European Patent Application EP 4 520 821 A1 - sequence listing, part 5

SEQ ID NO: 11499 - RNA, 6873 nt, Homo sapiens
  source 1..6873: mol_type = other RNA
ctgaatagctgggactacaggtgcctgccagcatgccgggctaatttttgtatttttagcaaagatagggtttcactatgtcagccaggctggtcttgaactcccgaccttgtgatctgcttgccttggcctcccaaagttctgggattacaggcatgagccactatgcctggcccagaaactgagtttctactctggcaagttaaacaaaaaattagtacatatcaggctgggtggctctaggccacatgcaagcaagctgcaaactgaattgcctctgcagctgcagaaggctaatttctacattgatatttggaaacactaacagctagaaaacaccactctactcatttttaaaaataagatcatattaaatgatgttacatgcatcatttatatattgctcgcagtgccagcatcctcaaatatggttttaattttggtagatatcttgctagggggagcacatttccaagttatccagatatagggccctctttccttctctttctgtccacgtgcaaccagatgctttgtggagttaaagttgacatttatttaaatgccacttggtgtctggtttttcacctttaatttagggttttctagctgggatgtaaaagaatcacttggagggatttttcaaaataccaatggccaggccactagccagtcaatcagaagcaaaatctccttggatgggacctggaagtctttacagttttccagcattttaatgaacatccctgattaagaaccaccgggtcttaagagtgtgccatatgtatttttcaagttcctagaggctctccaaaacaaaacaaaaaaaatctgctttattctctgcctggtgttgatgcatcagtctctttagccgttagtctgatcctggaaatttatggtcataatttgatgagcaatgttgggaatgacttcttcttctttttttttttttttttgttttgagacagagtctcactctgttgaccaggctggagtgtagtggggcgatctccgctcactgcaacctccaccccaatactttcatttttaaatattatttatggcatccagatttgcataagatggactgggtcaatggccatgccctttataaatcaatattcttaagttctgcaaattcagtttcctaaagagccaaatcacatcctactcatcagcaaggcgggtagacatcattttcacaatcacttctaattttccaccattgtaaaaaaaataaaatatgtaatcactttcttattgtaaaataaagaatttacttttccaggacctactgcctccctgttccccccccccttttttttttttcaaacaatcttgaaccctttgtcacgagtcagttgccaagagaagcctatttgttggtttgagagcagttcatgcagacacagaccacttcctctgagaattcatttgcttccccaggatggaatctggctgggcctctgaccttgctggtcacgtgggccggggcctccatcagtcataccctggactcctatctgtgtctaaacacacgccccacccccaactgcacggcagccactcgcatagcactctgggagggctgtgggcatgagcagcgaggactccatcagcagctcccccacataagccctgctgatgagggggcttgcgaagcagctttgatgtgctggtaaatccaggtgcaaaacagaactcaagttaaggcctccgcacagcactgcgttctaactgtgaaggattcttactctagtgtcctgtgtggaggtattggaattgtccattgctaagactcagaggagaaaagcacttagcatcgcaggacttggagcaccggtgctgaggcaacccttcattcattcgtcggatgtgtgttaaggcccagggcaggggtcagggtttctcctctcacacagcacgtgggtggcaggaccaacaccgggtctgacctcccagccgggggcacaggctgctaaccccaggcctggaatctgtcagatgcccttcccgtgctgacttgacttagacaggcctcctgaccttcccgcaaaggtcatgtgtgattcgcaggggttctggccgcttgaaaggttcctgagaaagtacatgcaatgaggacagagcttgcagagggaggacaggcatgcagaaggctctgtgtgcagccccagacctgggtaccttcgtcaccgtcctcaccccacctccgggtgcgcagatagggagcaggtctcctgtgttatggcccaagcagggctgttaggacactgagaacattccctcctcccgcaggagagagaggtccaaggtgccctacatcgtgcgccagtgcatggaggagatcgagcgccgaggcatggaggaggtgggcatctaccgcatgtctggggtggccgcagacatccaggcactgaaggcaggcttcaacgtcagtgagtgtcggcctgcgcaggacgggatggaggtgtgggcagtggtgtccccgatgagatctcagagtgctccatggcccaggcatgtcacatccttctctgtgtcttttcttcatttatcaggatcttcaaggaggccgctgcatttccgtgctctttccagataacaaggacgtgtcagtgatgatgagcgagatggacgtgaacgccatcgcaggcatgctgaagctgtacttccgtgagctgcccgagcccctcttcactgacgagttctaccccaacttcgcagagggcatcggtgagcactggaggccttggcctcatgggagacgtctcctccacgtgcactgctgccctcagaggctgtgaaaagtgaggtgtgggaacccgagctgtgcttcctctgccatggtcggaattttaacccaacctcaaaaagcaggggaccaaaactgagcctatcctggaaggccttgcccatccccagagggctccccatccatatttctcaaggaggccaagtgggtgaaatggtcagcactgccgtgctgtggggtcctaaagtctgctgtcctccttcctgcagaccagggctaaacactggtgcccaggtgctcttgccatgggtcctggtccagccaagcatggtttcaaacatgacctgacccttagtcaacctggaggctgatgtctagagtgggcgctggagcgtgcagcacctgtagcctgtgcatcacccttagggcaggtctgcctcccgggcccatgcacagaggacctggtctcccagcctgcaggtgcccctgtggtgtccaggatgtcgagggggtctctgcgtacttggtggggctgggaccctcccacttcccacctccttgtgtccctcactcccctgtttcattccatgctgagcctcccctgccttgggctccctggggagggggtggtggcaggagttgcccgagggcagctctgcccatgagcagctgctctagcggctcctcctgctgctgttcgccgggtgctgctgaccccaaggctggagtcagcttgcagcacagccagggtcgaggtcactccctccctgaggactctagcacggcacagcccctctgcctctctcctggtggtggcgttgaaacagcaccctctgcttcggtcctctacaggatggcagagaaggaggcagtcaataagatgtccctgcacaaccttggcacggtgtttggccccacgctgctccggccctccgagaaggagagcaagctccctgccaaccccagccagcccatcaccatgactgacagctggtccttggaggtcatgtcccaggtatgggaagacagcctccagcccatgcaaccccagcctgacagaggtggcctctgcctgccccacccccagtcctgcccatcttccgacttgcattgtatgtggtggtggctgagattcagagacagggacttgcctaggtttgcatggatgggagtgatagggggtgcctaggccacctcctggtcctgctggtgcaccttgctgggggcttaaaaccaccccaagtgttcgagtgtggtggctcatgcctgtaatcccagcactttgggaggccgaggcaggacaactgaacccaggtgtttgagaccagtctgggcaatgtagcaaaccccatctccagaaaaaatacaaagaaaaattaggcaggcattggggcacatatctgtaatcctaggtatctgggaggctgacacaggaggattgcttgagcccaggagttagaggctgcagtgatccatgatggagccactgtactccagcctgggggacagagcaaggccctgtgcatctctaaaataaataaccaccccccacccaacaagtcatgccttgtcaggaccccaccccacccccgtctcactgtaaggggttcatgacaccagcaggggtttctagcacctgaggtggacttgggatcttgggccccaaagacctcccaccagcagctgtgcgcccccttccgagccactctcctcttccccactccgcgagggcaggtcgaggtgctgctgtacttcttgcggctggaggccatccctgccctggacagcaagggacagagcatcctgttctccaccgatgtctaaaggtcccagtccatctcctggaggcggacagacggcctggaaacctctggctaatcaggccatctaataagatgctggaatgtaatccctggacaatccgtgtcctggcagcatttggtcttcctctaagcgcctggctccgctgttctcaggagtgggttctgaagtctctatctgggcccggtgggctcccttgtcctggcttccatctctgtctcagcgaccattcagccctgtggccaccgctctggcatgagcccctcagtcttgggtggtttctgcctggtccaggatttggtgttgctgctgagtccagcctttccaccacctccgcatgggctgtgggtgttgtcagctgcctcccgccttggcttcagtagctcacccagcttacaggggagctgccctgggctggagatgggcacgcaccctgggtcctatgtgtttcaggaactgagggtcagctggcagtgggatgaggctggcccccttctccgctttcgttccgggaggcctcccgtagagcggtaggggctcgagatggcatttcgtttggggcacgagctggtccgggaggtctgggatctctggttctgacctctgggcacctgctgcagctgtggctgaggcccagaaatgtgaagggcctccatccactccagtagtgaccccaacgtggggttcaatgtggaggggggaggggctgctgcggcagctgcaggagcagaagtgccacaccttgttcttctcatgcccgcatccatgcttgcagctgggaagggggcaggaatcagcgaggtgacctgggctgagtcctgggaatgggaagaggtggcaggaaggggatctgaggaggagaacagggggcctggtggtctgtgcttcttcccagacatgggagctgtagaggggacccctgcagcagatgctaagggggccagtaggcccaggcagtcttgggacttgtgtgtctcctgctgtgcatccatactgggtgctttagaaacggcaggcagaccagaagcccctgttgcaagtgaggacaaagtgtgggaaggccgtgagggtctgcagtccgagatggccttgtcctcaacctgcagtgcactgttgatgcgctggaatgccgcctccttctcccggtccaggtcttcaacagtgacccggtaccccagctctaagggaggtggcagcatcaaaggctcccctcgcctgcgtggcagcaggggaaacttgtgtgtactgggcctagaggcctcggatgtggaggagtcattcctgagggcgagtgtctaccctggtgctatatctgctgccttttcacactgggtgtgacctgaagagacagcctgaggcctgtcctcactcactgtctttgaggaactgagggtcagctggcagtgggatgaggctggccccctcctccgctttagccccggcaagcctcccgtggagctgtaggagctggagatggcatttcggttggtgcaggagctcgtccaggaggtctgggatgtctggttatatctgatttctgacctctgggcatggaggtctgtctgcagaggcccgggcccgggcacaaagggagagaggcctctattgtcccgcaggggccgaaatgcagacggtgcatccccggtgacctcggggacccttctctgatcaccaggattctcttggactctagggtccttgtcctgctcaggcatccctgccccgctctccttgagggccctcaacactatcttccctggacacaagtctggggacagccggctgttgtggaccccaaaggggtgactcccggctcctgggccccacagagagtccatgttctcagtgcagtggctgagctggaggacgccctggaactcggagcacgcagcactggcttgctgtggtacctgtgcaatcaaattgaaggcaggatcccaggaaggaaggcagggcttgcaggatcacggaaaaccttcttagagttgtcttgacaccactgatgtcaagtgtccgggtgcttgtaggatggcctgccactcagtccacgggcaggagcaacggggagatcccacaagcaaagtgaactgggggatgggctgaacgggctccaggcaactgagccctactggcaggtcctcggcctgggcccgaacaggaaggaggggcacagagtgcccaggtaaccgctcctgggagcagtggggaaccgtcggttgcttgaactctcgagagctgggctctgagcgtcctcgtccagccgccaactcggccaacggctaagccagcagttt

SEQ ID NO: 11500 - RNA, 4528 nt, Homo sapiens
  source 1..4528: mol_type = other RNA
ctgaatagctgggactacaggtgcctgccatcacacccagctaattttttgtatttttagtagagacggggtttcacggtgttaaccaggatggtctctatctcctgacctcgtgatccacccacctcggcctcccaaagtgctgggattacaggcgtgagccaccgcacccggcaccttttgctttttaacgagttaattatcactaagctcctcttttgagattttcagtagtgataatataaaaatggaaagtactaagtttactataatattcactatgcattagcatacatttagatgatactgagatatttttgcttttaatttgccacttattacaagtaaattaactgaataacaaaaccacaaactactgaagttaaaaagtaactggctatcagtgatttgagcagaagtgctatgccatctagtgtcatgacaaggcattgctttataaactagagtaggaaaaaatctgagcaatgttcatttatcaattttactgagcttttttactcggtctcatatagtatagatgtactggtaaggaaacaatttttttattatggaactcaaatcactcaagtaagtttaacttatcaatagacaaactttctaaattctaaaaagtgtaaactaaaaatcactatattaattatgcttttacaattaattattatacatgtcaataaagctacaactaataactaagctttgcttacctacattttacaaccactaaaaccagaagtggcagggtgcggtggctcacacctgtaatcccagcactttgggaggctgaagcgggcggatcacgaggtcaggagatcgagaccaccctggccaacatgctgaaaccccatctccactaaaaatacaaaaattagctgggcgtggtggcgtgtgcctgtagtcccagctacttggcaggctgaggcaggagaatcgcttgaacccgggaggcggaggttgcagtgagccgagatcacaccactgcactccagcctgggcgacagagcgagactccatctcaaaaaaaaaaaaaaacccgaagggctgataagcagcaagacccaatgatgagttctgaacctttcccagcccttcctctaaagtaactggaagacgttaaccggcaataaaaggccaaagggcagaatggggaagcaaaataaaaaagtcacttgctaatctaaaatctgggtaagagtgtagagtttctgatatatattttatgaatgaaaaagaaaggctaaaaaattatgacataattgattttataggaatctgaaaatcacttctaaaaaatgggtctgttatttgattttgcctgtatttgttttccaataaaggaccatcatgtgatcaaaaagacagaaattatctatgtgaatagcagtgttacctgccacatatttggaactccttctaacttaactcaaaagctaagctagaaaaagataattctttcttgcttgcttgccctggtgtataatcctggttttttccatataactacaaagatgtgagagcaccagcctatggaaatctagtttgagtatcaaccctagtatctttactgccattcgccctacagaagaatagctatatctcactgttgagaaatggctattcatcaggagaccaaatcccagtttaataaggcataatttctatttaaaggtctggatttgaatgcctactactctgtctcttctttagctgcgtgaatgaatttgggtaaagtccctaatctcagattgttttatcatctgtaaaacagtaataatgagtcatgtagcacttctgtatcaggttgctcggagtaataaattagaaaactgtgtgaaagtgcctattttagaatttggcattttctagtttgtgaccttggacaagttatgtaagctatcatttccacatttctctatcttatttcacaaggtgttgtaataaagattatttaagcaaatatatttttactaattatgaaaaggaatggccgggcacggtggctcacgcctgtaatcccagcactttgggaggccaaggcgggcagatcacgaggtcaggagatccagaccatcctggctaacacggtgaaaccccgtctctactaaaaatacaaaaaattagctgggtgtgatggcaggcacctgcagtcccagctgcttgggaggctgaggcgggagaatggcgtgaacccgggaggcggagcttgcagtgagccgagatggcgccactgcactccagcctgggcgactgaccgagactccgcctcaaaaaaaaaaaaaaaaaaaagaaaagaaaacaaaaagattgtacaatatgagatattataaatgtttacatcatttaaggtctgcaaaaagatgctacttactgaagatgctccttcattagtgactaatacatattagaagtcagcaaaagtaatggaaaagctaggtagaatcaaaattaaagaaagaactgccaatcagttctcctttctcttaaaacaaaacatcactccctgcatgactgttaaaaacgggctaagtagcccttgtattgtgggaagatcagaaatctgtttaacaaaaatggcatactttcttaaaaataatggtccaaaacattagttcaattcaacaattactgaatacttacaatgtactcgatacaaacacttcaaatcctgctgtttgaggaactcatcataaagcagacagacttttaaaaaaatcacatacaagtgatgagggcaatcaacagcattagcataaacaaggtacaaaggagcaaataattattagaggtgatacctgagatttcttcttttgatttggattttgaaggatgaattagtttactagccagagataagaaagaacactaaagaataaggtgcaacgtatactgaaaggcagggaaccatacaattcagttctggatttcaagatcttcaagtgctagaaaggggccattaaaaatgactgtggacagggagaaagggcctattaatacaaggccttgactttatcccgttgaagggttttaagcaggcaagttatataatcagatacgacttttagaaactcaacactagctgcagtgaaggatggtacagattggataagaatgtgtaggcaaagattactgtgacagtccaagtaagagacgaaattatgctattatgaactaaagtaaaacaactcagtcattatcttcctattactatgtagtaatgctcagttaaattcattttgtcatactaattttagctctgaagcacaactgctttaatagaaaatgaagccttcggccgggagcggtggctcacgcctgtaaatcccaacactttgggaggccgaggcaggtggatcacctgaggtcaggagttcaagaccagcctgaccaacatggtgaaaccccacctctacaaaaacaaaaaaaacaaaaaaaacaaaactagcccggcgtggtggcaggcgcctgtaatcccagctacttggaggctgaggcaggataatcgcttgaacctgggaggtggaggttcgcagtgagctgagatggcgccattgcactccagcctgggcaacaagagcgaaatgctgtctcaaaaaaaaagaaaaaaaaaaagaaaaagaagaaaaaaaagaaaattaagccttcagtactttgtagctacagtcacaagaaaccatgaattgatttgtgttgttctaataatgcatcataaatctgaccactggatgagatatcagatattttactttaaagcctgaataatttatgatctttcactaaaatacagcaactactactagctgagctatcagagacttcatgttaaagccaaatatgtatgatctttctcaaaagcagagcagtaagtatccaaagaccatcaaattagtttgtcaattcgctagatttaattttcattcattaaatatctcattctttttaagcccatcacggggatcaaaatagaccaccatcggattctgactttccttacctgattccaacgtctcctccccttctggtagaagcctagctttcttagcattctgtggagcatcatcaccattgtcctcatatatgttagaccattttattgccatgtcaagctctggaggcggaggcttcttctcagtggtgtaggtctcaggaggtggtacataatttgacttccatattttgaattcctttggaggctcctcaggcgccttgacgacgtgcctctcccagtctatctgtttgttgagcggattgtagagaaaggccgggcgagtcacgctcctaaacagctcgtcaggtcccgggagccgcttctccgccttgttcctacagccgcccgccgacttcgccggatccggggttctgcgactcgtctcctccggctcgatgttatcctcctcgtccgaggagcctgagctgctgctcccgtatgccgcaaaatagctcagagggtccttctcctccgctgccatgacggctgcgagcgacaacccagcactccgccggaagccggaaa

SEQ ID NO: 11501 - RNA, 2572 nt, Homo sapiens
  source 1..2572: mol_type = other RNA
ctgaatagctgggactacaggtgcctgccatcacgcccggctactttttgtatttttagtagagatgggggtttcaccatgttggccaggctagtcttgaactcctgacctcgagtgatgtgccagccttggcctcccaaaatgctgagattacaggcatgagccactgcacctagccacatcccataaatttcggtatgttgtgtttccattttcatttgtcttaagatatttctgatttcttctttgacccattggttgttcaggagtgttaattccacatacttgcaaattttccaagttttctcctgttaattatttccagtttcataccagtgtgtgaaacctttccttgatgtagtaatagatataaatacacacatatgtataggtttccatctatgattcctggctcataactcccagagtccttgttacagtcttttgttacaatgttggtatgttaggcctctctgactttctccagtgttcctttcacctgccccaaggcaggtctgtaatctgattgtgggtcataagaccaccattccagagagggtcccatcccataccctgggggaaggaatgctaacgtcacgaagcttctataaaaagccaggatgactggatttagagagcttctggatagctgaacacatgcaagttcctggagggcagctcgcccagggagggcatgggagttctgtgccccttcccccatacctcaccctgagcatctcttcatctgtatcctttgtaataaaataaattggtaaacatgtttccctgagttctgtgagtcactatagccaattaattgaaccccaagagggattgtgggaaccccaacttgaagccagttgtcagaagttccagaggccccagacctgtgactggtgtctagcagtgttgggagagggaaagaggacaatctttggggggctgagcccttaccctgtgggatcagacactatttccaggtagatagtgttggaattgaattggaagacatccagtcagtgtttgttgccaaactgattgcttgcttgttgctagggagaaatccccacatagtttggggtcacagaagtcttctgtgctgattgatggttcttgtgcttcaaactctcaggctcaagggatcctccttcctcagccttctgagtagccagggccacaggtacacgccaccacacccaaactgagaatatgcctgagacctcagggaagaaaggggacaagggaagagcacactaggtgagtggcagcatcgagcaggatgtggaacagacatcatgagcctgggcattaatcagtatgtgtcagaacagaaagctatactgaaaaaaataaattttattaaataaatctgtatttttgaaatttgaattttcttttttgtagtttgtttaacttccttttggaatccataatgttttaataaaactcactttgaaaaaaatctcaaatacactaacaagggaaatacattttgttatttacaaatatgggccagggagaaatgtgagacagtgtaacttggggccaggcacagagttattcatttattcaataaatatttactgaatgcctactatgtgccaggcattatgctaagatgctggggatatacctagtaatgaagaaggaagaaattgtctctgcctacatgtaactaaaagtccttgggagaagaaagatagtgaaaaataaatccaaatgcgatgtgttatgaaagaggaagtataaagtgccatgagtatgagtggaaagagcagttaaaggtgagcagaggagcagctctcagtggaaagaaatcaaaagctaagataaaaaccagtaacactctggatgggtgggaatagattgaaatccataaagccaaagagatttgaattacttgacttcaaataggttgaatatttcagtaaggtaaggactctattctttttctttctcggcctttgtccagagagtgggaaaagtttgaaagatttggtctgaatccaggttttaaaaattatttttatggattgattaatattgttatgcacaacaggactacagaatgtaggagatggggtaactgtccccaaaagaggtcatagccttgttggagagacaacatataaacatagaaaaaaataaaagaggtctcttaggagactataaatgattaaagccttaatgaaggcagaggaagaagtttctatgggcacaaataataagtaatgatgtcttgctagagatgtcctattttagaacttattggtgaattatgacattctaagataggcctaagtgtacaagacttaggtctaaaattaggcattagaaactgcctccctgtttggcctggctgatggcagaggaaggttcagaaatacaggggagattcagtagccaaagatgggttcatctatagctatgatgagataaacagtttacaccaagattatacattctggtgtctagaagggggatcttcgtgtattcatccattctcacactgctataaagatactacctgagactaagtaatttataaagaaaagaggttaattgactcaca

SEQ ID NO: 11502 - RNA, 4645 nt, Homo sapiens
  source 1..4645: mol_type = other RNA
ctgaatagctgggactacaggtgcctgtcaccacgcctggctaatttttttgtacttgtagtacacacggggtttcaccgtgttagccaggatggtctcaatctcctgacctcgtgatccacccgcctcagcctcccaaagtgctgggattacaggcttgagccaccgcgcccagccatgaaaaactttttaataagtgaaaggaatatgataccgtatgagaaagagaattcaaacaagcagtgtgggaccaagagatatttgcgcaaagacaccattcatctctggatgaaacctgatatttgtgagatgaaacttggtttcatgagagctgaaactgaaatttcttgcagtcttttatctgtgtctggtcacacagcagagacaagatctgtaattatctcatatggaagctatcaataaacaaattgaccctggattccactgagggattttgaactttaaagaactcaccataaaccatttgttagctagttagttagcctactacccatatcatggccaagagtcaaaaacagacacctaggcatctctggaaataagcaaagagctgtcccagttcagctgtaaaataactcactttcttatgcatgcaatatgagaatacagatgtcactaactgatatggcttggctgtgtccccacccaaatctcatcttgaattgtagtgcccctaatcctcacgtatcatgtgagggaactggtaggaggtaatttaatcatgggggtagttacctctttgctgttctcatgatagtgagtgagttctcactagatctgatgatttaataagagggtatttttccttttgctcagcacgtctcctttctgctgccatgcgtagagggatgtgtttgctttcccttctgtcattactgtaagtttcctgaggcttctccaaccctgcagaactgtgagtcaattaaatgtctttattttataaatttcccagtcttgggtatatctttagtagcagcataagaacggactaatacactaatgttgtgggtgagcaacggctacctgggccggtggcattgaggtaaaagaatttaccaagacagctgtaggtaaaggaaggcagatttattaaagaaaagtaggaaaatatgtttccagggaggcaacaggcagcatcagcagaagaaaagctgactgcaaagaaacaaaggcttgcttaggattttatggaatagtgtttatgctgtatgctgcagagggctttgtccagtactgataatgccaaggttgcggtgaggtaacttgcaggtgtctggtaatagtttagcacatggcccatatcctggaccatgaagaaaggcagactcatagcttatctgctttctctttctgcttttccctgctcccgccagcctaactccttttccctaattaggacttcacaactaacggaggaactaataattaatgtattgagaaaaacagaaaataattacttgtcctcacatgcacacgtatgtttattgcagcactatttaccatagcaaagacttggaaccaacccaaatgcccatcagtgatagactggataaagaaaatatggcacatatacaccatggaatactatgcagccataaaaagaatgagttcatgtcctttgcagcgacatggatgaagctggaaaccatcattctcagcaaactaacacaggaacagaaaaccaaacaccacatgttcttactaataagtgggagttgaacaatgagaacacatggacacagggaggtgaacatcacagaccaaggcctgtcggggggtggggggcaaggggaggaagagcattaggacaaatacctaatgcatgtgggacttaaaacctagatgatgggtcaataggtgcagcaaaccaccttggaacatgtatacctatgtaacaaacctgcaggttctgcacatgtaacccagaacttaaagtaaaataaaataaaataataattacttgtcctagcatatgggaatcaaggaaccaaaaggcagtgtttaaattatataaactggccgggcacagtggcttatgcctgtaattccagccctttaggaggccaaggcgggcagaatccttgaccccaggagttcaagatcagcctgggcaacaatacaaaaccccatttctacaaatgatacaaaaaattagctgagcatgatggctcgcacctgagtcccaagtactcagaaggctgaggtgggaggatcccttgagcctgggaagttgaagctgcagtgaaccatgattgcatcattgcactacagcctgggcaatgggaatgaaaccgtgtctcagaaaaaaaaataataaaagtaaaaaataaaataagtggcataaactatgaagtagcagttgtaacatatttttaggattatgtgggtacagtaggcataactctaaagtggtttctaattggtacaccagtggcctagtgtacacctgcataatcccttccccttttgtttgagtaggatttgggattatgatgggatgttactccgtggttggagtacactaaataacaaaggtgaggcagtttttcagatgcaattaaggttccaaatcctttcatcttttttttttttttttttttttggagaggagtctggctctgtcacccaggctggagtgcagtggtgcaatctcgactcactgcaacctccacctcctaggttcaagcgatcctctcgactcagcctcccaaatagctgggattacaggtgtgcactaccacacccagccaatttttgtatttttagtagagacagggtttcaccatgttggccaggctggtctcaaactcctgacctcaagtgatccacccgccttggcctcccaaagtgctgcgattacaggcataaaccaccacacccagtccaaatccttccatcctaagtcaatcaaaattaattttttcatcacaaaaatgatgaaaatagatcagctttgattcataacagagaaaaccactctaagtgttaaaatcaaaacagaagataatgcctaatgaaaggaggtcaggggtataggatagttggtggaaaaaaatattgataatcattacatgcttgcctgtattattttaaattttttaattaaaaaatatattattttgtagtcacatggacaacaaaaccaaaacattacaaatctccagaaagtgcaatgcataagctctcttagttcaaattaaacatttgaaagatattatttttcatcctatatcttttgtcagttacctgaaatgcatttttcccaaatcaatcttcatacaagaatgtgaagagggccagggatggtggttcacacctataatcccagcactttgggaatccaaggtgggagaatcccttgaggccaggagttcaagaccagcctgggcaacatagcaagaccttgtcttgacaaaaaattaaaaattaaaaattagtcgggcatagtgacatggtgcctgcagtcctagctacttgggaggctgagtcaggaggatcacttgagcttgcaatgagctatgatcttgccactatgctccagcctgggcagtgtgagttaaattttattttctaaattttatttgatgtgaattaaatcttatttaaatttctgctgagaattagcaagaatgtaaataaaattacataaatgtgtaataaaactacattgaatttaacattaaatatatacattaaatgaaaatacaaaattctttatgttaattttataattctcaaatgtaggtgaacgaatttcatcaattttaaaacacattgtttcacatacatgacaattgtatatgacactgtttaaaaacattttatagactccagaagtagacaattagtaataatataacatgcaactgtatcattgttagtaatgttgggtctttactctccaccttctctgccccaagaaacatttaaatgagctgttgcttacagatataacgatttttatcttcacaggattcatctaaagcatttccatttggattatacgctatgcagttctttgtattaaaagtttcaaatgatggaaatagatactgggagagtgcagagccattctcccacaaccaggcggtgtgctcctcacagttcatctgtgttttgaagctgaagcaggctggatttctgagaagcacagagatgccgactttcgttccaagttttctgttcactggaaatgaagtaacagttgcaccggtacccaacccatttttcttggcaagaacagcagtcagagtctttctggagttctatgttgggtcctggagtaaatgctggctcaatactcagtttagtaaaagaatttttcaacaaaattcccaacgtagacatcaacgaaaggcatattatccctaaggtcccagaaattaacctccacagagtggtcttaaacactgccatgagaaattatgttccaagagcgaagtagagaaggcacgatgtgtactttttcagaaagaacagcgttgaattgttgaagctgagctggagattaaagaatctgaaagttgagtatgaagaaatttagcaaaaatagagaatgaaaaattgtgtatttaaatgatgttcttgaatcatctattggtgagacatgtattatagtgtgaat

SEQ ID NO: 11503 - RNA, 4699 nt, Homo sapiens
  source 1..4699: mol_type = other RNA
ctgaatagctgggactacaggtgcctgtcaccacgcctggctaatttttttgtacttgtagtacacacggggtttcaccgtgttagccaggatggtctcaatctcctgacctcgtgatccacccgcctcagcctcccaaagtgctgggattacaggcttgagccaccgcgcccagccatgaaaaactttttaataagtgaaaggaatatgataccgtatgagaaagagaattcaaacaagcagtgtgggaccaagagatatttgcgcaaagacaccattcatctctggatgaaacctgatatttgtgagatgaaacttggtttcatgagagctgaaactgaaatttcttgcagtcttttatctgtgtctggtcacacagcagagacaagatctgtaattatctcatatggaagctatcaataaacaaattgaccctggattccactgagggattttgaactttaaagaactcaccataaaccatttgttagctagttagttagcctactacccatatcatggccaagagtcaaaaacagacacctaggcatctctggaaataagcaaagagctgtcccagttcagctgtaaaataactcactttcttatgcatgcaatatgagaatacagatgtcactaactgatatggcttggctgtgtccccacccaaatctcatcttgaattgtagtgcccctaatcctcacgtatcatgtgagggaactggtaggaggtaatttaatcatgggggtagttacctctttgctgttctcatgatagtgagtgagttctcactagatctgatgatttaataagagggtatttttccttttgctcagcacgtctcctttctgctgccatgcgtagagggatgtgtttgctttcccttctgtcattactgtaagtttcctgaggcttctccaaccctgcagaactgtgagtcaattaaatgtctttattttataaatttcccagtcttgggtatatctttagtagcagcataagaacggactaatacactaatgttgtgggtgagcaacggctacctgggccggtggcattgaggtaaaagaatttaccaagacagctgtaggtaaaggaaggcagatttattaaagaaaagtaggaaaatatgtttccagggaggcaacaggcagcatcagcagaagaaaagctgactgcaaagaaacaaaggcttgcttaggattttatggaatagtgtttatgctgtatgctgcagagggctttgtccagtactgataatgccaaggttgcggtgaggtaacttgcaggtgtctggtaatagtttagcacatggcccatatcctggaccatgaagaaaggcagactcatagcttatctgctttctctttctgcttttccctgctcccgccagcctaactccttttccctaattaggacttcacaactaacggaggaactaataattaatgtattgagaaaaacagaaaataattacttgtcctcacatgcacacgtatgtttattgcagcactatttaccatagcaaagacttggaaccaacccaaatgcccatcagtgatagactggataaagaaaatatggcacatatacaccatggaatactatgcagccataaaaagaatgagttcatgtcctttgcagcgacatggatgaagctggaaaccatcattctcagcaaactaacacaggaacagaaaaccaaacaccacatgttcttactaataagtgggagttgaacaatgagaacacatggacacagggaggtgaacatcacagaccaaggcctgtcggggggtggggggcaaggggaggaagagcattaggacaaatacctaatgcatgtgggacttaaaacctagatgatgggtcaataggtgcagcaaaccaccttggaacatgtatacctatgtaacaaacctgcaggttctgcacatgtaacccagaacttaaagtaaaataaaataaaataataattacttgtcctagcatatgggaatcaaggaaccaaaaggcagtgtttaaattatataaactggccgggcacagtggcttatgcctgtaattccagccctttaggaggccaaggcgggcagaatccttgaccccaggagttcaagatcagcctgggcaacaatacaaaaccccatttctacaaatgatacaaaaaattagctgagcatgatggctcgcacctgagtcccaagtactcagaaggctgaggtgggaggatcccttgagcctgggaagttgaagctgcagtgaaccatgattgcatcattgcactacagcctgggcaatgggaatgaaaccgtgtctcagaaaaaaaaataataaaagtaaaaaataaaataagtggcataaactatgaagtagcagttgtaacatatttttaggattatgtgggtacagtaggcataactctaaagtggtttctaattggtacaccagtggcctagtgtacacctgcataatcccttccccttttgtttgagtaggatttgggattatgatgggatgttactccgtggttggagtacactaaataacaaaggtgaggcagtttttcagatgcaattaaggttccaaatcctttcatcttttttttttttttttttttttggagaggagtctggctctgtcacccaggctggagtgcagtggtgcaatctcgactcactgcaacctccacctcctaggttcaagcgatcctctcgactcagcctcccaaatagctgggattacaggtgtgcactaccacacccagccaatttttgtatttttagtagagacagggtttcaccatgttggccaggctggtctcaaactcctgacctcaagtgatccacccgccttggcctcccaaagtgctgcgattacaggcataaaccaccacacccagtccaaatccttccatcctaagtcaatcaaaattaattttttcatcacaaaaatgatgaaaatagatcagctttgattcataacagagaaaaccactctaagtgttaaaatcaaaacagaagataatgcctaatgaaaggaggtcaggggtataggatagttggtggaaaaaaatattgataatcattacatgcttgcctgtattattttaaattttttaattaaaaaatatattattttgtagtcacatggacaacaaaaccaaaacattacaaatctccagaaagtgcaatgcataagctctcttagttcaaattaaacatttgaaagatattatttttcatcctatatcttttgtcagttacctgaaatgcatttttcccaaatcaatcttcatacaagaatgtgaagagggccagggatggtggttcacacctataatcccagcactttgggaatccaaggtgggagaatcccttgaggccaggagttcaagaccagcctgggcaacatagcaagaccttgtcttgacaaaaaattaaaaattaaaaattagtcgggcatagtgacatggtgcctgcagtcctagctacttgggaggctgagtcaggaggatcacttgagcttgcaatgagctatgatcttgccactatgctccagcctgggcagtgtgagttaaattttattttctaaattttatttgatgtgaattaaatcttatttaaatttctgctgagaattagcaagaatgtaaataaaattacataaatgtgtaataaaactacattgaatttaacattaaatatatacattaaatgaaaatacaaaattctttatgttaattttataattctcaaatgtaggtgaacgaatttcatcaattttaaaacacattgtttcacatacatgacaattgtatatgacactgtttaaaaacattttatagactccagaagtagacaattagtaataatataacatgcaactgtatcattgttagtaatgttgggtctttactctccaccttctctgccccaagaaacatttaaatgagctgttgcttacagatataacgatttttatcttcacaggattcatctaaagcatttccatttggattatacgctatgcagttctttgtattaaaagtttcaaatgatggaaatagatactgggagagtgcagagccattctcccacaaccaggcggtgtgctcctcactgtaagagagtccaatccagtaaaattgttgactggagctcataaaatcatgccagttcatctgtgttttgaagctgaagcaggctggatttctgagaagcacagagatgccgactttcgttccaagttttctgttcactggaaatgaagtaacagttgcaccggtacccaacccatttttcttggcaagaacagcagtcagagtctttctggagttctatgttgggtcctggagtaaatgctggctcaatactcagtttagtaaaagaatttttcaacaaaattcccaacgtagacatcaacgaaaggcatattatccctaaggtcccagaaattaacctccacagagtggtcttaaacactgccatgagaaattatgttccaagagcgaagtagagaaggcacgatgtgtactttttcagaaagaacagcgttgaattgttgaagctgagctggagattaaagaatctgaaagttgagtatgaagaaatttagcaaaaatagagaatgaaaaattgtgtatttaaatgatgttcttgaatcatctattggtgagacatgtattatagtgtgaat

SEQ ID NO: 11504 - RNA, 4632 nt, Homo sapiens
  source 1..4632: mol_type = other RNA
ctgaatagctgggactacaggtgcctgtcaccacgcctggctaatttttttgtacttgtagtacacacggggtttcaccgtgttagccaggatggtctcaatctcctgacctcgtgatccacccgcctcagcctcccaaagtgctgggattacaggcttgagccaccgcgcccagccatgaaaaactttttaataagtgaaaggaatatgataccgtatgagaaagagaattcaaacaagcagtgtgggaccaagagatatttgcgcaaagacaccattcatctctggatgaaacctgatatttgtgagatgaaacttggtttcatgagagctgaaactgaaatttcttgcagtcttttatctgtgtctggtcacacagcagagacaagatctgtaattatctcatatggaagctatcaataaacaaattgaccctggattccactgagggattttgaactttaaagaactcaccataaaccatttgttagctagttagttagcctactacccatatcatggccaagagtcaaaaacagacacctaggcatctctggaaataagcaaagagctgtcccagttcagctgtaaaataactcactttcttatgcatgcaatatgagaatacagatgtcactaactgatatggcttggctgtgtccccacccaaatctcatcttgaattgtagtgcccctaatcctcacgtatcatgtgagggaactggtaggaggtaatttaatcatgggggtagttacctctttgctgttctcatgatagtgagtgagttctcactagatctgatgatttaataagagggtatttttccttttgctcagcacgtctcctttctgctgccatgcgtagagggatgtgtttgctttcccttctgtcattactgtaagtttcctgaggcttctccaaccctgcagaactgtgagtcaattaaatgtctttattttataaatttcccagtcttgggtatatctttagtagcagcataagaacggactaatacactaatgttgtgggtgagcaacggctacctgggccggtggcattgaggtaaaagaatttaccaagacagctgtaggtaaaggaaggcagatttattaaagaaaagtaggaaaatatgtttccagggaggcaacaggcagcatcagcagaagaaaagctgactgcaaagaaacaaaggcttgcttaggattttatggaatagtgtttatgctgtatgctgcagagggctttgtccagtactgataatgccaaggttgcggtgaggtaacttgcaggtgtctggtaatagtttagcacatggcccatatcctggaccatgaagaaaggcagactcatagcttatctgctttctctttctgcttttccctgctcccgccagcctaactccttttccctaattaggacttcacaactaacggaggaactaataattaatgtattgagaaaaacagaaaataattacttgtcctcacatgcacacgtatgtttattgcagcactatttaccatagcaaagacttggaaccaacccaaatgcccatcagtgatagactggataaagaaaatatggcacatatacaccatggaatactatgcagccataaaaagaatgagttcatgtcctttgcagcgacatggatgaagctggaaaccatcattctcagcaaactaacacaggaacagaaaaccaaacaccacatgttcttactaataagtgggagttgaacaatgagaacacatggacacagggaggtgaacatcacagaccaaggcctgtcggggggtggggggcaaggggaggaagagcattaggacaaatacctaatgcatgtgggacttaaaacctagatgatgggtcaataggtgcagcaaaccaccttggaacatgtatacctatgtaacaaacctgcaggttctgcacatgtaacccagaacttaaagtaaaataaaataaaataataattacttgtcctagcatatgggaatcaaggaaccaaaaggcagtgtttaaattatataaactggccgggcacagtggcttatgcctgtaattccagccctttaggaggccaaggcgggcagaatccttgaccccaggagttcaagatcagcctgggcaacaatacaaaaccccatttctacaaatgatacaaaaaattagctgagcatgatggctcgcacctgagtcccaagtactcagaaggctgaggtgggaggatcccttgagcctgggaagttgaagctgcagtgaaccatgattgcatcattgcactacagcctgggcaatgggaatgaaaccgtgtctcagaaaaaaaaataataaaagtaaaaaataaaataagtggcataaactatgaagtagcagttgtaacatatttttaggattatgtgggtacagtaggcataactctaaagtggtttctaattggtacaccagtggcctagtgtacacctgcataatcccttccccttttgtttgagtaggatttgggattatgatgggatgttactccgtggttggagtacactaaataacaaaggtgaggcagtttttcagatgcaattaaggttccaaatcctttcatcttttttttttttttttttttttggagaggagtctggctctgtcacccaggctggagtgcagtggtgcaatctcgactcactgcaacctccacctcctaggttcaagcgatcctctcgactcagcctcccaaatagctgggattacaggtgtgcactaccacacccagccaatttttgtatttttagtagagacagggtttcaccatgttggccaggctggtctcaaactcctgacctcaagtgatccacccgccttggcctcccaaagtgctgcgattacaggcataaaccaccacacccagtccaaatccttccatcctaagtcaatcaaaattaattttttcatcacaaaaatgatgaaaatagatcagctttgattcataacagagaaaaccactctaagtgttaaaatcaaaacagaagataatgcctaatgaaaggaggtcaggggtataggatagttggtggaaaaaaatattgataatcattacatgcttgcctgtattattttaaattttttaattaaaaaatatattattttgtagtcacatggacaacaaaaccaaaacattacaaatctccagaaagtgcaatgcataagctctcttagttcaaattaaacatttgaaagatattatttttcatcctatatcttttgtcagttacctgaaatgcatttttcccaaatcaatcttcatacaagaatgtgaagagggccagggatggtggttcacacctataatcccagcactttgggaatccaaggtgggagaatcccttgaggccaggagttcaagaccagcctgggcaacatagcaagaccttgtcttgacaaaaaattaaaaattaaaaattagtcgggcatagtgacatggtgcctgcagtcctagctacttgggaggctgagtcaggaggatcacttgagcttgcaatgagctatgatcttgccactatgctccagcctgggcagtgtgagttaaattttattttctaaattttatttgatgtgaattaaatcttatttaaatttctgctgagaattagcaagaatgtaaataaaattacataaatgtgtaataaaactacattgaatttaacattaaatatatacattaaatgaaaatacaaaattctttatgttaattttataattctcaaatgtaggtgaacgaatttcatcaattttaaaacacattgtttcacatacatgacaattgtatatgacactgtttaaaaacattttatagactccagaagtagacaattagtaataatataacatgcaactgtatcattgttagtaatgttgggtctttactctccaccttctctgccccaagaaacatttaaatgagctgttgcttacagatataacgatttttatcttcacaggattcatctaaagcatttccatttggattatacgctatgcagttctttgtattaaaagtttcaaatgatggaaatagatactgggagagtgcagagccattctcccacaaccaggcggtgtgctcctcactgtaagagagtccaatccagtaaaattgttgactggagctcataaaatccagttcatctgtgttttgaagctgaagcaggctggatttctgagaagcacagagatgccgactttcgttccaagttttctgttcactggaaatgaagtaacagttgcaccggtacccaacccatttttcttggcaagaacagcagtcagagtaatttttcaacaaaattcccaacgtagacatcaacgaaaggcatattatccctaaggtcccagaaattaacctccacagagtggtcttaaacactgccatgagaaattatgttccaagagcgaagtagagaaggcacgatgtgtactttttcagaaagaacagcgttgaattgttgaagctgagctggagattaaagaatctgaaagttgagtatgaagaaatttagcaaaaatagagaatgaaaaattgtgtatttaaatgatgttcttgaatcatctattggtgagacatgtattatagtgtgaat

SEQ ID NO: 11505 - RNA, 4660 nt, Homo sapiens
  source 1..4660: mol_type = other RNA
ctgaatagctgggactacaggtgcctgtcaccacgcctggctaatttttttgtacttgtagtacacacggggtttcaccgtgttagccaggatggtctcaatctcctgacctcgtgatccacccgcctcagcctcccaaagtgctgggattacaggcttgagccaccgcgcccagccatgaaaaactttttaataagtgaaaggaatatgataccgtatgagaaagagaattcaaacaagcagtgtgggaccaagagatatttgcgcaaagacaccattcatctctggatgaaacctgatatttgtgagatgaaacttggtttcatgagagctgaaactgaaatttcttgcagtcttttatctgtgtctggtcacacagcagagacaagatctgtaattatctcatatggaagctatcaataaacaaattgaccctggattccactgagggattttgaactttaaagaactcaccataaaccatttgttagctagttagttagcctactacccatatcatggccaagagtcaaaaacagacacctaggcatctctggaaataagcaaagagctgtcccagttcagctgtaaaataactcactttcttatgcatgcaatatgagaatacagatgtcactaactgatatggcttggctgtgtccccacccaaatctcatcttgaattgtagtgcccctaatcctcacgtatcatgtgagggaactggtaggaggtaatttaatcatgggggtagttacctctttgctgttctcatgatagtgagtgagttctcactagatctgatgatttaataagagggtatttttccttttgctcagcacgtctcctttctgctgccatgcgtagagggatgtgtttgctttcccttctgtcattactgtaagtttcctgaggcttctccaaccctgcagaactgtgagtcaattaaatgtctttattttataaatttcccagtcttgggtatatctttagtagcagcataagaacggactaatacactaatgttgtgggtgagcaacggctacctgggccggtggcattgaggtaaaagaatttaccaagacagctgtaggtaaaggaaggcagatttattaaagaaaagtaggaaaatatgtttccagggaggcaacaggcagcatcagcagaagaaaagctgactgcaaagaaacaaaggcttgcttaggattttatggaatagtgtttatgctgtatgctgcagagggctttgtccagtactgataatgccaaggttgcggtgaggtaacttgcaggtgtctggtaatagtttagcacatggcccatatcctggaccatgaagaaaggcagactcatagcttatctgctttctctttctgcttttccctgctcccgccagcctaactccttttccctaattaggacttcacaactaacggaggaactaataattaatgtattgagaaaaacagaaaataattacttgtcctcacatgcacacgtatgtttattgcagcactatttaccatagcaaagacttggaaccaacccaaatgcccatcagtgatagactggataaagaaaatatggcacatatacaccatggaatactatgcagccataaaaagaatgagttcatgtcctttgcagcgacatggatgaagctggaaaccatcattctcagcaaactaacacaggaacagaaaaccaaacaccacatgttcttactaataagtgggagttgaacaatgagaacacatggacacagggaggtgaacatcacagaccaaggcctgtcggggggtggggggcaaggggaggaagagcattaggacaaatacctaatgcatgtgggacttaaaacctagatgatgggtcaataggtgcagcaaaccaccttggaacatgtatacctatgtaacaaacctgcaggttctgcacatgtaacccagaacttaaagtaaaataaaataaaataataattacttgtcctagcatatgggaatcaaggaaccaaaaggcagtgtttaaattatataaactggccgggcacagtggcttatgcctgtaattccagccctttaggaggccaaggcgggcagaatccttgaccccaggagttcaagatcagcctgggcaacaatacaaaaccccatttctacaaatgatacaaaaaattagctgagcatgatggctcgcacctgagtcccaagtactcagaaggctgaggtgggaggatcccttgagcctgggaagttgaagctgcagtgaaccatgattgcatcattgcactacagcctgggcaatgggaatgaaaccgtgtctcagaaaaaaaaataataaaagtaaaaaataaaataagtggcataaactatgaagtagcagttgtaacatatttttaggattatgtgggtacagtaggcataactctaaagtggtttctaattggtacaccagtggcctagtgtacacctgcataatcccttccccttttgtttgagtaggatttgggattatgatgggatgttactccgtggttggagtacactaaataacaaaggtgaggcagtttttcagatgcaattaaggttccaaatcctttcatcttttttttttttttttttttttggagaggagtctggctctgtcacccaggctggagtgcagtggtgcaatctcgactcactgcaacctccacctcctaggttcaagcgatcctctcgactcagcctcccaaatagctgggattacaggtgtgcactaccacacccagccaatttttgtatttttagtagagacagggtttcaccatgttggccaggctggtctcaaactcctgacctcaagtgatccacccgccttggcctcccaaagtgctgcgattacaggcataaaccaccacacccagtccaaatccttccatcctaagtcaatcaaaattaattttttcatcacaaaaatgatgaaaatagatcagctttgattcataacagagaaaaccactctaagtgttaaaatcaaaacagaagataatgcctaatgaaaggaggtcaggggtataggatagttggtggaaaaaaatattgataatcattacatgcttgcctgtattattttaaattttttaattaaaaaatatattattttgtagtcacatggacaacaaaaccaaaacattacaaatctccagaaagtgcaatgcataagctctcttagttcaaattaaacatttgaaagatattatttttcatcctatatcttttgtcagttacctgaaatgcatttttcccaaatcaatcttcatacaagaatgtgaagagggccagggatggtggttcacacctataatcccagcactttgggaatccaaggtgggagaatcccttgaggccaggagttcaagaccagcctgggcaacatagcaagaccttgtcttgacaaaaaattaaaaattaaaaattagtcgggcatagtgacatggtgcctgcagtcctagctacttgggaggctgagtcaggaggatcacttgagcttgcaatgagctatgatcttgccactatgctccagcctgggcagtgtgagttaaattttattttctaaattttatttgatgtgaattaaatcttatttaaatttctgctgagaattagcaagaatgtaaataaaattacataaatgtgtaataaaactacattgaatttaacattaaatatatacattaaatgaaaatacaaaattctttatgttaattttataattctcaaatgtaggtgaacgaatttcatcaattttaaaacacattgtttcacatacatgacaattgtatatgacactgtttaaaaacattttatagactccagaagtagacaattagtaataatataacatgcaactgtatcattgttagtaatgttgggtctttactctccaccttctctgccccaagaaacatttaaatgagctgttgcttacagatataacgatttttatcttcacaggattcatctaaagcatttccatttggattatacgctatgcagttctttgtattaaaagtttcaaatgatggaaatagatactgggagagtgcagagccattctcccacaaccaggcggtgtgctcctcactgtaagagagtccaatccagtaaaattgttgactggagctcataaaatccagttcatctgtgttttgaagctgaagcaggctggatttctgagaagcacagagatgccgactttcgttccaagttttctgttcactggaaatgaagtaacagttgcaccggtacccaacccatttttcttggcaagaacagcagtcagagtctttctggagttctatgttgggtcctggagtaaatgctggctcaatactcagtttagtaaaagaatttttcaacaaaattcccaacgtagacatcaacgaaaggcatattatccctaaggtcccagaaattaacctccacagagtggtcttaaacactgccatgagaaattatgttccaagagcgaagtagagaaggcacgatgtgtactttttcagaaagaacagcgttgaattgttgaagctgagctggagattaaagaatctctttaactctttctgagctgccaactctgattgttctttttttgtttgtttttgtttgtttgttttttgag

SEQ ID NO: 11506 - RNA, 4695 nt, Homo sapiens
  source 1..4695: mol_type = other RNA
ctgaatagctgggactacaggtgcctgtcaccacgcctggctaatttttttgtacttgtagtacacacggggtttcaccgtgttagccaggatggtctcaatctcctgacctcgtgatccacccgcctcagcctcccaaagtgctgggattacaggcttgagccaccgcgcccagccatgaaaaactttttaataagtgaaaggaatatgataccgtatgagaaagagaattcaaacaagcagtgtgggaccaagagatatttgcgcaaagacaccattcatctctggatgaaacctgatatttgtgagatgaaacttggtttcatgagagctgaaactgaaatttcttgcagtcttttatctgtgtctggtcacacagcagagacaagatctgtaattatctcatatggaagctatcaataaacaaattgaccctggattccactgagggattttgaactttaaagaactcaccataaaccatttgttagctagttagttagcctactacccatatcatggccaagagtcaaaaacagacacctaggcatctctggaaataagcaaagagctgtcccagttcagctgtaaaataactcactttcttatgcatgcaatatgagaatacagatgtcactaactgatatggcttggctgtgtccccacccaaatctcatcttgaattgtagtgcccctaatcctcacgtatcatgtgagggaactggtaggaggtaatttaatcatgggggtagttacctctttgctgttctcatgatagtgagtgagttctcactagatctgatgatttaataagagggtatttttccttttgctcagcacgtctcctttctgctgccatgcgtagagggatgtgtttgctttcccttctgtcattactgtaagtttcctgaggcttctccaaccctgcagaactgtgagtcaattaaatgtctttattttataaatttcccagtcttgggtatatctttagtagcagcataagaacggactaatacactaatgttgtgggtgagcaacggctacctgggccggtggcattgaggtaaaagaatttaccaagacagctgtaggtaaaggaaggcagatttattaaagaaaagtaggaaaatatgtttccagggaggcaacaggcagcatcagcagaagaaaagctgactgcaaagaaacaaaggcttgcttaggattttatggaatagtgtttatgctgtatgctgcagagggctttgtccagtactgataatgccaaggttgcggtgaggtaacttgcaggtgtctggtaatagtttagcacatggcccatatcctggaccatgaagaaaggcagactcatagcttatctgctttctctttctgcttttccctgctcccgccagcctaactccttttccctaattaggacttcacaactaacggaggaactaataattaatgtattgagaaaaacagaaaataattacttgtcctcacatgcacacgtatgtttattgcagcactatttaccatagcaaagacttggaaccaacccaaatgcccatcagtgatagactggataaagaaaatatggcacatatacaccatggaatactatgcagccataaaaagaatgagttcatgtcctttgcagcgacatggatgaagctggaaaccatcattctcagcaaactaacacaggaacagaaaaccaaacaccacatgttcttactaataagtgggagttgaacaatgagaacacatggacacagggaggtgaacatcacagaccaaggcctgtcggggggtggggggcaaggggaggaagagcattaggacaaatacctaatgcatgtgggacttaaaacctagatgatgggtcaataggtgcagcaaaccaccttggaacatgtatacctatgtaacaaacctgcaggttctgcacatgtaacccagaacttaaagtaaaataaaataaaataataattacttgtcctagcatatgggaatcaaggaaccaaaaggcagtgtttaaattatataaactggccgggcacagtggcttatgcctgtaattccagccctttaggaggccaaggcgggcagaatccttgaccccaggagttcaagatcagcctgggcaacaatacaaaaccccatttctacaaatgatacaaaaaattagctgagcatgatggctcgcacctgagtcccaagtactcagaaggctgaggtgggaggatcccttgagcctgggaagttgaagctgcagtgaaccatgattgcatcattgcactacagcctgggcaatgggaatgaaaccgtgtctcagaaaaaaaaataataaaagtaaaaaataaaataagtggcataaactatgaagtagcagttgtaacatatttttaggattatgtgggtacagtaggcataactctaaagtggtttctaattggtacaccagtggcctagtgtacacctgcataatcccttccccttttgtttgagtaggatttgggattatgatgggatgttactccgtggttggagtacactaaataacaaaggtgaggcagtttttcagatgcaattaaggttccaaatcctttcatcttttttttttttttttttttttggagaggagtctggctctgtcacccaggctggagtgcagtggtgcaatctcgactcactgcaacctccacctcctaggttcaagcgatcctctcgactcagcctcccaaatagctgggattacaggtgtgcactaccacacccagccaatttttgtatttttagtagagacagggtttcaccatgttggccaggctggtctcaaactcctgacctcaagtgatccacccgccttggcctcccaaagtgctgcgattacaggcataaaccaccacacccagtccaaatccttccatcctaagtcaatcaaaattaattttttcatcacaaaaatgatgaaaatagatcagctttgattcataacagagaaaaccactctaagtgttaaaatcaaaacagaagataatgcctaatgaaaggaggtcaggggtataggatagttggtggaaaaaaatattgataatcattacatgcttgcctgtattattttaaattttttaattaaaaaatatattattttgtagtcacatggacaacaaaaccaaaacattacaaatctccagaaagtgcaatgcataagctctcttagttcaaattaaacatttgaaagatattatttttcatcctatatcttttgtcagttacctgaaatgcatttttcccaaatcaatcttcatacaagaatgtgaagagggccagggatggtggttcacacctataatcccagcactttgggaatccaaggtgggagaatcccttgaggccaggagttcaagaccagcctgggcaacatagcaagaccttgtcttgacaaaaaattaaaaattaaaaattagtcgggcatagtgacatggtgcctgcagtcctagctacttgggaggctgagtcaggaggatcacttgagcttgcaatgagctatgatcttgccactatgctccagcctgggcagtgtgagttaaattttattttctaaattttatttgatgtgaattaaatcttatttaaatttctgctgagaattagcaagaatgtaaataaaattacataaatgtgtaataaaactacattgaatttaacattaaatatatacattaaatgaaaatacaaaattctttatgttaattttataattctcaaatgtaggtgaacgaatttcatcaattttaaaacacattgtttcacatacatgacaattgtatatgacactgtttaaaaacattttatagactccagaagtagacaattagtaataatataacatgcaactgtatcattgttagtaatgttgggtctttactctccaccttctctgccccaagaaacatttaaatgagctgttgcttacagatataacgatttttatcttcacaggattcatctaaagcatttccatttggattatacgctatgcagttctttgtattaaaagtttcaaatgatggaaatagatactgggagagtgcagagccattctcccacaaccaggcggtgtgctcctcactgtaagagagtccaatccagtaaaattgttgactggagctcataaaatccagttcatctgtgttttgaagctgaagcaggctggatttctgagaagcacagagatgccgactttcgttccaagttttctgttcactggaaatgaagtaacagttgcaccggtacccaacccatttttcttggcaagaacagcagtcagagtctttctggagttctatgttgggtcctggagtaaatgctggctcaatactcagtttagtaaaagaatttttcaacaaaattcccaacgtagacatcaacgaaaggcatattatccctaaggtcccagaaattaacctccacagagtggtcttaaacactgccatgagaaattatgttccaagagcgaagtagagaaggcacgatgtgtactttttcagaaagaacagcgttgaattgttgaagctgagctggagattaaagaatctgaaagttgagtatgaagaaatttagcaaaaatagagaatgaaaaattgtgtatttaaatgatgttcttgaatcatctattggtgagacatgtattatagtgtgaat

SEQ ID NO: 11507 - RNA, 4689 nt, Homo sapiens
  source 1..4689: mol_type = other RNA
ctgaatagctgggactacaggtgcctgtcaccacgcctggctaatttttttgtacttgtagtacacacggggtttcaccgtgttagccaggatggtctcaatctcctgacctcgtgatccacccgcctcagcctcccaaagtgctgggattacaggcttgagccaccgcgcccagccatgaaaaactttttaataagtgaaaggaatatgataccgtatgagaaagagaattcaaacaagcagtgtgggaccaagagatatttgcgcaaagacaccattcatctctggatgaaacctgatatttgtgagatgaaacttggtttcatgagagctgaaactgaaatttcttgcagtcttttatctgtgtctggtcacacagcagagacaagatctgtaattatctcatatggaagctatcaataaacaaattgaccctggattccactgagggattttgaactttaaagaactcaccataaaccatttgttagctagttagttagcctactacccatatcatggccaagagtcaaaaacagacacctaggcatctctggaaataagcaaagagctgtcccagttcagctgtaaaataactcactttcttatgcatgcaatatgagaatacagatgtcactaactgatatggcttggctgtgtccccacccaaatctcatcttgaattgtagtgcccctaatcctcacgtatcatgtgagggaactggtaggaggtaatttaatcatgggggtagttacctctttgctgttctcatgatagtgagtgagttctcactagatctgatgatttaataagagggtatttttccttttgctcagcacgtctcctttctgctgccatgcgtagagggatgtgtttgctttcccttctgtcattactgtaagtttcctgaggcttctccaaccctgcagaactgtgagtcaattaaatgtctttattttataaatttcccagtcttgggtatatctttagtagcagcataagaacggactaatacactaatgttgtgggtgagcaacggctacctgggccggtggcattgaggtaaaagaatttaccaagacagctgtaggtaaaggaaggcagatttattaaagaaaagtaggaaaatatgtttccagggaggcaacaggcagcatcagcagaagaaaagctgactgcaaagaaacaaaggcttgcttaggattttatggaatagtgtttatgctgtatgctgcagagggctttgtccagtactgataatgccaaggttgcggtgaggtaacttgcaggtgtctggtaatagtttagcacatggcccatatcctggaccatgaagaaaggcagactcatagcttatctgctttctctttctgcttttccctgctcccgccagcctaactccttttccctaattaggacttcacaactaacggaggaactaataattaatgtattgagaaaaacagaaaataattacttgtcctcacatgcacacgtatgtttattgcagcactatttaccatagcaaagacttggaaccaacccaaatgcccatcagtgatagactggataaagaaaatatggcacatatacaccatggaatactatgcagccataaaaagaatgagttcatgtcctttgcagcgacatggatgaagctggaaaccatcattctcagcaaactaacacaggaacagaaaaccaaacaccacatgttcttactaataagtgggagttgaacaatgagaacacatggacacagggaggtgaacatcacagaccaaggcctgtcggggggtggggggcaaggggaggaagagcattaggacaaatacctaatgcatgtgggacttaaaacctagatgatgggtcaataggtgcagcaaaccaccttggaacatgtatacctatgtaacaaacctgcaggttctgcacatgtaacccagaacttaaagtaaaataaaataaaataataattacttgtcctagcatatgggaatcaaggaaccaaaaggcagtgtttaaattatataaactggccgggcacagtggcttatgcctgtaattccagccctttaggaggccaaggcgggcagaatccttgaccccaggagttcaagatcagcctgggcaacaatacaaaaccccatttctacaaatgatacaaaaaattagctgagcatgatggctcgcacctgagtcccaagtactcagaaggctgaggtgggaggatcccttgagcctgggaagttgaagctgcagtgaaccatgattgcatcattgcactacagcctgggcaatgggaatgaaaccgtgtctcagaaaaaaaaataataaaagtaaaaaataaaataagtggcataaactatgaagtagcagttgtaacatatttttaggattatgtgggtacagtaggcataactctaaagtggtttctaattggtacaccagtggcctagtgtacacctgcataatcccttccccttttgtttgagtaggatttgggattatgatgggatgttactccgtggttggagtacactaaataacaaaggtgaggcagtttttcagatgcaattaaggttccaaatcctttcatcttttttttttttttttttttttggagaggagtctggctctgtcacccaggctggagtgcagtggtgcaatctcgactcactgcaacctccacctcctaggttcaagcgatcctctcgactcagcctcccaaatagctgggattacaggtgtgcactaccacacccagccaatttttgtatttttagtagagacagggtttcaccatgttggccaggctggtctcaaactcctgacctcaagtgatccacccgccttggcctcccaaagtgctgcgattacaggcataaaccaccacacccagtccaaatccttccatcctaagtcaatcaaaattaattttttcatcacaaaaatgatgaaaatagatcagctttgattcataacagagaaaaccactctaagtgttaaaatcaaaacagaagataatgcctaatgaaaggaggtcaggggtataggatagttggtggaaaaaaatattgataatcattacatgcttgcctgtattattttaaattttttaattaaaaaatatattattttgtagtcacatggacaacaaaaccaaaacattacaaatctccagaaagtgcaatgcataagctctcttagttcaaattaaacatttgaaagatattatttttcatcctatatcttttgtcagttacctgaaatgcatttttcccaaatcaatcttcatacaagaatgtgaagagggccagggatggtggttcacacctataatcccagcactttgggaatccaaggtgggagaatcccttgaggccaggagttcaagaccagcctgggcaacatagcaagaccttgtcttgacaaaaaattaaaaattaaaaattagtcgggcatagtgacatggtgcctgcagtcctagctacttgggaggctgagtcaggaggatcacttgagcttgcaatgagctatgatcttgccactatgctccagcctgggcagtgtgagttaaattttattttctaaattttatttgatgtgaattaaatcttatttaaatttctgctgagaattagcaagaatgtaaataaaattacataaatgtgtaataaaactacattgaatttaacattaaatatatacattaaatgaaaatacaaaattctttatgttaattttataattctcaaatgtaggtgaacgaatttcatcaattttaaaacacattgtttcacatacatgacaattgtatatgacactgtttaaaaacattttatagactccagaagtagacaattagtaataatataacatgcaactgtatcattgttagtaatgttgggtctttactctccaccttctctgccccaagaaacatttaaatgagctgttgcttacagatataacgatttttatcttcacaggattcatctaaagcatttccatttggattatacgctatgcagttctttgtattaaaagtttcaaatgatggaaatagatactgggagagtgcagagccattctcccacaaccaggcggtgtgctcctcactgtaagagagtccaatccagtaaaattgttgactggagctcataaaatccagttcatctgtgttttgaagctgaagcaggctggatttctgagaagcacagagatgccgactttcgttccaagttttctgttcactggaaatgaagtaacagttgcaccggtacccaacccatttttcttggcaagaacagcagtcagagtctttctggagttctatgttgggtcctggagtaaatgctggctcaatactcagtttagtaaaagaatttttcaacaaaattcccaacgtagacatcaacgaaaggcatattatccctaaggtcccagaaattaacctccacagagtggtcttaaacactgccatgagaaattatgttccaagagcgaagtagagaaggcacgatgtgtactttttcagaaagaacagcgttgaattgttgaagctgagctggagattaaagaatctgtaacccctgctacttgggaggctgaggcattagagtctcttgaacttgatgagctgagatcgcaccattgcactccagcctgggtgacaagagcaaaac

SEQ ID NO: 11508 - RNA, 4602 nt, Homo sapiens
  source 1..4602: mol_type = other RNA
ctgaatagctgggactacaggtgcctgtcaccacgcctggctaatttttttgtacttgtagtacacacggggtttcaccgtgttagccaggatggtctcaatctcctgacctcgtgatccacccgcctcagcctcccaaagtgctgggattacaggcttgagccaccgcgcccagccatgaaaaactttttaataagtgaaaggaatatgataccgtatgagaaagagaattcaaacaagcagtgtgggaccaagagatatttgcgcaaagacaccattcatctctggatgaaacctgatatttgtgagatgaaacttggtttcatgagagctgaaactgaaatttcttgcagtcttttatctgtgtctggtcacacagcagagacaagatctgtaattatctcatatggaagctatcaataaacaaattgaccctggattccactgagggattttgaactttaaagaactcaccataaaccatttgttagctagttagttagcctactacccatatcatggccaagagtcaaaaacagacacctaggcatctctggaaataagcaaagagctgtcccagttcagctgtaaaataactcactttcttatgcatgcaatatgagaatacagatgtcactaactgatatggcttggctgtgtccccacccaaatctcatcttgaattgtagtgcccctaatcctcacgtatcatgtgagggaactggtaggaggtaatttaatcatgggggtagttacctctttgctgttctcatgatagtgagtgagttctcactagatctgatgatttaataagagggtatttttccttttgctcagcacgtctcctttctgctgccatgcgtagagggatgtgtttgctttcccttctgtcattactgtaagtttcctgaggcttctccaaccctgcagaactgtgagtcaattaaatgtctttattttataaatttcccagtcttgggtatatctttagtagcagcataagaacggactaatacactaatgttgtgggtgagcaacggctacctgggccggtggcattgaggtaaaagaatttaccaagacagctgtaggtaaaggaaggcagatttattaaagaaaagtaggaaaatatgtttccagggaggcaacaggcagcatcagcagaagaaaagctgactgcaaagaaacaaaggcttgcttaggattttatggaatagtgtttatgctgtatgctgcagagggctttgtccagtactgataatgccaaggttgcggtgaggtaacttgcaggtgtctggtaatagtttagcacatggcccatatcctggaccatgaagaaaggcagactcatagcttatctgctttctctttctgcttttccctgctcccgccagcctaactccttttccctaattaggacttcacaactaacggaggaactaataattaatgtattgagaaaaacagaaaataattacttgtcctcacatgcacacgtatgtttattgcagcactatttaccatagcaaagacttggaaccaacccaaatgcccatcagtgatagactggataaagaaaatatggcacatatacaccatggaatactatgcagccataaaaagaatgagttcatgtcctttgcagcgacatggatgaagctggaaaccatcattctcagcaaactaacacaggaacagaaaaccaaacaccacatgttcttactaataagtgggagttgaacaatgagaacacatggacacagggaggtgaacatcacagaccaaggcctgtcggggggtggggggcaaggggaggaagagcattaggacaaatacctaatgcatgtgggacttaaaacctagatgatgggtcaataggtgcagcaaaccaccttggaacatgtatacctatgtaacaaacctgcaggttctgcacatgtaacccagaacttaaagtaaaataaaataaaataataattacttgtcctagcatatgggaatcaaggaaccaaaaggcagtgtttaaattatataaactggccgggcacagtggcttatgcctgtaattccagccctttaggaggccaaggcgggcagaatccttgaccccaggagttcaagatcagcctgggcaacaatacaaaaccccatttctacaaatgatacaaaaaattagctgagcatgatggctcgcacctgagtcccaagtactcagaaggctgaggtgggaggatcccttgagcctgggaagttgaagctgcagtgaaccatgattgcatcattgcactacagcctgggcaatgggaatgaaaccgtgtctcagaaaaaaaaataataaaagtaaaaaataaaataagtggcataaactatgaagtagcagttgtaacatatttttaggattatgtgggtacagtaggcataactctaaagtggtttctaattggtacaccagtggcctagtgtacacctgcataatcccttccccttttgtttgagtaggatttgggattatgatgggatgttactccgtggttggagtacactaaataacaaaggtgaggcagtttttcagatgcaattaaggttccaaatcctttcatcttttttttttttttttttttttggagaggagtctggctctgtcacccaggctggagtgcagtggtgcaatctcgactcactgcaacctccacctcctaggttcaagcgatcctctcgactcagcctcccaaatagctgggattacaggtgtgcactaccacacccagccaatttttgtatttttagtagagacagggtttcaccatgttggccaggctggtctcaaactcctgacctcaagtgatccacccgccttggcctcccaaagtgctgcgattacaggcataaaccaccacacccagtccaaatccttccatcctaagtcaatcaaaattaattttttcatcacaaaaatgatgaaaatagatcagctttgattcataacagagaaaaccactctaagtgttaaaatcaaaacagaagataatgcctaatgaaaggaggtcaggggtataggatagttggtggaaaaaaatattgataatcattacatgcttgcctgtattattttaaattttttaattaaaaaatatattattttgtagtcacatggacaacaaaaccaaaacattacaaatctccagaaagtgcaatgcataagctctcttagttcaaattaaacatttgaaagatattatttttcatcctatatcttttgtcagttacctgaaatgcatttttcccaaatcaatcttcatacaagaatgtgaagagggccagggatggtggttcacacctataatcccagcactttgggaatccaaggtgggagaatcccttgaggccaggagttcaagaccagcctgggcaacatagcaagaccttgtcttgacaaaaaattaaaaattaaaaattagtcgggcatagtgacatggtgcctgcagtcctagctacttgggaggctgagtcaggaggatcacttgagcttgcaatgagctatgatcttgccactatgctccagcctgggcagtgtgagttaaattttattttctaaattttatttgatgtgaattaaatcttatttaaatttctgctgagaattagcaagaatgtaaataaaattacataaatgtgtaataaaactacattgaatttaacattaaatatatacattaaatgaaaatacaaaattctttatgttaattttataattctcaaatgtaggtgaacgaatttcatcaattttaaaacacattgtttcacatacatgacaattgtatatgacactgtttaaaaacattttatagactccagaagtagacaattagtaataatataacatgcaactgtatcattgttagtaatgttgggtctttactctccaccttctctgccccaagaaacatttaaatgagctgttgcttacagatataacgatttttatcttcacaggattcatctaaagcatttccatttggattatacgctatgcagttctttgtattaaaagtttcaaatgatggaaatagatactgggagagtgcagagccattctcccacaaccaggcggtgtgctcctcactgtaagagagtccaatccagtaaaattgttgactggagctcataaaatccagttcatctgtgttttgaagctgaagcaggctggatttctgagaagcacagagatgccgactttcgttccaagttttctgttcactggaaatgaagtaacagttgcaccggtacccaacccatttttcttggcaagaacagcagtcagagtctttctggagttctatgttgggtcctggagtaaatgctggctcaatactcagtttagtaaaagctgccatgagaaattatgttccaagagcgaagtagagaaggcacgatgtgtactttttcagaaagaacagcgttgaattgttgaagctgagctggagattaaagaatctgaaagttgagtatgaagaaatttagcaaaaatagagaatgaaaaattgtgtatttaaatgatgttcttgaatcatctattggtgagacatgtattatagtgtgaat

SEQ ID NO: 11509 - RNA, 4546 nt, Homo sapiens
  source 1..4546: mol_type = other RNA
ctgaatagctgggactacaggtgcctgtcaccacgcctggctaatttttttgtacttgtagtacacacggggtttcaccgtgttagccaggatggtctcaatctcctgacctcgtgatccacccgcctcagcctcccaaagtgctgggattacaggcttgagccaccgcgcccagccatgaaaaactttttaataagtgaaaggaatatgataccgtatgagaaagagaattcaaacaagcagtgtgggaccaagagatatttgcgcaaagacaccattcatctctggatgaaacctgatatttgtgagatgaaacttggtttcatgagagctgaaactgaaatttcttgcagtcttttatctgtgtctggtcacacagcagagacaagatctgtaattatctcatatggaagctatcaataaacaaattgaccctggattccactgagggattttgaactttaaagaactcaccataaaccatttgttagctagttagttagcctactacccatatcatggccaagagtcaaaaacagacacctaggcatctctggaaataagcaaagagctgtcccagttcagctgtaaaataactcactttcttatgcatgcaatatgagaatacagatgtcactaactgatatggcttggctgtgtccccacccaaatctcatcttgaattgtagtgcccctaatcctcacgtatcatgtgagggaactggtaggaggtaatttaatcatgggggtagttacctctttgctgttctcatgatagtgagtgagttctcactagatctgatgatttaataagagggtatttttccttttgctcagcacgtctcctttctgctgccatgcgtagagggatgtgtttgctttcccttctgtcattactgtaagtttcctgaggcttctccaaccctgcagaactgtgagtcaattaaatgtctttattttataaatttcccagtcttgggtatatctttagtagcagcataagaacggactaatacactaatgttgtgggtgagcaacggctacctgggccggtggcattgaggtaaaagaatttaccaagacagctgtaggtaaaggaaggcagatttattaaagaaaagtaggaaaatatgtttccagggaggcaacaggcagcatcagcagaagaaaagctgactgcaaagaaacaaaggcttgcttaggattttatggaatagtgtttatgctgtatgctgcagagggctttgtccagtactgataatgccaaggttgcggtgaggtaacttgcaggtgtctggtaatagtttagcacatggcccatatcctggaccatgaagaaaggcagactcatagcttatctgctttctctttctgcttttccctgctcccgccagcctaactccttttccctaattaggacttcacaactaacggaggaactaataattaatgtattgagaaaaacagaaaataattacttgtcctcacatgcacacgtatgtttattgcagcactatttaccatagcaaagacttggaaccaacccaaatgcccatcagtgatagactggataaagaaaatatggcacatatacaccatggaatactatgcagccataaaaagaatgagttcatgtcctttgcagcgacatggatgaagctggaaaccatcattctcagcaaactaacacaggaacagaaaaccaaacaccacatgttcttactaataagtgggagttgaacaatgagaacacatggacacagggaggtgaacatcacagaccaaggcctgtcggggggtggggggcaaggggaggaagagcattaggacaaatacctaatgcatgtgggacttaaaacctagatgatgggtcaataggtgcagcaaaccaccttggaacatgtatacctatgtaacaaacctgcaggttctgcacatgtaacccagaacttaaagtaaaataaaataaaataataattacttgtcctagcatatgggaatcaaggaaccaaaaggcagtgtttaaattatataaactggccgggcacagtggcttatgcctgtaattccagccctttaggaggccaaggcgggcagaatccttgaccccaggagttcaagatcagcctgggcaacaatacaaaaccccatttctacaaatgatacaaaaaattagctgagcatgatggctcgcacctgagtcccaagtactcagaaggctgaggtgggaggatcccttgagcctgggaagttgaagctgcagtgaaccatgattgcatcattgcactacagcctgggcaatgggaatgaaaccgtgtctcagaaaaaaaaataataaaagtaaaaaataaaataagtggcataaactatgaagtagcagttgtaacatatttttaggattatgtgggtacagtaggcataactctaaagtggtttctaattggtacaccagtggcctagtgtacacctgcataatcccttccccttttgtttgagtaggatttgggattatgatgggatgttactccgtggttggagtacactaaataacaaaggtgaggcagtttttcagatgcaattaaggttccaaatcctttcatcttttttttttttttttttttttggagaggagtctggctctgtcacccaggctggagtgcagtggtgcaatctcgactcactgcaacctccacctcctaggttcaagcgatcctctcgactcagcctcccaaatagctgggattacaggtgtgcactaccacacccagccaatttttgtatttttagtagagacagggtttcaccatgttggccaggctggtctcaaactcctgacctcaagtgatccacccgccttggcctcccaaagtgctgcgattacaggcataaaccaccacacccagtccaaatccttccatcctaagtcaatcaaaattaattttttcatcacaaaaatgatgaaaatagatcagctttgattcataacagagaaaaccactctaagtgttaaaatcaaaacagaagataatgcctaatgaaaggaggtcaggggtataggatagttggtggaaaaaaatattgataatcattacatgcttgcctgtattattttaaattttttaattaaaaaatatattattttgtagtcacatggacaacaaaaccaaaacattacaaatctccagaaagtgcaatgcataagctctcttagttcaaattaaacatttgaaagatattatttttcatcctatatcttttgtcagttacctgaaatgcatttttcccaaatcaatcttcatacaagaatgtgaagagggccagggatggtggttcacacctataatcccagcactttgggaatccaaggtgggagaatcccttgaggccaggagttcaagaccagcctgggcaacatagcaagaccttgtcttgacaaaaaattaaaaattaaaaattagtcgggcatagtgacatggtgcctgcagtcctagctacttgggaggctgagtcaggaggatcacttgagcttgcaatgagctatgatcttgccactatgctccagcctgggcagtgtgagttaaattttattttctaaattttatttgatgtgaattaaatcttatttaaatttctgctgagaattagcaagaatgtaaataaaattacataaatgtgtaataaaactacattgaatttaacattaaatatatacattaaatgaaaatacaaaattctttatgttaattttataattctcaaatgtaggtgaacgaatttcatcaattttaaaacacattgtttcacatacatgacaattgtatatgacactgtttaaaaacattttatagactccagaagtagacaattagtaataatataacatgcaactgtatcattgttagtaatgttgggtctttactctccaccttctctgccccaagaaacatttaaatgagctgttgcttacagatataacgatttttatcttcacaggattcatctaaagcatttccatttggattatacgctatgcagttctttgtattaaaagtttcaaatgatggaaatagatactgggagagtgcagagccattctcccacaaccaggcggtgtgctcctcactgtaagagagtccaatccagtaaaattgttgactggagctcataaaatcctgctttctggagttctatgttgggtcctggagtaaatgctggctcaatactcagtttagtaaaagaatttttcaacaaaattcccaacgtagacatcaacgaaaggcatattatccctaaggtcccagaaattaacctccacagagtggtcttaaacactgccatgagaaattatgttccaagagcgaagtagagaaggcacgatgtgtactttttcagaaagaacagcgttgaattgttgaagctgagctggagattaaagaatctgaaagttgagtatgaagaaatttagcaaaaatagagaatgaaaaattgtgtatttaaatgatgttcttgaatcatctattggtgagacatgtattatagtgtgaat

SEQ ID NO: 11510 - RNA, 882 nt, Homo sapiens
  source 1..882: mol_type = other RNA
ctgaatagctgggactacaggtgcgcaccaccacgcccagctaatttttgtaattttagtagagatggggtgtcaccatgttggccaggctggtctcgaactcctgaccttgtaatctgcccaccttggcctcccaacgtgctgggattacaagtgtgagccaccgtgcccggccacaggctgtttgtttttaaatgaaacaaaaaatccaaactggcttttagaattaactgttgtctttcctcacatttttgtcaatttaaagaactgttaagctcctgtaaaaaagatgttatgtaatctgtaactacatttgagaatgttagtcaacttcaaataaattcttaccaaaatacctttttcttgttaacactaattgttgctgaaatattaacctgaacttgcatatcattctatctggcaacttttcagaatagattcataccagcttcacatgccatttattaattcatcaattaattgattcagtaattattagtgaacactaaatgtcaggcacttttctagatgtttgggaatatcagtaaataaaacagattcttgccctcaaggaaatatttatagaactgctgttgtataaacagtactcatcaaatattccactgctcccctgcttttcccagcatcccttacagttaggtttggatcatgtgattacagcaagctaatggcctatcaaggaaatgacatgtatcatttttaggctgaggaaggtataagctaatgtgctccccaaccctgttattacctgtcacacaaccccagaggttaatattccacatggttcagccacaagatataatttgagtcattttggttactgagtctcatagtccgtttgtgctgctatagcaacatacc

SEQ ID NO: 11511 - RNA, 1570 nt, Homo sapiens
  source 1..1570: mol_type = other RNA
ctgaatagctgggactacaggtgcgcaccaccacgcccagctaatttttgtatttttaatagagacagggtttcaccatgttgatcaggctggtctcaaactcctgacctcagatgatccacccgcctcagctaaaaacaatacaaaaaattagccaggcatggtggtgcatgcctgtaatcccagctacttggaaggctgaagcacgagaatcacttgaacctggaaggcagaggttgcagtgagccaagatcgcgccactgaactccagcctgggtgacagagtgagactctgtctcaaaaaaagaaaagaaaagaaaagaaaggccctatattttataggaaatgatacctgaaactgcatttatatatttatagtcttcaaattcataaaaatatataaacatgtaaatatcccttaaaaagcaacatgttcttatactgtcaaatttcagtattttaaaaattacttacttttcagaaaactggataaaccacatggatgccacgagaaggtgtcaggagagccagcaatcctagccaggtggtccctcccaatctctccatcatcaggaggagtgcacagtactggtgtaaggggggatccatacaccacatgctcctggcattgaaagaacaaaccacaattataaaatagcaggacctcacctggaattaataggaagcctgctgttatttctagaagcaatctgacatgcaaaataaacaaaacctacccactttgttatgagttagtcctggctttgtctctgtgtacccttgggcaagtaacttaatctctctcagccttagtttcctcacctctaaaatgctgtgcagcagggtagttgtgaagattaaaggagatgctatacataaagtgccaagaatctagcaaatatggtgctggaacagactttcccatttcctctgcctggccatcttcctctcaagatttgccctaagggtcacggcctctatgaagctttccctgaccctcccacactgggttagttgatcctctggggtcctctgcacccctttccagtgggtgtctctctcagagctcttaaaaggtaaaacgattgctggctgcatagcatggcgcttcccctgcgtttcgtggggcttgaggcctgggatggtgtcttaatcatctctttgctcccggcaccatggccgaccgacaagagccctcacgatggcctctttgactgcatctctcatccttgttccccttgctcactgtgacttagctgccgtggactcttgctggaacttgcgtgtatcaggcagtctcctgtctcagggtcttccatttgctgtttctgaaaaagcgattttaaattaaagagtcttggccaggcacggtaactcatgcctataataccagcactttgggaggccgaacactttgggaggatcgcttgagcccaggagtttgaaaccagcctggcaacatgaagaaaccctgtctctacaaaaaatacaaaaattagctgggcatggtggcacgtgcctgcagtcccagctactcaagggagtggggatgctgaggttggaggattgc

SEQ ID NO: 11512 - RNA, 9760 nt, Homo sapiens
  source 1..9760: mol_type = other RNA
ctgaatagctgggactacaggtgcgcaccaccatgcccggctcagtttccggttcttgaactagactttcctactgagtgtcacatgaaaaaaaacaaacaaaaaagactgaggcacagggacaaaggaaagagtatttagctggcacactctcaccttagttctccatctaccttaaaatgtcccgggggcagagggtgcttgttacaatgaggattctcggtccacaccctagatctgtggactcagaatctttggagggaaactcaggaatcagcctgtaaacaaatatccaagatgattttcgtggcccacctgggatccaaccatatgcccccaagaagcaagatccctgccccagttagagaacctacttttttccccagattccatttctcttgtattcattcttgccttgtttcttcattagcatttcatgttaaccattttgtatgtgatcttgtctggaaagttttctacttttgagcaaacttttaggctccggatataaggaataaggcttttaggctcaggatgtaaggaataagctttcaacttgcacaactgccagtaagttcactggacactttcatttccattgctttttcaaaactaggtttagtaactttgtttccagatggggagagaggatattagcagaattggaaaagcagcattcttgagcactgggtgtttcaaatgtttgtgacacaaaagtggggttggggtggggggatgataaataaatcagcataggctacttccctgatcatcatcatcaaaatatcatttcaagagcagtcattctggataccgacggctttgtcagtgagtctttcattacacagaagagaaaaacacttcccagggtttcctcagcgccaccaccaagtggtgttacatcaccagaagcatggaaattaatccattaatttacttggacattttgacataaaaaaataaatgattgttttctaagcatttcaaatctaaattttttaaataattttttttcatttttgggggaaaatctaaaatttgtaccgggctaccagaactaggacttaatgggattctttctgttacaacatgttactacttgatggcggatactggggtaatggaaggggagggtgcatatgcacgtggccttctagaaaaatcccatatgcaatacatataagaaaatacgctaacttttaaaaataataaaagcagatcaatggttgcctcaggatagaggatggggaaggattacaaaggggcaggggaaacttttggggatgatagatatgttcactattttgattatgtcaagggtatatacatacatcaaactgtatcaagtactgttcaaatatgcgaagtgtattatatgtcggttataccttaatcaagctttaaaaagaacttgagtccaggcgcggttgctcacacctgtaatcccagcactttggggggctgaggcgggtgaaacacttgaggtcaggagttcgagaccagcctggccaacatggcaaaacccccgtctctaactaaaatacaaaaattagctaggtgggtggcacacgcctgtaaacccagctactcgggaggctgaggcacaagaatcccttgaacctgggaggcggaggctgcagtgagccgagattgtgccattgcgctccagcctgggtgacagagcactcaagactctgtctcaaaaaaaaaaaaaaaagtacagcaatatcaataaaattaacaaaaaaagaacttgaaaagacaaaaaaattctagcaacaattttattaaaaaactaaatagatgagaattaagggaaagtgggtgtctaagataaaagaagtaatagttctagcatattctctaacagtattaagaagttcaattgctcactttatgaattaagtgttagaagaaacaggtggaacacaaataagatgatactttgctttatgaaaacttaatattcctctctctacaattgccctcacttctatttgggaggaaggaatggctagaaaaaaaaattgcagaaaataagaacatttttgttttatgtttttttcttaccaatttgaagataccaaagtaactaataaaatgtatttatggggtcatatggtaatatgtaatccatgaaaaattaatagtattcactaggaggctaactgaagtggttttcaatattgaatgtctctgaaactgtacataaatactgtatattttacaaacaatgacacagtgtaaaagaacatacatgtgtatctatgcctttcactatgttaggagcaaggctggagaaaatgaactaaatcagatgttgttttggaaaacaaaaggatgcatatgacaggtaagttcttttccacttatctgtaagctgccttaatcatgaagcttcatttgcttaagatgttggacatgttggtccatcacaacaatttttaaagacctccttctttagatctcattttggacgtaataaagctaagtctttcttagataatttgccatcttctttaaaagcaaaagctacaaaaaaagtctttcaattcaataacaaatatatgctcttacaattatgtattaaacaaaggtttagtttaacagaatgattatgcaatgtacagtttaaacgtatcagttttacaaaagaaattcagttaggacttacaggaccgaatcctactttggatagtattatttctaaacaactgggaagcttttggggaaaaaaaaccccaaatactttaatcttaactccatttatacatttctttccatctttccccaaaagaacatttctagagcacaaaatagattcaaaattgtttaattagatacattttatatatcctgaacataatggctcccatagaaataaactagtattttgtacacaaactttatttactgtgccacattcataatatactgggccaagtgcaaacatttattacatcccctggtgtgtgcagagctctgctcccacaaacacctcattatctaggatgacagagaacaagattagacaagatggataattaaaatccacaaggtaataacaaaaatgtactttatgattataaactcttctccagctacagctgtaaccagtactaagcaaaacagtttaatcaggttttcctccctaaatccagcccccaagccactgctccttggggcaggatctaataattgattagtggggttgctgaaaggcctagggccagaataatctagaggaaaaggtttagaaaattgacaacctggcatctcatatattgaaaatcctttggtttctcttgcccagaaaattgcattttttccccacatatagttgatatgtaccattaaaagttatcttaaataaggtttatttttacaattgcctgaaaattatggggtaggtattttaaaaataatccatgaaaaacaatggcttaatttaagaaaaacaataaaataacagcaaaagagagtaaatctgcaccctgggtgacagcatatggaatcgatgagcttctggtcagcctctaccagtgctggtgtgtgccattgatccgctcagtctagccaagtcctcagaatcatcgtcacttattactgctctcctcaatgaccatctccaatgagatgaagcagcttatgaataaaccatgggagaagtatacaggcatattatgttctcctctatcctagatccttttaggaaaaaacaagaaagtaggcctgaaataaaaaggtttgtataacatcctaaggaataaatcaggtcttattaagagaatgatctaatattctacccttttgctatttagtcttgacagcccaaatactacgtagatgaaaattccaatagagtaagtctcttcattttataaccaccatgtcaataaaaagtaaaaaaggggatgaggccatcgcaccaatgaatattccacaggagatatgatattagtgaattgggtattataggaatagtaactaaaacttaactgaacacttgaattggaataatcagactatctgaatcccaaaagagattctaaatctgagatattatcaaatgtagtgattttaatagacatttttctcattctcatcttgaagtcctcatcagagtgtcaggctacctctgaccaacattcactcacctgatttgtaccatgaccttactgtctggtaaagatcctttctactattttttcttttttgtaattataacccaaattgctaagtacagtcgttgcttccctgatgggtcctggatcctcttccagctacctgataccacatctgatggtcagctgctgctccctttccttcatctctgcttgtaaaaacctttactttgcaggattgttttcttatgtttaggctattttgagactgttcagggaagtgctagtaagtacagaccagaaccactttaaatagtatttaaagctttatcaaccataggagaacagactcccgtgaggaagtcaataggattcttattaaaattaacgacatgtatctcaggatgcagaaaaagaacatcaagatgaatgagcagaaaaagaatcaatatcaaggggaagattttactgccgcagggcaagccacctatggatttaaaatgggaatgagaggaatagagagggtattgttgaagcagaatgcttagatctggtgatggattcgaaaatttacctgagaatgaaattccattctaagctaatgcagactgtacacataacataaaaactcagatgcaagggaggagttttggataaataaaatattgcgccatctagtggaaacgttagcgctttctcttacactctcatcagcagtttttcatttgatggtgtattagccattattaggaatgctttgctgaggagaaataccactaaaatcaacacctcataataaaatgtaaagtgtctgtaactgtatcagagttttaaataacacttaaattctaatggtaagaatccaagaataaacatctaactaacaataaaatatatgtaattttataattccctaggaaaatctctgaggagatattttaaaaaaaacatacaggcatttatatagtcacctacgtgcagaaacaggaatactgatgcaagttttctgcaaaagcctctgtatattagtggaggaaaaacaaatcctgaagtatgcaaaacacacttctgctttcctgctttgggatggatacattccttagcttaagtttcatatctctgccaatagcaaggtaaatgcttaatatgtagccatgtaccatatggaatcacttgatgaaaatttgaaatatgattttgcatagaattcatttaaacaatgcaaataaactactattattcttgcttctgttctcagtggaattcgactagtgtcagtggagcgggcatgggattgagacatggattacatggtgcttcactcaaaaacaattacatttatagtactactaagcccacacaggaattccatatgctttttgttatttccttttaaggttttaacactgatgaccaaatgtccaaatcaaagacagatttttccaaataatagggcacactgtgaggttaggtggaagagggatggtttattatctggacgcaggacaggaaattaacgagccacgtaaatacagagatctacttagcacgtcttttccttctttcccttcagacataccatatggtaactgacttatcagagtaaagcacgtgttgttcacttttaaaaaacccatttaagttagtctcataattgtcctgattgagaaagtgaatcatgccatgattcaaaaaatctgttcttcacataaacctatgagcacacattttaaaaatgatttattgtacatctttgcatttcttaaggcatgaacaatggcatacagatggaacaggttctgagaagcatcacatctttttcgacaaggccagcacaatcacaccacatcaaacagacacacttgaagtctgcactgaccgactgcttgtggcccaggagtcctgcgataggggatggtgcttccagacagtggaacaatcgtgtggtttctatgttgttgttaactttcttgatcagctttaagcaccagttaccatttgtttttctttacaaactggtcagactttggattttatattctgctccttttattctgctttccaaggacggtgtggattttttttttttttttttttttttttttaaggaatatggttgcagcaaaacagaaaggatcccaaagtggttaggggccttgtctaatgcacttctgaaagtccattataaagatgaatagaaaagcaaatggtaggttttcagttgacccagaaaccacacatagctataagaaacataattgtgcatagttatttattcattcagaatgtgatatgttggctagctctacattcccagtctaccaaagaacagggctgtctactttgctaaacccagggtcctttcgaagctcccagtaggtgtcgttagaaacccaggcttctctttgattggcatcaataacttttttaaaaaattttggtatatgttcaagattgttttcttccatatatcgtctccgagatctctggagttcctctactctttgcttctctgatgctgcagcttctaaatttccttcttccaaaaatctttgatctggccggaaccgggcgtctgttggtggaaggagatcttttagtactggatctaactcattgagctcaatagcaaaccttgtgaagccatagtacagctcatagtttgttggcatggaacctggtctccaaatgcactttgcagagggggccacaccacagtagagtccttcatgccactttccaaacagccggtacaccgccttcccctcctgatctatcaccaccccctggacttcattcatgttagaattccaataattcaccttgacaaatgtgagtttgcaaatgcaaacactgcttttggtatttctgatggttacttctccataatgttctatccatcttctcccactgaggatgttgtgtatgcaagtggtgactttattccacacatagtaatctccatactttggaagcatgacattcagtgttccaacaggcaggatttccatcgacttcccccagaacttgtttttccatctgatatcttgccaaaacacaaaattctttgattcacagtgacaggcagaaatgggtggatgatggctaacctgttctgagaaaaagcggaatcccttgtcttctctaatgcattcataagtctccccaaggactgggttgaatggcttacttcctgctctgaaataggtggagcagtatcctgaaactgcaaatgcggcaacgagaaccatgcgctcatatggatcatcagtttccgaagccttgtccaggagctcgctgtattccatttcctcacagaggtgctgcagggtgttgagcggctcgtttagctccacaggcatagagactttagacaggtctttaccaatgttgttcctcaagatattccacaggttaatgttactggtgtcaggacaaggagctggcaggcatgctcgacgcccatttcggaaggcccctcctgtaagctccccattcaggatttgccgagaaatattgtctgcaacactggtgttgtcttcagatatattatcactcacatcactgatgtaagactcatcatctgaagcctcattctctgacgaacttgcagagaggagcacctcttgggcatcaaagaactcagaaacagactctgacatggagaggcggctctcattggctacttgctgtgataaggggagactgacatggatttgctcaccagcctcatcagggctaggaataatatttacactgacaacctgatcacaaataatagactctgaatgtattctgttcaaccgactccttagttcagcattctggttgagtgcctgagacagtgactgtcggagccgtgccatctgcgtgctgtggcctttactgtgatcctgctcggaaaccatctgcttcagcttctccttctctatagctatgctattaaatgcagacttcaaaagagaatgcactttctgtgcgattagacaaaattcttcttgcagctttgtataatctgttgaactttccagagggtcagtgaggtggctagggggagtctgaaattcaatatctgcacaaaggttggggttggaggaatgcaagcgaactggtgacatggtagcactgaaaggaacctgcagttgtatttttgtatctttgctgacactttttgttctccatcgtcttgtgacccgcttgtctttctttgaaatatctacacagttagcctgcatgtcagtaaagttaggtgccgactgagttctctgaagtatttccaaattttgcaggagtttgctaagttccacaaggtttgactggcaatgtgcaagatcttctgcacacctgtccatctcttccgagtcctgtaaccaggctgccactttactctggccagttgtgcacgttgcagggaggctattgctgcatggtaaaggggactgccacggaaagctgtttggttgcatctttccatccattacagaaacattagcagctggtgaggattcagctgtggacgttgaaggaaatatgtgaaaactagcatctcttggtgatctcacaatttcattctgacgatacaaccgatgatgtcgcagtttggagacccatgcatcaaaccagtcctgggatttcaccttcaaatgatagatgtgctcttcggtgtcaaggtctattcttcgagctttctttttaattgacatgactgagagtcccacatctatgctcccatggacctttcctttctgaatatcgagtggtgcctttgaatactttaacattccattatccaggacaaaaaaacgcttgtgccagccttttaaaggccattttcttttcttcagcataaagccctcatgtttgtctggtttctggacattggtttggcctattttcagcccttctataatttcccagctgtcagcttccttggagagggggactggctccggttctagcaattgccgacttacagagggctcggtgctagaggaagcagtcctctccagtatgtgaatactctgcctactgtccctttgggaggatgttgaagaggaggcacttctatgggttggagtggatgttttatgagcaggggaaatgcccttctcatctgaactcatcgctgcagttagagtctcgttttatgcacttaagaccatcccaatcttctctcaaatccacaaacaaagaagtagatgatttttcagcttcattccatttcatgaatcaggtttgactagaaaagagcaggcaatattgagggtgtccaaaccaccttgcaccttggagtcaaagtcttccaagtcagctttatggtcaaagctgtttcacagtgatttatcctcagatgcctgcagcttttctccttgggacatgatatgtctttgaccttgctggggctatctgggtaaattataggggtggctccttaatatccttctgttgctgttttcccagcaagtggcagaacctggagggcgagcggtggcgccgcggactctgcggcggctgcgcggctgcgacgggaggcaggaggcggagagccggccccggcaggcggactggcgcgcgggctagtggaggagaggaggcatgggcgccgcctgcaccgagccgcgatctccagcaccgac

SEQ ID NO: 11513 - RNA, 9667 nt, Homo sapiens
  source 1..9667: mol_type = other RNA
ctgaatagctgggactacaggtgcgcaccaccatgcccggctcagtttccggttcttgaactagactttcctactgagtgtcacatgaaaaaaaacaaacaaaaaagactgaggcacagggacaaaggaaagagtatttagctggcacactctcaccttagttctccatctaccttaaaatgtcccgggggcagagggtgcttgttacaatgaggattctcggtccacaccctagatctgtggactcagaatctttggagggaaactcaggaatcagcctgtaaacaaatatccaagatgattttcgtggcccacctgggatccaaccatatgcccccaagaagcaagatccctgccccagttagagaacctacttttttccccagattccatttctcttgtattcattcttgccttgtttcttcattagcatttcatgttaaccattttgtatgtgatcttgtctggaaagttttctacttttgagcaaacttttaggctccggatataaggaataaggcttttaggctcaggatgtaaggaataagctttcaacttgcacaactgccagtaagttcactggacactttcatttccattgctttttcaaaactaggtttagtaactttgtttccagatggggagagaggatattagcagaattggaaaagcagcattcttgagcactgggtgtttcaaatgtttgtgacacaaaagtggggttggggtggggggatgataaataaatcagcataggctacttccctgatcatcatcatcaaaatatcatttcaagagcagtcattctggataccgacggctttgtcagtgagtctttcattacacagaagagaaaaacacttcccagggtttcctcagcgccaccaccaagtggtgttacatcaccagaagcatggaaattaatccattaatttacttggacattttgacataaaaaaataaatgattgttttctaagcatttcaaatctaaattttttaaataattttttttcatttttgggggaaaatctaaaatttgtaccgggctaccagaactaggacttaatgggattctttctgttacaacatgttactacttgatggcggatactggggtaatggaaggggagggtgcatatgcacgtggccttctagaaaaatcccatatgcaatacatataagaaaatacgctaacttttaaaaataataaaagcagatcaatggttgcctcaggatagaggatggggaaggattacaaaggggcaggggaaacttttggggatgatagatatgttcactattttgattatgtcaagggtatatacatacatcaaactgtatcaagtactgttcaaatatgcgaagtgtattatatgtcggttataccttaatcaagctttaaaaagaacttgagtccaggcgcggttgctcacacctgtaatcccagcactttggggggctgaggcgggtgaaacacttgaggtcaggagttcgagaccagcctggccaacatggcaaaacccccgtctctaactaaaatacaaaaattagctaggtgggtggcacacgcctgtaaacccagctactcgggaggctgaggcacaagaatcccttgaacctgggaggcggaggctgcagtgagccgagattgtgccattgcgctccagcctgggtgacagagcactcaagactctgtctcaaaaaaaaaaaaaaaagtacagcaatatcaataaaattaacaaaaaaagaacttgaaaagacaaaaaaattctagcaacaattttattaaaaaactaaatagatgagaattaagggaaagtgggtgtctaagataaaagaagtaatagttctagcatattctctaacagtattaagaagttcaattgctcactttatgaattaagtgttagaagaaacaggtggaacacaaataagatgatactttgctttatgaaaacttaatattcctctctctacaattgccctcacttctatttgggaggaaggaatggctagaaaaaaaaattgcagaaaataagaacatttttgttttatgtttttttcttaccaatttgaagataccaaagtaactaataaaatgtatttatggggtcatatggtaatatgtaatccatgaaaaattaatagtattcactaggaggctaactgaagtggttttcaatattgaatgtctctgaaactgtacataaatactgtatattttacaaacaatgacacagtgtaaaagaacatacatgtgtatctatgcctttcactatgttaggagcaaggctggagaaaatgaactaaatcagatgttgttttggaaaacaaaaggatgcatatgacaggtaagttcttttccacttatctgtaagctgccttaatcatgaagcttcatttgcttaagatgttggacatgttggtccatcacaacaatttttaaagacctccttctttagatctcattttggacgtaataaagctaagtctttcttagataatttgccatcttctttaaaagcaaaagctacaaaaaaagtctttcaattcaataacaaatatatgctcttacaattatgtattaaacaaaggtttagtttaacagaatgattatgcaatgtacagtttaaacgtatcagttttacaaaagaaattcagttaggacttacaggaccgaatcctactttggatagtattatttctaaacaactgggaagcttttggggaaaaaaaaccccaaatactttaatcttaactccatttatacatttctttccatctttccccaaaagaacatttctagagcacaaaatagattcaaaattgtttaattagatacattttatatatcctgaacataatggctcccatagaaataaactagtattttgtacacaaactttatttactgtgccacattcataatatactgggccaagtgcaaacatttattacatcccctggtgtgtgcagagctctgctcccacaaacacctcattatctaggatgacagagaacaagattagacaagatggataattaaaatccacaaggtaataacaaaaatgtactttatgattataaactcttctccagctacagctgtaaccagtactaagcaaaacagtttaatcaggttttcctccctaaatccagcccccaagccactgctccttggggcaggatctaataattgattagtggggttgctgaaaggcctagggccagaataatctagaggaaaaggtttagaaaattgacaacctggcatctcatatattgaaaatcctttggtttctcttgcccagaaaattgcattttttccccacatatagttgatatgtaccattaaaagttatcttaaataaggtttatttttacaattgcctgaaaattatggggtaggtattttaaaaataatccatgaaaaacaatggcttaatttaagaaaaacaataaaataacagcaaaagagagtaaatctgcaccctgggtgacagcatatggaatcgatgagcttctggtcagcctctaccagtgctggtgtgtgccattgatccgctcagtctagccaagtcctcagaatcatcgtcacttattactgctctcctcaatgaccatctccaatgagatgaagcagcttatgaataaaccatgggagaagtatacaggcatattatgttctcctctatcctagatccttttaggaaaaaacaagaaagtaggcctgaaataaaaaggtttgtataacatcctaaggaataaatcaggtcttattaagagaatgatctaatattctacccttttgctatttagtcttgacagcccaaatactacgtagatgaaaattccaatagagtaagtctcttcattttataaccaccatgtcaataaaaagtaaaaaaggggatgaggccatcgcaccaatgaatattccacaggagatatgatattagtgaattgggtattataggaatagtaactaaaacttaactgaacacttgaattggaataatcagactatctgaatcccaaaagagattctaaatctgagatattatcaaatgtagtgattttaatagacatttttctcattctcatcttgaagtcctcatcagagtgtcaggctacctctgaccaacattcactcacctgatttgtaccatgaccttactgtctggtaaagatcctttctactattttttcttttttgtaattataacccaaattgctaagtacagtcgttgcttccctgatgggtcctggatcctcttccagctacctgataccacatctgatggtcagctgctgctccctttccttcatctctgcttgtaaaaacctttactttgcaggattgttttcttatgtttaggctattttgagactgttcagggaagtgctagtaagtacagaccagaaccactttaaatagtatttaaagctttatcaaccataggagaacagactcccgtgaggaagtcaataggattcttattaaaattaacgacatgtatctcaggatgcagaaaaagaacatcaagatgaatgagcagaaaaagaatcaatatcaaggggaagattttactgccgcagggcaagccacctatggatttaaaatgggaatgagaggaatagagagggtattgttgaagcagaatgcttagatctggtgatggattcgaaaatttacctgagaatgaaattccattctaagctaatgcagactgtacacataacataaaaactcagatgcaagggaggagttttggataaataaaatattgcgccatctagtggaaacgttagcgctttctcttacactctcatcagcagtttttcatttgatggtgtattagccattattaggaatgctttgctgaggagaaataccactaaaatcaacacctcataataaaatgtaaagtgtctgtaactgtatcagagttttaaataacacttaaattctaatggtaagaatccaagaataaacatctaactaacaataaaatatatgtaattttataattccctaggaaaatctctgaggagatattttaaaaaaaacatacaggcatttatatagtcacctacgtgcagaaacaggaatactgatgcaagttttctgcaaaagcctctgtatattagtggaggaaaaacaaatcctgaagtatgcaaaacacacttctgctttcctgctttgggatggatacattccttagcttaagtttcatatctctgccaatagcaaggtaaatgcttaatatgtagccatgtaccatatggaatcacttgatgaaaatttgaaatatgattttgcatagaattcatttaaacaatgcaaataaactactattattcttgcttctgttctcagtggaattcgactagtgtcagtggagcgggcatgggattgagacatggattacatggtgcttcactcaaaaacaattacatttatagtactactaagcccacacaggaattccatatgctttttgttatttccttttaaggttttaacactgatgaccaaatgtccaaatcaaagacagatttttccaaataatagggcacactgtgaggttaggtggaagagggatggtttattatctggacgcaggacaggaaattaacgagccacgtaaatacagagatctacttagcacgtcttttccttctttcccttcagacataccatatggtaactgacttatcagagtaaagcacgtgttgttcacttttaaaaaacccatttaagttagtctcataattgtcctgattgagaaagtgaatcatgccatgattcaaaaaatctgttcttcacataaacctatgagcacacattttaaaaatgatttattgtacatctttgcatttcttaaggcatgaacaatggcatacagatggaacaggttctgagaagcatcacatctttttcgacaaggccagcacaatcacaccacatcaaacagacacacttgaagtctgcactgaccgactgcttgtggcccaggagtcctgcgataggggatggtgcttccagacagtggaacaatcgtgtggtttctatgttgttgttaactttcttgatcagctttaagcaccagttaccatttgtttttctttacaaactggtcagactttggattttatattctgctccttttattctgctttccaaggacggtgtggattttttttttttttttttttttttttttaaggaatatggttgcagcaaaacagaaaggatcccaaagtggttaggggccttgtctaatgcacttctgaaagtccattataaagatgaatagaaaagcaaatggtaggttttcagttgacccagaaaccacacatagctataagaaacataattgtgcatagttatttattcattcagaatgtgatatgttggctagctctacattcccagtctaccaaagaacagggctgtctactttgctaaacccagggtcctttcgaagctcccagtaggtgtcgttagaaacccaggcttctctttgattggcatcaataacttttttaaaaaattttggtatatgttcaagattgttttcttccatatatcgtctccgagatctctggagttcctctactctttgcttctctgatgctgcagcttctaaatttccttcttccaaaaatctttgatctggccggaaccgggcgtctgttggtggaaggagatcttttagtactggatctaactcattgagctcaatagcaaaccttgtgaagccatagtacagctcatagtttgttggcatggaacctggtctccaaatgcactttgcagagggggccacaccacagtagagtccttcatgccactttccaaacagccggtacaccgccttcccctcctgatctatcaccaccccctggacttcattcatgttagaattccaataattcaccttgacaaatgtgagtttgcaaatgcaaacactgcttttggtatttctgatggttacttctccataatgttctatccatcttctcccactgaggatgttgtgtatgcaagtggtgactttattccacacatagtaatctccatactttggaagcatgacattcagtgttccaacaggcaggatttccatcgacttcccccagaacttgtttttccatctgatatcttgccaaaacacaaaattctttgattcacagtgacaggcagaaatgggtggatgatggctaacctgttctgagaaaaagcggaatcccttgtcttctctaatgcattcataagtctccccaaggactgggttgaatggcttacttcctgctctgaaataggtggagcagtatcctgaaactgcaaatgcggcaacgagaaccatgcgctcatatggatcatcagtttccgaagccttgtccaggagctcgctgtattccatttcctcacagaggtgctgcagggtgttgagcggctcgtttagctccacaggcatagagactttagacaggtctttaccaatgttgttcctcaagatattccacaggttaatgttactggtgtcaggacaaggagctggcaggcatgctcgacgcccatttcggaaggcccctcctgtaagctccccattcaggatttgccgagaaatattgtctgcaacactggtgttgtcttcagatatattatcactcacatcactgatgtaagactcatcatctgaagcctcattctctgacgaacttgcagagaggagcacctcttgggcatcaaagaactcagaaacagactctgacatggagaggcggctctcattggctacttgctgtgataaggggagactgacatggatttgctcaccagcctcatcagggctaggaataatatttacactgacaacctgatcacaaataatagactctgaatgtattctgttcaaccgactccttagttcagcattctggttgagtgcctgagacagtgactgtcggagccgtgccatctgcgtgctgtggcctttactgtgatcctgctcggaaaccatctgcttcagcttctccttctctatagctatgctattaaatgcagacttcaaaagagaatgcactttctgtgcgattagacaaaattcttcttgcagctttgtataatctgttgaactttccagagggtcagtgaggtggctagggggagtctgaaattcaatatctgcacaaaggttggggttggaggaatgcaagcgaactggtgacatggtagcactgaaaggaacctgcatgtcagtaaagttaggtgccgactgagttctctgaagtatttccaaattttgcaggagtttgctaagttccacaaggtttgactggcaatgtgcaagatcttctgcacacctgtccatctcttccgagtcctgtaaccaggctgccactttactctggccagttgtgcacgttgcagggaggctattgctgcatggtaaaggggactgccacggaaagctgtttggttgcatctttccatccattacagaaacattagcagctggtgaggattcagctgtggacgttgaaggaaatatgtgaaaactagcatctcttggtgatctcacaatttcattctgacgatacaaccgatgatgtcgcagtttggagacccatgcatcaaaccagtcctgggatttcaccttcaaatgatagatgtgctcttcggtgtcaaggtctattcttcgagctttctttttaattgacatgactgagagtcccacatctatgctcccatggacctttcctttctgaatatcgagtggtgcctttgaatactttaacattccattatccaggacaaaaaaacgcttgtgccagccttttaaaggccattttcttttcttcagcataaagccctcatgtttgtctggtttctggacattggtttggcctattttcagcccttctataatttcccagctgtcagcttccttggagagggggactggctccggttctagcaattgccgacttacagagggctcggtgctagaggaagcagtcctctccagtatgtgaatactctgcctactgtccctttgggaggatgttgaagaggaggcacttctatgggttggagtggatgttttatgagcaggggaaatgcccttctcatctgaactcatcgctgcagttagagtctcgttttatgcacttaagaccatcccaatcttctctcaaatccacaaacaaagaagtagatgatttttcagcttcattccatttcatgaatcaggtttgactagaaaagagcaggcaatattgagggtgtccaaaccaccttgcaccttggagtcaaagtcttccaagtcagctttatggtcaaagctgtttcacagtgatttatcctcagatgcctgcagcttttctccttgggacatgatatgtctttgaccttgctggggctatctgggtaaattataggggtggctccttaatatccttctgttgctgttttcccagcaagtggcagaacctggagggcgagcggtggcgccgcggactctgcggcggctgcgcggctgcgacgggaggcaggaggcggagagccggccccggcaggcggactggcgcgcgggctagtggaggagaggaggcatgggcgccgcctgcaccgagccgcgatctccagcaccgac

SEQ ID NO: 11514 - RNA, 9381 nt, Homo sapiens
  source 1..9381: mol_type = other RNA
ctgaatagctgggactacaggtgcgcaccaccatgcccggctcagtttccggttcttgaactagactttcctactgagtgtcacatgaaaaaaaacaaacaaaaaagactgaggcacagggacaaaggaaagagtatttagctggcacactctcaccttagttctccatctaccttaaaatgtcccgggggcagagggtgcttgttacaatgaggattctcggtccacaccctagatctgtggactcagaatctttggagggaaactcaggaatcagcctgtaaacaaatatccaagatgattttcgtggcccacctgggatccaaccatatgcccccaagaagcaagatccctgccccagttagagaacctacttttttccccagattccatttctcttgtattcattcttgccttgtttcttcattagcatttcatgttaaccattttgtatgtgatcttgtctggaaagttttctacttttgagcaaacttttaggctccggatataaggaataaggcttttaggctcaggatgtaaggaataagctttcaacttgcacaactgccagtaagttcactggacactttcatttccattgctttttcaaaactaggtttagtaactttgtttccagatggggagagaggatattagcagaattggaaaagcagcattcttgagcactgggtgtttcaaatgtttgtgacacaaaagtggggttggggtggggggatgataaataaatcagcataggctacttccctgatcatcatcatcaaaatatcatttcaagagcagtcattctggataccgacggctttgtcagtgagtctttcattacacagaagagaaaaacacttcccagggtttcctcagcgccaccaccaagtggtgttacatcaccagaagcatggaaattaatccattaatttacttggacattttgacataaaaaaataaatgattgttttctaagcatttcaaatctaaattttttaaataattttttttcatttttgggggaaaatctaaaatttgtaccgggctaccagaactaggacttaatgggattctttctgttacaacatgttactacttgatggcggatactggggtaatggaaggggagggtgcatatgcacgtggccttctagaaaaatcccatatgcaatacatataagaaaatacgctaacttttaaaaataataaaagcagatcaatggttgcctcaggatagaggatggggaaggattacaaaggggcaggggaaacttttggggatgatagatatgttcactattttgattatgtcaagggtatatacatacatcaaactgtatcaagtactgttcaaatatgcgaagtgtattatatgtcggttataccttaatcaagctttaaaaagaacttgagtccaggcgcggttgctcacacctgtaatcccagcactttggggggctgaggcgggtgaaacacttgaggtcaggagttcgagaccagcctggccaacatggcaaaacccccgtctctaactaaaatacaaaaattagctaggtgggtggcacacgcctgtaaacccagctactcgggaggctgaggcacaagaatcccttgaacctgggaggcggaggctgcagtgagccgagattgtgccattgcgctccagcctgggtgacagagcactcaagactctgtctcaaaaaaaaaaaaaaaagtacagcaatatcaataaaattaacaaaaaaagaacttgaaaagacaaaaaaattctagcaacaattttattaaaaaactaaatagatgagaattaagggaaagtgggtgtctaagataaaagaagtaatagttctagcatattctctaacagtattaagaagttcaattgctcactttatgaattaagtgttagaagaaacaggtggaacacaaataagatgatactttgctttatgaaaacttaatattcctctctctacaattgccctcacttctatttgggaggaaggaatggctagaaaaaaaaattgcagaaaataagaacatttttgttttatgtttttttcttaccaatttgaagataccaaagtaactaataaaatgtatttatggggtcatatggtaatatgtaatccatgaaaaattaatagtattcactaggaggctaactgaagtggttttcaatattgaatgtctctgaaactgtacataaatactgtatattttacaaacaatgacacagtgtaaaagaacatacatgtgtatctatgcctttcactatgttaggagcaaggctggagaaaatgaactaaatcagatgttgttttggaaaacaaaaggatgcatatgacaggtaagttcttttccacttatctgtaagctgccttaatcatgaagcttcatttgcttaagatgttggacatgttggtccatcacaacaatttttaaagacctccttctttagatctcattttggacgtaataaagctaagtctttcttagataatttgccatcttctttaaaagcaaaagctacaaaaaaagtctttcaattcaataacaaatatatgctcttacaattatgtattaaacaaaggtttagtttaacagaatgattatgcaatgtacagtttaaacgtatcagttttacaaaagaaattcagttaggacttacaggaccgaatcctactttggatagtattatttctaaacaactgggaagcttttggggaaaaaaaaccccaaatactttaatcttaactccatttatacatttctttccatctttccccaaaagaacatttctagagcacaaaatagattcaaaattgtttaattagatacattttatatatcctgaacataatggctcccatagaaataaactagtattttgtacacaaactttatttactgtgccacattcataatatactgggccaagtgcaaacatttattacatcccctggtgtgtgcagagctctgctcccacaaacacctcattatctaggatgacagagaacaagattagacaagatggataattaaaatccacaaggtaataacaaaaatgtactttatgattataaactcttctccagctacagctgtaaccagtactaagcaaaacagtttaatcaggttttcctccctaaatccagcccccaagccactgctccttggggcaggatctaataattgattagtggggttgctgaaaggcctagggccagaataatctagaggaaaaggtttagaaaattgacaacctggcatctcatatattgaaaatcctttggtttctcttgcccagaaaattgcattttttccccacatatagttgatatgtaccattaaaagttatcttaaataaggtttatttttacaattgcctgaaaattatggggtaggtattttaaaaataatccatgaaaaacaatggcttaatttaagaaaaacaataaaataacagcaaaagagagtaaatctgcaccctgggtgacagcatatggaatcgatgagcttctggtcagcctctaccagtgctggtgtgtgccattgatccgctcagtctagccaagtcctcagaatcatcgtcacttattactgctctcctcaatgaccatctccaatgagatgaagcagcttatgaataaaccatgggagaagtatacaggcatattatgttctcctctatcctagatccttttaggaaaaaacaagaaagtaggcctgaaataaaaaggtttgtataacatcctaaggaataaatcaggtcttattaagagaatgatctaatattctacccttttgctatttagtcttgacagcccaaatactacgtagatgaaaattccaatagagtaagtctcttcattttataaccaccatgtcaataaaaagtaaaaaaggggatgaggccatcgcaccaatgaatattccacaggagatatgatattagtgaattgggtattataggaatagtaactaaaacttaactgaacacttgaattggaataatcagactatctgaatcccaaaagagattctaaatctgagatattatcaaatgtagtgattttaatagacatttttctcattctcatcttgaagtcctcatcagagtgtcaggctacctctgaccaacattcactcacctgatttgtaccatgaccttactgtctggtaaagatcctttctactattttttcttttttgtaattataacccaaattgctaagtacagtcgttgcttccctgatgggtcctggatcctcttccagctacctgataccacatctgatggtcagctgctgctccctttccttcatctctgcttgtaaaaacctttactttgcaggattgttttcttatgtttaggctattttgagactgttcagggaagtgctagtaagtacagaccagaaccactttaaatagtatttaaagctttatcaaccataggagaacagactcccgtgaggaagtcaataggattcttattaaaattaacgacatgtatctcaggatgcagaaaaagaacatcaagatgaatgagcagaaaaagaatcaatatcaaggggaagattttactgccgcagggcaagccacctatggatttaaaatgggaatgagaggaatagagagggtattgttgaagcagaatgcttagatctggtgatggattcgaaaatttacctgagaatgaaattccattctaagctaatgcagactgtacacataacataaaaactcagatgcaagggaggagttttggataaataaaatattgcgccatctagtggaaacgttagcgctttctcttacactctcatcagcagtttttcatttgatggtgtattagccattattaggaatgctttgctgaggagaaataccactaaaatcaacacctcataataaaatgtaaagtgtctgtaactgtatcagagttttaaataacacttaaattctaatggtaagaatccaagaataaacatctaactaacaataaaatatatgtaattttataattccctaggaaaatctctgaggagatattttaaaaaaaacatacaggcatttatatagtcacctacgtgcagaaacaggaatactgatgcaagttttctgcaaaagcctctgtatattagtggaggaaaaacaaatcctgaagtatgcaaaacacacttctgctttcctgctttgggatggatacattccttagcttaagtttcatatctctgccaatagcaaggtaaatgcttaatatgtagccatgtaccatatggaatcacttgatgaaaatttgaaatatgattttgcatagaattcatttaaacaatgcaaataaactactattattcttgcttctgttctcagtggaattcgactagtgtcagtggagcgggcatgggattgagacatggattacatggtgcttcactcaaaaacaattacatttatagtactactaagcccacacaggaattccatatgctttttgttatttccttttaaggttttaacactgatgaccaaatgtccaaatcaaagacagatttttccaaataatagggcacactgtgaggttaggtggaagagggatggtttattatctggacgcaggacaggaaattaacgagccacgtaaatacagagatctacttagcacgtcttttccttctttcccttcagacataccatatggtaactgacttatcagagtaaagcacgtgttgttcacttttaaaaaacccatttaagttagtctcataattgtcctgattgagaaagtgaatcatgccatgattcaaaaaatctgttcttcacataaacctatgagcacacattttaaaaatgatttattgtacatctttgcatttcttaaggcatgaacaatggcatacagatggaacaggttctgagaagcatcacatctttttcgacaaggccagcacaatcacaccacatcaaacagacacacttgaagtctgcactgaccgactgcttgtggcccaggagtcctgcgataggggatggtgcttccagacagtggaacaatcgtgtggtttctatgttgttgttaactttcttgatcagctttaagcaccagttaccatttgtttttctttacaaactggtcagactttggattttatattctgctccttttattctgctttccaaggacggtgtggattttttttttttttttttttttttttttaaggaatatggttgcagcaaaacagaaaggatcccaaagtggttaggggccttgtctaatgcacttctgaaagtccattataaagatgaatagaaaagcaaatggtaggttttcagttgacccagaaaccacacatagctataagaaacataattgtgcatagttatttattcattcagaatgtgatatgttggctagctctacattcccagtctaccaaagaacagggctgtctactttgctaaacccagggtcctttcgaagctcccagtaggtgtcgttagaaacccaggcttctctttgattggcatcaataacttttttaaaaaattttggtatatgttcaagattgttttcttccatatatcgtctccgagatctctggagttcctctactctttgcttctctgatgctgcagcttctaaatttccttcttccaaaaatctttgatctggccggaaccgggcgtctgttggtggaaggagatcttttagtactggatctaactcattgagctcaatagcaaaccttgtgaagccatagtacagctcatagtttgttggcatggaacctggtctccaaatgcactttgcagagggggccacaccacagtagagtccttcatgccactttccaaacagccggtacaccgccttcccctcctgatctatcaccaccccctggacttcattcatgttagaattccaataattcaccttgacaaatgtgagtttgcaaatgcaaacactgcttttggtatttctgatggttacttctccataatgttctatccatcttctcccactgaggatgttgtgtatgcaagtggtgactttattccacacatagtaatctccatactttggaagcatgacattcagtgttccaacaggcaggatttccatcgacttcccccagaacttgtttttccatctgatatcttgccaaaacacaaaattctttgattcacagtgacaggcagaaatgggtggatgatggctaacctgttctgagaaaaagcggaatcccttgtcttctctaatgcattcataagtctccccaaggactgggttgaatggcttacttcctgctctgaaataggtggagcagtatcctgaaactgcaaatgcggcaacgagaaccatgcgctcatatggatcatcagtttccgaagccttgtccaggagctcgctgtattccatttcctcacagaggtgctgcagggtgttgagcggctcgtttagctccacaggcatagagactttagacaggtctttaccaatgttgttcctcaagatattccacaggttaatgttactggtgtcaggacaaggagctggcaggcatgctcgacgcccatttcggaaggcccctcctgtaagctccccattcaggatttgccgagaaatattgtctgcaacactggtgttgtcttcagatatattatcactcacatcactgatgtaagactcatcatctgaagcctcattctctgacgaacttgcagagaggagcacctcttgggcatcaaagaactcagaaacagactctgacatggagaggcggctctcattggctacttgctgtgataaggggagactgacatggatttgctcaccagcctcatcagggctaggaataatatttacactgacaacctgatcacaaataatagactctgaatgtattctgttcaaccgactccttagttcagcattctggttgagtgcctgagacagtgactgtcggagccgtgccatctgcgtgctgtggcctttactgtgatcctgctcggaaaccatctgcttcagcttctccttctctatagctatgctattaaatgcagacttcaaaagagaatgcactttctgtgcgattagacaaaattcttcttgcagctttgtataatctgttgaactttccagagggtcagtgaggtggctagggggagtctgaaattcaatatctgcacaaaggttggggttggaggaatgcaagcgaactggtgacatggtagcactgaaaggaactgttgtagccactgctgccgctagcctctgccggcgccgagttgtgctgaactggcccttcgcgggtggcccttcctgcagttgtatttttgtatctttgctgacactttttgttctccatcgtcttgtgacccgcttgtctttctttgaaatatctacacagttagcctgcatgtcagtaaagttaggtgccgactgagttctctgaagtatttccaaattttgcaggagtttgctaagttccacaaggtttgactggcaatgtgcaagatcttctgcacacctgtccatctcttccgagtcctgtaaccaggctgccactttactctggccagttgtgcacgttgcagggaggctattgctgcatggtaaaggggactgccacggaaagctgtttggttgcatctttccatccattacagaaacattagcagctggtgaggattcagctgtggacgttgaaggaaatatgtgaaaactagcatctcttggtgatctcacaatttcattctgacgatacaaccgatgatgtcgcagtttggagacccatgcatcaaaccagtcctgggatttcaccttcaaatgatagatgtgctcttcggtgtcaaggtctattcttcgagctttctttttaattgacatgactgagagtcccacatctatgctcccatggacctttcctttctgaatatcgagtggtgcctttgaatactttaacattccattatccaggacaaaaaaacgcttgtgccagccttttaaaggccattttcttttcttcagcataaagccctcatgtttgtctggtttctggacattggtttggcctattttcagcccttctataatttcccagctgtcagcttccttggagagggggactggctccggttctagcaattgccgacttacagagggctcggtgctagaggaagcagtcctctccagtatgtgaatactccgccctctgtttcccctgatcagagataactgatgcatatttagcttaaaaccaggaacctggaacacatatttcactgtagctctttaatttggtaaaaatatgctcctcaggttagtgttcattgatctcaatacctcctgagcagcaagtggaaatg

SEQ ID NO: 11515 - RNA, 9835 nt, Homo sapiens
  source 1..9835: mol_type = other RNA
ctgaatagctgggactacaggtgcgcaccaccatgcccggctcagtttccggttcttgaactagactttcctactgagtgtcacatgaaaaaaaacaaacaaaaaagactgaggcacagggacaaaggaaagagtatttagctggcacactctcaccttagttctccatctaccttaaaatgtcccgggggcagagggtgcttgttacaatgaggattctcggtccacaccctagatctgtggactcagaatctttggagggaaactcaggaatcagcctgtaaacaaatatccaagatgattttcgtggcccacctgggatccaaccatatgcccccaagaagcaagatccctgccccagttagagaacctacttttttccccagattccatttctcttgtattcattcttgccttgtttcttcattagcatttcatgttaaccattttgtatgtgatcttgtctggaaagttttctacttttgagcaaacttttaggctccggatataaggaataaggcttttaggctcaggatgtaaggaataagctttcaacttgcacaactgccagtaagttcactggacactttcatttccattgctttttcaaaactaggtttagtaactttgtttccagatggggagagaggatattagcagaattggaaaagcagcattcttgagcactgggtgtttcaaatgtttgtgacacaaaagtggggttggggtggggggatgataaataaatcagcataggctacttccctgatcatcatcatcaaaatatcatttcaagagcagtcattctggataccgacggctttgtcagtgagtctttcattacacagaagagaaaaacacttcccagggtttcctcagcgccaccaccaagtggtgttacatcaccagaagcatggaaattaatccattaatttacttggacattttgacataaaaaaataaatgattgttttctaagcatttcaaatctaaattttttaaataattttttttcatttttgggggaaaatctaaaatttgtaccgggctaccagaactaggacttaatgggattctttctgttacaacatgttactacttgatggcggatactggggtaatggaaggggagggtgcatatgcacgtggccttctagaaaaatcccatatgcaatacatataagaaaatacgctaacttttaaaaataataaaagcagatcaatggttgcctcaggatagaggatggggaaggattacaaaggggcaggggaaacttttggggatgatagatatgttcactattttgattatgtcaagggtatatacatacatcaaactgtatcaagtactgttcaaatatgcgaagtgtattatatgtcggttataccttaatcaagctttaaaaagaacttgagtccaggcgcggttgctcacacctgtaatcccagcactttggggggctgaggcgggtgaaacacttgaggtcaggagttcgagaccagcctggccaacatggcaaaacccccgtctctaactaaaatacaaaaattagctaggtgggtggcacacgcctgtaaacccagctactcgggaggctgaggcacaagaatcccttgaacctgggaggcggaggctgcagtgagccgagattgtgccattgcgctccagcctgggtgacagagcactcaagactctgtctcaaaaaaaaaaaaaaaagtacagcaatatcaataaaattaacaaaaaaagaacttgaaaagacaaaaaaattctagcaacaattttattaaaaaactaaatagatgagaattaagggaaagtgggtgtctaagataaaagaagtaatagttctagcatattctctaacagtattaagaagttcaattgctcactttatgaattaagtgttagaagaaacaggtggaacacaaataagatgatactttgctttatgaaaacttaatattcctctctctacaattgccctcacttctatttgggaggaaggaatggctagaaaaaaaaattgcagaaaataagaacatttttgttttatgtttttttcttaccaatttgaagataccaaagtaactaataaaatgtatttatggggtcatatggtaatatgtaatccatgaaaaattaatagtattcactaggaggctaactgaagtggttttcaatattgaatgtctctgaaactgtacataaatactgtatattttacaaacaatgacacagtgtaaaagaacatacatgtgtatctatgcctttcactatgttaggagcaaggctggagaaaatgaactaaatcagatgttgttttggaaaacaaaaggatgcatatgacaggtaagttcttttccacttatctgtaagctgccttaatcatgaagcttcatttgcttaagatgttggacatgttggtccatcacaacaatttttaaagacctccttctttagatctcattttggacgtaataaagctaagtctttcttagataatttgccatcttctttaaaagcaaaagctacaaaaaaagtctttcaattcaataacaaatatatgctcttacaattatgtattaaacaaaggtttagtttaacagaatgattatgcaatgtacagtttaaacgtatcagttttacaaaagaaattcagttaggacttacaggaccgaatcctactttggatagtattatttctaaacaactgggaagcttttggggaaaaaaaaccccaaatactttaatcttaactccatttatacatttctttccatctttccccaaaagaacatttctagagcacaaaatagattcaaaattgtttaattagatacattttatatatcctgaacataatggctcccatagaaataaactagtattttgtacacaaactttatttactgtgccacattcataatatactgggccaagtgcaaacatttattacatcccctggtgtgtgcagagctctgctcccacaaacacctcattatctaggatgacagagaacaagattagacaagatggataattaaaatccacaaggtaataacaaaaatgtactttatgattataaactcttctccagctacagctgtaaccagtactaagcaaaacagtttaatcaggttttcctccctaaatccagcccccaagccactgctccttggggcaggatctaataattgattagtggggttgctgaaaggcctagggccagaataatctagaggaaaaggtttagaaaattgacaacctggcatctcatatattgaaaatcctttggtttctcttgcccagaaaattgcattttttccccacatatagttgatatgtaccattaaaagttatcttaaataaggtttatttttacaattgcctgaaaattatggggtaggtattttaaaaataatccatgaaaaacaatggcttaatttaagaaaaacaataaaataacagcaaaagagagtaaatctgcaccctgggtgacagcatatggaatcgatgagcttctggtcagcctctaccagtgctggtgtgtgccattgatccgctcagtctagccaagtcctcagaatcatcgtcacttattactgctctcctcaatgaccatctccaatgagatgaagcagcttatgaataaaccatgggagaagtatacaggcatattatgttctcctctatcctagatccttttaggaaaaaacaagaaagtaggcctgaaataaaaaggtttgtataacatcctaaggaataaatcaggtcttattaagagaatgatctaatattctacccttttgctatttagtcttgacagcccaaatactacgtagatgaaaattccaatagagtaagtctcttcattttataaccaccatgtcaataaaaagtaaaaaaggggatgaggccatcgcaccaatgaatattccacaggagatatgatattagtgaattgggtattataggaatagtaactaaaacttaactgaacacttgaattggaataatcagactatctgaatcccaaaagagattctaaatctgagatattatcaaatgtagtgattttaatagacatttttctcattctcatcttgaagtcctcatcagagtgtcaggctacctctgaccaacattcactcacctgatttgtaccatgaccttactgtctggtaaagatcctttctactattttttcttttttgtaattataacccaaattgctaagtacagtcgttgcttccctgatgggtcctggatcctcttccagctacctgataccacatctgatggtcagctgctgctccctttccttcatctctgcttgtaaaaacctttactttgcaggattgttttcttatgtttaggctattttgagactgttcagggaagtgctagtaagtacagaccagaaccactttaaatagtatttaaagctttatcaaccataggagaacagactcccgtgaggaagtcaataggattcttattaaaattaacgacatgtatctcaggatgcagaaaaagaacatcaagatgaatgagcagaaaaagaatcaatatcaaggggaagattttactgccgcagggcaagccacctatggatttaaaatgggaatgagaggaatagagagggtattgttgaagcagaatgcttagatctggtgatggattcgaaaatttacctgagaatgaaattccattctaagctaatgcagactgtacacataacataaaaactcagatgcaagggaggagttttggataaataaaatattgcgccatctagtggaaacgttagcgctttctcttacactctcatcagcagtttttcatttgatggtgtattagccattattaggaatgctttgctgaggagaaataccactaaaatcaacacctcataataaaatgtaaagtgtctgtaactgtatcagagttttaaataacacttaaattctaatggtaagaatccaagaataaacatctaactaacaataaaatatatgtaattttataattccctaggaaaatctctgaggagatattttaaaaaaaacatacaggcatttatatagtcacctacgtgcagaaacaggaatactgatgcaagttttctgcaaaagcctctgtatattagtggaggaaaaacaaatcctgaagtatgcaaaacacacttctgctttcctgctttgggatggatacattccttagcttaagtttcatatctctgccaatagcaaggtaaatgcttaatatgtagccatgtaccatatggaatcacttgatgaaaatttgaaatatgattttgcatagaattcatttaaacaatgcaaataaactactattattcttgcttctgttctcagtggaattcgactagtgtcagtggagcgggcatgggattgagacatggattacatggtgcttcactcaaaaacaattacatttatagtactactaagcccacacaggaattccatatgctttttgttatttccttttaaggttttaacactgatgaccaaatgtccaaatcaaagacagatttttccaaataatagggcacactgtgaggttaggtggaagagggatggtttattatctggacgcaggacaggaaattaacgagccacgtaaatacagagatctacttagcacgtcttttccttctttcccttcagacataccatatggtaactgacttatcagagtaaagcacgtgttgttcacttttaaaaaacccatttaagttagtctcataattgtcctgattgagaaagtgaatcatgccatgattcaaaaaatctgttcttcacataaacctatgagcacacattttaaaaatgatttattgtacatctttgcatttcttaaggcatgaacaatggcatacagatggaacaggttctgagaagcatcacatctttttcgacaaggccagcacaatcacaccacatcaaacagacacacttgaagtctgcactgaccgactgcttgtggcccaggagtcctgcgataggggatggtgcttccagacagtggaacaatcgtgtggtttctatgttgttgttaactttcttgatcagctttaagcaccagttaccatttgtttttctttacaaactggtcagactttggattttatattctgctccttttattctgctttccaaggacggtgtggattttttttttttttttttttttttttttaaggaatatggttgcagcaaaacagaaaggatcccaaagtggttaggggccttgtctaatgcacttctgaaagtccattataaagatgaatagaaaagcaaatggtaggttttcagttgacccagaaaccacacatagctataagaaacataattgtgcatagttatttattcattcagaatgtgatatgttggctagctctacattcccagtctaccaaagaacagggctgtctactttgctaaacccagggtcctttcgaagctcccagtaggtgtcgttagaaacccaggcttctctttgattggcatcaataacttttttaaaaaattttggtatatgttcaagattgttttcttccatatatcgtctccgagatctctggagttcctctactctttgcttctctgatgctgcagcttctaaatttccttcttccaaaaatctttgatctggccggaaccgggcgtctgttggtggaaggagatcttttagtactggatctaactcattgagctcaatagcaaaccttgtgaagccatagtacagctcatagtttgttggcatggaacctggtctccaaatgcactttgcagagggggccacaccacagtagagtccttcatgccactttccaaacagccggtacaccgccttcccctcctgatctatcaccaccccctggacttcattcatgttagaattccaataattcaccttgacaaatgtgagtttgcaaatgcaaacactgcttttggtatttctgatggttacttctccataatgttctatccatcttctcccactgaggatgttgtgtatgcaagtggtgactttattccacacatagtaatctccatactttggaagcatgacattcagtgttccaacaggcaggatttccatcgacttcccccagaacttgtttttccatctgatatcttgccaaaacacaaaattctttgattcacagtgacaggcagaaatgggtggatgatggctaacctgttctgagaaaaagcggaatcccttgtcttctctaatgcattcataagtctccccaaggactgggttgaatggcttacttcctgctctgaaataggtggagcagtatcctgaaactgcaaatgcggcaacgagaaccatgcgctcatatggatcatcagtttccgaagccttgtccaggagctcgctgtattccatttcctcacagaggtgctgcagggtgttgagcggctcgtttagctccacaggcatagagactttagacaggtctttaccaatgttgttcctcaagatattccacaggttaatgttactggtgtcaggacaaggagctggcaggcatgctcgacgcccatttcggaaggcccctcctgtaagctccccattcaggatttgccgagaaatattgtctgcaacactggtgttgtcttcagatatattatcactcacatcactgatgtaagactcatcatctgaagcctcattctctgacgaacttgcagagaggagcacctcttgggcatcaaagaactcagaaacagactctgacatggagaggcggctctcattggctacttgctgtgataaggggagactgacatggatttgctcaccagcctcatcagggctaggaataatatttacactgacaacctgatcacaaataatagactctgaatgtattctgttcaaccgactccttagttcagcattctggttgagtgcctgagacagtgactgtcggagccgtgccatctgcgtgctgtggcctttactgtgatcctgctcggaaaccatctgcttcagcttctccttctctatagctatgctattaaatgcagacttcaaaagagaatgcactttctgtgcgattagacaaaattcttcttgcagctttgtataatctgttgaactttccagagggtcagtgaggtggctagggggagtctgaaattcaatatctgcacaaaggttggggttggaggaatgcaagcgaactggtgacatggtagcactgaaaggaactgttgtagccactgctgccgctagcctctgccggcgccgagttgtgctgaactggcccttcgcgggtggcccttcctgcagttgtatttttgtatctttgctgacactttttgttctccatcgtcttgtgacccgcttgtctttctttgaaatatctacacagttagcctgcatgtcagtaaagttaggtgccgactgagttctctgaagtatttccaaattttgcaggagtttgctaagttccacaaggtttgactggcaatgtgcaagatcttctgcacacctgtccatctcttccgagtcctgtaaccaggctgccactttactctggccagttgtgcacgttgcagggaggctattgctgcatggtaaaggggactgccacggaaagctgtttggttgcatctttccatccattacagaaacattagcagctggtgaggattcagctgtggacgttgaaggaaatatgtgaaaactagcatctcttggtgatctcacaatttcattctgacgatacaaccgatgatgtcgcagtttggagacccatgcatcaaaccagtcctgggatttcaccttcaaatgatagatgtgctcttcggtgtcaaggtctattcttcgagctttctttttaattgacatgactgagagtcccacatctatgctcccatggacctttcctttctgaatatcgagtggtgcctttgaatactttaacattccattatccaggacaaaaaaacgcttgtgccagccttttaaaggccattttcttttcttcagcataaagccctcatgtttgtctggtttctggacattggtttggcctattttcagcccttctataatttcccagctgtcagcttccttggagagggggactggctccggttctagcaattgccgacttacagagggctcggtgctagaggaagcagtcctctccagtatgtgaatactctgcctactgtccctttgggaggatgttgaagaggaggcacttctatgggttggagtggatgttttatgagcaggggaaatgcccttctcatctgaactcatcgctgcagttagagtctcgttttatgcacttaagaccatcccaatcttctctcaaatccacaaacaaagaagtagatgatttttcagcttcattccatttcatgaatcaggtttgactagaaaagagcaggcaatattgagggtgtccaaaccaccttgcaccttggagtcaaagtcttccaagtcagctttatggtcaaagctgtttcacagtgatttatcctcagatgcctgcagcttttctccttgggacatgatatgtctttgaccttgctggggctatctgggtaaattataggggtggctccttaatatccttctgttgctgttttcccagcaagtggcagaacctggagggcgagcggtggcgccgcggactctgcggcggctgcgcggctgcgacgggaggcaggaggcggagagccggccccggcaggcggactggcgcgcgggctagtggaggagaggaggcatgggcgccgcctgcaccgagccgcgatctccagcaccgac

SEQ ID NO: 11516 - RNA, 9652 nt, Homo sapiens
  source 1..9652: mol_type = other RNA
ctgaatagctgggactacaggtgcgcaccaccatgcccggctcagtttccggttcttgaactagactttcctactgagtgtcacatgaaaaaaaacaaacaaaaaagactgaggcacagggacaaaggaaagagtatttagctggcacactctcaccttagttctccatctaccttaaaatgtcccgggggcagagggtgcttgttacaatgaggattctcggtccacaccctagatctgtggactcagaatctttggagggaaactcaggaatcagcctgtaaacaaatatccaagatgattttcgtggcccacctgggatccaaccatatgcccccaagaagcaagatccctgccccagttagagaacctacttttttccccagattccatttctcttgtattcattcttgccttgtttcttcattagcatttcatgttaaccattttgtatgtgatcttgtctggaaagttttctacttttgagcaaacttttaggctccggatataaggaataaggcttttaggctcaggatgtaaggaataagctttcaacttgcacaactgccagtaagttcactggacactttcatttccattgctttttcaaaactaggtttagtaactttgtttccagatggggagagaggatattagcagaattggaaaagcagcattcttgagcactgggtgtttcaaatgtttgtgacacaaaagtggggttggggtggggggatgataaataaatcagcataggctacttccctgatcatcatcatcaaaatatcatttcaagagcagtcattctggataccgacggctttgtcagtgagtctttcattacacagaagagaaaaacacttcccagggtttcctcagcgccaccaccaagtggtgttacatcaccagaagcatggaaattaatccattaatttacttggacattttgacataaaaaaataaatgattgttttctaagcatttcaaatctaaattttttaaataattttttttcatttttgggggaaaatctaaaatttgtaccgggctaccagaactaggacttaatgggattctttctgttacaacatgttactacttgatggcggatactggggtaatggaaggggagggtgcatatgcacgtggccttctagaaaaatcccatatgcaatacatataagaaaatacgctaacttttaaaaataataaaagcagatcaatggttgcctcaggatagaggatggggaaggattacaaaggggcaggggaaacttttggggatgatagatatgttcactattttgattatgtcaagggtatatacatacatcaaactgtatcaagtactgttcaaatatgcgaagtgtattatatgtcggttataccttaatcaagctttaaaaagaacttgagtccaggcgcggttgctcacacctgtaatcccagcactttggggggctgaggcgggtgaaacacttgaggtcaggagttcgagaccagcctggccaacatggcaaaacccccgtctctaactaaaatacaaaaattagctaggtgggtggcacacgcctgtaaacccagctactcgggaggctgaggcacaagaatcccttgaacctgggaggcggaggctgcagtgagccgagattgtgccattgcgctccagcctgggtgacagagcactcaagactctgtctcaaaaaaaaaaaaaaaagtacagcaatatcaataaaattaacaaaaaaagaacttgaaaagacaaaaaaattctagcaacaattttattaaaaaactaaatagatgagaattaagggaaagtgggtgtctaagataaaagaagtaatagttctagcatattctctaacagtattaagaagttcaattgctcactttatgaattaagtgttagaagaaacaggtggaacacaaataagatgatactttgctttatgaaaacttaatattcctctctctacaattgccctcacttctatttgggaggaaggaatggctagaaaaaaaaattgcagaaaataagaacatttttgttttatgtttttttcttaccaatttgaagataccaaagtaactaataaaatgtatttatggggtcatatggtaatatgtaatccatgaaaaattaatagtattcactaggaggctaactgaagtggttttcaatattgaatgtctctgaaactgtacataaatactgtatattttacaaacaatgacacagtgtaaaagaacatacatgtgtatctatgcctttcactatgttaggagcaaggctggagaaaatgaactaaatcagatgttgttttggaaaacaaaaggatgcatatgacaggtaagttcttttccacttatctgtaagctgccttaatcatgaagcttcatttgcttaagatgttggacatgttggtccatcacaacaatttttaaagacctccttctttagatctcattttggacgtaataaagctaagtctttcttagataatttgccatcttctttaaaagcaaaagctacaaaaaaagtctttcaattcaataacaaatatatgctcttacaattatgtattaaacaaaggtttagtttaacagaatgattatgcaatgtacagtttaaacgtatcagttttacaaaagaaattcagttaggacttacaggaccgaatcctactttggatagtattatttctaaacaactgggaagcttttggggaaaaaaaaccccaaatactttaatcttaactccatttatacatttctttccatctttccccaaaagaacatttctagagcacaaaatagattcaaaattgtttaattagatacattttatatatcctgaacataatggctcccatagaaataaactagtattttgtacacaaactttatttactgtgccacattcataatatactgggccaagtgcaaacatttattacatcccctggtgtgtgcagagctctgctcccacaaacacctcattatctaggatgacagagaacaagattagacaagatggataattaaaatccacaaggtaataacaaaaatgtactttatgattataaactcttctccagctacagctgtaaccagtactaagcaaaacagtttaatcaggttttcctccctaaatccagcccccaagccactgctccttggggcaggatctaataattgattagtggggttgctgaaaggcctagggccagaataatctagaggaaaaggtttagaaaattgacaacctggcatctcatatattgaaaatcctttggtttctcttgcccagaaaattgcattttttccccacatatagttgatatgtaccattaaaagttatcttaaataaggtttatttttacaattgcctgaaaattatggggtaggtattttaaaaataatccatgaaaaacaatggcttaatttaagaaaaacaataaaataacagcaaaagagagtaaatctgcaccctgggtgacagcatatggaatcgatgagcttctggtcagcctctaccagtgctggtgtgtgccattgatccgctcagtctagccaagtcctcagaatcatcgtcacttattactgctctcctcaatgaccatctccaatgagatgaagcagcttatgaataaaccatgggagaagtatacaggcatattatgttctcctctatcctagatccttttaggaaaaaacaagaaagtaggcctgaaataaaaaggtttgtataacatcctaaggaataaatcaggtcttattaagagaatgatctaatattctacccttttgctatttagtcttgacagcccaaatactacgtagatgaaaattccaatagagtaagtctcttcattttataaccaccatgtcaataaaaagtaaaaaaggggatgaggccatcgcaccaatgaatattccacaggagatatgatattagtgaattgggtattataggaatagtaactaaaacttaactgaacacttgaattggaataatcagactatctgaatcccaaaagagattctaaatctgagatattatcaaatgtagtgattttaatagacatttttctcattctcatcttgaagtcctcatcagagtgtcaggctacctctgaccaacattcactcacctgatttgtaccatgaccttactgtctggtaaagatcctttctactattttttcttttttgtaattataacccaaattgctaagtacagtcgttgcttccctgatgggtcctggatcctcttccagctacctgataccacatctgatggtcagctgctgctccctttccttcatctctgcttgtaaaaacctttactttgcaggattgttttcttatgtttaggctattttgagactgttcagggaagtgctagtaagtacagaccagaaccactttaaatagtatttaaagctttatcaaccataggagaacagactcccgtgaggaagtcaataggattcttattaaaattaacgacatgtatctcaggatgcagaaaaagaacatcaagatgaatgagcagaaaaagaatcaatatcaaggggaagattttactgccgcagggcaagccacctatggatttaaaatgggaatgagaggaatagagagggtattgttgaagcagaatgcttagatctggtgatggattcgaaaatttacctgagaatgaaattccattctaagctaatgcagactgtacacataacataaaaactcagatgcaagggaggagttttggataaataaaatattgcgccatctagtggaaacgttagcgctttctcttacactctcatcagcagtttttcatttgatggtgtattagccattattaggaatgctttgctgaggagaaataccactaaaatcaacacctcataataaaatgtaaagtgtctgtaactgtatcagagttttaaataacacttaaattctaatggtaagaatccaagaataaacatctaactaacaataaaatatatgtaattttataattccctaggaaaatctctgaggagatattttaaaaaaaacatacaggcatttatatagtcacctacgtgcagaaacaggaatactgatgcaagttttctgcaaaagcctctgtatattagtggaggaaaaacaaatcctgaagtatgcaaaacacacttctgctttcctgctttgggatggatacattccttagcttaagtttcatatctctgccaatagcaaggtaaatgcttaatatgtagccatgtaccatatggaatcacttgatgaaaatttgaaatatgattttgcatagaattcatttaaacaatgcaaataaactactattattcttgcttctgttctcagtggaattcgactagtgtcagtggagcgggcatgggattgagacatggattacatggtgcttcactcaaaaacaattacatttatagtactactaagcccacacaggaattccatatgctttttgttatttccttttaaggttttaacactgatgaccaaatgtccaaatcaaagacagatttttccaaataatagggcacactgtgaggttaggtggaagagggatggtttattatctggacgcaggacaggaaattaacgagccacgtaaatacagagatctacttagcacgtcttttccttctttcccttcagacataccatatggtaactgacttatcagagtaaagcacgtgttgttcacttttaaaaaacccatttaagttagtctcataattgtcctgattgagaaagtgaatcatgccatgattcaaaaaatctgttcttcacataaacctatgagcacacattttaaaaatgatttattgtacatctttgcatttcttaaggcatgaacaatggcatacagatggaacaggttctgagaagcatcacatctttttcgacaaggccagcacaatcacaccacatcaaacagacacacttgaagtctgcactgaccgactgcttgtggcccaggagtcctgcgataggggatggtgcttccagacagtggaacaatcgtgtggtttctatgttgttgttaactttcttgatcagctttaagcaccagttaccatttgtttttctttacaaactggtcagactttggattttatattctgctccttttattctgctttccaaggacggtgtggattttttttttttttttttttttttttttaaggaatatggttgcagcaaaacagaaaggatcccaaagtggttaggggccttgtctaatgcacttctgaaagtccattataaagatgaatagaaaagcaaatggtaggttttcagttgacccagaaaccacacatagctataagaaacataattgtgcatagttatttattcattcagaatgtgatatgttggctagctctacattcccagtctaccaaagaacagggctgtctactttgctaaacccagggtcctttcgaagctcccagtaggtgtcgttagaaacccaggcttctctttgattggcatcaataacttttttaaaaaattttggtatatgttcaagattgttttcttccatatatcgtctccgagatctctggagttcctctactctttgcttctctgatgctgcagcttctaaatttccttcttccaaaaatctttgatctggccggaaccgggcgtctgttggtggaaggagatcttttagtactggatctaactcattgagctcaatagcaaaccttgtgaagccatagtacagctcatagtttgttggcatggaacctggtctccaaatgcactttgcagagggggccacaccacagtagagtccttcatgccactttccaaacagccggtacaccgccttcccctcctgatctatcaccaccccctggacttcattcatgttagaattccaataattcaccttgacaaatgtgagtttgcaaatgcaaacactgcttttggtatttctgatggttacttctccataatgttctatccatcttctcccactgaggatgttgtgtatgcaagtggtgactttattccacacatagtaatctccatactttggaagcatgacattcagtgttccaacaggcaggatttccatcgacttcccccagaacttgtttttccatctgatatcttgccaaaacacaaaattctttgattcacagtgacaggcagaaatgggtggatgatggctaacctgttctgagaaaaagcggaatcccttgtcttctctaatgcattcataagtctccccaaggactgggttgaatggcttacttcctgctctgaaataggtggagcagtatcctgaaactgcaaatgcggcaacgagaaccatgcgctcatatggatcatcagtttccgaagccttgtccaggagctcgctgtattccatttcctcacagaggtgctgcagggtgttgagcggctcgtttagctccacaggcatagagactttagacaggtctttaccaatgttgttcctcaagatattccacaggttaatgttactggtgtcaggacaaggagctggcaggcatgctcgacgcccatttcggaaggcccctcctgtaagctccccattcaggatttgccgagaaatattgtctgcaacactggtgttgtcttcagatatattatcactcacatcactgatgtaagactcatcatctgaagcctcattctctgacgaacttgcagagaggagcacctcttgggcatcaaagaactcagaaacagactctgacatggagaggcggctctcattggctacttgctgtgataaggggagactgacatggatttgctcaccagcctgagacagtgactgtcggagccgtgccatctgcgtgctgtggcctttactgtgatcctgctcggaaaccatctgcttcagcttctccttctctatagctatgctattaaatgcagacttcaaaagagaatgcactttctgtgcgattagacaaaattcttcttgcagctttgtataatctgttgaactttccagagggtcagtgaggtggctagggggagtctgaaattcaatatctgcacaaaggttggggttggaggaatgcaagcgaactggtgacatggtagcactgaaaggaacctgcagttgtatttttgtatctttgctgacactttttgttctccatcgtcttgtgacccgcttgtctttctttgaaatatctacacagttagcctgcatgtcagtaaagttaggtgccgactgagttctctgaagtatttccaaattttgcaggagtttgctaagttccacaaggtttgactggcaatgtgcaagatcttctgcacacctgtccatctcttccgagtcctgtaaccaggctgccactttactctggccagttgtgcacgttgcagggaggctattgctgcatggtaaaggggactgccacggaaagctgtttggttgcatctttccatccattacagaaacattagcagctggtgaggattcagctgtggacgttgaaggaaatatgtgaaaactagcatctcttggtgatctcacaatttcattctgacgatacaaccgatgatgtcgcagtttggagacccatgcatcaaaccagtcctgggatttcaccttcaaatgatagatgtgctcttcggtgtcaaggtctattcttcgagctttctttttaattgacatgactgagagtcccacatctatgctcccatggacctttcctttctgaatatcgagtggtgcctttgaatactttaacattccattatccaggacaaaaaaacgcttgtgccagccttttaaaggccattttcttttcttcagcataaagccctcatgtttgtctggtttctggacattggtttggcctattttcagcccttctataatttcccagctgtcagcttccttggagagggggactggctccggttctagcaattgccgacttacagagggctcggtgctagaggaagcagtcctctccagtatgtgaatactctgcctactgtccctttgggaggatgttgaagaggaggcacttctatgggttggagtggatgttttatgagcaggggaaatgcccttctcatctgaactcatcgctgcagttagagtctcgttttatgcacttaagaccatcccaatcttctctcaaatccacaaacaaagaagtagatgatttttcagcttcattccatttcatgaatcaggtttgactagaaaagagcaggcaatattgagggtgtccaaaccaccttgcaccttggagtcaaagtcttccaagtcagctttatggtcaaagctgtttcacagtgatttatcctcagatgcctgcagcttttctccttgggacatgatatgtctttgaccttgctggggctatctgggtaaattataggggtggctccttaatatccttctgttgctgttttcccagcaagtggcagaacctggagggcgagcggtggcgccgcggactctgcggcggctgcgcggctgcgacgggaggcaggaggcggagagccggccccggcaggcggactggcgcgcgggctagtggaggagaggaggcatgggcgccgcctgcaccgagccgcgatctccagcaccgac

SEQ ID NO: 11517 - RNA, 3401 nt, Homo sapiens
  source 1..3401: mol_type = other RNA
ctgaatagctgggactacaggtgcgcaccaccatgcctggctaatttttgtatttttagtaggcagggttttgccacactggccaggctggtctcgaactcctgacctcaggtgacctgcccaccctggcctctcaaagtgctgggattagaggcgtgagccactgcgcctggccaagattcattttaattgtgtatttttctttaacccaatatttccaatgttaacatttcaacatgtaatcaatacaaaaaattaggagatatttaaccttttattgtcctttagagcacatctcaatttggactaaccatatttcaaatgctcaacagctacatatgggtagtggctactgcactggacatcgaagttctagaactctctcttacaaatgaacactatcactgtcgttgaaaactttcttgagatagtttattttatacaaacaaactgtatttcttattattcctgaaatatctcatattggcatcctgccatttcattgtagtgcctatcatttttccattgatactgataaagttgcctaagacacaacttcctacatagaggaaataagaggaacaaaccccttttggacagaatctattaaaactcattccactatccctatgtacataaataacattgcctctgctgagtggaatttgcattcgttacttcaaaattcagactcatctacctttccaagttagacagttggggaaagaacttcctaaatcttaaggttgaaggcagagggctcaaccccactccagattcaggcaaggggaataggaaagaaagtgcgagataagagcatggtggcctcttggggtcccttgatgggggctgttgggaagtggaaggcattcttttaaggggataagaagcaaatggaagacttgctccaactctagagttttcagagagttagaggaggtggagagatttactcctgccatggatcatatgcatttctaccatcaactcctggttttgcagtatttttataaatggagtttggaccttggtgacactcagcctctcttccccttttcctatgttgctcaatcttcctttccctcctaggttcttacacatttcaaacccttgccaataacagtattttagttatcaggtctcaccattccctctggttgttgagcctttggataaaaatccacatggctatggagtgggttttgttggaaaaagtgaccgtcctctaactgcacctctatttctggctcctcaaacagcaaagggtaataataaggcatggtagaggttttcccatttttcagtgactagactgtgaatatttacagatgaattttctattattaatgttattgtggttgttttaaaataaaagttctgaatgtatatatgaccaaaacaaacaaacaaaaagagcacagtgaactcaaatcatattccattacaatagtcccaggacttcattagacagactcccagtaattaagcctccaatcttaaaatgttaaacatttcaacatgtattgactaattcctgtaaaatacagaaagtgcaacatcaccaaacgtgcatttcccaggattcattttagaattctcatgaaaatttaataatagtatttcagttaattatggcatttgagaaaaagatactaatggggaaagatcacatacatgctttgggtgatacgttaaaaaaacctacaataattagtagtattgccttaacatttctaaaatcacataaaaatgatcatctttgattgccatttcagtaattttgaatacagggtatgttattttctgctcactagtaatcaaaacacataaaacagacttgtaacaaatattcagagtcgattattttcataagctaaacagttccgatactttaagatttgtgtttgagcatacagtactgcaatgttggctacataaaataaaaaaatctttttaagaggaagctcaataatcagaggctgtattgcatttaaggatttaacactggctatatacaaaagggaaagcatttcaatgagaaatacttcacgttaccaagttctctcctttaatatggcaacattcagcagcttatgctactcttttatcctttggttcccagtgacaaacaatgcagtaataatgcctctggttttagttcctcttggatgacatttattagcagagagagagacctgatgctttagctgaaatttggcagcccaagaagtgcaccaactgctccaaagtaaccctcatgttctagaaacaatgcttttagttgaccttttgaccagtaatccagtgcatatgccaaaagtttcattgagagggtattgacacgtaaaaagtttccaacaaagacaactctgtttattttctcattaacagcacacattcgtgccacagaaccaatgttattggtgatagtaactaaagtagctcttgccagatcttctttactaacagattctcgcttctccttataaatcatattcccaaaactagatgctacagcccaacctggcaaaccaaatctttcataatctcctccataaatatcacggaccagcttgtcagcttgtgtgctatcacctttggatgccatttcaagagcctcttcaaaactttcacagccagtcaataaactgcataaacccagaaaggtaccccctccaaggcttgtcccagtcactcgtttatagttgtctttggaatggactgctaaaatactgactcctgagccaatgttcactacaagcagtggatagggatcatccaggttaaaaggcatcttttggcatcgctcaggttctgaggcattagcaaaataatagcactcggcttgtccattgaaactgacagagtctatatacagcaagccctttacaaggcagtcaagttcatccagtttgtgcaggtggaggtttccaattgtgcgaaaatctttttcaaacttgtaagcaccacctcctgtagcacatagcaccgtctgcaatgttgagaagtttttatctcttcccatttggataaaagtaggcaggtcctgggttggaaacctgataaagtgcaagttccctcttcggccaaaaagtgttaaatctttcagttcaaggtgtacatcccgaatgccggtggatccatatgccacgttagaagtcaaatatttccgaatactttttaaactctcaacttcttcttgctcttcctctgctgtgatatcaataggttcaaagtacgagagctttactagagttcccccaatgtccatgccaaaccatgggaaagagggtttcttggcatctttgatcttcatggcgtcggcccgaggggcgatggacggcctccgatccggggcactgagagcagaggcggcgactccggaggtggctgggccgcgc

SEQ ID NO: 11518 - RNA, 573 nt, Homo sapiens
  source 1..573: mol_type = other RNA
ctgaatagctgggactacaggtgcgcatcaccacactggattcatttttaaattttttgtagagataggtcctcgatatgctgcccaagctgctctcaaagtccttggctcaagcgatcttcccaccttggcttctcaaagtgttgggattacaggcgtgagccactaagccctggctcccttagcagtttccaaacccaccctgtggttttcccaatacctgcagaaccagctttaaagtgaccacagcagagatgccagtgcagatgctggagcctttcctcagaagtctgagtttcaattatgcagagggctcttcctccaacttctaagctttagtggttcaacttcttcctttgttctctcagcccgagtgggtagctgcttcttgcagttactaacttaagtgatactgcagatttgtttttttgacttttcagttatctagttaataaccataaacctagttaacagttctctgtattacattgtctctgttaaataattggtatagtttctgtcccctgactgatgtatctttataagcttaattctctattacgatacatttgt

SEQ ID NO: 11519 - RNA, 2018 nt, Homo sapiens
  source 1..2018: mol_type = other RNA
ctgaatagctgggactacaggtgcgccaccacacccagctaattttttgtatccttagtagagatggggtttcaccatgttgcccaggctggtcttaactcctgaattcaagtgatccacctgccttggcctcagcctcccaaagtgcttagattacaggtgtgagccactacacccagcctctttcaggacaactttatatgcagtctactggcatgcctaggtgaaaataaactaaatgactgaaaatgttagtattttgacccttataaattcaaaaggcagagagagcattttggatgggacagatggcaattgaaaataagcttgtttaccttgtgagagtctttccccctggggactgataagttgtggcttctgggtcattgcattccaacactgaggcttccctggcaacacccctagtccaaggtaaccaggatagagctctggaaaccactccagccccatgcagctgcgaagagtcttcctgccagcagctgcagcatgattggtgaaggggctctgaggagtgtgacgctgggctgaacataaagggctctggcacccagtgtgtgatgcttggaactgactatcagatttgggctccagagataactgtccctcgggactctccattaatgcctttacatcagggacacaatgatgattctgggcttctgctttcttttcttgaagaaatgttgtagctagagaggcaagactttgactacttgactgcgatacagaatgaaactggtaagtcgtctccctcggaatgaacaaacttaaatgtggtctttccccttgagactcctttcctgtgactgaatccctggtgttgaagttctcacagccatggctcatgacagtccgttcctgcttttctgttgcagacatacttttctctgcatttcctttgctcccacacgtctctactcccagggtaagtcctttctcttgtttctccatgacttggattttacctaatgagctcattttaaggcttaaaatgagggattctgtgttcttttctggagtctcagtaactgtaacatcagtagggactcctgagaggtgatccctgcctttggaatctctctcattgcttaataatgttcttacccttttaaccccatcactgacattctttggagaaatatgacaatcaccagtaggcacatctagtaattttactagaagttcctgtctttggggatcaattttgtccaatttgagatcaccagaggtagtttgtacatcattaggtagagttgaggaatattttctatcttgatttgacaaagaaggttctattgagccaaccagtaaagacgctccagcttctgaaggattacatcgactttctcctgatttaggcaaatctttggcaagttctcttttaggagaggttttctctgatgcgtaaaactgagccttggtttcttcttggaaagtagtcattggtttagtattttttaacattttgaaggatggttggattggattcttgatgtctttatctgcctttgtagtagctgctctttccaaaccaacagctggcagtggaaaggtcttcactgtctgttctggtttgtccaccaccaacttagaatttctttcttcattctctgtctctaactctttccctttagctttaattaaatctttgattggtcctttcatctttttagcacgtgggagtgtagctggcttggactgataaactttttgatcagtaggtatggttggtcctatcatcttacagtatggcaagtgggattttaatcgtttaaatggcttcttacagtaaggacacacttccattctgggtggattatcactcatcctattcccgagctcctccaggaggatgctagttttgtgggtgcttctcccggatccccatgcttccccgatcaccgttcccgagtgtggcagaatgaaacgtgaatgtcagccctccgttggctgtgaacaggcgagcgcttctgccaccccaggggaggtcctttctc

SEQ ID NO: 11520 - RNA, 2018 nt, Homo sapiens
  source 1..2018: mol_type = other RNA
ctgaatagctgggactacaggtgcgccaccacacccagctaattttttgtatccttagtagagatggggtttcaccatgttgcccaggctggtcttaactcctgaattcaagtgatccacctgccttggcctcagcctcccaaagtgcttagattacaggtgtgagccactacacccagcctctttcaggacaactttatatgcagtctactggcatgcctaggtgaaaataaactaaatgactgaaaatgttagtattttgacccttataaattcaaaaggcagagagagcattttggatgggacagatggcaattgaaaataagcttgtttaccttgtgagagtctttccccctggggactgataagttgtggcttctgggtcattgcattccaacactgaggcttccctggcaacacccctagtccaaggtaaccaggatagagctctggaaaccactccagccccatgcagctgcgaagagtcttcctgccagcagctgcagcatgattggtgaaggggctctgaggagtgtgacgctgggctgaacataaagggctctggcacccagtgtgtgatgcttggaactgactatcagatttgggctccagagataactgtccctcgggactctccattaatgcctttacatcagggacacaatgatgattctgggcttctgctttcttttcttgaagaaatgttgtagctagagaggcaagactttgactacttgactgcgatacagaatgaaactggtaagtcgtctccctcggaatgaacaaacttaaatgtggtctttccccttgagactcctttcctgtgactgaatccctggtgttgaagttctcacagccatggctcatgacagtccgttcctgcttttctgttgcagacatacttttctctgcatttcctttgctcccacacgtctctactcccagggtaagtcctttctcttgtttctccatgacttggattttacctaatgagctcattttaaggcttaaaatgagggattctgtgttcttttctggagtctcagtaactgtaacatcagtagggactcctgagaggtgatccctgcctttggaatctctctcattgcttaataatgttcttacccttttaaccccatcactgacattctttggagaaatatgacaatcaccagtaggcacatctagtaattttactagaagttcctgtctttggggatcaattttgtccaatttgagatcaccagaggtagtttgtacatcattaggtagagttgaggaatattttctatcttgatttgacaaagaaggttctattgagccaaccagtaaagacgctccagcttctgaaggattacatcgactttctcctgatttaggcaaatctttggcaagttctcttttaggagaggttttctctgatgcgtaaaactgagccttggtttcttcttggaaagtagtcattggtttagtattttttaacattttgaaggatggttggattggattcttgatgtctttatctgcctttgtagtagctgctctttccaaaccaacagctggcagtggaaaggtcttcactgtctgttctggtttgtccaccaccaacttagaatttctttcttcattctctgtctctaactctttccctttagctttaattaaatctttgattggtcctttcatctttttagcacgtgggagtgtagctggcttggactgataaactttttgatcagtaggtatggttggtcctatcatcttacagtatggcaagtgggattttaatcgtttaaatggcttcttacagtaaggacacacttccattctgggtggattatcactcatcctattcccgagctcctccaggaggatgctagttttgtgggtgcttctcccggatccccatgcttccccgatcaccgttcccgagtgtggcagaatgaaacgtgaatgtcagcctcggaagacctgaaagcccaggcggccccggcgacaagccccccagggaagccccc

SEQ ID NO: 11521 - RNA, 4004 nt, Homo sapiens
  source 1..4004: mol_type = other RNA
ctgaatagctgggactacaggtgcgcgccaccacacccagctaatttttgtatttttagtagagatggggtttcaccatgttggccagcctggtctcgaactcctgacctcaggtgatccacctgtctcggtctcccaaagtgctgggattataggcgtgagccaccgtacccagccacttttgtcatcttgtgttggctttggcagcgacaccattcactggggtgggaattcgggacagggtcttgcccctgtgcccgggatttgacatttgggaaacaaatgttaaaaccctaccatgtccctaaatgtcccagcctccccagggcaatgctgagacccagaggtgtcccgtcacagccggtggctccacaggaacctgcaggcataagcctgctcagaaaccccgtcttcctcatggcaggagctgctggcttttggggatgggactcgcgcaggaccctgtcccacagggcaaatctttctgtatcactgcccctcagcactaaataccaccagttccctgccatcatcgttggaataaccccaaatgcaattccttgctgtctcaggtcaagatgcactggacgctttcactgaggctcagttaattgtgggtctggttggcccagcctggatagcacttgctgagaggtcaaccacagagctaggaagaagggcctggagaatgtgcccgccctactcaccgtctgctcagactgatagacatgaagacatttaggattagagggaaactcgtgagcaactctctgcaaacactgtccattcttttcttttctttttattttgagacggagttttgctcttgttgcccaggctggagtgcagtggcatgatcttggatcactgcaacctctgcctcctgggttcaagcagttctcctgcctcagcctcccgagtagctgggattacaggcatgcaccaccatgcccggctaatttttgtatttttattagagacggggtttcgccatgttcaccaggctggtcttgaactcctgacctcaggtgatccacccacctcagcctcccagagtgctgggattacaggcatgagccactgtgccctgattattttttattttttttgagacagagtcttgctctgtcgcccaggctggaatgcagtggcacgatcttggctcactgtaacctctgcctctcaggtttaagtgattctcatgcctcagcctcccaagtagctgggattacaggcacctgccaccacgcctggctaatttttgtatttttagtagagatgaggtttcaccatgttggccaggctgttctcaaactcctcacctcaggtgatccgcctgcctcggcctcccaaagtctgggattacaggcgtgagccatcgtgcctggcccagccttttcttaaatacttccagagacagggagctcagtgcttctagagtccatctgaccagtgatccgcatttggaccacattagaaaagtctgtcttctttttcctagggaaatttgcctcccgaacaagaacccgctggtccaagctttgaatgcaggtggctgcggccagcgcactggatttatcttcccgaatgacttctgaaacactcaaacgcccgataccctgtatcttcctcttgctaggtctgcctatttcagagccagtttctgagcctctgctgttccaacccggaacagcgttggcgtgtcccagcctgacgctgggttgggggagcagtgaggtccacatatctcattccttggtgggaggtattgacggggtttgcccggtggcttgacatctgagttaaaggggcttgagaatgttctagattactggggtgtcattttgcaatcggaggacaaggatggttggcagcggctcttcttgtgcaatgggctctgatcctctcaaaggagctgggtgtcattatgagcgagaagggggcgggtcaaatgaaaaaccatgggtgtgaaatttggacataaggtcggaggtcaggagctaccccaggacgtggccctcataggggggttgagcttctaggtctgaggccgcattctggagggaaaggcacaggaaaggacgcagacccagccggggtggcggtgggtgtctgtggctccaacctggagcgggtgacaagcaagagaagggtcttgaatcttgtatccagctctgaccacagaggctgcgagcaggagcggaggccaccgacgccacgcgggccaccccctgcgcttcttgccttcctcggctgagagttcgtgagtgtggaagggtgaggggctcagagctgggcccttttctggaacgcacaaatactgcatcgttaaaaaaaaaaaatacaatgttttcaagcagctgaaaaggatgctgggtttcagagatgaacggaggggctggcacccttggaagattgggactcaggatgaggcaggatgagatctggggccagtgggcgtctgacagaggttttctggcatctggaatcttcttccatgtcctttgttatgctcacgtcgcctcaggacatgcttgtttcctgatcttctgagaccagagcagacctgttttccactggtgccacctctggcttctcttcagacctgggcagcacaaactccggctggggcctcgcgctctccctcctggccttcagtctttcctcttcgtattgcaggacgcagtctgggatctggacgtgttccatagggatgagttgctccaggtcttccaagctgtgcacgtactggatcttgttgatgaacttgacgctgatgaaagggcgagagatggccagcacagtccgaatgaaccacgaggggtggacgatgatcaaggacttcaggtttttccgcaacctccggtcgatcatctggtagcacttcttcagccagccgattccaggcatcctccgccggggcgtggcaccgttcaggtacacgatcatgtagtcctcagccaccaggagctctaagctgctgatgacgtacaggaagaggttctccatgatgtagtggtagtcggggaggctgctgtctggaaggaagcaggctgcgaagacgatgatggcgttgaggccttcgccgtagtaccctccgtgggtgaccactttcatgtaaggccggatcatgtgcaggtctatacggtgctcttgctccccgatgatcactgtccgccacaggcgcccgttggcggcgctgccgtcctccgtcgtgccgtccccaaatagatccgcgctgtccccgggcatgttcttggcggtggccacgggggtgtcgtcttcccactccagttcgttgccattccccaggaactccagcgagtcggtctcatcgggggtctcgatgtcatccacgttaatatccaggtcatcaggggtatccaagaagtcatcggacagcagggacccctcactctgatccagagaaatgttgatctctggggccaccagcgtcttcctcttacgatgcgctccgttgaaatttagcgtgttgggaggagaggatgtgtcttccaccgggctgccaagcagttccacccccgtctcttctgggagtggcctgggaagatcttcgtcctgccattcctccttcacgtccacgttttccatccggagcgtggcttcggtggtccccatgggagctgggaagaggcactggcttgaagcagggatgacccctctgcagctgagacagcctctcctccttactggcaaacaaaggcgagccctgcccgggtgcagctgggcatcgctcacgctccccgggccttcagagcctaggaggaagaggatgctcgcaggggcggattctgcatccgaggaaggtcacccagggcgacgtggccagcgcccgccagctcttttgtgcaggggtgggtggggtgcagggttagcggtgggctccccagcgcggggctgcggctgcgccccctctcatcgccgcccgcctgcgcgccctgcctccgaggtagctgcttcttcccagctcagggctggcagag

SEQ ID NO: 11522 - RNA, 5814 nt, Homo sapiens
  source 1..5814: mol_type = other RNA
ctgaatagctgggactacaggtgcgcgccaccatgcacagctaatttttgtatttttagtagagacggtgtttcaccgtgttagccaggatggtctcgatctcctgacctcgtgatccgcccgtctcggcctcccaaagtgctgggattacaggcgtgagccaccgcgcccggcccaactctgttattttctaaattattttggcaattcgagttcccttgccttgccatataaattctagagtgagcttgtcaatgtgaagcaatactgaggctctcaatccatgaacatctaattgaggctcaatccaggaacatctgtttacgcctcccaacccaggaacatctgtttacgcctctcattccaggatcatctgtttacgcctcccaatccaggaatatctgtttacgtctctcaaaccatgaacatctgcttacgcctctcaatccaggaatatgggtttatgcctctcaatccatgaacatctgtttatgcctccgaatccaggaacatctgtttatgtctctcaatccaggaacatcagtttacgtctctcaaaccatgaacatctgcttacgcctctcaatccaggaatatgggtttacgcctctcaatccaggaacatcagtttacgcctctcaatccatgaacatctgtttatgcctctcaatccatgaacatctgtttacgtctctcaatccaggaacatctgtttatgcctcttgatccaggaacatctgtttatgcctcccattccaggaacatctgtttacgtctctcaatccaggaacatctgtttacgccttttacagtttctttcctcaatgttgttggtttccagcacacagatcttgggtgtattttgttagaggtacacttcagtgtctcactttcttgtattataaatgcttaaatgtattattataaatgtttacaaattttttcaaaccccaattattcattgctagtgtacagaatcaaaaatgattttgaaaaattattccttgtatcctgaaactttatgaagtttacaagtataggaggttgtatgtgtgtggattccttggaattttctacatagaaaattatagcatccacaaacagagatatttttatttcctccttcctaatctcaatgttttaaatttccttttattgtcttattcactattattttgaaaagaatataagtatacaaatatacatttcaaaagataaaaccatttgagagtattctacagaaaataaaaattagtgaaggggtccgaatggttcaatacctaatggcaccagagatttcatgaagaactgtatattacctacttgatatctttacaattagcacaactacaaatcaaatgtctctggagttagctggtaatgtaagattatgaattggtaacaaaattcacagccacagtctgagatattttgggaccacgtgagctggctcacttaaccagggtcaccttactagtcctgatgcctggatcttggagtaactagcttccctaagcggttacacaccattcagaatgaatgaagacatgtgcagagttaggagagagatgagtaggtcagtttcccgtcttactggcatccagaaaattaagtgcctgaactcatcgtgagtaaagtttaataattcaaagcagaatttgagcttcaaaagaataacaaaatagtgttgcaaatataccattttctgtaaagaataaaagctacacagttttaggaaagcgaaggaaatcctgactctttgtttaactgattcattcactgcctcatttgtttatcaaatacttacttaacagatactgtgtcgatgtgtggctcaggccatcgagacacagcaggggacaaatgtttatacttgaggttggctaactcattaggacaataagtgagatttataatgcgtgccttatttgtacttttagattataaagactggttatcaaatacacataaaaaagaggagattttctttccaattgagtcttctcctgtgtgcagggaatgcatgccttgcctccctggctcgcctctgaaggtattttataaatttacggtgacctgagatatgtgactcagaactgactggaccggcactcgccggtcagccactcacatttcagtccgcggccctttatgctgttgttactcacactgcaggccgcggccctttatgctgttgctctatgccactgattcactgctttctcatcctgactagaatacagacttgttgagagcagggctatgttgtcctacatcgcaggagcttgagccgacggactggggacttggtgtccactgacactgaccggtgtggataaactgcgttggcacatccagtctccagctgccccgatcatcagacaacaacgcagagtgctgcagtctgtgctaccttggcgaacttggtgaggtccttgtacagctccgggtagagcatcgccatctctggcttcacgtcctggtccagcactaaggagaacactgggaacatggtgtatatggtggcataccccaccatgaggaagccctgatacaaagggacggatgcgaagtagaagactgaggaaaacacagcctgcatggtggagatgataaggcccctgtgcatgacgaactggccgagtgccgccgacctcttgtagctgttccgcccgtgcaccatgagcagcctgcctatgtgccggaactgcgtgatggagaagtcggccgccagcgaggcctgtttaccctcctttccctcaatcccaatcccacagtctgctgcctgaatcatgctgacatcatttcctccatcaccgatggcgcaggtgcgtctccctgtgtgctgctgcagcagtgtcacaatgcgggccttctgggtgggtgagcagcggcagcaaaccacggcagggcactggcaggccagctccacaaattcatgctcgtagtactttagacaaacctccagagagtccccagatatgactagtgcacaatcatgcttccttcgaaatgcattcagctccaaatgtgcctctccccgactggttacctgtctgaaaatatgaatatcttgtgttctagacacgagatgtgaacttttggcaatgcaggtagctgtctcgagtttatcgcctgttagcatccatatcttgatcccggcgttgcgcagcatctccagcgtgggccgcacgtctgcctgcagctggtcctccacgccggtgaggcacagcagttccatctccctctccaggctctcgactaccgcggccaccttgagggacctgtcgtgcatgctcagcttggcttgagtgtatcggctctggggacagagggggaggcgcctgtgtgcacacgtgtacgtgctgtgtgtggactccacagagctggactgcatgggctcaaagtcctggtactgctcctctgtcaacgccttctttgcaaccacgagggtccgcagtccttcgcgagccatgtttccgcactcctcttccagccagtcattatactgcacgataggagacatggccacgtcagcgcccttcatgtagaatgtgatttctgccgtggattcatccctgacgatgacgcccatccgcttgctctcggaggtgaagggaaacagctgcagaatgcagaagctgaggacctggccactgggggtcttcagctgcatggaggtgaggtccctgctgaccagcgtgaggcccacactctctgtccactgcaccagagcgacctcatccgggctggaagcctggtaggtgcgattctcatcactgaagtcttggtcagcctctgcgaactcagtctcctcagtaacgccggcccgagactcatacacgggggtcacgttgtgacacagcacgatggctttcacggcttcatggattcgactactgacacttttcctaactttgggagctgaagattgggcttttcttagtggagttgaaccagtattgtttccaccagcttgagactgcatctgtgagtaggagtccctgacatggctctggatctcatccatcgtgtcggcgccataggacacggtgcccaggtgcagccgcttaaatatcatttcattctgggtgagggttcctgttttgtctgtcaataaatacaccaggcgcccaagttcctctgggatagtgctggtccgaacgaccgtgccagggatgttctcatctttcatcatcatccatccatacaccgctttgcccatgtccaagttcacacgcaaacttatgggaatgatgtaagaaaagaggagaaggaaccgaaaaagattgcggtaccatggacccacaaatccttgtaaggttaccataacaatggaaagagcaactaaagccaaaaatagcgctttcgtcagccgattgagttcaaggtccaacaaaccaaccttattttttggattggatgtgttcattacacttcgagtctcttttccggtataaatgacaacacctattacagtacctgatgcaacaatggtgcttgcccacaatgtattttctatgctgagactttcatgaatgggcgggtcactgtcttccctggtaaatgtgccttcgaaactgtgaatgtccatttgtggtttctgagcataaacataagcactgatagaaaaaaggtcccccagagccggcagctgttgcgtgcagctcactgccaccttcagcttccagtcagtttcaccatctagttgatcagttcgaataaaacacgaacctgctttttctgaagtcctaagaaacaccatgtccgatggaattctttgattcttttccactatgatgaggtctccaacttgtatgtctgaactcttaacttgcactttacctcttactgtaagcttgctatatagttgtgaattcacttccttgtcacgctgaaaacgccgaaattcatcaattgcttcccgtgtcatagtaacagccaagacaaatcccagaggagcccagtaggtgtagagatagcctattttcaatgctggtacaaactgtgagcaggatattactagaaaatagagattcaagaaaaacttgaattgttcatacaaaaccccaggtataaaggtaaacacattgtatttttgattttttatagaattcctgggatgtttttcttcacacttttcaggacatccaagccatactgtgcgagctttcagctctttctttcttcgacaaatatttatcagccaaccacagcaactggtacagaggaacttccagccatcacagacaaaccactccagtcctcttttcctttgcattatcctggctcgtggtaaggtgtggtaatcactttcctcattctcaaagccttcttcagacatcattagtggcatttcatccaaatgcgcagactcatcctccagctggtacctacattgaacagcaaagagtgcgtgaagcctggactcccacacgccccagccgtaggaagacactctccccattgcccaggtggtgtcagggcagaccaagtcaggagtggggacatccatccaagcctggcagtcattgtagggtacatgcacaagggtgccggatgctcgttcctgctgtgccggtcggctcccggcctgggccccgcggcgctgtagtaggccgcgcgtttgcggttggctgcggccgccgctgcgctacgcaccgggtaaagcgggatctggtccgccatgttccgaccgcccctttcccgcccctcccactttcccctcaattcgccaccttttccccgccctctcccctcagcgccaaccccggctgaggcgccgcctgcgggccttccccgcctccgccaagc

SEQ ID NO: 11523 - RNA, 5749 nt, Homo sapiens
  source 1..5749: mol_type = other RNA
ctgaatagctgggactacaggtgcgcgccaccatgcacagctaatttttgtatttttagtagagacggtgtttcaccgtgttagccaggatggtctcgatctcctgacctcgtgatccgcccgtctcggcctcccaaagtgctgggattacaggcgtgagccaccgcgcccggcccaactctgttattttctaaattattttggcaattcgagttcccttgccttgccatataaattctagagtgagcttgtcaatgtgaagcaatactgaggctctcaatccatgaacatctaattgaggctcaatccaggaacatctgtttacgcctcccaacccaggaacatctgtttacgcctctcattccaggatcatctgtttacgcctcccaatccaggaatatctgtttacgtctctcaaaccatgaacatctgcttacgcctctcaatccaggaatatgggtttatgcctctcaatccatgaacatctgtttatgcctccgaatccaggaacatctgtttatgtctctcaatccaggaacatcagtttacgtctctcaaaccatgaacatctgcttacgcctctcaatccaggaatatgggtttacgcctctcaatccaggaacatcagtttacgcctctcaatccatgaacatctgtttatgcctctcaatccatgaacatctgtttacgtctctcaatccaggaacatctgtttatgcctcttgatccaggaacatctgtttatgcctcccattccaggaacatctgtttacgtctctcaatccaggaacatctgtttacgccttttacagtttctttcctcaatgttgttggtttccagcacacagatcttgggtgtattttgttagaggtacacttcagtgtctcactttcttgtattataaatgcttaaatgtattattataaatgtttacaaattttttcaaaccccaattattcattgctagtgtacagaatcaaaaatgattttgaaaaattattccttgtatcctgaaactttatgaagtttacaagtataggaggttgtatgtgtgtggattccttggaattttctacatagaaaattatagcatccacaaacagagatatttttatttcctccttcctaatctcaatgttttaaatttccttttattgtcttattcactattattttgaaaagaatataagtatacaaatatacatttcaaaagataaaaccatttgagagtattctacagaaaataaaaattagtgaaggggtccgaatggttcaatacctaatggcaccagagatttcatgaagaactgtatattacctacttgatatctttacaattagcacaactacaaatcaaatgtctctggagttagctggtaatgtaagattatgaattggtaacaaaattcacagccacagtctgagatattttgggaccacgtgagctggctcacttaaccagggtcaccttactagtcctgatgcctggatcttggagtaactagcttccctaagcggttacacaccattcagaatgaatgaagacatgtgcagagttaggagagagatgagtaggtcagtttcccgtcttactggcatccagaaaattaagtgcctgaactcatcgtgagtaaagtttaataattcaaagcagaatttgagcttcaaaagaataacaaaatagtgttgcaaatataccattttctgtaaagaataaaagctacacagttttaggaaagcgaaggaaatcctgactctttgtttaactgattcattcactgcctcatttgtttatcaaatacttacttaacagatactgtgtcgatgtgtggctcaggccatcgagacacagcaggggacaaatgtttatacttgaggttggctaactcattaggacaataagtgagatttataatgcgtgccttatttgtacttttagattataaagactggttatcaaatacacataaaaaagaggagattttctttccaattgagtcttctcctgtgtgcagggaatgcatgccttgcctccctggctcgcctctgaaggtattttataaatttacggtgacctgagatatgtgactcagaactgactggaccggcactcgccggtcagccactcacatttcagtccgcggccctttatgctgttgttactcacactgcaggccgcggccctttatgctgttgctctatgccactgattcactgctttctcatcctgactagaatacagacttgttgagagcagggctatgttgtcctacatcgcaggagcttgagccgacggactggggacttggtgtccactgacactgaccggtgtggataaactgcgttggcacatccagtctccagctgccccgatcatcagacaacaacgcagagtgctgcagtctgtgctaccttggcgaacttggtgaggtccttgtacagctccgggtagagcatcgccatctctggcttcacgtcctggtccagcactaaggagaacactgggaacatggtgtatatggtggcatacctgcatggtggagatgataaggcccctgtgcatgacgaactggccgagtgccgccgacctcttgtagctgttccgcccgtgcaccatgagcagcctgcctatgtgccggaactgcgtgatggagaagtcggccgccagcgaggcctgtttaccctcctttccctcaatcccaatcccacagtctgctgcctgaatcatgctgacatcatttcctccatcaccgatggcgcaggtgcgtctccctgtgtgctgctgcagcagtgtcacaatgcgggccttctgggtgggtgagcagcggcagcaaaccacggcagggcactggcaggccagctccacaaattcatgctcgtagtactttagacaaacctccagagagtccccagatatgactagtgcacaatcatgcttccttcgaaatgcattcagctccaaatgtgcctctccccgactggttacctgtctgaaaatatgaatatcttgtgttctagacacgagatgtgaacttttggcaatgcaggtagctgtctcgagtttatcgcctgttagcatccatatcttgatcccggcgttgcgcagcatctccagcgtgggccgcacgtctgcctgcagctggtcctccacgccggtgaggcacagcagttccatctccctctccaggctctcgactaccgcggccaccttgagggacctgtcgtgcatgctcagcttggcttgagtgtatcggctctggggacagagggggaggcgcctgtgtgcacacgtgtacgtgctgtgtgtggactccacagagctggactgcatgggctcaaagtcctggtactgctcctctgtcaacgccttctttgcaaccacgagggtccgcagtccttcgcgagccatgtttccgcactcctcttccagccagtcattatactgcacgataggagacatggccacgtcagcgcccttcatgtagaatgtgatttctgccgtggattcatccctgacgatgacgcccatccgcttgctctcggaggtgaagggaaacagctgcagaatgcagaagctgaggacctggccactgggggtcttcagctgcatggaggtgaggtccctgctgaccagcgtgaggcccacactctctgtccactgcaccagagcgacctcatccgggctggaagcctggtaggtgcgattctcatcactgaagtcttggtcagcctctgcgaactcagtctcctcagtaacgccggcccgagactcatacacgggggtcacgttgtgacacagcacgatggctttcacggcttcatggattcgactactgacacttttcctaactttgggagctgaagattgggcttttcttagtggagttgaaccagtattgtttccaccagcttgagactgcatctgtgagtaggagtccctgacatggctctggatctcatccatcgtgtcggcgccataggacacggtgcccaggtgcagccgcttaaatatcatttcattctgggtgagggttcctgttttgtctgtcaataaatacaccaggcgcccaagttcctctgggatagtgctggtccgaacgaccgtgccagggatgttctcatctttcatcatcatccatccatacaccgctttgcccatgtccaagttcacacgcaaacttatgggaatgatgtaagaaaagaggagaaggaaccgaaaaagattgcggtaccatggacccacaaatccttgtaaggttaccataacaatggaaagagcaactaaagccaaaaatagcgctttcgtcagccgattgagttcaaggtccaacaaaccaaccttattttttggattggatgtgttcattacacttcgagtctcttttccggtataaatgacaacacctattacagtacctgatgcaacaatggtgcttgcccacaatgtattttctatgctgagactttcatgaatgggcgggtcactgtcttccctggtaaatgtgccttcgaaactgtgaatgtccatttgtggtttctgagcataaacataagcactgatagaaaaaaggtcccccagagccggcagctgttgcgtgcagctcactgccaccttcagcttccagtcagtttcaccatctagttgatcagttcgaataaaacacgaacctgctttttctgaagtcctaagaaacaccatgtccgatggaattctttgattcttttccactatgatgaggtctccaacttgtatgtctgaactcttaacttgcactttacctcttactgtaagcttgctatatagttgtgaattcacttccttgtcacgctgaaaacgccgaaattcatcaattgcttcccgtgtcatagtaacagccaagacaaatcccagaggagcccagtaggtgtagagatagcctattttcaatgctggtacaaactgtgagcaggatattactagaaaatagagattcaagaaaaacttgaattgttcatacaaaaccccaggtataaaggtaaacacattgtatttttgattttttatagaattcctgggatgtttttcttcacacttttcaggacatccaagccatactgtgcgagctttcagctctttctttcttcgacaaatatttatcagccaaccacagcaactggtacagaggaacttccagccatcacagacaaaccactccagtcctcttttcctttgcattatcctggctcgtggtaaggtgtggtaatcactttcctcattctcaaagccttcttcagacatcattagtggcatttcatccaaatgcgcagactcatcctccagctggtacctacattgaacagcaaagagtgcgtgaagcctggactcccacacgccccagccgtaggaagacactctccccattgcccaggtggtgtcagggcagaccaagtcaggagtggggacatccatccaagcctggcagtcattgtagggtacatgcacaagggtgccggatgctcgttcctgctgtgccggtcggctcccggcctgggccccgcggcgctgtagtaggccgcgcgtttgcggttggctgcggccgccgctgcgctacgcaccgggtaaagcgggatctggtccgccatgttccgaccgcccctttcccgcccctcccactttcccctcaattcgccaccttttccccgccctctcccctcagcgccaaccccggctgaggcgccgcctgcgggccttccccgcctccgccaagc

SEQ ID NO: 11524 - RNA, 5867 nt, Homo sapiens
  source 1..5867: mol_type = other RNA
ctgaatagctgggactacaggtgcgcgccaccatgcccagctcacttttgtatttttaaatagagacagggtttcaccatgatggccaggctggtcttgaattcctgaccttgtgatctgcccgccttggcctcccaaagtactgggattacaggcgtgagccaccgcacctggccgaagtattttataacatagtttaaaatccttaaattctacttaaatggctgaaatgatattagctcgtttacaaaagtttctagtgtaagctgaggttctgcaactacatgctctttcagaaggcagtccgtatcagaatgcagatgtatctgatctcgtgatgattgcaaaggaaataactaagccaatctaaatttcactctagaattagttaaagttttgattaaaaggaggagtttattttgaattaaattagtaaagagagtgagaaatctgataggagttaacatcaacacatacaccacaggctttggttgcaagtaggccatgctaacaattctactgggatctgactactttctcctggcagtatcttattcatgaaagctataacaagatgtcaataagacagcatattaaagaaaagacaaactcactatcagcaggaactcttagcagaggaggctttagacaggttggctaatgcctgtgctttgatttgtagtgagctggtaattacaaacaactgaaagtgacaaattggtttaaaggtatcctcctccaacctttgacattccatgtttctgtggaatgagtaagatgagcattatgcttactcctaggctgaacactgagtttgatgtataatgaactgatagctgttatgaacttctaaggaagatttaagttatatgtgggggttagttttcttaaaaacatggtctttaatgctacttcatgattagcaacaatagcaaagtttctaaggacttatactggccacagttgtgacaatttgagcatcgaaaagaacataatggattgaaacccattaaaactataaaaattcacaagaccaccatcacaccagaaaagggaaatctaaaaaaaaaaaaaaacactaatttgtcaccatctaataaaccagttatttactttgaagttgataattaaatgaaaataataaagcattcaacctgcccttctggtagaactgtaggtaaggatgaccaaatagctcaagtggagaagggaaagcttagttcacatagaataaccaactaacaaacggagaagaaatgaaagaactagacaaccaactcacaaactttaacaaagttaatgatttaggcaagaattaccacctaatgttaaaactcctgggtaaatggtaattcattcaatgccaaaggaataccacacagataagtctgtagtcacaaaggggaaaaatctaactggatgatcagactgtcatgctgatccagtaatcaaacttagatcaatagattagttaatggtagatcaactagatattacgttttctgaagtgatgcgatatgaagcatgtatcttatctatgatataatctagcacaaaatgttttaacttgaacctataaaggctttagatataacttccagattgcaggtagtacaggcaatataaaaacaagttaaacaacaccatgaaaaagaaactaggcaaattcacaagacaggattctacaggaccgctgccccagtctctttaacaagtcaatgtcataaaaaaggaactgtgctagattaaaatagatgtaagggactttaaaggacatgaccagttgcaatgtaaggtcatagaatgaatatcagtttgcacaaaccaactgcaaatctggggacaattggggaaatttaaatatggtctaagatcaaaaatgtgctggaatgagaaagtggagattgttgattaaagaaaaatcggttataaaacactatagatgtggtcttactttggttaaaaatgtaaatgtatatgtatggaaaaagatctggaaggatattaacagtggtaatctctgagtggtggaaatatgttttatgttcttatttttgcttgtctacttttttaaaatgtcctcaatgcatttatactgcttctataataaataaaaggttattttaaaacaagaacttctagaaaattgcagttcctgtcttctgttagataactgattatagacagtctgtagaccaacaagtacaaaaacaaagaaccactacttatctgtagatcaacaagtacaaaaacaaagaaccactatgtaatatcttatttgtgggtaaaatacttgactgaaataaatttttcgatgcttagcttacaaagataatactagaatgtagcagaaatgtctctccataataaatgcaggcaacaggccaatttatctttgaagtattcaattaaaaaaacacaagtacaatacatcttgctaggcgtcattcaccctccaaatcaagcctggactactagtattcacccttagaaaaaaaaatctagcgtctagtatttaaaacgtgtaaattatgaacttcatgagaggcttataaccccatcctagggtgaggtcctcatctatgcctcaggagtggcaggagtggcattgggctccaagtcctcctgggaagggggagccgaggcttcctgttcagcaagtgcctctctaagttggctgcctaaaactgcatcatgaatgctgtggaacagcagctcccatagggcaggattttcaaaaaatctattccgagtgaggtcattcacaacttgtgcactgcatcctgctaagtatacatatataccgacgtctccatattcttttacaatccctgccagagttttcactccaacagaatcaataaaattgacttgagtgaaatccaaaatgacagtgtggacgttatcccctgggggcataaatctttgcatttcctcaggaaatgtgcttttgatcactattgggggatattttacttcaccatcctcttcttcaggcttggtagcatcctctccatctacttctgcatctgctttgacaacagttgcgttggccatatttgcatttccgacttccttagcgtacttccgcatggcctttctccttgctcccatgatgactgctgggttcactccagtctttcgttttaatgcattgctatacaagtcgctatttgcatagtaaattggtgcatttatttgaaatatttttattccaggaatttctttcacctcctcatatgcgtctatatcaatatacacatcagtttcaggaagctttccaaggactttgtagcttggactctgtgttctgtaaatcacagtcagcagagcaatgatcacagcagtgatcaaaccatagtccaatcccaggaacaaggaggacacaaaagtggtaagccagatggtcagctctattttgctggttctccagaaaaaggggagatctgagaactgcataaacattcccttcaggttgacaatcacaatggccgacagcacagcctggggcaatgattcaaagaggaatccagttgctaatatgaccagcagaatcattaatgaggccaaacaacctgcaagctgtgtcttcccaccggttccctcctgaacaaggcttcgagacaaggagcatgaaattgaaaaggtctggaagagtgagccaatggaattgcacagtcccagggcaatgagctcctgattgccgtcaacctggtagccatgtttatttgctaaggtcttggccatggagatggtcactgaaaatccaacgatggctatggcaatggcatctacgtacacaaggtggaagaggctggtgtccggattggctggaggtagcagccctagaggaagtgttccaacgacatccacattgtatgattctttcaagttaaacccagctgaaatgccagttcccattacgaccgcaaagaactctaaaggaataggcgccggcaatttctctttaaatctctcattaaactccttgccacccaacagcaaaccaaaaaccatcagcccgacgcctagggaacacacgttgaggtttttaacattctgcaacacagcaactgtactatacaccacggaaaagattccactgtaccgctttgttttaactccaaacagatattttaacatggaggtgaagacatgcacagctgctgcggtggtaaacccacggaccagaggctctgtgagatatatggccacaaatccaaacctacagacacctaggcaaaactgaatgattcctgaaagtaaggtcacagacatggcgactttcactctcaaggcatctctggcctctgtgccattggttgcatttactcctcctggaatgactatatcatctggtactaatcgaacagctacaccaccaatcatcaggctaataacagcaaaaggacctatggatatgtgtctggaggttccaagaaaacaatacatgataacagggtaaaatgaagagtacaggccaaatattggaggcacagctgccagcattgcaaaggctaagccttgaggaagctgaagcacccctgtgcttatgcctgagaccaagtcacccaacacatattccttgaatttgtatgctggcagccatttagttatgggtaggaacatataaatgatatttcttatttttttaggagtacatgtgaatgcctgtttcagcttatccgcaatggaatcaggaaccttgtcctttgtgtgtagtctttcctggaggaccggatgactaaagataggcctttccacatagtacctctgggttgctgcaaggatttcattttcttcagcatgatccatagtactctgaaattattccttaacagccggagacaagcatttcctgagtgtcaccagatccaatgtgcagcacaaaagtcgggacaggggacaagatcccccgctgggagctccagtgcagttcactgaagccttgatcactgaggctgagagcaggagaagggagagctcgctccttggcccccacagcgtatctgaggctttcttcacagctagctgatcggatccttgcagctgtttcttctgtaggtctcggagctcactgagaacgtccagcacgccttcccggcggggcccggcccaggtgcgcactagatgaggcagtcaaccaagtcaattggttcccgatcaactaaatctctcctaaaaataaacactgccgcgagcttcgagagttcagcgtgtcagagcctctatgatggcagagcacctgccgcgatgcctgattggtagggagaaggatttcccgggagggggccaataccaaattttagggctgttaggctctgagcagtcccttcgtgaccggataagtcagagacccggggtttgagccttgcccggcgctgagcggagggcccagtttcgggaccacagccttgctccctgggagctccgggcggccaatgccgggcaagcccagcccggcacaggaggaggcagggcccgtctccggaaagagggccagaggcagaactgagggcctggttttgtgtaattcgatttggatacaaacaggccagacccaaactggaaacggcgaagggctggattagcaccgaagggattcgaggaggcaaacgggaagtaaaaatgctgtgtggagctgcagagggcaaggggacaggggttgcaaaggaaagagcttcgtgagactttctccttcccggcgtagggaccagcagagtgcgggcaggtcagccctgtcaccggttcgtttagggaaaaagcgcgacatggggcctgggagacaggggcagaggcggtgacagcgagggcccctgctcgggtgggcccgcgggcctcagctcagtcccctcccgagggaccgc

SEQ ID NO: 11525 - RNA, 5007 nt, Homo sapiens
  source 1..5007: mol_type = other RNA
ctgaatagctgggactacaggtgcgcgccaccatgcccagctcacttttgtatttttaaatagagacagggtttcaccatgatggccaggctggtcttgaattcctgaccttgtgatctgcccgccttggcctcccaaagtactgggattacaggcgtgagccaccgcacctggccgaagtattttataacatagtttaaaatccttaaattctacttaaatggctgaaatgatattagctcgtttacaaaagtttctagtgtaagctgaggttctgcaactacatgctctttcagaaggcagtccgtatcagaatgcagatgtatctgatctcgtgatgattgcaaaggaaataactaagccaatctaaatttcactctagaattagttaaagttttgattaaaaggaggagtttattttgaattaaattagtaaagagagtgagaaatctgataggagttaacatcaacacatacaccacaggctttggttgcaagtaggccatgctaacaattctactgggatctgactactttctcctggcagtatcttattcatgaaagctataacaagatgtcaataagacagcatattaaagaaaagacaaactcactatcagcaggaactcttagcagaggaggctttagacaggttggctaatgcctgtgctttgatttgtagtgagctggtaattacaaacaactgaaagtgacaaattggtttaaaggtatcctcctccaacctttgacattccatgtttctgtggaatgagtaagatgagcattatgcttactcctaggctgaacactgagtttgatgtataatgaactgatagctgttatgaacttctaaggaagatttaagttatatgtgggggttagttttcttaaaaacatggtctttaatgctacttcatgattagcaacaatagcaaagtttctaaggacttatactggccacagttgtgacaatttgagcatcgaaaagaacataatggattgaaacccattaaaactataaaaattcacaagaccaccatcacaccagaaaagggaaatctaaaaaaaaaaaaaaacactaatttgtcaccatctaataaaccagttatttactttgaagttgataattaaatgaaaataataaagcattcaacctgcccttctggtagaactgtaggtaaggatgaccaaatagctcaagtggagaagggaaagcttagttcacatagaataaccaactaacaaacggagaagaaatgaaagaactagacaaccaactcacaaactttaacaaagttaatgatttaggcaagaattaccacctaatgttaaaactcctgggtaaatggtaattcattcaatgccaaaggaataccacacagataagtctgtagtcacaaaggggaaaaatctaactggatgatcagactgtcatgctgatccagtaatcaaacttagatcaatagattagttaatggtagatcaactagatattacgttttctgaagtgatgcgatatgaagcatgtatcttatctatgatataatctagcacaaaatgttttaacttgaacctataaaggctttagatataacttccagattgcaggtagtacaggcaatataaaaacaagttaaacaacaccatgaaaaagaaactaggcaaattcacaagacaggattctacaggaccgctgccccagtctctttaacaagtcaatgtcataaaaaaggaactgtgctagattaaaatagatgtaagggactttaaaggacatgaccagttgcaatgtaaggtcatagaatgaatatcagtttgcacaaaccaactgcaaatctggggacaattggggaaatttaaatatggtctaagatcaaaaatgtgctggaatgagaaagtggagattgttgattaaagaaaaatcggttataaaacactatagatgtggtcttactttggttaaaaatgtaaatgtatatgtatggaaaaagatctggaaggatattaacagtggtaatctctgagtggtggaaatatgttttatgttcttatttttgcttgtctacttttttaaaatgtcctcaatgcatttatactgcttctataataaataaaaggttattttaaaacaagaacttctagaaaattgcagttcctgtcttctgttagataactgattatagacagtctgtagaccaacaagtacaaaaacaaagaaccactacttatctgtagatcaacaagtacaaaaacaaagaaccactatgtaatatcttatttgtgggtaaaatacttgactgaaataaatttttcgatgcttagcttacaaagataatactagaatgtagcagaaatgtctctccataataaatgcaggcaacaggccaatttatctttgaagtattcaattaaaaaaacacaagtacaatacatcttgctaggcgtcattcaccctccaaatcaagcctggactactagtattcacccttagaaaaaaaaatctagcgtctagtatttaaaacgtgtaaattatgaacttcatgagaggcttataaccccatcctagggtgaggtcctcatctatgcctcaggagtggcaggagtggcattgggctccaagtcctcctgggaagggggagccgaggcttcctgttcagcaagtgcctctctaagttggctgcctaaaactgcatcatgaatgctgtggaacagcagctcccatagggcaggattttcaaaaaatctattccgagtgaggtcattcacaacttgtgcactgcatcctgctaagtatacatatataccgacgtctccatattcttttacaatccctgccagagttttcactccaacagaatcaataaaattgacttgagtgaaatccaaaatgacagtgtggacgttatcccctgggggcataaatctttgcatttcctcaggaaatgtgcttttgatcactattgggggatattttacttcaccatcctcttcttcaggcttggtagcatcctctccatctacttctgcatctgctttgacaacagttgcgttggccatatttgcatttccgacttccttagcgtacttccgcatggcctttctccttgctcccatgatgactgctgggttcactccagtctttcgttttaatgcattgctatacaagtcgctatttgcatagtaaattggtgcatttatttgaaatatttttattccaggaatttctttcacctctgtgttctgtaaatcacagtcagcagagcaatgatcacagcagtgatcaaaccatagtccaatcccaggaacaaggaggacacaaaagtggtaagccagatggtcagctctattttgctggttctccagaaaaaggggagatctgagaactgcataaacattcccttcaggttgacaatcacaatggccgacagcacagcctggggcaatgattcaaagaggaatccagttgctaatatgaccagcagaatcattaatgaggccaaacaacctgcaagctgtgtcttcccaccggttccctcctgaacaaggcttcgagacaaggagcatgaaattgaaaaggtctggaagagtgagccaatggaattgcacagtcccagggcaatgagctcctgattgccgtcaacctggtagccatgtttatttgctaaggtcttggccatggagatggtcactgaaaatccaacgatggctatggcaatggcatctacgtacacaaggtggaagaggctggtgtccggattggctggaggtagcagccctagaggaagtgttccaacgacatccacattgtatgattctttcaagttaaacccagctgaaatgccagttcccattacgaccgcaaagaactctaaaggaataggcgccggcaatttctctttaaatctctcattaaactccttgccacccaacagcaaaccaaaaaccatcagcccgacgcctagggaacacacgttgaggtttttaacattctgcaacacagcaactgtactatacaccacggaaaagattccactgtaccgctttgttttaactccaaacagatattttaacatggaggtgaagacatgcacagctgctgcggtggtaaacccacggaccagaggctctgtgagatatatggccacaaatccaaacctacagacacctaggcaaaactgaatgattcctgaaagtaaggtcacagacatggcgactttcactctcaaggcatctctggcctctgtgccattggttgcatttactcctcctggaatgactatatcatctggtactaatcgaacagctacaccaccaatcatcaggctaataacagcaaaaggacctatggatatgtgtctggaggttccaagaaaacaatacatgataacagggtaaaatgaagagtacaggccaaatattggaggcacagctgccagcattgcaaaggctaagccttgaggaagctgaagcacccctgtgcttatgcctgagaccaagtcacccaacacatattccttgaatttgtatgctggcagccatttagttatgggtaggaacatataaatgatatttcttatttttttaggagtacatgtgaatgcctgtttcagcttatccgcaatggaatcaggaaccttgtcctttgtgtgtagtctttcctggaggaccggatgactaaagataggcctttccacatagtacctctgggttgctgcaaggatttcattttcttcagcatgatccatagtactctgaaattattccttaacagccggagacaagcatttcctgagtgtcaccagatccaatgtgcagcacaaaagtcgggacaggggacaagatcccccgctgggagctccagtgcagttcactgaagccttgatcactgaggctgagagcaggagaagggagagctcgctccttggcccagcccgggctgccctgggcggagccgccccgccgcgctccacagccgctgcctcttcgacgcgcgcgctgcctccaggt

SEQ ID NO: 11526 - RNA, 4911 nt, Homo sapiens
  source 1..4911: mol_type = other RNA
ctgaatagctgggactacaggtgcgcgccaccatgcccagctcacttttgtatttttaaatagagacagggtttcaccatgatggccaggctggtcttgaattcctgaccttgtgatctgcccgccttggcctcccaaagtactgggattacaggcgtgagccaccgcacctggccgaagtattttataacatagtttaaaatccttaaattctacttaaatggctgaaatgatattagctcgtttacaaaagtttctagtgtaagctgaggttctgcaactacatgctctttcagaaggcagtccgtatcagaatgcagatgtatctgatctcgtgatgattgcaaaggaaataactaagccaatctaaatttcactctagaattagttaaagttttgattaaaaggaggagtttattttgaattaaattagtaaagagagtgagaaatctgataggagttaacatcaacacatacaccacaggctttggttgcaagtaggccatgctaacaattctactgggatctgactactttctcctggcagtatcttattcatgaaagctataacaagatgtcaataagacagcatattaaagaaaagacaaactcactatcagcaggaactcttagcagaggaggctttagacaggttggctaatgcctgtgctttgatttgtagtgagctggtaattacaaacaactgaaagtgacaaattggtttaaaggtatcctcctccaacctttgacattccatgtttctgtggaatgagtaagatgagcattatgcttactcctaggctgaacactgagtttgatgtataatgaactgatagctgttatgaacttctaaggaagatttaagttatatgtgggggttagttttcttaaaaacatggtctttaatgctacttcatgattagcaacaatagcaaagtttctaaggacttatactggccacagttgtgacaatttgagcatcgaaaagaacataatggattgaaacccattaaaactataaaaattcacaagaccaccatcacaccagaaaagggaaatctaaaaaaaaaaaaaaacactaatttgtcaccatctaataaaccagttatttactttgaagttgataattaaatgaaaataataaagcattcaacctgcccttctggtagaactgtaggtaaggatgaccaaatagctcaagtggagaagggaaagcttagttcacatagaataaccaactaacaaacggagaagaaatgaaagaactagacaaccaactcacaaactttaacaaagttaatgatttaggcaagaattaccacctaatgttaaaactcctgggtaaatggtaattcattcaatgccaaaggaataccacacagataagtctgtagtcacaaaggggaaaaatctaactggatgatcagactgtcatgctgatccagtaatcaaacttagatcaatagattagttaatggtagatcaactagatattacgttttctgaagtgatgcgatatgaagcatgtatcttatctatgatataatctagcacaaaatgttttaacttgaacctataaaggctttagatataacttccagattgcaggtagtacaggcaatataaaaacaagttaaacaacaccatgaaaaagaaactaggcaaattcacaagacaggattctacaggaccgctgccccagtctctttaacaagtcaatgtcataaaaaaggaactgtgctagattaaaatagatgtaagggactttaaaggacatgaccagttgcaatgtaaggtcatagaatgaatatcagtttgcacaaaccaactgcaaatctggggacaattggggaaatttaaatatggtctaagatcaaaaatgtgctggaatgagaaagtggagattgttgattaaagaaaaatcggttataaaacactatagatgtggtcttactttggttaaaaatgtaaatgtatatgtatggaaaaagatctggaaggatattaacagtggtaatctctgagtggtggaaatatgttttatgttcttatttttgcttgtctacttttttaaaatgtcctcaatgcatttatactgcttctataataaataaaaggttattttaaaacaagaacttctagaaaattgcagttcctgtcttctgttagataactgattatagacagtctgtagaccaacaagtacaaaaacaaagaaccactacttatctgtagatcaacaagtacaaaaacaaagaaccactatgtaatatcttatttgtgggtaaaatacttgactgaaataaatttttcgatgcttagcttacaaagataatactagaatgtagcagaaatgtctctccataataaatgcaggcaacaggccaatttatctttgaagtattcaattaaaaaaacacaagtacaatacatcttgctaggcgtcattcaccctccaaatcaagcctggactactagtattcacccttagaaaaaaaaatctagcgtctagtatttaaaacgtgtaaattatgaacttcatgagaggcttataaccccatcctagggtgaggtcctcatctatgcctcaggagtggcaggagtggcattgggctccaagtcctcctgggaagggggagccgaggcttcctgttcagcaagtgcctctctaagttggctgcctaaaactgcatcatgaatgctgtggaacagcagctcccatagggcaggattttcaaaaaatctattccgagtgaggtcattcacaacttgtgcactgcatcctgctaagtatacatatataccgacgtctccatattcttttacaatccctgccagagttttcactccaacagaatcaataaaattgacttgagtgaaatccaaaatgacagtgtggacgttatcccctgggggcataaatctttgcatttcctcaggaaatgtgcttttgatcactattgggggatattttacttcaccatcctcttcttcaggcttggtagcatcctctccatctacttctgcatctgctttgacaacagttgcgttggccatatttgcatttccgacttccttagcgtacttccgcatggcctttctccttgctcccatgatgactgctgggttcactccagtctttcgttttaatgcattgctatacaagtcgctatttgcatagtaaattggtgcatttatttgaaatatttttattccaggaatttctttcacctctgtgttctgtaaatcacagtcagcagagcaatgatcacagcagtgatcaaaccatagtccaatcccaggaacaaggaggacacaaaagtggtaagccagatggtctggggcaatgattcaaagaggaatccagttgctaatatgaccagcagaatcattaatgaggccaaacaacctgcaagctgtgtcttcccaccggttccctcctgaacaaggcttcgagacaaggagcatgaaattgaaaaggtctggaagagtgagccaatggaattgcacagtcccagggcaatgagctcctgattgccgtcaacctggtagccatgtttatttgctaaggtcttggccatggagatggtcactgaaaatccaacgatggctatggcaatggcatctacgtacacaaggtggaagaggctggtgtccggattggctggaggtagcagccctagaggaagtgttccaacgacatccacattgtatgattctttcaagttaaacccagctgaaatgccagttcccattacgaccgcaaagaactctaaaggaataggcgccggcaatttctctttaaatctctcattaaactccttgccacccaacagcaaaccaaaaaccatcagcccgacgcctagggaacacacgttgaggtttttaacattctgcaacacagcaactgtactatacaccacggaaaagattccactgtaccgctttgttttaactccaaacagatattttaacatggaggtgaagacatgcacagctgctgcggtggtaaacccacggaccagaggctctgtgagatatatggccacaaatccaaacctacagacacctaggcaaaactgaatgattcctgaaagtaaggtcacagacatggcgactttcactctcaaggcatctctggcctctgtgccattggttgcatttactcctcctggaatgactatatcatctggtactaatcgaacagctacaccaccaatcatcaggctaataacagcaaaaggacctatggatatgtgtctggaggttccaagaaaacaatacatgataacagggtaaaatgaagagtacaggccaaatattggaggcacagctgccagcattgcaaaggctaagccttgaggaagctgaagcacccctgtgcttatgcctgagaccaagtcacccaacacatattccttgaatttgtatgctggcagccatttagttatgggtaggaacatataaatgatatttcttatttttttaggagtacatgtgaatgcctgtttcagcttatccgcaatggaatcaggaaccttgtcctttgtgtgtagtctttcctggaggaccggatgactaaagataggcctttccacatagtacctctgggttgctgcaaggatttcattttcttcagcatgatccatagtactctgaaattattccttaacagccggagacaagcatttcctgagtgtcaccagatccaatgtgcagcacaaaagtcgggacaggggacaagatcccccgctgggagctccagtgcagttcactgaagccttgatcactgaggctgagagcaggagaagggagagctcgctccttggcccagcccgggctgccctgggcggagccgccccgccgcgctccacagccgctgcctcttcgacgcgcgcgctgcctccaggt

SEQ ID NO: 11527 - RNA, 2667 nt, Homo sapiens
  source 1..2667: mol_type = other RNA
ctgaatagctgggactacaggtgcgcgccaccatgcccggctaattttgtgtattttagcagagatggggtttcaccatgttgcccggggtggtcttgaactcctgaactcaggcgatacacccacctcggccccccaaagtgctgggattaacaggcgtgagccaccgcaaccggccttggttatattttcaaaatagtgaaggtttgaaaaattagatcgtaaattatgagaagttgcccatcacagtatttgggataaaatggagtgccaccagctcggatgagaattaagctaacagttcaacaaggaaaccaattcacaaggaacatactggaagtcaatcacaaaaaggaataagctggaatgaaggtattctctggttctctcacttcgagtgttgatacaaaaacacaacttcacagtgaccctctggatctcacctccttagcagcaagatcctcccataacatccgtttccctggaccttctttgggtcatgatgaaagttagcagaagaaaacctcagatgacccatccttgactaggccctgcagggtcattatgcccatcctcatgaccacctcacacgctccttaaggtgtctcatcatagcccccactggcaaggtgaaggtcacatataccactgatatatctgaaaagtaaacacttttgtagcccaaggaattagaaataccttcctctgttttttttttaatggtctttacatcaaggtgctgcagccagtggggcatgaggcagagttttcacctgggtcagaaggttttggaactcttccactgcctgtgaatgtgccttggggttgagcaccaggtgttggaagagattgaccggctcagcattcctaaatgtcttagggattgggatggtcaggggcagaaaattgttaccaatgaggaaatgatggagggacctttgctggaggccacggcccaagaaccagagaatgtcctggagccgctgagagagcatgttgtgggcccagtccgtgaggggcagccgtagcaagaggtgcatgagagctgttttaaaatggtaagaagtgaggatggggcgggatgctccatggggtaagctctgatgctgccggagacttaaaatgatctggaggcacttgaggtgacaggtgttctcgggggcaaagcgccccaccagcttcaggaacaggtgctcacaggccacaaaggactcaggccagtccacactggtgagctgctcctggtcaggagcctgactcaccaggtagaccaaggtgtcttctcgttgcacccccaggaccaagtggattgagagaaagcggcctgagcgatagtccagccggagcttgcaggaggtggtagacggtgggagactgagtttaaagtcatacttgtgggccacaagggcccaggcattgcccatcatgttccggaaccactgcacagtcttgcacacgtctaggtggaagccggtgcagagagctgccttgatggagctactacacttccccaagactgccgaggggtccctgtggtggtgcaccaggcacagcacgtcccctaggagtttctcacgcttgcacacacattctgactccaccagcacacagccacagcggcggcccagggctgggtccctcatctccaggacaaacatggtgccctgtggggggacaatgggcaccaggatatcaaatttctgggtctcatggagggttccccatttctcaaaggcagccccgatgcccaggcagtcttccaattgtgggtgagcctcttggcggctgagcacccgacaggcctcaatgagatcatccacaaaactctccacaaactcacaggtgcagggcaggtcacggatggcattttggacatagtgtttgtaaaaggagtccagggcctcctgggaggggaagtcagtaagccagttgtaagaggtgacagggacaacacggacttcctcctcctcctcctcactgctggaatcaaaggccggttcatgctgcatgttctgtcgcaggagctcaaagacgagaaaaaggcaaaagaggccagtgttccacaggtttcccagcatccagcccagaggcccttcctggccatcggcctggaacggccaccccatgtctttcttccccagcactaactggtcactggatgtgtctcctgtccagaagttctctgccttctgcctctgctcagcggctcgctttctctcttcaaactccatctctagcaggcgcatctcctcactcattcgcttctccagctgccgactcctggctaatgtgtccaggtccatccgatcactgaccatcagagggtggtgaacaacatacatcactgccaagaacagcaggcttatcacagccatggaggcctctgcatcaacattcatgaaggactatgccgtgtggacgctgaagccagctgggcctatcctccctttggaacttggccttgcttcgtctccccgccctctctaggagccctgttaaaatgtacaaggtacctgggggctttggctcaaatcggaacccgaccctccccccattcataacttccccaaattccacgcccagagatttgtactctcacccgcctatccgtaggaggccaagggcccatcctacctcgggatgtctcccgggacccagggccaggtt

SEQ ID NO: 11528 - RNA, 2816 nt, Homo sapiens
  source 1..2816: mol_type = other RNA
ctgaatagctgggactacaggtgcgcgccaccatgcccggctaattttgtgtattttagcagagatggggtttcaccatgttgcccggggtggtcttgaactcctgaactcaggcgatacacccacctcggccccccaaagtgctgggattaacaggcgtgagccaccgcaaccggccttggttatattttcaaaatagtgaaggtttgaaaaattagatcgtaaattatgagaagttgcccatcacagtatttgggataaaatggagtgccaccagctcggatgagaattaagctaacagttcaacaaggaaaccaattcacaaggaacatactggaagtcaatcacaaaaaggaataagctggaatgaaggtattctctggttctctcacttcgagtgttgatacaaaaacacaacttcacagtgaccctctggatctcacctccttagcagcaagatcctcccataacatccgtttccctggaccttctttgggtcatgatgaaagttagcagaagaaaacctcagatgacccatccttgactaggccctgcagggtcattatgcccatcctcatgaccacctcacacgctccttaaggtgtctcatcatagcccccactggcaaggtgaaggtcacatataccactgatatatctgaaaagtaaacacttttgtagcccaaggaattagaaataccttcctctgttttttttttaatggtctttacatcaaggtgctgcagccagtggggcatgaggcagagttttcacctgggtcagaaggttttggaactcttccactgcctgtgaatgtgccttggggttgagcaccaggtgttggaagagattgaccggctcagcattcctaaatgtcttagggattgggatggtcaggggcagaaaattgttaccaatgaggaaatgatggagggacctttgctggaggccacggcccaagaaccagagaatgtcctggagccgctgagagagcatgttgtgggcccagtccgtgaggggcagccgtagcaagaggtgcatgagagctgttttaaaatggtaagaagtgaggatggggcgggatgctccatggggtaagctctgatgctgccggagacttaaaatgatctggaggcacttgaggtgacaggtgttctcgggggcaaagcgccccaccagcttcaggaacaggtgctcacaggccacaaaggactcaggccagtccacactggtgagctgctcctggtcaggagcctgactcaccaggtagaccaaggtgtcttctcgttgcacccccaggaccaagtggattgagagaaagcggcctgagcgatagtccagccggagcttgcaggaggtggtagacggtgggagactgagtttaaagtcatacttgtgggccacaagggcccaggcattgcccatcatgttccggaaccactgcacagtcttgcacacgtctaggtggaagccggtgcagagagctgccttgatggagctactacacttccccaagactgccgaggggtccctgtggtggtgcaccaggcacagcacgtcccctaggagtttctcacgcttgcacacacattctgactccaccagcacacagccacagcggcggcccagggctgggtccctcatctccaggacaaacatggtgccctgtggggggacaatgggcaccaggatatcaaatttctgggtctcatggagggttccccatttctcaaaggcagccccgatgcccaggcagtcttccaattgtgggtgagcctcttggcggctgagcacccgacaggcctcaatgagatcatccacaaaactctccacaaactcacaggtgcagggcaggtcacggatggcattttggacatagtgtttgtaaaaggagtccagggcctcctgggaggggaagtcagtaagccagttgtaagaggtgacagggacaacacggacttcctcctcctcctcctcactgctggaatcaaaggccggttcatgctgcatgttctgtcgcaggagctcaaagacgagaaaaaggcaaaagaggccagtgttccacaggtttcccagcatccagcccagaggcccttcctggccatcggcctggaacggccaccccatgtctttcttccccagcactaactggtcactggatgtgtctcctgtccagaagttctctgccttctgcctctgctcagcggctcgctttctctcttcaaactccatctctagcaggcgcatctcctcactcattcgcttctccagctgccgactcctggctaatgtgtccaggtccatccgatcactgaccatcagagggtggtgaacaacatacatcactgccaagaacagcaggcttatcacagccatggaggcctctgcatctggagaagtaggagagtaggagtcagtggtcatcttccagacttatctgctctctagctcacattccccagagccctggtaccccaaattctgaaaatcagctactcaggaggaacagaaagcccacagagcttggcttggacacagcaagggtggtcggcctgggaggaggttcgagagaaaagagggcgaaaggatgtgccactcagtctctctcctgctttccttccacatggtgtgggtggtatttaggcttccagaaagtgtacatgggactgttttcattcctgtgtaggatggggagggggacccttgtggtagggtggcctcacccgactcctcagtcaaccatgggcaccagatatgacctgctgatcccagaggctcccttttatagccagaaagccctgaacctgcctgggtgac

SEQ ID NO: 11529 - RNA, 1657 nt, Homo sapiens
  source 1..1657: mol_type = other RNA
ctgaatagctgggactacaggtgcgtgccacacccggctaatttcttatttttagtagagacggggtttcaccatgttggctaggttggtctcgaactcctgaccttgtgatccgcccaccttggcctcccaaagtgctgggattacaggcgtgagccaccgcgcccagcccaggtgggctttctcaggaagccatggaagcagagacatgctttccttctaccctactctactgtgaacttggacaaaatacactgggggtctgggctggaaggcagattcctacaagtcccctcctctggaggaagctaaacagcaaaggcatcgagcggccctgcccgctcctttttgtgtgtatatacgaagaacacaggaacagctgttcttctttcagtcattccaactaaaacagacattttgcatagagagaataccagcccacttggtttcttgttttttattattggcgtcagctaggactatacgtggccttaaacgtcatgcactgatggacagaagagaaaaaaggatgaaaaaaaagacaaaggaggggaaagaggagcagcagtgaaaatttgtaataaaaactcttcttaatttataggtaagttttggcatttttaaatccaacgccccctcccaccccctaaagttccaaccaaagtgagagggtcacagggtgacccggccaggtgttctgcactccctcacaggctgctgtcagaggcagcttgtgggtttaattcttttgtatgtgttttacatttttcactttctttaaataattgcttcttgactcttagacgttccggttcacgggggtgacataattgcggggaaacatgccggtctgcccgtggcaagctcctttccaccagttggggtctgagttatccatgacatggataaaatctccccggcggaagcccagctctccatcctcctggggatcaaagtcaaagagggcctggacgtatgtcggctgctgtggcacctgttctatgtcccgcaggaatatctgctggtttctggagacagatgtagatctgtgataatccaccagctcattcaaagaattgaacttcaccacccagaggaagtacttcccggctccatctcggagcaccttgaagtgctgcacatcgtttccaaacggatgtggtttcatttctatgtagttcttgggaatgaagccgtcttttccattaagctctgccttgtaccagttctgatcacattcttcgttcaaaaccttgaggatgtccccccttttgaagctcagctcgtcgtctgcagtagctttgaagtcatatttggcgatggcttccattctgagcgctgctcagtgctcagcagcctgaagcagggggaagggagtcttccctgctgaagcaacccagcgctctgggcttagcctcgcctctcttctgggactcgctccggcactctgggacacacaatgccacccgtggcgcagctgctccgctcagcgtccggcccgcccctccacaacgctgcgagcggccggcgaccccaaggctgctctgcgagggcagcgcttgctcccgccgccgtcaccgccacaggcacagactctgccacagccgccgccgccgctgccgccgcccggtcgccgaagcagcaatacctcctggct

SEQ ID NO: 11530 - RNA, 1780 nt, Homo sapiens
  source 1..1780: mol_type = other RNA
ctgaatagctgggactacaggtgcgtgccacacccggctaatttcttatttttagtagagacggggtttcaccatgttggctaggttggtctcgaactcctgaccttgtgatccgcccaccttggcctcccaaagtgctgggattacaggcgtgagccaccgcgcccagcccaggtgggctttctcaggaagccatggaagcagagacatgctttccttctaccctactctactgtgaacttggacaaaatacactgggggtctgggctggaaggcagattcctacaagtcccctcctctggaggaagctaaacagcaaaggcatcgagcggccctgcccgctcctttttgtgtgtatatacgaagaacacaggaacagctgttcttctttcagtcattccaactaaaacagacattttgcatagagagaataccagcccacttggtttcttgttttttattattggcgtcagctaggactatacgtggccttaaacgtcatgcactgatggacagaagagaaaaaaggatgaaaaaaaagacaaaggaggggaaagaggagcagcagtgaaaatttgtaataaaaactcttcttaatttataggtaagttttggcatttttaaatccaacgccccctcccaccccctaaagttccaaccaaagtgagagggtcacagggtgacccggccaggtgttctgcactccctcacaggctgctgtcagaggcagcttgtgggtttaattcttttgtatgtgttttacatttttcactttctttaaataattgcttcttgactcttagacgttccggttcacgggggtgacataattgcggggaaacatgccggtctgcccgtggcaagctcctttccaccagttggggtctgagttatccatgacatggataaaatctccccggcggaagcccagctctccatcctcctggggatcaaagtcaaagagggcctggacgtatgtcggctgctgtggcacctgttctatgtcccgcaggaatatctgctggtttctggagacagatgtagatctgtgataatccaccagctcattcaaagaattgaacttcaccacccagaggaagtacttcccggctccatctcggagcaccttgaagtgctgcacatcgtttccaaacttgacagagagggagaagtccccaggagcgctctcactctctcggataagaaaggccccatcgtgccgctgtttgctaagcatttcttctgccttggctctggggattttgccaaaaaaccacggatgtggtttcatttctatgtagttcttgggaatgaagccgtcttttccattaagctctgccttgtaccagttctgatcacattcttcgttcaaaaccttgaggatgtccccccttttgaagctcagctcgtcgtctgcagtagctttgaagtcatatttggcgatggcttccattctgagcgctgctcagtgctcagcagcctgaagcagggggaagggagtcttccctgctgaagcaacccagcgctctgggcttagcctcgcctctcttctgggactcgctccggcactctgggacacacaatgccacccgtggcgcagctgctccgctcagcgtccggcccgcccctccacaacgctgcgagcggccggcgaccccaaggctgctctgcgagggcagcgcttgctcccgccgccgtcaccgccacaggcacagactctgccacagccgccgccgccgctgccgccgcccggtcgccgaagcagcaatacctcctggct

SEQ ID NO: 11531 - RNA, 3728 nt, Homo sapiens
  source 1..3728: mol_type = other RNA
ctgaatagctgggactacaggtgcgtgccaccacaccaggctaatttttgtatttttagtagagacggggtttcaccacgttggccaggctggtctcaaactcctggcctcaagtgatccacccgcctcggcctcccaacatgctgggattacaggcataagccactacgcctggcctgagctgtcttgactgtcactgcaaactgaggctcaggtggccagtgacttgcccaagtccacaaggctgtgggaggtggagcagggattcaagggaggccctgaggccacccagcctgggtgggtctcaaaagcaattttcttctcttccctcctccacccattcatagtggaaagcaagcctgcaccccaggagctcccattcataccctctctgtcccctctctgttcttcctcctcccgcctgccccatgcacctcccaccctgaagttccctgccacccctcgccctgtgccagcttgtctctgcaggctctcagtcctgggggctggagaacaggtgctcagtcctctttgctgcccacagaagtctcagaacattcttgccccaccctcccttgggccaaagccctttagggtcccgtcctttcatgctgtgctctcctcctcctcctcctcctccctgcctctctccttgctcactgaagacctcagcacccactgcctcccagccttgccctgaaccaagcacagacgaccaccacgctggcaatgtctctgtccaccagaggggtgatgggtcagcccccaagaacctcctacgccacagggaggagttggaattttattccaagtgaggcaaaaaccatgcaaggtatagagcaggggaggccaaggccaggtgtgggtttaatcggggtctgtcggtggcagggcagctgcagggaggccgtgttggtgatgcctgggccagggcacagtggtaaagtttaacccaggctcccctgtctacccctgaaaaagactggaaaatgctgagtcccagccaagggtccagggtctaggagctgaggtcagagaggcccaggaggtgggggaggcaggcccagtgaggtggccctctcctggtcttgctggcttcggttttcccaggggagctcactgcaccctgagcggcattgtcccccattgccctgacccttgcccccacctccttggctggtggagccaggagcctgggaggcccctgtgcacacctggcagcttcacctccccaaacaggcccggagttcattcaaatccagcctctgggagcaggggccttgccactcggttatgtgagcctgctaaagccctccttgccatgtgtgcttgcaggcgggggcccagaaccaagttgggaggccactggctgtcctgtgggaccagagaagtctggtgccaccctagcagggccaagggacttcttctggacgtcagtctgtgcccagcctctaccaccagctttcccttccctgcagggaggggcatgacctgcagaaccaaaggtgcttctgtgagccagtagcccagtgctgcttgggggcaggggcggggcctgtgccttgggttcccccccctccctgggcacatttggggttggggcagcccacacggtggggtgggaagattgacctgcccattttacaaatgagcaaaggtgggagaactcagggagacatgggggagcagagggaggaagcagagcccaacagcccggggcacccggaccccagccactgcctgcctgtggatgggtttctggccacggtgcagggctactgcgaggaggaaatgagggtgatgtgggcacctgaaacagcagaaatggctcagggccaggcactggggagccactgtccccatggggcttgagcttctgcctcagagggaccttccggctgccattgagggtcccagcaccaaaccccacagctggaccacttgggacctcaatccacagggggccagggctgcggcctatggcagataaagatagaggaggagggctggatgaagccacaggtggtgggcacaggataggccagacagaagggactttgggggactccaccttgggtagaaggagggacagctgaggtcctgtggtggagaaggcctggagcagagggtgaccaaggagatgacagagtgcacgtacagggccaggccaatgggagtgggaacccttgggagagggagcttcaggccattcattcagttcctgtttagccagcaccctcctcccctcatctgtccctctgccctcaccccaacatgccagaatctccttcctctccagcttgtacccaagccctctctgctccatgcccccagcctgctgaccacctctcagccatgtcctgggcctccagatctgtccctgatcctagtcttgcctctgaggggtccatcatccttgtctgtcccccagacctcccacgccagcccctgctcccaccctgcctggctgcctcgtgcctctggcccagctgggtaggtagggatttgcatagctgctccccagctcctccatacctcggctccccacacagcactgctaggcgcccctgcagggtcctccctcagctcagaggctgccctactggctgaggtgcaggctggtgccaagagagcatgctgctctgtcagcatgaggcagtgagcagggctctgggcaagggtggcatccaggaaagcccttgaagactgaggggcgctttgctggttgggccaagggaggaagggcctgcctggcagaaggaacagcctgggcaaaggccccaagatgggaaagccttggtggttggggcatagaatgggggggcagtggggccggccaagacaggaagggccttgaatgtgagggtgaaatgatggggtgtccctgggggccttactcccaactcagatcaagtcctttggtggcaggggctgccccggtcctctgacccagggcaagctctatgagcggtggagcccatcctagagattttcatagaccaggttaagttcgccatcatcttcgaatctatgcggtctctcctgggagagggggctctgcttggcggtgggtgagctgccatcctcattctcgatgcaggcatagacctcggtctcgcggcgctgcagagctgtgtagacagattctgaaggatgctgcttggggctgctggcagatcttggatctgggcacttcctggtggggtccttccctggaccccgcatccgcttctctgaccaggatgaaggtgccgctgcctctcaccgtggagtgtggccagtggacagagcagtagtaggtgccagtggccgatgctcccggcagcacaagggtgacctggcagtccagggtgtggctctggttctctgtgcccagtccagggtggcagtttgttggcttcttagggctcctctgtccctggagatcttcatgaaagtagctgactgtgaaaaccttgaattggggagtgtatggataggtgatcctgcagctgaaggagatagctgtgttggccagggaggccatgatgggcaggccggtgtgggtcactgactgtcctcctgccagtcgcagggtcccgggcagcagcagcacgccaaggaggagccagggggctgcggggagcccaggagggcgtgggaggcctggcagggcccgccacctcacaggctggttctccatctgggggcctgcttgtctgcggcgactctttagttcacaggagggg

SEQ ID NO: 11532 - RNA, 3841 nt, Homo sapiens
  source 1..3841: mol_type = other RNA
ctgaatagctgggactacaggtgcgtgccaccacaccaggctaatttttgtatttttagtagagacggggtttcaccacgttggccaggctggtctcaaactcctggcctcaagtgatccacccgcctcggcctcccaacatgctgggattacaggcataagccactacgcctggcctgagctgtcttgactgtcactgcaaactgaggctcaggtggccagtgacttgcccaagtccacaaggctgtgggaggtggagcagggattcaagggaggccctgaggccacccagcctgggtgggtctcaaaagcaattttcttctcttccctcctccacccattcatagtggaaagcaagcctgcaccccaggagctcccattcataccctctctgtcccctctctgttcttcctcctcccgcctgccccatgcacctcccaccctgaagttccctgccacccctcgccctgtgccagcttgtctctgcaggctctcagtcctgggggctggagaacaggtgctcagtcctctttgctgcccacagaagtctcagaacattcttgccccaccctcccttgggccaaagccctttagggtcccgtcctttcatgctgtgctctcctcctcctcctcctcctccctgcctctctccttgctcactgaagacctcagcacccactgcctcccagccttgccctgaaccaagcacagacgaccaccacgctggcaatgtctctgtccaccagaggggtgatgggtcagcccccaagaacctcctacgccacagggaggagttggaattttattccaagtgaggcaaaaaccatgcaaggtatagagcaggggaggccaaggccaggtgtgggtttaatcggggtctgtcggtggcagggcagctgcagggaggccgtgttggtgatgcctgggccagggcacagtggtaaagtttaacccaggctcccctgtctacccctgaaaaagactggaaaatgctgagtcccagccaagggtccagggtctaggagctgaggtcagagaggcccaggaggtgggggaggcaggcccagtgaggtggccctctcctggtcttgctggcttcggttttcccaggggagctcactgcaccctgagcggcattgtcccccattgccctgacccttgcccccacctccttggctggtggagccaggagcctgggaggcccctgtgcacacctggcagcttcacctccccaaacaggcccggagttcattcaaatccagcctctgggagcaggggccttgccactcggttatgtgagcctgctaaagccctccttgccatgtgtgcttgcaggcgggggcccagaaccaagttgggaggccactggctgtcctgtgggaccagagaagtctggtgccaccctagcagggccaagggacttcttctggacgtcagtctgtgcccagcctctaccaccagctttcccttccctgcagggaggggcatgacctgcagaaccaaaggtgcttctgtgagccagtagcccagtgctgcttgggggcaggggcggggcctgtgccttgggttcccccccctccctgggcacatttggggttggggcagcccacacggtggggtgggaagattgacctgcccattttacaaatgagcaaaggtgggagaactcagggagacatgggggagcagagggaggaagcagagcccaacagcccggggcacccggaccccagccactgcctgcctgtggatgggtttctggccacggtgcagggctactgcgaggaggaaatgagggtgatgtgggcacctgaaacagcagaaatggctcagggccaggcactggggagccactgtccccatggggcttgagcttctgcctcagagggaccttccggctgccattgagggtcccagcaccaaaccccacagctggaccacttgggacctcaatccacagggggccagggctgcggcctatggcagataaagatagaggaggagggctggatgaagccacaggtggtgggcacaggataggccagacagaagggactttgggggactccaccttgggtagaaggagggacagctgaggtcctgtggtggagaaggcctggagcagagggtgaccaaggagatgacagagtgcacgtacagggccaggccaatgggagtgggaacccttgggagagggagcttcaggccattcattcagttcctgtttagccagcaccctcctcccctcatctgtccctctgccctcaccccaacatgccagaatctccttcctctccagcttgtacccaagccctctctgctccatgcccccagcctgctgaccacctctcagccatgtcctgggcctccagatctgtccctgatcctagtcttgcctctgaggggtccatcatccttgtctgtcccccagacctcccacgccagcccctgctcccaccctgcctggctgcctcgtgcctctggcccagctgggtaggtagggatttgcatagctgctccccagctcctccatacctcggctccccacacagcactgctaggcgcccctgcagggtcctccctcagctcagaggctgccctactggctgaggtgcaggctggtgccaagagagcatgctgctctgtcagcatgaggcagtgagcagggctctgggcaagggtggcatccaggaaagcccttgaagactgaggggcgctttgctggttgggccaagggaggaagggcctgcctggcagaaggaacagcctgggcaaaggccccaagatgggaaagccttggtggttggggcatagaatgggggggcagtggggccggccaagacaggaagggccttgaatgtgagggtgaaatgatggggtgtccctgggggccttactcccaactcagatcaagtcctttggtggcaggggctgccccggtcctctgacccagggcaagctctatgagcggtggagcccatcctagagattttcatagaccaggttaagttcgccatcatcttcgaatctatgcggtctctcctgggagagggggctctgcttggcggtgggtgagctgccatcctcattctcgatgcaggcatagacctcggtctcgcggcgctgcagagctgtgtagacagattctgaaggatgctgcttggggctgctggcagatcttggatctgggcacttcctggtggggtccttccctggaccccgcatccgcttcttgttccagagcagcagggccgtgcccactacactcaggacactcaggaggccggtgaagccaaagagcaggagcttctgtggactctgcgggggctctcggtaccctgcgtctctgaccaggatgaaggtgccgctgcctctcaccgtggagtgtggccagtggacagagcagtagtaggtgccagtggccgatgctcccggcagcacaagggtgacctggcagtccagggtgtggctctggttctctgtgcccagtccagggtggcagtttgttggcttcttagggctcctctgtccctggagatcttcatgaaagtagctgactgtgaaaaccttgaattggggagtgtatggataggtgatcctgcagctgaaggagatagctgtgttggccagggaggccatgatgggcaggccggtgtgggtcactgactgtcctcctgccagtcgcagggtcccgggcagcagcagcacgccaaggaggagccagggggctgcggggagcccaggagggcgtgggaggcctggcagggcccgccacctcacaggctggttctccatctgggggcctgcttgtctgcggcgactctttagttcacaggagggg

SEQ ID NO: 11533 - RNA, 4291 nt, Homo sapiens
  source 1..4291: mol_type = other RNA
ctgaatagctgggactacaggtgcgtgccaccacaccaggctaatttttgtatttttagtagagacggggtttcaccacgttggccaggctggtctcaaactcctggcctcaagtgatccacccgcctcggcctcccaacatgctgggattacaggcataagccactacgcctggcctgagctgtcttgactgtcactgcaaactgaggctcaggtggccagtgacttgcccaagtccacaaggctgtgggaggtggagcagggattcaagggaggccctgaggccacccagcctgggtgggtctcaaaagcaattttcttctcttccctcctccacccattcatagtggaaagcaagcctgcaccccaggagctcccattcataccctctctgtcccctctctgttcttcctcctcccgcctgccccatgcacctcccaccctgaagttccctgccacccctcgccctgtgccagcttgtctctgcaggctctcagtcctgggggctggagaacaggtgctcagtcctctttgctgcccacagaagtctcagaacattcttgccccaccctcccttgggccaaagccctttagggtcccgtcctttcatgctgtgctctcctcctcctcctcctcctccctgcctctctccttgctcactgaagacctcagcacccactgcctcccagccttgccctgaaccaagcacagacgaccaccacgctggcaatgtctctgtccaccagaggggtgatgggtcagcccccaagaacctcctacgccacagggaggagttggaattttattccaagtgaggcaaaaaccatgcaaggtatagagcaggggaggccaaggccaggtgtgggtttaatcggggtctgtcggtggcagggcagctgcagggaggccgtgttggtgatgcctgggccagggcacagtggtaaagtttaacccaggctcccctgtctacccctgaaaaagactggaaaatgctgagtcccagccaagggtccagggtctaggagctgaggtcagagaggcccaggaggtgggggaggcaggcccagtgaggtggccctctcctggtcttgctggcttcggttttcccaggggagctcactgcaccctgagcggcattgtcccccattgccctgacccttgcccccacctccttggctggtggagccaggagcctgggaggcccctgtgcacacctggcagcttcacctccccaaacaggcccggagttcattcaaatccagcctctgggagcaggggccttgccactcggttatgtgagcctgctaaagccctccttgccatgtgtgcttgcaggcgggggcccagaaccaagttgggaggccactggctgtcctgtgggaccagagaagtctggtgccaccctagcagggccaagggacttcttctggacgtcagtctgtgcccagcctctaccaccagctttcccttccctgcagggaggggcatgacctgcagaaccaaaggtgcttctgtgagccagtagcccagtgctgcttgggggcaggggcggggcctgtgccttgggttcccccccctccctgggcacatttggggttggggcagcccacacggtggggtgggaagattgacctgcccattttacaaatgagcaaaggtgggagaactcagggagacatgggggagcagagggaggaagcagagcccaacagcccggggcacccggaccccagccactgcctgcctgtggatgggtttctggccacggtgcagggctactgcgaggaggaaatgagggtgatgtgggcacctgaaacagcagaaatggctcagggccaggcactggggagccactgtccccatggggcttgagcttctgcctcagagggaccttccggctgccattgagggtcccagcaccaaaccccacagctggaccacttgggacctcaatccacagggggccagggctgcggcctatggcagataaagatagaggaggagggctggatgaagccacaggtggtgggcacaggataggccagacagaagggactttgggggactccaccttgggtagaaggagggacagctgaggtcctgtggtggagaaggcctggagcagagggtgaccaaggagatgacagagtgcacgtacagggccaggccaatgggagtgggaacccttgggagagggagcttcaggccattcattcagttcctgtttagccagcaccctcctcccctcatctgtccctctgccctcaccccaacatgccagaatctccttcctctccagcttgtacccaagccctctctgctccatgcccccagcctgctgaccacctctcagccatgtcctgggcctccagatctgtccctgatcctagtcttgcctctgaggggtccatcatccttgtctgtcccccagacctcccacgccagcccctgctcccaccctgcctggctgcctcgtgcctctggcccagctgggtaggtagggatttgcatagctgctccccagctcctccatacctcggctccccacacagcactgctaggcgcccctgcagggtcctccctcagctcagaggctgccctactggctgaggtgcaggctggtgccaagagagcatgctgctctgtcagcatgaggcagtgagcagggctctgggcaagggtggcatccaggaaagcccttgaagactgaggggcgctttgctggttgggccaagggaggaagggcctgcctggcagaaggaacagcctgggcaaaggccccaagatgggaaagccttggtggttggggcatagaatgggggggcagtggggccggccaagacaggaagggccttgaatgtgagggtgaaatgatggggtgtccctgggggccttactcccaactcagatcaagtcctttggtggcaggggctgccccggtcctctgacccagggcaagctctatgagcggtggagcccatcctagagattttcatagaccaggttaagttcgccatcatcttcgaatctatgcggtctctcctgggagagggggctctgcttggcggtgggtgagctgccatcctcattctcgatgcaggcatagacctcggtctcgcggcgctgcagagctgtgtagacagattctgaaggatgctgcttggggctgctggcagatcttggatctgggcacttcctggtggggtccttccctggaccccgcatccgcttcttgttccagagcagcagggccgtgcccactacactcaggacactcaggaggccggtgaagccaaagagcaggagcttctgtggactctgcgggggctctcggtaccctgcgtctctgaccaggatgaaggtgccgctgcctctcaccgtggagtgtggccagtggacagagcagtagtaggtgccagtggccgatgctcccggcagcacaagggtgacctggcagtccagggtgtggctctggttctctgtgcccagtccagggtggcagtttgttggcttcttagggctcctctgtccctggagatcttcatgaaagtagctgactgtgaaaaccttgaattggggagtgtatggataggtgatcctgcagctgaaggagatagctgtgttggccagggaggccatgatgggcaggccggtgtgggtcactgactgtcctcctgcttgaggtcacagaggggacccgggcttttctactggacacataccatggtccccctgctatgctcagtttctgggaggcagcaaggagctagtgccaactccccaaccccgccacaccaaaaggaatcttcaagatcatgttggccaggctggtctcgaactcctggcctcaagtgatctgcccgcctcggtctcccaaagtgctgggattacaggtgtgacctaccatacccggccacaattttcaacatttattccacgtccaccatgtgccaaggttctgggaggctcgggcccttgacacaaccatgtccctgagatttcctctccgtgacccttcttccccctctaggggtcctgggctgccctgaggccaccgcctagcaagatcaagatagggcttgagcggcagtgggatagggcagtgggggttccgggggggtccggtgcaggcagaaccaagagtgtgccggcggagggctgtcggtacagggtgcagggcgtggcggctgcaggacctcagcttgcctctttaaatcccttcctgggcaccgcggtggcccggccctttcccctcgtgctgtttctgctggaaacgccgcacagtctcctc

SEQ ID NO: 11534 - RNA, 3148 nt, Homo sapiens
  source 1..3148: mol_type = other RNA
ctgaatagctgggactacaggtgcgtgccaccacacccagctaatttttgtatttttagaagagacggggtttcaccgtgttagccaggatggtctcgatctcctgaccttgtgatccgcccgccttggcctcccaaagtgctgggattacaggcgtgagccaccatacctggccatctaaacttaattatctcccaaatgtcccatttccaaatatcatcacattgggggttagggcttcaacatatgaattttagggggatataattcagtccatagcactttgtcttttggtggacctgggtgctgggtgtggtcattactattggagtgtcattgctctcacatcagtgcaaaggactatacatacaaaaacatatttacatctatctctatagactgaaatacacgagttcacactgatatctccaattcgacaccacagggtttattctagttttctccctttccatatttgtgggagccaggtttttatgagacaattttattgggagataattctgtgtctcttgtgggtgtcttaattgtcagattttgtacgctttgaccaccatttaaattttttaaatgcaacaaaatatcaattttgttgatactttgtgggctgagatgttgacagattttgttccagactatttcaaggattttttttttcttgagatggagtttcactcttgttgcccaggctggagtgcaacggcgtgatcttggctcaccacaacctccgcctcctgggttcaagcgattctcctgcctcagcctcccgagtagctggattacaggctcgcgccaccacgcttggctaatttttgtatttttagtagagacgggatttctccatgttggtcaggctggtctggaactcccaacctcaggtgatccgcctgcctcagcctcccaaagtgctaggattataggtgtgccactgtgcccaggtatttcaaggatttttgtacagcaaatggccttagaagacagagatagtatctccctaagattgtggttccttagccgtcatgcaaacctgcagtgtgtaacactttcctgggcctgccagtattgccctgtgggacttggagggcaagggagaccaaggctaacacactgcctgctgtgccctgagcagtagtctctgcccaagtaatcctgtgttttctgccagcattcatgaagctggctccctaacacaagaagttgttgaaagttctactcagcttcttagctgcctcttccagaatcagcaggtgcccttatgggaaaagtagctctaagtcccaggctcacttctcttgagtttccttcgtgtcctgaattttggttctatattgccagctgatgctttcagatagatgctgtttatattttgcacagcttttctagttgttctctatgttcagtgggtccaaatttcctggtctaccattagtgaaagtggcagatggtgaaggcaattttcaactcaaaggtttcaaggccaccaaaaagagaaatacacatgtactgagaaagaaaagtcaagacctgtaagaagtgtcacaggtttcttaggtcacacatacaaaactgacccatatattcctgaaaatgaacagactgtctagtgccccagacccctgctatggataccctatttgaccttcaggcttagttccaaagccagctatatcttttataaaagactttccaccctatctccttcacctcctcacccagccaaaggaaaccttctttcctctgttctcccacaggactttatacctctgttagggcacttctccatctctgccacgttatagctggctgaccacccaaattcataattagcaacttgaggacccaatcatgtcttaaccatctttgcatttttcagtatgtcttgaatagagaatttatgaaaataaatgtttgcataagctgataaaggagatgaagaaaaacacacagaaggagaaaaccaagggtgtgggatcagaaaatccaagagaagagagtgtttctggagaatgaagcaataactgaatgctgctgagaagtcagaatgatgaagcctgaaaagtttcccctaaatgtggcagcataaaggattcaggagaacactgacttttattgaggaagacaggtcaaatgttgtttggagtcactgcattttttaggcaagtcaattagacaagcttctttttttttttttttgagacagaatgtcgcccaggctggagtgcaatggcacgatctcggctcactgcaccctctgcctcccaggttcaagcaattctcctgcctcagcctctgagtagctgggattacaggcatgcaccaccatgcctggctaattgttgtatttttagtagagatggggtttcaccatgttggtcaggctggtctcgaattcctgaccttgtgatccgcctgcctcggcctcccaaagtgctgggattataggcgtgagccaccgtgcccggcctggcaagcttcttcttgaagaaggatgaacagttctcagcaaagaggagtcatcattcttctgaaccaccataaacattccagagaagaggtagatagaaggctagatcctggaggatgtgctgtggtgagctaggccctcaggcaggtggtggtgcccagcagaaatggcactgtaagccaggcttccctggtcctaggagaatgttttagactagatgtctaggagaagtctgggcactaccactggtcttcatagacctgcatcaggctggtcctaggcctcctgttccagctacatagtggacacctccctctgggctatagcacacagggccacagcgcaactggggctcttcctcctcataccagcgctgttcactgaagtcagggaagaaggctgcaatctctctgctggctgaaaccacagagtccgaaccatgggtggtgttgcgggtgtcagtgaggccgaaactcccacggatagaatctggggccacatggcgtgctcggaacactctggtgggtcccatgagcgtcctccagagctggatggcatccttgtgggcaaggatgtaggctcggattggcccgcccagattctgggtcattcggagccccagtgcagcagaagtccggctgcgggttcaccttgtcctccggcaca

SEQ ID NO: 11535 - RNA, 3277 nt, Homo sapiens
  source 1..3277: mol_type = other RNA
ctgaatagctgggactacaggtgcgtgccaccacacccagctaatttttgtatttttagaagagacggggtttcaccgtgttagccaggatggtctcgatctcctgaccttgtgatccgcccgccttggcctcccaaagtgctgggattacaggcgtgagccaccatacctggccatctaaacttaattatctcccaaatgtcccatttccaaatatcatcacattgggggttagggcttcaacatatgaattttagggggatataattcagtccatagcactttgtcttttggtggacctgggtgctgggtgtggtcattactattggagtgtcattgctctcacatcagtgcaaaggactatacatacaaaaacatatttacatctatctctatagactgaaatacacgagttcacactgatatctccaattcgacaccacagggtttattctagttttctccctttccatatttgtgggagccaggtttttatgagacaattttattgggagataattctgtgtctcttgtgggtgtcttaattgtcagattttgtacgctttgaccaccatttaaattttttaaatgcaacaaaatatcaattttgttgatactttgtgggctgagatgttgacagattttgttccagactatttcaaggattttttttttcttgagatggagtttcactcttgttgcccaggctggagtgcaacggcgtgatcttggctcaccacaacctccgcctcctgggttcaagcgattctcctgcctcagcctcccgagtagctggattacaggctcgcgccaccacgcttggctaatttttgtatttttagtagagacgggatttctccatgttggtcaggctggtctggaactcccaacctcaggtgatccgcctgcctcagcctcccaaagtgctaggattataggtgtgccactgtgcccaggtatttcaaggatttttgtacagcaaatggccttagaagacagagatagtatctccctaagattgtggttccttagccgtcatgcaaacctgcagtgtgtaacactttcctgggcctgccagtattgccctgtgggacttggagggcaagggagaccaaggctaacacactgcctgctgtgccctgagcagtagtctctgcccaagtaatcctgtgttttctgccagcattcatgaagctggctccctaacacaagaagttgttgaaagttctactcagcttcttagctgcctcttccagaatcagcaggtgcccttatgggaaaagtagctctaagtcccaggctcacttctcttgagtttccttcgtgtcctgaattttggttctatattgccagctgatgctttcagatagatgctgtttatattttgcacagcttttctagttgttctctatgttcagtgggtccaaatttcctggtctaccattagtgaaagtggcagatggtgaaggcaattttcaactcaaaggtttcaaggccaccaaaaagagaaatacacatgtactgagaaagaaaagtcaagacctgtaagaagtgtcacaggtttcttaggtcacacatacaaaactgacccatatattcctgaaaatgaacagactgtctagtgccccagacccctgctatggataccctatttgaccttcaggcttagttccaaagccagctatatcttttataaaagactttccaccctatctccttcacctcctcacccagccaaaggaaaccttctttcctctgttctcccacaggactttatacctctgttagggcacttctccatctctgccacgttatagctggctgaccacccaaattcataattagcaacttgaggacccaatcatgtcttaaccatctttgcatttttcagtatgtcttgaatagagaatttatgaaaataaatgtttgcataagctgataaaggagatgaagaaaaacacacagaaggagaaaaccaagggtgtgggatcagaaaatccaagagaagagagtgtttctggagaatgaagcaataactgaatgctgctgagaagtcagaatgatgaagcctgaaaagtttcccctaaatgtggcagcataaaggattcaggagaacactgacttttattgaggaagacaggtcaaatgttgtttggagtcactgcattttttaggcaagtcaattagacaagcttctttttttttttttttgagacagaatgtcgcccaggctggagtgcaatggcacgatctcggctcactgcaccctctgcctcccaggttcaagcaattctcctgcctcagcctctgagtagctgggattacaggcatgcaccaccatgcctggctaattgttgtatttttagtagagatggggtttcaccatgttggtcaggctggtctcgaattcctgaccttgtgatccgcctgcctcggcctcccaaagtgctgggattataggcgtgagccaccgtgcccggcctggcaagcttcttcttgaagaaggatgaacagttctcagcaaagaggagtcatcattcttctgaaccaccataaacattccagagaagaggtagatagaaggctagatcctggaggatgtgctgtggtgagctaggccctcaggcaggtggtggtgcccagcagaaatggcactgtaagccaggcttccctggtcctaggagaatgttttagactagatgtctaggagaagtctgggcactaccactggtcttcatagacctgcatcaggctggtcctaggcctcctgttccagctacatagtggacacctccctctgggctatagcacacagggccacagcgcaactggggctcttcctcctcataccagcgctgttcactgaagtcagggaagaaggctgcaatctctctgctggctgaaaccacagagtccgaaccatgggtggtgttgcgggtgtcagtgaggccgaaactcccacggatagaatctggggccacatggcgtgctcggaacactctggtgggtcccatgagcgtcctccagagctggatggcatccttgtgggcaaggatgtaggctcggattggcccgctggccatgaactccaccagcctctgatagaaaaaacgccctgcaaagagagaggaccttcatcaagataccttcatcctggtgcccaaggcaactttctgtacttctacctccttaccttcatgctctcggtaaaacctctggcaatcttcctttctccacagtagttctctcattcgtacaatcaggaacttgttgctta

SEQ ID NO: 11536 - RNA, 3373 nt, Homo sapiens
  source 1..3373: mol_type = other RNA
ctgaatagctgggactacaggtgcgtgccaccacacccagctaatttttgtatttttagaagagacggggtttcaccgtgttagccaggatggtctcgatctcctgaccttgtgatccgcccgccttggcctcccaaagtgctgggattacaggcgtgagccaccatacctggccatctaaacttaattatctcccaaatgtcccatttccaaatatcatcacattgggggttagggcttcaacatatgaattttagggggatataattcagtccatagcactttgtcttttggtggacctgggtgctgggtgtggtcattactattggagtgtcattgctctcacatcagtgcaaaggactatacatacaaaaacatatttacatctatctctatagactgaaatacacgagttcacactgatatctccaattcgacaccacagggtttattctagttttctccctttccatatttgtgggagccaggtttttatgagacaattttattgggagataattctgtgtctcttgtgggtgtcttaattgtcagattttgtacgctttgaccaccatttaaattttttaaatgcaacaaaatatcaattttgttgatactttgtgggctgagatgttgacagattttgttccagactatttcaaggattttttttttcttgagatggagtttcactcttgttgcccaggctggagtgcaacggcgtgatcttggctcaccacaacctccgcctcctgggttcaagcgattctcctgcctcagcctcccgagtagctggattacaggctcgcgccaccacgcttggctaatttttgtatttttagtagagacgggatttctccatgttggtcaggctggtctggaactcccaacctcaggtgatccgcctgcctcagcctcccaaagtgctaggattataggtgtgccactgtgcccaggtatttcaaggatttttgtacagcaaatggccttagaagacagagatagtatctccctaagattgtggttccttagccgtcatgcaaacctgcagtgtgtaacactttcctgggcctgccagtattgccctgtgggacttggagggcaagggagaccaaggctaacacactgcctgctgtgccctgagcagtagtctctgcccaagtaatcctgtgttttctgccagcattcatgaagctggctccctaacacaagaagttgttgaaagttctactcagcttcttagctgcctcttccagaatcagcaggtgcccttatgggaaaagtagctctaagtcccaggctcacttctcttgagtttccttcgtgtcctgaattttggttctatattgccagctgatgctttcagatagatgctgtttatattttgcacagcttttctagttgttctctatgttcagtgggtccaaatttcctggtctaccattagtgaaagtggcagatggtgaaggcaattttcaactcaaaggtttcaaggccaccaaaaagagaaatacacatgtactgagaaagaaaagtcaagacctgtaagaagtgtcacaggtttcttaggtcacacatacaaaactgacccatatattcctgaaaatgaacagactgtctagtgccccagacccctgctatggataccctatttgaccttcaggcttagttccaaagccagctatatcttttataaaagactttccaccctatctccttcacctcctcacccagccaaaggaaaccttctttcctctgttctcccacaggactttatacctctgttagggcacttctccatctctgccacgttatagctggctgaccacccaaattcataattagcaacttgaggacccaatcatgtcttaaccatctttgcatttttcagtatgtcttgaatagagaatttatgaaaataaatgtttgcataagctgataaaggagatgaagaaaaacacacagaaggagaaaaccaagggtgtgggatcagaaaatccaagagaagagagtgtttctggagaatgaagcaataactgaatgctgctgagaagtcagaatgatgaagcctgaaaagtttcccctaaatgtggcagcataaaggattcaggagaacactgacttttattgaggaagacaggtcaaatgttgtttggagtcactgcattttttaggcaagtcaattagacaagcttctttttttttttttttgagacagaatgtcgcccaggctggagtgcaatggcacgatctcggctcactgcaccctctgcctcccaggttcaagcaattctcctgcctcagcctctgagtagctgggattacaggcatgcaccaccatgcctggctaattgttgtatttttagtagagatggggtttcaccatgttggtcaggctggtctcgaattcctgaccttgtgatccgcctgcctcggcctcccaaagtgctgggattataggcgtgagccaccgtgcccggcctggcaagcttcttcttgaagaaggatgaacagttctcagcaaagaggagtcatcattcttctgaaccaccataaacattccagagaagaggtagatagaaggctagatcctggaggatgtgctgtggtgagctaggccctcaggcaggtggtggtgcccagcagaaatggcactgtaagccaggcttccctggtcctaggagaatgttttagactagatgtctaggagaagtctgggcactaccactggtcttcatagacctgcatcaggctggtcctaggcctcctgttccagctacatagtggacacctccctctgggctatagcacacagggccacagcgcaactggggctcttcctcctcataccagcgctgttcactgaagtcagggaagaaggctgcaatctctctgctggctgaaaccacagagtccgaaccatgggtggtgttgcgggtgtcagtgaggccgaaactcccacggatagaatctggggccacatggcgtgctcggaacactctggtgggtcccatgagcgtcctccagagctggatggcatccttgtgggcaaggatgtaggctcggattggcccgctggccatgaactccaccagcctctgatagaaaaaacgcccttcatgctctcggtaaaacctctggcaatcttcctttctccacagtagttctctcattcgtacaatcaggaacttgttgcttagaatctgctgatgaacagcctccagaatcagtggatgggcgactgcgtcaggcttgatcagggctagagtgagctggagagcctgagggcttcgcaagattgaggccatctcactcctcatccagccattccaaggccaggctgctaggggttctcgtggcaagaacacgcggc

SEQ ID NO: 11537 - RNA, 3630 nt, Homo sapiens
  source 1..3630: mol_type = other RNA
ctgaatagctgggactacaggtgcgtgccaccacacccagctaatttttgtatttttagaagagacggggtttcaccgtgttagccaggatggtctcgatctcctgaccttgtgatccgcccgccttggcctcccaaagtgctgggattacaggcgtgagccaccatacctggccatctaaacttaattatctcccaaatgtcccatttccaaatatcatcacattgggggttagggcttcaacatatgaattttagggggatataattcagtccatagcactttgtcttttggtggacctgggtgctgggtgtggtcattactattggagtgtcattgctctcacatcagtgcaaaggactatacatacaaaaacatatttacatctatctctatagactgaaatacacgagttcacactgatatctccaattcgacaccacagggtttattctagttttctccctttccatatttgtgggagccaggtttttatgagacaattttattgggagataattctgtgtctcttgtgggtgtcttaattgtcagattttgtacgctttgaccaccatttaaattttttaaatgcaacaaaatatcaattttgttgatactttgtgggctgagatgttgacagattttgttccagactatttcaaggattttttttttcttgagatggagtttcactcttgttgcccaggctggagtgcaacggcgtgatcttggctcaccacaacctccgcctcctgggttcaagcgattctcctgcctcagcctcccgagtagctggattacaggctcgcgccaccacgcttggctaatttttgtatttttagtagagacgggatttctccatgttggtcaggctggtctggaactcccaacctcaggtgatccgcctgcctcagcctcccaaagtgctaggattataggtgtgccactgtgcccaggtatttcaaggatttttgtacagcaaatggccttagaagacagagatagtatctccctaagattgtggttccttagccgtcatgcaaacctgcagtgtgtaacactttcctgggcctgccagtattgccctgtgggacttggagggcaagggagaccaaggctaacacactgcctgctgtgccctgagcagtagtctctgcccaagtaatcctgtgttttctgccagcattcatgaagctggctccctaacacaagaagttgttgaaagttctactcagcttcttagctgcctcttccagaatcagcaggtgcccttatgggaaaagtagctctaagtcccaggctcacttctcttgagtttccttcgtgtcctgaattttggttctatattgccagctgatgctttcagatagatgctgtttatattttgcacagcttttctagttgttctctatgttcagtgggtccaaatttcctggtctaccattagtgaaagtggcagatggtgaaggcaattttcaactcaaaggtttcaaggccaccaaaaagagaaatacacatgtactgagaaagaaaagtcaagacctgtaagaagtgtcacaggtttcttaggtcacacatacaaaactgacccatatattcctgaaaatgaacagactgtctagtgccccagacccctgctatggataccctatttgaccttcaggcttagttccaaagccagctatatcttttataaaagactttccaccctatctccttcacctcctcacccagccaaaggaaaccttctttcctctgttctcccacaggactttatacctctgttagggcacttctccatctctgccacgttatagctggctgaccacccaaattcataattagcaacttgaggacccaatcatgtcttaaccatctttgcatttttcagtatgtcttgaatagagaatttatgaaaataaatgtttgcataagctgataaaggagatgaagaaaaacacacagaaggagaaaaccaagggtgtgggatcagaaaatccaagagaagagagtgtttctggagaatgaagcaataactgaatgctgctgagaagtcagaatgatgaagcctgaaaagtttcccctaaatgtggcagcataaaggattcaggagaacactgacttttattgaggaagacaggtcaaatgttgtttggagtcactgcattttttaggcaagtcaattagacaagcttctttttttttttttttgagacagaatgtcgcccaggctggagtgcaatggcacgatctcggctcactgcaccctctgcctcccaggttcaagcaattctcctgcctcagcctctgagtagctgggattacaggcatgcaccaccatgcctggctaattgttgtatttttagtagagatggggtttcaccatgttggtcaggctggtctcgaattcctgaccttgtgatccgcctgcctcggcctcccaaagtgctgggattataggcgtgagccaccgtgcccggcctggcaagcttcttcttgaagaaggatgaacagttctcagcaaagaggagtcatcattcttctgaaccaccataaacattccagagaagaggtagatagaaggctagatcctggaggatgtgctgtggtgagctaggccctcaggcaggtggtggtgcccagcagaaatggcactgtaagccaggcttccctggtcctaggagaatgttttagactagatgtctaggagaagtctgggcactaccactggtcttcatagacctgcatcaggctggtcctaggcctcctgttccagctacatagtggacacctccctctgggctatagcacacagggccacagcgcaactggggctcttcctcctcataccagcgctgttcactgaagtcagggaagaaggctgcaatctctctgctggctgaaaccacagagtccgaaccatgggtggtgttgcgggtgtcagtgaggccgaaactcccacggatagaatctggggccacatggcgtgctcggaacactctggtgggtcccatgagcgtcctccagagctggatggcatccttgtgggcaaggatgtaggctcggattggcccgctggccatgaactccaccagcctctgatagaaaaaacgcccttcatgctctcggtaaaacctctggcaatcttcctttctccacagtagttctctcattcgtacaatcaggaacttgttgcttagaatctgctgatgaacagcctccagaatcagtggatgggcgactgcgtcaggcttgatcagggctagagtgagctggagagcctgagggcttcgcaagattgaggccatctcactccttagtgatcttagctcacttcccgttacactttctcacagctccttgcaagttcccttcagttccgtcttcaccaccagaaggtgtaagcagtacctagcacacagctggctcttaacagtatctgaatgaaccaacgaatgcacctcatccagccattccaaggccaggctgctaggggttctcgtggcaagaacacgcggcccctcgtacccggggcctaagcccaccccagattctgggtcattcggagccccagtgcagcagaagtccggctgcgggttcaccttgtcctccggcacagggcccggccac

SEQ ID NO: 11538 - RNA, 3386 nt, Homo sapiens
  source 1..3386: mol_type = other RNA
ctgaatagctgggactacaggtgcgtgccaccacacccagctaatttttgtatttttagaagagacggggtttcaccgtgttagccaggatggtctcgatctcctgaccttgtgatccgcccgccttggcctcccaaagtgctgggattacaggcgtgagccaccatacctggccatctaaacttaattatctcccaaatgtcccatttccaaatatcatcacattgggggttagggcttcaacatatgaattttagggggatataattcagtccatagcactttgtcttttggtggacctgggtgctgggtgtggtcattactattggagtgtcattgctctcacatcagtgcaaaggactatacatacaaaaacatatttacatctatctctatagactgaaatacacgagttcacactgatatctccaattcgacaccacagggtttattctagttttctccctttccatatttgtgggagccaggtttttatgagacaattttattgggagataattctgtgtctcttgtgggtgtcttaattgtcagattttgtacgctttgaccaccatttaaattttttaaatgcaacaaaatatcaattttgttgatactttgtgggctgagatgttgacagattttgttccagactatttcaaggattttttttttcttgagatggagtttcactcttgttgcccaggctggagtgcaacggcgtgatcttggctcaccacaacctccgcctcctgggttcaagcgattctcctgcctcagcctcccgagtagctggattacaggctcgcgccaccacgcttggctaatttttgtatttttagtagagacgggatttctccatgttggtcaggctggtctggaactcccaacctcaggtgatccgcctgcctcagcctcccaaagtgctaggattataggtgtgccactgtgcccaggtatttcaaggatttttgtacagcaaatggccttagaagacagagatagtatctccctaagattgtggttccttagccgtcatgcaaacctgcagtgtgtaacactttcctgggcctgccagtattgccctgtgggacttggagggcaagggagaccaaggctaacacactgcctgctgtgccctgagcagtagtctctgcccaagtaatcctgtgttttctgccagcattcatgaagctggctccctaacacaagaagttgttgaaagttctactcagcttcttagctgcctcttccagaatcagcaggtgcccttatgggaaaagtagctctaagtcccaggctcacttctcttgagtttccttcgtgtcctgaattttggttctatattgccagctgatgctttcagatagatgctgtttatattttgcacagcttttctagttgttctctatgttcagtgggtccaaatttcctggtctaccattagtgaaagtggcagatggtgaaggcaattttcaactcaaaggtttcaaggccaccaaaaagagaaatacacatgtactgagaaagaaaagtcaagacctgtaagaagtgtcacaggtttcttaggtcacacatacaaaactgacccatatattcctgaaaatgaacagactgtctagtgccccagacccctgctatggataccctatttgaccttcaggcttagttccaaagccagctatatcttttataaaagactttccaccctatctccttcacctcctcacccagccaaaggaaaccttctttcctctgttctcccacaggactttatacctctgttagggcacttctccatctctgccacgttatagctggctgaccacccaaattcataattagcaacttgaggacccaatcatgtcttaaccatctttgcatttttcagtatgtcttgaatagagaatttatgaaaataaatgtttgcataagctgataaaggagatgaagaaaaacacacagaaggagaaaaccaagggtgtgggatcagaaaatccaagagaagagagtgtttctggagaatgaagcaataactgaatgctgctgagaagtcagaatgatgaagcctgaaaagtttcccctaaatgtggcagcataaaggattcaggagaacactgacttttattgaggaagacaggtcaaatgttgtttggagtcactgcattttttaggcaagtcaattagacaagcttctttttttttttttttgagacagaatgtcgcccaggctggagtgcaatggcacgatctcggctcactgcaccctctgcctcccaggttcaagcaattctcctgcctcagcctctgagtagctgggattacaggcatgcaccaccatgcctggctaattgttgtatttttagtagagatggggtttcaccatgttggtcaggctggtctcgaattcctgaccttgtgatccgcctgcctcggcctcccaaagtgctgggattataggcgtgagccaccgtgcccggcctggcaagcttcttcttgaagaaggatgaacagttctcagcaaagaggagtcatcattcttctgaaccaccataaacattccagagaagaggtagatagaaggctagatcctggaggatgtgctgtggtgagctaggccctcaggcaggtggtggtgcccagcagaaatggcactgtaagccaggcttccctggtcctaggagaatgttttagactagatgtctaggagaagtctgggcactaccactggtcttcatagacctgcatcaggctggtcctaggcctcctgttccagctacatagtggacacctccctctgggctatagcacacagggccacagcgcaactggggctcttcctcctcataccagcgctgttcactgaagtcagggaagaaggctgcaatctctctgctggctgaaaccacagagtccgaaccatgggtggtgttgcgggtgtcagtgaggccgaaactcccacggatagaatctggggccacatggcgtgctcggaacactctggtgggtcccatgagcgtcctccagagctggatggcatccttgtgggcaaggatgtaggctcggattggcccgcttcatgctctcggtaaaacctctggcaatcttcctttctccacagtagttctctcattcgtacaatcaggaacttgttgcttagaatctgctgatgaacagcctccagaatcagtggatgggcgactgcgtcaggcttgatcagggctagagtgagctggagagcctgagggcttcgcaagattgaggccatctcactcccctcgtacccggggcctaagcccaccccagattctgggtcattcggagccccagtgcagcagaagtccggctgcgggttcaccttgtcctccggcacagggcccggccac

SEQ ID NO: 11539 - RNA, 4627 nt, Homo sapiens
  source 1..4627: mol_type = other RNA
ctgaatagctgggactacaggtgcgtgccaccacacccagctaatttttgtatttttagaagagacggggtttcaccgtgttagccaggatggtctcgatctcctgaccttgtgatccgcccgccttggcctcccaaagtgctgggattacaggcgtgagccaccatacctggccatctaaacttaattatctcccaaatgtcccatttccaaatatcatcacattgggggttagggcttcaacatatgaattttagggggatataattcagtccatagcactttgtcttttggtggacctgggtgctgggtgtggtcattactattggagtgtcattgctctcacatcagtgcaaaggactatacatacaaaaacatatttacatctatctctatagactgaaatacacgagttcacactgatatctccaattcgacaccacagggtttattctagttttctccctttccatatttgtgggagccaggtttttatgagacaattttattgggagataattctgtgtctcttgtgggtgtcttaattgtcagattttgtacgctttgaccaccatttaaattttttaaatgcaacaaaatatcaattttgttgatactttgtgggctgagatgttgacagattttgttccagactatttcaaggattttttttttcttgagatggagtttcactcttgttgcccaggctggagtgcaacggcgtgatcttggctcaccacaacctccgcctcctgggttcaagcgattctcctgcctcagcctcccgagtagctggattacaggctcgcgccaccacgcttggctaatttttgtatttttagtagagacgggatttctccatgttggtcaggctggtctggaactcccaacctcaggtgatccgcctgcctcagcctcccaaagtgctaggattataggtgtgccactgtgcccaggtatttcaaggatttttgtacagcaaatggccttagaagacagagatagtatctccctaagattgtggttccttagccgtcatgcaaacctgcagtgtgtaacactttcctgggcctgccagtattgccctgtgggacttggagggcaagggagaccaaggctaacacactgcctgctgtgccctgagcagtagtctctgcccaagtaatcctgtgttttctgccagcattcatgaagctggctccctaacacaagaagttgttgaaagttctactcagcttcttagctgcctcttccagaatcagcaggtgcccttatgggaaaagtagctctaagtcccaggctcacttctcttgagtttccttcgtgtcctgaattttggttctatattgccagctgatgctttcagatagatgctgtttatattttgcacagcttttctagttgttctctatgttcagtgggtccaaatttcctggtctaccattagtgaaagtggcagatggtgaaggcaattttcaactcaaaggtttcaaggccaccaaaaagagaaatacacatgtactgagaaagaaaagtcaagacctgtaagaagtgtcacaggtttcttaggtcacacatacaaaactgacccatatattcctgaaaatgaacagactgtctagtgccccagacccctgctatggataccctatttgaccttcaggcttagttccaaagccagctatatcttttataaaagactttccaccctatctccttcacctcctcacccagccaaaggaaaccttctttcctctgttctcccacaggactttatacctctgttagggcacttctccatctctgccacgttatagctggctgaccacccaaattcataattagcaacttgaggacccaatcatgtcttaaccatctttgcatttttcagtatgtcttgaatagagaatttatgaaaataaatgtttgcataagctgataaaggagatgaagaaaaacacacagaaggagaaaaccaagggtgtgggatcagaaaatccaagagaagagagtgtttctggagaatgaagcaataactgaatgctgctgagaagtcagaatgatgaagcctgaaaagtttcccctaaatgtggcagcataaaggattcaggagaacactgacttttattgaggaagacaggtcaaatgttgtttggagtcactgcattttttaggcaagtcaattagacaagcttctttttttttttttttgagacagaatgtcgcccaggctggagtgcaatggcacgatctcggctcactgcaccctctgcctcccaggttcaagcaattctcctgcctcagcctctgagtagctgggattacaggcatgcaccaccatgcctggctaattgttgtatttttagtagagatggggtttcaccatgttggtcaggctggtctcgaattcctgaccttgtgatccgcctgcctcggcctcccaaagtgctgggattataggcgtgagccaccgtgcccggcctggcaagcttcttcttgaagaaggatgaacagttctcagcaaagaggagtcatcattcttctgaaccaccataaacattccagagaagaggtagatagaaggctagatcctggaggatgtgctgtggtgagctaggccctcaggcaggtggtggtgcccagcagaaatggcactgtaagccaggcttccctggtcctaggagaatgttttagactagatgtctaggagaagtctgggcactaccactggtcttcatagacctgcatcaggctggtcctaggcctcctgttccagctacatagtggacacctccctctgggctatagcacacagggccacagcgcaactggggctcttcctcctcataccagcgctgttcactgaagtcagggaagaaggctgcaatctctctgctggctgaaaccacagagtccgaaccatgggtggtgttgcgggtgtcagtgaggccgaaactcccacggatagaatctggggccacatggcgtgctcggaacactctggtgggtcccatgagcgtcctccagagctggatggcatccttgtgggcaaggatgtaggctcggattggcccgcttgtcctccggcacagggcccggccaccaggcgccacgctggatagcctgcggccctcgcagggtccttcaggcgctccctgggcagccctgctcggggtcctagtccggttgcgccgcggcgtgaggtgaggtgtgagttgccctggagggtggcgggttttccaggcgcatgcatttgccgcggacgggacgagaggatgaagccgttctgggcgccggaactcgcttgtgggaaccgcccctcggaagccggcctgggcgccctcggaagccggcctgggcgccctcggcgggagggagtgctgggccgggtgctggcgcagcgctacgcagggtggcggaacccagaggaccggacgggctcgttcagggtggcggcccggcgggggcgatgcccgccagcagagacaccgatggaaaccttgcccagttattttctttgcccagggtagttcctggaacatggttgatgcccagtatttgtcaaaagtacgcggagggcaaagaacttaagcgctcgatagcgaaggcacaggcccttcaaagtcttttgagctctgagcgatacattagcatgaaggatcgtagctaatatgggggttgatgaaggaggatccttggctggagcccaggtgtgcatagggcatgaggaaagcaagtcataacggcctttcacgtgtcattaggaatctgggcagcagggtgtggtttgggttactctggagtctattgacgcagcccagggtgaggagatgagaactgggggtattcctggtgtgtactgtgatgtatggagaggatggggacagggagaatggatcgggggtcagctgtggcaggtgaccagaaacttggtgacaggttgaataaagatggttaaaaaaaaaaaaagtgttttggtttcttgggtttttttttttttttttgagggaaatcactgagaatgagaagaatgaaaataaacgataactgtcatcaatgtaaagacttacttgcacatttaactgacttcggtgtctgcctacacaggtgttgccctcttggaaggtttatccccaactcatggcttctgtccctgcagcaataagaagccacttcccaatagtttcctgatacccagtcacctttgggaacttacgaggaaagtttttccagtctctccgcagacccttgcatctcttctctttttgtttagacccttgaccaccaccccctattctaatcttaactcctctgctactcagttccaatcctaacccaagccctagtccctaaatttataatcctttaatcctagacctggtctctagatcctgagcccttgatgcttatcttctaacctcctaatcccaacctcaaatccctaaacctcaacccatgaattctgacctgattctcaaaccccaggcccccaaccctgactccaaaaatgacaacccattacttctccctacacggaatcactgacggagttgtagcaactgaatctgcagtaggccaaaggacccagtgagttagccagcaaactactctaaataaaagatatggt

SEQ ID NO: 11540 - RNA, 2529 nt, Homo sapiens
  source 1..2529: mol_type = other RNA
ctgaatagctgggactacaggtgcgtgccaccacacccagctaatttttgtatttttggtagagacggggtttcaccatgttggtcaggatagtctcaatctcttgaccttgtgatccacctgcctcagcctcccaaactgctaggattacaggcgtgagccactgcgccaggccttctcagcagctcttgtgggaacacagaaagggaattcaaaatttggctacctctcccactcatgtgatcagggaagaataggcttatgagagacctaaaaaaatcttccgagcagccttggatttaaagtcatagcgctgtttaaaataaagtaatatggcaatctggaatgtctccaagaaaagtcattttgttctgtcactgacatctgtactatttgtttgaatgttgtttttgtaaacagttgtagattaaagaagtttttacagatcaatgagtaaaatgttcatttaataactttctaactgtatacagtatatgcttgatagttcaaaattctccaaatgtagatattatacaataattattttaaattattaaatgagtatttaatccttttaaattacattttgaaaatttaatggcaattacacacaaattttaatttaaaataatattaaggacttaatctgatttacagaaatgaaatgcaatgaagagattaagggctaacctccattactataaaattctctggctaccatctagcacaggagcaactggattgctttcagcagtcttgaagcactaaaatatcttaaaattcatatggagaaatagtatgtatctctacattaaatttagatttgatatttattctctgacagatcagacccagaatattaatttttatgtaattgaaccaaaaacatttagcaatccttcatttagtaatcttttgtataaatataaaaatctctgataagtgaaatgttttttcaaattatacttctatttttcacagctttataggtaattataattttcaaactttaaatatttcatgtgatttgatatatctgtacagaaagagtaagataaaaacatttaataagattaaatctaatttgcaaaaattggtatctgacatttgttgtgtgctcttgcaaagagtgcataggacatttctgcagcaatcaaaaaggtaaaatctttttaaactcagatttcaagtttcctctaatattccttctaatcctaatccctggaaatactttcaagttttgatttctagatgcaatgtgttttgttacatatacacatgtcttatccttaaacttttaaaaaacagtatgatcagattcagcatgatgatatcttctcagactctgtagaagtcctctgtgcaagattaatgtcgagattcctagtgccccatcgtgaaaaaccagttaaagatagtatacaactatgctttagtgggatttcctgcaggtttgggatcataaccatacaaaaaagtagctgttattacaaggatggctccaaggaaaaagacacaagctgaatatttcttatccacactgattgttttgtttcttttaagattttctcaaagtaaaccccagcaaagccacttgaaaaacatgctgtgagaactgccatgagtcctacaaattgagaaccagctgaaagttccttagaatcaagctgagaatctgagggccactgtacaaaagcaactcctgtcatcaaaattactagggacagccactggtatacacccaattttttactaagcatagacacagaaaataatgctgttgtaagaatttttaactgatacgtgacctgataagtagctgcatctagatttgatagtgccacatacagtaaattattctgaagagtatagatccctgatggaatagcaagtttaagtgtttccataggtttattaagaatttcatcatgtagtactcgattcagtgctcttagactacatttgctgtctttgtagaccaataaaatgcaggccattatcttcaaaagttcagcaacaaccactgctgtagaagatagataacgaggtccttcttcttttaaagttctggaataacgcattgttagaaccaaactggtagtctgaaagaccaaaattcccagggaaacgtattttaggttggcgaacattgttttatcttcatttgccaagggcagcctttccatttctttaagttcctgcggcttcttgagctccaggtgctggtcgggtgcatctgtgcctaccacagggctcaacaccgagcgagagctcatgggatgttcactgaaggaatgacgggccccagccgggcccacccgtcactagctccgcacgcaccaggcgctgaggcacacactgccgtcttcattcgcttgacacacccctctcctcgggccttttttcctcctccacccagtacattccgcacgtcgtccgtcggagttacaacgtgtcacctcatctgctcccacccctacttagctagcactgtatttcaggtcttcgataccgtccccttcaccccta

SEQ ID NO: 11541 - RNA, 2335 nt, Homo sapiens
  source 1..2335: mol_type = other RNA
ctgaatagctgggactacaggtgcgtgccaccacacccagctaatttttgtatttttggtagagacggggtttcaccatgttggtcaggatagtctcaatctcttgaccttgtgatccacctgcctcagcctcccaaactgctaggattacaggcgtgagccactgcgccaggccttctcagcagctcttgtgggaacacagaaagggaattcaaaatttggctacctctcccactcatgtgatcagggaagaataggcttatgagagacctaaaaaaatcttccgagcagccttggatttaaagtcatagcgctgtttaaaataaagtaatatggcaatctggaatgtctccaagaaaagtcattttgttctgtcactgacatctgtactatttgtttgaatgttgtttttgtaaacagttgtagattaaagaagtttttacagatcaatgagtaaaatgttcatttaataactttctaactgtatacagtatatgcttgatagttcaaaattctccaaatgtagatattatacaataattattttaaattattaaatgagtatttaatccttttaaattacattttgaaaatttaatggcaattacacacaaattttaatttaaaataatattaaggacttaatctgatttacagaaatgaaatgcaatgaagagattaagggctaacctccattactataaaattctctggctaccatctagcacaggagcaactggattgctttcagcagtcttgaagcactaaaatatcttaaaattcatatggagaaatagtatgtatctctacattaaatttagatttgatatttattctctgacagatcagacccagaatattaatttttatgtaattgaaccaaaaacatttagcaatccttcatttagtaatcttttgtataaatataaaaatctctgataagtgaaatgttttttcaaattatacttctatttttcacagctttataggtaattataattttcaaactttaaatatttcatgtgatttgatatatctgtacagaaagagtaagataaaaacatttaataagattaaatctaatttgcaaaaattggtatctgacatttgttgtgtgctcttgcaaagagtgcataggacatttctgcagcaatcaaaaaggtaaaatctttttaaactcagatttcaagtttcctctaatattccttctaatcctaatccctggaaatactttcaagttttgatttctagatgcaatgtgttttgttacatatacacatgtcttatccttaaacttttaaaaaacagtatgatcagattcagcatgatgatatcttctcagactctgtagaagtcctctgtgcaagattaatgtcgagattcctagtgccccatcgtgaaaaaccagttaaagatagtatacaactatgctttagtgggatttcctgcaggtttgggatcataaccatacaaaaaagtagctgttattacaaggatggctccaaggaaaaagacacaagctgaatatttcttatccacactgattgttttgtttcttttaagattttctcaaagtaaaccccagcaaagccacttgaaaaacatgctgtgagaactgccatgagtcctacaaattgagaaccagctgaaagttccttagaatcaagctgagaatctgagggccactgtacaaaagcaactcctgtcatcaaaattactagggacagccactggtatacacccaattttttactaagcatagacacagaaaataatgctgttgtaagaatttttaactgatacgtgacctgataagtagctgcatctagatttgatagtgccacatacagtaaattattctgaagagtatagatccctgatggaatagcaagtttaagtgtttccataggtttattaagaatttcatcatgtagtactcgattcagtgctcttagactacatttgctgtctttgtagaccaataaaatgcaggccattatcttcaaaagttcagcaacaaccactgctgtagaagatagataacgaggtccttcttcttttaaagttctggaataacgcattgttagaaccaaactggtagtctgaaagaccaaaattcccagggaaacgtattttaggttggcgaacattgttttatcttcatttgcctcccgcgcagctcgaccggctgagcccaccaccgggggccgcggttcagctccgccgggcgccccaggctgccgagtccgctgggtcctacgcgaccgctgacccgcagcgccgccggctcccgtcgccgtagccaccgccagctcggtgcagcccaggcgtttcc

SEQ ID NO: 11542 - RNA, 3926 nt, Homo sapiens
  source 1..3926: mol_type = other RNA
ctgaatagctgggactacaggtgcgtgccaccacacccagctaatttttgtatttttggtagagacggggtttcaccatgttggtcaggatagtctcaatctcttgaccttgtgatccacctgcctcagcctcccaaactgctaggattacaggcgtgagccactgcgccaggccttctcagcagctcttgtgggaacacagaaagggaattcaaaatttggctacctctcccactcatgtgatcagggaagaataggcttatgagagacctaaaaaaatcttccgagcagccttggatttaaagtcatagcgctgtttaaaataaagtaatatggcaatctggaatgtctccaagaaaagtcattttgttctgtcactgacatctgtactatttgtttgaatgttgtttttgtaaacagttgtagattaaagaagtttttacagatcaatgagtaaaatgttcatttaataactttctaactgtatacagtatatgcttgatagttcaaaattctccaaatgtagatattatacaataattattttaaattattaaatgagtatttaatccttttaaattacattttgaaaatttaatggcaattacacacaaattttaatttaaaataatattaaggacttaatctgatttacagaaatgaaatgcaatgaagagattaagggctaacctccattactataaaattctctggctaccatctagcacaggagcaactggattgctttcagcagtcttgaagcactaaaatatcttaaaattcatatggagaaatagtatgtatctctacattaaatttagatttgatatttattctctgacagatcagacccagaatattaatttttatgtaattgaaccaaaaacatttagcaatccttcatttagtaatcttttgtataaatataaaaatctctgataagtgaaatgttttttcaaattatacttctatttttcacagctttataggtaattataattttcaaactttaaatatttcatgtgatttgatatatctgtacagaaagagtaagataaaaacatttaataagattaaatctaatttgcaaaaattggtatctgacatttgttgtgtgctcttgcaaagagtgcataggacatttctgcagcaatcaaaaaggtaaaatctttttaaactcagatttcaagtttcctctaatattccttctaatcctaatccctggaaatactttcaagttttgatttctagatgcaatgtgttttgttacatatacacatgtcttatccttaaacttttaaaaaacagtatgatcagattcagcatgatgatatcttctcagactctgtagaagtcctctgtgcaagattaatgtcgagattcctagtgccccatcgtgaaaaaccagttaaagatagtatacaactatgctttagtgggatttcctgcaggtttgggatcataaccatacaaaaaagtagctgttattacaaggatggctccaaggaaaaagacactgaagaacaactactatccaggtcagtcggttatatccctgaaaaaatccattctttgataccagttctccatcataaatgtatacacccattaatccaaatatacttccaaagaaaccaagctgaatatttcttatccacactgattgttttgtttcttttaagattttctcaaagtaaaccccagcaaagccacttgaaaaacatgctgtgagaactgccatgagtcctacaaattgagaaccagctgaaagttccttagaatcaagctgagaatctgagggccactgataagtagctgcatctagatttgatagtgccacatacagtaaattattctgaagagtatagatccctgatggaatagcaagtttaagtgtttccataggtttattaagaatttcatcatgtagtactcgattcagtgctcttagactacatttgctgtctttgtagaccaataaaatgcaggccattatcttcaaaagttcagcaacaaccactgctgtagaagatagataacgaggtccttcttcttttaaagttctggaataacgcattgttagaaccaaactggtagtctgaaagaccaaaattcccagggaaacgtattttaggttggcgaacattgttttatcttcatttgcctcccgcgcagctcgaccggctgagcccaccaccgggggccgcggttcagctccgccgggcgccccaggctgccgagtccgctgggtcctacgcgaccgctgacccgcagcgccgccggctcccgtcgccgtagccaccgccagctcggtgcagcccaggcgtttccgggttcccgcggtcccgtcccccaaatgctccggcttccgcctcggctctggcaaatgccgttcccggctcggctctggcagccccagctcggcacttggcagctctgtccctaaggcgacgcacctgggctgctctgctggcagcccctggttcctgcttcaccgtcgcgtggaggcctggggcactgctttctgctacacctctcctaggagcgcgaaacagatggagtgacactcgtcgagggcctctgcgggactgtctgtttgcagagggtgccaaggtgtccactgcgtaaggaagggcaaagtcctttggggcaaagaaccctgagaggaacggggagatggattttgaaagcaaacgaaccctctcctaaaagtgactgtcactgacctgaaaacaaccagattagctatggcaaaggctgccaaccaaccagtggtctgcaagaaggcttgttcttccacttcacccaccctgactgagatcttgagactgaaggaaacccaaagccgtaccaccaatgggcctagtgtcatcaaccgggagaggaaaaagaaaactgggcccagaggattgcagagttatgagggaccaaccccttcctggctgcatggatcacagcattaccttttaaaagtgttccagtagctgtgttggaaaccctctaaccacggcagcccattcaggtgatgaacaggctgaaatcagtacttcaggttcagctggattatcaaataagcgaataggattatctctttttgttaactcagggctgctataaattaagcctatgtctctttatattgcaaatgattaaaaccatgtccaagagagacatacttagaaaaaaagtgatattgaagaaaaataagtaactgtattagagtagaataactggttttaaaattttctgcaatacagtcttgagaaaattcctggatggtaaaatacatattagatcttaatacatgcccagttttttttgaaaccaaaatgtgcctgttagatgatgataacagcatgcctcgttttattgtgatttgctttattgctcttcacagacattgcttttgtttttttgttttttttttttacaaattgaaggtttgtggcaaccttgcctcaagcacatctattggtgccatttttccaacagcatgtgctcactttgtgtctctgtgtcacataatattcaataatttttgcaatatttaaatttgttcatcattattatatctggtatagtgctttgtgatcaatgatctttgatgttactatggtaattgttttggggtgctgatatggtttggctgtgtccccacccaaatctcaacttgaactgtatctcccagaattcccacgtgttgagggagagacctagggggagataattgaatcatgggggccagtctttcctgtgctattctcatgatagtgaataagtctcatgaaatccgatgggtttatctggggtttctgattttgcttcttcctcatttttctcttgctgcagccatgtaagcaagtacctttcacctcccgccatgattctgaggcctcccccgccatgtggaactgtaggtccaatta

SEQ ID NO: 11543 - RNA, 2638 nt, Homo sapiens
  source 1..2638: mol_type = other RNA
ctgaatagctgggactacaggtgcgtgccaccacacccagctaatttttgtatttttggtagagacggggtttcaccatgttggtcaggatagtctcaatctcttgaccttgtgatccacctgcctcagcctcccaaactgctaggattacaggcgtgagccactgcgccaggccttctcagcagctcttgtgggaacacagaaagggaattcaaaatttggctacctctcccactcatgtgatcagggaagaataggcttatgagagacctaaaaaaatcttccgagcagccttggatttaaagtcatagcgctgtttaaaataaagtaatatggcaatctggaatgtctccaagaaaagtcattttgttctgtcactgacatctgtactatttgtttgaatgttgtttttgtaaacagttgtagattaaagaagtttttacagatcaatgagtaaaatgttcatttaataactttctaactgtatacagtatatgcttgatagttcaaaattctccaaatgtagatattatacaataattattttaaattattaaatgagtatttaatccttttaaattacattttgaaaatttaatggcaattacacacaaattttaatttaaaataatattaaggacttaatctgatttacagaaatgaaatgcaatgaagagattaagggctaacctccattactataaaattctctggctaccatctagcacaggagcaactggattgctttcagcagtcttgaagcactaaaatatcttaaaattcatatggagaaatagtatgtatctctacattaaatttagatttgatatttattctctgacagatcagacccagaatattaatttttatgtaattgaaccaaaaacatttagcaatccttcatttagtaatcttttgtataaatataaaaatctctgataagtgaaatgttttttcaaattatacttctatttttcacagctttataggtaattataattttcaaactttaaatatttcatgtgatttgatatatctgtacagaaagagtaagataaaaacatttaataagattaaatctaatttgcaaaaattggtatctgacatttgttgtgtgctcttgcaaagagtgcataggacatttctgcagcaatcaaaaaggtaaaatctttttaaactcagatttcaagtttcctctaatattccttctaatcctaatccctggaaatactttcaagttttgatttctagatgcaatgtgttttgttacatatacacatgtcttatccttaaacttttaaaaaacagtatgatcagattcagcatgatgatatcttctcagactctgtagaagtcctctgtgcaagattaatgtcgagattcctagtgccccatcgtgaaaaaccagttaaagatagtatacaactatgctttagtgggatttcctgcaggtttgggatcataaccatacaaaaaagtagctgttattacaaggatggctccaaggaaaaagacactgaagaacaactactatccaggtcagtcggttatatccctgaaaaaatccattctttgataccagttctccatcataaatgtatacacccattaatccaaatatacttccaaagaaaccaagctgaatatttcttatccacactgattgttttgtttcttttaagattttctcaaagtaaaccccagcaaagccacttgaaaaacatgctgtgagaactgccatgagtcctacaaattgagaaccagctgaaagttccttagaatcaagctgagaatctgagggccactgtacaaaagcaactcctgtcatcaaaattactagggacagccactggtatacacccaattttttactaagcatagacacagaaaataatgctgttgtaagaatttttaactgatacgtgacctgataagtagctgcatctagatttgatagtgccacatacagtaaattattctgaagagtatagatccctgatggaatagcaagtttaagtgtttccataggtttattaagaatttcatcatgtagtactcgattcagtgctcttagactacatttgctgtctttgtagaccaataaaatgcaggccattatcttcaaaagttcagcaacaaccactgctgtagaagatagataacgaggtccttcttcttttaaagttctggaataacgcattgttagaaccaaactggtagtctgaaagaccaaaattcccagggaaacgtattttaggttggcgaacattgttttatcttcatttgccaagggcagcctttccatttctttaagttcctgcggcttcttgagctccaggtgctggtcgggtgcatctgtgcctaccacagggctcaacaccgagcgagagctcatgggatgttcactgaaggaatgacgggccccagccgggcccacccgtcactagctccgcacgcaccaggcgctgaggcacacactgccgtcttcattcgcttgacacacccctctcctcgggccttttttcctcctccacccagtacattccgcacgtcgtccgtcggagttacaacgtgtcacctcatctgctcccacccctacttagctagcactgtatttcaggtcttcgataccgtcccc

SEQ ID NO: 11544 - RNA, 2419 nt, Homo sapiens
  source 1..2419: mol_type = other RNA
ctgaatagctgggactacaggtgcgtgccaccacacccagctaatttttgtatttttggtagagacggggtttcaccatgttggtcaggatagtctcaatctcttgaccttgtgatccacctgcctcagcctcccaaactgctaggattacaggcgtgagccactgcgccaggccttctcagcagctcttgtgggaacacagaaagggaattcaaaatttggctacctctcccactcatgtgatcagggaagaataggcttatgagagacctaaaaaaatcttccgagcagccttggatttaaagtcatagcgctgtttaaaataaagtaatatggcaatctggaatgtctccaagaaaagtcattttgttctgtcactgacatctgtactatttgtttgaatgttgtttttgtaaacagttgtagattaaagaagtttttacagatcaatgagtaaaatgttcatttaataactttctaactgtatacagtatatgcttgatagttcaaaattctccaaatgtagatattatacaataattattttaaattattaaatgagtatttaatccttttaaattacattttgaaaatttaatggcaattacacacaaattttaatttaaaataatattaaggacttaatctgatttacagaaatgaaatgcaatgaagagattaagggctaacctccattactataaaattctctggctaccatctagcacaggagcaactggattgctttcagcagtcttgaagcactaaaatatcttaaaattcatatggagaaatagtatgtatctctacattaaatttagatttgatatttattctctgacagatcagacccagaatattaatttttatgtaattgaaccaaaaacatttagcaatccttcatttagtaatcttttgtataaatataaaaatctctgataagtgaaatgttttttcaaattatacttctatttttcacagctttataggtaattataattttcaaactttaaatatttcatgtgatttgatatatctgtacagaaagagtaagataaaaacatttaataagattaaatctaatttgcaaaaattggtatctgacatttgttgtgtgctcttgcaaagagtgcataggacatttctgcagcaatcaaaaaggtaaaatctttttaaactcagatttcaagtttcctctaatattccttctaatcctaatccctggaaatactttcaagttttgatttctagatgcaatgtgttttgttacatatacacatgtcttatccttaaacttttaaaaaacagtatgatcagattcagcatgatgatatcttctcagactctgtagaagtcctctgtgcaagattaatgtcgagattcctagtgccccatcgtgaaaaaccagttaaagatagtatacaactatgctttagtgggatttcctgcaggtttgggatcataaccatacaaaaaagtagctgttattacaaggatggctccaaggaaaaagacactgaagaacaactactatccaggtcagtcggttatatccctgaaaaaatccattctttgataccagttctccatcataaatgtatacacccattaatccaaatatacttccaaagaaaccaagctgaatatttcttatccacactgattgttttgtttcttttaagattttctcaaagtaaaccccagcaaagccacttgaaaaacatgctgtgagaactgccatgagtcctacaaattgagaaccagctgaaagttccttagaatcaagctgagaatctgagggccactgtacaaaagcaactcctgtcatcaaaattactagggacagccactggtatacacccaattttttactaagcatagacacagaaaataatgctgttgtaagaatttttaactgatacgtgacctgataagtagctgcatctagatttgatagtgccacatacagtaaattattctgaagagtatagatccctgatggaatagcaagtttaagtgtttccataggtttattaagaatttcatcatgtagtactcgattcagtgctcttagactacatttgctgtctttgtagaccaataaaatgcaggccattatcttcaaaagttcagcaacaaccactgctgtagaagatagataacgaggtccttcttcttttaaagttctggaataacgcattgttagaaccaaactggtagtctgaaagaccaaaattcccagggaaacgtattttaggttggcgaacattgttttatcttcatttgcctcccgcgcagctcgaccggctgagcccaccaccgggggccgcggttcagctccgccgggcgccccaggctgccgagtccgctgggtcctacgcgaccgctgacccgcagcgccgccggctcccgtcgccgt

SEQ ID NO: 11545 - RNA, 2650 nt, Homo sapiens
  source 1..2650: mol_type = other RNA
ctgaatagctgggactacaggtgcgtgccaccacacccagctaatttttgtatttttggtagagacggggtttcaccatgttggtcaggatagtctcaatctcttgaccttgtgatccacctgcctcagcctcccaaactgctaggattacaggcgtgagccactgcgccaggccttctcagcagctcttgtgggaacacagaaagggaattcaaaatttggctacctctcccactcatgtgatcagggaagaataggcttatgagagacctaaaaaaatcttccgagcagccttggatttaaagtcatagcgctgtttaaaataaagtaatatggcaatctggaatgtctccaagaaaagtcattttgttctgtcactgacatctgtactatttgtttgaatgttgtttttgtaaacagttgtagattaaagaagtttttacagatcaatgagtaaaatgttcatttaataactttctaactgtatacagtatatgcttgatagttcaaaattctccaaatgtagatattatacaataattattttaaattattaaatgagtatttaatccttttaaattacattttgaaaatttaatggcaattacacacaaattttaatttaaaataatattaaggacttaatctgatttacagaaatgaaatgcaatgaagagattaagggctaacctccattactataaaattctctggctaccatctagcacaggagcaactggattgctttcagcagtcttgaagcactaaaatatcttaaaattcatatggagaaatagtatgtatctctacattaaatttagatttgatatttattctctgacagatcagacccagaatattaatttttatgtaattgaaccaaaaacatttagcaatccttcatttagtaatcttttgtataaatataaaaatctctgataagtgaaatgttttttcaaattatacttctatttttcacagctttataggtaattataattttcaaactttaaatatttcatgtgatttgatatatctgtacagaaagagtaagataaaaacatttaataagattaaatctaatttgcaaaaattggtatctgacatttgttgtgtgctcttgcaaagagtgcataggacatttctgcagcaatcaaaaaggtaaaatctttttaaactcagatttcaagtttcctctaatattccttctaatcctaatccctggaaatactttcaagttttgatttctagatgcaatgtgttttgttacatatacacatgtcttatccttaaacttttaaaaaacagtatgatcagattcagcatgatgatatcttctcagactctgtagaagtcctctgtgcaagattaatgtcgagattcctagtgccccatcgtgaaaaaccagttaaagatagtatacaactatgctttagtgggatttcctgcaggtttgggatcataaccatacaaaaaagtagctgttattacaaggatggctccaaggaaaaagacactggttggcacaaaatcttgaagccaaaaataggagatcaatgttgataatattatcgataaagaggttgcaaatccttttaaaatattatctgcatacttaataacagcagctattacaaggcctccaagtgcctgaagaacaactactatccaggtcagtcggttatatccctgaaaaaatccattctttgataccagttctccatcataaatgtatacacccattaatccaaatatacttccaaagaaaccaagctgaatatttcttatccacactgattgttttgtttcttttaagattttctcaaagtaaaccccagcaaagccacttgaaaaacatgctgtgagaactgccatgagtcctacaaattgagaaccagctgaaagttccttagaatcaagctgagaatctgagggccactgataagtagctgcatctagatttgatagtgccacatacagtaaattattctgaagagtatagatccctgatggaatagcaagtttaagtgtttccataggtttattaagaatttcatcatgtagtactcgattcagtgctcttagactacatttgctgtctttgtagaccaataaaatgcaggccattatcttcaaaagttcagcaacaaccactgctgtagaagatagataacgaggtccttcttcttttaaagttctggaataacgcattgttagaaccaaactggtagtctgaaagaccaaaattcccagggaaacgtattttaggttggcgaacattgttttatcttcatttgccaagggcagcctttccatttctttaagttcctgcggcttcttgagctccaggtgctggtcgggtgcatctgtgcctaccacagggctcaacaccgagcgagagctcatgggatgttcactgaaggaatgacgggccccagccgggcccacccgtcactagctccgcacgcaccaggcgctgaggcacacactgccgtcttcattcgcttgacacacccctctcctcgggccttttttcctcctccacccagtacattccgcacgtcgtccgtcggagttacaacgtgtcacctcatctgctcccacccctacttagctagcactgtatttcaggtcttcgataccgtcccct

SEQ ID NO: 11546 - RNA, 4060 nt, Homo sapiens
  source 1..4060: mol_type = other RNA
ctgaatagctgggactacaggtgcgtgccaccacacccagctaatttttgtatttttggtagagacggggtttcaccatgttggtcaggatagtctcaatctcttgaccttgtgatccacctgcctcagcctcccaaactgctaggattacaggcgtgagccactgcgccaggccttctcagcagctcttgtgggaacacagaaagggaattcaaaatttggctacctctcccactcatgtgatcagggaagaataggcttatgagagacctaaaaaaatcttccgagcagccttggatttaaagtcatagcgctgtttaaaataaagtaatatggcaatctggaatgtctccaagaaaagtcattttgttctgtcactgacatctgtactatttgtttgaatgttgtttttgtaaacagttgtagattaaagaagtttttacagatcaatgagtaaaatgttcatttaataactttctaactgtatacagtatatgcttgatagttcaaaattctccaaatgtagatattatacaataattattttaaattattaaatgagtatttaatccttttaaattacattttgaaaatttaatggcaattacacacaaattttaatttaaaataatattaaggacttaatctgatttacagaaatgaaatgcaatgaagagattaagggctaacctccattactataaaattctctggctaccatctagcacaggagcaactggattgctttcagcagtcttgaagcactaaaatatcttaaaattcatatggagaaatagtatgtatctctacattaaatttagatttgatatttattctctgacagatcagacccagaatattaatttttatgtaattgaaccaaaaacatttagcaatccttcatttagtaatcttttgtataaatataaaaatctctgataagtgaaatgttttttcaaattatacttctatttttcacagctttataggtaattataattttcaaactttaaatatttcatgtgatttgatatatctgtacagaaagagtaagataaaaacatttaataagattaaatctaatttgcaaaaattggtatctgacatttgttgtgtgctcttgcaaagagtgcataggacatttctgcagcaatcaaaaaggtaaaatctttttaaactcagatttcaagtttcctctaatattccttctaatcctaatccctggaaatactttcaagttttgatttctagatgcaatgtgttttgttacatatacacatgtcttatccttaaacttttaaaaaacagtatgatcagattcagcatgatgatatcttctcagactctgtagaagtcctctgtgcaagattaatgtcgagattcctagtgccccatcgtgaaaaaccagttaaagatagtatacaactatgctttagtgggatttcctgcaggtttgggatcataaccatacaaaaaagtagctgttattacaaggatggctccaaggaaaaagacactggttggcacaaaatcttgaagccaaaaataggagatcaatgttgataatattatcgataaagaggttgcaaatccttttaaaatattatctgcatacttaataacagcagctattacaaggcctccaagtgcctgaagaacaactactatccaggtcagtcggttatatccctgaaaaaatccattctttgataccagttctccatcataaatgtatacacccattaatccaaatatacttccaaagaaaccaagctgaatatttcttatccacactgattgttttgtttcttttaagattttctcaaagtaaaccccagcaaagccacttgaaaaacatgctgtgagaactgccatgagtcctacaaattgagaaccagctgaaagttccttagaatcaagctgagaatctgagggccactgataagtagctgcatctagatttgatagtgccacatacagtaaattattctgaagagtatagatccctgatggaatagcaagtttaagtgtttccataggtttattaagaatttcatcatgtagtactcgattcagtgctcttagactacatttgctgtctttgtagaccaataaaatgcaggccattatcttcaaaagttcagcaacaaccactgctgtagaagatagataacgaggtccttcttcttttaaagttctggaataacgcattgttagaaccaaactggtagtctgaaagaccaaaattcccagggaaacgtattttaggttggcgaacattgttttatcttcatttgcctcccgcgcagctcgaccggctgagcccaccaccgggggccgcggttcagctccgccgggcgccccaggctgccgagtccgctgggtcctacgcgaccgctgacccgcagcgccgccggctcccgtcgccgtagccaccgccagctcggtgcagcccaggcgtttccgggttcccgcggtcccgtcccccaaatgctccggcttccgcctcggctctggcaaatgccgttcccggctcggctctggcagccccagctcggcacttggcagctctgtccctaaggcgacgcacctgggctgctctgctggcagcccctggttcctgcttcaccgtcgcgtggaggcctggggcactgctttctgctacacctctcctaggagcgcgaaacagatggagtgacactcgtcgagggcctctgcgggactgtctgtttgcagagggtgccaaggtgtccactgcgtaaggaagggcaaagtcctttggggcaaagaaccctgagaggaacggggagatggattttgaaagcaaacgaaccctctcctaaaagtgactgtcactgacctgaaaacaaccagattagctatggcaaaggctgccaaccaaccagtggtctgcaagaaggcttgttcttccacttcacccaccctgactgagatcttgagactgaaggaaacccaaagccgtaccaccaatgggcctagtgtcatcaaccgggagaggaaaaagaaaactgggcccagaggattgcagagttatgagggaccaaccccttcctggctgcatggatcacagcattaccttttaaaagtgttccagtagctgtgttggaaaccctctaaccacggcagcccattcaggtgatgaacaggctgaaatcagtacttcaggttcagctggattatcaaataagcgaataggattatctctttttgttaactcagggctgctataaattaagcctatgtctctttatattgcaaatgattaaaaccatgtccaagagagacatacttagaaaaaaagtgatattgaagaaaaataagtaactgtattagagtagaataactggttttaaaattttctgcaatacagtcttgagaaaattcctggatggtaaaatacatattagatcttaatacatgcccagttttttttgaaaccaaaatgtgcctgttagatgatgataacagcatgcctcgttttattgtgatttgctttattgctcttcacagacattgcttttgtttttttgttttttttttttacaaattgaaggtttgtggcaaccttgcctcaagcacatctattggtgccatttttccaacagcatgtgctcactttgtgtctctgtgtcacataatattcaataatttttgcaatatttaaatttgttcatcattattatatctggtatagtgctttgtgatcaatgatctttgatgttactatggtaattgttttggggtgctgatatggtttggctgtgtccccacccaaatctcaacttgaactgtatctcccagaattcccacgtgttgagggagagacctagggggagataattgaatcatgggggccagtctttcctgtgctattctcatgatagtgaataagtctcatgaaatccgatgggtttatctggggtttctgattttgcttcttcctcatttttctcttgctgcagccatgtaagcaagtacctttcacctcccgccatgattctgaggcctcccccgccatgtggaactgtaggtccaatta

SEQ ID NO: 11547 - RNA, 2549 nt, Homo sapiens
  source 1..2549: mol_type = other RNA
ctgaatagctgggactacaggtgcgtgccaccacacccagctaatttttgtatttttggtagagacggggtttcaccatgttggtcaggatagtctcaatctcttgaccttgtgatccacctgcctcagcctcccaaactgctaggattacaggcgtgagccactgcgccaggccttctcagcagctcttgtgggaacacagaaagggaattcaaaatttggctacctctcccactcatgtgatcagggaagaataggcttatgagagacctaaaaaaatcttccgagcagccttggatttaaagtcatagcgctgtttaaaataaagtaatatggcaatctggaatgtctccaagaaaagtcattttgttctgtcactgacatctgtactatttgtttgaatgttgtttttgtaaacagttgtagattaaagaagtttttacagatcaatgagtaaaatgttcatttaataactttctaactgtatacagtatatgcttgatagttcaaaattctccaaatgtagatattatacaataattattttaaattattaaatgagtatttaatccttttaaattacattttgaaaatttaatggcaattacacacaaattttaatttaaaataatattaaggacttaatctgatttacagaaatgaaatgcaatgaagagattaagggctaacctccattactataaaattctctggctaccatctagcacaggagcaactggattgctttcagcagtcttgaagcactaaaatatcttaaaattcatatggagaaatagtatgtatctctacattaaatttagatttgatatttattctctgacagatcagacccagaatattaatttttatgtaattgaaccaaaaacatttagcaatccttcatttagtaatcttttgtataaatataaaaatctctgataagtgaaatgttttttcaaattatacttctatttttcacagctttataggtaattataattttcaaactttaaatatttcatgtgatttgatatatctgtacagaaagagtaagataaaaacatttaataagattaaatctaatttgcaaaaattggtatctgacatttgttgtgtgctcttgcaaagagtgcataggacatttctgcagcaatcaaaaaggtaaaatctttttaaactcagatttcaagtttcctctaatattccttctaatcctaatccctggaaatactttcaagttttgatttctagatgcaatgtgttttgttacatatacacatgtcttatccttaaacttttaaaaaacagtatgatcagattcagcatgatgatatcttctcagactctgtagaagtcctctgtgcaagattaatgtcgagattcctagtgccccatcgtgaaaaaccagttaaagatagtatacaactatgctttagtgggatttcctgcaggtttgggatcataaccatacaaaaaagtagctgttattacaaggatggctccaaggaaaaagacactggttggcacaaaatcttgaagccaaaaataggagatcaatgttgataatattatcgataaagaggttgcaaatccttttaaaatattatctgcatacttaataacagcagctattacaaggcctccaagtgcctgaagaacaactactatccaggtcagtcggttatatccctgaaaaaatccattctttgataccagttctccatcataaatgtatacacccattaatccaaatatacttccaaagaaaccaagctgaatatttcttatccacactgattgttttgtttcttttaagattttctcaaagtaaaccccagcaaagccacttgaaaaacatgctgtgagaactgccatgagtcctacaaattgagaaccagctgaaagttccttagaatcaagctgagaatctgagggccactgtacaaaagcaactcctgtcatcaaaattactagggacagccactggtatacacccaattttttactaagcatagacacagaaaataatgctgttgtaagaatttttaactgatacgtgacctgataagtagctgcatctagatttgatagtgccacatacagtaaattattctgaagagtatagatccctgatggaatagcaagtttaagtgtttccataggtttattaagaatttcatcatgtagtactcgattcagtgctcttagactacatttgctgtctttgtagaccaataaaatgcaggccattatcttcaaaagttcagcaacaaccactgctgtagaagatagataacgaggtccttcttcttttaaagttctggaataacgcattgttagaaccaaactggtagtctgaaagaccaaaattcccagggaaacgtattttaggttggcgaacattgttttatcttcatttgccaagggcagcctttccatttctttaagttcctgcggcttcttgagctccaggtgctggtcgggtgcatctgtgcctaccacagggctcaacaccgagcgagagctcatgggatgttcactgaaggaat

SEQ ID NO: 11548 - RNA, 2588 nt, Homo sapiens
  source 1..2588: mol_type = other RNA
ctgaatagctgggactacaggtgcgtgccaccacacccagctaatttttgtatttttggtagagacggggtttcaccatgttggtcaggatagtctcaatctcttgaccttgtgatccacctgcctcagcctcccaaactgctaggattacaggcgtgagccactgcgccaggccttctcagcagctcttgtgggaacacagaaagggaattcaaaatttggctacctctcccactcatgtgatcagggaagaataggcttatgagagacctaaaaaaatcttccgagcagccttggatttaaagtcatagcgctgtttaaaataaagtaatatggcaatctggaatgtctccaagaaaagtcattttgttctgtcactgacatctgtactatttgtttgaatgttgtttttgtaaacagttgtagattaaagaagtttttacagatcaatgagtaaaatgttcatttaataactttctaactgtatacagtatatgcttgatagttcaaaattctccaaatgtagatattatacaataattattttaaattattaaatgagtatttaatccttttaaattacattttgaaaatttaatggcaattacacacaaattttaatttaaaataatattaaggacttaatctgatttacagaaatgaaatgcaatgaagagattaagggctaacctccattactataaaattctctggctaccatctagcacaggagcaactggattgctttcagcagtcttgaagcactaaaatatcttaaaattcatatggagaaatagtatgtatctctacattaaatttagatttgatatttattctctgacagatcagacccagaatattaatttttatgtaattgaaccaaaaacatttagcaatccttcatttagtaatcttttgtataaatataaaaatctctgataagtgaaatgttttttcaaattatacttctatttttcacagctttataggtaattataattttcaaactttaaatatttcatgtgatttgatatatctgtacagaaagagtaagataaaaacatttaataagattaaatctaatttgcaaaaattggtatctgacatttgttgtgtgctcttgcaaagagtgcataggacatttctgcagcaatcaaaaaggtaaaatctttttaaactcagatttcaagtttcctctaatattccttctaatcctaatccctggaaatactttcaagttttgatttctagatgcaatgtgttttgttacatatacacatgtcttatccttaaacttttaaaaaacagtatgatcagattcagcatgatgatatcttctcagactctgtagaagtcctctgtgcaagattaatgtcgagattcctagtgccccatcgtgaaaaaccagttaaagatagtatacaactatgctttagtgggatttcctgcaggtttgggatcataaccatacaaaaaagtagctgttattacaaggatggctccaaggaaaaagacactggttggcacaaaatcttgaagccaaaaataggagatcaatgttgataatattatcgataaagaggttgcaaatccttttaaaatattatctgcatacttaataacagcagctattacaaggcctccaagtgcctgaagaacaactactatccaggtcagtcggttatatccctgaaaaaatccattctttgataccagttctccatcataaatgtatacacccattaatccaaatatacttccaaagaaaccaagctgaatatttcttatccacactgattgttttgtttcttttaagattttctcaaagtaaaccccagcaaagccacttgaaaaacatgctgtgagaactgccatgagtcctacaaattgagaaccagctgaaagttccttagaatcaagctgagaatctgagggccactgtacaaaagcaactcctgtcatcaaaattactagggacagccactggtatacacccaattttttactaagcatagacacagaaaataatgctgttgtaagaatttttaactgatacgtgacctgataagtagctgcatctagatttgatagtgccacatacagtaaattattctgaagagtatagatccctgatggaatagcaagtttaagtgtttccataggtttattaagaatttcatcatgtagtactcgattcagtgctcttagactacatttgctgtctttgtagaccaataaaatgcaggccattatcttcaaaagttcagcaacaaccactgctgtagaagatagataacgaggtccttcttcttttaaagttctggaataacgcattgttagaaccaaactggtagtctgaaagaccaaaattcccagggaaacgtattttaggttggcgaacattgttttatcttcatttgcctcccgcgcagctcgaccggctgagcccaccaccgggggccgcggttcagctccgccgggcgccccaggctgccgagtccgctgggtcctacgcgaccgctgacccgcagcgccgccggctcccgtcgccgtagccaccgccagctcggtgcagcccaggcgtttcc

SEQ ID NO: 11549 - RNA, 2712 nt, Homo sapiens
  source 1..2712: mol_type = other RNA
ctgaatagctgggactacaggtgcgtgccaccacacccagctaatttttgtatttttggtagagacggggtttcaccatgttggtcaggatagtctcaatctcttgaccttgtgatccacctgcctcagcctcccaaactgctaggattacaggcgtgagccactgcgccaggccttctcagcagctcttgtgggaacacagaaagggaattcaaaatttggctacctctcccactcatgtgatcagggaagaataggcttatgagagacctaaaaaaatcttccgagcagccttggatttaaagtcatagcgctgtttaaaataaagtaatatggcaatctggaatgtctccaagaaaagtcattttgttctgtcactgacatctgtactatttgtttgaatgttgtttttgtaaacagttgtagattaaagaagtttttacagatcaatgagtaaaatgttcatttaataactttctaactgtatacagtatatgcttgatagttcaaaattctccaaatgtagatattatacaataattattttaaattattaaatgagtatttaatccttttaaattacattttgaaaatttaatggcaattacacacaaattttaatttaaaataatattaaggacttaatctgatttacagaaatgaaatgcaatgaagagattaagggctaacctccattactataaaattctctggctaccatctagcacaggagcaactggattgctttcagcagtcttgaagcactaaaatatcttaaaattcatatggagaaatagtatgtatctctacattaaatttagatttgatatttattctctgacagatcagacccagaatattaatttttatgtaattgaaccaaaaacatttagcaatccttcatttagtaatcttttgtataaatataaaaatctctgataagtgaaatgttttttcaaattatacttctatttttcacagctttataggtaattataattttcaaactttaaatatttcatgtgatttgatatatctgtacagaaagagtaagataaaaacatttaataagattaaatctaatttgcaaaaattggtatctgacatttgttgtgtgctcttgcaaagagtgcataggacatttctgcagcaatcaaaaaggtaaaatctttttaaactcagatttcaagtttcctctaatattccttctaatcctaatccctggaaatactttcaagttttgatttctagatgcaatgtgttttgttacatatacacatgtcttatccttaaacttttaaaaaacagtatgatcagattcagcatgatgatatcttctcagactctgtagaagtcctctgtgcaagattaatgtcgagattcctagtgccccatcgtgaaaaaccagttaaagatagtatacaactatgctttagtgggatttcctgcaggtttgggatcataaccatacaaaaaagtagctgttattacaaggatggctccaaggaaaaagacactggttggcacaaaatcttgaagccaaaaataggagatcaatgttgataatattatcgataaagaggttgcaaatccttttaaaatattatctgcatacttaataacagcagctattacaaggcctccaagtgcctgaagaacaactactatccaggtcagtcggttatatccctgaaaaaatccattctttgataccagttctccatcataaatgtatacacccattaatccaaatatacttccaaagaaaccaagctgaatatttcttatccacactgattgttttgtttcttttaagattttctcaaagtaaaccccagcaaagccacttgaaaaacatgctgtgagaactgccatgagtcctacaaattgagaaccagctgaaagttccttagaatcaagctgagaatctgagggccactgtacaaaagcaactcctgtcatcaaaattactagggacagccactggtatacacccaattttttactaagcatagacacagaaaataatgctgttgtaagaatttttaactgatacgtgacctgataagtagctgcatctagatttgatagtgccacatacagtaaattattctgaagagtatagatccctgatggaatagcaagtttaagtgtttccataggtttattaagaatttcatcatgtagtactcgattcagtgctcttagactacatttgctgtctttgtagaccaataaaatgcaggccattatcttcaaaagttcagcaacaaccactgctgtagaagatagataacgaggtccttcttcttttaaagttctggaataacgcattgttagaaccaaactggtagtctgaaagaccaaaattcccagggaaacgtattttaggttggcgaacattgttttatcttcatttgcttgggaggctaaggtgggagatcacttgagccagggaggtggaagttgcagtgagctgagattgcgcctctgtactccagccaaggtgacagtgagacccaagggcagcctttccatttctttaagttcctgcggcttcttgagctccaggtgctggtcgggtgcatctgtgcctaccacagggctcaacaccgagcgagagctcatgggatgttcactgaaggaatgacgggccccagccgggcccacccgtcactagctccgcacgcaccaggcgctgaggcacacact

SEQ ID NO: 11550 - RNA, 4282 nt, Homo sapiens
  source 1..4282: mol_type = other RNA
ctgaatagctgggactacaggtgcgtgccaccacacccagctaatttttgtatttttggtagagacggggtttcaccatgttggtcaggatagtctcaatctcttgaccttgtgatccacctgcctcagcctcccaaactgctaggattacaggcgtgagccactgcgccaggccttctcagcagctcttgtgggaacacagaaagggaattcaaaatttggctacctctcccactcatgtgatcagggaagaataggcttatgagagacctaaaaaaatcttccgagcagccttggatttaaagtcatagcgctgtttaaaataaagtaatatggcaatctggaatgtctccaagaaaagtcattttgttctgtcactgacatctgtactatttgtttgaatgttgtttttgtaaacagttgtagattaaagaagtttttacagatcaatgagtaaaatgttcatttaataactttctaactgtatacagtatatgcttgatagttcaaaattctccaaatgtagatattatacaataattattttaaattattaaatgagtatttaatccttttaaattacattttgaaaatttaatggcaattacacacaaattttaatttaaaataatattaaggacttaatctgatttacagaaatgaaatgcaatgaagagattaagggctaacctccattactataaaattctctggctaccatctagcacaggagcaactggattgctttcagcagtcttgaagcactaaaatatcttaaaattcatatggagaaatagtatgtatctctacattaaatttagatttgatatttattctctgacagatcagacccagaatattaatttttatgtaattgaaccaaaaacatttagcaatccttcatttagtaatcttttgtataaatataaaaatctctgataagtgaaatgttttttcaaattatacttctatttttcacagctttataggtaattataattttcaaactttaaatatttcatgtgatttgatatatctgtacagaaagagtaagataaaaacatttaataagattaaatctaatttgcaaaaattggtatctgacatttgttgtgtgctcttgcaaagagtgcataggacatttctgcagcaatcaaaaaggtaaaatctttttaaactcagatttcaagtttcctctaatattccttctaatcctaatccctggaaatactttcaagttttgatttctagatgcaatgtgttttgttacatatacacatgtcttatccttaaacttttaaaaaacagtatgatcagattcagcatgatgatatcttctcagactctgtagaagtcctctgtgcaagattaatgtcgagattcctagtgccccatcgtgaaaaaccagttaaagatagtatacaactatgctttagtgggatttcctgcaggtttgggatcataaccatacaaaaaagtagctgttattacaaggatggctccaaggaaaaagacactggttggcacaaaatcttgaagccaaaaataggagatcaatgttgataatattatcgataaagaggttgcaaatccttttaaaatattatctgcatacttaataacagcagctattacaaggcctccaagtgcctgaagaacaactactatccaggtcagtcggttatatccctgaaaaaatccattctttgataccagttctccatcataaatgtatacacccattaatccaaatatacttccaaagaaaccaagctgaatatttcttatccacactgattgttttgtttcttttaagattttctcaaagtaaaccccagcaaagccacttgaaaaacatgctgtgagaactgccatgagtcctacaaattgagaaccagctgaaagttccttagaatcaagctgagaatctgagggccactgtacaaaagcaactcctgtcatcaaaattactagggacagccactggtatacacccaattttttactaagcatagacacagaaaataatgctgttgtaagaatttttaactgatacgtgacctgataagtagctgcatctagatttgatagtgccacatacagtaaattattctgaagagtatagatccctgatggaatagcaagtttaagtgtttccataggtttattaagaatttcatcatgtagtactcgattcagtgctcttagactacatttgctgtctttgtagaccaataaaatgcaggccattatcttcaaaagttcagcaacaaccactgctgtagaagatagataacgaggtccttcttcttttaaagttctggaataacgcattgttagaaccaaactggtagtctgaaagaccaaaattcccagggaaacgtattttaggttggcgaacattgttttatcttcatttgcttgggaggctaaggtgggagatcacttgagccagggaggtggaagttgcagtgagctgagattgcgcctctgtactccagccaaggtgacagtgagaccctcccgcgcagctcgaccggctgagcccaccaccgggggccgcggttcagctccgccgggcgccccaggctgccgagtccgctgggtcctacgcgaccgctgacccgcagcgccgccggctcccgtcgccgtagccaccgccagctcggtgcagcccaggcgtttccgggttcccgcggtcccgtcccccaaatgctccggcttccgcctcggctctggcaaatgccgttcccggctcggctctggcagccccagctcggcacttggcagctctgtccctaaggcgacgcacctgggctgctctgctggcagcccctggttcctgcttcaccgtcgcgtggaggcctggggcactgctttctgctacacctctcctaggagcgcgaaacagatggagtgacactcgtcgagggcctctgcgggactgtctgtttgcagagggtgccaaggtgtccactgcgtaaggaagggcaaagtcctttggggcaaagaaccctgagaggaacggggagatggattttgaaagcaaacgaaccctctcctaaaagtgactgtcactgacctgaaaacaaccagattagctatggcaaaggctgccaaccaaccagtggtctgcaagaaggcttgttcttccacttcacccaccctgactgagatcttgagactgaaggaaacccaaagccgtaccaccaatgggcctagtgtcatcaaccgggagaggaaaaagaaaactgggcccagaggattgcagagttatgagggaccaaccccttcctggctgcatggatcacagcattaccttttaaaagtgttccagtagctgtgttggaaaccctctaaccacggcagcccattcaggtgatgaacaggctgaaatcagtacttcaggttcagctggattatcaaataagcgaataggattatctctttttgttaactcagggctgctataaattaagcctatgtctctttatattgcaaatgattaaaaccatgtccaagagagacatacttagaaaaaaagtgatattgaagaaaaataagtaactgtattagagtagaataactggttttaaaattttctgcaatacagtcttgagaaaattcctggatggtaaaatacatattagatcttaatacatgcccagttttttttgaaaccaaaatgtgcctgttagatgatgataacagcatgcctcgttttattgtgatttgctttattgctcttcacagacattgcttttgtttttttgttttttttttttacaaattgaaggtttgtggcaaccttgcctcaagcacatctattggtgccatttttccaacagcatgtgctcactttgtgtctctgtgtcacataatattcaataatttttgcaatatttaaatttgttcatcattattatatctggtatagtgctttgtgatcaatgatctttgatgttactatggtaattgttttggggtgctgatatggtttggctgtgtccccacccaaatctcaacttgaactgtatctcccagaattcccacgtgttgagggagagacctagggggagataattgaatcatgggggccagtctttcctgtgctattctcatgatagtgaataagtctcatgaaatccgatgggtttatctggggtttctgattttgcttcttcctcatttttctcttgctgcagccatgtaagcaagtacctttcacctcccgccatgattctgaggcctcccccgccatgtggaactgtaggtccaatta

SEQ ID NO: 11551 - RNA, 617 nt, Homo sapiens
  source 1..617: mol_type = other RNA
ctgaatagctgggactacaggtgcgtgccaccacaccgcactaatttttttcctttttttttttttttctttttggtagagacgggtttctcactatgttgcccaggctggtctcgaactcccgggctcaagcgatcctcccgccgcggcctcccaaagcgctgggattacaggtacggccactgcgaccagctgcttctccttggtggactgatcaacaccaacaaggcggcgcacgtccctattactcacgccttcgtcaggctcctggagaatattcatccagtcttccagaggcatgacgctccgcctcctcttgacaggtggctggcccaggatcaagattcccctccaggccaccgctccacctggggaggcctcagccgcggccgtagccgcggtggcctccataacggctgcagtcgtccccgcctagagcctggttttggagcctcgaggacgccgacgaggctgtttaacttcccgtgagtccccaccctcgccgctccgctggccgggaatttggcaaggctttgccctacgcggtaaacacgtaagcctactggcctccgcatttccctgagcagcgacctagatgacgccagactgagggagcc

SEQ ID NO: 11552 - RNA, 259 nt, Homo sapiens
  source 1..259: mol_type = other RNA
ctgaatagctgggactacaggtgcgtgccaccacacctggctaattttttgtatttttagtatagatggggtttcaccatgttagccaggatggtctccatctcctgacctcgtgatccacccacctcggcctcccaaagtgctgggattacaggtgtgagccacagtgccgggctggattccatctcctcctcctcctcctccttgtctctccctcctggccaccggcgcggcccagccggcgacgcgctgacgccgt

SEQ ID NO: 11553 - RNA, 7028 nt, Homo sapiens
  source 1..7028: mol_type = other RNA
ctgaatagctgggactacaggtgcgtgccaccacatccagctaattttttatatttttagtagagactgggtttcactgtgttagccagggtggtctcaatcacctgaccttgtgatccaccagcctcagcctcccaaagtgctgggattacaggcgtgagccatcatgaccggcccaccagctcaactctttagccctatctcctactattcttctacctatactcagtacccaccctggtcactattccttaatgtagtgccatatctagactgccctgtcaccaagcaaattcttattcatccttgggccagcatcagatgttacctggtttcaccaaaacatggtataatgggggctttaaaccctttccataaatctcattagtcctccctaagcaacccaaatcaaaatttaaaaaaatatttcgtatggatggagttttgcaatctcatgtaaactatgtacaaaaagcatctttaaaaagatttgtatttttattatctgcaacatactaagtaaaagcaaagtactcgctatacaagtgcatcttcaagataagtcccttggcctaactttcaactagattgcagctaataaaactcctccacagaaattctgaagcagtcacagactattacttgccctaagaagttttctctaacctcttcctgacaagctgtccttctgggctcccatacaaacaatagtgtagtgtgttactttctcctttggtttcttctacaatggtagcacatccaggttaaggattctacattagattccttacgtgtaaaataaagataagaagacatatctcatagaattaaatgtgttaatgcgtacttaaagcacttagcatagcatctagcatgttgtaagtgctatatcaatgtcagcaattctttttcaatttttgtttgttgaatgatgaggcactagtacaaagagtcccacagcaaacagactggtagatgtgtggttcacaaaagagcatgctatgaaaacacaatatgtcctgaaattctctgggtggttattacataagcaaaatgccttcctagttagttatctacttgcagatgtgatgtgaaactgagtagattttaatgtttagcagtttaagaagattttaagacctcaaagctgggaaaagaaattttcaattataaatttgtgaacttctgaggaagttttttgaaaataacacttaacagtttcatatttgaagaaaaagaaaacagtgtcttgggaatttgtgctgtctttgactctatcatataatacttctttatactgcaaactacctgtaaatgtatttgatcgcaggtttgtgagaaaaataaagtgtgttgtgtggtagaaataataccaaagtggtattattgtgggctacagatattgaatcctagcccacaaattagctgtgggatcttgggcaagctcttaattcctctgggcatcagagcccttctttggaatttgaagagagaaaacgaaataatctctaaattcccatccagctctaagttacaaagtttttgtaatactatattttgaactttttcttacattatacccccatgtcctcttactagaaactaaactatttatttatttatatatttttagagcaggaatcaagtcttattttctttacacccaagtgcctaaatccagagcctgtttcttgactttgaatgaatgagttagtaaccgtttcttgaacgagtgcccctcttcacagagctagtttaaaaaaaggcatagcaaatttatggtataataggttagcagctaaccgtaacataactatgttattagaacaaataattgtgcattaatatgacttggtattcaatacagttatagatcatattattttttgaagactttactaatttagaaaaggagttctaaactatttccttgcttcagacatatttcagagaattatgagtcacaaagctttgagagaggcttatttatgaaatctcataatcccattggcaatatcaaaagtacccaagtactcgctaccaggtagcattttgtagcaaaggtttttatctttgacttactaccaaaattacagactgaaagacaatctgatccaggaaataaggaactggtgtctaatgacacaccaagaaagcaaacgtgtgtgtgcacatacatacacatacacacaatttaaactccgtaactcaattgccttatatactcattttcaagtttatatttagtgctggcttattgcaggtgcagttccaacatatccctaacatggaatggaaaatggagaatgagtgactacctgtaaaggaagtctatgcttttgaacaagggcagattcccttctgtggatatatccccaaaagagagagacaggaaattccatttctcttgttttagtaatgatgtggttgaaatttgagatgtacttgcttcagaatttcctgggcctgaattgttgggaaagctaagattttccccagcactcagctatcagcctcaatcacctaaatgtgagtttgaatgttagtcacagaaaactctacatgaatggacacaagcacggtaagtttttattgttaaattactatgttaccctatgcagagcaaaaagtaaagggactgatctacttctgcattcacattttaaattcttgaataatgattaagtgaacaaatcatcagctaggaaaggaaaactgaagctagggtttccttataagtcttctaatttctctaataattagagaaaacatgctcaaaaactttagaaaaacatttttctatatgtgatatattaataaataaactatgtttacctcattaaattggaaagactcaatattaaagaaagtttatatccggctaatgcaattatcatttggatataatataggcatcaaaaaataaaggagtggcataaatttttccaaaatgttaacacttaatgctgagtttccagttccagaattgtccactcgccttgaggcgaacaatcttcagaggaaaaactagccatggtgatgctcgctgaggaatcaagtggagatgttagttcactccatctgttcaaagtgtcaatatgtgttataccctgaggttttgagctatctcgtgctaaaagtagtgtctgattgattagatactgtgctaaacttaagtcttcaggaacggaatttgtaacatctaagtttgaatcctgttcagagagcagttgctttagtagtgtccaatcttgttttgcaaaatgttggtcatcttcaaaatccatatctgtaacatgtgtttctgattccactttctgctcaaatgcttctattacatccatctcatatattggagacagggtttttgaaggccgatggtcatacatgcgggtttgtgccagtgtgtcacaatcatctatgtctcctgcagataaagcaatattagctttttcagtagttgtagaatggctctctttcactggaccttcctgaggcagaacttgactccgaaaggagtctagagattttgtagagctgttctttggtatgtcagaattgggttctctttgatgaagatccaagtgacatggtctttcttgagattttacatcactatccaagaatttgctgcgttgctgaatgtcattttccacattgcttccattgtttacttttttatcttctcgaagaagctgtctgcttctactggataggacgtctattgtgttctttttttctgtggctgaaacactctgtttattttttcttgaagagtcaatgctactaagatccaagacagtgctttcatttttacatacactattgcctttattttgtttacattctaaaatattatcttcactttctcgtgagaatctggaatagcaggtccttccatgatgttcatgagaaatgccatcaaaaacatcagaaggtgaaaaagaatctacagaagcctgaaagggagtatggacttctccttcatctgatcccagctcttcacattcatcgactgaaagtaaaactgaccttttaaactttttagttgcagaaaattcacgacattcattttcagttgcatcttcaaaagctaaattaattattccctgaaactgctgaggagctgggttagatatagagaaattttctgcaacgttttcagcttcagatctttcatcttctgtttcatctgctgaagaagatacctgatctatttcctgagcaaactggacactgcctcgtggaatattttctctttccctagagtgaactattgcagatcgagaccaaatttctggccttttcctagggatttcatcatcactcgttgaattaacttggaaaagatcattattactttgctttttcatttttacttcaattcttaaattactatcataaatttttaattcttcaggagtactggtatcactgctacttcttccaagaaaatcatggcacagcatagtgccacatttagagatacctctgtcatttgacccatcatcatcctgagaccctccagcatcatagtcttcagatctgggctttatgtcatcggaggaggtggtagcactgccagtgtcagattcaggactctctcgctgatgcagaacaccagtactcaaattccagtgacccacaaatggagtttctggagtttcatggctctctggagattctgatgtttccatatttttaggagaatttttttctgatagctgtcccgaaaaacacttggaagatacatctgagtctgctgtagcatgtttgtcttcatccatagcagattcatctgacaacttactaggaattgtcagtccttccacaggaactttcgattttttgtcttcttgagcagaatttaaggtaccatttgtcctttcaggattacacagtgaaacatcttccacacatttaatacttgattgtttgtttgtatcttttctccctacttggttctccctatctgatatcaaatggatttgccctgcacttgttgagtctaaatcacaaactggattagagttcaaggagttttcatttggatttgaaaccatgtattttagggctgtggtgctataaaattttgaatttacattatcactcccaacagaatgacaacatatgttagctgcatcgcaatcatctgtttctttgtgattgggaaattttgtttcacttttatctaaacaaatctgttttgattccagttcgtgttttaatgatttatccagctttgaaatattttggcattctaacgccaacttctctttttcttgatcgtttaatggcttttgtgggtcaggcctgcaggatgactggagtgcttctgcatcacttatttcagatgcaagattaatgagaggtttgtgaggcttctgttcagaaacactgtccttgttgttattatcacgcacatcatgaaacatacttttttggacagtagatgtttcatgttttaaaggtctttgggaggaaggctgagtttttgatataacctgtccaggaggcattttctgttttgaatctttattattcaaagtttcacctttctttgactgatttagatttttaggcattgccactatttttgcattaaccttaggcaaagctgtgtgtacttgcttgaccatttttctcttaggtgcttgtttctctgtagttgtattgtggtccaactttgccacattttcatcagactgccttgaagagactgaagattttactgagtttggtgactctccttgggatccttgagttttagtaagattagatggggtactctttgtcctctgctgagctgcagtacatccattgctagttcctcttttcttcaaaattgcctgtggtactggctcactacatcctttgccactgactttctttagtacactgttatttacattagtgtcttgttcatgaatactttttttattggaagttccattggtaactcttgaaacaggtcgagattttatggctacagtggaatttttgacactatctacactgtttttcatcatctgtcctggagaatcacaaaaggatagtttatgtccagaaggcttttcttcttctgttgatccattttctttcggttcatccagacattcagtggaaattgagaattccatacttgaatctgtggatctgctggagggtcctgcgatgctgaggcatggtgaatccttccctgtagctttcttcaaaggctttgctttggcttgcacatttaagtttcctgtgagtaccttgggtctggcacctgaaatttgcccttcctgatttctcactccttttccatttagtaaattcttctgtccagttgctgctgctgctgctgttgctgatctttctacaacttgtctaggtgacatgttttccaaccgtgccttatcaccattttctgttttggattttgttacagttttgggctttccagaaacattttttcccccagtttttagttcttttgtaatcttagatgctatttttgtaccatctttttcctttacatcatcttgcttcagagttttatttatactatttctattggtacttgacgaatgtccagatgctcctaatccatcagatttcatctttttattagtagagagataactccaacactctttcttgttatttcccctccaagatttgatttttatatcaccagagtcagaaacttgtttcctttgctcagcctcctaaagtgctgggattacaggtgtgagccaccgcgcccgtcctattgtcattctttatgtaagtatgcaaacggttttttttttcctttggaagctgtatgagattgtagaggtctgaggcagagcctgtgctctcttcatcttttgtatccctcggcaccatgtcacatattggatactgcgagctactgaatataggctttttgccaagtcttcgatcatcacctttgtcaaatgcagctgcttggattttctgttgatcatctgtgctcatcagcttccagctttctgtgtgacgaacagcatagaaagact

SEQ ID NO: 11554 - RNA, 4232 nt, Homo sapiens
  source 1..4232: mol_type = other RNA
ctgaatagctgggactacaggtgcgtgccaccacgcctggctaatttttgtattttttgtttttttttagtagagacggggttttgccatgttggccacgctggtcttgaacttctggtcttgattaacccatctcagcctgccaaagtgctgggattacaggcatgagccactgtgcctggctccactttatcttcaatgtctctatttcctcttgtttaaatacaatggctaataagtctagaataacgctaagtaataacaccacactatggtcatgagttcaggttgggctatttataatataatcaatacctatgatgaaaccactgtccaacctcaaactagataattgctgataacaatacagacttattttacttgccatcctcttctcaccaccaaagtaaacattattgggaatttttatcattcttttgttttttatcatatatataatatacacacacataatagtcaattctcattttttgcagactccgtatgtgtgaatttacctcttgctaaaatttatttctaactccagtatcagtacttgctgggcttttgcagccatttgcggacatgcagcatgtgaaaaaatttgaattgcctgctctccatgttcccagctgaggtggaacaaggccttcttgtttcagttcttataaacaagtatccttttcagtctatttagtgccatgtcttttgcatttttgtggattttgctgcttaaagtgacccccacgcacagtgccaagtgttcctaagtgcaagaagactgtgatgtgccgcctggagaaactgaggtaagcttcattcaggaataagtgtcgtgggctaagttcagtgttaatgggtcaaccatatatactaaggtgtcttcaaacagaaacacatgtaacaagtttatgtactgatgggttgatgaaactgtgcccagaggttcataggaacccaaccctgtatttcccttgggaataatggttcagtactctctaattcagtgttcatggtgactttataaaacataactactatagataatgagaacagactatacatatatatatacacacacagtcaccgtttagtatccgtggaggattggttccagaaccttccttggatataaaaatcctctgatgctcaagtccctaatatgaagtatttggatataacctgtgcataccttctcatatacttttaagtcatctctagattacttataataccgaatacagtataaacaccatctaatactttgtattgtttagggaaaaatgacaaggaaaaatgtctgtacaggtttagtccagacacaattttccccctcaatattttcaacctgtagttggttgagtccatagatgtggaacccacatatacagacagccaaccgcatgtctaaacaagtttcacttgtttttgaacttctggagtatcataatgtacatgtcttctgacaccagcttttttcattcaacattattattaacattcacctatattgttactcacagctgcaggacaactttatgtccttgttttagatgtgtctcctgtaaacagcatatgattggggtttgttttaatattcaatttttccttgggctagtttaatacttatacatttattgtaattactgatctatttggacttgttttgccatcttttgttttatccaccttttctatgcttatttctcaaatttaaaattttgtttcttccctattatcccaccatctctcatcactattcattgagagattatatatacttctagcaattaacctcggaattttatcatgcatacttaaaaagactaagttgatattaactggctactcccaaaaatgtaagaacactgaaacattttgactctgattaaccttcccaccatgctgtctacttttaacctacctttaacaatttggcctgtcattatcattttgccgataagatctgtttacatttccctacctgtaagaaattatctatcattactatccacactttatgactcccataacttatatttcctgaggtacatatctcagaactgagttccaggctggggttcatgttgcttattactttcaaactattcacctttaggcatcatagtatctaccacttatctgtgcttactacataccaggtgatattctccacaagtgttgattaacctgacatttattaattcatggaatcctcataataccctaatggactatgtatgtttatgatccatatcttatgactcttataatttatctttcctaaggctacacatacctcagaactaggatccaggcctttttgattccccattgccttcactcaccttttcactccaacgtataatttcctgagttcttgaataatgacttatttctaagacacacagtggcgaggcggaactccaggataccagaggaaatggatgtctgaagttacacaggcaagtactctagcctacaaggcctctgggaaatgccatctagtctttgcttaaattgagccactggcagacctcagtataactcaaggctctatcctcgagttacagatagcacctaagaattttctgaagttttggggaaacctctttaatctttaacccacagatcttaattctgcctccccgaaccaaagtggcaaagagctccatcttactattaatgtattttaagatagtgactacacactctactcttttagttcagattaagcatccaattttcttagctattttttctccatggattcttattttcatttcctgtagaaatcacatgaatcctcaagaaaaggttgttttgccaatggacacctttccatattgaaaaccaaaagaacagtttggtaaaacagtaacatgccaaacacataaccaacttctctacctacaatattcacttcctagtttctgtgtgatctaaaacattttcctcccttccacccggcaataaactcacataagatgaaattaatttacaaaaggtaggctccgtttattagagtcacacacaactgactatctcagtgtgactcaagaccacaaaaaacccatttctccttcacttctgagtcctggggttaatacctagaccagcaagtgtactgcttggggtccattcacaggtttacaagtttttcattgagtgcaatctgtgactgtgtgaggttggccaggtaggtcaccatcaaaaggtcattgatgttgctgttgagcatggtctcaaagtcatcgggaactattttcggtacttggttaaccaggctcatcaggaagcggcccacagtattgtcagctgacacctttccagacagtacatcctctgcatattgcaacactgtactcagggcatcctggatgcgagctgatgcccctcctacttgctgcaagtcacttgagagtccaatcactctgttggggctaaagcaggtcttcatgatcaggtcaactccgatgcgttcagtgtcgtagtacgcgtatttcactgtcagaggcgtgaacatcactcccatggtcctcccagggactcccattaaagtgctgacgtaggctttgatgctcatgcggccgttctggagacttgtgtccacagtgaggtggatggggttgggggcctctcggctgtagtactcgtggatcagcacagagtgctctgtgatgtcatggcccgtagcgtaccagcccaggatgagctcatttggagaaacttttttatgcagttcatacatattcttagcaaattccatgtcaacagccacttcatcttctgactcattgtgcggcactgaaaagcaattggtgacctccactgagtgtttgtcgacagttcccaacagggtcccgataactcgggcagcaccctcgttgcgtctctcgtagctgtccacaatggaggccaaaatgactgggtgcagcctgaccacgcggccgccggggaagggccctggaagagcaggaccaggcagagcgggcgctggggtctgcgctggagcttgcgctgaggccggggtctggccaggagccgcagttgcagccgctgctgccgcagggtctgaggatgaggctggagccgcagcgggaaccggagccgcagccggtgctggcgttggcgctggaactgaggctggggccgccgccgggactggggttggcgtggccggaggagcacttactggtaccgccggtgtggccatcttgtcgagaaagaag

SEQ ID NO: 11555 - RNA, 6939 nt, Homo sapiens
  source 1..6939: mol_type = other RNA
ctgaatagctgggactacaggtgcgtgccaccaggcctggctaatttttctatttttactaagacagggtttcaccatattggccaagttggtctcaaactcctgacctcgtatttttttttttcttcaacagtcagtatctgttttcgtgcttacaaccaatacccccaacttttacagacacaaaagcaaacataatagacttattattccttgttatgggcactcgttaaacatttacaacacggaaacacatgtccttttgttctggaaaatgttttagagtggattctaggtttcatgtattcctccccctttttctggatgaagggagacaccaggatggcagttgtgtgcctctccttctagccccaagtcaagcttctaatggagtctttctaaggaagttgacgttggtagaattcctgctgcatcacaggggagtttcaggtcaatttatggtaaatacagaaaaagtcagtccccagaatgacaattattagctctaggtggaaaaaaagttatgtaggagggaaagcaaaatcatttttaccatgtagtttaactaagagtactggcaaggtcataagaaataaatgccaaatattgatataatcatattttaatacaaatatttctgaaagagacatgagaagagtattttatgtggtgagtttggggagagaaagacatctaaatgaataatgaatgtctaaaattgaaaaaaaaagtattagtgtcataagcatgctattcagaaaagtgaacataaataaaataatgagttagaagtagtaaaatttgttgtctcaaggtaacaaaaatgaggaagggcaagggactactatgtttcgggaaaaacaaaaacaaacaaacaaaaaacctgtaaagccctttgaccctttgcactacatgcacttataaaatacaaagaacaaggccaggagtggtcgctcatgcctgtaatcccagcaatttaggaggctgaggcaggtggatcacctgaggtccagagttcaagacaagtctgaccaacgtggagaaaccccgtctccactaaaaatacaaaattagccaggcatgttggcatatgcctgtaatcccagctattcaggaggctgaggcaggagaatcacttgaatccgggaggcagaggttgtggtgagccgagattgtgccattgcactccagcccgggcaacaaaagtgaaactccgtctcaaaaaaataataataaaataaaatacaaagaacattgcattgagataaaaattacaatgtatcattgatttgaattttttctgcatgtaattcatcagttaattttattctgtagaaatttttccctgctatttctccatggcaaatgaaagtagtgatcgtgaaacattgtgttttattcattcaaaacaacagaatacaagacaaaggaaaatatttctataccctacaagaaccaaaaatccaaaagtacacactaacactagaaaaagtgttctgaacaggttgaccatataacttattctaacaaggataatacgaaataaaccagaattatcccagacatttattactcatacttccaaatggaccttttcttacatcttacaagatagttagtgctctgaatctggaaaaatatgtgtaaaccgaccttgaggatttataaaatttccttagaaagcattgcagttaattctagaagctatttttctacctattgaatcactagaaatagagaagcttttaaaaaaattaacttgtttttagttttcagatacatgttttaagagcccagagtcttggctggaagaactctaatgaacagatcagtgaaaaaatatacttatacagaagtctgaaggtggagatcagtactttctagatgttacattttaatagtagctaaactaatgatgacatgtttatattgtcttatattttttaaagatattttcttatcactgttgtgaaaaagaaactttgtactcacaatttagcgtctccacttacactttataagcatctttataatatcgtcaatcttgctgaaatttcatataagcagtacaaaatacagtacatcattataaatcaaggagaagcattttggtcacagtgatctctaattacaatgtggactctctcaatttagaaaactactgttatacagctgtaatttttacttaatgccattctatacaaaccaatataacttggatgttcacaatccacgaatgcctactaaaagtatttttacttactttgtcttttaaattgataacccatgtattttaagtttatatatatagtattttagtaatacactgaattacttaaaacataaattggagtttttactaaaaattatatcttcacctacctgcctcccattttaagcatgattacaagtaaatgaaatttctattttattttctcaacatattatacctaaagttctttaaataaagtttgaaggtatctcttataataatatagtcaatgcatagtcatcatagttcaataagatgtgttctttccctgacaaaactgtgtactccattaacaagtcttcctatcttattataacaaagtaatttcctttcattggttactttaacataaatattaatggcattcaaaggaagcatagattcttaatgtattatccatcgatataaattatatgtgtatatatatatgtatatatatatatatatatgtaaaacttaagaagcattttgcttccaaagcagcaacttgtaaaaagtatctgtatttaaaatagaatttactggaattctgatcgtttattctgtggatctgtttttcatctgctttcttagtaacaatcagaatcataggtgcaaaagagtagagggggagaaacatacactagggagagtcccaaaactatcacgaattaagaatgatgttaaaaagatgacaatgaaagtgctttggtaagtaaagatgtccagagaaagaaaatgaatgaatggaatttcacaagcattacccctgagggtataacaggagcatcagaagacgtcagagaatttttgggaggacttcagatggctccaaattcctgaaaaaaccctacactctgtagaggaagaatatatagagaagaaaggacagagtaaatagttctcatcaatattttgaatgagagaccaaaaacacaaacacacacaaggaaaaagagacaagttccaaatgttctggaggctttgcaatactgcagtggtttgctacaaaagtctttcatgaagttcccagtaaaaaccaccatgacaatggtatctgactatactgtcccttccacacccagtcataattttctctcttaaaattggatttatatttccccatactacaactgtaaaaatgttttcctgctcacatacactaatcattgagaatttggttattggagttttccagaaagtaatattttgattgtctttaccattcagaaaagaaattatttaccttttaattgatgctaagcttgcttcaccatgcaaaccaataaattcactcacagaatctttgattgatctgatagtagagtgctttcttgtaaactgcctttcaagtttgttacactaatatatttgtggaaacatttcatgaatccaggtataaaaagatctttaagcaaacataataaaaatgagagtttacccttcttgcatatacttaagcacaaccaggaaatggtcgtttttattttttcactcctgaaaagggttaaaagaaactcacaaattttataattcacagaaatgtgggcacttaccatttctgtaattcacaaaacaagtgcattatttggcatacatggtgtttaaggctaaaatcataaaatactcactaattagcttaaaagtgtaaattacatcttagaatctgtctaggcaacaggagaatttggatttgctttatttaagattatcatgaagtccacaactttgatatttaaatacagccttcataatgaatcttttctagatggtggtctttagaaatctttagagataaataatgaatcttttagacatgaatgatcactatatttaacaataaccattgtcctttcaaggtaaccatgacagttttattcagtttggcaaatacttttcattgttagcctacatctagaatttaaacaatattaggtatggtctctaattgctttgactgttggtgatgtcattagggctgtctttgtctgaatagtgaagcagaagtttccctttgtatttttctgtggtttgattcctttctcctgttgcctgtaccctcccaatttcttttttccctcccaaatttctaccctaccgtcctatgccaccactttcaactgtcacttttagtggtatattatattcaactttcacataatcattaaaaaataataactaggtgcctgacccttttgagagaatttacatattaaaaataattctcaaaagtagacaaaatatgtccaaaacattaagttatttattattcgactatctactacatttgctcctaaggctagacctgggatggcggcaagaattctatacagaatgagagataaataaatatgagaatagtaaaggattgccctctcgcatttatcttcctcttgaatattcatttcttctactgccaggtattcttctggactatgctgatagagtggattctagaagtatggacagagataccccatttctagaatccatcccatatttcactttttagttaacaaaaatgtcttggttaatcactgcagtcaatatttgttggtaaactctccagctttgagactcccctttcctcttctaaccatgctctgaattgcccagtattgtgctttgaccctgcttctcagctctagaagtgaacccttagtttacttaagccattccatcctttctggtcatgttgcctatttaacaatgaaaaaataatcaaatttgtttgctccatttgagaagcaaactctctaccagacagaaacaaggatgtatgaattgccaagagttggcagccatcttgccaacacaagaggaaagcctgcatgagagtgaggccaagaccagggaaatggatccaacactctggaaagggattcagaagccagtttatgcccatacttaattctagacacaacatttaagccctggtaaatagcccttgcccaaagcttaatctcccctggatcattctgttatatgatacagtaagttttcttttgtatataaaccagttagagtcaggttttctgaaacagttctatgaaaaatgattttaggtaatgaagtatttttcctatcaaagtaactcaattcagacaactagtatctaaggtagaccttgggtagtggaaaaaaattgcataaagatccatgcatgagtacataagagtcattactaatgcactcatgtcaagaataagcttaaactctagtctttggtctgcgagagaaggttggatagttgacataaatatcctctcttgtatcatccatggattgattggtaggttgactggtagagatgggacttctatagttattgggtgccttctgtgtatcccaggactctgtaaatagatctcttctctctctccttctccttctgttaaggaaaatgacaatgatggtggtaattgagataacaaacaacaacaataaaactgtccctccagccacaaagagggtatattggttatcggttttaccctcggctacagtcaatctcatcacgaaggtttcgttttctcctgcgctggcctgcaagtagcagcggtaaagccccgagtctgagactgtgacatcggggatgacgatgacgctccaccttccgtggctgcagttgctcactatttgtcttgggaacttggaggtgaaatttctgccatggaccaagttgcagtaagttaagaggtcgatctgacggggctggatcttttcccacctcactgcctgcacaggccacgtcatctgaggctgacaagtgagtgtgacattctttccaggttccgaaacaatgtggctatttgatggcacagctgcctcaaaactatctgactgaaccacctgtatcaccttctgccaagttccctgtgggtaagtgtaaagagagcaggaatagtagccaacatcatcttcagaggcattccgaaagaaaagagtcatgttattggaagccatcgttgaattcaaaaagtaaaccctctcagcatagggcttccttatgaccatgccatgagtagggctgaaaatggctatggaatcctgctgggtcccgatcttgaaccactccacctgtgttaagatgcccattgatggatacacacattctagagacatgttctcggcaaagggaactgatgtatgccaaagcacctcttcacatagagctctgtatacatgaagaagagccaaaagtaaagtaggataatccatctctggaaactgtttgaaaggctggttctattaaaaaaaaaaattgctttttataatgtgacatgcagatccccagcacaatgcagtttccttcctctcagatgttatcagtcgtgtcttctttttctgaagtatgaacacaggaaaaaggccttagcttaaaagacaggtttgctcctttatgaggatgggcagatttgagtttcttctctctcggggaaccagtcggcttattttcgggctttcattttctacaaggagtcattcattcaacaaacatgtgctgcatgcattctctgtgcctaactcagctgtaggcaatgaggatacaataatacaaaaaaaaaaaaatattgccatgatagaacttacattctatgtggaggaggcagaaactaaaataaagatgtaaaaatataaataataagtgaaaggtggtgcatgcatggagcagagaagtcctcact

SEQ ID NO: 11556 - RNA, 6544 nt, Homo sapiens
  source 1..6544: mol_type = other RNA
ctgaatagctgggactacaggtgcgtgccaccaggcctggctaatttttctatttttactaagacagggtttcaccatattggccaagttggtctcaaactcctgacctcgtatttttttttttcttcaacagtcagtatctgttttcgtgcttacaaccaatacccccaacttttacagacacaaaagcaaacataatagacttattattccttgttatgggcactcgttaaacatttacaacacggaaacacatgtccttttgttctggaaaatgttttagagtggattctaggtttcatgtattcctccccctttttctggatgaagggagacaccaggatggcagttgtgtgcctctccttctagccccaagtcaagcttctaatggagtctttctaaggaagttgacgttggtagaattcctgctgcatcacaggggagtttcaggtcaatttatggtaaatacagaaaaagtcagtccccagaatgacaattattagctctaggtggaaaaaaagttatgtaggagggaaagcaaaatcatttttaccatgtagtttaactaagagtactggcaaggtcataagaaataaatgccaaatattgatataatcatattttaatacaaatatttctgaaagagacatgagaagagtattttatgtggtgagtttggggagagaaagacatctaaatgaataatgaatgtctaaaattgaaaaaaaaagtattagtgtcataagcatgctattcagaaaagtgaacataaataaaataatgagttagaagtagtaaaatttgttgtctcaaggtaacaaaaatgaggaagggcaagggactactatgtttcgggaaaaacaaaaacaaacaaacaaaaaacctgtaaagccctttgaccctttgcactacatgcacttataaaatacaaagaacaaggccaggagtggtcgctcatgcctgtaatcccagcaatttaggaggctgaggcaggtggatcacctgaggtccagagttcaagacaagtctgaccaacgtggagaaaccccgtctccactaaaaatacaaaattagccaggcatgttggcatatgcctgtaatcccagctattcaggaggctgaggcaggagaatcacttgaatccgggaggcagaggttgtggtgagccgagattgtgccattgcactccagcccgggcaacaaaagtgaaactccgtctcaaaaaaataataataaaataaaatacaaagaacattgcattgagataaaaattacaatgtatcattgatttgaattttttctgcatgtaattcatcagttaattttattctgtagaaatttttccctgctatttctccatggcaaatgaaagtagtgatcgtgaaacattgtgttttattcattcaaaacaacagaatacaagacaaaggaaaatatttctataccctacaagaaccaaaaatccaaaagtacacactaacactagaaaaagtgttctgaacaggttgaccatataacttattctaacaaggataatacgaaataaaccagaattatcccagacatttattactcatacttccaaatggaccttttcttacatcttacaagatagttagtgctctgaatctggaaaaatatgtgtaaaccgaccttgaggatttataaaatttccttagaaagcattgcagttaattctagaagctatttttctacctattgaatcactagaaatagagaagcttttaaaaaaattaacttgtttttagttttcagatacatgttttaagagcccagagtcttggctggaagaactctaatgaacagatcagtgaaaaaatatacttatacagaagtctgaaggtggagatcagtactttctagatgttacattttaatagtagctaaactaatgatgacatgtttatattgtcttatattttttaaagatattttcttatcactgttgtgaaaaagaaactttgtactcacaatttagcgtctccacttacactttataagcatctttataatatcgtcaatcttgctgaaatttcatataagcagtacaaaatacagtacatcattataaatcaaggagaagcattttggtcacagtgatctctaattacaatgtggactctctcaatttagaaaactactgttatacagctgtaatttttacttaatgccattctatacaaaccaatataacttggatgttcacaatccacgaatgcctactaaaagtatttttacttactttgtcttttaaattgataacccatgtattttaagtttatatatatagtattttagtaatacactgaattacttaaaacataaattggagtttttactaaaaattatatcttcacctacctgcctcccattttaagcatgattacaagtaaatgaaatttctattttattttctcaacatattatacctaaagttctttaaataaagtttgaaggtatctcttataataatatagtcaatgcatagtcatcatagttcaataagatgtgttctttccctgacaaaactgtgtactccattaacaagtcttcctatcttattataacaaagtaatttcctttcattggttactttaacataaatattaatggcattcaaaggaagcatagattcttaatgtattatccatcgatataaattatatgtgtatatatatatgtatatatatatatatatatgtaaaacttaagaagcattttgcttccaaagcagcaacttgtaaaaagtatctgtatttaaaatagaatttactggaattctgatcgtttattctgtggatctgtttttcatctgctttcttagtaacaatcagaatcataggtgcaaaagagtagagggggagaaacatacactagggagagtcccaaaactatcacgaattaagaatgatgttaaaaagatgacaatgaaagtgctttggtaagtaaagatgtccagagaaagaaaatgaatgaatggaatttcacaagcattacccctgagggtataacaggagcatcagaagacgtcagagaatttttgggaggacttcagatggctccaaattcctgaaaaaaccctacactctgtagaggaagaatatatagagaagaaaggacagagtaaatagttctcatcaatattttgaatgagagaccaaaaacacaaacacacacaaggaaaaagagacaagttccaaatgttctggaggctttgcaatactgcagtggtttgctacaaaagtctttcatgaagttcccagtaaaaaccaccatgacaatggtatctgactatactgtcccttccacacccagtcataattttctctcttaaaattggatttatatttccccatactacaactgtaaaaatgttttcctgctcacatacactaatcattgagaatttggttattggagttttccagaaagtaatattttgattgtctttaccattcagaaaagaaattatttaccttttaattgatgctaagcttgcttcaccatgcaaaccaataaattcactcacagaatctttgattgatctgatagtagagtgctttcttgtaaactgcctttcaagtttgttacactaatatatttgtggaaacatttcatgaatccaggtataaaaagatctttaagcaaacataataaaaatgagagtttacccttcttgcatatacttaagcacaaccaggaaatggtcgtttttattttttcactcctgaaaagggttaaaagaaactcacaaattttataattcacagaaatgtgggcacttaccatttctgtaattcacaaaacaagtgcattatttggcatacatggtgtttaaggctaaaatcataaaatactcactaattagcttaaaagtgtaaattacatcttagaatctgtctaggcaacaggagaatttggatttgctttatttaagattatcatgaagtccacaactttgatatttaaatacagccttcataatgaatcttttctagatggtggtctttagaaatctttagagataaataatgaatcttttagacatgaatgatcactatatttaacaataaccattgtcctttcaaggtaaccatgacagttttattcagtttggcaaatacttttcattgttagcctacatctagaatttaaacaatattaggtatggtctctaattgctttgactgttggtgatgtcattagggctgtctttgtctgaatagtgaagcagaagtttccctttgtatttttctgtggtttgattcctttctcctgttgcctgtaccctcccaatttcttttttccctcccaaatttctaccctaccgtcctatgccaccactttcaactgtcacttttagtggtatattatattcaactttcacataatcattaaaaaataataactaggtgcctgacccttttgagagaatttacatattaaaaataattctcaaaagtagacaaaatatgtccaaaacattaagttatttattattcgactatctactacatttgctcctaaggctagacctgggatggcggcaagaattctatacagaatgagagataaataaatatgagaatagtaaaggattgccctctcgcatttatcttcctcttgaatattcatttcttctactgccaggtattcttctggactatgctgatagagtggattctagaagtatggacagagataccccatttctagaatccatcccatatttcactttttagttaacaaaaatgtcttggttaatcactgcagtcaatatttgttggtaaactctccagctttgagactcccctttcctcttctaaccatgctctgaattgcccagtattgtgctttgaccctgcttctcagctctagaagtgaacccttagtttacttaagccattccatcctttctggtcatgttgcctatttaacaatgaaaaaataatcaaatttgtttgctccatttgagaagcaaactctctaccagacagaaacaaggatgtatgaattgccaagagttggcagccatcttgccaacacaagaggaaagcctgcatgagagtgaggccaagaccagggaaatggatccaacactctggaaagggattcagaagccagtttatgcccatacttaattctagacacaacatttaagccctggtaaatagcccttgcccaaagcttaatctcccctggatcattctgttatatgatacagtaagttttcttttgtatataaaccagttagagtcaggttttctgaaacagttctatgaaaaatgattttaggtaatgaagtatttttcctatcaaagtaactcaattcagacaactagtatctaaggtagaccttgggtagtggaaaaaaattgcataaagatccatgcatgagtacataagagtcattactaatgcactcatgtcaagaataagcttaaactctagtctttggtctgcgagagaaggttggatagttgacataaatatcctctcttgtatcatccatggattgattggtaggttgactggtagagatgggacttctatagttattgggtgccttctgtgtatcccaggactctgtaaatagatctcttctctctctccttctccttctgttaaggaaaatgacaatgatggtggtaattgagataacaaacaacaacaataaaactgtccctccagccacaaagagggtatattggttatcggttttaccctcggctacagtcaatctcatcacgaaggtttcgttttctcctgcgctggcctgcaagtagcagcggtaaagccccgagtctgagactgtgacatcggggatgacgatgacgctccaccttccgtggctgcagttgctcactatttgtcttgggaacttggaggtgaaatttctgccatggaccaagttgcagtaagttaagaggtcgatctgacggggctggatcttttcccacctcactgcctgcacaggccacgtcatctgaggctgacaagtgagtgtgacattctttccaggttccgaaacaatgtggctatttgatggcacagctgcctcaaaactatctgactgaaccacctgtatcaccttctgccaagttccctgtgggtaagtgtaaagagagcaggaatagtagccaacatcatcttcagaggcattccgaaagaaaagagtcatgttattggaagccatcgttgaattcaaaaagtaaaccctctcagcatagggcttccttatgaccatgccatgagtagggctgaaaatggctatggaatcctgctgggtcccgatcttgaaccactccacctgtgttaagatgcccattgatggatacacacattctagagacatgttctcggcaaagggaactgatgtatgccaaagcacctcttcacatagagctctgtatacatgaagaagagccaaaagtaaagtaggataatccatctctggaaactgtttgaaaggctggttcttgagatgtgagtgctgctcgctctaacgcttcttcccatctgc

SEQ ID NO: 11557 - RNA, 6135 nt, Homo sapiens
  source 1..6135: mol_type = other RNA
ctgaatagctgggactacaggtgcgtgccaccaggcctggctaatttttctatttttactaagacagggtttcaccatattggccaagttggtctcaaactcctgacctcgtatttttttttttcttcaacagtcagtatctgttttcgtgcttacaaccaatacccccaacttttacagacacaaaagcaaacataatagacttattattccttgttatgggcactcgttaaacatttacaacacggaaacacatgtccttttgttctggaaaatgttttagagtggattctaggtttcatgtattcctccccctttttctggatgaagggagacaccaggatggcagttgtgtgcctctccttctagccccaagtcaagcttctaatggagtctttctaaggaagttgacgttggtagaattcctgctgcatcacaggggagtttcaggtcaatttatggtaaatacagaaaaagtcagtccccagaatgacaattattagctctaggtggaaaaaaagttatgtaggagggaaagcaaaatcatttttaccatgtagtttaactaagagtactggcaaggtcataagaaataaatgccaaatattgatataatcatattttaatacaaatatttctgaaagagacatgagaagagtattttatgtggtgagtttggggagagaaagacatctaaatgaataatgaatgtctaaaattgaaaaaaaaagtattagtgtcataagcatgctattcagaaaagtgaacataaataaaataatgagttagaagtagtaaaatttgttgtctcaaggtaacaaaaatgaggaagggcaagggactactatgtttcgggaaaaacaaaaacaaacaaacaaaaaacctgtaaagccctttgaccctttgcactacatgcacttataaaatacaaagaacaaggccaggagtggtcgctcatgcctgtaatcccagcaatttaggaggctgaggcaggtggatcacctgaggtccagagttcaagacaagtctgaccaacgtggagaaaccccgtctccactaaaaatacaaaattagccaggcatgttggcatatgcctgtaatcccagctattcaggaggctgaggcaggagaatcacttgaatccgggaggcagaggttgtggtgagccgagattgtgccattgcactccagcccgggcaacaaaagtgaaactccgtctcaaaaaaataataataaaataaaatacaaagaacattgcattgagataaaaattacaatgtatcattgatttgaattttttctgcatgtaattcatcagttaattttattctgtagaaatttttccctgctatttctccatggcaaatgaaagtagtgatcgtgaaacattgtgttttattcattcaaaacaacagaatacaagacaaaggaaaatatttctataccctacaagaaccaaaaatccaaaagtacacactaacactagaaaaagtgttctgaacaggttgaccatataacttattctaacaaggataatacgaaataaaccagaattatcccagacatttattactcatacttccaaatggaccttttcttacatcttacaagatagttagtgctctgaatctggaaaaatatgtgtaaaccgaccttgaggatttataaaatttccttagaaagcattgcagttaattctagaagctatttttctacctattgaatcactagaaatagagaagcttttaaaaaaattaacttgtttttagttttcagatacatgttttaagagcccagagtcttggctggaagaactctaatgaacagatcagtgaaaaaatatacttatacagaagtctgaaggtggagatcagtactttctagatgttacattttaatagtagctaaactaatgatgacatgtttatattgtcttatattttttaaagatattttcttatcactgttgtgaaaaagaaactttgtactcacaatttagcgtctccacttacactttataagcatctttataatatcgtcaatcttgctgaaatttcatataagcagtacaaaatacagtacatcattataaatcaaggagaagcattttggtcacagtgatctctaattacaatgtggactctctcaatttagaaaactactgttatacagctgtaatttttacttaatgccattctatacaaaccaatataacttggatgttcacaatccacgaatgcctactaaaagtatttttacttactttgtcttttaaattgataacccatgtattttaagtttatatatatagtattttagtaatacactgaattacttaaaacataaattggagtttttactaaaaattatatcttcacctacctgcctcccattttaagcatgattacaagtaaatgaaatttctattttattttctcaacatattatacctaaagttctttaaataaagtttgaaggtatctcttataataatatagtcaatgcatagtcatcatagttcaataagatgtgttctttccctgacaaaactgtgtactccattaacaagtcttcctatcttattataacaaagtaatttcctttcattggttactttaacataaatattaatggcattcaaaggaagcatagattcttaatgtattatccatcgatataaattatatgtgtatatatatatgtatatatatatatatatatgtaaaacttaagaagcattttgcttccaaagcagcaacttgtaaaaagtatctgtatttaaaatagaatttactggaattctgatcgtttattctgtggatctgtttttcatctgctttcttagtaacaatcagaatcataggtgcaaaagagtagagggggagaaacatacactagggagagtcccaaaactatcacgaattaagaatgatgttaaaaagatgacaatgaaagtgctttggtaagtaaagatgtccagagaaagaaaatgaatgaatggaatttcacaagcattacccctgagggtataacaggagcatcagaagacgtcagagaatttttgggaggacttcagatggctccaaattcctgaaaaaaccctacactctgtagaggaagaatatatagagaagaaaggacagagtaaatagttctcatcaatattttgaatgagagaccaaaaacacaaacacacacaaggaaaaagagacaagttccaaatgttctggaggctttgcaatactgcagtggtttgctacaaaagtctttcatgaagttcccagtaaaaaccaccatgacaatggtatctgactatactgtcccttccacacccagtcataattttctctcttaaaattggatttatatttccccatactacaactgtaaaaatgttttcctgctcacatacactaatcattgagaatttggttattggagttttccagaaagtaatattttgattgtctttaccattcagaaaagaaattatttaccttttaattgatgctaagcttgcttcaccatgcaaaccaataaattcactcacagaatctttgattgatctgatagtagagtgctttcttgtaaactgcctttcaagtttgttacactaatatatttgtggaaacatttcatgaatccaggtataaaaagatctttaagcaaacataataaaaatgagagtttacccttcttgcatatacttaagcacaaccaggaaatggtcgtttttattttttcactcctgaaaagggttaaaagaaactcacaaattttataattcacagaaatgtgggcacttaccatttctgtaattcacaaaacaagtgcattatttggcatacatggtgtttaaggctaaaatcataaaatactcactaattagcttaaaagtgtaaattacatcttagaatctgtctaggcaacaggagaatttggatttgctttatttaagattatcatgaagtccacaactttgatatttaaatacagccttcataatgaatcttttctagatggtggtctttagaaatctttagagataaataatgaatcttttagacatgaatgatcactatatttaacaataaccattgtcctttcaaggtaaccatgacagttttattcagtttggcaaatacttttcattgttagcctacatctagaatttaaacaatattaggtatggtctctaattgctttgactgttggtgatgtcattagggctgtctttgtctgaatagtgaagcagaagtttccctttgtatttttctgtggtttgattcctttctcctgttgcctgtaccctcccaatttcttttttccctcccaaatttctaccctaccgtcctatgccaccactttcaactgtcacttttagtggtatattatattcaactttcacataatcattaaaaaataataactaggtgcctgacccttttgagagaatttacatattaaaaataattctcaaaagtagacaaaatatgtccaaaacattaagttatttattattcgactatctactacatttgctcctaaggctagacctgggatggcggcaagaattctatacagaatgagagataaataaatatgagaatagtaaaggattgccctctcgcatttatcttcctcttgaatattcatttcttctactgccaggtattcttctggactatgctgatagagtggattctagaagtatggacagagataccccatttctagaatccatcccatatttcactttttagttaacaaaaatgtcttggttaatcactgcagtcaatatttgttggtaaactctccagctttgagactcccctttcctcttctaaccatgctctgaattgcccagtattgtgctttgaccctgcttctcagctctagaagtgaacccttagtttacttaagccattccatcctttctggtcatgttgcctatttaacaatgaaaaaataatcaaatttgtttgctccatttgagaagcaaactctctaccagacagaaacaaggatgtatgaattgccaagagttggcagccatcttgccaacacaagaggaaagcctgcatgagagtgaggccaagaccagggaaatggatccaacactctggaaagggattcagaagccagtttatgcccatacttaattctagacacaacatttaagccctggtaaatagcccttgcccaaagcttaatctcccctggatcattctgttatatgatacagtaagttttcttttgtatataaaccagttagagtcaggttttctgaaacagttctatgaaaaatgattttaggtaatgaagtatttttcctatcaaagtaactcaattcagacaactagtatctaaggtagaccttgggtagtggaaaaaaattgcataaagatccatgcatgagtacataagagtcattactaatgcactcatgtcaagaataagcttaaactctagtctttggtctgcgagagaaggttggatagttgacataaatatcctctcttgtatcatccatggattgattggtaggttgactggtagagatgggacttctatagttattgggtgccttctgtgtatcccaggactctgtaaatagatctcttctctctctccttctccttctgttaaggaaaatgacaatgatggtggtaattgagataacaaacaacaacaataaaactgtccctccagccacaaagagggtatattggttatcggttttaccctcggctacagtcaatctcatcacgaaggtttcgttttctcctgcgctggcctgcaagtagcagcggtaaagccccgagtctgagactgtgacatcggggatgacgatgacgctccaccttccgtggctgcagttgctcactatttgtcttgggaacttggaggtgaaatttctgccatggaccaagttgcagtaagttaagaggtcgatctgacggggctggatcttttcccacctcactgcctgcacaggccacgtcatctgaggctgacaagtgagtgtgacattctttccaggttccgaaacaatgtggctatttgatggcacagctgcctcaaaactatcttgagatgtgagtgctgctcgctctaacgcttcttcccatctgc

SEQ ID NO: 11558 - RNA, 3470 nt, Homo sapiens
  source 1..3470: mol_type = other RNA
ctgaatagctgggactacaggtgcgtgccaccatgcctggctagtttttgtatttttagtggagatgaggtttctccattttggccaggctcttgacctcaagtgatccacccacctcagcctcccaagtgctgggatacaggcctaagatgctgcacctggccccgtgcccatcttttcttatgagaaagcccacagtgttctgtacacacactaatagttcagcataatttggccttcaacaggggcactgagatgataaggaatgtccttttttaccccatccccaaggttcttctcaagagtgtcaccagccctccctctacctggcttttttccccagccctccctctacctggctttttttctgttctgcagaaacactgtgctcctgttctggcaaagctgcgcccaccgcctgacaatcaggacgcctatcgggcagaattcgggtcccttgggcccctcctctgctcccaggtggtcaaggctcgggcccaggctgctctgcaggctcagcaggtcaacaggaccactctgaccatcacgcaggtccgtggccgggtggggaggaggaataggaggaagcagaggagaacccctgtgtgggacaggcacttgcacacagccacatgtgccctcagtcagtagtctcagggcaaccaggccctgagtgaggatgccccagccctagtgagagccactgaggaagagcgaggggagcccaggcctctcccttcagactcctcttcttagtagatggtgccacttccccctttcctcttctccccgcagccccggcccacgctgaccctctcgcaggccccacagcctggccctcgcacccctggcttgctgaaggttcctggctccatcgcacttcctgtccagacactggtgtctgcacgagcggctgccccaccacagccttcccctcctccaaccaagtttattgtaatgtcatcgtcctccagcgccccatccacccagcaggtatgcagagctgtgggacagggagcatctggagggcctgggttacctcagagcaccctggggaggcccaggagtagagcacagtcccctctgggccccaagtcaagagctggaagaggcgcccaccagggtcctgcagggctgtagctgccctgcatgaacaaggtctccagccatagctgtctacagggtgaactacaggaacaacttgttcaggcagggagcgagtgaagcgtcctcgccaggcctctggggggcagggagggcacagggcaagcggcctgcctttcctttctatccaggtcctgtccctcagcacctcggcccccggctcaggttccaccaccacttcgcccgtcaccaccaccgtccccagcgtgcagcccatcgtcaagttggtctccaccgccaccaccgcaccccccagcactgctccctctggtcctgggagtgtccagaagtacatcgtggtctcacttcccccaacaggggagggcaaaggaggccccacctcccatccttctccagttcctcccccggcatcgtccccgtccccactcagcggcagtgccctttgtggggggaagcaggaggctggggacagtccccctccagctccagggactccaaaagccaatggctcccagcccaactccggctcccctcagcctgctccgtgatgctccacctgccagcccccggattcccacacatgcagacatgtacacacgtgcacgtacacacatgcatgctcgctaagcggaaggaagttgtagattgcttccttcatgtcactttctttttagatattgtacagccagtttctcagaataaaagtttggtttgtaagttctgatccactgcagtccttcctgcatcagataccacagaaaggctgggcccattgccccctcctggtcttgggactgaggactcttcctgcccagattcagagtccgaaggccaggaggctggaaaagaaacgactgtcctcccgtgggacaaactgccaccttggccgtcgtgtcctcgtttggggagcctcagatccgaatgacataggcgtcgctgtggcttaggtgtcgcacccacttgtgggggttggcattgccgcatggcctgaaggccagcctgaggaatcggacctggaggccagagcacgtgtgccggggaagctcgaaggagagactggcagggcccagccccagaggagaggccgaggtggagagcccatggctgggaggtcctgggggccctgggacgtccatctggaaaaggcctgagagttgagagcctccttgcacccgaggcaggtcccagcgaagggctccctctgccagctcagccttctgctctgggctgctcagctcctgagacaggctgaccacccctcgaggcagggggaggtgcagcctgacattgagggcttggctctttgagagcaggtcacatcgcaactttagataaacctggagccggcctgagcctcggtcccactgcacagaggggaagagccggaaggggagcggtgaggggaggtcatcggagagttggtaccgcatcacagtcagctcgccctgaggtggttgcaagcggaggattcgatgagactcaaattcgtccagattcacagagctgtgaaacgagacttcatcgacccggattcctggcccataacctctcagctctgacttccccacacaaaactcttccgtcaagccaatgcgcatctcagagccgctaggaaggaagctcttgagccgaatctctccctgcacatccaccttcagcagggatccattagatgctatcagtacagacaatctctcgaccacatccaaaaaaacttcattcttttggctctggtcagagcgactggacaggacggggcggctggctgcactgctgggggccactttgctctgttgtgtctcagccccaaacaagccaacgctgctgaggtcaaagaggctgaagggcttgctgaccacagcttccgtctggatgaaattcctcagcatctccgtggatgtggtctgtacatagccatagtccagcacttcatccaggagttcgtataccagagccacattgcgggagatggtcccctcgcccagggagccacagtaatcgcccagaagggtggccaacctggagagcagttctaggaggctgaagggagaaacgttttctgaagttgtgaccaccaaatagaggccgctgtgtctgatgtgaatgaaatgacggccatggtgatgcatgacaaccggggactcgtctcctggcagtcccgtcagcttccggtagaagagctcggccacatcccggccgccactgtccccgcggaagtctttgtagatgagcgggtcccccttggaggacagaatgaagaattgggaaatcatggccgttctggagagtagacaagaagacggcgaaagtcgggcctgccccgccctgcggccccggaacaaaag

SEQ ID NO: 11559 - RNA, 3491 nt, Homo sapiens
  source 1..3491: mol_type = other RNA
ctgaatagctgggactacaggtgcgtgccaccatgcctggctagtttttgtatttttagtggagatgaggtttctccattttggccaggctcttgacctcaagtgatccacccacctcagcctcccaagtgctgggatacaggcctaagatgctgcacctggccccgtgcccatcttttcttatgagaaagcccacagtgttctgtacacacactaatagttcagcataatttggccttcaacaggggcactgagatgataaggaatgtccttttttaccccatccccaaggttcttctcaagagtgtcaccagccctccctctacctggcttttttccccagccctccctctacctggctttttttctgttctgcagaaacactgtgctcctgttctggcaaagctgcgcccaccgcctgacaatcaggacgcctatcgggcagaattcgggtcccttgggcccctcctctgctcccaggtggtcaaggctcgggcccaggctgctctgcaggctcagcaggtcaacaggaccactctgaccatcacgcaggtccgtggccgggtggggaggaggaataggaggaagcagaggagaacccctgtgtgggacaggcacttgcacacagccacatgtgccctcagtcagtagtctcagggcaaccaggccctgagtgaggatgccccagccctagtgagagccactgaggaagagcgaggggagcccaggcctctcccttcagactcctcttcttagtagatggtgccacttccccctttcctcttctccccgcagccccggcccacgctgaccctctcgcaggccccacagcctggccctcgcacccctggcttgctgaaggttcctggctccatcgcacttcctgtccagacactggtgtctgcacgagcggctgccccaccacagccttcccctcctccaaccaagtttattgtaatgtcatcgtcctccagcgccccatccacccagcaggtatgcagagctgtgggacagggagcatctggagggcctgggttacctcagagcaccctggggaggcccaggagtagagcacagtcccctctgggccccaagtcaagagctggaagaggcgcccaccagggtcctgcagggctgtagctgccctgcatgaacaaggtctccagccatagctgtctacagggtgaactacaggaacaacttgttcaggcagggagcgagtgaagcgtcctcgccaggcctctggggggcagggagggcacagggcaagcggcctgcctttcctttctatccaggtcctgtccctcagcacctcggcccccggctcaggttccaccaccacttcgcccgtcaccaccaccgtccccagcgtgcagcccatcgtcaagttggtctccaccgccaccaccgcaccccccagcactgctccctctggtcctgggagtgtccagaagtacatcgtggtctcacttcccccaacaggggagggcaaaggaggccccacctcccatccttctccagttcctcccccggcatcgtccccgtccccactcagcggcagtgccctttgtggggggaagcaggaggctggggacagtccccctccagctccagggactccaaaagccaatggctcccagcccaactccggctcccctcagcctgctccgtgatgctccacctgccagcccccggattcccacacatgcagacatgtacacacgtgcacgtacacacatgcatgctcgctaagcggaaggaagttgtagattgcttccttcatgtcactttctttttagatattgtacagccagtttctcagaataaaagtttggtttgtaagttctgatccactgcagtccttcctgcatcagataccacagaaaggctgggcccattgccccctcctggtcttgggactgaggactcttcctgcccagattcagagtccgaaggccaggaggctggaaaagaaacgactgtcctcccgtgggacaaactgccaccttggccgtcgtgtcctcgtttggggagcctcagatccgaatgacataggcgtcgctgtggcttaggtgtcgcacccacttgtgggggttggcattgccgcatggcctgaaggccagcctgaggaatcggacctggaggccagagcacgtgtgccggggaagctcgaaggagagactggcagggcccagccccagaggagaggccgaggtggagagcccatggctgggaggtcctgggggccctgggacgtccatctggaaaaggcctgagagttgagagcctccttgcacccgaggcaggtcccagcgaagggctccctctgccagctcagccttctgctctgggctgctcagctcctgagacaggctgaccacccctcgaggcagggggaggtgcagcctgacattgagggcttggctctttgagagcaggtcacatcgcaactttagataaacctggagccggcctgagcctcggtcccactgcacagaggggaagagccggaaggggagcggtgaggggaggtcatcggagagttggtaccgcatcacagtcagctcgccctgaggtggttgcaagcggaggattcgatgagactcaaattcgtccagattcacagagctgtgaaacgagacttcatcgacccggattcctggcccataacctctcagctctgacttccccacacaaaactcttccgtcaagccaatgcgcatctcagagccgctaggaaggaagctcttgagccgaatctctccctgcacatccaccttcagcagggatccattagatgctatcagtacagacaatctctcgaccacatccaaaaaaacttcattcttttggctctggtcagagcgactggacaggacggggcggctggctgcactgctgggggccactttgctctgttgtgtctcagccccaaacaagccaacgctgctgaggtcaaagaggctgaagggcttgctgaccacagcttccgtctggatgaaattcctcagcatctccgtggatgtggtctgtacatagccatagtccagcacttcatccaggagttcgtataccagagccacattgcgggagatggtcccctcgcccagggagccacagtaatcgcccagaagggtggccaacctggagagcagttctaggaggctgaagggagaaacgttttctgaagttgtgaccaccaaatagaggccgctgtgtctgatgtgaatgaaatgacggccatggtgatgccgcctcccgccactggttaccatgacaaccggggactcgtctcctggcagtcccgtcagcttccggtagaagagctcggccacatcccggccgccactgtccccgcggaagtctttgtagatgagcgggtcccccttggaggacagaatgaagaattgggaaatcatggccgttctggagagtagacaagaagacggcgaaagtcgggcctgccccgccctgcggccccggaacaaaag

SEQ ID NO: 11560 - RNA, 8887 nt, Homo sapiens
  source 1..8887: mol_type = other RNA
ctgaatagctgggactacaggtgcgtgccaccatgctcagctaatttttgcattttttgtagagatggtgtctcattatgttacccaggctggtcttgaactcctgggctcaagcgatcctgaaaccttggcctcccagagtgctgggattataggtatgagccaccactaggtctactttaaaagaaatgcttaatggagtttttcaagtaaaaatgaaagaaagcagctgggtgtggtggctcatgcctgtaatcccagcattttgggaggccaaggagggtggatcacttgaggtcaggaggtcaagtccagccaggccaacatggcaaaaacccacgccttctaaaaatgcaaaaaattaaccaggtgtggtggcgggtgcctgtaatcccaactactcagggggctgaggcaggagaatcaattaaaccatgaagcagaggttgcagtgagccgagatcacaccactgccctccagcctgggcgacagcaacactctgtctcaaaaagaaaaaaaaaaagaatgctaatcaatcacatgaaagcataagaaaatatataatattcagcagtaaaggtgcatatacatgggaggctgaggccggagaattgcttgaacccaggaagtggaggtttcagtgagctgagatcgcaccactgcactccagcctgccaaactgcatctcaaaaaaaaaaaaaacaaaaacaaaaacttgaggcctggcctcatgctccccttccatccccacttccgtgggtccaagctgccttggctgaggagggggctgaggaggtgtgagcccctgccaggaaccccctgcccagaccatgtacttggcccacaggcccctgatgtctgcgtccagcgaggcctccagtggcgtcagcatgtttgtgtggaggaacgtggaaccttgctctgtggctgtgttctcctggtactctgtccccttcctgacccctccctgcagctatgtgaggtccagcaacctgccagtcactcagtggcctccaaccagagcaaagaacctgccaagtcagcagctgttgctcatgagtgtccaccaggtgggacagggagtgctgaccctgggtggccccctggagccacctgccctgaaagcccagggcccgcaaccccacacactttgggggtggtggaacctggtaaaagctcacctcccaccatggaggaggagccctgggcccctcaggggagtccctgctggacagtgagacagagaatgaccatgatgatgctttcctctccatcatgtctcctgacacccagttgcctctaccagccagatgatgtcaggcccagtccctcagtgccctgcgcaaggaacaggactcatcttctgagaaggatggatgcagccccaacaaatgggacaaggaccacatccggtggcccatgagtggcggtcatgatcttcagcaagcggcaccaggccctggcagggcgcaccagggtcaccccaaccaggacaaccggaccgtcagccagatgctgagcaagcggtggtacaccctggggcccaatgagacgcagaaataccacgacctggccttccaggtgaaggtggcccacttgcaacaaggaccgaaagaagtccagctcagaggccaagcccacaagccaggggctagcaggagtgtaacaagggctcgtgggagcggagaatatcagagacgggcactgccactgcccctggggtgtcctctgaactcctgtcagttgcagcccaaacactccagagctcggataccaaggagcagcttctgtggggcagaatggctgcacacagtcagggaacctggcttagcctggcccaagccttctcccacagtggggtacacagcctggacggcagggaaatagaccgtcaggcactacgggaactgacacaggtggtgtctggcactgcatcatactctggcccaaagccttctactcagtatggagctccaggccactttgcagcccctggtgagggaggtgaccagtgggcagccctgctgctgcccacctgagctgctcattcccagcacatggccagtgaggacatagcaagtgacgaggagcacacggtcatccatgaggaggagggggtgatgatgtcattgctgatgatggctttagcaccactgacaccgatctcaagttcaaggagtgggtgaccgactgagagtggggacaactctggggaggagccagagggcaacaagggctttggtgggaaggtatttgcacctgtcattccttcctcctttactcctgccgccccttgctggatcctgagcccccagggtcccccgatccacctgcagcttttggcaaagtctatggtcccaccttgtcctcctcctacacatactcggatgcttcctcctcaaccttggcacccacctccttcttactgggcccaggagccttcaatgcccaggagtctggtcaaggcagcagagcgggccccctacggcccctacccctggggatgggggcccagggacgccttccaaggtgacctgtttcctcccaatggatcctgccaccttctggtgcaagagacctgaaagtgtgggcgacctggagctaccaggctcctcagtcatcagggtccctcccaacactaaggctttcctaggcaggagctgggctgagccacccggggggcagagcctgaagagaaactgactgggctttcggggtcggggcagagggaaccccacggacatggatcccacactggaggaccccaccacgcccaaatgcaagatgagaagatgctccagctgcagtccaaagcccaacacccccaagtgtgccatgtgtgatggggacagcttcccctttgcctgtacaggtggagaagccaaggacaggctcagggaaccggagaccgagaaggcgctgtcctcttcactgcacgtgccctggaccagtgccggccctgatcatgcagctcttccaggcccactgcttcttcctgtccactaggccacagccgccctccaggcccactatgcacacatcttcccctccaaggtttgttctgcccctgccctgactcccagccctgtgggggtcctgaccgcacctcacctggctcagactcttgacgctgccctggctgccccaccactgcctctgcccgagagtcacgtgaggctgagagtaggggcaggggcagcagtggtgccagttggggggcggtccagtgggaggagcctcagcctcacgggctgctccgtgggactgatgactgcatgatcttctgggcacctcacggatcttcaactgcaggtgaaacggatgctggtggtgggtgcagggccgctgggagctgctgcatggttcccagaggctggactggggcaggtgccaactgaagctgctggggcagcatgggcaggatgttctgcacacaaaccttggagaagacgatgtgtgcatagcgggtccactgctgctgcccctgccctgactcccagccctgcctgaccccacctcaacctgctcaggctctggcgcaaccctggctgccctgccactgcctctgccccagagttggggccttgacagcctggttggaaggggacaccccagccctgcctaaacacctggggggtctccataactaccacaggcaggtgggcaaccccaaagatcccaggactcacagtaccccctgagaacatggacagtatgtgggggtagcaatggagggcaggatggttatcttctcccaggtaaagccatttaatcctttcagtttgggacggagtaaggcctgcctttttttttttttttttttttttttgagaccgagtcttgctctgtcgcccaggctggagtgcagtggtgcgatcttggctcactgcaaactcttcccaccgggttcacgccattctcctgcctcagccttccgggtagctaggattacaggtgcacgctaccacgtccggctaatttttgtatttttagtacagacggggcttcatcatcttggccaggctgatttcgatctcctgacatcgtgatctgcctgcctccccctcccaaagtgctgggattacaggcgtgagccaccacgcctggccaaggcctgctcctcttatctataccccctacccctgcagctgtgccgggggaaagctgggcagtttccctcctccgagcccctgtacataccatgaattgtgggaccttcagagcttttcacttttcggaaaatagctcctgctggggctacaagatggagtgtgaagagggccttgggccacagggaggcgcctgtggactaaggggagttcatgcaccccttctttccccagaggggctggactcaggtgagtatgggggtgggggctcctgcacttcgacacaggcagcggaagggttttctccccattccctctgcactcccaacttgagctatactttttaagaaagtgattcaccctgcctttgcccccttccccagaacagaacacgttgatcatgggcgatatttttcattgtgccaaaaagttgccatgaccgtcattaaacctgtttaacaccaaataataaggaaaataaaacaaaaagttcgggcatggtgcagaaactcactccaaataaattacctaccaaaatatataatggtggaaatattccaaaattccatattttgggatttatacacaaaagataaacaaattagaggccaagaggctgccggaagggaaaaacggggcctggaaaggccgttgtgaggaatgagcttggcctaaagaggccactggcaggcagtagctggacctgccgaagtggccgaaaggcaggagctttggacgggggaggccgcagtgaggcgagagctagctgggcgtggagagtccactgtgaggccaaggccaaggccaggcccgtgcaggcctttgagaggcaggaggccgggcctgcaaaggccgactggagatcaagttctgcgcctgaagaggctgccaaaagtcaaaagcggggcctgggaaggccgccgagagccatgaactgggctgggccgaaagaggccactgggaggcaggaagagctgggcctggagaggctgactcgaggaagttttgcacctggagaggccgccgagaggacggagctgggcccggggaggccgacttgctgctcttccaggcccacttccaggccgacttgaggacgacttgggcctgcagaggccgctgggaggccggagctgggcctggagaggccgacttcgggacgatttgggcctgcagaggccaccgggaggcccaagctgggcctagagaagcccaccaaccggaggccgtttggggcctgcagatgccatcggagggcaggagctgagcctggagaggccaccgtgaggcctgagctgggcctggggagcttggcttagggaagttgtgggcctaccagggcctctgggagctgggcaggagctgagtccaaagacgttgttgggacctggagtcgggccagagtccggcctggagacgcagccgggaggaagagctgggcccggagaggacgctgggaggctgcaagtgggtctgagaggccgacttgaggaggcccggcctctgcctcccgcatggcccagctgttcctcctggctgcatctcccgcctcccagcaaacaagctcttttggctcagctcccgccggcctttgtagaccccgaagtttctgcaaccaagctcttcagacccacatcccttctcccagtgactgaacagtcccagctccagctggagaagggtgtctgcagaccccgctgttgcctcccaggggagtctccaggcccagctctcgccccaccgcgacctcccaggcccaagtccctgcctacctcccagcagcccgcgtgcgaccctgctcctccctcacggtggcctgttgaggcaggggctcacactgacctctctcagcgtgggaggggccggtgtgaggcaaggggctcaggctgacctctgtccgcgtgggaggggccggtgtgaggcaaggggctcaggctgacctctgtccgcgtgggagggtgggcatcaacaggccaccgtgagagaggagctgggccgcacgtgggctgctgggaggcaggcagggacttggccccgggaggccgccgtgggggcaagagctgcgcctggagaggcccctggtaggcaagggcggggcctgcagaggctgttctccaaccagtgctgggcctgtacaggccaccaggaggcaggaggtgggccctcagagcttggctggagaaagttcggggcctagaaaggcggttgggagctgggcaggagttgagccaaaagagcttgcttacttgctgggaggcagggccaggagaggccgacttcaggacaacttgggcctgcagcggtcgccgggaggcccaagcttggcgtggaggagcccaccgaccggagaccatttggggcctggagatgccatcggagggcaggagctcatcctggagaggccaccgtgaggcctgacctgggcctggggagcttggcttgaggaagctgtgggccgaccaatgccgccaggagatgggtaggcactgagtccaaagaggttgttgagaggcaggagtcgggcctggagacgcaaccaggaagaagagctgggcccggagaggacgcccggagggtgcaagtggctctggagaggccgacttgaggaggttctgggcccggagaggccgccggaagggaaaaactgggcctggaaaggccgttgtgaggaacgagccccatgggcctgaagaggccactggcaggtgggagctgggcctgccgaagcggccgagaggcaggagctttggactcgggaggccgcaatgaggcgacagctagctgggcgtggagagtccgctgtgaggcagaggctgggcctgtgcaggccttcgggaggcaggaggctgggccttgtcgaggcctgcagaggccaccgaaagtcaaaagcggggcttgggaaggccgccgggaggcatgagctgggctgggccgaaagaggccactgggaggcaggaggagctgggcctggagaggctgccgaaaggcaggagcttcgactgaggatgccacagtgagacaccatctgggtctggagggtccactgtgaggcagaggctggcctgtagagtccgacagtagacagaagttgggcaaaaggctgatttgaggaagttttgggcttcaagagtcagccacgaggcaggcactaggcctggaaatggcccgacagtcatgagttgggcctaaatgggccactgtgagggaggagctatgcctgttgaggctgctggcaggcaggcagaaatttggcctggggcagctgccatgaggcaagagctgggcctggaaaaagcccctgggaggcaagagcagggcctgcagaggctgttctcaagtcaaagctgggcctgttcatgccactgggaagcagaaggtgggcctggagagtttgacttgaggaagttttgggcctacattggccgccatgagctggacaggaactgggccaaaaaaggctgttgtgaggcagcagttgtgcctgtagacccagccaagaggaagaggtgggcctggagaagcccccatgacgtagaggttgggcctgtagacgctgacaggaggcaggagctgggcctggaaaggtcaacttgaggagattttgggccttcataggccaccaggaggcagcagttgggactacagagtctgacttgagtaagttttgggcccggagatgacgtcctgggacaggagttgggcctggagaggccaccgtgaggcataagctgcatgtagagaggccctgggcctgtctaggctgctgggagacaggcaggaatctggccagggaaggttgccatgagacaaaagttgggcctggaaaggcccttgtgaagcatgagcttggcctaaagaggccactgggtggcaggagctgggtgtgtagaagctgctgaaaggttgggagcttggcttggggggtccacagtgaggcagatgctgggcgtgaagaatctgctgtgaggcagatgttgggactgtagaggccgacgggaggcagaggctgggcctggaggggccaccaagatgcaggagctgggcctggagaggctgcaaagaagcatgagctgggcctggtgaggtcgacttgagaaagttcagggcctggagagaaggctgggaggcaggagctgggtctaaagaggccattgtaacgatggagctgtgcctgtggaggctgttgtggggcagtaggctcatctgcggagactgccgtgacgtagggtatgggcctaaataggccattgtgagtcatgagcttggtctgtagaggctgattggagaaagttctgggcctggagaggctgccgggaggtaggagcataatgtagaatcagtgggcgtcttaagcttgttttcctgcaactggatggtcccacgtttcactgtcacccctctggaatccacgtatacgaaaattccaaatattagttgggcatagtggcaagcacctgtagtctcagccacgtgggaggttgagatgggaggatcgcttcagcctggaaggttgaggctgcagtcagctgtgatagcactactacactccagccttggacaacagatggagaccctgaataacatgttgctcagtcagtctctcttcctggattcagaggtctttcatggtagatccagctccagctctgtggccctgtggttggagaccgctgctcaagtgcattcgaaaggatccatcccatgccattcttcagagtcatctttactgctgcagtggtcaacttgtagcacccctaagctcgcaggacaggtgctt

SEQ ID NO: 11561 - RNA, 4575 nt, Homo sapiens
  source 1..4575: mol_type = other RNA
ctgaatagctgggactacaggtgcgtgccaccatgctcagtacacttttttcctggtgtctgtggcattctctgacctcattattattggtcactcttctcaagatcagaaatgagaatattttcttctaaatatactgtactaaagttggttgcaggatagtaaggattccgaaaccctgcaagtctcctgaagaagccaccgttatgcttgtatatgcagaaggaaagtgtgcaaatggccacaatgactatcagtgtcagtacaaccgcaagaggaatgatgctgtgacttggtcctttttctggcagcgcctctgcagtgtgaatatctgcctccattttacatataaagccttttttttcttgacacggggatagctgccataatccttcagggatcctcaaggcaacacaatgatggggcttgaagtagtctgtgtctggcttccgaatgccccagtttgactggtctgtgggagttccatcaaaccactttatggtttcattgttaccatcaaattgagcattcaaccaaaccatctggacagaagaaccaaaagcaaacagctcttctaggagaaatgcattttcagcctcatccttgattgttaaaagattagaaccttcctttttgcaaaattcatgagcagcctcaaaactcatactgtctaggactgtagaaaaactgtagcaattacttttaaattttatccagggaatagatgtttctgagcacaactctgggtgttcagattgtcttgtttcaggtggcacatgacaaatggcaccttgcagaaatgactcgcaggctgtgctatgccagcgtccgttgctgtcggcaaaaacgcagtcaccaaggagggaggactcctcatctttccaaaaagtgaaagaagatttggtgccatcagaccagtcaaaattaagaccattatctgtggtgaacagtccaatccagtgggcatatcctagccggttgaggacaacagtgaggaaggactggtgatactggtctgtgatgctgaccagttgtgctttgtgcatcaggcaggtttttattgctgcataccaagtcatatttgcattaattattttgtaagttctgtttccatattctaaggtattgggcattggatacatatcagatgtatttacaccgtgtccagaagtatcttgcattttttcacaaacaaacccatagccttcctttccacagtcttcaaaataccattttccagtgaaatgaaaattaggattacttgagagtaaggcacagagaggaatgtgtttctgaacttcagtggtattgtgacttggaatatttattatatcaaatggagaccagttagaatataccacaggctttccatttagccatgtttcataatcatcattttgtaaacctatccacacactggtggtctggccaaaaagattcatagtaatgaaagcttgctccacctcactttcaatggcgaccagggtccccccttcttcagcacagaaatgttgagcatgcgtccagttcttccaactgcttgggtctttggggatattcagcagaaggcacttatagttaaaatatagccatcctttgggacacgttccatgttgttttggtgtatctttctttttctctatgagccaaaccttttttcgcttacagatactaggcatagaaactgaacactcttcactaccccagagtcctgttatagaagaaataaagccacatctctggctctgattattcacagttctttctcttcctgtgtcccagttctggtatatcactggtgttccatctctccagcgaaattcatcattggctctttcttcttgaagtccaatccaccaacttgcaccatactttgatagcgcttttattttgctgtggatgaattcttgctcatgtgcagaatgaattgtgagaagatcactgtgcagccagctacagacaaactcaaagttcaaccattctgaggcaaaggtatgaaaaaggtattctgcatcctgataaaagagccagggtacatcgtactggtaccagaacggaatcttgggtttcacatctcttgggattttgcatatccattcacgtttggaaccacagtgtaagggcagcaatgttttgtttgccttataaacagcacagtttcttgcatcttctccaaaataagtgttgtctaaaaacgaagagacaacaggagttctatcagaccactcccatgagccggcattcagtgggtttcttttattaaatccaatccagaactgcctttcttctgtccaattaaattttgaatgtaagagctcattcacaaaattctcttcctcaatatgggcaaagcttgcaagatgagctccaaattcttcgcaaaatgcttcagcttctctccatgttcttttcatcagaactttttcactatgaaataccttgaagcaactggccagaccaggctctgactcccagtccaaatagcaggggtgaaagggccatctctcttcatactctgctttttcctgattttcaactggctgcttgcacaaggacattgccttaaagtgccgacagtgcttcacttcccagcgaccaagtggatgccttcctcgcatggcaacacagccaccactgtagcgcggctggtgtgtgttccagtgtgtgtactgcaccggctcgggtttctgccctactggcttccaagtgtattctcccgtatcattttggtcctgaagagctatccaaaaataactgtccttcatttttaccacactactgatcaaactggtaataaaagcctgttcaaacctgtttgtaatggttacaagtgcaggaggacagtaataaccgctggaagcttggtcaaagcttcgaaggactgtgtcaattttgtaacagaatccaccatgtctctcccatccctcttgacatcctgattcagcatcagagaggacatggcctgcttttttacaaatgtaaaaaagtctttcttcacaatttttgactttccagtgtccctcagactgctctgctgagacacacagctggcttctatttggaaaaatgtggggctcaagtgtgtgccaattagtaaagatgactgaagagtcattagaccattcaaaggaaactggaattttattgctgctcaaaccaatccatgtttctgatgcattttcatctccaaggagggttacaagaaactccacctctgctaatgaggttatgtctattaatgcactgttatcagcctgacaagaacgcagagcctcatgccaggtcttttcttctttctgaagtttgtagcaattacgattgtagggattccagccaggctcacagtgggtagcataatatttccacgcatctttttcaactatttcatgatcaatgtggtttagatattttttacatatatatggcaaggtggactcacaatcccgactcctccaggcacttggcataaatgaactaaatgttccacagtgatcttcaacaaatggctcaaaatttacctctgggctccaattcagatagttgagcggcgttccatcagaccactgccagccagcgtgttcatccagctgattgaggcccatccacacctccactgttttactgctcatgtgctcccttatgaaattttcttcagtttcatctgtaatacttaacagcgtacctccttgcatctggcatgaagaatgtgcctcactccaagagagagatgaaagcaggttgaactggtagcaaatgtgtgaattgaggtccttctcccaaatagtatcacaacctacttctgcagaggtgggatcagggcaaaatccccacttttcatctctttcataacggcttgtcgtggcacaccacagtaagtcatcttcccgaccttcacgggtacattcatgatgccactgatggttatactggaagggaaacatacacggcatcccgtgggtgttccctttgattgtatgcaaatctttgtgtagatattcacaaatgtctccaccacctgacccataagaaatccacttatgaatatacttccgtgaggccaccactgtgttgtcatgcgccacctggacagagtactgcagcgggcctgtgatcatcttcctgttacagcgccaccgtaaggaaacgagggtggagtcacattcatataagcttaatggctgctctggggcggagaaattcaggcccaggcaaccactgcctcctatgttaaagaggccatggtttgaaacccatttccacagcatgtgcttgtttgcttgcttgcagttctccagggtcagaaccgatttacctgcttgaatgcatttcttgagactctcactttggataacaaatattcctttatcctgccactccaggagccgctcgggggtaagcgccgccgccacaccctcggcgcagccccgcggcgcccccagcagcagcagcagcagcagcgacggcgacagcagcatcgctaaccactgggctctccgggagccccttgtcccgggagccccttatcccgggagcccagagccgcgtcccaagcacccggccccgccgcgcggaagc

SEQ ID NO: 11562 - RNA, 5859 nt, Homo sapiens
  source 1..5859: mol_type = other RNA
ctgaatagctgggactacaggtgcgtgccaccatgctcagtacacttttttcttgataaaattcaataaacagttatgtaatgagtaaatttttagatattgattatgaagctgttttctttataaggaactaataaaggaaaataaaatctgtaattttttatttacagacagtatcataatcattatttaccatctacactaactagactaatataaaaggagatcgttcccagaaaatagtttattaaatagaacacctaaactcatttacataataaagatatctagattactaatttatttagtacttctcaacaacatctgtctggttctaatgagactataattcagatctttagctcttctcctttaaatccaagttacattttatatcttccagttattaagagtgttacatattattttatatatttagtttttcagaaagtccatgagttttaacagtacaactgttaaagtttcaatatattactttaagcttatgtataagacattttaaaatatccaacttaatcatcatttagtaattgaaagtttaaggccacattttaactatatggttgtttataaaagtgtgctgctaatgaaggtctttgccatttaaaagaaggtatttttctttctcctttagcttgagatgttagacctaataaaaatgaatgtcaccttaaatatcagttgagagcccagaacctgtgacccttaagcacagaaattagtattttccaaatcctgctattaaaagtgaattcaaaagaaacaactaagaatcctctcagaagccctttccttttcctctcatatacaagattaatttttttttgcttctttctgtctttcttaatggtacgagtgcaggtaaatgtctgaatagataccagattagttttaaaattcccccaaattttagtagagatacattaatgcaaaaactattattcgcattgatttcagagttttcaatagggagtttcttttaatagttcttgtctttctgaaaaataaccaatgcataatttaccccttttaagaatggatcacagtttagggaaatgaataaatcaaaacccatctgatttggttaagattcaaaaccagtaatcacttcaagaataattaaaatagtgacccaattcacattctaatggcatctgtgctgtaaagggaaagacagatgagactcctgtttagtcttctttacttaccctggtgtctgtggcattctctgacctcattattattggtcactcttctcaagatcagaaatgagaatattttcttctaaatatactgtactaaagttggttgcaggatagtaaggattccgaaaccctgcaagtctcctgaagaagccaccgttatgcttgtatatgcagaaggaaagtgtgcaaatggccacaatgactatcagtgtcagtacaaccgcaagaggaatgatgctgtgacttggtcctttttctggcagcgcctctgcagtgtgaatatctgcctccattttacatataaagccttttttttcttgacacggggatagctgccataatccttcagggatcctcaaggcaacacaatgatggggcttgaagtagtctgtgtctggcttccgaatgccccagtttgactggtctgtgggagttccatcaaaccactttatggtttcatcatcaaattgagcattcaaccaaaccatctggacagaagaaccaaaagcaaacagctcttctaggagaaatgcattttcagcctcatccttgattgttaaaagattagaaccttcctttttgcaaaattcatgagcagcctcaaaactcatactgtctaggactgtagaaaaactgtagcaattacttttaaattttatccagggaatagatgtttctgagcacaactctgggtgttcagattgtcttgtttcaggtggcacatgacaaatggcaccttgcagaaatgactcgcaggctgtgctatgccagcgtccgttgctgtcggcaaaaacgcagtcaccaaggagggaggactcctcatctttccaaaaagtgaaagaagatttggtgccatcagaccagtcaaaattaagaccattatctgtggtgaacagtccaatccagtgggcatatcctagccggttgaggacaacagtgaggaaggactggtgatactggtctgtgatgctgaccagttgtgctttgtgcatcaggcaggtttttattgctgcataccaagtcatatttgcattaattattttgtaagttctgtttccatattctaaggtattgggcattggatacatatcagatgtatttacaccgtgtccagaagtatcttgcattttttcacaaacaaacccatagccttcctttccacagtcttcaaaataccattttccagtgaaatgaaaattaggattacttgagagtaaggcacagagaggaatgtgtttctgaacttcagtggtattgtgacttggaatatttattatatcaaatggagaccagttagaatataccacaggctttccatttagccatgtttcataatcatcattttgtaaacctatccacacactggtggtctggccaaaaagattcatagtaatgaaagcttgctccacctcactttcaatggcgaccagggtccccccttcttcagcacagaaatgttgagcatgcgtccagttcttccaactgcttgggtctttggggatattcagcagaaggcacttatagttaaaatatagccatcctttgggacacgttccatgttgttttggtgtatctttctttttctctatgagccaaaccttttttcgcttacagatactaggcatagaaactgaacactcttcactaccccagagtcctgttatagaagaaataaagccacatctctggctctgattattcacagttctttctcttcctgtgtcccagttctggtatatcactggtgttccatctctccagcgaaattcatcattggctctttcttcttgaagtccaatccaccaacttgcaccatactttgatagcgcttttattttgctgtggatgaattcttgctcatgtgcagaatgaattgtgagaagatcactgtgcagccagctacagacaaactcaaagttcaaccattctgaggcaaaggtatgaaaaaggtattctgcatcctgataaaagagccagggtacatcgtactggtaccagaacggaatcttgggtttcacatctcttgggattttgcatatccattcacgtttggaaccacagtgtaagggcagcaatgttttgtttgccttataaacagcacagtttcttgcatcttctccaaaataagtgttgtctaaaaacgaagagacaacaggagttctatcagaccactcccatgagccggcattcagtgggtttcttttattaaatccaatccagaactgcctttcttctgtccaattaaattttgaatgtaagagctcattcacaaaattctcttcctcaatatgggcaaagcttgcaagatgagctccaaattcttcgcaaaatgcttcagcttctctccatgttcttttcatcagaactttttcactatgaaataccttgaagcaactggccagaccaggctctgactcccagtccaaatagcaggggtgaaagggccatctctcttcatactctgctttttcctgattttcaactggctgcttgcacaaggacattgccttaaagtgccgacagtgcttcacttcccagcgaccaagtggatgccttcctcgcatggcaacacagccaccactgtagcgcggctggtgtgtgttccagtgtgtgtactgcaccggctcgggtttctgccctactggcttccaagtgtattctcccgtatcattttggtcctgaagagctatccaaaaataactgtccttcatttttaccacactactgatcaaactggtaataaaagcctgttcaaacctgtttgtaatggttacaagtgcaggaggacagtaataaccgctggaagcttggtcaaagcttcgaaggactgtgtcaattttgtaacagaatccaccatgtctctcccatccctcttgacatcctgattcagcatcagagaggacatggcctgcttttttacaaatgtaaaaaagtctttcttcacaatttttgactttccagtgtccctcagactgctctgctgagacacacagctggcttctatttggaaaaatgtggggctcaagtgtgtgccaattagtaaagatgactgaagagtcattagaccattcaaaggaaactggaattttattgctgctcaaaccaatccatgtttctgatgcattttcatctccaaggagggttacaagaaactccacctctgctaatgaggttatgtctattaatgcactgttatcagcctgacaagaacgcagagcctcatgccaggtcttttcttctttctgaagtttgtagcaattacgattgtagggattccagccaggctcacagtgggtagcataatatttccacgcatctttttcaactatttcatgatcaatgtggtttagatattttttacatatatatggcaaggtggactcacaatcccgactcctccaggcacttggcataaatgaactaaatgttccacagtgatcttcaacaaatggctcaaaatttacctctgggctccaattcagatagttgagcggcgttccatcagaccactgccagccagcgtgttcatccagctgattgaggcccatccacacctccactgttttactgctcatgtgctcccttatgaaattttcttcagtttcatctgtaatacttaacagcgtacctccttgcatctggcatgaagaatgtgcctcactccaagagagagatgaaagcaggttgaactggtagcaaatgtgtgaattgaggtccttctcccaaatagtatcacaacctacttctgcagaggtgggatcagggcaaaatccccacttttcatctctttcataacggcttgtcgtggcacaccacagtaagtcatcttcccgaccttcacgggtacattcatgatgccactgatggttatactggaagggaaacatacacggcatcccgtgggtgttccctttgattgtatgcaaatctttgtgtagatattcacaaatgtctccaccacctgacccataagaaatccacttatgaatatacttccgtgaggccaccactgtgttgtcatgcgccacctggacagagtactgcagcgggcctgtgatcatcttcctgttacagcgccaccgtaaggaaacgagggtggagtcacattcatataagcttaatggctgctctggggcggagaaattcaggcccaggcaaccactgcctcctatgttaaagaggccatggtttgaaacccatttccacagcatgtgcttgtttgcttgcttgcagttctccagggtcagaaccgatttacctgcttgaatgcatttcttgagactctcactttggataacaaatattcctttatcctgccactccaggagccgctcgggggtaagcgccgccgccacaccctcggcgcagccccgcggcgcccccagcagcagcagcagcagcagcgacggcgacagcagcatcgctaaccactgggctctccgggagccccttgtcccgggagccccttatcccgggagcccagagccgcgtcccaagcacccggccccgccgcgcggaagcggatccgtagcctcctccgcgccccaccccctccgggggccttgccagcccagagccctggagacccactccgccaccgctgtctccacagtgaaccgacactcggggctct

SEQ ID NO: 11563 - RNA, 5865 nt, Homo sapiens
  source 1..5865: mol_type = other RNA
ctgaatagctgggactacaggtgcgtgccaccatgctcagtacacttttttcttgataaaattcaataaacagttatgtaatgagtaaatttttagatattgattatgaagctgttttctttataaggaactaataaaggaaaataaaatctgtaattttttatttacagacagtatcataatcattatttaccatctacactaactagactaatataaaaggagatcgttcccagaaaatagtttattaaatagaacacctaaactcatttacataataaagatatctagattactaatttatttagtacttctcaacaacatctgtctggttctaatgagactataattcagatctttagctcttctcctttaaatccaagttacattttatatcttccagttattaagagtgttacatattattttatatatttagtttttcagaaagtccatgagttttaacagtacaactgttaaagtttcaatatattactttaagcttatgtataagacattttaaaatatccaacttaatcatcatttagtaattgaaagtttaaggccacattttaactatatggttgtttataaaagtgtgctgctaatgaaggtctttgccatttaaaagaaggtatttttctttctcctttagcttgagatgttagacctaataaaaatgaatgtcaccttaaatatcagttgagagcccagaacctgtgacccttaagcacagaaattagtattttccaaatcctgctattaaaagtgaattcaaaagaaacaactaagaatcctctcagaagccctttccttttcctctcatatacaagattaatttttttttgcttctttctgtctttcttaatggtacgagtgcaggtaaatgtctgaatagataccagattagttttaaaattcccccaaattttagtagagatacattaatgcaaaaactattattcgcattgatttcagagttttcaatagggagtttcttttaatagttcttgtctttctgaaaaataaccaatgcataatttaccccttttaagaatggatcacagtttagggaaatgaataaatcaaaacccatctgatttggttaagattcaaaaccagtaatcacttcaagaataattaaaatagtgacccaattcacattctaatggcatctgtgctgtaaagggaaagacagatgagactcctgtttagtcttctttacttaccctggtgtctgtggcattctctgacctcattattattggtcactcttctcaagatcagaaatgagaatattttcttctaaatatactgtactaaagttggttgcaggatagtaaggattccgaaaccctgcaagtctcctgaagaagccaccgttatgcttgtatatgcagaaggaaagtgtgcaaatggccacaatgactatcagtgtcagtacaaccgcaagaggaatgatgctgtgacttggtcctttttctggcagcgcctctgcagtgtgaatatctgcctccattttacatataaagccttttttttcttgacacggggatagctgccataatccttcagggatcctcaaggcaacacaatgatggggcttgaagtagtctgtgtctggcttccgaatgccccagtttgactggtctgtgggagttccatcaaaccactttatggtttcattgttaccatcaaattgagcattcaaccaaaccatctggacagaagaaccaaaagcaaacagctcttctaggagaaatgcattttcagcctcatccttgattgttaaaagattagaaccttcctttttgcaaaattcatgagcagcctcaaaactcatactgtctaggactgtagaaaaactgtagcaattacttttaaattttatccagggaatagatgtttctgagcacaactctgggtgttcagattgtcttgtttcaggtggcacatgacaaatggcaccttgcagaaatgactcgcaggctgtgctatgccagcgtccgttgctgtcggcaaaaacgcagtcaccaaggagggaggactcctcatctttccaaaaagtgaaagaagatttggtgccatcagaccagtcaaaattaagaccattatctgtggtgaacagtccaatccagtgggcatatcctagccggttgaggacaacagtgaggaaggactggtgatactggtctgtgatgctgaccagttgtgctttgtgcatcaggcaggtttttattgctgcataccaagtcatatttgcattaattattttgtaagttctgtttccatattctaaggtattgggcattggatacatatcagatgtatttacaccgtgtccagaagtatcttgcattttttcacaaacaaacccatagccttcctttccacagtcttcaaaataccattttccagtgaaatgaaaattaggattacttgagagtaaggcacagagaggaatgtgtttctgaacttcagtggtattgtgacttggaatatttattatatcaaatggagaccagttagaatataccacaggctttccatttagccatgtttcataatcatcattttgtaaacctatccacacactggtggtctggccaaaaagattcatagtaatgaaagcttgctccacctcactttcaatggcgaccagggtccccccttcttcagcacagaaatgttgagcatgcgtccagttcttccaactgcttgggtctttggggatattcagcagaaggcacttatagttaaaatatagccatcctttgggacacgttccatgttgttttggtgtatctttctttttctctatgagccaaaccttttttcgcttacagatactaggcatagaaactgaacactcttcactaccccagagtcctgttatagaagaaataaagccacatctctggctctgattattcacagttctttctcttcctgtgtcccagttctggtatatcactggtgttccatctctccagcgaaattcatcattggctctttcttcttgaagtccaatccaccaacttgcaccatactttgatagcgcttttattttgctgtggatgaattcttgctcatgtgcagaatgaattgtgagaagatcactgtgcagccagctacagacaaactcaaagttcaaccattctgaggcaaaggtatgaaaaaggtattctgcatcctgataaaagagccagggtacatcgtactggtaccagaacggaatcttgggtttcacatctcttgggattttgcatatccattcacgtttggaaccacagtgtaagggcagcaatgttttgtttgccttataaacagcacagtttcttgcatcttctccaaaataagtgttgtctaaaaacgaagagacaacaggagttctatcagaccactcccatgagccggcattcagtgggtttcttttattaaatccaatccagaactgcctttcttctgtccaattaaattttgaatgtaagagctcattcacaaaattctcttcctcaatatgggcaaagcttgcaagatgagctccaaattcttcgcaaaatgcttcagcttctctccatgttcttttcatcagaactttttcactatgaaataccttgaagcaactggccagaccaggctctgactcccagtccaaatagcaggggtgaaagggccatctctcttcatactctgctttttcctgattttcaactggctgcttgcacaaggacattgccttaaagtgccgacagtgcttcacttcccagcgaccaagtggatgccttcctcgcatggcaacacagccaccactgtagcgcggctggtgtgtgttccagtgtgtgtactgcaccggctcgggtttctgccctactggcttccaagtgtattctcccgtatcattttggtcctgaagagctatccaaaaataactgtccttcatttttaccacactactgatcaaactggtaataaaagcctgttcaaacctgtttgtaatggttacaagtgcaggaggacagtaataaccgctggaagcttggtcaaagcttcgaaggactgtgtcaattttgtaacagaatccaccatgtctctcccatccctcttgacatcctgattcagcatcagagaggacatggcctgcttttttacaaatgtaaaaaagtctttcttcacaatttttgactttccagtgtccctcagactgctctgctgagacacacagctggcttctatttggaaaaatgtggggctcaagtgtgtgccaattagtaaagatgactgaagagtcattagaccattcaaaggaaactggaattttattgctgctcaaaccaatccatgtttctgatgcattttcatctccaaggagggttacaagaaactccacctctgctaatgaggttatgtctattaatgcactgttatcagcctgacaagaacgcagagcctcatgccaggtcttttcttctttctgaagtttgtagcaattacgattgtagggattccagccaggctcacagtgggtagcataatatttccacgcatctttttcaactatttcatgatcaatgtggtttagatattttttacatatatatggcaaggtggactcacaatcccgactcctccaggcacttggcataaatgaactaaatgttccacagtgatcttcaacaaatggctcaaaatttacctctgggctccaattcagatagttgagcggcgttccatcagaccactgccagccagcgtgttcatccagctgattgaggcccatccacacctccactgttttactgctcatgtgctcccttatgaaattttcttcagtttcatctgtaatacttaacagcgtacctccttgcatctggcatgaagaatgtgcctcactccaagagagagatgaaagcaggttgaactggtagcaaatgtgtgaattgaggtccttctcccaaatagtatcacaacctacttctgcagaggtgggatcagggcaaaatccccacttttcatctctttcataacggcttgtcgtggcacaccacagtaagtcatcttcccgaccttcacgggtacattcatgatgccactgatggttatactggaagggaaacatacacggcatcccgtgggtgttccctttgattgtatgcaaatctttgtgtagatattcacaaatgtctccaccacctgacccataagaaatccacttatgaatatacttccgtgaggccaccactgtgttgtcatgcgccacctggacagagtactgcagcgggcctgtgatcatcttcctgttacagcgccaccgtaaggaaacgagggtggagtcacattcatataagcttaatggctgctctggggcggagaaattcaggcccaggcaaccactgcctcctatgttaaagaggccatggtttgaaacccatttccacagcatgtgcttgtttgcttgcttgcagttctccagggtcagaaccgatttacctgcttgaatgcatttcttgagactctcactttggataacaaatattcctttatcctgccactccaggagccgctcgggggtaagcgccgccgccacaccctcggcgcagccccgcggcgcccccagcagcagcagcagcagcagcgacggcgacagcagcatcgctaaccactgggctctccgggagccccttgtcccgggagccccttatcccgggagcccagagccgcgtcccaagcacccggccccgccgcgcggaagcggatccgtagcctcctccgcgccccaccccctccgggggccttgccagcccagagccctggagacccactccgccaccgctgtctccacagtgaaccgacactcggggctct

SEQ ID NO: 11564 - RNA, 2626 nt, Homo sapiens
  source 1..2626: mol_type = other RNA
ctgaatagctgggactacaggtgcgtgccgccacatccagctaatgtttttattttttgtagagacagggtcttgctctgttgtccaggctggtctcgaattcctgtcctcaagtgatcctcttaacttgtcctcccacagtgctgagattacaggcctgagcccaaatatccatttttaatcagtacttttgtttaagactctattgttatattggaggaaaacaaaaaacaaaaaacttttgtaacatttcatatatgacaaatcccaagaagtaaaaaaaaggactttccaggtcccagggcttcaggaagtgggagtgggctcatggggtgaggacattgtacccagcactaagcaaagtagagtcttaagcctgtttcttgcctgggggctatttatgcttcaacacggtacctgaaatattgggtattccaatatgcaagaggcagaactgaaaattccacaaatccgttctgacatacggataaacttttattgacataccaaagagaaaccaatattcactgaaggctgccgaatccgtatttctaagagtaaaggtgtttaattgactctccacacttaaagcactttgtatgaaatatagctacaaatatacataaagaattcagatcacaaaactctctaggacattggctgggcgcggtggcccaagcctgtaatcccagcactttgggaggctgaggcaggcggatcacaaggtcaggagatcaagaccatcctggctaacacggtcaaaccccgtctctactaaaaatacaaaaaattagccggatgtggtggcgggtgcctgtagtcccagctactcgggaggctgaggcaggagaatggcgtgaacctgggaggcagagcttgcagtgagccgagaccgcgccactgcactccagcctgggcaacagagcaagattctgtctcaaaaaaaaaaaaaacctctccaggaaatcaatagtcatcatataatactggaactacagttaaaaaaaaaaaaaaagcaatcttctaggattcctaactgtagtttaaagtacagatcatttgtaccaactttctatagcaagttgtaataggcaactgtaagcaaacagtatcaatctgtataacttgtaaaaattcatctgaagttgtttggagctgtacgacaatggatgttattcttccagttctcccagcagctctacaaaatcagtgatataccatttggcgttatccttgacttgttgcctgatcacatttcctccaaatccaatgaaagcatcagcaggaggacaggcttccatatctgtggcaccatctccaatcatgattattttcttaaaatgaaatttttcctttaaaagtttaatcacttttccttttccaccagattcagctgttggctgcgtctcatcaaaacctgcatattcaccgttaaagtagaatttcagcctattggcaaatacattggttgctgggatattgagctttgaagcaacatgctctacaatactcctaaagccaccagatattaggaaaacctgaacatttcgctcctgtaggcgacttaccagctccatttctgacaccgcgtcctcaacgccacagattttggctagctcatcgattccttcttctctgatgaccgtgctgtcaacatcaaaacacacagcatctgctgagtagaaaagcttcctcagctctgagtgggagaccatcgctggaagaattttcctcgtttctccagtgctagatttctaggagacgacactcttctgttccttccctagataaaaacgcagcacaaagttctgtctacagatttcctcaagaaagacctgtggattctgcaagagcaagagcccagatactcaggaggctgaggcaggagaatcccttgaaccctgtaggcggaggttgaagtgagccgagatcacaccactgcactccagcctgggcgacagaacgagactctgtcctgtgtcctgggcctccggggctcctgcggctgcaaccttccggctgcagggggccagcgccggctccgacgctcgggcgagcagttcccagggaggtgagctgtgcagacccagggcctccaccgaacgctctcttgagatctgctgataagcggggtggcttctgatgagttctgcaagtgcttctgtaaacttaaaagggagtccgctcaaaggcaggaatgactctacaagggtgaattttcaaatctgccataggggcctcgggcctcagcagcatccagagccctacggacgggcaggttcttacgtctcaactcccatcgcaccagtcctgcagctttctaaaggtatccagcactttctaccttgcattctatcttcatcttcgctaggcctcacagcaccgcatgattccgggggagggtgcttatcagactcgcgtgtggccccacggcacctagggcaccgtcgagcacacggtccgggaagctccaatgaaacggaacaaaccgcgagatcaggggaggtaggaggcccaccctacgccctgcccccgcggagcacaagccccgcctgcgtcccgagctcccgggtccgcaaagctgggccccaaagagctccaacgccggaaccaaggagcacggaat

SEQ ID NO: 11565 - RNA, 2578 nt, Homo sapiens
  source 1..2578: mol_type = other RNA
ctgaatagctgggactacaggtgcgtgccgccacatccagctaatgtttttattttttgtagagacagggtcttgctctgttgtccaggctggtctcgaattcctgtcctcaagtgatcctcttaacttgtcctcccacagtgctgagattacaggcctgagcccaaatatccatttttaatcagtacttttgtttaagactctattgttatattggaggaaaacaaaaaacaaaaaacttttgtaacatttcatatatgacaaatcccaagaagtaaaaaaaaggactttccaggtcccagggcttcaggaagtgggagtgggctcatggggtgaggacattgtacccagcactaagcaaagtagagtcttaagcctgtttcttgcctgggggctatttatgcttcaacacggtacctgaaatattgggtattccaatatgcaagaggcagaactgaaaattccacaaatccgttctgacatacggataaacttttattgacataccaaagagaaaccaatattcactgaaggctgccgaatccgtatttctaagagtaaaggtgtttaattgactctccacacttaaagcactttgtatgaaatatagctacaaatatacataaagaattcagatcacaaaactctctaggacattggctgggcgcggtggcccaagcctgtaatcccagcactttgggaggctgaggcaggcggatcacaaggtcaggagatcaagaccatcctggctaacacggtcaaaccccgtctctactaaaaatacaaaaaattagccggatgtggtggcgggtgcctgtagtcccagctactcgggaggctgaggcaggagaatggcgtgaacctgggaggcagagcttgcagtgagccgagaccgcgccactgcactccagcctgggcaacagagcaagattctgtctcaaaaaaaaaaaaaacctctccaggaaatcaatagtcatcatataatactggaactacagttaaaaaaaaaaaaaaagcaatcttctaggattcctaactgtagtttaaagtacagatcatttgtaccaactttctatagcaagttgtaataggcaactgtaagcaaacagtatcaatctgtataacttgtaaaaattcatctgaagttgtttggagctgtacgacaatggatgttattcttccagttctcccagcagctctacaaaatcagtgatataccatttggcgttatccttgacttgttgcctgatcacatttcctccaaatccaatgaaagcatcagcaggaggacaggcttccatatctgtggcaccatctccaatcatgattattttcttaaaatgaaatttttcctttaaaagtttaatcacttttccttttccaccagattcagctgttggctgcgtctcatcaaaacctgcatattcaccgttaaagtagaatttcagcctattggcaaatacattggttgctgggatattgagctttgaagcaacatgctctacaatactcctaaagccaccagatattaggaaaacctgaacatttcgctcctgtaggcgacttaccagctccatttctgacaccgcgtcctcaacgccacagattttggctagctcatcgattccttcttctctgatgaccgtgctgtcaacatcaaaacacacagcatctgctgagtagaaaagcttcctcagctctgagtgggagaccatcgctggaagaattttcctcgtttctccagtgctagatttctaggagacgacactcttctgttccttccctagataaaaacgcagcacaaagttctgtctacagatttcctcaagaaagacctgtggattctgcaagagcaagagcccagatactcaggaggctgaggcaggagaatcccttgaaccctgtaggcggaggttgaagtgagccgagatcacaccactgcactccagcctgggcgacagaacgagactctgtcctgtgtcctgggcctccggggctcctgcggctgcaaccttccggctgcagggggccagcgccggctccgacgctcgggcgagcagttcccagggaggtgagctgtgcagacccagggcctccaccgaacgctctcttgagatctgcttaaaagggagtccgctcaaaggcaggaatgactctacaagggtgaattttcaaatctgccataggggcctcgggcctcagcagcatccagagccctacggacgggcaggttcttacgtctcaactcccatcgcaccagtcctgcagctttctaaaggtatccagcactttctaccttgcattctatcttcatcttcgctaggcctcacagcaccgcatgattccgggggagggtgcttatcagactcgcgtgtggccccacggcacctagggcaccgtcgagcacacggtccgggaagctccaatgaaacggaacaaaccgcgagatcaggggaggtaggaggcccaccctacgccctgcccccgcggagcacaagccccgcctgcgtcccgagctcccgggtccgcaaagctgggccccaaagagctccaacgccggaaccaaggagcacggaat

SEQ ID NO: 11566 - RNA, 2512 nt, Homo sapiens
  source 1..2512: mol_type = other RNA
ctgaatagctgggactacaggtgcgtgccgccacatccagctaatgtttttattttttgtagagacagggtcttgctctgttgtccaggctggtctcgaattcctgtcctcaagtgatcctcttaacttgtcctcccacagtgctgagattacaggcctgagcccaaatatccatttttaatcagtacttttgtttaagactctattgttatattggaggaaaacaaaaaacaaaaaacttttgtaacatttcatatatgacaaatcccaagaagtaaaaaaaaggactttccaggtcccagggcttcaggaagtgggagtgggctcatggggtgaggacattgtacccagcactaagcaaagtagagtcttaagcctgtttcttgcctgggggctatttatgcttcaacacggtacctgaaatattgggtattccaatatgcaagaggcagaactgaaaattccacaaatccgttctgacatacggataaacttttattgacataccaaagagaaaccaatattcactgaaggctgccgaatccgtatttctaagagtaaaggtgtttaattgactctccacacttaaagcactttgtatgaaatatagctacaaatatacataaagaattcagatcacaaaactctctaggacattggctgggcgcggtggcccaagcctgtaatcccagcactttgggaggctgaggcaggcggatcacaaggtcaggagatcaagaccatcctggctaacacggtcaaaccccgtctctactaaaaatacaaaaaattagccggatgtggtggcgggtgcctgtagtcccagctactcgggaggctgaggcaggagaatggcgtgaacctgggaggcagagcttgcagtgagccgagaccgcgccactgcactccagcctgggcaacagagcaagattctgtctcaaaaaaaaaaaaaacctctccaggaaatcaatagtcatcatataatactggaactacagttaaaaaaaaaaaaaaagcaatcttctaggattcctaactgtagtttaaagtacagatcatttgtaccaactttctatagcaagttgtaataggcaactgtaagcaaacagtatcaatctgtataacttgtaaaaattcatctgaagttgtttggagctgtacgacaatggatgttattcttccagttctcccagcagctctacaaaatcagtgatataccatttggcgttatccttgacttgttgcctgatcacatttcctccaaatccaatgaaagcatcagcaggaggacaggcttccatatctgtggcaccatctccaatcatgattattttcttaaaatgaaatttttcctttaaaagtttaatcacttttccttttccaccagattcagctgttggctgcgtctcatcaaaacctgcatattcaccgttaaagtagaatttcagcctattggcaaatacattggttgctgggatattgagctttgaagcaacatgctctacaatactcctaaagccaccagatattaggaaaacctgaacatttcgctcctgtaggcgacttaccagctccatttctgacaccgcgtcctcaacgccacagattttggctagctcatcgattccttcttctctgatgaccgtgctgtcaacatcaaaacacacagcatctgctgagtagaaaagcttcctcagctctgagtgggagaccatcgctggaagaattttcctcgtttctccagtgctagatttctaggagacgacactcttctgttccttccctagataaaaacgcagcacaaagttctgtctacagatttcctcaagaaagacctgtggattctgcaagagcaagagccctgtgtcctgggcctccggggctcctgcggctgcaaccttccggctgcagggggccagcgccggctccgacgctcgggcgagcagttcccagggaggtgagctgtgcagacccagggcctccaccgaacgctctcttgagatctgctgataagcggggtggcttctgatgagttctgcaagtgcttctgtaaacttaaaagggagtccgctcaaaggcaggaatgactctacaagggtgaattttcaaatctgccataggggcctcgggcctcagcagcatccagagccctacggacgggcaggttcttacgtctcaactcccatcgcaccagtcctgcagctttctaaaggtatccagcactttctaccttgcattctatcttcatcttcgctaggcctcacagcaccgcatgattccgggggagggtgcttatcagactcgcgtgtggccccacggcacctagggcaccgtcgagcacacggtccgggaagctccaatgaaacggaacaaaccgcgagatcaggggaggtaggaggcccaccctacgccctgcccccgcggagcacaagccccgcctgcgtcccgagctcccgggtccgcaaagctgggccccaaagagctccaacgccggaaccaaggagcacggaat

SEQ ID NO: 11567 - RNA, 2975 nt, Homo sapiens
  source 1..2975: mol_type = other RNA
ctgaatagctgggactacaggtgcgtgccgccacatccagctaatgtttttattttttgtagagacagggtcttgctctgttgtccaggctggtctcgaattcctgtcctcaagtgatcctcttaacttgtcctcccacagtgctgagattacaggcctgagcccaaatatccatttttaatcagtacttttgtttaagactctattgttatattggaggaaaacaaaaaacaaaaaacttttgtaacatttcatatatgacaaatcccaagaagtaaaaaaaaggactttccaggtcccagggcttcaggaagtgggagtgggctcatggggtgaggacattgtacccagcactaagcaaagtagagtcttaagcctgtttcttgcctgggggctatttatgcttcaacacggtacctgaaatattgggtattccaatatgcaagaggcagaactgaaaattccacaaatccgttctgacatacggataaacttttattgacataccaaagagaaaccaatattcactgaaggctgccgaatccgtatttctaagagtaaaggtgtttaattgactctccacacttaaagcactttgtatgaaatatagctacaaatatacataaagaattcagatcacaaaactctctaggacattggctgggcgcggtggcccaagcctgtaatcccagcactttgggaggctgaggcaggcggatcacaaggtcaggagatcaagaccatcctggctaacacggtcaaaccccgtctctactaaaaatacaaaaaattagccggatgtggtggcgggtgcctgtagtcccagctactcgggaggctgaggcaggagaatggcgtgaacctgggaggcagagcttgcagtgagccgagaccgcgccactgcactccagcctgggcaacagagcaagattctgtctcaaaaaaaaaaaaaacctctccaggaaatcaatagtcatcatataatactggaactacagttaaaaaaaaaaaaaaagcaatcttctaggattcctaactgtagtttaaagtacagatcatttgtaccaactttctatagcaagttgtaataggcaactgtaagcaaacagtatcaatctgtataacttgtaaaaattcatctgaagttgtttggagctgtacgacaatggatgttattcttccagttctcccagcagctctacaaaatcagtgatataccatttggcgttatccttgacttgttgcctgatcacatttcctccaaatccaatgaaagcatcagcaggaggacaggcttccatatctgtggcaccatctccaatcatgattattttcttaaaatgaaatttttcctttaaaagtttaatcacttttccttttccaccagattcagctgttggctgcgtctcatcaaaacctgcatattcaccgttaaagtagaatttcagcctattggcaaatacattggttgctgggatattgagctttgaagcaacatgctctacaatactcctaaagccaccagatattaggaaaacctgaacatttcgctcctgtaggcgacttaccagctcccttatgccgggggtcaggtgtgggggttgctctgctatgagtctctgcacctgctccctggagggctggatgagggctaagcgctctgtgagagcagctttgaaaggcactgccccgcccatggctcgccgtgtcatttctgacaccgcgtcctcaacgccacagattttggctagctcatcgattccttcttctctgatgaccgtgctgtcaacatcaaaacacacagcatctgctgagtagaaaagcttcctcagctctgagtgggagaccatcgctggaagaattttcctcgtttctccagtgctagatttctaggagacgacactcttctgttccttccctagataaaaacgcagcacaaagttctgtctacagatttcctcaagaaagacctgtggattctgcaagagcaagagcccagatactcaggaggctgaggcaggagaatcccttgaaccctgtaggcggaggttgaagtgagccgagatcacaccactgcactccagcctgggcgacagaacgagactctgtcctgtgtcctgggcctccggggctcctgcggctgcaaccttccggctgcagggggccagcgccggctccgacgctcgggcgagcagttcccagggaggtgagctgtgcagacccagggcctccaccgaacgctctcttgagatctgctgtaatctcagcaatctgggaggccaaagcagaaggattgcttgaggccaggagttcaagaccagcacaggcaacaaactgaagcactgtctctacaaaacatcaaaaaattatccaggtgtggtgacgagtgcttgtggtcccagctacacaggaggctgaggcaggaggaaagcttgagcccaggaggttgaggctgcagtgagacatgttcgtgccactgcactccagcttcggcaacagagtgggacccttaaaagggagtccgctcaaaggcaggaatgactctacaagggtgaattttcaaatctgccataggggcctcgggcctcagcagcatccagagccctacggacgggcaggttcttacgtctcaactcccatcgcaccagtcctgcagctttctaaaggtatccagcactttctaccttgcattctatcttcatcttcgctaggcctcacagcaccgcatgattccgggggagggtgcttatcagactcgcgtgtggccccacggcacctagggcaccgtcgagcacacggtccgggaagctccaatgaaacggaacaaaccgcgagatcaggggaggtaggaggcccaccctacgccctgcccccgcggagcacaagccccgcctgcgtcccgagctcccgggtccgcaaagctgggccccaaagagctccaacgccggaaccaaggagcacggaatgccgggaac

SEQ ID NO: 11568 - RNA, 1797 nt, Homo sapiens
  source 1..1797: mol_type = other RNA
ctgaatagctgggactacaggtgcgtgctaccacacccagctaattttttatgtagagacggggtttcaccgtgttagccaggatggtctcgatctcctgacctcgtgatccgcctgcctcggccttccaaagtgctgggattacaggcgtgagccaccgtgcccggcctcaactttttatttattagcttgttggtcttcaacctctgtaagcctcagtttcctcacttatcaatcatctactgctgtatagagacaggtccatctcctagcatgcagggtgaggctaatgtgacatttgaaaactccagagtgctgctgacagtggttggaggtgaaggaggaggaaataaaagcaatgtgagaatagctttaaagaaaggaagggcaaaaagttgaaaagaaagaggcagtgtggagagatggagccaacagcagcatgggagtccctggctagggtcagggcttagatgacgacattgttggttgggttcacttgccctctgaactgcacagggaatcgagctggtcattagacatggcctggagccagtcactggaaaaggaaatcaatacccagactgattctcagaacagccaccatttgtatgattttaatccatagaatcattctgaaagcttcttaatcttcaccttttttctggacaggagacaggtggctgagcctagccctggactggatcatatcttcacacttccttaagccacagaaaacttgaaccaggtggtgtggtcatactcctcaccaggcctcagcagcacaggagggaagcggggctgattgactgcatcaggccagttctgagtctccaggcagaaaccggagtgcttgggatagacagctccattcttgccctttaatgtgccatccaggaagttgcccgtgtaaaactggaccccgggctgggtggtgtatacttctagtacccgcccgcttgcagcatgatgcacccttgcacaaaaatgcttttctttagatcccttcagacagaaattgtggtcaaaaccattgagatggaagtcctgcaggtgttttccaagctccactggctttctcaggtcgaatgcagtgccttgcactggggcaacttctcctgtaggaatcagggtttcatccacaggcaaataagtatccgcttctatggtgacttcatggtcatttatatttggggaagcctggcctgccaggttgaagtaagaatggttggtcaggttgactggtgtggcctgactggcttgtgctctgtagttgactatgagctctccgccatccagggtgtatgtcacccagacttttaactctccggggtagccttcttcaccatctggactgatgcgcgagaactggacgccatttgacagcacccgaggggtccagagcactttatcaaaccctctgactcctccatgcagactgttgggttccttgttaatggccaggtgatactccttcccatccaccttgaaggttcctttggcgattcggttggccaccctcccaataactgctccaaagtatggctgcttttggaggtatccttccaactcggcgaagccaagcaccacgtccgaggctctcccctgcctgtctttgacctctagggctgtgatcgtgcagccccaggagatgatgtccactctcaagaggtctgactgcagctggaacttctccactgtccctcctcccgagggcagctctccaaacacggccctggtcaccgaagccatagggaaagtttggcgtgtgcagccactgcccgctcttcaaactccagc

SEQ ID NO: 11569 - RNA, 737 nt, Homo sapiens
  source 1..737: mol_type = other RNA
ctgaatagctgggactacaggtgcgtgtcaccacacccagataattttttgtatttttagtagcgatagggtttcaccgtgttagccaggagggtctcgatctcctgacctcatgatccacccacctcgggctcccaaagtgctggaattacaggcatgagccactgcacccagcctttttttaattattatttgaagaatttaagattggaattaattgctccttgaatgtttggtagactcatctgtaataccatttgagcctagaatattctggtttttttgagacggagtcttgccctattgcccaggccggagtgcagtgggattacacgcgtgagccaccatgcctggccagaatattctttattgtaaaatttaaagctgtaatttcaatgtcttgaagagttatagatctaattagattttccatttctcctggagtcaatttggtacaaacagtcaataaagactacaagaccagtttaagtagatttttcagtttgagtgtcctggatcatgtacacaatcatgaatgtgaagtctgtctgcatgaagaatcatctgtggttataaattcttaggaggttttttccttcttccctctggaacaacggttgaagcaggcaagtttcctaatcaccttctctcctttagtagggcagcatttttcttttttataaatagttggcctggccaggcatggtggctcacgcctataatcctagcactttggg

SEQ ID NO: 11570 - RNA, 5118 nt, Homo sapiens
  source 1..5118: mol_type = other RNA
ctgaatagctgggactacaggtgcttgacaccacaactggctaatttttttttttaatttctgtagagatggggtctcgccatgttgcccagggctggtctcgaactcccgggctcaagcaatcctcccacctcagcctcccaaagcactgggatcacagacatgaaccatctccaggattcccctccttgccgagaaactactgccatctgggacatttccttcacacatctggctctgatggggaagctgtgatttcggcccccaccccctgtccctgcccagccctgcctctccaagtggcctcaggtttgttccagcccttgattggagcaggtgggctaggtggccccaagctcagcccacccaccttgaattcctgcttcttcctttctttcctttccactccatcttatttcttttttgagctacatccccacacgcatgcaactgaccttctttggggtggggagggggtgctaggggccgaataaaggaataaaagtgcgcagacttgggcatcttaaaagagatgccatcatcaagttggtcagggtaccaggtgccctgatcactgtccctgcacccctgttccctgcctcagcaccctccatgaggactcatcagggaagcccccccaatcacttctcacctttctcccccagccttcccaccacacccctcagcctgtcttttcaccattgacacttgccacccctattcctcttcccaacacctgccaagtcccacccaccttgcagacccttcctatgccacctgtagcccctaccccaggctctgaaaatgaggcaagagggaatgggacttggtccttcccttcttgcatgaggattttttttttttttttttttgagacagagtcttgctgtgtcacccgggctggactacagtggtgtgatcatggctcactggggcttcaacctcccaggcataggtgatcctcctgcctcagcctcctgagtatctgggaccacaggcatgcaccaccacatctggctaattcttgtatgttttggtagatatgggatctcttgctatgttgcccaggctggtcttgaactcctggctcaagggattctcctgcctcaacctcccaaagtgctaggattacaggtgtgagtaaccacacctagcccacatgaggatattttaagccaagacccaacaaaggtggaaaaacacaccagagagtgcacagatgagttccaccaaaagaaaaatatttgtaaaaaacttggccaggcgcagtagctcacacctgtaatcccagcactttgggaggccaaggcaggcagatcacctgaggtcaggatttcaagaccagcctggccaacatggtgaagctgcatctctactaaaaatacaaaaattagccaggtgtggtgacgggcgcctgtaatcccagctactcgggaggctgaggcaggagaattgtgtaaacccaggaggtggaggttgcagtgagccgagatcacgccattgcactctagcccgagtaacagtgtgagaatccatctcaaaaaataaaaataaaaaataacaatgagaaaaataaaatgagccaaatgttgtgcattatgaggaaggatgggatactggcttgactgggtaaggaaatgtgaaaccactgcaagaatacaaagatgacacacacacacgtgacaatgagcagacaataggttatatctctaaggagctatgtcacacagtgctttaaacacagaggtgaaatgaagacaaaagaaagatggaagtgtggagcccggggcaggtgcttagctcagttcaggcctggcacatccccttccccattttgtccctgtcttggctagacctgttttctcctcagaggcccacagaccagacctttgaggaatagagcaagatgaaacctgaagttgctttccaccagacctctgggtgacccctgagtcttcagttgttccccacattcaaaagaggccacagcttcccttcacagaagctggggggacagatgcagtgatgtctcccacactctggatttctcaggacacagagctaccaggggtgtggagggggcatttccagcaaaaaaaaaagctggcatggagggaacaatagtgtccctactcatttccacctgtcagttacagtccacacccactgccaggcgcccactgcaagtcacccgccagcatccaccttcccctccagagaaagcccaagacttggaaaatgtgtttcacagaaacccatcaaccccgttcccaaactatctagaaacccaacagaggtaggaaccactgccagcatcggaactggagacaaggaaggtgaacgctgaagaaaacaaaactctcagctgttttaagaaagaactgggctgggtgcagtggctcatgcctgtaatcccagcactttgggaggccgagaaaggaggatcagtttgagtccaggagttcgagaccagcctgggcaacatggtgaaaccctgtctgtataaaaaatttaaaaattagccaggtgtggtggtgcatgcctgtagtcccagctactcaggaggctgagatgggaggatcacttgagcccaggaggtagaggctgcagtgatccatgatcacactactgtactccagcctggtcaacagaacaagaccctatcataaaaacaaacaaacaaacaaaaacctagatgttgggaaaccaacaagattagattccaactgtgtcacactcagggaagcagtatagccacattcctccaggccaaaatagaaactgatttccagaacgtgcatttcactcaattactttcactgtgggggtcgtcctctctccctaatgggcagcaagatgtggctgaacttacatcatctgaggaagtttacgtcatctcatccctgcctggtaagttcaaggttaccaggaagtgagataaaaatcaactcctgactcctgggcgagtgtccaaaagcaatctacataaaaccctttggccgcccggaattcctcctgctcagacatgccgggacatgcagagctctgccaactccagcccccgcgcccccgttttgagccccccgcgccaccccgctaaggagaacaacaaactcgtcccagcaccaaaaccctgaagctccaggccagaagtaggggggggtttccgctgatgtggagttttacatattaaaaaagaaaagtcaaaagcagacaaaatccgcctttccacaggtggccctggtctccatggcgacagctcatagcttggtgttgaaaggaccacgacccccatggccacatctggggcagcagtcccaccccgttgcctggccacggaccccatgccttaagcaagggggcctcatttttggccctaaaacaaagacatgccatcttaagtccaattgttttgagacagagtctcgctctgtcacccaggctggagtgcagctgtgcaatctcagctcactgcaacctctgcctcccaagttcaagcgattctccagcctcagcctcccgagtagctgggactacaggcactcatcaccatgcccggctaatttttgtatttttagtagaggcagggtttcaccatgttggccaggctgatcttgaactcctgatctcaggtgatccgcccaccctggccttccaaagtgctgggattacaggcatgagccactgcgcctggccaagacatggcatcttaagtccaattttcagggcaggaggcaaaagtggcatcaccctggtgggcgagtgggggtggggggaaaacacttttgttgttggctaaaaagcctgcattttaaccaaagggaatataaattactctgtgcccaaactagcactatttaaaaaaaaaaaaaaagagagagagagaagaaagaaagcaagaaagaaagaaagcaagaaagaaagaaagaaagaaagaaagaaagccagccagccagccatatcccagggtggccccagaaagggccaggctgttgagcacagttcaaggtcgaggacgcattgagaggcttttaaatttggtaaaagccagtcttggatataaaatgaattctgaaattccttcaccaacggacaggaaagcaggtgaacatatggccccagccgtggtatcgcagctcatggattcaccagaccaagattctccctgggcatctggacctcccaggctggcctccctggtcacggcagctgtgtccccagatgcagggaggaaaatgggagaaaaaaaaattttcaccacttccctcgaatcaaccggagcttttgtagagaaggaggaagaggaggtgggcagatcagaatctctcttccagatcggatccccaagctgaagagcttgtcttttcctggccacaccccagagggtggatgtcccctcgtggggtccccagcaggatgaggtcttaggagacctgagcgtccctcagtgtttgtggcaatagttgattttgccctctgactgctccaggaggtccaacatctcctcaatgatggctctcagtgccctgcccagctggtccgcgttgtacggcttccccagtgggggcacgtggacgaaggctgatcgaccgtgactctgccggcatcctgcgagatggtcaccgacacatccaggcccaacgtggtgactcgcttgcacacagcatccatgtcgatgatggagtcaatgctttcaggcccgtcctccacgcagcactgggagccggggcaaaagcggcagttgtccagccccttgtagcccttgttgtgtccacatttctccagtgtgactgtggtcgccatgcctgacacccccacatgcaccaccagctgtggactgtgcttctcccacagggcggggatgagtctctggactgtttggtactcaaccggaatctcgtacacatgcaggtccacgctgtcgccaaggcctagcttttctagctcctgaactgcaatccaactggcgttcacggtgtgttccccaaaagggccaaatcccgtcactaccaccgccttcctcggctgctccatggcgggatcgggctgtgcctcggacctgcttctgttgcgactggcgcgacagctgctgccgctgcagcctctcggccgcgcgag

SEQ ID NO: 11571 - RNA, 5239 nt, Homo sapiens
  source 1..5239: mol_type = other RNA
ctgaatagctgggactacaggtgcttgacaccacaactggctaatttttttttttaatttctgtagagatggggtctcgccatgttgcccagggctggtctcgaactcccgggctcaagcaatcctcccacctcagcctcccaaagcactgggatcacagacatgaaccatctccaggattcccctccttgccgagaaactactgccatctgggacatttccttcacacatctggctctgatggggaagctgtgatttcggcccccaccccctgtccctgcccagccctgcctctccaagtggcctcaggtttgttccagcccttgattggagcaggtgggctaggtggccccaagctcagcccacccaccttgaattcctgcttcttcctttctttcctttccactccatcttatttcttttttgagctacatccccacacgcatgcaactgaccttctttggggtggggagggggtgctaggggccgaataaaggaataaaagtgcgcagacttgggcatcttaaaagagatgccatcatcaagttggtcagggtaccaggtgccctgatcactgtccctgcacccctgttccctgcctcagcaccctccatgaggactcatcagggaagcccccccaatcacttctcacctttctcccccagccttcccaccacacccctcagcctgtcttttcaccattgacacttgccacccctattcctcttcccaacacctgccaagtcccacccaccttgcagacccttcctatgccacctgtagcccctaccccaggctctgaaaatgaggcaagagggaatgggacttggtccttcccttcttgcatgaggattttttttttttttttttttgagacagagtcttgctgtgtcacccgggctggactacagtggtgtgatcatggctcactggggcttcaacctcccaggcataggtgatcctcctgcctcagcctcctgagtatctgggaccacaggcatgcaccaccacatctggctaattcttgtatgttttggtagatatgggatctcttgctatgttgcccaggctggtcttgaactcctggctcaagggattctcctgcctcaacctcccaaagtgctaggattacaggtgtgagtaaccacacctagcccacatgaggatattttaagccaagacccaacaaaggtggaaaaacacaccagagagtgcacagatgagttccaccaaaagaaaaatatttgtaaaaaacttggccaggcgcagtagctcacacctgtaatcccagcactttgggaggccaaggcaggcagatcacctgaggtcaggatttcaagaccagcctggccaacatggtgaagctgcatctctactaaaaatacaaaaattagccaggtgtggtgacgggcgcctgtaatcccagctactcgggaggctgaggcaggagaattgtgtaaacccaggaggtggaggttgcagtgagccgagatcacgccattgcactctagcccgagtaacagtgtgagaatccatctcaaaaaataaaaataaaaaataacaatgagaaaaataaaatgagccaaatgttgtgcattatgaggaaggatgggatactggcttgactgggtaaggaaatgtgaaaccactgcaagaatacaaagatgacacacacacacgtgacaatgagcagacaataggttatatctctaaggagctatgtcacacagtgctttaaacacagaggtgaaatgaagacaaaagaaagatggaagtgtggagcccggggcaggtgcttagctcagttcaggcctggcacatccccttccccattttgtccctgtcttggctagacctgttttctcctcagaggcccacagaccagacctttgaggaatagagcaagatgaaacctgaagttgctttccaccagacctctgggtgacccctgagtcttcagttgttccccacattcaaaagaggccacagcttcccttcacagaagctggggggacagatgcagtgatgtctcccacactctggatttctcaggacacagagctaccaggggtgtggagggggcatttccagcaaaaaaaaaagctggcatggagggaacaatagtgtccctactcatttccacctgtcagttacagtccacacccactgccaggcgcccactgcaagtcacccgccagcatccaccttcccctccagagaaagcccaagacttggaaaatgtgtttcacagaaacccatcaaccccgttcccaaactatctagaaacccaacagaggtaggaaccactgccagcatcggaactggagacaaggaaggtgaacgctgaagaaaacaaaactctcagctgttttaagaaagaactgggctgggtgcagtggctcatgcctgtaatcccagcactttgggaggccgagaaaggaggatcagtttgagtccaggagttcgagaccagcctgggcaacatggtgaaaccctgtctgtataaaaaatttaaaaattagccaggtgtggtggtgcatgcctgtagtcccagctactcaggaggctgagatgggaggatcacttgagcccaggaggtagaggctgcagtgatccatgatcacactactgtactccagcctggtcaacagaacaagaccctatcataaaaacaaacaaacaaacaaaaacctagatgttgggaaaccaacaagattagattccaactgtgtcacactcagggaagcagtatagccacattcctccaggccaaaatagaaactgatttccagaacgtgcatttcactcaattactttcactgtgggggtcgtcctctctccctaatgggcagcaagatgtggctgaacttacatcatctgaggaagtttacgtcatctcatccctgcctggtaagttcaaggttaccaggaagtgagataaaaatcaactcctgactcctgggcgagtgtccaaaagcaatctacataaaaccctttggccgcccggaattcctcctgctcagacatgccgggacatgcagagctctgccaactccagcccccgcgcccccgttttgagccccccgcgccaccccgctaaggagaacaacaaactcgtcccagcaccaaaaccctgaagctccaggccagaagtaggggggggtttccgctgatgtggagttttacatattaaaaaagaaaagtcaaaagcagacaaaatccgcctttccacaggtggccctggtctccatggcgacagctcatagcttggtgttgaaaggaccacgacccccatggccacatctggggcagcagtcccaccccgttgcctggccacggaccccatgccttaagcaagggggcctcatttttggccctaaaacaaagacatgccatcttaagtccaattgttttgagacagagtctcgctctgtcacccaggctggagtgcagctgtgcaatctcagctcactgcaacctctgcctcccaagttcaagcgattctccagcctcagcctcccgagtagctgggactacaggcactcatcaccatgcccggctaatttttgtatttttagtagaggcagggtttcaccatgttggccaggctgatcttgaactcctgatctcaggtgatccgcccaccctggccttccaaagtgctgggattacaggcatgagccactgcgcctggccaagacatggcatcttaagtccaattttcagggcaggaggcaaaagtggcatcaccctggtgggcgagtgggggtggggggaaaacacttttgttgttggctaaaaagcctgcattttaaccaaagggaatataaattactctgtgcccaaactagcactatttaaaaaaaaaaaaaaagagagagagagaagaaagaaagcaagaaagaaagaaagcaagaaagaaagaaagaaagaaagaaagaaagccagccagccagccatatcccagggtggccccagaaagggccaggctgttgagcacagttcaaggtcgaggacgcattgagaggcttttaaatttggtaaaagccagtcttggatataaaatgaattctgaaattccttcaccaacggacaggaaagcaggtgaacatatggccccagccgtggtatcgcagctcatggattcaccagaccaagattctccctgggcatctggacctcccaggctggcctccctggtcacggcagctgtgtccccagatgcagggaggaaaatgggagaaaaaaaaattttcaccacttccctcgaatcaaccggagcttttgtagagaaggaggaagaggaggtgggcagatcagaatctctcttccagatcggatccccaagctgaagagcttgtcttttcctggccacaccccagagggtggatgtcccctcgtggggtccccagcaggatgaggtcttaggagacctgagcgtccctcagtgtttgtggcaatagttgattttgccctctgactgctccaggaggtccaacatctcctcaatgatggctctcagtgccctgcccagctggtccgcgttgtacggcttccccagtgggggcacgtggacgaaggctgatcgaccgtgactctgccggcatcctgcgagatggtcaccgacacatccaggcccaacgtggtgactcgcttgcacacagcatccatgtcgatgatggagtcaatgctttcaggcccgtcctccacgcagcactgggagccggggcaaaagcggcagttgtccagccccttgtagcccttgttgtgtccacatttctccagtgtgactgtggtcgccatgcctgacacccccacatgcaccaccagctgtggactgtgcttctcccacagggcggggatgagtctctggactgtttggtactcaaccggaatctcgtacacatgcaggtccacgctgtcgccaaggcctagcttttctagctcctgatggcagggctcggtggctcacacctataatcccagcttctttgggaggccgaggtggaaggatcatttgagcccggaagttcaagaccagccagggcaatatagtgagatcccatctctgaactgcaatccaactggcgttcacggtgtgttccccaaaagggccaaatcccgtcactaccaccgccttcctcggctgctccatggcgggatcgggctgtgcctcggacctgcttctgttgcgactggcgcgacagctgctgccgctgcagcctctcggccgcgcgag

SEQ ID NO: 11572 - RNA, 5105 nt, Homo sapiens
  source 1..5105: mol_type = other RNA
ctgaatagctgggactacaggtgcttgacaccacaactggctaatttttttttttaatttctgtagagatggggtctcgccatgttgcccagggctggtctcgaactcccgggctcaagcaatcctcccacctcagcctcccaaagcactgggatcacagacatgaaccatctccaggattcccctccttgccgagaaactactgccatctgggacatttccttcacacatctggctctgatggggaagctgtgatttcggcccccaccccctgtccctgcccagccctgcctctccaagtggcctcaggtttgttccagcccttgattggagcaggtgggctaggtggccccaagctcagcccacccaccttgaattcctgcttcttcctttctttcctttccactccatcttatttcttttttgagctacatccccacacgcatgcaactgaccttctttggggtggggagggggtgctaggggccgaataaaggaataaaagtgcgcagacttgggcatcttaaaagagatgccatcatcaagttggtcagggtaccaggtgccctgatcactgtccctgcacccctgttccctgcctcagcaccctccatgaggactcatcagggaagcccccccaatcacttctcacctttctcccccagccttcccaccacacccctcagcctgtcttttcaccattgacacttgccacccctattcctcttcccaacacctgccaagtcccacccaccttgcagacccttcctatgccacctgtagcccctaccccaggctctgaaaatgaggcaagagggaatgggacttggtccttcccttcttgcatgaggattttttttttttttttttttgagacagagtcttgctgtgtcacccgggctggactacagtggtgtgatcatggctcactggggcttcaacctcccaggcataggtgatcctcctgcctcagcctcctgagtatctgggaccacaggcatgcaccaccacatctggctaattcttgtatgttttggtagatatgggatctcttgctatgttgcccaggctggtcttgaactcctggctcaagggattctcctgcctcaacctcccaaagtgctaggattacaggtgtgagtaaccacacctagcccacatgaggatattttaagccaagacccaacaaaggtggaaaaacacaccagagagtgcacagatgagttccaccaaaagaaaaatatttgtaaaaaacttggccaggcgcagtagctcacacctgtaatcccagcactttgggaggccaaggcaggcagatcacctgaggtcaggatttcaagaccagcctggccaacatggtgaagctgcatctctactaaaaatacaaaaattagccaggtgtggtgacgggcgcctgtaatcccagctactcgggaggctgaggcaggagaattgtgtaaacccaggaggtggaggttgcagtgagccgagatcacgccattgcactctagcccgagtaacagtgtgagaatccatctcaaaaaataaaaataaaaaataacaatgagaaaaataaaatgagccaaatgttgtgcattatgaggaaggatgggatactggcttgactgggtaaggaaatgtgaaaccactgcaagaatacaaagatgacacacacacacgtgacaatgagcagacaataggttatatctctaaggagctatgtcacacagtgctttaaacacagaggtgaaatgaagacaaaagaaagatggaagtgtggagcccggggcaggtgcttagctcagttcaggcctggcacatccccttccccattttgtccctgtcttggctagacctgttttctcctcagaggcccacagaccagacctttgaggaatagagcaagatgaaacctgaagttgctttccaccagacctctgggtgacccctgagtcttcagttgttccccacattcaaaagaggccacagcttcccttcacagaagctggggggacagatgcagtgatgtctcccacactctggatttctcaggacacagagctaccaggggtgtggagggggcatttccagcaaaaaaaaaagctggcatggagggaacaatagtgtccctactcatttccacctgtcagttacagtccacacccactgccaggcgcccactgcaagtcacccgccagcatccaccttcccctccagagaaagcccaagacttggaaaatgtgtttcacagaaacccatcaaccccgttcccaaactatctagaaacccaacagaggtaggaaccactgccagcatcggaactggagacaaggaaggtgaacgctgaagaaaacaaaactctcagctgttttaagaaagaactgggctgggtgcagtggctcatgcctgtaatcccagcactttgggaggccgagaaaggaggatcagtttgagtccaggagttcgagaccagcctgggcaacatggtgaaaccctgtctgtataaaaaatttaaaaattagccaggtgtggtggtgcatgcctgtagtcccagctactcaggaggctgagatgggaggatcacttgagcccaggaggtagaggctgcagtgatccatgatcacactactgtactccagcctggtcaacagaacaagaccctatcataaaaacaaacaaacaaacaaaaacctagatgttgggaaaccaacaagattagattccaactgtgtcacactcagggaagcagtatagccacattcctccaggccaaaatagaaactgatttccagaacgtgcatttcactcaattactttcactgtgggggtcgtcctctctccctaatgggcagcaagatgtggctgaacttacatcatctgaggaagtttacgtcatctcatccctgcctggtaagttcaaggttaccaggaagtgagataaaaatcaactcctgactcctgggcgagtgtccaaaagcaatctacataaaaccctttggccgcccggaattcctcctgctcagacatgccgggacatgcagagctctgccaactccagcccccgcgcccccgttttgagccccccgcgccaccccgctaaggagaacaacaaactcgtcccagcaccaaaaccctgaagctccaggccagaagtaggggggggtttccgctgatgtggagttttacatattaaaaaagaaaagtcaaaagcagacaaaatccgcctttccacaggtggccctggtctccatggcgacagctcatagcttggtgttgaaaggaccacgacccccatggccacatctggggcagcagtcccaccccgttgcctggccacggaccccatgccttaagcaagggggcctcatttttggccctaaaacaaagacatgccatcttaagtccaattgttttgagacagagtctcgctctgtcacccaggctggagtgcagctgtgcaatctcagctcactgcaacctctgcctcccaagttcaagcgattctccagcctcagcctcccgagtagctgggactacaggcactcatcaccatgcccggctaatttttgtatttttagtagaggcagggtttcaccatgttggccaggctgatcttgaactcctgatctcaggtgatccgcccaccctggccttccaaagtgctgggattacaggcatgagccactgcgcctggccaagacatggcatcttaagtccaattttcagggcaggaggcaaaagtggcatcaccctggtgggcgagtgggggtggggggaaaacacttttgttgttggctaaaaagcctgcattttaaccaaagggaatataaattactctgtgcccaaactagcactatttaaaaaaaaaaaaaaagagagagagagaagaaagaaagcaagaaagaaagaaagcaagaaagaaagaaagaaagaaagaaagaaagccagccagccagccatatcccagggtggccccagaaagggccaggctgttgagcacagttcaaggtcgaggacgcattgagaggcttttaaatttggtaaaagccagtcttggatataaaatgaattctgaaattccttcaccaacggacaggaaagcaggtgaacatatggccccagccgtggtatcgcagctcatggattcaccagaccaagattctccctgggcatctggacctcccaggctggcctccctggtcacggcagctgtgtccccagatgcagggaggaaaatgggagaaaaaaaaattttcaccacttccctcgaatcaaccggagcttttgtagagaaggaggaagaggaggtgggcagatcagaatctctcttccagatcggatccccaagctgaagagcttgtcttttcctggccacaccccagagggtggatgtcccctcgtggggtccccagcaggatgaggtcttaggagacctgagcgtccctcagtgtttgtggcaatagttgattttgccctctgactgctccaggaggtccaacatctcctcaatgatggctctcagtgccctgcccagctggtccgcgttgtacggcttccccagtgggggcacgtggacgaaggctgatcgaccgtgactctggtacaaagaggtgtagtaggtaaagtcgcagagatatctgccggcatcctgcgagatggtcaccgacacatccaggcccaacgtggtgactcgcttgcacacagcatccatgtcgatgatggagtcaatgctttcaggcccgtcctccacgcagcactgggagccggggcaaaagcggcagttgtccagccccttgtagcccttgttgtgtccacatttctccagtgtgactgtggtcgccatgcctgacacccccacatgcaccaccagctgtggactgtgcttctcccacagggcggggatgagtctctggactgtttggtactcaaccggaatctcgtacacatgcaggtccacgctgtcgccaaggcctagcttttctagctcccgtcactaccaccgccttcctcggctgctccatggcgggatcgggctgtgcctcggacctgcttctgttgcgactggcgcgacagctgctgccgctgcagcctctcggccgcgcgag

SEQ ID NO: 11573 - RNA, 5158 nt, Homo sapiens
  source 1..5158: mol_type = other RNA
ctgaatagctgggactacaggtgcttgacaccacaactggctaatttttttttttaatttctgtagagatggggtctcgccatgttgcccagggctggtctcgaactcccgggctcaagcaatcctcccacctcagcctcccaaagcactgggatcacagacatgaaccatctccaggattcccctccttgccgagaaactactgccatctgggacatttccttcacacatctggctctgatggggaagctgtgatttcggcccccaccccctgtccctgcccagccctgcctctccaagtggcctcaggtttgttccagcccttgattggagcaggtgggctaggtggccccaagctcagcccacccaccttgaattcctgcttcttcctttctttcctttccactccatcttatttcttttttgagctacatccccacacgcatgcaactgaccttctttggggtggggagggggtgctaggggccgaataaaggaataaaagtgcgcagacttgggcatcttaaaagagatgccatcatcaagttggtcagggtaccaggtgccctgatcactgtccctgcacccctgttccctgcctcagcaccctccatgaggactcatcagggaagcccccccaatcacttctcacctttctcccccagccttcccaccacacccctcagcctgtcttttcaccattgacacttgccacccctattcctcttcccaacacctgccaagtcccacccaccttgcagacccttcctatgccacctgtagcccctaccccaggctctgaaaatgaggcaagagggaatgggacttggtccttcccttcttgcatgaggattttttttttttttttttttgagacagagtcttgctgtgtcacccgggctggactacagtggtgtgatcatggctcactggggcttcaacctcccaggcataggtgatcctcctgcctcagcctcctgagtatctgggaccacaggcatgcaccaccacatctggctaattcttgtatgttttggtagatatgggatctcttgctatgttgcccaggctggtcttgaactcctggctcaagggattctcctgcctcaacctcccaaagtgctaggattacaggtgtgagtaaccacacctagcccacatgaggatattttaagccaagacccaacaaaggtggaaaaacacaccagagagtgcacagatgagttccaccaaaagaaaaatatttgtaaaaaacttggccaggcgcagtagctcacacctgtaatcccagcactttgggaggccaaggcaggcagatcacctgaggtcaggatttcaagaccagcctggccaacatggtgaagctgcatctctactaaaaatacaaaaattagccaggtgtggtgacgggcgcctgtaatcccagctactcgggaggctgaggcaggagaattgtgtaaacccaggaggtggaggttgcagtgagccgagatcacgccattgcactctagcccgagtaacagtgtgagaatccatctcaaaaaataaaaataaaaaataacaatgagaaaaataaaatgagccaaatgttgtgcattatgaggaaggatgggatactggcttgactgggtaaggaaatgtgaaaccactgcaagaatacaaagatgacacacacacacgtgacaatgagcagacaataggttatatctctaaggagctatgtcacacagtgctttaaacacagaggtgaaatgaagacaaaagaaagatggaagtgtggagcccggggcaggtgcttagctcagttcaggcctggcacatccccttccccattttgtccctgtcttggctagacctgttttctcctcagaggcccacagaccagacctttgaggaatagagcaagatgaaacctgaagttgctttccaccagacctctgggtgacccctgagtcttcagttgttccccacattcaaaagaggccacagcttcccttcacagaagctggggggacagatgcagtgatgtctcccacactctggatttctcaggacacagagctaccaggggtgtggagggggcatttccagcaaaaaaaaaagctggcatggagggaacaatagtgtccctactcatttccacctgtcagttacagtccacacccactgccaggcgcccactgcaagtcacccgccagcatccaccttcccctccagagaaagcccaagacttggaaaatgtgtttcacagaaacccatcaaccccgttcccaaactatctagaaacccaacagaggtaggaaccactgccagcatcggaactggagacaaggaaggtgaacgctgaagaaaacaaaactctcagctgttttaagaaagaactgggctgggtgcagtggctcatgcctgtaatcccagcactttgggaggccgagaaaggaggatcagtttgagtccaggagttcgagaccagcctgggcaacatggtgaaaccctgtctgtataaaaaatttaaaaattagccaggtgtggtggtgcatgcctgtagtcccagctactcaggaggctgagatgggaggatcacttgagcccaggaggtagaggctgcagtgatccatgatcacactactgtactccagcctggtcaacagaacaagaccctatcataaaaacaaacaaacaaacaaaaacctagatgttgggaaaccaacaagattagattccaactgtgtcacactcagggaagcagtatagccacattcctccaggccaaaatagaaactgatttccagaacgtgcatttcactcaattactttcactgtgggggtcgtcctctctccctaatgggcagcaagatgtggctgaacttacatcatctgaggaagtttacgtcatctcatccctgcctggtaagttcaaggttaccaggaagtgagataaaaatcaactcctgactcctgggcgagtgtccaaaagcaatctacataaaaccctttggccgcccggaattcctcctgctcagacatgccgggacatgcagagctctgccaactccagcccccgcgcccccgttttgagccccccgcgccaccccgctaaggagaacaacaaactcgtcccagcaccaaaaccctgaagctccaggccagaagtaggggggggtttccgctgatgtggagttttacatattaaaaaagaaaagtcaaaagcagacaaaatccgcctttccacaggtggccctggtctccatggcgacagctcatagcttggtgttgaaaggaccacgacccccatggccacatctggggcagcagtcccaccccgttgcctggccacggaccccatgccttaagcaagggggcctcatttttggccctaaaacaaagacatgccatcttaagtccaattgttttgagacagagtctcgctctgtcacccaggctggagtgcagctgtgcaatctcagctcactgcaacctctgcctcccaagttcaagcgattctccagcctcagcctcccgagtagctgggactacaggcactcatcaccatgcccggctaatttttgtatttttagtagaggcagggtttcaccatgttggccaggctgatcttgaactcctgatctcaggtgatccgcccaccctggccttccaaagtgctgggattacaggcatgagccactgcgcctggccaagacatggcatcttaagtccaattttcagggcaggaggcaaaagtggcatcaccctggtgggcgagtgggggtggggggaaaacacttttgttgttggctaaaaagcctgcattttaaccaaagggaatataaattactctgtgcccaaactagcactatttaaaaaaaaaaaaaaagagagagagagaagaaagaaagcaagaaagaaagaaagcaagaaagaaagaaagaaagaaagaaagaaagccagccagccagccatatcccagggtggccccagaaagggccaggctgttgagcacagttcaaggtcgaggacgcattgagaggcttttaaatttggtaaaagccagtcttggatataaaatgaattctgaaattccttcaccaacggacaggaaagcaggtgaacatatggccccagccgtggtatcgcagctcatggattcaccagaccaagattctccctgggcatctggacctcccaggctggcctccctggtcacggcagctgtgtccccagatgcagggaggaaaatgggagaaaaaaaaattttcaccacttccctcgaatcaaccggagcttttgtagagaaggaggaagaggaggtgggcagatcagaatctctcttccagatcggatccccaagctgaagagcttgtcttttcctggccacaccccagagggtggatgtcccctcgtggggtccccagcaggatgaggtcttaggagacctgagcgtccctcagtgtttgtggcaatagttgattttgccctctgactgctccaggaggtccaacatctcctcaatgatggctctcagtgccctgcccagctggtccgcgttgtacggcttccccagtgggggcacgtggacgaaggctgatcgaccgtgactctggtacaaagaggtgtagtaggtaaagtcgcagagatatctgccggcatcctgcgagatggtcaccgacacatccaggcccaacgtggtgactcgcttgcacacagcatccatgtcgatgatggagtcaatgctttcaggcccgtcctccacgcagcactgggagccggggcaaaagcggcagttgtccagccccttgtagcccttgttgtgtccacatttctccagtgtgactgtggtcgccatgcctgacacccccacatgcaccaccagctgtggactgtgcttctcccacagggcggggatgagtctctggactgtttggtactcaaccggaatctcgtacacatgcaggtccacgctgtcgccaaggcctagcttttctagctcctgaactgcaatccaactggcgttcacggtgtgttccccaaaagggccaaatcccgtcactaccaccgccttcctcggctgctccatggcgggatcgggctgtgcctcggacctgcttctgttgcgactggcgcgacagctgctgccgctgcagcctctcggccgcgcgag

SEQ ID NO: 11574 - RNA, 5279 nt, Homo sapiens
  source 1..5279: mol_type = other RNA
ctgaatagctgggactacaggtgcttgacaccacaactggctaatttttttttttaatttctgtagagatggggtctcgccatgttgcccagggctggtctcgaactcccgggctcaagcaatcctcccacctcagcctcccaaagcactgggatcacagacatgaaccatctccaggattcccctccttgccgagaaactactgccatctgggacatttccttcacacatctggctctgatggggaagctgtgatttcggcccccaccccctgtccctgcccagccctgcctctccaagtggcctcaggtttgttccagcccttgattggagcaggtgggctaggtggccccaagctcagcccacccaccttgaattcctgcttcttcctttctttcctttccactccatcttatttcttttttgagctacatccccacacgcatgcaactgaccttctttggggtggggagggggtgctaggggccgaataaaggaataaaagtgcgcagacttgggcatcttaaaagagatgccatcatcaagttggtcagggtaccaggtgccctgatcactgtccctgcacccctgttccctgcctcagcaccctccatgaggactcatcagggaagcccccccaatcacttctcacctttctcccccagccttcccaccacacccctcagcctgtcttttcaccattgacacttgccacccctattcctcttcccaacacctgccaagtcccacccaccttgcagacccttcctatgccacctgtagcccctaccccaggctctgaaaatgaggcaagagggaatgggacttggtccttcccttcttgcatgaggattttttttttttttttttttgagacagagtcttgctgtgtcacccgggctggactacagtggtgtgatcatggctcactggggcttcaacctcccaggcataggtgatcctcctgcctcagcctcctgagtatctgggaccacaggcatgcaccaccacatctggctaattcttgtatgttttggtagatatgggatctcttgctatgttgcccaggctggtcttgaactcctggctcaagggattctcctgcctcaacctcccaaagtgctaggattacaggtgtgagtaaccacacctagcccacatgaggatattttaagccaagacccaacaaaggtggaaaaacacaccagagagtgcacagatgagttccaccaaaagaaaaatatttgtaaaaaacttggccaggcgcagtagctcacacctgtaatcccagcactttgggaggccaaggcaggcagatcacctgaggtcaggatttcaagaccagcctggccaacatggtgaagctgcatctctactaaaaatacaaaaattagccaggtgtggtgacgggcgcctgtaatcccagctactcgggaggctgaggcaggagaattgtgtaaacccaggaggtggaggttgcagtgagccgagatcacgccattgcactctagcccgagtaacagtgtgagaatccatctcaaaaaataaaaataaaaaataacaatgagaaaaataaaatgagccaaatgttgtgcattatgaggaaggatgggatactggcttgactgggtaaggaaatgtgaaaccactgcaagaatacaaagatgacacacacacacgtgacaatgagcagacaataggttatatctctaaggagctatgtcacacagtgctttaaacacagaggtgaaatgaagacaaaagaaagatggaagtgtggagcccggggcaggtgcttagctcagttcaggcctggcacatccccttccccattttgtccctgtcttggctagacctgttttctcctcagaggcccacagaccagacctttgaggaatagagcaagatgaaacctgaagttgctttccaccagacctctgggtgacccctgagtcttcagttgttccccacattcaaaagaggccacagcttcccttcacagaagctggggggacagatgcagtgatgtctcccacactctggatttctcaggacacagagctaccaggggtgtggagggggcatttccagcaaaaaaaaaagctggcatggagggaacaatagtgtccctactcatttccacctgtcagttacagtccacacccactgccaggcgcccactgcaagtcacccgccagcatccaccttcccctccagagaaagcccaagacttggaaaatgtgtttcacagaaacccatcaaccccgttcccaaactatctagaaacccaacagaggtaggaaccactgccagcatcggaactggagacaaggaaggtgaacgctgaagaaaacaaaactctcagctgttttaagaaagaactgggctgggtgcagtggctcatgcctgtaatcccagcactttgggaggccgagaaaggaggatcagtttgagtccaggagttcgagaccagcctgggcaacatggtgaaaccctgtctgtataaaaaatttaaaaattagccaggtgtggtggtgcatgcctgtagtcccagctactcaggaggctgagatgggaggatcacttgagcccaggaggtagaggctgcagtgatccatgatcacactactgtactccagcctggtcaacagaacaagaccctatcataaaaacaaacaaacaaacaaaaacctagatgttgggaaaccaacaagattagattccaactgtgtcacactcagggaagcagtatagccacattcctccaggccaaaatagaaactgatttccagaacgtgcatttcactcaattactttcactgtgggggtcgtcctctctccctaatgggcagcaagatgtggctgaacttacatcatctgaggaagtttacgtcatctcatccctgcctggtaagttcaaggttaccaggaagtgagataaaaatcaactcctgactcctgggcgagtgtccaaaagcaatctacataaaaccctttggccgcccggaattcctcctgctcagacatgccgggacatgcagagctctgccaactccagcccccgcgcccccgttttgagccccccgcgccaccccgctaaggagaacaacaaactcgtcccagcaccaaaaccctgaagctccaggccagaagtaggggggggtttccgctgatgtggagttttacatattaaaaaagaaaagtcaaaagcagacaaaatccgcctttccacaggtggccctggtctccatggcgacagctcatagcttggtgttgaaaggaccacgacccccatggccacatctggggcagcagtcccaccccgttgcctggccacggaccccatgccttaagcaagggggcctcatttttggccctaaaacaaagacatgccatcttaagtccaattgttttgagacagagtctcgctctgtcacccaggctggagtgcagctgtgcaatctcagctcactgcaacctctgcctcccaagttcaagcgattctccagcctcagcctcccgagtagctgggactacaggcactcatcaccatgcccggctaatttttgtatttttagtagaggcagggtttcaccatgttggccaggctgatcttgaactcctgatctcaggtgatccgcccaccctggccttccaaagtgctgggattacaggcatgagccactgcgcctggccaagacatggcatcttaagtccaattttcagggcaggaggcaaaagtggcatcaccctggtgggcgagtgggggtggggggaaaacacttttgttgttggctaaaaagcctgcattttaaccaaagggaatataaattactctgtgcccaaactagcactatttaaaaaaaaaaaaaaagagagagagagaagaaagaaagcaagaaagaaagaaagcaagaaagaaagaaagaaagaaagaaagaaagccagccagccagccatatcccagggtggccccagaaagggccaggctgttgagcacagttcaaggtcgaggacgcattgagaggcttttaaatttggtaaaagccagtcttggatataaaatgaattctgaaattccttcaccaacggacaggaaagcaggtgaacatatggccccagccgtggtatcgcagctcatggattcaccagaccaagattctccctgggcatctggacctcccaggctggcctccctggtcacggcagctgtgtccccagatgcagggaggaaaatgggagaaaaaaaaattttcaccacttccctcgaatcaaccggagcttttgtagagaaggaggaagaggaggtgggcagatcagaatctctcttccagatcggatccccaagctgaagagcttgtcttttcctggccacaccccagagggtggatgtcccctcgtggggtccccagcaggatgaggtcttaggagacctgagcgtccctcagtgtttgtggcaatagttgattttgccctctgactgctccaggaggtccaacatctcctcaatgatggctctcagtgccctgcccagctggtccgcgttgtacggcttccccagtgggggcacgtggacgaaggctgatcgaccgtgactctggtacaaagaggtgtagtaggtaaagtcgcagagatatctgccggcatcctgcgagatggtcaccgacacatccaggcccaacgtggtgactcgcttgcacacagcatccatgtcgatgatggagtcaatgctttcaggcccgtcctccacgcagcactgggagccggggcaaaagcggcagttgtccagccccttgtagcccttgttgtgtccacatttctccagtgtgactgtggtcgccatgcctgacacccccacatgcaccaccagctgtggactgtgcttctcccacagggcggggatgagtctctggactgtttggtactcaaccggaatctcgtacacatgcaggtccacgctgtcgccaaggcctagcttttctagctcctgatggcagggctcggtggctcacacctataatcccagcttctttgggaggccgaggtggaaggatcatttgagcccggaagttcaagaccagccagggcaatatagtgagatcccatctctgaactgcaatccaactggcgttcacggtgtgttccccaaaagggccaaatcccgtcactaccaccgccttcctcggctgctccatggcgggatcgggctgtgcctcggacctgcttctgttgcgactggcgcgacagctgctgccgctgcagcctctcggccgcgcgag

SEQ ID NO: 11575 - RNA, 4925 nt, Homo sapiens
  source 1..4925: mol_type = other RNA
ctgaatagctgggactacaggtgcttgacaccacaactggctaatttttttttttaatttctgtagagatggggtctcgccatgttgcccagggctggtctcgaactcccgggctcaagcaatcctcccacctcagcctcccaaagcactgggatcacagacatgaaccatctccaggattcccctccttgccgagaaactactgccatctgggacatttccttcacacatctggctctgatggggaagctgtgatttcggcccccaccccctgtccctgcccagccctgcctctccaagtggcctcaggtttgttccagcccttgattggagcaggtgggctaggtggccccaagctcagcccacccaccttgaattcctgcttcttcctttctttcctttccactccatcttatttcttttttgagctacatccccacacgcatgcaactgaccttctttggggtggggagggggtgctaggggccgaataaaggaataaaagtgcgcagacttgggcatcttaaaagagatgccatcatcaagttggtcagggtaccaggtgccctgatcactgtccctgcacccctgttccctgcctcagcaccctccatgaggactcatcagggaagcccccccaatcacttctcacctttctcccccagccttcccaccacacccctcagcctgtcttttcaccattgacacttgccacccctattcctcttcccaacacctgccaagtcccacccaccttgcagacccttcctatgccacctgtagcccctaccccaggctctgaaaatgaggcaagagggaatgggacttggtccttcccttcttgcatgaggattttttttttttttttttttgagacagagtcttgctgtgtcacccgggctggactacagtggtgtgatcatggctcactggggcttcaacctcccaggcataggtgatcctcctgcctcagcctcctgagtatctgggaccacaggcatgcaccaccacatctggctaattcttgtatgttttggtagatatgggatctcttgctatgttgcccaggctggtcttgaactcctggctcaagggattctcctgcctcaacctcccaaagtgctaggattacaggtgtgagtaaccacacctagcccacatgaggatattttaagccaagacccaacaaaggtggaaaaacacaccagagagtgcacagatgagttccaccaaaagaaaaatatttgtaaaaaacttggccaggcgcagtagctcacacctgtaatcccagcactttgggaggccaaggcaggcagatcacctgaggtcaggatttcaagaccagcctggccaacatggtgaagctgcatctctactaaaaatacaaaaattagccaggtgtggtgacgggcgcctgtaatcccagctactcgggaggctgaggcaggagaattgtgtaaacccaggaggtggaggttgcagtgagccgagatcacgccattgcactctagcccgagtaacagtgtgagaatccatctcaaaaaataaaaataaaaaataacaatgagaaaaataaaatgagccaaatgttgtgcattatgaggaaggatgggatactggcttgactgggtaaggaaatgtgaaaccactgcaagaatacaaagatgacacacacacacgtgacaatgagcagacaataggttatatctctaaggagctatgtcacacagtgctttaaacacagaggtgaaatgaagacaaaagaaagatggaagtgtggagcccggggcaggtgcttagctcagttcaggcctggcacatccccttccccattttgtccctgtcttggctagacctgttttctcctcagaggcccacagaccagacctttgaggaatagagcaagatgaaacctgaagttgctttccaccagacctctgggtgacccctgagtcttcagttgttccccacattcaaaagaggccacagcttcccttcacagaagctggggggacagatgcagtgatgtctcccacactctggatttctcaggacacagagctaccaggggtgtggagggggcatttccagcaaaaaaaaaagctggcatggagggaacaatagtgtccctactcatttccacctgtcagttacagtccacacccactgccaggcgcccactgcaagtcacccgccagcatccaccttcccctccagagaaagcccaagacttggaaaatgtgtttcacagaaacccatcaaccccgttcccaaactatctagaaacccaacagaggtaggaaccactgccagcatcggaactggagacaaggaaggtgaacgctgaagaaaacaaaactctcagctgttttaagaaagaactgggctgggtgcagtggctcatgcctgtaatcccagcactttgggaggccgagaaaggaggatcagtttgagtccaggagttcgagaccagcctgggcaacatggtgaaaccctgtctgtataaaaaatttaaaaattagccaggtgtggtggtgcatgcctgtagtcccagctactcaggaggctgagatgggaggatcacttgagcccaggaggtagaggctgcagtgatccatgatcacactactgtactccagcctggtcaacagaacaagaccctatcataaaaacaaacaaacaaacaaaaacctagatgttgggaaaccaacaagattagattccaactgtgtcacactcagggaagcagtatagccacattcctccaggccaaaatagaaactgatttccagaacgtgcatttcactcaattactttcactgtgggggtcgtcctctctccctaatgggcagcaagatgtggctgaacttacatcatctgaggaagtttacgtcatctcatccctgcctggtaagttcaaggttaccaggaagtgagataaaaatcaactcctgactcctgggcgagtgtccaaaagcaatctacataaaaccctttggccgcccggaattcctcctgctcagacatgccgggacatgcagagctctgccaactccagcccccgcgcccccgttttgagccccccgcgccaccccgctaaggagaacaacaaactcgtcccagcaccaaaaccctgaagctccaggccagaagtaggggggggtttccgctgatgtggagttttacatattaaaaaagaaaagtcaaaagcagacaaaatccgcctttccacaggtggccctggtctccatggcgacagctcatagcttggtgttgaaaggaccacgacccccatggccacatctggggcagcagtcccaccccgttgcctggccacggaccccatgccttaagcaagggggcctcatttttggccctaaaacaaagacatgccatcttaagtccaattgttttgagacagagtctcgctctgtcacccaggctggagtgcagctgtgcaatctcagctcactgcaacctctgcctcccaagttcaagcgattctccagcctcagcctcccgagtagctgggactacaggcactcatcaccatgcccggctaatttttgtatttttagtagaggcagggtttcaccatgttggccaggctgatcttgaactcctgatctcaggtgatccgcccaccctggccttccaaagtgctgggattacaggcatgagccactgcgcctggccaagacatggcatcttaagtccaattttcagggcaggaggcaaaagtggcatcaccctggtgggcgagtgggggtggggggaaaacacttttgttgttggctaaaaagcctgcattttaaccaaagggaatataaattactctgtgcccaaactagcactatttaaaaaaaaaaaaaaagagagagagagaagaaagaaagcaagaaagaaagaaagcaagaaagaaagaaagaaagaaagaaagaaagccagccagccagccatatcccagggtggccccagaaagggccaggctgttgagcacagttcaaggtcgaggacgcattgagaggcttttaaatttggtaaaagccagtcttggatataaaatgaattctgaaattccttcaccaacggacaggaaagcaggtgaacatatggccccagccgtggtatcgcagctcatggattcaccagaccaagattctccctgggcatctggacctcccaggctggcctccctggtcacggcagctgtgtccccagatgcagggaggaaaatgggagaaaaaaaaattttcaccacttccctcgaatcaaccggagcttttgtagagaaggaggaagaggaggtgggcagatcagaatctctcttccagatcggatccccaagctgaagagcttgtcttttcctggccacaccccagagggtggatgtcccctcgtggggtccccagcaggatgaggtcttaggagacctgagcgtccctcagtgtttgtggcaatagttgattttgccctctgactgctccaggaggtccaacatctcctcaatgatggctctcagtgccctgcccagctggtccgcgttgtacggcttccccagtgggggcacgtggacgaaggctgatcgaccgtgactctggtacaaagaggtgtagtaggtaaagtcgcagagatatctgtggactgtgcttctcccacagggcggggatgagtctctggactgtttggtactcaaccggaatctcgtacacatgcaggtccacgctgtcgccaaggcctagcttttctagctcctgaactgcaatccaactggcgttcacggtgtgttccccaaaagggccaaatcccgtcactaccaccgccttcctcggctgctccatggcgggatcgggctgtgcctcggacctgcttctgttgcgactggcgcgacagctgctgccgctgcagcctctcggccgcgcgag

SEQ ID NO: 11576 - RNA, 1855 nt, Homo sapiens
  source 1..1855: mol_type = other RNA
ctgaatagctgggactacaggtgggagccacctggcccagcctataagcatttatccaatcaatgttaaacgttgcataatgaatagaagctgtagatattgccatactgtaatccaattttatggatatgagaagaaactcttggggttactaaaatagctgttttaactactagagagactacacaggtggttcaacagaatttacttgtatattttccattttctatactatttgaaggcataggatagttttgtattagctttctacaatactgtgttttaaatttatccagtaaactaagatgcagtacaacttttatacaactcaggagattaaaaaaaaaatctccacaagaagaagcaactcagcaggccctggcattaaaacatttcccagaataaacagatatgcattgcattaaaggtaattttcaaatatttaagttacaccaagatttccctccaatatgtgcctttctcaaaccaatgcaactaattcattgctaatactggggcatgaatttttggcaaatgtttatggttttactttcttcattaatcaaaaaattttttaaagtgctaccaagcagcaaaacaagtcgcatcagttctctgctcatggcagaagtgccaactgtgaaatcgcaaaaggtacagttttaacagtaagtaatgcatgaagaaactgtaacaaatggcctaaatacagagttggacagagtcaaaccagttatgtctagaattactcaattgaaactaatagaggtacattcaaaataaagttggagattataatcgctatttagaatcaaatttgaagacttccttgataaaatataagaatgttcttttgaaattgtaaatgaaactatcaatagatggagagctagagacttattaacccctcctacacacataaggaaataagtgacaaagtctcttgcactgaagttatgtattttaacagctttacatgtaatattcatatataaaaaactttaagtgcttttctccaatttaaaaatctaaagaattcaaaaataaggcattcaatatttgaaaaaagtacagatttacaaaatgtgtatattctgtcatgaaaactccacaccaacattatacacttggaaaaaaatacaaacaggatatattacaaatttatgcagcaataacttagttcacaccatgcaataaaaagtacattaatcaagatacacaagcttttgtaggttctaaactgaaggacttttttcttttttttctgcagaatccttaaaacctgtggcacttaaaatttgttagcctttctaatgagaggtaaattatacacaacaatgatgaaaaagattaacagaccagttgtctattatgaatcattccagctttgttcaacaatggccgaaactcttttctcatattctcgtttgttttcctgataaagctgtgctgcctggctattggctggactgttaggattcggttcatccagcagagactgaattgatgttaagatagaagatacatcatatgttggactccatcgattctgaaggatatctaaacatatgctaccatcagcatacacatttggatgaaacattttggataaaaacctaacagttggtggtttatttggatattcttcagaaaattctattactagtttaaaagtaccatcttcaaaaggtgtcccttctggtccaaatataactgcattccactgcatgatgttgttttcagatggtgcgccactgacacccacaggtgggtcctcttgtaaccgcttgaaatcccgcatgagcctcctccgggccggggtcgacatgctccgcagctgccccgcggtcagtct

SEQ ID NO: 11577 - RNA, 6276 nt, Homo sapiens
  source 1..6276: mol_type = other RNA
ctgaatagctgggactacaggtgggcaccagcactcctcgctaattttttttgtgtgtgtgtgttttgtttgcttgtttgtttgttgttgttttggttttttggggttttttttgtttttttttttttttttgcagagatggggttttgtcatgttgcctaggctggtctcaaactcctggactcaagcaatctgcccacctctgcctcccaaagtcctgggattacaggagtgagccactgcgcctagccctcctatctgctgctttgtatcctctgacctacatctctccaccctcctccacctcaggttttgttatctctgtatacctgtatttgagtgttttctttagattccccatgtgagtgaaatcgtgtaatatttttctttctgtatctgccttatttcacttaatatcctccagtttcatccatgttgtggcaaatggcaagatattctttttagggctgaataatattccattgtgtgtgtgtgtgtgtgtatacagtttctttatccattcattcttcaacaggcatttaggttgcttccctatattggctgcaatgctgcaatgaacgtgggatcacatttatctctacaaggtggctatctcattttatttgtgtatatcccctaaagagggattgttgggtcatatgtagccctattttcagtttatttagaaacctccatactgttttccacaatggctgtacattctcaccaacaatgcacaaaggttttctgttctcttcacccttatccacgtttatgattaatatcttttgactttttgataatagtcatcctattattatctagtgtctcataatggtttcaattcacatttcccttatgattagtgatgttgaacaccttttcatatccatcttggccatttttcttcttggagaaatgtcttttcaggtttttgcccatttttaactgggatcatttgttttcctgctattgagttgtatgagttctttatcaatttgttgtatcttattagatatatagtttgcaaatattttttccaatccataggttgccatttcattttgttgcttgttgtctttgctatgcagaagcttttcagcttgatgtagtcccatttatttatttttgcttttgtggcctgggcttttgatgtgatagccaaaaaatcattgctaaggccaaggttcaggagcttatcattacattttaacagctggaagagctcttccactctcatcagaatttttcttatctgtctcacttttgttttttagttgaggattagtatcattttgtcaagttaaaaaattgtatattgattaatttagggagaattgacatctttacaatactgagtcttcctatccaaagcaatatgtcttctttacattattttttactttgataagtgtggtttaaatgtagcttttattaatttactaaatgatacattttatttattcttgttaattattattgtcctaactcactattatttgtataaaagaaagttattttttattttaatatttcctttcactttactgaattttatcttaccacttttaccactttatttattattattattatttttattattttgagacagagttttgctcttgttgtctagactggagtgcaatggtgcgatctcggctcaccacaacttctgcctcccaggttcaagcaattctcccgcctcagcctcccgagtagctgggattacaggcatgcaccactacgcccggctaatttttattttaagtagagatggagtttctccatgttgtcaagctggtctcgaactcctgacctcaggtgatccgcccgacttggcctcccaaagtgctgagattacaggtgtgagccaccacgccctgcctattattattatttttattattttccagacagagtcttgctctgtcactaggctggagtgctctggtgcgaccttggctcactgcaacctctgcctcccaggatcaagcacttctcatgcttcagcctcctgagtagctgggactacaggtgtgtgccaccaaaccaggctaatttttgtatttttagaagagatggggtttcgccatgttggccaggctggtcttgaactcctgacctcaggtgatccacccacctcagcctcccaaaatgctgggattataggcatgaaccactgcgcctggccataatactttattattatttggttctcatggatttcctaggtgtataatcacttacaaataaaagtaattttggcatttctttaaatattataacttatttttcttgtataattggattggccacctgttctaaaacactgtaaaataagatagatagtaatcaatttttttcatgttcctaactttagtaggaatgcttctgtttcttcatcattaggtatgtattagcttttgtttacatgtatataaaattatggccaaataacatctgtctatcctattttagtaactaatttaataattaagaatggatgttgaatatttttgttttagcccagttgtctaagacttccaggaatatacctgtagtgtaataaaattaggtttattgatccattgcaatgagacagactgcgtcccaggggagccatggggtatctcaccaaacaaaggaaaaggcagagttataggatttggggtaagtttaggttaatattaaataaggcagatcgttgataggctcagaggaaagcagggctgtgtgtaaaacggtccatatcaggtctggactgcaaagtggacccagagtcctattttcttgaatactagacagttgagagaggtgtggaatgttgtgtccagataccccttatctgcacttctgtatttgagtataagatgaggctgtgttaggagtcaggaaaagaaaggagccaactgaagttatttagaaagcaaaatcaacagaacttggtgacgctggatgtagtgtgagggaaaatggcgaactgaaatttcacccctctatttatggcttatgtgattgggtagatgaccaggtcttcagctgatatggaatatactataacaacagttggtttagggaagcaagagagagaagaacaggatgatcacttcaatttttgatttgttgggtttctgactgctgcaagactcgagtatagacccacaggtaggtagtaggatgtataagtgcagggatactgctggaggctggggtcacagctatagatacagatgcctaggagtcatgagcatcactgaaggagggcctgcaaagtgagaggagcactgaccagatcaagagaaaaccccaggaagatttccctaaggtttccaggccagtaggatgagcccacagtgaagactacaaatgaacagagagaggtaggaatcaaagcagagacctgccatgtcagagaaactgaggaaaagagttccaaggaggagggagtggtcaactttatcaactgcaggaaatgggctcaggaatggaagacctgaattggtttaacagttggcaggtagacggtgacttttgccagggtacattcaggtaagttggtgaagcagaagaccaaattctgtatgttcagccaataataagtgagacagaaaagtcagcctccaccttacaggaagctgggctgagaagggcaggagacagggcagtaactgctgtggcatcaagctcagggaatgcttttcagcaaaaaagatgtcagtgtttcacttttttcagctagttagaatcaggacctcagcctgatggaattcatttaaaataccaaataaaggtaagtcttctgtagtctttctgtactcacttgagtacttgatctctgtaactcactctgcatcctccttcttgccccttccttagcatgacacacgcacgcgcacgtgcacacacacaccagtatacatttgattatattttaatgatcacgcagacccttttagaaaagatgtctccttgaactgtacccaggagatgtggccatggcacacacaaagctgtagggaaagaccagacgaatcttgagctgagaaggaagggctcagttgcataggtatttaggcagaatgcataaagaaatcctttgttgaaaatatttaggaaagaatggagtttttgaaatataaaatcaataataatttttattttttgttcagcacacatggcaacacagagctgtgaagacagacgtggttagcacaaaccacttgggccagtgaaaccagggcaaactcatggatcatctgcgttcccatcttcaccttggtggcagccctacctctgagattttaaggtctacggaaagtgcaggcttccaggagtgatgaggtggagcattttctcaggttaccaacagccttgacatattcttctcctaagtatttttcatatgtgtttctgtcatgaagtttggccaaacatactgtgtcatctctgaacagaaggtccttggtttccgaccggaacaaacaaaagttgcccgagcagtcagttacgttgcttccaaataggtgctgctgttgacgtaatatcttgtggacgcaagcttccttatctttccgtgtgaccacagcgtgattcggggctctggccaggtggcagttcgcatactcctccacaggtttcctggtaccatcaaggcacagcaactcatagtctttttcattcagattcttagcccatggatcagggttttttcccccagtgttctgtgggacagtctggtgtttcacaaaggccacatctcccttctcaaccagacacctgaaagcgcctgtgtagccgtagtatccctctttgttgttgggttcacacaggtttaggcctgagcccatacacagcttacagagactggagtctttcttagacccaggggcacaaccttcactgaaaaattcatcaaatctgcagtggttgatcttattgtagagcaggcccatggggatgttccagccagcggttctgccaactgccgtatggcaggacttcttgcctttcagattgtcccaggtgaggtcagaagctgatttcttcaccactgctatagcaaaataccctgcctctggtgtatcctcacaattatcgctcttattgtagttttctgccaagacaggcaccagaccacacttgcccgctatgtagacaaaccctccatccaagctcatggcatcagcttctccattcatgatcttggcgatgcagtcttcggtggtctctgctgatacacactctattttccctacactgttaacactccactcatcacacttgagcctctcgtggtggctcagcgcacaccacttcacaggcttgcattcatctgttggggcttctgggcatgtgccttcccgtagattccggatggcagtgacatactcatagcccaggtacatcttggcatccatcctgggggggacttttaaaaacccgtgggcagagtccttaaacagcaggtccttcccatgaggagagctgaatagttggaattcttttgatttgtctttgccaaaatgttcctgggcctggttgagaagctcccagatcaagtcctccttgccgcccatacttcgggccacgacggtatgagaagggacctgggccaagtggcagtccttgtattcatctaccggcttccgggtgttgtccaggcaaagcagctcatactggtccctgtcagccttgtttgccaagttctcaaatatagtcgagtgcttgacaaaggccacatccccagcaccatccttcagacacttgaaggctcccgagtagccgaagtattggttaagggtggagcagccacaccctggacacagttgacacagctgggggaagtccgtcccatccgcacaaggggcacagctgcccgagaagaaattggccactgctttctcaagaggtttacgtggctcaggtaagtcacagtaaagtaagcctatggggatgttccacccagcggacctgcctagacccgtgtggcaggacttcttgcctcgaagctggttcatctggaagccactatccttcttcaccacagcaacagcataatagaaagtctgtggatcctcttttgacccatagaactctgccaccacaggcttcaggttattgggagccaggtaagcatcatacaccaaacctgcatccagtgtcacagcatccgcttcgtttgcccaggacggcgcagaccagcagggctcccacggcgagcctcatcttccgggtgcggcgctgagcagcgagcacagtcggactcgcttctgt

SEQ ID NO: 11578 - RNA, 7417 nt, Homo sapiens
  source 1..7417: mol_type = other RNA
ctgaatagctgggactacaggtgggcaccagcactcctcgctaattttttttgtgtgtgtgtgttttgtttgcttgtttgtttgttgttgttttggttttttggggttttttttgtttttttttttttttttgcagagatggggttttgtcatgttgcctaggctggtctcaaactcctggactcaagcaatctgcccacctctgcctcccaaagtcctgggattacaggagtgagccactgcgcctagccctcctatctgctgctttgtatcctctgacctacatctctccaccctcctccacctcaggttttgttatctctgtatacctgtatttgagtgttttctttagattccccatgtgagtgaaatcgtgtaatatttttctttctgtatctgccttatttcacttaatatcctccagtttcatccatgttgtggcaaatggcaagatattctttttagggctgaataatattccattgtgtgtgtgtgtgtgtgtatacagtttctttatccattcattcttcaacaggcatttaggttgcttccctatattggctgcaatgctgcaatgaacgtgggatcacatttatctctacaaggtggctatctcattttatttgtgtatatcccctaaagagggattgttgggtcatatgtagccctattttcagtttatttagaaacctccatactgttttccacaatggctgtacattctcaccaacaatgcacaaaggttttctgttctcttcacccttatccacgtttatgattaatatcttttgactttttgataatagtcatcctattattatctagtgtctcataatggtttcaattcacatttcccttatgattagtgatgttgaacaccttttcatatccatcttggccatttttcttcttggagaaatgtcttttcaggtttttgcccatttttaactgggatcatttgttttcctgctattgagttgtatgagttctttatcaatttgttgtatcttattagatatatagtttgcaaatattttttccaatccataggttgccatttcattttgttgcttgttgtctttgctatgcagaagcttttcagcttgatgtagtcccatttatttatttttgcttttgtggcctgggcttttgatgtgatagccaaaaaatcattgctaaggccaaggttcaggagcttatcattacattttaacagctggaagagctcttccactctcatcagaatttttcttatctgtctcacttttgttttttagttgaggattagtatcattttgtcaagttaaaaaattgtatattgattaatttagggagaattgacatctttacaatactgagtcttcctatccaaagcaatatgtcttctttacattattttttactttgataagtgtggtttaaatgtagcttttattaatttactaaatgatacattttatttattcttgttaattattattgtcctaactcactattatttgtataaaagaaagttattttttattttaatatttcctttcactttactgaattttatcttaccacttttaccactttatttattattattattatttttattattttgagacagagttttgctcttgttgtctagactggagtgcaatggtgcgatctcggctcaccacaacttctgcctcccaggttcaagcaattctcccgcctcagcctcccgagtagctgggattacaggcatgcaccactacgcccggctaatttttattttaagtagagatggagtttctccatgttgtcaagctggtctcgaactcctgacctcaggtgatccgcccgacttggcctcccaaagtgctgagattacaggtgtgagccaccacgccctgcctattattattatttttattattttccagacagagtcttgctctgtcactaggctggagtgctctggtgcgaccttggctcactgcaacctctgcctcccaggatcaagcacttctcatgcttcagcctcctgagtagctgggactacaggtgtgtgccaccaaaccaggctaatttttgtatttttagaagagatggggtttcgccatgttggccaggctggtcttgaactcctgacctcaggtgatccacccacctcagcctcccaaaatgctgggattataggcatgaaccactgcgcctggccataatactttattattatttggttctcatggatttcctaggtgtataatcacttacaaataaaagtaattttggcatttctttaaatattataacttatttttcttgtataattggattggccacctgttctaaaacactgtaaaataagatagatagtaatcaatttttttcatgttcctaactttagtaggaatgcttctgtttcttcatcattaggtatgtattagcttttgtttacatgtatataaaattatggccaaataacatctgtctatcctattttagtaactaatttaataattaagaatggatgttgaatatttttgttttagcccagttgtctaagacttccaggaatatacctgtagtgtaataaaattaggtttattgatccattgcaatgagacagactgcgtcccaggggagccatggggtatctcaccaaacaaaggaaaaggcagagttataggatttggggtaagtttaggttaatattaaataaggcagatcgttgataggctcagaggaaagcagggctgtgtgtaaaacggtccatatcaggtctggactgcaaagtggacccagagtcctattttcttgaatactagacagttgagagaggtgtggaatgttgtgtccagataccccttatctgcacttctgtatttgagtataagatgaggctgtgttaggagtcaggaaaagaaaggagccaactgaagttatttagaaagcaaaatcaacagaacttggtgacgctggatgtagtgtgagggaaaatggcgaactgaaatttcacccctctatttatggcttatgtgattgggtagatgaccaggtcttcagctgatatggaatatactataacaacagttggtttagggaagcaagagagagaagaacaggatgatcacttcaatttttgatttgttgggtttctgactgctgcaagactcgagtatagacccacaggtaggtagtaggatgtataagtgcagggatactgctggaggctggggtcacagctatagatacagatgcctaggagtcatgagcatcactgaaggagggcctgcaaagtgagaggagcactgaccagatcaagagaaaaccccaggaagatttccctaaggtttccaggccagtaggatgagcccacagtgaagactacaaatgaacagagagaggtaggaatcaaagcagagacctgccatgtcagagaaactgaggaaaagagttccaaggaggagggagtggtcaactttatcaactgcaggaaatgggctcaggaatggaagacctgaattggtttaacagttggcaggtagacggtgacttttgccagggtacattcaggtaagttggtgaagcagaagaccaaattctgtatgttcagccaataataagtgagacagaaaagtcagcctccaccttacaggaagctgggctgagaagggcaggagacagggcagtaactgctgtggcatcaagctcagggaatgcttttcagcaaaaaagatgtcagtgtttcacttttttcagctagttagaatcaggacctcagcctgatggaattcatttaaaataccaaataaaggtaagtcttctgtagtctttctgtactcacttgagtacttgatctctgtaactcactctgcatcctccttcttgccccttccttagcatgacacacgcacgcgcacgtgcacacacacaccagtatacatttgattatattttaatgatcacgcagacccttttagaaaagatgtctccttgaactgtacccaggagatgtggccatggcacacacaaagctgtagggaaagaccagacgaatcttgagctgagaaggaagggctcagttgcataggtatttaggcagaatgcataaagaaatcctttgttgaaaatatttaggaaagaatggagtttttgaaatataaaatcaataataatttttattttttgttcagcacacatggcaacacagagctgtgaagacagacgtggttagcacaaaccacttgggccagtgaaaccagggcaaactcatggatcatctgcgttcccatcttcaccttggtggcagccctacctctgagattttaaggtctacggaaagtgcaggcttccaggagtgatgaggtggagcattttctcaggttaccaacagccttgacatattcttctcctaagtatttttcatatgtgtttctgtcatgaagtttggccaaacatactgtgtcatctctgaacagaaggtccttggtttccgaccggaacaaacaaaagttgcccgagcagtcagttacgttgcttccaaataggtgctgctgttgacgtaatatcttgtggacgcaagcttccttatctttccgtgtgaccacagcgtgattcggggctctggccaggtggcagttcgcatactcctccacaggtttcctggtaccatcaaggcacagcaactcatagtctttttcattcagattcttagcccatggatcagggttttttcccccagtgttctgtgggacagtctggtgtttcacaaaggccacatctcccttctcaaccagacacctgaaagcgcctgtgtagccgtagtatccctctttgttgttgggttcacacaggtttaggcctgagcccatacacagcttacagagactggagtctttcttagacccaggggcacaaccttcactgaaaaattcatcaaatctgcagtggttgatcttattgtagagcaggcccatggggatgttccagccagcggttctgccaactgccgtatggcaggacttcttgcctttcagattgtcccaggtgaggtcagaagctgatttcttcaccactgctatagcaaaataccctgcctctggtgtatcctcacaattatcgctcttattgtagttttctgccaagacaggcaccagaccacacttgcccgctatgtagacaaaccctccatccaagctcatggcatcagcttctccattcatgatcttggcgatgcagtcttcggtggtctctgctgatacacactctattttccctacactgttaacactccactcatcacacttgagcctctcgtggtggctcagcgcacaccacttcacaggcttgcattcatctgttggggcttctgggcatgtgccttcccgtagattccggatggcagtgacatactcatagcccaggtacatcttggcatccatcctgggggggacttttaaaaacccgtgggcagagtccttaaacagcaggtccttcccatgaggagagctgaatagttggaattcttttgatttgtctttgccaaaatgttcctgggcctggttgagaagctcccagatcaagtcctccttgccgcccatacttcgggccacgacggtatgagaagggacctgggccaagtggcagtccttgtattcatctaccggcttccgggtgttgtccaggcaaagcagctcatactggtccctgtcagccttgtttgccaagttctcaaatatagtcgagtgcttgacaaaggccacatccccagcaccatccttcagacacttgaaggctcccgagtagccgaagtattggttaagggtggagcagccacaccctggacacagttgacacagctgggggaagtccgtcccatccgcacaaggggcacagctgcccgagaagaaattggccactgctttctcaagaggtttacgtggctcaggtaagtcacagtaaagtaagcctatggggatgttccacccagcggacctgcctagacccgtgtggcaggacttcttgcctcgaagctggttcatctggaagccactatccttcttcaccacagcaacagcataatagaaagtctgtggatcctcttttgacccatagaactctgccaccacaggcttcaggttattgggagccaggtaagcatcatacaccaaacctgcatccagtgtcacagcatccgcttcgtttgccgcaatggccctgatgcaatcaaggtaggaggctttcttcacacaagcaacactgggaccatcggatggaatgacgcttttcatatggtcgcggaaactctggcacttagtggcctcatgctccgacactgcacaccatctcacagttttatcagggacagccagacacagcccagccaagtgtaagaagtgaggtgtctggtgtcccccctgtgattttaaaccaaggctctgatggattcttgacttgtccacagtcacacagaagaaagtggcaaaagtagaactagagttgtgactctgccgccatcattcttgcttctccctaggtgccctaaggtgccctaaatcatctgggtctgcaggagagtgccctgaaagccccactggagccgtagtatctctcctggctgttgtaagcccatatgtgggcaggattgcacctgccaccacacagagcacagagaggggaatccggattagacccaggggcacaactgcgactgaagaaatcatcacatttacaggacccggtttgattgtatattaagcccatggggatgttccagcttgcagaagtgccaactgcagtgtggcaggacttcttgcctcaaagagagttccaggtgacatcagcatctgatttcttaaccacagccatgacataatagccttttctctgtgttgtagatcaggtctctacaaattcaaacttggagaagttgggagtcaacatggcagatggaaggtccgtcttgtccttcttaggtgacctcagacacgtccttatcatctaggagcctaaatttttcttcagttaaatggtggcagtggaacccctcctggagtgactctttttggatcctgagtcgcggaaaaatactcatatcccaggtacagcttggcatctatcttaggtgggaccattaaaaacccatgggcagcatcagtaaacagcagatctgtctcatgaggagagccaaagagctgaaattctgacgacttgtcttttccaaaatgttctgtgatggctttaatgtactcaagggaagacgctctctccacgcaggtgacaaggggaccatctgctggaaacacttttttcatattgtctcggaaactggtgcacttcgtggcctcgtgatctgacatggcacaccatcttccagttttctcaggagcagccaggcacagccctccacgtttgacatttccgctcttctgctgcagct

SEQ ID NO: 11579 - RNA, 6449 nt, Homo sapiens
  source 1..6449: mol_type = other RNA
ctgaatagctgggactacaggtgggcaccagcactcctcgctaattttttttgtgtgtgtgtgttttgtttgcttgtttgtttgttgttgttttggttttttggggttttttttgtttttttttttttttttgcagagatggggttttgtcatgttgcctaggctggtctcaaactcctggactcaagcaatctgcccacctctgcctcccaaagtcctgggattacaggagtgagccactgcgcctagccctcctatctgctgctttgtatcctctgacctacatctctccaccctcctccacctcaggttttgttatctctgtatacctgtatttgagtgttttctttagattccccatgtgagtgaaatcgtgtaatatttttctttctgtatctgccttatttcacttaatatcctccagtttcatccatgttgtggcaaatggcaagatattctttttagggctgaataatattccattgtgtgtgtgtgtgtgtgtatacagtttctttatccattcattcttcaacaggcatttaggttgcttccctatattggctgcaatgctgcaatgaacgtgggatcacatttatctctacaaggtggctatctcattttatttgtgtatatcccctaaagagggattgttgggtcatatgtagccctattttcagtttatttagaaacctccatactgttttccacaatggctgtacattctcaccaacaatgcacaaaggttttctgttctcttcacccttatccacgtttatgattaatatcttttgactttttgataatagtcatcctattattatctagtgtctcataatggtttcaattcacatttcccttatgattagtgatgttgaacaccttttcatatccatcttggccatttttcttcttggagaaatgtcttttcaggtttttgcccatttttaactgggatcatttgttttcctgctattgagttgtatgagttctttatcaatttgttgtatcttattagatatatagtttgcaaatattttttccaatccataggttgccatttcattttgttgcttgttgtctttgctatgcagaagcttttcagcttgatgtagtcccatttatttatttttgcttttgtggcctgggcttttgatgtgatagccaaaaaatcattgctaaggccaaggttcaggagcttatcattacattttaacagctggaagagctcttccactctcatcagaatttttcttatctgtctcacttttgttttttagttgaggattagtatcattttgtcaagttaaaaaattgtatattgattaatttagggagaattgacatctttacaatactgagtcttcctatccaaagcaatatgtcttctttacattattttttactttgataagtgtggtttaaatgtagcttttattaatttactaaatgatacattttatttattcttgttaattattattgtcctaactcactattatttgtataaaagaaagttattttttattttaatatttcctttcactttactgaattttatcttaccacttttaccactttatttattattattattatttttattattttgagacagagttttgctcttgttgtctagactggagtgcaatggtgcgatctcggctcaccacaacttctgcctcccaggttcaagcaattctcccgcctcagcctcccgagtagctgggattacaggcatgcaccactacgcccggctaatttttattttaagtagagatggagtttctccatgttgtcaagctggtctcgaactcctgacctcaggtgatccgcccgacttggcctcccaaagtgctgagattacaggtgtgagccaccacgccctgcctattattattatttttattattttccagacagagtcttgctctgtcactaggctggagtgctctggtgcgaccttggctcactgcaacctctgcctcccaggatcaagcacttctcatgcttcagcctcctgagtagctgggactacaggtgtgtgccaccaaaccaggctaatttttgtatttttagaagagatggggtttcgccatgttggccaggctggtcttgaactcctgacctcaggtgatccacccacctcagcctcccaaaatgctgggattataggcatgaaccactgcgcctggccataatactttattattatttggttctcatggatttcctaggtgtataatcacttacaaataaaagtaattttggcatttctttaaatattataacttatttttcttgtataattggattggccacctgttctaaaacactgtaaaataagatagatagtaatcaatttttttcatgttcctaactttagtaggaatgcttctgtttcttcatcattaggtatgtattagcttttgtttacatgtatataaaattatggccaaataacatctgtctatcctattttagtaactaatttaataattaagaatggatgttgaatatttttgttttagcccagttgtctaagacttccaggaatatacctgtagtgtaataaaattaggtttattgatccattgcaatgagacagactgcgtcccaggggagccatggggtatctcaccaaacaaaggaaaaggcagagttataggatttggggtaagtttaggttaatattaaataaggcagatcgttgataggctcagaggaaagcagggctgtgtgtaaaacggtccatatcaggtctggactgcaaagtggacccagagtcctattttcttgaatactagacagttgagagaggtgtggaatgttgtgtccagataccccttatctgcacttctgtatttgagtataagatgaggctgtgttaggagtcaggaaaagaaaggagccaactgaagttatttagaaagcaaaatcaacagaacttggtgacgctggatgtagtgtgagggaaaatggcgaactgaaatttcacccctctatttatggcttatgtgattgggtagatgaccaggtcttcagctgatatggaatatactataacaacagttggtttagggaagcaagagagagaagaacaggatgatcacttcaatttttgatttgttgggtttctgactgctgcaagactcgagtatagacccacaggtaggtagtaggatgtataagtgcagggatactgctggaggctggggtcacagctatagatacagatgcctaggagtcatgagcatcactgaaggagggcctgcaaagtgagaggagcactgaccagatcaagagaaaaccccaggaagatttccctaaggtttccaggccagtaggatgagcccacagtgaagactacaaatgaacagagagaggtaggaatcaaagcagagacctgccatgtcagagaaactgaggaaaagagttccaaggaggagggagtggtcaactttatcaactgcaggaaatgggctcaggaatggaagacctgaattggtttaacagttggcaggtagacggtgacttttgccagggtacattcaggtaagttggtgaagcagaagaccaaattctgtatgttcagccaataataagtgagacagaaaagtcagcctccaccttacaggaagctgggctgagaagggcaggagacagggcagtaactgctgtggcatcaagctcagggaatgcttttcagcaaaaaagatgtcagtgtttcacttttttcagctagttagaatcaggacctcagcctgatggaattcatttaaaataccaaataaaggtaagtcttctgtagtctttctgtactcacttgagtacttgatctctgtaactcactctgcatcctccttcttgccccttccttagcatgacacacgcacgcgcacgtgcacacacacaccagtatacatttgattatattttaatgatcacgcagacccttttagaaaagatgtctccttgaactgtacccaggagatgtggccatggcacacacaaagctgtagggaaagaccagacgaatcttgagctgagaaggaagggctcagttgcataggtatttaggcagaatgcataaagaaatcctttgttgaaaatatttaggaaagaatggagtttttgaaatataaaatcaataataatttttattttttgttcagcacacatggcaacacagagctgtgaagacagacgtggttagcacaaaccacttgggccagtgaaaccagggcaaactcatggatcatctgcgttcccatcttcaccttggtggcagccctacctctgagattttaaggtctacggaaagtgcaggcttccaggagtgatgaggtggagcattttctcaggttaccaacagccttgacatattcttctcctaagtatttttcatatgtgtttctgtcatgaagtttggccaaacatactgtgtcatctctgaacagaaggtccttggtttccgaccggaacaaacaaaagttgcccgagcagtcagttacgttgcttccaaataggtgctgctgttgacgtaatatcttgtggacgcaagcttccttatctttccgtgtgaccacagcgtgattcggggctctggccaggtggcagttcgcatactcctccacaggtttcctggtaccatcaaggcacagcaactcatagtctttttcattcagattcttagcccatggatcagggttttttcccccagtgttctgtgggacagtctggtgtttcacaaaggccacatctcccttctcaaccagacacctgaaagcgcctgtgtagccgtagtatccctctttgttgttgggttcacacaggtttaggcctgagcccatacacagcttacagagactggagtctttcttagacccaggggcacaaccttcactgaaaaattcatcaaatctgcagtggttgatcttattgtagagcaggcccatggggatgttccagccagcggttctgccaactgccgtatggcaggacttcttgcctttcagattgtcccaggtgaggtcagaagctgatttcttcaccactgctatagcaaaataccctgcctctggtgtatcctcacaattatcgctcttattgtagttttctgccaagacaggcaccagaccacacttgcccgctatgtagacaaaccctccatccaagctcatggcatcagcttctccattcatgatcttggcgatgcagtcttcggtggtctctgctgatacacactctattttccctacactgttaacactccactcatcacacttgagcctctcgtggtggctcagcgcacaccacttcacaggcttgcattcatctgttggggcttctgggcatgtgccttcccgtagattccggatggcagtgacatactcatagcccaggtacatcttggcatccatcctgggggggacttttaaaaacccgtgggcagagtccttaaacagcaggtccttcccatgaggagagctgaatagttggaattcttttgatttgtctttgccaaaatgttcctgggcctggttgagaagctcccagatcaagtcctccttgccgcccatacttcgggccacgacggtatgagaagggacctgggccaagtggcagtccttgtattcatctaccggcttccgggtgttgtccaggcaaagcagctcatactggtccctgtcagccttgtttgccaagttctcaaatatagtcgagtgcttgacaaaggccacatccccagcaccatccttcagacacttgaaggctcccgagtagccgaagtattggttaagggtggagcagccacaccctggacacagttgacacagctgggggaagtccgtcccatccgcacaaggggcacagctgcccgagaagaaattggccactgctttctcaagaggtttacgtggctcaggtaagtcacagtaaagtaagcctatggggatgttccacccagcggacctgcctagacccgtgtggcaggacttcttgcctcgaagctggttcatctggaagccactatccttcttcaccacagcaacagcataatagaaagtctgtggatcctcttttgacccatagaactctgccaccacaggcttcaggttattgggagccaggtaagcatcatacaccaaacctgcatccagtgtcacagcatccgcttcgtttgccgcaatggccctgatgcaatcaaggtaggaggctttcttcacacaagcaacactgggaccatcggatggaatgacgcttttcatatggtcgcggaaactctggcacttagtggcctcatgctccgacactgcacaccatctcacagttttatcagggacagccagacacagccccaggacggcgcagaccagcagggctcccacggcgagcctcatcttccgggtgcggcgctgagcagcgagcacagtcggactcgcttctgt

SEQ ID NO: 11580 - RNA, 2922 nt, Homo sapiens
  source 1..2922: mol_type = other RNA
ctgaatagctgggactacaggtgggtgtcactatgcccagctaattaaaaacttttttttttttttcagtagagatggggtcttgatatgttgcccaggctggtctccaactcctcgcctcaagtgatactcctgactcagcttcccaaagtgctgggattataggcatgagccactgtttcaggccataattttcttcattctttacaacaatcctgtgagaggaaggctttagggctgccctttcaagtcttaagagtccaagtagcttactggaggctacctggctggtctgacagttgaattcgtcctgtgtgactttaaaacgaatgctcttaactccatcctttgtccccattgtggctccattgcttgccacacagctggcttcttgctggataaaggctttgcccatgggacagacgctgatccaaaggctggcagattcctcttctccctgccctgtgagaaacagcttcgggaaaccagagagagttgcaaaccctagatcaatgtctcttatcagctctcagcttcaggagcctactcagcctaaaacaatcaggtgctggcctcatccacccaggtgaggaactggatggagcccgacttctggtttcttctttgctgttctgtgcagtcaaaactctgggatccagggaacagcagttaatgactctttggggcccagaattggagctccttggtggcatttgcatcctctttcaccagatgacttaggcagcgcttcctgacctttgtcatgctgtagttctcatagaaaatgaaactttttacagccactgcagtaaagaaccaaggctgcctctggcccctgaggccaatattggcccaactggaatccactagagggctgcacgttggctaggaagctctgactgatggcatgggcttccctgccagggctcatggtgcataggcgaaggaagaggggcgtgatctctctcagacgctgagaattatttgggttgctcataattacttggcctagggtcacccagaaagttactgaagacaagagatggtatccaagatccctagcggcagggactgaatctcactcatctttgtctccgcagtgcctagcactgtgcccggccccaagcagtactcagtaagaacttgtggacccaattcaagtgtcctagttggtgattctgatggatgattgattggagtaggagtctaatccactttgtccttcccacctggtccttttacttctatccccatgacccccgactctcctaaccctcacagcacaggatggggggcctcttgaccaccagaattccattttgcggcgggcgcagcgttcccggtctaggccttagctctctcatttcaatgagggcaacatctacggagaactcccgtgcattcttggtggaaggaaacaaacttgagacttggattctgctgtcaggcagcagacagtttaatgagaagtgtggaatgaggctcagtggaaatatcacatataagacatgatgcacgtccagaggaggtacaagcaggaagttccagttggtaaggaccaccgcaggcttggaagagagagatgttcagggcgaggggaaggccctatagaagagggggcgtgtgaccaagaccttgaggaggggctgaggccattagaaggggagaggagaggaagggtggggggtgttccatgtaaggtgctgtgatcatttcccctcctctttatgttaactttgttgttttcatctctgaaactagaacccgttagcactgtccacccgggactgtggtgcctggcctaggcctaggcctgcccatcgcttgttgtctgaacaaggaaccctggagggagaggtggaaggcagaaggaagccctggacatacactggatcccacatagacatttgggcacctaccagaaggtgagctccaggaaggcttgggtctgtgaccttcactgccctgcctcagcatctagcccctggctctgggggagctcaacaatacttgttgaagactgaatgtggcagacactctttcaggacccgagagtactggcaggaacaggaaaggggctaactccaggtatgaaatccaggagaaaggaggagcctgcgggagtccaaggaaggggtgtcagggggcaacatggctccaaggcagggggcagggggcagattaatcagacctaaactccagtggtaacagctccgttaattgagtggtaatgatccttggtacttctcatcttcaaagccaggaacaaactgtaatgaatactcttgccacccgggggcagggtgcggagggtggtggggagaatcttatgctactggtactcagttggggaaactgaggcactggcagaaaaatggtccttaggagagcgaatgtgaagcccagcagagcttggaatcttcaggggtgtcttgaacacaccagagagtggccccttcaaaatccaggcccctggggagcccaggccatgagtagggaggaaggtagtgctggaaccccttgcaggcctgactaaaagttgcagtggagaagtcgggtctgcaggaggcttggctggtgtgcgccgggtttcccagggtgggtcggggtgcccggggcgtagaccctgcggccctgcagcacgcagccacgctctccgcgttccaggggcggcgcgggagtggcgcgcggctgggagggcacccgggcgtccttcgcgcccagcgctgcatactcactgtgactcaccggctgctccgagatgcctcccggttttctcatcgcagtctggctgctctgagccccgagggcgtttttcattagggtgattaccctgccgtcattaaaagccggtaaatagcacccagggacgaggccgcgcggccgcgtctgaaccgcagcccgggttcacaggcgcccccc

SEQ ID NO: 11581 - RNA, 418 nt, Homo sapiens
  source 1..418: mol_type = other RNA
ctgaatagctgggactacaggtgtacacaaccatgcccagctaagttaaaatttttttttttgtaaagatggaatcacactatgttgcccaggtttgtctctgactcctggcctcaagcgatcctcctgtctcagcctcccaaagtgttgggattactagcagaagccattgtgtccagtggttcatttttttttttgtatgagcgaaagacaatcaaaaagtgtccagcacctgaacttcatgccttcaagaggtggattccggcttctttacagcgcaatcactagcaggtcatttccgtctagcttgcagatttcccattactgacacaaacgctccctcagggcgtccccgtctggactacaggagaaagtttgggaggcaggttcaacttttcaacttggcggggaattcctc

SEQ ID NO: 11582 - RNA, 9374 nt, Homo sapiens
  source 1..9374: mol_type = other RNA
ctgaatagctgggactacaggtgtacacaatcacacccggctttttcatttttgtattttttttgtagagatggggtttagacatattgcccaggctgctctcgaacttctaggctcaaatgatacctctggctccgcctctcaaagtgttgggattacaggcgtgaaccactgtgcctggccaccagtacttcttacgtaatacttgctgtagagaatctctttctactcaagggaagatgctaaaactggtgttcatgcaattaaagatgacatgaacatagacattcagaagcaacactgtcatcttgagagccacatcattccagtgtcacatttctagaaccaaaatatgagtccgtgtgggctgctataacgaaatgccttagtctggtttataaagtttataagcaagaactgtgaacaataaatttgttactataaaaaaacttcttgcttatagttctggaggctgggaagccaatcagtgtgctggcatatttggtgtttgtggagggtctgctttctggttcatgaacagtggcttcttgctttgtcctcacgtggtggttggggcaagtcggctgtctggggccccttttacgagggcattaatcccattcatgaaggctccactctcatgacctaatcacctcccaaaggccccacatcctgtcacactgatgatcagatttcaacatatgaattttgtggccagggggacacaaacattcagaccacagcacaaaggttagggacaacttcttaagtaattgtgtgatgcagcaaacacatgcataaaaaaaaaatcagaaataatgaaagtaaacaagggcaacattatcttaggtttgtctctgaaaacattcaggacgcatcactgagtagtgcacagttttagtctgtgagcacgcttcagtgaaattatatcaccactgaccacaaaatcttcaaatcccagagttgaagaaaacacttttagtcagttactaatggagaaaaaataaatataatttggttgcaacctcgtaagttgcttcctgttctataatttaaaataactatcttaaattagtagtttaatgagtgagcaatttagcacctgatactgctgagaaattaatgactctgcactgcattaaatttaaaaaatgagctttaataaaattacagtaaattttaaatatgatttcctacttattcatggattctagaagcttattttatgatggtaatcttcagtttaggtcttggtgaaataatttcaagccttagccattggcatttggtcagtatgtgtatgtagtgtactatgaatgtgactcagccatatactacaactgagacaaggcaatcaccaaggtcacatacctagtacaaccccatctccaggccacccatttaccaagtttgtggccctcatgtaagaggtgaccaagatgcacctgcaccaagagcaccaagaggattgtctcaatccttaagagaaagaagaaggtaagggctggggatgaggggtgcacttaaaccagaaatgagacatggccctctgtggctaggatcctaacttcagattgctaatttatcccattttacttaggcccaaaatgacaggctgaatacttttattggaaatgaaacattccagagttagacatgtttactctggacagtcaaggacagcgatgtgtagggaaagtttggttcatgcaaaaatgaatgaaattttaatacacttaaagttacttctcactctgaaaataataccaaagtagagtcaataaatattaaatttccttccaattccacaggaccaattaacgaaaaacataatttttgtactacagaataaaaattttaaaatctcaaatattttttcccaaaggcagaggtcatggcaaatcttcggagaaagagagcattttgtctatttgaaaattcaggctcaggccttcaaatgaaatgatggttcatgctgtcatttcaagtgactacaaagaagaaatgaaagaaagatgtaaggagtcactactttaaggattattcacaaaagtcttaggaataatacaggtgaagtctcagaaaggcaagtccttataacagaatgggcatggatcatgtactaatcagtaggttacaattcactaccttacagaatttgggcttcatttagaaggcctgatggtgtacaacagactttacattttcacattaatgcaagagcctatcagtgaattcatgttcatttcctttattaaccagcctacattagatttaatttgtgaactctgctatataagcaaagaagaaagcaagcaagcacatgatcagaagagaaaaagagctagatagcccataaggctcctagagggaacttgagcactcctcatgacagagacacagatgacacacttctaacttctcaaacatgccaagtttgtgcttgccttctgggtctttgcctttattattcctcccctcagcccacttgtggttccttctaatccttcacgtaccagctcaaatgttttctcttacacagatgacactttcttctaacactttcttctaaagtagtttcaccactgcctccccacattatcctgtatactttccagtcaccatcagaagtttgctcatggctgggcgtggtggctcatgcctgtaatcccagcactttgggaggctgaggtgggtggatcacctgaggtcaggagttcgagaccagcctggccaacatggtaaaaccccatctctactaaaaataccaaaaattaactgggcgtagtggcgggcgcctgtaatctcagctactcaggaggctgagatgggagaattgcttgaacccgggaggcggaggttacagtgagccgagatcaggccattgcccatttcctgggcaacaagagtgaaactccgtctcaagaagctggtttgtttattgtataccatcactaaaatccaagctcaactataaaagggtcacctttttgctcaccattacatgcaggcatctaaaaatacttgcttaaataagtgaatgaaaaagcagcagaaaggaagcaattttacttctgaaaaattattctaaaaaaataacaggtcaactttaccaagatatagatatacatttataataatgaaaagaaattgtctaaaaatctatccaatctatccaaatgagtattttctttttttttttgagacagtctcattctgtcatccaggctggagtgcagtggtgtgatctcagctcacagcaacctcctccttccgggttcaaacaattcttccacctcagcctcccatgtagccaggatgataggtgtgcaccatcatacctgggtaatttttgtatttttagtagtgtcagggttttgccatgttggccaggctggtgttgaactcctgacctcaagtgatccatccgccttggcctcccaaagtgctgaaataggcgtgtgccactacgcctggccatgaaattgttaaattagttatggtatctataaaggtattaaaaagaatattaaagacattttttctactactgagtgaaataagcagattacaggccagtatgtatggtatgatcacattaatgtagagaaaacaacaaaaatagtatgttgttgtgtaagtttagaagaaaataaaacaaacaagatattaaaaatagtagttgtcaatttacttttaactttttcctccaagttacctttgccacgcctcctcccccgcctttgctgtatgagaaaaaatttggacaaaaacttcaggtgactatgaggagcgatttttttctcagcctagcagtggtagagaatgccttattttcatccttatgccctttcacatatgattccaaagtgtacatatccaaattcctactttacctctccagagatcactgccaacaaagttattacctctctaagatcctaatatttcaaaacaaacggcattaaatcttagttttgactgctcactgtgtaaatcagactatttcaggtctgaactatgccattttaaaatttccctttttaaaaaatctttatggaacaagtacaatttttcgacagatagtgacaactactccctactttaaatataggctggacaaatcatacacaaaataatagcataatctcatagtacttcaatttcattctactctctatgtttgaagaaagaaaaacattataactgagttcacagcagccttcttttatcttaacacaagttaccagtgtatacataagaagctgtgaacagaagctctttatgatattcatatacaaagctgctgagaaacagcctcaacaatgccaatcaaagagcaaaacattgggttagttttcaaactaaatgagctgctttgccctccatgccaactattaagcaataggcccttttatgtctttcccattcattactgactaatgcagcagttctcaacattctcactagtcccatgatcactcaattttttttccctattcttttaaataactctatttggttacagataaaatgagcaagttgacagcatacaagttttctttaagttcttaatttttaagaagtattgtgtaattttattttctaattttggtatttttttcaataaaatgttttttaaaacatttaaacaaatcatataatagctgacctggtatcgaatgctgtacttagacattcctaaaccattattttttatatttcaaactaagtttaaacaaaaactttattattattgaacgaatatccaaggatcttaaagaaatcaatcgaagtgtgatacagtctagtgtttattttatgttatggcaggtacacttgaatttcaaaaatttaaaacatatataaaaagtggttagggactaacatttgtatcaacagttgataaatgtctaagattgtttattatacagcagggtacaatggtagtgctaatgccaacagggcaccatggaagttagtctaaaaattatcgctaggctttatacaagcaacaacatatgctgctgctcttagaattttgggaaatgatctgcttctaatactaagcagttctttaacatttttaaatgttatacagtgttacagtatttagtttggcaaatgtttcaaaataaagtagaaatgtattcataacatcacagaaatgcacatccaatgttgttttcaataagaaccataggtacagatcagaactcttccctatatgaaataatttacacacagatgaatactataatatcactatctaaaataatcactaaatacagttctttttcagaaataaacaagcaaagatttttttcattatcaaatatcaaaaacatgttgataatgtatgtttttcaaataaatgatactttaaaattataggaataatctcagtgaattcagtgaatgtgcaacctaaatcaaccaagtatactgtagtacaaccatattaagaaaccaatgatcagaaaatacaaccgtatgaaagaaatttataatccacaaaactttttcaggtcttaaggtaaaatagttccacagtctacaggtaaaaccaaggcaacaaaaatgcgtgcttatcttgattaagtaggtaattttatgcagaagatgtaacactttgtttgtagacagcatggtatgcatttctcagcaagacataaggaaaacaagattccaaaagatccattgtaaggaatggagattcttgtacaatcatatctagcagtaaataaacagattctctatttcttgttgtagttttatctgtctcctggccaattttcagtagactggaggatgcaagcgccagaaattctttaagacggtcttcaatgcttcctttgtgaattgtaaacaaagctgcagcaatctggttgatggctttggccaagcaatgtatgttgttgcaatgcccttctatagcagggctgtactgagacatcacattactggccagtgttggcaaagaaactgccacaaacaccatgagaaggcaggcaattttatactcttcttctggactaatgttttccgatttttgtgaagaaagagctacgaccaatgcaggatcaatctcacaaggtaatccggcagctgatgataactcatacacattcattgcaaccttcatatcagtttcccttggaatgtgatccttaaaatcttcaattgaacttacaagaaaaggaatgtggtaggataagacatctctaagtgcttcttgtgccaatgatcggaaggataaaattacaccaattattgtcatcctcttcaagacactgtcaacagatgataatcttttaaacagtgcagccatctggtctggtttgtcaaagctggtcctcatttgtgttaacacatcaacattctccaccacaagtttcttaagttcagcaacttgtgatgaaatatgccacataaggctttcacttagaaacttcataccatatgggcctagtagttctgataatgacctcatttctgatatgtcagaatattcctctgcattgaatgttaattcattttctgtaggtaagttcacaaacgctttcattgcaggaaaatatgctatatggccattgctgacttgtcgtaacaaagtttccaaataccaatttgtgtatagacttgtaatggttggctctccatgactgtctaaatgttgtgtttgttgaagaagcacattattaaatactcttgtaatatcaatctgcacatagttttctattgactggagtacggtcatgtatgctcttacacttgttagaagttctgaaggttttgcaatttcctgtgtggcttgattatacatagtcatcccaacaattgacttggtaaagcgtatttccagatgagaagtcaaatattctcgtggggtaaaggtatgttcccataccaccatgtttggtacataatttatagagaagcataactcagaaagtgcagtgtgcaatttatcaaggttggtcacaaccagcctgtttttcctcatgctctcaacacctggtttctccctttcaggttcccctttcttaccagtctgcttttttgatttcttattcactgcttgactgatagttttggcacaatgcttgggtagcaactggtcactaagggtacactgttctgtgcaaatatcagtgatgagatttcgagcttgtttggccatttcatctaggaacatattacataaggaaagactgcgatctccaatatgatgtcgctcttctggacatagttcatgcgtgcaactcataaaatgagtgcaaagtagtggaaatgcaattgagtatcttgattgagagggtaactccaaacactgttgaaacatcttctcaaaagcacgactataaaaacaaaatatggagagatctgatgtttccaccaacatttccaccaaggaatctaccatttttgtatgaaaaattattgtattcatcatctttccaagttctctgtgatctgcaaggccaagtgaagcctttgagacactagtatatgcctgtaacctaaaccaatctaatctcattcctctgaaatcaaatacttccccatcttcaacttgttttacacttagggaagtcatagtgttaacaaaagaggacatgatgattgattcatcttcagggcaaacagaaagattctgcacgagttcattgaggacaacagcatcaaagccagaaaggtactgcacgtaatacctctgcattacaggtccgtatttcctcacatgtgctctaagttcttccatgtaaaatattaattcagcaatgtgcttatctataaagtcgtctgcactcttctttggcatgttatctgcatgacgaagtagccagatgatttcatcacgggcaaaggataatgccataaaaacaaaaagtgccttgggacctagcaatccaggttgatcagagaggacagtagccaattccttcagtgcagatcttaaaaacttgcgtctttctctgtgcattgaaccagcatgtgacacggctgcctccttgcattctcttatgtcattaatacgtttattatagcctcgtatgtttacaaataagtcttctgcagctttgtgaatgtggaaaacttcatcccgaaagagagagaggcaagagctactttgaagagctagtttccaaaggttcagtgctgtagcgtcagtatttaggatcccatggcacaaaataaagccaaagataatccacttttccattgcatccaaagagaggtattcacaaggcatagtgtcggactgtgctggattaagcattgtactaggtgcactgatgaggctcaataactgggcatttctccactggtcagctgaaagattccttcgaggatataccatttgaagagaaattagtgcatctgaaagagacttgctatggggtacaaattcttccatcatcttctttaaagggttttcataatccacaatcatctggccaaggcgtgggtattctctgtcacttgctccatgagtcatttcatgggcatagttgtataatccaatgattgccttcctttcttcaattcgagacagcagtatcattagtgttgtataggttataattaaatctaagtagttctttgttaaatcaaagtttacagtaatatcaaagaagacttggcaaacgtcaatagtattcagcaattcacaaacatggtccttaaattccataacatctacaaatgtgaagtaatataatgccagatttttcagaatctctgatttttctttctgtagttgtgcaagctgttgattgttgttgcgggtttctacagcagggaattttctgactatgaatttcacagcagattccaggtttttgtcgataagataggatggttttgccttggggtctccacatgccttccaaacttgtccttgcttcttgatgttgtagaggcgggtgagcatgccgacgccccggtcgttgaggatggtgagcttctccgccagcttctgctgactgggctgcagcactgagcgcgacatggtggtgctggtgccgccgccgccgccggccgcctcgcgcccagtcacgggcccgcggccttcgcagcagcctctctcgggcctcctcccctcccgcccgcgacctccgccttaggagagcgcgcccatggccctcgcgccccaatcccgcgccggcgacagagcgagccgcggcggactcctcggagccccttctcccgcagcagcccgcgccccggcagcctcctgccttccgcccgccgcccttccgcccccacccccggcgctctccgccccagcccccaacgagccgccttccccggctgctccactaggtgtggcggcggcggcggcggcggcggcgtctccggcggctgag

SEQ ID NO: 11583 - RNA, 9356 nt, Homo sapiens
  source 1..9356: mol_type = other RNA
ctgaatagctgggactacaggtgtacacaatcacacccggctttttcatttttgtattttttttgtagagatggggtttagacatattgcccaggctgctctcgaacttctaggctcaaatgatacctctggctccgcctctcaaagtgttgggattacaggcgtgaaccactgtgcctggccaccagtacttcttacgtaatacttgctgtagagaatctctttctactcaagggaagatgctaaaactggtgttcatgcaattaaagatgacatgaacatagacattcagaagcaacactgtcatcttgagagccacatcattccagtgtcacatttctagaaccaaaatatgagtccgtgtgggctgctataacgaaatgccttagtctggtttataaagtttataagcaagaactgtgaacaataaatttgttactataaaaaaacttcttgcttatagttctggaggctgggaagccaatcagtgtgctggcatatttggtgtttgtggagggtctgctttctggttcatgaacagtggcttcttgctttgtcctcacgtggtggttggggcaagtcggctgtctggggccccttttacgagggcattaatcccattcatgaaggctccactctcatgacctaatcacctcccaaaggccccacatcctgtcacactgatgatcagatttcaacatatgaattttgtggccagggggacacaaacattcagaccacagcacaaaggttagggacaacttcttaagtaattgtgtgatgcagcaaacacatgcataaaaaaaaaatcagaaataatgaaagtaaacaagggcaacattatcttaggtttgtctctgaaaacattcaggacgcatcactgagtagtgcacagttttagtctgtgagcacgcttcagtgaaattatatcaccactgaccacaaaatcttcaaatcccagagttgaagaaaacacttttagtcagttactaatggagaaaaaataaatataatttggttgcaacctcgtaagttgcttcctgttctataatttaaaataactatcttaaattagtagtttaatgagtgagcaatttagcacctgatactgctgagaaattaatgactctgcactgcattaaatttaaaaaatgagctttaataaaattacagtaaattttaaatatgatttcctacttattcatggattctagaagcttattttatgatggtaatcttcagtttaggtcttggtgaaataatttcaagccttagccattggcatttggtcagtatgtgtatgtagtgtactatgaatgtgactcagccatatactacaactgagacaaggcaatcaccaaggtcacatacctagtacaaccccatctccaggccacccatttaccaagtttgtggccctcatgtaagaggtgaccaagatgcacctgcaccaagagcaccaagaggattgtctcaatccttaagagaaagaagaaggtaagggctggggatgaggggtgcacttaaaccagaaatgagacatggccctctgtggctaggatcctaacttcagattgctaatttatcccattttacttaggcccaaaatgacaggctgaatacttttattggaaatgaaacattccagagttagacatgtttactctggacagtcaaggacagcgatgtgtagggaaagtttggttcatgcaaaaatgaatgaaattttaatacacttaaagttacttctcactctgaaaataataccaaagtagagtcaataaatattaaatttccttccaattccacaggaccaattaacgaaaaacataatttttgtactacagaataaaaattttaaaatctcaaatattttttcccaaaggcagaggtcatggcaaatcttcggagaaagagagcattttgtctatttgaaaattcaggctcaggccttcaaatgaaatgatggttcatgctgtcatttcaagtgactacaaagaagaaatgaaagaaagatgtaaggagtcactactttaaggattattcacaaaagtcttaggaataatacaggtgaagtctcagaaaggcaagtccttataacagaatgggcatggatcatgtactaatcagtaggttacaattcactaccttacagaatttgggcttcatttagaaggcctgatggtgtacaacagactttacattttcacattaatgcaagagcctatcagtgaattcatgttcatttcctttattaaccagcctacattagatttaatttgtgaactctgctatataagcaaagaagaaagcaagcaagcacatgatcagaagagaaaaagagctagatagcccataaggctcctagagggaacttgagcactcctcatgacagagacacagatgacacacttctaacttctcaaacatgccaagtttgtgcttgccttctgggtctttgcctttattattcctcccctcagcccacttgtggttccttctaatccttcacgtaccagctcaaatgttttctcttacacagatgacactttcttctaacactttcttctaaagtagtttcaccactgcctccccacattatcctgtatactttccagtcaccatcagaagtttgctcatggctgggcgtggtggctcatgcctgtaatcccagcactttgggaggctgaggtgggtggatcacctgaggtcaggagttcgagaccagcctggccaacatggtaaaaccccatctctactaaaaataccaaaaattaactgggcgtagtggcgggcgcctgtaatctcagctactcaggaggctgagatgggagaattgcttgaacccgggaggcggaggttacagtgagccgagatcaggccattgcccatttcctgggcaacaagagtgaaactccgtctcaagaagctggtttgtttattgtataccatcactaaaatccaagctcaactataaaagggtcacctttttgctcaccattacatgcaggcatctaaaaatacttgcttaaataagtgaatgaaaaagcagcagaaaggaagcaattttacttctgaaaaattattctaaaaaaataacaggtcaactttaccaagatatagatatacatttataataatgaaaagaaattgtctaaaaatctatccaatctatccaaatgagtattttctttttttttttgagacagtctcattctgtcatccaggctggagtgcagtggtgtgatctcagctcacagcaacctcctccttccgggttcaaacaattcttccacctcagcctcccatgtagccaggatgataggtgtgcaccatcatacctgggtaatttttgtatttttagtagtgtcagggttttgccatgttggccaggctggtgttgaactcctgacctcaagtgatccatccgccttggcctcccaaagtgctgaaataggcgtgtgccactacgcctggccatgaaattgttaaattagttatggtatctataaaggtattaaaaagaatattaaagacattttttctactactgagtgaaataagcagattacaggccagtatgtatggtatgatcacattaatgtagagaaaacaacaaaaatagtatgttgttgtgtaagtttagaagaaaataaaacaaacaagatattaaaaatagtagttgtcaatttacttttaactttttcctccaagttacctttgccacgcctcctcccccgcctttgctgtatgagaaaaaatttggacaaaaacttcaggtgactatgaggagcgatttttttctcagcctagcagtggtagagaatgccttattttcatccttatgccctttcacatatgattccaaagtgtacatatccaaattcctactttacctctccagagatcactgccaacaaagttattacctctctaagatcctaatatttcaaaacaaacggcattaaatcttagttttgactgctcactgtgtaaatcagactatttcaggtctgaactatgccattttaaaatttccctttttaaaaaatctttatggaacaagtacaatttttcgacagatagtgacaactactccctactttaaatataggctggacaaatcatacacaaaataatagcataatctcatagtacttcaatttcattctactctctatgtttgaagaaagaaaaacattataactgagttcacagcagccttcttttatcttaacacaagttaccagtgtatacataagaagctgtgaacagaagctctttatgatattcatatacaaagctgctgagaaacagcctcaacaatgccaatcaaagagcaaaacattgggttagttttcaaactaaatgagctgctttgccctccatgccaactattaagcaataggcccttttatgtctttcccattcattactgactaatgcagcagttctcaacattctcactagtcccatgatcactcaattttttttccctattcttttaaataactctatttggttacagataaaatgagcaagttgacagcatacaagttttctttaagttcttaatttttaagaagtattgtgtaattttattttctaattttggtatttttttcaataaaatgttttttaaaacatttaaacaaatcatataatagctgacctggtatcgaatgctgtacttagacattcctaaaccattattttttatatttcaaactaagtttaaacaaaaactttattattattgaacgaatatccaaggatcttaaagaaatcaatcgaagtgtgatacagtctagtgtttattttatgttatggcaggtacacttgaatttcaaaaatttaaaacatatataaaaagtggttagggactaacatttgtatcaacagttgataaatgtctaagattgtttattatacagcagggtacaatggtagtgctaatgccaacagggcaccatggaagttagtctaaaaattatcgctaggctttatacaagcaacaacatatgctgctgctcttagaattttgggaaatgatctgcttctaatactaagcagttctttaacatttttaaatgttatacagtgttacagtatttagtttggcaaatgtttcaaaataaagtagaaatgtattcataacatcacagaaatgcacatccaatgttgttttcaataagaaccataggtacagatcagaactcttccctatatgaaataatttacacacagatgaatactataatatcactatctaaaataatcactaaatacagttctttttcagaaataaacaagcaaagatttttttcattatcaaatatcaaaaacatgttgataatgtatgtttttcaaataaatgatactttaaaattataggaataatctcagtgaattcagtgaatgtgcaacctaaatcaaccaagtatactgtagtacaaccatattaagaaaccaatgatcagaaaatacaaccgtatgaaagaaatttataatccacaaaactttttcaggtcttaaggtaaaatagttccacagtctacaggtaaaaccaaggcaacaaaaatgcgtgcttatcttgattaagtaggtaattttatgcagaagatgtaacactttgtttgtagacagcatggtatgcatttctcagcaagacataaggaaaacaagattccaaaagatccattgtaaggaatggagattcttgtacaatcatatctagcagtaaataaacagattctctatttcttgttgtagttttatctgtctcctggccaattttcagtagactggaggatgcaagcgccagaaattctttaagacggtcttcaatgcttcctttgtgaattgtaaacaaagctgcagcaatctggttgatggctttggccaagcaatgtatgttgttgcaatgcccttctatagcagggctgtactgagacatcacattactggccagtgttggcaaagaaactgccacaaacaccatgagaaggcaggcaattttatactcttcttctggactaatgttttccgatttttgtgaagaaagagctacgaccaatgcaggatcaatctcacaaggtaatccggcagctgatgataactcatacacattcattgcaaccttcatatcagtttcccttggaatgtgatccttaaaatcttcaattgaacttacaagaaaaggaatgtggtaggataagacatctctaagtgcttcttgtgccaatgatcggaaggataaaattacaccaattattgtcatcctcttcaagacactgtcaacagatgataatcttttaaacagtgcagccatctggtctggtttgtcaaagctggtcctcatttgtgttaacacatcaacattctccaccacaagtttcttaagttcagcaacttgtgatgaaatatgccacataaggctttcacttagaaacttcataccatatgggcctagtagttctgataatgacctcatttctgatatgtcagaatattcctctgcattgaatgttaattcattttctgtaggtaagttcacaaacgctttcattgcaggaaaatatgctatatggccattgctgacttgtcgtaacaaagtttccaaataccaatttgtgtatagacttgtaatggttggctctccatgactgtctaaatgttgtgtttgttgaagaagcacattattaaatactcttgtaatatcaatctgcacatagttttctattgactggagtacggtcatgtatgctcttacacttgttagaagttctgaaggttttgcaatttcctgtgtggcttgattatacatagtcatcccaacaattgacttggtaaagcgtatttccagatgagaagtcaaatattctcgtggggtaaaggtatgttcccataccaccatgtttggtacataatttatagagaagcataactcagaaagtgcagtgtgcaatttatcaaggttggtcacaaccagcctgtttttcctcatgctctcaacacctggtttctccctttcaggttcccctttcttaccagtctgcttttttgatttcttattcactgcttgactgatagttttggcacaatgcttgggtagcaactggtcactaagggtacactgttctgtgcaaatatcagtgatgagatttcgagcttgtttggccatttcatctaggaacatattacataaggaaagactgcgatctccaatatgatgtcgctcttctggacatagttcatgcgtgcaactcataaaatgagtgcaaagtagtggaaatgcaattgagtatcttgattgagagggtaactccaaacactgttgaaacatcttctcaaaagcacgactataaaaacaaaatatggagagatctgatgtttccaccaacatttccaccaaggaatctaccatttttgtatgaaaaattattgtattcatcatctttccaagttctctgtgatctgcaaggccaagtgaagcctttgagacactagtatatgcctgtaacctaaaccaatctaatctcattcctctgaaatcaaatacttccccatcttcaacttgttttacacttagggaagtcatagtgttaacaaaagaggacatgatgattgattcatcttcagggcaaacagaaagattctgcacgagttcattgaggacaacagcatcaaagccagaaaggtactgcacgtaatacctctgcattacaggtccgtatttcctcacatgtgctctaagttcttccatgtaaaatattaattcagcaatgtgcttatctataaagtcgtctgcactcttctttggcatgttatctgcatgacgaagtagccagatgatttcatcacgggcaaaggataatgccataaaaacaaaaagtgccttgggacctagcaatccaggttgatcagagaggacagtagccaattccttcagtgcagatcttaaaaacttgcgtctttctctgtgcattgaaccagcatgtgacacggctgcctccttgcattctcttatgtcattaatacgtttattatagcctcgtatgtttacaaataagtcttctgcagctttgtgaatgtggaaaacttcatcccgaaagagagagaggcaagagctactttgaagagctagtttccaaaggttcagtgctgtagcgtcagtatttaggatcccatggcacaaaataaagccaaagataatccacttttccattgcatccaaagagaggtattcacaaggcatagtgtcggactgtgctggattaagcattgtactaggtgcactgatgaggctcaataactgggcatttctccactggtcagctgaaagattccttcgaggatataccatttgaagagaaattagtgcatctgaaagagacttgctatggggtacaaattcttccatcatcttctttaaagggttttcataatccacaatcatctggccaaggcgtgggtattctctgtcacttgctccatgagtcatttcatgggcatagttgtataatccaatgattgccttcctttcttcaattcgagacagcagtatcattagtgttgtataggttataattaaatctaagtagttctttgttaaatcaaagtttacagtaatatcaaagaagacttggcaaacgtcaatagtattcagcaattcacaaacatggtccttaaattccataacatctacaaatgtgaagtaatataatgccagatttttcagaatctctgatttttctttctgtagttgtgcaagctgttgattgttgttgcgggtttctacagcagggaattttctgactatgaatttcacagcagattccaggtttttgtcgataagataggatggttttgccttggggtctccacatgccttcttgatgttgtagaggcgggtgagcatgccgacgccccggtcgttgaggatggtgagcttctccgccagcttctgctgactgggctgcagcactgagcgcgacatggtggtgctggtgccgccgccgccgccggccgcctcgcgcccagtcacgggcccgcggccttcgcagcagcctctctcgggcctcctcccctcccgcccgcgacctccgccttaggagagcgcgcccatggccctcgcgccccaatcccgcgccggcgacagagcgagccgcggcggactcctcggagccccttctcccgcagcagcccgcgccccggcagcctcctgccttccgcccgccgcccttccgcccccacccccggcgctctccgccccagcccccaacgagccgccttccccggctgctccactaggtgtggcggcggcggcggcggcggcggcgtctccggcggctgag

SEQ ID NO: 11584 - RNA, 3002 nt, Homo sapiens
  source 1..3002: mol_type = other RNA
ctgaatagctgggactacaggtgtacaccaccacgcccagctaatttttgtatgtttagtagagacggggtttcactgtgttggccaggctggtctcgaactcctgactgcaagtgatctgcctgcctcagcctcccaaactgctgggattataggtgtgagccaccgcgcccagcccttagatgtggtctttaaagtataatccttttttaaaaaatacttccaagggaattttcagggtttgttagattagtcctcatcataggtttgattccttctcatcaaaagctgtcatcccactgtctctccttatagccaagtatcctaaactgtgcaagctgaagtgccttggagtacctcaggaaaaacacttgacactgacgcatcttttgtataaactactagttccaggaagttcagtttcaatatgatatggcactacattccctttgatggcatcctatccttgtgaagctgggtttggagccactgctatgacaaaaagcaccatgcaaaaatcaatgtggaagaaataaggacaatggtgtccaatctgatttcaattttgagaaactgtatggagcccaaaaggcacacacattccattagtaactgtgatgatttaaggatgagataaaaattatcacatcaggctgggcacagtggctcacacctgtaatcccagcactttggtaggccaaggcagatcacctgaggccaggagttccttacagcctgggcaacacagccagagccccatctctacaaaaaaattaggcgggcgtggtggcacgtgcctgaagtctccgctactcaggaggcagaggtgggaggcttgcttgagcccaggagtttgaggtcacaatgagctatgaccctccaacctgggcaatagagccaagacactgtctctatttttaaaaaaatcatcacatcacttttgctcttgtgtgtgtatagtttttttcaaatggctactagagttgttagaacataagttaataaatgtaactgttaggtatttcttttggccaaggaatggcctgaaaaaaattactgagattctaatgatgtcagaaactaaaagtctgagaatctctgggtcatctacatatatatgtatatatatatattttttttttctttttttttttgagacggagtttcgtgcttgttgcccaggctagagtgcaatggcacgatcttggctcaccacaacctccacctcccaggttcaagcgaattctcctgcctcagcctcccgagttagctgagattacaggcatgcaccaccacgcccagctaattttgcatttttagtagagacggggtttttccatgttggtcaggctggtcttgaactcccgacctcaggtgatccacctgcctcaggctcccaaagtgctgggattacaggtgtgagccactgcgcccagccttccttatacaactatatacaccccaaacttgccatcattctttagttcttgtgcaacagttctctgatttaagcagtatgtaagaggatcagttgctcacattagaggcctacctgttgataggaaatgcctgttttaaatacctgccacaaggtaacaaatcaaatagaagcagagtagaaactggactatcttcctagtccaatgaggagttgtatagtgagtggatacactccccgtctcagctccccaggattacttcataaactatgaaaatgacaatgaggcaggcaccagaaccactcaacacacatctgtagtcaggagtgctcacctatctgggccagagaattcaacaccatctactatccccaaccaggacttctgcgggtaaatcatgccacttcagatttctcctcaaattttctaccctaaaaaggagcttccaataaataactcacaccccagctagcagttactgtcctaaattatatagtagtatagcaaggccacataaatccaaggcattacactgtgatcaatatgtatttttttgaaactattctttttaattatagtttaagttctggggtacacgtgcaggacgtgcaaaatatgtacttctttaagatgtttccacaggtacaacagcagaactacatttagaattcacaaataatagactttacatctgtaatcctttaatcccattcatagcaatttggaaaaggaatgaaaataaaatatttagggtttctactcttgaaaatgagacacaaattagccaggcatggtggtgtgtgcctataatcccagctacttgggaggacaaggcaagagaattgcttggacctgggaggcggaggttgcagtgagccgagatcgcaccactgcactccagcttgagtgacagagcaggactctctctctcaaaaaaaaaaaaaaagacacaaactaatcagaataaattttaaaatgtttaaaccaaattcatatacaccatatatataaatgtatggcatactcaaatatattttaaaaaaagaaaaagaggggatttgcccataatcaaaactttattgaaaaactgacaccaaaataggagattactgctgtataccttacaaaaccaaatgtaattacattatcttggtaaattaattagaattatggaatttatgataaggctttctgtgagacaacacaaaattaaaattcaggaagctgtttgaatcattagtgttgctttcttctaaatgaacacccttctgtgagtctggcctttcctcctgtaggctggcacaacactgttgaacaacctacacaaagaaccactgtctgagcatggctgaaaaccgtggtgatcttgtagcaacctggacattttacatccataaagtaagaatttggactttgtactaggcgtttctttttatgttttttcttttcctcttccaaggacggatgtagtaaatctctagccaaaggcatgttgatcctcttgcaagctcagccctaccagacctcccagcccacacagctagcaagctgcaagcgatctgc

SEQ ID NO: 11585 - RNA, 3339 nt, Homo sapiens
  source 1..3339: mol_type = other RNA
ctgaatagctgggactacaggtgtacaccaccatacctggctaatttttatttttcatagaaacaatctccttatgttgcccaggcttaaaactttttaagaagtttctcctcttttcttgcaggcaggctggcactgctctctagggacctgttactggcaatgcttccccttttaatttgtatcttatttggaaagagcttcaaaattaggtagttgaacttggtaacaatatacaacagcaacacataggctaagactaagggaaaaagaagctcacctttgaacaaccacaagagttttgagtaaagggtcattcctgtgtcatgaataagtgagagtactgaaaagctccatttcaaattgatatgtatgattatatttaagctgattcaaaaacacctactgaccatcaagctctatatgtaatgctggaagagtttcttcctctccattgataaaccaataatttcactgtttgtcttgagtcttcaaaactgctgatttataaagtcaaagagcgtctaaggataaaagacattgagaacagagacatagtagcccagaaaggcactcttctagcactcttctggtcccacatttattcattcaataaaaatttattgagccacgctgtttccaaggaattgtactaggtgctgcaatgcaaagggttatgacaaaactgtctgtaaatgtaggatctgaattggtctttgatagttttcctgatttgagaaagaagtctctatttggctaatttagggagctaagagaatggacaaggtctgcttatgtccttctggcagcctagcatagcttttgcctccctcaaatcagttataagtcaaaacaaataaggcacattttttaaaaaaattcccccctttaattgaccaaagtaaagccatgacatttcatttggtaacctgtttagaattataaaaatcatttcatttggcccagcccatactgcccaagacaaaacttccagacaattctgatgccatccagttttgttcttacaaactgcatattaaaaaaaaaaaaaaaaaaaaatcttcaacgtcctaaatgtgatgtgctcagtgcgaagcatatcagagctggacgtgacatttatgtccttgacaagcctcgattatccaggtcctttaccttgtatatcctgaccagccaatgttctgtggtatatgcttcctccaggacatcaagctcaaagtctttattcccaatctcagcatttcggacacggtcaaagcctggaggacgcttggcttctgtgtaaacctgtccaaagcgatagtaacacatcttgtacatgaggcagttgagcagcactggagaaccttcacggtccacacggaactccccagttggagtataatagtcattctccttgatatgtttgcctgtatctgtgctccctccaatccggaccatccaaagaaacttgttgatatcatcagaggaatacccagtgaggcctccaaaaatgaccagcacatagctgacatcgagctccctcatgatctcataggctttttcctctgtggacgccattgcctgccctactcgagaaatatgggtattattccatgtgttattgtccactaaaattgttcggtttgccatagctgtaatctgatagccataatcccaccaggacatgaccttcgcatcctctggagtattatgacgaagccaataatatgcttctcggaagtcatcaaatatgatcctactgccatccccaccacgggcagatagtacaatggacggagaagagtaggcctcactggtcacccaggttgaatgaaaggtgtaggtgatgagaaagaaagccatgaccagtatcatcccacttgccacttcattcttaatagggtaggtggaatcctgttgcttcttgctcttcttgtctggacgacttatgtccagattcttcatgtatgtggacagcacctgggagactccaatgccagagagaatgcacataacaggtgccaacactagcattagacgcaccattacagctgaaaagtacatgctggtcacaccatacatgatgataaaaatccgggcatcagacaggttgctaaagcagtaatagaggccaactggaaacatgaagacgaggagctgcaggtcaaaatagtatgaggaccaggttgtgggctgatgctcagacacagaagcaatgatggggatgttgttcttagcataagagggatccagcagcgagtagaaacgccccgtccagggagatatttttcctgtcagcatgaggagagctcccacggtgagaaggacaaagcctaccagagagatgacgctccggaaaagaacttcaaattgttgtggattcaacttgctgcgcaggtaatccacaaaggcatggatctggcagagaccaaagaccccaaaggctgccatgtgctctgatgaaaggacaggctggaaacccacaaaggagatctgcatagaaagtatagtgcccaggcagtaaacagtacagtaggccacatagatccggtgagagaaacggcctgtgagcatcagcacgaggacgtggagaggaattaagttgatcaggaacacataacctccccatgacgagaccatgtagaaataagcaagggcacacttagctgcccaacagatggaaccagtctttactgccttgatccacatgtagtaggtgagtagcatgcaaaagatggcaatcccttcattatcataggagccagccacagatcgggagatatatccaggaactacagcaatcatggcagcagcaagaagcccagcccctgcatccttgagctctttggtaaggtggtacgtgacgatggtggtgaaggaggagaagagaggggccaggaacacacagacattccgaatgtcgatggtgatgtggaaaaaatggagtacatggtagattgcagcagaggtgatcattaaacctgggtaaattgttcctccaatgattcgtcccaaagggtaccaggctcggtcatcaaaccagttatggaatttataaaacccctcctcagccaggaacctggtagtccgataattaaagtacggatcaaactcatggataacactttcaaatctcaggacagcaaacagacgagtggagaaggataatacagcagccattgacagaatgagaagcttcaaaagtgtgtcctgcttctcataggacaatcgcaaaaatccaaacttagtcatcttgacatgaatgggtggcaacacacgacgatcagctggccggctttcctaaacgatccgcggggctccctcagccatccgttcagcggcgcacccaaccct

SEQ ID NO: 11586 - RNA, 3427 nt, Homo sapiens
  source 1..3427: mol_type = other RNA
ctgaatagctgggactacaggtgtacaccaccatacctggctaatttttatttttcatagaaacaatctccttatgttgcccaggcttaaaactttttaagaagtttctcctcttttcttgcaggcaggctggcactgctctctagggacctgttactggcaatgcttccccttttaatttgtatcttatttggaaagagcttcaaaattaggtagttgaacttggtaacaatatacaacagcaacacataggctaagactaagggaaaaagaagctcacctttgaacaaccacaagagttttgagtaaagggtcattcctgtgtcatgaataagtgagagtactgaaaagctccatttcaaattgatatgtatgattatatttaagctgattcaaaaacacctactgaccatcaagctctatatgtaatgctggaagagtttcttcctctccattgataaaccaataatttcactgtttgtcttgagtcttcaaaactgctgatttataaagtcaaagagcgtctaaggataaaagacattgagaacagagacatagtagcccagaaaggcactcttctagcactcttctggtcccacatttattcattcaataaaaatttattgagccacgctgtttccaaggaattgtactaggtgctgcaatgcaaagggttatgacaaaactgtctgtaaatgtaggatctgaattggtctttgatagttttcctgatttgagaaagaagtctctatttggctaatttagggagctaagagaatggacaaggtctgcttatgtccttctggcagcctagcatagcttttgcctccctcaaatcagttataagtcaaaacaaataaggcacattttttaaaaaaattcccccctttaattgaccaaagtaaagccatgacatttcatttggtaacctgtttagaattataaaaatcatttcatttggcccagcccatactgcccaagacaaaacttccagacaattctgatgccatccagttttgttcttacaaactgcatattaaaaaaaaaaaaaaaaaaaaatcttcaacgtcctaaatgtgatgtgctcagtgcgaagcatatcagagctggacgtgacatttatgtccttgacaagcctcgattatccaggtcctttaccttgtatatcctgaccagccaatgttctgtggtatatgcttcctccaggacatcaagctcaaagtctttattcccaatctcagcatttcggacacggtcaaagcctggaggacgcttggcttctgtgtaaacctgtccaaagcgatagtaacacatcttgtacatgaggcagttgagcagcactggagaaccttcacggtccacacggaactccccagttggagtataatagtcattctccttgatatgtttgcctgtatctgtgctccctccaatccggaccatccaaagaaacttgttgatatcatcagaggaatacccagtgaggcctccaaaaatgaccagcacatagctgacatcgagctccctcatgatctcataggctttttcctctgtggacgccattgcctgccctactcgagaaatatgggtattattccatgtgttattgtccactaaaattgttcggtttgccatagctgtaatctgatagccataatcccaccaggacatgaccttcgcatcctctggagtattatgacgaagccaataatatgcttctcggaagtcatcaaatatgatcctactgccatccccaccacgggcagatagtacaatggacggagaagagtaggcctcactggtcacccaggttgaatgaaaggtgtaggtgatgagaaagaaagccatgaccagtatcatcccacttgccacttcattcttaatagggtaggtggaatcctgttgcttcttgctcttcttgtctggacgacttatgtccagattcttcatgtatgtggacagcacctgggagactccaatgccagagagaatgcacataacaggtgccaacactagcattagacgcaccattacagctgaaaagtacatgctggtcacaccatacatgatgataaaaatccgggcatcagacaggttgctaaagcagtaatagaggccaactggaaacatgaagacgaggagctgcaggtcaaaatagtatgaggaccaggttgtgggctgatgctcagacacagaagcaatgatggggatgttgttcttagcataagagggatccagcagcgagtagaaacgccccgtccagggagatatttttcctgtcagcatgaggagagctcccacggtgagaaggacaaagcctaccagagagatgacgctccggaaaagaacttcaaattgttgtggattcaacttgctgcgcaggtaatccacaaaggcatggatctggcagagaccaaagaccccaaaggctgccatgtgctctgatgaaaggacaggctggaaacccacaaaggagatctgcatagaaagtatagtgcccaggcagtaaacagtacagtaggccacatagatccggtgagagaaacggcctgtgagcatcagcacgaggacgtggagaggaattaagttgatcaggaacacataacctccccatgacgagaccatgtagaaataagcaagggcacacttagctgcccaacagatggaaccagtctttactgccttgatccacatgtagtaggtgagtagcatgcaaaagatggcaatcccttcattatcataggagccagccacagatcgggagatatatccaggaactacagcaatcatggcagcagcaagaagcccagcccctgcatccttgagctctttggtaaggtggtacgtgacgatggtggtgaaggaggagaagagaggggccaggaacacacagacattccgaatgtcgatggtgatgtggaaaaaatggagtacatggtagattgcagcagaggtgatcattaaacctgggtaaattgttcctccaatgattcgtcccaaagggtaccaggctcggtcatcaaaccagttatggaatttataaaacccctcctcagccaggaacctggtagtccgataattaaagtacggatcaaactcatggataacactttcaaatctcaggacagcaaacagacgagtggagaaggataatacagcagccattgacagaatgagaagcttcaaaagtgtgtcctgcttctcataggacaatcgcaaaaatccaaacttagtcatcttgacatgaatgggtggcaacacacgacgatcagtttgcaactaaaaataaaggcctaactactccaggaggtcaacaatccagccatatctctcagggtttgcagctgttttctggaatgcctggccggctttcctaaacgatccgcggggctccctcagccatccgttcagcggcgcacccaaccct

SEQ ID NO: 11587 - RNA, 3216 nt, Homo sapiens
  source 1..3216: mol_type = other RNA
ctgaatagctgggactacaggtgtacaccaccatacctggctaatttttatttttcatagaaacaatctccttatgttgcccaggcttaaaactttttaagaagtttctcctcttttcttgcaggcaggctggcactgctctctagggacctgttactggcaatgcttccccttttaatttgtatcttatttggaaagagcttcaaaattaggtagttgaacttggtaacaatatacaacagcaacacataggctaagactaagggaaaaagaagctcacctttgaacaaccacaagagttttgagtaaagggtcattcctgtgtcatgaataagtgagagtactgaaaagctccatttcaaattgatatgtatgattatatttaagctgattcaaaaacacctactgaccatcaagctctatatgtaatgctggaagagtttcttcctctccattgataaaccaataatttcactgtttgtcttgagtcttcaaaactgctgatttataaagtcaaagagcgtctaaggataaaagacattgagaacagagacatagtagcccagaaaggcactcttctagcactcttctggtcccacatttattcattcaataaaaatttattgagccacgctgtttccaaggaattgtactaggtgctgcaatgcaaagggttatgacaaaactgtctgtaaatgtaggatctgaattggtctttgatagttttcctgatttgagaaagaagtctctatttggctaatttagggagctaagagaatggacaaggtctgcttatgtccttctggcagcctagcatagcttttgcctccctcaaatcagttataagtcaaaacaaataaggcacattttttaaaaaaattcccccctttaattgaccaaagtaaagccatgacatttcatttggtaacctgtttagaattataaaaatcatttcatttggcccagcccatactgcccaagacaaaacttccagacaattctgatgccatccagttttgttcttacaaactgcatattaaaaaaaaaaaaaaaaaaaaatcttcaacgtcctaaatgtgatgtgctcagtgcgaagcatatcagagctggacgtgacatttatgtccttgacaagcctcgattatccaggtcctttaccttgtatatcctgaccagccaatgttctgtggtatatgcttcctccaggacatcaagctcaaagtctttattcccaatctcagcatttcggacacggtcaaagcctggaggacgcttggcttctgtgtaaacctgtccaaagcgatagtaacacatcttgtacatgaggcagttgagcagcactggagaaccttcacggtccacacggaactccccagttggagtataatagtcattctccttgatatgtttgcctgtatctgtgctccctccaatccggaccatccaaagaaacttgttgatatcatcagaggaatacccagtgaggcctccaaaaatgaccagcacatagctgacatcgagctccctcatgatctcataggctttttcctctgtggacgccattgcctgccctactcgagaaatatgggtattattccatgtgttattgtccactaaaattgttcggtttgccatagctgtaatctgatagccataatcccaccaggacatgaccttcgcatcctctggagtattatgacgaagccaataatatgcttctcggaagtcatcaaatatgatcctactgccatccccaccacgggcagatagtacaatggacggagaagagtaggcctcactggtcacccaggttgaatgaaaggtgtaggtgatgagaaagaaagccatgaccagtatcatcccacttgccacttcattcttaatagggtaggtggaatcctgttgcttcttgctcttcttgtctggacgacttatgtccagattcttcatgtatgtggacagcacctgggagactccaatgccagagagaatgcacataacaggtgccaacactagcattagacgcaccattacagctgaaaagtacatgctggtcacaccatacatgatgataaaaatccgggcatcagacaggttgctaaagcagtaatagaggccaactggaaacatgaagacgaggagctgcaggtcaaaatagtatgaggaccaggttgtgggctgatgctcagacacagaagcaatgatggggatgttgttcttagcataagagggatccagcagcgagtagaaacgccccgtccagggagatatttttcctgtcagcatgaggagagctcccacggtgagaaggacaaagcctaccagagagatgacgctccggaaaagaacttcaaattgttgtggattcaacttgctgcgcaggtaatccacaaaggcatggatctggcagagaccaaagaccccaaaggctgccatgtgctctgatgaaaggacaggctggaaacccacaaaggagatctgcatagaaagtatagtgcccaggcagtaaacagtacagtaggccacatagatccggtgagagaaacggcctgtgagcatcagcacgaggacgtggagaggaattaagttgatcaggaacacataacctccccatgacgagaccatgtagaaataagcaagggcacacttagctgcccaacagatggaaccagtctttactgccttgatccacatgtagtaggtgagtagcatgcaaaagatggcaatcccttcattatcataggagccagccacagatcgggagatatatccaggaactacagcaatcatggcagcagcaagaagcccagcccctgcatccttgagctctttggtaaggtggtacgtgacgatggtggtgaaggaggagaagagaggggccaggaacacacagacattccgaatgtcgatggtgatgtggaaaaaatggagtacatggtagattgcagcagaggtgatcattaaacctgggtaaattgttcctccaatgattcgtcccaaagggtaccaggctcggtcatcaaaccagttatggaatttataaaacccctcctcagccaggaacctggtagtccgataattaaagtacggatcaaactcatggataacactttcaaatctcaggacagcaaacagacgagtggagaaggctggccggctttcctaaacgatccgcggggctccctcagccatccgttcagcggcgcacccaaccct

SEQ ID NO: 11588 - RNA, 4138 nt, Homo sapiens
  source 1..4138: mol_type = other RNA
ctgaatagctgggactacaggtgtacaccactacaagtggctaatttttgtcagtttttgcagagaagagggtctcactatgttgcccaagctggtcttgaaatcctgggctcaagagatcctcccatcttggcctcccgaagtgttgggattacaggcgtgaaccacggtgactagctcaatccaagcttttctgatttctgatgtaatctaattcatggcactttaaatgttttggtgccttggtgtattaacatgtaacatgagaacaagatttatttacttacctcaagaagctagtacatgggttattgaatgcactcttaaactttgagcccctcagatgaaaagcactgtggaaacaattacagctgaagaaaacccttccaatgcctcagaatcctgacttactgtgccttgtgtctcaatggcacattgagaaacaatgtgcactagttagtggcatcacatcccttcatatatgttgtttggcacacaaatgtttatacatttaaaatagctgtcatactacctattcaaaagcatttactagttttctaataaagctaatgaaatgtacccattatggagtactccgtgtcaagtttagagaaactttagctttctctgaagtacatgtaacataataaaaagtttatttaaaaaattgaactagtgttgtatgaagccataagtttttaatgaaaaaaaatgtatgccacagtgtctatatattcatctgaagagtacaaagatggagttctgagaaaaaagggtttatcactatagaaaataaatctggttcttaaattatgttcaaagcaaacattaaaacagtaatgtctcatacactgaaataaagcaattagaggtaataaattataaatacagtagttcaaatattgttttaagcattagtttttctaaacaagttaaattcaaaacattttaaatctgttatattttttcaaagggatgtacaaatgaaagccttcatagaaatctaaaacgataccaccttgtgatcttcatatagaatatgctgaaccttgaccatttttgatttataacatactttggttaatacattatgttccatatgcctttatatttgggaggaatcagattgtgatttgtagcctttacatgcagtttacccaaaccttcttcacatccaggtcttgcttgattctctggagaaggttttgtcagactcataattaaaatgatgcaaactgtaaatgacttcttcagaactgaaaacttcttttttttttaaataaagtgcttttaaattcaaatatatgttgccctaaagaaaactgaaatatactttaaccctgaaatctccgtatcttgacacacacattttaacggaaaaaaaaaaaatcagttttaggccattcatgtccttcaagagagttcagattggatctaaattgggttttgcatcatcatcgtgctcatgtttatacatgaaggttaaaagaaaaagggcaacatccaaggatgaccaataggcagtatgcgacgtgacagctgaccaatagcggctctccacaaggccttctctgagttcaaaatcaatcctgtgatccaactccaatgcagaatcgaggaagccagaactgctatgtggaagggtctgtgtccctacggtggtagcagaaggtgaggcaactggcttcttctcatcttccattgagtcttttgatgtttcagatgactgtgttgtagatgaacgtccaaatcttgagaacaacattcctccaagtccctttccaatgctagcagcccctaatatgcttgctttgcctatatttgttatagattctccatagtgtcggcgggacaaaactggtgaggtcacagggcttggtatggttgaaatgccttcattctctgaaactgaggtaggttctttagctgggttgagaaagcttggcttcatatgttcataaggtaaaggatttgaagtattgtaccagtggatctggacaggtgaaatgttgctgtagtgtttcagtattaatggttctaatctataagccactggatctgtaggatgaaaaatatttagtaaccggttacaaatctctctaggcaaaatatggtcttgacttccagtatttcctgggcggatgccacgcaacgccaagaaaactgctaatggggatcccatacagaagaaattctcaaccttaaattttaaggcaggtgtttgtgtcatagatgatgctttcaatccgtgaagccgttcttctatttccttcagccgtcgtttagttatatagagttcatcaagaagatgtcgttcttcatagctcatccatcgttcatcaggcaactcttcttccttttgcagcaactgttcatacagccgaactggattccagccagtcattatgtcataagtaattacacatcccaaggaatgtgatactattgagactttaccccctttttcttcaaagtctggattccgagaacagaaaagggaatacaatcgattcagctcttgctgaaggcctttaactagttcatctctataaagtggactagtataatacattatgtccattgcactgctgttcagcatatcccttaaacctcgtactttgtcaggagtaatggaatcaacagtgtctccatcaagagtaagttttgaccgccactcaacaggcagaaattcaacatgtgttgcatggttggaaaaatgcctttcttctatttttcttgcagcttctctcatcatagctgtatttttgataattcttccttggtccattttctgcccaatgccatgcacaacaaatacaatatgggtagtctgtgatggcttgtcttctaatgtggcttcttctacataacctctatgaagtctggtaccactacttgatgcatcttttccatctatggattttgacacttcaatatcgaaattttcctgcatctgctggcccctaaaacaattgagatgttcttgctcaattaaattactttcttcctcttctagaggctgccaagtgccgtcaataaaccactgtccacgcattactggtattttatcagcctggttccagtacaccgggtagcactctccttgggtcacatccacctcgtagaggccgccccgcacgcacacaggctcgatgttcacaagctccaccatctccggctcgtgccccgtcgtactctggcagaagccgcaggcgcggtcctcatcgtcatcttctccggaactggaggctgggcccgtgggggagcacacatggtcgccgtcccggtccccgccctggggccgggcacccgtggtctgcagcagggtccggaaggcgagctcgatgcggagcgagtcgtagccgatgaagggcttccaggtcttcttgtcctccttgtagaaccagcgtacctcctccgggcccagctccgtcactacctcatagcggtgccgggccgccgggccgccaagccgggtacgtttcctttccccgggggaccctcctgtcgcgccgccgccccccgagttcgtcgggaccagcggaggctgctgcggcgggtgcagcgacaaggagctgccgccgccgccgctctcaccctcgctgtagtagcgcagcgaggagcccgactcggcggagctgaagtcatagttctcgtcactgaggcaggggtccagcgcgaggtggtggttgtggtcgtcggtgcccggcgccaaatgcagcccgggttccccgcgcagcagggccaggggcacgtcgccgtcgtccgggtccccgccgggcaggtgctcgaagcagcagacgccgccgccgaacgctggcctcgcgtctgagcccagctcccaggcgccgccgccgccgcctcggccgttatgctcggggctccgtggggacccgcggcccgggtaattcatgctgtggagacgccgccggctgtccggcggcgcgcggagccgtgacccccagcgcttccgccacacattcaacgccgccgccctctccacccgaagtttctaatctttcaaatcccgacccgagctgcggcggcagcggcgaccgctccgcccccacgagacccgcagccgccgcagctgcgttctgccgccggccccattgtcacgcagcccgacgtaggcggt

SEQ ID NO: 11589 - RNA, 4288 nt, Homo sapiens
  source 1..4288: mol_type = other RNA
ctgaatagctgggactacaggtgtacaccactacaagtggctaatttttgtcagtttttgcagagaagagggtctcactatgttgcccaagctggtcttgaaatcctgggctcaagagatcctcccatcttggcctcccgaagtgttgggattacaggcgtgaaccacggtgactagctcaatccaagcttttctgatttctgatgtaatctaattcatggcactttaaatgttttggtgccttggtgtattaacatgtaacatgagaacaagatttatttacttacctcaagaagctagtacatgggttattgaatgcactcttaaactttgagcccctcagatgaaaagcactgtggaaacaattacagctgaagaaaacccttccaatgcctcagaatcctgacttactgtgccttgtgtctcaatggcacattgagaaacaatgtgcactagttagtggcatcacatcccttcatatatgttgtttggcacacaaatgtttatacatttaaaatagctgtcatactacctattcaaaagcatttactagttttctaataaagctaatgaaatgtacccattatggagtactccgtgtcaagtttagagaaactttagctttctctgaagtacatgtaacataataaaaagtttatttaaaaaattgaactagtgttgtatgaagccataagtttttaatgaaaaaaaatgtatgccacagtgtctatatattcatctgaagagtacaaagatggagttctgagaaaaaagggtttatcactatagaaaataaatctggttcttaaattatgttcaaagcaaacattaaaacagtaatgtctcatacactgaaataaagcaattagaggtaataaattataaatacagtagttcaaatattgttttaagcattagtttttctaaacaagttaaattcaaaacattttaaatctgttatattttttcaaagggatgtacaaatgaaagccttcatagaaatctaaaacgataccaccttgtgatcttcatatagaatatgctgaaccttgaccatttttgatttataacatactttggttaatacattatgttccatatgcctttatatttgggaggaatcagattgtgatttgtagcctttacatgcagtttacccaaaccttcttcacatccaggtcttgcttgattctctggagaaggttttgtcagactcataattaaaatgatgcaaactgtaaatgacttcttcagaactgaaaacttcttttttttttaaataaagtgcttttaaattcaaatatatgttgccctaaagaaaactgaaatatactttaaccctgaaatctccgtatcttgacacacacattttaacggaaaaaaaaaaaatcagttttaggccattcatgtccttcaagagagttcagattggatctaaattgggttttgcatcatcatcgtgctcatgtttatacatgaaggttaaaagaaaaagggcaacatccaaggatgaccaataggcagtatgcgacgtgacagctgaccaatagcggctctccacaaggccttctctgagttcaaaatcaatcctgtgatccaactccaatgcagaatcgaggaagccagaactgctatgtggaagggtctgtgtccctacggtggtagcagaaggtgaggcaactggcttcttctcatcttccattgagtcttttgatgtttcagatgactgtgttgtagatgaacgtccaaatcttgagaacaacattcctccaagtccctttccaatgctagcagcccctaatatgcttgctttgcctatatttgttatagattctccatagtgtcggcgggacaaaactggtgaggtcacagggcttggtatggttgaaatgccttcattctctgaaactgaggtaggttctttagctgggttgagaaagcttggcttcatatgttcataaggtaaaggatttgaagtattgtaccagtggatctggacaggtgaaatgttgctgtagtgtttcagtattaatggttctaatctataagccactggatctgtaggatgaaaaatatttagtaaccggttacaaatctctctaggcaaaatatggtcttgacttccagtatttcctgggcggatgccacgcaacgccaagaaaactgctaatggggatcccatacagaagaaattctcaaccttaaattttaaggcaggtgtttgtgtcatagatgatgctttcaatccgtgaagccgttcttctatttccttcagccgtcgtttagttatatagagttcatcaagaagatgtcgttcttcatagctcatccatcgttcatcaggcaactcttcttccttttgcagcaactgttcatacagccgaactggattccagccagtcattatgtcataagtaattacacatcccaaggaatgtgatactattgagactttaccccctttttcttcaaagtctggattccgagaacagaaaagggaatacaatcgattcagctcttgctgaaggcctttaactagttcatctctataaagtggactagtataatacattatgtccattgcactgctgttcagcatatcccttaaacctcgtactttgtcaggagtaatggaatcaacagtgtctccatcaagagtaagttttgaccgccactcaacaggcagaaattcaacatgtgttgcatggttggaaaaatgcctttcttctatttttcttgcagcttctctcatcatagctgtatttttgataattcttccttggtccattttctgcccaatgccatgcacaacaaatacaatatgggtagtctgtgatggcttgtcttctaatgtggcttcttctacataacctctatgaagtctggtaccactacttgatgctttagaaaatcccagtttttgggtaactgttcttgcaattttagatgttgttgcatcactataaagatatacttcatccacactgtgccagtccacatggtttcgactcaacttgaaactatgaacagcagaatagttgatcccactgccatcttttccatctatggattttgacacttcaatatcgaaattttcctgcatctgctggcccctaaaacaattgagatgttcttgctcaattaaattactttcttcctcttctagaggctgccaagtgccgtcaataaaccactgtccacgcattactggtattttatcagcctggttccagtacaccgggtagcactctccttgggtcacatccacctcgtagaggccgccccgcacgcacacaggctcgatgttcacaagctccaccatctccggctcgtgccccgtcgtactctggcagaagccgcaggcgcggtcctcatcgtcatcttctccggaactggaggctgggcccgtgggggagcacacatggtcgccgtcccggtccccgccctggggccgggcacccgtggtctgcagcagggtccggaaggcgagctcgatgcggagcgagtcgtagccgatgaagggcttccaggtcttcttgtcctccttgtagaaccagcgtacctcctccgggcccagctccgtcactacctcatagcggtgccgggccgccgggccgccaagccgggtacgtttcctttccccgggggaccctcctgtcgcgccgccgccccccgagttcgtcgggaccagcggaggctgctgcggcgggtgcagcgacaaggagctgccgccgccgccgctctcaccctcgctgtagtagcgcagcgaggagcccgactcggcggagctgaagtcatagttctcgtcactgaggcaggggtccagcgcgaggtggtggttgtggtcgtcggtgcccggcgccaaatgcagcccgggttccccgcgcagcagggccaggggcacgtcgccgtcgtccgggtccccgccgggcaggtgctcgaagcagcagacgccgccgccgaacgctggcctcgcgtctgagcccagctcccaggcgccgccgccgccgcctcggccgttatgctcggggctccgtggggacccgcggcccgggtaattcatgctgtggagacgccgccggctgtccggcggcgcgcggagccgtgacccccagcgcttccgccacacattcaacgccgccgccctctccacccgaagtttctaatctttcaaatcccgacccgagctgcggcggcagcggcgaccgctccgcccccacgagacccgcagccgccgcagctgcgttctgccgccggccccattgtcacgcagcccgacgtaggcggt

SEQ ID NO: 11590 - RNA, 4267 nt, Homo sapiens
  source 1..4267: mol_type = other RNA
ctgaatagctgggactacaggtgtacaccactacaagtggctaatttttgtcagtttttgcagagaagagggtctcactatgttgcccaagctggtcttgaaatcctgggctcaagagatcctcccatcttggcctcccgaagtgttgggattacaggcgtgaaccacggtgactagctcaatccaagcttttctgatttctgatgtaatctaattcatggcactttaaatgttttggtgccttggtgtattaacatgtaacatgagaacaagatttatttacttacctcaagaagctagtacatgggttattgaatgcactcttaaactttgagcccctcagatgaaaagcactgtggaaacaattacagctgaagaaaacccttccaatgcctcagaatcctgacttactgtgccttgtgtctcaatggcacattgagaaacaatgtgcactagttagtggcatcacatcccttcatatatgttgtttggcacacaaatgtttatacatttaaaatagctgtcatactacctattcaaaagcatttactagttttctaataaagctaatgaaatgtacccattatggagtactccgtgtcaagtttagagaaactttagctttctctgaagtacatgtaacataataaaaagtttatttaaaaaattgaactagtgttgtatgaagccataagtttttaatgaaaaaaaatgtatgccacagtgtctatatattcatctgaagagtacaaagatggagttctgagaaaaaagggtttatcactatagaaaataaatctggttcttaaattatgttcaaagcaaacattaaaacagtaatgtctcatacactgaaataaagcaattagaggtaataaattataaatacagtagttcaaatattgttttaagcattagtttttctaaacaagttaaattcaaaacattttaaatctgttatattttttcaaagggatgtacaaatgaaagccttcatagaaatctaaaacgataccaccttgtgatcttcatatagaatatgctgaaccttgaccatttttgatttataacatactttggttaatacattatgttccatatgcctttatatttgggaggaatcagattgtgatttgtagcctttacatgcagtttacccaaaccttcttcacatccaggtcttgcttgattctctggagaaggttttgtcagactcataattaaaatgatgcaaactgtaaatgacttcttcagaactgaaaacttcttttttttttaaataaagtgcttttaaattcaaatatatgttgccctaaagaaaactgaaatatactttaaccctgaaatctccgtatcttgacacacacattttaacggaaaaaaaaaaaatcagttttaggccattcatgtccttcaagagagttcagattggatctaaattgggttttgcatcatcatcgtgctcatgtttatacatgaaggttaaaagaaaaagggcaacatccaaggatgaccaataggcagtatgcgacgtgacagctgaccaatagcggctctccacaaggccttctctgagttcaaaatcaatcctgtgatccaactccaatgcagaatcgaggaagccagaactgctatgtggaagggtctgtgtccctacggtggtagcagaaggtgaggcaactggcttcttctcatcttccattgagtcttttgatgtttcagatgactgtgttgtagatgaacgtccaaatcttgagaacaacattcctccaagtccctttccaatgctagcagcccctaatatgcttgctttgcctatatttgttatagattctccatagtgtcggcgggacaaaactggtgaggtcacagggcttggtatggttgaaatgccttcattctctgaaactgaggtaggttctttagctgggttgagaaagcttggcttcatatgttcataaggtaaaggatttgaagtattgtaccagtggatctggacaggtgaaatgttgctgtagtgtttcagtattaatggttctaatctataagccactggatctgtaggatgaaaaatatttagtaaccggttacaaatctctctaggcaaaatatggtcttgacttccagtatttcctgggcggatgccacgcaacgccaagaaaactgctaatggggatcccatacagaagaaattctcaaccttaaattttaaggcaggtgtttgtgtcatagatgatgctttcaatccgtgaagccgttcttctatttccttcagccgtcgtttagttatatagagttcatcaagaagatgtcgttcttcatagctcatccatcgttcatcaggcaactcttcttccttttgcagcaactgttcatacagccgaactggattccagccagtcattatgtcataagtaattacacatcccaaggaatgtgatactattgagactttaccccctttttcttcaaagtctggattccgagaacagaaaagggaatacaatcgattcagctcttgctgaaggcctttaactagttcatctctataaagtggactagtataatacattatgtccattgcactgctgttcagcatatcccttaaacctcgtactttgtcaggagtaatggaatcaacagtgtctccatcaagagtaagttttgaccgccactcaacaggcagaaattcaacatgtgttgcatggttggaaaaatgcctttcttctatttttcttgcagcttctctcatcatagctgtatttttgataattcttccttggtccattttctgcccaatgccatgcacaacaaatacaatatgggtagtctgtgatggcttgtcttctaatgtggcttcttctacataacctctatgaagtctggtaccactacttgatgctttagaaaatcccagtttttgggtaactgttcttgcaattttagatgttgttgcatcactataaagatatacttcatccacactgtgccagtccacatggtttcgactcaacttgaaactatgaacagcatcttttccatctatggattttgacacttcaatatcgaaattttcctgcatctgctggcccctaaaacaattgagatgttcttgctcaattaaattactttcttcctcttctagaggctgccaagtgccgtcaataaaccactgtccacgcattactggtattttatcagcctggttccagtacaccgggtagcactctccttgggtcacatccacctcgtagaggccgccccgcacgcacacaggctcgatgttcacaagctccaccatctccggctcgtgccccgtcgtactctggcagaagccgcaggcgcggtcctcatcgtcatcttctccggaactggaggctgggcccgtgggggagcacacatggtcgccgtcccggtccccgccctggggccgggcacccgtggtctgcagcagggtccggaaggcgagctcgatgcggagcgagtcgtagccgatgaagggcttccaggtcttcttgtcctccttgtagaaccagcgtacctcctccgggcccagctccgtcactacctcatagcggtgccgggccgccgggccgccaagccgggtacgtttcctttccccgggggaccctcctgtcgcgccgccgccccccgagttcgtcgggaccagcggaggctgctgcggcgggtgcagcgacaaggagctgccgccgccgccgctctcaccctcgctgtagtagcgcagcgaggagcccgactcggcggagctgaagtcatagttctcgtcactgaggcaggggtccagcgcgaggtggtggttgtggtcgtcggtgcccggcgccaaatgcagcccgggttccccgcgcagcagggccaggggcacgtcgccgtcgtccgggtccccgccgggcaggtgctcgaagcagcagacgccgccgccgaacgctggcctcgcgtctgagcccagctcccaggcgccgccgccgccgcctcggccgttatgctcggggctccgtggggacccgcggcccgggtaattcatgctgtggagacgccgccggctgtccggcggcgcgcggagccgtgacccccagcgcttccgccacacattcaacgccgccgccctctccacccgaagtttctaatctttcaaatcccgacccgagctgcggcggcagcggcgaccgctccgcccccacgagacccgcagccgccgcagctgcgttctgccgccggccccattgtcacgcagcccgacgtaggcggt

SEQ ID NO: 11591 - RNA, 4390 nt, Homo sapiens
  source 1..4390: mol_type = other RNA
ctgaatagctgggactacaggtgtacaccactacaagtggctaatttttgtcagtttttgcagagaagagggtctcactatgttgcccaagctggtcttgaaatcctgggctcaagagatcctcccatcttggcctcccgaagtgttgggattacaggcgtgaaccacggtgactagctcaatccaagcttttctgatttctgatgtaatctaattcatggcactttaaatgttttggtgccttggtgtattaacatgtaacatgagaacaagatttatttacttacctcaagaagctagtacatgggttattgaatgcactcttaaactttgagcccctcagatgaaaagcactgtggaaacaattacagctgaagaaaacccttccaatgcctcagaatcctgacttactgtgccttgtgtctcaatggcacattgagaaacaatgtgcactagttagtggcatcacatcccttcatatatgttgtttggcacacaaatgtttatacatttaaaatagctgtcatactacctattcaaaagcatttactagttttctaataaagctaatgaaatgtacccattatggagtactccgtgtcaagtttagagaaactttagctttctctgaagtacatgtaacataataaaaagtttatttaaaaaattgaactagtgttgtatgaagccataagtttttaatgaaaaaaaatgtatgccacagtgtctatatattcatctgaagagtacaaagatggagttctgagaaaaaagggtttatcactatagaaaataaatctggttcttaaattatgttcaaagcaaacattaaaacagtaatgtctcatacactgaaataaagcaattagaggtaataaattataaatacagtagttcaaatattgttttaagcattagtttttctaaacaagttaaattcaaaacattttaaatctgttatattttttcaaagggatgtacaaatgaaagccttcatagaaatctaaaacgataccaccttgtgatcttcatatagaatatgctgaaccttgaccatttttgatttataacatactttggttaatacattatgttccatatgcctttatatttgggaggaatcagattgtgatttgtagcctttacatgcagtttacccaaaccttcttcacatccaggtcttgcttgattctctggagaaggttttgtcagactcataattaaaatgatgcaaactgtaaatgacttcttcagaactgaaaacttcttttttttttaaataaagtgcttttaaattcaaatatatgttgccctaaagaaaactgaaatatactttaaccctgaaatctccgtatcttgacacacacattttaacggaaaaaaaaaaaatcagttttaggccattcatgtccttcaagagagttcagattggatctaaattgggttttgcatcatcatcgtgctcatgtttatacatgaaggttaaaagaaaaagggcaacatccaaggatgaccaataggcagtatgcgacgtgacagctgaccaatagcggctctccacaaggccttctctgagttcaaaatcaatcctgtgatccaactccaatgcagaatcgaggaagccagaactgctatgtggaagggtctgtgtccctacggtggtagcagaaggtgaggcaactggcttcttctcatcttccattgagtcttttgatgtttcagatgactgtgttgtagatgaacgtccaaatcttgagaacaacattcctccaagtccctttccaatgctagcagcccctaatatgcttgctttgcctatatttgttatagattctccatagtgtcggcgggacaaaactggtgaggtcacagggcttggtatggttgaaatgccttcattctctgaaactgaggtaggttctttagctgggttgagaaagcttggcttcatatgttcataaggtaaaggatttgaagtattgtaccagtggatctggacaggtgaaatgttgctgtagtgtttcagtattaatggttctaatctataagccactggatctgtaggatgaaaaatatttagtaaccggttacaaatctctctaggcaaaatatggtcttgacttccagtatttcctgggcggatgccacgcaacgccaagaaaactgctaatggggatcccatacagaagaaattctcaaccttaaattttaaggcaggtgtttgtgtcatagatgatgctttcaatccgtgaagccgttcttctatttccttcagccgtcgtttagttatatagagttcatcaagaagatgtcgttcttcatagctcatccatcgttcatcaggcaactcttcttccttttgcagcaactgttcatacagccgaactggattccagccagtcattatgtcataagtaattacacatcccaaggaatgtgatactattgagactttaccccctttttcttcaaagtctggattccgagaacagaaaagggaatacaatcgattcagctcttgctgaaggcctttaactagttcatctctataaagtggactagtataatacattatgtccattgcactgctgttcagcatatcccttaaacctcgtactttgtcaggagtaatggaatcaacagtgtctccatcaagagtaagttttgaccgccactcaacaggcagaaattcaacatgtgttgcatggttggaaaaatgcctttcttctatttttcttgcagcttctctcatcatagctgtatttttgataattcttccttggtccattttctgcccaatgccatgcacaacaaatacaatatgggtagtctgtgatggcttgtcttctaatgtggcttcttctacataacctctatgaagtctggtaccactacttgatgctttagaaaatcccagtttttgggtaactgttcttgcaattttagatgttgttgcatcactataaagatatacttcatccacactgtgccagtccacatggtttcgactcaacttgaaactatgaacagcttgggaatgctttcgtttaagacctgtcgcatctgtactctccttatatcttctccatttgaacagagaagggagggagaagggagggaggtggtagacaacagaatagttgatcccactgccatcttttccatctatggattttgacacttcaatatcgaaattttcctgcatctgctggcccctaaaacaattgagatgttcttgctcaattaaattactttcttcctcttctagaggctgccaagtgccgtcaataaaccactgtccacgcattactggtattttatcagcctggttccagtacaccgggtagcactctccttgggtcacatccacctcgtagaggccgccccgcacgcacacaggctcgatgttcacaagctccaccatctccggctcgtgccccgtcgtactctggcagaagccgcaggcgcggtcctcatcgtcatcttctccggaactggaggctgggcccgtgggggagcacacatggtcgccgtcccggtccccgccctggggccgggcacccgtggtctgcagcagggtccggaaggcgagctcgatgcggagcgagtcgtagccgatgaagggcttccaggtcttcttgtcctccttgtagaaccagcgtacctcctccgggcccagctccgtcactacctcatagcggtgccgggccgccgggccgccaagccgggtacgtttcctttccccgggggaccctcctgtcgcgccgccgccccccgagttcgtcgggaccagcggaggctgctgcggcgggtgcagcgacaaggagctgccgccgccgccgctctcaccctcgctgtagtagcgcagcgaggagcccgactcggcggagctgaagtcatagttctcgtcactgaggcaggggtccagcgcgaggtggtggttgtggtcgtcggtgcccggcgccaaatgcagcccgggttccccgcgcagcagggccaggggcacgtcgccgtcgtccgggtccccgccgggcaggtgctcgaagcagcagacgccgccgccgaacgctggcctcgcgtctgagcccagctcccaggcgccgccgccgccgcctcggccgttatgctcggggctccgtggggacccgcggcccgggtaattcatgctgtggagacgccgccggctgtccggcggcgcgcggagccgtgacccccagcgcttccgccacacattcaacgccgccgccctctccacccgaagtttctaatctttcaaatcccgacccgagctgcggcggcagcggcgaccgctccgcccccacgagacccgcagccgccgcagctgcgttctgccgccggccccattgtcacgcagcccgacgtaggcggt

SEQ ID NO: 11592 - RNA, 4369 nt, Homo sapiens
  source 1..4369: mol_type = other RNA
ctgaatagctgggactacaggtgtacaccactacaagtggctaatttttgtcagtttttgcagagaagagggtctcactatgttgcccaagctggtcttgaaatcctgggctcaagagatcctcccatcttggcctcccgaagtgttgggattacaggcgtgaaccacggtgactagctcaatccaagcttttctgatttctgatgtaatctaattcatggcactttaaatgttttggtgccttggtgtattaacatgtaacatgagaacaagatttatttacttacctcaagaagctagtacatgggttattgaatgcactcttaaactttgagcccctcagatgaaaagcactgtggaaacaattacagctgaagaaaacccttccaatgcctcagaatcctgacttactgtgccttgtgtctcaatggcacattgagaaacaatgtgcactagttagtggcatcacatcccttcatatatgttgtttggcacacaaatgtttatacatttaaaatagctgtcatactacctattcaaaagcatttactagttttctaataaagctaatgaaatgtacccattatggagtactccgtgtcaagtttagagaaactttagctttctctgaagtacatgtaacataataaaaagtttatttaaaaaattgaactagtgttgtatgaagccataagtttttaatgaaaaaaaatgtatgccacagtgtctatatattcatctgaagagtacaaagatggagttctgagaaaaaagggtttatcactatagaaaataaatctggttcttaaattatgttcaaagcaaacattaaaacagtaatgtctcatacactgaaataaagcaattagaggtaataaattataaatacagtagttcaaatattgttttaagcattagtttttctaaacaagttaaattcaaaacattttaaatctgttatattttttcaaagggatgtacaaatgaaagccttcatagaaatctaaaacgataccaccttgtgatcttcatatagaatatgctgaaccttgaccatttttgatttataacatactttggttaatacattatgttccatatgcctttatatttgggaggaatcagattgtgatttgtagcctttacatgcagtttacccaaaccttcttcacatccaggtcttgcttgattctctggagaaggttttgtcagactcataattaaaatgatgcaaactgtaaatgacttcttcagaactgaaaacttcttttttttttaaataaagtgcttttaaattcaaatatatgttgccctaaagaaaactgaaatatactttaaccctgaaatctccgtatcttgacacacacattttaacggaaaaaaaaaaaatcagttttaggccattcatgtccttcaagagagttcagattggatctaaattgggttttgcatcatcatcgtgctcatgtttatacatgaaggttaaaagaaaaagggcaacatccaaggatgaccaataggcagtatgcgacgtgacagctgaccaatagcggctctccacaaggccttctctgagttcaaaatcaatcctgtgatccaactccaatgcagaatcgaggaagccagaactgctatgtggaagggtctgtgtccctacggtggtagcagaaggtgaggcaactggcttcttctcatcttccattgagtcttttgatgtttcagatgactgtgttgtagatgaacgtccaaatcttgagaacaacattcctccaagtccctttccaatgctagcagcccctaatatgcttgctttgcctatatttgttatagattctccatagtgtcggcgggacaaaactggtgaggtcacagggcttggtatggttgaaatgccttcattctctgaaactgaggtaggttctttagctgggttgagaaagcttggcttcatatgttcataaggtaaaggatttgaagtattgtaccagtggatctggacaggtgaaatgttgctgtagtgtttcagtattaatggttctaatctataagccactggatctgtaggatgaaaaatatttagtaaccggttacaaatctctctaggcaaaatatggtcttgacttccagtatttcctgggcggatgccacgcaacgccaagaaaactgctaatggggatcccatacagaagaaattctcaaccttaaattttaaggcaggtgtttgtgtcatagatgatgctttcaatccgtgaagccgttcttctatttccttcagccgtcgtttagttatatagagttcatcaagaagatgtcgttcttcatagctcatccatcgttcatcaggcaactcttcttccttttgcagcaactgttcatacagccgaactggattccagccagtcattatgtcataagtaattacacatcccaaggaatgtgatactattgagactttaccccctttttcttcaaagtctggattccgagaacagaaaagggaatacaatcgattcagctcttgctgaaggcctttaactagttcatctctataaagtggactagtataatacattatgtccattgcactgctgttcagcatatcccttaaacctcgtactttgtcaggagtaatggaatcaacagtgtctccatcaagagtaagttttgaccgccactcaacaggcagaaattcaacatgtgttgcatggttggaaaaatgcctttcttctatttttcttgcagcttctctcatcatagctgtatttttgataattcttccttggtccattttctgcccaatgccatgcacaacaaatacaatatgggtagtctgtgatggcttgtcttctaatgtggcttcttctacataacctctatgaagtctggtaccactacttgatgctttagaaaatcccagtttttgggtaactgttcttgcaattttagatgttgttgcatcactataaagatatacttcatccacactgtgccagtccacatggtttcgactcaacttgaaactatgaacagcttgggaatgctttcgtttaagacctgtcgcatctgtactctccttatatcttctccatttgaacagagaagggagggagaagggagggaggtggtagacaacatcttttccatctatggattttgacacttcaatatcgaaattttcctgcatctgctggcccctaaaacaattgagatgttcttgctcaattaaattactttcttcctcttctagaggctgccaagtgccgtcaataaaccactgtccacgcattactggtattttatcagcctggttccagtacaccgggtagcactctccttgggtcacatccacctcgtagaggccgccccgcacgcacacaggctcgatgttcacaagctccaccatctccggctcgtgccccgtcgtactctggcagaagccgcaggcgcggtcctcatcgtcatcttctccggaactggaggctgggcccgtgggggagcacacatggtcgccgtcccggtccccgccctggggccgggcacccgtggtctgcagcagggtccggaaggcgagctcgatgcggagcgagtcgtagccgatgaagggcttccaggtcttcttgtcctccttgtagaaccagcgtacctcctccgggcccagctccgtcactacctcatagcggtgccgggccgccgggccgccaagccgggtacgtttcctttccccgggggaccctcctgtcgcgccgccgccccccgagttcgtcgggaccagcggaggctgctgcggcgggtgcagcgacaaggagctgccgccgccgccgctctcaccctcgctgtagtagcgcagcgaggagcccgactcggcggagctgaagtcatagttctcgtcactgaggcaggggtccagcgcgaggtggtggttgtggtcgtcggtgcccggcgccaaatgcagcccgggttccccgcgcagcagggccaggggcacgtcgccgtcgtccgggtccccgccgggcaggtgctcgaagcagcagacgccgccgccgaacgctggcctcgcgtctgagcccagctcccaggcgccgccgccgccgcctcggccgttatgctcggggctccgtggggacccgcggcccgggtaattcatgctgtggagacgccgccggctgtccggcggcgcgcggagccgtgacccccagcgcttccgccacacattcaacgccgccgccctctccacccgaagtttctaatctttcaaatcccgacccgagctgcggcggcagcggcgaccgctccgcccccacgagacccgcagccgccgcagctgcgttctgccgccggccccattgtcacgcagcccgacgtaggcggt

SEQ ID NO: 11593 - RNA, 4222 nt, Homo sapiens
  source 1..4222: mol_type = other RNA
ctgaatagctgggactacaggtgtacaccactacaagtggctaatttttgtcagtttttgcagagaagagggtctcactatgttgcccaagctggtcttgaaatcctgggctcaagagatcctcccatcttggcctcccgaagtgttgggattacaggcgtgaaccacggtgactagctcaatccaagcttttctgatttctgatgtaatctaattcatggcactttaaatgttttggtgccttggtgtattaacatgtaacatgagaacaagatttatttacttacctcaagaagctagtacatgggttattgaatgcactcttaaactttgagcccctcagatgaaaagcactgtggaaacaattacagctgaagaaaacccttccaatgcctcagaatcctgacttactgtgccttgtgtctcaatggcacattgagaaacaatgtgcactagttagtggcatcacatcccttcatatatgttgtttggcacacaaatgtttatacatttaaaatagctgtcatactacctattcaaaagcatttactagttttctaataaagctaatgaaatgtacccattatggagtactccgtgtcaagtttagagaaactttagctttctctgaagtacatgtaacataataaaaagtttatttaaaaaattgaactagtgttgtatgaagccataagtttttaatgaaaaaaaatgtatgccacagtgtctatatattcatctgaagagtacaaagatggagttctgagaaaaaagggtttatcactatagaaaataaatctggttcttaaattatgttcaaagcaaacattaaaacagtaatgtctcatacactgaaataaagcaattagaggtaataaattataaatacagtagttcaaatattgttttaagcattagtttttctaaacaagttaaattcaaaacattttaaatctgttatattttttcaaagggatgtacaaatgaaagccttcatagaaatctaaaacgataccaccttgtgatcttcatatagaatatgctgaaccttgaccatttttgatttataacatactttggttaatacattatgttccatatgcctttatatttgggaggaatcagattgtgatttgtagcctttacatgcagtttacccaaaccttcttcacatccaggtcttgcttgattctctggagaaggttttgtcagactcataattaaaatgatgcaaactgtaaatgacttcttcagaactgaaaacttcttttttttttaaataaagtgcttttaaattcaaatatatgttgccctaaagaaaactgaaatatactttaaccctgaaatctccgtatcttgacacacacattttaacggaaaaaaaaaaaatcagttttaggccattcatgtccttcaagagagttcagattggatctaaattgggttttgcatcatcatcgtgctcatgtttatacatgaaggttaaaagaaaaagggcaacatccaaggatgaccaataggcagtatgcgacgtgacagctgaccaatagcggctctccacaaggccttctctgagttcaaaatcaatcctgtgatccaactccacgagggcattatctttattctgcattacattttccggaaaaagaagttgtgggagattaaagaacgattcttgaagtctgaaatatgcagaatcgaggaagccagaactgctatgtggaagggtctgtgtccctacggtggtagcagaaggtgaggcaactggcttcttctcatcttccattgagtcttttgatgtttcagatgactgtgttgtagatgaacgtccaaatcttgagaacaacattcctccaagtccctttccaatgctagcagcccctaatatgcttgctttgcctatatttgttatagattctccatagtgtcggcgggacaaaactggtgaggtcacagggcttggtatggttgaaatgccttcattctctgaaactgaggtaggttctttagctgggttgagaaagcttggcttcatatgttcataaggtaaaggatttgaagtattgtaccagtggatctggacaggtgaaatgttgctgtagtgtttcagtattaatggttctaatctataagccactggatctgtaggatgaaaaatatttagtaaccggttacaaatctctctaggcaaaatatggtcttgacttccagtatttcctgggcggatgccacgcaacgccaagaaaactgctaatggggatcccatacagaagaaattctcaaccttaaattttaaggcaggtgtttgtgtcatagatgatgctttcaatccgtgaagccgttcttctatttccttcagccgtcgtttagttatatagagttcatcaagaagatgtcgttcttcatagctcatccatcgttcatcaggcaactcttcttccttttgcagcaactgttcatacagccgaactggattccagccagtcattatgtcataagtaattacacatcccaaggaatgtgatactattgagactttaccccctttttcttcaaagtctggattccgagaacagaaaagggaatacaatcgattcagctcttgctgaaggcctttaactagttcatctctataaagtggactagtataatacattatgtccattgcactgctgttcagcatatcccttaaacctcgtactttgtcaggagtaatggaatcaacagtgtctccatcaagagtaagttttgaccgccactcaacaggcagaaattcaacatgtgttgcatggttggaaaaatgcctttcttctatttttcttgcagcttctctcatcatagctgtatttttgataattcttccttggtccattttctgcccaatgccatgcacaacaaatacaatatgggtagtctgtgatggcttgtcttctaatgtggcttcttctacataacctctatgaagtctggtaccactacttgatgcatcttttccatctatggattttgacacttcaatatcgaaattttcctgcatctgctggcccctaaaacaattgagatgttcttgctcaattaaattactttcttcctcttctagaggctgccaagtgccgtcaataaaccactgtccacgcattactggtattttatcagcctggttccagtacaccgggtagcactctccttgggtcacatccacctcgtagaggccgccccgcacgcacacaggctcgatgttcacaagctccaccatctccggctcgtgccccgtcgtactctggcagaagccgcaggcgcggtcctcatcgtcatcttctccggaactggaggctgggcccgtgggggagcacacatggtcgccgtcccggtccccgccctggggccgggcacccgtggtctgcagcagggtccggaaggcgagctcgatgcggagcgagtcgtagccgatgaagggcttccaggtcttcttgtcctccttgtagaaccagcgtacctcctccgggcccagctccgtcactacctcatagcggtgccgggccgccgggccgccaagccgggtacgtttcctttccccgggggaccctcctgtcgcgccgccgccccccgagttcgtcgggaccagcggaggctgctgcggcgggtgcagcgacaaggagctgccgccgccgccgctctcaccctcgctgtagtagcgcagcgaggagcccgactcggcggagctgaagtcatagttctcgtcactgaggcaggggtccagcgcgaggtggtggttgtggtcgtcggtgcccggcgccaaatgcagcccgggttccccgcgcagcagggccaggggcacgtcgccgtcgtccgggtccccgccgggcaggtgctcgaagcagcagacgccgccgccgaacgctggcctcgcgtctgagcccagctcccaggcgccgccgccgccgcctcggccgttatgctcggggctccgtggggacccgcggcccgggtaattcatgctgtggagacgccgccggctgtccggcggcgcgcggagccgtgacccccagcgcttccgccacacattcaacgccgccgccctctccacccgaagtttctaatctttcaaatcccgacccgagctgcggcggcagcggcgaccgctccgcccccacgagacccgcagccgccgcagctgcgttctgccgccggccccattgtcacgcagcccgacgtaggcggt

SEQ ID NO: 11594 - RNA, 4372 nt, Homo sapiens
  source 1..4372: mol_type = other RNA
ctgaatagctgggactacaggtgtacaccactacaagtggctaatttttgtcagtttttgcagagaagagggtctcactatgttgcccaagctggtcttgaaatcctgggctcaagagatcctcccatcttggcctcccgaagtgttgggattacaggcgtgaaccacggtgactagctcaatccaagcttttctgatttctgatgtaatctaattcatggcactttaaatgttttggtgccttggtgtattaacatgtaacatgagaacaagatttatttacttacctcaagaagctagtacatgggttattgaatgcactcttaaactttgagcccctcagatgaaaagcactgtggaaacaattacagctgaagaaaacccttccaatgcctcagaatcctgacttactgtgccttgtgtctcaatggcacattgagaaacaatgtgcactagttagtggcatcacatcccttcatatatgttgtttggcacacaaatgtttatacatttaaaatagctgtcatactacctattcaaaagcatttactagttttctaataaagctaatgaaatgtacccattatggagtactccgtgtcaagtttagagaaactttagctttctctgaagtacatgtaacataataaaaagtttatttaaaaaattgaactagtgttgtatgaagccataagtttttaatgaaaaaaaatgtatgccacagtgtctatatattcatctgaagagtacaaagatggagttctgagaaaaaagggtttatcactatagaaaataaatctggttcttaaattatgttcaaagcaaacattaaaacagtaatgtctcatacactgaaataaagcaattagaggtaataaattataaatacagtagttcaaatattgttttaagcattagtttttctaaacaagttaaattcaaaacattttaaatctgttatattttttcaaagggatgtacaaatgaaagccttcatagaaatctaaaacgataccaccttgtgatcttcatatagaatatgctgaaccttgaccatttttgatttataacatactttggttaatacattatgttccatatgcctttatatttgggaggaatcagattgtgatttgtagcctttacatgcagtttacccaaaccttcttcacatccaggtcttgcttgattctctggagaaggttttgtcagactcataattaaaatgatgcaaactgtaaatgacttcttcagaactgaaaacttcttttttttttaaataaagtgcttttaaattcaaatatatgttgccctaaagaaaactgaaatatactttaaccctgaaatctccgtatcttgacacacacattttaacggaaaaaaaaaaaatcagttttaggccattcatgtccttcaagagagttcagattggatctaaattgggttttgcatcatcatcgtgctcatgtttatacatgaaggttaaaagaaaaagggcaacatccaaggatgaccaataggcagtatgcgacgtgacagctgaccaatagcggctctccacaaggccttctctgagttcaaaatcaatcctgtgatccaactccacgagggcattatctttattctgcattacattttccggaaaaagaagttgtgggagattaaagaacgattcttgaagtctgaaatatgcagaatcgaggaagccagaactgctatgtggaagggtctgtgtccctacggtggtagcagaaggtgaggcaactggcttcttctcatcttccattgagtcttttgatgtttcagatgactgtgttgtagatgaacgtccaaatcttgagaacaacattcctccaagtccctttccaatgctagcagcccctaatatgcttgctttgcctatatttgttatagattctccatagtgtcggcgggacaaaactggtgaggtcacagggcttggtatggttgaaatgccttcattctctgaaactgaggtaggttctttagctgggttgagaaagcttggcttcatatgttcataaggtaaaggatttgaagtattgtaccagtggatctggacaggtgaaatgttgctgtagtgtttcagtattaatggttctaatctataagccactggatctgtaggatgaaaaatatttagtaaccggttacaaatctctctaggcaaaatatggtcttgacttccagtatttcctgggcggatgccacgcaacgccaagaaaactgctaatggggatcccatacagaagaaattctcaaccttaaattttaaggcaggtgtttgtgtcatagatgatgctttcaatccgtgaagccgttcttctatttccttcagccgtcgtttagttatatagagttcatcaagaagatgtcgttcttcatagctcatccatcgttcatcaggcaactcttcttccttttgcagcaactgttcatacagccgaactggattccagccagtcattatgtcataagtaattacacatcccaaggaatgtgatactattgagactttaccccctttttcttcaaagtctggattccgagaacagaaaagggaatacaatcgattcagctcttgctgaaggcctttaactagttcatctctataaagtggactagtataatacattatgtccattgcactgctgttcagcatatcccttaaacctcgtactttgtcaggagtaatggaatcaacagtgtctccatcaagagtaagttttgaccgccactcaacaggcagaaattcaacatgtgttgcatggttggaaaaatgcctttcttctatttttcttgcagcttctctcatcatagctgtatttttgataattcttccttggtccattttctgcccaatgccatgcacaacaaatacaatatgggtagtctgtgatggcttgtcttctaatgtggcttcttctacataacctctatgaagtctggtaccactacttgatgctttagaaaatcccagtttttgggtaactgttcttgcaattttagatgttgttgcatcactataaagatatacttcatccacactgtgccagtccacatggtttcgactcaacttgaaactatgaacagcagaatagttgatcccactgccatcttttccatctatggattttgacacttcaatatcgaaattttcctgcatctgctggcccctaaaacaattgagatgttcttgctcaattaaattactttcttcctcttctagaggctgccaagtgccgtcaataaaccactgtccacgcattactggtattttatcagcctggttccagtacaccgggtagcactctccttgggtcacatccacctcgtagaggccgccccgcacgcacacaggctcgatgttcacaagctccaccatctccggctcgtgccccgtcgtactctggcagaagccgcaggcgcggtcctcatcgtcatcttctccggaactggaggctgggcccgtgggggagcacacatggtcgccgtcccggtccccgccctggggccgggcacccgtggtctgcagcagggtccggaaggcgagctcgatgcggagcgagtcgtagccgatgaagggcttccaggtcttcttgtcctccttgtagaaccagcgtacctcctccgggcccagctccgtcactacctcatagcggtgccgggccgccgggccgccaagccgggtacgtttcctttccccgggggaccctcctgtcgcgccgccgccccccgagttcgtcgggaccagcggaggctgctgcggcgggtgcagcgacaaggagctgccgccgccgccgctctcaccctcgctgtagtagcgcagcgaggagcccgactcggcggagctgaagtcatagttctcgtcactgaggcaggggtccagcgcgaggtggtggttgtggtcgtcggtgcccggcgccaaatgcagcccgggttccccgcgcagcagggccaggggcacgtcgccgtcgtccgggtccccgccgggcaggtgctcgaagcagcagacgccgccgccgaacgctggcctcgcgtctgagcccagctcccaggcgccgccgccgccgcctcggccgttatgctcggggctccgtggggacccgcggcccgggtaattcatgctgtggagacgccgccggctgtccggcggcgcgcggagccgtgacccccagcgcttccgccacacattcaacgccgccgccctctccacccgaagtttctaatctttcaaatcccgacccgagctgcggcggcagcggcgaccgctccgcccccacgagacccgcagccgccgcagctgcgttctgccgccggccccattgtcacgcagcccgacgtaggcggt

SEQ ID NO: 11595 - RNA, 4351 nt, Homo sapiens
  source 1..4351: mol_type = other RNA
ctgaatagctgggactacaggtgtacaccactacaagtggctaatttttgtcagtttttgcagagaagagggtctcactatgttgcccaagctggtcttgaaatcctgggctcaagagatcctcccatcttggcctcccgaagtgttgggattacaggcgtgaaccacggtgactagctcaatccaagcttttctgatttctgatgtaatctaattcatggcactttaaatgttttggtgccttggtgtattaacatgtaacatgagaacaagatttatttacttacctcaagaagctagtacatgggttattgaatgcactcttaaactttgagcccctcagatgaaaagcactgtggaaacaattacagctgaagaaaacccttccaatgcctcagaatcctgacttactgtgccttgtgtctcaatggcacattgagaaacaatgtgcactagttagtggcatcacatcccttcatatatgttgtttggcacacaaatgtttatacatttaaaatagctgtcatactacctattcaaaagcatttactagttttctaataaagctaatgaaatgtacccattatggagtactccgtgtcaagtttagagaaactttagctttctctgaagtacatgtaacataataaaaagtttatttaaaaaattgaactagtgttgtatgaagccataagtttttaatgaaaaaaaatgtatgccacagtgtctatatattcatctgaagagtacaaagatggagttctgagaaaaaagggtttatcactatagaaaataaatctggttcttaaattatgttcaaagcaaacattaaaacagtaatgtctcatacactgaaataaagcaattagaggtaataaattataaatacagtagttcaaatattgttttaagcattagtttttctaaacaagttaaattcaaaacattttaaatctgttatattttttcaaagggatgtacaaatgaaagccttcatagaaatctaaaacgataccaccttgtgatcttcatatagaatatgctgaaccttgaccatttttgatttataacatactttggttaatacattatgttccatatgcctttatatttgggaggaatcagattgtgatttgtagcctttacatgcagtttacccaaaccttcttcacatccaggtcttgcttgattctctggagaaggttttgtcagactcataattaaaatgatgcaaactgtaaatgacttcttcagaactgaaaacttcttttttttttaaataaagtgcttttaaattcaaatatatgttgccctaaagaaaactgaaatatactttaaccctgaaatctccgtatcttgacacacacattttaacggaaaaaaaaaaaatcagttttaggccattcatgtccttcaagagagttcagattggatctaaattgggttttgcatcatcatcgtgctcatgtttatacatgaaggttaaaagaaaaagggcaacatccaaggatgaccaataggcagtatgcgacgtgacagctgaccaatagcggctctccacaaggccttctctgagttcaaaatcaatcctgtgatccaactccacgagggcattatctttattctgcattacattttccggaaaaagaagttgtgggagattaaagaacgattcttgaagtctgaaatatgcagaatcgaggaagccagaactgctatgtggaagggtctgtgtccctacggtggtagcagaaggtgaggcaactggcttcttctcatcttccattgagtcttttgatgtttcagatgactgtgttgtagatgaacgtccaaatcttgagaacaacattcctccaagtccctttccaatgctagcagcccctaatatgcttgctttgcctatatttgttatagattctccatagtgtcggcgggacaaaactggtgaggtcacagggcttggtatggttgaaatgccttcattctctgaaactgaggtaggttctttagctgggttgagaaagcttggcttcatatgttcataaggtaaaggatttgaagtattgtaccagtggatctggacaggtgaaatgttgctgtagtgtttcagtattaatggttctaatctataagccactggatctgtaggatgaaaaatatttagtaaccggttacaaatctctctaggcaaaatatggtcttgacttccagtatttcctgggcggatgccacgcaacgccaagaaaactgctaatggggatcccatacagaagaaattctcaaccttaaattttaaggcaggtgtttgtgtcatagatgatgctttcaatccgtgaagccgttcttctatttccttcagccgtcgtttagttatatagagttcatcaagaagatgtcgttcttcatagctcatccatcgttcatcaggcaactcttcttccttttgcagcaactgttcatacagccgaactggattccagccagtcattatgtcataagtaattacacatcccaaggaatgtgatactattgagactttaccccctttttcttcaaagtctggattccgagaacagaaaagggaatacaatcgattcagctcttgctgaaggcctttaactagttcatctctataaagtggactagtataatacattatgtccattgcactgctgttcagcatatcccttaaacctcgtactttgtcaggagtaatggaatcaacagtgtctccatcaagagtaagttttgaccgccactcaacaggcagaaattcaacatgtgttgcatggttggaaaaatgcctttcttctatttttcttgcagcttctctcatcatagctgtatttttgataattcttccttggtccattttctgcccaatgccatgcacaacaaatacaatatgggtagtctgtgatggcttgtcttctaatgtggcttcttctacataacctctatgaagtctggtaccactacttgatgctttagaaaatcccagtttttgggtaactgttcttgcaattttagatgttgttgcatcactataaagatatacttcatccacactgtgccagtccacatggtttcgactcaacttgaaactatgaacagcatcttttccatctatggattttgacacttcaatatcgaaattttcctgcatctgctggcccctaaaacaattgagatgttcttgctcaattaaattactttcttcctcttctagaggctgccaagtgccgtcaataaaccactgtccacgcattactggtattttatcagcctggttccagtacaccgggtagcactctccttgggtcacatccacctcgtagaggccgccccgcacgcacacaggctcgatgttcacaagctccaccatctccggctcgtgccccgtcgtactctggcagaagccgcaggcgcggtcctcatcgtcatcttctccggaactggaggctgggcccgtgggggagcacacatggtcgccgtcccggtccccgccctggggccgggcacccgtggtctgcagcagggtccggaaggcgagctcgatgcggagcgagtcgtagccgatgaagggcttccaggtcttcttgtcctccttgtagaaccagcgtacctcctccgggcccagctccgtcactacctcatagcggtgccgggccgccgggccgccaagccgggtacgtttcctttccccgggggaccctcctgtcgcgccgccgccccccgagttcgtcgggaccagcggaggctgctgcggcgggtgcagcgacaaggagctgccgccgccgccgctctcaccctcgctgtagtagcgcagcgaggagcccgactcggcggagctgaagtcatagttctcgtcactgaggcaggggtccagcgcgaggtggtggttgtggtcgtcggtgcccggcgccaaatgcagcccgggttccccgcgcagcagggccaggggcacgtcgccgtcgtccgggtccccgccgggcaggtgctcgaagcagcagacgccgccgccgaacgctggcctcgcgtctgagcccagctcccaggcgccgccgccgccgcctcggccgttatgctcggggctccgtggggacccgcggcccgggtaattcatgctgtggagacgccgccggctgtccggcggcgcgcggagccgtgacccccagcgcttccgccacacattcaacgccgccgccctctccacccgaagtttctaatctttcaaatcccgacccgagctgcggcggcagcggcgaccgctccgcccccacgagacccgcagccgccgcagctgcgttctgccgccggccccattgtcacgcagcccgacgtaggcggt

SEQ ID NO: 11596 - RNA, 4474 nt, Homo sapiens
  source 1..4474: mol_type = other RNA
ctgaatagctgggactacaggtgtacaccactacaagtggctaatttttgtcagtttttgcagagaagagggtctcactatgttgcccaagctggtcttgaaatcctgggctcaagagatcctcccatcttggcctcccgaagtgttgggattacaggcgtgaaccacggtgactagctcaatccaagcttttctgatttctgatgtaatctaattcatggcactttaaatgttttggtgccttggtgtattaacatgtaacatgagaacaagatttatttacttacctcaagaagctagtacatgggttattgaatgcactcttaaactttgagcccctcagatgaaaagcactgtggaaacaattacagctgaagaaaacccttccaatgcctcagaatcctgacttactgtgccttgtgtctcaatggcacattgagaaacaatgtgcactagttagtggcatcacatcccttcatatatgttgtttggcacacaaatgtttatacatttaaaatagctgtcatactacctattcaaaagcatttactagttttctaataaagctaatgaaatgtacccattatggagtactccgtgtcaagtttagagaaactttagctttctctgaagtacatgtaacataataaaaagtttatttaaaaaattgaactagtgttgtatgaagccataagtttttaatgaaaaaaaatgtatgccacagtgtctatatattcatctgaagagtacaaagatggagttctgagaaaaaagggtttatcactatagaaaataaatctggttcttaaattatgttcaaagcaaacattaaaacagtaatgtctcatacactgaaataaagcaattagaggtaataaattataaatacagtagttcaaatattgttttaagcattagtttttctaaacaagttaaattcaaaacattttaaatctgttatattttttcaaagggatgtacaaatgaaagccttcatagaaatctaaaacgataccaccttgtgatcttcatatagaatatgctgaaccttgaccatttttgatttataacatactttggttaatacattatgttccatatgcctttatatttgggaggaatcagattgtgatttgtagcctttacatgcagtttacccaaaccttcttcacatccaggtcttgcttgattctctggagaaggttttgtcagactcataattaaaatgatgcaaactgtaaatgacttcttcagaactgaaaacttcttttttttttaaataaagtgcttttaaattcaaatatatgttgccctaaagaaaactgaaatatactttaaccctgaaatctccgtatcttgacacacacattttaacggaaaaaaaaaaaatcagttttaggccattcatgtccttcaagagagttcagattggatctaaattgggttttgcatcatcatcgtgctcatgtttatacatgaaggttaaaagaaaaagggcaacatccaaggatgaccaataggcagtatgcgacgtgacagctgaccaatagcggctctccacaaggccttctctgagttcaaaatcaatcctgtgatccaactccacgagggcattatctttattctgcattacattttccggaaaaagaagttgtgggagattaaagaacgattcttgaagtctgaaatatgcagaatcgaggaagccagaactgctatgtggaagggtctgtgtccctacggtggtagcagaaggtgaggcaactggcttcttctcatcttccattgagtcttttgatgtttcagatgactgtgttgtagatgaacgtccaaatcttgagaacaacattcctccaagtccctttccaatgctagcagcccctaatatgcttgctttgcctatatttgttatagattctccatagtgtcggcgggacaaaactggtgaggtcacagggcttggtatggttgaaatgccttcattctctgaaactgaggtaggttctttagctgggttgagaaagcttggcttcatatgttcataaggtaaaggatttgaagtattgtaccagtggatctggacaggtgaaatgttgctgtagtgtttcagtattaatggttctaatctataagccactggatctgtaggatgaaaaatatttagtaaccggttacaaatctctctaggcaaaatatggtcttgacttccagtatttcctgggcggatgccacgcaacgccaagaaaactgctaatggggatcccatacagaagaaattctcaaccttaaattttaaggcaggtgtttgtgtcatagatgatgctttcaatccgtgaagccgttcttctatttccttcagccgtcgtttagttatatagagttcatcaagaagatgtcgttcttcatagctcatccatcgttcatcaggcaactcttcttccttttgcagcaactgttcatacagccgaactggattccagccagtcattatgtcataagtaattacacatcccaaggaatgtgatactattgagactttaccccctttttcttcaaagtctggattccgagaacagaaaagggaatacaatcgattcagctcttgctgaaggcctttaactagttcatctctataaagtggactagtataatacattatgtccattgcactgctgttcagcatatcccttaaacctcgtactttgtcaggagtaatggaatcaacagtgtctccatcaagagtaagttttgaccgccactcaacaggcagaaattcaacatgtgttgcatggttggaaaaatgcctttcttctatttttcttgcagcttctctcatcatagctgtatttttgataattcttccttggtccattttctgcccaatgccatgcacaacaaatacaatatgggtagtctgtgatggcttgtcttctaatgtggcttcttctacataacctctatgaagtctggtaccactacttgatgctttagaaaatcccagtttttgggtaactgttcttgcaattttagatgttgttgcatcactataaagatatacttcatccacactgtgccagtccacatggtttcgactcaacttgaaactatgaacagcttgggaatgctttcgtttaagacctgtcgcatctgtactctccttatatcttctccatttgaacagagaagggagggagaagggagggaggtggtagacaacagaatagttgatcccactgccatcttttccatctatggattttgacacttcaatatcgaaattttcctgcatctgctggcccctaaaacaattgagatgttcttgctcaattaaattactttcttcctcttctagaggctgccaagtgccgtcaataaaccactgtccacgcattactggtattttatcagcctggttccagtacaccgggtagcactctccttgggtcacatccacctcgtagaggccgccccgcacgcacacaggctcgatgttcacaagctccaccatctccggctcgtgccccgtcgtactctggcagaagccgcaggcgcggtcctcatcgtcatcttctccggaactggaggctgggcccgtgggggagcacacatggtcgccgtcccggtccccgccctggggccgggcacccgtggtctgcagcagggtccggaaggcgagctcgatgcggagcgagtcgtagccgatgaagggcttccaggtcttcttgtcctccttgtagaaccagcgtacctcctccgggcccagctccgtcactacctcatagcggtgccgggccgccgggccgccaagccgggtacgtttcctttccccgggggaccctcctgtcgcgccgccgccccccgagttcgtcgggaccagcggaggctgctgcggcgggtgcagcgacaaggagctgccgccgccgccgctctcaccctcgctgtagtagcgcagcgaggagcccgactcggcggagctgaagtcatagttctcgtcactgaggcaggggtccagcgcgaggtggtggttgtggtcgtcggtgcccggcgccaaatgcagcccgggttccccgcgcagcagggccaggggcacgtcgccgtcgtccgggtccccgccgggcaggtgctcgaagcagcagacgccgccgccgaacgctggcctcgcgtctgagcccagctcccaggcgccgccgccgccgcctcggccgttatgctcggggctccgtggggacccgcggcccgggtaattcatgctgtggagacgccgccggctgtccggcggcgcgcggagccgtgacccccagcgcttccgccacacattcaacgccgccgccctctccacccgaagtttctaatctttcaaatcccgacccgagctgcggcggcagcggcgaccgctccgcccccacgagacccgcagccgccgcagctgcgttctgccgccggccccattgtcacgcagcccgacgtaggcggt

SEQ ID NO: 11597 - RNA, 4453 nt, Homo sapiens
  source 1..4453: mol_type = other RNA
ctgaatagctgggactacaggtgtacaccactacaagtggctaatttttgtcagtttttgcagagaagagggtctcactatgttgcccaagctggtcttgaaatcctgggctcaagagatcctcccatcttggcctcccgaagtgttgggattacaggcgtgaaccacggtgactagctcaatccaagcttttctgatttctgatgtaatctaattcatggcactttaaatgttttggtgccttggtgtattaacatgtaacatgagaacaagatttatttacttacctcaagaagctagtacatgggttattgaatgcactcttaaactttgagcccctcagatgaaaagcactgtggaaacaattacagctgaagaaaacccttccaatgcctcagaatcctgacttactgtgccttgtgtctcaatggcacattgagaaacaatgtgcactagttagtggcatcacatcccttcatatatgttgtttggcacacaaatgtttatacatttaaaatagctgtcatactacctattcaaaagcatttactagttttctaataaagctaatgaaatgtacccattatggagtactccgtgtcaagtttagagaaactttagctttctctgaagtacatgtaacataataaaaagtttatttaaaaaattgaactagtgttgtatgaagccataagtttttaatgaaaaaaaatgtatgccacagtgtctatatattcatctgaagagtacaaagatggagttctgagaaaaaagggtttatcactatagaaaataaatctggttcttaaattatgttcaaagcaaacattaaaacagtaatgtctcatacactgaaataaagcaattagaggtaataaattataaatacagtagttcaaatattgttttaagcattagtttttctaaacaagttaaattcaaaacattttaaatctgttatattttttcaaagggatgtacaaatgaaagccttcatagaaatctaaaacgataccaccttgtgatcttcatatagaatatgctgaaccttgaccatttttgatttataacatactttggttaatacattatgttccatatgcctttatatttgggaggaatcagattgtgatttgtagcctttacatgcagtttacccaaaccttcttcacatccaggtcttgcttgattctctggagaaggttttgtcagactcataattaaaatgatgcaaactgtaaatgacttcttcagaactgaaaacttcttttttttttaaataaagtgcttttaaattcaaatatatgttgccctaaagaaaactgaaatatactttaaccctgaaatctccgtatcttgacacacacattttaacggaaaaaaaaaaaatcagttttaggccattcatgtccttcaagagagttcagattggatctaaattgggttttgcatcatcatcgtgctcatgtttatacatgaaggttaaaagaaaaagggcaacatccaaggatgaccaataggcagtatgcgacgtgacagctgaccaatagcggctctccacaaggccttctctgagttcaaaatcaatcctgtgatccaactccacgagggcattatctttattctgcattacattttccggaaaaagaagttgtgggagattaaagaacgattcttgaagtctgaaatatgcagaatcgaggaagccagaactgctatgtggaagggtctgtgtccctacggtggtagcagaaggtgaggcaactggcttcttctcatcttccattgagtcttttgatgtttcagatgactgtgttgtagatgaacgtccaaatcttgagaacaacattcctccaagtccctttccaatgctagcagcccctaatatgcttgctttgcctatatttgttatagattctccatagtgtcggcgggacaaaactggtgaggtcacagggcttggtatggttgaaatgccttcattctctgaaactgaggtaggttctttagctgggttgagaaagcttggcttcatatgttcataaggtaaaggatttgaagtattgtaccagtggatctggacaggtgaaatgttgctgtagtgtttcagtattaatggttctaatctataagccactggatctgtaggatgaaaaatatttagtaaccggttacaaatctctctaggcaaaatatggtcttgacttccagtatttcctgggcggatgccacgcaacgccaagaaaactgctaatggggatcccatacagaagaaattctcaaccttaaattttaaggcaggtgtttgtgtcatagatgatgctttcaatccgtgaagccgttcttctatttccttcagccgtcgtttagttatatagagttcatcaagaagatgtcgttcttcatagctcatccatcgttcatcaggcaactcttcttccttttgcagcaactgttcatacagccgaactggattccagccagtcattatgtcataagtaattacacatcccaaggaatgtgatactattgagactttaccccctttttcttcaaagtctggattccgagaacagaaaagggaatacaatcgattcagctcttgctgaaggcctttaactagttcatctctataaagtggactagtataatacattatgtccattgcactgctgttcagcatatcccttaaacctcgtactttgtcaggagtaatggaatcaacagtgtctccatcaagagtaagttttgaccgccactcaacaggcagaaattcaacatgtgttgcatggttggaaaaatgcctttcttctatttttcttgcagcttctctcatcatagctgtatttttgataattcttccttggtccattttctgcccaatgccatgcacaacaaatacaatatgggtagtctgtgatggcttgtcttctaatgtggcttcttctacataacctctatgaagtctggtaccactacttgatgctttagaaaatcccagtttttgggtaactgttcttgcaattttagatgttgttgcatcactataaagatatacttcatccacactgtgccagtccacatggtttcgactcaacttgaaactatgaacagcttgggaatgctttcgtttaagacctgtcgcatctgtactctccttatatcttctccatttgaacagagaagggagggagaagggagggaggtggtagacaacatcttttccatctatggattttgacacttcaatatcgaaattttcctgcatctgctggcccctaaaacaattgagatgttcttgctcaattaaattactttcttcctcttctagaggctgccaagtgccgtcaataaaccactgtccacgcattactggtattttatcagcctggttccagtacaccgggtagcactctccttgggtcacatccacctcgtagaggccgccccgcacgcacacaggctcgatgttcacaagctccaccatctccggctcgtgccccgtcgtactctggcagaagccgcaggcgcggtcctcatcgtcatcttctccggaactggaggctgggcccgtgggggagcacacatggtcgccgtcccggtccccgccctggggccgggcacccgtggtctgcagcagggtccggaaggcgagctcgatgcggagcgagtcgtagccgatgaagggcttccaggtcttcttgtcctccttgtagaaccagcgtacctcctccgggcccagctccgtcactacctcatagcggtgccgggccgccgggccgccaagccgggtacgtttcctttccccgggggaccctcctgtcgcgccgccgccccccgagttcgtcgggaccagcggaggctgctgcggcgggtgcagcgacaaggagctgccgccgccgccgctctcaccctcgctgtagtagcgcagcgaggagcccgactcggcggagctgaagtcatagttctcgtcactgaggcaggggtccagcgcgaggtggtggttgtggtcgtcggtgcccggcgccaaatgcagcccgggttccccgcgcagcagggccaggggcacgtcgccgtcgtccgggtccccgccgggcaggtgctcgaagcagcagacgccgccgccgaacgctggcctcgcgtctgagcccagctcccaggcgccgccgccgccgcctcggccgttatgctcggggctccgtggggacccgcggcccgggtaattcatgctgtggagacgccgccggctgtccggcggcgcgcggagccgtgacccccagcgcttccgccacacattcaacgccgccgccctctccacccgaagtttctaatctttcaaatcccgacccgagctgcggcggcagcggcgaccgctccgcccccacgagacccgcagccgccgcagctgcgttctgccgccggccccattgtcacgcagcccgacgtaggcggt

SEQ ID NO: 11598 - RNA, 11921 nt, Homo sapiens
  source 1..11921: mol_type = other RNA
ctgaatagctgggactacaggtgtacactaccacacccagctaacaactcattctaaagaaactgttttaactattttaaccttagccattttaaatttataggtaccaaattcaggtcagcttcaaatttgggacggtacagaaaatagttaaattgtatttgtttccgaggacaaaatgagcaacagaggaacaaaggactttttcctttgttgaggccactcctattctaaacttgtaactagggtgtttcaatctgactgtatataaatcaaaacaaaaatttagcttgagattatttccatttactcccaggttgatttaaccaaattaaagataatttgcatttttgatggccctaagttaattttaatcccaaactagataaatatttcattaaaaaccaggaatactgcatctaggtatttttagattaagtggctaatctgtttttctaataattcttatatataattgcagccctttaaataaaactagcttttgcagtagactgattaaaatccactgagtcaagaaatacctaagaatacatttttactcaataccatcttatcatgtgggctgctgacttaaaaatatgtggttttctgtttcaaataagattgttcttgttacattccctgaatcacacccaatttatatttcaaaaatcagttagaggccggacatggtggctcacacctgtaatctcagcactttggaaggctgaggcgggtgtatcacctgaggttaggagttcgagaccagcctgaccaaaatgaaaccccatctcttctaaaaatacaaaaattagccgggcatggtggcatacctctgtaatcccagctactcaggaggctgaggcatgagaactctttgaactctggaggcggagattgcagtgggccgagattgcaccactgcactccagcctgggtgacagagtggaactctgtctcaaaaaagaaagaaggaaaaaaatcagcgaggttggaaaaaatcacttcaagttaataatatatatatttttacttttgaaattttttataagtaaaatgaatacattacaatcaaacacagaacacatattaagtggacaataaatattttaatttgccttttgtgtgtatgtgagtgtgagtgtgttccatggtggtttatgttttagatatgtgtggtattacaggacaaagaaattaactcccccatgctcaaaatgtgatttccccctccctgtctaagcattgcaagaatgcagaccataatcacacaatgcatactttatcatatgaggccaaaacagcattttcctctcctgtgcctctggtctgatggatacccagggaaacaaatgttatctatgaatggtcttttctgcctgcccaaacatgtctgtctattatcaggactggcctggcaggacctggtttctgatcctaaccagctgtgtgagaactagaaacgtcatttcatctgtcacatggagttggactagactatctctcctgtcccttctaactttcaaatctcttgatttaatggttctgtcctatatgtatcctgatttcttttttttttttttttttttttttgagatggagttttgctctcgttgcccaggctgaagtgcagtggtgtgatctcagctcactgcaacctccacctcctgggctcaagcaattctccttcctcagcttcccaagtagctggaattacaggctaattttgtatatttttagtagagatggggtttcaccatgttggtcaggctggtctcaaactcctgacctcaagggatccacccaccttagcctcccaaaatgctgggattacaggcgtaagccccgacgcctggcatgtatcctgatttctggggtattaattagttcacatggccagccaagacccactccagatgcagtggggctcctccccatctgtcacagtacactggatcaacataatgggaagttatctgttgttgtcatttcatttttacttgaaaaataatttacatactatattattttttaaataagaaaaccatattattattattttttatttttttgagatggagtctcactccgtcgcccaggctggagtgcagtggcattatctcagctcactgcaacctctacctcccgagttcaagcgattctcctgttttgtatttttagtagagacggagtttcaccatgttggccaggctggtctttaactcctgacctcaggtgatccacccccgttgacctcccaaagtgctgggattacaggcatgagccactgctcccggccagaaaaccatattattttttaaaaaagaaaaccacccagtcaggcacagtggctcacgcctgtaatcccagcactttgggaggctgaggcaggcagatcacgaggtcaggagatcaagaccatcctggtcaacatggtgacacgccatctcttataaaatacaaaaaattagctgggcgtggtggcacacgcctgtagtgccagctactcgggaggctgaggcaggggaatcacttgaacctgggatacggaggttgcagtgagccaagatcgcgccactgcactccagcctggcgacagagtgagagtctgtcaaaaaaacaaaaaaaacaaacctgatgcatatttcctaaagactacaacattctgatattctatgtatagtatatatttttgcataactgaataaaacacataatttaaacactgttagtgaccaaagccaccatgtttgagaaaaggcaataaatttcagcaactgtttaaactgcttataaatatagtatgccaaagctggaagtttactggataggaagagtagcttagacagaaagcgtctctgaggctctatgactggctaggtacccgacccacgcgttctcagagtaccctgtgcttgtccctgttgtcacacccaacatgccgtgttataactgccagtctctgtgattacacactgcaggatccttgagggcagggatggtgctggttcactgaagtacccttcgtgcttgacatacagtaaagactccataaataattgtttgataactactgaatgagtaaccagccatcttcactcattgatctgctgggagcaacagaagcaggcaagagtagcaccacatgacacaggaataagaggcacggtttccaagagcaggccggacgcagtgactcacgcctgtaatcccagcactttgggaggcagaggcggattgcctgaggtcaggccgagatcagcctgaccaacatggtgaaaccctatctctactaaaaatacaaaaattagccgggcgtggtggcgggcgcctgtaatcccagctactcaggaggctgagacaggagaatcgcttcaatccaggaggcggaggttgtggtgagccgagattgcaccactgcactccagcctggcaacaagagtgaaactccatctttaaaaaaaaaaaaaaaaaaaaaaaggcacggttaccaagagcctgtgtttggtgtttgccagatggccaaaggctcccatcaaaatatgactgatggaatactcagacatgtccattcaataatgtccctacagtacgacatactatactcacctattatgagtgacaccaaaggatacatgatattttggctaggatcattttgactgttaagccaactcttacacacaccttaccaaaatttgcaaactgtctattaatcacaagcaactaagcaccaacaacactattcaagaaaggaaaaatgagttagggtgggttatattttactaggaaattcctctggctatattctataggaattaggtgtaatatctgttatgcaattgcttagcatagtgtttggcaaagtattaacaaagcctctttcccttctgcatgagaattttacctttgttaactttctagctctgttcccctggcaacctaataaaaattcatatgtcaactgctaggcaatgttacatatggtagacatgatgcccaattggtaaactgcatctggactgggagaactataaatgcctgataggaagcctcagctctgggcatccctaagtacagtgacgcttggaacaggcatgtcttttatagggacactggaggccatgtctatgaagctgttataagagatacttgttcctgtgggacaaggggctcttaagccggggaagcttccatacttgccccatgtagatctgtctccttgcacctgcactatgccacacagacagctgcagagactttcagagaagagcaactggttctgccttgctagtaagcagtgcttcccattctatatccttttaagtgaatctgatgccaagtgtggcagtttataaatttgaatgtttctaaaccttcagttgggcctaagacccttggagggcactgcagtattatttgcatgtttttctgatggcagtagatgctcctcaggggctatggatggtaaaagatgtgaaactgtttggtatgtttttctacttccaaaaaaatcctgaccatacccttcactgtatgcatgacagataatccatatccattacatgtcaccaagacctgtatatgaaattgatgccttccttcaaaatccccaagcttgttactactaaaccttcctcatcaaagcacataatccctgccctaacctccactgattaactgacaaaggtccagaaatcaaatgatggatataaaaattgccccccctaaaaccacaattgtcaatgaagaattggcagtagtaaaataatctacctggagggtcaagacggatgctaaatgttctccttcagttatgaagtttccatgtcatccgatcatgcagtcatgtgagttactgtcaccttttaaaactaggatatatttaggccgggcgcggtggctcacgcctgtaatcctagcactttgggaggccgaggcgggtggatcacaaggtcaggatattgagactatcctggctaacacggtgaaaccccgtctctactaaaaatacaaaaaattagctgggcatggtggcgggtgcctgtagtcccagctactcaggaggctgaggcaggagaatggcatgaacccaggaggcggagcttgcagtgagccgagattgtgccactgcactccagcctgggcaacagagcgagactccgtctcagaaaaaaaaagaaaagaaaaacaacaacaacaacaaaaactaggacatgtttaggaaccaaccaaactactctgaccccaaaacacttttcgtttttctctacagaaacatcatttgaagaaaagaattcaaatttccagcactacaatgaaaggtttgtggaacacagtactgttgagtggagagaactacaaaagcaacagaaatcaatgaaaacagtgcccatcatatgcacctgaataaagtgtccctttatcaggttagaagatagtgtgatcacatgaaaacacaaggcaagctacaagagaccagcaacaacaggaagcacagtgggaatgctcaaaacagagcataataggaacttctcacccatcccaaccctttgcccctccctaccccattacactagacttcacagagatcattctcttaatgcacaagggacacacacaagaaaaatctagagttccaaataaaacagtctgagttcagttaaccaaaggccactccactctttcctacggctcccagaatcagtgcatgcagccctacctgttgcctttctctccctggggtttgtcacgacatcaatgaacaataacaaaaaaaacccatctcagtattccaaaccaccagaatactcaattccataacatgttgcagaacactaggtcagcagcttccttaaggaatattcaaagtctggtggccaccaaaatatttacatcagaacggcatctttctgccaaatgatcagaatcatgatgcactatgtcatttcttaattattataggtaaggccctatttacattccttctcaacttttgagaagggggtcctcatcccccaagagaaataacttcccaagaatgccattttggaattccattacaagtaagagtcctgttcccattcatgcaatacatctaatatgagacgaaaatatccctttgtgaacttgggtggaatgtgccagaatagaaactaaaccactaacggtctgtgttgggctcaactgtaaatttacttagtataaaaataccaccaaccccacaaattaaacctcaaagacactgtgattataaatactgaccacctaaaggggaccaatttatgatctgatagtctagacagaggaagtatctcctttaaaagtgatagaactcagtgatccagttattgccagtgcctatacacaaactccaaatagtccaccagaaatgcaacaatctgagatattacgaaagaaagagaatcatttaaacattaggtgtcacattctgttttcttcccagtgattctgctactttaaaaattaacaaaatgatcagaacctagtaacgattctgggtgtatgaatgagtcagaattttctaagtttccacattataaacctaaatcagatcttgggcaagctatgaaccatctggcctcagcgcttcattttactaatccactattttctaaaatttgcgagagtataaggggctactaaatattatgaaggtcagccaggcacggtggctcacgcctgtaatcccagcactttgggaggctgaggcaggcggatcacttgaggtcaggagttcaagaccagcctggccaacatggtgaaaccccatttctactaaaaatacaaaaattggccaggcgtggtggcgcgtgcctataatcccaactactcaagaggctgagacagaagaatctcttgaacctgggaggtggaggttgcagtgagccgagatcacgccattgcactccagcctgggtgacaaagatgaaactccatctcaaaataaataaataaatacataaaataaaattaaaaataaataaatattatgcaggtaaaaggtagcttaaaatagaacacaaaattaagtccactcattaaagatcctttaaaaaatcctactttatcttacagcagagtttctcaacattggtattactgacattttgaattggagaattcattgttgtggggactgtcctgtgcatttcaggatgtttggcagcttccctggcctctacccactagatgccagtagccacctgcaaggcacgaaatcacccccaactgagaatcactgtcctacagtgaaatctctaatgtaaaatgttttacccagggatatgaagaggtcacggaatcactgaagaggatcatagctccactggagaaagcaggcaaagaggctgaactatgaggtagaaaagtcattaaaacatcagagataatttaaacagagaaagcaaaaatatcaaacactgttcctggccaagtaaatcttctacacatccatttaggtttcctttttgctgagatccctcttttaaaataacagcaaatatatgtatacatttttggagacagtttcgctcttgttgcccaggctggagtgcagtggtgtgatgtcggctcacagcaacctccgcctcctgggttcaagcgattctcctgcttcagcctcctgagtagctggaattacaggcatgcgccaccatgcctggctaattttgtatttttagtagagacggggtttctccatgttggccaggctggtcttgaactcccgacctcaggtgatccacctgccttggcctcccaaagtgttgggattacaggcgtgagccactgcgcctggccacagctagtatttttatttcagataagacaaatatctctggtccctgataattttcaatgagtaactcttgatctagaatatttttcttttatttatttattttattattatttttttgagacaaggtctcacactgttgcccaggctggagtggagtggcacgattccagctcactgcaaccttttccaggctcaagtgttcctctcgccacagcctcctgagtagctgggattacaggcacatgccaccactcctgactaatttttgtatttttgctagagacggggtttcgccatgttggtcaggctggtatcgaactcctgacctcaagtgttccatctgccttggcctcccaaagtgctgggattataggcgtgagccaccgcacacagccaagaatgatatttatcgaactacctgtgataagagaagttttaaattttccattctactgcagaccaatacgtggtcctgctgtacaggctggtatccaacctctgcaccatgtggccctctagctgaccagaactgaactggtccatacctcactcaagaagacaaagccatgagtcacagcaatgtcaaagtgttatcaacatttctatatgtgtattcttaatttctgactttccttgtagcagactggtagaaaacagtttacagaacagggcctctctgtgggccagagtttgagttgcactgttccagttttaactactattgagaagtacgacttaaacacctgtctaatgctttggctaacatttacaagccaatttataatgtttttgacttttttgttgttcaagaggtagaaataaaagtgacttttaccaccttttgaaagacaactacacttaaaggaagacaagaagatttcttttaaaatccattttggatattttaacataagacaaaattatggaaattgccttcaattacattccgaattcctaacactgcctgccctttagccctttaaagagttcagcctcttttgttacaataattgtgtggctggaaagtgggcgaaaggtagactgcttttaaaaacctgttctgctactaaccttccctttccctcatgaagatcttttaaaagatgaacattttagaaatgttacttggcattatgggcttatactttccctccaattaaagttctaggcaaggaggtagaaggcaggactcaactccaaaggccggactcggacatggaccaaattgaggactagctaaaacagggcggtggtgggagggtggtgcaggaagcagatttccataagaaacacttatcactgtgccatgtcaattaccattgccatggcaacacctggaagtcactgccccttatcatggcaaccacccagcggcttggaagttaccaccattttcctaaatattgctgcataatctgccccttaatttgcatgtaactaaaagtgggtataaatataagtgccgacctgcctctgagctactactctgggcacactgcctatggtgtagccctgctccacgaggagcggccccttagctgctgttgggcactgctgcttcaatacaagctgctgtctaacaccactggcttgcccttgaattctttcctgggtgaagccaagaactcctctgggctaagccccaatttttgggctcacctgccctacatcagcataaactaagtaaaagaatgccagaggcagctacatttccaagttacacagctccagcttttggaaattgctggaaaaagtaggggagcattttgagttttgcccaaatgagttgttttatgataacagaacaggttgtatgtgtagaatcgtcaaatgccaaaccagacagggaaaccatccagacctggggtcatagcctcccttctcagggctaacttaaaatttaattcaactgggcaagtcaggatgccataatgagcctttcagatcattcccatgttcgtctgcccataagtattccaagcctttaaaattgttctagatttagggagtaccttttatgatcatgtagccagaccgccctgcctgctttatatcaatgaaggtttctctttaatactttgccagaaaatttaatgtggaattcattaggaaaggcttggcaaaggtaaacttgatcccaaaacttaatggtttttagagaaagaggatgataacaaaggaatgcagaggactgaatcaatataaaaacaagcctggagattttcttatctttctcctaaccagagtttggacacacagcaagaaaaacaggagacctcagggcctgctttgactcactcagaattaaggagtggccagcaaagccctcagaaaccaagggcaccacacaaaaaggttatctgtcctttgagtcacaaaatccaacctctatcagatagtctaataaaaatgcacatataataacagtgaaaaaatgttcctctcagggttccacaaaattggacaaatggtatctttcaacaacagaacgagcactaacaagttttaaaacctcctcttccccaccaatttattgctacgtaagtgtctctcggtctgataagttaggctgaatttgtggtttgtcatcagaatcatctccagcagggtcattttcctcacccgactccacatagattggccagtcattgtctgtgtcgctcttttcttggctttcagatgaagcctccaccaagctaaggttgatgggcatcaaatcatcatcatcatcgggtgtgtctgtaacgcaggtgcagctgtcacacagcccgaagcgccgcagcccctgggacaggtgactcgtgaatgttctcctgcagcccttgcagatgattggacggttggatctgtggacactcagtgcgtggctccgcaggtgctcttgtcgagtgaacctcttgccgcaggtctcacaggggtagggccgctcgcctgtgtgtgaacggatgtgccgcttgaggatgcccttctgtttggcagtgtaagggcagaaaggacacttgtggagcttgatggggaccaccagcacatcacctgagtcctctccataccagtcagcctggacatccatcatggaactcatggctactcctgcaccttctggtcttccttccaaactcctagaaaagtgatggtctgcatcatccttgctcggggcagcgctgttgcgcaagagcgcctccaggaactgcttcacgtggtagttgctgtaagccaagtcaaccgcctggccgcttggcaaggcctcctccacgtgggccaggttcagcggggcagcatactgctgcagctgttcaccaacgtccacctccacttcatcagcatcaaattccaccttgggctctatccgtttgggtggagtagagaggttgctgtcagccgagccaccgccaaggctgtctctcaccaccagttccaaggggtggcagtctccgcagtcaccgcaaggggactctctcaggcactccacgctcttttctccctcggctggagaggagaccaagctcttggtaccacaggaggtcccctcccggcctgaactggggctttcactgtcaacctgatgagccgccgctgctgccgccgctgcagccgccgccgctgccgccgccactgctgcagccacagcagcctccttctccatctttcggcaaatgtcgagggatgacctaatgtatgtcttgcagaagttcaccacgtcattcatctgcaggtagctggcagccgacatcacttcaatcacattctccccacacaaatccaacttcccagaatagaggaaatctaagatgatggagaaggcatcagaggtgacaatgtccaaggaggcggtgctatgccgcccgctgtcctggatatagtgaatgagcagggctcggaagtagccgctgttagcaaacaaaatgttcctgtgggccttgaagatccgcccttccacaatgatgctgcagtcacagaaaaagtccctctttctctgttcattcagctcccccaaaagcttggcataataggattgcatctccattgctccgccagctgctgctgctccagagcaaacctgtatctcttccagcgggttccagcagcgcagccacggagc

SEQ ID NO: 11599 - RNA, 3600 nt, Homo sapiens
  source 1..3600: mol_type = other RNA
ctgaatagctgggactacaggtgtacgccacacatctggctacttttttttctttttggtagagacagagtcacccaggctggtctcaaactcctggtctcaagggatcctcctgcctcagcctcctgaagaggtgggattacaggcgtgaaccaccatgctagctaaaaccaagatcttgatctttaacactgacctaaattaaggttattttttttcccacattagaaaaagaaagaaccttacaaatgtcacatagtaggaaaaaacctaagaaacgagatgtactcaatccaagacacaaatagtttgccaagaagagaaaggtaaagaaaaactaggacatgcattattttcccccacaaaattaagacttcagaacattcttttgatataaaagaaaaacattagaattatgtgactctctgcaaagggctaagaaaactaagcactaatcaaagacaatcttgaattttcctgtcaaccaataaaaacgataccctcggccgggcgcggtggctcacgcctgtaatcccagcactttgggaggccgaggcgggtggatcatgaggtcaggagatcgagaccatcctggctaacaaggtgaaaccccgtctctactaaaaatacaaaaaaattagccgggcgcggtggcgggcgcctgtagtcccagctactagggaggctgaggcaggagaatggcgtgaacccgggaagcggagcttgcagtgagccgagattgcgccactgcagtccgcagtccggcctgggcgacagagcgagactccgtctcaaaaaaaaaaaaaaaaaaaaacgataccctcacctgaacaagggagtcttccactttacaaaatcacgaatcttcctgtaccaaaagaggttcgcttctataacagccgatctagctgatgagcctgtctgattagttgggttgcgggaagatcagattactcttcccgcttaggcggaaagaaactcacctgaagttgcctgggttctcctttcgtttcaagtaaatcctgagttatcagaagaggctcgcttttctcatagctctcctggttgataagcgtgtcggcatagttgggctgggggaaaatcagatgactcttacgcgagtctgcagtgagtgagacctcgtgggaataggtctgcaggaaagcccgaaccccttccacgcccacaaagtgcgagccgggcatgctcgctaagccacctcccgaagcctgcagcaggcgtgacttgtgccagcgctgcagtctgagcgccagcagcacgatgacgaaggccaggaagacgcaggagaccgcggccaccgccaccaccaggtacagagtgaggtccgaatcgttgggtttggcggagggctcgaggctgcccaggtcggccaggatgtcggggatcctgtcggccacggccacggtgagcgtgacagtggcggagagagggggctggccgtggtcctggacggccaccactaggctctgcttgagcgcgtctctgtccagcagggcgcgcgccgtgcgcacctcgcccgtgtgcaggcccactgagaaaagtcctggctcgctggccttgagcaggcggtaggacagccaggcgttctggcccgagtctctgtccaccgccaccaccttggtcaccaggtagccgggctctgcggagcggggcgccagctccacgccagtggaaccgtctgtggggagggcggggtacaggatctcgggcgcattgtcattctggtccagcacaaacaggctcagtgacacgttgctgctaagaggcgggtccccgctgtcgctggctgtcacccacagctgtaggtctctcaactgctcatagtcgaaggagcgcagggcgtacagaatcccagtgtcggagttgatggacacgtaggaggacaggggcgccccctggagggtgtcttctgccagtgagtaggagacttgggcgttctggtccacgtcagggtccagtgcattcacagagaagatggaggcacccctggggttgttttcaaggacatagactgagtaggatgaatgggggaaggtgggcgggttgtcgttggtgtctgccacatttagagagatgattgtttctgtagacagaggtggtgttcctttgtccgtggctgtcacagtgatgttgtacaagaatacctcttcccggtctagagctgcatttgtcactaatcgataataattgccaactgatttttccaattcaaatgggagacttctcgggatggaacaggttaccaggccattcaggccagagtctcgatcgaacacttgaaaaagggcgattactgttcctggaggtgcactttcagcaattgttctgcttccagatgtaacaaccacttctggtacattatcattgacatccaagatagttattaagactttcgctctgtctcgaagacctggcccatcccgggcttcaacacccagctcataaaaactcgagtcctcatagtctagatttgcagaagttgaaatttctccagtcaaaacattcaaacagaaaatttgtgagatcttttctgtaatcttcacaaaggaataagttacttccccgtggactccttcatcctggtcggtggcagtcactgccaacactggtgtgcctactggcaggttttcaggaacacttacacggtagacaggctgagtaaacattggagtgttgtcattcacatctagaactgttaccagaatttgggcgacgcttgagcggacagggtcgccgccatccatggcagtaaggaccaggcggtaaacggcttctccttcccggtccagtgtgccctccagcaccagctccgggtacttgggcccatgggcttcgctttgcacgtccactgagaagtgactattaccactgagcttaaatccctgaagggagttcattcccacatcagggtcatagacctccattagtggaaaacgagaggatggagctgcgttttcgagaattttcacttccaattcttcctttaagaatcggggtgtattgtcattaatgtccactatttccacttccacgggataaagattcagtttatcctcgacaaggatgttaaaactcaccagacaccgcgggctctgagcacagagctcctcgcggtctatcctacccgcggtgaccaagctgccgtttcgcggattcagagagaaaagctgcatcctacctctggagacgatgcggactccgtgctccgccaactcctggggctccagtcccagatccttgacgatgttgcctacgaaggagcctttctccagctcctcgggaatagagtagcggatctgcgctgccgcggccccccacagcgtccccaggagcgtgaggagcaggacctgctcgctgcgctgcggatgcctctgcggaggcgccattactggcttattaggaacttctctgggattaagaagaggaagaacagatctgcatcacttttgctcttctcagaaatagcggtgaaggtccttcaacaagcagagaccggatgcgaagcgtttcaggtcagaatttctgcacagctttcctgctttcccgtctaatttgctttgttgttggaggatgtaactt

SEQ ID NO: 11600 - RNA, 33 nt, Homo sapiens
  source 1..33: mol_type = other RNA
ctgaatagctgggactacaggtgtacgccacca

SEQ ID NO: 11601 - RNA, 2025 nt, Homo sapiens
  source 1..2025: mol_type = other RNA
ctgaatagctgggactacaggtgtaggccaccatgactggctgattttttctctctgtattttgtagagacagggcttctccatgttgcccaggctagtctcgaacttctgggctcaagtgatccttcctcctcagcctcccaaagtgctaggattacaggcgtgagccactgtgcccagacattatttactttttacatggcttacacttactatcatgtacaatcagagccatagagacctcaaagggaaagaattaggatcagtgagcttttcatggaatttgtacttaagcatgactttacaaagtaccatatagacaatgtcaaagcaattattttttcatttccttctatccacatgtaggggtgaggctatttcacagagatagtgtatcattttactaaaacattatttattttaactatatttaggacttaaattaaaaaaaataattttctcattcatctagggacaatttctgacccgcgacagaaagaggactccagtggagagctcaggaaactcctagaatggtgttgctgtaataagaagatgtcaacagcagtagaaaggtttggttgcctcaaactgaaaatgactttggtttggtaacttttaagatcacagtgtaagaaaaccgagatcatgggctggagagattacaaatatctttctcttattgcttcttcttcagtaagtgtttattactagccaagttgggggtggggagacaaaattcaaacagcagaaaataacatctttgggtctactctttcctttcaaaagttttcttggggataagctgggaaatagatcatcaatgggtttattgactaggaggaagagggggagtctgtctaaatcatcaaaatgtgagagagagattaaaaccacattctctcatcagagtagaaagttatatttaaaaaaagaaatagaggattgaaaatgtgagctatagcctctaattcataaataactcagctgttttatggtggaatatttagagacagagactgaggctaagaccatttggcctctccaaagatgaaatcgaggcttttctaacttccagctgtgagtcaaaagcaagaagaaatctagatgggatctccttgttttttgggtgagctctccgggagtttcttccgcccgtgctgagaggtcttagagcattacacatagtcgtgcttggaaggataagattgtacctcgtcctctgtgcgggcacctccatcgtatatcttcttgtttttggtgttggacccaaagccagtgctggccttgaagcctccaggcttgtaggcaacactgtggcctgaggcatgataagaaacggctttgtagttggtttcttctggtgccaggccccggcaggcgatgcacatcatcacacccccaattagtgtgaggcctccagcgacccagcccacgaacagagccgcaccaaatgtgtacctggtctgaacagtctgcaccatcccacccatgccggtgtacatgttagctgtggacatccagaagttagtcaccagcatgttggcaaacacagacactccagcaattgcacaaagacctgagacaatgaacatgatcccggaggtcagtgtcatgttggctttggcagagtcctccatgctgccaatgcggatgcatttcagggcaaagatggataccaggaggccaatggcacccaggacgatgcctacgatcatcagggctcgcactgcctgcagcatggctggaagtcccaggatggtgaaatagggcctgcattcggtgaagcctgaactctgcctcacgcagctcctccagagcccttcgtactggaacacggaggtgacggggttgtcgtacaggtcctgggtgctccacatgtccatcccggtggccgcgatgcagccggccagccccaggatggacaggaggaacgccaccacttggcatgtggtggtggacatgatcctggccgcccgccctgccgcctgcgagaagctgccgccctcctgctgccgaaggtgt

SEQ ID NO: 11602 - RNA, 2017 nt, Homo sapiens
  source 1..2017: mol_type = other RNA
ctgaatagctgggactacaggtgtaggccaccatgactggctgattttttctctctgtattttgtagagacagggcttctccatgttgcccaggctagtctcgaacttctgggctcaagtgatccttcctcctcagcctcccaaagtgctaggattacaggcgtgagccactgtgcccagacattatttactttttacatggcttacacttactatcatgtacaatcagagccatagagacctcaaagggaaagaattaggatcagtgagcttttcatggaatttgtacttaagcatgactttacaaagtaccatatagacaatgtcaaagcaattattttttcatttccttctatccacatgtaggggtgaggctatttcacagagatagtgtatcattttactaaaacattatttattttaactatatttaggacttaaattaaaaaaaataattttctcattcatctagggacaatttctgacccgcgacagaaagaggactccagtggagagctcaggaaactcctagaatggtgttgctgtaataagaagatgtcaacagcagtagaaaggtttggttgcctcaaactgaaaatgactttggtttggtaacttttaagatcacagtgtaagaaaaccgagatcatgggctggagagattacaaatatctttctcttattgcttcttcttcagtaagtgtttattactagccaagttgggggtggggagacaaaattcaaacagcagaaaataacatctttgggtctactctttcctttcaaaagttttcttggggataagctgggaaatagatcatcaatgggtttattgactaggaggaagagggggagtctgtctaaatcatcaaaatgtgagagagagattaaaaccacattctctcatcagagtagaaagttatatttaaaaaaagaaatagaggattgaaaatgtgagctatagcctctaattcataaataactcagctgttttatggtggaatatttagagacagagactgaggctaagaccatttggcctctccaaagatgaaatcgaggcttttctaacttccagctgtgagtcaaaagcaagaagaaatctagatgggatctccttgttttttgggtgagctctccgggagtttcttccgcccgtgctgagaggtcttagagcattacacatagtcgtgcttggaaggataagattgtacctcgtcctctgtgcgggcacctccatcgtatatcttcttgtttttggtgttggacccaaagccagtgctggccttgaagcctccaggcttgtaggcaacactgtggcctgaggcatgataagaaacggctttgtagttggtttcttctggtgccaggccccggcaggcgatgcacatcatcacacccccaattagtgtgaggcctccagcgacccagcccacgaacagagccgcaccaaatgtgtacctggtctgaacagtctgcaccatcccacccatgccggtgtacatgttagctgtggacatccagaagttagtcaccagcatgttggcaaacacagacactccagcaattgcacaaagacctgagacaatgaacatgatcccggaggtcagtgtcatgttggctttggcagagtcctccatgctgccaatgcggatgcatttcagggcaaagatggataccaggaggccaatggcacccaggacgatgcctacgatcatcagggctcgcactgcctgcagcatggctggcagccccagcagggtgaagtagccccggcactcggtgaagccagagctctctcggacacaggagcgccacagcccctggtagttgaaaacagctgttacggggttgttgtacaagtcttgggtgctccactggtccatgcaggtggcagcaatgatgcccgcaatcccaatcagtgaaaccacgaaccccaagccctgacaggcagtcacggccatggtggcgcacagtgtcgacacagagccacacgacaagtggacagcgcaattct

SEQ ID NO: 11603 - RNA, 2978 nt, Homo sapiens
  source 1..2978: mol_type = other RNA
ctgaatagctgggactacaggtgtatgccaccatgcctggctaaatttttgtatttttagtagagacagggtttcaccatgttggccaggctggtctcgaactcctgacctcaagtgatctgcctgcctcagccttccaaagtgctgggattacaggcatgagccaccatgccgggccgagactctgtctgtttaaaaaaagaagaagaagaagaagtaaaagaaggcagctcagctggtacagtagaaagcctattctggaaactgccatgatggatggctaataaaatattggagatacttaacccttagccaaacagtatgtgtctgtgtggtgtgtgtgagtatgtacatgtatgatagactgtgtgtgtgtgtgtgtgtgtgtgtgtgtgtttgtgtggtgggggtatgtgtgtgaaggccccagaaggtggccctgggacaaagcgctcctaccacttgtccccagcataggacagccacacaattcagagcacaggagagcccacacctggaggctgggctgcccttgcgggtggggttagcaatagctaacatgaaaacttccagatagcaaacctcccctggccacctgactacatatttcaaacattacctgaagcaatgaaattcaagagcattcatagtcttttttaaacttctgactacgacccacattgaggttagttacatggctgccaagggggtggggacacaggataggtaacaagagttcagactcagcctgatggcacagggtgcgctttgccctgtcccagtccactgtgtttgtggtggtgacccactaaattgattttgtgacccacttgtgggttctactgcagcttggacccgcagtctccgtgcacatggaaaatcattccctccacggaagtgggtggacctccccgcagcaggccccggcctcagtgaggatcaccaagtgccaccaggcccccacaaccccgctcaggaggaggaagcaggcttccctgaccatctttaaagaaaagggggcaccatgatgggcccactcaggtccaggctggcaaccacaggtccacccgtccaagacgcaaggcgaggctgggccattccctgcaagtgcgtgttggtcccttagggcttgcccaggggcgcccccgcgctctggcatctctgtaccaggaggatgagcctggcgaggtctgagagctccgggaacgcggccatcacgcggtccacctggtcacgcgggaagacgctgtagagcgcgatgcgagcccgggcgcgcgcgtccccctcgtcgtcctcggtcgcgtacactgaaagtcccccagtggcgccgtcgccccaggccggctccgcccagacggagcgcccagggaagcggtcggagcggggtggacgggcccacgggtcgtcgggtggcctgcgcggggaaagcaagtcgccgtgcaggtccctagggcggtgttcgccccgcggctggagctgcaggccgggcggaggcgggaggtcgcccggggagaactggctctccgggctagggaggctgagcgggcctggcacccggccgcccgcggacacccagtcgggcccgcccagtcggggcgtgaggctgcaggcggggaccgggagaggcggccccaggggccccaggtcgtcgctgaaggccagccgagagaagctccctcgcagggcggccaggtccggggacccccgcgccggcgggaggctgtgcgcaaatggttcccggggggccgcccgggctcctgcggagccgcccggggctctcggtggccgctgctcctcggcgcccgcgccaggccgggcccctgtcttggcgcggagctcgtcggccaccgccagttgcgcgtggtgcggcctctccgggtggtagaacttgcacttgatgccataggtgcatttcttgccataaggacaatgctgccaggatggctctgggggcttcggcttcctgctcaggaagttgctcagggagggtccatggcggcccagggggtcatcaggcggcatgaaccggtcgttgacgaaggagaacatgagcagcctctgctcgatgaaccacttccactcggggttctcgctctgcaggtcccggtagttgtcgttggagacgatgacgccgtcctgctcgtaggccaccttcacgatgtagcggtcgtcgtagcagaccaggcgcttgccgtgcaccttgcgggacggcgtgtacaccagcaccgcctgccgctccagctccgccagcacgtgctgctctctgataggggtgtcagctcttggtgggtccttcctccaggatggaacaaaaactttgatgtaggtgtgtcctctgtccctgaaccagtcaacagccagcttgattccccggcaagagaaggtttctttatttccatggctcatcgccacgttgctgccatcaatcactatgggtcgcagagaactggccagggttctgaagtcctcttccagggctgtccccgggccacgctgggcagagtccgggaccccacaggagccccgaggcactagcctgggtgcagccgggtgctccagggcacccgggcggctgcccgtgcggataagctcctgcagcacgtcgttgaccagggcgccctcgcccagcttgcccaacacccggagcacatcctcccggtcatagcccagcttctggaagaattccatcttgctggggtgctccatgctgtgcccagcggccactggcgcaggtcctgccccaggcttcctcctctcagagccctgcagacatgagcagcagggtgtgtccctccggtcttcacaatgaatgctggcccagtcgccagcagccttcacgccaatgttctcccgtcagtgaggccaggcccccaggtgccactggagtcagaggagggcagctggcgtgcgccaagcagccactaggagccacttcatgccaatgctccacttcctgcacgccacagtcacgttcagct

SEQ ID NO: 11604 - RNA, 4133 nt, Homo sapiens
  source 1..4133: mol_type = other RNA
ctgaatagctgggactacaggtgtatgccaccatgcctggctaatctttttgtatttttagtagagatagggtttcaccacgttggccaggctggtctcaaactcctgacctcaggtgatctgcccgcctcggcctcccaaagtgctgggattactggcgtgagccactacacctggccaaaagcattctgaagagaatcaaattctgataaactctggtttgtaaaaattaattcagtggtataggcctcccaggggagaagcagtttgcctttttaccatcagttaaaaatcaaaagagcatatatattttttccttatctagtcgtgaccattacagcactgtttacatgtacaaatccaaatcctttaatcagaaaacacagtaaactacaaaaaaaactctggtatttaacagagtacttacatataatatgtactacaagacattttctttcgaaaataaaagtctatttccacagtatcaaacaattgaaacaaatataaatgggaacaaaatttctaaacagcagttcaaaaaccttggcaaagccagttatcaaataacatctagcttcatttatcaactaaaagactcactaaaaagaatgatttctgtacgtgtaaactgagtgtaacacttcaatatttcaatggaaattgctcttttgtcacacattattaaagtctgttctctgaataatttgaagaaatgtcagttataaggcaaattaagacttaaaaaaatagaaacagtgcatcttaaagtttttcagagacctacatataatttacaaacacataatttattatatggttatagtttggaacaaattttccctgagcactctttctgcctggctagaaaaatttaaacatgatttataaaatagaattttattttgatttttcttgaatatatgcaaattttcacctatctaatgtatttggaaaattttagaccgaactagcaagtataactgttttaaggagttatttgaatggttacagaaatatggttgggttttagagccctgagaactgtacagtgggtgtctcatataacagaaatgatttactatcctaaaactatcaatggttattttaccaaattcagaatgccactagtttcacagaggacagagtaataatcagtaattccagctcagatgatcaatagataagcattaaaaactgaaagaaaaaaaagttggattaacattgtactttccacgatataatgctgaaaaaaattaacccttctgcccaacacagtactgaaataccttaccctgaaacttcatttaatgcagtcttgagacctgtcactccttaatattcatgcagacttaaaattagcatcattgggaatttcgtcacacaacctgcagttctcaatgctatctcaagatttacagctccaaagacatactacaatcagtgccatgcatggtaacactaccagttgtgttcccctaacttttaaggtcttaaaaaaacttggctacctgacagtttaggcctttctttttcaaataaataaaggaaaacactgggagtctcaactatgcaaatttgtaaataattgctttctacatagcctagaatgatattagaagaaaatcagatttaaaaagtttcatatttacaattagattttcataaaacctaactatgcatttcttttagaattatgatttatgtggattaaaataataataacataaaacagttggaagtcattgttctgaagatcttcaagaagtgagcaatttcagatgtccagaagagtgccttctctctttttacttatattttaaggtactttatgcaggacgcccttgaccaaaacgacttttagaccttgtgtttttctctgagctgctttggcgtgcactaactggcactgaggccttgatttgtgcttccagcctggaataaatacctcctgcaaattcttttgcttcctttgacttgactcggtccagatcccccaatctcatttttattaggtgccctgtaatttcagtcattcgccgttgatcgtcttctctttgtgcatcctggttgaatctcaaggatcttgtggcatcccacttattcttctgcatactcataacgaaaggagacacatctctagaagctgacttctccaatgccttttctttcctctgggcacagggtgaagatacctgcttttttggttgtctagtgaacttctttggcttctcctttttcctttgtttcttggatacttcttcttcatctccaacttcatcttcagtgacctcagatccagtggtatattcttcttcttctgaaaacagtgactgttgtttcagttgtagagtccagtttttcaatgacaagaaagcattgagctccccagttttgggaccccatggtgtatttggctccagtaaaacatcacattctatacccttttcatcacagaggccaaccccaacatcactaactgtatcttttgaaaaaggcacaacaatgacatctctgtacttgtgcaaatcgtccaacattctagcagtgggacaggacggcaaatctccgccttcaccttgatcacgaagtgtaaccatgtggtccctcactttacagccctgataacatcttgaacaagtcagccaattgattgttccccacaatcgccagtatacatctctccaagattttaattcttcgaaaagactattcaaatactcatgaacatcccatgtcttatctcttatgtgaatatagacaatatttccacgtcgatccacattgatttttccaggaatgcaaggaattcttctttctgtttcttttgttaaaagtttcttacacaaacagcatctatacaatgttgctgcattactccgagaatctggattcaagtactcaggatcaaacagtctttcaatcttcttacaaaaaagtttgcttttaaatttatcttttttgtcctttaaatcatcaacttcattgtgtgagaacagatcagctatacgtgtgagaagatttgcattaatacagttcatgttgcatggggtagctactatggcattcatatttttgtggcaatactgaatacactgttcaactagtgaatccatttttaaaaactccgaagaaataagaattgaaatgacatttcctggctctaaagtgggcatctcacaatctttattctccttagtgttccttttaatgtattttatcaaccagttgaaaatgtgaacgtcgcaatgaactgaaatgtccacctcttcccagcgctgggcatccatagataaatattcagcaaagtacttcatttctgatatcaaaagatctcgcgggcaagtaaaatcttctttcaagttttttgcttcatcacacacatggatcaccatgtttggcccttcagattcttcagtcatttctccaccattatgagtagtacaattttcactttctgaagaacaattccttgtggaagctatactatgtcttccagttttggaaactgcatcatgtccaactggagtctcctgaaattctccatgtatgtcaagaagtgaggatttgatatatgtggctaaagtttcaacaggactctctccagcagccattagggaattatactggttgtcaacaggcgagcttccactgctctttaattcatcaaacctttttgcacactcttttggtgttaatccaggcacgagccttgctatagtttcccagttgatagtctgagggattccaattaatggataaaggatcatgtccaataccatttggttattattgttcaggaaattgttgttttctgaatatccacgactcatcttttggaacttgtagaaggccagaatagtggagtggttaagtgtgcagactctggagtcagactgtccaagtttgcatcgcagttctactacttatggcattatctggttcagattagttaatctctgtgcctcaatttcctcatctccacagggccgcggctgccctcgcagcgcctctgttacctgcagtggtcggcaccgcccgcgctcgcgccctgaagctgccgctaccgagcccgcaaccccgtccgcagcgcctcacaccccgcccccgcccgcttgcaggcggctgcggagact

SEQ ID NO: 11605 - RNA, 4192 nt, Homo sapiens
  source 1..4192: mol_type = other RNA
ctgaatagctgggactacaggtgtatgccaccatgcctggctaatctttttgtatttttagtagagatagggtttcaccacgttggccaggctggtctcaaactcctgacctcaggtgatctgcccgcctcggcctcccaaagtgctgggattactggcgtgagccactacacctggccaaaagcattctgaagagaatcaaattctgataaactctggtttgtaaaaattaattcagtggtataggcctcccaggggagaagcagtttgcctttttaccatcagttaaaaatcaaaagagcatatatattttttccttatctagtcgtgaccattacagcactgtttacatgtacaaatccaaatcctttaatcagaaaacacagtaaactacaaaaaaaactctggtatttaacagagtacttacatataatatgtactacaagacattttctttcgaaaataaaagtctatttccacagtatcaaacaattgaaacaaatataaatgggaacaaaatttctaaacagcagttcaaaaaccttggcaaagccagttatcaaataacatctagcttcatttatcaactaaaagactcactaaaaagaatgatttctgtacgtgtaaactgagtgtaacacttcaatatttcaatggaaattgctcttttgtcacacattattaaagtctgttctctgaataatttgaagaaatgtcagttataaggcaaattaagacttaaaaaaatagaaacagtgcatcttaaagtttttcagagacctacatataatttacaaacacataatttattatatggttatagtttggaacaaattttccctgagcactctttctgcctggctagaaaaatttaaacatgatttataaaatagaattttattttgatttttcttgaatatatgcaaattttcacctatctaatgtatttggaaaattttagaccgaactagcaagtataactgttttaaggagttatttgaatggttacagaaatatggttgggttttagagccctgagaactgtacagtgggtgtctcatataacagaaatgatttactatcctaaaactatcaatggttattttaccaaattcagaatgccactagtttcacagaggacagagtaataatcagtaattccagctcagatgatcaatagataagcattaaaaactgaaagaaaaaaaagttggattaacattgtactttccacgatataatgctgaaaaaaattaacccttctgcccaacacagtactgaaataccttaccctgaaacttcatttaatgcagtcttgagacctgtcactccttaatattcatgcagacttaaaattagcatcattgggaatttcgtcacacaacctgcagttctcaatgctatctcaagatttacagctccaaagacatactacaatcagtgccatgcatggtaacactaccagttgtgttcccctaacttttaaggtcttaaaaaaacttggctacctgacagtttaggcctttctttttcaaataaataaaggaaaacactgggagtctcaactatgcaaatttgtaaataattgctttctacatagcctagaatgatattagaagaaaatcagatttaaaaagtttcatatttacaattagattttcataaaacctaactatgcatttcttttagaattatgatttatgtggattaaaataataataacataaaacagttggaagtcattgttctgaagatcttcaagaagtgagcaatttcagatgtccagaagagtgccttctctctttttacttatattttaaggtactttatgcaggacgcccttgaccaaaacgacttttagaccttgtgtttttctctgagctgctttggcgtgcactaactggcactgaggccttgatttgtgcttccagcctggaataaatacctcctgcaaattcttttgcttcctttgacttgactcggtccagatcccccaatctcatttttattaggtgccctgtaatttcagtcattcgccgttgatcgtcttctctttgtgcatcctggttgaatctcaaggatcttgtggcatcccacttattcttctgcatactcataacgaaaggagacacatctctagaagctgacttctccaatgccttttctttcctctgggcacagggtgaagatacctgcttttttggttgtctagtgaacttctttggcttctcctttttcctttgtttcttggatacttcttcttcatctccaacttcatcttcagtgacctcagatccagtggtatattcttcttcttctgaaaacagtgactgttgtttcagttgtagagtccagtttttcaatgacaagaaagcattgagctccccagttttgggaccccatggtgtatttggctccagtaaaacatcacattctatacccttttcatcacagaggccaaccccaacatcactaactgtatcttttgaaaaaggcacaacaatgacatctctgtacttgtgcaaatcgtccaacattctagcagtgggacaggacggcaaatctccgccttcaccttgatcacgaagtgtaaccatgtggtccctcactttacagccctttgtaagctgagtaggatcaaaccgaagaaccttttggttacagcagggataaattccagtgccaacagtattcaatgaacttgctgcagtaggataaaccactgtttctgagtggtattgacaatgtgaaaattcaatacagagaaaggcctgataacatcttgaacaagtcagccaattgattgttccccacaatcgccagtatacatctctccaagattttaattcttcgaaaagactattcaaatactcatgaacatcccatgtcttatctcttatgtgaatatagacaatatttccacgtcgatccacattgatttttccaggaatgcaaggaattcttctttctgtttcttttgttaaaagtttcttacacaaacagcatctatacaatgttgctgcattactccgagaatctggattcaagtactcaggatcaaacagtctttcaatcttcttacaaaaaagtttgcttttaaatttatcttttttgtcctttaaatcatcaacttcattgtgtgagaacagatcagctatacgtgtgagaagatttgcattaatacagttcatgttgcatggggtagctactatggcattcatatttttgtggcaatactgaatacactgttcaactagtgaatccatttttaaaaactccgaagaaataagaattgaaatgacatttcctggctctaaagtgggcatctcacaatctttattctccttagtgttccttttaatgtattttatcaaccagttgaaaatgtgaacgtcgcaatgaactgaaatgtccacctcttcccagcgctgggcatccatagataaatattcagcaaagtacttcatttctgatatcaaaagatctcgcgggcaagtaaaatcttctttcaagttttttgcttcatcacacacatggatcaccatgtttggccagttttggaaactgcatcatgtccaactggagtctcctgaaattctccatgtatgtcaagaagtgaggatttgatatatgtggctaaagtttcaacaggactctctccagcagccattagggaattatactggttgtcaacaggcgagcttccactgctctttaattcatcaaacctttttgcacactcttttggtgttaatccaggcacgagccttgctatagtttcccagttgatagtctgagggattccaattaatggataaaggatcatgtccaataccatttggttattattgttcaggaaattgttgttttctgaatatccacgactcatcttttggaacttgtagaaggccagaatagtggagtggttaagtgtgcagactctggagtcagactgtccaagtttgcatcgcagttctactacttatggcattatctggttcagattagttaatctctgtgcctcaatttcctcatctccacagggccgcggctgccctcgcagcgcctctgttacctgcagtggtcggcaccgcccgcgctcgcgccctgaagctgccgctaccgagcccgcaaccccgtccgcagcgcctcacaccccgcccccgcccgcttgcaggcggctgcggagact

SEQ ID NO: 11606 - RNA, 4286 nt, Homo sapiens
  source 1..4286: mol_type = other RNA
ctgaatagctgggactacaggtgtatgccaccatgcctggctaatctttttgtatttttagtagagatagggtttcaccacgttggccaggctggtctcaaactcctgacctcaggtgatctgcccgcctcggcctcccaaagtgctgggattactggcgtgagccactacacctggccaaaagcattctgaagagaatcaaattctgataaactctggtttgtaaaaattaattcagtggtataggcctcccaggggagaagcagtttgcctttttaccatcagttaaaaatcaaaagagcatatatattttttccttatctagtcgtgaccattacagcactgtttacatgtacaaatccaaatcctttaatcagaaaacacagtaaactacaaaaaaaactctggtatttaacagagtacttacatataatatgtactacaagacattttctttcgaaaataaaagtctatttccacagtatcaaacaattgaaacaaatataaatgggaacaaaatttctaaacagcagttcaaaaaccttggcaaagccagttatcaaataacatctagcttcatttatcaactaaaagactcactaaaaagaatgatttctgtacgtgtaaactgagtgtaacacttcaatatttcaatggaaattgctcttttgtcacacattattaaagtctgttctctgaataatttgaagaaatgtcagttataaggcaaattaagacttaaaaaaatagaaacagtgcatcttaaagtttttcagagacctacatataatttacaaacacataatttattatatggttatagtttggaacaaattttccctgagcactctttctgcctggctagaaaaatttaaacatgatttataaaatagaattttattttgatttttcttgaatatatgcaaattttcacctatctaatgtatttggaaaattttagaccgaactagcaagtataactgttttaaggagttatttgaatggttacagaaatatggttgggttttagagccctgagaactgtacagtgggtgtctcatataacagaaatgatttactatcctaaaactatcaatggttattttaccaaattcagaatgccactagtttcacagaggacagagtaataatcagtaattccagctcagatgatcaatagataagcattaaaaactgaaagaaaaaaaagttggattaacattgtactttccacgatataatgctgaaaaaaattaacccttctgcccaacacagtactgaaataccttaccctgaaacttcatttaatgcagtcttgagacctgtcactccttaatattcatgcagacttaaaattagcatcattgggaatttcgtcacacaacctgcagttctcaatgctatctcaagatttacagctccaaagacatactacaatcagtgccatgcatggtaacactaccagttgtgttcccctaacttttaaggtcttaaaaaaacttggctacctgacagtttaggcctttctttttcaaataaataaaggaaaacactgggagtctcaactatgcaaatttgtaaataattgctttctacatagcctagaatgatattagaagaaaatcagatttaaaaagtttcatatttacaattagattttcataaaacctaactatgcatttcttttagaattatgatttatgtggattaaaataataataacataaaacagttggaagtcattgttctgaagatcttcaagaagtgagcaatttcagatgtccagaagagtgccttctctctttttacttatattttaaggtactttatgcaggacgcccttgaccaaaacgacttttagaccttgtgtttttctctgagctgctttggcgtgcactaactggcactgaggccttgatttgtgcttccagcctggaataaatacctcctgcaaattcttttgcttcctttgacttgactcggtccagatcccccaatctcatttttattaggtgccctgtaatttcagtcattcgccgttgatcgtcttctctttgtgcatcctggttgaatctcaaggatcttgtggcatcccacttattcttctgcatactcataacgaaaggagacacatctctagaagctgacttctccaatgccttttctttcctctgggcacagggtgaagatacctgcttttttggttgtctagtgaacttctttggcttctcctttttcctttgtttcttggatacttcttcttcatctccaacttcatcttcagtgacctcagatccagtggtatattcttcttcttctgaaaacagtgactgttgtttcagttgtagagtccagtttttcaatgacaagaaagcattgagctccccagttttgggaccccatggtgtatttggctccagtaaaacatcacattctatacccttttcatcacagaggccaaccccaacatcactaactgtatcttttgaaaaaggcacaacaatgacatctctgtacttgtgcaaatcgtccaacattctagcagtgggacaggacggcaaatctccgccttcaccttgatcacgaagtgtaaccatgtggtccctcactttacagccctttgtaagctgagtaggatcaaaccgaagaaccttttggttacagcagggataaattccagtgccaacagtattcaatgaacttgctgcagtaggataaaccactgtttctgagtggtattgacaatgtgaaaattcaatacagagaaaggcctgataacatcttgaacaagtcagccaattgattgttccccacaatcgccagtatacatctctccaagattttaattcttcgaaaagactattcaaatactcatgaacatcccatgtcttatctcttatgtgaatatagacaatatttccacgtcgatccacattgatttttccaggaatgcaaggaattcttctttctgtttcttttgttaaaagtttcttacacaaacagcatctatacaatgttgctgcattactccgagaatctggattcaagtactcaggatcaaacagtctttcaatcttcttacaaaaaagtttgcttttaaatttatcttttttgtcctttaaatcatcaacttcattgtgtgagaacagatcagctatacgtgtgagaagatttgcattaatacagttcatgttgcatggggtagctactatggcattcatatttttgtggcaatactgaatacactgttcaactagtgaatccatttttaaaaactccgaagaaataagaattgaaatgacatttcctggctctaaagtgggcatctcacaatctttattctccttagtgttccttttaatgtattttatcaaccagttgaaaatgtgaacgtcgcaatgaactgaaatgtccacctcttcccagcgctgggcatccatagataaatattcagcaaagtacttcatttctgatatcaaaagatctcgcgggcaagtaaaatcttctttcaagttttttgcttcatcacacacatggatcaccatgtttggcccttcagattcttcagtcatttctccaccattatgagtagtacaattttcactttctgaagaacaattccttgtggaagctatactatgtcttccagttttggaaactgcatcatgtccaactggagtctcctgaaattctccatgtatgtcaagaagtgaggatttgatatatgtggctaaagtttcaacaggactctctccagcagccattagggaattatactggttgtcaacaggcgagcttccactgctctttaattcatcaaacctttttgcacactcttttggtgttaatccaggcacgagccttgctatagtttcccagttgatagtctgagggattccaattaatggataaaggatcatgtccaataccatttggttattattgttcaggaaattgttgttttctgaatatccacgactcatcttttggaacttgtagaaggccagaatagtggagtggttaagtgtgcagactctggagtcagactgtccaagtttgcatcgcagttctactacttatggcattatctggttcagattagttaatctctgtgcctcaatttcctcatctccacagggccgcggctgccctcgcagcgcctctgttacctgcagtggtcggcaccgcccgcgctcgcgccctgaagctgccgctaccgagcccgcaaccccgtccgcagcgcctcacaccccgcccccgcccgcttgcaggcggctgcggagact

SEQ ID NO: 11607 - RNA, 4379 nt, Homo sapiens
  source 1..4379: mol_type = other RNA
ctgaatagctgggactacaggtgtatgccaccatgcctggctaatctttttgtatttttagtagagatagggtttcaccacgttggccaggctggtctcaaactcctgacctcaggtgatctgcccgcctcggcctcccaaagtgctgggattactggcgtgagccactacacctggccaaaagcattctgaagagaatcaaattctgataaactctggtttgtaaaaattaattcagtggtataggcctcccaggggagaagcagtttgcctttttaccatcagttaaaaatcaaaagagcatatatattttttccttatctagtcgtgaccattacagcactgtttacatgtacaaatccaaatcctttaatcagaaaacacagtaaactacaaaaaaaactctggtatttaacagagtacttacatataatatgtactacaagacattttctttcgaaaataaaagtctatttccacagtatcaaacaattgaaacaaatataaatgggaacaaaatttctaaacagcagttcaaaaaccttggcaaagccagttatcaaataacatctagcttcatttatcaactaaaagactcactaaaaagaatgatttctgtacgtgtaaactgagtgtaacacttcaatatttcaatggaaattgctcttttgtcacacattattaaagtctgttctctgaataatttgaagaaatgtcagttataaggcaaattaagacttaaaaaaatagaaacagtgcatcttaaagtttttcagagacctacatataatttacaaacacataatttattatatggttatagtttggaacaaattttccctgagcactctttctgcctggctagaaaaatttaaacatgatttataaaatagaattttattttgatttttcttgaatatatgcaaattttcacctatctaatgtatttggaaaattttagaccgaactagcaagtataactgttttaaggagttatttgaatggttacagaaatatggttgggttttagagccctgagaactgtacagtgggtgtctcatataacagaaatgatttactatcctaaaactatcaatggttattttaccaaattcagaatgccactagtttcacagaggacagagtaataatcagtaattccagctcagatgatcaatagataagcattaaaaactgaaagaaaaaaaagttggattaacattgtactttccacgatataatgctgaaaaaaattaacccttctgcccaacacagtactgaaataccttaccctgaaacttcatttaatgcagtcttgagacctgtcactccttaatattcatgcagacttaaaattagcatcattgggaatttcgtcacacaacctgcagttctcaatgctatctcaagatttacagctccaaagacatactacaatcagtgccatgcatggtaacactaccagttgtgttcccctaacttttaaggtcttaaaaaaacttggctacctgacagtttaggcctttctttttcaaataaataaaggaaaacactgggagtctcaactatgcaaatttgtaaataattgctttctacatagcctagaatgatattagaagaaaatcagatttaaaaagtttcatatttacaattagattttcataaaacctaactatgcatttcttttagaattatgatttatgtggattaaaataataataacataaaacagttggaagtcattgttctgaagatcttcaagaagtgagcaatttcagatgtccagaagagtgccttctctctttttacttatattttaaggtactttatgcaggacgcccttgaccaaaacgacttttagaccttgtgtttttctctgagctgctttggcgtgcactaactggcactgaggccttgatttgtgcttccagcctggaataaatacctcctgcaaattcttttgcttcctttgacttgactcggtccagatcccccaatctcatttttattaggtgccctgtaatttcagtcattcgccgttgatcgtcttctctttgtgcatcctggttgaatctcaaggatcttgtggcatcccacttattcttctgcatactcataacgaaaggagacacatctctagaagctgacttctccaatgccttttctttcctctgggcacagggtgaagatacctgcttttttggttgtctagtgaacttctttggcttctcctttttcctttgtttcttggatacttcttcttcatctccaacttcatcttcagtgacctcagatccagtggtatattcttcttcttctgaaaacagtgactgttgtttcagttgtagagtccagtttttcaatgacaagaaagcattgagctccccagttttgggaccccatggtgtatttggctccagtaaaacatcacattctatacccttttcatcacagaggccaaccccaacatcactaactgtatcttttgaaaaaggcacaacaatgacatctctgtacttgtgcaaatcgtccaacattctagcagtgggacaggacggcaaatctccgccttcaccttgatcacgaagtgtaaccatgtggtccctcactttacagccctttgtaagctgagtaggatcaaaccgaagaaccttttggttacagcagggataaattccagtgccaacagtattcaatgaacttgctgcagtaggataaaccactgtttctgagtggtattgacaatgtgaaaattcaatacagagaaaggcctgataacatcttgaacaagtcagccaattgattgttccccacaatcgccagtatacatctctccaagattttaattcttcgaaaagactattcaaatactcatgaacatcccatgtcttatctcttatgtgaatatagacaatatttccacgtcgatccacattgatttttccaggaatgcaaggaattcttctttctgtttcttttgttaaaagtttcttacacaaacagcatctatacaatgttgctgcattactccgagaatctggattcaagtactcaggatcaaacagtctttcaatcttcttacaaaaaagtttgcttttaaatttatcttttttgtcctttaaatcatcaacttcattgtgtgagaacagatcagctatacgtgtgagaagatttgcattaatacagttcatgttgcatggggtagctactatggcattcatatttttgtggcaatactgaatacactgttcaactagtgaatccatttttaaaaactccgaagaaataagaattgaaatgacatttcctggctctaaagtgggcatctcacaatctttattctccttagtgttccttttaatgtattttatcaaccagttgaaaatgtgaacgtcgcaatgaactgaaatgtccacctcttcccagcgctgggcatccatagataaatattcagcaaagtacttcatttctgatatcaaaagatctcgcgggcaagtaaaatcttctttcaagttttttgcttcatcacacacatggatcaccatgtttggcccttcagattcttcagtcatttctccaccattatgagtagtacaattttcactttctgaagaacaattccttgtggaagctatactatgtcttccagttttggaaactgcatcatgtccaactggagtctcctgaaattctccatgtatgtcaagaagtgaggatttgatatatgtggctaaagtttcaacaggactctctccagcagccattagggaattatactggttgtcaacaggcgagcttccactgctctttaattcatcaaacctttttgcacactcttttggtgttaatccaggcacgagccttgctatagtttcccagttgatagtctgagggattccaattaatggataaaggatcatgtccaataccatttggttattattgttcaggaaattgttgttttctgaatatccacgactcatcttttggaacttgtagaaggccagaatagtggagtggttaagtgtgcagactctggagtcagactgtccaagtttgcatcgcagttctactacttatggcattatctggttcagattagttaatctctgtgcctcaatttcctcatcttgggcccggaggctcactacgcggcgcgtcctcggggcacccccagaccttcgcgccccgctcccgcccgtggaggcacagaaactccaggggcgcagagcggacaaaggcgccgggcagcgggagcgaggcggggcagaggcccggggcgcggccgggcgcgcagaagctggggttcccgccgctgtgcgcgggcgggacggtctgcagggacatggaccgggcgggtgacgggacgcgggccagct

SEQ ID NO: 11608 - RNA, 1693 nt, Homo sapiens
  source 1..1693: mol_type = other RNA
ctgaatagctgggactacaggtgtatgccactgcgcccagcctacatcacgattttattatatcttgactgttgataattaaaatttcctgggatataaataaggcaatatgaagttgccctttctcagtatttttctttgtactgcctgttatttgaaaaagcattttctccctcaggggagttaggaaaggttagagagctgagagaacagggtttccctgggcagaggccgagtaggggagagcaggcaggggtctgtcagcagagtagtactggggccatgcatgagtggggccttgggggctctagggtcagcaggcagcacactggcatgttctccaggtagcagcagaaacattagggtgttagaggtttggggtctgcaggcatatctggggatcagaacaagctaatggccagcattggctgaagcaaggctttgagactcacagaattgggctgtcagtcaagcagggatctaagagatggggccagccaagcagaagtcaaaggctggtgccagcatcaaaatctgctctgatgctcctttgggagactgattcttcaagtctcaaatgctgttcacacctgtctctggatgctgttggctacctgggtgtggcttagcagggggagggtagcgtggtaggctgagcagaaagcctggctggcttcccaggcctgcgcttctgcagagaagtagtaacagtgctcctcggacaacacccagcctggggggcactgctggcatctggctcctgctcttgaggccaggaccacaatgacaaccccagagactgccaggagcacagccatgaacgccagggcccagtacagggacttcacgtacatgggtagccccgtaagcgttacggcccggggcagcttctcgtcgccgtccaaccccgcgcggggcaacagcgccgcatcctccttctccagccccagctccttgcagcggcagcacgtgggggagcccggggagccggcgcttccttccgcggggctggcccggccctctgcgtcgcagccgctctccgtccgggctgcagccagcggcgagcggcggccccacgtgccgccctgggatggtgcgcgcagcaggagctggtgcgccgggtccgcgtggcgggagaaggcaggggactcgggcaccggcaccttgaggaagcgcgtggagggcctgggcgatggcgtgctgctgccaccggccgcgcccacgggcttcacgcgcacatctacctgcagctccatgggcgcccaggcgctgggcgcaggctcagccccgggcgcctcgccattccggggcagcttgaccaaggcagggcccggtgacggcggctcggggcagaccccgtagcccaggctgagcggcggcacgcgcggggacccggggcgaggcgaaggcggctttttcttgctcgagggctccaggcctgcgcccgccgccttctccacggccccggccggacttgggctgctttcgggaccttcaggttgtcgcaccttcgcgggcacctgcggctgctccagcgtggggaccaggcttcccacgggctccattgggagctctgccccggcttggcctccgggcgcagcctcccaagactcctccatcccgcgcgccccgccacccggagacgctgaggagcgcacctgggcccagtgcagaggagcttcgctctcctccg

SEQ ID NO: 11609 - RNA, 6612 nt, Homo sapiens
  source 1..6612: mol_type = other RNA
ctgaatagctgggactacaggtgtatgcccatgtacaaatttttttgcagagatgggatctcattatgttgcccaggctaggagcaaacttttaataaaaggacttgtgtactcttaaattgaattttatgattttgtcctactgtttttgctgtgatatcctcaatgattcccatagaacacacaataatggtaataataacctacagaagcctcctctcatgtacaattttatttttcttttaaggagataaggaaggggaaaaagtagttgatttcctgtgtttcttatttagaaaaaattaaattatactgcatttttctagtattctgttagaaatttactttattaaaccttgataacttcagctataaacctaaaatattcttcttatactgatagaccaaacaaaagggctaaaaacaaatctatcatctaatttagattatatgtaagttagtaagtctcttcaaaataaagaaaggtagttttaggacagagatttttatatagattgaaagttatcttccctggaagaaaggtgaatctgagaatctagccgcacttcaaaaatgtgtgcaagtgtttatttggaatcccttctattttattagaaacagaaacagtaatttcaccagtaggaattgcgtgtgctctcaatacaagtaagtttgccactccttcaattgttgtccattgcagacactttggattcaaggttaagaatccaaatgagaaataagaaatatccggtccctgatgattcgtttaagtcctgttcaactcgatgaaagcttccacccgaaggaagagttactgttcctcctggctggctttgtgtttctttcagtgctctaaagaactttgtatttgggcagctgtgctctgtcatgtcaggctgctggacaggagttgatgcttacggcgccgctgaccagggctgctttactgaagctcactgggtgtccatcaatcacaaagtggcgtatgcagcctgtgaagggtttgctgggggccaagcgtggtgtcagtagagattctggaacacctccaacaaacacaggctccctgtgatcaattggttttggattcaggggtccaaccacatggttcacttcagagtccacatccaactgaaccacattagaatctctaataactgtaattctgtgccatctgccatcacagagactctgcttgggtgtaactgaggtggaaaaatctctgatgccattattgactttcactatgacctgtccatttttcatgtgaacatttaggtactccccattgacactgtggccgtggaccagggttccggaactgcttctgggacggacttcaaatgcaatttcaaacttcaatccaatattgaaagattcatctagaaccacgtatcctccttctgttgaaaagtaagttcctgtttccatggggccttcaaagcaaggggtcacactgaatgtctgagaagcagaggtgatggaggccccattgagctggagattgctgagacagccactaaaactgtagatggagttaatctgaacatttttcacagcctttccaggagccacacctcccaaataaatgggacccttgattttccaggtagcttcagtaggaggaagactttcttctaggactcggagaccatcaattaccagtcggccactgctcctttctcgaataaatatcacatcatgccacaggccatcattgtatttctcctggcttctaatcttcagttttttgtgaccaacattaaacatgtaaaccaagcggccatgggccaaaaatagagtcatgaagtcattctcttcttgatctgagacatagaagatcatgccatgggaggaacgagttctcagacgaatggaaaactgagatttggcaccaaaatctccttttaagtgttcaaactcttggcggctgttggctgttcctccatattgataggcgtgctctattgctctagggctgttggaaaggtggcaatgagagtttcttggagtattccgctctgggagtttcagagcaacaggatcccatgaaggtgcatctttacttttccctccctttttattctgacttgctttaggcttggataaattttttccttttttatggaggagaaacaatggtgaagactcaatgggacactcataaagagaagtgtggaccttttcagtataccgttggaaatcttcaacctccacatctctatccaccctggtaaagtaggcattacttatgcagccagtgaaattagcatactgagcactgattggtgagccaccgaagtaaaacttcttttcacttgcttgtgtctgttctattttccctttggtaggattcttactcccaactctgcttttatctactatcagttcatatcttgtgggtgagacagagctaatgacgaagtgggacagcccatcattgtactgcttatctactgactgaactttgattccctttacatccatgatgacagtaccattatccagtgagatggagaacacgtctgaccctgaagcataatagaatagtaacccatttggttgtaatgttcggaaattaaaacctccttcaaagccatcaaagaaagatattttctgaattgaagcaatgaagctctgtccattgaaatatgctctgcgagatataagtgagtcttctgggcatccataaccaactcccagggtttctgtctgctccagtaaattgaagtccttcttttggaactggaagcccttcatgcatcctctgaagttgatatctaggggaaggtgtgctctgagggccctggattgtaagatttctggaggagctcctccaatgtatatatctgtaaaaggtattttcatcttttcattatccatgctcttgacatgccttctgtcaactaccaagatcattttcttatcattgtggtaaatgattgagatctcatggtattttgcatcattaatttgagctttctttaacgtatcttcaagatgcacagggccaccgctgaatccaaaatcatagaacacatgtaggtaaccattgcgcatttccagtctgaaaaacatacttccattgaccatcaggagaataaggccgttgtcagctggtgttcgaacttctatgtcaaagcgagtcacctgaccaaatttccctctccttgtgatgtctctcaccacggcataaccggagccatcgaagaagtaactggcagcccgactctgagtgaaggccagcttatctcgggcacatggcactgatgtggaggggtccatattatagatgtgcttaaagttgtacaagctgatcacatcattattcaaagtggccagttccaggcagccaacaaagccaggcaggtttaagctggtagggagcttgaagttggaaggcactccaccaacataaaacactgtgtcctcagggtccaggtccagcagagagtcatctcccgaaaattccccctttttaatgaacttttcctctgctgtgctacttagactcgggactgttaaaaacacctttccatgttttcccaccctttcaatcttgacaatgctgaagtaagcaggccaggaactgacgggcttggagtccaggggaatctccacatctttagttcccaaattatagacgtataccagattatcatttttgattgcaagacccatatactcttttttggcgtttttgcttccgaggtacaggataaactgatctgcagtctcggtcagttccggccgcttcacagggggtttcatgtacaggctcagagacgtgaaggcctttaagtcatccatactggttctcgagtgcacttccacagctgactggccatcaaacatcatggagacttggatcttgctggcaacacttctggtctgagcaatgagctctcggatcctctggatgctggcagaaacgttgcttgcaggtcgcttctgctcaaccgtacgaagctgatccaggagctgagggacaacctcggtcagatttcttactgcatccctagcagagttcactgcagtgttgtaagcagaagagtcaaaatgttgaagattctgtgaccagttggttagattgttggccatgggggcagtggcctgctgcacctccatcgtcgtcctgttggcttcctcggtgatcagtctagactgccccaggcgctgctgggcatcccctctctctgctgcttgtagttgcttaacggcatcactgagtctggttttaagggcacttttccttgctagggctccacccacacgcctgctagtgtcagccactgcttcatcactgctagactctgcctttgcttgcagttctctggcttgattgaggaggttctcactttcatctttatggtaaatgatttgagtatcaatcccactcaccgcatcataaattcggtcagtggtgttcaaagcaaattctgctgtttcattggcttcactaacataattaacaatattttcatagacatttgatgcatccaaagccttctgtaccagcccgttcatatctgaactgtgcaacttcctgctcaattcattagcttcttgttgaaggtcctgtgcatggtcaatagcttcttggactaaatcatggctgaggttacttaggttagatagttttacttgtagttcacttttggctccatctatttctgcataaatccctgacgcattctttattatatcatcaagttctgaaagagttagacgaggtgttgtcagagagtccgcagatgtgctcagagacatgttcaccacttccatttgttccctcactctttcctgttgtttctcatggtcccgctgcctggctgctgtggccctgttcatgtcttcggcatccctgacatagttaagggcctggtcaagtgcttcctggagatctgacaacttagcattgtagtcatccagctgctccaggacgacaggaaacagagtgcgggtctcattgtgcagccgctgccagctctcagcctggctcagtagttcgtaagcctcatctgcctcctcatccacgagctcccgttgggtgaaaaatggttgacggcttctaatctcttcaagcatcttctgggccaacaccagcttctcagagatttccttggggctaagttcatgctcttccccataatagagcatcttgttgttgatctcttggattttatccctcatatcatgggcttgctctaccagctgacttgcgtggttaatggtgtccatgctttccttctgaacaagttgtccttttctggaggcttgattttccttttcaactaattcctctacgtcagacagaaggcttttcatcgtgttctcagcattgttgatttgtatctttcttagggcgtattggttttctctttctgacaattttgttttgaggaggtagatggtggcgttgatttcattcacgtgcctatgagcggcggccccagaggatacgctcagcaccccggatttgccttcctcgatggagagcgctgctaaccgcaggtcatcagtcaggtcccagacgcacttatcacagcctgtagggggttcaaaaccttcttccaagcattctccggttacactgtcacatgggcctcccccgcagttgcacactgcacagttcttggctatcctggcgtccccatagtagccaggagcgcaacgttcacacttgaatccggtggtgttgcgtaagcaattcctacactggccagtgacttcatcacaatcttcaaagatcaggttgggatctgaatttccactgcagtcacatttcttacaggtgcttccaatgagtaaggggtttccatagtaaccgggagcacatctttcacagttaggtccagcataattttcgttacaaatgcaccgaacagctccatttttcctatagcaggattctgcaaaattggccaagtggggcaggggacaggggcacggctggcagaattggggtgctcccctgatggaatctccgatataaccatccagacacttttcacagtgctctcctgttgtgttccgctggcagtgcacacagtatcctgagccgtccaaacactcgttggaattgccattacagtcgcagggcacacattctcccgacagggtgtgaaagaatccagcattgcatttctcggccgcaggcggcaggcgtcccagagccacgcggggttcgctcgtctcaggcgggtcttgcctgccaaccgctgagctcccttcaatgtcaaaaggaaaagcgttgtcgtccccggacgcggcgcgggagcaggcagcgctccagaggagccacagaggcagaaccgagcgccaggctgagctcaaagccatttctccgctgacatccagtagtgctcttccagggctcgggcgctgtgggtctccgtaggtctcccgcgtggtgcggcggtgcctcgcttattttccctcctctccgtgtgcagtatcccgaggtggctgcgcaaccagcagagatggacggagcttacagtacggcatcaaaaggcagacggattggggtgagccccgccagcgctaggccacctcctctccctggccgttcgggactggggactgcgctgtcctggcttccttctc

SEQ ID NO: 11610 - RNA, 6595 nt, Homo sapiens
  source 1..6595: mol_type = other RNA
ctgaatagctgggactacaggtgtatgcccatgtacaaatttttttgcagagatgggatctcattatgttgcccaggctaggagcaaacttttaataaaaggacttgtgtactcttaaattgaattttatgattttgtcctactgtttttgctgtgatatcctcaatgattcccatagaacacacaataatggtaataataacctacagaagcctcctctcatgtacaattttatttttcttttaaggagataaggaaggggaaaaagtagttgatttcctgtgtttcttatttagaaaaaattaaattatactgcatttttctagtattctgttagaaatttactttattaaaccttgataacttcagctataaacctaaaatattcttcttatactgatagaccaaacaaaagggctaaaaacaaatctatcatctaatttagattatatgtaagttagtaagtctcttcaaaataaagaaaggtagttttaggacagagatttttatatagattgaaagttatcttccctggaagaaaggtgaatctgagaatctagccgcacttcaaaaatgtgtgcaagtgtttatttggaatcccttctattttattagaaacagaaacagtaatttcaccagtaggaattgcgtgtgctctcaatacaagtaagtttgccactccttcaattgttgtccattgcagacactttggattcaaggttaagaatccaaatgagaaataagaaatatccggtccctgatgattcgtttaagtcctgttcaactcgatgaaagcttccacccgaaggaagagttactgttcctcctggctggctttgtgtttctttcagtgctctaaagaactttgtatttgggcagctgtgctctgtcatgtcaggctgctggacaggagttgatgcttacggcgccgctgaccagggctgctttactgaagctcactgggtgtccatcaatcacaaagtggcgtatgcagcctgtgaagggtttgctgggggccaagcgtggtgtcagtagagattctggaacacctccaacaaacacaggctccctgtgatcaattggttttggattcaggggtccaaccacatggttcacttcagagtccacatccaactgaaccacattagaatctctaataactgtaattctgtgccatctgccatcacagagactctgcttgggtgtaactgaggtggaaaaatctctgatgccattattgactttcactatgacctgtccatttttcatgtgaacatttaggtactccccattgacactgtggccgtggaccagggttccggaactgcttctgggacggacttcaaatgcaatttcaaacttcaatccaatattgaaagattcatctagaaccacgtatcctccttctgttgaaaagtaagttcctgtttccatggggccttcaaagcaaggggtcacactgaatgtctgagaagcagaggtgatggaggccccattgagctggagattgctgagacagccactaaaactgtagatggagttaatctgaacatttttcacagcctttccaggagccacacctcccaaataaatgggacccttgattttccaggtagcttcagtaggaggaagactttcttctaggactcggagaccatcaattaccagtcggccactgctcctttctcgaataaatatcacatcatgccacaggccatcattgtatttctcctggcttctaatcttcagttttttgtgaccaacattaaacatgtaaaccaagcggccatgggccaaaaatagagtcatgaagtcattctcttcttgatctgagacatagaagatcatgccatgggaggaacgagttctcagacgaatggaaaactgagatttggcaccaaaatctccttttaagtgttcaaactcttggcggctgttggctgttcctccatattgataggcgtgctctattgctctagggctgttggaaaggtggcaatgagagtttcttggagtattccgctctgggagtttcagagcaacaggatcccatgaaggtgcatctttacttttccctccctttttattctgacttgctttaggcttggataaattttttccttttttatggaggagaaacaatggtgaagactcaatgggacactcataaagagaagtgtggaccttttcagtataccgttggaaatcttcaacctccacatctctatccaccctggtaaagtaggcattacttatgcagccagtgaaattagcatactgagcactgattggtgagccaccgaagtaaaacttcttttcacttgcttgtgtctgttctattttccctttggtaggattcttactcccaactctgcttttatctactatcagttcatatcttgtgggtgagacagagctaatgacgaagtgggacagcccatcattgtactgcttatctactgactgaactttgattccctttacatccatgatgacagtaccattatccagtgagatggagaacacgtctgaccctgaagcataatagaatagtaacccatttggttgtaatgttcggaaattaaaacctccttcaaagccatcaaagaaagatattttctgaattgaagcaatgaagctctgtccattgaaatatgctctgcgagatataagtgagtcttctgggcatccataaccaactcccagggtttctgtctgctccagtaaattgaagtccttcttttggaactggaagcccttcatgcatcctctgaagttgatatctaggggaaggtgtgctctgagggccctggattgtaagatttctggaggagctcctccaatgtatatatctgtaaaaggtattttcatcttttcattatccatgctcttgacatgccttctgtcaactaccaagatcattttcttatcattgtggtaaatgattgagatctcatggtattttgcatcattaatttgagctttctttaacgtatcttcaagatgcacagggccaccgctgaatccaaaatcatagaacacatgtaggtaaccattgcgcatttccagtctgaaaaacatacttccattgaccatcaggagaataaggccgttgtcagctggtgttcgaacttctatgtcaaagcgagtcacctgaccaaatttccctctccttgtgatgtctctcaccacggcataaccggagccatcgaagaagtaactggcagcccgactctgagtgaaggccagcttatctcgggcacatggcactgatgtggaggggtccatattatagatgtgcttaaagttgtacaagctgatcacatcattattcaaagtggccagttccaggcagccaacaaagccaggcaggtttaagctggtagggagcttgaagttggaaggcactccaccaacataaaacactgtgtcctcagggtccaggtccagcagagagtcatctcccgaaaattccccctttttaatgaacttttcctctgctgtgctacttagactcgggactgttaaaaacacctttccatgttttcccaccctttcaatcttgacaatgctgaagtaagcaggccaggaactgacgggcttggagtccaggggaatctccacatctttagttcccaaattatagacgtataccagattatcatttttgattgcaagacccatatactcttttttggcgtttttgcttccgaggtacaggataaactgatctgcagtctcggtcagttccggccgcttcacagggggtttcatgtacaggctcagagacgtgaaggcctttaagtcatccatactggttctcgagtgcacttccacagctgactggccatcaaacatcatggagacttggatcttgctggcaacacttctggtctgagcaatgagctctcggatcctctggatgctggcagaaacgttgcttgcaggtcgcttctgctcaaccgtacgaagctgatccaggagctgagggacaacctcggtcagatttcttactgcatccctagcagagttcactgcagtgttgtaagcagaagagtcaaaatgttgaagattctgtgaccagttggttagattgttggccatgggggcagtggcctgctgcacctccatcgtcgtcctgttggcttcctcggtgatcagtctagactgccccaggcgctgctgggcatcccctctctctgctgcttgtagttgcttaacggcatcactgagtctggttttaagggcacttttccttgctagggctccacccacacgcctgctagtgtcagccactgcttcatcactgctagactctgcctttgcttgcagttctctggcttgattgaggaggttctcactttcatctttatggtaaatgatttgagtatcaatcccactcaccgcatcataaattcggtcagtggtgttcaaagcaaattctgctgtttcattggcttcactaacataattaacaatattttcatagacatttgatgcatccaaagccttctgtaccagcccgttcatatctgaactgtgcaacttcctgctcaattcattagcttcttgttgaaggtcctgtgcatggtcaatagcttcttggactaaatcatggctgaggttacttaggttagatagttttacttgtagttcacttttggctccatctatttctgcataaatccctgacgcattctttattatatcatcaagttctgaaagagttagacgaggtgttgtcagagagtccgcagatgtgctcagagacatgttcaccacttccatttgttccctcactctttcctgttgtttctcatggtcccgctgcctggctgctgtggccctgttcatgtcttcggcatccctgacatagttaagggcctggtcaagtgcttcctggagatctgacaacttagcattgtagtcatccagctgctccaggacgacaggaaacagagtgcgggtctcattgtgcagccgctgccagctctcagcctggctcagtagttcgtaagcctcatctgcctcctcatccacgagctcccgttgggtgaaaaatggttgacggcttctaatctcttcaagcatcttctgggccaacaccagcttctcagagatttccttggggctaagttcatgctcttccccataatagagcatcttgttgttgatctcttggattttatccctcatatcatgggcttgctctaccagctgacttgcgtggttaatggtgtccatgctttccttctgaacaagttgtccttttctggaggcttgattttccttttcaactaattcctctacgtcagacagaaggcttttcatcgtgttctcagcattgttgatttgtatctttcttagggcgtattggttttctctttctgacaattttgttttgaggaggtagatggtggcgttgatttcattcacgtgcctatgagcggcggccccagaggatacgctcagcaccccggatttgccttcctcgatggagagcgctgctaaccgcaggtcatcagtcaggtcccagacgcacttatcacagcctgtagggggttcaaaaccttcttccaagcattctccggttacactgtcacatgggcctcccccgcagttgcacactgcacagttcttggctatcctggcgtccccatagtagccaggagcgcaacgttcacacttgaatccggtggtgttgcgtaagcaattcctacactggccagtgacttcatcacaatcttcaaagatcaggttgggatctgaatttccactgcagtcacatttcttacaggtgcttccaatgagtaaggggtttccatagtaaccgggagcacatctttcacagttaggtccagcataattttcgttacaaatgcaccgaacagctccatttttcctatagcaggattctgcaaaattggccaagtggggcaggggacaggggcacggctggcagaattggggtgctcccctgatggaatctccgatataaccatccagacacttttcacagtgctctcctgttgtgttccgctggcagtgcacacagtatcctgagccgtccaaacactcgttggaattgccattacagtcgcagggcacacattctcccgacagggtgtgaaagaatccagcattgcatttctcggccgcaggcggcaggcgtcccagagccacgcggggttcgctcgtctcaggcgggtcttgcctgccaaccgctgagctcccttcaatgtcaaaaggaaaagcgttgtcgtccccggacgcggcgcgggagcaggcagcgctccagaggagccacagaggcagaaccgagcgccaggctgagctcaaagccatttctccgctgacatccagtagtgctcttccagggctcgggcgctgtgggtctccgtaggtctcccgcgtggtgcggcggtgcctcgcttattttccctcctctccgtgtgcagtatcccgaggtggctgcgcaaccagcagagtacggcatcaaaaggcagacggattggggtgagccccgccagcgctaggccacctcctctccctggccgttcgggactggggactgcgctgtcctggcttccttctc

SEQ ID NO: 11611 - RNA, 6616 nt, Homo sapiens
  source 1..6616: mol_type = other RNA
ctgaatagctgggactacaggtgtatgcccatgtacaaatttttttgcagagatgggatctcattatgttgcccaggctaggagcaaacttttaataaaaggacttgtgtactcttaaattgaattttatgattttgtcctactgtttttgctgtgatatcctcaatgattcccatagaacacacaataatggtaataataacctacagaagcctcctctcatgtacaattttatttttcttttaaggagataaggaaggggaaaaagtagttgatttcctgtgtttcttatttagaaaaaattaaattatactgcatttttctagtattctgttagaaatttactttattaaaccttgataacttcagctataaacctaaaatattcttcttatactgatagaccaaacaaaagggctaaaaacaaatctatcatctaatttagattatatgtaagttagtaagtctcttcaaaataaagaaaggtagttttaggacagagatttttatatagattgaaagttatcttccctggaagaaaggtgaatctgagaatctagccgcacttcaaaaatgtgtgcaagtgtttatttggaatcccttctattttattagaaacagaaacagtaatttcaccagtaggaattgcgtgtgctctcaatacaagtaagtttgccactccttcaattgttgtccattgcagacactttggattcaaggttaagaatccaaatgagaaataagaaatatccggtccctgatgattcgtttaagtcctgttcaactcgatgaaagcttccacccgaaggaagagttactgttcctcctggctggctttgtgtttctttcagtgctctaaagaactttgtatttgggcagctgtgctctgtcatgtcaggctgctggacaggagttgatgcttacggcgccgctgaccagggctgctttactgaagctcactgggtgtccatcaatcacaaagtggcgtatgcagcctgtgaagggtttgctgggggccaagcgtggtgtcagtagagattctggaacacctccaacaaacacaggctccctgtgatcaattggttttggattcaggggtccaaccacatggttcacttcagagtccacatccaactgaaccacattagaatctctaataactgtaattctgtgccatctgccatcacagagactctgcttgggtgtaactgaggtggaaaaatctctgatgccattattgactttcactatgacctgtccatttttcatgtgaacatttaggtactccccattgacactgtggccgtggaccagggttccggaactgcttctgggacggacttcaaatgcaatttcaaacttcaatccaatattgaaagattcatctagaaccacgtatcctccttctgttgaaaagtaagttcctgtttccatggggccttcaaagcaaggggtcacactgaatgtctgagaagcagaggtgatggaggccccattgagctggagattgctgagacagccactaaaactgtagatggagttaatctgaacatttttcacagcctttccaggagccacacctcccaaataaatgggacccttgattttccaggtagcttcagtaggaggaagactttcttctaggactcggagaccatcaattaccagtcggccactgctcctttctcgaataaatatcacatcatgccacaggccatcattgtatttctcctggcttctaatcttcagttttttgtgaccaacattaaacatgtaaaccaagcggccatgggccaaaaatagagtcatgaagtcattctcttcttgatctgagacatagaagatcatgccatgggaggaacgagttctcagacgaatggaaaactgagatttggcaccaaaatctccttttaagtgttcaaactcttggcggctgttggctgttcctccatattgataggcgtgctctattgctctagggctgttggaaaggtggcaatgagagtttcttggagtattccgctctgggagtttcagagcaacaggatcccatgaaggtgcatctttacttttccctccctttttattctgacttgctttaggcttggataaattttttccttttttatggaggagaaacaatggtgaagactcaatgggacactcataaagagaagtgtggaccttttcagtataccgttggaaatcttcaacctccacatctctatccaccctggtaaagtaggcattacttatgcagccagtgaaattagcatactgagcactgattggtgagccaccgaagtaaaacttcttttcacttgcttgtgtctgttctattttccctttggtaggattcttactcccaactctgcttttatctactatcagttcatatcttgtgggtgagacagagctaatgacgaagtgggacagcccatcattgtactgcttatctactgactgaactttgattccctttacatccatgatgacagtaccattatccagtgagatggagaacacgtctgaccctgaagcataatagaatagtaacccatttggttgtaatgttcggaaattaaaacctccttcaaagccatcaaagaaagatattttctgaattgaagcaatgaagctctgtccattgaaatatgctctgcgagatataagtgagtcttctgggcatccataaccaactcccagggtttctgtctgctccagtaaattgaagtccttcttttggaactggaagcccttcatgcatcctctgaagttgatatctaggggaaggtgtgctctgagggccctggattgtaagatttctggaggagctcctccaatgtatatatctgtaaaaggtattttcatcttttcattatccatgctcttgacatgccttctgtcaactaccaagatcattttcttatcattgtggtaaatgattgagatctcatggtattttgcatcattaatttgagctttctttaacgtatcttcaagatgcacagggccaccgctgaatccaaaatcatagaacacatgtaggtaaccattgcgcatttccagtctgaaaaacatacttccattgaccatcaggagaataaggccgttgtcagctggtgttcgaacttctatgtcaaagcgagtcacctgaccaaatttccctctccttgtgatgtctctcaccacggcataaccggagccatcgaagaagtaactggcagcccgactctgagtgaaggccagcttatctcgggcacatggcactgatgtggaggggtccatattatagatgtgcttaaagttgtacaagctgatcacatcattattcaaagtggccagttccaggcagccaacaaagccaggcaggtttaagctggtagggagcttgaagttggaaggcactccaccaacataaaacactgtgtcctcagggtccaggtccagcagagagtcatctcccgaaaattccccctttttaatgaacttttcctctgctgtgctacttagactcgggactgttaaaaacacctttccatgttttcccaccctttcaatcttgacaatgctgaagtaagcaggccaggaactgacgggcttggagtccaggggaatctccacatctttagttcccaaattatagacgtataccagattatcatttttgattgcaagacccatatactcttttttggcgtttttgcttccgaggtacaggataaactgatctgcagtctcggtcagttccggccgcttcacagggggtttcatgtacaggctcagagacgtgaaggcctttaagtcatccatactggttctcgagtgcacttccacagctgactggccatcaaacatcatggagacttggatcttgctggcaacacttctggtctgagcaatgagctctcggatcctctggatgctggcagaaacgttgcttgcaggtcgcttctgctcaaccgtacgaagctgatccaggagctgagggacaacctcggtcagatttcttactgcatccctagcagagttcactgcagtgttgtaagcagaagagtcaaaatgttgaagattctgtgaccagttggttagattgttggccatgggggcagtggcctgctgcacctccatcgtcgtcctgttggcttcctcggtgatcagtctagactgccccaggcgctgctgggcatcccctctctctgctgcttgtagttgcttaacggcatcactgagtctggttttaagggcacttttccttgctagggctccacccacacgcctgctagtgtcagccactgcttcatcactgctagactctgcctttgcttgcagttctctggcttgattgaggaggttctcactttcatctttatggtaaatgatttgagtatcaatcccactcaccgcatcataaattcggtcagtggtgttcaaagcaaattctgctgtttcattggcttcactaacataattaacaatattttcatagacatttgatgcatccaaagccttctgtaccagcccgttcatatctgaactgtgcaacttcctgctcaattcattagcttcttgttgaaggtcctgtgcatggtcaatagcttcttggactaaatcatggctgaggttacttaggttagatagttttacttgtagttcacttttggctccatctatttctgcataaatccctgacgcattctttattatatcatcaagttctgaaagagttagacgaggtgttgtcagagagtccgcagatgtgctcagagacatgttcaccacttccatttgttccctcactctttcctgttgtttctcatggtcccgctgcctggctgctgtggccctgttcatgtcttcggcatccctgacatagttaagggcctggtcaagtgcttcctggagatctgacaacttagcattgtagtcatccagctgctccaggacgacaggaaacagagtgcgggtctcattgtgcagccgctgccagctctcagcctggctcagtagttcgtaagcctcatctgcctcctcatccacgagctcccgttgggtgaaaaatggttgacggcttctaatctcttcaagcatcttctgggccaacaccagcttctcagagatttccttggggctaagttcatgctcttccccataatagagcatcttgttgttgatctcttggattttatccctcatatcatgggcttgctctaccagctgacttgcgtggttaatggtgtccatgctttccttctgaacaagttgtccttttctggaggcttgattttccttttcaactaattcctctacgtcagacagaaggcttttcatcgtgttctcagcattgttgatttgtatctttcttagggcgtattggttttctctttctgacaattttgttttgaggaggtagatggtggcgttgatttcattcacgtgcctatgagcggcggccccagaggatacgctcagcaccccggatttgccttcctcgatggagagcgctgctaaccgcaggtcatcagtcaggtcccagacgcacttatcacagcttatggttgggcagtccatgcctgtagggggttcaaaaccttcttccaagcattctccggttacactgtcacatgggcctcccccgcagttgcacactgcacagttcttggctatcctggcgtccccatagtagccaggagcgcaacgttcacacttgaatccggtggtgttgcgtaagcaattcctacactggccagtgacttcatcacaatcttcaaagatcaggttgggatctgaatttccactgcagtcacatttcttacaggtgcttccaatgagtaaggggtttccatagtaaccgggagcacatctttcacagttaggtccagcataattttcgttacaaatgcaccgaacagctccatttttcctatagcaggattctgcaaaattggccaagtggggcaggggacaggggcacggctggcagaattggggtgctcccctgatggaatctccgatataaccatccagacacttttcacagtgctctcctgttgtgttccgctggcagtgcacacagtatcctgagccgtccaaacactcgttggaattgccattacagtcgcagggcacacattctcccgacagggtgtgaaagaatccagcattgcatttctcggccgcaggcggcaggcgtcccagagccacgcggggttcgctcgtctcaggcgggtcttgcctgccaaccgctgagctcccttcaatgtcaaaaggaaaagcgttgtcgtccccggacgcggcgcgggagcaggcagcgctccagaggagccacagaggcagaaccgagcgccaggctgagctcaaagccatttctccgctgacatccagtagtgctcttccagggctcgggcgctgtgggtctccgtaggtctcccgcgtggtgcggcggtgcctcgcttattttccctcctctccgtgtgcagtatcccgaggtggctgcgcaaccagcagagtacggcatcaaaaggcagacggattggggtgagccccgccagcgctaggccacctcctctccctggccgttcgggactggggactgcgctgtcctggcttccttctc

SEQ ID NO: 11612 - RNA, 16348 nt, Homo sapiens
  source 1..16348: mol_type = other RNA
ctgaatagctgggactacaggtgtatttttgtatttttagtagaggtggggtttcaccatgttgaccaggctggtcttgaactcctgacctcaagtggcgcacccaccttggcctcccaaagtgctcggattacaggcatgaaccacttctcctggcctctactttatatatttctatagatgtgcctattctgcgtatttttaaaattttatttattttattttttgagacaatatctcactcttgctcaggctggagtgcaatggtgcaatctcagctcactgcagcctcaacctccctggctcaagtgatcttccctcctccctccctcgagtagctgggaccacaggtgtgcaccaccatgccccaataatttttgtgtattttggttgagatggggttttgctatattgcccaggctggtctcaaactccagacgtcaagtgatccacctgcctcggctcccccaggtgctgggattacaggcgtgagccacagtgcctggcctattctgggtattttaataaacagaatcatagaatatatgaccttctgtttttattttcttttattcagcataatgttttcaagtttcattcatgtcatagcatgtatctgtacttcattcctttttattgccaaataatattccattgtataggatataccacatttccttaatccatccagtgatggacatttggcttgtttccacttttggctgtcatcagtaatgctgctatgaacatttatgtacaggattttctgtaaacatgttttcatttctgttgggtatatacctaagtgtgaaatttctgggtcatatggtaactctggttaattttttgaggaactgccaaattgttttccaaagtggcagcagcattttacgttcccaccagcaactggaactaaggttccagtttccccacatcctcaaccgaacttgttactgcctctcattttttattctatcccatacaaagtaggtatgaactggtatgtcatggttttgagttgcattttcctaatgactaatgatgttgagcatcttttcaagtgctctctctccagtttttaaaataaaactttgcaaacattcagaaaatctgaaagaattgtacagagaacattggtgtacatcggccgggcacggtggctgacgcctgtaatcccagcactttgggaggccaaggcaggcggatcacgaggtcaggagatcgagaccatcctggctaacacggtgaaaccccgtctctactaaaaatacaaaaaaaattagccgggcatggtggcgggcgcctgtagtcccagctactcaggaggctgaggcaggagaatggcgtgaacccaggaggcggagcttgcagtgagccgagatagcgccactgcactccagcctgggagacagagcgagactccatctctaaaaaaaaaaccaaaaaacaaaacattggtgtacattggtgtacatttcagctagattcagttattaacatttagcagtgtatacacttttattactttcactctctatacatatatatgtgcacatctatacacacgtatatctaactttttgctgatttaaatcttgtatcgtgacacttcatagatcaaaataatcccttaaccacattcttctacatacccacaatagcagaattatatgtaagaaaatttaaaattccatcactcatattcatagattcatattcaaatatcaattgtcacaaggtttttttttttagtagcattttttttcaaagaccagaatccatccaaaattcacaaactgcatttggttgttgtatcttattgtaattgctgacaatcaagttttaatttggttggaacatcaatcttttctagttagtccttttctgtgtctcatttaagaaatcctttccaaccctggaattacaaagatatttacctacatatcttccaaacatttaaattgttttgcacttctgacaaaaatgtagtataaattagggattcaatttcatttttctgcatatgaataaccaaatgtctcagcctcttcttttcctcagtaacatataatgctggttttcctatgctgtgtgtgtctgttggtcaatttgttcacatttgggctaattccgtactgtattaattatagctataaaatattaaatttattaaattaatattgaattaattcttaatttagcttatgaatattaattatagctatagctttgaaataaacattgatatctggcagagcaagaaccatcattattccctaagtcattaccatcacaactttattcttatttttcagtagtatttcgattattcctggcccttgtcaatttctgtaaaaaatataggtgtgagccatgtatttctcttcagtcattttggtaacttattctccagatatttgtctatttcatctaaggtctcagttggctggcataaagtttttagggtattaacaataaatttattcaggatctgtagctattacatgttttttcatttttaattttatcgttgacttgtctcttttttattttattttattttattttattttttgagacgcagtctcgctctgtcgcccaggctggagtgcaatggcacgatctcagctcacggcaagctccgcctcccgggttcaagtcattctcctgtctcagcctcctgagtagcttgggactacaggcgcccgccaccatgcccggctaattttttgtatttttagtagagacggtgtttcaccgtgttagccaggatagtctcaatttcctgacctggtgatccgcctgcctcagccttccaaagtgctgggattacatgagccaccgcgcccggccgccttgtctcttattctctaaatcttactattgacgtccaagttactatttttgagagagggtctcactctgtctcccaggctggagtgcagtggtgtgatcttggctcactgcaacctctgcctcccaggctcgagccatcctcccacctcagcctcccaagtagatggaactacaggcacaacaccatgtccagctaattttgtaatttttttttttttttttttttttttttttgtgacggagtctcgctctgtcgcccaggctggagcacagtggcgcgatcttggctcactgcaagctccgaccccgggttcacgccattctcctgcctcagcctcccaagtagctgggactacaggcgcccgccaccgtgcccaggtaattttttgtatttttaatagagatggggtttcaccgtgttagccaggatggtctcaatctcctgacctcgtgatccgcccgcctcggcctcccaaagtgctgggattacaggcgtgagccaccgcgcctggcctgtactctttttttttttatagagacggggttttgccatgttgcccaagctggtttcaaactcctggactcaggcgatccatctgccttggcctcccaaagtgcagggattataggcatgaaccactgtggcaggctaacatccaaattattttgtcttaaaacaccaacttttacctttttttaaatcttctgtattacatctttgttttctgctttatgggttattcctcttacagtgttatctcttccctctactcttttagggtttattctgttatgttttaatgttttaaactgagtgtccagtgtattaacactcagtctatcctttaagatataagtatttaaaactacaaatgtctatctcccactttctctgcctttttttattatagaatatttcaaacatatacaaaattggacagcataacaaaccgccatgcatccatcaactagcttgctgaagcaagatatttgaatataaaataaatgatcaattcatcttaatactgacccactctcttcttggcatcgtattatttttaagacattctcagacatcagtgcatcccatgttttgatatagtattttcattactatttacttctaagtgttttacttttataatttatttataaagttacttagaagtgtttttttaatttccaaaagtattgattttttgtgggggtatcattttgtattgactgctaattgtattgtgttcaaagactagggtctaaattaaactaatctttttttttttttttttttttttttgagacagagtcttgcactgtcgcccgggctagagtgcactggcaccatctcggctcactgcaacctccgccgcccagtttcaagcgattttcctgcttcagcctcctcagtagctgggattacaggcagccgacaccatgcccagctaattttttgtatttttagtagagacggggtttctccatgttggccaggctggtctcgaactcctgacctcgtgattcgcctgccttggcctcccaaagtgctgggattacaggcatgagccaccgtgcctggcctaaactaactcttttacatttgttgagacagtgcacttctatttcaggagtcagatactcatctaagtatatattgtaaaagctgtatctatactaatatttttgtctgcttgatcaatagttgaaatcttccattatgatggtagacttgtcaaaacttccctatagttctgtcatttgtttttaacaagtctgttttgttaggtaggtagcagtttcaaattatacaatttgggtgatttaaaccttttttcattataaagtgactcatttacaatgcattctatcttagggaccattttagctgatgtatagctacttcagctttctcttggtcatatctacctacgacaagttgagcatccctaatctgaaaatccaaaatgctccaaaatctgaaacattttaagcaccaacatgatgctcaagggaaatacaccttttctgagttctaaatgttatatagtgcatagaactggatttgttgttgttgttgttttgttttagagacagagtctcactctgtgccccaggctggagtgcagtggcatgatcttggctcactgcaacctccacctcccaggttcaagcaactctcctgcctcagcttcccaagtagttgggattactggcatgtgccaccagacccagctaatttttgtatttttagtagagaccgggttttgccatgttggccagggtggtctggaactcctgatctcaggtgatccgcctgccttggcctcccaaagtgttgggattacaggcatgagccaccacacttggcctaaaactggatttttttttttttttttttttttttttttttttgagatgaagtctcgctctgtcgcccaggctggaatgcagtggcacgatctcggctcactgcaagcttcacctcctgggttcatgccattctcctgcctcagcctccggagtagctgggactataggcgcctgccaccatgcccggctaattttttgtatttttgtagagatgaggtttcaccgtgttggccaggatagtcttgatctcctgacctcgtgatccgcccccctcggcctccccaagtgctgagattatagacgtgagccatcgcgcctggctagaactggatatttaaaatccagtaaatatttggtaaatttactacatcccatatatttcaactagtaataaattcggatttacttgtcgtcatcttcttttgtgtttatgttagccttatttttctaattcggcagtccccaaccttgttggcaccagggactgatttttgtggaagacaatttttccactgatgcggtttttttcccatggatgggggccggggcgggcatggttttgggattaaactgttccacctcagaaaatcaggcagtagattctcataaggagcacgcaacctagatccctcacatgcgcagttcacaatagagtttgtgctgctgtgagaatctaatgcagcagctgatctgacaggaggcggtgctcagggtaggtttgccgctcgcttcctgctgtgcagccaggtcctgaacaggtcagggacaggcagcctgggggggttggggacctctgctgtgttgttttcccctgttgttcttgctgctactaaactgataaagctttctttattttccctctacaactttggaagttacacattttgattctttagtaattatgctaaaaaacgacagctttcatacttaaagcctaaagttaatcaagatctttatactctgctcccaaagaaatggaaagctcttagaacactgtaattctgatcactgaactactgttttcagcatcttttgtttttgagacagggtctcactctgttgcccagactggagtgcactagtgcaatgaatcatagctcactacagttttgaactctgggcttaagggatcctcctgcctctgcctgccaagtagctgggactacaggcatgctactgtgcatggccaacttttttattttttttagagaccaggtctcactatgttgcccaggctggtctcaaactcctgggctcaaacgatcctcctgccttggccttccaaagtgctgggattacaggtgtgaaccaccatgcccagccggtttttaattttttaatatgcctccaaaggagacattatcatggttttctactgttcatattgggttatatttgcccggatcttcatcagtcttttttgttaatcactgtctattatgtatcacttcttccttcattgagtttttaaaattcatgtggcatatatttcagtaggcttttcagtgagggtctgttatcctgaagtctctcagtctttgagaagtctttaattcactttcattcttggatgataactagaaatcaaattccagattgacagttatttttctctattattttgaagctactgtattgtctctgatttctatggctgctatggagaacttctaccagcaggttagattcttgtgggtaaactctctttttctttctggttgcttttaagctttttctctttgtctctgttgttctgcagtattatttttatttatccctggctcgctgcatttcctaaatgtgaagattcatgtctcattaatcattttcagccattatcacttttaatattgccttgctcccctactcgattctctcctcctagaacttctacaggacatacgctgaatattctcattcaatttttcatgcctcttaacacgtattctccatcactactccattcttgctaatttccccaacttcattttatagtttattcttttttttttttttttgagatggagtctcactctgtcacccacactggagtgcaatggcacgatcttggctcactgcaacctccacctcccgggttcaagcgattctcctgcttcagcctctcaagtagctgggattacaggtgcacgccaccaggcccagctaattttttttgttttttttaatagagacagggtttcaccatgtgtaccaggttggtcttgaactcctgacctcatggtccacccgcctcagcctcccaaagtgctaggattacaggcatgagccaccgcgcccagtccggtttattcattttctgtgtcctaatatcttcattaagttaatttccagtacagttgtacctcagtatctgcagggagttggttccaggatccctttgactatcaaaatccacagatgctcaagggccctatataaaatggtgtcttttctggtgttttttgtttttgttttttgagacaaggtctcattctgttgccaggctggagagcagtggctcagtcacagctcactgtagcctcgacctcctgggctcaggtgattctcccacctcaacctaccaagtagctgggactataggcacgtgccactatgcctggtcaatttttgtattttgtgtagacagggttttgccatgttgcccaggctggtctacaactcctgggctcaagcagtctgcccacctccatcccccaaaaacgttgggattacacgtgtgagccaccatgccaggcctggagtagtatttgcatgtaacctatgcacatcctcccatatactttaagtcatctctggattacttataatatctaatacaatataaatactatgtaaatagttgttacactgtattttaaaatatgtatatttttattgttgtattattttttcaaatctttcccatcacattagttgattctgaagatgcagagcccgtaaatatggacggccaactatgttgtatttctcatttctgaaaattctatttagtttctaaagtttgtttccttcttctaaatatatttaaatatactttatttgtagcctctgcttaataattctattatctaaagtccttgggggtttaaatcttattgccttctgactcttatgataaattgtttccttgcatgttctattattttgaattgtgatctcaacttcattggggtttcatatgtggatatcctgttaggtctgagttaacatgcaacaatctagaaattctgtttccttctggcaactgccctagaaatacttttcatattaagttcacaggattcgcagaccacacaggtagtataaatttgaatcccaaactggtgaaaaggtaggtctatggtgacaaattcccaggaatgacttttattctctgtaccatgagtccaagctaacacaagcactagagggtggattttgttttttaatccttccattgagggtgaatgtctttaaaggtcctggctttgtatgtggatctcaatccaacttctcaccttgtaggggggcctaagactttacctcgagtgtccttgcgtgacctttaaaacccgagcatactggttacagaaactagggactgtctttacgcccaggcagtcacaaagcataaaccacacaccatactgttgttaaatttcctgtttagggctccgcccaggctggaatgcaatggcatgatctcagctcactgcaacctccatctcccaggttcaaatgattctgcctcagcctcccaagtagctgggattaccggcatgcgccaccatgcccagctaatttttatatttttagaagagatggattttcaccatgttggccaggctagtctcaaactcctgacctcaagtgatccgcctgcctcagcctcccaaagtgctgggattacaggcgtgagccaccaggcctggcggaaccttgatcttttaaatgtgaatttcagatatttctattacctgtaaggagagaggtggggaagacgaaggttgaagggaatattgaataaataactcctgtgtactagccctcaatacatgagatatttgataacagctatacaaaacaagccatgttaatagatgagaaattaaagctcagaaaggtcaaataatttcgctaaggtcacaatgtactattacacccgaattcacgttggaattaactagtcagatccattttcattctggacatggtggtgtatgcctgtagtcccagctatttgggggcctgaagtgagaggactgcttgtgcctaggaattcatgtacagcctgggcaacatagcaagaaactgcttctaaaaataaataggctgggtgcagtggctcacgcctgtaatcccagcactttgggaggtggaggcaggtggatcacttgaggtcaggagttcaagaccagcctggccaacacggcgaaaccccatctctactaaaaatacaaaaaattagctgggtgtggtggtgcgtgcctgtaatcccagttacttgggaggctgaggcaggagaagagctttaacccaggaagcagaggttgtggtgagctgagatcacgtcactgcactccagcctgggcaacagagcaagactctgtctcaaataaaaataaataactttgggaggccgaagtgggaggatcccgaggtcgagatcgagaccatcctggctaacacagtgaaaccccatctctactaaaaatacaaaaaattagctgggcatggtggcaggcacctgtagtctcccagctacttggaaggctgaggcagaagaattgcttgaacctgggaggcggaggttgcagtgagccgagatcgtgccactgcattccagcctgggcaacagagagagactccatctcaaaaaattaaaaataagttaacaaataatcaattttcttcctctacagcagaggtcagcaaacttattctgttaaaggccaaacagtaaatattttaggcctcataagccatatggtattggctgcaactattcagttttactgttgtatcattaaagcagccactgaaaagtgtaaacaaatgagcatgactgtgttcccataaaactttaaggacattgacatttgaatttcataaaattttcacatataacaatactattattacttggatcttttccccaaccatataaaaatttaaaacccgttgctaatgcatgggtcttacaaaaacagcctggagttgacccacgggccgtggtttgctgacccttatcatacaccataacacctccttggaagtacacctctctaatgcctttgttccaaacaatactgggttaggaaagacatggaaaaaggaaaatgagatacattattttttgtaccctatgggggattgaggggttgttgctacatagccccctcaatttgtgctgtagcaatatgcagttaagatccttattctaatgttaaatgtctcttctgtggcttatcctaactttaaaaaaaaaaaaaagaagccatcttacgtaaatgaacttacaattttaagacagggtctcactctgtcacccaggctggagtgcagtggtacaatcacggctcattgcagcctcgacctctcaggctcgagagatcctcccaccccaacttcccaagtagctgggactacaggtgtgcaccactatgcctagctcatcttttttttttttttttttttcctttaaaagatatggagtctcgctattttgcccaggctggtcttgaactcctggactcaagcaatccacctgcctcagcctcccagagtgttgggattacaggtgtgagccactgtgcccggcctgaattatcttcttattgtaaaatttcctttaatgcttaatagttgatgtatattaagtgctaactaaatgttcactgataaacattaatcagatgctgctaaatattgtctttctttattcacagatgatagtcaatgggcacaacatataagtagttacaatgaaatgagaagcaatatagcagtcaggctatatgcatgatttaacaacaaaattatcacttccttttaatttagaataagggacaatttaaaaagcatctcttggccctatcatttctgttccagtagttagtgttcatatgtgaatactaagtttgacattcctttctcccatagaaccattttggtgatttggatggtggccactacactgctttctgcaagaattcagtcacccaggcctgatatagctttgataacacacgagtcagtgagattccagatacttctgttcaaaatgctatggatctcctgttctatagctgccagcccttttccataccaatacaaaagcgttaagagccaggaaaatggtgtttcctgaacactgcaaaacaagcagtcagcatctggtggtagagttttgcttggtcattaaactcttagaacttacttgcatcattaacatttttatgccttgtgggcatgttatacaacctttcatcttaagataaatctgtcgtccagaagatgggtcttggttcactaaaaaaggcagtgtgaatataatgcaatgctaatggatgcaggccttcaaaacactgcaattatatagtgagttcaggtttcaaaattcagtgtttatcagaaaatatctcataatcatatatattcaacaaattattttccaaagatactcatgaagctaaacaaaaataatttttgttcaaatggctcgatgagtttaagaatatgatttgaatatatttgatataataatttagccaagaagtggtctcttagactaattgtaaaacatgaaaagttgtcagcttcacaatttgaaccccatcctttcatcttctccctgagagcctgctaatggtggtctctttctgaagcacttttagaatcttatttttatatggagtgttttactgactatatatatagcaactgagtccctcggttaaataaattataagctcctttaaccctcttaatacatcactctgtaaagatgtagtttataatgcagttcactttgcaatcatgcctgactcccggcatttttactttaatatttagaatgaatattctcaatatgtgagaatactagtcttgaaagaatgactctgggtgttattatatagcacgtgtgtatataaaatctatggttttactgtcctatatttgataatacaatattaaagacagaacacccacagggttataaattatttttctcattaagattttaatgtagctgtaaatgaaattctcgttttaaaaaaattaaagtttccatttttttttttagaataaagatttagtgcacaaatacagcccaaagccaacagaaaaattgctttgccctgtcatttccctaagaaagcactgaagttaactcaaaataggctgaaagaaaaaaagcaatcctctgagttctaggtttcacaaaaggaccacgtgttaaactatgtacatcgatttgatgtgcaagtatgcaataaatatgtacacatacattcctatctgctttacatcattctagagtattcatagtatatcaagatgggatttagaaatgtgaaaaggccataacagtgaaaaggaaaaaaaaaagataacaatagtttttagaccagtcgaataataatgcttagctagttaattattttaactttggagcagactaaaaaagttgttttgaaataaatggtacctgtaagtgatgattactgcaatacttgttaaatgttatttgtcagcactgaccggaattatatagtgctagtaacacagctcccactgtcctagaattcctctaaatggccagctatagctaccattatcctgataagcatttcaagagttgtgttgctgagccttttaaaagataactagtttataacctatgtctccttatgtggctacatcagttactcgtggtcccaatgaagtataaaagaggatataagctgctgaagatttcacagaagaaacggagatatcagaaacttcatgatcatcaaacttaaaccaccgttgtcttgctgcatttttacaataggctgtgtagtggcctccatccagcccaccgtagtgatttgaaacagaaaacaaattatatttcttcaaattgttctttggaccaataacatactgtgacaagtcaagattttctaacgggaagtccacagatgtctgtaatttttgtttccacctgccatcgtaggaaaaacgtttcagatgcactaaaagcacaggtggtaacttccagatttctatcttttttagagaatcccgtcgagctctgcaatgactgcagtaaaatctgttgttatctgtgagtttttcttctttggaaaataatctaaggcaatcctgtaatgtacatttacttgtggatgctagtggtagagacaaatacatgaaggcctcaaatgtcctagactttttgtgacatgtgaggcactgtactgtagatttgaattgaccctgaaaaagtgcaacaataatagactcattgagctgcttgtgtttctgccaggcatgttctgcagctttaaagtcatcgagatgatcattattttcttctttatatctcttccgattatcagctttatttagatcttcatggagaccatccattaggaacagaagcaattcttgtgaatcttgctgactgtatcctgcaaactggtcattgatcttcccaatggtgattttaaagtcctttggactgatatatctatactgtcctgtccacagggctttcatgattataccaaattcttctgccacttcacctttatgccccaacaaatttgacctgttaatatcatcctgataacagtttcggttgaaataatcagccaaatgtggagcgttacataggcactgcaatattgagttcatataacaagtatttcctaagttacgaagtccagtaagagctggtccagaacctccaaaaacaggattgaggttccgaatctgagaagcagaaagccttgagatctcagctttaggataacatgttggcttgttttcccgattaactgttggagttactgttggcttcctcttctcttcctcttgaatagcctgggttatatctggggaggagtaggagcgcttcagtttggaaggttccctatcccgctcagcaggaatctgtggcttggctttatgagttggaggggtggaaggaggtgcagatgaaggagccatttccggtgggtacatatgaacagtgttggtgggtgaatgataataacgaaaggttccagtgattgggtcaagaaacttggcccagcctgaaggcagtcctggtacgatcctccccatttcttcacttcgtgctcttgtcaaaggttctcgttgagccttgcctgaacctgaatcccctgtcacagatgtatggggcacatctcctgttgactttttctgtatttctggggttggacaccttttccccctatcttctacagatttcttggcatcagaagtttcatgttcacttttactttgtctttttactcctgttatttctttgcccctctttgctgaggtttctttatcttctttcttggcctgttcactttctttcttctccatttcttcttttgctttttgttgcttctctgtaatttcattttcttcagcttcttgtttctttttggctttttgttcttgttcttccttcctcagtttctctttctgttcctcttgctgcctttcccgaagttctttttcttgtttgtttttttccattagaagagcagtttctgcatgaatacgagccttttcttcatctgttaacatgagagttggagaaaaaactactggcttggtggaacgatcaggaataacttttccactctgaggagattgttgctcatggtttgtactttcagattttattctatgctcttcaggcaatttgactgctggttttttagtacgatcaatctgtggaacattctttatactaggcactggctgaattatgggtgaaacatcagatttagaagcagcaactggttcaactggagttgatatattcagtggtcccattctctcattttgaccacttatcaattctatattttcatctacttctatagatgcaggtggcgtctgggcagcaggtttagaaggaattgattcttccaatgagggataagtaaaatccaatgagatagacacctcttcattctggcgtcgtgggggtggagtgaccttagcatttgttgtatactggggataacaaaggagccagttttcatagcctccctctaaaaccaaaggctcattgcgcaggacagttttactttcccacttgaaaagtgcatctttcagactccggagagttgttccaatctgtaaatctttggcagaactaaaccagtcaagaagtaccacatactccacattccccctcttcttccatgtgtctttagaatcatctggcaggtgtgcttcaatccaactagcagtgactcctggactgatggcttcttcaggaacactgagagaatgtaaaatacaggaatcctgataatcctgcattcttcgagcatccattataatcaagctgatgtttttatccgtcatcattgtgtatagttcctttgctgtgattgctcctttctctttggtctcacatttttcattcttttcaccattgctcttttgggttttgtctttggaatccaaaacattctccaaagagcctttagccaatgtgccaccatcctctcttcctgtttcctgccttttttgttgtagccgctgtgcttcctcctgcctgtctttttcctcaagttttttccggacttcagcttcttcatatctcttagtgcttattttctctggtttaacttctgtcttcttattaaggtcttttagtgaagaactgaggtagagttctttaggaactgaagccacagcaggcatgatgaattatctttacttttccactttcacaatggatgctatatttccttacaagtgcttctttccgtgacgccgggcgcgcttcactaacgccagccttctcgccaaatgcccatctcccaagaactcgagggagaattagccttggctaccaggacggaagccagcccagctc

SEQ ID NO: 11613 - RNA, 16666 nt, Homo sapiens
  source 1..16666: mol_type = other RNA
ctgaatagctgggactacaggtgtatttttgtatttttagtagaggtggggtttcaccatgttgaccaggctggtcttgaactcctgacctcaagtggcgcacccaccttggcctcccaaagtgctcggattacaggcatgaaccacttctcctggcctctactttatatatttctatagatgtgcctattctgcgtatttttaaaattttatttattttattttttgagacaatatctcactcttgctcaggctggagtgcaatggtgcaatctcagctcactgcagcctcaacctccctggctcaagtgatcttccctcctccctccctcgagtagctgggaccacaggtgtgcaccaccatgccccaataatttttgtgtattttggttgagatggggttttgctatattgcccaggctggtctcaaactccagacgtcaagtgatccacctgcctcggctcccccaggtgctgggattacaggcgtgagccacagtgcctggcctattctgggtattttaataaacagaatcatagaatatatgaccttctgtttttattttcttttattcagcataatgttttcaagtttcattcatgtcatagcatgtatctgtacttcattcctttttattgccaaataatattccattgtataggatataccacatttccttaatccatccagtgatggacatttggcttgtttccacttttggctgtcatcagtaatgctgctatgaacatttatgtacaggattttctgtaaacatgttttcatttctgttgggtatatacctaagtgtgaaatttctgggtcatatggtaactctggttaattttttgaggaactgccaaattgttttccaaagtggcagcagcattttacgttcccaccagcaactggaactaaggttccagtttccccacatcctcaaccgaacttgttactgcctctcattttttattctatcccatacaaagtaggtatgaactggtatgtcatggttttgagttgcattttcctaatgactaatgatgttgagcatcttttcaagtgctctctctccagtttttaaaataaaactttgcaaacattcagaaaatctgaaagaattgtacagagaacattggtgtacatcggccgggcacggtggctgacgcctgtaatcccagcactttgggaggccaaggcaggcggatcacgaggtcaggagatcgagaccatcctggctaacacggtgaaaccccgtctctactaaaaatacaaaaaaaattagccgggcatggtggcgggcgcctgtagtcccagctactcaggaggctgaggcaggagaatggcgtgaacccaggaggcggagcttgcagtgagccgagatagcgccactgcactccagcctgggagacagagcgagactccatctctaaaaaaaaaaccaaaaaacaaaacattggtgtacattggtgtacatttcagctagattcagttattaacatttagcagtgtatacacttttattactttcactctctatacatatatatgtgcacatctatacacacgtatatctaactttttgctgatttaaatcttgtatcgtgacacttcatagatcaaaataatcccttaaccacattcttctacatacccacaatagcagaattatatgtaagaaaatttaaaattccatcactcatattcatagattcatattcaaatatcaattgtcacaaggtttttttttttagtagcattttttttcaaagaccagaatccatccaaaattcacaaactgcatttggttgttgtatcttattgtaattgctgacaatcaagttttaatttggttggaacatcaatcttttctagttagtccttttctgtgtctcatttaagaaatcctttccaaccctggaattacaaagatatttacctacatatcttccaaacatttaaattgttttgcacttctgacaaaaatgtagtataaattagggattcaatttcatttttctgcatatgaataaccaaatgtctcagcctcttcttttcctcagtaacatataatgctggttttcctatgctgtgtgtgtctgttggtcaatttgttcacatttgggctaattccgtactgtattaattatagctataaaatattaaatttattaaattaatattgaattaattcttaatttagcttatgaatattaattatagctatagctttgaaataaacattgatatctggcagagcaagaaccatcattattccctaagtcattaccatcacaactttattcttatttttcagtagtatttcgattattcctggcccttgtcaatttctgtaaaaaatataggtgtgagccatgtatttctcttcagtcattttggtaacttattctccagatatttgtctatttcatctaaggtctcagttggctggcataaagtttttagggtattaacaataaatttattcaggatctgtagctattacatgttttttcatttttaattttatcgttgacttgtctcttttttattttattttattttattttattttttgagacgcagtctcgctctgtcgcccaggctggagtgcaatggcacgatctcagctcacggcaagctccgcctcccgggttcaagtcattctcctgtctcagcctcctgagtagcttgggactacaggcgcccgccaccatgcccggctaattttttgtatttttagtagagacggtgtttcaccgtgttagccaggatagtctcaatttcctgacctggtgatccgcctgcctcagccttccaaagtgctgggattacatgagccaccgcgcccggccgccttgtctcttattctctaaatcttactattgacgtccaagttactatttttgagagagggtctcactctgtctcccaggctggagtgcagtggtgtgatcttggctcactgcaacctctgcctcccaggctcgagccatcctcccacctcagcctcccaagtagatggaactacaggcacaacaccatgtccagctaattttgtaatttttttttttttttttttttttttttttgtgacggagtctcgctctgtcgcccaggctggagcacagtggcgcgatcttggctcactgcaagctccgaccccgggttcacgccattctcctgcctcagcctcccaagtagctgggactacaggcgcccgccaccgtgcccaggtaattttttgtatttttaatagagatggggtttcaccgtgttagccaggatggtctcaatctcctgacctcgtgatccgcccgcctcggcctcccaaagtgctgggattacaggcgtgagccaccgcgcctggcctgtactctttttttttttatagagacggggttttgccatgttgcccaagctggtttcaaactcctggactcaggcgatccatctgccttggcctcccaaagtgcagggattataggcatgaaccactgtggcaggctaacatccaaattattttgtcttaaaacaccaacttttacctttttttaaatcttctgtattacatctttgttttctgctttatgggttattcctcttacagtgttatctcttccctctactcttttagggtttattctgttatgttttaatgttttaaactgagtgtccagtgtattaacactcagtctatcctttaagatataagtatttaaaactacaaatgtctatctcccactttctctgcctttttttattatagaatatttcaaacatatacaaaattggacagcataacaaaccgccatgcatccatcaactagcttgctgaagcaagatatttgaatataaaataaatgatcaattcatcttaatactgacccactctcttcttggcatcgtattatttttaagacattctcagacatcagtgcatcccatgttttgatatagtattttcattactatttacttctaagtgttttacttttataatttatttataaagttacttagaagtgtttttttaatttccaaaagtattgattttttgtgggggtatcattttgtattgactgctaattgtattgtgttcaaagactagggtctaaattaaactaatctttttttttttttttttttttttttgagacagagtcttgcactgtcgcccgggctagagtgcactggcaccatctcggctcactgcaacctccgccgcccagtttcaagcgattttcctgcttcagcctcctcagtagctgggattacaggcagccgacaccatgcccagctaattttttgtatttttagtagagacggggtttctccatgttggccaggctggtctcgaactcctgacctcgtgattcgcctgccttggcctcccaaagtgctgggattacaggcatgagccaccgtgcctggcctaaactaactcttttacatttgttgagacagtgcacttctatttcaggagtcagatactcatctaagtatatattgtaaaagctgtatctatactaatatttttgtctgcttgatcaatagttgaaatcttccattatgatggtagacttgtcaaaacttccctatagttctgtcatttgtttttaacaagtctgttttgttaggtaggtagcagtttcaaattatacaatttgggtgatttaaaccttttttcattataaagtgactcatttacaatgcattctatcttagggaccattttagctgatgtatagctacttcagctttctcttggtcatatctacctacgacaagttgagcatccctaatctgaaaatccaaaatgctccaaaatctgaaacattttaagcaccaacatgatgctcaagggaaatacaccttttctgagttctaaatgttatatagtgcatagaactggatttgttgttgttgttgttttgttttagagacagagtctcactctgtgccccaggctggagtgcagtggcatgatcttggctcactgcaacctccacctcccaggttcaagcaactctcctgcctcagcttcccaagtagttgggattactggcatgtgccaccagacccagctaatttttgtatttttagtagagaccgggttttgccatgttggccagggtggtctggaactcctgatctcaggtgatccgcctgccttggcctcccaaagtgttgggattacaggcatgagccaccacacttggcctaaaactggatttttttttttttttttttttttttttttttttgagatgaagtctcgctctgtcgcccaggctggaatgcagtggcacgatctcggctcactgcaagcttcacctcctgggttcatgccattctcctgcctcagcctccggagtagctgggactataggcgcctgccaccatgcccggctaattttttgtatttttgtagagatgaggtttcaccgtgttggccaggatagtcttgatctcctgacctcgtgatccgcccccctcggcctccccaagtgctgagattatagacgtgagccatcgcgcctggctagaactggatatttaaaatccagtaaatatttggtaaatttactacatcccatatatttcaactagtaataaattcggatttacttgtcgtcatcttcttttgtgtttatgttagccttatttttctaattcggcagtccccaaccttgttggcaccagggactgatttttgtggaagacaatttttccactgatgcggtttttttcccatggatgggggccggggcgggcatggttttgggattaaactgttccacctcagaaaatcaggcagtagattctcataaggagcacgcaacctagatccctcacatgcgcagttcacaatagagtttgtgctgctgtgagaatctaatgcagcagctgatctgacaggaggcggtgctcagggtaggtttgccgctcgcttcctgctgtgcagccaggtcctgaacaggtcagggacaggcagcctgggggggttggggacctctgctgtgttgttttcccctgttgttcttgctgctactaaactgataaagctttctttattttccctctacaactttggaagttacacattttgattctttagtaattatgctaaaaaacgacagctttcatacttaaagcctaaagttaatcaagatctttatactctgctcccaaagaaatggaaagctcttagaacactgtaattctgatcactgaactactgttttcagcatcttttgtttttgagacagggtctcactctgttgcccagactggagtgcactagtgcaatgaatcatagctcactacagttttgaactctgggcttaagggatcctcctgcctctgcctgccaagtagctgggactacaggcatgctactgtgcatggccaacttttttattttttttagagaccaggtctcactatgttgcccaggctggtctcaaactcctgggctcaaacgatcctcctgccttggccttccaaagtgctgggattacaggtgtgaaccaccatgcccagccggtttttaattttttaatatgcctccaaaggagacattatcatggttttctactgttcatattgggttatatttgcccggatcttcatcagtcttttttgttaatcactgtctattatgtatcacttcttccttcattgagtttttaaaattcatgtggcatatatttcagtaggcttttcagtgagggtctgttatcctgaagtctctcagtctttgagaagtctttaattcactttcattcttggatgataactagaaatcaaattccagattgacagttatttttctctattattttgaagctactgtattgtctctgatttctatggctgctatggagaacttctaccagcaggttagattcttgtgggtaaactctctttttctttctggttgcttttaagctttttctctttgtctctgttgttctgcagtattatttttatttatccctggctcgctgcatttcctaaatgtgaagattcatgtctcattaatcattttcagccattatcacttttaatattgccttgctcccctactcgattctctcctcctagaacttctacaggacatacgctgaatattctcattcaatttttcatgcctcttaacacgtattctccatcactactccattcttgctaatttccccaacttcattttatagtttattcttttttttttttttttgagatggagtctcactctgtcacccacactggagtgcaatggcacgatcttggctcactgcaacctccacctcccgggttcaagcgattctcctgcttcagcctctcaagtagctgggattacaggtgcacgccaccaggcccagctaattttttttgttttttttaatagagacagggtttcaccatgtgtaccaggttggtcttgaactcctgacctcatggtccacccgcctcagcctcccaaagtgctaggattacaggcatgagccaccgcgcccagtccggtttattcattttctgtgtcctaatatcttcattaagttaatttccagtacagttgtacctcagtatctgcagggagttggttccaggatccctttgactatcaaaatccacagatgctcaagggccctatataaaatggtgtcttttctggtgttttttgtttttgttttttgagacaaggtctcattctgttgccaggctggagagcagtggctcagtcacagctcactgtagcctcgacctcctgggctcaggtgattctcccacctcaacctaccaagtagctgggactataggcacgtgccactatgcctggtcaatttttgtattttgtgtagacagggttttgccatgttgcccaggctggtctacaactcctgggctcaagcagtctgcccacctccatcccccaaaaacgttgggattacacgtgtgagccaccatgccaggcctggagtagtatttgcatgtaacctatgcacatcctcccatatactttaagtcatctctggattacttataatatctaatacaatataaatactatgtaaatagttgttacactgtattttaaaatatgtatatttttattgttgtattattttttcaaatctttcccatcacattagttgattctgaagatgcagagcccgtaaatatggacggccaactatgttgtatttctcatttctgaaaattctatttagtttctaaagtttgtttccttcttctaaatatatttaaatatactttatttgtagcctctgcttaataattctattatctaaagtccttgggggtttaaatcttattgccttctgactcttatgataaattgtttccttgcatgttctattattttgaattgtgatctcaacttcattggggtttcatatgtggatatcctgttaggtctgagttaacatgcaacaatctagaaattctgtttccttctggcaactgccctagaaatacttttcatattaagttcacaggattcgcagaccacacaggtagtataaatttgaatcccaaactggtgaaaaggtaggtctatggtgacaaattcccaggaatgacttttattctctgtaccatgagtccaagctaacacaagcactagagggtggattttgttttttaatccttccattgagggtgaatgtctttaaaggtcctggctttgtatgtggatctcaatccaacttctcaccttgtaggggggcctaagactttacctcgagtgtccttgcgtgacctttaaaacccgagcatactggttacagaaactagggactgtctttacgcccaggcagtcacaaagcataaaccacacaccatactgttgttaaatttcctgtttagggctccgcccaggctggaatgcaatggcatgatctcagctcactgcaacctccatctcccaggttcaaatgattctgcctcagcctcccaagtagctgggattaccggcatgcgccaccatgcccagctaatttttatatttttagaagagatggattttcaccatgttggccaggctagtctcaaactcctgacctcaagtgatccgcctgcctcagcctcccaaagtgctgggattacaggcgtgagccaccaggcctggcggaaccttgatcttttaaatgtgaatttcagatatttctattacctgtaaggagagaggtggggaagacgaaggttgaagggaatattgaataaataactcctgtgtactagccctcaatacatgagatatttgataacagctatacaaaacaagccatgttaatagatgagaaattaaagctcagaaaggtcaaataatttcgctaaggtcacaatgtactattacacccgaattcacgttggaattaactagtcagatccattttcattctggacatggtggtgtatgcctgtagtcccagctatttgggggcctgaagtgagaggactgcttgtgcctaggaattcatgtacagcctgggcaacatagcaagaaactgcttctaaaaataaataggctgggtgcagtggctcacgcctgtaatcccagcactttgggaggtggaggcaggtggatcacttgaggtcaggagttcaagaccagcctggccaacacggcgaaaccccatctctactaaaaatacaaaaaattagctgggtgtggtggtgcgtgcctgtaatcccagttacttgggaggctgaggcaggagaagagctttaacccaggaagcagaggttgtggtgagctgagatcacgtcactgcactccagcctgggcaacagagcaagactctgtctcaaataaaaataaataactttgggaggccgaagtgggaggatcccgaggtcgagatcgagaccatcctggctaacacagtgaaaccccatctctactaaaaatacaaaaaattagctgggcatggtggcaggcacctgtagtctcccagctacttggaaggctgaggcagaagaattgcttgaacctgggaggcggaggttgcagtgagccgagatcgtgccactgcattccagcctgggcaacagagagagactccatctcaaaaaattaaaaataagttaacaaataatcaattttcttcctctacagcagaggtcagcaaacttattctgttaaaggccaaacagtaaatattttaggcctcataagccatatggtattggctgcaactattcagttttactgttgtatcattaaagcagccactgaaaagtgtaaacaaatgagcatgactgtgttcccataaaactttaaggacattgacatttgaatttcataaaattttcacatataacaatactattattacttggatcttttccccaaccatataaaaatttaaaacccgttgctaatgcatgggtcttacaaaaacagcctggagttgacccacgggccgtggtttgctgacccttatcatacaccataacacctccttggaagtacacctctctaatgcctttgttccaaacaatactgggttaggaaagacatggaaaaaggaaaatgagatacattattttttgtaccctatgggggattgaggggttgttgctacatagccccctcaatttgtgctgtagcaatatgcagttaagatccttattctaatgttaaatgtctcttctgtggcttatcctaactttaaaaaaaaaaaaaagaagccatcttacgtaaatgaacttacaattttaagacagggtctcactctgtcacccaggctggagtgcagtggtacaatcacggctcattgcagcctcgacctctcaggctcgagagatcctcccaccccaacttcccaagtagctgggactacaggtgtgcaccactatgcctagctcatcttttttttttttttttttttcctttaaaagatatggagtctcgctattttgcccaggctggtcttgaactcctggactcaagcaatccacctgcctcagcctcccagagtgttgggattacaggtgtgagccactgtgcccggcctgaattatcttcttattgtaaaatttcctttaatgcttaatagttgatgtatattaagtgctaactaaatgttcactgataaacattaatcagatgctgctaaatattgtctttctttattcacagatgatagtcaatgggcacaacatataagtagttacaatgaaatgagaagcaatatagcagtcaggctatatgcatgatttaacaacaaaattatcacttccttttaatttagaataagggacaatttaaaaagcatctcttggccctatcatttctgttccagtagttagtgttcatatgtgaatactaagtttgacattcctttctcccatagaaccattttggtgatttggatggtggccactacactgctttctgcaagaattcagtcacccaggcctgatatagctttgataacacacgagtcagtgagattccagatacttctgttcaaaatgctatggatctcctgttctatagctgccagcccttttccataccaatacaaaagcgttaagagccaggaaaatggtgtttcctgaacactgcaaaacaagcagtcagcatctggtggtagagttttgcttggtcattaaactcttagaacttacttgcatcattaacatttttatgccttgtgggcatgttatacaacctttcatcttaagataaatctgtcgtccagaagatgggtcttggttcactaaaaaaggcagtgtgaatataatgcaatgctaatggatgcaggccttcaaaacactgcaattatatagtgagttcaggtttcaaaattcagtgtttatcagaaaatatctcataatcatatatattcaacaaattattttccaaagatactcatgaagctaaacaaaaataatttttgttcaaatggctcgatgagtttaagaatatgatttgaatatatttgatataataatttagccaagaagtggtctcttagactaattgtaaaacatgaaaagttgtcagcttcacaatttgaaccccatcctttcatcttctccctgagagcctgctaatggtggtctctttctgaagcacttttagaatcttatttttatatggagtgttttactgactatatatatagcaactgagtccctcggttaaataaattataagctcctttaaccctcttaatacatcactctgtaaagatgtagtttataatgcagttcactttgcaatcatgcctgactcccggcatttttactttaatatttagaatgaatattctcaatatgtgagaatactagtcttgaaagaatgactctgggtgttattatatagcacgtgtgtatataaaatctatggttttactgtcctatatttgataatacaatattaaagacagaacacccacagggttataaattatttttctcattaagattttaatgtagctgtaaatgaaattctcgttttaaaaaaattaaagtttccatttttttttttagaataaagatttagtgcacaaatacagcccaaagccaacagaaaaattgctttgccctgtcatttccctaagaaagcactgaagttaactcaaaataggctgaaagaaaaaaagcaatcctctgagttctaggtttcacaaaaggaccacgtgttaaactatgtacatcgatttgatgtgcaagtatgcaataaatatgtacacatacattcctatctgctttacatcattctagagtattcatagtatatcaagatgggatttagaaatgtgaaaaggccataacagtgaaaaggaaaaaaaaaagataacaatagtttttagaccagtcgaataataatgcttagctagttaattattttaactttggagcagactaaaaaagttgttttgaaataaatggtacctgtaagtgatgattactgcaatacttgttaaatgttatttgtcagcactgaccggaattatatagtgctagtaacacagctcccactgtcctagaattcctctaaatggccagctatagctaccattatcctgataagcatttcaagagttgtgttgctgagccttttaaaagataactagtttataacctatgtctccttatgtggctacatcagttactcgtggtcccaatgaagtataaaagaggatataagctgctgaagatttcacagaagaaacggagatatcagaaacttcatgatcatcaaacttaaaccaccgttgtcttgctgcatttttacaataggctgtgtagtggcctccatccagcccaccgtagtgatttgaaacagaaaacaaattatatttcttcaaattgttctttggaccaataacatactgtgacaagtcaagattttctaacgggaagtccacagatgtctgtaatttttgtttccacctgccatcgtaggaaaaacgtttcagatgcactaaaagcacaggtggtaacttccagatttctatcttttttagagaatcccgtcgagctctgcaatgactgcagtaaaatctgttgttatctgtgagtttttcttctttggaaaataatctaaggcaatcctgtaatgtacatttacttgtggatgctagtggtagagacaaatacatgaaggcctcaaatgtcctagactttttgtgacatgtgaggcactgtactgtagatttgaattgaccctgaaaaagtgcaacaataatagactcattgagctgcttgtgtttctgccaggcatgttctgcagctttaaagtcatcgagatgatcattattttcttctttatatctcttccgattatcagctttatttagatcttcatggagaccatccattaggaacagaagcaattcttgtgaatcttgctgactgtatcctgcaaactggtcattgatcttcccaatggtgattttaaagtcctttggactgatatatctatactgtcctgtccacagggctttcatgattataccaaattcttctgccacttcacctttatgccccaacaaatttgacctgttaatatcatcctgataacagtttcggttgaaataatcagccaaatgtggagcgttacataggcactgcaatattgagttcatataacaagtatttcctaagttacgaagtccagtaagagctggtccagaacctccaaaaacaggattgaggttccgaatctgagaagcagaaagccttgagatctcagctttaggataacatgttggcttgttttcccgattaactgttggagttactgttggcttcctcttctcttcctcttgaatagcctgggttatatctggggaggagtaggagcgcttcagtttggaaggttccctatcccgctcagcaggaatctgtggcttggctttatgagttggaggggtggaaggaggtgcagatgaaggagccatttccggtgggtacatatgaacagtgttggtgggtgaatgataataacgaaaggttccagtgattgggtcaagaaacttggcccagcctgaaggcagtcctggtacgatcctccccatttcttcacttcgtgctcttgtcaaaggttctcgttgagctttatttctttcggtatcgtctgtatcctctctaaaagttcctgtccttagaattccactttctggttgtcctttaatcttaaatggcttgcctgaacctgaatcccctgtcacagatgtatggggcacatctcctgttgactttttctgtatttctggggttggacaccttttccccctatcttctacagatttcttggcatcagaagtttcatgttcacttttactttgtctttttactcctgttatttctttgcccctctttgctgaggtttctttatcttctttcttggcctgttcactttctttcttctccatttcttcttttgctttttgttgcttctctgtaatttcattttcttcagcttcttgtttctttttggctttttgttcttgttcttccttcctcagtttctctttctgttcctcttgctgcctttcccgaagttctttttcttgtttgtttttttccattagaagagcagtttctgcatgaatacgagccttttcttcatctgttaacatgagagttggagaaaaaactactggcttggtggaacgatcaggaataacttttccactctgaggagattgttgctcatggtttgtactttcagattttattctatgctcttcaggcaatttgactgctggttttttagtacgatcaatctgtggaacattctttatactaggcactggctgaattatgggtgaaacatcagatttagaagcagcaactggttcaactggagttgatatattcagtggtcccattctctcattttgaccacttatcaattctatattttcatctacttctatagatgcaggtggcgtctgggcagcaggtttagaaggaattgattcttccaatgagggataagtaaaatccaatgagatagacacctcttcattctggcgtcgtgggggtggagtgaccttagcatttgttgtatactggggataacaaaggagccagttttcatagcctccctctaaaaccaaaggctcattgcgcaggacagttttactttcccacttgaaaagtgcatctttcagactccggagagttgttccaatctgtaaatctttggcagaactaaaccagtcaagaagtaccacatactccacattccccctcttcttccatgtgtctttagaatcatctggcaggtgtgcttcaatccaactagcagtgactcctggactgatggcttcttcaggaacactgagagaatgtaaaatacaggaatcctgataatcctgcattcttcgagcatccattataatcaagctgatgtttttatccgtcatcattgtgtatagttcctttgctgtgattgctcctttctctttggtctcacatttttcattcttttcaccattgctcttttgggttttgtctttggaatccaaaacattctccaaagagcctttagccaatgtgccaccatcctctcttcctgtttcctgccttttttgttgtagccgctgtgcttcctcctgcctgtctttttcctcaagttttttccggacttcagcttcttcatatcttaatttaaggctttcagagagtctttcagcttcttcgacagcttttttgatgtttccaggtccaagtattgaatggaaataatcctgctgttgcttgaaatcaggtctttttttgataagattataaacagtcacgtatttcatatatagtacataggccctttcctcatcacgatctaatctgcattcttctgctgtcttaaagatcttcagggcactgtgcacataactcttagtgcttattttctctggtttaacttctgtcttcttattaaggtcttttagtgaagaactgaggtagagttctttaggaactgaagccacagcaggcatgatgaattatctttacttttccactttcacaatggatgctatatttccttacaagtgcttctttccgtgacgccgggcgcgcttcactaacgccagccttctcgccaaatgcccatctcccaagaactcgagggagaattagccttggctaccaggacggaagccagcccagctc

SEQ ID NO: 11614 - RNA, 16806 nt, Homo sapiens
  source 1..16806: mol_type = other RNA
ctgaatagctgggactacaggtgtatttttgtatttttagtagaggtggggtttcaccatgttgaccaggctggtcttgaactcctgacctcaagtggcgcacccaccttggcctcccaaagtgctcggattacaggcatgaaccacttctcctggcctctactttatatatttctatagatgtgcctattctgcgtatttttaaaattttatttattttattttttgagacaatatctcactcttgctcaggctggagtgcaatggtgcaatctcagctcactgcagcctcaacctccctggctcaagtgatcttccctcctccctccctcgagtagctgggaccacaggtgtgcaccaccatgccccaataatttttgtgtattttggttgagatggggttttgctatattgcccaggctggtctcaaactccagacgtcaagtgatccacctgcctcggctcccccaggtgctgggattacaggcgtgagccacagtgcctggcctattctgggtattttaataaacagaatcatagaatatatgaccttctgtttttattttcttttattcagcataatgttttcaagtttcattcatgtcatagcatgtatctgtacttcattcctttttattgccaaataatattccattgtataggatataccacatttccttaatccatccagtgatggacatttggcttgtttccacttttggctgtcatcagtaatgctgctatgaacatttatgtacaggattttctgtaaacatgttttcatttctgttgggtatatacctaagtgtgaaatttctgggtcatatggtaactctggttaattttttgaggaactgccaaattgttttccaaagtggcagcagcattttacgttcccaccagcaactggaactaaggttccagtttccccacatcctcaaccgaacttgttactgcctctcattttttattctatcccatacaaagtaggtatgaactggtatgtcatggttttgagttgcattttcctaatgactaatgatgttgagcatcttttcaagtgctctctctccagtttttaaaataaaactttgcaaacattcagaaaatctgaaagaattgtacagagaacattggtgtacatcggccgggcacggtggctgacgcctgtaatcccagcactttgggaggccaaggcaggcggatcacgaggtcaggagatcgagaccatcctggctaacacggtgaaaccccgtctctactaaaaatacaaaaaaaattagccgggcatggtggcgggcgcctgtagtcccagctactcaggaggctgaggcaggagaatggcgtgaacccaggaggcggagcttgcagtgagccgagatagcgccactgcactccagcctgggagacagagcgagactccatctctaaaaaaaaaaccaaaaaacaaaacattggtgtacattggtgtacatttcagctagattcagttattaacatttagcagtgtatacacttttattactttcactctctatacatatatatgtgcacatctatacacacgtatatctaactttttgctgatttaaatcttgtatcgtgacacttcatagatcaaaataatcccttaaccacattcttctacatacccacaatagcagaattatatgtaagaaaatttaaaattccatcactcatattcatagattcatattcaaatatcaattgtcacaaggtttttttttttagtagcattttttttcaaagaccagaatccatccaaaattcacaaactgcatttggttgttgtatcttattgtaattgctgacaatcaagttttaatttggttggaacatcaatcttttctagttagtccttttctgtgtctcatttaagaaatcctttccaaccctggaattacaaagatatttacctacatatcttccaaacatttaaattgttttgcacttctgacaaaaatgtagtataaattagggattcaatttcatttttctgcatatgaataaccaaatgtctcagcctcttcttttcctcagtaacatataatgctggttttcctatgctgtgtgtgtctgttggtcaatttgttcacatttgggctaattccgtactgtattaattatagctataaaatattaaatttattaaattaatattgaattaattcttaatttagcttatgaatattaattatagctatagctttgaaataaacattgatatctggcagagcaagaaccatcattattccctaagtcattaccatcacaactttattcttatttttcagtagtatttcgattattcctggcccttgtcaatttctgtaaaaaatataggtgtgagccatgtatttctcttcagtcattttggtaacttattctccagatatttgtctatttcatctaaggtctcagttggctggcataaagtttttagggtattaacaataaatttattcaggatctgtagctattacatgttttttcatttttaattttatcgttgacttgtctcttttttattttattttattttattttattttttgagacgcagtctcgctctgtcgcccaggctggagtgcaatggcacgatctcagctcacggcaagctccgcctcccgggttcaagtcattctcctgtctcagcctcctgagtagcttgggactacaggcgcccgccaccatgcccggctaattttttgtatttttagtagagacggtgtttcaccgtgttagccaggatagtctcaatttcctgacctggtgatccgcctgcctcagccttccaaagtgctgggattacatgagccaccgcgcccggccgccttgtctcttattctctaaatcttactattgacgtccaagttactatttttgagagagggtctcactctgtctcccaggctggagtgcagtggtgtgatcttggctcactgcaacctctgcctcccaggctcgagccatcctcccacctcagcctcccaagtagatggaactacaggcacaacaccatgtccagctaattttgtaatttttttttttttttttttttttttttttgtgacggagtctcgctctgtcgcccaggctggagcacagtggcgcgatcttggctcactgcaagctccgaccccgggttcacgccattctcctgcctcagcctcccaagtagctgggactacaggcgcccgccaccgtgcccaggtaattttttgtatttttaatagagatggggtttcaccgtgttagccaggatggtctcaatctcctgacctcgtgatccgcccgcctcggcctcccaaagtgctgggattacaggcgtgagccaccgcgcctggcctgtactctttttttttttatagagacggggttttgccatgttgcccaagctggtttcaaactcctggactcaggcgatccatctgccttggcctcccaaagtgcagggattataggcatgaaccactgtggcaggctaacatccaaattattttgtcttaaaacaccaacttttacctttttttaaatcttctgtattacatctttgttttctgctttatgggttattcctcttacagtgttatctcttccctctactcttttagggtttattctgttatgttttaatgttttaaactgagtgtccagtgtattaacactcagtctatcctttaagatataagtatttaaaactacaaatgtctatctcccactttctctgcctttttttattatagaatatttcaaacatatacaaaattggacagcataacaaaccgccatgcatccatcaactagcttgctgaagcaagatatttgaatataaaataaatgatcaattcatcttaatactgacccactctcttcttggcatcgtattatttttaagacattctcagacatcagtgcatcccatgttttgatatagtattttcattactatttacttctaagtgttttacttttataatttatttataaagttacttagaagtgtttttttaatttccaaaagtattgattttttgtgggggtatcattttgtattgactgctaattgtattgtgttcaaagactagggtctaaattaaactaatctttttttttttttttttttttttttgagacagagtcttgcactgtcgcccgggctagagtgcactggcaccatctcggctcactgcaacctccgccgcccagtttcaagcgattttcctgcttcagcctcctcagtagctgggattacaggcagccgacaccatgcccagctaattttttgtatttttagtagagacggggtttctccatgttggccaggctggtctcgaactcctgacctcgtgattcgcctgccttggcctcccaaagtgctgggattacaggcatgagccaccgtgcctggcctaaactaactcttttacatttgttgagacagtgcacttctatttcaggagtcagatactcatctaagtatatattgtaaaagctgtatctatactaatatttttgtctgcttgatcaatagttgaaatcttccattatgatggtagacttgtcaaaacttccctatagttctgtcatttgtttttaacaagtctgttttgttaggtaggtagcagtttcaaattatacaatttgggtgatttaaaccttttttcattataaagtgactcatttacaatgcattctatcttagggaccattttagctgatgtatagctacttcagctttctcttggtcatatctacctacgacaagttgagcatccctaatctgaaaatccaaaatgctccaaaatctgaaacattttaagcaccaacatgatgctcaagggaaatacaccttttctgagttctaaatgttatatagtgcatagaactggatttgttgttgttgttgttttgttttagagacagagtctcactctgtgccccaggctggagtgcagtggcatgatcttggctcactgcaacctccacctcccaggttcaagcaactctcctgcctcagcttcccaagtagttgggattactggcatgtgccaccagacccagctaatttttgtatttttagtagagaccgggttttgccatgttggccagggtggtctggaactcctgatctcaggtgatccgcctgccttggcctcccaaagtgttgggattacaggcatgagccaccacacttggcctaaaactggatttttttttttttttttttttttttttttttttgagatgaagtctcgctctgtcgcccaggctggaatgcagtggcacgatctcggctcactgcaagcttcacctcctgggttcatgccattctcctgcctcagcctccggagtagctgggactataggcgcctgccaccatgcccggctaattttttgtatttttgtagagatgaggtttcaccgtgttggccaggatagtcttgatctcctgacctcgtgatccgcccccctcggcctccccaagtgctgagattatagacgtgagccatcgcgcctggctagaactggatatttaaaatccagtaaatatttggtaaatttactacatcccatatatttcaactagtaataaattcggatttacttgtcgtcatcttcttttgtgtttatgttagccttatttttctaattcggcagtccccaaccttgttggcaccagggactgatttttgtggaagacaatttttccactgatgcggtttttttcccatggatgggggccggggcgggcatggttttgggattaaactgttccacctcagaaaatcaggcagtagattctcataaggagcacgcaacctagatccctcacatgcgcagttcacaatagagtttgtgctgctgtgagaatctaatgcagcagctgatctgacaggaggcggtgctcagggtaggtttgccgctcgcttcctgctgtgcagccaggtcctgaacaggtcagggacaggcagcctgggggggttggggacctctgctgtgttgttttcccctgttgttcttgctgctactaaactgataaagctttctttattttccctctacaactttggaagttacacattttgattctttagtaattatgctaaaaaacgacagctttcatacttaaagcctaaagttaatcaagatctttatactctgctcccaaagaaatggaaagctcttagaacactgtaattctgatcactgaactactgttttcagcatcttttgtttttgagacagggtctcactctgttgcccagactggagtgcactagtgcaatgaatcatagctcactacagttttgaactctgggcttaagggatcctcctgcctctgcctgccaagtagctgggactacaggcatgctactgtgcatggccaacttttttattttttttagagaccaggtctcactatgttgcccaggctggtctcaaactcctgggctcaaacgatcctcctgccttggccttccaaagtgctgggattacaggtgtgaaccaccatgcccagccggtttttaattttttaatatgcctccaaaggagacattatcatggttttctactgttcatattgggttatatttgcccggatcttcatcagtcttttttgttaatcactgtctattatgtatcacttcttccttcattgagtttttaaaattcatgtggcatatatttcagtaggcttttcagtgagggtctgttatcctgaagtctctcagtctttgagaagtctttaattcactttcattcttggatgataactagaaatcaaattccagattgacagttatttttctctattattttgaagctactgtattgtctctgatttctatggctgctatggagaacttctaccagcaggttagattcttgtgggtaaactctctttttctttctggttgcttttaagctttttctctttgtctctgttgttctgcagtattatttttatttatccctggctcgctgcatttcctaaatgtgaagattcatgtctcattaatcattttcagccattatcacttttaatattgccttgctcccctactcgattctctcctcctagaacttctacaggacatacgctgaatattctcattcaatttttcatgcctcttaacacgtattctccatcactactccattcttgctaatttccccaacttcattttatagtttattcttttttttttttttttgagatggagtctcactctgtcacccacactggagtgcaatggcacgatcttggctcactgcaacctccacctcccgggttcaagcgattctcctgcttcagcctctcaagtagctgggattacaggtgcacgccaccaggcccagctaattttttttgttttttttaatagagacagggtttcaccatgtgtaccaggttggtcttgaactcctgacctcatggtccacccgcctcagcctcccaaagtgctaggattacaggcatgagccaccgcgcccagtccggtttattcattttctgtgtcctaatatcttcattaagttaatttccagtacagttgtacctcagtatctgcagggagttggttccaggatccctttgactatcaaaatccacagatgctcaagggccctatataaaatggtgtcttttctggtgttttttgtttttgttttttgagacaaggtctcattctgttgccaggctggagagcagtggctcagtcacagctcactgtagcctcgacctcctgggctcaggtgattctcccacctcaacctaccaagtagctgggactataggcacgtgccactatgcctggtcaatttttgtattttgtgtagacagggttttgccatgttgcccaggctggtctacaactcctgggctcaagcagtctgcccacctccatcccccaaaaacgttgggattacacgtgtgagccaccatgccaggcctggagtagtatttgcatgtaacctatgcacatcctcccatatactttaagtcatctctggattacttataatatctaatacaatataaatactatgtaaatagttgttacactgtattttaaaatatgtatatttttattgttgtattattttttcaaatctttcccatcacattagttgattctgaagatgcagagcccgtaaatatggacggccaactatgttgtatttctcatttctgaaaattctatttagtttctaaagtttgtttccttcttctaaatatatttaaatatactttatttgtagcctctgcttaataattctattatctaaagtccttgggggtttaaatcttattgccttctgactcttatgataaattgtttccttgcatgttctattattttgaattgtgatctcaacttcattggggtttcatatgtggatatcctgttaggtctgagttaacatgcaacaatctagaaattctgtttccttctggcaactgccctagaaatacttttcatattaagttcacaggattcgcagaccacacaggtagtataaatttgaatcccaaactggtgaaaaggtaggtctatggtgacaaattcccaggaatgacttttattctctgtaccatgagtccaagctaacacaagcactagagggtggattttgttttttaatccttccattgagggtgaatgtctttaaaggtcctggctttgtatgtggatctcaatccaacttctcaccttgtaggggggcctaagactttacctcgagtgtccttgcgtgacctttaaaacccgagcatactggttacagaaactagggactgtctttacgcccaggcagtcacaaagcataaaccacacaccatactgttgttaaatttcctgtttagggctccgcccaggctggaatgcaatggcatgatctcagctcactgcaacctccatctcccaggttcaaatgattctgcctcagcctcccaagtagctgggattaccggcatgcgccaccatgcccagctaatttttatatttttagaagagatggattttcaccatgttggccaggctagtctcaaactcctgacctcaagtgatccgcctgcctcagcctcccaaagtgctgggattacaggcgtgagccaccaggcctggcggaaccttgatcttttaaatgtgaatttcagatatttctattacctgtaaggagagaggtggggaagacgaaggttgaagggaatattgaataaataactcctgtgtactagccctcaatacatgagatatttgataacagctatacaaaacaagccatgttaatagatgagaaattaaagctcagaaaggtcaaataatttcgctaaggtcacaatgtactattacacccgaattcacgttggaattaactagtcagatccattttcattctggacatggtggtgtatgcctgtagtcccagctatttgggggcctgaagtgagaggactgcttgtgcctaggaattcatgtacagcctgggcaacatagcaagaaactgcttctaaaaataaataggctgggtgcagtggctcacgcctgtaatcccagcactttgggaggtggaggcaggtggatcacttgaggtcaggagttcaagaccagcctggccaacacggcgaaaccccatctctactaaaaatacaaaaaattagctgggtgtggtggtgcgtgcctgtaatcccagttacttgggaggctgaggcaggagaagagctttaacccaggaagcagaggttgtggtgagctgagatcacgtcactgcactccagcctgggcaacagagcaagactctgtctcaaataaaaataaataactttgggaggccgaagtgggaggatcccgaggtcgagatcgagaccatcctggctaacacagtgaaaccccatctctactaaaaatacaaaaaattagctgggcatggtggcaggcacctgtagtctcccagctacttggaaggctgaggcagaagaattgcttgaacctgggaggcggaggttgcagtgagccgagatcgtgccactgcattccagcctgggcaacagagagagactccatctcaaaaaattaaaaataagttaacaaataatcaattttcttcctctacagcagaggtcagcaaacttattctgttaaaggccaaacagtaaatattttaggcctcataagccatatggtattggctgcaactattcagttttactgttgtatcattaaagcagccactgaaaagtgtaaacaaatgagcatgactgtgttcccataaaactttaaggacattgacatttgaatttcataaaattttcacatataacaatactattattacttggatcttttccccaaccatataaaaatttaaaacccgttgctaatgcatgggtcttacaaaaacagcctggagttgacccacgggccgtggtttgctgacccttatcatacaccataacacctccttggaagtacacctctctaatgcctttgttccaaacaatactgggttaggaaagacatggaaaaaggaaaatgagatacattattttttgtaccctatgggggattgaggggttgttgctacatagccccctcaatttgtgctgtagcaatatgcagttaagatccttattctaatgttaaatgtctcttctgtggcttatcctaactttaaaaaaaaaaaaaagaagccatcttacgtaaatgaacttacaattttaagacagggtctcactctgtcacccaggctggagtgcagtggtacaatcacggctcattgcagcctcgacctctcaggctcgagagatcctcccaccccaacttcccaagtagctgggactacaggtgtgcaccactatgcctagctcatcttttttttttttttttttttcctttaaaagatatggagtctcgctattttgcccaggctggtcttgaactcctggactcaagcaatccacctgcctcagcctcccagagtgttgggattacaggtgtgagccactgtgcccggcctgaattatcttcttattgtaaaatttcctttaatgcttaatagttgatgtatattaagtgctaactaaatgttcactgataaacattaatcagatgctgctaaatattgtctttctttattcacagatgatagtcaatgggcacaacatataagtagttacaatgaaatgagaagcaatatagcagtcaggctatatgcatgatttaacaacaaaattatcacttccttttaatttagaataagggacaatttaaaaagcatctcttggccctatcatttctgttccagtagttagtgttcatatgtgaatactaagtttgacattcctttctcccatagaaccattttggtgatttggatggtggccactacactgctttctgcaagaattcagtcacccaggcctgatatagctttgataacacacgagtcagtgagattccagatacttctgttcaaaatgctatggatctcctgttctatagctgccagcccttttccataccaatacaaaagcgttaagagccaggaaaatggtgtttcctgaacactgcaaaacaagcagtcagcatctggtggtagagttttgcttggtcattaaactcttagaacttacttgcatcattaacatttttatgccttgtgggcatgttatacaacctttcatcttaagataaatctgtcgtccagaagatgggtcttggttcactaaaaaaggcagtgtgaatataatgcaatgctaatggatgcaggccttcaaaacactgcaattatatagtgagttcaggtttcaaaattcagtgtttatcagaaaatatctcataatcatatatattcaacaaattattttccaaagatactcatgaagctaaacaaaaataatttttgttcaaatggctcgatgagtttaagaatatgatttgaatatatttgatataataatttagccaagaagtggtctcttagactaattgtaaaacatgaaaagttgtcagcttcacaatttgaaccccatcctttcatcttctccctgagagcctgctaatggtggtctctttctgaagcacttttagaatcttatttttatatggagtgttttactgactatatatatagcaactgagtccctcggttaaataaattataagctcctttaaccctcttaatacatcactctgtaaagatgtagtttataatgcagttcactttgcaatcatgcctgactcccggcatttttactttaatatttagaatgaatattctcaatatgtgagaatactagtcttgaaagaatgactctgggtgttattatatagcacgtgtgtatataaaatctatggttttactgtcctatatttgataatacaatattaaagacagaacacccacagggttataaattatttttctcattaagattttaatgtagctgtaaatgaaattctcgttttaaaaaaattaaagtttccatttttttttttagaataaagatttagtgcacaaatacagcccaaagccaacagaaaaattgctttgccctgtcatttccctaagaaagcactgaagttaactcaaaataggctgaaagaaaaaaagcaatcctctgagttctaggtttcacaaaaggaccacgtgttaaactatgtacatcgatttgatgtgcaagtatgcaataaatatgtacacatacattcctatctgctttacatcattctagagtattcatagtatatcaagatgggatttagaaatgtgaaaaggccataacagtgaaaaggaaaaaaaaaagataacaatagtttttagaccagtcgaataataatgcttagctagttaattattttaactttggagcagactaaaaaagttgttttgaaataaatggtacctgtaagtgatgattactgcaatacttgttaaatgttatttgtcagcactgaccggaattatatagtgctagtaacacagctcccactgtcctagaattcctctaaatggccagctatagctaccattatcctgataagcatttcaagagttgtgttgctgagccttttaaaagataactagtttataacctatgtctccttatgtggctacatcagttactcgtggtcccaatgaagtataaaagaggatataagctgctgaagatttcacagaagaaacggagatatcagaaacttcatgatcatcaaacttaaaccaccgttgtcttgctgcatttttacaataggctgtgtagtggcctccatccagcccaccgtagtgatttgaaacagaaaacaaattatatttcttcaaattgttctttggaccaataacatactgtgacaagtcaagattttctaacgggaagtccacagatgtctgtaatttttgtttccacctgccatcgtaggaaaaacgtttcagatgcactaaaagcacaggtggtaacttccagatttctatcttttttagagaatcccgtcgagctctgcaatgactgcagtaaaatctgttgttatctgtgagtttttcttctttggaaaataatctaaggcaatcctgtaatgtacatttacttgtggatgctagtggtagagacaaatacatgaaggcctcaaatgtcctagactttttgtgacatgtgaggcactgtactgtagatttgaattgaccctgaaaaagtgcaacaataatagactcattgagctgcttgtgtttctgccaggcatgttctgcagctttaaagtcatcgagatgatcattattttcttctttatatctcttccgattatcagctttatttagatcttcatggagaccatccattaggaacagaagcaattcttgtgaatcttgctgactgtatcctgcaaactggtcattgatcttcccaatggtgattttaaagtcctttggactgatatatctatactgtcctgtccacagggctttcatgattataccaaattcttctgccacttcacctttatgccccaacaaatttgacctgttaatatcatcctgataacagtttcggttgaaataatcagccaaatgtggagcgttacataggcactgcaatattgagttcatataacaagtatttcctaagttacgaagtccagtaagagctggtccagaacctccaaaaacaggattgaggttccgaatctgagaagcagaaagccttgagatctcagctttaggataacatgttggcttgttttcccgattaactgttggagttactgttggcttcctcttctcttcctcttgaatagcctgggttatatctggggaggagtaggagcgcttcagtttggaaggttccctatcccgctcagcaggaatctgtggcttggctttatgagttggaggggtggaaggaggtgcagatgaaggagccatttccggtgggtacatatgaacagtgttggtgggtgaatgataataacgaaaggttccagtgattgggtcaagaaacttggcccagcctgaaggcagtcctggtacgatcctccccatttcttcacttcgtgctcttgtcaaaggttctcgttgagctttatttctttcggtatcgtctgtatcctctctaaaagttcctgtccttagaattccactttctggttgtcctttaatcttaaatggcttgcctgaacctgaatcccctgtcacagatgtatggggcacatctcctgttgactttttctgtatttctggggttggacaccttttccccctatcttctacagatttcttggcatcagaagtttcatgttcacttttactttgtctttttactcctgttatttctttgcccctctttgctgaggtttctttatcttctttcttggcctgttcactttctttcttctccatttcttcttttgctttttgttgcttctctgtaatttcattttcttcagcttcttgtttctttttggctttttgttcttgttcttccttcctcagtttctctttctgttcctcttgctgcctttcccgaagttctttttcttgtttgtttttttccattagaagagcagtttctgcatgaatacgagccttttcttcatctgttaacatgagagttggagaaaaaactactggcttggtggaacgatcaggaataacttttccactctgaggagattgttgctcatggtttgtactttcagattttattctatgctcttcaggcaatttgactgctggttttttagtacgatcaatctgtggaacattctttatactaggcactggctgaattatgggtgaaacatcagatttagaagcagcaactggttcaactggagttgatatattcagtggtcccattctctcattttgaccacttatcaattctatattttcatctacttctatagatgcaggtggcgtctgggcagcaggtttagaaggaattgattcttccaatgagggataagtaaaatccaatgagatagacacctcttcattctggcgtcgtgggggtggagtgaccttagcatttgttgtatactggggataacaaaggagccagttttcatagcctccctctaaaaccaaaggctcattgcgcaggacagttttactttcccacttgaaaagtgcatctttcagactccggagagttgttccaatctgtaaatctttggcagaactaaaccagtcaagaagtaccacatactccacattccccctcttcttccatgtgtctttagaatcatctggcaggtgtgcttcaatccaactagcagtgactcctggactgatggcttcttcaggaacactgagagaatgtaaaatacaggaatcctgataatcctgcattcttcgagcatccattataatcaagctgatgtttttatccgtcatcattgtgtatagttcctttgctgtgattgctcctttctctttggtctcacatttttcattcttttcaccattgctcttttgggttttgtctttggaatccaaaacattctccaaagagcctttagccaatgtgccaccatcctctcttcctgtttcctgccttttttgttgtagccgctgtgcttcctcctgcctgtctttttcctcaagttttttccggacttcagcttcttcatatcttaatttaaggctttcagagagtctttcagcttcttcgacagcttttttgatgtttccaggtccaagtattgaatggaaataatcctgctgttgcttgaaatcaggtctttttttgataagattataaacagtcacgtatttcatatatagtacataggccctttcctcatcacgatctaatctgcattcttctgctgtcttaaagatcttcagggcactgtgcacataactcttagtgcttattttctctggtttaacttctgtcttcttattaaggtcttttagtgaagaactgaggtagagttctttaggaactgaagccacagcaggcatgatgaattatctttacttttccactttcacaatggatgctatatttccttacaagtgcttctttcctttaggagttgtcccactcctctccgcggacagagcttgtctccggggtaaccagcagctggtggaaggaaaggcgttcatcgttcacagcggacgacttcccagagaacaggtgctagggcccaagacccgcactcaccgtgacgccgggcgcgcttcactaacgccagccttctcgccaaatgcccatctcccaagaactcgagggagaattagccttggctaccaggacggaagccagcccagctc

SEQ ID NO: 11615 - RNA, 4508 nt, Homo sapiens
  source 1..4508: mol_type = other RNA
ctgaatagctgggactacaggtgtccaccaccaaacccagctaatttttgtatttttagtagagatggggttttgccatgttggccaggctggtcttgaactcctgacctcaggtgatcctctcgccttgcccaaagtcctgggattacaggcatgagccaccgcacctggctatatataccagattcttgagcagataattaaacctcctccaccacaaaacttgaaaataaggtacaagaaggcatgacatgagaatccacctgccccttttcccatctgactgtgatgctgaggtgtggtggaattagccaaaagatgtaggaagaaaacttgggtgagctacacccagaataattaatacttaagtcatcaagggttgattgtacttgcaggagaacgggtaactttcccacataaagctgaaatgctagtacagagaaatagccttccatttgctattacaggatcaatgtgcaggtttgatcactttttttttgaagcattttcttttgccaagaataaaaatcatgtatagctattgcactaccaataggtcaattcatgctacaaatgtccatgtgtttctaggatgccagtggctactgctaccagaaataactccagtcactcccttgactagtgttgctagtttggtctttagggtttacctaagtgagagcatcaatgatgggttaaagtcacagaccacaatgaataaatcacagtctgtgcacacttttggccaggaagagtggcagtggaatcttgcatgtcatttggttgaaattaagactaaatctctatatgtgcacacacccacactcacacccacacgcacacatatcacagggttatagcagaatgaaaacggtgggtaggaatcaccagttgaaggctgtaggtttaaatgatcaggattggcacactcagatcagcccaccagtggtcttcactttgtgaaatggaactaatgccacaaggaaactgcatggttacttcatctgtttacacatctgcttatatgttcagctgaactgtcactgaaaacaggagcaccattcttgggacatgaaacaaggaggaggggaaacattcagataatcaacagttaatagaacaagtaaaaaaataagccaacagcaggtgcggcatctctggtatgcaaaacaactaatgaaagtgttcaaaggaattatcaaggcaggccattaagactataaaccatcaaaagagcagcagcaatagcaagagagaaagaagagggttagcaagagactagatcttcctgaaaaagtggccttggctctacaattgtctaccttgtgctgtccttagaagaacaggcccagtgctacagaataaaaatctccatgccaagccactgccttcagaatggtgatgatgtcttcttacaaaggtaaacccaagatgacaaccacaagcaaaaaaatcacccttttgttttaccatcaacagatgaaatagtccatacagtgccattcaatttcccacaggcagaaaccaaagacctcagaatgagaaagtcatggttttcacgtcacaaatgttacgtgtggtcagattatggagcaatgaaaacatttttctgcgccgctcattacactaaatcttgatgtttctgaagtctcttggagtttgagatgtattggaatagtttttcgcaccaagattaacatggcacagtaggaacaggctactgacaaatccatgtccacttaccttacccacaaggttccctaagggttcccttcattctcacaatatttcattttgagatgacttaaggtcaggtagaagggaccacataggccactcttcatcacttctcctcctagctcagaggctcacaattgaggcacttggcccttttgcactactaacatctggggctggaaacctgttgctggataaatacagctcagcaaatccccaaccatatttctattcactaaggtgttattggattgctcctgtttgtgcatgtctgcacacacatgcacaatttcttgtcctctccctccacacttacagacatacacctggtcatgtggaccatcgaaacacaacttgtttggatggaagaagaaaactctgcagatgctgttatttttagaagcctgcttatccctcctgaatgccaacaattttggcttggcatccatttcaaatcaagcaaggtgcatatccaggacaaagcaatgtgcattatgtctgaagggatccacatcttcagtgaaactcagaatgtggccagaactagctaactacctgaactgaaagcaccccatgttcagattcagaccaactcaaaacacatgtaaggggtgcctattgtatgcagggtaaggtgtcaagtccctttttatttggattaagctcaaataagaaaggacctgaagcgaacgtgggatgtgtatgtgtgtacatgtacacgtttgcaaacacacaggtttatgtgggtattaatatcgagtggaaaatctggctttttatttgtctgtgtctttttttttttttttcagtctgattcgagtatatctgttttggcaagttgtgggcagctctcttttacttttgtcacccagaggcttccgtagacaaaaggaaaggagagaggtgtgttcaaagacccccatggcgaagagcccatcccccaagcctgacacaaccctccctcccagcggacccctcttctggactggcttcgctgttggctacttcagtgcatctgacccccaccccccgcgtgaagacctgagattgagcgtggatttctgttctccaccaactctgcagcaagggccctgccagaggcgtcgcttcctgtcatctcctcttcccgctcccaagtagaggcacctaaacagagattagatttctggtttcaaggcatgtcggaccaagcacgctgaatgaacatgagttagttaattagctcggtctctcttctttccgttccctggtctgaatgtttcttgatggcaaagcgaccaggagagagttgatttgcatcttaagacctatgggtaatgcttctggagtggggagatttatttagcaactgcttgaacttgtgtacggggtcgggaaggaggtggagctgaccccaatggggctatcggagattggggtgtgggtggtgcccactgccacgctgacaccccgggcctcgatgatggcagacaggagctgctgctgctgctggcgcagggtgtcggcgatgagcagcggcagggagttgaagctggcggtgagatgctccagcttcgactccaggctgccaatctgcttctccaggtcttcgctccggtcattgagttctgtgattaagtcatacatgacattctgcatcttggaaaggtccaccagagtgttggcttggtcactcagcttcctctgttccatcttgacgctcctcaactggtggatagcttggaggaacttcctctggtgtttcctcactttggcatggtcaatcttctttagcagctttgtgtgtttatagattaaccatgtttcccgaaggacattggctgcagcattcttgatccgcttggtgagctgagtgtccatcatgaagttatgaacgtgcttctccgctttggtgagttccagctttcgggccaccacggccaccacaagggcagtgcagcctgcacccatgatgccagtgaggagacagacacctttcccacagtatgtgtggggcaccatgtccccataaccaatggaaaggaatgtgatggagatgagccacatggcacccagaaagttactagttacgtcctgctggtcatggtaccaagcaggaagtgatgagccagaaggctgggctggtgattcaggactttcacagacacggacggtccaggcagcaatgatccacagagagatgctgaacacgagcagcacagtgccagggcagatggtcatgagcgtcttcatgacaaagcgggtgttgaagttgatcttgttgagggccccgatgctgcgggacgaggcatcggtgaagagcttgctgtgcagcagcatgactcgggcgatcaggtacaggcgcaggaacatggggatagacaggatgatgtccacatcggcctccgcccgggagggtgtgtaggagaaggccaggcgtgccgtccagaagaacttgtactcgccaggaatggggtggatggcgcacaccagcatctccaggctgatgtacaggatgcgctcgtaggtcatggctatccgccagtcatccgcgccattgtcgatcacgaagagctggacttcacgtgtgtggtaggcgatgatcaagcccaaaaggatgatggtggacagactgataaggcatttcagggccaacgaaaacatggagtccttcctccatctccactccctctgggagggaaaccccctcctccgtcttggggctggactgagaggctggagcagtggggccagctccccgctaaagccagtgcctgctgttctccatccgg

SEQ ID NO: 11616 - RNA, 5636 nt, Homo sapiens
  source 1..5636: mol_type = other RNA
ctgaatagctgggactacaggtgtccaccaccaaacccagctaatttttgtatttttagtagagatggggttttgccatgttggccaggctggtcttgaactcctgacctcaggtgatcctctcgccttgcccaaagtcctgggattacaggcatgagccaccgcacctggctatatataccagattcttgagcagataattaaacctcctccaccacaaaacttgaaaataaggtacaagaaggcatgacatgagaatccacctgccccttttcccatctgactgtgatgctgaggtgtggtggaattagccaaaagatgtaggaagaaaacttgggtgagctacacccagaataattaatacttaagtcatcaagggttgattgtacttgcaggagaacgggtaactttcccacataaagctgaaatgctagtacagagaaatagccttccatttgctattacaggatcaatgtgcaggtttgatcactttttttttgaagcattttcttttgccaagaataaaaatcatgtatagctattgcactaccaataggtcaattcatgctacaaatgtccatgtgtttctaggatgccagtggctactgctaccagaaataactccagtcactcccttgactagtgttgctagtttggtctttagggtttacctaagtgagagcatcaatgatgggttaaagtcacagaccacaatgaataaatcacagtctgtgcacacttttggccaggaagagtggcagtggaatcttgcatgtcatttggttgaaattaagactaaatctctatatgtgcacacacccacactcacacccacacgcacacatatcacagggttatagcagaatgaaaacggtgggtaggaatcaccagttgaaggctgtaggtttaaatgatcaggattggcacactcagatcagcccaccagtggtcttcactttgtgaaatggaactaatgccacaaggaaactgcatggttacttcatctgtttacacatctgcttatatgttcagctgaactgtcactgaaaacaggagcaccattcttgggacatgaaacaaggaggaggggaaacattcagataatcaacagttaatagaacaagtaaaaaaataagccaacagcaggtgcggcatctctggtatgcaaaacaactaatgaaagtgttcaaaggaattatcaaggcaggccattaagactataaaccatcaaaagagcagcagcaatagcaagagagaaagaagagggttagcaagagactagatcttcctgaaaaagtggccttggctctacaattgtctaccttgtgctgtccttagaagaacaggcccagtgctacagaataaaaatctccatgccaagccactgccttcagaatggtgatgatgtcttcttacaaaggtaaacccaagatgacaaccacaagcaaaaaaatcacccttttgttttaccatcaacagatgaaatagtccatacagtgccattcaatttcccacaggcagaaaccaaagacctcagaatgagaaagtcatggttttcacgtcacaaatgttacgtgtggtcagattatggagcaatgaaaacatttttctgcgccgctcattacactaaatcttgatgtttctgaagtctcttggagtttgagatgtattggaatagtttttcgcaccaagattaacatggcacagtaggaacaggctactgacaaatccatgtccacttaccttacccacaaggttccctaagggttcccttcattctcacaatatttcattttgagatgacttaaggtcaggtagaagggaccacataggccactcttcatcacttctcctcctagctcagaggctcacaattgaggcacttggcccttttgcactactaacatctggggctggaaacctgttgctggataaatacagctcagcaaatccccaaccatatttctattcactaaggtgttattggattgctcctgtttgtgcatgtctgcacacacatgcacaatttcttgtcctctccctccacacttacagacatacacctggtcatgtggaccatcgaaacacaacttgtttggatggaagaagaaaactctgcagatgctgttatttttagaagcctgcttatccctcctgaatgccaacaattttggcttggcatccatttcaaatcaagcaaggtgcatatccaggacaaagcaatgtgcattatgtctgaagggatccacatcttcagtgaaactcagaatgtggccagaactagctaactacctgaactgaaagcaccccatgttcagattcagaccaactcaaaacacatgtaaggggtgcctattgtatgcagggtaaggtgtcaagtccctttttatttggattaagctcaaataagaaaggacctgaagcgaacgtgggatgtgtatgtgtgtacatgtacacgtttgcaaacacacaggtttatgtgggtattaatatcgagtggaaaatctggctttttatttgtctgtgtctttttttttttttttcagtctgattcgagtatatctgttttggcaagttgtgggcagctctcttttacttttgtcacccagaggcttccgtagacaaaaggaaaggagagaggtgtgttcaaagacccccatggcgaagagcccatcccccaagcctgacacaaccctccctcccagcggacccctcttctggactggcttcgctgttggctacttcagtgcatctgacccccaccccccgcgtgaagacctgagattgagcgtggatttctgttctccaccaactctgcagcaagggccctgccagaggcgtcgcttcctgtcatctcctcttcccgctcccaagtagaggcacctaaacagagattagatttctggtttcaaggcatgtcggaccaagcacgctgaatgaacatgagttagttaattagctcggtctctcttctttccgttccctggtctgaatgtttcttgatggcaaagcgaccaggagagagttgatttgcatcttaagacctatgggtaatgcttctggagtggggagatttatttagcaactgcttgaacttgtgtacggggtcgggaaggaggtggagctgaccccaatggggctatcggagattggggtgtgggtggtgcccactgccacgctgacaccccgggcctcgatgatggcagacaggagctgctgctgctgctggcgcagggtgtcggcgatgagcagcggcagggagttgaagctggcggtgagatgctccagcttcgactccaggctgccaatctgcttctccaggtcttcgctccggtcattgagttctgtgattaagtcatacatgacattctgcatcttggaaaggtccaccagagtgttggcttggtcactcagcttcctctgttccatcttgacgctcctcaactggtggatagcttggaggaacttcctctggtgtttcctcactttggcatggtcaatcttctttagcagctttgtgtgtttatagattaaccatgtttcccgaaggacattggctgcagcattcttgatccgcttggtgagctgagtgtccatcatgaagttatgaacgtgcttctccgctttggtgagttccagctttcgggccaccacggccaccacaagggcagtgcagcctgcacccatgatgccagtgaggagacagacacctttcccacagtatgtgtggggcaccatgtccccataaccaatggaaaggaatgtgatggagatgagccacatggcacccagaaagttactagttacgtcctgctggtcatggtaccaagcaggaagtgatgagccagaaggctgggctggtgattcaggactttcacagacacggacggtccaggcagcaatgatccacagagagatgctgaacacgagcagcacagtgccagggcagatggtcatgagcgtcttcatgacaaagcgggtgttgaagttgatcttgttgagggccccgatgctgcgggacgaggcatcggtgaagagcttgctgtgcagcagcatgactcgggcgatcaggtacaggcgcaggaacatggggatagacaggatgatgtccacatcggcctccgcccgggagggtgtgtaggagaaggccaggcgtgccgtccagaagaacttgtactcgccaggaatggggtggatggcgcacaccagcatctccaggctgatgtacaggatgcgctcgtaggtcatggctatccgccagtcatccgcgccattgtcgatcacgaagagctggacttcacgtgtgtggtaggcgatgatcaagcccaaaaggatgatggtggacagactgataaggcatttcagggccaacgaaaacatggagtcctttgagtacaaaccccaagagagctcggtctctatcaccataacaacaattccaaacatcccaaaaatcagagcatagtcactcagtcgctttctcttttcaaacagggccctcctgtgtcccagcttatagccaatgttttggtttttccgcttgttggctttggggaaggtggtgctgctggcggtggtgccggcatgctggtggttgtgggtggcattagggtgatggagcagggtctggtgggcatggttgtcctcccgggaggagatgacgatctccggggggttgctagggctgaaaagctggaggggttggccctcagtctcggcctcgatgaggttcctccgggaggcgctgaggcggctgaggggcttcatgaccccaccgctatacttgcaggagctcatggcgatctccgtgaaggggttgctgtcccgccggtgcaccagggggctggcctgtcggtgccggctgcctccgccaggcccacttgtagctgtggaacttggagagtggccaagcaagtggtcattgagattgagctggctgccttgcctggaggaagggtggaggatggcggtggagttggacgaagggggggccctgaaagcggtgggagaggagtgcagcaggccagggtggacgggctggctctggagttgggcgagctgagacaggggatgcggtggctgctgctgctgctgctgctgctgctgctgctgctgctgctgaagctgcggaggctgaggctgcagcgagggtcccaggggctgctggggggctgctggtggcgctggcggtggtggctgctgctgctgttgctgctgctgctgctgctgctgctcatccccagaggatggacaggggcacttggggtcttcatccaagtcccccacccccgagtcatggaagtgcccagaagtgtccatcttggggcctggctgtattccctgcagcacaagcccccaccccaaagccaccctcgctccaaagatgtcctcaaagaaagccaggcatccaatctcccccaccagtatcttggctccagtcctctctttggcttgcttcggttctctggggctgcctggagtccagacgctgccactcaagaatgcattgtattgggcagggagggagagcaggaggggagcttggagaaagaagagggggtgaaagaactctctcaggaggtggtcctctaggagcgtgtgaggccaggctcagcttcactcctcgctggctcaat

SEQ ID NO: 11617 - RNA, 4463 nt, Homo sapiens
  source 1..4463: mol_type = other RNA
ctgaatagctgggactacaggtgtccaccaccaaacccagctaatttttgtatttttagtagagatggggttttgccatgttggccaggctggtcttgaactcctgacctcaggtgatcctctcgccttgcccaaagtcctgggattacaggcatgagccaccgcacctggctatatataccagattcttgagcagataattaaacctcctccaccacaaaacttgaaaataaggtacaagaaggcatgacatgagaatccacctgccccttttcccatctgactgtgatgctgaggtgtggtggaattagccaaaagatgtaggaagaaaacttgggtgagctacacccagaataattaatacttaagtcatcaagggttgattgtacttgcaggagaacgggtaactttcccacataaagctgaaatgctagtacagagaaatagccttccatttgctattacaggatcaatgtgcaggtttgatcactttttttttgaagcattttcttttgccaagaataaaaatcatgtatagctattgcactaccaataggtcaattcatgctacaaatgtccatgtgtttctaggatgccagtggctactgctaccagaaataactccagtcactcccttgactagtgttgctagtttggtctttagggtttacctaagtgagagcatcaatgatgggttaaagtcacagaccacaatgaataaatcacagtctgtgcacacttttggccaggaagagtggcagtggaatcttgcatgtcatttggttgaaattaagactaaatctctatatgtgcacacacccacactcacacccacacgcacacatatcacagggttatagcagaatgaaaacggtgggtaggaatcaccagttgaaggctgtaggtttaaatgatcaggattggcacactcagatcagcccaccagtggtcttcactttgtgaaatggaactaatgccacaaggaaactgcatggttacttcatctgtttacacatctgcttatatgttcagctgaactgtcactgaaaacaggagcaccattcttgggacatgaaacaaggaggaggggaaacattcagataatcaacagttaatagaacaagtaaaaaaataagccaacagcaggtgcggcatctctggtatgcaaaacaactaatgaaagtgttcaaaggaattatcaaggcaggccattaagactataaaccatcaaaagagcagcagcaatagcaagagagaaagaagagggttagcaagagactagatcttcctgaaaaagtggccttggctctacaattgtctaccttgtgctgtccttagaagaacaggcccagtgctacagaataaaaatctccatgccaagccactgccttcagaatggtgatgatgtcttcttacaaaggtaaacccaagatgacaaccacaagcaaaaaaatcacccttttgttttaccatcaacagatgaaatagtccatacagtgccattcaatttcccacaggcagaaaccaaagacctcagaatgagaaagtcatggttttcacgtcacaaatgttacgtgtggtcagattatggagcaatgaaaacatttttctgcgccgctcattacactaaatcttgatgtttctgaagtctcttggagtttgagatgtattggaatagtttttcgcaccaagattaacatggcacagtaggaacaggctactgacaaatccatgtccacttaccttacccacaaggttccctaagggttcccttcattctcacaatatttcattttgagatgacttaaggtcaggtagaagggaccacataggccactcttcatcacttctcctcctagctcagaggctcacaattgaggcacttggcccttttgcactactaacatctggggctggaaacctgttgctggataaatacagctcagcaaatccccaaccatatttctattcactaaggtgttattggattgctcctgtttgtgcatgtctgcacacacatgcacaatttcttgtcctctccctccacacttacagacatacacctggtcatgtggaccatcgaaacacaacttgtttggatggaagaagaaaactctgcagatgctgttatttttagaagcctgcttatccctcctgaatgccaacaattttggcttggcatccatttcaaatcaagcaaggtgcatatccaggacaaagcaatgtgcattatgtctgaagggatccacatcttcagtgaaactcagaatgtggccagaactagctaactacctgaactgaaagcaccccatgttcagattcagaccaactcaaaacacatgtaaggggtgcctattgtatgcagggtaaggtgtcaagtccctttttatttggattaagctcaaataagaaaggacctgaagcgaacgtgggatgtgtatgtgtgtacatgtacacgtttgcaaacacacaggtttatgtgggtattaatatcgagtggaaaatctggctttttatttgtctgtgtctttttttttttttttcagtctgattcgagtatatctgttttggcaagttgtgggcagctctcttttacttttgtcacccagaggcttccgtagacaaaaggaaaggagagaggtgtgttcaaagacccccatggcgaagagcccatcccccaagcctgacacaaccctccctcccagcggacccctcttctggactggcttcgctgttggctacttcagtgcatctgacccccaccccccgcgtgaagacctgagattgagcgtggatttctgttctccaccaactctgcagcaagggccctgccagaggcgtcgcttcctgtcatctcctcttcccgctcccaagtagaggcacctaaacagagattagatttctggtttcaaggcatgtcggaccaagcacgctgaatgaacatgagttagttaattagctcggtctctcttctttccgttccctggtctgaatgtttcttgatggcaaagcgaccaggagagagttgatttgcatcttaagacctatgggtaatgcttctggagtggggagatttatttagcaactgcttgaacttgtgtacggggtcgggaaggaggtggagctgaccccaatggggctatcggagattggggtgtgggtggtgcccactgccacgctgacaccccgggcctcgatgatggcagacaggagctgctgctgctgctggcgcagggtgtcggcgatgagcagcggcagggagttgaagctggcggtgagatgctccagcttcgactccaggctgccaatctgcttctccaggtcttcgctccggtcattgagttctgtgattaagtcatacatgacattctgcatcttggaaaggtccaccagagtgttggcttggtcactcagcttcctctgttccatcttgacgctcctcaactggtggatagcttggaggaacttcctctggtgtttcctcactttggcatggtcaatcttctttagcagctttgtgtgtttatagattaaccatgtttcccgaaggacattggctgcagcattcttgatccgcttggtgagctgagtgtccatcatgaagttatgaacgtgcttctccgctttggtgagttccagctttcgggccaccacggccaccacaagggcagtgcagcctgcacccatgatgccagtgaggagacagacacctttcccacagtatgtgtggggcaccatgtccccataaccaatggaaaggaatgtgatggagatgagccacatggcacccagaaagttactagttacgtcctgctggtcatggtacctttcacagacacggacggtccaggcagcaatgatccacagagagatgctgaacacgagcagcacagtgccagggcagatggtcatgagcgtcttcatgacaaagcgggtgttgaagttgatcttgttgagggccccgatgctgcgggacgaggcatcggtgaagagcttgctgtgcagcagcatgactcgggcgatcaggtacaggcgcaggaacatggggatagacaggatgatgtccacatcggcctccgcccgggagggtgtgtaggagaaggccaggcgtgccgtccagaagaacttgtactcgccaggaatggggtggatggcgcacaccagcatctccaggctgatgtacaggatgcgctcgtaggtcatggctatccgccagtcatccgcgccattgtcgatcacgaagagctggacttcacgtgtgtggtaggcgatgatcaagcccaaaaggatgatggtggacagactgataaggcatttcagggccaacgaaaacatggagtccttcctccatctccactccctctgggagggaaaccccctcctccgtcttggggctggactgagaggctggagcagtggggccagctccccgctaaagccagtgcctgctgttctccatccgg

SEQ ID NO: 11618 - RNA, 4523 nt, Homo sapiens
  source 1..4523: mol_type = other RNA
ctgaatagctgggactacaggtgtccaccaccaaacccagctaatttttgtatttttagtagagatggggttttgccatgttggccaggctggtcttgaactcctgacctcaggtgatcctctcgccttgcccaaagtcctgggattacaggcatgagccaccgcacctggctatatataccagattcttgagcagataattaaacctcctccaccacaaaacttgaaaataaggtacaagaaggcatgacatgagaatccacctgccccttttcccatctgactgtgatgctgaggtgtggtggaattagccaaaagatgtaggaagaaaacttgggtgagctacacccagaataattaatacttaagtcatcaagggttgattgtacttgcaggagaacgggtaactttcccacataaagctgaaatgctagtacagagaaatagccttccatttgctattacaggatcaatgtgcaggtttgatcactttttttttgaagcattttcttttgccaagaataaaaatcatgtatagctattgcactaccaataggtcaattcatgctacaaatgtccatgtgtttctaggatgccagtggctactgctaccagaaataactccagtcactcccttgactagtgttgctagtttggtctttagggtttacctaagtgagagcatcaatgatgggttaaagtcacagaccacaatgaataaatcacagtctgtgcacacttttggccaggaagagtggcagtggaatcttgcatgtcatttggttgaaattaagactaaatctctatatgtgcacacacccacactcacacccacacgcacacatatcacagggttatagcagaatgaaaacggtgggtaggaatcaccagttgaaggctgtaggtttaaatgatcaggattggcacactcagatcagcccaccagtggtcttcactttgtgaaatggaactaatgccacaaggaaactgcatggttacttcatctgtttacacatctgcttatatgttcagctgaactgtcactgaaaacaggagcaccattcttgggacatgaaacaaggaggaggggaaacattcagataatcaacagttaatagaacaagtaaaaaaataagccaacagcaggtgcggcatctctggtatgcaaaacaactaatgaaagtgttcaaaggaattatcaaggcaggccattaagactataaaccatcaaaagagcagcagcaatagcaagagagaaagaagagggttagcaagagactagatcttcctgaaaaagtggccttggctctacaattgtctaccttgtgctgtccttagaagaacaggcccagtgctacagaataaaaatctccatgccaagccactgccttcagaatggtgatgatgtcttcttacaaaggtaaacccaagatgacaaccacaagcaaaaaaatcacccttttgttttaccatcaacagatgaaatagtccatacagtgccattcaatttcccacaggcagaaaccaaagacctcagaatgagaaagtcatggttttcacgtcacaaatgttacgtgtggtcagattatggagcaatgaaaacatttttctgcgccgctcattacactaaatcttgatgtttctgaagtctcttggagtttgagatgtattggaatagtttttcgcaccaagattaacatggcacagtaggaacaggctactgacaaatccatgtccacttaccttacccacaaggttccctaagggttcccttcattctcacaatatttcattttgagatgacttaaggtcaggtagaagggaccacataggccactcttcatcacttctcctcctagctcagaggctcacaattgaggcacttggcccttttgcactactaacatctggggctggaaacctgttgctggataaatacagctcagcaaatccccaaccatatttctattcactaaggtgttattggattgctcctgtttgtgcatgtctgcacacacatgcacaatttcttgtcctctccctccacacttacagacatacacctggtcatgtggaccatcgaaacacaacttgtttggatggaagaagaaaactctgcagatgctgttatttttagaagcctgcttatccctcctgaatgccaacaattttggcttggcatccatttcaaatcaagcaaggtgcatatccaggacaaagcaatgtgcattatgtctgaagggatccacatcttcagtgaaactcagaatgtggccagaactagctaactacctgaactgaaagcaccccatgttcagattcagaccaactcaaaacacatgtaaggggtgcctattgtatgcagggtaaggtgtcaagtccctttttatttggattaagctcaaataagaaaggacctgaagcgaacgtgggatgtgtatgtgtgtacatgtacacgtttgcaaacacacaggtttatgtgggtattaatatcgagtggaaaatctggctttttatttgtctgtgtctttttttttttttttcagtctgattcgagtatatctgttttggcaagttgtgggcagctctcttttacttttgtcacccagaggcttccgtagacaaaaggaaaggagagaggtgtgttcaaagacccccatggcgaagagcccatcccccaagcctgacacaaccctccctcccagcggacccctcttctggactggcttcgctgttggctacttcagtgcatctgacccccaccccccgcgtgaagacctgagattgagcgtggatttctgttctccaccaactctgcagcaagggccctgccagaggcgtcgcttcctgtcatctcctcttcccgctcccaagtagaggcacctaaacagagattagatttctggtttcaaggcatgtcggaccaagcacgctgaatgaacatgagttagttaattagctcggtctctcttctttccgttccctggtctgaatgtttcttgatggcaaagcgaccaggagagagttgatttgcatcttaagacctatgggtaatgcttctggagtggggagatttatttagcaactgcttgaacttgtgtacggggtcgggaaggaggtggagctgaccccaatggggctatcggagattggggtgtgggtggtgcccactgccacgctgacaccccgggcctcgatgatggcagacaggagctgctgctgctgctggcgcagggtgtcggcgatgagcagcggcagggagttgaagctggcggtgagatgctccagcttcgactccaggctgccaatctgcttctccaggtcttcgctccggtcattgagttctgtgattaagtcatacatgacattctgcatcttggaaaggtccaccagagtgttggcttggtcactcagcttcctctgttccatcttgacgctcctcaactggtggatagcttggaggaacttcctctggtgtttcctcactttggcatggtcaatcttctttagcagctttgtgtgtttatagattaaccatgtttcccgaaggacattggctgcagcattcttgatccgcttggtgagctgagtgtccatcatgaagttatgaacgtgcttctccgctttggtgagttccagctttcgggccaccacggccaccacaagggcagtgcagcctgcacccatgatgccagtgaggagacagacacctttcccacagtatgtgtggggcaccatgtccccataaccaatggaaaggaatgtgatggagatgagccacatggcacccagaaagttactagttacgtcctgctggtcatggtacctttcacagacacggacggtccaggcagcaatgatccacagagagatgctgaacacgagcagcacagtgccagggcagatggtcatgagcgtcttcatgacaaagcgggtgttgaagttgatcttgttgagggccccgatgctgcgggacgaggcatcggtgaagagcttgctgtgcagcagcatgactcgggcgatcaggtacaggcgcaggaacatggggatagacaggatgatgtccacatcggcctccgcccgggagggtgtgtaggagaaggccaggcgtgccgtccagaagaacttgtactcgccaggaatggggtggatggcgcacaccagcatctccaggctgatgtacaggatgcgctcgtaggtcatggctatccgccagtcatccgcgccattgtcgatcacgaagagctggacttcacgtgtgtggtaggcgatgatcaagcccaaaaggatgatggtggacagactgataaggcatttcagggccaacgaaaacatggagtcctttataggtctctccatctataacctgaagcaaaacaccaaacaactgtccttgcagatgtcgcgtggcaggcctggtatcagcaagctctaaggagtaggtgccagctcagtccctgcaaggagtgtcctttaagctgactttcctgttaatttgacactgagcagcactcctgtccttt

SEQ ID NO: 11619 - RNA, 5591 nt, Homo sapiens
  source 1..5591: mol_type = other RNA
ctgaatagctgggactacaggtgtccaccaccaaacccagctaatttttgtatttttagtagagatggggttttgccatgttggccaggctggtcttgaactcctgacctcaggtgatcctctcgccttgcccaaagtcctgggattacaggcatgagccaccgcacctggctatatataccagattcttgagcagataattaaacctcctccaccacaaaacttgaaaataaggtacaagaaggcatgacatgagaatccacctgccccttttcccatctgactgtgatgctgaggtgtggtggaattagccaaaagatgtaggaagaaaacttgggtgagctacacccagaataattaatacttaagtcatcaagggttgattgtacttgcaggagaacgggtaactttcccacataaagctgaaatgctagtacagagaaatagccttccatttgctattacaggatcaatgtgcaggtttgatcactttttttttgaagcattttcttttgccaagaataaaaatcatgtatagctattgcactaccaataggtcaattcatgctacaaatgtccatgtgtttctaggatgccagtggctactgctaccagaaataactccagtcactcccttgactagtgttgctagtttggtctttagggtttacctaagtgagagcatcaatgatgggttaaagtcacagaccacaatgaataaatcacagtctgtgcacacttttggccaggaagagtggcagtggaatcttgcatgtcatttggttgaaattaagactaaatctctatatgtgcacacacccacactcacacccacacgcacacatatcacagggttatagcagaatgaaaacggtgggtaggaatcaccagttgaaggctgtaggtttaaatgatcaggattggcacactcagatcagcccaccagtggtcttcactttgtgaaatggaactaatgccacaaggaaactgcatggttacttcatctgtttacacatctgcttatatgttcagctgaactgtcactgaaaacaggagcaccattcttgggacatgaaacaaggaggaggggaaacattcagataatcaacagttaatagaacaagtaaaaaaataagccaacagcaggtgcggcatctctggtatgcaaaacaactaatgaaagtgttcaaaggaattatcaaggcaggccattaagactataaaccatcaaaagagcagcagcaatagcaagagagaaagaagagggttagcaagagactagatcttcctgaaaaagtggccttggctctacaattgtctaccttgtgctgtccttagaagaacaggcccagtgctacagaataaaaatctccatgccaagccactgccttcagaatggtgatgatgtcttcttacaaaggtaaacccaagatgacaaccacaagcaaaaaaatcacccttttgttttaccatcaacagatgaaatagtccatacagtgccattcaatttcccacaggcagaaaccaaagacctcagaatgagaaagtcatggttttcacgtcacaaatgttacgtgtggtcagattatggagcaatgaaaacatttttctgcgccgctcattacactaaatcttgatgtttctgaagtctcttggagtttgagatgtattggaatagtttttcgcaccaagattaacatggcacagtaggaacaggctactgacaaatccatgtccacttaccttacccacaaggttccctaagggttcccttcattctcacaatatttcattttgagatgacttaaggtcaggtagaagggaccacataggccactcttcatcacttctcctcctagctcagaggctcacaattgaggcacttggcccttttgcactactaacatctggggctggaaacctgttgctggataaatacagctcagcaaatccccaaccatatttctattcactaaggtgttattggattgctcctgtttgtgcatgtctgcacacacatgcacaatttcttgtcctctccctccacacttacagacatacacctggtcatgtggaccatcgaaacacaacttgtttggatggaagaagaaaactctgcagatgctgttatttttagaagcctgcttatccctcctgaatgccaacaattttggcttggcatccatttcaaatcaagcaaggtgcatatccaggacaaagcaatgtgcattatgtctgaagggatccacatcttcagtgaaactcagaatgtggccagaactagctaactacctgaactgaaagcaccccatgttcagattcagaccaactcaaaacacatgtaaggggtgcctattgtatgcagggtaaggtgtcaagtccctttttatttggattaagctcaaataagaaaggacctgaagcgaacgtgggatgtgtatgtgtgtacatgtacacgtttgcaaacacacaggtttatgtgggtattaatatcgagtggaaaatctggctttttatttgtctgtgtctttttttttttttttcagtctgattcgagtatatctgttttggcaagttgtgggcagctctcttttacttttgtcacccagaggcttccgtagacaaaaggaaaggagagaggtgtgttcaaagacccccatggcgaagagcccatcccccaagcctgacacaaccctccctcccagcggacccctcttctggactggcttcgctgttggctacttcagtgcatctgacccccaccccccgcgtgaagacctgagattgagcgtggatttctgttctccaccaactctgcagcaagggccctgccagaggcgtcgcttcctgtcatctcctcttcccgctcccaagtagaggcacctaaacagagattagatttctggtttcaaggcatgtcggaccaagcacgctgaatgaacatgagttagttaattagctcggtctctcttctttccgttccctggtctgaatgtttcttgatggcaaagcgaccaggagagagttgatttgcatcttaagacctatgggtaatgcttctggagtggggagatttatttagcaactgcttgaacttgtgtacggggtcgggaaggaggtggagctgaccccaatggggctatcggagattggggtgtgggtggtgcccactgccacgctgacaccccgggcctcgatgatggcagacaggagctgctgctgctgctggcgcagggtgtcggcgatgagcagcggcagggagttgaagctggcggtgagatgctccagcttcgactccaggctgccaatctgcttctccaggtcttcgctccggtcattgagttctgtgattaagtcatacatgacattctgcatcttggaaaggtccaccagagtgttggcttggtcactcagcttcctctgttccatcttgacgctcctcaactggtggatagcttggaggaacttcctctggtgtttcctcactttggcatggtcaatcttctttagcagctttgtgtgtttatagattaaccatgtttcccgaaggacattggctgcagcattcttgatccgcttggtgagctgagtgtccatcatgaagttatgaacgtgcttctccgctttggtgagttccagctttcgggccaccacggccaccacaagggcagtgcagcctgcacccatgatgccagtgaggagacagacacctttcccacagtatgtgtggggcaccatgtccccataaccaatggaaaggaatgtgatggagatgagccacatggcacccagaaagttactagttacgtcctgctggtcatggtacctttcacagacacggacggtccaggcagcaatgatccacagagagatgctgaacacgagcagcacagtgccagggcagatggtcatgagcgtcttcatgacaaagcgggtgttgaagttgatcttgttgagggccccgatgctgcgggacgaggcatcggtgaagagcttgctgtgcagcagcatgactcgggcgatcaggtacaggcgcaggaacatggggatagacaggatgatgtccacatcggcctccgcccgggagggtgtgtaggagaaggccaggcgtgccgtccagaagaacttgtactcgccaggaatggggtggatggcgcacaccagcatctccaggctgatgtacaggatgcgctcgtaggtcatggctatccgccagtcatccgcgccattgtcgatcacgaagagctggacttcacgtgtgtggtaggcgatgatcaagcccaaaaggatgatggtggacagactgataaggcatttcagggccaacgaaaacatggagtcctttgagtacaaaccccaagagagctcggtctctatcaccataacaacaattccaaacatcccaaaaatcagagcatagtcactcagtcgctttctcttttcaaacagggccctcctgtgtcccagcttatagccaatgttttggtttttccgcttgttggctttggggaaggtggtgctgctggcggtggtgccggcatgctggtggttgtgggtggcattagggtgatggagcagggtctggtgggcatggttgtcctcccgggaggagatgacgatctccggggggttgctagggctgaaaagctggaggggttggccctcagtctcggcctcgatgaggttcctccgggaggcgctgaggcggctgaggggcttcatgaccccaccgctatacttgcaggagctcatggcgatctccgtgaaggggttgctgtcccgccggtgcaccagggggctggcctgtcggtgccggctgcctccgccaggcccacttgtagctgtggaacttggagagtggccaagcaagtggtcattgagattgagctggctgccttgcctggaggaagggtggaggatggcggtggagttggacgaagggggggccctgaaagcggtgggagaggagtgcagcaggccagggtggacgggctggctctggagttgggcgagctgagacaggggatgcggtggctgctgctgctgctgctgctgctgctgctgctgctgctgctgaagctgcggaggctgaggctgcagcgagggtcccaggggctgctggggggctgctggtggcgctggcggtggtggctgctgctgctgttgctgctgctgctgctgctgctgctcatccccagaggatggacaggggcacttggggtcttcatccaagtcccccacccccgagtcatggaagtgcccagaagtgtccatcttggggcctggctgtattccctgcagcacaagcccccaccccaaagccaccctcgctccaaagatgtcctcaaagaaagccaggcatccaatctcccccaccagtatcttggctccagtcctctctttggcttgcttcggttctctggggctgcctggagtccagacgctgccactcaagaatgcattgtattgggcagggagggagagcaggaggggagcttggagaaagaagagggggtgaaagaactctctcaggaggtggtcctctaggagcgtgtgaggccaggctcagcttcactcctcgctggctcaat

SEQ ID NO: 11620 - RNA, 5418 nt, Homo sapiens
  source 1..5418: mol_type = other RNA
ctgaatagctgggactacaggtgtccaccaccacacccagctaatttttgtatttttagtagagatggggtttcaccatattggccaggctggtctcaatctcctggccttgtgatccgcctgcctcggcctcccaaagtgctgggattacaggtgtgagccaccgcacctggccaaaatcgaggctctttagggagcagagtgtggggaaagacaatgaaagtcgaatatggaacctgatcaagtaggcaccaaacagaaacagacattcactcaatgaagttaaatttgcctaagaaggacctcacgggacgctcaacacaactgcagtaatgggaaggtctcataaactccgtgaagctcagtgcaggttcaattccctgtgagttgcagggaaatgcagattctctttggagaagcttggaagtttttgtgggtgttttgttttgcataaggctgggaagctcattgctccatcttttttttccagagcctgcagcagagacatccctcaggggatcggcttggcttagtggctggatctgagtggaatgggctctcacttgccatgtgtgcagtggtgcttgccagccccatatactcagccagggccatgctggctccctctgtcataagaccacttacgatgctctttcctcatccccagggatggccagctactccaaagccaatcaagaatcaacctgagggctgttgaacccagggagatactggaaccagatgcacttcaactagagtcactccaaaaagccactttgaatcacatctctaaggcaaggtccaggtccctggaggttctgtcagtccgtcctacatgctattctgtccttctggatggagaagagaaactcttctcagtcaacagcattcctccagagacctgaagtggccactgaagcctcccctagacccggctcaacagctgccttttcccatcatgtatcagacaacaggtggctgccattttagaaacagagtgttacaatgttacaattattctctcatgactggggaatgcagccacccactgcctgtcagaacagcacctcttcctgctcatctggaatgacacacgacacaaactagaagaaaagagggaaaaccaccaggccggaaggcaggcctgctagtgtcttcaatgaaacaggcacctcaaatacaactgcactcatacaactgcaacatcaagaggtatttctattagccaaactcaaaaacatttcttttttaaactgctcagtggtttgagacaccaagaacagttaatatcatacacaccagattatataacaaaaaaaatcaagtatttaaaagagtagcctgtatttttgttccttcaccttgttttttttcttgatacagggtctggctctgtcacccaggctggagtgcagtggctcaagagatcctcccacctcagcctcccaagtagctgggactgcaggcatgtgccaccacacctaattcttgtattttttgtagaaatgggctttcgccatgttgccaatgctggtctcaaactcctggactcaagcgatccgcccgcttcagcctccaaaagtgctgggattacaggcatgagccaccgcaccccgcctgttccctgaccttttaaacgaattcacgtattaacggagaatcaacatctaaatagacttttatttttattttacttgtttggacagaaaagaaaattcatcagctttcattagagtctccttaagtgttggaaacacattaaactcagaaatagtggaccttgtagaaaagcatcacaaattaaaaatatatttctccatgtggtaaaagtgctttcaatcccattaaagggcacagcaagggtgtttggaaacacgatctgaaatttggcctgcaatccgtggcatcgattccaaccacagggcgggggagtcaccatgatctagagcacaggagccacgtggggcccggagcatgcggacagcaacactcgcaataactgagtgaggacgaggcccatagcctgagtagaatagattctgtatttgtaaaaaatgaggtggttacatcaactgggttgaagggggactgggtaatcccagaaattccttgtttctggtctgtggggatggtcagatctgcccaccactctggcaccgaggcttccctggagacgcataaacctgggttgggaaagtgcccagatctgcctgggggacacacgagcctcgctgccagtgccgggcacgcagcctctccagtcctgccgtcagcaaccgcctccggccctcatgtcaaatcacacctgaccagagttgtcaccacagtcctgttttggggtttttccaaggccagccctgttgttctgaggggccactctgagcaggcaaacactgccagggtcactcactacacacagaggaaagacaatgagcaaatggccatcgtagagaattcggttgtgtgtttcagcaatgctacttatttttcaagacaagtaattctgccaatgatgacatctgcgacaaagcttagggcccgcgggctccccatgcgcctcgtggagagcaaccacgtctgttcggaagccagcggcccttcccggccctgccacaggccagaacacagaactgtgatcatgcaaagagccgtgactgaggccggggtcagcgtcgggggtggagaggaggggacatctgccttttacattagatctgaagcaacagtaagaaaataacctgaagatatatttaaaaataaaaaatagcatcatccttcactccaagtttttggcatttccctctctcccctgcccaccagctaagcagagggaatgagcaggaatgcctcgtttttcagaatgggcacccactccccatttcaccactgtacacccaggatgtgtgtcttcttctaagagaccggttcaaaggtgctggcatgaggcaaatgctggaaaaccctccggcctcccctgacacctgagccattgtaaccatgcagggcgtctttgcttccttcaagtcttgaacttgaaccacgtcccagattgctgtagatctttaggaagcaggcatctctcttagagcgtgctccagctcattctaccacgggggccttccttcacagtcaccagtccacgctgcctcgcaagctccacggatgtcatgagagaatctgcccttgagaacgtgggtgtaagtgctcatcacaccggcggcactgtttctcgagggaggacatgctcttcttggaatgcaaatgaggacagcaaccgtcctctgaccaggtccatcctgtccctccagaggccctgtgcatccctcccaggcagcaagccacacaccaggccgtgtccgggtctctgatgggcaagttggaacggcaggctctcctcctcctcttgcccctcccttgaccgagtcctgcgcccccagcatcagtgggtcggagaggcatcctccaagcccagcagctctctgacgagtctctctccaaactgcgcccggctgtacctcttcacgtggtaggcgtctgacattttgtacaggatgtaggcattgttgatggcgatgctgatggcgaaccagaacacctgctgccaggtcttgtttggtttatgagaaatgaaatacttgctgtatttgtcatcgtatctgcagatgtagctcaggtgagcggcaaacgcctccacggccaaggggcatgggatctccccactcttccttttgatgatgactccctgctgcaccggggagtaggcgttggtcaggaagcggaagtgtcctttgttgtaccagcagatcaaggacatgttccccttcatcttgatttggtactggccccgggccgggggtgtggctgggttggtcagcatggacagtgggaggccggtgcagtcactcttccgcgcgcggagcaagccgcagcagtaaatcccttgcttctcaaactcttcaaacagcgtcaggctggtgatgctgggccccgtgaaaatgatgtagttcttgcctgccgcgttccggcacaggctcctggccaccatgctgtggagctggggcttattcttcagcgcatccaggccatctgggcccccaccttccttcaggtggacataaatctggatgatgaagccagtggaagaacattgtctgacccagaggctgaatttccgctttttcctctttcgcagctcccgctctgtgcacgtggcaatgaatacaggatcctcatcgatcaggggttcatgtagcacctgggtttgggaaggcctgaaggcagagtcgaagctgttctgcagggagtcgaggaagggctggaccttgtagagcccgtgcgtggtctggctggagcggaaggccacgacgtggaagtacttgaggatcttctcgaagcgggcctggctcatgacgagggcgaggctgcggttgctgtagaagcctccgctccagatgctgaggacggactcgcagtgggagatgctggtggagatcatgtagcccaggaacgccttcatctccgtcagcgtcacctccacccaggctccgtcgctcccaaaccgctcctggaacttcttggcatacatgtttgtctgcaccaccatgttcttgaggacgttgtctgggacaaagagctggaagaagtccacggcactggcgctggggggcatctttcgggtgggaccgccggtatcctcgaagcgcgggggcgggcggtcccgcagcgctgcgctccagcccgcgccggcctcgtcctcctccggctcctgtgcgtccggggcgcggggcggtggcggggcggcccctgggggtcccgggggctcgcgctcgtcgtccgaggaggcggccgaggaggagcgcgaggcggccgaggtgctgtagaaggggttcccgccgctgtccgggccggactcgccgaacacgtcgtccgagatgtgcaggctctcgtagcgcgcgcgggcagcctcgagcagcgccggcgccctcctccgcgcgcccccgccgccctcggccatggccccggccgccgcccgcgcgcccgcccccacagtgcctcccagccgcacacgccgggccctgggcccgcgccgcggcccgccgccccccaccagcgcagcccgcagcacagcgcccgccgccccgtgcccggccggcccgccgtcttggccgcctcgggcccagcgcccggggaagcgccctcggagctcgggcgccgcaggctgcgggccgcggcgggaggcgagccgcgcgcggggctggcaggggcgacccagagcgggcgggacgcagaggctgcggccgagaccaggcgccgccgccgccaccgccgccaccaccgccaccaccgccgccgctgcgtctcctcggcgcccgccgcctccctgcccgccctctccacggcctccggcgctcggctgcc

SEQ ID NO: 11621 - RNA, 2578 nt, Homo sapiens
  source 1..2578: mol_type = other RNA
ctgaatagctgggactacaggtgtccaccaccacgctcgtctaatttttgtatttttagtagagacggggtttcaccatgttggccaggccggtcttgaactcttgacctcaggtgatctgcctgcctcggcctcccaaagtgctgggatttacaggtatgagccaccacatccagccaatgtgacccattatctcacagttctatatattagaagtccagcacagaacagatagattctcatactgaggatcatgcaaagctgaaatccaggtgtcagcccaggctgtggttatcatctgaagcttggagtactcttctaagctgactcagatttttggcagaattcagttccttgtggttgcaactgaggtcccaatttttttttcctgcttgctgacaactggaaggtaggtctcatctcctagaggccacctttaggttttagccaatgtggccctctcacatacttcttcaaggcttacaaggagaattcttcttgcaagggttcacttgattaggtcaggccctttcaacagtctcaaagtgagttgtttaggaaccttaactgcatctgccaaattccttcaactttgtcatgtaacataatctaataatggacatatcattatggcagtatcatcaagggatattttatttgtggttaaatgattgctgtgaacacaatctataaatatatgactaataggattttgtaactggctctataaactttaaattttgtatcattttacaatttacaaagtgcttgtatatattttgcatcatttgattttcatgactacctgtcagagaagcacagcagatattagcccaatgttattagtggctcacagcagctaagtgtatgtccaaagctttacagcaaattagtagtggagtcagctgggcttcagatcagagtgtttccaccctacatacagcccaggctctttttgctaaccctgtaattttcaaactgtgtttggtgatgcttgaaggagatttctcagggattactgtaagaactgggggtgatactaatgggtagggctaagtgttgatatggtggctctatttttatattttggaagttcaacccatgctttaataaccactgtcctgcaacagcctatgccttgttaaaggtaaagaagaatatttaggaaaaaaatcagttaaaaaaatggttgagataggtgtatataaaaagtcaagagtcttttccaataaagttttaagaagctgtcatctcttgcagcagctgttgaaccttcttaatgtctggtctcttatttttcttttcatgcagacattgactagcaacagagtacatagcttcaactgaagtggaatcagcatcattcatctttttatcaatataatcttcaattgtcttttcttcatcttcaatttcttctttaatatctagcaataactgaggttcacggtgttcatccacagctggaagtccagttattatttctagtaaaaccacaccaaagctgtaaatatcagatttgggtgttatttctccacgcaaagcttctggtgccatataagctgttgttcccacaattctgctagtcatgactgtctgggcaaacttctcagaagcccgtgcaaggccaaagtcagatattttagcagtaaaagcttcatccagtaagatatttgcacttttaatatctctatgaatatgatgattttcatgtagaaaattgatgccattagctgcaccctgagcaatcttgcatctcatgtgccaagaaagtggtggagtaccatccaagcaagagagtctgtctagcaatgaaccattaggcatgtaaacatatactaagcagaggtcatctccatcacttgagaaaccaagtagttctactaagttttcatgttgacactttgccattacttttatttcttgatcaaactgctgtttcagttcttcagtagtaatgtcaaccatcaccaacagaaatgggtcgttcatcaaagttatttgtgacattcttcaattcataaaatgaaaaactgtgaaaacgtgtatcactaacttctaaacttttattttctggacttgaggagtcaggtggcatatagctttgttcaagattctgcacaggtgtcatcaatgtcctgtctttgtcacagaaaggcatctgtttttgctgaactgttatagcttctttagaaggtagtgtattagcagttttgggaacagcatctgggagcaaaagactcgcaggagcaaaaaattcattttggatcaaaagatccacaagatcaccaactgtgcaatttgtggtgccccagtcaaacagtaattcagaagtgggactttttccagtttgaagtaatgcttcaaatctccttatgtgaaactgattgtatctatcatcaccagatggttttttaatagctacagctaacttcttccatccttcttgaggatcaataaaatctgacagcttcctaattagtccaacattgaggcagcgcacatatgttgatggtgttatgggtttgttcatcttctattcctgcccgggcgcgggctgctgaagccggcgacagaa

SEQ ID NO: 11622 - RNA, 2467 nt, Homo sapiens
  source 1..2467: mol_type = other RNA
ctgaatagctgggactacaggtgtccaccaccacgctcgtctaatttttgtatttttagtagagacggggtttcaccatgttggccaggccggtcttgaactcttgacctcaggtgatctgcctgcctcggcctcccaaagtgctgggatttacaggtatgagccaccacatccagccaatgtgacccattatctcacagttctatatattagaagtccagcacagaacagatagattctcatactgaggatcatgcaaagctgaaatccaggtgtcagcccaggctgtggttatcatctgaagcttggagtactcttctaagctgactcagatttttggcagaattcagttccttgtggttgcaactgaggtcccaatttttttttcctgcttgctgacaactggaaggtaggtctcatctcctagaggccacctttaggttttagccaatgtggccctctcacatacttcttcaaggcttacaaggagaattcttcttgcaagggttcacttgattaggtcaggccctttcaacagtctcaaagtgagttgtttaggaaccttaactgcatctgccaaattccttcaactttgtcatgtaacataatctaataatggacatatcattatggcagtatcatcaagggatattttatttgtggttaaatgattgctgtgaacacaatctataaatatatgactaataggattttgtaactggctctataaactttaaattttgtatcattttacaatttacaaagtgcttgtatatattttgcatcatttgattttcatgactacctgtcagagaagcacagcagatattagcccaatgttattagtggctcacagcagctaagtgtatgtccaaagctttacagcaaattagtagtggagtcagctgggcttcagatcagagtgtttccaccctacatacagcccaggctctttttgctaaccctgtaattttcaaactgtgtttggtgatgcttgaaggagatttctcagggattactgtaagaactgggggtgatactaatgggtagggctaagtgttgatatggtggctctatttttatattttggaagttcaacccatgctttaataaccactgtcctgcaacagcctatgccttgttaaaggtaaagaagaatatttaggaaaaaaatcagttaaaaaaatggttgagataggtgtatataaaaagtcaagagtcttttccaataaagttttaagaagctgtcatctcttgcagcagctgttgaaccttcttaatgtctggtctcttatttttcttttcatgcagacattgactagcaacagagtacatagcttcaactgaagtggaatcagcatcattcatctttttatcaatataatcttcaattgtcttttcttcatcttcaatttcttctttaatatctagcaataactgaggttcacggtgttcatccacagctggaagtccagttattatttctagtaaaaccacaccaaagctgtaaatatcagatttgggtgttatttctccacgcaaagcttctggtgccatataagctgttgttcccacaattctgctagtcatgactgtctgggcaaacttctcagaagcccgtgcaaggccaaagtcagatattttagcagtaaaagcttcatccagtaagatatttgcacttttaatatctctatgaatatgatgattttcatgtagaaaattgatgccattagctgcaccctgagcaatcttgcatctcatgtgccaagaaagtggtggagtaccatccaagcaagagagtctgtctagcaatgaaccattaggcatgtaaacatatactaagcagaggtcatctccatcacttgagaaaccaagtagttctactaagttttcatgttgacactttgccattacttttatttcttgatcaaactgctgtttcagttcttcagtagtaatgtcaaccatcaccaacagaaatgggtcgttcatcaaagttatttgtgacattcttcaattcataaaatgaaaaactgtgaaaacgtgtatcactaacttctaaacttttattttctggacttgaggagtcaggtggcatatagctttgttcaagattctgcacaggtgtcatcaatgtcctgtctttgtcacagaaaggcatctgtttttgctgaactgttatagcttctttagaaggtagtgtattagcagttttgggaacagcatcttatgtgaaactgattgtatctatcatcaccagatggttttttaatagctacagctaacttcttccatccttcttgaggatcaataaaatctgacagcttcctaattagtccaacattgaggcagcgcacatatgttgatggtgttatgggtttgttcatcttctattccaaatatttactgagtgtctactttgtgctagatactgctccaggcccctgcccgggcgcgggctgctgaa

SEQ ID NO: 11623 - RNA, 2646 nt, Homo sapiens
  source 1..2646: mol_type = other RNA
ctgaatagctgggactacaggtgtccaccaccacgctcgtctaatttttgtatttttagtagagacggggtttcaccatgttggccaggccggtcttgaactcttgacctcaggtgatctgcctgcctcggcctcccaaagtgctgggatttacaggtatgagccaccacatccagccaatgtgacccattatctcacagttctatatattagaagtccagcacagaacagatagattctcatactgaggatcatgcaaagctgaaatccaggtgtcagcccaggctgtggttatcatctgaagcttggagtactcttctaagctgactcagatttttggcagaattcagttccttgtggttgcaactgaggtcccaatttttttttcctgcttgctgacaactggaaggtaggtctcatctcctagaggccacctttaggttttagccaatgtggccctctcacatacttcttcaaggcttacaaggagaattcttcttgcaagggttcacttgattaggtcaggccctttcaacagtctcaaagtgagttgtttaggaaccttaactgcatctgccaaattccttcaactttgtcatgtaacataatctaataatggacatatcattatggcagtatcatcaagggatattttatttgtggttaaatgattgctgtgaacacaatctataaatatatgactaataggattttgtaactggctctataaactttaaattttgtatcattttacaatttacaaagtgcttgtatatattttgcatcatttgattttcatgactacctgtcagagaagcacagcagatattagcccaatgttattagtggctcacagcagctaagtgtatgtccaaagctttacagcaaattagtagtggagtcagctgggcttcagatcagagtgtttccaccctacatacagcccaggctctttttgctaaccctgtaattttcaaactgtgtttggtgatgcttgaaggagatttctcagggattactgtaagaactgggggtgatactaatgggtagggctaagtgttgatatggtggctctatttttatattttggaagttcaacccatgctttaataaccactgtcctgcaacagcctatgccttgttaaaggtaaagaagaatatttaggaaaaaaatcagttaaaaaaatggttgagataggtgtatataaaaagtcaagagtcttttccaataaagttttaagaagctgtcatctcttgcagcagctgttgaaccttcttaatgtctggtctcttatttttcttttcatgcagacattgactagcaacagagtacatagcttcaactgaagtggaatcagcatcattcatctttttatcaatataatcttcaattgtcttttcttcatcttcaatttcttctttaatatctagcaataactgaggttcacggtgttcatccacagctggaagtccagttattatttctagtaaaaccacaccaaagctgtaaatatcagatttgggtgttatttctccacgcaaagcttctggtgccatataagctgttgttcccacaattctgctagtcatgactgtctgggcaaacttctcagaagcccgtgcaaggccaaagtcagatattttagcagtaaaagcttcatccagtaagatatttgcacttttaatatctctatgaatatgatgattttcatgtagaaaattgatgccattagctgcaccctgagcaatcttgcatctcatgtgccaagaaagtggtggagtaccatccaagcaagagagtctgtctagcaatgaaccattaggcatgtaaacatatactaagcagaggtcatctccatcacttgagaaaccaagtagttctactaagttttcatgttgacactttgccattacttttatttcttgatcaaactgctgtttcagttcttcagtagtaatgtcaaccatcaccaacagaaatgggtcgttcatcaaagttatttgtgacattcttcaattcataaaatgaaaaactgtgaaaacgtgtatcactaacttctaaacttttattttctggacttgaggagtcaggtggcatatagctttgttcaagattctgcacaggtgtcatcaatgtcctgtctttgtcacagaaaggcatctgtttttgctgaactgttatagcttctttagaaggtagtgtattagcagttttgggaacagcatcttatgtgaaactgattgtatctatcatcaccagatggttttttaatagctacagctaacttcttccatccttcttgaggatcaataaaatctgacagcttcctaattagtccaacattgaggcagcgcacatatgttgatggtgttatgggtttgttcatcttctattcccaagtctttcttctggagtaagctctgtcaaaggaacccacttcctctctaacttttctcacggatgataaagagatttccgttccgcagccgaccccagcaaccctggggcagaggtgccgaggcctggaagcggacctcggacgacgtttgaccgaggcattaaggcggggaatgccttacctgcccgggcgcgggctgctgaagccggcgacagaagaaccagccgaactaggaagcgccgcgaag

SEQ ID NO: 11624 - RNA, 2462 nt, Homo sapiens
  source 1..2462: mol_type = other RNA
ctgaatagctgggactacaggtgtccaccaccacgctcgtctaatttttgtatttttagtagagacggggtttcaccatgttggccaggccggtcttgaactcttgacctcaggtgatctgcctgcctcggcctcccaaagtgctgggatttacaggtatgagccaccacatccagccaatgtgacccattatctcacagttctatatattagaagtccagcacagaacagatagattctcatactgaggatcatgcaaagctgaaatccaggtgtcagcccaggctgtggttatcatctgaagcttggagtactcttctaagctgactcagatttttggcagaattcagttccttgtggttgcaactgaggtcccaatttttttttcctgcttgctgacaactggaaggtaggtctcatctcctagaggccacctttaggttttagccaatgtggccctctcacatacttcttcaaggcttacaaggagaattcttcttgcaagggttcacttgattaggtcaggccctttcaacagtctcaaagtgagttgtttaggaaccttaactgcatctgccaaattccttcaactttgtcatgtaacataatctaataatggacatatcattatggcagtatcatcaagggatattttatttgtggttaaatgattgctgtgaacacaatctataaatatatgactaataggattttgtaactggctctataaactttaaattttgtatcattttacaatttacaaagtgcttgtatatattttgcatcatttgattttcatgactacctgtcagagaagcacagcagatattagcccaatgttattagtggctcacagcagctaagtgtatgtccaaagctttacagcaaattagtagtggagtcagctgggcttcagatcagagtgtttccaccctacatacagcccaggctctttttgctaaccctgtaattttcaaactgtgtttggtgatgcttgaaggagatttctcagggattactgtaagaactgggggtgatactaatgggtagggctaagtgttgatatggtggctctatttttatattttggaagttcaacccatgctttaataaccactgtcctgcaacagcctatgccttgttaaaggtaaagaagaatatttaggaaaaaaatcagttaaaaaaatggttgagataggtgtatataaaaagtcaagagtcttttccaataaagttttaagaagctgtcatctcttgcagcagctgttgaaccttcttaatgtctggtctcttatttttcttttcatgcagacattgactagcaacagagtacatagcttcaactgaagtggaatcagcatcattcatctttttatcaatataatcttcaattgtcttttcttcatcttcaatttcttctttaatatctagcaataactgaggttcacggtgttcatccacagctggaagtccagttattatttctagtaaaaccacaccaaagctgtaaatatcagatttgggtgttatttctccacgcaaagcttctggtgccatataagctgttgttcccacaattctgctagtcatgactgtctgggcaaacttctcagaagcccgtgcaaggccaaagtcagatattttagcagtaaaagcttcatccagtaagatatttgcacttttaatatctctatgaatatgatgattttcatgtagaaaattgatgccattagctgcaccctgagcaatcttgcatctcatgtgccaagaaagtggtggagtaccatccaagcaagagagtctgtctagcaatgaaccattaggcatgtaaacatatactaagcagaggtcatctccatcacttgagaaaccaagtagttctactaagttttcatgttgacactttgccattacttttatttcttgatcaaactgctgtttcagttcttcagtagtaatgtcaaccatcaccaacagaaatgggtcgttcatcaaagttatttgtgacattcttcaattcataaaatgaaaaactgtgaaaacgtgtatcactaacttctaaacttttattttctggacttgaggagtcaggtggcatatagctttgttcaagattctgcacaggtgtcatcaatgtcctgtctttgtcacagaaaggcatctgtttttgctgaactgttatagcttctttagaaggtagtgtattagcagttttgggaacagcatcttatgtgaaactgattgtatctatcatcaccagatggttttttaatagctacagctaacttcttccatccttcttgaggatcaataaaatctgacagcttcctaattagtccaacattgaggcagcgcacatatgttgatggtgttatgggtttgttcatcttctattcctgcccgggcgcgggctgctgaagccggcgacagaagaaccagccgaactaggaagcgccgcgaag

SEQ ID NO: 11625 - RNA, 2378 nt, Homo sapiens
  source 1..2378: mol_type = other RNA
ctgaatagctgggactacaggtgtccaccaccacgctcgtctaatttttgtatttttagtagagacggggtttcaccatgttggccaggccggtcttgaactcttgacctcaggtgatctgcctgcctcggcctcccaaagtgctgggatttacaggtatgagccaccacatccagccaatgtgacccattatctcacagttctatatattagaagtccagcacagaacagatagattctcatactgaggatcatgcaaagctgaaatccaggtgtcagcccaggctgtggttatcatctgaagcttggagtactcttctaagctgactcagatttttggcagaattcagttccttgtggttgcaactgaggtcccaatttttttttcctgcttgctgacaactggaaggtaggtctcatctcctagaggccacctttaggttttagccaatgtggccctctcacatacttcttcaaggcttacaaggagaattcttcttgcaagggttcacttgattaggtcaggccctttcaacagtctcaaagtgagttgtttaggaaccttaactgcatctgccaaattccttcaactttgtcatgtaacataatctaataatggacatatcattatggcagtatcatcaagggatattttatttgtggttaaatgattgctgtgaacacaatctataaatatatgactaataggattttgtaactggctctataaactttaaattttgtatcattttacaatttacaaagtgcttgtatatattttgcatcatttgattttcatgactacctgtcagagaagcacagcagatattagcccaatgttattagtggctcacagcagctaagtgtatgtccaaagctttacagcaaattagtagtggagtcagctgggcttcagatcagagtgtttccaccctacatacagcccaggctctttttgctaaccctgtaattttcaaactgtgtttggtgatgcttgaaggagatttctcagggattactgtaagaactgggggtgatactaatgggtagggctaagtgttgatatggtggctctatttttatattttggaagttcaacccatgctttaataaccactgtcctgcaacagcctatgccttgttaaaggtaaagaagaatatttaggaaaaaaatcagttaaaaaaatggttgagataggtgtatataaaaagtcaagagtcttttccaataaagttttaagaagctgtcatctcttgcagcagctgttgaaccttcttaatgtctggtctcttatttttcttttcatgcagacattgactagcaacagagtacatagcttcaactgaagtggaatcagcatcattcatctttttatcaatataatcttcaattgtcttttcttcatcttcaatttcttctttaatatctagcaataactgaggttcacggtgttcatccacagctggaagtccagttattatttctagtaaaaccacaccaaagctgtaaatatcagatttgggtgttatttctccacgcaaagcttctggtgccatataagctgttgttcccacaattctgctagtcatgactgtctgggcaaacttctcagaagcccgtgcaaggccaaagtcagatattttagcagtaaaagcttcatccagtaagatatttgcacttttaatatctctatgaatatgatgattttcatgtagaaaattgatgccattagctgcaccctgagcaatcttgcatctcatgtgccaagaaagtggtggagtaccatccaagcaagagagtctgtctagcaatgaaccattaggcatgtaaacatatactaagcagaggtcatctccatcacttgagaaaccaagtagttctactaagttttcatgttgacactttgccattacttttatttcttgatcaaactgctgtttcagttcttcagtagtaatgtcaaccattgctgcaagcttcttcactgccacagttgtgttatttacgtagcctttatatacaactccaaatcctccctctcccattttattaccaccaacagaaatgggtcgttcatcaaagttatttgtgacattcttcaattcataaaatgaaaaactgtgaaaacgtgtatcactaacttctaaacttttattttctggacttgaggagtcaggtggcatatagctttgttcaagattctgcacaggtgtcatcaatgtcctgtctttgtcacagaaaggcatctgtttttgctgaactgttatagcttctttagaaggtagtgtattagcagttttgggaacagcatctgcccgggcgcgggctgctgaagccggcgacagaagaaccagccgaactaggaagcgccgcgaag

SEQ ID NO: 11626 - RNA, 2818 nt, Homo sapiens
  source 1..2818: mol_type = other RNA
ctgaatagctgggactacaggtgtccaccaccacgctcgtctaatttttgtatttttagtagagacggggtttcaccatgttggccaggccggtcttgaactcttgacctcaggtgatctgcctgcctcggcctcccaaagtgctgggatttacaggtatgagccaccacatccagccaatgtgacccattatctcacagttctatatattagaagtccagcacagaacagatagattctcatactgaggatcatgcaaagctgaaatccaggtgtcagcccaggctgtggttatcatctgaagcttggagtactcttctaagctgactcagatttttggcagaattcagttccttgtggttgcaactgaggtcccaatttttttttcctgcttgctgacaactggaaggtaggtctcatctcctagaggccacctttaggttttagccaatgtggccctctcacatacttcttcaaggcttacaaggagaattcttcttgcaagggttcacttgattaggtcaggccctttcaacagtctcaaagtgagttgtttaggaaccttaactgcatctgccaaattccttcaactttgtcatgtaacataatctaataatggacatatcattatggcagtatcatcaagggatattttatttgtggttaaatgattgctgtgaacacaatctataaatatatgactaataggattttgtaactggctctataaactttaaattttgtatcattttacaatttacaaagtgcttgtatatattttgcatcatttgattttcatgactacctgtcagagaagcacagcagatattagcccaatgttattagtggctcacagcagctaagtgtatgtccaaagctttacagcaaattagtagtggagtcagctgggcttcagatcagagtgtttccaccctacatacagcccaggctctttttgctaaccctgtaattttcaaactgtgtttggtgatgcttgaaggagatttctcagggattactgtaagaactgggggtgatactaatgggtagggctaagtgttgatatggtggctctatttttatattttggaagttcaacccatgctttaataaccactgtcctgcaacagcctatgccttgttaaaggtaaagaagaatatttaggaaaaaaatcagttaaaaaaatggttgagataggtgtatataaaaagtcaagagtcttttccaataaagttttaagaagctgtcatctcttgcagcagctgttgaaccttcttaatgtctggtctcttatttttcttttcatgcagacattgactagcaacagagtacatagcttcaactgaagtggaatcagcatcattcatctttttatcaatataatcttcaattgtcttttcttcatcttcaatttcttctttaatatctagcaataactgaggttcacggtgttcatccacagctggaagtccagttattatttctagtaaaaccacaccaaagctgtaaatatcagatttgggtgttatttctccacgcaaagcttctggtgccatataagctgttgttcccacaattctgctagtcatgactgtctgggcaaacttctcagaagcccgtgcaaggccaaagtcagatattttagcagtaaaagcttcatccagtaagatatttgcacttttaatatctctatgaatatgatgattttcatgtagaaaattgatgccattagctgcaccctgagcaatcttgcatctcatgtgccaagaaagtggtggagtaccatccaagcaagagagtctgtctagcaatgaaccattaggcatgtaaacatatactaagcagaggtcatctccatcacttgagaaaccaagtagttctactaagttttcatgttgacactttgccattacttttatttcttgatcaaactgctgtttcagttcttcagtagtaatgtcaaccattgctgcaagcttcttcactgccacagttgtgttatttacgtagcctttatatacaactccaaatcctccctctcccattttattaccaccaacagaaatgggtcgttcatcaaagttatttgtgacattcttcaattcataaaatgaaaaactgtgaaaacgtgtatcactaacttctaaacttttattttctggacttgaggagtcaggtggcatatagctttgttcaagattctgcacaggtgtcatcaatgtcctgtctttgtcacagaaaggcatctgtttttgctgaactgttatagcttctttagaaggtagtgtattagcagttttgggaacagcatctgggagcaaaagactcgcaggagcaaaaaattcattttggatcaaaagatccacaagatcaccaactgtgcaatttgtggtgccccagtcaaacagtaattcagaagtgggactttttccagtttgaagtaatgcttcaaatctccttatgtgaaactgattgtatctatcatcaccagatggttttttaatagctacagctaacttcttccatccttcttgaggatcaataaaatctgacagcttcctaattagtccaacattgaggcagcgcacatatgttgatggtgttatgggtttgttcatcttctattccaaatatttactgagtgtctactttgtgctagatactgctccaggccccaggggccttgggcagttacgtttttgaagcactaatagcgccgtttgttcccattctaaatgctcaaagtgctttctcgctttctcagggtttgcttttttttttttttttttcttttgagacggagtctccctctgttgc

SEQ ID NO: 11627 - RNA, 2926 nt, Homo sapiens
  source 1..2926: mol_type = other RNA
ctgaatagctgggactacaggtgtccaccaccacgctcgtctaatttttgtatttttagtagagacggggtttcaccatgttggccaggccggtcttgaactcttgacctcaggtgatctgcctgcctcggcctcccaaagtgctgggatttacaggtatgagccaccacatccagccaatgtgacccattatctcacagttctatatattagaagtccagcacagaacagatagattctcatactgaggatcatgcaaagctgaaatccaggtgtcagcccaggctgtggttatcatctgaagcttggagtactcttctaagctgactcagatttttggcagaattcagttccttgtggttgcaactgaggtcccaatttttttttcctgcttgctgacaactggaaggtaggtctcatctcctagaggccacctttaggttttagccaatgtggccctctcacatacttcttcaaggcttacaaggagaattcttcttgcaagggttcacttgattaggtcaggccctttcaacagtctcaaagtgagttgtttaggaaccttaactgcatctgccaaattccttcaactttgtcatgtaacataatctaataatggacatatcattatggcagtatcatcaagggatattttatttgtggttaaatgattgctgtgaacacaatctataaatatatgactaataggattttgtaactggctctataaactttaaattttgtatcattttacaatttacaaagtgcttgtatatattttgcatcatttgattttcatgactacctgtcagagaagcacagcagatattagcccaatgttattagtggctcacagcagctaagtgtatgtccaaagctttacagcaaattagtagtggagtcagctgggcttcagatcagagtgtttccaccctacatacagcccaggctctttttgctaaccctgtaattttcaaactgtgtttggtgatgcttgaaggagatttctcagggattactgtaagaactgggggtgatactaatgggtagggctaagtgttgatatggtggctctatttttatattttggaagttcaacccatgctttaataaccactgtcctgcaacagcctatgccttgttaaaggtaaagaagaatatttaggaaaaaaatcagttaaaaaaatggttgagataggtgtatataaaaagtcaagagtcttttccaataaagttttaagaagctgtcatctcttgcagcagctgttgaaccttcttaatgtctggtctcttatttttcttttcatgcagacattgactagcaacagagtacatagcttcaactgaagtggaatcagcatcattcatctttttatcaatataatcttcaattgtcttttcttcatcttcaatttcttctttaatatctagcaataactgaggttcacggtgttcatccacagctggaagtccagttattatttctagtaaaaccacaccaaagctgtaaatatcagatttgggtgttatttctccacgcaaagcttctggtgccatataagctgttgttcccacaattctgctagtcatgactgtctgggcaaacttctcagaagcccgtgcaaggccaaagtcagatattttagcagtaaaagcttcatccagtaagatatttgcacttttaatatctctatgaatatgatgattttcatgtagaaaattgatgccattagctgcaccctgagcaatcttgcatctcatgtgccaagaaagtggtggagtaccatccaagcaagagagtctgtctagcaatgaaccattaggcatgtaaacatatactaagcagaggtcatctccatcacttgagaaaccaagtagttctactaagttttcatgttgacactttgccattacttttatttcttgatcaaactgctgtttcagttcttcagtagtaatgtcaaccattgctgcaagcttcttcactgccacagttgtgttatttacgtagcctttatatacaactccaaatcctccctctcccattttattaccaccaacagaaatgggtcgttcatcaaagttatttgtgacattcttcaattcataaaatgaaaaactgtgaaaacgtgtatcactaacttctaaacttttattttctggacttgaggagtcaggtggcatatagctttgttcaagattctgcacaggtgtcatcaatgtcctgtctttgtcacagaaaggcatctgtttttgctgaactgttatagcttctttagaaggtagtgtattagcagttttgggaacagcatctgggagcaaaagactcgcaggagcaaaaaattcattttggatcaaaagatccacaagatcaccaactgtgcaatttgtggtgccccagtcaaacagtaattcagaagtgggactttttccagtttgaagtaatgcttcaaatctccttatgtgaaactgattgtatctatcatcaccagatggttttttaatagctacagctaacttcttccatccttcttgaggatcaataaaatctgacagcttcctaattagtccaacattgaggcagcgcacatatgttgatggtgttatgggtttgttcatcttctattccaaatatttactgagtgtctactttgtgctagatactgctccaggcccccaagtctttcttctggagtaagctctgtcaaaggaacccacttcctctctaacttttctcacggatgataaagagatttccgttccgcagccgaccccagcaaccctggggcagaggtgccgaggcctggaagcggacctcggacgacgtttgaccgaggcattaaggcggggaatgccttacctgcccgggcgcgggctgctgaagccggcgacagaagaaccagccgaactaggaagcgccgcgaag

SEQ ID NO: 11628 - RNA, 2742 nt, Homo sapiens
  source 1..2742: mol_type = other RNA
ctgaatagctgggactacaggtgtccaccaccacgctcgtctaatttttgtatttttagtagagacggggtttcaccatgttggccaggccggtcttgaactcttgacctcaggtgatctgcctgcctcggcctcccaaagtgctgggatttacaggtatgagccaccacatccagccaatgtgacccattatctcacagttctatatattagaagtccagcacagaacagatagattctcatactgaggatcatgcaaagctgaaatccaggtgtcagcccaggctgtggttatcatctgaagcttggagtactcttctaagctgactcagatttttggcagaattcagttccttgtggttgcaactgaggtcccaatttttttttcctgcttgctgacaactggaaggtaggtctcatctcctagaggccacctttaggttttagccaatgtggccctctcacatacttcttcaaggcttacaaggagaattcttcttgcaagggttcacttgattaggtcaggccctttcaacagtctcaaagtgagttgtttaggaaccttaactgcatctgccaaattccttcaactttgtcatgtaacataatctaataatggacatatcattatggcagtatcatcaagggatattttatttgtggttaaatgattgctgtgaacacaatctataaatatatgactaataggattttgtaactggctctataaactttaaattttgtatcattttacaatttacaaagtgcttgtatatattttgcatcatttgattttcatgactacctgtcagagaagcacagcagatattagcccaatgttattagtggctcacagcagctaagtgtatgtccaaagctttacagcaaattagtagtggagtcagctgggcttcagatcagagtgtttccaccctacatacagcccaggctctttttgctaaccctgtaattttcaaactgtgtttggtgatgcttgaaggagatttctcagggattactgtaagaactgggggtgatactaatgggtagggctaagtgttgatatggtggctctatttttatattttggaagttcaacccatgctttaataaccactgtcctgcaacagcctatgccttgttaaaggtaaagaagaatatttaggaaaaaaatcagttaaaaaaatggttgagataggtgtatataaaaagtcaagagtcttttccaataaagttttaagaagctgtcatctcttgcagcagctgttgaaccttcttaatgtctggtctcttatttttcttttcatgcagacattgactagcaacagagtacatagcttcaactgaagtggaatcagcatcattcatctttttatcaatataatcttcaattgtcttttcttcatcttcaatttcttctttaatatctagcaataactgaggttcacggtgttcatccacagctggaagtccagttattatttctagtaaaaccacaccaaagctgtaaatatcagatttgggtgttatttctccacgcaaagcttctggtgccatataagctgttgttcccacaattctgctagtcatgactgtctgggcaaacttctcagaagcccgtgcaaggccaaagtcagatattttagcagtaaaagcttcatccagtaagatatttgcacttttaatatctctatgaatatgatgattttcatgtagaaaattgatgccattagctgcaccctgagcaatcttgcatctcatgtgccaagaaagtggtggagtaccatccaagcaagagagtctgtctagcaatgaaccattaggcatgtaaacatatactaagcagaggtcatctccatcacttgagaaaccaagtagttctactaagttttcatgttgacactttgccattacttttatttcttgatcaaactgctgtttcagttcttcagtagtaatgtcaaccattgctgcaagcttcttcactgccacagttgtgttatttacgtagcctttatatacaactccaaatcctccctctcccattttattaccaccaacagaaatgggtcgttcatcaaagttatttgtgacattcttcaattcataaaatgaaaaactgtgaaaacgtgtatcactaacttctaaacttttattttctggacttgaggagtcaggtggcatatagctttgttcaagattctgcacaggtgtcatcaatgtcctgtctttgtcacagaaaggcatctgtttttgctgaactgttatagcttctttagaaggtagtgtattagcagttttgggaacagcatctgggagcaaaagactcgcaggagcaaaaaattcattttggatcaaaagatccacaagatcaccaactgtgcaatttgtggtgccccagtcaaacagtaattcagaagtgggactttttccagtttgaagtaatgcttcaaatctccttatgtgaaactgattgtatctatcatcaccagatggttttttaatagctacagctaacttcttccatccttcttgaggatcaataaaatctgacagcttcctaattagtccaacattgaggcagcgcacatatgttgatggtgttatgggtttgttcatcttctattccaaatatttactgagtgtctactttgtgctagatactgctccaggcccctgcccgggcgcgggctgctgaagccggcgacagaagaaccagccgaactaggaagcgccgcgaag

SEQ ID NO: 11629 - RNA, 3062 nt, Homo sapiens
  source 1..3062: mol_type = other RNA
ctgaatagctgggactacaggtgtccaccaccacgctcgtctaatttttgtatttttagtagagacggggtttcaccatgttggccaggccggtcttgaactcttgacctcaggtgatctgcctgcctcggcctcccaaagtgctgggatttacaggtatgagccaccacatccagccaatgtgacccattatctcacagttctatatattagaagtccagcacagaacagatagattctcatactgaggatcatgcaaagctgaaatccaggtgtcagcccaggctgtggttatcatctgaagcttggagtactcttctaagctgactcagatttttggcagaattcagttccttgtggttgcaactgaggtcccaatttttttttcctgcttgctgacaactggaaggtaggtctcatctcctagaggccacctttaggttttagccaatgtggccctctcacatacttcttcaaggcttacaaggagaattcttcttgcaagggttcacttgattaggtcaggccctttcaacagtctcaaagtgagttgtttaggaaccttaactgcatctgccaaattccttcaactttgtcatgtaacataatctaataatggacatatcattatggcagtatcatcaagggatattttatttgtggttaaatgattgctgtgaacacaatctataaatatatgactaataggattttgtaactggctctataaactttaaattttgtatcattttacaatttacaaagtgcttgtatatattttgcatcatttgattttcatgactacctgtcagagaagcacagcagatattagcccaatgttattagtggctcacagcagctaagtgtatgtccaaagctttacagcaaattagtagtggagtcagctgggcttcagatcagagtgtttccaccctacatacagcccaggctctttttgctaaccctgtaattttcaaactgtgtttggtgatgcttgaaggagatttctcagggattactgtaagaactgggggtgatactaatgggtagggctaagtgttgatatggtggctctatttttatattttggaagttcaacccatgctttaataaccactgtcctgcaacagcctatgccttgttaaaggtaaagaagaatatttaggaaaaaaatcagttaaaaaaatggttgagataggtgtatataaaaagtcaagagtcttttccaataaagttttaagaagctgtcatctcttgcagcagctgttgaaccttcttaatgtctggtctcttatttttcttttcatgcagacattgactagcaacagagtacatagcttcaactgaagtggaatcagcatcattcatctttttatcaatataatcttcaattgtcttttcttcatcttcaatttcttctttaatatctagcaataactgaggttcacggtgttcatccacagctggaagtccagttattatttctagtaaaaccacaccaaagctgtaaatatcagatttgggtgttatttctccacgcaaagcttctggtgccatataagctgttgttcccacaattctgctagtcatgactgtctgggcaaacttctcagaagcccgtgcaaggccaaagtcagatattttagcagtaaaagcttcatccagtaagatatttgcacttttaatatctctatgaatatgatgattttcatgtagaaaattgatgccattagctgcaccctgagcaatcttgcatctcatgtgccaagaaagtggtggagtaccatccaagcaagagagtctgtctagcaatgaaccattaggcatgtaaacatatactaagcagaggtcatctccatcacttgagaaaccaagtagttctactaagttttcatgttgacactttgccattacttttatttcttgatcaaactgctgtttcagttcttcagtagtaatgtcaaccattgctgcaagcttcttcactgccacagttgtgttatttacgtagcctttatatacaactccaaatcctccctctcccattttattaccaccaacagaaatgggtcgttcatcaaagttatttgtgacattcttcaattcataaaatgaaaaactgtgaaaacgtgtatcactaacttctaaacttttattttctggacttgaggagtcaggtggcatatagctttgttcaagattctgcacaggtgtcatcaatgtcctgtctttgtcacagaaaggcatctgtttttgctgaactgttatagcttctttagaaggtagtgtattagcagttttgggaacagcatctgggagcaaaagactcgcaggagcaaaaaattcattttggatcaaaagatccacaagatcaccaactgtgcaatttgtggtgccccagtcaaacagtaattcagaagtgggactttttccagtttgaagtaatgcttcaaatctccttatgtgaaactgattgtatctatcatcaccagatggttttttaatagctacagctaacttcttccatccttcttgaggatcaataaaatctgacagcttcctaattagtccaacattgaggcagcgcacatatgttgatggtgttatgggtttgttcatcttctattccaaatatttactgagtgtctactttgtgctagatactgctccaggcccctggacagggtttgcttttatccctttgtctccctctggcttccaagctgacaggtacacttttttcccccatctgcgaatgtactcatctgatcccataagccgcctccactttctaattccctggaagcttggaggccggagaaacaagcgaattacaatcgtgtggaggctcagcgagctgctggcgccacaggcatctgtcaggtgctggcctgacttcctggttctggggaaaagagacttcatttcgcagtcgggttcacggaatccagggcctgagaggtgagaaacttgaggtccgactgcgccccagaacagctgggtgacgtccctccaagcctcaggctcttcctcagggccgacgaacttcttgattaccgggg

SEQ ID NO: 11630 - RNA, 2770 nt, Homo sapiens
  source 1..2770: mol_type = other RNA
ctgaatagctgggactacaggtgtccaccaccacgctcgtctaatttttgtatttttagtagagacggggtttcaccatgttggccaggccggtcttgaactcttgacctcaggtgatctgcctgcctcggcctcccaaagtgctgggatttacaggtatgagccaccacatccagccaatgtgacccattatctcacagttctatatattagaagtccagcacagaacagatagattctcatactgaggatcatgcaaagctgaaatccaggtgtcagcccaggctgtggttatcatctgaagcttggagtactcttctaagctgactcagatttttggcagaattcagttccttgtggttgcaactgaggtcccaatttttttttcctgcttgctgacaactggaaggtaggtctcatctcctagaggccacctttaggttttagccaatgtggccctctcacatacttcttcaaggcttacaaggagaattcttcttgcaagggttcacttgattaggtcaggccctttcaacagtctcaaagtgagttgtttaggaaccttaactgcatctgccaaattccttcaactttgtcatgtaacataatctaataatggacatatcattatggcagtatcatcaagggatattttatttgtggttaaatgattgctgtgaacacaatctataaatatatgactaataggattttgtaactggctctataaactttaaattttgtatcattttacaatttacaaagtgcttgtatatattttgcatcatttgattttcatgactacctgtcagagaagcacagcagatattagcccaatgttattagtggctcacagcagctaagtgtatgtccaaagctttacagcaaattagtagtggagtcagctgggcttcagatcagagtgtttccaccctacatacagcccaggctctttttgctaaccctgtaattttcaaactgtgtttggtgatgcttgaaggagatttctcagggattactgtaagaactgggggtgatactaatgggtagggctaagtgttgatatggtggctctatttttatattttggaagttcaacccatgctttaataaccactgtcctgcaacagcctatgccttgttaaaggtaaagaagaatatttaggaaaaaaatcagttaaaaaaatggttgagataggtgtatataaaaagtcaagagtcttttccaataaagttttaagaagctgtcatctcttgcagcagctgttgaaccttcttaatgtctggtctcttatttttcttttcatgcagacattgactagcaacagagtacatagcttcaactgaagtggaatcagcatcattcatctttttatcaatataatcttcaattgtcttttcttcatcttcaatttcttctttaatatctagcaataactgaggttcacggtgttcatccacagctggaagtccagttattatttctagtaaaaccacaccaaagctgtaaatatcagatttgggtgttatttctccacgcaaagcttctggtgccatataagctgttgttcccacaattctgctagtcatgactgtctgggcaaacttctcagaagcccgtgcaaggccaaagtcagatattttagcagtaaaagcttcatccagtaagatatttgcacttttaatatctctatgaatatgatgattttcatgtagaaaattgatgccattagctgcaccctgagcaatcttgcatctcatgtgccaagaaagtggtggagtaccatccaagcaagagagtctgtctagcaatgaaccattaggcatgtaaacatatactaagcagaggtcatctccatcacttgagaaaccaagtagttctactaagttttcatgttgacactttgccattacttttatttcttgatcaaactgctgtttcagttcttcagtagtaatgtcaaccattgctgcaagcttcttcactgccacagttgtgttatttacgtagcctttatatacaactccaaatcctccctctcccattttattaccaccaacagaaatgggtcgttcatcaaagttatttgtgacattcttcaattcataaaatgaaaaactgtgaaaacgtgtatcactaacttctaaacttttattttctggacttgaggagtcaggtggcatatagctttgttcaagattctgcacaggtgtcatcaatgtcctgtctttgtcacagaaaggcatctgtttttgctgaactgttatagcttctttagaaggtagtgtattagcagttttgggaacagcatctgggagcaaaagactcgcaggagcaaaaaattcattttggatcaaaagatccacaagatcaccaactgtgcaatttgtggtgccccagtcaaacagtaattcagaagtgggactttttccagtttgaagtaatgcttcaaatctccttatgtgaaactgattgtatctatcatcaccagatggttttttaatagctacagctaacttcttccatccttcttgaggatcaataaaatctgacagcttcctaattagtccaacattgaggcagcgcacatatgttgatggtgttatgggtttgttcatcttctattccaggggccttgggcagttacgtttttgaagcactaatagcgccgtttgttcccattctaaatgctcaaagtgctttctcgctttctcagggtttgcttttttttttttttttttcttttgagacggagtctccctctgttgc

SEQ ID NO: 11631 - RNA, 2806 nt, Homo sapiens
  source 1..2806: mol_type = other RNA
ctgaatagctgggactacaggtgtccaccaccacgctcgtctaatttttgtatttttagtagagacggggtttcaccatgttggccaggccggtcttgaactcttgacctcaggtgatctgcctgcctcggcctcccaaagtgctgggatttacaggtatgagccaccacatccagccaatgtgacccattatctcacagttctatatattagaagtccagcacagaacagatagattctcatactgaggatcatgcaaagctgaaatccaggtgtcagcccaggctgtggttatcatctgaagcttggagtactcttctaagctgactcagatttttggcagaattcagttccttgtggttgcaactgaggtcccaatttttttttcctgcttgctgacaactggaaggtaggtctcatctcctagaggccacctttaggttttagccaatgtggccctctcacatacttcttcaaggcttacaaggagaattcttcttgcaagggttcacttgattaggtcaggccctttcaacagtctcaaagtgagttgtttaggaaccttaactgcatctgccaaattccttcaactttgtcatgtaacataatctaataatggacatatcattatggcagtatcatcaagggatattttatttgtggttaaatgattgctgtgaacacaatctataaatatatgactaataggattttgtaactggctctataaactttaaattttgtatcattttacaatttacaaagtgcttgtatatattttgcatcatttgattttcatgactacctgtcagagaagcacagcagatattagcccaatgttattagtggctcacagcagctaagtgtatgtccaaagctttacagcaaattagtagtggagtcagctgggcttcagatcagagtgtttccaccctacatacagcccaggctctttttgctaaccctgtaattttcaaactgtgtttggtgatgcttgaaggagatttctcagggattactgtaagaactgggggtgatactaatgggtagggctaagtgttgatatggtggctctatttttatattttggaagttcaacccatgctttaataaccactgtcctgcaacagcctatgccttgttaaaggtaaagaagaatatttaggaaaaaaatcagttaaaaaaatggttgagataggtgtatataaaaagtcaagagtcttttccaataaagttttaagaagctgtcatctcttgcagcagctgttgaaccttcttaatgtctggtctcttatttttcttttcatgcagacattgactagcaacagagtacatagcttcaactgaagtggaatcagcatcattcatctttttatcaatataatcttcaattgtcttttcttcatcttcaatttcttctttaatatctagcaataactgaggttcacggtgttcatccacagctggaagtccagttattatttctagtaaaaccacaccaaagctgtaaatatcagatttgggtgttatttctccacgcaaagcttctggtgccatataagctgttgttcccacaattctgctagtcatgactgtctgggcaaacttctcagaagcccgtgcaaggccaaagtcagatattttagcagtaaaagcttcatccagtaagatatttgcacttttaatatctctatgaatatgatgattttcatgtagaaaattgatgccattagctgcaccctgagcaatcttgcatctcatgtgccaagaaagtggtggagtaccatccaagcaagagagtctgtctagcaatgaaccattaggcatgtaaacatatactaagcagaggtcatctccatcacttgagaaaccaagtagttctactaagttttcatgttgacactttgccattacttttatttcttgatcaaactgctgtttcagttcttcagtagtaatgtcaaccattgctgcaagcttcttcactgccacagttgtgttatttacgtagcctttatatacaactccaaatcctccctctcccattttattaccaccaacagaaatgggtcgttcatcaaagttatttgtgacattcttcaattcataaaatgaaaaactgtgaaaacgtgtatcactaacttctaaacttttattttctggacttgaggagtcaggtggcatatagctttgttcaagattctgcacaggtgtcatcaatgtcctgtctttgtcacagaaaggcatctgtttttgctgaactgttatagcttctttagaaggtagtgtattagcagttttgggaacagcatctgggagcaaaagactcgcaggagcaaaaaattcattttggatcaaaagatccacaagatcaccaactgtgcaatttgtggtgccccagtcaaacagtaattcagaagtgggactttttccagtttgaagtaatgcttcaaatctccttatgtgaaactgattgtatctatcatcaccagatggttttttaatagctacagctaacttcttccatccttcttgaggatcaataaaatctgacagcttcctaattagtccaacattgaggcagcgcacatatgttgatggtgttatgggtttgttcatcttctattcccaagtctttcttctggagtaagctctgtcaaaggaacccacttcctctctaacttttctcacggatgataaagagatttccgttccgcagccgaccccagcaaccctggggcagaggtgccgaggcctggaagcggacctcggacgacgtttgaccgaggcattaaggcggggaatg

SEQ ID NO: 11632 - RNA, 2694 nt, Homo sapiens
  source 1..2694: mol_type = other RNA
ctgaatagctgggactacaggtgtccaccaccacgctcgtctaatttttgtatttttagtagagacggggtttcaccatgttggccaggccggtcttgaactcttgacctcaggtgatctgcctgcctcggcctcccaaagtgctgggatttacaggtatgagccaccacatccagccaatgtgacccattatctcacagttctatatattagaagtccagcacagaacagatagattctcatactgaggatcatgcaaagctgaaatccaggtgtcagcccaggctgtggttatcatctgaagcttggagtactcttctaagctgactcagatttttggcagaattcagttccttgtggttgcaactgaggtcccaatttttttttcctgcttgctgacaactggaaggtaggtctcatctcctagaggccacctttaggttttagccaatgtggccctctcacatacttcttcaaggcttacaaggagaattcttcttgcaagggttcacttgattaggtcaggccctttcaacagtctcaaagtgagttgtttaggaaccttaactgcatctgccaaattccttcaactttgtcatgtaacataatctaataatggacatatcattatggcagtatcatcaagggatattttatttgtggttaaatgattgctgtgaacacaatctataaatatatgactaataggattttgtaactggctctataaactttaaattttgtatcattttacaatttacaaagtgcttgtatatattttgcatcatttgattttcatgactacctgtcagagaagcacagcagatattagcccaatgttattagtggctcacagcagctaagtgtatgtccaaagctttacagcaaattagtagtggagtcagctgggcttcagatcagagtgtttccaccctacatacagcccaggctctttttgctaaccctgtaattttcaaactgtgtttggtgatgcttgaaggagatttctcagggattactgtaagaactgggggtgatactaatgggtagggctaagtgttgatatggtggctctatttttatattttggaagttcaacccatgctttaataaccactgtcctgcaacagcctatgccttgttaaaggtaaagaagaatatttaggaaaaaaatcagttaaaaaaatggttgagataggtgtatataaaaagtcaagagtcttttccaataaagttttaagaagctgtcatctcttgcagcagctgttgaaccttcttaatgtctggtctcttatttttcttttcatgcagacattgactagcaacagagtacatagcttcaactgaagtggaatcagcatcattcatctttttatcaatataatcttcaattgtcttttcttcatcttcaatttcttctttaatatctagcaataactgaggttcacggtgttcatccacagctggaagtccagttattatttctagtaaaaccacaccaaagctgtaaatatcagatttgggtgttatttctccacgcaaagcttctggtgccatataagctgttgttcccacaattctgctagtcatgactgtctgggcaaacttctcagaagcccgtgcaaggccaaagtcagatattttagcagtaaaagcttcatccagtaagatatttgcacttttaatatctctatgaatatgatgattttcatgtagaaaattgatgccattagctgcaccctgagcaatcttgcatctcatgtgccaagaaagtggtggagtaccatccaagcaagagagtctgtctagcaatgaaccattaggcatgtaaacatatactaagcagaggtcatctccatcacttgagaaaccaagtagttctactaagttttcatgttgacactttgccattacttttatttcttgatcaaactgctgtttcagttcttcagtagtaatgtcaaccattgctgcaagcttcttcactgccacagttgtgttatttacgtagcctttatatacaactccaaatcctccctctcccattttattaccaccaacagaaatgggtcgttcatcaaagttatttgtgacattcttcaattcataaaatgaaaaactgtgaaaacgtgtatcactaacttctaaacttttattttctggacttgaggagtcaggtggcatatagctttgttcaagattctgcacaggtgtcatcaatgtcctgtctttgtcacagaaaggcatctgtttttgctgaactgttatagcttctttagaaggtagtgtattagcagttttgggaacagcatctgggagcaaaagactcgcaggagcaaaaaattcattttggatcaaaagatccacaagatcaccaactgtgcaatttgtggtgccccagtcaaacagtaattcagaagtgggactttttccagtttgaagtaatgcttcaaatctccttatgtgaaactgattgtatctatcatcaccagatggttttttaatagctacagctaacttcttccatccttcttgaggatcaataaaatctgacagcttcctaattagtccaacattgaggcagcgcacatatgttgatggtgttatgggtttgttcatcttctattcctgcccgggcgcgggctgctgaagccggcgacagaagaaccagccgaactaggaagcgccgcgaag

SEQ ID NO: 11633 - RNA, 3433 nt, Homo sapiens
  source 1..3433: mol_type = other RNA
ctgaatagctgggactacaggtgtccaccaccacgctcgtctaatttttgtatttttagtagagacggggtttcaccatgttggccaggccggtcttgaactcttgacctcaggtgatctgcctgcctcggcctcccaaagtgctgggatttacaggtatgagccaccacatccagccaatgtgacccattatctcacagttctatatattagaagtccagcacagaacagatagattctcatactgaggatcatgcaaagctgaaatccaggtgtcagcccaggctgtggttatcatctgaagcttggagtactcttctaagctgactcagatttttggcagaattcagttccttgtggttgcaactgaggtcccaatttttttttcctgcttgctgacaactggaaggtaggtctcatctcctagaggccacctttaggttttagccaatgtggccctctcacatacttcttcaaggcttacaaggagaattcttcttgcaagggttcacttgattaggtcaggccctttcaacagtctcaaagtgagttgtttaggaaccttaactgcatctgccaaattccttcaactttgtcatgtaacataatctaataatggacatatcattatggcagtatcatcaagggatattttatttgtggttaaatgattgctgtgaacacaatctataaatatatgactaataggattttgtaactggctctataaactttaaattttgtatcattttacaatttacaaagtgcttgtatatattttgcatcatttgattttcatgactacctgtcagagaagcacagcagatattagcccaatgttattagtggctcacagcagctaagtgtatgtccaaagctttacagcaaattagtagtggagtcagctgggcttcagatcagagtgtttccaccctacatacagcccaggctctttttgctaaccctgtaattttcaaactgtgtttggtgatgcttgaaggagatttctcagggattactgtaagaactgggggtgatactaatgggtagggctaagtgttgatatggtggctctatttttatattttggaagttcaacccatgctttaataaccactgtcctgcaacagcctatgccttgttaaaggtaaagaagaatatttaggaaaaaaatcagttaaaaaaatggttgagataggtgtatataaaaagtcaagagtcttttccaataaagttttaagaagctgtcatctcttgcagcagctgttgaaccttcttaatgtctggtctcttatttttcttttcatgcagacattgactagcaacagagtacatagcttcaactgaagtggaatcagcatcattcatctttttatcaatataatcttcaattgtcttttcttcatcttcaatttcttctttaatatctagcaataactgaggttcacggtgttcatccacagctggaagtccagttattatttctagtaaaaccacaccaaagctgtaaatatcagatttgggtgttatttctccacgcaaagcttctggtgccatataagctgttgttcccacaattctgctagtcatgactgtctgggcaaacttctcagaagcccgtgcaaggccaaagtcagatattttagcagtaaaagcttcatccagtaagatatttgcacttttaatatctctatgaatatgatgattttcatgtagaaaattgatgccattagctgcaccctgagcaatcttgcatctcatgtgccaagaaagtggtggagtaccatccaagcaagagagtctgtctagcaatgaaccattaggcatgtaaacatatactaagcagaggtcatctccatcacttgagaaaccaagtagttctactaagttttcatgttgacactttgccattacttttatttcttgatcaaactgctgtttcagttcttcagtagtaatgtcaaccattgctgcaagcttcttcactgccacagttgtgttatttacgtagcctttatatacaactccaaatcctccctctcccattttattaccaccaacagaaatgggtcgttcatcaaagttatttgtgacattcttcaattcataaaatgaaaaactgtgaaaacgtgtatcactaacttctaaacttttattttctggacttgaggagtcaggtggcatatagctttgttcaagattctgcacaggtgtcatcaatgtcctgtctttgtcacagaaaggcatctgtttttgctgaactgttatagcttctttagaaggtagtgtattagcagttttgggaacagcatctgggagcaaaagactcgcaggagcaaaaaattcattttggatcaaaagatccacaagatcaccaactgtgcaatttgtggtgccccagtcaaacagtaattcagaagtgggactttttccagtttgaagtaatgcttcaaatctccttatgtgaaactgattgtatctatcatcaccagatggttttttaatagctacagctaacttcttccatccttcttgaggatcaataaaatctgacagcttcctaattagtccaacattgaggcagcgcacatatgttgatggtgttatgggtttgttcatcttctattcctgcttatggaatccaatgccttcccaaagtactgtgcccaaaacaggagggcaaaagattcttgtcaaatgtgttaataaagttttaagactgcttcattagcactttgatcagaggaaaagattgtgcaggggtggagggaagatgaactttgaggttgcacaggcctaagttctaaccaaagccaactgtgaccagagctagtaaatacatttctctgcaccttgcttttctttatctgaaaaacagagatagtaatacctaagaattgctgtaagaattaaaatcaacacatgcaaagggccaaatcttgtcacataataataggtggtcaaaaaaaaaaaggagcaattattatttcctggcagaaattattcttatatcacattatttttaaagatatgtgcagactgtatttaggttcaatttccagaacagtagtgaggatctactgaaagcgtacaaataacaagtctgagaaaatagctaagcttttgagatggtggctgtcttatttgatcaaccatggtaattttaatgtatttatatcctttctaaaatacactatttacttccatatattcttagcaaaatatgctgtataaccattaatctttatttttagatactttaacatcatcattatgaacaaaagctggtgagggcttccagagctattaaattagatagggctgcctattacaaactgggatatgtgctggtgtaccataaattaaacttaacatatctttcttgaacattgatccaacacaacagtaagtaattgaaaatgctttgcatata

SEQ ID NO: 11634 - RNA, 3014 nt, Homo sapiens
  source 1..3014: mol_type = other RNA
ctgaatagctgggactacaggtgtccaccaccacgctcgtctaatttttgtatttttagtagagacggggtttcaccatgttggccaggccggtcttgaactcttgacctcaggtgatctgcctgcctcggcctcccaaagtgctgggatttacaggtatgagccaccacatccagccaatgtgacccattatctcacagttctatatattagaagtccagcacagaacagatagattctcatactgaggatcatgcaaagctgaaatccaggtgtcagcccaggctgtggttatcatctgaagcttggagtactcttctaagctgactcagatttttggcagaattcagttccttgtggttgcaactgaggtcccaatttttttttcctgcttgctgacaactggaaggtaggtctcatctcctagaggccacctttaggttttagccaatgtggccctctcacatacttcttcaaggcttacaaggagaattcttcttgcaagggttcacttgattaggtcaggccctttcaacagtctcaaagtgagttgtttaggaaccttaactgcatctgccaaattccttcaactttgtcatgtaacataatctaataatggacatatcattatggcagtatcatcaagggatattttatttgtggttaaatgattgctgtgaacacaatctataaatatatgactaataggattttgtaactggctctataaactttaaattttgtatcattttacaatttacaaagtgcttgtatatattttgcatcatttgattttcatgactacctgtcagagaagcacagcagatattagcccaatgttattagtggctcacagcagctaagtgtatgtccaaagctttacagcaaattagtagtggagtcagctgggcttcagatcagagtgtttccaccctacatacagcccaggctctttttgctaaccctgtaattttcaaactgtgtttggtgatgcttgaaggagatttctcagggattactgtaagaactgggggtgatactaatgggtagggctaagtgttgatatggtggctctatttttatattttggaagttcaacccatgctttaataaccactgtcctgcaacagcctatgccttgttaaaggtaaagaagaatatttaggaaaaaaatcagttaaaaaaatggttgagataggtgtatataaaaagtcaagagtcttttccaataaagttttaagaagctgtcatctcttgcagcagctgttgaaccttcttaatgtctggtctcttatttttcttttcatgcagacattgactagcaacagagtacatagcttcaactgaagtggaatcagcatcattcatctttttatcaatataatcttcaattgtcttttcttcatcttcaatttcttctttaatatctagcaataactgaggttcacggtgttcatccacagctggaagtccagttattatttctagtaaaaccacaccaaagctgtaaatatcagatttgggtgttatttctccacgcaaagcttctggtgccatataagctgttgttcccacaattctgctagtcatgactgtctgggcaaacttctcagaagcccgtgcaaggccaaagtcagatattttagcagtaaaagcttcatccagtaagatatttgcacttttaatatctctatgaatatgatgattttcatgtagaaaattgatgccattagctgcaccctgagcaatcttgcatctcatgtgccaagaaagtggtggagtaccatccaagcaagagagtctgtctagcaatgaaccattaggcatgtaaacatatactaagcagaggtcatctccatcacttgagaaaccaagtagttctactaagttttcatgttgacactttgccattacttttatttcttgatcaaactgctgtttcagttcttcagtagtaatgtcaaccattgctgcaagcttcttcactgccacagttgtgttatttacgtagcctttatatacaactccaaatcctccctctcccattttattaccaccaacagaaatgggtcgttcatcaaagttatttgtgacattcttcaattcataaaatgaaaaactgtgaaaacgtgtatcactaacttctaaacttttattttctggacttgaggagtcaggtggcatatagctttgttcaagattctgcacaggtgtcatcaatgtcctgtctttgtcacagaaaggcatctgtttttgctgaactgttatagcttctttagaaggtagtgtattagcagttttgggaacagcatctgggagcaaaagactcgcaggagcaaaaaattcattttggatcaaaagatccacaagatcaccaactgtgcaatttgtggtgccccagtcaaacagtaattcagaagtgggactttttccagtttgaagtaatgcttcaaatctccttatgtgaaactgattgtatctatcatcaccagatggttttttaatagctacagctaacttcttccatccttcttgaggatcaataaaatctgacagcttcctaattagtccaacattgaggcagcgcacatatgttgatggtgttatgggtttgttcatcttctattcctggacagggtttgcttttatccctttgtctccctctggcttccaagctgacaggtacacttttttcccccatctgcgaatgtactcatctgatcccataagccgcctccactttctaattccctggaagcttggaggccggagaaacaagcgaattacaatcgtgtggaggctcagcgagctgctggcgccacaggcatctgtcaggtgctggcctgacttcctggttctggggaaaagagacttcatttcgcagtcgggttcacggaatccagggcctgagaggtgagaaacttgaggtccgactgcgccccagaacagctgggtgacgtccctccaagcctcaggctcttcctcagggccgacgaacttcttgattaccgggg

SEQ ID NO: 11635 - RNA, 2939 nt, Homo sapiens
  source 1..2939: mol_type = other RNA
ctgaatagctgggactacaggtgtccaccaccacgctcgtctaatttttgtatttttagtagagacggggtttcaccatgttggccaggccggtcttgaactcttgacctcaggtgatctgcctgcctcggcctcccaaagtgctgggatttacaggtatgagccaccacatccagccaatgtgacccattatctcacagttctatatattagaagtccagcacagaacagatagattctcatactgaggatcatgcaaagctgaaatccaggtgtcagcccaggctgtggttatcatctgaagcttggagtactcttctaagctgactcagatttttggcagaattcagttccttgtggttgcaactgaggtcccaatttttttttcctgcttgctgacaactggaaggtaggtctcatctcctagaggccacctttaggttttagccaatgtggccctctcacatacttcttcaaggcttacaaggagaattcttcttgcaagggttcacttgattaggtcaggccctttcaacagtctcaaagtgagttgtttaggaaccttaactgcatctgccaaattccttcaactttgtcatgtaacataatctaataatggacatatcattatggcagtatcatcaagggatattttatttgtggttaaatgattgctgtgaacacaatctataaatatatgactaataggattttgtaactggctctataaactttaaattttgtatcattttacaatttacaaagtgcttgtatatattttgcatcatttgattttcatgactacctgtcagagaagcacagcagatattagcccaatgttattagtggctcacagcagctaagtgtatgtccaaagctttacagcaaattagtagtggagtcagctgggcttcagatcagagtgtttccaccctacatacagcccaggctctttttgctaaccctgtaattttcaaactgtgtttggtgatgcttgaaggagatttctcagggattactgtaagaactgggggtgatactaatgggtagggctaagtgttgatatggtggctctatttttatattttggaagttcaacccatgctttaataaccactgtcctgcaacagcctatgccttgttaaaggtaaagaagaatatttaggaaaaaaatcagttaaaaaaatggttgagataggtgtatataaaaagtcaagagtcttttccaataaagttttaagaagctgtcatctcttgcagcagctgttgaaccttcttaatgtctggtctcttatttttcttttcatgcagacattgactagcaacagagtacatagcttcaactgaagtggaatcagcatcattcatctttttatcaatataatcttcaattgtcttttcttcatcttcaatttcttctttaatatctagcaataactgaggttcacggtgttcatccacagctggaagtccagttattatttctagtaaaaccacaccaaagctgtaaatatcagatttgggtgttatttctccacgcaaagcttctggtgccatataagctgttgttcccacaattctgctagtcatgactgtctgggcaaacttctcagaagcccgtgcaaggccaaagtcagatattttagcagtaaaagcttcatccagtaagatatttgcacttttaatatctctatgaatatgatgattttcatgtagaaaattgatgccattagctgcaccctgagcaatcttgcatctcatgtgccaagaaagtggtggagtaccatccaagcaagagagtctgtctagcaatgaaccattaggcatgtaaacatatactaagcagaggtcatctccatcacttgagaaaccaagtagttctactaagttttcatgttgacactttgccattacttttatttcttgatcaaactgctgtttcagttcttcagtagtaatgtcaaccattgctgcaagcttcttcactgccacagttgtgttatttacgtagcctttatatacaactccaaatcctccctctcccattttattaccaccaacagaaatgggtcgttcatcaaagttatttgtgacattcttcaattcataaaatgaaaaactgtgaaaacgtgtatcactaacttctaaacttttattttctggacttgaggagtcaggtggcatatagctttgttcaagattctgcacaggtgtcatcaatgtcctgtctttgtcacagaaaggcatctgtttttgctgaactgttatagcttctttagaaggtagtgtattagcagttttgggaacagcatctgggagcaaaagactcgcaggagcaaaaaattcattttggatcaaaagatccacaagatcaccaactgtgcaatttgtggtgccccagtcaaacagtaattcagaagtgggactttttccagtttgaagtaatgcttcaaatctccttatgtgaaactgattgtatctatcatcaccagatggttttttaatagctacagctaacttcttccatccttcttgaggatcaataaaatctgacagcttcctaattagtccaacattgaggcagcgcacatatgttgatggtgttatgggtttgttcatcttctattccttttcctcaaaaacagaagaacaacattgttttaaagttttgctaatctcttcaatatttaacttaatagaagagagctgaattcttgtatctgcttctgcactcaacccactgcagcatgttgttttggttgatgtatatgaagaaaatccagcaaatatttactgagtgtctactttgtgctagatactgctccaggcccctgcccgggcgcgggctgctgaagccggcgacagaagaaccagccgaactaggaagcgccgcgaaggggcggggcctgccgggttggccccgccccacttccccgatg

SEQ ID NO: 11636 - RNA, 2591 nt, Homo sapiens
  source 1..2591: mol_type = other RNA
ctgaatagctgggactacaggtgtccaccaccacgctcgtctaatttttgtatttttagtagagacggggtttcaccatgttggccaggccggtcttgaactcttgacctcaggtgatctgcctgcctcggcctcccaaagtgctgggatttacaggtatgagccaccacatccagccaatgtgacccattatctcacagttctatatattagaagtccagcacagaacagatagattctcatactgaggatcatgcaaagctgaaatccaggtgtcagcccaggctgtggttatcatctgaagcttggagtactcttctaagctgactcagatttttggcagaattcagttccttgtggttgcaactgaggtcccaatttttttttcctgcttgctgacaactggaaggtaggtctcatctcctagaggccacctttaggttttagccaatgtggccctctcacatacttcttcaaggcttacaaggagaattcttcttgcaagggttcacttgattaggtcaggccctttcaacagtctcaaagtgagttgtttaggaaccttaactgcatctgccaaattccttcaactttgtcatgtaacataatctaataatggacatatcattatggcagtatcatcaagggatattttatttgtggttaaatgattgctgtgaacacaatctataaatatatgactaataggattttgtaactggctctataaactttaaattttgtatcattttacaatttacaaagtgcttgtatatattttgcatcatttgattttcatgactacctgtcagagaagcacagcagatattagcccaatgttattagtggctcacagcagctaagtgtatgtccaaagctttacagcaaattagtagtggagtcagctgggcttcagatcagagtgtttccaccctacatacagcccaggctctttttgctaaccctgtaattttcaaactgtgtttggtgatgcttgaaggagatttctcagggattactgtaagaactgggggtgatactaatgggtagggctaagtgttgatatggtggctctatttttatattttggaagttcaacccatgctttaataaccactgtcctgcaacagcctatgccttgttaaaggtaaagaagaatatttaggaaaaaaatcagttaaaaaaatggttgagataggtgtatataaaaagtcaagagtcttttccaataaagttttaagaagctgtcatctcttgcagcagctgttgaaccttcttaatgtctggtctcttatttttcttttcatgcagacattgactagcaacagagtacatagcttcaactgaagtggaatcagcatcattcatctttttatcaatataatcttcaattgtcttttcttcatcttcaatttcttctttaatatctagcaataactgaggttcacggtgttcatccacagctggaagtccagttattatttctagtaaaaccacaccaaagctgtaaatatcagatttgggtgttatttctccacgcaaagcttctggtgccatataagctgttgttcccacaattctgctagtcatgactgtctgggcaaacttctcagaagcccgtgcaaggccaaagtcagatattttagcagtaaaagcttcatccagtaagatatttgcacttttaatatctctatgaatatgatgattttcatgtagaaaattgatgccattagctgcaccctgagcaatcttgcatctcatgtgccaagaaagtggtggagtaccatccaagcaagagagtctgtctagcaatgaaccattaggcatgtaaacatatactaagcagaggtcatctccatcacttgagaaaccaagtagttctactaagttttcatgttgacactttgccattacttttatttcttgatcaaactgctgtttcagttcttcagtagtaatgtcaaccattgctgcaagcttcttcactgccacagttgtgttatttacgtagcctttatatacaactccaaatcctccctctcccattttattaccaccaacagaaatgggtcgttcatcaaagttatttgtgacattcttcaattcataaaatgaaaaactgtgaaaacgtgtatcactaacttctaaacttttattttctggacttgaggagtcaggtggcatatagctttgttcaagattctgcacaggtgtcatcaatgtcctgtctttgtcacagaaaggcatctgtttttgctgaactgttatagcttctttagaaggtagtgtattagcagttttgggaacagcatctgggagcaaaagactcgcaggagcaaaaaattcattttggatcaaaagatccacaagatcaccaactgtgcaatttgtggtgccccagtcaaacagtaattcagaagtgggactttttccagtttgaagtaatgcttcaaatctcggttctggaggctgggaagtccaagatcgagaggctgcatctggttagggccttcttgctacatcatctgcccgggcgcgggctgctgaagccggcgacagaagaaccagccgaactaggaagcgccgcgaag

SEQ ID NO: 11637 - RNA, 2809 nt, Homo sapiens
  source 1..2809: mol_type = other RNA
ctgaatagctgggactacaggtgtccaccaccacgctcgtctaatttttgtatttttagtagagacggggtttcaccatgttggccaggccggtcttgaactcttgacctcaggtgatctgcctgcctcggcctcccaaagtgctgggatttacaggtatgagccaccacatccagccaatgtgacccattatctcacagttctatatattagaagtccagcacagaacagatagattctcatactgaggatcatgcaaagctgaaatccaggtgtcagcccaggctgtggttatcatctgaagcttggagtactcttctaagctgactcagatttttggcagaattcagttccttgtggttgcaactgaggtcccaatttttttttcctgcttgctgacaactggaaggtaggtctcatctcctagaggccacctttaggttttagccaatgtggccctctcacatacttcttcaaggcttacaaggagaattcttcttgcaagggttcacttgattaggtcaggccctttcaacagtctcaaagtgagttgtttaggaaccttaactgcatctgccaaattccttcaactttgtcatgtaacataatctaataatggacatatcattatggcagtatcatcaagggatattttatttgtggttaaatgattgctgtgaacacaatctataaatatatgactaataggattttgtaactggctctataaactttaaattttgtatcattttacaatttacaaagtgcttgtatatattttgcatcatttgattttcatgactacctgtcagagaagcacagcagatattagcccaatgttattagtggctcacagcagctaagtgtatgtccaaagctttacagcaaattagtagtggagtcagctgggcttcagatcagagtgtttccaccctacatacagcccaggctctttttgctaaccctgtaattttcaaactgtgtttggtgatgcttgaaggagatttctcagggattactgtaagaactgggggtgatactaatgggtagggctaagtgttgatatggtggctctatttttatattttggaagttcaacccatgctttaataaccactgtcctgcaacagcctatgccttgttaaaggtaaagaagaatatttaggaaaaaaatcagttaaaaaaatggttgagataggtgtatataaaaagtcaagagtcttttccaataaagttttaagaagctgtcatctcttgcagcagctgttgaaccttcttaatgtctggtctcttatttttcttttcatgcagacattgactagcaacagagtacatagcttcaactgaagtggaatcagcatcattcatctttttatcaatataatcttcaattgtcttttcttcatcttcaatttcttctttaatatctagcaataactgaggttcacggtgttcatccacagctggaagtccagttattatttctagtaaaaccacaccaaagctgtaaatatcagatttgggtgttatttctccacgcaaagcttctggtgccatataagctgttgttcccacaattctgctagtcatgactgtctgggcaaacttctcagaagcccgtgcaaggccaaagtcagatattttagcagtaaaagcttcatccagtaagatatttgcacttttaatatctctatgaatatgatgattttcatgtagaaaattgatgccattagctgcaccctgagcaatcttgcatctcatgtgccaagaaagtggtggagtaccatccaagcaagagagtctgtctagcaatgaaccattaggcatgtaaacatatactaagcagaggtcatctccatcacttgagaaaccaagtagttctactaagttttcatgttgacactttgccattacttttatttcttgatcaaactgctgtttcagttcttcagtagtaatgtcaaccattgctgcaagcttcttcactgccacagttgtgttatttacgtagcctttatatacaactccaaatcctccctctcccattttattaccaccaacagaaatgggtcgttcatcaaagttatttgtgacattcttcaattcataaaatgaaaaactgtgaaaacgtgtatcactaacttctaaacttttattttctggacttgaggagtcaggtggcatatagctttgttcaagattctgcacaggtgtcatcaatgtcctgtctttgtcacagaaaggcatctgtttttgctgaactgttatagcttctttagaaggtagtgtattagcagttttgggaacagcatctgggagcaaaagactcgcaggagcaaaaaattcattttggatcaaaagatccacaagatcaccaactgtgcaatttgtggtgccccagtcaaacagtaattcagaagtgggactttttccagtttgaagtaatgcttcaaatctcggttctggaggctgggaagtccaagatcgagaggctgcatctggttagggccttcttgctacatcatcttatgtgaaactgattgtatctatcatcaccagatggttttttaatagctacagctaacttcttccatccttcttgaggatcaataaaatctgacagcttcctaattagtccaacattgaggcagcgcacatatgttgatggtgttatgggtttgttcatcttctattccaaatatttactgagtgtctactttgtgctagatactgctccaggcccctgcccgggcgcgggctgctgaagccggcgacagaagaaccagccgaactaggaagcgccgcgaag

SEQ ID NO: 11638 - RNA, 2945 nt, Homo sapiens
  source 1..2945: mol_type = other RNA
ctgaatagctgggactacaggtgtccaccaccacgctcgtctaatttttgtatttttagtagagacggggtttcaccatgttggccaggccggtcttgaactcttgacctcaggtgatctgcctgcctcggcctcccaaagtgctgggatttacaggtatgagccaccacatccagccaatgtgacccattatctcacagttctatatattagaagtccagcacagaacagatagattctcatactgaggatcatgcaaagctgaaatccaggtgtcagcccaggctgtggttatcatctgaagcttggagtactcttctaagctgactcagatttttggcagaattcagttccttgtggttgcaactgaggtcccaatttttttttcctgcttgctgacaactggaaggtaggtctcatctcctagaggccacctttaggttttagccaatgtggccctctcacatacttcttcaaggcttacaaggagaattcttcttgcaagggttcacttgattaggtcaggccctttcaacagtctcaaagtgagttgtttaggaaccttaactgcatctgccaaattccttcaactttgtcatgtaacataatctaataatggacatatcattatggcagtatcatcaagggatattttatttgtggttaaatgattgctgtgaacacaatctataaatatatgactaataggattttgtaactggctctataaactttaaattttgtatcattttacaatttacaaagtgcttgtatatattttgcatcatttgattttcatgactacctgtcagagaagcacagcagatattagcccaatgttattagtggctcacagcagctaagtgtatgtccaaagctttacagcaaattagtagtggagtcagctgggcttcagatcagagtgtttccaccctacatacagcccaggctctttttgctaaccctgtaattttcaaactgtgtttggtgatgcttgaaggagatttctcagggattactgtaagaactgggggtgatactaatgggtagggctaagtgttgatatggtggctctatttttatattttggaagttcaacccatgctttaataaccactgtcctgcaacagcctatgccttgttaaaggtaaagaagaatatttaggaaaaaaatcagttaaaaaaatggttgagataggtgtatataaaaagtcaagagtcttttccaataaagttttaagaagctgtcatctcttgcagcagctgttgaaccttcttaatgtctggtctcttatttttcttttcatgcagacattgactagcaacagagtacatagcttcaactgaagtggaatcagcatcattcatctttttatcaatataatcttcaattgtcttttcttcatcttcaatttcttctttaatatctagcaataactgaggttcacggtgttcatccacagctggaagtccagttattatttctagtaaaaccacaccaaagctgtaaatatcagatttgggtgttatttctccacgcaaagcttctggtgccatataagctgttgttcccacaattctgctagtcatgactgtctgggcaaacttctcagaagcccgtgcaaggccaaagtcagatattttagcagtaaaagcttcatccagtaagatatttgcacttttaatatctctatgaatatgatgattttcatgtagaaaattgatgccattagctgcaccctgagcaatcttgcatctcatgtgccaagaaagtggtggagtaccatccaagcaagagagtctgtctagcaatgaaccattaggcatgtaaacatatactaagcagaggtcatctccatcacttgagaaaccaagtagttctactaagttttcatgttgacactttgccattacttttatttcttgatcaaactgctgtttcagttcttcagtagtaatgtcaaccattgctgcaagcttcttcactgccacagttgtgttatttacgtagcctttatatacaactccaaatcctccctctcccattttattaccaccaacagaaatgggtcgttcatcaaagttatttgtgacattcttcaattcataaaatgaaaaactgtgaaaacgtgtatcactaacttctaaacttttattttctggacttgaggagtcaggtggcatatagctttgttcaagattctgcacaggtgtcatcaatgtcctgtctttgtcacagaaaggcatctgtttttgctgaactgttatagcttctttagaaggtagtgtattagcagttttgggaacagcatctgggagcaaaagactcgcaggagcaaaaaattcattttggatcaaaagatccacaagatcaccaactgtgcaatttgtggtgccccagtcaaacagtaattcagaagtgggactttttccagtttgaagtaatgcttcaaatctcggttctggaggctgggaagtccaagatcgagaggctgcatctggttagggccttcttgctacatcatcttatgtgaaactgattgtatctatcatcaccagatggttttttaatagctacagctaacttcttccatccttcttgaggatcaataaaatctgacagcttcctaattagtccaacattgaggcagcgcacatatgttgatggtgttatgggtttgttcatcttctattcccaagtctttcttctggagtaagctctgtcaaaggaacccacttcctctctaacttttctcacggatgataaagagatttccgttccgcagccgaccccagcaaccctggggcagaggtgccgaggcctggaagcggacctcggacgacgtttgaccgaggcattaaggcggggaatgccttacctgcccgggcgcgggctgctgaagccggcgacagaagaaccagccgaactaggaagcgccgcgaag

SEQ ID NO: 11639 - RNA, 2761 nt, Homo sapiens
  source 1..2761: mol_type = other RNA
ctgaatagctgggactacaggtgtccaccaccacgctcgtctaatttttgtatttttagtagagacggggtttcaccatgttggccaggccggtcttgaactcttgacctcaggtgatctgcctgcctcggcctcccaaagtgctgggatttacaggtatgagccaccacatccagccaatgtgacccattatctcacagttctatatattagaagtccagcacagaacagatagattctcatactgaggatcatgcaaagctgaaatccaggtgtcagcccaggctgtggttatcatctgaagcttggagtactcttctaagctgactcagatttttggcagaattcagttccttgtggttgcaactgaggtcccaatttttttttcctgcttgctgacaactggaaggtaggtctcatctcctagaggccacctttaggttttagccaatgtggccctctcacatacttcttcaaggcttacaaggagaattcttcttgcaagggttcacttgattaggtcaggccctttcaacagtctcaaagtgagttgtttaggaaccttaactgcatctgccaaattccttcaactttgtcatgtaacataatctaataatggacatatcattatggcagtatcatcaagggatattttatttgtggttaaatgattgctgtgaacacaatctataaatatatgactaataggattttgtaactggctctataaactttaaattttgtatcattttacaatttacaaagtgcttgtatatattttgcatcatttgattttcatgactacctgtcagagaagcacagcagatattagcccaatgttattagtggctcacagcagctaagtgtatgtccaaagctttacagcaaattagtagtggagtcagctgggcttcagatcagagtgtttccaccctacatacagcccaggctctttttgctaaccctgtaattttcaaactgtgtttggtgatgcttgaaggagatttctcagggattactgtaagaactgggggtgatactaatgggtagggctaagtgttgatatggtggctctatttttatattttggaagttcaacccatgctttaataaccactgtcctgcaacagcctatgccttgttaaaggtaaagaagaatatttaggaaaaaaatcagttaaaaaaatggttgagataggtgtatataaaaagtcaagagtcttttccaataaagttttaagaagctgtcatctcttgcagcagctgttgaaccttcttaatgtctggtctcttatttttcttttcatgcagacattgactagcaacagagtacatagcttcaactgaagtggaatcagcatcattcatctttttatcaatataatcttcaattgtcttttcttcatcttcaatttcttctttaatatctagcaataactgaggttcacggtgttcatccacagctggaagtccagttattatttctagtaaaaccacaccaaagctgtaaatatcagatttgggtgttatttctccacgcaaagcttctggtgccatataagctgttgttcccacaattctgctagtcatgactgtctgggcaaacttctcagaagcccgtgcaaggccaaagtcagatattttagcagtaaaagcttcatccagtaagatatttgcacttttaatatctctatgaatatgatgattttcatgtagaaaattgatgccattagctgcaccctgagcaatcttgcatctcatgtgccaagaaagtggtggagtaccatccaagcaagagagtctgtctagcaatgaaccattaggcatgtaaacatatactaagcagaggtcatctccatcacttgagaaaccaagtagttctactaagttttcatgttgacactttgccattacttttatttcttgatcaaactgctgtttcagttcttcagtagtaatgtcaaccattgctgcaagcttcttcactgccacagttgtgttatttacgtagcctttatatacaactccaaatcctccctctcccattttattaccaccaacagaaatgggtcgttcatcaaagttatttgtgacattcttcaattcataaaatgaaaaactgtgaaaacgtgtatcactaacttctaaacttttattttctggacttgaggagtcaggtggcatatagctttgttcaagattctgcacaggtgtcatcaatgtcctgtctttgtcacagaaaggcatctgtttttgctgaactgttatagcttctttagaaggtagtgtattagcagttttgggaacagcatctgggagcaaaagactcgcaggagcaaaaaattcattttggatcaaaagatccacaagatcaccaactgtgcaatttgtggtgccccagtcaaacagtaattcagaagtgggactttttccagtttgaagtaatgcttcaaatctcggttctggaggctgggaagtccaagatcgagaggctgcatctggttagggccttcttgctacatcatcttatgtgaaactgattgtatctatcatcaccagatggttttttaatagctacagctaacttcttccatccttcttgaggatcaataaaatctgacagcttcctaattagtccaacattgaggcagcgcacatatgttgatggtgttatgggtttgttcatcttctattcctgcccgggcgcgggctgctgaagccggcgacagaagaaccagccgaactaggaagcgccgcgaag

SEQ ID NO: 11640 - RNA, 2596 nt, Homo sapiens
  source 1..2596: mol_type = other RNA
ctgaatagctgggactacaggtgtccaccaccacgctcgtctaatttttgtatttttagtagagacggggtttcaccatgttggccaggccggtcttgaactcttgacctcaggtgatctgcctgcctcggcctcccaaagtgctgggatttacaggtatgagccaccacatccagccaatgtgacccattatctcacagttctatatattagaagtccagcacagaacagatagattctcatactgaggatcatgcaaagctgaaatccaggtgtcagcccaggctgtggttatcatctgaagcttggagtactcttctaagctgactcagatttttggcagaattcagttccttgtggttgcaactgaggtcccaatttttttttcctgcttgctgacaactggaaggtaggtctcatctcctagaggccacctttaggttttagccaatgtggccctctcacatacttcttcaaggcttacaaggagaattcttcttgcaagggttcacttgattaggtcaggccctttcaacagtctcaaagtgagttgtttaggaaccttaactgcatctgccaaattccttcaactttgtcatgtaacataatctaataatggacatatcattatggcagtatcatcaagggatattttatttgtggttaaatgattgctgtgaacacaatctataaatatatgactaataggattttgtaactggctctataaactttaaattttgtatcattttacaatttacaaagtgcttgtatatattttgcatcatttgattttcatgactacctgtcagagaagcacagcagatattagcccaatgttattagtggctcacagcagctaagtgtatgtccaaagctttacagcaaattagtagtggagtcagctgggcttcagatcagagtgtttccaccctacatacagcccaggctctttttgctaaccctgtaattttcaaactgtgtttggtgatgcttgaaggagatttctcagggattactgtaagaactgggggtgatactaatgggtagggctaagtgttgatatggtggctctatttttatattttggaagttcaacccatgctttaataaccactgtcctgcaacagcctatgccttgttaaaggtaaagaagaatatttaggaaaaaaatcagttaaaaaaatggttgagataggtgtatataaaaagtcaagagtcttttccaataaagttttaagaagctgtcatctcttgcagcagctgttgaaccttcttaatgtctggtctcttatttttcttttcatgcagacattgactagcaacagagtacatagcttcaactgaagtggaatcagcatcattcatctttttatcaatataatcttcaattgtcttttcttcatcttcaatttcttctttaatatctagcaataactgaggttcacggtgttcatccacagctggaagtccagttattatttctagtaaaaccacaccaaagctgtaaatatcagatttgggtgttatttctccacgcaaagcttctggtgccatataagctgttgttcccacaattctgctagtcatgactgtctgggcaaacttctcagaagcccgtgcaaggccaaagtcagatattttagcagtaaaagcttcatccagtaagatatttgcacttttaatatctctatgaatatgatgattttcatgtagaaaattgatgccattagctgcaccctgagcaatcttgcatctcatgtgccaagaaagtggtggagtaccatccaagcaagagagtctgtctagcaatgaaccattaggcatgtaaacatatactaagcagaggtcatctccatcacttgagaaaccaagtagttctactaagttttcatgttgacactttgccattacttttatttcttgatcaaactgctgtttcagttcttcagtagtaatgtcaaccattgctgcaagcttcttcactgccacagttgtgttatttacgtagcctttatatacaactccaaatcctccctctcccattttattaccaccaacagaaatgggtcgttcatcaaagttatttgtgacattcttcaattcataaaatgaaaaactgtgaaaacgtgtatcactaacttctaaacttttattttctggacttgaggagtcaggtggcatatagctttgttcaagattctgcacaggtgtcatcaatgtcctgtctttgtcacagaaaggcatctgtttttgctgaactgttatagcttctttagaaggtagtgtattagcagttttgggaacagcatcttatgtgaaactgattgtatctatcatcaccagatggttttttaatagctacagctaacttcttccatccttcttgaggatcaataaaatctgacagcttcctaattagtccaacattgaggcagcgcacatatgttgatggtgttatgggtttgttcatcttctattccaaatatttactgagtgtctactttgtgctagatactgctccaggcccctgcccgggcgcgggctgctgaagccggcgacagaagaaccagccgaactaggaagcgccgcgaag

SEQ ID NO: 11641 - RNA, 3172 nt, Homo sapiens
  source 1..3172: mol_type = other RNA
ctgaatagctgggactacaggtgtccaccaccacgctcgtctaatttttgtatttttagtagagacggggtttcaccatgttggccaggccggtcttgaactcttgacctcaggtgatctgcctgcctcggcctcccaaagtgctgggatttacaggtatgagccaccacatccagccaatgtgacccattatctcacagttctatatattagaagtccagcacagaacagatagattctcatactgaggatcatgcaaagctgaaatccaggtgtcagcccaggctgtggttatcatctgaagcttggagtactcttctaagctgactcagatttttggcagaattcagttccttgtggttgcaactgaggtcccaatttttttttcctgcttgctgacaactggaaggtaggtctcatctcctagaggccacctttaggttttagccaatgtggccctctcacatacttcttcaaggcttacaaggagaattcttcttgcaagggttcacttgattaggtcaggccctttcaacagtctcaaagtgagttgtttaggaaccttaactgcatctgccaaattccttcaactttgtcatgtaacataatctaataatggacatatcattatggcagtatcatcaagggatattttatttgtggttaaatgattgctgtgaacacaatctataaatatatgactaataggattttgtaactggctctataaactttaaattttgtatcattttacaatttacaaagtgcttgtatatattttgcatcatttgattttcatgactacctgtcagagaagcacagcagatattagcccaatgttattagtggctcacagcagctaagtgtatgtccaaagctttacagcaaattagtagtggagtcagctgggcttcagatcagagtgtttccaccctacatacagcccaggctctttttgctaaccctgtaattttcaaactgtgtttggtgatgcttgaaggagatttctcagggattactgtaagaactgggggtgatactaatgggtagggctaagtgttgatatggtggctctatttttatattttggaagttcaacccatgctttaataaccactgtcctgcaacagcctatgccttgttaaaggtaaagaagaatatttaggaaaaaaatcagttaaaaaaatggttgagataggtgtatataaaaagtcaagagtcttttccaataaagttttaagaagctgtcatctcttgcagcagctgttgaaccttcttaatgtctggtctcttatttttcttttcatgcagacattgactagcaacagagtacatagcttcaactgaagtggaatcagcatcattcatctttttatcaatataatcttcaattgtcttttcttcatcttcaatttcttctttaatatctagcaataactgaggttcacggtgttcatccacagctggaagtccagttattatttctagtaaaaccacaccaaagctgtaaatatcagatttgggtgttatttctccacgcaaagcttctggtgccatataagctgttgttcccacaattctgctagtcatgactgtctgggcaaacttctcagaagcccgtgcaaggccaaagtcagatattttagcagtaaaagcttcatccagtaagatatttgcacttttaatatctctatgaatatgatgattttcatgtagaaaattgatgccattagctgcaccctgagcaatcttgcatctcatgtgccaagaaagtggtggagtaccatccaagcaagagagtctgtctagcaatgaaccattaggcatgtaaacatatactaagcagaggtcatctccatcacttgagaaaccaagtagttctactaagttttcatgttgacactttgccattacttttatttcttgatcaaactgctgtttcagttcttcagtagtaatgtcaaccattgctgcaagcttcttcactgccacagttgtgttatttacgtagcctttatatacaactccaaatcctccctctcccattttattaccaccaacagaaatgggtcgttcatcaaagttatttgtgacattcttcaattcataaaatgaaaaactgtgaaaacgtgtatcactaacttctaaacttttattttctggacttgaggagtcaggtggcatatagctttgttcaagattctgcacaggtgtcatcaatgtcctgtctttgtcacagaaaggcatctgtttttgctgaactgttatagcttctttagaaggtagtgtattagcagttttgggaacagcatcttatgtgaaactgattgtatctatcatcaccagatggttttttaatagctacagctaacttcttccatccttcttgaggatcaataaaatctgacagcttcctaattagtccaacattgaggcagcgcacatatgttgatggtgttatgggtttgttcatcttctattccaaatatttactgagtgtctactttgtgctagatactgctccaggcccctggacagggtttgcttttatccctttgtctccctctggcttccaagctgacaggtacacttttttcccccatctgcgaatgtactcatctgatcccataagccgcctccactttctaattccctggaagcttggaggccggagaaacaagcgaattacaatcgtgtggaggctcagcgagctgctggcgccacaggcatctgtcaggtgctggcctgacttcctggttctggggaaaagagacttcatttcgcagtcgggttcacggaatccagggcctgagaggtgagaaacttgaggtccgactgcgccccagaacagctgggtgacgtccctccaagcctcaggctcttcctcagggccgacgaacttcttgattaccggggacctacccaagtctttcttctggagtaagctctgtcaaaggaacccacttcctctctaacttttctcacggatgataaagagatttccgttccgcagccgaccccagcaaccctggggcagaggtgccgaggcctggaagcggacctcggacgacgtttgaccgaggcattaaggcggggaatgccttacctgcccgggcgcgggctgctgaagccggcgacagaagaaccagccgaactaggaagcgccgcgaag

SEQ ID NO: 11642 - RNA, 2660 nt, Homo sapiens
  source 1..2660: mol_type = other RNA
ctgaatagctgggactacaggtgtccaccaccacgctcgtctaatttttgtatttttagtagagacggggtttcaccatgttggccaggccggtcttgaactcttgacctcaggtgatctgcctgcctcggcctcccaaagtgctgggatttacaggtatgagccaccacatccagccaatgtgacccattatctcacagttctatatattagaagtccagcacagaacagatagattctcatactgaggatcatgcaaagctgaaatccaggtgtcagcccaggctgtggttatcatctgaagcttggagtactcttctaagctgactcagatttttggcagaattcagttccttgtggttgcaactgaggtcccaatttttttttcctgcttgctgacaactggaaggtaggtctcatctcctagaggccacctttaggttttagccaatgtggccctctcacatacttcttcaaggcttacaaggagaattcttcttgcaagggttcacttgattaggtcaggccctttcaacagtctcaaagtgagttgtttaggaaccttaactgcatctgccaaattccttcaactttgtcatgtaacataatctaataatggacatatcattatggcagtatcatcaagggatattttatttgtggttaaatgattgctgtgaacacaatctataaatatatgactaataggattttgtaactggctctataaactttaaattttgtatcattttacaatttacaaagtgcttgtatatattttgcatcatttgattttcatgactacctgtcagagaagcacagcagatattagcccaatgttattagtggctcacagcagctaagtgtatgtccaaagctttacagcaaattagtagtggagtcagctgggcttcagatcagagtgtttccaccctacatacagcccaggctctttttgctaaccctgtaattttcaaactgtgtttggtgatgcttgaaggagatttctcagggattactgtaagaactgggggtgatactaatgggtagggctaagtgttgatatggtggctctatttttatattttggaagttcaacccatgctttaataaccactgtcctgcaacagcctatgccttgttaaaggtaaagaagaatatttaggaaaaaaatcagttaaaaaaatggttgagataggtgtatataaaaagtcaagagtcttttccaataaagttttaagaagctgtcatctcttgcagcagctgttgaaccttcttaatgtctggtctcttatttttcttttcatgcagacattgactagcaacagagtacatagcttcaactgaagtggaatcagcatcattcatctttttatcaatataatcttcaattgtcttttcttcatcttcaatttcttctttaatatctagcaataactgaggttcacggtgttcatccacagctggaagtccagttattatttctagtaaaaccacaccaaagctgtaaatatcagatttgggtgttatttctccacgcaaagcttctggtgccatataagctgttgttcccacaattctgctagtcatgactgtctgggcaaacttctcagaagcccgtgcaaggccaaagtcagatattttagcagtaaaagcttcatccagtaagatatttgcacttttaatatctctatgaatatgatgattttcatgtagaaaattgatgccattagctgcaccctgagcaatcttgcatctcatgtgccaagaaagtggtggagtaccatccaagcaagagagtctgtctagcaatgaaccattaggcatgtaaacatatactaagcagaggtcatctccatcacttgagaaaccaagtagttctactaagttttcatgttgacactttgccattacttttatttcttgatcaaactgctgtttcagttcttcagtagtaatgtcaaccattgctgcaagcttcttcactgccacagttgtgttatttacgtagcctttatatacaactccaaatcctccctctcccattttattaccaccaacagaaatgggtcgttcatcaaagttatttgtgacattcttcaattcataaaatgaaaaactgtgaaaacgtgtatcactaacttctaaacttttattttctggacttgaggagtcaggtggcatatagctttgttcaagattctgcacaggtgtcatcaatgtcctgtctttgtcacagaaaggcatctgtttttgctgaactgttatagcttctttagaaggtagtgtattagcagttttgggaacagcatcttatgtgaaactgattgtatctatcatcaccagatggttttttaatagctacagctaacttcttccatccttcttgaggatcaataaaatctgacagcttcctaattagtccaacattgaggcagcgcacatatgttgatggtgttatgggtttgttcatcttctattcccaagtctttcttctggagtaagctctgtcaaaggaacccacttcctctctaacttttctcacggatgataaagagatttccgttccgcagccgaccccagcaaccctggggcagaggtgccgaggcctggaagcggacctcggacgacgtttgaccgaggcattaaggcggggaatg

SEQ ID NO: 11643 - RNA, 2548 nt, Homo sapiens
  source 1..2548: mol_type = other RNA
ctgaatagctgggactacaggtgtccaccaccacgctcgtctaatttttgtatttttagtagagacggggtttcaccatgttggccaggccggtcttgaactcttgacctcaggtgatctgcctgcctcggcctcccaaagtgctgggatttacaggtatgagccaccacatccagccaatgtgacccattatctcacagttctatatattagaagtccagcacagaacagatagattctcatactgaggatcatgcaaagctgaaatccaggtgtcagcccaggctgtggttatcatctgaagcttggagtactcttctaagctgactcagatttttggcagaattcagttccttgtggttgcaactgaggtcccaatttttttttcctgcttgctgacaactggaaggtaggtctcatctcctagaggccacctttaggttttagccaatgtggccctctcacatacttcttcaaggcttacaaggagaattcttcttgcaagggttcacttgattaggtcaggccctttcaacagtctcaaagtgagttgtttaggaaccttaactgcatctgccaaattccttcaactttgtcatgtaacataatctaataatggacatatcattatggcagtatcatcaagggatattttatttgtggttaaatgattgctgtgaacacaatctataaatatatgactaataggattttgtaactggctctataaactttaaattttgtatcattttacaatttacaaagtgcttgtatatattttgcatcatttgattttcatgactacctgtcagagaagcacagcagatattagcccaatgttattagtggctcacagcagctaagtgtatgtccaaagctttacagcaaattagtagtggagtcagctgggcttcagatcagagtgtttccaccctacatacagcccaggctctttttgctaaccctgtaattttcaaactgtgtttggtgatgcttgaaggagatttctcagggattactgtaagaactgggggtgatactaatgggtagggctaagtgttgatatggtggctctatttttatattttggaagttcaacccatgctttaataaccactgtcctgcaacagcctatgccttgttaaaggtaaagaagaatatttaggaaaaaaatcagttaaaaaaatggttgagataggtgtatataaaaagtcaagagtcttttccaataaagttttaagaagctgtcatctcttgcagcagctgttgaaccttcttaatgtctggtctcttatttttcttttcatgcagacattgactagcaacagagtacatagcttcaactgaagtggaatcagcatcattcatctttttatcaatataatcttcaattgtcttttcttcatcttcaatttcttctttaatatctagcaataactgaggttcacggtgttcatccacagctggaagtccagttattatttctagtaaaaccacaccaaagctgtaaatatcagatttgggtgttatttctccacgcaaagcttctggtgccatataagctgttgttcccacaattctgctagtcatgactgtctgggcaaacttctcagaagcccgtgcaaggccaaagtcagatattttagcagtaaaagcttcatccagtaagatatttgcacttttaatatctctatgaatatgatgattttcatgtagaaaattgatgccattagctgcaccctgagcaatcttgcatctcatgtgccaagaaagtggtggagtaccatccaagcaagagagtctgtctagcaatgaaccattaggcatgtaaacatatactaagcagaggtcatctccatcacttgagaaaccaagtagttctactaagttttcatgttgacactttgccattacttttatttcttgatcaaactgctgtttcagttcttcagtagtaatgtcaaccattgctgcaagcttcttcactgccacagttgtgttatttacgtagcctttatatacaactccaaatcctccctctcccattttattaccaccaacagaaatgggtcgttcatcaaagttatttgtgacattcttcaattcataaaatgaaaaactgtgaaaacgtgtatcactaacttctaaacttttattttctggacttgaggagtcaggtggcatatagctttgttcaagattctgcacaggtgtcatcaatgtcctgtctttgtcacagaaaggcatctgtttttgctgaactgttatagcttctttagaaggtagtgtattagcagttttgggaacagcatcttatgtgaaactgattgtatctatcatcaccagatggttttttaatagctacagctaacttcttccatccttcttgaggatcaataaaatctgacagcttcctaattagtccaacattgaggcagcgcacatatgttgatggtgttatgggtttgttcatcttctattcctgcccgggcgcgggctgctgaagccggcgacagaagaaccagccgaactaggaagcgccgcgaag

SEQ ID NO: 11644 - RNA, 4205 nt, Homo sapiens
  source 1..4205: mol_type = other RNA
ctgaatagctgggactacaggtgtccactaccacggctggccaattttttgtatttttagtagagatgggttttcactgtgttagctaggatggtctcgatctcctgacctcgtgatctgcccgcctcggcctcccaaagtgctgggattacaggcgtgagccaccgcacctggccaaccttaacctatttttaaaaaagatgtttatggctttgctgatagcaggctggaaagctagctgaatttgcaggcaacctcaagtagttaatgaaaaattattgtggcttgtccaaagggattgagttttccaaataaaaaagtgggcttcagttttatgtcattgtaagaggccatgtgagggatgtttggatgctcgctttgaatctgtaggaccactcaatgattttttaaaaccattggtttctggcaggcaaaacattcaaaatctaggctatcccaggaaatctagcataagggctgtcctgcagtaatgcattaaaccacgtaacaaacgaactcaagaagagggatgtggctctggatttgtgaccctcaacataacatttaccaccttgggcttcggcttcaacatcagttaaatggagggacacagacgactctttggctcttatactctatgacatgatcactggccaccttagaaaatcaagcctatttagaccacggtttgtgagaagtcagactctctgaggctcagtttccttatctataaaaaagaagatgataacattgggagaagccatcttaagcagcgaggaaagaaaaggacagtggagtcaagtgaacagtctcagatctcagccccgtgtaatctaagggaaggttactggagctgggtctactttcgtcatctgcaaaatggggataagaatgcctgttgtaaggacagttgaatgatcttgctcatgccaacttacagaaggtacgaaataaacgccgatctcctttattctgatctcacattcagcaaatgtgagagaaatgtgaatgtactgaaatgtctgccagaaaaaagaaaatccaacccctcaaaagaatgacatcaggggttttgatatctattcacctacacttccctcttccacaggaagcggcccaccttctgacccacactgcccatctctgtgcttatcatggagctttcaagagtgaggatcggaggctgtattgagcagtgggcacaaaccacagggagcgctgttcaaaaatggaaaacaaggtggccctgacaccgggtgctgctgggcaccctctcagacctgccctgcaacagcatcaggaggctgagggtccccagccagaaggcccaagaggggcccaggctggaaactttactgcgaagcagccctcatcttaaggtggctcaacaccacacctgagatctagcccatgcgacagtatggaagcaggaggccctactccaccacagaaagaacatttatgggcgcctaagccctgggagaatggcacctgagggaacagagcgtgcccacaagcagaccttggggagggagaagaggcagccctgctcctagtcgcagccagcgtgcgtcatgtccaggccccacaagggtgaccctggctcaggttctcatgctccagaagctggcccaggtggcagtgggttccctatggaggcagctcatcattcacaacacagcaacaaaccttctgctctcatgaggagaatgtattttaaacttgggaagagtcataattctgggatgtttcacatgttgtcagctttaaccttctacagacacaggccctctcctctgtgaggagggacctctggcatgtgtgggtgtgtggtgggtccctctccctattagcagaaatgtgttgggcatgagccaggtttatgatttggattgtgtcctgcacataacacctgtgagaatacaactgggactaggacaatgcgggaagcatattcttcatgaggcggtaaccaaaaggcttggctataccaaaggattctggtggccgggcacggtggctcacacctgtaatgccagcactttgggaggccaaggcgggtagatcacttgaggtccaggagttcgagcccagcctggccaacatggtgaaaccctgtctctactaaacatacaacaattagctgggcatggtggtgggtgcctgtaatcccagctactggggaggctgagacaggagaaatgcttgaacccgggaagcagaggttgcagtgagccgagattgcaccacagcactccagcctgggtgacagagcaagactccacctcaaaaaaaaaaaaccacaaaaaaacacaaaaggattctgggtgtaacaatctcagtagagccagcgggtgactctggttctcctaaaattctgcccttacttgccactcaccacacccccagatctgaagggccagcccttttctacctatgacacctcaccagcaagtaaagggcacaggacctcagaagtctgtggtgctaaggatgaagactctactcagagaaggtgctcagccctagtgaggaggttctgggaagcaggtgggcctgctcaatgcagtccctaacccttgggagcatccatgtgagaggtaaaggtgcaaatgacttgggcatgttgactccctactgaggaaggcagggcccctcacatctgcagtggccgtatgcatcagagaacggcatgactgcacatgtgagaactgggtgcacccgagcagtgtcaataggaatcccttccctattccatgccaaacagtcttccccagacacaaagtttccaggtcctgaggcttgactcttctaaggctcaaaatgggttctgtttccagacgtgcttgccttgcttgtctttgcttgtcttaaggactctatttcaggccaatacttgatcctcagacaaactgggacaggttgggaactttgatgttgagatcgccaatgttgatgttccgaggaatctctggcaggttgatgtttttcacagcagacacagcccgcgcaggggctgctgaaaggccaccctcggatttctccagcctgttttgagcctcaatctgagccacgatttcattcatgtttgtttccaacaccatcccacccatcaccacctcctggaggatgtagtgcaccttatccatatggaagatcaaatccaattcacacacattttcgaaacacttatccagagtttccacaaaaacctggatgaggtccaagattccaagttcactctctgaggaatccacacaaaatacaaagtagagggtagcatagtgccggtagatcagtttgtagtcagagccaccaatcaaacttccaccctccaagaagttacagatgttgtcatcccgcttgaggactagatggaaagtctctcgaacaatctgctgttgaatttcttctggccactcctcgtcctctgccccatccccctgctctcggatctccgctgcagcccccttcgaacacttttgggccatgatgttgtctgtccaggatgcccctgtctttccatcaccagtgaaattacacttggtcactgttccagcctcaagtttggccaatgaatccaggaagggaccatcgccccgagtcttcagccgtaccccggcccccagctcgagttccatcacctccatctctgactcgggcatccagaacgccactgtgtggtcgggggtgaggctctctgtcagcgcgagcagctctggcttgttgaccagccccttcagcgcctcgggcgtgagcctgtcagtgtcccccttggcttccaccttgtaggacgacatgaggaagcccgtgttcaccttcctggtggcgctgaagttgggctcgatttcatttcccttggcgtcgaatttacggcgatggatgtgactgggccggatatacagcacgtagtagcgctccttcctgccatgagtgtccaagatgctgtgccgagatacatcgatcagttctccctccagcaggacaccatttcccccctggtgggcggcggggtcccaggcccctggcagccggacgctctgcaccgccttgttccggagcgcgccgtcgtggtagatgcggctcattctcccgaccgcccgggcaccccggcacagagccggcgcactgggctgggggcgcggcgcgggaagtgctgcaggacgcgcggggacccgcgattcccagccggcggatccgggaat

SEQ ID NO: 11645 - RNA, 3530 nt, Homo sapiens
  source 1..3530: mol_type = other RNA
ctgaatagctgggactacaggtgtccactaccacggctggccaattttttgtatttttagtagagatgggttttcactgtgttagctaggatggtctcgatctcctgacctcgtgatctgcccgcctcggcctcccaaagtgctgggattacaggcgtgagccaccgcacctggccaaccttaacctatttttaaaaaagatgtttatggctttgctgatagcaggctggaaagctagctgaatttgcaggcaacctcaagtagttaatgaaaaattattgtggcttgtccaaagggattgagttttccaaataaaaaagtgggcttcagttttatgtcattgtaagaggccatgtgagggatgtttggatgctcgctttgaatctgtaggaccactcaatgattttttaaaaccattggtttctggcaggcaaaacattcaaaatctaggctatcccaggaaatctagcataagggctgtcctgcagtaatgcattaaaccacgtaacaaacgaactcaagaagagggatgtggctctggatttgtgaccctcaacataacatttaccaccttgggcttcggcttcaacatcagttaaatggagggacacagacgactctttggctcttatactctatgacatgatcactggccaccttagaaaatcaagcctatttagaccacggtttgtgagaagtcagactctctgaggctcagtttccttatctataaaaaagaagatgataacattgggagaagccatcttaagcagcgaggaaagaaaaggacagtggagtcaagtgaacagtctcagatctcagccccgtgtaatctaagggaaggttactggagctgggtctactttcgtcatctgcaaaatggggataagaatgcctgttgtaaggacagttgaatgatcttgctcatgccaacttacagaaggtacgaaataaacgccgatctcctttattctgatctcacattcagcaaatgtgagagaaatgtgaatgtactgaaatgtctgccagaaaaaagaaaatccaacccctcaaaagaatgacatcaggggttttgatatctattcacctacacttccctcttccacaggaagcggcccaccttctgacccacactgcccatctctgtgcttatcatggagctttcaagagtgaggatcggaggctgtattgagcagtgggcacaaaccacagggagcgctgttcaaaaatggaaaacaaggtggccctgacaccgggtgctgctgggcaccctctcagacctgccctgcaacagcatcaggaggctgagggtccccagccagaaggcccaagaggggcccaggctggaaactttactgcgaagcagccctcatcttaaggtggctcaacaccacacctgagatctagcccatgcgacagtatggaagcaggaggccctactccaccacagaaagaacatttatgggcgcctaagccctgggagaatggcacctgagggaacagagcgtgcccacaagcagaccttggggagggagaagaggcagccctgctcctagtcgcagccagcgtgcgtcatgtccaggccccacaagggtgaccctggctcaggttctcatgctccagaagctggcccaggtggcagtgggttccctatggaggcagctcatcattcacaacacagcaacaaaccttctgctctcatgaggagaatgtattttaaacttgggaagagtcataattctgggatgtttcacatgttgtcagctttaaccttctacagacacaggccctctcctctgtgaggagggacctctggcatgtgtgggtgtgtggtgggtccctctccctattagcagaaatgtgttgggcatgagccaggtttatgatttggattgtgtcctgcacataacacctgtgagaatacaactgggactaggacaatgcgggaagcatattcttcatgaggcggtaaccaaaaggcttggctataccaaaggattctggtggccgggcacggtggctcacacctgtaatgccagcactttgggaggccaaggcgggtagatcacttgaggtccaggagttcgagcccagcctggccaacatggtgaaaccctgtctctactaaacatacaacaattagctgggcatggtggtgggtgcctgtaatcccagctactggggaggctgagacaggagaaatgcttgaacccgggaagcagaggttgcagtgagccgagattgcaccacagcactccagcctgggtgacagagcaagactccacctcaaaaaaaaaaaaccacaaaaaaacacaaaaggattctgggtgtaacaatctcagtagagccagcgggtgactctggttctcctaaaattctgcccttacttgccactcaccacacccccagatctgaagggccagcccttttctacctatgacacctcaccagcaagtaaagggcacaggacctcagaagtctgtggtgctaaggatgaagactctactcagagaaggtgctcagccctagtgaggaggttctgggaagcaggtgggcctgctcaatgcagtccctaacccttgggagcatccatgtgagaggtaaaggtgcaaatgacttgggcatgttgactccctactgaggaaggcagggcccctcacatctgcagtggccgtatgcatcagagaacggcatgactgcacatgtgagaactgggtgcacccgagcagtgtcaataggaatcccttccctattccatgccaaacagtcttccccagacacaaagtttccaggtcctgaggcttgactcttctaaggctcaaaatgggttctgtttccagacgtgcttgccttgcttgtctttgcttgtcttaaggactctatttcaggccaatacttgatcctcagacaaactgggacaggttgggaactttgatgttgagatcgccaatgttgatgttccgaggaatctctggcaggttgatgtttttcacagcagacacagcccgcgcaggggctgctgaaaggccaccctcggatttctccagcctgttttgagcctcaatctgagccacgatttcattcatgtttgtttccaacaccatcccacccatcaccacctcctggaggatgtagtgcaccttatccatatggaagatcaaatccaattcacacacattttcgaaacacttatccagagtttccacaaaaacctggatgaggtccaagattccaagttcactctctgaggaatccacacaaaatacaaagtagagggtagcatagtgccggtagatcagtttgtagtcagagccaccaatcaaacttccaccctccaagaagttacagatgttgtcatcccgcttgaggactagatggaaagtctctcgaacaatctgctgttgaatttcttctgggaaacgctggtagaagcggactagccgtggcttcccatggttgttgaaaaccagaatcgcctgaatcatctttgccagccacggttctctcagcaccggctactcccagaaagc

SEQ ID NO: 11646 - RNA, 3526 nt, Homo sapiens
  source 1..3526: mol_type = other RNA
ctgaatagctgggactacaggtgtccactaccacggctggccaattttttgtatttttagtagagatgggttttcactgtgttagctaggatggtctcgatctcctgacctcgtgatctgcccgcctcggcctcccaaagtgctgggattacaggcgtgagccaccgcacctggccaaccttaacctatttttaaaaaagatgtttatggctttgctgatagcaggctggaaagctagctgaatttgcaggcaacctcaagtagttaatgaaaaattattgtggcttgtccaaagggattgagttttccaaataaaaaagtgggcttcagttttatgtcattgtaagaggccatgtgagggatgtttggatgctcgctttgaatctgtaggaccactcaatgattttttaaaaccattggtttctggcaggcaaaacattcaaaatctaggctatcccaggaaatctagcataagggctgtcctgcagtaatgcattaaaccacgtaacaaacgaactcaagaagagggatgtggctctggatttgtgaccctcaacataacatttaccaccttgggcttcggcttcaacatcagttaaatggagggacacagacgactctttggctcttatactctatgacatgatcactggccaccttagaaaatcaagcctatttagaccacggtttgtgagaagtcagactctctgaggctcagtttccttatctataaaaaagaagatgataacattgggagaagccatcttaagcagcgaggaaagaaaaggacagtggagtcaagtgaacagtctcagatctcagccccgtgtaatctaagggaaggttactggagctgggtctactttcgtcatctgcaaaatggggataagaatgcctgttgtaaggacagttgaatgatcttgctcatgccaacttacagaaggtacgaaataaacgccgatctcctttattctgatctcacattcagcaaatgtgagagaaatgtgaatgtactgaaatgtctgccagaaaaaagaaaatccaacccctcaaaagaatgacatcaggggttttgatatctattcacctacacttccctcttccacaggaagcggcccaccttctgacccacactgcccatctctgtgcttatcatggagctttcaagagtgaggatcggaggctgtattgagcagtgggcacaaaccacagggagcgctgttcaaaaatggaaaacaaggtggccctgacaccgggtgctgctgggcaccctctcagacctgccctgcaacagcatcaggaggctgagggtccccagccagaaggcccaagaggggcccaggctggaaactttactgcgaagcagccctcatcttaaggtggctcaacaccacacctgagatctagcccatgcgacagtatggaagcaggaggccctactccaccacagaaagaacatttatgggcgcctaagccctgggagaatggcacctgagggaacagagcgtgcccacaagcagaccttggggagggagaagaggcagccctgctcctagtcgcagccagcgtgcgtcatgtccaggccccacaagggtgaccctggctcaggttctcatgctccagaagctggcccaggtggcagtgggttccctatggaggcagctcatcattcacaacacagcaacaaaccttctgctctcatgaggagaatgtattttaaacttgggaagagtcataattctgggatgtttcacatgttgtcagctttaaccttctacagacacaggccctctcctctgtgaggagggacctctggcatgtgtgggtgtgtggtgggtccctctccctattagcagaaatgtgttgggcatgagccaggtttatgatttggattgtgtcctgcacataacacctgtgagaatacaactgggactaggacaatgcgggaagcatattcttcatgaggcggtaaccaaaaggcttggctataccaaaggattctggtggccgggcacggtggctcacacctgtaatgccagcactttgggaggccaaggcgggtagatcacttgaggtccaggagttcgagcccagcctggccaacatggtgaaaccctgtctctactaaacatacaacaattagctgggcatggtggtgggtgcctgtaatcccagctactggggaggctgagacaggagaaatgcttgaacccgggaagcagaggttgcagtgagccgagattgcaccacagcactccagcctgggtgacagagcaagactccacctcaaaaaaaaaaaaccacaaaaaaacacaaaaggattctgggtgtaacaatctcagtagagccagcgggtgactctggttctcctaaaattctgcccttacttgccactcaccacacccccagatctgaagggccagcccttttctacctatgacacctcaccagcaagtaaagggcacaggacctcagaagtctgtggtgctaaggatgaagactctactcagagaaggtgctcagccctagtgaggaggttctgggaagcaggtgggcctgctcaatgcagtccctaacccttgggagcatccatgtgagaggtaaaggtgcaaatgacttgggcatgttgactccctactgaggaaggcagggcccctcacatctgcagtggccgtatgcatcagagaacggcatgactgcacatgtgagaactgggtgcacccgagcagtgtcaataggaatcccttccctattccatgccaaacagtcttccccagacacaaagtttccaggtcctgaggcttgactcttctaaggctcaaaatgggttctgtttccagacgtgcttgccttgcttgtctttgcttgtcttaaggactctatttcaggccaatacttgatcctcagacaaactgggacaggttgggaactttgatgttgagatcgccaatgttgatgttccgaggaatctctggcaggttgatgtttttcacagcagacacagcccgcgcaggggctgctgaaaggccaccctcggatttctccagcctgttttgagcctcaatctgagccacgatttcattcatgtttgtttccaacaccatcccacccatcaccacctcctggaggatgtagtgcaccttatccatatggaagatcaaatccaattcacacacattttcgaaacacttatccagagtttccacaaaaacctggatgaggtccaagattccaagttcactctctgaggaatccacacaaaatacaaagtagagggtagcatagtgccggtagatcagtttgtagtcagagccaccaatcaaacttccaccctccaagaagttacagatgttgtcatcccgcttgaggactagatggaaagtctctcgaacaatctgctgttgaatttcttgaaacgctggtagaagcggactagccgtggcttcccatggttgttgaaaaccagaatcgcctgaatcatctttgccagccacggttctctcagcaccggctactcccagaaagc

SEQ ID NO: 11647 - RNA, 3649 nt, Homo sapiens
  source 1..3649: mol_type = other RNA
ctgaatagctgggactacaggtgtccactaccacggctggccaattttttgtatttttagtagagatgggttttcactgtgttagctaggatggtctcgatctcctgacctcgtgatctgcccgcctcggcctcccaaagtgctgggattacaggcgtgagccaccgcacctggccaaccttaacctatttttaaaaaagatgtttatggctttgctgatagcaggctggaaagctagctgaatttgcaggcaacctcaagtagttaatgaaaaattattgtggcttgtccaaagggattgagttttccaaataaaaaagtgggcttcagttttatgtcattgtaagaggccatgtgagggatgtttggatgctcgctttgaatctgtaggaccactcaatgattttttaaaaccattggtttctggcaggcaaaacattcaaaatctaggctatcccaggaaatctagcataagggctgtcctgcagtaatgcattaaaccacgtaacaaacgaactcaagaagagggatgtggctctggatttgtgaccctcaacataacatttaccaccttgggcttcggcttcaacatcagttaaatggagggacacagacgactctttggctcttatactctatgacatgatcactggccaccttagaaaatcaagcctatttagaccacggtttgtgagaagtcagactctctgaggctcagtttccttatctataaaaaagaagatgataacattgggagaagccatcttaagcagcgaggaaagaaaaggacagtggagtcaagtgaacagtctcagatctcagccccgtgtaatctaagggaaggttactggagctgggtctactttcgtcatctgcaaaatggggataagaatgcctgttgtaaggacagttgaatgatcttgctcatgccaacttacagaaggtacgaaataaacgccgatctcctttattctgatctcacattcagcaaatgtgagagaaatgtgaatgtactgaaatgtctgccagaaaaaagaaaatccaacccctcaaaagaatgacatcaggggttttgatatctattcacctacacttccctcttccacaggaagcggcccaccttctgacccacactgcccatctctgtgcttatcatggagctttcaagagtgaggatcggaggctgtattgagcagtgggcacaaaccacagggagcgctgttcaaaaatggaaaacaaggtggccctgacaccgggtgctgctgggcaccctctcagacctgccctgcaacagcatcaggaggctgagggtccccagccagaaggcccaagaggggcccaggctggaaactttactgcgaagcagccctcatcttaaggtggctcaacaccacacctgagatctagcccatgcgacagtatggaagcaggaggccctactccaccacagaaagaacatttatgggcgcctaagccctgggagaatggcacctgagggaacagagcgtgcccacaagcagaccttggggagggagaagaggcagccctgctcctagtcgcagccagcgtgcgtcatgtccaggccccacaagggtgaccctggctcaggttctcatgctccagaagctggcccaggtggcagtgggttccctatggaggcagctcatcattcacaacacagcaacaaaccttctgctctcatgaggagaatgtattttaaacttgggaagagtcataattctgggatgtttcacatgttgtcagctttaaccttctacagacacaggccctctcctctgtgaggagggacctctggcatgtgtgggtgtgtggtgggtccctctccctattagcagaaatgtgttgggcatgagccaggtttatgatttggattgtgtcctgcacataacacctgtgagaatacaactgggactaggacaatgcgggaagcatattcttcatgaggcggtaaccaaaaggcttggctataccaaaggattctggtggccgggcacggtggctcacacctgtaatgccagcactttgggaggccaaggcgggtagatcacttgaggtccaggagttcgagcccagcctggccaacatggtgaaaccctgtctctactaaacatacaacaattagctgggcatggtggtgggtgcctgtaatcccagctactggggaggctgagacaggagaaatgcttgaacccgggaagcagaggttgcagtgagccgagattgcaccacagcactccagcctgggtgacagagcaagactccacctcaaaaaaaaaaaaccacaaaaaaacacaaaaggattctgggtgtaacaatctcagtagagccagcgggtgactctggttctcctaaaattctgcccttacttgccactcaccacacccccagatctgaagggccagcccttttctacctatgacacctcaccagcaagtaaagggcacaggacctcagaagtctgtggtgctaaggatgaagactctactcagagaaggtgctcagccctagtgaggaggttctgggaagcaggtgggcctgctcaatgcagtccctaacccttgggagcatccatgtgagaggtaaaggtgcaaatgacttgggcatgttgactccctactgaggaaggcagggcccctcacatctgcagtggccgtatgcatcagagaacggcatgactgcacatgtgagaactgggtgcacccgagcagtgtcaataggaatcccttccctattccatgccaaacagtcttccccagacacaaagtttccaggtcctgaggcttgactcttctaaggctcaaaatgggttctgtttccagacgtgcttgccttgcttgtctttgcttgtcttaaggactctatttcaggccaatacttgatcctcagacaaactgggacaggttgggaactttgatgttgagatcgccaatgttgatgttccgaggaatctctggcaggttgatgtttttcacagcagacacagcccgcgcaggggctgctgaaaggccaccctcggatttctccagcctgttttgagcctcaatctgagccacgatttcattcatgtttgtttccaacaccatcccacccatcaccacctcctggaggatgtagtgcaccttatccatatggaagatcaaatccaattcacacacattttcgaaacacttatccagagtttccacaaaaacttttaaggtttgggaacttatagccttcttgttctgatgtcaggtccttgttcccaaagagctagtgttccagtttgtagggtgttgcactggcttttcttcctctctctttttttaagctggatgaggtccaagattccaagttcactctctgaggaatccacacaaaatacaaagtagagggtagcatagtgccggtagatcagtttgtagtcagagccaccaatcaaacttccaccctccaagaagttacagatgttgtcatcccgcttgaggactagatggaaagtctctcgaacaatctgctgttgaatttcttctgggaaacgctggtagaagcggactagccgtggcttcccatggttgttgaaaaccagaatcgcctgaatcatctttgccagccacggttctctcagcaccggctactcccagaaagc

SEQ ID NO: 11648 - RNA, 16142 nt, Homo sapiens
  source 1..16142: mol_type = other RNA
ctgaatagctgggactacaggtgtctaccaccatgcccggctaattttataaaattttttatagagacgggggtcttgctgtgttgctcaggtcttgaactcctggcctcaagtgcacctcctgccttggcctcccaaaacactgggattacagatgcaggccactgtacctggcccccatatttattaatcacattttattcattcattcatttaactttcctgtgaagttttgcaaatggcttcctcaattcccccttgttaagctttttttccttctcaaaccatgcttatatcctttctggttccagccacatattttgggtcagacagtcctagcactgtacttttaatatcacctggagtgacttcagagacttctttgaagccacaagaccatctggttcaataccaatattttgaaatctaatgactcactattctagaacattctcaacattaagtttcttaaagatggcttaaatactttttaaatttaaataaatgtacagaaaacaaaaatcttttcatttaaaacctaccaaatatagccacacatggtagggcatacctatagtcccagttactcaggaggctgaggcaggaggattacttgagccaaggagttcagggctgcagtgcactatgattgtgcctgcaaaaaggcactgcactccagcgtcggccacagagaaagacctagttttttgtttttgtttttgtttttgagacagagtcttgttctgtcgcccaggctggaatgcagtctggagtgcagtggctcattgcaacctccacctcctgggttcaagcaattctcctgcctcagcctcctgagtagctgggattacaggggcacaccaccacgcccaactaacttttgtatttttagtagagatggagtttcgccatgttggccaggttggtctcaaactcctgggctcaagtgattcacctaccttggcctcccaaagtgctgggattacaggcgtgagccactgcatccagccataagactcagtttcttttcttttttttttttggagatggagttttgctcttttgtccaggctggagtgaagtggtgcgaccatggttcactgcaacctctaccctcccggttcaagcaattctcctgcctcagcctcccaagtagctgggattataggcacccactactacgcccagctaatttttgtatttttagtagagacgaggtttcgccatgttggctaggctggtctcaaactcctgacctcaggtgatccacccgcttcggccttgcaaagtgctgagattacaggcatgagtcaccacgcctggccggcaagaccctgtttctaaaaaacaaaataaaaaataaatcttccaactatttataatatgatctctgttcatctttactgttataaacattcctcaggtacttgaaaggagtgtgtgttctaggcttgttgagtacagataacctattagacaaggttactaacttccctgctgcctgctctatcacctctattagaagtatttaaaatctcaattttccttttaattttcatgctgttttctgggttgttcatgattgctatgtttgtggtggattgttctttaaaaaaaaaaatcttgatcctattaacactttttgcctcaaattctattttgtctgctattgatattactacccaaaatccccgcaccccgcccttttttttgagacaggatctcactctgtcactcaagctggagtgcagttcaccatcacggtggctcattgcagcctcgacctccctgggcttgggtgatcctcccacctcagcctcccgagtagctgggatcacaggcacataccaccatacctggctaatttttgtactttttatagagacggggattcaccatgttggccaggctggtcttaaactcctgatctcaagtgatccgcccaccttggcctcccaaagtgctgggattataggcatgagccaccacacccagccggcagcaaactgtttatggactggtactggggcccagaccctaccttgagtggtactgggctagaggacttattaattgcatgatctaggagtagttcataaattctgtgatggtcattctttgggtgaactccatttctagcagattctagataagcagcatgacttcctctgattctctgacacctgagggtggggaaattcagactgtcccacttgggttgtgcgtcttcacgctggggaagagggtgaggccaaagttgtgttgggagataaataatgaaattcaagaactccatggtaacagcccttgtctttcctctctggggccacacagtgcagtgtggggagaggagtggacagaaggaatgtcagcatttccttggcaaaatctcttgcgtttcagaacagcagtgagattttggaggtatgagagagtcacaggtgtgacattcctgtgaggaatgctatttgagtacaagcagtggatgtcctcatgatgttatgatttcagaagaatagcactgtgcttggctgaaaagttctgcattcaataactccatgccaataagcagccatttcctcccagcacacagttgctcaccaatgtccatggtcctatggcactgggaggcctctgatgcagctgtctcccactatggtcttaggaaattcctggaacgttattagagtgagtttttcctagatctgcttactgaatacctgttgaactttcacactgatggccagttccaagacttaagcatgaccttgcgaccattggtgatagtgctttcttgatctgctgaatcaaattgaagcagaactgggggtactactaggaatgaggggtgactagggatggggctggggcgaggggtatattgggtaactgaggatgaccagtgtcagagagcacaaagatgatggtgaagggcaggtagaccacctcccacttggtgggaaagtctgttcctggctggaactggttcattcattccaagccagcaacagctccaggtttggacgccatttatgaatctacatgccaccagaccagtccctgtcttccacacaccccactctctggagtctggaaaaatggcgggggtggggctagctactagtttttgtttttttttttctttttgagacacagtttcattctgtcatccaggctggagtgcagtggcatgatctcagctcactgcaacctccgcctcccaggttcaagcgattctcgtgccttagctttcagagtagctgggactacaggtgcacaccatcacagctgactaatttttcttttctttttttttttttgagacggagtctcactctgtctcccaggctggagtgcagtgatgtgatctcagctcactgcaacctacgtctccagggttcatgtgagtttcctgcctcagcctcctgagtgagtagctgggattacaggcgcctgccaccacgtccagctaatttttgtatttttagtagagattgggtttcaccatgttggccaggctggtctccaactcctgacctcaagtgatccacctgcctcggcctcccaaatcgctgggattacaggcgtgagtcatcatgcctggccttttttttttttttgtgagacagagttttgctcttgtcacccaggctggagtgtaatggcatgatctcggctcactgaaacctctgccaggcacacgtcaccatgcccggctaatttttgtatttttggtagaaacggggtttcaccatgttggccaggctggtctccaactcctgacctcaagtgatcctcctgccttggcctcccaaagtgctgggattacaggtgttagctaccaagtctggcctttttttttttttttttttttttttttttttgagacagagtttcgctcttgtcacccaggctggagtgtaatagtgtgattccagcttactgcaacctctgcctctcgggttcaagccattctcctgcctcagcctcctgagcagctgggattacaggcacacgccagcatgcctggctaatttttatatttttagtagagacggggtttcaccatgttggccaggctggtctcgaactcctgacctcaggtgatccatctgcctcagcctcccaaactgctgggatgacaggcgtgagccaccacgccaggccctatttttatttttaaccagtgctgtagtttgaatatttgtctcctccaaaactcatctggaaacatccccaatgtggcaatattgagagatggcgcctttaaaaggtgactgggtcatgaaggctctgcccagtgagactggtgcctttataagaagaggaagagagacctgagctaccatgctcaagtccctcaccacgtgaggccctctgccaccttgggtctctgcagagagttcccaggaacaagaagtctctcaccagatgtggaccctgtaccttggacttctcagtctccactattgtaagaaataaattccttttctttataaatgacccagtttcaggtattctgttctatgcaacacaaaatggactaagacaacgagtacgcttagttgttgcttcctgagttccaaagtccgacagacagagcaggtcctccattcttgcccctttttaccccaaatgctcattggcattcttgcagctacgagtaataattaaaagtggctaagccaggctggcatggttgctcacgcctgtaatatcagcactttgggaggctgaggcaggaggatcacttgaacccaggagtgagaccagccagggcaacatagcaacaccctgtctctaattattattatttttttaagtgagtaagccaaataggggtttacttttcatctagaacaagaagacgtgttggccaggctggtctcaaactactgggctcaagtgatccacccacctcagcctcccaaagtgttgggattatgcgtgagccaccgcacctggccacaagacccaatttcttttattttatctttttttttttttttttaagagatagggcatctaacggcattgttttagctgctcaacacttttttttttttgcttatttttgtttgttttgtttgtttttgagacagggtctccctctgttgcccagcatatagtgcagtggcatgatcatggctcactgcagcctcaacctcccaggatcaggcaatcctcctgcttcagcttcctgagtagctgagaccacaggtgcacaccaatatacctaatttttttttttttgagatggagtttcactcttgttgcccaggctggagtgcaatggcgtggtctcagctcactgcaacctctgcctccctggttcaagcgattctcctgtctcagcctgccgagtagctggggttacaggcataagccactacgcccagctaattttgtatttttagtagagacagggtttctccatgttggtcaggctggtctcgaactcctgacctcaggtgatccacccacctcagccttccaaagtgctgagattgcaggtgtgaaccactacgcctggccacctgactaatttttaagttattcacagagaacaggttttgcaatgttgcccaggctggtctcaaactcctgggctcaaatgatcctcctccctcggcctcccaaagtgctggggttacaggtgtgccactgtgcctggtcggctcaccactttcagatctggctctcttcacctctcttttatagtcataagctgattagcacaattctagacatccgcagctacatttaaggcaggaaggaggtggtaatagacactaccagccacatctgtcccttttaatcaggataccctagaaatcctcagcagactttgaattatgtgccattggtgaaatgtcatatgatcatccctctacaaggcaacgaggtaaaaagagaatttagtatttctagcctctagagtggagatgaacaaagaataggaatgggcatttgcttaggaaaccaactgtgccttacaacatttttgcacttttttctgtaacattttgtgttaaatcatataaaaatgctgatcctaacaaatatggtcaatgagtcacaccataattctctaagaactccagtccaaaaaggttaatcttgcttttaaactccaggcgcggtgtttcacagctgtaattttagcacttcgggaggcagagcaagaggatcacttgaggccaggagttggagaccagcctggcaacatagcaagaccccgtctctacaaaaaataaaattatctgggcctgttggtgcacacctgtagtcccagctactcaggaggctgaggtgggaggatcacttgagcctaggaattcgaggctgcagtgagctgtgattgcaccactgcactccagcctgggtgacagagggagaacctatctccaaaacaaaacaaaataaaaacaaaacaaaactccaagcagagaaagacttgacgagtcggatgagtctgatgattcctaaaggaaatcctttttgagattccaggagattccatctcctcaacagagtaattgattttgagcctcccacctcctgaattaaggcccacccatccctatcctgcactgaactgtagactcttttttacttccttacaaaagtttattcttaaatgtacaacagactccaagacgacactttattgtagctataggtggcaaaagatgttatggcagagaatccagatgtttaaataggaatggggtcaagggtcaccgccccaagcacggataacaaaatttattttttgccagatttctttaattccacctgtgactggtgagggctggtggcggggtggctttcacttttagctcctctttttgtttctgcttgaacgtcccatcttccttacccacccccttgacctgcttcttgagctttctcagggcttcttgccacctttgcagctgtacatggcacctgccatagggctctaattttaaactgagaaattgagaaaacaggaaactgactctttttggggggagagtaagacaaacaggaaaaggaaaatgaagacgtggttgatacagatcgttggatttcaaaaggaaaagtctacggataaccgaaaaaaataaatatttagaaatgcatagtcttggctggttaaataagtatccatgcttgttcttgtggcatagtagttacgagacatttttagttaaatggaaaaatgtgaattactatagtttgagtgatatgctgctttccaaattaaaagcagcataacaaaaacattcccctaatactcataaataattcattgaattggcaataattcacctcctaatgacttcatatgaagtataaagtaacttcgatacatcagaagaaatcctatcttctaatataagaaagtaatatgattacattaaatgcgtctcatataagttataaaaatggtatctatgagtaaagaaatgcttgtgaacaaaaaaattgatcttataaaggtcaaacaggccaggcgtggtggctcacacctgtaatcccagcactttgggaggctgaggtgggcggagtacctgaggtcaggagttcaagaccagcctggccaacatggtgataccctgtctctacaaaaatacaaaaaattagctgggcatgatggtgggtgcctgtaatctcagctactcgggaggcagaggcgggagaatcgcttgaacccgggaggcggaggttgcagtgaactgagattgagccacaacaaccaagcctgggagacagaggaaactctgtctcaaaaaataaaaaataaaaattaaaattaaaaaaaaggtcaaacaaaccaaacccttctgattaatttattcaatctacttttattataagcaaatgagaaattataattttaatctgaaaaagcagaatcaggggattttggagctggacagtcccctggaaattatttggatcaaagccctcattttataggtgaagaaactgagaagtaagatttgagcaagctgcccaaaggctttgccaaaggctataccagtgaatggcagagtctggactggaagtcccagtgctgccgtccaggtgagacctgttccactgcatgctactagctcccgggctgagaccggacttttgcttggcaggtttctttctttcgaaactattaattattgtattttttgtagagacagggttttgccatgatgcccaggctggtcttgaactcctgagctcaagagatccacccagcttggcctctcaaaaatgttgggattacaggcataagccacagtgcccggcccattttcctcccacctctttgttccttctctgtttcttttgcagcattatgttctatcattgtataccagagttcctcaacttcagttatagtctgttcttgctttatgctatcttcttcagcaagctcatcttggtctgttttcctccttatcaggcataccccagaaactcctgttttatctccacctcaactaaacattttcctgagttctgggcctctataaactaattatttgattaacatcttttttttttttttctgagatagagtctctctctgtcacccaggctggagtgcagtggtgcaatctcagatcactgcagcttctgcctcccagattcaagcgattctcctgcctcagcctcctaagtagctgggattataggcatgcaccaccgcacacagctaatttttgtacttttagtagagacggggtttcaccatgttggtcaggctggtctcaaactcctgatctgaagtgatctgactgcctcagcttcccaaagtgctgggattacaagcctgagccaccatgcctggccaacatctttaattggatatctcagtatcaagaaggcccataatattcctctgcctcatccctctcctcagtcctcttcttgtgtttcctagttcagagaatggcaccattctctatcaagctgcgcaaatcagacatgtgtgattttttgttgttgttgagacagggactcactctgtcacccaggctagagtgcagtggcgtgatcatggcgcactgaagcctcaaactcctgggctcaggagatcctcccgcctcagcctcctgagtagctgggaccacaggcccacaccaccatgcccagctaattttgtattctttgtagagatggggtttcatcatgtttgcccaggctggtctcgaactcctggactcaagcaatccacccacctcagcctcccaaagtgctgggattacaggcatgagccactgtgcccagctgaagtgtgatccttaacttcaccccttctcatgccctccatttccaatccatctccagtccagttgactccagctactcaattatttccacttatctcattccactacctttgaagctaccaccatctctaactacagtcatctcccaactaactggtctcctggcatctctctggttctcctccactaatttcaaaaaaagaaatttactgtgacagtgctcacaacactcccccttgctcttactaaagatgcttaccatagcctccaggtattgtatggcctgaggtctatctacatttccaggtgcaggacacaccatgtctccccactcccaaatttagtctccagactccatcctttttacagttctttaaaagcatcacaattcctccaaccactaggcatttgtatgtgctattccctctttccagaatgcaataccctccctctgcctagctagctaacttctatgtatctatgactgcagctcaaactttcctcatggactccctccacaagtgccaagcctgggccagattcttttgttatgtgctcacagaacgatgttccctttagcattcattgagtttgctgtttaattattcttgtcttgtttttgtttaattagtcctatctctaatactagacaaatgttccttaagatcacaggaaatataggactgtctctacataaaaactgttttatatccataatgcctaggacagtacctggcacacagtatatgctcaataaatttttgttgaatgaatgcaattatcattatattcctgatattagcaggtataatccagtttaagtttgggaacagaaagacaaaacggaccacatctaataaatccggtctcctttcttttattatttatttatttgagacagttttgctcttgttgcccaggctgcagtgcaatggcatgatcttggctcactgaaacctccgcctcccaagttcaagggattctccagcctcagcctcccaagtagctgggattacaggcatccaccaccacgcccagctaatttttttgtatttttagtagagatggggtttcaccatgttggccaggctggtctcgaactcctgacctcaggtgatccacccacctcagcctcccaaagtgttgggattacaggcgtgagccaccgtgcccggccaaggtctcctttcttttaatcaaactctcacctttggccattctgcagtcattcacccgacagtatttactgacggagtgaatacagagtgcttgattaatgttgctgctttgttattattattattattattgagatggagtcttgctctgttgcccaggctggagtgcagtggcgtgatctcggctcactgcaacctccgcctcccgggttcaagccattctcctgcctcagcctcccaagtagctgggactacaggcatgcaacaccacacctggctaatttttgtatttttagtagagacaaggtttcaccatattggccaggctggtcttgaactcctgacctcaggtgatctgcccacctcagcttcccaaagtgctgggattacaggcgtgagccaccatacccaacctaatgtttctgctttgaaatacaatttcaaaaagtcattaataggttgaaaacagcaagattttaaaagtattttaaaaagtgaaacagaagaatgcttacttcatttcacagagatagatttctcctttatgttatttctaaaaggagatggaattttgtttcattcatttctgcttatttggacaggccaaatatgaacagctgaacacgtcagcgttaccatgcatatgttacacagatgccatccttcttccatcagctctcatatgcaatacagaagtaaaaagaggttctctttatttttaaaaggtaaaaattgaaattcagtcacttaacacagaataaacaataattacaattacactggtaacaaaggacagcaagcatgttttctttgaaagcactgtatctggtttgtctccgtgcttggtcctagtatctggcatattttccccagagttttcttttcagtgggatgattatcttcggggcaaaaaagtttatcagactcaagttttagcagtacttattttattcatttatatacatgtaaccccatcctgtcttactccaatcttcttactgccttcctactgacacatatattatataacaccctccccaagttctatttacggttaaaaatttctttttttttttctttttttgagacagagtttcactctcgtcacccaggctggtgtgcaatggcgcagtctcggctcactgcaacctccgactccctggttcaagtgattctcctgtctcagcctcccgagtagctggaattacaggcgcccgccaccatgcccagctaatttttgtatttttagtagagacagtgtttcgccatgttggccaggctggtctcaaactcctgacctcaggtgatccacccgccttggcctctcaaagtgctgggattataggcgtaagccactgcgcccagcctacagttacgaatttctaaatggcacaaataaactcagctgttctcagtgcagacgtcaaatcctcactgtgctgaaacattttcctcagcttttgggaaataattacaatttaaacatacacagagaatgtttcttagacaaacataatacccgaggcttatctggtaaaaactaattgctctgtccttagcacaaaaaatatatatctttgtaaaatgagaagaaccaaagaatatttaaaacaaagaaggaagccacacgtactaattacacaagagactgactgacaaactggaattctccaaaacagattttcagcgaggcttctcatttcagagtccaggaaaaaaaaatcctaaaaaccccaaaggtatattatatgtgtgtatatatatttttattgtgttaaaaaacacaaaacataaaatttactgtcttatcaaaaggtatattttgtcgctcttccctttttttttttttttttttcccgagacagagtccagtctgtcgcccaggctgaagtgcagtggcatgatctcggctcactgcaacctgcatcttctgggctcaagcaatcctcccacctcagcctcctgagtagatggagctacaggcacgtgccactaggcccggctaatttttgtattttttgcagacagggttttgccatgttgcccgggctggtctttgttctcctaagagttgttttctccatgaaagttgataaataacatttagaaaatgaattattacaagagtaatgatatgtctcaatttattatatgaaattatcaacaactgcttttaatattcagatgtcaagaagatgaaaagcagaaatacattttgcaaacatgtagcactccataaatggaaatcatgtatttcctctaatatcccaatttttctatattgggatcttatatggctgtttctatatggctattttgtcccaacttgctgtacaagaattttccccagccaccttagaaaggttggatgtagttcactccaagtttgcagttcactccaagtgtttcagtaccacagaaagctccatggaagcctcaaatgtacgggctaggcaatagaagcagggaggtaggattaagaaattactggccaggtgtggtggctcaggcctgtaatcccagcacttcgagaggctgaggcagacagatggcttgagctcaagagtttgagatcagcctgagcaacatggcaaaactctgtctctacaaaaaatataaaaatcagccaggtatgttggtgtgcacctgtagtcccagctactggggaggttgaggcaggaggattgcttgagcccaggaggctgaggctgcagtgagccatgattgtgccactgcattccagcctggtcgactgtaagacaaaaaataagaaaataaaaaatttaccaatataaaatgctcaaacagctaacaaacatgttcaattccatttatagtcttttctttgagccatttaaacatagggctattttttttttttttttttgagatggagtttcactcttgttgcccaggctggagagcaatggcatgatctcggctcaccacaacctctgcctcctgggttcaagcgattctcctgcctcagcctcccgagcagctgggattacaggcatgtgccaccatgcctggctaattttgtatttttagtagagacgggattcctccatgttggtcagactggtcttgaactcccaacctcaggtgatctgcctgcctcaaccttccaaagtgctgggattacaggtgtgagccactgagattggctgccgttttgttttttaactccatatagtttctatagttcactgaaaactcaaagagatgacctataaatgtatgaataatgtatgatttcttacatcaattttctactagaaaaaaatcatacttttagaattggattttgtcttacagtcatctttattatactttataaatgagatttcatttatataaatcaggaagctaaactaaaatagaaacactagatttaaattctgatttgaatactctgatcaaaataacaaatctcacactgggaaaccatctatcagcaagcagagagctactgtgtgtccttccttagaagagtttgaacaccgagaacccacagcatatttgcagtacagtaacagcaattcctttgtcattatcacagaactttaattttcatatactttgctgggaccaaccaaaccatcccatatatataaccatatccatatatatatatatatatatcccacatatatatgggatggtatatatatacacatgtatatgtatgtgtgtgtgtatatatgtgtatatatgtatacacacacacacacacacatatatatatatatacacacacacacatatatatatggagagagagagagagacagtgtcttgctctgtcgcccaggctggagtgcagtggtacgatcttggctcattgcaacctccgcctcccaggctcaagcgattctcatgtctcagtctcccaagtagctgggattacaggtgtgcaccaccacaccaggctaaccattccatacattttatacaatcatttttaaaaagaagcatgaaccatttcggttttagagaattaagtttttttaaaaaagagactcttaaaaaaaagtcattatatgaataaaatctgctttgtgttaattccgacaaatcattccatcattgagtctgtcaccaattttttttttttgaaatggagtttcgctcttgttgcccaggctggagtgcaatggtacgatctcggctcactgcaaccgccgcctcccgggttcaagtgattctcctgcctcagcctcccgagtagctgggattacaggcatgcgccaccacgcctggctaattttgtattattagttgagacagggtttctccatgttggtcaggctggtctcgaactcctgacctcaagtgatccgctggccttggcctcccaaagtgctgggattacaggcgtgagccaccgtgcctggcccaattttttttttttaataacttgcacacttaacaatattttttatcttcttgggacaacattcttttctccacaaaaacccaattaaggacgttgtgccagtttactcctacttccttcctgttcactgagcttaaagtgggtataggcgagaatgccaaataatgtacataaaatgccaagggcctgattaatggacagtggatccttaaataaaacatatcctccgaataaagtaatgcagaacttgaagtgtccgaacatgttataggtgacaggtgaagtgttcccaatgatccaataaattgataagttcaccatgaaagctattactccagatagcagcaccataagcaaagcagaaactgaccagggaccaaatattcctccttctccaaacactggctcaaagaagggcacagcaaccagcaacatggcagatgacatcggagcctggtagtacagcagctgcattgagttcacttgtaattcatgctgtttggctcctacccaaaacaggtaggtatttggtgagcatcacacacccaagtttctctgtctcctttcttctcttcaccttgagtcagacaacttatgcaattatgctttcttcccaacagtctattgtctctatactgtattttctaaaccttggaatacagcttcaaaatttatgaaatcagcgtgagctggattctggtggagaaggttttctggtagcagaaggtctggatggctatgatcaccggcgtggtcatggccttggccagctgataggtgcctatggtgttgttctgcagagaaaggttagtgaagaccacaaagccacagaagctgagggccaggaggaggagcctggagggcggcagacttttgggggcaaagatgtccagcttctggcagatatacaagcccagccaggtgaccacgaagtgcaccagggtcaggctcatgttggggaagccgtggtacacataaatccatttgttgaggaacacaatgcagatggacaccagcaggttgaacaggagcccggcggcgattcgccagtggccccgcactcggtccaccagcaatgccatgatccccgcgaagctggggccgtctagcctcggaaggggcgccgggcctgtctccggctgcccttctactccaccgccgcgtcctcgcagacgccgacctcaccgtctgacccaggagtggcatgcacagatcaaccccgggcgagtagcactcttaacagaggacacacaccccgccgccgccctgtaagccagctaggac

SEQ ID NO: 11649 - RNA, 16145 nt, Homo sapiens
  source 1..16145: mol_type = other RNA
ctgaatagctgggactacaggtgtctaccaccatgcccggctaattttataaaattttttatagagacgggggtcttgctgtgttgctcaggtcttgaactcctggcctcaagtgcacctcctgccttggcctcccaaaacactgggattacagatgcaggccactgtacctggcccccatatttattaatcacattttattcattcattcatttaactttcctgtgaagttttgcaaatggcttcctcaattcccccttgttaagctttttttccttctcaaaccatgcttatatcctttctggttccagccacatattttgggtcagacagtcctagcactgtacttttaatatcacctggagtgacttcagagacttctttgaagccacaagaccatctggttcaataccaatattttgaaatctaatgactcactattctagaacattctcaacattaagtttcttaaagatggcttaaatactttttaaatttaaataaatgtacagaaaacaaaaatcttttcatttaaaacctaccaaatatagccacacatggtagggcatacctatagtcccagttactcaggaggctgaggcaggaggattacttgagccaaggagttcagggctgcagtgcactatgattgtgcctgcaaaaaggcactgcactccagcgtcggccacagagaaagacctagttttttgtttttgtttttgtttttgagacagagtcttgttctgtcgcccaggctggaatgcagtctggagtgcagtggctcattgcaacctccacctcctgggttcaagcaattctcctgcctcagcctcctgagtagctgggattacaggggcacaccaccacgcccaactaacttttgtatttttagtagagatggagtttcgccatgttggccaggttggtctcaaactcctgggctcaagtgattcacctaccttggcctcccaaagtgctgggattacaggcgtgagccactgcatccagccataagactcagtttcttttcttttttttttttggagatggagttttgctcttttgtccaggctggagtgaagtggtgcgaccatggttcactgcaacctctaccctcccggttcaagcaattctcctgcctcagcctcccaagtagctgggattataggcacccactactacgcccagctaatttttgtatttttagtagagacgaggtttcgccatgttggctaggctggtctcaaactcctgacctcaggtgatccacccgcttcggccttgcaaagtgctgagattacaggcatgagtcaccacgcctggccggcaagaccctgtttctaaaaaacaaaataaaaaataaatcttccaactatttataatatgatctctgttcatctttactgttataaacattcctcaggtacttgaaaggagtgtgtgttctaggcttgttgagtacagataacctattagacaaggttactaacttccctgctgcctgctctatcacctctattagaagtatttaaaatctcaattttccttttaattttcatgctgttttctgggttgttcatgattgctatgtttgtggtggattgttctttaaaaaaaaaaatcttgatcctattaacactttttgcctcaaattctattttgtctgctattgatattactacccaaaatccccgcaccccgcccttttttttgagacaggatctcactctgtcactcaagctggagtgcagttcaccatcacggtggctcattgcagcctcgacctccctgggcttgggtgatcctcccacctcagcctcccgagtagctgggatcacaggcacataccaccatacctggctaatttttgtactttttatagagacggggattcaccatgttggccaggctggtcttaaactcctgatctcaagtgatccgcccaccttggcctcccaaagtgctgggattataggcatgagccaccacacccagccggcagcaaactgtttatggactggtactggggcccagaccctaccttgagtggtactgggctagaggacttattaattgcatgatctaggagtagttcataaattctgtgatggtcattctttgggtgaactccatttctagcagattctagataagcagcatgacttcctctgattctctgacacctgagggtggggaaattcagactgtcccacttgggttgtgcgtcttcacgctggggaagagggtgaggccaaagttgtgttgggagataaataatgaaattcaagaactccatggtaacagcccttgtctttcctctctggggccacacagtgcagtgtggggagaggagtggacagaaggaatgtcagcatttccttggcaaaatctcttgcgtttcagaacagcagtgagattttggaggtatgagagagtcacaggtgtgacattcctgtgaggaatgctatttgagtacaagcagtggatgtcctcatgatgttatgatttcagaagaatagcactgtgcttggctgaaaagttctgcattcaataactccatgccaataagcagccatttcctcccagcacacagttgctcaccaatgtccatggtcctatggcactgggaggcctctgatgcagctgtctcccactatggtcttaggaaattcctggaacgttattagagtgagtttttcctagatctgcttactgaatacctgttgaactttcacactgatggccagttccaagacttaagcatgaccttgcgaccattggtgatagtgctttcttgatctgctgaatcaaattgaagcagaactgggggtactactaggaatgaggggtgactagggatggggctggggcgaggggtatattgggtaactgaggatgaccagtgtcagagagcacaaagatgatggtgaagggcaggtagaccacctcccacttggtgggaaagtctgttcctggctggaactggttcattcattccaagccagcaacagctccaggtttggacgccatttatgaatctacatgccaccagaccagtccctgtcttccacacaccccactctctggagtctggaaaaatggcgggggtggggctagctactagtttttgtttttttttttctttttgagacacagtttcattctgtcatccaggctggagtgcagtggcatgatctcagctcactgcaacctccgcctcccaggttcaagcgattctcgtgccttagctttcagagtagctgggactacaggtgcacaccatcacagctgactaatttttcttttctttttttttttttgagacggagtctcactctgtctcccaggctggagtgcagtgatgtgatctcagctcactgcaacctacgtctccagggttcatgtgagtttcctgcctcagcctcctgagtgagtagctgggattacaggcgcctgccaccacgtccagctaatttttgtatttttagtagagattgggtttcaccatgttggccaggctggtctccaactcctgacctcaagtgatccacctgcctcggcctcccaaatcgctgggattacaggcgtgagtcatcatgcctggccttttttttttttttgtgagacagagttttgctcttgtcacccaggctggagtgtaatggcatgatctcggctcactgaaacctctgccaggcacacgtcaccatgcccggctaatttttgtatttttggtagaaacggggtttcaccatgttggccaggctggtctccaactcctgacctcaagtgatcctcctgccttggcctcccaaagtgctgggattacaggtgttagctaccaagtctggcctttttttttttttttttttttttttttttttgagacagagtttcgctcttgtcacccaggctggagtgtaatagtgtgattccagcttactgcaacctctgcctctcgggttcaagccattctcctgcctcagcctcctgagcagctgggattacaggcacacgccagcatgcctggctaatttttatatttttagtagagacggggtttcaccatgttggccaggctggtctcgaactcctgacctcaggtgatccatctgcctcagcctcccaaactgctgggatgacaggcgtgagccaccacgccaggccctatttttatttttaaccagtgctgtagtttgaatatttgtctcctccaaaactcatctggaaacatccccaatgtggcaatattgagagatggcgcctttaaaaggtgactgggtcatgaaggctctgcccagtgagactggtgcctttataagaagaggaagagagacctgagctaccatgctcaagtccctcaccacgtgaggccctctgccaccttgggtctctgcagagagttcccaggaacaagaagtctctcaccagatgtggaccctgtaccttggacttctcagtctccactattgtaagaaataaattccttttctttataaatgacccagtttcaggtattctgttctatgcaacacaaaatggactaagacaacgagtacgcttagttgttgcttcctgagttccaaagtccgacagacagagcaggtcctccattcttgcccctttttaccccaaatgctcattggcattcttgcagctacgagtaataattaaaagtggctaagccaggctggcatggttgctcacgcctgtaatatcagcactttgggaggctgaggcaggaggatcacttgaacccaggagtgagaccagccagggcaacatagcaacaccctgtctctaattattattatttttttaagtgagtaagccaaataggggtttacttttcatctagaacaagaagacgtgttggccaggctggtctcaaactactgggctcaagtgatccacccacctcagcctcccaaagtgttgggattatgcgtgagccaccgcacctggccacaagacccaatttcttttattttatctttttttttttttttttaagagatagggcatctaacggcattgttttagctgctcaacacttttttttttttgcttatttttgtttgttttgtttgtttttgagacagggtctccctctgttgcccagcatatagtgcagtggcatgatcatggctcactgcagcctcaacctcccaggatcaggcaatcctcctgcttcagcttcctgagtagctgagaccacaggtgcacaccaatatacctaatttttttttttttgagatggagtttcactcttgttgcccaggctggagtgcaatggcgtggtctcagctcactgcaacctctgcctccctggttcaagcgattctcctgtctcagcctgccgagtagctggggttacaggcataagccactacgcccagctaattttgtatttttagtagagacagggtttctccatgttggtcaggctggtctcgaactcctgacctcaggtgatccacccacctcagccttccaaagtgctgagattgcaggtgtgaaccactacgcctggccacctgactaatttttaagttattcacagagaacaggttttgcaatgttgcccaggctggtctcaaactcctgggctcaaatgatcctcctccctcggcctcccaaagtgctggggttacaggtgtgccactgtgcctggtcggctcaccactttcagatctggctctcttcacctctcttttatagtcataagctgattagcacaattctagacatccgcagctacatttaaggcaggaaggaggtggtaatagacactaccagccacatctgtcccttttaatcaggataccctagaaatcctcagcagactttgaattatgtgccattggtgaaatgtcatatgatcatccctctacaaggcaacgaggtaaaaagagaatttagtatttctagcctctagagtggagatgaacaaagaataggaatgggcatttgcttaggaaaccaactgtgccttacaacatttttgcacttttttctgtaacattttgtgttaaatcatataaaaatgctgatcctaacaaatatggtcaatgagtcacaccataattctctaagaactccagtccaaaaaggttaatcttgcttttaaactccaggcgcggtgtttcacagctgtaattttagcacttcgggaggcagagcaagaggatcacttgaggccaggagttggagaccagcctggcaacatagcaagaccccgtctctacaaaaaataaaattatctgggcctgttggtgcacacctgtagtcccagctactcaggaggctgaggtgggaggatcacttgagcctaggaattcgaggctgcagtgagctgtgattgcaccactgcactccagcctgggtgacagagggagaacctatctccaaaacaaaacaaaataaaaacaaaacaaaactccaagcagagaaagacttgacgagtcggatgagtctgatgattcctaaaggaaatcctttttgagattccaggagattccatctcctcaacagagtaattgattttgagcctcccacctcctgaattaaggcccacccatccctatcctgcactgaactgtagactcttttttacttccttacaaaagtttattcttaaatgtacaacagactccaagacgacactttattgtagctataggtggcaaaagatgttatggcagagaatccagatgtttaaataggaatggggtcaagggtcaccgccccaagcacggataacaaaatttattttttgccagatttctttaattccacctgtgactggtgagggctggtggcggggtggctttcacttttagctcctctttttgtttctgcttgaacgtcccatcttccttacccacccccttgacctgcttcttgagctttctcagggcttcttgccacctttgcagctgtacatggcacctgccatagggctctaattttaaactgagaaattgagaaaacaggaaactgactctttttggggggagagtaagacaaacaggaaaaggaaaatgaagacgtggttgatacagatcgttggatttcaaaaggaaaagtctacggataaccgaaaaaaataaatatttagaaatgcatagtcttggctggttaaataagtatccatgcttgttcttgtggcatagtagttacgagacatttttagttaaatggaaaaatgtgaattactatagtttgagtgatatgctgctttccaaattaaaagcagcataacaaaaacattcccctaatactcataaataattcattgaattggcaataattcacctcctaatgacttcatatgaagtataaagtaacttcgatacatcagaagaaatcctatcttctaatataagaaagtaatatgattacattaaatgcgtctcatataagttataaaaatggtatctatgagtaaagaaatgcttgtgaacaaaaaaattgatcttataaaggtcaaacaggccaggcgtggtggctcacacctgtaatcccagcactttgggaggctgaggtgggcggagtacctgaggtcaggagttcaagaccagcctggccaacatggtgataccctgtctctacaaaaatacaaaaaattagctgggcatgatggtgggtgcctgtaatctcagctactcgggaggcagaggcgggagaatcgcttgaacccgggaggcggaggttgcagtgaactgagattgagccacaacaaccaagcctgggagacagaggaaactctgtctcaaaaaataaaaaataaaaattaaaattaaaaaaaaggtcaaacaaaccaaacccttctgattaatttattcaatctacttttattataagcaaatgagaaattataattttaatctgaaaaagcagaatcaggggattttggagctggacagtcccctggaaattatttggatcaaagccctcattttataggtgaagaaactgagaagtaagatttgagcaagctgcccaaaggctttgccaaaggctataccagtgaatggcagagtctggactggaagtcccagtgctgccgtccaggtgagacctgttccactgcatgctactagctcccgggctgagaccggacttttgcttggcaggtttctttctttcgaaactattaattattgtattttttgtagagacagggttttgccatgatgcccaggctggtcttgaactcctgagctcaagagatccacccagcttggcctctcaaaaatgttgggattacaggcataagccacagtgcccggcccattttcctcccacctctttgttccttctctgtttcttttgcagcattatgttctatcattgtataccagagttcctcaacttcagttatagtctgttcttgctttatgctatcttcttcagcaagctcatcttggtctgttttcctccttatcaggcataccccagaaactcctgttttatctccacctcaactaaacattttcctgagttctgggcctctataaactaattatttgattaacatcttttttttttttttctgagatagagtctctctctgtcacccaggctggagtgcagtggtgcaatctcagatcactgcagcttctgcctcccagattcaagcgattctcctgcctcagcctcctaagtagctgggattataggcatgcaccaccgcacacagctaatttttgtacttttagtagagacggggtttcaccatgttggtcaggctggtctcaaactcctgatctgaagtgatctgactgcctcagcttcccaaagtgctgggattacaagcctgagccaccatgcctggccaacatctttaattggatatctcagtatcaagaaggcccataatattcctctgcctcatccctctcctcagtcctcttcttgtgtttcctagttcagagaatggcaccattctctatcaagctgcgcaaatcagacatgtgtgattttttgttgttgttgagacagggactcactctgtcacccaggctagagtgcagtggcgtgatcatggcgcactgaagcctcaaactcctgggctcaggagatcctcccgcctcagcctcctgagtagctgggaccacaggcccacaccaccatgcccagctaattttgtattctttgtagagatggggtttcatcatgtttgcccaggctggtctcgaactcctggactcaagcaatccacccacctcagcctcccaaagtgctgggattacaggcatgagccactgtgcccagctgaagtgtgatccttaacttcaccccttctcatgccctccatttccaatccatctccagtccagttgactccagctactcaattatttccacttatctcattccactacctttgaagctaccaccatctctaactacagtcatctcccaactaactggtctcctggcatctctctggttctcctccactaatttcaaaaaaagaaatttactgtgacagtgctcacaacactcccccttgctcttactaaagatgcttaccatagcctccaggtattgtatggcctgaggtctatctacatttccaggtgcaggacacaccatgtctccccactcccaaatttagtctccagactccatcctttttacagttctttaaaagcatcacaattcctccaaccactaggcatttgtatgtgctattccctctttccagaatgcaataccctccctctgcctagctagctaacttctatgtatctatgactgcagctcaaactttcctcatggactccctccacaagtgccaagcctgggccagattcttttgttatgtgctcacagaacgatgttccctttagcattcattgagtttgctgtttaattattcttgtcttgtttttgtttaattagtcctatctctaatactagacaaatgttccttaagatcacaggaaatataggactgtctctacataaaaactgttttatatccataatgcctaggacagtacctggcacacagtatatgctcaataaatttttgttgaatgaatgcaattatcattatattcctgatattagcaggtataatccagtttaagtttgggaacagaaagacaaaacggaccacatctaataaatccggtctcctttcttttattatttatttatttgagacagttttgctcttgttgcccaggctgcagtgcaatggcatgatcttggctcactgaaacctccgcctcccaagttcaagggattctccagcctcagcctcccaagtagctgggattacaggcatccaccaccacgcccagctaatttttttgtatttttagtagagatggggtttcaccatgttggccaggctggtctcgaactcctgacctcaggtgatccacccacctcagcctcccaaagtgttgggattacaggcgtgagccaccgtgcccggccaaggtctcctttcttttaatcaaactctcacctttggccattctgcagtcattcacccgacagtatttactgacggagtgaatacagagtgcttgattaatgttgctgctttgttattattattattattattgagatggagtcttgctctgttgcccaggctggagtgcagtggcgtgatctcggctcactgcaacctccgcctcccgggttcaagccattctcctgcctcagcctcccaagtagctgggactacaggcatgcaacaccacacctggctaatttttgtatttttagtagagacaaggtttcaccatattggccaggctggtcttgaactcctgacctcaggtgatctgcccacctcagcttcccaaagtgctgggattacaggcgtgagccaccatacccaacctaatgtttctgctttgaaatacaatttcaaaaagtcattaataggttgaaaacagcaagattttaaaagtattttaaaaagtgaaacagaagaatgcttacttcatttcacagagatagatttctcctttatgttatttctaaaaggagatggaattttgtttcattcatttctgcttatttggacaggccaaatatgaacagctgaacacgtcagcgttaccatgcatatgttacacagatgccatccttcttccatcagctctcatatgcaatacagaagtaaaaagaggttctctttatttttaaaaggtaaaaattgaaattcagtcacttaacacagaataaacaataattacaattacactggtaacaaaggacagcaagcatgttttctttgaaagcactgtatctggtttgtctccgtgcttggtcctagtatctggcatattttccccagagttttcttttcagtgggatgattatcttcggggcaaaaaagtttatcagactcaagttttagcagtacttattttattcatttatatacatgtaaccccatcctgtcttactccaatcttcttactgccttcctactgacacatatattatataacaccctccccaagttctatttacggttaaaaatttctttttttttttctttttttgagacagagtttcactctcgtcacccaggctggtgtgcaatggcgcagtctcggctcactgcaacctccgactccctggttcaagtgattctcctgtctcagcctcccgagtagctggaattacaggcgcccgccaccatgcccagctaatttttgtatttttagtagagacagtgtttcgccatgttggccaggctggtctcaaactcctgacctcaggtgatccacccgccttggcctctcaaagtgctgggattataggcgtaagccactgcgcccagcctacagttacgaatttctaaatggcacaaataaactcagctgttctcagtgcagacgtcaaatcctcactgtgctgaaacattttcctcagcttttgggaaataattacaatttaaacatacacagagaatgtttcttagacaaacataatacccgaggcttatctggtaaaaactaattgctctgtccttagcacaaaaaatatatatctttgtaaaatgagaagaaccaaagaatatttaaaacaaagaaggaagccacacgtactaattacacaagagactgactgacaaactggaattctccaaaacagattttcagcgaggcttctcatttcagagtccaggaaaaaaaaatcctaaaaaccccaaaggtatattatatgtgtgtatatatatttttattgtgttaaaaaacacaaaacataaaatttactgtcttatcaaaaggtatattttgtcgctcttccctttttttttttttttttttcccgagacagagtccagtctgtcgcccaggctgaagtgcagtggcatgatctcggctcactgcaacctgcatcttctgggctcaagcaatcctcccacctcagcctcctgagtagatggagctacaggcacgtgccactaggcccggctaatttttgtattttttgcagacagggttttgccatgttgcccgggctggtctttgttctcctaagagttgttttctccatgaaagttgataaataacatttagaaaatgaattattacaagagtaatgatatgtctcaatttattatatgaaattatcaacaactgcttttaatattcagatgtcaagaagatgaaaagcagaaatacattttgcaaacatgtagcactccataaatggaaatcatgtatttcctctaatatcccaatttttctatattgggatcttatatggctgtttctatatggctattttgtcccaacttgctgtacaagaattttccccagccaccttagaaaggttggatgtagttcactccaagtttgcagttcactccaagtgtttcagtaccacagaaagctccatggaagcctcaaatgtacgggctaggcaatagaagcagggaggtaggattaagaaattactggccaggtgtggtggctcaggcctgtaatcccagcacttcgagaggctgaggcagacagatggcttgagctcaagagtttgagatcagcctgagcaacatggcaaaactctgtctctacaaaaaatataaaaatcagccaggtatgttggtgtgcacctgtagtcccagctactggggaggttgaggcaggaggattgcttgagcccaggaggctgaggctgcagtgagccatgattgtgccactgcattccagcctggtcgactgtaagacaaaaaataagaaaataaaaaatttaccaatataaaatgctcaaacagctaacaaacatgttcaattccatttatagtcttttctttgagccatttaaacatagggctattttttttttttttttttgagatggagtttcactcttgttgcccaggctggagagcaatggcatgatctcggctcaccacaacctctgcctcctgggttcaagcgattctcctgcctcagcctcccgagcagctgggattacaggcatgtgccaccatgcctggctaattttgtatttttagtagagacgggattcctccatgttggtcagactggtcttgaactcccaacctcaggtgatctgcctgcctcaaccttccaaagtgctgggattacaggtgtgagccactgagattggctgccgttttgttttttaactccatatagtttctatagttcactgaaaactcaaagagatgacctataaatgtatgaataatgtatgatttcttacatcaattttctactagaaaaaaatcatacttttagaattggattttgtcttacagtcatctttattatactttataaatgagatttcatttatataaatcaggaagctaaactaaaatagaaacactagatttaaattctgatttgaatactctgatcaaaataacaaatctcacactgggaaaccatctatcagcaagcagagagctactgtgtgtccttccttagaagagtttgaacaccgagaacccacagcatatttgcagtacagtaacagcaattcctttgtcattatcacagaactttaattttcatatactttgctgggaccaaccaaaccatcccatatatataaccatatccatatatatatatatatatatcccacatatatatgggatggtatatatatacacatgtatatgtatgtgtgtgtgtatatatgtgtatatatgtatacacacacacacacacacatatatatatatatacacacacacacatatatatatggagagagagagagagacagtgtcttgctctgtcgcccaggctggagtgcagtggtacgatcttggctcattgcaacctccgcctcccaggctcaagcgattctcatgtctcagtctcccaagtagctgggattacaggtgtgcaccaccacaccaggctaaccattccatacattttatacaatcatttttaaaaagaagcatgaaccatttcggttttagagaattaagtttttttaaaaaagagactcttaaaaaaaagtcattatatgaataaaatctgctttgtgttaattccgacaaatcattccatcattgagtctgtcaccaattttttttttttgaaatggagtttcgctcttgttgcccaggctggagtgcaatggtacgatctcggctcactgcaaccgccgcctcccgggttcaagtgattctcctgcctcagcctcccgagtagctgggattacaggcatgcgccaccacgcctggctaattttgtattattagttgagacagggtttctccatgttggtcaggctggtctcgaactcctgacctcaagtgatccgctggccttggcctcccaaagtgctgggattacaggcgtgagccaccgtgcctggcccaattttttttttttaataacttgcacacttaacaatattttttatcttcttgggacaacattcttttctccacaaaaacccaattaaggacgttgtgccagtttactcctacttccttcctgttcactgagcttaaagtgggtataggcgagaatgccaaataatgtacataaaatgccaagggcctgattaatggacagtggatccttaaataaaacatatcctccgaataaagtaatgcagaacttgaagtgtccgaacatgttataggtgacaggtgaagtgttcccaatgatccaataaattgataagttcaccatgaaagctattactccagatagcagcaccataagcaaagcagaaactgaccagggaccaaatattcctccttctccaaacactggctcaaagaagggcacagcaaccagcaacatggcagatgacatcggagcctggtagtacagcagctgcattgagttcacttgtaattcatgctgtttggctcctacccaaaacaggtaggtatttggtgagcatcacacacccaagtttctctgtctcctttcttctcttcaccttgagtcagacaacttatgcaattatgctttcttcccaacagtctattgtctctatactgtattttctaaaccttggaatacagcttcaaaatttatgaaatctgcagcgtgagctggattctggtggagaaggttttctggtagcagaaggtctggatggctatgatcaccggcgtggtcatggccttggccagctgataggtgcctatggtgttgttctgcagagaaaggttagtgaagaccacaaagccacagaagctgagggccaggaggaggagcctggagggcggcagacttttgggggcaaagatgtccagcttctggcagatatacaagcccagccaggtgaccacgaagtgcaccagggtcaggctcatgttggggaagccgtggtacacataaatccatttgttgaggaacacaatgcagatggacaccagcaggttgaacaggagcccggcggcgattcgccagtggccccgcactcggtccaccagcaatgccatgatccccgcgaagctggggccgtctagcctcggaaggggcgccgggcctgtctccggctgcccttctactccaccgccgcgtcctcgcagacgccgacctcaccgtctgacccaggagtggcatgcacagatcaaccccgggcgagtagcactcttaacagaggacacacaccccgccgccgccctgtaagccagctaggac

SEQ ID NO: 11650 - RNA, 16086 nt, Homo sapiens
  source 1..16086: mol_type = other RNA
ctgaatagctgggactacaggtgtctaccaccatgcccggctaattttataaaattttttatagagacgggggtcttgctgtgttgctcaggtcttgaactcctggcctcaagtgcacctcctgccttggcctcccaaaacactgggattacagatgcaggccactgtacctggcccccatatttattaatcacattttattcattcattcatttaactttcctgtgaagttttgcaaatggcttcctcaattcccccttgttaagctttttttccttctcaaaccatgcttatatcctttctggttccagccacatattttgggtcagacagtcctagcactgtacttttaatatcacctggagtgacttcagagacttctttgaagccacaagaccatctggttcaataccaatattttgaaatctaatgactcactattctagaacattctcaacattaagtttcttaaagatggcttaaatactttttaaatttaaataaatgtacagaaaacaaaaatcttttcatttaaaacctaccaaatatagccacacatggtagggcatacctatagtcccagttactcaggaggctgaggcaggaggattacttgagccaaggagttcagggctgcagtgcactatgattgtgcctgcaaaaaggcactgcactccagcgtcggccacagagaaagacctagttttttgtttttgtttttgtttttgagacagagtcttgttctgtcgcccaggctggaatgcagtctggagtgcagtggctcattgcaacctccacctcctgggttcaagcaattctcctgcctcagcctcctgagtagctgggattacaggggcacaccaccacgcccaactaacttttgtatttttagtagagatggagtttcgccatgttggccaggttggtctcaaactcctgggctcaagtgattcacctaccttggcctcccaaagtgctgggattacaggcgtgagccactgcatccagccataagactcagtttcttttcttttttttttttggagatggagttttgctcttttgtccaggctggagtgaagtggtgcgaccatggttcactgcaacctctaccctcccggttcaagcaattctcctgcctcagcctcccaagtagctgggattataggcacccactactacgcccagctaatttttgtatttttagtagagacgaggtttcgccatgttggctaggctggtctcaaactcctgacctcaggtgatccacccgcttcggccttgcaaagtgctgagattacaggcatgagtcaccacgcctggccggcaagaccctgtttctaaaaaacaaaataaaaaataaatcttccaactatttataatatgatctctgttcatctttactgttataaacattcctcaggtacttgaaaggagtgtgtgttctaggcttgttgagtacagataacctattagacaaggttactaacttccctgctgcctgctctatcacctctattagaagtatttaaaatctcaattttccttttaattttcatgctgttttctgggttgttcatgattgctatgtttgtggtggattgttctttaaaaaaaaaaatcttgatcctattaacactttttgcctcaaattctattttgtctgctattgatattactacccaaaatccccgcaccccgcccttttttttgagacaggatctcactctgtcactcaagctggagtgcagttcaccatcacggtggctcattgcagcctcgacctccctgggcttgggtgatcctcccacctcagcctcccgagtagctgggatcacaggcacataccaccatacctggctaatttttgtactttttatagagacggggattcaccatgttggccaggctggtcttaaactcctgatctcaagtgatccgcccaccttggcctcccaaagtgctgggattataggcatgagccaccacacccagccggcagcaaactgtttatggactggtactggggcccagaccctaccttgagtggtactgggctagaggacttattaattgcatgatctaggagtagttcataaattctgtgatggtcattctttgggtgaactccatttctagcagattctagataagcagcatgacttcctctgattctctgacacctgagggtggggaaattcagactgtcccacttgggttgtgcgtcttcacgctggggaagagggtgaggccaaagttgtgttgggagataaataatgaaattcaagaactccatggtaacagcccttgtctttcctctctggggccacacagtgcagtgtggggagaggagtggacagaaggaatgtcagcatttccttggcaaaatctcttgcgtttcagaacagcagtgagattttggaggtatgagagagtcacaggtgtgacattcctgtgaggaatgctatttgagtacaagcagtggatgtcctcatgatgttatgatttcagaagaatagcactgtgcttggctgaaaagttctgcattcaataactccatgccaataagcagccatttcctcccagcacacagttgctcaccaatgtccatggtcctatggcactgggaggcctctgatgcagctgtctcccactatggtcttaggaaattcctggaacgttattagagtgagtttttcctagatctgcttactgaatacctgttgaactttcacactgatggccagttccaagacttaagcatgaccttgcgaccattggtgatagtgctttcttgatctgctgaatcaaattgaagcagaactgggggtactactaggaatgaggggtgactagggatggggctggggcgaggggtatattgggtaactgaggatgaccagtgtcagagagcacaaagatgatggtgaagggcaggtagaccacctcccacttggtgggaaagtctgttcctggctggaactggttcattcattccaagccagcaacagctccaggtttggacgccatttatgaatctacatgccaccagaccagtccctgtcttccacacaccccactctctggagtctggaaaaatggcgggggtggggctagctactagtttttgtttttttttttctttttgagacacagtttcattctgtcatccaggctggagtgcagtggcatgatctcagctcactgcaacctccgcctcccaggttcaagcgattctcgtgccttagctttcagagtagctgggactacaggtgcacaccatcacagctgactaatttttcttttctttttttttttttgagacggagtctcactctgtctcccaggctggagtgcagtgatgtgatctcagctcactgcaacctacgtctccagggttcatgtgagtttcctgcctcagcctcctgagtgagtagctgggattacaggcgcctgccaccacgtccagctaatttttgtatttttagtagagattgggtttcaccatgttggccaggctggtctccaactcctgacctcaagtgatccacctgcctcggcctcccaaatcgctgggattacaggcgtgagtcatcatgcctggccttttttttttttttgtgagacagagttttgctcttgtcacccaggctggagtgtaatggcatgatctcggctcactgaaacctctgccaggcacacgtcaccatgcccggctaatttttgtatttttggtagaaacggggtttcaccatgttggccaggctggtctccaactcctgacctcaagtgatcctcctgccttggcctcccaaagtgctgggattacaggtgttagctaccaagtctggcctttttttttttttttttttttttttttttttgagacagagtttcgctcttgtcacccaggctggagtgtaatagtgtgattccagcttactgcaacctctgcctctcgggttcaagccattctcctgcctcagcctcctgagcagctgggattacaggcacacgccagcatgcctggctaatttttatatttttagtagagacggggtttcaccatgttggccaggctggtctcgaactcctgacctcaggtgatccatctgcctcagcctcccaaactgctgggatgacaggcgtgagccaccacgccaggccctatttttatttttaaccagtgctgtagtttgaatatttgtctcctccaaaactcatctggaaacatccccaatgtggcaatattgagagatggcgcctttaaaaggtgactgggtcatgaaggctctgcccagtgagactggtgcctttataagaagaggaagagagacctgagctaccatgctcaagtccctcaccacgtgaggccctctgccaccttgggtctctgcagagagttcccaggaacaagaagtctctcaccagatgtggaccctgtaccttggacttctcagtctccactattgtaagaaataaattccttttctttataaatgacccagtttcaggtattctgttctatgcaacacaaaatggactaagacaacgagtacgcttagttgttgcttcctgagttccaaagtccgacagacagagcaggtcctccattcttgcccctttttaccccaaatgctcattggcattcttgcagctacgagtaataattaaaagtggctaagccaggctggcatggttgctcacgcctgtaatatcagcactttgggaggctgaggcaggaggatcacttgaacccaggagtgagaccagccagggcaacatagcaacaccctgtctctaattattattatttttttaagtgagtaagccaaataggggtttacttttcatctagaacaagaagacgtgttggccaggctggtctcaaactactgggctcaagtgatccacccacctcagcctcccaaagtgttgggattatgcgtgagccaccgcacctggccacaagacccaatttcttttattttatctttttttttttttttttaagagatagggcatctaacggcattgttttagctgctcaacacttttttttttttgcttatttttgtttgttttgtttgtttttgagacagggtctccctctgttgcccagcatatagtgcagtggcatgatcatggctcactgcagcctcaacctcccaggatcaggcaatcctcctgcttcagcttcctgagtagctgagaccacaggtgcacaccaatatacctaatttttttttttttgagatggagtttcactcttgttgcccaggctggagtgcaatggcgtggtctcagctcactgcaacctctgcctccctggttcaagcgattctcctgtctcagcctgccgagtagctggggttacaggcataagccactacgcccagctaattttgtatttttagtagagacagggtttctccatgttggtcaggctggtctcgaactcctgacctcaggtgatccacccacctcagccttccaaagtgctgagattgcaggtgtgaaccactacgcctggccacctgactaatttttaagttattcacagagaacaggttttgcaatgttgcccaggctggtctcaaactcctgggctcaaatgatcctcctccctcggcctcccaaagtgctggggttacaggtgtgccactgtgcctggtcggctcaccactttcagatctggctctcttcacctctcttttatagtcataagctgattagcacaattctagacatccgcagctacatttaaggcaggaaggaggtggtaatagacactaccagccacatctgtcccttttaatcaggataccctagaaatcctcagcagactttgaattatgtgccattggtgaaatgtcatatgatcatccctctacaaggcaacgaggtaaaaagagaatttagtatttctagcctctagagtggagatgaacaaagaataggaatgggcatttgcttaggaaaccaactgtgccttacaacatttttgcacttttttctgtaacattttgtgttaaatcatataaaaatgctgatcctaacaaatatggtcaatgagtcacaccataattctctaagaactccagtccaaaaaggttaatcttgcttttaaactccaggcgcggtgtttcacagctgtaattttagcacttcgggaggcagagcaagaggatcacttgaggccaggagttggagaccagcctggcaacatagcaagaccccgtctctacaaaaaataaaattatctgggcctgttggtgcacacctgtagtcccagctactcaggaggctgaggtgggaggatcacttgagcctaggaattcgaggctgcagtgagctgtgattgcaccactgcactccagcctgggtgacagagggagaacctatctccaaaacaaaacaaaataaaaacaaaacaaaactccaagcagagaaagacttgacgagtcggatgagtctgatgattcctaaaggaaatcctttttgagattccaggagattccatctcctcaacagagtaattgattttgagcctcccacctcctgaattaaggcccacccatccctatcctgcactgaactgtagactcttttttacttccttacaaaagtttattcttaaatgtacaacagactccaagacgacactttattgtagctataggtggcaaaagatgttatggcagagaatccagatgtttaaataggaatggggtcaagggtcaccgccccaagcacggataacaaaatttattttttgccagatttctttaattccacctgtgactggtgagggctggtggcggggtggctttcacttttagctcctctttttgtttctgcttgaacgtcccatcttccttacccacccccttgacctgcttcttgagctttctcagggcttcttgccacctttgcagctgtacatggcacctgccatagggctctaattttaaactgagaaattgagaaaacaggaaactgactctttttggggggagagtaagacaaacaggaaaaggaaaatgaagacgtggttgatacagatcgttggatttcaaaaggaaaagtctacggataaccgaaaaaaataaatatttagaaatgcatagtcttggctggttaaataagtatccatgcttgttcttgtggcatagtagttacgagacatttttagttaaatggaaaaatgtgaattactatagtttgagtgatatgctgctttccaaattaaaagcagcataacaaaaacattcccctaatactcataaataattcattgaattggcaataattcacctcctaatgacttcatatgaagtataaagtaacttcgatacatcagaagaaatcctatcttctaatataagaaagtaatatgattacattaaatgcgtctcatataagttataaaaatggtatctatgagtaaagaaatgcttgtgaacaaaaaaattgatcttataaaggtcaaacaggccaggcgtggtggctcacacctgtaatcccagcactttgggaggctgaggtgggcggagtacctgaggtcaggagttcaagaccagcctggccaacatggtgataccctgtctctacaaaaatacaaaaaattagctgggcatgatggtgggtgcctgtaatctcagctactcgggaggcagaggcgggagaatcgcttgaacccgggaggcggaggttgcagtgaactgagattgagccacaacaaccaagcctgggagacagaggaaactctgtctcaaaaaataaaaaataaaaattaaaattaaaaaaaaggtcaaacaaaccaaacccttctgattaatttattcaatctacttttattataagcaaatgagaaattataattttaatctgaaaaagcagaatcaggggattttggagctggacagtcccctggaaattatttggatcaaagccctcattttataggtgaagaaactgagaagtaagatttgagcaagctgcccaaaggctttgccaaaggctataccagtgaatggcagagtctggactggaagtcccagtgctgccgtccaggtgagacctgttccactgcatgctactagctcccgggctgagaccggacttttgcttggcaggtttctttctttcgaaactattaattattgtattttttgtagagacagggttttgccatgatgcccaggctggtcttgaactcctgagctcaagagatccacccagcttggcctctcaaaaatgttgggattacaggcataagccacagtgcccggcccattttcctcccacctctttgttccttctctgtttcttttgcagcattatgttctatcattgtataccagagttcctcaacttcagttatagtctgttcttgctttatgctatcttcttcagcaagctcatcttggtctgttttcctccttatcaggcataccccagaaactcctgttttatctccacctcaactaaacattttcctgagttctgggcctctataaactaattatttgattaacatcttttttttttttttctgagatagagtctctctctgtcacccaggctggagtgcagtggtgcaatctcagatcactgcagcttctgcctcccagattcaagcgattctcctgcctcagcctcctaagtagctgggattataggcatgcaccaccgcacacagctaatttttgtacttttagtagagacggggtttcaccatgttggtcaggctggtctcaaactcctgatctgaagtgatctgactgcctcagcttcccaaagtgctgggattacaagcctgagccaccatgcctggccaacatctttaattggatatctcagtatcaagaaggcccataatattcctctgcctcatccctctcctcagtcctcttcttgtgtttcctagttcagagaatggcaccattctctatcaagctgcgcaaatcagacatgtgtgattttttgttgttgttgagacagggactcactctgtcacccaggctagagtgcagtggcgtgatcatggcgcactgaagcctcaaactcctgggctcaggagatcctcccgcctcagcctcctgagtagctgggaccacaggcccacaccaccatgcccagctaattttgtattctttgtagagatggggtttcatcatgtttgcccaggctggtctcgaactcctggactcaagcaatccacccacctcagcctcccaaagtgctgggattacaggcatgagccactgtgcccagctgaagtgtgatccttaacttcaccccttctcatgccctccatttccaatccatctccagtccagttgactccagctactcaattatttccacttatctcattccactacctttgaagctaccaccatctctaactacagtcatctcccaactaactggtctcctggcatctctctggttctcctccactaatttcaaaaaaagaaatttactgtgacagtgctcacaacactcccccttgctcttactaaagatgcttaccatagcctccaggtattgtatggcctgaggtctatctacatttccaggtgcaggacacaccatgtctccccactcccaaatttagtctccagactccatcctttttacagttctttaaaagcatcacaattcctccaaccactaggcatttgtatgtgctattccctctttccagaatgcaataccctccctctgcctagctagctaacttctatgtatctatgactgcagctcaaactttcctcatggactccctccacaagtgccaagcctgggccagattcttttgttatgtgctcacagaacgatgttccctttagcattcattgagtttgctgtttaattattcttgtcttgtttttgtttaattagtcctatctctaatactagacaaatgttccttaagatcacaggaaatataggactgtctctacataaaaactgttttatatccataatgcctaggacagtacctggcacacagtatatgctcaataaatttttgttgaatgaatgcaattatcattatattcctgatattagcaggtataatccagtttaagtttgggaacagaaagacaaaacggaccacatctaataaatccggtctcctttcttttattatttatttatttgagacagttttgctcttgttgcccaggctgcagtgcaatggcatgatcttggctcactgaaacctccgcctcccaagttcaagggattctccagcctcagcctcccaagtagctgggattacaggcatccaccaccacgcccagctaatttttttgtatttttagtagagatggggtttcaccatgttggccaggctggtctcgaactcctgacctcaggtgatccacccacctcagcctcccaaagtgttgggattacaggcgtgagccaccgtgcccggccaaggtctcctttcttttaatcaaactctcacctttggccattctgcagtcattcacccgacagtatttactgacggagtgaatacagagtgcttgattaatgttgctgctttgttattattattattattattgagatggagtcttgctctgttgcccaggctggagtgcagtggcgtgatctcggctcactgcaacctccgcctcccgggttcaagccattctcctgcctcagcctcccaagtagctgggactacaggcatgcaacaccacacctggctaatttttgtatttttagtagagacaaggtttcaccatattggccaggctggtcttgaactcctgacctcaggtgatctgcccacctcagcttcccaaagtgctgggattacaggcgtgagccaccatacccaacctaatgtttctgctttgaaatacaatttcaaaaagtcattaataggttgaaaacagcaagattttaaaagtattttaaaaagtgaaacagaagaatgcttacttcatttcacagagatagatttctcctttatgttatttctaaaaggagatggaattttgtttcattcatttctgcttatttggacaggccaaatatgaacagctgaacacgtcagcgttaccatgcatatgttacacagatgccatccttcttccatcagctctcatatgcaatacagaagtaaaaagaggttctctttatttttaaaaggtaaaaattgaaattcagtcacttaacacagaataaacaataattacaattacactggtaacaaaggacagcaagcatgttttctttgaaagcactgtatctggtttgtctccgtgcttggtcctagtatctggcatattttccccagagttttcttttcagtgggatgattatcttcggggcaaaaaagtttatcagactcaagttttagcagtacttattttattcatttatatacatgtaaccccatcctgtcttactccaatcttcttactgccttcctactgacacatatattatataacaccctccccaagttctatttacggttaaaaatttctttttttttttctttttttgagacagagtttcactctcgtcacccaggctggtgtgcaatggcgcagtctcggctcactgcaacctccgactccctggttcaagtgattctcctgtctcagcctcccgagtagctggaattacaggcgcccgccaccatgcccagctaatttttgtatttttagtagagacagtgtttcgccatgttggccaggctggtctcaaactcctgacctcaggtgatccacccgccttggcctctcaaagtgctgggattataggcgtaagccactgcgcccagcctacagttacgaatttctaaatggcacaaataaactcagctgttctcagtgcagacgtcaaatcctcactgtgctgaaacattttcctcagcttttgggaaataattacaatttaaacatacacagagaatgtttcttagacaaacataatacccgaggcttatctggtaaaaactaattgctctgtccttagcacaaaaaatatatatctttgtaaaatgagaagaaccaaagaatatttaaaacaaagaaggaagccacacgtactaattacacaagagactgactgacaaactggaattctccaaaacagattttcagcgaggcttctcatttcagagtccaggaaaaaaaaatcctaaaaaccccaaaggtatattatatgtgtgtatatatatttttattgtgttaaaaaacacaaaacataaaatttactgtcttatcaaaaggtatattttgtcgctcttccctttttttttttttttttttcccgagacagagtccagtctgtcgcccaggctgaagtgcagtggcatgatctcggctcactgcaacctgcatcttctgggctcaagcaatcctcccacctcagcctcctgagtagatggagctacaggcacgtgccactaggcccggctaatttttgtattttttgcagacagggttttgccatgttgcccgggctggtctttgttctcctaagagttgttttctccatgaaagttgataaataacatttagaaaatgaattattacaagagtaatgatatgtctcaatttattatatgaaattatcaacaactgcttttaatattcagatgtcaagaagatgaaaagcagaaatacattttgcaaacatgtagcactccataaatggaaatcatgtatttcctctaatatcccaatttttctatattgggatcttatatggctgtttctatatggctattttgtcccaacttgctgtacaagaattttccccagccaccttagaaaggttggatgtagttcactccaagtttgcagttcactccaagtgtttcagtaccacagaaagctccatggaagcctcaaatgtacgggctaggcaatagaagcagggaggtaggattaagaaattactggccaggtgtggtggctcaggcctgtaatcccagcacttcgagaggctgaggcagacagatggcttgagctcaagagtttgagatcagcctgagcaacatggcaaaactctgtctctacaaaaaatataaaaatcagccaggtatgttggtgtgcacctgtagtcccagctactggggaggttgaggcaggaggattgcttgagcccaggaggctgaggctgcagtgagccatgattgtgccactgcattccagcctggtcgactgtaagacaaaaaataagaaaataaaaaatttaccaatataaaatgctcaaacagctaacaaacatgttcaattccatttatagtcttttctttgagccatttaaacatagggctattttttttttttttttttgagatggagtttcactcttgttgcccaggctggagagcaatggcatgatctcggctcaccacaacctctgcctcctgggttcaagcgattctcctgcctcagcctcccgagcagctgggattacaggcatgtgccaccatgcctggctaattttgtatttttagtagagacgggattcctccatgttggtcagactggtcttgaactcccaacctcaggtgatctgcctgcctcaaccttccaaagtgctgggattacaggtgtgagccactgagattggctgccgttttgttttttaactccatatagtttctatagttcactgaaaactcaaagagatgacctataaatgtatgaataatgtatgatttcttacatcaattttctactagaaaaaaatcatacttttagaattggattttgtcttacagtcatctttattatactttataaatgagatttcatttatataaatcaggaagctaaactaaaatagaaacactagatttaaattctgatttgaatactctgatcaaaataacaaatctcacactgggaaaccatctatcagcaagcagagagctactgtgtgtccttccttagaagagtttgaacaccgagaacccacagcatatttgcagtacagtaacagcaattcctttgtcattatcacagaactttaattttcatatactttgctgggaccaaccaaaccatcccatatatataaccatatccatatatatatatatatatatcccacatatatatgggatggtatatatatacacatgtatatgtatgtgtgtgtgtatatatgtgtatatatgtatacacacacacacacacacatatatatatatatacacacacacacatatatatatggagagagagagagagacagtgtcttgctctgtcgcccaggctggagtgcagtggtacgatcttggctcattgcaacctccgcctcccaggctcaagcgattctcatgtctcagtctcccaagtagctgggattacaggtgtgcaccaccacaccaggctaaccattccatacattttatacaatcatttttaaaaagaagcatgaaccatttcggttttagagaattaagtttttttaaaaaagagactcttaaaaaaaagtcattatatgaataaaatctgctttgtgttaattccgacaaatcattccatcattgagtctgtcaccaattttttttttttgaaatggagtttcgctcttgttgcccaggctggagtgcaatggtacgatctcggctcactgcaaccgccgcctcccgggttcaagtgattctcctgcctcagcctcccgagtagctgggattacaggcatgcgccaccacgcctggctaattttgtattattagttgagacagggtttctccatgttggtcaggctggtctcgaactcctgacctcaagtgatccgctggccttggcctcccaaagtgctgggattacaggcgtgagccaccgtgcctggcccaattttttttttttaataacttgcacacttaacaatattttttatcttcttgggacaacattcttttctccacaaaaacccaattaaggacgttgtgccagtttactcctacttccttcctgttcactgagcttaaagtgggtataggcgagaatgccaaataatgtacataaaatgccaagggcctgattaatggacagtggatccttaaataaaacatatcctccgaataaagtaatgcagaacttgaagtgtccgaacatgttataggtgacaggtgaagtgttcccaatgatccaataaattgataagttcaccatgaaagctattactccagatagcagcaccataagcaaagcagaaactgaccagggaccaaatattcctccttctccaaacactggctcaaagaagggcacagcaaccagcaacatggcagatgacatcggagcctggtagtacagcagctgcattgagttcacttgtaattcatgctgtttggctcctacccacacttgataaagggatgtaactaaaacaccaagagcagcaaacaccattccaaggaaattaaacttcacatcgtaataagaatttaggattacacctaaagttataggaatcagcgtgagctggattctggtggagaaggttttctggtagcagaaggtctggatggctatgatcaccggcgtggtcatggccttggccagctgataggtgcctatggtgttgttctgcagagaaaggttagtgaagaccacaaagccacagaagctgagggccaggaggaggagcctggagggcggcagacttttgggggcaaagatgtccagcttctggcagatatacaagcccagccaggtgaccacgaagtgcaccagggtcaggctcatgttggggaagccgtggtacacataaatccatttgttgaggaacacaatgcagatggacaccagcaggttgaacaggagcccggcggcgattcgccagtggccccgcactcggtccaccagcaatgccatgatccccgcgaagctggggccgtctagcctcggaaggggcgccgggcctgtctccggctgcccttctactccaccgccgcgtcctcgcagacgccgacctcaccgtctgacccaggagtggcatgcacagatcaaccccgggcgagtagcactcttaacagaggacacacaccccgccgccgccctgtaagccagctaggac

SEQ ID NO: 11651 - RNA, 15975 nt, Homo sapiens
  source 1..15975: mol_type = other RNA
ctgaatagctgggactacaggtgtctaccaccatgcccggctaattttataaaattttttatagagacgggggtcttgctgtgttgctcaggtcttgaactcctggcctcaagtgcacctcctgccttggcctcccaaaacactgggattacagatgcaggccactgtacctggcccccatatttattaatcacattttattcattcattcatttaactttcctgtgaagttttgcaaatggcttcctcaattcccccttgttaagctttttttccttctcaaaccatgcttatatcctttctggttccagccacatattttgggtcagacagtcctagcactgtacttttaatatcacctggagtgacttcagagacttctttgaagccacaagaccatctggttcaataccaatattttgaaatctaatgactcactattctagaacattctcaacattaagtttcttaaagatggcttaaatactttttaaatttaaataaatgtacagaaaacaaaaatcttttcatttaaaacctaccaaatatagccacacatggtagggcatacctatagtcccagttactcaggaggctgaggcaggaggattacttgagccaaggagttcagggctgcagtgcactatgattgtgcctgcaaaaaggcactgcactccagcgtcggccacagagaaagacctagttttttgtttttgtttttgtttttgagacagagtcttgttctgtcgcccaggctggaatgcagtctggagtgcagtggctcattgcaacctccacctcctgggttcaagcaattctcctgcctcagcctcctgagtagctgggattacaggggcacaccaccacgcccaactaacttttgtatttttagtagagatggagtttcgccatgttggccaggttggtctcaaactcctgggctcaagtgattcacctaccttggcctcccaaagtgctgggattacaggcgtgagccactgcatccagccataagactcagtttcttttcttttttttttttggagatggagttttgctcttttgtccaggctggagtgaagtggtgcgaccatggttcactgcaacctctaccctcccggttcaagcaattctcctgcctcagcctcccaagtagctgggattataggcacccactactacgcccagctaatttttgtatttttagtagagacgaggtttcgccatgttggctaggctggtctcaaactcctgacctcaggtgatccacccgcttcggccttgcaaagtgctgagattacaggcatgagtcaccacgcctggccggcaagaccctgtttctaaaaaacaaaataaaaaataaatcttccaactatttataatatgatctctgttcatctttactgttataaacattcctcaggtacttgaaaggagtgtgtgttctaggcttgttgagtacagataacctattagacaaggttactaacttccctgctgcctgctctatcacctctattagaagtatttaaaatctcaattttccttttaattttcatgctgttttctgggttgttcatgattgctatgtttgtggtggattgttctttaaaaaaaaaaatcttgatcctattaacactttttgcctcaaattctattttgtctgctattgatattactacccaaaatccccgcaccccgcccttttttttgagacaggatctcactctgtcactcaagctggagtgcagttcaccatcacggtggctcattgcagcctcgacctccctgggcttgggtgatcctcccacctcagcctcccgagtagctgggatcacaggcacataccaccatacctggctaatttttgtactttttatagagacggggattcaccatgttggccaggctggtcttaaactcctgatctcaagtgatccgcccaccttggcctcccaaagtgctgggattataggcatgagccaccacacccagccggcagcaaactgtttatggactggtactggggcccagaccctaccttgagtggtactgggctagaggacttattaattgcatgatctaggagtagttcataaattctgtgatggtcattctttgggtgaactccatttctagcagattctagataagcagcatgacttcctctgattctctgacacctgagggtggggaaattcagactgtcccacttgggttgtgcgtcttcacgctggggaagagggtgaggccaaagttgtgttgggagataaataatgaaattcaagaactccatggtaacagcccttgtctttcctctctggggccacacagtgcagtgtggggagaggagtggacagaaggaatgtcagcatttccttggcaaaatctcttgcgtttcagaacagcagtgagattttggaggtatgagagagtcacaggtgtgacattcctgtgaggaatgctatttgagtacaagcagtggatgtcctcatgatgttatgatttcagaagaatagcactgtgcttggctgaaaagttctgcattcaataactccatgccaataagcagccatttcctcccagcacacagttgctcaccaatgtccatggtcctatggcactgggaggcctctgatgcagctgtctcccactatggtcttaggaaattcctggaacgttattagagtgagtttttcctagatctgcttactgaatacctgttgaactttcacactgatggccagttccaagacttaagcatgaccttgcgaccattggtgatagtgctttcttgatctgctgaatcaaattgaagcagaactgggggtactactaggaatgaggggtgactagggatggggctggggcgaggggtatattgggtaactgaggatgaccagtgtcagagagcacaaagatgatggtgaagggcaggtagaccacctcccacttggtgggaaagtctgttcctggctggaactggttcattcattccaagccagcaacagctccaggtttggacgccatttatgaatctacatgccaccagaccagtccctgtcttccacacaccccactctctggagtctggaaaaatggcgggggtggggctagctactagtttttgtttttttttttctttttgagacacagtttcattctgtcatccaggctggagtgcagtggcatgatctcagctcactgcaacctccgcctcccaggttcaagcgattctcgtgccttagctttcagagtagctgggactacaggtgcacaccatcacagctgactaatttttcttttctttttttttttttgagacggagtctcactctgtctcccaggctggagtgcagtgatgtgatctcagctcactgcaacctacgtctccagggttcatgtgagtttcctgcctcagcctcctgagtgagtagctgggattacaggcgcctgccaccacgtccagctaatttttgtatttttagtagagattgggtttcaccatgttggccaggctggtctccaactcctgacctcaagtgatccacctgcctcggcctcccaaatcgctgggattacaggcgtgagtcatcatgcctggccttttttttttttttgtgagacagagttttgctcttgtcacccaggctggagtgtaatggcatgatctcggctcactgaaacctctgccaggcacacgtcaccatgcccggctaatttttgtatttttggtagaaacggggtttcaccatgttggccaggctggtctccaactcctgacctcaagtgatcctcctgccttggcctcccaaagtgctgggattacaggtgttagctaccaagtctggcctttttttttttttttttttttttttttttttgagacagagtttcgctcttgtcacccaggctggagtgtaatagtgtgattccagcttactgcaacctctgcctctcgggttcaagccattctcctgcctcagcctcctgagcagctgggattacaggcacacgccagcatgcctggctaatttttatatttttagtagagacggggtttcaccatgttggccaggctggtctcgaactcctgacctcaggtgatccatctgcctcagcctcccaaactgctgggatgacaggcgtgagccaccacgccaggccctatttttatttttaaccagtgctgtagtttgaatatttgtctcctccaaaactcatctggaaacatccccaatgtggcaatattgagagatggcgcctttaaaaggtgactgggtcatgaaggctctgcccagtgagactggtgcctttataagaagaggaagagagacctgagctaccatgctcaagtccctcaccacgtgaggccctctgccaccttgggtctctgcagagagttcccaggaacaagaagtctctcaccagatgtggaccctgtaccttggacttctcagtctccactattgtaagaaataaattccttttctttataaatgacccagtttcaggtattctgttctatgcaacacaaaatggactaagacaacgagtacgcttagttgttgcttcctgagttccaaagtccgacagacagagcaggtcctccattcttgcccctttttaccccaaatgctcattggcattcttgcagctacgagtaataattaaaagtggctaagccaggctggcatggttgctcacgcctgtaatatcagcactttgggaggctgaggcaggaggatcacttgaacccaggagtgagaccagccagggcaacatagcaacaccctgtctctaattattattatttttttaagtgagtaagccaaataggggtttacttttcatctagaacaagaagacgtgttggccaggctggtctcaaactactgggctcaagtgatccacccacctcagcctcccaaagtgttgggattatgcgtgagccaccgcacctggccacaagacccaatttcttttattttatctttttttttttttttttaagagatagggcatctaacggcattgttttagctgctcaacacttttttttttttgcttatttttgtttgttttgtttgtttttgagacagggtctccctctgttgcccagcatatagtgcagtggcatgatcatggctcactgcagcctcaacctcccaggatcaggcaatcctcctgcttcagcttcctgagtagctgagaccacaggtgcacaccaatatacctaatttttttttttttgagatggagtttcactcttgttgcccaggctggagtgcaatggcgtggtctcagctcactgcaacctctgcctccctggttcaagcgattctcctgtctcagcctgccgagtagctggggttacaggcataagccactacgcccagctaattttgtatttttagtagagacagggtttctccatgttggtcaggctggtctcgaactcctgacctcaggtgatccacccacctcagccttccaaagtgctgagattgcaggtgtgaaccactacgcctggccacctgactaatttttaagttattcacagagaacaggttttgcaatgttgcccaggctggtctcaaactcctgggctcaaatgatcctcctccctcggcctcccaaagtgctggggttacaggtgtgccactgtgcctggtcggctcaccactttcagatctggctctcttcacctctcttttatagtcataagctgattagcacaattctagacatccgcagctacatttaaggcaggaaggaggtggtaatagacactaccagccacatctgtcccttttaatcaggataccctagaaatcctcagcagactttgaattatgtgccattggtgaaatgtcatatgatcatccctctacaaggcaacgaggtaaaaagagaatttagtatttctagcctctagagtggagatgaacaaagaataggaatgggcatttgcttaggaaaccaactgtgccttacaacatttttgcacttttttctgtaacattttgtgttaaatcatataaaaatgctgatcctaacaaatatggtcaatgagtcacaccataattctctaagaactccagtccaaaaaggttaatcttgcttttaaactccaggcgcggtgtttcacagctgtaattttagcacttcgggaggcagagcaagaggatcacttgaggccaggagttggagaccagcctggcaacatagcaagaccccgtctctacaaaaaataaaattatctgggcctgttggtgcacacctgtagtcccagctactcaggaggctgaggtgggaggatcacttgagcctaggaattcgaggctgcagtgagctgtgattgcaccactgcactccagcctgggtgacagagggagaacctatctccaaaacaaaacaaaataaaaacaaaacaaaactccaagcagagaaagacttgacgagtcggatgagtctgatgattcctaaaggaaatcctttttgagattccaggagattccatctcctcaacagagtaattgattttgagcctcccacctcctgaattaaggcccacccatccctatcctgcactgaactgtagactcttttttacttccttacaaaagtttattcttaaatgtacaacagactccaagacgacactttattgtagctataggtggcaaaagatgttatggcagagaatccagatgtttaaataggaatggggtcaagggtcaccgccccaagcacggataacaaaatttattttttgccagatttctttaattccacctgtgactggtgagggctggtggcggggtggctttcacttttagctcctctttttgtttctgcttgaacgtcccatcttccttacccacccccttgacctgcttcttgagctttctcagggcttcttgccacctttgcagctgtacatggcacctgccatagggctctaattttaaactgagaaattgagaaaacaggaaactgactctttttggggggagagtaagacaaacaggaaaaggaaaatgaagacgtggttgatacagatcgttggatttcaaaaggaaaagtctacggataaccgaaaaaaataaatatttagaaatgcatagtcttggctggttaaataagtatccatgcttgttcttgtggcatagtagttacgagacatttttagttaaatggaaaaatgtgaattactatagtttgagtgatatgctgctttccaaattaaaagcagcataacaaaaacattcccctaatactcataaataattcattgaattggcaataattcacctcctaatgacttcatatgaagtataaagtaacttcgatacatcagaagaaatcctatcttctaatataagaaagtaatatgattacattaaatgcgtctcatataagttataaaaatggtatctatgagtaaagaaatgcttgtgaacaaaaaaattgatcttataaaggtcaaacaggccaggcgtggtggctcacacctgtaatcccagcactttgggaggctgaggtgggcggagtacctgaggtcaggagttcaagaccagcctggccaacatggtgataccctgtctctacaaaaatacaaaaaattagctgggcatgatggtgggtgcctgtaatctcagctactcgggaggcagaggcgggagaatcgcttgaacccgggaggcggaggttgcagtgaactgagattgagccacaacaaccaagcctgggagacagaggaaactctgtctcaaaaaataaaaaataaaaattaaaattaaaaaaaaggtcaaacaaaccaaacccttctgattaatttattcaatctacttttattataagcaaatgagaaattataattttaatctgaaaaagcagaatcaggggattttggagctggacagtcccctggaaattatttggatcaaagccctcattttataggtgaagaaactgagaagtaagatttgagcaagctgcccaaaggctttgccaaaggctataccagtgaatggcagagtctggactggaagtcccagtgctgccgtccaggtgagacctgttccactgcatgctactagctcccgggctgagaccggacttttgcttggcaggtttctttctttcgaaactattaattattgtattttttgtagagacagggttttgccatgatgcccaggctggtcttgaactcctgagctcaagagatccacccagcttggcctctcaaaaatgttgggattacaggcataagccacagtgcccggcccattttcctcccacctctttgttccttctctgtttcttttgcagcattatgttctatcattgtataccagagttcctcaacttcagttatagtctgttcttgctttatgctatcttcttcagcaagctcatcttggtctgttttcctccttatcaggcataccccagaaactcctgttttatctccacctcaactaaacattttcctgagttctgggcctctataaactaattatttgattaacatcttttttttttttttctgagatagagtctctctctgtcacccaggctggagtgcagtggtgcaatctcagatcactgcagcttctgcctcccagattcaagcgattctcctgcctcagcctcctaagtagctgggattataggcatgcaccaccgcacacagctaatttttgtacttttagtagagacggggtttcaccatgttggtcaggctggtctcaaactcctgatctgaagtgatctgactgcctcagcttcccaaagtgctgggattacaagcctgagccaccatgcctggccaacatctttaattggatatctcagtatcaagaaggcccataatattcctctgcctcatccctctcctcagtcctcttcttgtgtttcctagttcagagaatggcaccattctctatcaagctgcgcaaatcagacatgtgtgattttttgttgttgttgagacagggactcactctgtcacccaggctagagtgcagtggcgtgatcatggcgcactgaagcctcaaactcctgggctcaggagatcctcccgcctcagcctcctgagtagctgggaccacaggcccacaccaccatgcccagctaattttgtattctttgtagagatggggtttcatcatgtttgcccaggctggtctcgaactcctggactcaagcaatccacccacctcagcctcccaaagtgctgggattacaggcatgagccactgtgcccagctgaagtgtgatccttaacttcaccccttctcatgccctccatttccaatccatctccagtccagttgactccagctactcaattatttccacttatctcattccactacctttgaagctaccaccatctctaactacagtcatctcccaactaactggtctcctggcatctctctggttctcctccactaatttcaaaaaaagaaatttactgtgacagtgctcacaacactcccccttgctcttactaaagatgcttaccatagcctccaggtattgtatggcctgaggtctatctacatttccaggtgcaggacacaccatgtctccccactcccaaatttagtctccagactccatcctttttacagttctttaaaagcatcacaattcctccaaccactaggcatttgtatgtgctattccctctttccagaatgcaataccctccctctgcctagctagctaacttctatgtatctatgactgcagctcaaactttcctcatggactccctccacaagtgccaagcctgggccagattcttttgttatgtgctcacagaacgatgttccctttagcattcattgagtttgctgtttaattattcttgtcttgtttttgtttaattagtcctatctctaatactagacaaatgttccttaagatcacaggaaatataggactgtctctacataaaaactgttttatatccataatgcctaggacagtacctggcacacagtatatgctcaataaatttttgttgaatgaatgcaattatcattatattcctgatattagcaggtataatccagtttaagtttgggaacagaaagacaaaacggaccacatctaataaatccggtctcctttcttttattatttatttatttgagacagttttgctcttgttgcccaggctgcagtgcaatggcatgatcttggctcactgaaacctccgcctcccaagttcaagggattctccagcctcagcctcccaagtagctgggattacaggcatccaccaccacgcccagctaatttttttgtatttttagtagagatggggtttcaccatgttggccaggctggtctcgaactcctgacctcaggtgatccacccacctcagcctcccaaagtgttgggattacaggcgtgagccaccgtgcccggccaaggtctcctttcttttaatcaaactctcacctttggccattctgcagtcattcacccgacagtatttactgacggagtgaatacagagtgcttgattaatgttgctgctttgttattattattattattattgagatggagtcttgctctgttgcccaggctggagtgcagtggcgtgatctcggctcactgcaacctccgcctcccgggttcaagccattctcctgcctcagcctcccaagtagctgggactacaggcatgcaacaccacacctggctaatttttgtatttttagtagagacaaggtttcaccatattggccaggctggtcttgaactcctgacctcaggtgatctgcccacctcagcttcccaaagtgctgggattacaggcgtgagccaccatacccaacctaatgtttctgctttgaaatacaatttcaaaaagtcattaataggttgaaaacagcaagattttaaaagtattttaaaaagtgaaacagaagaatgcttacttcatttcacagagatagatttctcctttatgttatttctaaaaggagatggaattttgtttcattcatttctgcttatttggacaggccaaatatgaacagctgaacacgtcagcgttaccatgcatatgttacacagatgccatccttcttccatcagctctcatatgcaatacagaagtaaaaagaggttctctttatttttaaaaggtaaaaattgaaattcagtcacttaacacagaataaacaataattacaattacactggtaacaaaggacagcaagcatgttttctttgaaagcactgtatctggtttgtctccgtgcttggtcctagtatctggcatattttccccagagttttcttttcagtgggatgattatcttcggggcaaaaaagtttatcagactcaagttttagcagtacttattttattcatttatatacatgtaaccccatcctgtcttactccaatcttcttactgccttcctactgacacatatattatataacaccctccccaagttctatttacggttaaaaatttctttttttttttctttttttgagacagagtttcactctcgtcacccaggctggtgtgcaatggcgcagtctcggctcactgcaacctccgactccctggttcaagtgattctcctgtctcagcctcccgagtagctggaattacaggcgcccgccaccatgcccagctaatttttgtatttttagtagagacagtgtttcgccatgttggccaggctggtctcaaactcctgacctcaggtgatccacccgccttggcctctcaaagtgctgggattataggcgtaagccactgcgcccagcctacagttacgaatttctaaatggcacaaataaactcagctgttctcagtgcagacgtcaaatcctcactgtgctgaaacattttcctcagcttttgggaaataattacaatttaaacatacacagagaatgtttcttagacaaacataatacccgaggcttatctggtaaaaactaattgctctgtccttagcacaaaaaatatatatctttgtaaaatgagaagaaccaaagaatatttaaaacaaagaaggaagccacacgtactaattacacaagagactgactgacaaactggaattctccaaaacagattttcagcgaggcttctcatttcagagtccaggaaaaaaaaatcctaaaaaccccaaaggtatattatatgtgtgtatatatatttttattgtgttaaaaaacacaaaacataaaatttactgtcttatcaaaaggtatattttgtcgctcttccctttttttttttttttttttcccgagacagagtccagtctgtcgcccaggctgaagtgcagtggcatgatctcggctcactgcaacctgcatcttctgggctcaagcaatcctcccacctcagcctcctgagtagatggagctacaggcacgtgccactaggcccggctaatttttgtattttttgcagacagggttttgccatgttgcccgggctggtctttgttctcctaagagttgttttctccatgaaagttgataaataacatttagaaaatgaattattacaagagtaatgatatgtctcaatttattatatgaaattatcaacaactgcttttaatattcagatgtcaagaagatgaaaagcagaaatacattttgcaaacatgtagcactccataaatggaaatcatgtatttcctctaatatcccaatttttctatattgggatcttatatggctgtttctatatggctattttgtcccaacttgctgtacaagaattttccccagccaccttagaaaggttggatgtagttcactccaagtttgcagttcactccaagtgtttcagtaccacagaaagctccatggaagcctcaaatgtacgggctaggcaatagaagcagggaggtaggattaagaaattactggccaggtgtggtggctcaggcctgtaatcccagcacttcgagaggctgaggcagacagatggcttgagctcaagagtttgagatcagcctgagcaacatggcaaaactctgtctctacaaaaaatataaaaatcagccaggtatgttggtgtgcacctgtagtcccagctactggggaggttgaggcaggaggattgcttgagcccaggaggctgaggctgcagtgagccatgattgtgccactgcattccagcctggtcgactgtaagacaaaaaataagaaaataaaaaatttaccaatataaaatgctcaaacagctaacaaacatgttcaattccatttatagtcttttctttgagccatttaaacatagggctattttttttttttttttttgagatggagtttcactcttgttgcccaggctggagagcaatggcatgatctcggctcaccacaacctctgcctcctgggttcaagcgattctcctgcctcagcctcccgagcagctgggattacaggcatgtgccaccatgcctggctaattttgtatttttagtagagacgggattcctccatgttggtcagactggtcttgaactcccaacctcaggtgatctgcctgcctcaaccttccaaagtgctgggattacaggtgtgagccactgagattggctgccgttttgttttttaactccatatagtttctatagttcactgaaaactcaaagagatgacctataaatgtatgaataatgtatgatttcttacatcaattttctactagaaaaaaatcatacttttagaattggattttgtcttacagtcatctttattatactttataaatgagatttcatttatataaatcaggaagctaaactaaaatagaaacactagatttaaattctgatttgaatactctgatcaaaataacaaatctcacactgggaaaccatctatcagcaagcagagagctactgtgtgtccttccttagaagagtttgaacaccgagaacccacagcatatttgcagtacagtaacagcaattcctttgtcattatcacagaactttaattttcatatactttgctgggaccaaccaaaccatcccatatatataaccatatccatatatatatatatatatatcccacatatatatgggatggtatatatatacacatgtatatgtatgtgtgtgtgtatatatgtgtatatatgtatacacacacacacacacacatatatatatatatacacacacacacatatatatatggagagagagagagagacagtgtcttgctctgtcgcccaggctggagtgcagtggtacgatcttggctcattgcaacctccgcctcccaggctcaagcgattctcatgtctcagtctcccaagtagctgggattacaggtgtgcaccaccacaccaggctaaccattccatacattttatacaatcatttttaaaaagaagcatgaaccatttcggttttagagaattaagtttttttaaaaaagagactcttaaaaaaaagtcattatatgaataaaatctgctttgtgttaattccgacaaatcattccatcattgagtctgtcaccaattttttttttttgaaatggagtttcgctcttgttgcccaggctggagtgcaatggtacgatctcggctcactgcaaccgccgcctcccgggttcaagtgattctcctgcctcagcctcccgagtagctgggattacaggcatgcgccaccacgcctggctaattttgtattattagttgagacagggtttctccatgttggtcaggctggtctcgaactcctgacctcaagtgatccgctggccttggcctcccaaagtgctgggattacaggcgtgagccaccgtgcctggcccaattttttttttttaataacttgcacacttaacaatattttttatcttcttgggacaacattcttttctccacaaaaacccaattaaggacgttgtgccagtttactcctacttccttcctgttcactgagcttaaagtgggtataggcgagaatgccaaataatgtacataaaatgccaagggcctgattaatggacagtggatccttaaataaaacatatcctccgaataaagtaatgcagaacttgaagtgtccgaacatgttataggtgacaggtgaagtgttcccaatgatccaataaattgataagttcaccatgaaagctattactccagatagcagcaccataagcaaagcagaaactgaccagggaccaaatattcctccttctccaaacactggctcaaagaagggcacagcaaccagcaacatggcagatgacatcggagcctggtagtacagcagctgcattgagttcacttgtaattcatgctgtttggctcctacccacagcgtgagctggattctggtggagaaggttttctggtagcagaaggtctggatggctatgatcaccggcgtggtcatggccttggccagctgataggtgcctatggtgttgttctgcagagaaaggttagtgaagaccacaaagccacagaagctgagggccaggaggaggagcctggagggcggcagacttttgggggcaaagatgtccagcttctggcagatatacaagcccagccaggtgaccacgaagtgcaccagggtcaggctcatgttggggaagccgtggtacacataaatccatttgttgaggaacacaatgcagatggacaccagcaggttgaacaggagcccggcggcgattcgccagtggccccgcactcggtccaccagcaatgccatgatccccgcgaagctggggccgtctagcctcggaaggggcgccgggcctgtctccggctgcccttctactccaccgccgcgtcctcgcagacgccgacctcaccgtctgacccaggagtggcatgcacagatcaaccccgggcgagtagcactcttaacagaggacacacaccccgccgccgccctgtaagccagctaggac

SEQ ID NO: 11652 - RNA, 10489 nt, Homo sapiens
  source 1..10489: mol_type = other RNA
ctgaatagctgggactacaggtgtctgccaccacaccccgctaacttttgtatttttagtagagacggggtttcaccaggctggtgaagctggtcttgaactcttgacctcaagtgatccacccacctcagcctcccaaagtgctgggattacaggcgtgagccaccacgcctggcctgatttcattttttggctcttgtggatagtgctgcaggaaacgtgagagtgcaggtgtctctttgatgtactgatttcctttcttttggcttttcacccagtagtggggttgctggatcgtataatagttctattttcagttgctttgaggagcctccatactgttctccatagtggctgtactaatttccactcccaccaacagtgtacgagggctgtccttcctccatatcctcaccagcatctgttctttcctgtctttctgatacaagccattttaactgaagagggatgatatctgattgtggttaatttgcatttctctgataagtggtgatattgagcattttttcatatacctgttagacatttgcatgtcttctctgagaaacgtctgtttggatcttttgcctactttataattggaatatctggagtttggggttttttttttgttatttttctttgtttttgctatagagttgtttgagctccctgtatattctggcaattaaccccttgtcaaatggatagtttgcaaatattttctcccaatctgtgggttgtctctttattttgttatttcctcggcagtatggaagcttcccagcttgatgtaatcccaattgtctatttataattgttacatcttcttgatgacttatctttacaaaatacttttctttatctctagtaaaacttttgttttaaactctattgtgtctgatattagaaagccactggagatttattatggttgctgtttgcgttttatatctttttccatcctttacttctaatccaattgtatctttgagtatgtatgtatgtcttctgtacatggttggatttttttttatcaccactttgacaatctgtgtcttttgatagtttaatctattcacatttaatgttattactggccaggtgcgctggctcatgcctataatcttgatgcttcgagagaccagaatgggaggattgcttgagccctggagtttgatacctccatctctataaataaataaataaaataaaataaaatagccaggtgggaggtgggagaattgcttgaagccaagagttcaaggctgcagtgagctatgatcatgcaactgcactccagcctgggcaatagagcaagaccctcttaaaaaaaagttattattgatatagttagatttacatatgctgctttcccttttgtattttatgtctcatgtatcttttgttcatctatttctccttcacttttgtcttaagtgcatattttgtaatgtaatattttatttatttaatgattccttacaatatttttgcagttatttctttagtgtttgttctaggaagtgttaaatacacattaacttatcagagtctacttcagatttatactaccttaattccaataagacttttataaacccattattcctatatagttctagcccccaccccgacttttgtgctggtattgatatatatatctatgttacaaatgcaacaacacattgctataaatattgctttatatattttataatttaaagaggctgagagatgaagagaaagtatatattaacagcttttgttacagtagcctatttatttcctatttctggttctctcagcttattcttgtggctttaagttgccatctagagccatttccttaccccaacacgactcttctcccatcctcctcctttgtggtgttattggtagacatattacacttctgtatgttatagtccaaacagtactgcatattgttttatataattgctttttttgttgctgttattgagacggagtctcactctgttgcccaggctgaagtgcggtggcgtgatctcggctcactgcaacctctgcctcctgggttcaagccattctcctgcctcagcctcccgagtagctgggactacaggcgcccgccaccacgccccgctaattttttgtgtttttaatagagatggggtttcaccatgttagtgaggatggtcttgacctccagaccttgtgatccgcccacctcggcctcccaaagtgctgggattacaggcgtgagccaccacgcctggcctataattattaatcagttactaataaaataagaaatctgcacttgcactatcttttattattacataattaccctttactggtgctctttgttttttctgtggaaacaaattactgcctggggtcattcctcagactgttgctcttcagtctccaaactgatcactggaaatgatgttaagtggagctgatcccgttcccactccttggctcttggacctgtgtacactccctattgaggaatcactaccagataaaagtctgtgattccaggactgcatcttggaggacggtgccctgtgcttgtcaagtactgccactaagctggtacttcaaaccaccttcagcaggtcatccaatgctctgtcacaccagccgcttctaggtggtggggtaagcataaggtgtgaccaatagatcagtcatgggaccaccactgaaccttatctgtggtaaagtgggtctccttgtctaatgccctgccatgtgggataatcagaatctctactcccctaaaaattattagacttcttccaatgttacatactgttattttctggggcttatttccatatttttgtaccatcaaattacatcttataatttttaagtctgtttagatttggccgagcatgactttttatttttttatgtttccaactttcttggtattaaatattttgtttaaaatgacattatttcaccctggtttgtgaataacccttctaggtagatattttctttcagaacattgaagacattcttttactgtcttctgatttttactgttgctattgagaagtcaacctaagcatgtaaaattggaaaagggcaactcaatgataaaatatcagactttcaactaatattcccatccttacaacctccaatgatggtatctcataacatattacaaataccaagagagtagaatttttttttttttttgagtcaaggtcttgctctgtcacccaggctggagtgcagtggtacaaatatggcttactgcagcttcaacctcctgggctcaagcaatcctcctgcctcagcctccagagtagctgggaccacagccctaagccaccatcccggggtattttttttttttcagagatggggttttgctttgttgtccagactggtctcaaattcctgagctcaagtgatcctcctgcctcccaaagtgttgggattataggcataagccactgcacccagccagagtagggctgattttaaattttagactttggccccaaagtgagctgttattttccttttactgtgatgctcttaaaatagttaaaaaaaaaaaaaaaaagtagctaaattgtttttaaaaattaaggatgctctggccgggtacgatggctcatgcctgtaatcctagcactttgggaggccaaggcgggtggatcacctgaggtcaggagtttgagaccatcctggccaaaatggtgaaaccccatctctactaaaaatacaaaaattagccaggtgtggtggcaggtgcctgtaatcccagctactcaggaggctgaggcaggagaatcacctgaaccccagaggcggaagttgcagtgagccgagatcacgccactgcactccagcatgggtgacacagtgagactctgtctcaaaaaaaaaaaaaaaaaaaaattacccctacactttttcacaataaaccttagatcttcaagacactcacaaaaccaaaagccacttccttctctcaacacttacccccaagacaaatgaagatatatggaaatatatggcatacctagttcagacttctattaaagagtcacacaaacattccatcaataaacatgcagcatgaatttctaaataaacgtctgcttgaagcacttttatttgccagtagaagtaatatttccaactgtctcaggtcaagagttccttttggcctccagcctgatctcagactggactttcctctttgggaactcctatgccctctactcagaagactgtcctcttggcttcttttggcttttcagcaacattgacatttgtcttctgtattattattatatagtttgtttatttatttttactttttacagatatgaggtcttgccctgtcatccaggctgaaacacaatcatggctcactgcatcctcaaccttctgggctgaagcgacactcctgcctcagcctcccaagtagctgggaccataggaaagcatcttattttttttcattttttagttctctttcttattcttttgccacaagttgataattgaggccgatgcaagtgaagacatagatacatgccacagttaggattgtgtcatatacacagaacatgtgtttgtcattttcttttctttttttttttttttttgagacagagtctcactctgtcacccaggctggagtgcaatggcgcaatctctgctcactgccacctccacctcccgggttccagcgattctcctgcctcagcctcccaagtagctgggattacaggcgcccgccaccatgcccgactaatttttgtatttttagttgagacgggatttcaccatattggccaggctgaactcgaactcccgaccttgtgatccacccaccttggcctcccaaagtgctgggattacaggcgtgagccaccacgcccggccagtagctactactttcaataacacacttttattgggtcttggtggagggagagggctgagggtcttaggaacacataatggatacaatccagcatgtcacaaagcattatcattctttcttctagattatggcaaagttcctgacttttgttcttccccttgccataagccagtgttggatctggtcttgccttagctgctacagctaacttttaaaaccatcatcatggtcaggcatggtggctcacgcctgtaatcccggcacttcgggaggccgaggcaggtggattacctgaggtcaggaattcaagaccagcctggccaacgtggtgaaaccccgtctctactaaaaatacaaaaattagccaggcgcggtggcacacacctgtaatcccagctactatggaggctgaggcaggagaatcgcttgaacccaggaggcggaggttgcagtgagccgagattgtgcaattcactccagcctgggtgacagaacaagactccgtctcaaaaaaaaaaaaaaacaaaacaaaacaaaaaaaaaaacagaaagcaaaaccatcatcactgctgggtgtcagtgcaccaagtatatgctgtaagtaattgcccttcactgaacaccctcaaaggatttcacaagtatctaccccctcccccaactttttttttgagacagggtctcactgttgcccagactggagtacagtgcagctcactgcatccttgacctcctgggctcaagtgatcctcctgcctcaacctcctgagtagctgggattgcaggtgtgcaccgctgtaaccagcttttaagaaacttttgtagacagggttttgtcacgttgccctgggtgttgtcatgctgagaagttttgatacattactcattcctgcaatgctctatgaattctacatattttcctaaatgagcaatcccatcccagggcatgtttagtgtagattattgttaccaaactggtaaaaataagccatggggaactggcagaataagcttcctcctgcaaggcaaattccacattttcccagaaaagggaaggggttctatctgtatcaggaggtggcaggttttttatacctcaactactcaactgtgccatggctgtgcaaaagcagtcaaataatacacaaatatatttagccatgttccaacaacagttatttatggacactcaagtttgaattttatatattgccaacatctactctatagccttaaatgaagcatctgcagtgcaaagtctatcagaagagtttgctaggctgagtcctcaggttcttcccagatactcctattcaaagtctatcagaagagtttgctaggctgagtcctcaggttcttcccagacattcctattcaaagtctatcagaagagtttgctaggctgagtcctcaggttcttcccagatactcctattcaaagtctatcagaagagtttgctaggctgagtcctcaggttcttcccagacattcctattcaaagtctatcagaagagtttgctaggctgaggcctcaggttcttcgcagatactgctattcaaagtctatcacaagagcttgctaggctgagtcctcaggttcttcccagatattcctattcaaattatcaagggataactttttgagggggggaagggtgaggataactttttcaacacatgtttacattaagggatttagtaaacatttgaggtgaactgactttaattcaccaagccaaatatactatttgattcccaccacctcactcctacagctgtaagaaactttttcagcaatgtcaaagttgccaagtctgacactccaccctgaggtgagatttcagggcttcaggcctgtcattctcatggtctaagatccagcaagatcaaaatcagccatctctgcccctgtctcagattttctcataaatttaaaattcttataatgctataattcttcagtgtttccaaaatttcagtatcaggcactacaacgttccaggtgtacagaaacaataaccatatttcacatgatggctaaaagttgctatcttcaaatataaacaagaatgtgattttcttgtctcaggaaaaacaaacaaacctaaatcatataccccactttgttaactacatgctaccaaggcaacaactgatcagttaaagcccttaggttataagaaatagaaagctggccgggctcggtggctcacacctgtaatcccatgactttgggaggctgaagtgggcagatcacctgaggtcaggagttcaagaccagcctggccaacatggtgaaaccccgtctatactaaaaatacaaatattagccaggcatgtaatcctagccacttgggaggctgaggcaaggaaattgcttgaacccaggaggtggaagttgcagtgagctgagatcatgccattgcattccagcctggaggacaagagtgaaacttagtctcaaaaaaaaaaaaaaaaaaaaaaaaaaaaaaacccaaacaacaaaaagcaaaagacatttttattgagaagtgaggaaacacacagatcagagaagcaggttctaaagggatcgtatccacagttattcttgtaatcaattagccagaatgaatggatgttctcaacagaattctgggacaagaatgaatgagttcccacattttctggttcatgtacaaatgaattacagactcaaaattctgaaaaagagattaccattatccaacaatgggtaaaatgctcacctgtagctagtggaacggatacctgaaagacactaccacaggaagcaccccagagaggggaggtatttctccagagaaaacaggggtgctcatgtcaatcaatggacaacaggcatggaactgcaaaatataataaacgttcattataatgagttctcttaagcggcagccctgtaataaatgccagatctgcttatgaaaaagaaatcaaaagataattagcatttaatatggaaaatactgggggatattattccacaaactatcaaatatatatatagatagatagaacaagttacattaaaaaataaagtacaaaaaattttagaaatactattcagtgttaactcaggaaagtcacattaaatatccattaactttaagactctgttccctgcgtttttcctgaacattatttacatatttttaaaaaaacaactttatactccaccatgaagtcaactgttcataccaagattttattttacaaaaacacagcttcaaatctggaatgtgactttccatggaacacactttcaatgggaaaatgcttccttaatttattcaacttataaggtgttcctagtgtaaattctctgaatcttcatgatgatactacaacatttgatacatttattgctccacattccttccattattttcatctacaaagatttgtaacttatttctgaaagcttttacactcatcccaaatatggttggtctctctcctctctgatttttgacatgagtgtaattttagggcctcctgcttgtaaatcctgtctatattatccgaagtctcctgaacatcagtttctcacattgcatcattctgatttctcatttatgagtcttccgatgtatacgaagccctgaattccaacagaaggatttcccacattcagagcatttccatggtttctctccggtgtgaactctctgatgttcactgagagatgacttctgagtgaaggcttttccacattcactgcatttaaaaggtttctctcccgaatgagttttctggtgtatctgaagtgatgccttcctagggtaggctttttcacattcattgcattcatagggcttctcagttgaatgagttctctgatgtataatcagctgtgattttccacaaaaggctctctcacacaaactacattcatagggtctctctccggtgtgtgttctcctatgtataacaaggtatgacttgctgctgaaagccttcccacattcactgcatccatagggcttctctcctgcatgagctctcagatgtgcagtgagctgttccttcctaccaaaggctttcccacattcaccgcattgataaggattatttcctgtgtgaactccctgatgtacaatgagttgtgtcttcatattgaaggctttcccacaatcactgcattgatagggtttttctcctgtatgcattcggatgtgaacaaggagataggacttactcctaaaggctttcccacattcactgcatttatggggtttcactcctgtatgagttctctggtgtacaacgaatggagacttcaaactaaaggctttcccacattcgctgcattcatacggtttcactcctgtgtgacttctctggtgtaaaagaagctgtgatttccaactgtaggctttcccacattcactgcagccatagggtttccctcctgtgtgaatttcctgatggacaatgagctgtgacctgaaagagaagaccttctcgcactcactacatgagtagggtttttctcctgtatgaactctctgatgagcattaaggtttgacttggcactgaaggctctttcacatttactgcattcataaggtctctctcctgtatgaattctgagatgtacaatgagctgtgacttacaacgaaaagctttcccacattcactacacacacagtttttttctatgctatgagctctttgatgcttaagaaaatatggttcttcataaccatgaaacttatcaggattctttcttaaataacttctgcttggagctgagttttgtgtcaaactttttccacgtgtgttatagagtctctgtcttgaagaatcatgggttttgctcagattaagtcttcccaacacactacaagcatagcttctttcaatactctcaagctcatcttgattgttctggtaccattcttcccagccatccactgatatcaggttatgatagttttccaatatcacatctctgtacaggtacttctgtgtagaatccagtagctgccattcatcccaggtgaactccatagatatatccttgaatgacaataatccccagcacgaagctgtccggaaactggtggccatccccacgcccacgttcgcgcgctgcctgcgggggcaggacccgcgggctgcggagagaccgtgagggatgcgtccgcccgaagacaggtgcgggaccagggccccaggctcctgaccgtcccggggccgagtcgttggcagggacgccggctcctcagctctcgcccaacacagaccgcgcgtgactagacaacctcccggtctgggtaccaggagtcgcacggatggatttgtgcctttccgtggccctgactcgggagagcaggaggctgatctggccccgtccacgccccggaccgacggaagtgtttagctggtcaagtctctggtctgcccaggataatccgagccgcttagctccgcgcctccgcggccacagagactcagccaggtacacccgctggccagattccggtccactgagtctaagccggaaacagccctgcacgcgcgcacccgactaaggccgggagt

SEQ ID NO: 11653 - RNA, 10788 nt, Homo sapiens
  source 1..10788: mol_type = other RNA
ctgaatagctgggactacaggtgtctgccaccacaccccgctaacttttgtatttttagtagagacggggtttcaccaggctggtgaagctggtcttgaactcttgacctcaagtgatccacccacctcagcctcccaaagtgctgggattacaggcgtgagccaccacgcctggcctgatttcattttttggctcttgtggatagtgctgcaggaaacgtgagagtgcaggtgtctctttgatgtactgatttcctttcttttggcttttcacccagtagtggggttgctggatcgtataatagttctattttcagttgctttgaggagcctccatactgttctccatagtggctgtactaatttccactcccaccaacagtgtacgagggctgtccttcctccatatcctcaccagcatctgttctttcctgtctttctgatacaagccattttaactgaagagggatgatatctgattgtggttaatttgcatttctctgataagtggtgatattgagcattttttcatatacctgttagacatttgcatgtcttctctgagaaacgtctgtttggatcttttgcctactttataattggaatatctggagtttggggttttttttttgttatttttctttgtttttgctatagagttgtttgagctccctgtatattctggcaattaaccccttgtcaaatggatagtttgcaaatattttctcccaatctgtgggttgtctctttattttgttatttcctcggcagtatggaagcttcccagcttgatgtaatcccaattgtctatttataattgttacatcttcttgatgacttatctttacaaaatacttttctttatctctagtaaaacttttgttttaaactctattgtgtctgatattagaaagccactggagatttattatggttgctgtttgcgttttatatctttttccatcctttacttctaatccaattgtatctttgagtatgtatgtatgtcttctgtacatggttggatttttttttatcaccactttgacaatctgtgtcttttgatagtttaatctattcacatttaatgttattactggccaggtgcgctggctcatgcctataatcttgatgcttcgagagaccagaatgggaggattgcttgagccctggagtttgatacctccatctctataaataaataaataaaataaaataaaatagccaggtgggaggtgggagaattgcttgaagccaagagttcaaggctgcagtgagctatgatcatgcaactgcactccagcctgggcaatagagcaagaccctcttaaaaaaaagttattattgatatagttagatttacatatgctgctttcccttttgtattttatgtctcatgtatcttttgttcatctatttctccttcacttttgtcttaagtgcatattttgtaatgtaatattttatttatttaatgattccttacaatatttttgcagttatttctttagtgtttgttctaggaagtgttaaatacacattaacttatcagagtctacttcagatttatactaccttaattccaataagacttttataaacccattattcctatatagttctagcccccaccccgacttttgtgctggtattgatatatatatctatgttacaaatgcaacaacacattgctataaatattgctttatatattttataatttaaagaggctgagagatgaagagaaagtatatattaacagcttttgttacagtagcctatttatttcctatttctggttctctcagcttattcttgtggctttaagttgccatctagagccatttccttaccccaacacgactcttctcccatcctcctcctttgtggtgttattggtagacatattacacttctgtatgttatagtccaaacagtactgcatattgttttatataattgctttttttgttgctgttattgagacggagtctcactctgttgcccaggctgaagtgcggtggcgtgatctcggctcactgcaacctctgcctcctgggttcaagccattctcctgcctcagcctcccgagtagctgggactacaggcgcccgccaccacgccccgctaattttttgtgtttttaatagagatggggtttcaccatgttagtgaggatggtcttgacctccagaccttgtgatccgcccacctcggcctcccaaagtgctgggattacaggcgtgagccaccacgcctggcctataattattaatcagttactaataaaataagaaatctgcacttgcactatcttttattattacataattaccctttactggtgctctttgttttttctgtggaaacaaattactgcctggggtcattcctcagactgttgctcttcagtctccaaactgatcactggaaatgatgttaagtggagctgatcccgttcccactccttggctcttggacctgtgtacactccctattgaggaatcactaccagataaaagtctgtgattccaggactgcatcttggaggacggtgccctgtgcttgtcaagtactgccactaagctggtacttcaaaccaccttcagcaggtcatccaatgctctgtcacaccagccgcttctaggtggtggggtaagcataaggtgtgaccaatagatcagtcatgggaccaccactgaaccttatctgtggtaaagtgggtctccttgtctaatgccctgccatgtgggataatcagaatctctactcccctaaaaattattagacttcttccaatgttacatactgttattttctggggcttatttccatatttttgtaccatcaaattacatcttataatttttaagtctgtttagatttggccgagcatgactttttatttttttatgtttccaactttcttggtattaaatattttgtttaaaatgacattatttcaccctggtttgtgaataacccttctaggtagatattttctttcagaacattgaagacattcttttactgtcttctgatttttactgttgctattgagaagtcaacctaagcatgtaaaattggaaaagggcaactcaatgataaaatatcagactttcaactaatattcccatccttacaacctccaatgatggtatctcataacatattacaaataccaagagagtagaatttttttttttttttgagtcaaggtcttgctctgtcacccaggctggagtgcagtggtacaaatatggcttactgcagcttcaacctcctgggctcaagcaatcctcctgcctcagcctccagagtagctgggaccacagccctaagccaccatcccggggtattttttttttttcagagatggggttttgctttgttgtccagactggtctcaaattcctgagctcaagtgatcctcctgcctcccaaagtgttgggattataggcataagccactgcacccagccagagtagggctgattttaaattttagactttggccccaaagtgagctgttattttccttttactgtgatgctcttaaaatagttaaaaaaaaaaaaaaaaagtagctaaattgtttttaaaaattaaggatgctctggccgggtacgatggctcatgcctgtaatcctagcactttgggaggccaaggcgggtggatcacctgaggtcaggagtttgagaccatcctggccaaaatggtgaaaccccatctctactaaaaatacaaaaattagccaggtgtggtggcaggtgcctgtaatcccagctactcaggaggctgaggcaggagaatcacctgaaccccagaggcggaagttgcagtgagccgagatcacgccactgcactccagcatgggtgacacagtgagactctgtctcaaaaaaaaaaaaaaaaaaaaattacccctacactttttcacaataaaccttagatcttcaagacactcacaaaaccaaaagccacttccttctctcaacacttacccccaagacaaatgaagatatatggaaatatatggcatacctagttcagacttctattaaagagtcacacaaacattccatcaataaacatgcagcatgaatttctaaataaacgtctgcttgaagcacttttatttgccagtagaagtaatatttccaactgtctcaggtcaagagttccttttggcctccagcctgatctcagactggactttcctctttgggaactcctatgccctctactcagaagactgtcctcttggcttcttttggcttttcagcaacattgacatttgtcttctgtattattattatatagtttgtttatttatttttactttttacagatatgaggtcttgccctgtcatccaggctgaaacacaatcatggctcactgcatcctcaaccttctgggctgaagcgacactcctgcctcagcctcccaagtagctgggaccataggaaagcatcttattttttttcattttttagttctctttcttattcttttgccacaagttgataattgaggccgatgcaagtgaagacatagatacatgccacagttaggattgtgtcatatacacagaacatgtgtttgtcattttcttttctttttttttttttttttgagacagagtctcactctgtcacccaggctggagtgcaatggcgcaatctctgctcactgccacctccacctcccgggttccagcgattctcctgcctcagcctcccaagtagctgggattacaggcgcccgccaccatgcccgactaatttttgtatttttagttgagacgggatttcaccatattggccaggctgaactcgaactcccgaccttgtgatccacccaccttggcctcccaaagtgctgggattacaggcgtgagccaccacgcccggccagtagctactactttcaataacacacttttattgggtcttggtggagggagagggctgagggtcttaggaacacataatggatacaatccagcatgtcacaaagcattatcattctttcttctagattatggcaaagttcctgacttttgttcttccccttgccataagccagtgttggatctggtcttgccttagctgctacagctaacttttaaaaccatcatcatggtcaggcatggtggctcacgcctgtaatcccggcacttcgggaggccgaggcaggtggattacctgaggtcaggaattcaagaccagcctggccaacgtggtgaaaccccgtctctactaaaaatacaaaaattagccaggcgcggtggcacacacctgtaatcccagctactatggaggctgaggcaggagaatcgcttgaacccaggaggcggaggttgcagtgagccgagattgtgcaattcactccagcctgggtgacagaacaagactccgtctcaaaaaaaaaaaaaaacaaaacaaaacaaaaaaaaaaacagaaagcaaaaccatcatcactgctgggtgtcagtgcaccaagtatatgctgtaagtaattgcccttcactgaacaccctcaaaggatttcacaagtatctaccccctcccccaactttttttttgagacagggtctcactgttgcccagactggagtacagtgcagctcactgcatccttgacctcctgggctcaagtgatcctcctgcctcaacctcctgagtagctgggattgcaggtgtgcaccgctgtaaccagcttttaagaaacttttgtagacagggttttgtcacgttgccctgggtgttgtcatgctgagaagttttgatacattactcattcctgcaatgctctatgaattctacatattttcctaaatgagcaatcccatcccagggcatgtttagtgtagattattgttaccaaactggtaaaaataagccatggggaactggcagaataagcttcctcctgcaaggcaaattccacattttcccagaaaagggaaggggttctatctgtatcaggaggtggcaggttttttatacctcaactactcaactgtgccatggctgtgcaaaagcagtcaaataatacacaaatatatttagccatgttccaacaacagttatttatggacactcaagtttgaattttatatattgccaacatctactctatagccttaaatgaagcatctgcagtgcaaagtctatcagaagagtttgctaggctgagtcctcaggttcttcccagatactcctattcaaagtctatcagaagagtttgctaggctgagtcctcaggttcttcccagacattcctattcaaagtctatcagaagagtttgctaggctgagtcctcaggttcttcccagatactcctattcaaagtctatcagaagagtttgctaggctgagtcctcaggttcttcccagacattcctattcaaagtctatcagaagagtttgctaggctgaggcctcaggttcttcgcagatactgctattcaaagtctatcacaagagcttgctaggctgagtcctcaggttcttcccagatattcctattcaaattatcaagggataactttttgagggggggaagggtgaggataactttttcaacacatgtttacattaagggatttagtaaacatttgaggtgaactgactttaattcaccaagccaaatatactatttgattcccaccacctcactcctacagctgtaagaaactttttcagcaatgtcaaagttgccaagtctgacactccaccctgaggtgagatttcagggcttcaggcctgtcattctcatggtctaagatccagcaagatcaaaatcagccatctctgcccctgtctcagattttctcataaatttaaaattcttataatgctataattcttcagtgtttccaaaatttcagtatcaggcactacaacgttccaggtgtacagaaacaataaccatatttcacatgatggctaaaagttgctatcttcaaatataaacaagaatgtgattttcttgtctcaggaaaaacaaacaaacctaaatcatataccccactttgttaactacatgctaccaaggcaacaactgatcagttaaagcccttaggttataagaaatagaaagctggccgggctcggtggctcacacctgtaatcccatgactttgggaggctgaagtgggcagatcacctgaggtcaggagttcaagaccagcctggccaacatggtgaaaccccgtctatactaaaaatacaaatattagccaggcatgtaatcctagccacttgggaggctgaggcaaggaaattgcttgaacccaggaggtggaagttgcagtgagctgagatcatgccattgcattccagcctggaggacaagagtgaaacttagtctcaaaaaaaaaaaaaaaaaaaaaaaaaaaaaaacccaaacaacaaaaagcaaaagacatttttattgagaagtgaggaaacacacagatcagagaagcaggttctaaagggatcgtatccacagttattcttgtaatcaattagccagaatgaatggatgttctcaacagaattctgggacaagaatgaatgagttcccacattttctggttcatgtacaaatgaattacagactcaaaattctgaaaaagagattaccattatccaacaatgggtaaaatgctcacctgtagctagtggaacggatacctgaaagacactaccacaggaagcaccccagagaggggaggtatttctccagagaaaacaggggtgctcatgtcaatcaatggacaacaggcatggaactgcaaaatataataaacgttcattataatgagttctcttaagcggcagccctgtaataaatgccagatctgcttatgaaaaagaaatcaaaagataattagcatttaatatggaaaatactgggggatattattccacaaactatcaaatatatatatagatagatagaacaagttacattaaaaaataaagtacaaaaaattttagaaatactattcagtgttaactcaggaaagtcacattaaatatccattaactttaagactctgttccctgcgtttttcctgaacattatttacatatttttaaaaaaacaactttatactccaccatgaagtcaactgttcataccaagattttattttacaaaaacacagcttcaaatctggaatgtgactttccatggaacacactttcaatgggaaaatgcttccttaatttattcaacttataaggtgttcctagtgtaaattctctgaatcttcatgatgatactacaacatttgatacatttattgctccacattccttccattattttcatctacaaagatttgtaacttatttctgaaagcttttacactcatcccaaatatggttggtctctctcctctctgatttttgacatgagtgtaattttagggcctcctgcttgtaaatcctgtctatattatccgaagtctcctgaacatcagtttctcacattgcatcattctgatttctcatttatgagtcttccgatgtatacgaagccctgaattccaacagaaggatttcccacattcagagcatttccatggtttctctccggtgtgaactctctgatgttcactgagagatgacttctgagtgaaggcttttccacattcactgcatttaaaaggtttctctcccgaatgagttttctggtgtatctgaagtgatgccttcctagggtaggctttttcacattcattgcattcatagggcttctcagttgaatgagttctctgatgtataatcagctgtgattttccacaaaaggctctctcacacaaactacattcatagggtctctctccggtgtgtgttctcctatgtataacaaggtatgacttgctgctgaaagccttcccacattcactgcatccatagggcttctctcctgcatgagctctcagatgtgcagtgagctgttccttcctaccaaaggctttcccacattcaccgcattgataaggattatttcctgtgtgaactccctgatgtacaatgagttgtgtcttcatattgaaggctttcccacaatcactgcattgatagggtttttctcctgtatgcattcggatgtgaacaaggagataggacttactcctaaaggctttcccacattcactgcatttatggggtttcactcctgtatgagttctctggtgtacaacgaatggagacttcaaactaaaggctttcccacattcgctgcattcatacggtttcactcctgtgtgacttctctggtgtaaaagaagctgtgatttccaactgtaggctttcccacattcactgcagccatagggtttccctcctgtgtgaatttcctgatggacaatgagctgtgacctgaaagagaagaccttctcgcactcactacatgagtagggtttttctcctgtatgaactctctgatgagcattaaggtttgacttggcactgaaggctctttcacatttactgcattcataaggtctctctcctgtatgaattctgagatgtacaatgagctgtgacttacaacgaaaagctttcccacattcactacacacacagtttttttctatgctatgagctctttgatgcttaagaaaatatggttcttcataaccatgaaacttatcaggattctttcttaaataacttctgcttggagctgagttttgtgtcaaactttttccacgtgtgttatagagtctctgtcttgaagaatcatgggttttgctcagattaagtcttcccaacacactacaagcatagcttctttcaatactctcaagctcatcttgattgttctggtaccattcttcccagccatctggacagctctgcctggaaattttggcatttattatccatggatcttctccttgttccaacttgaagattaagtcaggcttggtaccatgataccccactgatatcaggttatgatagttttccaatatcacatctctgtacaggtacttctgtgtagaatccagtagctgccattcatcccaggtgaactccatagatatatccttgaatgacaataatccaggagtctgaaggcaattggtctggggcttccatctcttgctccaccttacatggcttccacttccagggcaacccagtctaagatggctctagtcatcacatctgcattctaagcaacagcaaagagtgggggctgggagggaacagcagggaaattcagaaatggagtttctgtatatgcccaactgaaaaactggcaaatccagcacgaagctgtccggaaactggtggccatccccacgcccacgttcgcgcgctgcctgcgggggcaggacccgcgggctgcggagagaccgtgagggatgcgtccgcccgaagacaggtgcgggaccagggccccaggctcctgaccgtcccggggccgagtcgttggcagggacgccggctcctcagctctcgcccaacacagaccgcgcgtgactagacaacctcccggtctgggtaccaggagtcgcacggatggatttgtgcctttccgtggccctgactcgggagagcaggaggctgatctggccccgtccacgccccggaccgacggaagtgtttagctggtcaagtctctggtctgcccaggataatccgagccgcttagctccgcgcctccgcggccacagagactcagccaggtacacccgctggccagattccggtccactgagtctaagccggaaacagccctgcacgcgcgcacccgactaaggccgggagt

SEQ ID NO: 11654 - RNA, 10585 nt, Homo sapiens
  source 1..10585: mol_type = other RNA
ctgaatagctgggactacaggtgtctgccaccacaccccgctaacttttgtatttttagtagagacggggtttcaccaggctggtgaagctggtcttgaactcttgacctcaagtgatccacccacctcagcctcccaaagtgctgggattacaggcgtgagccaccacgcctggcctgatttcattttttggctcttgtggatagtgctgcaggaaacgtgagagtgcaggtgtctctttgatgtactgatttcctttcttttggcttttcacccagtagtggggttgctggatcgtataatagttctattttcagttgctttgaggagcctccatactgttctccatagtggctgtactaatttccactcccaccaacagtgtacgagggctgtccttcctccatatcctcaccagcatctgttctttcctgtctttctgatacaagccattttaactgaagagggatgatatctgattgtggttaatttgcatttctctgataagtggtgatattgagcattttttcatatacctgttagacatttgcatgtcttctctgagaaacgtctgtttggatcttttgcctactttataattggaatatctggagtttggggttttttttttgttatttttctttgtttttgctatagagttgtttgagctccctgtatattctggcaattaaccccttgtcaaatggatagtttgcaaatattttctcccaatctgtgggttgtctctttattttgttatttcctcggcagtatggaagcttcccagcttgatgtaatcccaattgtctatttataattgttacatcttcttgatgacttatctttacaaaatacttttctttatctctagtaaaacttttgttttaaactctattgtgtctgatattagaaagccactggagatttattatggttgctgtttgcgttttatatctttttccatcctttacttctaatccaattgtatctttgagtatgtatgtatgtcttctgtacatggttggatttttttttatcaccactttgacaatctgtgtcttttgatagtttaatctattcacatttaatgttattactggccaggtgcgctggctcatgcctataatcttgatgcttcgagagaccagaatgggaggattgcttgagccctggagtttgatacctccatctctataaataaataaataaaataaaataaaatagccaggtgggaggtgggagaattgcttgaagccaagagttcaaggctgcagtgagctatgatcatgcaactgcactccagcctgggcaatagagcaagaccctcttaaaaaaaagttattattgatatagttagatttacatatgctgctttcccttttgtattttatgtctcatgtatcttttgttcatctatttctccttcacttttgtcttaagtgcatattttgtaatgtaatattttatttatttaatgattccttacaatatttttgcagttatttctttagtgtttgttctaggaagtgttaaatacacattaacttatcagagtctacttcagatttatactaccttaattccaataagacttttataaacccattattcctatatagttctagcccccaccccgacttttgtgctggtattgatatatatatctatgttacaaatgcaacaacacattgctataaatattgctttatatattttataatttaaagaggctgagagatgaagagaaagtatatattaacagcttttgttacagtagcctatttatttcctatttctggttctctcagcttattcttgtggctttaagttgccatctagagccatttccttaccccaacacgactcttctcccatcctcctcctttgtggtgttattggtagacatattacacttctgtatgttatagtccaaacagtactgcatattgttttatataattgctttttttgttgctgttattgagacggagtctcactctgttgcccaggctgaagtgcggtggcgtgatctcggctcactgcaacctctgcctcctgggttcaagccattctcctgcctcagcctcccgagtagctgggactacaggcgcccgccaccacgccccgctaattttttgtgtttttaatagagatggggtttcaccatgttagtgaggatggtcttgacctccagaccttgtgatccgcccacctcggcctcccaaagtgctgggattacaggcgtgagccaccacgcctggcctataattattaatcagttactaataaaataagaaatctgcacttgcactatcttttattattacataattaccctttactggtgctctttgttttttctgtggaaacaaattactgcctggggtcattcctcagactgttgctcttcagtctccaaactgatcactggaaatgatgttaagtggagctgatcccgttcccactccttggctcttggacctgtgtacactccctattgaggaatcactaccagataaaagtctgtgattccaggactgcatcttggaggacggtgccctgtgcttgtcaagtactgccactaagctggtacttcaaaccaccttcagcaggtcatccaatgctctgtcacaccagccgcttctaggtggtggggtaagcataaggtgtgaccaatagatcagtcatgggaccaccactgaaccttatctgtggtaaagtgggtctccttgtctaatgccctgccatgtgggataatcagaatctctactcccctaaaaattattagacttcttccaatgttacatactgttattttctggggcttatttccatatttttgtaccatcaaattacatcttataatttttaagtctgtttagatttggccgagcatgactttttatttttttatgtttccaactttcttggtattaaatattttgtttaaaatgacattatttcaccctggtttgtgaataacccttctaggtagatattttctttcagaacattgaagacattcttttactgtcttctgatttttactgttgctattgagaagtcaacctaagcatgtaaaattggaaaagggcaactcaatgataaaatatcagactttcaactaatattcccatccttacaacctccaatgatggtatctcataacatattacaaataccaagagagtagaatttttttttttttttgagtcaaggtcttgctctgtcacccaggctggagtgcagtggtacaaatatggcttactgcagcttcaacctcctgggctcaagcaatcctcctgcctcagcctccagagtagctgggaccacagccctaagccaccatcccggggtattttttttttttcagagatggggttttgctttgttgtccagactggtctcaaattcctgagctcaagtgatcctcctgcctcccaaagtgttgggattataggcataagccactgcacccagccagagtagggctgattttaaattttagactttggccccaaagtgagctgttattttccttttactgtgatgctcttaaaatagttaaaaaaaaaaaaaaaaagtagctaaattgtttttaaaaattaaggatgctctggccgggtacgatggctcatgcctgtaatcctagcactttgggaggccaaggcgggtggatcacctgaggtcaggagtttgagaccatcctggccaaaatggtgaaaccccatctctactaaaaatacaaaaattagccaggtgtggtggcaggtgcctgtaatcccagctactcaggaggctgaggcaggagaatcacctgaaccccagaggcggaagttgcagtgagccgagatcacgccactgcactccagcatgggtgacacagtgagactctgtctcaaaaaaaaaaaaaaaaaaaaattacccctacactttttcacaataaaccttagatcttcaagacactcacaaaaccaaaagccacttccttctctcaacacttacccccaagacaaatgaagatatatggaaatatatggcatacctagttcagacttctattaaagagtcacacaaacattccatcaataaacatgcagcatgaatttctaaataaacgtctgcttgaagcacttttatttgccagtagaagtaatatttccaactgtctcaggtcaagagttccttttggcctccagcctgatctcagactggactttcctctttgggaactcctatgccctctactcagaagactgtcctcttggcttcttttggcttttcagcaacattgacatttgtcttctgtattattattatatagtttgtttatttatttttactttttacagatatgaggtcttgccctgtcatccaggctgaaacacaatcatggctcactgcatcctcaaccttctgggctgaagcgacactcctgcctcagcctcccaagtagctgggaccataggaaagcatcttattttttttcattttttagttctctttcttattcttttgccacaagttgataattgaggccgatgcaagtgaagacatagatacatgccacagttaggattgtgtcatatacacagaacatgtgtttgtcattttcttttctttttttttttttttttgagacagagtctcactctgtcacccaggctggagtgcaatggcgcaatctctgctcactgccacctccacctcccgggttccagcgattctcctgcctcagcctcccaagtagctgggattacaggcgcccgccaccatgcccgactaatttttgtatttttagttgagacgggatttcaccatattggccaggctgaactcgaactcccgaccttgtgatccacccaccttggcctcccaaagtgctgggattacaggcgtgagccaccacgcccggccagtagctactactttcaataacacacttttattgggtcttggtggagggagagggctgagggtcttaggaacacataatggatacaatccagcatgtcacaaagcattatcattctttcttctagattatggcaaagttcctgacttttgttcttccccttgccataagccagtgttggatctggtcttgccttagctgctacagctaacttttaaaaccatcatcatggtcaggcatggtggctcacgcctgtaatcccggcacttcgggaggccgaggcaggtggattacctgaggtcaggaattcaagaccagcctggccaacgtggtgaaaccccgtctctactaaaaatacaaaaattagccaggcgcggtggcacacacctgtaatcccagctactatggaggctgaggcaggagaatcgcttgaacccaggaggcggaggttgcagtgagccgagattgtgcaattcactccagcctgggtgacagaacaagactccgtctcaaaaaaaaaaaaaaacaaaacaaaacaaaaaaaaaaacagaaagcaaaaccatcatcactgctgggtgtcagtgcaccaagtatatgctgtaagtaattgcccttcactgaacaccctcaaaggatttcacaagtatctaccccctcccccaactttttttttgagacagggtctcactgttgcccagactggagtacagtgcagctcactgcatccttgacctcctgggctcaagtgatcctcctgcctcaacctcctgagtagctgggattgcaggtgtgcaccgctgtaaccagcttttaagaaacttttgtagacagggttttgtcacgttgccctgggtgttgtcatgctgagaagttttgatacattactcattcctgcaatgctctatgaattctacatattttcctaaatgagcaatcccatcccagggcatgtttagtgtagattattgttaccaaactggtaaaaataagccatggggaactggcagaataagcttcctcctgcaaggcaaattccacattttcccagaaaagggaaggggttctatctgtatcaggaggtggcaggttttttatacctcaactactcaactgtgccatggctgtgcaaaagcagtcaaataatacacaaatatatttagccatgttccaacaacagttatttatggacactcaagtttgaattttatatattgccaacatctactctatagccttaaatgaagcatctgcagtgcaaagtctatcagaagagtttgctaggctgagtcctcaggttcttcccagatactcctattcaaagtctatcagaagagtttgctaggctgagtcctcaggttcttcccagacattcctattcaaagtctatcagaagagtttgctaggctgagtcctcaggttcttcccagatactcctattcaaagtctatcagaagagtttgctaggctgagtcctcaggttcttcccagacattcctattcaaagtctatcagaagagtttgctaggctgaggcctcaggttcttcgcagatactgctattcaaagtctatcacaagagcttgctaggctgagtcctcaggttcttcccagatattcctattcaaattatcaagggataactttttgagggggggaagggtgaggataactttttcaacacatgtttacattaagggatttagtaaacatttgaggtgaactgactttaattcaccaagccaaatatactatttgattcccaccacctcactcctacagctgtaagaaactttttcagcaatgtcaaagttgccaagtctgacactccaccctgaggtgagatttcagggcttcaggcctgtcattctcatggtctaagatccagcaagatcaaaatcagccatctctgcccctgtctcagattttctcataaatttaaaattcttataatgctataattcttcagtgtttccaaaatttcagtatcaggcactacaacgttccaggtgtacagaaacaataaccatatttcacatgatggctaaaagttgctatcttcaaatataaacaagaatgtgattttcttgtctcaggaaaaacaaacaaacctaaatcatataccccactttgttaactacatgctaccaaggcaacaactgatcagttaaagcccttaggttataagaaatagaaagctggccgggctcggtggctcacacctgtaatcccatgactttgggaggctgaagtgggcagatcacctgaggtcaggagttcaagaccagcctggccaacatggtgaaaccccgtctatactaaaaatacaaatattagccaggcatgtaatcctagccacttgggaggctgaggcaaggaaattgcttgaacccaggaggtggaagttgcagtgagctgagatcatgccattgcattccagcctggaggacaagagtgaaacttagtctcaaaaaaaaaaaaaaaaaaaaaaaaaaaaaaacccaaacaacaaaaagcaaaagacatttttattgagaagtgaggaaacacacagatcagagaagcaggttctaaagggatcgtatccacagttattcttgtaatcaattagccagaatgaatggatgttctcaacagaattctgggacaagaatgaatgagttcccacattttctggttcatgtacaaatgaattacagactcaaaattctgaaaaagagattaccattatccaacaatgggtaaaatgctcacctgtagctagtggaacggatacctgaaagacactaccacaggaagcaccccagagaggggaggtatttctccagagaaaacaggggtgctcatgtcaatcaatggacaacaggcatggaactgcaaaatataataaacgttcattataatgagttctcttaagcggcagccctgtaataaatgccagatctgcttatgaaaaagaaatcaaaagataattagcatttaatatggaaaatactgggggatattattccacaaactatcaaatatatatatagatagatagaacaagttacattaaaaaataaagtacaaaaaattttagaaatactattcagtgttaactcaggaaagtcacattaaatatccattaactttaagactctgttccctgcgtttttcctgaacattatttacatatttttaaaaaaacaactttatactccaccatgaagtcaactgttcataccaagattttattttacaaaaacacagcttcaaatctggaatgtgactttccatggaacacactttcaatgggaaaatgcttccttaatttattcaacttataaggtgttcctagtgtaaattctctgaatcttcatgatgatactacaacatttgatacatttattgctccacattccttccattattttcatctacaaagatttgtaacttatttctgaaagcttttacactcatcccaaatatggttggtctctctcctctctgatttttgacatgagtgtaattttagggcctcctgcttgtaaatcctgtctatattatccgaagtctcctgaacatcagtttctcacattgcatcattctgatttctcatttatgagtcttccgatgtatacgaagccctgaattccaacagaaggatttcccacattcagagcatttccatggtttctctccggtgtgaactctctgatgttcactgagagatgacttctgagtgaaggcttttccacattcactgcatttaaaaggtttctctcccgaatgagttttctggtgtatctgaagtgatgccttcctagggtaggctttttcacattcattgcattcatagggcttctcagttgaatgagttctctgatgtataatcagctgtgattttccacaaaaggctctctcacacaaactacattcatagggtctctctccggtgtgtgttctcctatgtataacaaggtatgacttgctgctgaaagccttcccacattcactgcatccatagggcttctctcctgcatgagctctcagatgtgcagtgagctgttccttcctaccaaaggctttcccacattcaccgcattgataaggattatttcctgtgtgaactccctgatgtacaatgagttgtgtcttcatattgaaggctttcccacaatcactgcattgatagggtttttctcctgtatgcattcggatgtgaacaaggagataggacttactcctaaaggctttcccacattcactgcatttatggggtttcactcctgtatgagttctctggtgtacaacgaatggagacttcaaactaaaggctttcccacattcgctgcattcatacggtttcactcctgtgtgacttctctggtgtaaaagaagctgtgatttccaactgtaggctttcccacattcactgcagccatagggtttccctcctgtgtgaatttcctgatggacaatgagctgtgacctgaaagagaagaccttctcgcactcactacatgagtagggtttttctcctgtatgaactctctgatgagcattaaggtttgacttggcactgaaggctctttcacatttactgcattcataaggtctctctcctgtatgaattctgagatgtacaatgagctgtgacttacaacgaaaagctttcccacattcactacacacacagtttttttctatgctatgagctctttgatgcttaagaaaatatggttcttcataaccatgaaacttatcaggattctttcttaaataacttctgcttggagctgagttttgtgtcaaactttttccacgtgtgttatagagtctctgtcttgaagaatcatgggttttgctcagattaagtcttcccaacacactacaagcatagcttctttcaatactctcaagctcatcttgattgttctggtaccattcttcccagccatctggacagctctgcctggaaattttggcatttattatccatggatcttctccttgttccaacttgaagattaagtcaggcttggtaccatgataccccactgatatcaggttatgatagttttccaatatcacatctctgtacaggtacttctgtgtagaatccagtagctgccattcatcccaggtgaactccatagatatatccttgaatgacaataatccccagcacgaagctgtccggaaactggtggccatccccacgcccacgttcgcgcgctgcctgcgggggcaggacccgcgggctgcggagagaccgtgagggatgcgtccgcccgaagacaggtgcgggaccagggccccaggctcctgaccgtcccggggccgagtcgttggcagggacgccggctcctcagctctcgcccaacacagaccgcgcgtgactagacaacctcccggtctgggtaccaggagtcgcacggatggatttgtgcctttccgtggccctgactcgggagagcaggaggctgatctggccccgtccacgccccggaccgacggaagtgtttagctggtcaagtctctggtctgcccaggataatccgagccgcttagctccgcgcctccgcggccacagagactcagccaggtacacccgctggccagattccggtccactgagtctaagccggaaacagccctgcacgcgcgcacccgactaaggccgggagt

SEQ ID NO: 11655 - RNA, 10684 nt, Homo sapiens
  source 1..10684: mol_type = other RNA
ctgaatagctgggactacaggtgtctgccaccacaccccgctaacttttgtatttttagtagagacggggtttcaccaggctggtgaagctggtcttgaactcttgacctcaagtgatccacccacctcagcctcccaaagtgctgggattacaggcgtgagccaccacgcctggcctgatttcattttttggctcttgtggatagtgctgcaggaaacgtgagagtgcaggtgtctctttgatgtactgatttcctttcttttggcttttcacccagtagtggggttgctggatcgtataatagttctattttcagttgctttgaggagcctccatactgttctccatagtggctgtactaatttccactcccaccaacagtgtacgagggctgtccttcctccatatcctcaccagcatctgttctttcctgtctttctgatacaagccattttaactgaagagggatgatatctgattgtggttaatttgcatttctctgataagtggtgatattgagcattttttcatatacctgttagacatttgcatgtcttctctgagaaacgtctgtttggatcttttgcctactttataattggaatatctggagtttggggttttttttttgttatttttctttgtttttgctatagagttgtttgagctccctgtatattctggcaattaaccccttgtcaaatggatagtttgcaaatattttctcccaatctgtgggttgtctctttattttgttatttcctcggcagtatggaagcttcccagcttgatgtaatcccaattgtctatttataattgttacatcttcttgatgacttatctttacaaaatacttttctttatctctagtaaaacttttgttttaaactctattgtgtctgatattagaaagccactggagatttattatggttgctgtttgcgttttatatctttttccatcctttacttctaatccaattgtatctttgagtatgtatgtatgtcttctgtacatggttggatttttttttatcaccactttgacaatctgtgtcttttgatagtttaatctattcacatttaatgttattactggccaggtgcgctggctcatgcctataatcttgatgcttcgagagaccagaatgggaggattgcttgagccctggagtttgatacctccatctctataaataaataaataaaataaaataaaatagccaggtgggaggtgggagaattgcttgaagccaagagttcaaggctgcagtgagctatgatcatgcaactgcactccagcctgggcaatagagcaagaccctcttaaaaaaaagttattattgatatagttagatttacatatgctgctttcccttttgtattttatgtctcatgtatcttttgttcatctatttctccttcacttttgtcttaagtgcatattttgtaatgtaatattttatttatttaatgattccttacaatatttttgcagttatttctttagtgtttgttctaggaagtgttaaatacacattaacttatcagagtctacttcagatttatactaccttaattccaataagacttttataaacccattattcctatatagttctagcccccaccccgacttttgtgctggtattgatatatatatctatgttacaaatgcaacaacacattgctataaatattgctttatatattttataatttaaagaggctgagagatgaagagaaagtatatattaacagcttttgttacagtagcctatttatttcctatttctggttctctcagcttattcttgtggctttaagttgccatctagagccatttccttaccccaacacgactcttctcccatcctcctcctttgtggtgttattggtagacatattacacttctgtatgttatagtccaaacagtactgcatattgttttatataattgctttttttgttgctgttattgagacggagtctcactctgttgcccaggctgaagtgcggtggcgtgatctcggctcactgcaacctctgcctcctgggttcaagccattctcctgcctcagcctcccgagtagctgggactacaggcgcccgccaccacgccccgctaattttttgtgtttttaatagagatggggtttcaccatgttagtgaggatggtcttgacctccagaccttgtgatccgcccacctcggcctcccaaagtgctgggattacaggcgtgagccaccacgcctggcctataattattaatcagttactaataaaataagaaatctgcacttgcactatcttttattattacataattaccctttactggtgctctttgttttttctgtggaaacaaattactgcctggggtcattcctcagactgttgctcttcagtctccaaactgatcactggaaatgatgttaagtggagctgatcccgttcccactccttggctcttggacctgtgtacactccctattgaggaatcactaccagataaaagtctgtgattccaggactgcatcttggaggacggtgccctgtgcttgtcaagtactgccactaagctggtacttcaaaccaccttcagcaggtcatccaatgctctgtcacaccagccgcttctaggtggtggggtaagcataaggtgtgaccaatagatcagtcatgggaccaccactgaaccttatctgtggtaaagtgggtctccttgtctaatgccctgccatgtgggataatcagaatctctactcccctaaaaattattagacttcttccaatgttacatactgttattttctggggcttatttccatatttttgtaccatcaaattacatcttataatttttaagtctgtttagatttggccgagcatgactttttatttttttatgtttccaactttcttggtattaaatattttgtttaaaatgacattatttcaccctggtttgtgaataacccttctaggtagatattttctttcagaacattgaagacattcttttactgtcttctgatttttactgttgctattgagaagtcaacctaagcatgtaaaattggaaaagggcaactcaatgataaaatatcagactttcaactaatattcccatccttacaacctccaatgatggtatctcataacatattacaaataccaagagagtagaatttttttttttttttgagtcaaggtcttgctctgtcacccaggctggagtgcagtggtacaaatatggcttactgcagcttcaacctcctgggctcaagcaatcctcctgcctcagcctccagagtagctgggaccacagccctaagccaccatcccggggtattttttttttttcagagatggggttttgctttgttgtccagactggtctcaaattcctgagctcaagtgatcctcctgcctcccaaagtgttgggattataggcataagccactgcacccagccagagtagggctgattttaaattttagactttggccccaaagtgagctgttattttccttttactgtgatgctcttaaaatagttaaaaaaaaaaaaaaaaagtagctaaattgtttttaaaaattaaggatgctctggccgggtacgatggctcatgcctgtaatcctagcactttgggaggccaaggcgggtggatcacctgaggtcaggagtttgagaccatcctggccaaaatggtgaaaccccatctctactaaaaatacaaaaattagccaggtgtggtggcaggtgcctgtaatcccagctactcaggaggctgaggcaggagaatcacctgaaccccagaggcggaagttgcagtgagccgagatcacgccactgcactccagcatgggtgacacagtgagactctgtctcaaaaaaaaaaaaaaaaaaaaattacccctacactttttcacaataaaccttagatcttcaagacactcacaaaaccaaaagccacttccttctctcaacacttacccccaagacaaatgaagatatatggaaatatatggcatacctagttcagacttctattaaagagtcacacaaacattccatcaataaacatgcagcatgaatttctaaataaacgtctgcttgaagcacttttatttgccagtagaagtaatatttccaactgtctcaggtcaagagttccttttggcctccagcctgatctcagactggactttcctctttgggaactcctatgccctctactcagaagactgtcctcttggcttcttttggcttttcagcaacattgacatttgtcttctgtattattattatatagtttgtttatttatttttactttttacagatatgaggtcttgccctgtcatccaggctgaaacacaatcatggctcactgcatcctcaaccttctgggctgaagcgacactcctgcctcagcctcccaagtagctgggaccataggaaagcatcttattttttttcattttttagttctctttcttattcttttgccacaagttgataattgaggccgatgcaagtgaagacatagatacatgccacagttaggattgtgtcatatacacagaacatgtgtttgtcattttcttttctttttttttttttttttgagacagagtctcactctgtcacccaggctggagtgcaatggcgcaatctctgctcactgccacctccacctcccgggttccagcgattctcctgcctcagcctcccaagtagctgggattacaggcgcccgccaccatgcccgactaatttttgtatttttagttgagacgggatttcaccatattggccaggctgaactcgaactcccgaccttgtgatccacccaccttggcctcccaaagtgctgggattacaggcgtgagccaccacgcccggccagtagctactactttcaataacacacttttattgggtcttggtggagggagagggctgagggtcttaggaacacataatggatacaatccagcatgtcacaaagcattatcattctttcttctagattatggcaaagttcctgacttttgttcttccccttgccataagccagtgttggatctggtcttgccttagctgctacagctaacttttaaaaccatcatcatggtcaggcatggtggctcacgcctgtaatcccggcacttcgggaggccgaggcaggtggattacctgaggtcaggaattcaagaccagcctggccaacgtggtgaaaccccgtctctactaaaaatacaaaaattagccaggcgcggtggcacacacctgtaatcccagctactatggaggctgaggcaggagaatcgcttgaacccaggaggcggaggttgcagtgagccgagattgtgcaattcactccagcctgggtgacagaacaagactccgtctcaaaaaaaaaaaaaaacaaaacaaaacaaaaaaaaaaacagaaagcaaaaccatcatcactgctgggtgtcagtgcaccaagtatatgctgtaagtaattgcccttcactgaacaccctcaaaggatttcacaagtatctaccccctcccccaactttttttttgagacagggtctcactgttgcccagactggagtacagtgcagctcactgcatccttgacctcctgggctcaagtgatcctcctgcctcaacctcctgagtagctgggattgcaggtgtgcaccgctgtaaccagcttttaagaaacttttgtagacagggttttgtcacgttgccctgggtgttgtcatgctgagaagttttgatacattactcattcctgcaatgctctatgaattctacatattttcctaaatgagcaatcccatcccagggcatgtttagtgtagattattgttaccaaactggtaaaaataagccatggggaactggcagaataagcttcctcctgcaaggcaaattccacattttcccagaaaagggaaggggttctatctgtatcaggaggtggcaggttttttatacctcaactactcaactgtgccatggctgtgcaaaagcagtcaaataatacacaaatatatttagccatgttccaacaacagttatttatggacactcaagtttgaattttatatattgccaacatctactctatagccttaaatgaagcatctgcagtgcaaagtctatcagaagagtttgctaggctgagtcctcaggttcttcccagatactcctattcaaagtctatcagaagagtttgctaggctgagtcctcaggttcttcccagacattcctattcaaagtctatcagaagagtttgctaggctgagtcctcaggttcttcccagatactcctattcaaagtctatcagaagagtttgctaggctgagtcctcaggttcttcccagacattcctattcaaagtctatcagaagagtttgctaggctgaggcctcaggttcttcgcagatactgctattcaaagtctatcacaagagcttgctaggctgagtcctcaggttcttcccagatattcctattcaaattatcaagggataactttttgagggggggaagggtgaggataactttttcaacacatgtttacattaagggatttagtaaacatttgaggtgaactgactttaattcaccaagccaaatatactatttgattcccaccacctcactcctacagctgtaagaaactttttcagcaatgtcaaagttgccaagtctgacactccaccctgaggtgagatttcagggcttcaggcctgtcattctcatggtctaagatccagcaagatcaaaatcagccatctctgcccctgtctcagattttctcataaatttaaaattcttataatgctataattcttcagtgtttccaaaatttcagtatcaggcactacaacgttccaggtgtacagaaacaataaccatatttcacatgatggctaaaagttgctatcttcaaatataaacaagaatgtgattttcttgtctcaggaaaaacaaacaaacctaaatcatataccccactttgttaactacatgctaccaaggcaacaactgatcagttaaagcccttaggttataagaaatagaaagctggccgggctcggtggctcacacctgtaatcccatgactttgggaggctgaagtgggcagatcacctgaggtcaggagttcaagaccagcctggccaacatggtgaaaccccgtctatactaaaaatacaaatattagccaggcatgtaatcctagccacttgggaggctgaggcaaggaaattgcttgaacccaggaggtggaagttgcagtgagctgagatcatgccattgcattccagcctggaggacaagagtgaaacttagtctcaaaaaaaaaaaaaaaaaaaaaaaaaaaaaaacccaaacaacaaaaagcaaaagacatttttattgagaagtgaggaaacacacagatcagagaagcaggttctaaagggatcgtatccacagttattcttgtaatcaattagccagaatgaatggatgttctcaacagaattctgggacaagaatgaatgagttcccacattttctggttcatgtacaaatgaattacagactcaaaattctgaaaaagagattaccattatccaacaatgggtaaaatgctcacctgtagctagtggaacggatacctgaaagacactaccacaggaagcaccccagagaggggaggtatttctccagagaaaacaggggtgctcatgtcaatcaatggacaacaggcatggaactgcaaaatataataaacgttcattataatgagttctcttaagcggcagccctgtaataaatgccagatctgcttatgaaaaagaaatcaaaagataattagcatttaatatggaaaatactgggggatattattccacaaactatcaaatatatatatagatagatagaacaagttacattaaaaaataaagtacaaaaaattttagaaatactattcagtgttaactcaggaaagtcacattaaatatccattaactttaagactctgttccctgcgtttttcctgaacattatttacatatttttaaaaaaacaactttatactccaccatgaagtcaactgttcataccaagattttattttacaaaaacacagcttcaaatctggaatgtgactttccatggaacacactttcaatgggaaaatgcttccttaatttattcaacttataaggtgttcctagtgtaaattctctgaatcttcatgatgatactacaacatttgatacatttattgctccacattccttccattattttcatctacaaagatttgtaacttatttctgaaagcttttacactcatcccaaatatggttggtctctctcctctctgatttttgacatgagtgtaattttagggcctcctgcttgtaaatcctgtctatattatccgaagtctcctgaacatcagtttctcacattgcatcattctgatttctcatttatgagtcttccgatgtatacgaagccctgaattccaacagaaggatttcccacattcagagcatttccatggtttctctccggtgtgaactctctgatgttcactgagagatgacttctgagtgaaggcttttccacattcactgcatttaaaaggtttctctcccgaatgagttttctggtgtatctgaagtgatgccttcctagggtaggctttttcacattcattgcattcatagggcttctcagttgaatgagttctctgatgtataatcagctgtgattttccacaaaaggctctctcacacaaactacattcatagggtctctctccggtgtgtgttctcctatgtataacaaggtatgacttgctgctgaaagccttcccacattcactgcatccatagggcttctctcctgcatgagctctcagatgtgcagtgagctgttccttcctaccaaaggctttcccacattcaccgcattgataaggattatttcctgtgtgaactccctgatgtacaatgagttgtgtcttcatattgaaggctttcccacaatcactgcattgatagggtttttctcctgtatgcattcggatgtgaacaaggagataggacttactcctaaaggctttcccacattcactgcatttatggggtttcactcctgtatgagttctctggtgtacaacgaatggagacttcaaactaaaggctttcccacattcgctgcattcatacggtttcactcctgtgtgacttctctggtgtaaaagaagctgtgatttccaactgtaggctttcccacattcactgcagccatagggtttccctcctgtgtgaatttcctgatggacaatgagctgtgacctgaaagagaagaccttctcgcactcactacatgagtagggtttttctcctgtatgaactctctgatgagcattaaggtttgacttggcactgaaggctctttcacatttactgcattcataaggtctctctcctgtatgaattctgagatgtacaatgagctgtgacttacaacgaaaagctttcccacattcactacacacacagtttttttctatgctatgagctctttgatgcttaagaaaatatggttcttcataaccatgaaacttatcaggattctttcttaaataacttctgcttggagctgagttttgtgtcaaactttttccacgtgtgttatagagtctctgtcttgaagaatcatgggttttgctcagattaagtcttcccaacacactacaagcatagcttctttcaatactctcaagctcatcttgattgttctggtaccattcttcccagccatctggacagctctgcctggaaattttggcatttattatccatggatcttctccttgttccaacttgaagattaagtcaggcttggtaccatgataccccactgatatcaggttatgatagttttccaatatcacatctctgtacaggtacttctgtgtagaatccagtagctgccattcatcccaggtgaactccatagatatatccttgaatgacaataatccctcaggcagggcactgtttccctgggcccaaggaacacccagaagattcccgaacttgacacttgagctcattagcaggctcctcctcagcagcactacccagcacgaagctgtccggaaactggtggccatccccacgcccacgttcgcgcgctgcctgcgggggcaggacccgcgggctgcggagagaccgtgagggatgcgtccgcccgaagacaggtgcgggaccagggccccaggctcctgaccgtcccggggccgagtcgttggcagggacgccggctcctcagctctcgcccaacacagaccgcgcgtgactagacaacctcccggtctgggtaccaggagtcgcacggatggatttgtgcctttccgtggccctgactcgggagagcaggaggctgatctggccccgtccacgccccggaccgacggaagtgtttagctggtcaagtctctggtctgcccaggataatccgagccgcttagctccgcgcctccgcggccacagagactcagccaggtacacccgctggccagattccggtccactgagtctaagccggaaacagccctgcacgcgcgcacccgactaaggccgggagt

SEQ ID NO: 11656 - RNA, 10689 nt, Homo sapiens
  source 1..10689: mol_type = other RNA
ctgaatagctgggactacaggtgtctgccaccacaccccgctaacttttgtatttttagtagagacggggtttcaccaggctggtgaagctggtcttgaactcttgacctcaagtgatccacccacctcagcctcccaaagtgctgggattacaggcgtgagccaccacgcctggcctgatttcattttttggctcttgtggatagtgctgcaggaaacgtgagagtgcaggtgtctctttgatgtactgatttcctttcttttggcttttcacccagtagtggggttgctggatcgtataatagttctattttcagttgctttgaggagcctccatactgttctccatagtggctgtactaatttccactcccaccaacagtgtacgagggctgtccttcctccatatcctcaccagcatctgttctttcctgtctttctgatacaagccattttaactgaagagggatgatatctgattgtggttaatttgcatttctctgataagtggtgatattgagcattttttcatatacctgttagacatttgcatgtcttctctgagaaacgtctgtttggatcttttgcctactttataattggaatatctggagtttggggttttttttttgttatttttctttgtttttgctatagagttgtttgagctccctgtatattctggcaattaaccccttgtcaaatggatagtttgcaaatattttctcccaatctgtgggttgtctctttattttgttatttcctcggcagtatggaagcttcccagcttgatgtaatcccaattgtctatttataattgttacatcttcttgatgacttatctttacaaaatacttttctttatctctagtaaaacttttgttttaaactctattgtgtctgatattagaaagccactggagatttattatggttgctgtttgcgttttatatctttttccatcctttacttctaatccaattgtatctttgagtatgtatgtatgtcttctgtacatggttggatttttttttatcaccactttgacaatctgtgtcttttgatagtttaatctattcacatttaatgttattactggccaggtgcgctggctcatgcctataatcttgatgcttcgagagaccagaatgggaggattgcttgagccctggagtttgatacctccatctctataaataaataaataaaataaaataaaatagccaggtgggaggtgggagaattgcttgaagccaagagttcaaggctgcagtgagctatgatcatgcaactgcactccagcctgggcaatagagcaagaccctcttaaaaaaaagttattattgatatagttagatttacatatgctgctttcccttttgtattttatgtctcatgtatcttttgttcatctatttctccttcacttttgtcttaagtgcatattttgtaatgtaatattttatttatttaatgattccttacaatatttttgcagttatttctttagtgtttgttctaggaagtgttaaatacacattaacttatcagagtctacttcagatttatactaccttaattccaataagacttttataaacccattattcctatatagttctagcccccaccccgacttttgtgctggtattgatatatatatctatgttacaaatgcaacaacacattgctataaatattgctttatatattttataatttaaagaggctgagagatgaagagaaagtatatattaacagcttttgttacagtagcctatttatttcctatttctggttctctcagcttattcttgtggctttaagttgccatctagagccatttccttaccccaacacgactcttctcccatcctcctcctttgtggtgttattggtagacatattacacttctgtatgttatagtccaaacagtactgcatattgttttatataattgctttttttgttgctgttattgagacggagtctcactctgttgcccaggctgaagtgcggtggcgtgatctcggctcactgcaacctctgcctcctgggttcaagccattctcctgcctcagcctcccgagtagctgggactacaggcgcccgccaccacgccccgctaattttttgtgtttttaatagagatggggtttcaccatgttagtgaggatggtcttgacctccagaccttgtgatccgcccacctcggcctcccaaagtgctgggattacaggcgtgagccaccacgcctggcctataattattaatcagttactaataaaataagaaatctgcacttgcactatcttttattattacataattaccctttactggtgctctttgttttttctgtggaaacaaattactgcctggggtcattcctcagactgttgctcttcagtctccaaactgatcactggaaatgatgttaagtggagctgatcccgttcccactccttggctcttggacctgtgtacactccctattgaggaatcactaccagataaaagtctgtgattccaggactgcatcttggaggacggtgccctgtgcttgtcaagtactgccactaagctggtacttcaaaccaccttcagcaggtcatccaatgctctgtcacaccagccgcttctaggtggtggggtaagcataaggtgtgaccaatagatcagtcatgggaccaccactgaaccttatctgtggtaaagtgggtctccttgtctaatgccctgccatgtgggataatcagaatctctactcccctaaaaattattagacttcttccaatgttacatactgttattttctggggcttatttccatatttttgtaccatcaaattacatcttataatttttaagtctgtttagatttggccgagcatgactttttatttttttatgtttccaactttcttggtattaaatattttgtttaaaatgacattatttcaccctggtttgtgaataacccttctaggtagatattttctttcagaacattgaagacattcttttactgtcttctgatttttactgttgctattgagaagtcaacctaagcatgtaaaattggaaaagggcaactcaatgataaaatatcagactttcaactaatattcccatccttacaacctccaatgatggtatctcataacatattacaaataccaagagagtagaatttttttttttttttgagtcaaggtcttgctctgtcacccaggctggagtgcagtggtacaaatatggcttactgcagcttcaacctcctgggctcaagcaatcctcctgcctcagcctccagagtagctgggaccacagccctaagccaccatcccggggtattttttttttttcagagatggggttttgctttgttgtccagactggtctcaaattcctgagctcaagtgatcctcctgcctcccaaagtgttgggattataggcataagccactgcacccagccagagtagggctgattttaaattttagactttggccccaaagtgagctgttattttccttttactgtgatgctcttaaaatagttaaaaaaaaaaaaaaaaagtagctaaattgtttttaaaaattaaggatgctctggccgggtacgatggctcatgcctgtaatcctagcactttgggaggccaaggcgggtggatcacctgaggtcaggagtttgagaccatcctggccaaaatggtgaaaccccatctctactaaaaatacaaaaattagccaggtgtggtggcaggtgcctgtaatcccagctactcaggaggctgaggcaggagaatcacctgaaccccagaggcggaagttgcagtgagccgagatcacgccactgcactccagcatgggtgacacagtgagactctgtctcaaaaaaaaaaaaaaaaaaaaattacccctacactttttcacaataaaccttagatcttcaagacactcacaaaaccaaaagccacttccttctctcaacacttacccccaagacaaatgaagatatatggaaatatatggcatacctagttcagacttctattaaagagtcacacaaacattccatcaataaacatgcagcatgaatttctaaataaacgtctgcttgaagcacttttatttgccagtagaagtaatatttccaactgtctcaggtcaagagttccttttggcctccagcctgatctcagactggactttcctctttgggaactcctatgccctctactcagaagactgtcctcttggcttcttttggcttttcagcaacattgacatttgtcttctgtattattattatatagtttgtttatttatttttactttttacagatatgaggtcttgccctgtcatccaggctgaaacacaatcatggctcactgcatcctcaaccttctgggctgaagcgacactcctgcctcagcctcccaagtagctgggaccataggaaagcatcttattttttttcattttttagttctctttcttattcttttgccacaagttgataattgaggccgatgcaagtgaagacatagatacatgccacagttaggattgtgtcatatacacagaacatgtgtttgtcattttcttttctttttttttttttttttgagacagagtctcactctgtcacccaggctggagtgcaatggcgcaatctctgctcactgccacctccacctcccgggttccagcgattctcctgcctcagcctcccaagtagctgggattacaggcgcccgccaccatgcccgactaatttttgtatttttagttgagacgggatttcaccatattggccaggctgaactcgaactcccgaccttgtgatccacccaccttggcctcccaaagtgctgggattacaggcgtgagccaccacgcccggccagtagctactactttcaataacacacttttattgggtcttggtggagggagagggctgagggtcttaggaacacataatggatacaatccagcatgtcacaaagcattatcattctttcttctagattatggcaaagttcctgacttttgttcttccccttgccataagccagtgttggatctggtcttgccttagctgctacagctaacttttaaaaccatcatcatggtcaggcatggtggctcacgcctgtaatcccggcacttcgggaggccgaggcaggtggattacctgaggtcaggaattcaagaccagcctggccaacgtggtgaaaccccgtctctactaaaaatacaaaaattagccaggcgcggtggcacacacctgtaatcccagctactatggaggctgaggcaggagaatcgcttgaacccaggaggcggaggttgcagtgagccgagattgtgcaattcactccagcctgggtgacagaacaagactccgtctcaaaaaaaaaaaaaaacaaaacaaaacaaaaaaaaaaacagaaagcaaaaccatcatcactgctgggtgtcagtgcaccaagtatatgctgtaagtaattgcccttcactgaacaccctcaaaggatttcacaagtatctaccccctcccccaactttttttttgagacagggtctcactgttgcccagactggagtacagtgcagctcactgcatccttgacctcctgggctcaagtgatcctcctgcctcaacctcctgagtagctgggattgcaggtgtgcaccgctgtaaccagcttttaagaaacttttgtagacagggttttgtcacgttgccctgggtgttgtcatgctgagaagttttgatacattactcattcctgcaatgctctatgaattctacatattttcctaaatgagcaatcccatcccagggcatgtttagtgtagattattgttaccaaactggtaaaaataagccatggggaactggcagaataagcttcctcctgcaaggcaaattccacattttcccagaaaagggaaggggttctatctgtatcaggaggtggcaggttttttatacctcaactactcaactgtgccatggctgtgcaaaagcagtcaaataatacacaaatatatttagccatgttccaacaacagttatttatggacactcaagtttgaattttatatattgccaacatctactctatagccttaaatgaagcatctgcagtgcaaagtctatcagaagagtttgctaggctgagtcctcaggttcttcccagatactcctattcaaagtctatcagaagagtttgctaggctgagtcctcaggttcttcccagacattcctattcaaagtctatcagaagagtttgctaggctgagtcctcaggttcttcccagatactcctattcaaagtctatcagaagagtttgctaggctgagtcctcaggttcttcccagacattcctattcaaagtctatcagaagagtttgctaggctgaggcctcaggttcttcgcagatactgctattcaaagtctatcacaagagcttgctaggctgagtcctcaggttcttcccagatattcctattcaaattatcaagggataactttttgagggggggaagggtgaggataactttttcaacacatgtttacattaagggatttagtaaacatttgaggtgaactgactttaattcaccaagccaaatatactatttgattcccaccacctcactcctacagctgtaagaaactttttcagcaatgtcaaagttgccaagtctgacactccaccctgaggtgagatttcagggcttcaggcctgtcattctcatggtctaagatccagcaagatcaaaatcagccatctctgcccctgtctcagattttctcataaatttaaaattcttataatgctataattcttcagtgtttccaaaatttcagtatcaggcactacaacgttccaggtgtacagaaacaataaccatatttcacatgatggctaaaagttgctatcttcaaatataaacaagaatgtgattttcttgtctcaggaaaaacaaacaaacctaaatcatataccccactttgttaactacatgctaccaaggcaacaactgatcagttaaagcccttaggttataagaaatagaaagctggccgggctcggtggctcacacctgtaatcccatgactttgggaggctgaagtgggcagatcacctgaggtcaggagttcaagaccagcctggccaacatggtgaaaccccgtctatactaaaaatacaaatattagccaggcatgtaatcctagccacttgggaggctgaggcaaggaaattgcttgaacccaggaggtggaagttgcagtgagctgagatcatgccattgcattccagcctggaggacaagagtgaaacttagtctcaaaaaaaaaaaaaaaaaaaaaaaaaaaaaaacccaaacaacaaaaagcaaaagacatttttattgagaagtgaggaaacacacagatcagagaagcaggttctaaagggatcgtatccacagttattcttgtaatcaattagccagaatgaatggatgttctcaacagaattctgggacaagaatgaatgagttcccacattttctggttcatgtacaaatgaattacagactcaaaattctgaaaaagagattaccattatccaacaatgggtaaaatgctcacctgtagctagtggaacggatacctgaaagacactaccacaggaagcaccccagagaggggaggtatttctccagagaaaacaggggtgctcatgtcaatcaatggacaacaggcatggaactgcaaaatataataaacgttcattataatgagttctcttaagcggcagccctgtaataaatgccagatctgcttatgaaaaagaaatcaaaagataattagcatttaatatggaaaatactgggggatattattccacaaactatcaaatatatatatagatagatagaacaagttacattaaaaaataaagtacaaaaaattttagaaatactattcagtgttaactcaggaaagtcacattaaatatccattaactttaagactctgttccctgcgtttttcctgaacattatttacatatttttaaaaaaacaactttatactccaccatgaagtcaactgttcataccaagattttattttacaaaaacacagcttcaaatctggaatgtgactttccatggaacacactttcaatgggaaaatgcttccttaatttattcaacttataaggtgttcctagtgtaaattctctgaatcttcatgatgatactacaacatttgatacatttattgctccacattccttccattattttcatctacaaagatttgtaacttatttctgaaagcttttacactcatcccaaatatggttggtctctctcctctctgatttttgacatgagtgtaattttagggcctcctgcttgtaaatcctgtctatattatccgaagtctcctgaacatcagtttctcacattgcatcattctgatttctcatttatgagtcttccgatgtatacgaagccctgaattccaacagaaggatttcccacattcagagcatttccatggtttctctccggtgtgaactctctgatgttcactgagagatgacttctgagtgaaggcttttccacattcactgcatttaaaaggtttctctcccgaatgagttttctggtgtatctgaagtgatgccttcctagggtaggctttttcacattcattgcattcatagggcttctcagttgaatgagttctctgatgtataatcagctgtgattttccacaaaaggctctctcacacaaactacattcatagggtctctctccggtgtgtgttctcctatgtataacaaggtatgacttgctgctgaaagccttcccacattcactgcatccatagggcttctctcctgcatgagctctcagatgtgcagtgagctgttccttcctaccaaaggctttcccacattcaccgcattgataaggattatttcctgtgtgaactccctgatgtacaatgagttgtgtcttcatattgaaggctttcccacaatcactgcattgatagggtttttctcctgtatgcattcggatgtgaacaaggagataggacttactcctaaaggctttcccacattcactgcatttatggggtttcactcctgtatgagttctctggtgtacaacgaatggagacttcaaactaaaggctttcccacattcgctgcattcatacggtttcactcctgtgtgacttctctggtgtaaaagaagctgtgatttccaactgtaggctttcccacattcactgcagccatagggtttccctcctgtgtgaatttcctgatggacaatgagctgtgacctgaaagagaagaccttctcgcactcactacatgagtagggtttttctcctgtatgaactctctgatgagcattaaggtttgacttggcactgaaggctctttcacatttactgcattcataaggtctctctcctgtatgaattctgagatgtacaatgagctgtgacttacaacgaaaagctttcccacattcactacacacacagtttttttctatgctatgagctctttgatgcttaagaaaatatggttcttcataaccatgaaacttatcaggattctttcttaaataacttctgcttggagctgagttttgtgtcaaactttttccacgtgtgttatagagtctctgtcttgaagaatcatgggttttgctcagattaagtcttcccaacacactacaagcatagcttctttcaatactctcaagctcatcttgattgttctggtaccattcttcccagccatctggacagctctgcctggaaattttggcatttattatccatggatcttctccttgttccaacttgaagattaagtcaggcttggtaccatgataccccactgatatcaggttatgatagttttccaatatcacatctctgtacaggtacttctgtgtagaatccagtagctgccattcatcccaggtgaactccatagatatatccttgaatgacaataatccctcggtcctcttgagggttccagttggtcacactctgagcttccacgaatacaataaggtgtctttatgtatttccagtttagacctcccatgtgagttacaggccagcacgaagctgtccggaaactggtggccatccccacgcccacgttcgcgcgctgcctgcgggggcaggacccgcgggctgcggagagaccgtgagggatgcgtccgcccgaagacaggtgcgggaccagggccccaggctcctgaccgtcccggggccgagtcgttggcagggacgccggctcctcagctctcgcccaacacagaccgcgcgtgactagacaacctcccggtctgggtaccaggagtcgcacggatggatttgtgcctttccgtggccctgactcgggagagcaggaggctgatctggccccgtccacgccccggaccgacggaagtgtttagctggtcaagtctctggtctgcccaggataatccgagccgcttagctccgcgcctccgcggccacagagactcagccaggtacacccgctggccagattccggtccactgagtctaagccggaaacagccctgcacgcgcgcacccgactaaggccgggagt

SEQ ID NO: 11657 - RNA, 16352 nt, Homo sapiens
  source 1..16352: mol_type = other RNA
ctgaatagctgggactacaggtgtctgccaccatgcccagctaattttttgtagttttggtagagatgggctttcaccgtgttagccaggatggtcttgatctcctgacctcatgatccacccacctcagcctcccaaagtgctgggatttcaggcgtgagccactgcgcctggcagatgtgactcactttatgatcacatcacaagctaaaggaaaatggcgagccaggtgtggcggctcacgcctgtaatcccagcactttgggaggctgaggcgggtggatcacttggaaggatgtcttgatccagagtaaaggctccataggcatttattggttgacaaggttggcatatgttgtatgaataagagcttccgtatgtgataaggtttctctctgtggatgacatagccatggggtcgcctgctgcctcccggttacccatacaaaccatggaaacaggaatgggtgacagccccacgctcccctgctgtgagcctccaatcccctggctggctaaacagcagcaccagctcctccttctgtccagccggacagagagcctggaggaagctggagtctgggtttcagtggctacagacaaccctccaaatggtcagttaagaaccagggccacattgtgagtggacactttcacactctgcaggtgaccacgcaaagtggtagagcaacttattttatttttgtcattcttttgaggcagggtcttgctgtgtctcccaggctggggtgcagtggcataatcactgcagccttgacctcccactttgttacctgtttccgacggtgtgacccgagtgcgcttcgttacccgtttctgatggcatgacccgactgcactttgttacctgttttgatggttgtttctgatggcgtgacccaactgtgcctcgttacccgtttccgatggtgtgacctgactgtgctttgttacctgtttctgatggttgtttctgatggtgtgacccgactgtgttttgttacctgtttccgatggtgtgacctgactgcgctttgttacctgtttctgatggttgtttctgatggtgtgacccgactgtgttttgttacctgtttctgatggttgtttctggtggtgtgacccaactgcactttgttacctgtttctgatggtgtgacatgactgcgcttcgttacccatttccgatggtgtgacctgactacgctttgttacctgtttctggtggtgtgacccaactgtgatttgttacctgtttctgatgtttgtttctgatggtgtgacctgactgctttgttacctgtttccaatggcgtgacctgactgagctttgttacctgtttctgatggtgtgacctgactgctttgttacctgtttccaatggtgtgacctgactgcgctttgttacctgtttccgatggtgtgacctgactgctttgttacctgtttccaatggcgtgacctgactgcgctttgttacctgtttctgatggcgtgacctgactgcgctttgttacctctttccgatagcgggatctgactgcattttgcattcatgggggcaccgtctggcaaggtgagcttgtcagggagaggccgtagccctcaccaccgctaatgactggctaccacacagaggttccaggcagagtctagctactggagccaaccagcgtggcttcggccagttaacagaccacttcttggagtcatgaggattaactcagtgagcccatggaaaatgcacaaactaagccctcaataaatatagcctgatgaactgccattctgcctatccgaattctaccctaagatagataatcagagatgctaggagaaaacatgagcatgtgagtggctaagagtatggattctggagtcaggcaacctgggttcaaggcctgctgtagtattacccaaacttgggcaagtttgttcatcttctgaagagagcttcatttctcacctggacctgtatccgtaataactgtatgcatatcatagcactgtcatgaggattagatgagttaatacatgtcgaatgattggtgcataataaatgctcaataattgtgagctggcattacccattccattgtatgtggcatgacaatgtgaaaccacttaaatcattgacaataaagaaagggttaaacagtctgcagtgcatccatgtgaggggaggttatgctgtctctaagttatctagaaagatttttactgacaagagaatattaagtgaaaagatccatacggtgttatagatagtatgatttcacttcattaaatatctatacttggctgggcgctgtggctcacgcctgtaagtaatcccagcactttgggaggccgaggtgggcggatcacgaggtcaggagatcaagaccatcctggccaacacggcgaaaccccgtctctactaaaaatgcaaaaaattagccaggcgtggtggcacgtgcctgtaatcctagctactcgggaggctggggcaggagaatcacttgaacccgggaggtggaggttgcagtgagccgagatcgcaccactgcactccagcctgggcaattgagcgagactccatcccaaaaaacaaaaaaatctatactcatgggagaatgctgcaagacaacaggccaaaatgctgagaaggtgagcgctaaatagtggaatttaatgatcttagtcttcgtatgtctgaaattgtccccaaggtgactatggtaagtgaaatgatggtcccaaaagatgcctgcatcctactttctggaacctgtgaagatggtcacttacctggcaaaaggggctgtgcagatgccatttgatgagggatcttcagatggggagagtgtcttggattatccaggtaagaccaatgtaatcaggaggctcttacaagggaaagagggagacaggagggtcagaggcagagaaggaggagtcacagagatcgctctacagcagaggtcggagtgatgccactgccggcagtgaacatggccatgagccaagcacacccctgagaaactggaaagggcaaagtttgatgtctttcctagtacttccagaaagaacagccctgccgtcaccttgccttttgccccatgaggcccgttttagacttctgacccccagaactacatgtaagacaggaaatgtgcgttgttttattgggtgcagtgtatactgctcgggtgatgggtgcaccaaaatctcacaaatcaccactaaagaacttactcatgtaaccactgtgttccccaataacctatgaaaataaaaaattaaaattctatagaatttgaagaacaaaatgtaaatctgcataaatctctgttaatagatacaggatataaaatgatataattttaatattaatagctgaaaatgtaaagagttttgtattcagttgaagttgttatgagattaaaatatattgttataacttaaaaaagaaagaaaaaattgtatgctgttttaagccactatatttgtggcaatttgttgtagcagcaacaggcagctgatacagtgggtgtaggttttacgatcacaaaagaaaagaaaaagctgcttgcttaaacaaacaaacaaacaaacaaaaaaacagctgggcacagtggctcacgcctgtaatcccagcactttgggaggctgaggcgggcagatcacctgaagcaggagttcgagaccagcctgacctacatggtgaaactctgtctctactaagcacaaaaaatcaaaaatacaaaacaaaaaaacaaacaaaaaaaaaacaaaaaacaaaaatcagctggacgtgatggcgcatgcctgtaatcccagccactcgggaggctgagtcaggagaacagcttgaacccaggaggcggaggttgcagtgagtcgagattgtgccattgcgctccagcctggacaacaagagcgaaactccttctcaaaaaaaaaaaaaaaaaaaaaaaagccgtgggtgaactggcttcatttctatacaggagctctgtccatctgccagtgcagacaggcacagtccagatccaaaggacaagctggctcaagattttgaaagcaatgaagtgaaatttgaagttgaaatttttgaagtgaaattgtaaagttgaaagccagagaatctgaaaacactggactgaaaagtctcattgtgtctgagctctgcccctttcttatttaattttgtagttttaaaaactgctacataggccaggcacactgactcacacctgttatcccagacctttaagaggctgaggggaccagatcacttgagaccaggagttggagatcagcctaggcaacatggcaaaactctgtctctgaaaaaaattagtggggcttggcatctgtagtcccagctactcaggaggctgaggtgggaggatcacttgagcctgggaggtggaggctgcagtgaactgagatcgtgccactgtactccagcctcggtgacagagcaagaccccatctcaagtagaacaaaaacaaacaaataaaaaccaaaactacataaaactatttgtaaaactatataaaactacataaaaatatttgtaaaaattaacatagttacctttggacaacatattaaagaaagaaactctggagataatttaaagttgatcccctatttgtacattacaggatgctcttccctcttcacatggtctggtccttgctggcaatgtgaggatgggccaatgtgaggatgggccagcccttttgcaaactggctgggcctagtcatctggtacaaagtggcagaacctgacgcttttgggcttctgctcaccatccctcttaaaggtgaagaagcccagtgtcctccagggtgggcaccttcttgtcactcaatgtcactgtcttacagaggtgtccccgaccagccaatctaaagtaaccctccccctgtcacttcaaatttgctctaatcatctgccaagctggtaattatcttatttgtttacccctctgtttggggtctgtcttcccagtccccaataagaccaccagctccccagcccaggtacctgtgtctggccaggggtccttgatacaccgtggctgaacacaggcaggaaggcctcactgccacctgggtgggtggaggttcaggctgggctgggtgctcaggaagcctccatgggcttggggaggtcattttcctggtagctgtgccttcctgggtactgctgaatggcaggctaagctcaggctggaaaccctgacctcctgccatgcccgggggaggagccatgcaggggtagggctgggctgtgctcggccatgtgcttgtgttttacacaccctctgaatctttacaaccaccttgttctccccatttcacagatgaggaaaccgaggctcagagaggactagtgactcacctaaggctcctaggagagtaggtggccaggtcccgatgcaggctccagcccagcaggcccacaacccgagcccttgggccacaggcaccgcctcaggcagtggcggatgggagcctcctgtgctgtgaccaagtgggacagggatgcatgaccctcctcaggccttggctggacccagggcccgaggatgaccctgtggggtcaaggaggcaaagacaagagtggtggcggtcacagaggcccccagccatgcccatgctgaccaggcccctcacctcctcctccatgcagagcgggactcggactctgcctcagctgcagctagctctgcccttcctgccctgcttcagggacccctcagcacgtcccagcagccactcacccctcgcctgaggatagaagaaagaaggaaagactttatggtgcaccccgggggccccatgccctgtccaggttgacctctgttaatatccccaaaagcccgtaagggaagttactccccgaccatagagatgaggagacagagtgcttccccatcagaggtgacacggccaggcagaactgggattccagccagatctgtgtgacccacagcccagtggtcaccaggaaaccctattgtcctcagggggtcaagggccaaacagcagaagatgagggagacgaggagggtggtgggggctgtgggtggcccggatggtcagcgggagctgctggctccaggcagacctgcagaagatcccccaccaccttcctgccacctctccatagtcagccccactcagggcttgagtgtccaggaggagtcctgcctgctggcctggccctgaggccctgtgtggtggtcctgaggggcggtagccctcgtgtcccctacctggcacacaccacctctgacagctgcctgcagactcacatctcagcccagaaggcaggctgggcagaggtgactgtcctcatctgattctgagtccagggagggacagtggcacagtgaggatcacccccagcaggtgcagagctggagtgggtcccccacggtgtgaccttgagggggggcctcagcctggcccccaaaagaccttcaggaggagcacattcctgtctgaaatggtgcaggatgtcctttttctgttcctatctggctgcagcgtgggcaggggcagcaggaaatgcatgaccacaagtgtgggaggaatgttagtggcgggaacggccgcagccctaaggctcagccctggggctcggcccattttcctgtgtggggtcctcaggcccagtgcggctgctactgcccgcctcccccggaggactccggccaggcctcaaaggcttatggtcaagtgtgtggctgcttctggagtaggcaggatggacagggcaagcagacgctaggggagggatgggagcagccacctggtacagtgcccaagacacagtttacagaacttcaatatgagtggtgtcccctcactgggcaatgcccaccctgtcggccttgagaggtggtgggggaggagcaggaatgagaaggtggcgatatggagagagggggccgagtggcaggggccgagcgctgggagggtatgggggcattggagggagacagtggccagagtggctgaccctgccctgaaattccttcagtagggccgggtcacccattccagcctggagccggctgtgctgcagggacctgggctggggctggggcagcaggtgacaggctggtgacaggcccagcacggacagggcagacgtggagaactccaaggatgatggggagggtgcctgcaaaggggggacttcctgcaggcagagagtctgggcccgcaatgatgactgtgtggccgccggggagatgcgtggggccatctggaggagtctgggttgctccatgtgatcacagacacgcccacctgtgcacgagcatgcacctcccccaggccatgaccacaggtagggggcatggaggataacgggaggccttggttccctcctttccccaccgagggaggtccccacgcagccctgagggtgagcagagccctggccacagcccagggcccaggacctggaaggaggcagagagacagacagacgagcccatggatcccaaatggggctggggatgggaagtggcctgccccggccacacctgcccaggcccccagcctggctctgtcctgagatcctcttggctgagtggggcggctccttcaaagaagggcctcctccctcctctgcctcctccttcccttcctggtccattcgccaccccaccctgcccgaagttggctccctgctcactgaggagtgggtgccccgtccccagggctccctggcttgggggtacccaggcctctgcctccctgctgctgctgctctggggaaccaccaggcccccagccaaggcagcccccctcagcttccctctctccttcctcacgcctgccctgctggaaacacaaggtgctcagcgaggccgccttcaacactcaacacggccccttccccaccggactcctaacctgtgttctcagctcccctctgcagctacgctcttgaaagagacttcaccttttcctcccccttgagcccactccaacctggcttgaccccaccttagtcagcttgggctgccgtaagaaaaccgccacagacaggtggcttcaacaatgaacttaatttctcacagtcctggaggttcaaagaacaaagcaaaggttccagcccatctgggttcctgtgaggctccctcctggcttgcgggtggccgccttctccgtgtgtcctggcgtggctgagcgtgagctcacttgcactttagagtttcttctggtgaggacgccaatcctactgggccagggcccctcctgatgacctcacttcacctgaattacttccttaaggggcctatctccaaatatagtcacacaggggcgggggctccaccctatgaatctgggggagcaaaactgcatccccagcatggctctggtcaaggtcactgccaacctgcacaccaccaggcccacggtcagctctcaggccaccctgacggggtctccaggcattgagagagcccacccacctcctccaggaagctcaccctgcctgctctccgcctcccttgcagctgctcctgcgccttctttcctgatctcttcatttcccagcctgtaaaccccgccagccccggagctcagccctgacctcttcctctttgtctatgcttgtcccgaagtggccccgtcaggcccatggctcccagccccgcatccctgacacctcccacactctcgcctcatcttgggctctcgcctgggctcctgcccagccagctgcctccccctcagaggctccacaggcattttgtattcaacctgcctgaaagcagactcctgccttctcctctcctccccaacctattcttcctgtttcctggccatcatcgccatccttccagtagctcaggacaagaccctcaccctcatccctggcgtctcccctccctcacacccagctccatgtgtgagcaaccctcttggctctgtcttcagaatcttcacagtccagtgcctctcgccacttcctccacgccccttggtctaagcaccatggtcgctgtgtgacagcaggagcctgacagcctcccagctcccacgctgcggcctgcagaataacgtgctccccctgcccctcaaagacgtccacatcccgagccctggaacctgtgactatgttgccttccatgacagatggagcgatgcagatgtgattgaacgaaggctctcgaggtggggcaatggccctggactatccagggggcccagagcaaccagcagagtccttagagggaggcaggaggtcaaaggcagaaaggtgacgcagtgacggagcagaggaaggaaaggtgacgtgaggtggccacgagccaaggccgcaggaagcctctagccgctggagaagacggggacacccgtcctcctccagagcctggggaaggagcacagccccactgaaagcttgatttgacttctgacctccaaaacaaagagaataaatttgtgttaagacgctaagtttgcggtcatttaaaatttttaatttattttatttgtagagatagggtcttgctctctcatgcaggctggactgcggtggcgtgatcactcactgcagcctcaaccacctgggctcaagcaatcagcccatctcagcctcccaagcagctgggactacaggtgcacgccaccaaacctggctatttttttttttttgtagagatggggggggggtctcaccatgttgcccaggctggtcttgaactcctggcctcagctgattctcctgcctcagcctccctaagtgctgggattacaggcaggagccaccatgcccagccagtttatggtaatttgctgcaaccacaggcaattaatatacactgttagcatggtccacgaggccgcacctgtgtggcccctgttaaacttctgacctcttctcatccttcaccacctgaccatccccctcccctctgggcctttgcacctgctgttcctgcttcctgagatgtcctcctcccaggttacctgtctttcttcagccagatgtcaccttcttagcgaggcttccctagtcaccttctaaacagcagccctgccactccctacaccccttccctggcttcatctttctccatgcgtcaccccacctgccatactcctcatctgtctgtttccttctaccagaaggtaggtcctaagtggatgcagcatctgtgtcacacattgctgtgccctcagtgcctggaataagcatctggcatgttgtgagcattccatagatatttgttggatgaatgaatgagtgaatgaatgaatgaaatttcacagatggggagactaagaccagggaacaggaacgccttgcctaagttagggtcagcactagtcctggaatcaaacgcggcatctcctgcatctcactgtccaaaaaatgcctccactgggcagacctgggcacttttgaaatgtttatccctcaggcctgtctcaatcttagttctgccaggtaattccacaatgaccccaggcaggtgtcctgccgtcttagtgtctagcgtctgcgtcctcatctattaatggatggacggatggatggatggatggatggatggatggatggatggatggacggacggacggacgggtggacggatgaatggatggatggatggatggacggatggatgaatgtccttagttgggaaaggctcagcaggtcagaagactaggaagaaggccagagccatgagagggcttggggaaggagaggcagccaggcacacagggggctgggacacagagtctggttccaggcaagggcttgagaagccatcaggggtttatagagagaaccgactcaatcctcccttctaagaggactgtgcagacattggactgtgtggggctggggccaaggtactggggatgaagttgaatgggagagatttgagatgcgatttgggtagaaaagacaagatttactggaaaacagaatatgaggtgggtgagtgggattaaggtgggggactgaggagtctggaagagtgcccaaggggggagtaccaaggacggcaggactttcctgcatttcttaggtaccttttaggtagaagtgatggaaacccctgtgcttgcactaagcaagatgggaaactgtatggattcctatgatggaaaaatctcgggccgcagtgctccagcggtgacccggggcccggctctctttccacctcctcattctctttttctgtgttggcatcattctcaggcaggccaccccatataatgtcaaatggcacccacagccccccactggcatcctattaggacatcaaacccagcagaaagaggctttttttctaatgttttcataacaaaagtcccaggggtgcttctcattggccaagcatgggtcacatgcccaaacccaaaccagtcactgatactggggagctggagggctctggttgttaaggctgggcccatgtgtccatccttgagccatgtgggtggagagtgggggtggttccctgagggagatgaagacaatggagaggtgccgggcagacacacaggagccagcccccgcgccctgcagggctgatacgcacaggagtctctgaggtgagggcctggcagagaaggtctggtacagcgcctgcaccatctgccttggtggcccagcctcctcccttcctggtcctgatccagtgggccttgccccacgctcccgcatgggatggcagagcccagccctgtgcctccaatcagggcaagctgccaccacactgagtacctgccccaggtcctacattgcaaattccatgacttatgaccactcaaagccacaagtgctgcctggcagggtcagtgctgaggctggggctcctacctactgtctctccctccttggctgccccctagcccgcctgcctcagtgagccagagaggtcgtgcccagtttgaatgcagtcctctaggcttcagggcacctaagttcagagctcagccctccatatttccctgtgtcctggaaaggtggggccaccctacagctgtccctgagagactgcagatacctgctcagtttctctctggttccggatcttgctgtctactctgtgggattcggactttggctcaaacacctctacaccttcttctcatggtggcaagagggctgctgcagttccagcctcacttctcagcttgaaaggcagcaggaaagagcgacagccttctctgtggctcccgctctgactggaccgctttaggtcacatgctcactcctgaccctctgtggcccatgagtgcaggaggctgcttgggcaggactgaattgcatgctccaattccaaagccccatcgggggagagctaaggcgaattcccaaaccaaaaccagggctgttgctgcaaaaaggaggcctgggtgctgaggacgcaggaaacacgtccctacctagggatcatcttcaaattataagtgaggagatggccgggcatggtggctcacaccagcactttcggaggctgaggcgggagggctgcttgagtccaggagttcaggaccagcctgggtaacacagtgagatcccgtctctacaaaaacaaacaaacaaaattagccgggcatgctagtgtgcgcctgtgatcccagctactcaggaggctgaggtgggaggatcacctgaacctgggaagtcgaggctgcagtgatctgtgatcgcaccactgaactccagcctgggaaacagagtgagaccctgtctccaaaaaataaaaataaaataagtggggaaagagaggctgggctttctagtgtcaagggctgacatgtccagagtgggcccccaggtacagacagctccccaccccaggaactaagcctttctcaggtctttgagcttttacgaatgacacaggctatgagtccatttaaaaatcattttattattaacatcatcttcccatgtagccaagtgtctgtcatgtataaggaatgtcggtaaatattccatttgaagcttctttgtacatatttccctcgataaataaactctgaattcacataaaaaagttaaacttaaataactcatatttccttctcttgtaacaggcatatattggtaaaatataaatattctcggactcaggctttgttctaagtgaggacagtaattgatcacatggtacaattattgacagtaaaaccaagaaattgtcagctggtgtcctggcatggactagtgctgaggtgggagacaggaagttcacatttggtttctgggccaaagtggggcaggaggggtggtggggagaaaaggacagttgttttctttacagctctgataaaaataatctgtgctgccactgaattttaactttgaatatattcttctacatttgctgattaattccataatcattttactgaaaactcagatgtcaactaacaaaatatggcacatgatccattttgaacaatgtcaataggttcagaaactaccattgggctggcaaaaaaaacaagagaaacgcacatggcgagagcgatgattcggggttggtttggttggttcactgtggcccactgaacactcgtccctggcctcagtgtggcagattcatccccttggggcgatggcacaagccctggtgcccggcagggcctctgaggcctgagcggcaggtgaggctggcaggcgcctgctcagagcacgcgggggatgatggtgaagggcacggcggggctgctggcctccagctccaaggctgtcaggaagcactccgtagccgccgcatcgttgccctgagcttggaggacctcgcccagcccgttccagacctcgtgggctgtcgagttcacctgcaccgcgtcccggaggatcttctccgccagactgtagcggcctagctggtgaaggatcagggccagtcgctgcatgctcttcacgtgggtggggctgatggctaaggcctcttcataccaccgccgcgcctcgtccatgcttccccggagctcagcaatctggccgcgcatgtagaggacattgtgggacattgggaagaggttggcagcttcttgggtacaggctgtggcttctgcaggcttcccgatgccgatatagacttcagctgcatggagccagatctgtgccagcgtcatccaggggtgcagcgggccctgcttaggggcactgctctgcagagacgaagccacttccgacagtgcctgctccactcttgaggctgctaccgatgtggcatggacggagcctgtctcgggatcgctgaagtctggcaaagtaattgtattaagctgtcgtctgtcagcaatggttctatctaagaggctgctcccacgtccagaatcactggggttggtgaggttgtagcaggatttccatatctgcagcatgtgcttacaagtcagcagtgcctcgtccgggcctcggcagagtgactgcaacttcactttggaaaacagtagtatgaaattttctgggtattcactcagggccatgtcgatgatgttcagagcgtcatggtaatgcttctgtgctgacagcaggagggcaaggaggtgcagggagttggcatcgtcaccttgaagctgaagagcttggcggacataccccagagcctctgggatctgtctggagatggcaagctgcagagccaggtagaaagctgcttggtgatctgtgggtgacaggctgtgggccctctgaaatgcaagaagcgcctttctctgtaggacctcctgcatccctcgcaaagaagcgtcagtggcctgcagactgtacgtgagccccagagctaagtagcctttggccttgaactctgacgttttctctcccacatcaacgacagttttggcaaacttttcagcctcttccaaccagtgcagggagcccatgcagagcttggcagcgaggagagggatggtggcatcgtctggcttcaggcggatacactctttcagcaccttcacggcacgggcagattttccagcagccatcagggacagagcaaactggtaccacaggtggaattcctcaaaggcaaacttcatggctctttctaggcactctgacagcatctcatactggcctcttcttccaagagcaatggtgagtaagtcatagaccacagatgcactctgcagactgatgaggcggtcactcttgtgttcaggtatcctgctcagcacagcgtcccggttggccattgattcactaatcagcaataacaacagggcttcttccgtattttcttgaggacaaaaaatgttctctcctgagtagacacgggctctccgagtgagagtgtaggtttttgtgtttgctcctttgcggagaggatcgtccagaggtgactggcacggtggatcctccagagggttccagtagctctgctcacacataccccgcaacaagatctctgccagctgcctggctattgtcattcgcaggttttgagtcgttcttgtttcaactgctctgagaagctctctaaatcttccgactcctcttgtcaagttcccatttttgaaatagaggacatgggctctctgaagtcctgtttctaggaaaaaacctagttcttgatcgtggggagcagggccaggcttagggcttctgttttgaatattagaaagtattaccctttctatctcttggagatacaggagtgcgatgtcccctgctttctcataacaggtgatgacatcctgttcccggtccacatggagattactggtagaagaagaaataggcagcttctccaaacaaagtcctttggtagcgtaggcttctgcgatcacccgcagcctgtagggcgggacagctgtcagtggcagatcgtccaggcccacccgggcgtaaatgttcagagcttctttataatcaccttccacataattcaacttggccatgatcagattggattcttgtaggaattctgacttaaggttccctcggtccagggcggcggtcagatgcttgcggacctcagtcagctggggcttggggcctcggggactggccccctgcctcagggggtgttccttcaggtactgctccagcttcgactccccgaggagaagctctgccatgtcatcgttggcgatgagcttggccgacagctgcttgacgagctcagggatccgctcccactggcactcggagcggcagcgctcgatctccgtctccagccgcgagcctgccttcttggtcgccatcgcggcctggccgggcccggccgcccgccccgcaggccccaccgccgccgccgcggcgccccctcgccgcctcccgccgccgccgcgggctcgggctccggctcccggctccgcggcgtaacgggagcgccggct

SEQ ID NO: 11658 - RNA, 16399 nt, Homo sapiens
  source 1..16399: mol_type = other RNA
ctgaatagctgggactacaggtgtctgccaccatgcccagctaattttttgtagttttggtagagatgggctttcaccgtgttagccaggatggtcttgatctcctgacctcatgatccacccacctcagcctcccaaagtgctgggatttcaggcgtgagccactgcgcctggcagatgtgactcactttatgatcacatcacaagctaaaggaaaatggcgagccaggtgtggcggctcacgcctgtaatcccagcactttgggaggctgaggcgggtggatcacttggaaggatgtcttgatccagagtaaaggctccataggcatttattggttgacaaggttggcatatgttgtatgaataagagcttccgtatgtgataaggtttctctctgtggatgacatagccatggggtcgcctgctgcctcccggttacccatacaaaccatggaaacaggaatgggtgacagccccacgctcccctgctgtgagcctccaatcccctggctggctaaacagcagcaccagctcctccttctgtccagccggacagagagcctggaggaagctggagtctgggtttcagtggctacagacaaccctccaaatggtcagttaagaaccagggccacattgtgagtggacactttcacactctgcaggtgaccacgcaaagtggtagagcaacttattttatttttgtcattcttttgaggcagggtcttgctgtgtctcccaggctggggtgcagtggcataatcactgcagccttgacctcccactttgttacctgtttccgacggtgtgacccgagtgcgcttcgttacccgtttctgatggcatgacccgactgcactttgttacctgttttgatggttgtttctgatggcgtgacccaactgtgcctcgttacccgtttccgatggtgtgacctgactgtgctttgttacctgtttctgatggttgtttctgatggtgtgacccgactgtgttttgttacctgtttccgatggtgtgacctgactgcgctttgttacctgtttctgatggttgtttctgatggtgtgacccgactgtgttttgttacctgtttctgatggttgtttctggtggtgtgacccaactgcactttgttacctgtttctgatggtgtgacatgactgcgcttcgttacccatttccgatggtgtgacctgactacgctttgttacctgtttctggtggtgtgacccaactgtgatttgttacctgtttctgatgtttgtttctgatggtgtgacctgactgctttgttacctgtttccaatggcgtgacctgactgagctttgttacctgtttctgatggtgtgacctgactgctttgttacctgtttccaatggtgtgacctgactgcgctttgttacctgtttccgatggtgtgacctgactgctttgttacctgtttccaatggcgtgacctgactgcgctttgttacctgtttctgatggcgtgacctgactgcgctttgttacctctttccgatagcgggatctgactgcattttgcattcatgggggcaccgtctggcaaggtgagcttgtcagggagaggccgtagccctcaccaccgctaatgactggctaccacacagaggttccaggcagagtctagctactggagccaaccagcgtggcttcggccagttaacagaccacttcttggagtcatgaggattaactcagtgagcccatggaaaatgcacaaactaagccctcaataaatatagcctgatgaactgccattctgcctatccgaattctaccctaagatagataatcagagatgctaggagaaaacatgagcatgtgagtggctaagagtatggattctggagtcaggcaacctgggttcaaggcctgctgtagtattacccaaacttgggcaagtttgttcatcttctgaagagagcttcatttctcacctggacctgtatccgtaataactgtatgcatatcatagcactgtcatgaggattagatgagttaatacatgtcgaatgattggtgcataataaatgctcaataattgtgagctggcattacccattccattgtatgtggcatgacaatgtgaaaccacttaaatcattgacaataaagaaagggttaaacagtctgcagtgcatccatgtgaggggaggttatgctgtctctaagttatctagaaagatttttactgacaagagaatattaagtgaaaagatccatacggtgttatagatagtatgatttcacttcattaaatatctatacttggctgggcgctgtggctcacgcctgtaagtaatcccagcactttgggaggccgaggtgggcggatcacgaggtcaggagatcaagaccatcctggccaacacggcgaaaccccgtctctactaaaaatgcaaaaaattagccaggcgtggtggcacgtgcctgtaatcctagctactcgggaggctggggcaggagaatcacttgaacccgggaggtggaggttgcagtgagccgagatcgcaccactgcactccagcctgggcaattgagcgagactccatcccaaaaaacaaaaaaatctatactcatgggagaatgctgcaagacaacaggccaaaatgctgagaaggtgagcgctaaatagtggaatttaatgatcttagtcttcgtatgtctgaaattgtccccaaggtgactatggtaagtgaaatgatggtcccaaaagatgcctgcatcctactttctggaacctgtgaagatggtcacttacctggcaaaaggggctgtgcagatgccatttgatgagggatcttcagatggggagagtgtcttggattatccaggtaagaccaatgtaatcaggaggctcttacaagggaaagagggagacaggagggtcagaggcagagaaggaggagtcacagagatcgctctacagcagaggtcggagtgatgccactgccggcagtgaacatggccatgagccaagcacacccctgagaaactggaaagggcaaagtttgatgtctttcctagtacttccagaaagaacagccctgccgtcaccttgccttttgccccatgaggcccgttttagacttctgacccccagaactacatgtaagacaggaaatgtgcgttgttttattgggtgcagtgtatactgctcgggtgatgggtgcaccaaaatctcacaaatcaccactaaagaacttactcatgtaaccactgtgttccccaataacctatgaaaataaaaaattaaaattctatagaatttgaagaacaaaatgtaaatctgcataaatctctgttaatagatacaggatataaaatgatataattttaatattaatagctgaaaatgtaaagagttttgtattcagttgaagttgttatgagattaaaatatattgttataacttaaaaaagaaagaaaaaattgtatgctgttttaagccactatatttgtggcaatttgttgtagcagcaacaggcagctgatacagtgggtgtaggttttacgatcacaaaagaaaagaaaaagctgcttgcttaaacaaacaaacaaacaaacaaaaaaacagctgggcacagtggctcacgcctgtaatcccagcactttgggaggctgaggcgggcagatcacctgaagcaggagttcgagaccagcctgacctacatggtgaaactctgtctctactaagcacaaaaaatcaaaaatacaaaacaaaaaaacaaacaaaaaaaaaacaaaaaacaaaaatcagctggacgtgatggcgcatgcctgtaatcccagccactcgggaggctgagtcaggagaacagcttgaacccaggaggcggaggttgcagtgagtcgagattgtgccattgcgctccagcctggacaacaagagcgaaactccttctcaaaaaaaaaaaaaaaaaaaaaaaagccgtgggtgaactggcttcatttctatacaggagctctgtccatctgccagtgcagacaggcacagtccagatccaaaggacaagctggctcaagattttgaaagcaatgaagtgaaatttgaagttgaaatttttgaagtgaaattgtaaagttgaaagccagagaatctgaaaacactggactgaaaagtctcattgtgtctgagctctgcccctttcttatttaattttgtagttttaaaaactgctacataggccaggcacactgactcacacctgttatcccagacctttaagaggctgaggggaccagatcacttgagaccaggagttggagatcagcctaggcaacatggcaaaactctgtctctgaaaaaaattagtggggcttggcatctgtagtcccagctactcaggaggctgaggtgggaggatcacttgagcctgggaggtggaggctgcagtgaactgagatcgtgccactgtactccagcctcggtgacagagcaagaccccatctcaagtagaacaaaaacaaacaaataaaaaccaaaactacataaaactatttgtaaaactatataaaactacataaaaatatttgtaaaaattaacatagttacctttggacaacatattaaagaaagaaactctggagataatttaaagttgatcccctatttgtacattacaggatgctcttccctcttcacatggtctggtccttgctggcaatgtgaggatgggccaatgtgaggatgggccagcccttttgcaaactggctgggcctagtcatctggtacaaagtggcagaacctgacgcttttgggcttctgctcaccatccctcttaaaggtgaagaagcccagtgtcctccagggtgggcaccttcttgtcactcaatgtcactgtcttacagaggtgtccccgaccagccaatctaaagtaaccctccccctgtcacttcaaatttgctctaatcatctgccaagctggtaattatcttatttgtttacccctctgtttggggtctgtcttcccagtccccaataagaccaccagctccccagcccaggtacctgtgtctggccaggggtccttgatacaccgtggctgaacacaggcaggaaggcctcactgccacctgggtgggtggaggttcaggctgggctgggtgctcaggaagcctccatgggcttggggaggtcattttcctggtagctgtgccttcctgggtactgctgaatggcaggctaagctcaggctggaaaccctgacctcctgccatgcccgggggaggagccatgcaggggtagggctgggctgtgctcggccatgtgcttgtgttttacacaccctctgaatctttacaaccaccttgttctccccatttcacagatgaggaaaccgaggctcagagaggactagtgactcacctaaggctcctaggagagtaggtggccaggtcccgatgcaggctccagcccagcaggcccacaacccgagcccttgggccacaggcaccgcctcaggcagtggcggatgggagcctcctgtgctgtgaccaagtgggacagggatgcatgaccctcctcaggccttggctggacccagggcccgaggatgaccctgtggggtcaaggaggcaaagacaagagtggtggcggtcacagaggcccccagccatgcccatgctgaccaggcccctcacctcctcctccatgcagagcgggactcggactctgcctcagctgcagctagctctgcccttcctgccctgcttcagggacccctcagcacgtcccagcagccactcacccctcgcctgaggatagaagaaagaaggaaagactttatggtgcaccccgggggccccatgccctgtccaggttgacctctgttaatatccccaaaagcccgtaagggaagttactccccgaccatagagatgaggagacagagtgcttccccatcagaggtgacacggccaggcagaactgggattccagccagatctgtgtgacccacagcccagtggtcaccaggaaaccctattgtcctcagggggtcaagggccaaacagcagaagatgagggagacgaggagggtggtgggggctgtgggtggcccggatggtcagcgggagctgctggctccaggcagacctgcagaagatcccccaccaccttcctgccacctctccatagtcagccccactcagggcttgagtgtccaggaggagtcctgcctgctggcctggccctgaggccctgtgtggtggtcctgaggggcggtagccctcgtgtcccctacctggcacacaccacctctgacagctgcctgcagactcacatctcagcccagaaggcaggctgggcagaggtgactgtcctcatctgattctgagtccagggagggacagtggcacagtgaggatcacccccagcaggtgcagagctggagtgggtcccccacggtgtgaccttgagggggggcctcagcctggcccccaaaagaccttcaggaggagcacattcctgtctgaaatggtgcaggatgtcctttttctgttcctatctggctgcagcgtgggcaggggcagcaggaaatgcatgaccacaagtgtgggaggaatgttagtggcgggaacggccgcagccctaaggctcagccctggggctcggcccattttcctgtgtggggtcctcaggcccagtgcggctgctactgcccgcctcccccggaggactccggccaggcctcaaaggcttatggtcaagtgtgtggctgcttctggagtaggcaggatggacagggcaagcagacgctaggggagggatgggagcagccacctggtacagtgcccaagacacagtttacagaacttcaatatgagtggtgtcccctcactgggcaatgcccaccctgtcggccttgagaggtggtgggggaggagcaggaatgagaaggtggcgatatggagagagggggccgagtggcaggggccgagcgctgggagggtatgggggcattggagggagacagtggccagagtggctgaccctgccctgaaattccttcagtagggccgggtcacccattccagcctggagccggctgtgctgcagggacctgggctggggctggggcagcaggtgacaggctggtgacaggcccagcacggacagggcagacgtggagaactccaaggatgatggggagggtgcctgcaaaggggggacttcctgcaggcagagagtctgggcccgcaatgatgactgtgtggccgccggggagatgcgtggggccatctggaggagtctgggttgctccatgtgatcacagacacgcccacctgtgcacgagcatgcacctcccccaggccatgaccacaggtagggggcatggaggataacgggaggccttggttccctcctttccccaccgagggaggtccccacgcagccctgagggtgagcagagccctggccacagcccagggcccaggacctggaaggaggcagagagacagacagacgagcccatggatcccaaatggggctggggatgggaagtggcctgccccggccacacctgcccaggcccccagcctggctctgtcctgagatcctcttggctgagtggggcggctccttcaaagaagggcctcctccctcctctgcctcctccttcccttcctggtccattcgccaccccaccctgcccgaagttggctccctgctcactgaggagtgggtgccccgtccccagggctccctggcttgggggtacccaggcctctgcctccctgctgctgctgctctggggaaccaccaggcccccagccaaggcagcccccctcagcttccctctctccttcctcacgcctgccctgctggaaacacaaggtgctcagcgaggccgccttcaacactcaacacggccccttccccaccggactcctaacctgtgttctcagctcccctctgcagctacgctcttgaaagagacttcaccttttcctcccccttgagcccactccaacctggcttgaccccaccttagtcagcttgggctgccgtaagaaaaccgccacagacaggtggcttcaacaatgaacttaatttctcacagtcctggaggttcaaagaacaaagcaaaggttccagcccatctgggttcctgtgaggctccctcctggcttgcgggtggccgccttctccgtgtgtcctggcgtggctgagcgtgagctcacttgcactttagagtttcttctggtgaggacgccaatcctactgggccagggcccctcctgatgacctcacttcacctgaattacttccttaaggggcctatctccaaatatagtcacacaggggcgggggctccaccctatgaatctgggggagcaaaactgcatccccagcatggctctggtcaaggtcactgccaacctgcacaccaccaggcccacggtcagctctcaggccaccctgacggggtctccaggcattgagagagcccacccacctcctccaggaagctcaccctgcctgctctccgcctcccttgcagctgctcctgcgccttctttcctgatctcttcatttcccagcctgtaaaccccgccagccccggagctcagccctgacctcttcctctttgtctatgcttgtcccgaagtggccccgtcaggcccatggctcccagccccgcatccctgacacctcccacactctcgcctcatcttgggctctcgcctgggctcctgcccagccagctgcctccccctcagaggctccacaggcattttgtattcaacctgcctgaaagcagactcctgccttctcctctcctccccaacctattcttcctgtttcctggccatcatcgccatccttccagtagctcaggacaagaccctcaccctcatccctggcgtctcccctccctcacacccagctccatgtgtgagcaaccctcttggctctgtcttcagaatcttcacagtccagtgcctctcgccacttcctccacgccccttggtctaagcaccatggtcgctgtgtgacagcaggagcctgacagcctcccagctcccacgctgcggcctgcagaataacgtgctccccctgcccctcaaagacgtccacatcccgagccctggaacctgtgactatgttgccttccatgacagatggagcgatgcagatgtgattgaacgaaggctctcgaggtggggcaatggccctggactatccagggggcccagagcaaccagcagagtccttagagggaggcaggaggtcaaaggcagaaaggtgacgcagtgacggagcagaggaaggaaaggtgacgtgaggtggccacgagccaaggccgcaggaagcctctagccgctggagaagacggggacacccgtcctcctccagagcctggggaaggagcacagccccactgaaagcttgatttgacttctgacctccaaaacaaagagaataaatttgtgttaagacgctaagtttgcggtcatttaaaatttttaatttattttatttgtagagatagggtcttgctctctcatgcaggctggactgcggtggcgtgatcactcactgcagcctcaaccacctgggctcaagcaatcagcccatctcagcctcccaagcagctgggactacaggtgcacgccaccaaacctggctatttttttttttttgtagagatggggggggggtctcaccatgttgcccaggctggtcttgaactcctggcctcagctgattctcctgcctcagcctccctaagtgctgggattacaggcaggagccaccatgcccagccagtttatggtaatttgctgcaaccacaggcaattaatatacactgttagcatggtccacgaggccgcacctgtgtggcccctgttaaacttctgacctcttctcatccttcaccacctgaccatccccctcccctctgggcctttgcacctgctgttcctgcttcctgagatgtcctcctcccaggttacctgtctttcttcagccagatgtcaccttcttagcgaggcttccctagtcaccttctaaacagcagccctgccactccctacaccccttccctggcttcatctttctccatgcgtcaccccacctgccatactcctcatctgtctgtttccttctaccagaaggtaggtcctaagtggatgcagcatctgtgtcacacattgctgtgccctcagtgcctggaataagcatctggcatgttgtgagcattccatagatatttgttggatgaatgaatgagtgaatgaatgaatgaaatttcacagatggggagactaagaccagggaacaggaacgccttgcctaagttagggtcagcactagtcctggaatcaaacgcggcatctcctgcatctcactgtccaaaaaatgcctccactgggcagacctgggcacttttgaaatgtttatccctcaggcctgtctcaatcttagttctgccaggtaattccacaatgaccccaggcaggtgtcctgccgtcttagtgtctagcgtctgcgtcctcatctattaatggatggacggatggatggatggatggatggatggatggatggatggatggacggacggacggacgggtggacggatgaatggatggatggatggatggacggatggatgaatgtccttagttgggaaaggctcagcaggtcagaagactaggaagaaggccagagccatgagagggcttggggaaggagaggcagccaggcacacagggggctgggacacagagtctggttccaggcaagggcttgagaagccatcaggggtttatagagagaaccgactcaatcctcccttctaagaggactgtgcagacattggactgtgtggggctggggccaaggtactggggatgaagttgaatgggagagatttgagatgcgatttgggtagaaaagacaagatttactggaaaacagaatatgaggtgggtgagtgggattaaggtgggggactgaggagtctggaagagtgcccaaggggggagtaccaaggacggcaggactttcctgcatttcttaggtaccttttaggtagaagtgatggaaacccctgtgcttgcactaagcaagatgggaaactgtatggattcctatgatggaaaaatctcgggccgcagtgctccagcggtgacccggggcccggctctctttccacctcctcattctctttttctgtgttggcatcattctcaggcaggccaccccatataatgtcaaatggcacccacagccccccactggcatcctattaggacatcaaacccagcagaaagaggctttttttctaatgttttcataacaaaagtcccaggggtgcttctcattggccaagcatgggtcacatgcccaaacccaaaccagtcactgatactggggagctggagggctctggttgttaaggctgggcccatgtgtccatccttgagccatgtgggtggagagtgggggtggttccctgagggagatgaagacaatggagaggtgccgggcagacacacaggagccagcccccgcgccctgcagggctgatacgcacaggagtctctgaggtgagggcctggcagagaaggtctggtacagcgcctgcaccatctgccttggtggcccagcctcctcccttcctggtcctgatccagtgggccttgccccacgctcccgcatgggatggcagagcccagccctgtgcctccaatcagggcaagctgccaccacactgagtacctgccccaggtcctacattgcaaattccatgacttatgaccactcaaagccacaagtgctgcctggcagggtcagtgctgaggctggggctcctacctactgtctctccctccttggctgccccctagcccgcctgcctcagtgagccagagaggtcgtgcccagtttgaatgcagtcctctaggcttcagggcacctaagttcagagctcagccctccatatttccctgtgtcctggaaaggtggggccaccctacagctgtccctgagagactgcagatacctgctcagtttctctctggttccggatcttgctgtctactctgtgggattcggactttggctcaaacacctctacaccttcttctcatggtggcaagagggctgctgcagttccagcctcacttctcagcttgaaaggcagcaggaaagagcgacagccttctctgtggctcccgctctgactggaccgctttaggtcacatgctcactcctgaccctctgtggcccatgagtgcaggaggctgcttgggcaggactgaattgcatgctccaattccaaagccccatcgggggagagctaaggcgaattcccaaaccaaaaccagggctgttgctgcaaaaaggaggcctgggtgctgaggacgcaggaaacacgtccctacctagggatcatcttcaaattataagtgaggagatggccgggcatggtggctcacaccagcactttcggaggctgaggcgggagggctgcttgagtccaggagttcaggaccagcctgggtaacacagtgagatcccgtctctacaaaaacaaacaaacaaaattagccgggcatgctagtgtgcgcctgtgatcccagctactcaggaggctgaggtgggaggatcacctgaacctgggaagtcgaggctgcagtgatctgtgatcgcaccactgaactccagcctgggaaacagagtgagaccctgtctccaaaaaataaaaataaaataagtggggaaagagaggctgggctttctagtgtcaagggctgacatgtccagagtgggcccccaggtacagacagctccccaccccaggaactaagcctttctcaggtctttgagcttttacgaatgacacaggctatgagtccatttaaaaatcattttattattaacatcatcttcccatgtagccaagtgtctgtcatgtataaggaatgtcggtaaatattccatttgaagcttctttgtacatatttccctcgataaataaactctgaattcacataaaaaagttaaacttaaataactcatatttccttctcttgtaacaggcatatattggtaaaatataaatattctcggactcaggctttgttctaagtgaggacagtaattgatcacatggtacaattattgacagtaaaaccaagaaattgtcagctggtgtcctggcatggactagtgctgaggtgggagacaggaagttcacatttggtttctgggccaaagtggggcaggaggggtggtggggagaaaaggacagttgttttctttacagctctgataaaaataatctgtgctgccactgaattttaactttgaatatattcttctacatttgctgattaattccataatcattttactgaaaactcagatgtcaactaacaaaatatggcacatgatccattttgaacaatgtcaataggttcagaaactaccattgggctggcaaaaaaaacaagagaaacgcacatggcgagagcgatgattcggggttggtttggttggttcactgtggcccactgaacactcgtccctggcctcagtgtggcagattcatccccttggggcgatggcacaagccctggtgcccggcagggcctctgaggcctgagcggcaggtgaggctggcaggcgcctgctcagagcacgcgggggatgatggtgaagggcacggcggggctgctggcctccagctccaaggctgtcaggaagcactccgtagccgccgcatcgttgccctgagcttggaggacctcgcccagcccgttccagacctcgtgggctgtcgagttcacctgcaccgcgtcccggaggatcttctccgccagactgtagcggcctagctggtgaaggatcagggccagtcgctgcatgctcttcacgtgggtggggctgatggctaaggcctcttcataccaccgccgcgcctcgtccatgcttccccggagctcagcaatctggccgcgcatgtagaggacattgtgggacattgggaagaggttggcagcttcttgggtacaggctgtggcttctgcaggcttcccgatgccgatatagacttcagctgcatggagccagatctgtgccagcgtcatccaggggtgcagcgggccctgcttaggggcactgctctgcagagacgaagccacttccgacagtgcctgctccactcttgaggctgctaccgatgtggcatggacggagctaactgaaaaaagggaaggaaaaccatgaaagtatgcttctggagagttgcctgtctcgggatcgctgaagtctggcaaagtaattgtattaagctgtcgtctgtcagcaatggttctatctaagaggctgctcccacgtccagaatcactggggttggtgaggttgtagcaggatttccatatctgcagcatgtgcttacaagtcagcagtgcctcgtccgggcctcggcagagtgactgcaacttcactttggaaaacagtagtatgaaattttctgggtattcactcagggccatgtcgatgatgttcagagcgtcatggtaatgcttctgtgctgacagcaggagggcaaggaggtgcagggagttggcatcgtcaccttgaagctgaagagcttggcggacataccccagagcctctgggatctgtctggagatggcaagctgcagagccaggtagaaagctgcttggtgatctgtgggtgacaggctgtgggccctctgaaatgcaagaagcgcctttctctgtaggacctcctgcatccctcgcaaagaagcgtcagtggcctgcagactgtacgtgagccccagagctaagtagcctttggccttgaactctgacgttttctctcccacatcaacgacagttttggcaaacttttcagcctcttccaaccagtgcagggagcccatgcagagcttggcagcgaggagagggatggtggcatcgtctggcttcaggcggatacactctttcagcaccttcacggcacgggcagattttccagcagccatcagggacagagcaaactggtaccacaggtggaattcctcaaaggcaaacttcatggctctttctaggcactctgacagcatctcatactggcctcttcttccaagagcaatggtgagtaagtcatagaccacagatgcactctgcagactgatgaggcggtcactcttgtgttcaggtatcctgctcagcacagcgtcccggttggccattgattcactaatcagcaataacaacagggcttcttccgtattttcttgaggacaaaaaatgttctctcctgagtagacacgggctctccgagtgagagtgtaggtttttgtgtttgctcctttgcggagaggatcgtccagaggtgactggcacggtggatcctccagagggttccagtagctctgctcacacataccccgcaacaagatctctgccagctgcctggctattgtcattcgcaggttttgagtcgttcttgtttcaactgctctgagaagctctctaaatcttccgactcctcttgtcaagttcccatttttgaaatagaggacatgggctctctgaagtcctgtttctaggaaaaaacctagttcttgatcgtggggagcagggccaggcttagggcttctgttttgaatattagaaagtattaccctttctatctcttggagatacaggagtgcgatgtcccctgctttctcataacaggtgatgacatcctgttcccggtccacatggagattactggtagaagaagaaataggcagcttctccaaacaaagtcctttggtagcgtaggcttctgcgatcacccgcagcctgtagggcgggacagctgtcagtggcagatcgtccaggcccacccgggcgtaaatgttcagagcttctttataatcaccttccacataattcaacttggccatgatcagattggattcttgtaggaattcttaaggttccctcggtccagggcggcggtcagatgcttgcggacctcagtcagctggggcttggggcctcggggactggccccctgcctcagggggtgttccttcaggtactgctccagcttcgactccccgaggagaagctctgccatgtcatcgttggcgatgagcttggccgacagctgcttgacgagctcagggatccgctcccactggcactcggagcggcagcgctcgatctccgtctccagccgcgagcctgccttcttggtcgccatcgcggcctggccgggcccggccgcccgccccgcaggccccaccgccgccgccgcggcgccccctcgccgcctcccgccgccgccgcgggctcgggctccggctcccggctccgcggcgtaacgggagcgccggct

SEQ ID NO: 11659 - RNA, 1195 nt, Homo sapiens
  source 1..1195: mol_type = other RNA
ctgaatagctgggactacaggtgtgagccaacacgcccggcagttctgtgattcttagcagacacgggggcagggctggtgcagactatctcctgccagccctgtgctgcattccctgcccttaccctgttgccaagtccatgtgccatcagggcctctttgatggcttccacgcgtccatccatcatgtccgacggggctaccacctgacatcctgccttggcatacgccaatgccacctcagccagccgctggcggctctcctcagcccggaatgctccgttttcactcaggagcccgcagtgaccatgggaggtgtagggacacaggcagacatcacaggccaccaggaggttggggaaggtcttcctcaacagatggattgcctcaatagctggggactcctcggagtcagctgcggaaccccgctcgtccttgggaactctgctggggacgccaaagatcaagacacagcgtaggccctcttccaccaagggcctcagcatctcttccagccgcttcacaccatacctggccactcctgggaggctggtgataggctgtatgtcatcaggaacatccgtgacaaagatggggtagatgaggttggaggcattgagggtggtggtggctgtctgccaggcccgaagtagtgggtggaagtagccgctgtgcagaacggactggggctgcatggcgtgggccagtgggcacaggggcatcagttggttggaaccgagggctcctggggcattggctgcaggctctgtctcatgccagtagacagagcttctgcagggcaaggtccagagttggttcatttttgcctcccctacagtgctctgtcacacactgaccttggcacacagtaaatatttaattacgtgaagtacaaaaatatgctccaaatgccaaattagtggacacaagacagaaggaagctggggcattaacatttgtttcttgagcacctactgtgtgccagaccatgcctggcattttcacaggtgatttctcatcaagtgggcactacagtcctggcaggcagggctgattgagtgcatggagcctgaccagaagtgagccatggctccaatgggagtgaggaggtcagaagaggcatattagaagaagacaggcgccaggcgtagtggctcacacctgtaaccccagcactttgggaggctgaggcggg

SEQ ID NO: 11660 - RNA, 2747 nt, Homo sapiens
  source 1..2747: mol_type = other RNA
ctgaatagctgggactacaggtgtgagccaccatgcccagccatccaaaacaaatgaaaagctactcaacctcatcagtatccagggaaatgccaattaaaaccagtgtgcatctacctgacattttagccacagtagaccccaccctgctgggggcaacagttatctagtaaaattaaaggtatctcctgacttagcaattcaactcaatgttctgcaaaggaacttgtgcacatgtgcagaagactgcacaaagaattatgtggaatgaccaaaatcagaaacaataaaaatgaccatcaacaaggctgtatcacttgaggtattattcatacaacagaacaccatatagcattaaaaatgaactccaggacccaacaaggatggattatacaatgctgagtgacaaaaacgacacaaaagcacatacacaggattccatttatctaacactcaaaagcaaacacaactatgtcgtataaggctgcatacaagaatggtaaaattcaaacgaaagcagggaaatgactgacagaagacgatgacctggaatgtgccccaatctcagctgcacatcaaatgtacctgggatgaggtgggtggagctttgaatctaccactatccaggccacacacctagaagctctggtttcattgtttcattgatttcattgttttgattgatgctgaccttaggcagcagagttttcaatgctctccaggtgtttctaaagtgcagacaagtttaggaccgtgcttgagggtgaagggcaggactgtgatggggaggggcaaatatggggcccttggggtgcaggcaatggttttccttgacctgaatgggggtctcacaggtgttgcatatacatatacgtacacatgtcagctcttccctttctccacagcatacacgtaggtgttccacggcccacaggtgacagcctttacttggagttgcttatctacaaagtattccacacggcgaggccgatccaagctggtggtgtcctcgtggcccagctgtccatatttaccccagccccaggtgtagagctcccctgttcctgaaagcaaaaggacaatcgatagttgtcactacggttctttggcaaggcatctgtccagcccagcttggcacagcccacagctagcatattacaatcctcatgagatctgcctggcatggaacaacatattctcttaacaactggctgatcacacgtggcatggcagaggatcccgagggaaaaagtggcggatcttcctgtgtgccatgctaccgagcgccgcagtcttccatgccagactggacagtccctgctgtcagaggcggcggcgggcagggaatgtgtctgtggccgtgcagggaggacagaaagcatcagcctcccaccagaaggaagaaacttctgggcctgacaggctggggaactactgtgaaacaacaagggggttggggcttatccactgagcaaggtagctgctctgtatgagccacagaagccttaagacagaagtttttccgtcgaccacacccccttccgtaggcaccagctcgagtggagcagagtgcctcccagccccactcacgtgtcaccacagctgtgtgccgggatccacagctggccttgactgcatctgagcccatggggagatccagtaatgccgggaagggctggacagctatgaagggggcaggggctccatcctcagccccacccgttctcttcacctgagaaccatcttcattcagttctgtggcttcccttgcgacagtctctccatcctctgccaggttcctggtgggcagggccagctgccctgattcattccagccccagatataaatatccccagtctcactcacacacacagaatgccagccccccgcggccacctcagccatgactaggccctgcaacgcctccaacagccgtggctccagctctgcctccagggtcccatggcccagctgtccatgcctgcccccgccccaggagaacacctggccagcagcgtccagcagcaacgcgtgctcggcgcccagctccagctggcgtgcccgcagctccggagccagaggccggtagaagggcgcccgcgggctcacgtaggcacgggcgcagggcagcaggggtagcctcccagcctgggcctcaccggccggatcgtcttccccttcggcctcgggcaccacattctgggcccacaatggctccccacgcagcgccgattcggccgcccagacctgcagtaacgcctccggccccggcccggcgcgcagcaccgcgaggagcccctccgaggcccacgcgtccttgcagcggcccgccgcgccgctggctgagcccgacagctccaagcggcctccacgggtcacgaaagcggtgtagctccagctcgcgctcacgcggcagatgtcgacgcccgcccgcagcggactggggctgtgcacctggcgcccgcgtccggagcccagctcctgcccgaagccgcagaaaccgaagccgaaccaggcccccggccgctcctccgccatgcccgagcagcgccctctgccggccgccgcctggctgcggcgggcccggggggattcttgcgaagagcccgctagtgggacactggcaagtctctggccttccaggggctggagctgccttatctcagtcccgggaccgcggcagctcaaaacccgacacgcgccggactcatgccccaacaggaagcagcttttaccttccacggat

SEQ ID NO: 11661 - RNA, 2823 nt, Homo sapiens
  source 1..2823: mol_type = other RNA
ctgaatagctgggactacaggtgtgagccaccatgcccagccatccaaaacaaatgaaaagctactcaacctcatcagtatccagggaaatgccaattaaaaccagtgtgcatctacctgacattttagccacagtagaccccaccctgctgggggcaacagttatctagtaaaattaaaggtatctcctgacttagcaattcaactcaatgttctgcaaaggaacttgtgcacatgtgcagaagactgcacaaagaattatgtggaatgaccaaaatcagaaacaataaaaatgaccatcaacaaggctgtatcacttgaggtattattcatacaacagaacaccatatagcattaaaaatgaactccaggacccaacaaggatggattatacaatgctgagtgacaaaaacgacacaaaagcacatacacaggattccatttatctaacactcaaaagcaaacacaactatgtcgtataaggctgcatacaagaatggtaaaattcaaacgaaagcagggaaatgactgacagaagacgatgacctggaatgtgccccaatctcagctgcacatcaaatgtacctgggatgaggtgggtggagctttgaatctaccactatccaggccacacacctagaagctctggtttcattgtttcattgatttcattgttttgattgatgctgaccttaggcagcagagttttcaatgctctccaggtgtttctaaagtgcagacaagtttaggaccgtgcttgagggtgaagggcaggactgtgatggggaggggcaaatatggggcccttggggtgcaggcaatggttttccttgacctgaatgggggtctcacaggtgttgcatatacatatacgtacacatgtcagctcttccctttctccacagcatacacgtaggtgttccacggcccacaggtgacagcctttacttggagttgcttatctacaaagtattccacacggcgaggccgatccaagctggtggtgtcctcgtggcccagctgtccatatttaccccagccccaggtgtagagctcccctgttcctgaaagcaaaaggacaatcgatagttgtcactacggttctttggcaaggcatctgtccagcccagcttggcacagcccacagctagcatattacaatcctcatgagatctgcctggcatggaacaacatattctcttaacaactggctgatcacacgtggcatggcagaggatcccgagggaaaaagtggcggatcttcctgtgtgccatgctaccgagcgccgcagtcttccatgccagactggacagtccctgctgtcagaggcggcggcgggcagggaatgtgtctgtggccgtgcagggaggacagaaagcatcagcctcccaccagaaggaagaaacttctgggcctgacaggctggggaactactgtgaaacaacaagggggttggggcttatccactgagcaaggtagctgctctgtatgagccacagaagccttaagacagaagtttttccgtcgaccacacccccttccgtaggcaccagctcgagtggagcagagtgcctcccagccccactcacgtgtcaccacagctgtgtgccgggatccacagctggccttgactgcatctgagcccatggggagatccagtaatgccgggaagggctggacagctatgaagggggcaggggctccatcctcagccccacccgttctcttcacctgagaaccatcttcattcagttctgtggcttcccttgcgacagtctctccatcctctgccaggttcctggtgggcagggccagctgccctgattcattccagccccagatataaatatccccagtctcactcacacacacagaatgccagccccccgcggccacctcagccatgactaggccctgcaacgcctccaacagccgtggctccagctctgcctccagggtcccatggcccagctgtccatgcctgcccccgccccaggagaacacctggccagcagcgtccagcagcaacgcgtgctcggcgcccagctccagctggcgtgcccgcagctccggagccagaggccggtagaagggcgcccgcgggctcacgtaggcacgggcgcagggcagcaggggtagcctcccagcctgggcctcaccggccggatcgtcttccccttcggcctcgggcaccacattctgggcccacaatggctccccacgcagcgccgattcggccgcccagacctgcagtaacgcctccggccccggcccggcgcgcagcaccgcgaggagcccctccgaggcccacgcgtccttgcagcggcccgccgcgccgctggctgagcccgacagctccaagcggcctccacgggtcacgaaagcggtgtagctccagctcgcgctcacgcggcagatgtcgacgcccgcccgcagcggactggggctgtgcacctggcgcccgcgtccggagcccagctcctgcccgaagccgcagaaaccgaagccgaaccaggcccccggccgctcctccgccatgcccgagcagcgccctctgccggccgccgcctggctgcggcgggcccggggggattcttgcgaagagcccgctagtgggacactggcaagtctctggccttccaggggctggagctgccttatcttatctagccatttattcgtccagcgagcatttactgagcgctcctcctctgccagtgaggacagctgtctgctcccaaggagctcagtcccgggaccgcggcagctcaaaacccgacacgcgccggactcatgccccaacaggaagcagcttttacctt

SEQ ID NO: 11662 - RNA, 2846 nt, Homo sapiens
  source 1..2846: mol_type = other RNA
ctgaatagctgggactacaggtgtgagccaccatgcccagccatccaaaacaaatgaaaagctactcaacctcatcagtatccagggaaatgccaattaaaaccagtgtgcatctacctgacattttagccacagtagaccccaccctgctgggggcaacagttatctagtaaaattaaaggtatctcctgacttagcaattcaactcaatgttctgcaaaggaacttgtgcacatgtgcagaagactgcacaaagaattatgtggaatgaccaaaatcagaaacaataaaaatgaccatcaacaaggctgtatcacttgaggtattattcatacaacagaacaccatatagcattaaaaatgaactccaggacccaacaaggatggattatacaatgctgagtgacaaaaacgacacaaaagcacatacacaggattccatttatctaacactcaaaagcaaacacaactatgtcgtataaggctgcatacaagaatggtaaaattcaaacgaaagcagggaaatgactgacagaagacgatgacctggaatgtgccccaatctcagctgcacatcaaatgtacctgggatgaggtgggtggagctttgaatctaccactatccaggccacacacctagaagctctggtttcattgtttcattgatttcattgttttgattgatgctgaccttaggcagcagagttttcaatgctctccaggtgtttctaaagtgcagacaagtttaggaccgtgcttgagggtgaagggcaggactgtgatggggaggggcaaatatggggcccttggggtgcaggcaatggttttccttgacctgaatgggggtctcacaggtgttgcatatacatatacgtacacatgtcagctcttccctttctccacagcatacacgtaggtgttccacggcccacaggtgacagcctttacttggagttgcttatctacaaagtattccacacggcgaggccgatccaagctggtggtgtcctcgtggcccagctgtccatatttaccccagccccaggtgtagagctcccctgttcctgaaagcaaaaggacaatcgatagttgtcactacggttctttggcaaggcatctgtccagcccagcttggcacagcccacagctagcatattacaatcctcatgagatctgcctggcatggaacaacatattctcttaacaactggctgatcacacgtggcatggcagaggatcccgagggaaaaagtggcggatcttcctgtgtgccatgctaccgagcgccgcagtcttccatgccagactggacagtccctgctgtcagaggcggcggcgggcagggaatgtgtctgtggccgtgcagggaggacagaaagcatcagcctcccaccagaaggaagaaacttctgggcctgacaggctggggaactactgtgaaacaacaagggggttggggcttatccactgagcaaggtagctgctctgtatgagccacagaagccttaagacagaagtttttccgtcgaccacacccccttccgtaggcaccagctcgagtggagcagagtgcctcccagccccactcacgtgtcaccacagctgtgtgccgggatccacagctggccttgactgcatctgagcccatggggagatccagtaatgccgggaagggctggacagctatgaagggggcaggggctccatcctcagccccacccgttctcttcacctgagaaccatcttcattcagttctgtggcttcccttgcgacagtctctccatcctctgccaggttcctggtgggcagggccagctgccctgattcattccagccccagatataaatatccccagtctcactcacacacacagaatgccagccccccgcggccacctcagccatgactaggccctgcaacgcctccaacagccgtggctccagctctgcctccagggtcccatggcccagctgtccatgcctgcccccgccccaggagaacacctggccagcagcgtccagcagcaacgcgtgctcggcgcccagctccagctggcgtgcccgcagctccggagccagaggccggtagaagggcgcccgcgggctcacgtaggcacgggcgcagggcagcaggggtagcctcccagcctgggcctcaccggccggatcgtcttccccttcggcctcgggcaccacattctgggcccacaatggctccccacgcagcgccgattcggccgcccagacctgcagtaacgcctccggccccggcccggcgcgcagcaccgcgaggagcccctccgaggcccacgcgtccttgcagcggcccgccgcgccgctggctgagcccgacagctccaagcggcctccacgggtcacgaaagcggtgtagctccagctcgcgctcacgcggcagatgtcgacgcccgcccgcagcggactggggctgtgcacctggcgcccgcgtccggagcccagctcctgcccgaagccgcagaaaccgaagccgaaccaggcccccggccgctcctccgccatgcccgagcagcgccctctgccggccgccgcctggctgcggcgggcccggggggattcttgcgaagagcccgctagtgggacactggcaagtctctggccttccaggggctggagctgccttatcttatctagccatttattcgtccagcgagcatttactgagcgctcctcctctgccagtgaggacagctgtctgctcccaaggagcttgatcttgaccctatgccctctaccctctcgggcaggtccttctggtgggcagccttggaggaaacgccgaggcgcagagcggccgcctccggaaagg

SEQ ID NO: 11663 - RNA, 2762 nt, Homo sapiens
  source 1..2762: mol_type = other RNA
ctgaatagctgggactacaggtgtgagccaccatgcccagccatccaaaacaaatgaaaagctactcaacctcatcagtatccagggaaatgccaattaaaaccagtgtgcatctacctgacattttagccacagtagaccccaccctgctgggggcaacagttatctagtaaaattaaaggtatctcctgacttagcaattcaactcaatgttctgcaaaggaacttgtgcacatgtgcagaagactgcacaaagaattatgtggaatgaccaaaatcagaaacaataaaaatgaccatcaacaaggctgtatcacttgaggtattattcatacaacagaacaccatatagcattaaaaatgaactccaggacccaacaaggatggattatacaatgctgagtgacaaaaacgacacaaaagcacatacacaggattccatttatctaacactcaaaagcaaacacaactatgtcgtataaggctgcatacaagaatggtaaaattcaaacgaaagcagggaaatgactgacagaagacgatgacctggaatgtgccccaatctcagctgcacatcaaatgtacctgggatgaggtgggtggagctttgaatctaccactatccaggccacacacctagaagctctggtttcattgtttcattgatttcattgttttgattgatgctgaccttaggcagcagagttttcaatgctctccaggtgtttctaaagtgcagacaagtttaggaccgtgcttgagggtgaagggcaggactgtgatggggaggggcaaatatggggcccttggggtgcaggcaatggttttccttgacctgaatgggggtctcacaggtgttgcatatacatatacgtacacatgtcagctcttccctttctccacagcatacacgtaggtgttccacggcccacaggtgacagcctttacttggagttgcttatctacaaagtattccacacggcgaggccgatccaagctggtggtgtcctcgtggcccagctgtccatatttaccccagccccaggtgtagagctcccctgttcctgaaagcaaaaggacaatcgatagttgtcactacggttctttggcaaggcatctgtccagcccagcttggcacagcccacagctagcatattacaatcctcatgagatctgcctggcatggaacaacatattctcttaacaactggctgatcacacgtggcatggcagaggatcccgagggaaaaagtggcggatcttcctgtgtgccatgctaccgagcgccgcagtcttccatgccagactggacagtccctgctgtcagaggcggcggcgggcagggaatgtgtctgtggccgtgcagggaggacagaaagcatcagcctcccaccagaaggaagaaacttctgggcctgacaggctggggaactactgtgaaacaacaagggggttggggcttatccactgagcaaggtagctgctctgtatgagccacagaagccttaagacagaagtttttccgtcgaccacacccccttccgtaggcaccagctcgagtggagcagagtgcctcccagccccactcacgtgtcaccacagctgtgtgccgggatccacagctggccttgactgcatctgagcccatggggagatccagtaatgccgggaagggctggacagctatgaagggggcaggggctccatcctcagccccacccgttctcttcacctgagaaccatcttcattcagttctgtggcttcccttgcgacagtctctccatcctctgccaggttcctggtgggcagggccagctgccctgattcattccagccccagatataaatatccccagtctcactcacacacacagaatgccagccccccgcggccacctcagccatgactaggccctgcaacgcctccaacagccgtggctccagctctgcctccagggtcccatggcccagctgtccatgcctgcccccgccccaggagaacacctggccagcagcgtccagcagcaacgcgtgctcggcgcccagctccagctggcgtgcccgcagctccggagccagaggccggtagaagggcgcccgcgggctcacgtaggcacgggcgcagggcagcaggggtagcctcccagcctgggcctcaccggccggatcgtcttccccttcggcctcgggcaccacattctgggcccacaatggctccccacgcagcgccgattcggccgcccagacctgcagtaacgcctccggccccggcccggcgcgcagcaccgcgaggagcccctccgaggcccacgcgtccttgcagcggcccgccgcgccgctggctgagcccgacagctccaagcggcctccacgggtcacgaaagcggtgtagctccagctcgcgctcacgcggcagatgtcgacgcccgcccgcagcggactggggctgtgcacctggcgcccgcgtccggagcccagctcctgcccgaagccgcagaaaccgaagccgaaccaggcccccggccgctcctccgccatgcccgagcagcgccctctgccggccgccgcctggctgcggcgggcccggggggattcttgcgaagagcccgctagtgggacactggcaagtctctggccttccaggggctggagctgccttatcttgatcttgaccctatgccctctaccctctcgggcaggtccttctggtgggcagccttggaggaaacgccgaggcgcagagcggccgcctccggaaagg

SEQ ID NO: 11664 - RNA, 2201 nt, Homo sapiens
  source 1..2201: mol_type = other RNA
ctgaatagctgggactacaggtgtgagccaccatgcccagccatccaaaacaaatgaaaagctactcaacctcatcagtatccagggaaatgccaattaaaaccagtgtgcatctacctgacattttagccacagtagaccccaccctgctgggggcaacagttatctagtaaaattaaaggtatctcctgacttagcaattcaactcaatgttctgcaaaggaacttgtgcacatgtgcagaagactgcacaaagaattatgtggaatgaccaaaatcagaaacaataaaaatgaccatcaacaaggctgtatcacttgaggtattattcatacaacagaacaccatatagcattaaaaatgaactccaggacccaacaaggatggattatacaatgctgagtgacaaaaacgacacaaaagcacatacacaggattccatttatctaacactcaaaagcaaacacaactatgtcgtataaggctgcatacaagaatggtaaaattcaaacgaaagcagggaaatgactgacagaagacgatgacctggaatgtgccccaatctcagctgcacatcaaatgtacctgggatgaggtgggtggagctttgaatctaccactatccaggccacacacctagaagctctggtttcattgtttcattgatttcattgttttgattgatgctgaccttaggcagcagagttttcaatgctctccaggtgtttctaaagtgcagacaagtttaggaccgtgcttgagggtgaagggcaggactgtgatggggaggggcaaatatggggcccttggggtgcaggcaatggttttccttgacctgaatgggggtctcacaggtgttgcatatacatatacgtacacatgtcagctcttccctttctccacagcatacacgtaggtgttccacggcccacaggtgacagcctttacttggagttgcttatctacaaagtattccacacggcgaggccgatccaagctggtggtgtcctcgtggcccagctgtccatatttaccccagccccaggtgtagagctcccctgttcgtgtcaccacagctgtgtgccgggatccacagctggccttgactgcatctgagcccatggggagatccagtaatgccgggaagggctggacagctatgaagggggcaggggctccatcctcagccccacccgttctcttcacctgagaaccatcttcattcagttctgtggcttcccttgcgacagtctctccatcctctgccaggttcctggtgggcagggccagctgccctgattcattccagccccagatataaatatccccagtctcactcacacacacagaatgccagccccccgcggccacctcagccatgactaggccctgcaacgcctccaacagccgtggctccagctctgcctccagggtcccatggcccagctgtccatgcctgcccccgccccaggagaacacctggccagcagcgtccagcagcaacgcgtgctcggcgcccagctccagctggcgtgcccgcagctccggagccagaggccggtagaagggcgcccgcgggctcacgtaggcacgggcgcagggcagcaggggtagcctcccagcctgggcctcaccggccggatcgtcttccccttcggcctcgggcaccacattctgggcccacaatggctccccacgcagcgccgattcggccgcccagacctgcagtaacgcctccggccccggcccggcgcgcagcaccgcgaggagcccctccgaggcccacgcgtccttgcagcggcccgccgcgccgctggctgagcccgacagctccaagcggcctccacgggtcacgaaagcggtgtagctccagctcgcgctcacgcggcagatgtcgacgcccgcccgcagcggactggggctgtgcacctggcgcccgcgtccggagcccagctcctgcccgaagccgcagaaaccgaagccgaaccaggcccccggccgctcctccgccatgcccgagcagcgccctctgccggccgccgcctggctgcggcgggcccggggggattcttgcgaagagcccgctagtgggacactggcaagtctctggccttccaggggctggagctgccttatctcagtcccgggaccgcggcagctcaaaacccgacacgcgccggactcatgccccaacaggaagc

SEQ ID NO: 11665 - RNA, 2285 nt, Homo sapiens
  source 1..2285: mol_type = other RNA
ctgaatagctgggactacaggtgtgagccaccatgcccagccatccaaaacaaatgaaaagctactcaacctcatcagtatccagggaaatgccaattaaaaccagtgtgcatctacctgacattttagccacagtagaccccaccctgctgggggcaacagttatctagtaaaattaaaggtatctcctgacttagcaattcaactcaatgttctgcaaaggaacttgtgcacatgtgcagaagactgcacaaagaattatgtggaatgaccaaaatcagaaacaataaaaatgaccatcaacaaggctgtatcacttgaggtattattcatacaacagaacaccatatagcattaaaaatgaactccaggacccaacaaggatggattatacaatgctgagtgacaaaaacgacacaaaagcacatacacaggattccatttatctaacactcaaaagcaaacacaactatgtcgtataaggctgcatacaagaatggtaaaattcaaacgaaagcagggaaatgactgacagaagacgatgacctggaatgtgccccaatctcagctgcacatcaaatgtacctgggatgaggtgggtggagctttgaatctaccactatccaggccacacacctagaagctctggtttcattgtttcattgatttcattgttttgattgatgctgaccttaggcagcagagttttcaatgctctccaggtgtttctaaagtgcagacaagtttaggaccgtgcttgagggtgaagggcaggactgtgatggggaggggcaaatatggggcccttggggtgcaggcaatggttttccttgacctgaatgggggtctcacaggtgttgcatatacatatacgtacacatgtcagctcttccctttctccacagcatacacgtaggtgttccacggcccacaggtgacagcctttacttggagttgcttatctacaaagtattccacacggcgaggccgatccaagctggtggtgtcctcgtggcccagctgtccatatttaccccagccccaggtgtagagctcccctgttcgtgtcaccacagctgtgtgccgggatccacagctggccttgactgcatctgagcccatggggagatccagtaatgccgggaagggctggacagctatgaagggggcaggggctccatcctcagccccacccgttctcttcacctgagaaccatcttcattcagttctgtggcttcccttgcgacagtctctccatcctctgccaggttcctggtgggcagggccagctgccctgattcattccagccccagatataaatatccccagtctcactcacacacacagaatgccagccccccgcggccacctcagccatgactaggccctgcaacgcctccaacagccgtggctccagctctgcctccagggtcccatggcccagctgtccatgcctgcccccgccccaggagaacacctggccagcagcgtccagcagcaacgcgtgctcggcgcccagctccagctggcgtgcccgcagctccggagccagaggccggtagaagggcgcccgcgggctcacgtaggcacgggcgcagggcagcaggggtagcctcccagcctgggcctcaccggccggatcgtcttccccttcggcctcgggcaccacattctgggcccacaatggctccccacgcagcgccgattcggccgcccagacctgcagtaacgcctccggccccggcccggcgcgcagcaccgcgaggagcccctccgaggcccacgcgtccttgcagcggcccgccgcgccgctggctgagcccgacagctccaagcggcctccacgggtcacgaaagcggtgtagctccagctcgcgctcacgcggcagatgtcgacgcccgcccgcagcggactggggctgtgcacctggcgcccgcgtccggagcccagctcctgcccgaagccgcagaaaccgaagccgaaccaggcccccggccgctcctccgccatgcccgagcagcgccctctgccggccgccgcctggctgcggcgggcccggggggattcttgcgaagagcccgctagtgggacactggcaagtctctggccttccaggggctggagctgccttatcttatctagccatttattcgtccagcgagcatttactgagcgctcctcctctgccagtgaggacagctgtctgctcccaaggagctcagtcccgggaccgcggcagctcaaaacccgacacgcgccggactcatgccccaacaggaagc

SEQ ID NO: 11666 - RNA, 2662 nt, Homo sapiens
  source 1..2662: mol_type = other RNA
ctgaatagctgggactacaggtgtgagccaccgtgctggctccattccattttgtccactcgtatctgcagcctgctggaaatgtgtagccagtgatgtctcgtcctggaagacttcattacactccaaacattttagactatgtctacacagtttggaggggtcttcatctaggggcatggctggggtgatgggagtgcttgaaggagccgatatgactgtcccagttatgccagactgaatttttgtgacagtgtgtgtgccagctcccacagggctctgaagagtggaagttgaagtggaagtattgcttgacggagaaactatcatttgatctgctgggactggctttaaaattaagtgggagcattgcattaccacccctttctccttatgcccacgggcatgggaaaggaggctgcatttgttgtaaaaaacgaggttctttgtacaatggttgcacgttacttcgatgcgcacgctccgtctgtcgtagtgctgggtcagactcttttcaagtgcaaaggagtccccacactccaagcacttgtacccacgcgtcggtaacgtgatccctgcattggcgggaggactgaggtttgggatgtaaacagggactggattgacactgctcagcaccttgttgaaagcttccaccacagaactctgcaaggacgacaccacctggactcgagacacctttttggggggttgcgaggctgctgcattgattattgcctgctttatttgttgctgaggtttggttagcacttggcggagttcagaggtggcctgggcaccctgaggcaaaaggttaaggttggcaaggtgcacagtctttggcacgagtttggcattggccaggctggatgccggcaccacgacagtttgctgctggatggcgttggcagctttaatgatggcgctgctggcactctggacagaggcagcagatatgaccgtggctttcaccgtggtgttgttagcgagcttcaaattaatgacttgggatcctgccgtcttcacagcagacactgggaggaaagcagtagccacaggcttgattgtgacctgtttgggggtgagctctgcaggggaaactgcattggtcacgaccgcagactggagaggcgccctggggggagaggaaaggacggcggctgatgctggagacgacagaagggatgtcacagaggccatcacggacgctgtctgctcggaaggtttctttccagagtcaagatccacttctggcaataccctggtcactgttctcttgatttccccagaagatgtcttaatggtttttatgcggactttggggattgctggtgtggaccctgcgggagaggacggggatcctttgctgctgttctcacttgagatgcttctgggactatccggttgcttcagggatggttttttggtcccgtcgatgagattctgggattcaggagacttgtcagcggctctcggactgtcatttacttcttttggtaacggggaggattccctcgaattggccactggttctttgcaggagtctgaagccgcctttttagcgctgagagccgcgatggcagcgatgcaggacgagagcttggaggacgactttgtctttgatggcgcaacgctggggaggctggtgtcattcttctcggagctcagcttcccatctaggactctgttttccagcaccttgtcagagctttccttcaatttatcctctgcttttctgactttaaaaggttcataaacactcaggtttatagaactggcttctgtttctctcttaacagctttgtttttctccacattgcctgacgtagagagtccagttttgctggagttttcccctccgagtgccttcagcttatcgtagtcctgctggggagccgaccccgtcaacacattcgacctgaagcttgatcgcatgtcctccttgtcaggggggtcatccacctcaatcttctcgtcgtcatcaaactcttcagcactggagatcg[450 bp omitted]cggtatttgctgtgtcattatccttccttcgaatctgctttagtggtccctgacacgttgcctccttccacatcttactgaagcacttgattttttttttcttgtacaatctagaaaacatcacacattcctaataaaagtaactattccagggtcaagagagaatttctactcagtgagaatacacatgcctgagaaaactcata

SEQ ID NO: 11667 - RNA, 489 nt, Homo sapiens
  source 1..489: mol_type = other RNA
ctgaatagctgggactacaggtgtgagccacctcacaaggcttcacacaaaatagatgccatctatctgattgggactatccttaccttgcttgcttacctgcaactgttgtagcactgtccggttgagctttctatactgctgggtaagtaccgtatatctttgctgttcaatatggtagccattagctacagggggctatcaaaatatggcttgtacagctgtaggtatgctagtttacaaggactccagatggcctgggagcttcagaaccttttgccaattatcagaggaaggtaaagcctctgtgcatctttgcccggctgtttcatacttttgcttctgcagattactgttctcagcttctccatgcatacgatggttatgtcaaatcagttccagtcacctcggcctccgcaagtgctgggatgacaggtgtgagccaccgcccccggcccctcgcccgccttttgaaggagcctttcgtcc

SEQ ID NO: 11668 - RNA, 205 nt, Homo sapiens
  source 1..205: mol_type = other RNA
ctgaatagctgggactacaggtgtgagccacggctcctggccaagaaatttctgataacttgttcaccaccaagaatcaagggtactcagcccaacagtatacaaagaaagtatcacttaatagatttcttctctaacttctctataacttattattagctttgctttagttcaaaaaagaaatacctcactggctttattaatt

SEQ ID NO: 11669 - RNA, 4320 nt, Homo sapiens
  source 1..4320: mol_type = other RNA
ctgaatagctgggactacaggtgtgagccactgtgcccagcccgtacactttttaaaaaacttaattcttcaaattcacgaataataattctacatattcgtggggtagaatactttgatacaaagaatgtacagttatcagctcagggtaacaagcatatccatcatctcaaacacctataatttctttgtgttgggaacattcaatattcttctattttaaagtatatattaactatagtcatgctatagtggtacacaacactagggcttattcctatgttattttgcatcctcccacaaatctctccctatcccttccttccccctatcttctcagcctctagtatgcgctgtcctaatttttacttctataagattaactttttaaaacttccacatgagtgagaacatgcattgtttaattttccattgctggcttatttcacctactataaagtcctccagttccttccatgttgctgcaaatgaaaggacattctttttttatggctgaatagtatcccattgtgtataataccacatcttgtttagccattcacctgttgatgcacctgttgattctgggttgattccatgtcttggctaatgaatagtgctacaataaacatgggggtgccaatgtctgacttttaatcatatgtaaatgagataaaatctcttccctgaacttccaacttactcattgtggttttgatgtgcattaccctgatgcttagtgtttagaattttttcatacatttattggccatttgtacgtcttcttttgagaaatgtctgttcagatgatttgcccatttttaatctagatttgttttgctattaagatgtttgaatatcttctatattctgaatattaatcctctgttgcatgagtagtttacaaatattttctcccattctgtaagctgtcttttcactgttgatggtttcctctgctgcacagaagctttttaatttgatatgatcccatgtttttgttgcctgtgcttttaggtctcagtcataaaatcttttcccagaccaatgtcctgaagtgcttcttgttttctcttatggtagttttattgttttaggtcttacatttaggtctttcatccattttgagttggtttttgtacagggtgggaggtgcggatctagtttcattcttctgcatatggatacccagttttctcagcaccatttattgaagagactgtcccttttttttttgtccctccaatgagtattcttgccacctttgtaaaaaatcagttggctgtagatacgtggattaatttctggttctctgttctgttccattgctctgtatctatttttatgccagtatcaggctgttttggttactacatttttgatttatattttgagatctggtagtgtgataactccagctttgttctttttgctcagtattgctttggctatttggggtcttgtggttccatataaattttaagaattttttttggtggcaatttctgtgaagaatgtcagttattttgatagaagttgtattgaatctggagatcactttgggtagcatggtcatttaaaatatattaattcctctaatccatgagtacggagtgtctttcaatttgtttgtatctccttcaatttctttcatcagtgttttgtagttttccttgtatagaaatattttaccttcttggttaatttattcctagatttttttcacagctattataaatggggttaccttgatttctttttcagctagttcactgttcatgcatagaaatgctactgatttttgtatactaattttgtatcttctaacttttctaaatttatcagttctatgagttttttggtagagtctttagttttgtttttatatatataacatcatgtcatctgcatagagaacaatttgacttctccattctagtttggatgccctttatttctttctcttatctacctgctctggctatgactttcatgacaacttcttagttctttatttattgtctatcattactaaaggtaactcatataactatgaaaaatatcttaaattatcaataatcaatttcgaaaatcaggttagactacaaaatgtccctttgaatgcaataaatatgcaatttttgttttgatcacagtatttcacgcaactggactcacacaaatgtagatctaaaggctgagtttttttcactgctttatcagctacataagcttctcagaatactgccaaataggtgctatgtgtgtatgtgcgtctgagtgtgtttcagctactgatataaactaagcatatcttttgctgaaaaatcaagtcacttgtgatgtacagaacaagagtctctcatccattggtcagtcacttttatagccacagagaaatggtcctcaaaggtgtcgtcccatgaagaaaactgatcgaagttatcacaaggctggacttttaatcatatgtaaatgagatcaaatctcttcattaacttctaaacttcctcattatagcaatcttgttagcaacaatagagagagcttggttttgctgtttttgatccacaatcttggaggcttgaaaaataccttttcagtcaattttgcaatcaatttttttgccattatgtcttactagggtgatgtcttgatgtcttttttgacccccctttcataattaaagttgcccaaattgctgctatatttcccactgggagggttataaatctgcctggcatctctttttggtcctgctgaagatttcttgggtggtgaacctgaagttgtatcttcactggctctcttttgcccaatctcaaccttttgtacaggtttccaggatagtgttactgtgctcttataagaaggaggaatgtggaagagatccttgattaaaacattgatattgtttgttattttcaatgcaacgactttaatcttgttctcttctgtttttaaggcctcacccgttttaccctggagagctaagcgaagttgtctgatataaacttgcaggccccgtgcaaagtactgcagcctgattttgaaatctttgagcttttctgcattcagtttggctgttaagaaatctggaagttttcggcccaactggtgaaaactgtacaacaaacattccacataactgaactgtagcttgggttcttcattaccagcattctctccattttctgcctcttctggagggaggggcatgtattccaataacttatcaaatagtttccttaaatttgtttctagtttttccatgtcaccacaaaatgaactcatctccgccaacaatttcaatacctccaactgtatatcaagaccttccactggggtagtcaaggtaccgaggttagggagaacctgctcacagaaatatgtcacaaaccttgtggaatggacatttttagagaagaggggtactgcctgccgagtgcactgtaagagcctgtccacacagtcaggatccgagggattgaaggtctgttctaggtcggcctgttcagccaccaactctacaagttgctgtcttccactcactgtctgtaagctttttaacccagacagtatcttcataaatagaacaaattcttcaccagtcacatcttctaggacctttttggattcagttagtataagctcttccacttcctttgttaagacttcatctggtaaagtcttaagttttgtagaaaggaatttaattgctcgttctctaacaatgtcctctccttgaagtatttggctgaacaacccacctaaagtcccttttgcatccattttaaatatacttaatagggcattgttcactaggttaaattctgcagagtcatctgtctgcaaaagttgcgttagtatatctgccactcgaggaagattttctccagtggcaaattgaggcagttctttaattgcttgacgtcgaatagatacatcttcatcctcacagaggtctaactgtgcattgatagcagaatcagccaattctggaaaatgcttaaagaatttcggaataaattgagctgctaatcgcttttccttagtaccacctttcacaccatccaatatcacttgataggcatctttatgctggcccacttgctccgtggcatcggccaggatgccataattgcggtaaagctcctctactgtcggcatggtgagcgacaagcccagggcccggttccgctatccttgtcctgaccggcgccaccgccgcctcggaacttctccaaacccactacccgcactattacacctccagctgccgccagtgcagccgccagtcaccgcgcacagcgcggctgc

SEQ ID NO: 11670 - RNA, 4390 nt, Homo sapiens
  source 1..4390: mol_type = other RNA
ctgaatagctgggactacaggtgtgagccactgtgcccagcccgtacactttttaaaaaacttaattcttcaaattcacgaataataattctacatattcgtggggtagaatactttgatacaaagaatgtacagttatcagctcagggtaacaagcatatccatcatctcaaacacctataatttctttgtgttgggaacattcaatattcttctattttaaagtatatattaactatagtcatgctatagtggtacacaacactagggcttattcctatgttattttgcatcctcccacaaatctctccctatcccttccttccccctatcttctcagcctctagtatgcgctgtcctaatttttacttctataagattaactttttaaaacttccacatgagtgagaacatgcattgtttaattttccattgctggcttatttcacctactataaagtcctccagttccttccatgttgctgcaaatgaaaggacattctttttttatggctgaatagtatcccattgtgtataataccacatcttgtttagccattcacctgttgatgcacctgttgattctgggttgattccatgtcttggctaatgaatagtgctacaataaacatgggggtgccaatgtctgacttttaatcatatgtaaatgagataaaatctcttccctgaacttccaacttactcattgtggttttgatgtgcattaccctgatgcttagtgtttagaattttttcatacatttattggccatttgtacgtcttcttttgagaaatgtctgttcagatgatttgcccatttttaatctagatttgttttgctattaagatgtttgaatatcttctatattctgaatattaatcctctgttgcatgagtagtttacaaatattttctcccattctgtaagctgtcttttcactgttgatggtttcctctgctgcacagaagctttttaatttgatatgatcccatgtttttgttgcctgtgcttttaggtctcagtcataaaatcttttcccagaccaatgtcctgaagtgcttcttgttttctcttatggtagttttattgttttaggtcttacatttaggtctttcatccattttgagttggtttttgtacagggtgggaggtgcggatctagtttcattcttctgcatatggatacccagttttctcagcaccatttattgaagagactgtcccttttttttttgtccctccaatgagtattcttgccacctttgtaaaaaatcagttggctgtagatacgtggattaatttctggttctctgttctgttccattgctctgtatctatttttatgccagtatcaggctgttttggttactacatttttgatttatattttgagatctggtagtgtgataactccagctttgttctttttgctcagtattgctttggctatttggggtcttgtggttccatataaattttaagaattttttttggtggcaatttctgtgaagaatgtcagttattttgatagaagttgtattgaatctggagatcactttgggtagcatggtcatttaaaatatattaattcctctaatccatgagtacggagtgtctttcaatttgtttgtatctccttcaatttctttcatcagtgttttgtagttttccttgtatagaaatattttaccttcttggttaatttattcctagatttttttcacagctattataaatggggttaccttgatttctttttcagctagttcactgttcatgcatagaaatgctactgatttttgtatactaattttgtatcttctaacttttctaaatttatcagttctatgagttttttggtagagtctttagttttgtttttatatatataacatcatgtcatctgcatagagaacaatttgacttctccattctagtttggatgccctttatttctttctcttatctacctgctctggctatgactttcatgacaacttcttagttctttatttattgtctatcattactaaaggtaactcatataactatgaaaaatatcttaaattatcaataatcaatttcgaaaatcaggttagactacaaaatgtccctttgaatgcaataaatatgcaatttttgttttgatcacagtatttcacgcaactggactcacacaaatgtagatctaaaggctgagtttttttcactgctttatcagctacataagcttctcagaatactgccaaataggtgctatgtgtgtatgtgcgtctgagtgtgtttcagctactgatataaactaagcatatcttttgctgaaaaatcaagtcacttgtgatgtacagaacaagagtctctcatccattggtcagtcacttttatagccacagagaaatggtcctcaaaggtgtcgtcccatgaagaaaactgatcgaagttatcacaaggctggacttttaatcatatgtaaatgagatcaaatctcttcattaacttctaaacttcctcattatagcaatcttgttagcaacaatagagagagcttggttttgctgtttttgatccacaatcttggaggcttgaaaaataccttttcagtcaattttgcaatcaatttttttgccattatgtcttactagggtgatgtcttgatgtcttttttgacccccctttcataattaaagttgcccaaattgctgctatatttcccactgggagggttataaatctgcctggcatctctttttggtcctgctgaagatttcttgggtggtgaacctgaagttgtatcttcactggctctcttttgcccaatctcaaccttttgtacaggtttccaggatagtgttactgtgctcttataagaaggaggaatgtggaagagatccttgattaaaacattgatattgtttgttattttcaatgcaacgactttaatcttgttctcttctgtttttaaggcctcacccgttttaccctggagagctaagcgaagttgtctgatataaacttgcaggccccgtgcaaagtactgcagcctgattttgaaatctttgagcttttctgcattcagtttggctgttaagaaatctggaagttttcggcccaactggtgaaaactgtacaacaaacattccacataactgaactgtagcttgggttcttcattaccagcattctctccattttctgcctcttctggagggaggggcatgtattccaataacttatcaaatagtttccttaaatttgtttctagtttttccatgtcaccacaaaatgaactcatctccgccaacaatttcaatacctccaactgtatatcaagaccttccactggggtagtcaaggtaccgaggttagggagaacctgctcacagaaatatgtcacaaaccttgtggaatggacatttttagagaagaggggtactgcctgccgagtgcactgtaagagcctgtccacacagtcaggatccgagggattgaaggtctgttctaggtcggcctgttcagccaccaactctacaagttgctgtcttccactcactgtctgtaagctttttaacccagacagtatcttcataaatagaacaaattcttcaccagtcacatcttctaggacctttttggattcagttagtataagctcttccacttcctttgttaagacttcatctggtaaagtcttaagttttgtagaaaggaatttaattgctcgttctctaacaatgtcctctccttgaagtatttggctgaacaacccacctaaagtcccttttgcatccattttaaatatacttaatagggcattgttcactaggttaaattctgcagagtcatctgtctgcaaaagttgcgttagtatatctgccactcgaggaagattttctccagtggcaaattgaggcagttctttaattgcttgacgtcgaatagatacatcttcatcctcacagaggtctaactgtgcattgatagcagaatcagccaattctggaaaatgcttaaagaatttcggaataaattgagctgctaatcgcttttccttagtaccacctttcacaccatccaatatcacttgataggcatctttatgcttcccaattccgttctccctccatctttgtttcatttttgagttgggggagatggatgagtctggcccacttgctccgtggcatcggccaggatgccataattgcggtaaagctcctctactgtcggcatggtgagcgacaagcccagggcccggttccgctatccttgtcctgaccggcgccaccgccgcctcggaacttctccaaacccactacccgcactattacacctccagctgccgccagtgcagccgccagtcaccgcgcacagcgcggctgcgcccccga

SEQ ID NO: 11671 - RNA, 3270 nt, Homo sapiens
  source 1..3270: mol_type = other RNA
ctgaatagctgggactacaggtgtgagccactgtgcctggcctggacctttcatttaaaccagctcacttcctctggattgagaaatgtaggcccttctccatccccctcctggttagggaagctggcagaaacccgtgtcctaaactgtatcccatggaaaaagtctacgagggtggtcatggcccttccccaactccgaaaatcgggaggcaaggtcgaccactgtgagcgtggggttcagagctgtctgaaccaagatatttgggagggcagttagtgcagagatggctccagcttccctaaaggacaggtgaagccactgtcttcctccttcggtagctgacaagggcctgaaggaatcaaagttcatgcattccaagagaggagacagagcatgtatgtgagaggaaagaggggagagaaccttggtttggtatgtgtgaaactggggtacttgaggatcagccctagggtcgaggctccctggagtcctagccatcagtggggaggtctctgagcactctttccagaggctgacctccacggatgagtctgagatggggcgtggccagaatctggtccgattccagggggccgagatataggaaggtgtccagaggcaggcagtgtggtcctgctggcagaattggaggtcccagggccctgcgccttcttgtccatggcctggctttggctggcagagggaggagtggtctcttccttggtgagttggagctgggtggcatttttggagctgcttttaggtgtgtcctctgaatctctggctgtggctttgccttttacagatttgtgactcttctcaacttcacggagcacttggattttcttcctcagctgggcattagctcgggaaaggcttttggaaactgagttcaggtagtaaatggccaagaacatcagcaggatggctgggatgatcaggcctggattggcgaggaaagcaaagatcttgcccaggaaggttgggaaatcgttttcaatggtctcttggaggacatcgtacattctgtttttcccactgaacggcccgcagtcaaaggagggtgggagggacatgatggtgtaggccaccggcaggaggctgaggaagagcaccagcagcaggaggcccatgtagaagttgttggatcgggaggctttgaacacgcgttcatggggtacgttgctgctcatcaccgcccagcactggaagtacatggaggtcagcaggcgcagcacattaatgcccaccaggcctggagcatagaaggagcccatccagatcattccttggttgaagatcaaacccagcacatttccactaatatcaaactcagcatatgaaggaaatccagcctccaagtcccagcaccagcagtagttcatgaaccgcacaaaacaagcccgtaggaagtcccccagcaggatggtgatgtacgttaccagcatgtcagacaccgtcagcctcatgaattcaatgcccacagctgtctcccagcaagaaccccggggcacatctgcagggtgcaggggtggtcgggggacactctcgttccaaccagaagagttgtaatagttaaacagagtccagtgagtgatgttctttattgtctcttcattagcaagcttgaggtggacgtcatccatcagggccaagagaaatgtgtagaggttccccaggaagagtgcaaagatgcgtcccagctgccacttcagtccagtgcgtgggtggtaattctccagggcagcgatggtttcaaacagagggggacaaaacattccaagcagggacatcacgatctctacctcattcctttcataccagctgacattctgcattttggagaattgctgagatcgcttaaccacaaagtaaatgaggtacccacttccacacaaacagcagatgatgagaaagttggccaggacacgaagaaatcttgtcagatggatattttcttctttgttactctcttgttcatccactattgattccttgaagctggtggtgatggatgcatatttgttatcagctgtctctgaattcccgatcaggtagtcccagctggtgaacatcttgaagctgaatgtgaagttgtcactctccccttcgcctgtgcttccttgggtattgctggccatcgatcgaatgacaataatcaggctgtagccgaacacgctgacccccaccataaagtaagccataggcagccggtacctcagccacccgatggtcctctggttgttgtagtagccatagaagagtgcagagtacttgatatagccctcaaaatcccaaaggacagaaaaatccatggccttttcttcctcagcccgaggcactgtctttctgggaatactcccatagggcatgcccatcagtacctctgggattatgactagaccaaatattaagccaaaaaggacaaggttaactccatacatccatcggagaaagatgaaatacgatgccactgaagaaccaaagtgactttcaatgtccttgatcttcatttcccaggggatacattgagtcttgaaattatcaaagtctctcttaaatttgacccatttcttggccatcagcatcttgtaggcatatagttgcttgcctttcccctttcccaaggcaccttcatacttctccacaaattcctgggcctccctgagctctgtcagcttcttcgccatgggccagggcttgctccgcatggtggcaatgagcttctttttttcttccacctgctccaggatctgggccagttcctcctcggacagggactccccaccagaggcactggaggccaaggaggatgacctgggtttcttctgccgcttcgacttctcctccctcctcggaatctccttttccctctttggggctgctgtccgctcctggaaggaggccctctcgtcgcgctttctcctgccctcgcaggtcctctctgcctcgccccgctcctgctcccccagctcttctctgtgtctcctgcgccctgtttgcttcctccggggagaccccgggcttgggctgcccccggcgcgctccttctggcttcgctgagctccgcgcctgcctggggtcccctcggctttgagagcccgcttgcttgaggatctccttcccagcctgtcacctgtgtgtggagagccgctcttcacccgccctttcactccgcctcgtgcttcctctttcaggccctttacctggtggctcatggtcagcagcactgctggggtcctgcacaggctcacgcagcgtgctcct

SEQ ID NO: 11672 - RNA, 2229 nt, Homo sapiens
  source 1..2229: mol_type = other RNA
ctgaatagctgggactacaggtgtgagccactgtgcctggcctgtgtctattttttgaatgggcaatttgtaccttttgatccccagcccctgcttccctcactagatgcagctgctgccatcattttcttgtatccttccattgttgggcctttcatatacaaacacagcctgttctgcctcatgcatgttgagttttcaactttaaattttttttttttttttttgagatggagtctcactctgtcatccaggctggagtgcagtggtgcaatctcggcccattgcaacctccacctcctgggttcaagcgattctcgtgcctcagtctcctgagtagttgggattacaggtgtgtgccaccacacccagctaatttttgtatttttagtagagacagggcttcaccatgtcggccaggatggtctggatctcctgaccttgtgattcaccccccttggcctcccaaagtgctgggattacaggtgtgagccactatgcccggccgttgagttttcaactttaagtgggaacttcagacttcatactttctgtgtgcagaagacatatgcagtgattataaacaaactgtacatctgccaaaaaaaaaggccggggggagggaggaacaaaggaaaggaggaaggaactgttgcgcagttatttatttacattggaaacagccctcgcagtacgggtatatgaaggccagacctgatgaacagcaggtgaaactctgggaacccagggcttaggatacacagtgcttccttgtacatttgtttccttcagatggtcacatccaccactgaagctttttagaaggcactttccatgacagatgcaggtcaaggtcgcacattaaaatcggccctaatgctttttgctgagtgtgagtccctgactctcttgcgaagatcccaccagcccttttcgtcttagcagaatgaaggcagtgccctctgcggcccactaacttcacaagctgaactcagacgctaaggcaggacgacccacgggctccattcaagcctcgcctcatctttcactggttgctgctggagaaaatcctttttcttttttttttttttttgttgttttctttgagacggagtctcgctctggtgcccaggctggagtgcagtggcacgatctcagctcactgcaacctccgcctcccgggttcaagtgattctcatgcctcggcctcccaagtagctgggattacaggcacctgtcaccatgcctggctaattgttcctatttttaggggtttctccatgttggccaggctggtcttgaactcctgacctcagatgatccgctgtcttcggcctcccaaagtgctgagattagaggcgtgagccagtgcacccggcccattctcttggtttttaaagctgaaaacaagatcctggtgtttgtggtctcaggagaagatgccgtggccctgaggccagccctcacctgggctgcgtgaagaaggcatggatctgctgtgccactgcttgtccgaccacctgctccagttccccaatggaagcattactcagttgctggatgcttggaaacttctggaggagaaggggagctttaacttttccaactcctgggatctgctgcacggttcgaaggagcgaaggctcagacagcagcagggcccgtttcttcccgagaagagggttcttactgggctctttggtttgctcttgaaccaactggatgacgaggcaggatgcttccatctggctggccactggaagcagcaccattccaaggtccagcacagtaaacttctgtagggctgggaagtattgttcactcatccgggttttttcaacgactacaattcctttaagattattggaatttctaacccgaacaagcctctttctgtagccatttcctgccaccaaatcagcttcggtgacataaagaatgcagcatctgttcgacagataaaagtctggtgtcaagccatcctcgaaaatgagcttaattttcccttgcatctcctgcgccagctgtgacccgcgccatttctcattggccacaatatgccccaaaggcacgtgcacggggcccgtatcatcaggggggttcttttccatggatggtctccaccgtagcttctcagtccagtccaaggcccgaatacagccggcaggaaccccaccgtcccagtctagagatcatgttactggtggccgcgccaccttccgggttcac

SEQ ID NO: 11673 - RNA, 1973 nt, Homo sapiens
  source 1..1973: mol_type = other RNA
ctgaatagctgggactacaggtgtgagccactgtgcctggcctgtgtctattttttgaatgggcaatttgtaccttttgatccccagcccctgcttccctcactagatgcagctgctgccatcattttcttgtatccttccattgttgggcctttcatatacaaacacagcctgttctgcctcatgcatgttgagttttcaactttaaattttttttttttttttttgagatggagtctcactctgtcatccaggctggagtgcagtggtgcaatctcggcccattgcaacctccacctcctgggttcaagcgattctcgtgcctcagtctcctgagtagttgggattacaggtgtgtgccaccacacccagctaatttttgtatttttagtagagacagggcttcaccatgtcggccaggatggtctggatctcctgaccttgtgattcaccccccttggcctcccaaagtgctgggattacaggtgtgagccactatgcccggccgttgagttttcaactttaagtgggaacttcagacttcatactttctgtgtgcagaagacatatgcagtgattataaacaaactgtacatctgccaaaaaaaaaggccggggggagggaggaacaaaggaaaggaggaaggaactgttgcgcagttatttatttacattggaaacagccctcgcagtacgggtatatgaaggccagacctgatgaacagcaggtgaaactctgggaacccagggcttaggatacacagtgcttccttgtacatttgtttccttcagatggtcacatccaccactgaagctttttagaaggcactttccatgacagatgcaggtcaaggtcgcacattaaaatcggccctaatgctttttgctgagtgtgagtccctgactctcttgcgaagatcccaccagcccttttcgtcttagcagaatgaaggcagtgccctctgcggcccactaacttcacaagctgaactcagacgctaaggcaggacgacccacgggctccattcaagcctcgcctcatctttcactggttgctgctggagaaaatcctttttcttttttttttttttttgttgttttctttgagacggagtctcgctctggtgcccaggctggagtgcagtggcacgatctcagctcactgcaacctccgcctcccgggttcaagtgattctcatgcctcggcctcccaagtagctgggattacaggcacctgtcaccatgcctggctaattgttcctatttttaggggtttctccatgttggccaggctggtcttgaactcctgacctcagatgatccgctgtcttcggcctcccaaagtgctgagattagaggcgtgagccagtgcacccggcccattctcttggtttttaaagctgaaaacaagatcctggtgtttgtggtctcaggagaagatgccgtggccctgaggccagccctcacctgggctgcgtgaagaaggcatggatctgctgtgccactgcttgtccgaccacctgctccagttccccaatggaagcattactcagttgctggatgcttggaaacttctggaggagaaggggagctttaacttttccaactcctgggatctgctgcacggttcgaaggagcgaaggctcagacagcagcagggcccgtttcttcccgagaagagggttcttactgggctctttggtttgctcttgaaccaactggatgacgaggcaggatgcttccatctggctggccactggaagcagcaccattccaaggtccagcacagtaaacttctgtagggctgggaagtattgttcactcatccgggttttttcaacgactacaattcctttaagattattggacgtagcttctcagtccagtccaaggcccgaatacagccggcaggaaccccaccgtcccagtctagagatcatgttactggtggccgcgccaccttccgggttcac

SEQ ID NO: 11674 - RNA, 2080 nt, Homo sapiens
  source 1..2080: mol_type = other RNA
ctgaatagctgggactacaggtgtgagctactatgccacgcttatttttgtatttttagtaaagacagggtttcaccatgttggtcaggctggtcttgaactcctgacctcaggtgatccacccacctcagcctcccaaagtgctgggattacaggcgtgagccactgtgcctggcccattattttcaatataatagattatctaccatactgccttgtgaggattaaataagaatacctgtaaagcacttagcacaatatccaagttactaaatatcagtaaaaaagaagaaaagtccccccagacatattatgctctagtcaacacaagacttcctctacatggacttgaaattcagcatctctttagataatgaagagctcattgcttgataaggtgtcctatctcatggttagctcaaattgttagaagttcacactgaaattacagtgatttaatgatatgaacctccacttctctatactttacatgaaaaggaagctttgagtttgccacatcttttgctacaactcccaaaatcatgcccaaccaacttttaagtaagggccacaatcttgaccccagcatttaagacccttaacaatcaggtcctaccctgccattcgtcctggctttatttcctggtatatctctatataggccccatatttctgcccagctggatcacttctccttccttgagctctgattttacttttctacttgtgcacctgcacttatgatgtttcatctccaattcgtttagcaaaattctgcctatgttagtcttataccatctcatcttcccttcacctattgaatcctagtatctcagaagtccaactcagaatatctccattctctgactacctaagtcaaaaatgatacctgactttgtattcctgtagcagaatatttataccactcgcattgtacttttagtgttttatctcacagaataggcatttgtatcagttgcaggttagtttccccaggaaacagactcctgagatgaagattgcatggaggaagtttactggaaaggaatctcaggatcagcatctgtggaggaatgaaggaagaaggcttgggcagaggagaaactgacctgtgatgtaatcacaactatggcctcacctgttcctgtggagagccttgaggctgggttggcctggtaaagttgtcccaaactggggcaagcaggcatgcctttgtaacccctgtttattagtcactgggtgtggattgtaccttggaggaggcatcatgttgggcagcacagctctcttcaggcaagggcaagtcctagaaagggactcaggtgagaatatcagctgccaaccctcccagaagctgaggagacaaagaagctgaggaaataagagttcatccctggatggagatctaggcagcaaaacgtgacatctactacagtccaaccctttgtgtcactcaggtcaattttcttcataaaataagctttgagatcaactcttctggggttttgcttggtccctcttccacccagtgactagctggtctctatgaggaatggtgctgattccggggctcaactttggtctccgttgctggcaagttagacatggggcagcaacagtagctagatcagccttaatgagaggagtccgtgctgctggagccatgcacacttcatctctgccatcaggctattctgttctagtgccttttgtgccagcattggggtggctgttgacacaggctgactgacatcaactggctgagtcatttgtttatgcagctgtttaatgtctattctgttgtgggtgctcctgaggaaatttccataggtctctttgggaaaggactgaaggagtcatgatctttttagattctttttttatacagttgcagggtctttccttgtggggacctgattcctccttcaggcaagaaattctgggtctaagaacagctcagatttaaattcacttttaattgggaattttagttctcccgggctcccagtttcctttcctaggatctctcacagagcacagattcgatttccaagtcccgccgcactcttaccgctcgcat

SEQ ID NO: 11675 - RNA, 1790 nt, Homo sapiens
  source 1..1790: mol_type = other RNA
ctgaatagctgggactacaggtgtgagctactatgccacgcttatttttgtatttttagtaaagacagggtttcaccatgttggtcaggctggtcttgaactcctgacctcaggtgatccacccacctcagcctcccaaagtgctgggattacaggcgtgagccactgtgcctggcccattattttcaatataatagattatctaccatactgccttgtgaggattaaataagaatacctgtaaagcacttagcacaatatccaagttactaaatatcagtaaaaaagaagaaaagtccccccagacatattatgctctagtcaacacaagacttcctctacatggacttgaaattcagcatctctttagataatgaagagctcattgcttgataaggtgtcctatctcatggttagctcaaattgttagaagttcacactgaaattacagtgatttaatgatatgaacctccacttctctatactttacatgaaaaggaagctttgagtttgccacatcttttgctacaactcccaaaatcatgcccaaccaacttttaagtaagggccacaatcttgaccccagcatttaagacccttaacaatcaggtcctaccctgccattcgtcctggctttatttcctggtatatctctatataggccccatatttctgcccagctggatcacttctccttccttgagctctgattttacttttctacttgtgcacctgcacttatgatgtttcatctccaattcgtttagcaaaattctgcctatgttagtcttataccatctcatcttcccttcacctattgaatcctagtatctcagaagtccaactcagaatatctccattctctgactacctaagtcaaaaatgatacctgactttgtattcctgtagcagaatatttataccactcgcattgtacttttagtgttttatctcacagaataggcatttgtatcagttgcaggttagtttccccaggaaacagactcctgagatgaagattgcatggaggaagtttactggaaaggaatctcaggatcagcatctgtggaggaatgaaggaagaaggcttgggcagaggagaaactgacctgtgatgtaatcacaactatggcctcacctgttcctgtggagagccttgaggctgggttggcctggtaaagttgtcccaaactggggcaagcaggcatgcctttgtaacccctgtttattagtcactgggtgtggattgtaccttggaggaggcatcatgttgggcagcacagctctcttcaggcaagggcaagtcctagaaagggactcaggtgagaatatcagctgccaaccctcccagaagctgaggagacaaagaagctgaggaaataagagttcatccctggatggagatctaggcagcaaaacgtgacatctactacagtccaaccctttgtgtcactcaggtcaattttcttcataaaataagctttgagatcaactcttctggggttttgcttggtccctcttcctgaggaaatttccataggtctctttgggaaaggactgaaggagtcatgatctttttagattctttttttatacagttgcagggtctttccttgtggggacctgattcctccttcaggcaagaaattctgggtctaagaacagctcagatttaaattcacttttaattgggaattttagttctcccgggctcccagtttcctttcctaggatctctcacagagcacagattcgatttccaagtcccgccgcactcttaccgctcgcat

SEQ ID NO: 11676 - RNA, 2573 nt, Homo sapiens
  source 1..2573: mol_type = other RNA
ctgaatagctgggactacaggtgtgcaacaccacacccagctaatttttgtatttttttagtagacacaaggtttcaccatgttggccacgctggtctcgaactcttgacctcaactgatctgcccaccttggcctcccaaataaccttaaatcttaaggttgatgcatgcctcttaatctcttggtttgcccatcagaaactgaatcatgggctcactaggagaaattgtcagtttaaaaatcctatgcttttcaaagaggttttattttggataactgttgcaattatagacctagagaagacatttaacccacccatgtttcagtttctattttcttcctcactagattattttattcacttttcaatttttaaaaattagatttattgcagactggcctcaagctcccagactatattttttagctgcattatttaggggttgaaatgccagcttttgagacttttgaaaaattcacaggctgggtgtggaggctcatgcctgtgaaggttgcagtgagctgagatcgtgccactgcactccaacctgggtgacgagagtgagaccctatctcaaaaaaaaaaaaaaaaaaaaaaaaaaagggtctggtgcagtggctcacacctacctgtaattccagcactttgggaggccaaggcaggccgatcacttgaggtcaggagtttgagatcagcctggccaacatggtgaaccctgtctctactaaaaaatacaaaaattagctgggcataatggtgtgcatttgtaatcccagctactcgggaggctgaggcatgaaaatcacttcaacccaggagacggaggttgcagtgagctgagaacgcaccactgcactccagcctgggcaacagagtgagactctgtctcaaaaaaaaaaaaaaaattcatattgcttctgacaagcctattaaacacatcaatagcaccctgggagcccatgaagtattattattgctcaagaaaggaaacatggcagagaaacaagcagaagcagctctggctgacagcctgagggtaaagagcactggagaagtaaagaaaaggaaaaggtcaccaccctgatctgacatgttgaattgagaggtaggttgtatgatagggaaggaatagggccagctgtggctgccagtagcagaatgtccaggttggaactctggtctaaagcctaggagagcagaacggtaagaggctacaaaataaaaacaaactggattatcaaggtggtcatactgagtaggcagggatggagatcttcaggctcccagccgggccccaatttacagtagagaggctcaagcagggatagggtagagcaagaaggactccagatcacagtcaaagtcgtcaaagggcatggtctccgctgaactgggctgggtagcttgtgtctccgtgacaaagttcactggctgcttctgtaggagctctgggtcgaaggccacaccccgaaagaaagggtggacctggaagtgatgcagataacgtagacgatggagggggttctggcataagagctcatggagcaggagtgagaggccctggttaagagaagctgggatctcagagtcactgtgggtcacacttgccaacatggccacatgatctctctctgcagccactggaaactttccagtcgccagagagaaaagcaagacacccagggaccaccaatcagcagcatggttgtaaggtcctccacttaggacctctggggccatgtactgaagagtgccacagatagtgtaggcttgagctccctggggcacgtggcgggacagaccaaagtctgtcagtttcagatggcctcgttcatctagaagaatattctccatcttcacatctcgatgcatgatgcccaagtcatggagataacacagtaccagcaccaactcggcagcaaagagacggatggaagcctcaggaaagcagccaacagccgaccaaagggagtacagatctgtgctgcagtagctacacataatgaaaaggtgccgttttccctgccagctgtcccccaagctgtgtacaaagggatggttgatctgtcgctggatgctaacctcctctttgcactgcctcacggtatccctctgtaggacctttaccttgggcaccaccttcactgcaaatacagctttctgggtgcaatctagcaccttgaggacagttccaaaggagcctttagccacgaggcctaaaatcttcagctgctgctgccccctaatgggcctaatgggaaactctggtagaaagaggttgatgaactgaggcactggccactctggcagaggcttctctaccagtactggggctggctttagggattcctggtgcagatagtggtgcccccgtagttcccagagttcttccagatctgacctgatggttcccaaacctgtccagaggctcttccagcctcgggcccagggaccccggatgttgccaccctgcttgtgagggacagccacccgggtgtgttccccctgctgggtgtgctgcccctgccgacagcttactgctcccattcccagcctctgcctcctctctct

SEQ ID NO: 11677 - RNA, 4162 nt, Homo sapiens
  source 1..4162: mol_type = other RNA
ctgaatagctgggactacaggtgtgcacaacacacttggttaatttttgtattttttatttagagacgaggttttgccatgttgcccaggctggtcttgaactcctgagctcaagtgatctgcctgtctcagctcacaaagtgttaggattacaaccaccgtgcccggccaatagctttttcaaactagctttttcaaaggtcaaatgcatcctcaccaaggggacaagattgaaagtagaatggcctgggcttaataaatcaatgatttgaaactatcagaagaaaacatggagaaaatgctccatgacattggtctgggcaatgatttttttggatacgatctcaaaagcacagtaacaaaagcacaagtacagaaatgaaattacatgaaactaaaaagcttctgcacagcaaaggaaacaattaatagggtgaagagacaacctacagaatggagaaaaaatattaactatagatctgatagggggttaatatccaaaatacataaggaactcaatagcaggaaaacaacccatttaaaaatgggcaaagaacctgaaaagacagttctcaaaagaagacatgcaaatggccagcagatatatgaaaaaattatcaacatcagcagtcaccagggaaatgcaaattaaaacaacgagataccacctaacacctgttagaatggctactatcaataacacaaaagataacaagtgttggcaaggatgtgaagaaaaaggatttcttgcattattgtgaagaaaaaggaattcttgcatattcttggtaggaatgtaaattagtacagccattatggaagacagtatggagtttctgcaaaaagttaaaaatagaactacatatgatccagcaatcctaatactgggcttatatccaaaggatatgaaatcagtatgtcaaagagatatctgcactaccaggttcactgcagcattattcacaatagccaggatatggtatcaacctaagcatctgtcaatggttgaatggataaagaaaatgtagtacatatacacaaacagctgatctcatagaagtagagagtagaatggtggttaccaggagctagggttgttggagaaacattggtcaaaggatacaaaatttcagttaaaaagggggaattagtgcaagagacctattgcacaacatagtaactatagttacaattacaagattactattaattttgaaaaataagagaatggatgtaaagtgttcttaccacaaaatggtaaccatgtgaggcatatgtcagttagctagatttagtcattctataatgtatatatgcttcaaaacagtatgttgtacatggtaaatacatacaattttatctgccaattggaaaaaaaaatcaattgtaaaagcaagtgtttggaaaacatttagctggaaaggtctgataggaggtctaacccttatacacttaaaaactcaacaactggctgggtgcagtggctcaagcttataattccagcactttgagaggccgaggcgggtggatcatttgaggtcagcagttcgcaaccagcctggccaacatggtgaaaccccatctctactgaaaatacaaaaaaattaaccgggcgcagtggcgggagcctgtaatcccagctactcaggaggcttaggcaggagaattgcttgaacctgggaggtgaaggttgcagtgagctgagatcaaaacactgcactccggcctgagcgacagagtgaaactccatctcaggaaaaaaacaaaaaaacaaaaaaccctcaacaactgtttacttttggtattcaagctcataaaagcctcatttactagtctactgctggtaaggatcaggaagggaaaattaagattaccttcatgataatcacgtgtgggttgacacagacggagacaataacatagaaattttattacagcatttcatgtttaagccagattccctgccaggatattttctgcttgaattaatgaggcaggatttggtcataccttaatgagtttcacagaaaaagagttcaagcattagcgcaaactgccttctgacattaaaataaaataaagcaaacatgggattttcacaaagttaaaagcctcctgtgatgcacattttggatagtaggagacattgagccccaaaatgtttaacataaagcatggttaattaaatgaaaccactgaaaaatgtgaatacatgaagaagaaagaataaaataattttgatgttaccatttcaactactatttttgatataatcattcttggcaaaatcattcttaaaggtggaaacgagcaggctgatagtacagcaagtaagagaaagtcaatactgatggcctccacttgctgatcctctgagactgcatcttatagttcataaaatctgctgaaggtcacaactgaggtacaacgacttgtgttacttgtactgtagcaatgagggctttcccaggccacaacatctgggatcaaggaacacattttgactaaataaactatacagaagtctgttttaggattttatgcaaatattaacctcattttaaaacatgaggaaaaatattacccacatttagggctaatttagctgtcaggaatagaccatacagttgaaaaaaacacagtctcatttaaaaagtttcagcagagacaaaaaggtactaaagatgatattcatccttcttcatcactgctgctccaggcatcttcaaaggccggatttaattgtgattttgttgtagtctcatcatcatcaggaactggttcatataaggatggaacccaagccagaatgttgcagtctctgctaccactataaagttcctggaaatttgactgaaatacacagcagtcaacagttttataatgtcccttaagcatagttatctgttctcctgagtaaactgtataaacagcaatggtgctaccatatggtacaaaaacaaattctgaactgcagccacaggagacagtgaatttcaatccttttttactgttattacaaacttttccatagttcacaagtgtgttttctccattggaactattccagagcctcattcgattatctgtaccaacagtgaggaggtgaagtccatcacttgtaaaacataagccattaactttcccattatgagcagtgtttgctgattcaacagcttgtgactttttcccattatgttgatcaagagtaatcaaacatcctgatgctcttctcacatcccataattttactctactgtcagcacttgctgttgccaagatatagtcataacgtggagaccaggaaactgctaatatttcttgtctgtgaccctgtagaatgtgagaacaggatccagacttcaagtcacaaagttgtactttgggtcctctagtaccaactgctaccaaacagtgcttggtggagactggagacatatgatgactataaactgtttcctcaaaattaaatacatctgcagtttgtaatgtatttgtatcccatactttcagagttttatcaaatgagcttgatgtgaacatgccagtgtcatgaggataccactgtacagtctccacactgtatctgtgaacatcaggatgatctctgccaatggaacacactgctttacatgtgtaataagattgtctgctggagttctcaaggtcataaagtacaatcacaccatctgaaccacctgataacatgcgtcaatccttaagttgctgtctctcttgtcattctggttgaatgatttcattctctggttgattcctaaggaatggctaatgagaacaacagtctctgaattcttgtgttgttgacaatttatccgtcctttttgtatctgaaatcagtttggctggatataaaatccttgactcacattttatttccttgagcatcttggataagaagcttcattttatctcccttcaacaggttcaatgtcaagggtgttaattccaccgccgtggattctttcaacatctctgtctttatttaattccagtcccaaaactctccgtgttgactctgctctccgaaggcgaagagggtcctccaaacccgtttggcgtgcggacaaaaaccccagcatatcgtgtcctcacaccggctggagcactggacgtcgccatgacagagctcaggggcgggact

SEQ ID NO: 11678 - RNA, 3944 nt, Homo sapiens
  source 1..3944: mol_type = other RNA
ctgaatagctgggactacaggtgtgcacaacacacttggttaatttttgtattttttatttagagacgaggttttgccatgttgcccaggctggtcttgaactcctgagctcaagtgatctgcctgtctcagctcacaaagtgttaggattacaaccaccgtgcccggccaatagctttttcaaactagctttttcaaaggtcaaatgcatcctcaccaaggggacaagattgaaagtagaatggcctgggcttaataaatcaatgatttgaaactatcagaagaaaacatggagaaaatgctccatgacattggtctgggcaatgatttttttggatacgatctcaaaagcacagtaacaaaagcacaagtacagaaatgaaattacatgaaactaaaaagcttctgcacagcaaaggaaacaattaatagggtgaagagacaacctacagaatggagaaaaaatattaactatagatctgatagggggttaatatccaaaatacataaggaactcaatagcaggaaaacaacccatttaaaaatgggcaaagaacctgaaaagacagttctcaaaagaagacatgcaaatggccagcagatatatgaaaaaattatcaacatcagcagtcaccagggaaatgcaaattaaaacaacgagataccacctaacacctgttagaatggctactatcaataacacaaaagataacaagtgttggcaaggatgtgaagaaaaaggatttcttgcattattgtgaagaaaaaggaattcttgcatattcttggtaggaatgtaaattagtacagccattatggaagacagtatggagtttctgcaaaaagttaaaaatagaactacatatgatccagcaatcctaatactgggcttatatccaaaggatatgaaatcagtatgtcaaagagatatctgcactaccaggttcactgcagcattattcacaatagccaggatatggtatcaacctaagcatctgtcaatggttgaatggataaagaaaatgtagtacatatacacaaacagctgatctcatagaagtagagagtagaatggtggttaccaggagctagggttgttggagaaacattggtcaaaggatacaaaatttcagttaaaaagggggaattagtgcaagagacctattgcacaacatagtaactatagttacaattacaagattactattaattttgaaaaataagagaatggatgtaaagtgttcttaccacaaaatggtaaccatgtgaggcatatgtcagttagctagatttagtcattctataatgtatatatgcttcaaaacagtatgttgtacatggtaaatacatacaattttatctgccaattggaaaaaaaaatcaattgtaaaagcaagtgtttggaaaacatttagctggaaaggtctgataggaggtctaacccttatacacttaaaaactcaacaactggctgggtgcagtggctcaagcttataattccagcactttgagaggccgaggcgggtggatcatttgaggtcagcagttcgcaaccagcctggccaacatggtgaaaccccatctctactgaaaatacaaaaaaattaaccgggcgcagtggcgggagcctgtaatcccagctactcaggaggcttaggcaggagaattgcttgaacctgggaggtgaaggttgcagtgagctgagatcaaaacactgcactccggcctgagcgacagagtgaaactccatctcaggaaaaaaacaaaaaaacaaaaaaccctcaacaactgtttacttttggtattcaagctcataaaagcctcatttactagtctactgctggtaaggatcaggaagggaaaattaagattaccttcatgataatcacgtgtgggttgacacagacggagacaataacatagaaattttattacagcatttcatgtttaagccagattccctgccaggatattttctgcttgaattaatgaggcaggatttggtcataccttaatgagtttcacagaaaaagagttcaagcattagcgcaaactgccttctgacattaaaataaaataaagcaaacatgggattttcacaaagttaaaagcctcctgtgatgcacattttggatagtaggagacattgagccccaaaatgtttaacataaagcatggttaattaaatgaaaccactgaaaaatgtgaatacatgaagaagaaagaataaaataattttgatgttaccatttcaactactatttttgatataatcattcttggcaaaatcattcttaaaggtggaaacgagcaggctgatagtacagcaagtaagagaaagtcaatactgatggcctccacttgctgatcctctgagactgcatcttatagttcataaaatctgctgaaggtcacaactgaggtacaacgacttgtgttacttgtactgtagcaatgagggctttcccaggccacaacatctgggatcaaggaacacattttgactaaataaactatacagaagtctgttttaggattttatgcaaatattaacctcattttaaaacatgaggaaaaatattacccacatttagggctaatttagctgtcaggaatagaccatacagttgaaaaaaacacagtctcatttaaaaagtttcagcagagacaaaaaggtactaaagatgatattcatccttcttcatcactgctgctccaggcatcttcaaaggccggatttaattgtgattttgttgtagtctcatcatcatcaggaactggttcatataaggatggaacccaagccagaatgttgcagtctctgctaccactataaagttcctggaaatttgactgaaatacacagcagtcaacagttttataatgtcccttaagcatagttatctgttctcctgagtaaactgtataaacagcaatggtgctaccatatggtacaaaaacaaattctgaactgcagccacaggagacagtgaatttcaatccttttttactgttattacaaacttttccatagttcacaagtgtgttttctccattggaactattccagagcctcattcgattatctgtaccaacagtgaggaggtgaagtccatcacttgtaaaacataagccattaactttcccattatgagcagtgtttgctgattcaacagcttgtgactttttcccattatgttgatcaagagtaatcaaacatcctgatgctcttctcacatcccataattttactctactgtcagcacttgctgttgccaagatatagtcataacgtggagaccaggaaactgctaatatttcttgtctgtgaccctgtagaatgtgagaacaggatccagacttcaagtcacaaagttgtactttgggtcctctagtaccaactgctaccaaacagtgcttggtggagactggagacatatgatgactataaactgtttcctcaaaattaaatacatctgcagtttgtaatgtatttgtatcccatactttcagagttttatcaaatgagcttgatgtgaacatgccagtgtcatgaggataccactgtacagtctccacactgtatctgtgaacatcaggatgatctctgccaatggaacacactgctttacatgtgtaataagattgtctgctggagttctcaaggtcataaagtacaatcacaccatctgaaccacctgataacatgtatctcccttcaacaggttcaatgtcaagggtgttaattccaccgccgtggattctttcaacatctctgtctttatttaattccagtcccaaaactctccgtgttgactctgctctccgaaggcgaagagggtcctccaaacccgtttggcgtgcggacaaaaaccccagcatatcgtgtcctcacaccggctggagcactggacgtcgccatgacagagctcaggggcgggact

SEQ ID NO: 11679 - RNA, 3862 nt, Homo sapiens
  source 1..3862: mol_type = other RNA
ctgaatagctgggactacaggtgtgcacaacacacttggttaatttttgtattttttatttagagacgaggttttgccatgttgcccaggctggtcttgaactcctgagctcaagtgatctgcctgtctcagctcacaaagtgttaggattacaaccaccgtgcccggccaatagctttttcaaactagctttttcaaaggtcaaatgcatcctcaccaaggggacaagattgaaagtagaatggcctgggcttaataaatcaatgatttgaaactatcagaagaaaacatggagaaaatgctccatgacattggtctgggcaatgatttttttggatacgatctcaaaagcacagtaacaaaagcacaagtacagaaatgaaattacatgaaactaaaaagcttctgcacagcaaaggaaacaattaatagggtgaagagacaacctacagaatggagaaaaaatattaactatagatctgatagggggttaatatccaaaatacataaggaactcaatagcaggaaaacaacccatttaaaaatgggcaaagaacctgaaaagacagttctcaaaagaagacatgcaaatggccagcagatatatgaaaaaattatcaacatcagcagtcaccagggaaatgcaaattaaaacaacgagataccacctaacacctgttagaatggctactatcaataacacaaaagataacaagtgttggcaaggatgtgaagaaaaaggatttcttgcattattgtgaagaaaaaggaattcttgcatattcttggtaggaatgtaaattagtacagccattatggaagacagtatggagtttctgcaaaaagttaaaaatagaactacatatgatccagcaatcctaatactgggcttatatccaaaggatatgaaatcagtatgtcaaagagatatctgcactaccaggttcactgcagcattattcacaatagccaggatatggtatcaacctaagcatctgtcaatggttgaatggataaagaaaatgtagtacatatacacaaacagctgatctcatagaagtagagagtagaatggtggttaccaggagctagggttgttggagaaacattggtcaaaggatacaaaatttcagttaaaaagggggaattagtgcaagagacctattgcacaacatagtaactatagttacaattacaagattactattaattttgaaaaataagagaatggatgtaaagtgttcttaccacaaaatggtaaccatgtgaggcatatgtcagttagctagatttagtcattctataatgtatatatgcttcaaaacagtatgttgtacatggtaaatacatacaattttatctgccaattggaaaaaaaaatcaattgtaaaagcaagtgtttggaaaacatttagctggaaaggtctgataggaggtctaacccttatacacttaaaaactcaacaactggctgggtgcagtggctcaagcttataattccagcactttgagaggccgaggcgggtggatcatttgaggtcagcagttcgcaaccagcctggccaacatggtgaaaccccatctctactgaaaatacaaaaaaattaaccgggcgcagtggcgggagcctgtaatcccagctactcaggaggcttaggcaggagaattgcttgaacctgggaggtgaaggttgcagtgagctgagatcaaaacactgcactccggcctgagcgacagagtgaaactccatctcaggaaaaaaacaaaaaaacaaaaaaccctcaacaactgtttacttttggtattcaagctcataaaagcctcatttactagtctactgctggtaaggatcaggaagggaaaattaagattaccttcatgataatcacgtgtgggttgacacagacggagacaataacatagaaattttattacagcatttcatgtttaagccagattccctgccaggatattttctgcttgaattaatgaggcaggatttggtcataccttaatgagtttcacagaaaaagagttcaagcattagcgcaaactgccttctgacattaaaataaaataaagcaaacatgggattttcacaaagttaaaagcctcctgtgatgcacattttggatagtaggagacattgagccccaaaatgtttaacataaagcatggttaattaaatgaaaccactgaaaaatgtgaatacatgaagaagaaagaataaaataattttgatgttaccatttcaactactatttttgatataatcattcttggcaaaatcattcttaaaggtggaaacgagcaggctgatagtacagcaagtaagagaaagtcaatactgatggcctccacttgctgatcctctgagactgcatcttatagttcataaaatctgctgaaggtcacaactgaggtacaacgacttgtgttacttgtactgtagcaatgagggctttcccaggccacaacatctgggatcaaggaacacattttgactaaataaactatacagaagtctgttttaggattttatgcaaatattaacctcattttaaaacatgaggaaaaatattacccacatttagggctaatttagctgtcaggaatagaccatacagttgaaaaaaacacagtctcatttaaaaagtttcagcagagacaaaaaggtactaaagatgatattcatccttcttcatcactgctgctccaggcatcttcaaaggccggatttaattgtgattttgttgtagtctcatcatcatcaggaactggttcatataaggatggaacccaagccagaatgttgcagtctctgctaccactataaagttcctggaaatttgactgaaatacacagcagtcaacagttttataatgtcccttaagcatagttatctgttctcctgagtaaactgtataaacagcaatggtgctaccatatggtacaaaaacaaattctgaactgcagccacaggagacagtgaatttcaatccttttttactgttattacaaacttttccatagttcacaagtgtgttttctccattggaactattccagagcctcattcgattatctgtaccaacagtgaggaggtgaagtccatcacttgtaaaacataagccattaactttcccattatgagcagtgtttgctgattcaacagcttgtgactttttcccattatgttgatcaagagtaatcaaacatcctgatgctcttctcacatcccataattttactctactgtcagcacttgctgttgccaagatatagtcataacgtggagaccaggaaactgctaatatttcttgtctgtgaccctgtagaatgtgagaacaggatccagacttcaagtcacaaagttgtactttgggtcctctagtaccaattgtaatgtatttgtatcccatactttcagagttttatcaaatgagcttgatgtgaacatgccagtgtcatgaggataccactgtacagtctccacactgtatctgtgaacatcaggatgatctctgccaatggaacacactgctttacatgtgtaataagattgtctgctggagttctcaaggtcataaagtacaatcacaccatctgaaccacctgataacatgtatctcccttcaacaggttcaatgtcaagggtgttaattccaccgccgtggattctttcaacatctctgtctttatttaattccagtcccaaaactctccgtgttgactctgctctccgaaggcgaagagggtcctccaaacccgtttggcgtgcggacaaaaaccccagcatatcgtgtcctcacaccggctggagcactggacgtcgccatgacagagctcaggggcgggact

SEQ ID NO: 11680 - RNA, 8691 nt, Homo sapiens
  source 1..8691: mol_type = other RNA
ctgaatagctgggactacaggtgtgcaccaccacacccagctaattttttgtatttttagtagagagacggggtttcactgtgttagccaggatggtctcgatctcctgaccttgtgatctgcccgccctggcctcccaaagtgctgggattataggtgtgagccaccacacccggccgcataagcactttccaagcctctgcttgtatcatgtttgctattgttctagtggctgaagcaaaccacatagtcaaacctagaaggagagcaacaatccaagggcatggctacagaaaggctggcccagttggggtcattaatgggtatacctggctccagaactaaggcgctttaccatcataagctcccaatgtttaaacagtaagtctgcccgcactccttccagggtggaaaaactcagatactgataaattctcttgatcacagcccagtttttcccagcggattccccaccatccctcctatccccagacgctggagtctaggtttccagcccagtcaaaatctcaaggatctttcttttccctcaaactccaaaagaacagacacgcaataggatttctattcatttttattcattcctccaaagagcaccacaggccaaccacacccttgatgtgtccttcatggttccccactgcagtggacacaaatccctccatcattatccaggcatggatggaactctgctgtggtgaggaggttgtctcgcccactcacccaagttttccatgcctgttctgcttttgatggcaatgccaaaattcatcatacatttccttgaattcctgccttcaagggtcttccagccctgtggtgccatgcagacacacttcagtggcggccagtgatctgtctacaagggagtcttagtcttttctgcttggatgctcccagggacagatgcctgccaacaaccttatgtcttcacaaagactaaaatggaatcccattaaaagttatgatttaaaaggcgaccacccccaaaagaagtcataacactcaagggtgtcaatatatacaactgtgtaaacacaaccaatctacaactatatcaacacaaccagcactcctctatgggcacagacacacacacaaaattgtcttgctttctcagatatgatctctggcatgactcctgctggcatgagggcagaggaaattgagaggagcaaagcatatagcagtgatgtcagacaggaccaaatcagagacagggtcaaagtggcagaaaaatgaggagcacactccgagcaaaggcatgggggtgagacaaaggcacccagactagagccatcttggtgctgcccaggggtgggtggcactcatgtttgagctccatgtgtcaggcttttcaggaaagggtgtactatgttatgtgtctgtgtgcatattgtgtgcctgcatgtacatacatacgctgaattctcaccataaccatgtgaggtagatgccatttgtagagtgacttgcccaagtcagtggaaggactatctgcccctagagctagactgatagaattttctatgttgatggaagtattctgtaccttccctgtccaataccatagccactaatcacatgtggctactcagtattaatgttgcactactgccaatgaaacatagaattttaagttgtatttacttttaattgaacagctgaggccaggtgtggtggcccatgcctgtaataccagcactttgggaggccgaggtgggcggatcacctgaggtcagcagttcaagaccagcatgcccaacatggtgaaaccccgtctctgagaaaaataccaaaattagccaggcatggtggcatacacctgtagtcccagctactcaggaggatgatgcaagagaatcagttgaacctgggaggcagaggttgcagtgagctgaggtcatgccactgcactccagcctgggtgacaaagtgagactctgtctcaaaacaaaacaaaacaacccagcaacttggtcaacataaccagacctgcatctttacttaaaaaaaaaatggacacccatctcagtttttggaaaactattatataattggaacaacttggatatgtgaatctacttctccaactatgaattttatgaaatcaaaataaaggtcaagcatttcagataaaaatgtaccatggtaattgagatttggtgtaagtgtaaaatatataacagattttgaagacagcacaaaagaacgtaacataattcatttaaataataccgatgacgccaggcacggtgcctcacgcctgtaatcctagcactttgggaggccgaggtgggtggatcacctgaggtcaggagtttgagactagcctggccaacatggcgaaaccccatctctaaccaaaaatacaaaaattagtgggcatggtggcgggtgcctgtaatcccagctactcgggaggctgaggcaggagaatcacttgaacctggaaggtggaggttgcagtgagccgagattgtgccactgcactccagcctgggcaacaaagcgaagcactatctcaaaaaaaaaaaaaactaaaaaaccgatgacatgttgaaatgctattttggatacattgggttaagtaaaacatgttaaaatgaatttaacctgtttccttttacttgtctaatgtggctattagaaaacttggcttactcagcactttgggaggctgaggtgggcagataacttgaggccatgagttccagaccagcttagccaacatggtgaaaccccatctctactaaaaatacaaaaattaggacgggtgcagtggctcacgcctataatcccagcactttgggaggctgaggccggtggatcacctgaggtcaggagttcaagaccagcctggccaacacagtgaaaccccatctctactaaaaatacaaaaattagctgggcatgatggtgcatgcctgtaatcccagctacttgggaggctgaggttgcagtgagccaagatcgcacaactgcactccagcctgggtgacagagcaagactccgtctcccaaaaaataaataaataaataaaataaaaatacaaaaattagctgggcgcggtggctcatgcctgtaatcccagcactttgggaggccaaggcgggtggcctgaggtcagtagttccagaccagcctgatcaacatggtgaaaccccatctctactaaaaatacaaaaattagccaggcatggtggcatatgcctgtaatcccagctactcaggaggctgaggcaggagaatcacatgaacctgggaggcggaggttgcagtgaggcgagatcgtgccactgcactccagcctgggtgatggagtgaaactccatctcaaaaaaagaaaacttaaaatgacatatgtggcttgcatttcgtttctactggacagtgctgccctgcagccctcccattccatcacgtggctgacatgcctgattgcagggcttagacactaatatgatggggtaaagatatggatgaatattcttccccaaagctgaaagagctttcatgaaaatgcctggagccattcagtatagaactaagtgctcttccccatggtagctatctcaactttgaagggacaaattttgtcagcagtgggagtccaagctggagatgatggtaccatcccttgtctgcccttggatcagttacctttgtcttcagcttttaagggagacaggatctcaaaactaaggttcttatccagctcttttatttcacagatgggaaaataaggcactgtccaagtaacacacagtgacagtggcaaagtcgtgcttgcttcccaggtccctgacctcagacaagggtgttctctcccattaaatgcttttttctcctcatcttgctccattttcctatcttgtggcaagagattaacaatctaaattccaatcctagttctgacactgaccaatgaaataaacatttaggctgggtgtggtggctcacacctgtaatcccatcaaggcaggaggatcacttgaggccaggagttcaacactagtgtgggctacaaagcaagacccccgtctctacagaaaatttggtgctgtgtacctatagtcccagctactctgtaggcggaggtgggaggatcgtttgagcccaggagttggagatggcagtgagccatgatcatcccactgtattccagccggggcaacagagcaagaccctgtctctaaaataataataataataataaatatttacgaagcacctattgtgtcaggcacctattgttctagatgctggggaaacaacagagaacaggacaggcaacgggtcaaaagccaataaacaggtaaataaataagatcatttttgacagtaataattgctacaaggaaactcaactggccgaaatgaatagtgggggaatgtgagctacttcagatagggtggtcagggaggggaagtcctctctgaggggatacgtgagctgagatctgactgagcccgtcacaggaaggtttgagagtagaacaggaagttgtgagtagagccttgaaggaaagagaacagcaggtgcatgggtccccaggcaggactcaaggtagccactcaggcatcagaaagagtcaggcggccatgatggctcacacctgtaatcccagcactttgggagtctgagtcgggtggatcacctgaggtcaggagttcgagaccagcctgaccaacagggtgaaatcccttctctactaaactacaaaaattagccaggtgtggtggcacatgcctgtcatctcagctacagtcatcacatccctgtactccagactgggtgacaaggtgagactccatttcaaaaaaaaaaagaaggaaagtctatcaggctggacaggagtgggaaggggcagtgaatgagaataggcaagggccagacccacagggccttactgtgtgctgttgggcctcaagcctgccctctctggactttgctctttctgtctacgacaaaagggattctatcgcttggattctcagatcctccttttctgtttttgacactgaagaattctgtaacctgcaacttttcccccacatgtggctagcagcctagaacattccaggcactgtggtttctgcctttgcttcattcactcctggcatattcccatggtctcaagtgcctgaccacccatttggtgggcccctggctcaatgcagcaccctctatgtacatcagaaagcagagcctcttggggatacccgaggtgtccatacagaagtgtttggaccagtgcagcagtacagctgctcttctgaaaaggaaggtgcacaaaacaccaaggccataaagggttatggttaaataccaggagaaaaaggccaaaaaaagatagaaactcctaaagaaaagagacagagaaacagactccccagagatcacctgaattgctcagcacctagaagatgaaggcagtcatatcccttcccagtcacactcacagaggcagttgccgggatcccaatacaaggtttggaggagctgtctctgaggtatgctttactgcccttccacacccaaaagacctcattcctggtccctggctactcccagagcccaccatgcccagacctcttacccacctcacctcatttttgtgggaccaccctccctacatgcttttggagggcaattatagaaacccatccactccccaggagagatcaagaagtctccagctttctcgcacaagcccccgatccctcctccagatgcagacctccccttacccaatatttaggaaccaaggtccacagccatcttagaaccccggaagtctcagaccccaggggcctccgccaccccatcaagattcaaagcccactgctccttggggacctgtgtgcaggctttttctcccagagaaatgtagaccctgtttccctctgaggctctgaagcccaagagttccagctccctggggcgctcaggtctccctcccctatactggagttcaggtcccagtcatggacacctccccaccaattaggaaacaggacttctaccagcctccctggaggactaaacatccagtaactccagtttctactccctaggagacaaagacatagtccctgctagagtctgggccaccaactcccttcaggacagaagggtctagatgtcattcaccatggttcccaaaggtatcaggattcctggccaggggcggtggctcacgcctgtaatcctagcactttgggaggccggagcgggtcgatcgcctgaggtcaggagttcgaggccagcctggccaacatggtgaaaccccgtctctactaaaaatacaaaaattagccaggtgtggtggcaggcacctgtaatcccagctactccggacgctgaggcaggagaatcgcttgaacccgggaggcggaggttgcagtgagccgaggtcgcgccattgcactccagcctgggcaacaagagacttcgtctcacaaaaaaaagaaaaaaaaaaaaaaaaatcaggattcctgtcccccagactctctgaatccaggtgataagaagtcacacatcccagctggaagtcaagagtccacatccccttcaagcacccaggattaagcccaggcatcccctgtcagagtctggactcccaagccccctcccactcctcactgggcaggctcagggggtgccagcacagcctcagcatcagcccgcatctcatcgagagcctgcagcaggacgccgtgagccgctcggtagcccaggccacctgtcgccgctgcaccacccgcaggccacaggaaggagagagcccccagtgctgcgcccccagcagtgccctcgcccgcccaggcgcccagtcttgcttccacctcggcgcgcgtcaccgggcctgggaaatgagcgcgcgctgccagctctccagaagccaggcccagggcacgctcacgtcgagccagtgccgtgggttccagccccaggccccgtcgccactccgccagctgaccccgcagaagtgccacgtcgcatgcccagcccagccctgggagtggtgccgccgccgccgccagactagccagcagagctggcctccacgccccggctcgcaacgccgcagccttggttcgggcagcgctgggagatgctggtggcaacgccagcagcagtgcccctgcctgggctggggggagcgctcgccgcagccattcgcatagccctgggagtccgccaggccgtagggggaacactggcggcggcgcctcctccagcacctcccacgtctcgtcctccgggcttaacgcagcggcccgctctgagtcgccaccacctgatttcttcatgccgacaacctgctgcaaaccctcgctgccagctttcccaggaccttccccgctgcctgctttctgcgatccagcgctacatttctcccttcccttactgagtgcattctccaatccccctccacctgcgttctttaagctctcgcccttgggattctccatcttgccttctcccagacactccggatcctcgccctcgccgtctgtgcgcacgcagacaagaggcgcatctggtagcagcaaggcctggacctgggcccagtccttctcagtgggggccccaggggtgacgaggatgagggcgtcgtagtgcgttgggtgagaggcggcggccgcggtggtggcagtgcccgtgtggcccagaggcacggtccagagcaccacattcgggcgctctggggctgggaagggagtgggtgctgtggggaccgaagcaggcgcagcgcctgggtcgccaggatccaatccaagcagcatgtccaccacaaggcccacgtcagccttgccagccacggccaggtctagccgtgcgctgcccaggcgctccaggcctgagcgcacccacgacagcgcagcctcaaggccgccggtctcaaaggcctcacgcacagcctctagctctgctgcacccaacacctcgaagccatcctgcgccggtggcaggagcctccgcagcgcttctgcctggctctgcagcgccgcccggaggcgctctagctcctcgcagccgtcgctgctgccgcagttcgccggtagcacaaacagatccgcagctcctaaccccgcgctgttcagcagagctgctgtctgatcacgggcctgggcggcagtctgtgaatccccaggacggaggttccgcacagccagtagcggggtccctcgggccagggcggccagcgctgcctctcccagggctggagccaacggttccccgttcccctcgggtccgggcagcaccagtaccagcacgttggcttccgccgcccagggccccggcgctgcgggtgggcagctcagctcgcccagaaaaaggcctgggcccgcagctcttaggctgggaaccccggagtccggccgtccctcgggggcctcgagcgtctccacatccttgtcgcacagcgctgcgatcagcgcggacttccccaagcccggaggccccaggaacaaggcggtcacgtcaccctgcggcggaggcatggcgagcaaaaagccgacccacgggagagagcgcagtcggtggcagtaggtcagcagctgagaagcccggcccctgggccgcggcggacggaggccgaagaggccagggagcggtgatttagagatgccgggacccgtcccggtagctttaacct

SEQ ID NO: 11681 - RNA, 8671 nt, Homo sapiens
  source 1..8671: mol_type = other RNA
ctgaatagctgggactacaggtgtgcaccaccacacccagctaattttttgtatttttagtagagagacggggtttcactgtgttagccaggatggtctcgatctcctgaccttgtgatctgcccgccctggcctcccaaagtgctgggattataggtgtgagccaccacacccggccgcataagcactttccaagcctctgcttgtatcatgtttgctattgttctagtggctgaagcaaaccacatagtcaaacctagaaggagagcaacaatccaagggcatggctacagaaaggctggcccagttggggtcattaatgggtatacctggctccagaactaaggcgctttaccatcataagctcccaatgtttaaacagtaagtctgcccgcactccttccagggtggaaaaactcagatactgataaattctcttgatcacagcccagtttttcccagcggattccccaccatccctcctatccccagacgctggagtctaggtttccagcccagtcaaaatctcaaggatctttcttttccctcaaactccaaaagaacagacacgcaataggatttctattcatttttattcattcctccaaagagcaccacaggccaaccacacccttgatgtgtccttcatggttccccactgcagtggacacaaatccctccatcattatccaggcatggatggaactctgctgtggtgaggaggttgtctcgcccactcacccaagttttccatgcctgttctgcttttgatggcaatgccaaaattcatcatacatttccttgaattcctgccttcaagggtcttccagccctgtggtgccatgcagacacacttcagtggcggccagtgatctgtctacaagggagtcttagtcttttctgcttggatgctcccagggacagatgcctgccaacaaccttatgtcttcacaaagactaaaatggaatcccattaaaagttatgatttaaaaggcgaccacccccaaaagaagtcataacactcaagggtgtcaatatatacaactgtgtaaacacaaccaatctacaactatatcaacacaaccagcactcctctatgggcacagacacacacacaaaattgtcttgctttctcagatatgatctctggcatgactcctgctggcatgagggcagaggaaattgagaggagcaaagcatatagcagtgatgtcagacaggaccaaatcagagacagggtcaaagtggcagaaaaatgaggagcacactccgagcaaaggcatgggggtgagacaaaggcacccagactagagccatcttggtgctgcccaggggtgggtggcactcatgtttgagctccatgtgtcaggcttttcaggaaagggtgtactatgttatgtgtctgtgtgcatattgtgtgcctgcatgtacatacatacgctgaattctcaccataaccatgtgaggtagatgccatttgtagagtgacttgcccaagtcagtggaaggactatctgcccctagagctagactgatagaattttctatgttgatggaagtattctgtaccttccctgtccaataccatagccactaatcacatgtggctactcagtattaatgttgcactactgccaatgaaacatagaattttaagttgtatttacttttaattgaacagctgaggccaggtgtggtggcccatgcctgtaataccagcactttgggaggccgaggtgggcggatcacctgaggtcagcagttcaagaccagcatgcccaacatggtgaaaccccgtctctgagaaaaataccaaaattagccaggcatggtggcatacacctgtagtcccagctactcaggaggatgatgcaagagaatcagttgaacctgggaggcagaggttgcagtgagctgaggtcatgccactgcactccagcctgggtgacaaagtgagactctgtctcaaaacaaaacaaaacaacccagcaacttggtcaacataaccagacctgcatctttacttaaaaaaaaaatggacacccatctcagtttttggaaaactattatataattggaacaacttggatatgtgaatctacttctccaactatgaattttatgaaatcaaaataaaggtcaagcatttcagataaaaatgtaccatggtaattgagatttggtgtaagtgtaaaatatataacagattttgaagacagcacaaaagaacgtaacataattcatttaaataataccgatgacgccaggcacggtgcctcacgcctgtaatcctagcactttgggaggccgaggtgggtggatcacctgaggtcaggagtttgagactagcctggccaacatggcgaaaccccatctctaaccaaaaatacaaaaattagtgggcatggtggcgggtgcctgtaatcccagctactcgggaggctgaggcaggagaatcacttgaacctggaaggtggaggttgcagtgagccgagattgtgccactgcactccagcctgggcaacaaagcgaagcactatctcaaaaaaaaaaaaaactaaaaaaccgatgacatgttgaaatgctattttggatacattgggttaagtaaaacatgttaaaatgaatttaacctgtttccttttacttgtctaatgtggctattagaaaacttggcttactcagcactttgggaggctgaggtgggcagataacttgaggccatgagttccagaccagcttagccaacatggtgaaaccccatctctactaaaaatacaaaaattaggacgggtgcagtggctcacgcctataatcccagcactttgggaggctgaggccggtggatcacctgaggtcaggagttcaagaccagcctggccaacacagtgaaaccccatctctactaaaaatacaaaaattagctgggcatgatggtgcatgcctgtaatcccagctacttgggaggctgaggttgcagtgagccaagatcgcacaactgcactccagcctgggtgacagagcaagactccgtctcccaaaaaataaataaataaataaaataaaaatacaaaaattagctgggcgcggtggctcatgcctgtaatcccagcactttgggaggccaaggcgggtggcctgaggtcagtagttccagaccagcctgatcaacatggtgaaaccccatctctactaaaaatacaaaaattagccaggcatggtggcatatgcctgtaatcccagctactcaggaggctgaggcaggagaatcacatgaacctgggaggcggaggttgcagtgaggcgagatcgtgccactgcactccagcctgggtgatggagtgaaactccatctcaaaaaaagaaaacttaaaatgacatatgtggcttgcatttcgtttctactggacagtgctgccctgcagccctcccattccatcacgtggctgacatgcctgattgcagggcttagacactaatatgatggggtaaagatatggatgaatattcttccccaaagctgaaagagctttcatgaaaatgcctggagccattcagtatagaactaagtgctcttccccatggtagctatctcaactttgaagggacaaattttgtcagcagtgggagtccaagctggagatgatggtaccatcccttgtctgcccttggatcagttacctttgtcttcagcttttaagggagacaggatctcaaaactaaggttcttatccagctcttttatttcacagatgggaaaataaggcactgtccaagtaacacacagtgacagtggcaaagtcgtgcttgcttcccaggtccctgacctcagacaagggtgttctctcccattaaatgcttttttctcctcatcttgctccattttcctatcttgtggcaagagattaacaatctaaattccaatcctagttctgacactgaccaatgaaataaacatttaggctgggtgtggtggctcacacctgtaatcccatcaaggcaggaggatcacttgaggccaggagttcaacactagtgtgggctacaaagcaagacccccgtctctacagaaaatttggtgctgtgtacctatagtcccagctactctgtaggcggaggtgggaggatcgtttgagcccaggagttggagatggcagtgagccatgatcatcccactgtattccagccggggcaacagagcaagaccctgtctctaaaataataataataataataaatatttacgaagcacctattgtgtcaggcacctattgttctagatgctggggaaacaacagagaacaggacaggcaacgggtcaaaagccaataaacaggtaaataaataagatcatttttgacagtaataattgctacaaggaaactcaactggccgaaatgaatagtgggggaatgtgagctacttcagatagggtggtcagggaggggaagtcctctctgaggggatacgtgagctgagatctgactgagcccgtcacaggaaggtttgagagtagaacaggaagttgtgagtagagccttgaaggaaagagaacagcaggtgcatgggtccccaggcaggactcaaggtagccactcaggcatcagaaagagtcaggcggccatgatggctcacacctgtaatcccagcactttgggagtctgagtcgggtggatcacctgaggtcaggagttcgagaccagcctgaccaacagggtgaaatcccttctctactaaactacaaaaattagccaggtgtggtggcacatgcctgtcatctcagctacagtcatcacatccctgtactccagactgggtgacaaggtgagactccatttcaaaaaaaaaaagaaggaaagtctatcaggctggacaggagtgggaaggggcagtgaatgagaataggcaagggccagacccacagggccttactgtgtgctgttgggcctcaagcctgccctctctggactttgctctttctgtctacgacaaaagggattctatcgcttggattctcagatcctccttttctgtttttgacactgaagaattctgtaacctgcaacttttcccccacatgtggctagcagcctagaacattccaggcactgtggtttctgcctttgcttcattcactcctggcatattcccatggtctcaagtgcctgaccacccatttggtgggcccctggctcaatgcagcaccctctatgtacatcagaaagcagagcctcttggggatacccgaggtgtccatacagaagtgtttggaccagtgcagcagtacagctgctcttctgaaaaggaaggtgcacaaaacaccaaggccataaagggttatggttaaataccaggagaaaaaggccaaaaaaagatagaaactcctaaagaaaagagacagagaaacagactccccagagatcacctgaattgctcagcacctagaagatgaaggcagtcatatcccttcccagtcacactcacagaggcagttgccgggatcccaatacaaggtttggaggagctgtctctgaggtatgctttactgcccttccacacccaaaagacctcattcctggtccctggctactcccagagcccaccatgcccagacctcttacccacctcacctcatttttgtgggaccaccctccctacatgcttttggagggcaattatagaaacccatccactccccaggagagatcaagaagtctccagctttctcgcacaagcccccgatccctcctccagatgcagacctccccttacccaatatttaggaaccaaggtccacagccatcttagaaccccggaagtctcagaccccaggggcctccgccaccccatcaagattcaaagcccactgctccttggggacctgtgtgcaggctttttctcccagagaaatgtagaccctgtttccctctgaggctctgaagcccaagagttccagctccctggggcgctcaggtctccctcccctatactggagttcaggtcccagtcatggacacctccccaccaattaggaaacaggacttctaccagcctccctggaggactaaacatccagtaactccagtttctactccctaggagacaaagacatagtccctgctagagtctgggccaccaactcccttcaggacagaagggtctagatgtcattcaccatggttcccaaaggtatcaggattcctggccaggggcggtggctcacgcctgtaatcctagcactttgggaggccggagcgggtcgatcgcctgaggtcaggagttcgaggccagcctggccaacatggtgaaaccccgtctctactaaaaatacaaaaattagccaggtgtggtggcaggcacctgtaatcccagctactccggacgctgaggcaggagaatcgcttgaacccgggaggcggaggttgcagtgagccgaggtcgcgccattgcactccagcctgggcaacaagagacttcgtctcacaaaaaaaagaaaaaaaaaaaaaaaaatcaggattcctgtcccccagactctctgaatccaggtgataagaagtcacacatcccagctggaagtcaagagtccacatccccttcaagcacccaggattaagcccaggcatcccctgtcagagtctggactcccaagccccctcccactcctcactgggcaggctcagggggtgccagcacagcctcagcatcagcccgcatctcatcgagagcctgcagcaggacgccgtgagccgctcggtagcccaggccacctgtcgccgctgcaccacccgcaggccacaggaaggagagagcccccagtgctgcgcccccagcagtgccctcgcccgcccaggcgcccagtcttgcttccacctcggcgcgcgtcaccgggcctgggaaatgagcgcgcgctgccagctctccagaagccaggcccagggcacgctcacgtcgagccagtgccgtgggttccagccccaggccccgtcgccactccgccagctgaccccgcagaagtgccacgtcgcatgcccagcccagccctgggagtggtgccgccgccgccgccagactagccagcagagctggcctccacgccccggctcgcaacgccgcagccttggttcgggcagcgctgggagatgctggtggcaacgccagcagcagtgcccctgcctgggctggggggagcgctcgccgcagccattcgcatagccctgggagtccgccaggccgtagggggaacactggcggcggcgcctcctccagcacctcccacgtctcgtcctccgggcttaacgcagcggcccgctctgagtcgccaccacctgatttcttcatgccgacaacctgctgcaaaccctcgctgccagctttcccaggaccttccccgctgcctgctttctgcgatccagcgctacatttctcccttcccttactgagtgcattctccaatccccctccacctgcgttctttaagctctcgcccttgggattctccatcttgccttctcccagacactccggatcctcgccctcgccgtctgtgcgcacgcagacaagaggcgcatctggtagcagcaaggcctggacctgggcccagtccttctcagtgggggccccaggggtgacgaggatgagggcgtcgtagtgcgttgggtgagaggcggcggccgcggtggtggcagtgcccgtgtggcccagaggcacggtccagagcaccacattcgggcgctctggggctgggaagggagtgggtgctgtggggaccgaagcaggcgcagcgcctgggtcgccaggatccaatccaagcagcatgtccaccacaaggcccacgtcagccttgccagccacggccaggtctagccgtgcgctgcccaggcgctccaggcctgagcgcacccacgacagcgcagcctcaaggccgccggtctcaaaggcctcacgcacagcctctagctctgctgcacccaacacctcgaagccatcctgcgccggtggcaggagcctccgcagcgcttctgcctggctctgcagcgccgcccggaggcgctctagctcctcgcagccgtcgctgctgccgcagttcgccggtagcacaaacagatccgcagctcctaaccccgcgctgttcagcagagctgctgtctgatcacgggcctgggcggcagtctgtgaatccccaggacggaggttccgcacagccagtagcggggtccctcgggccagggcggccagcgctgcctctcccagggctggagccaacggttccccgttcccctcgggtccgggcagcaccagtaccagcacgttggcttccgccgcccagggccccggcgctgcgggtgggcagctcagctcgcccagaaaaaggcctgggcccgcagctcttaggctgggaaccccggagtccggccgtccctcgggggcctcgagcgtctccacatccttgtcgcacagcgctgcgatcagcgcggacttccccaagcccggaggccccaggaacaaggcggtcacgtcaccctgcggcggaggcatgggggagagagcgcagtcggtggcagtaggtcagcagctgagaagcccggcccctgggccgcggcggacggaggccgaagaggccagggagcggtgatttagagatgccgggacccgtcccggtagctttaacct

SEQ ID NO: 11682 - RNA, 889 nt, Homo sapiens
  source 1..889: mol_type = other RNA
ctgaatagctgggactacaggtgtgcaccaccacacccttctgattttttgtagtgatggagggttatcactatgttgcccaggctattctcaaactcctgggctcaagcgaccctcctgcctgggcctcccaaaacgctgggattacgggtgtgagcctctgtgcctggcccatttttagcactcttcaaatggtctctggcatctggaggatgtgaaatagctgctagttgttataatgatgatcatcaatgtcatagttacagcatccttatttcttactccacgaaaaagatttattgtcatctctattttggaggtgacaaaactgaagctcacagaggtcaattgcatgcccaaagccacatggagagcggatcagagatggctttcaataccagagctctcttttagtgccgagcaatttctgaaactttattttcctctgtacgtccaggacacacaacacttgggctgtctcttcccagtgatccgattcccaggcccttgggctctgtcagttccaattcccagcatgctcagaggctctgtccttcgataatgagttctctgtcaattaccagctcctgcccagcagcctccggggcagtgtgggccaattgtcctgtcaggctgggggctgagcagagcgtctcaacttgggcagctactcagtggtcaatcacaatctcttagctggagatggtttctcatcagcccaggatcctagtaacggcacagagctggagctgtctgtggtcacaaaacacttgtcacagctatgatcctatttggtcctgagagtaagtcttcaaagtagcggttatttttatctcagacaatgatctaggccccaggagcccagcagcaatgaaatggtttccaccct

SEQ ID NO: 11683 - RNA, 2419 nt, Homo sapiens
  source 1..2419: mol_type = other RNA
ctgaatagctgggactacaggtgtgcaccaccacatccagctaatttttgtattttgggtagagacagggctttgccatgttggccaggctggtctcgaagtcctgacctcaagtgatctgcacaccttagcctcccaaagtgctgggattacaggcaagagccaccgcgcccagccaaagactcaatttcttgcttgatatagtggagcaacacaaaggaatcttccagctggttaccatccttctcaggatttcttttattttgggcttgcagtagctcaacctctatttccccctgcccctttgaaagttgatttctcctcagaggccctttccaagccagccttggactggctttcttggctttgcttggctattgtgtggtttcaactgagcagactgatatatgatttggatctgtctccctgcccaaatctcatgttgaatttaatccccagtgttggaggaggtgcctggtgggaggtgattggatcatgggggtggatttcctccttgctgttctcatgatagtgagttctcacgagatttggttgtttaaaagtgcatagcacctcccacttctttctttctcctgctccagactcgtaggacaggtctgcttctcttttgccttctgccttgattgtaagtttcctgaggcctccccagtcatgcttcctgtacagcctggggaaccatgagccaattaaacctcttttctttataaattacccagactcgaggctgggcctggtggctcacgcctgtaatcctaaccctttgagaggccaatgtgactggatggcctgagctcaggagctggagaccagcctgggcaacgtggtgaaaccccatctctactaaaatataaaaacttagccaggtgtagtgtgtgcctgtagtcccagctacttgggaggctgaggctggagaattgcttgaacccaggaggtggaggttgcagtgagccatgatcgcaccactgtactccagcctggagacagagcaagactctatctccaaaataaataaataaataaataaataaataaataaaattacccagtctcaggtagttctctgtacacacagacagtaacttttcccacctatttttccaaaaactgctcctgttctcagtcagtcctttcccaaactggagcctccctatagcccaacctgcaaaaattagggactcacttggaagtttattggtggaagtagagaagcaccttgttggaaacaccatcttacctctcccaaggtcacttggctcacagtggaaaaggagcattataagaggtggtagcaagtacacgtatgcaaggaagagcatgttttgcctaggtgtcaggctcccaagaagtgctctcctaggtaactggctatatgaacttgtagaaggtgctcattccagtcctcttgttcccagaggctgtggctcaaggcagctctcatgggtatattcaaattgattggagatgccactggagagggtatcttgtagctgctgcagttgtctatttcaatggcagtgtcattgttcctgtctgctgtgagctggggctttcctgagagctgtgagaaactgccactggtctgctcagccgccagcagcacgaggggctcgctgggctggggggatgacaggaggctgttttcaggtgttgtttctgtggagttggtgggcatcttgggcaccaggcagtgagtgaatttgattctcgggtctttggtggtgatggacaggcctttctgcagaattttcaccaagcggacccagaattgaaacacaatctctgggtgtttttcgtggagcttcagatagtagatcttttcggtcactgtcctaaccctcaggatgcgctggagccggtcgtagattcgtagctccacgtacttcagggggagaagcctgctgaggttgatgactggggcgtcaccaggtgtgctccaggtggtaaatggaccctggggccaggtaacattggccatcaggaggacattggggagtggcagggagggcaccgaggaggtgaccccgaggatcacggtggcagacccttcacagacatctctccagttcccgggcttagtgaccaaaatctcagcagtctctcaaagaatggcttaagacccttctggaaagccttcttcaactggataaagttgctttcaaacaccaccgagttggagaacaaattgaattctggagaatgaatcagttgacaaagaaggccattttccaccccaagttccactccagggcctggttccctgacctcaggtgggaggcccctgattttactcattggttcttggtaagaatgggcttgggaacatttctggggctccacgccgacccagcccaatgccaggatgttgatgtgatctgcccccacctccccagcatttcct

SEQ ID NO: 11684 - RNA, 2446 nt, Homo sapiens
  source 1..2446: mol_type = other RNA
ctgaatagctgggactacaggtgtgcaccaccacatccagctaatttttgtattttgggtagagacagggctttgccatgttggccaggctggtctcgaagtcctgacctcaagtgatctgcacaccttagcctcccaaagtgctgggattacaggcaagagccaccgcgcccagccaaagactcaatttcttgcttgatatagtggagcaacacaaaggaatcttccagctggttaccatccttctcaggatttcttttattttgggcttgcagtagctcaacctctatttccccctgcccctttgaaagttgatttctcctcagaggccctttccaagccagccttggactggctttcttggctttgcttggctattgtgtggtttcaactgagcagactgatatatgatttggatctgtctccctgcccaaatctcatgttgaatttaatccccagtgttggaggaggtgcctggtgggaggtgattggatcatgggggtggatttcctccttgctgttctcatgatagtgagttctcacgagatttggttgtttaaaagtgcatagcacctcccacttctttctttctcctgctccagactcgtaggacaggtctgcttctcttttgccttctgccttgattgtaagtttcctgaggcctccccagtcatgcttcctgtacagcctggggaaccatgagccaattaaacctcttttctttataaattacccagactcgaggctgggcctggtggctcacgcctgtaatcctaaccctttgagaggccaatgtgactggatggcctgagctcaggagctggagaccagcctgggcaacgtggtgaaaccccatctctactaaaatataaaaacttagccaggtgtagtgtgtgcctgtagtcccagctacttgggaggctgaggctggagaattgcttgaacccaggaggtggaggttgcagtgagccatgatcgcaccactgtactccagcctggagacagagcaagactctatctccaaaataaataaataaataaataaataaataaataaaattacccagtctcaggtagttctctgtacacacagacagtaacttttcccacctatttttccaaaaactgctcctgttctcagtcagtcctttcccaaactggagcctccctatagcccaacctgcaaaaattagggactcacttggaagtttattggtggaagtagagaagcaccttgttggaaacaccatcttacctctcccaaggtcacttggctcacagtggaaaaggagcattataagaggtggtagcaagtacacgtatgcaaggaagagcatgttttgcctaggtgtcaggctcccaagaagtgctctcctaggtaactggctatatgaacttgtagaaggtgctcattccagtcctcttgttcccagaggctgtggctcaaggcagctctcatgggtatattcaaattgattggagatgccactggagagggtatcttgtagctgctgcagttgtctatttcaatggcagtgtcattgttcctgtctgctgtgagctggggctttcctgagagctgtgagaaactgccactggtctgctcagccgccagcagcacgaggggctcgctgggctggggggatgacaggaggctgttttcaggtgttgtttctgtggagttggtgggcatcttgggcaccaggcagtgagtgaatttgattctcgggtctttggtggtgatggacaggcctttctgcagaattttcaccaagcggacccagaattgaaacacaatctctgggtgtttttcgtggagcttcagatagtagatcttttcggtcactgtcctaaccctcaggatgcgctggagccggtcgtagattcgtagctccacgtacttcagggggagaagcctgctgaggttgatgactggggcgtcaccaggtgtgctccaggtggtaaatggaccctggggccaggtaacattggccatcaggaggacattggggagtggcagggagggcaccgaggaggtgaccccgaggatcacggtggcagacccttcacagacatctctccagttcccgggcttagtgacctggaaatcagcctcaggtacatgggtcaaaatctcagcagtctctcaaagaatggcttaagacccttctggaaagccttcttcaactggataaagttgctttcaaacaccaccgagttggagaacaaattgaattctggagaatgaatcagttgacaaagaaggccattttccaccccaagttccactccagggcctggttccctgacctcaggtgggaggcccctgattttactcattggttcttggtaagaatgggcttgggaacatttctggggctccacgccgacccagcccaatgccaggatgttgatgtgatctgcccccacctccccagcatttcct

SEQ ID NO: 11685 - RNA, 2387 nt, Homo sapiens
  source 1..2387: mol_type = other RNA
ctgaatagctgggactacaggtgtgcaccaccacatccagctaatttttgtattttgggtagagacagggctttgccatgttggccaggctggtctcgaagtcctgacctcaagtgatctgcacaccttagcctcccaaagtgctgggattacaggcaagagccaccgcgcccagccaaagactcaatttcttgcttgatatagtggagcaacacaaaggaatcttccagctggttaccatccttctcaggatttcttttattttgggcttgcagtagctcaacctctatttccccctgcccctttgaaagttgatttctcctcagaggccctttccaagccagccttggactggctttcttggctttgcttggctattgtgtggtttcaactgagcagactgatatatgatttggatctgtctccctgcccaaatctcatgttgaatttaatccccagtgttggaggaggtgcctggtgggaggtgattggatcatgggggtggatttcctccttgctgttctcatgatagtgagttctcacgagatttggttgtttaaaagtgcatagcacctcccacttctttctttctcctgctccagactcgtaggacaggtctgcttctcttttgccttctgccttgattgtaagtttcctgaggcctccccagtcatgcttcctgtacagcctggggaaccatgagccaattaaacctcttttctttataaattacccagactcgaggctgggcctggtggctcacgcctgtaatcctaaccctttgagaggccaatgtgactggatggcctgagctcaggagctggagaccagcctgggcaacgtggtgaaaccccatctctactaaaatataaaaacttagccaggtgtagtgtgtgcctgtagtcccagctacttgggaggctgaggctggagaattgcttgaacccaggaggtggaggttgcagtgagccatgatcgcaccactgtactccagcctggagacagagcaagactctatctccaaaataaataaataaataaataaataaataaataaaattacccagtctcaggtagttctctgtacacacagacagtaacttttcccacctatttttccaaaaactgctcctgttctcagtcagtcctttcccaaactggagcctccctatagcccaacctgcaaaaattagggactcacttggaagtttattggtggaagtagagaagcaccttgttggaaacaccatcttacctctcccaaggtcacttggctcacagtggaaaaggagcattataagaggtggtagcaagtacacgtatgcaaggaagagcatgttttgcctaggtgtcaggctcccaagaagtgctctcctaggtaactggctatatgaacttgtagaaggtgctcattccagtcctcttgttcccagaggctgtggctcaaggcagctctcatgggtatattcaaattgattggagatgccactggagagggtatcttgtagctgctgcagttgtctatttcaatggcagtgtcattgttcctgtctgctgtgagctggggctttcctgagagctgtgagaaactgccactggtctgctcagccgccagcagcacgaggggctcgctgggctggggggatgacaggaggctgttttcaggtgttgtttctgtggagttggtgggcatcttgggcaccaggcagtgagtgaatttgattctcgggtctttggtggtgatggacaggcctttctgcagaattttcaccaagcggacccagaattgaaacacaatctctgggtgtttttcgtggagcttcagatagtagatcttttcggtcactgtcctaaccctcaggatgcgctggagccggtcgtagattcgtagctccacgtacttcagggggagaagcctgctgaggttgatgactggggcgtcaccaggtgtgctccaggtggtaaatggaccctggggccaggtaacattggccatcaggaggacattggggagtggcagggagggcaccgaggaggtgaccccgaggatcacggtggcagacccttcacagacatctctccagttcccgggcttagtgacctggaaatcagcctcaggtacatgggtctggataaagttgctttcaaacaccaccgagttggagaacaaattgaattctggagaatgaatcagttgacaaagaaggccattttccaccccaagttccactccagggcctggttccctgacctcaggtgggaggcccctgattttactcattggttcttggtaagaatgggcttgggaacatttctggggctccacgccgacccagcccaatgccaggatgttgatgtgatctgcccccacctccccagcatttcct

SEQ ID NO: 11686 - RNA, 2360 nt, Homo sapiens
  source 1..2360: mol_type = other RNA
ctgaatagctgggactacaggtgtgcaccaccacatccagctaatttttgtattttgggtagagacagggctttgccatgttggccaggctggtctcgaagtcctgacctcaagtgatctgcacaccttagcctcccaaagtgctgggattacaggcaagagccaccgcgcccagccaaagactcaatttcttgcttgatatagtggagcaacacaaaggaatcttccagctggttaccatccttctcaggatttcttttattttgggcttgcagtagctcaacctctatttccccctgcccctttgaaagttgatttctcctcagaggccctttccaagccagccttggactggctttcttggctttgcttggctattgtgtggtttcaactgagcagactgatatatgatttggatctgtctccctgcccaaatctcatgttgaatttaatccccagtgttggaggaggtgcctggtgggaggtgattggatcatgggggtggatttcctccttgctgttctcatgatagtgagttctcacgagatttggttgtttaaaagtgcatagcacctcccacttctttctttctcctgctccagactcgtaggacaggtctgcttctcttttgccttctgccttgattgtaagtttcctgaggcctccccagtcatgcttcctgtacagcctggggaaccatgagccaattaaacctcttttctttataaattacccagactcgaggctgggcctggtggctcacgcctgtaatcctaaccctttgagaggccaatgtgactggatggcctgagctcaggagctggagaccagcctgggcaacgtggtgaaaccccatctctactaaaatataaaaacttagccaggtgtagtgtgtgcctgtagtcccagctacttgggaggctgaggctggagaattgcttgaacccaggaggtggaggttgcagtgagccatgatcgcaccactgtactccagcctggagacagagcaagactctatctccaaaataaataaataaataaataaataaataaataaaattacccagtctcaggtagttctctgtacacacagacagtaacttttcccacctatttttccaaaaactgctcctgttctcagtcagtcctttcccaaactggagcctccctatagcccaacctgcaaaaattagggactcacttggaagtttattggtggaagtagagaagcaccttgttggaaacaccatcttacctctcccaaggtcacttggctcacagtggaaaaggagcattataagaggtggtagcaagtacacgtatgcaaggaagagcatgttttgcctaggtgtcaggctcccaagaagtgctctcctaggtaactggctatatgaacttgtagaaggtgctcattccagtcctcttgttcccagaggctgtggctcaaggcagctctcatgggtatattcaaattgattggagatgccactggagagggtatcttgtagctgctgcagttgtctatttcaatggcagtgtcattgttcctgtctgctgtgagctggggctttcctgagagctgtgagaaactgccactggtctgctcagccgccagcagcacgaggggctcgctgggctggggggatgacaggaggctgttttcaggtgttgtttctgtggagttggtgggcatcttgggcaccaggcagtgagtgaatttgattctcgggtctttggtggtgatggacaggcctttctgcagaattttcaccaagcggacccagaattgaaacacaatctctgggtgtttttcgtggagcttcagatagtagatcttttcggtcactgtcctaaccctcaggatgcgctggagccggtcgtagattcgtagctccacgtacttcagggggagaagcctgctgaggttgatgactggggcgtcaccaggtgtgctccaggtggtaaatggaccctggggccaggtaacattggccatcaggaggacattggggagtggcagggagggcaccgaggaggtgaccccgaggatcacggtggcagacccttcacagacatctctccagttcccgggcttagtgacctggataaagttgctttcaaacaccaccgagttggagaacaaattgaattctggagaatgaatcagttgacaaagaaggccattttccaccccaagttccactccagggcctggttccctgacctcaggtgggaggcccctgattttactcattggttcttggtaagaatgggcttgggaacatttctggggctccacgccgacccagcccaatgccaggatgttgatgtgatctgcccccacctccccagcatttcct

SEQ ID NO: 11687 - RNA, 2441 nt, Homo sapiens
  source 1..2441: mol_type = other RNA
ctgaatagctgggactacaggtgtgcaccaccacgcccagctaatttttgtatttttttgtaaagatagggtttcattatgttgcccaggctggtctcaaactcctgggctcaagcgatccacccacctcgatttcccaaagtgctgagattataggcctgagccaccatgcctggctgcagatccttcataggtttcttaatcttaagaacaaaaagctcacctggaaagcaagaacacatcaatttggcagtatctggtcactaaaagaactgtatctctggaggcaagcatgggctctaataaaccccacaaagtattgccgtctaattcccaaatattcctgactgtctctttccacagagctaaggagggttcaattcaaagaacattaaagtccctttggcttgcatagcagacgagaaaccagactcttcttgccaagcatgcctcaggcccacaaatacccatggaaataggtatatatttctgagtaaaaagccaccatccatgtcagaaaagatttgaatctacctcagctgtctttcttctcttagatctgtctgcctcatactttgtggatgactactttggaaaagtgaaactcaggtaagacactaagctctctaagcctcaattttctcacaggtaaaatggggatagtgtatttacctcagagagtcattgtgagacaacacatgtaaagcactgagcctagtatatagaacacatttaatgagcagaaactagttgctgagtgcttctacgtagacagaagtagagaaacgagcagattcatgagaggagaaaaaagaaacaaatatatagtgcatgtggacaggaactacacagaggatttctaaaagctgcctccaagaccaattcaggtcctagagggaaaaatgtacaacattgagttctgagaaggctgggcagatacatcacagacaatgcatggtttggaggcatgaaactaaacaaatgccttcccaatactctacatccacagggatacaaatgcagtgtcatctgtgggcagtcttcctgttaacttgacacaagatcagccctccatctgcaggtgtcaaagctcccttaataattagttcctgagtcaaatataatactgacaaaaacattgtagatctttcatcttttgggggaatttttagtcataaatttaggattccactgtttctttaaagcaaagccactagtagctgagggtgatggtgtgtgcctgcttcattacagacggtatgacacatcttgagataaaaactaggatggctttcttatctgggttcctgactgctccttagctttgagttcttctagcttcttctcatagcgactcataaagtaatcatctggttcaatctctgcattcttcaagttttccatgatcttttccagtctgagcactgatcgggctccttcaatctttcttgtactcaagtacaaggtgaactcctggaaatccaggagcttacaggtgtccacagagcagatattccggatatcactagttctatccaaatgaggaaaaaacaccagtcctgacaacttctctaggtcctggaggctcacttggaattcagttaactggggctggaagccgatggcttcattgggtaccacaaaggcccctagcgccagtggttcggtagatactgagcttctgcgggccaggattaccttataaaggtgtgaggggactgccacgttgtcctcgccaatcactaggtatctcctccactataatgcatgctccatgagggtactcttttctgccttgtttaatgctgtatcagaagcacccagaacagcaccaggtacctagtaaaagcttagttaagtctctggtaactaactattttctttccatcgcctctagtctgaggtaaggtcaaaggcccagataccacccaaacatcttcaaacctttctgtcagctctcgacagtacatttctattctgttccaatatccagaattattatcaaaatcctgaggcacaatgttagaaaggtaaaaggtttcagccatggctttacttgaaaatttgttatttcctgctggagccatgtgtcctcgtgaccacccacttccaacataatcttcattgaaggcactgaaggttggagggatattgggatcaggcttaaatttacaatgctttctgtctgcatcacctctgttccagttaaagggaatccaaattgttccaagacagccttttctgcagatccatccggctgcttccctgtcaacgctccctcagcgccctgactccggaagaactgcagggccgcgagcccagctcccgcagcgcccactacagccccagccacgaagccgctcagaaaacgacgggaaccccggaggcgggaagcgatactcttgatagccatcttgcccgaggtaccggccttttaccac

SEQ ID NO: 11688 - RNA, 2529 nt, Homo sapiens
  source 1..2529: mol_type = other RNA
ctgaatagctgggactacaggtgtgcaccaccacgcccagctaatttttgtatttttttgtaaagatagggtttcattatgttgcccaggctggtctcaaactcctgggctcaagcgatccacccacctcgatttcccaaagtgctgagattataggcctgagccaccatgcctggctgcagatccttcataggtttcttaatcttaagaacaaaaagctcacctggaaagcaagaacacatcaatttggcagtatctggtcactaaaagaactgtatctctggaggcaagcatgggctctaataaaccccacaaagtattgccgtctaattcccaaatattcctgactgtctctttccacagagctaaggagggttcaattcaaagaacattaaagtccctttggcttgcatagcagacgagaaaccagactcttcttgccaagcatgcctcaggcccacaaatacccatggaaataggtatatatttctgagtaaaaagccaccatccatgtcagaaaagatttgaatctacctcagctgtctttcttctcttagatctgtctgcctcatactttgtggatgactactttggaaaagtgaaactcaggtaagacactaagctctctaagcctcaattttctcacaggtaaaatggggatagtgtatttacctcagagagtcattgtgagacaacacatgtaaagcactgagcctagtatatagaacacatttaatgagcagaaactagttgctgagtgcttctacgtagacagaagtagagaaacgagcagattcatgagaggagaaaaaagaaacaaatatatagtgcatgtggacaggaactacacagaggatttctaaaagctgcctccaagaccaattcaggtcctagagggaaaaatgtacaacattgagttctgagaaggctgggcagatacatcacagacaatgcatggtttggaggcatgaaactaaacaaatgccttcccaatactctacatccacagggatacaaatgcagtgtcatctgtgggcagtcttcctgttaacttgacacaagatcagccctccatctgcaggtgtcaaagctcccttaataattagttcctgagtcaaatataatactgacaaaaacattgtagatctttcatcttttgggggaatttttagtcataaatttaggattccactgtttctttaaagcaaagccactagtagctgagggtgatggtgtgtgcctgtagtcccagctgctcagggggcagaggcaggaggattgcttaagcccagaagtttgaggctatagtgagctatgattccaccactgcactccagcctggatgacacggcgagaccacatctcttaaagagaaaaactttttaaaaagcaaaaagcaaagccactaaaatatgttagcctaaagagggcatgcctgcttcattacagacggtatgacacatcttgagataaaaactaggatggctttcttatctgggttcctgactgctccttagctttgagttcttctagcttcttctcatagcgactcataaagtaatcatctggttcaatctctgcattcttcaagttttccatgatcttttccagtctgagcactgatcgggctccttcaatctttcttgtactcaagtacaaggtgaactcctggaaatccaggagcttacaggtgtccacagagcagatattccggatatcactagttctatccaaatgaggaaaaaacaccagtcctgacaacttctctaggtcctggaggctcacttggaattcagttaactggggctggaagccgatggcttcattgggtaccacaaaggcccctagcgccagtggttcggtagatactgagcttctgcgggccaggattaccttataaaggtgtgaggggactgccacgttgtcctcgccaatcacctggtaactaactattttctttccatcgcctctagtctgaggtaaggtcaaaggcccagataccacccaaacatcttcaaacctttctgtcagctctcgacagtacatttctattctgttccaatatccagaattattatcaaaatcctgaggcacaatgttagaaaggtaaaaggtttcagccatggctttacttgaaaatttgttatttcctgctggagccatgtgtcctcgtgaccacccacttccaacataatcttcattgaaggcactgaaggttggagggatattgggatcaggcttaaatttacaatgctttctgtctgcatcaccataggtgaaggttgagagagagaagaaacaatgatgctaggagtgtaaacttgaagaatctacccattatcttgcttttggaaatatgttcaagaacccatctaggcacccgctttgcctgatcataagacaaagcgtgattagtgtaacaccttgcctctgttccagttaaagggaatccaaattgttccaagacagccttttctgcagatccatccggctgcttccctgtcaacgctccctcagcgccctgactcc

SEQ ID NO: 11689 - RNA, 2975 nt, Homo sapiens
  source 1..2975: mol_type = other RNA
ctgaatagctgggactacaggtgtgcaccaccacgcccagctaatttttgtatttttttgtaaagatagggtttcattatgttgcccaggctggtctcaaactcctgggctcaagcgatccacccacctcgatttcccaaagtgctgagattataggcctgagccaccatgcctggctgcagatccttcataggtttcttaatcttaagaacaaaaagctcacctggaaagcaagaacacatcaatttggcagtatctggtcactaaaagaactgtatctctggaggcaagcatgggctctaataaaccccacaaagtattgccgtctaattcccaaatattcctgactgtctctttccacagagctaaggagggttcaattcaaagaacattaaagtccctttggcttgcatagcagacgagaaaccagactcttcttgccaagcatgcctcaggcccacaaatacccatggaaataggtatatatttctgagtaaaaagccaccatccatgtcagaaaagatttgaatctacctcagctgtctttcttctcttagatctgtctgcctcatactttgtggatgactactttggaaaagtgaaactcaggtaagacactaagctctctaagcctcaattttctcacaggtaaaatggggatagtgtatttacctcagagagtcattgtgagacaacacatgtaaagcactgagcctagtatatagaacacatttaatgagcagaaactagttgctgagtgcttctacgtagacagaagtagagaaacgagcagattcatgagaggagaaaaaagaaacaaatatatagtgcatgtggacaggaactacacagaggatttctaaaagctgcctccaagaccaattcaggtcctagagggaaaaatgtacaacattgagttctgagaaggctgggcagatacatcacagacaatgcatggtttggaggcatgaaactaaacaaatgccttcccaatactctacatccacagggatacaaatgcagtgtcatctgtgggcagtcttcctgttaacttgacacaagatcagccctccatctgcaggtgtcaaagctcccttaataattagttcctgagtcaaatataatactgacaaaaacattgtagatctttcatcttttgggggaatttttagtcataaatttaggattccactgtttctttaaagcaaagccactagtagctgagggtgatggtgtgtgcctgtagtcccagctgctcagggggcagaggcaggaggattgcttaagcccagaagtttgaggctatagtgagctatgattccaccactgcactccagcctggatgacacggcgagaccacatctcttaaagagaaaaactttttaaaaagcaaaaagcaaagccactaaaatatgttagcctaaagagggcatgcctgcttcattacagacggtatgacacatcttgagataaaaactaggatggctttcttatctgggttcctgactgctccttagctttgagttcttctagcttcttctcatagcgactcataaagtaatcatctggttcaatctctgcattcttcaagttttccatgatcttttccagtctgagcactgatcgggctccttcaatctttcttgtactcaagtacaaggtgaactcctggaaatccaggagcttacaggtgtccacagagcagatattccggatatcactagttctatccaaatgaggaaaaaacaccagtcctgacaacttctctaggtcctggaggctcacttggaattcagttaactggggctggaagccgatggcttcattgggtaccacaaaggcccctagcgccagtggttcggtagatactgagcttctgcgggccaggattaccttataaaggtgtgaggggactgccacgttgtcctcgccaatcacctggtaactaactattttctttccatcgcctctagtctgaggtaaggtcaaaggcccagataccacccaaacatcttcaaacctttctgtcagctctcgacagtacatttctattctgttccaatatccagaattattatcaaaatcctgaggcacaatgttagaaaggtaaaaggtttcagccatggctttacttgaaaatttgttatttcctgctggagccatgtgtcctcgtgaccacccacttccaacataatcttcattgaaggcactgaaggttggagggatattgggatcaggcttaaatttacaatgctttctgtctgcatcaccataggtgaaggttgagagagagaagaaacaatgatgctaggagtgtaaacttgaagaatctacccattatcttgcttttggaaatatgttcaagaacccatctaggcacccgctttgcctgatcataagacaaagcgtgattagtgtaacaccttgcctctgttccagttaaagggaatccaaattgttccaagacagccttttctgcagatctgaatgccaattatgtaccaggtactgtgctggttagatgatggagaccaaaacagacatagtctcaagtcttatggagctaacaatcatccggctgcttccctgtcaacgctccctcagcgccctgactccggaagaactgcagggccgcgagcccagctcccgcagcgcccactacagccccagccacgaagccgctcagaaaacgacgggaaccccggaggcgggaagcgatactcttgatagccatcttgcccgaggtaccggccttttaccacggcgcatgcgcgcgcatgccggcccccgccatccccccgtcaccccacgcctcaccgcccgccaagctgagggcctcgcacgccccctggtgacaaaccgggatgcctagcgcatccccgcttcatccctggtccactggacggggcgatggatggggaatatgatgtctagagggcttagtggtatgctatatatagtcatgagaagaaaat

SEQ ID NO: 11690 - RNA, 2581 nt, Homo sapiens
  source 1..2581: mol_type = other RNA
ctgaatagctgggactacaggtgtgcaccaccacgcccagctaatttttgtatttttttgtaaagatagggtttcattatgttgcccaggctggtctcaaactcctgggctcaagcgatccacccacctcgatttcccaaagtgctgagattataggcctgagccaccatgcctggctgcagatccttcataggtttcttaatcttaagaacaaaaagctcacctggaaagcaagaacacatcaatttggcagtatctggtcactaaaagaactgtatctctggaggcaagcatgggctctaataaaccccacaaagtattgccgtctaattcccaaatattcctgactgtctctttccacagagctaaggagggttcaattcaaagaacattaaagtccctttggcttgcatagcagacgagaaaccagactcttcttgccaagcatgcctcaggcccacaaatacccatggaaataggtatatatttctgagtaaaaagccaccatccatgtcagaaaagatttgaatctacctcagctgtctttcttctcttagatctgtctgcctcatactttgtggatgactactttggaaaagtgaaactcaggtaagacactaagctctctaagcctcaattttctcacaggtaaaatggggatagtgtatttacctcagagagtcattgtgagacaacacatgtaaagcactgagcctagtatatagaacacatttaatgagcagaaactagttgctgagtgcttctacgtagacagaagtagagaaacgagcagattcatgagaggagaaaaaagaaacaaatatatagtgcatgtggacaggaactacacagaggatttctaaaagctgcctccaagaccaattcaggtcctagagggaaaaatgtacaacattgagttctgagaaggctgggcagatacatcacagacaatgcatggtttggaggcatgaaactaaacaaatgccttcccaatactctacatccacagggatacaaatgcagtgtcatctgtgggcagtcttcctgttaacttgacacaagatcagccctccatctgcaggtgtcaaagctcccttaataattagttcctgagtcaaatataatactgacaaaaacattgtagatctttcatcttttgggggaatttttagtcataaatttaggattccactgtttctttaaagcaaagccactagtagctgagggtgatggtgtgtgcctgtagtcccagctgctcagggggcagaggcaggaggattgcttaagcccagaagtttgaggctatagtgagctatgattccaccactgcactccagcctggatgacacggcgagaccacatctcttaaagagaaaaactttttaaaaagcaaaaagcaaagccactaaaatatgttagcctaaagagggcatgcctgcttcattacagacggtatgacacatcttgagataaaaactaggatggctttcttatctgggttcctgactgctccttagctttgagttcttctagcttcttctcatagcgactcataaagtaatcatctggttcaatctctgcattcttcaagttttccatgatcttttccagtctgagcactgatcgggctccttcaatctttcttgtactcaagtacaaggtgaactcctggaaatccaggagcttacaggtgtccacagagcagatattccggatatcactagttctatccaaatgaggaaaaaacaccagtcctgacaacttctctaggtcctggaggctcacttggaattcagttaactggggctggaagccgatggcttcattgggtaccacaaaggcccctagcgccagtggttcggtagatactgagcttctgcgggccaggattaccttataaaggtgtgaggggactgccacgttgtcctcgccaatcacctggtaactaactattttctttccatcgcctctagtctgaggtaaggtcaaaggcccagataccacccaaacatcttcaaacctttctgtcagctctcgacagtacatttctattctgttccaatatccagaattattatcaaaatcctgaggcacaatgttagaaaggtaaaaggtttcagccatggctttacttgaaaatttgttatttcctgctggagccatgtgtcctcgtgaccacccacttccaacataatcttcattgaaggcactgaaggttggagggatattgggatcaggcttaaatttacaatgctttctgtctgcatcaccataggtgaaggttgagagagagaagaaacaatgatgctaggagtgtaaacttgaagaatctacctctgttccagttaaagggaatccaaattgttccaagacagccttttctgcagatccatccggctgcttccctgtcaacgctccctcagcgccctgactccggaagaactgcagggccgcgagcccagctcccgcagcgcccactacagccccagccacgaagccgctcagaaaacgacgggaaccccggaggcgggaagcgatactcttgatagccatcttgcccgaggtaccggccttttaccac

SEQ ID NO: 11691 - RNA, 2730 nt, Homo sapiens
  source 1..2730: mol_type = other RNA
ctgaatagctgggactacaggtgtgcaccaccacgcccagctaatttttgtatttttttgtaaagatagggtttcattatgttgcccaggctggtctcaaactcctgggctcaagcgatccacccacctcgatttcccaaagtgctgagattataggcctgagccaccatgcctggctgcagatccttcataggtttcttaatcttaagaacaaaaagctcacctggaaagcaagaacacatcaatttggcagtatctggtcactaaaagaactgtatctctggaggcaagcatgggctctaataaaccccacaaagtattgccgtctaattcccaaatattcctgactgtctctttccacagagctaaggagggttcaattcaaagaacattaaagtccctttggcttgcatagcagacgagaaaccagactcttcttgccaagcatgcctcaggcccacaaatacccatggaaataggtatatatttctgagtaaaaagccaccatccatgtcagaaaagatttgaatctacctcagctgtctttcttctcttagatctgtctgcctcatactttgtggatgactactttggaaaagtgaaactcaggtaagacactaagctctctaagcctcaattttctcacaggtaaaatggggatagtgtatttacctcagagagtcattgtgagacaacacatgtaaagcactgagcctagtatatagaacacatttaatgagcagaaactagttgctgagtgcttctacgtagacagaagtagagaaacgagcagattcatgagaggagaaaaaagaaacaaatatatagtgcatgtggacaggaactacacagaggatttctaaaagctgcctccaagaccaattcaggtcctagagggaaaaatgtacaacattgagttctgagaaggctgggcagatacatcacagacaatgcatggtttggaggcatgaaactaaacaaatgccttcccaatactctacatccacagggatacaaatgcagtgtcatctgtgggcagtcttcctgttaacttgacacaagatcagccctccatctgcaggtgtcaaagctcccttaataattagttcctgagtcaaatataatactgacaaaaacattgtagatctttcatcttttgggggaatttttagtcataaatttaggattccactgtttctttaaagcaaagccactagtagctgagggtgatggtgtgtgcctgtagtcccagctgctcagggggcagaggcaggaggattgcttaagcccagaagtttgaggctatagtgagctatgattccaccactgcactccagcctggatgacacggcgagaccacatctcttaaagagaaaaactttttaaaaagcaaaaagcaaagccactaaaatatgttagcctaaagagggcatgcctgcttcattacagacggtatgacacatcttgagataaaaactaggatggctttcttatctgggttcctgactgctccttagctttgagttcttctagcttcttctcatagcgactcataaagtaatcatctggttcaatctctgcattcttcaagttttccatgatcttttccagtctgagcactgatcgggctccttcaatctttcttgtactcaagtacaaggtgaactcctggaaatccaggagcttacaggtgtccacagagcagatattccggatatcactagttctatccaaatgaggaaaaaacaccagtcctgacaacttctctaggtcctggaggctcacttggaattcagttaactggggctggaagccgatggcttcattgggtaccacaaaggcccctagcgccagtggttcggtagatactgagcttctgcgggccaggattaccttataaaggtgtgaggggactgccacgttgtcctcgccaatcacctggtaactaactattttctttccatcgcctctagtctgaggtaaggtcaaaggcccagataccacccaaacatcttcaaacctttctgtcagctctcgacagtacatttctattctgttccaatatccagaattattatcaaaatcctgaggcacaatgttagaaaggtaaaaggtttcagccatggctttacttgaaaatttgttatttcctgctggagccatgtgtcctcgtgaccacccacttccaacataatcttcattgaaggcactgaaggttggagggatattgggatcaggcttaaatttacaatgctttctgtctgcatcaccataggtgaaggttgagagagagaagaaacaatgatgctaggagtgtaaacttgaagaatctacctgcttacttctccagcatcatttcacatcaccttccccctcattcatctactggcactcttttagttccccattatcttgcttttggaaatatgttcaagaacccatctaggcacccgctttgcctgatcataagacaaagcgtgattagtgtaacaccttgcctctgttccagttaaagggaatccaaattgttccaagacagccttttctgcagatccatccggctgcttccctgtcaacgctccctcagcgccctgactccggaagaactgcagggccgcgagcccagctcccgcagcgcccactacagccccagccacgaagccgctcagaaaacgacgggaaccccggaggcgggaagcgatactcttgatagccatcttgcccgaggta

SEQ ID NO: 11692 - RNA, 3273 nt, Homo sapiens
  source 1..3273: mol_type = other RNA
ctgaatagctgggactacaggtgtgcaccaccacgcccagctaatttttgtatttttttgtaaagatagggtttcattatgttgcccaggctggtctcaaactcctgggctcaagcgatccacccacctcgatttcccaaagtgctgagattataggcctgagccaccatgcctggctgcagatccttcataggtttcttaatcttaagaacaaaaagctcacctggaaagcaagaacacatcaatttggcagtatctggtcactaaaagaactgtatctctggaggcaagcatgggctctaataaaccccacaaagtattgccgtctaattcccaaatattcctgactgtctctttccacagagctaaggagggttcaattcaaagaacattaaagtccctttggcttgcatagcagacgagaaaccagactcttcttgccaagcatgcctcaggcccacaaatacccatggaaataggtatatatttctgagtaaaaagccaccatccatgtcagaaaagatttgaatctacctcagctgtctttcttctcttagatctgtctgcctcatactttgtggatgactactttggaaaagtgaaactcaggtaagacactaagctctctaagcctcaattttctcacaggtaaaatggggatagtgtatttacctcagagagtcattgtgagacaacacatgtaaagcactgagcctagtatatagaacacatttaatgagcagaaactagttgctgagtgcttctacgtagacagaagtagagaaacgagcagattcatgagaggagaaaaaagaaacaaatatatagtgcatgtggacaggaactacacagaggatttctaaaagctgcctccaagaccaattcaggtcctagagggaaaaatgtacaacattgagttctgagaaggctgggcagatacatcacagacaatgcatggtttggaggcatgaaactaaacaaatgccttcccaatactctacatccacagggatacaaatgcagtgtcatctgtgggcagtcttcctgttaacttgacacaagatcagccctccatctgcaggtgtcaaagctcccttaataattagttcctgagtcaaatataatactgacaaaaacattgtagatctttcatcttttgggggaatttttagtcataaatttaggattccactgtttctttaaagcaaagccactagtagctgagggtgatggtgtgtgcctgtagtcccagctgctcagggggcagaggcaggaggattgcttaagcccagaagtttgaggctatagtgagctatgattccaccactgcactccagcctggatgacacggcgagaccacatctcttaaagagaaaaactttttaaaaagcaaaaagcaaagccactaaaatatgttagcctaaagagggcatgcctgcttcattacagacggtatgacacatcttgagataaaaactaggatggctttcttatctgggttcctgactgctccttagctttgagttcttctagcttcttctcatagcgactcataaagtaatcatctggttcaatctctgcattcttcaagttttccatgatcttttccagtctgagcactgatcgggctccttcaatctttcttgtactcaagtacaaggtgaactcctggaaatccaggagcttacaggtgtccacagagcagatattccggatatcactagttctatccaaatgaggaaaaaacaccagtcctgacaacttctctaggtcctggaggctcacttggaattcagttaactggggctggaagccgatggcttcattgggtaccacaaaggcccctagcgccagtggttcggtagatactgagcttctgcgggccaggattaccttataaaggtgtgaggggactgccacgttgtcctcgccaatcacctggtaactaactattttctttccatcgcctctagtctgaggtaaggtcaaaggcccagataccacccaaacatcttcaaacctttctgtcagctctcgacagtacatttctattctgttccaatatccagaattattatcaaaatcctgaggcacaatgttagaaaggtaaaaggtttcagccatggctttacttgaaaatttgttatttcctgctggagccatgtgtcctcgtgaccacccacttccaacataatcttcattgaaggcactgaaggttggagggatattgggatcaggcttaaatttacaatgctttctgtctgcatcaccataggtgaaggttgagagagagaagaaacaatgatgctaggagtgtaaacttgaagaatctacctgcttacttctccagcatcatttcacatcaccttccccctcattcatctactggcactcttttagttccctaaaagaacaaaactcctgtccacattgggggcctccgaagatgcaaatgttcctttcttcctagaatgctcttctccatatcccatggcacattcaaccccttgcctaagtaatttccgttcactcttcagtccacttttccagagaagccttactaatcaaaatcaggttcttgtgttataatctctcatcacacttttttttttttttgagacacattctccctctgttgcctaagctggagtgtggtgctgcgatcttggctcactgcaacccccacctcctgggctcaagagatcctcccatctcagtcccccaagtagctggaaccacagaggtgcaccaccacgcccagctaatttttgtattttttgtagaaacgcggttttgccatgttggccaggctcatctcaaactcctgagctcaaacgcctcagcctcccaaagtactgggattacaggtgtgagccaccacgcccagcctctcatcaaactttttactgttccttaattatactacactaacttgcaatcacctcctttggaaaaattattgtaattatacatctaaaattatttgtttgatgggtcaacccactctcccaactcaaagtgtcactggggtagagatcctctactctggtcacacataggtccccaagggttaccacagtgccagacacatagcaggcacataaatatttgttaaggtaaaactgaatggtgctcattgctgtaatatttatgacagagcctcccaactagtgtgtcaagatatgggtattttcagccctgagacagctggaaagggtctggctttctggctgccaggcagggttgatttaaccagtaagttatataaatata

SEQ ID NO: 11693 - RNA, 2641 nt, Homo sapiens
  source 1..2641: mol_type = other RNA
ctgaatagctgggactacaggtgtgcaccaccacgcccagctaatttttgtatttttttgtaaagatagggtttcattatgttgcccaggctggtctcaaactcctgggctcaagcgatccacccacctcgatttcccaaagtgctgagattataggcctgagccaccatgcctggctgcagatccttcataggtttcttaatcttaagaacaaaaagctcacctggaaagcaagaacacatcaatttggcagtatctggtcactaaaagaactgtatctctggaggcaagcatgggctctaataaaccccacaaagtattgccgtctaattcccaaatattcctgactgtctctttccacagagctaaggagggttcaattcaaagaacattaaagtccctttggcttgcatagcagacgagaaaccagactcttcttgccaagcatgcctcaggcccacaaatacccatggaaataggtatatatttctgagtaaaaagccaccatccatgtcagaaaagatttgaatctacctcagctgtctttcttctcttagatctgtctgcctcatactttgtggatgactactttggaaaagtgaaactcaggtaagacactaagctctctaagcctcaattttctcacaggtaaaatggggatagtgtatttacctcagagagtcattgtgagacaacacatgtaaagcactgagcctagtatatagaacacatttaatgagcagaaactagttgctgagtgcttctacgtagacagaagtagagaaacgagcagattcatgagaggagaaaaaagaaacaaatatatagtgcatgtggacaggaactacacagaggatttctaaaagctgcctccaagaccaattcaggtcctagagggaaaaatgtacaacattgagttctgagaaggctgggcagatacatcacagacaatgcatggtttggaggcatgaaactaaacaaatgccttcccaatactctacatccacagggatacaaatgcagtgtcatctgtgggcagtcttcctgttaacttgacacaagatcagccctccatctgcaggtgtcaaagctcccttaataattagttcctgagtcaaatataatactgacaaaaacattgtagatctttcatcttttgggggaatttttagtcataaatttaggattccactgtttctttaaagcaaagccactagtagctgagggtgatggtgtgtgcctgtagtcccagctgctcagggggcagaggcaggaggattgcttaagcccagaagtttgaggctatagtgagctatgattccaccactgcactccagcctggatgacacggcgagaccacatctcttaaagagaaaaactttttaaaaagcaaaaagcaaagccactaaaatatgttagcctaaagagggcatgcctgcttcattacagacggtatgacacatcttgagataaaaactaggatggctttcttatctgggttcctgactgctccttagctttgagttcttctagcttcttctcatagcgactcataaagtaatcatctggttcaatctctgcattcttcaagttttccatgatcttttccagtctgagcactgatcgggctccttcaatctttcttgtactcaagtacaaggtgaactcctggaaatccaggagcttacaggtgtccacagagcagatattccggatatcactagttctatccaaatgaggaaaaaacaccagtcctgacaacttctctaggtcctggaggctcacttggaattcagttaactggggctggaagccgatggcttcattgggtaccacaaaggcccctagcgccagtggttcggtagatactgagcttctgcgggccaggattaccttataaaggtgtgaggggactgccacgttgtcctcgccaatcacctggtaactaactattttctttccatcgcctctagtctgaggtaaggtcaaaggcccagataccacccaaacatcttcaaacctttctgtcagctctcgacagtacatttctattctgttccaatatccagaattattatcaaaatcctgaggcacaatgttagaaaggtaaaaggtttcagccatggctttacttgaaaatttgttatttcctgctggagccatgtgtcctcgtgaccacccacttccaacataatcttcattgaaggcactgaaggttggagggatattgggatcaggcttaaatttacaatgctttctgtctgcatcaccataggtgaaggttgagagagagaagaaacaatgatgctaggagtgtaaacttgaagaatctacctgcttacttctccagcatcatttcacatcaccttccccctcattcatctactggcactcttttagttcccttgcctctgttccagttaaagggaatccaaattgttccaagacagccttttctgcagatccatccggctgcttccctgtcaacgctccctcagcgccctgactccggaagaactgcagggccgcgagcccagctcccgcagcgcccactacagccccagccacgaagccgctcagaaaacgacgggaaccccggaggcgggaagcgatactcttgatagccatcttgcccgaggta

SEQ ID NO: 11694 - RNA, 2461 nt, Homo sapiens
  source 1..2461: mol_type = other RNA
ctgaatagctgggactacaggtgtgcaccaccacgcccagctaatttttgtatttttttgtaaagatagggtttcattatgttgcccaggctggtctcaaactcctgggctcaagcgatccacccacctcgatttcccaaagtgctgagattataggcctgagccaccatgcctggctgcagatccttcataggtttcttaatcttaagaacaaaaagctcacctggaaagcaagaacacatcaatttggcagtatctggtcactaaaagaactgtatctctggaggcaagcatgggctctaataaaccccacaaagtattgccgtctaattcccaaatattcctgactgtctctttccacagagctaaggagggttcaattcaaagaacattaaagtccctttggcttgcatagcagacgagaaaccagactcttcttgccaagcatgcctcaggcccacaaatacccatggaaataggtatatatttctgagtaaaaagccaccatccatgtcagaaaagatttgaatctacctcagctgtctttcttctcttagatctgtctgcctcatactttgtggatgactactttggaaaagtgaaactcaggtaagacactaagctctctaagcctcaattttctcacaggtaaaatggggatagtgtatttacctcagagagtcattgtgagacaacacatgtaaagcactgagcctagtatatagaacacatttaatgagcagaaactagttgctgagtgcttctacgtagacagaagtagagaaacgagcagattcatgagaggagaaaaaagaaacaaatatatagtgcatgtggacaggaactacacagaggatttctaaaagctgcctccaagaccaattcaggtcctagagggaaaaatgtacaacattgagttctgagaaggctgggcagatacatcacagacaatgcatggtttggaggcatgaaactaaacaaatgccttcccaatactctacatccacagggatacaaatgcagtgtcatctgtgggcagtcttcctgttaacttgacacaagatcagccctccatctgcaggtgtcaaagctcccttaataattagttcctgagtcaaatataatactgacaaaaacattgtagatctttcatcttttgggggaatttttagtcataaatttaggattccactgtttctttaaagcaaagccactagtagctgagggtgatggtgtgtgcctgtagtcccagctgctcagggggcagaggcaggaggattgcttaagcccagaagtttgaggctatagtgagctatgattccaccactgcactccagcctggatgacacggcgagaccacatctcttaaagagaaaaactttttaaaaagcaaaaagcaaagccactaaaatatgttagcctaaagagggcatgcctgcttcattacagacggtatgacacatcttgagataaaaactaggatggctttcttatctgggttcctgactgctccttagctttgagttcttctagcttcttctcatagcgactcataaagtaatcatctggttcaatctctgcattcttcaagttttccatgatcttttccagtctgagcactgatcgggctccttcaatctttcttgtactcaagtacaaggtgaactcctggaaatccaggagcttacaggtgtccacagagcagatattccggatatcactagttctatccaaatgaggaaaaaacaccagtcctgacaacttctctaggtcctggaggctcacttggaattcagttaactggggctggaagccgatggcttcattgggtaccacaaaggcccctagcgccagtggttcggtagatactgagcttctgcgggccaggattaccttataaaggtgtgaggggactgccacgttgtcctcgccaatcacctggtaactaactattttctttccatcgcctctagtctgaggtaaggtcaaaggcccagataccacccaaacatcttcaaacctttctgtcagctctcgacagtacatttctattctgttccaatatccagaattattatcaaaatcctgaggcacaatgttagaaaggtaaaaggtttcagccatggctttacttgaaaatttgttatttcctgctggagccatgtgtcctcgtgaccacccacttccaacataatcttcattgaaggcactgaaggttggagggatattgggatcaggcttaaatttacaatgctttctgtctgcatcaccatccggctgcttccctgtcaacgctccctcagcgccctgactccggaagaactgcagggccgcgagcccagctcccgcagcgcccactacagccccagccacgaagccgctcagaaaacgacgggaaccccggaggcgggaagcgatactcttgatagccatcttgcccgaggtaccggccttttaccac

SEQ ID NO: 11695 - RNA, 2611 nt, Homo sapiens
  source 1..2611: mol_type = other RNA
ctgaatagctgggactacaggtgtgcaccaccacgcccagctaatttttgtatttttttgtaaagatagggtttcattatgttgcccaggctggtctcaaactcctgggctcaagcgatccacccacctcgatttcccaaagtgctgagattataggcctgagccaccatgcctggctgcagatccttcataggtttcttaatcttaagaacaaaaagctcacctggaaagcaagaacacatcaatttggcagtatctggtcactaaaagaactgtatctctggaggcaagcatgggctctaataaaccccacaaagtattgccgtctaattcccaaatattcctgactgtctctttccacagagctaaggagggttcaattcaaagaacattaaagtccctttggcttgcatagcagacgagaaaccagactcttcttgccaagcatgcctcaggcccacaaatacccatggaaataggtatatatttctgagtaaaaagccaccatccatgtcagaaaagatttgaatctacctcagctgtctttcttctcttagatctgtctgcctcatactttgtggatgactactttggaaaagtgaaactcaggtaagacactaagctctctaagcctcaattttctcacaggtaaaatggggatagtgtatttacctcagagagtcattgtgagacaacacatgtaaagcactgagcctagtatatagaacacatttaatgagcagaaactagttgctgagtgcttctacgtagacagaagtagagaaacgagcagattcatgagaggagaaaaaagaaacaaatatatagtgcatgtggacaggaactacacagaggatttctaaaagctgcctccaagaccaattcaggtcctagagggaaaaatgtacaacattgagttctgagaaggctgggcagatacatcacagacaatgcatggtttggaggcatgaaactaaacaaatgccttcccaatactctacatccacagggatacaaatgcagtgtcatctgtgggcagtcttcctgttaacttgacacaagatcagccctccatctgcaggtgtcaaagctcccttaataattagttcctgagtcaaatataatactgacaaaaacattgtagatctttcatcttttgggggaatttttagtcataaatttaggattccactgtttctttaaagcaaagccactagtagctgagggtgatggtgtgtgcctgtagtcccagctgctcagggggcagaggcaggaggattgcttaagcccagaagtttgaggctatagtgagctatgattccaccactgcactccagcctggatgacacggcgagaccacatctcttaaagagaaaaactttttaaaaagcaaaaagcaaagccactaaaatatgttagcctaaagagggcatgcctgcttcattacagacggtatgacacatcttgagataaaaactaggatggctttcttatctgggttcctgactgctccttagctttgagttcttctagcttcttctcatagcgactcataaagtaatcatctggttcaatctctgcattcttcaagttttccatgatcttttccagtctgagcactgatcgggctccttcaatctttcttgtactcaagtacaaggtgaactcctggaaatccaggagcttacaggtgtccacagagcagatattccggatatcactagttctatccaaatgaggaaaaaacaccagtcctgacaacttctctaggtcctggaggctcacttggaattcagttaactggggctggaagccgatggcttcattgggtaccacaaaggcccctagcgccagtggttcggtagatactgagcttctgcgggccaggattaccttataaaggtgtgaggggactgccacgttgtcctcgccaatcacctggtaactaactattttctttccatcgcctctagtctgaggtaaggtcaaaggcccagataccacccaaacatcttcaaacctttctgtcagctctcgacagtacatttctattctgttccaatatccagaattattatcaaaatcctgaggcacaatgttagaaaggtaaaaggtttcagccatggctttacttgaaaatttgttatttcctgctggagccatgtgtcctcgtgaccacccacttccaacataatcttcattgaaggcactgaaggttggagggatattgggatcaggcttaaatttacaatgctttctgtctgcatcacccattatcttgcttttggaaatatgttcaagaacccatctaggcacccgctttgcctgatcataagacaaagcgtgattagtgtaacaccttgcctctgttccagttaaagggaatccaaattgttccaagacagccttttctgcagatccatccggctgcttccctgtcaacgctccctcagcgccctgactccggaagaactgcagggccgcgagcccagctcccgcagcgcccactacagccccagccacgaagccgctcagaaaacgacgggaaccccggaggcgggaagcgatactcttgatagccatcttgcccgaggtaccggccttttaccac

SEQ ID NO: 11696 - RNA, 2911 nt, Homo sapiens
  source 1..2911: mol_type = other RNA
ctgaatagctgggactacaggtgtgcaccaccacgcccagctaatttttgtatttttttgtaaagatagggtttcattatgttgcccaggctggtctcaaactcctgggctcaagcgatccacccacctcgatttcccaaagtgctgagattataggcctgagccaccatgcctggctgcagatccttcataggtttcttaatcttaagaacaaaaagctcacctggaaagcaagaacacatcaatttggcagtatctggtcactaaaagaactgtatctctggaggcaagcatgggctctaataaaccccacaaagtattgccgtctaattcccaaatattcctgactgtctctttccacagagctaaggagggttcaattcaaagaacattaaagtccctttggcttgcatagcagacgagaaaccagactcttcttgccaagcatgcctcaggcccacaaatacccatggaaataggtatatatttctgagtaaaaagccaccatccatgtcagaaaagatttgaatctacctcagctgtctttcttctcttagatctgtctgcctcatactttgtggatgactactttggaaaagtgaaactcaggtaagacactaagctctctaagcctcaattttctcacaggtaaaatggggatagtgtatttacctcagagagtcattgtgagacaacacatgtaaagcactgagcctagtatatagaacacatttaatgagcagaaactagttgctgagtgcttctacgtagacagaagtagagaaacgagcagattcatgagaggagaaaaaagaaacaaatatatagtgcatgtggacaggaactacacagaggatttctaaaagctgcctccaagaccaattcaggtcctagagggaaaaatgtacaacattgagttctgagaaggctgggcagatacatcacagacaatgcatggtttggaggcatgaaactaaacaaatgccttcccaatactctacatccacagggatacaaatgcagtgtcatctgtgggcagtcttcctgttaacttgacacaagatcagccctccatctgcaggtgtcaaagctcccttaataattagttcctgagtcaaatataatactgacaaaaacattgtagatctttcatcttttgggggaatttttagtcataaatttaggattccactgtttctttaaagcaaagccactagtagctgagggtgatggtgtgtgcctgtagtcccagctgctcagggggcagaggcaggaggattgcttaagcccagaagtttgaggctatagtgagctatgattccaccactgcactccagcctggatgacacggcgagaccacatctcttaaagagaaaaactttttaaaaagcaaaaagcaaagccactaaaatatgttagcctaaagagggcatgcctgcttcattacagacggtatgacacatcttgagataaaaactaggatggctttcttatctgggttcctgactgctccttagctttgagttcttctagcttcttctcatagcgactcataaagtaatcatctggttcaatctctgcattcttcaagttttccatgatcttttccagtctgagcactgatcgggctccttcaatctttcttgtactcaagtacaaggtgaactcctggaaatccaggagcttacaggtgtccacagagcagatattccggatatcactagttctatccaaatgaggaaaaaacaccagtcctgacaacttctctaggtcctggaggctcacttggaattcagttaactggggctggaagccgatggcttcattgggtaccacaaaggcccctagcgccagtggttcggtagatactgagcttctgcgggccaggattaccttataaaggtgtgaggggactgccacgttgtcctcgccaatcacctggtaactaactattttctttccatcgcctctagtctgaggtaaggtcaaaggcccagataccacccaaacatcttcaaacctttctgtcagctctcgacagtacatttctattctgttccaatatccagaattattatcaaaatcctgaggcacaatgttagaaaggtaaaaggtttcagccatggctttacttgaaaatttgttatttcctgctggagccatgtgtcctcgtgaccacccacttccaacataatcttcattgaaggcactgaaggttggagggatattgggatcaggcttaaatttacaatgctttctgtctgcatcacccattatcttgcttttggaaatatgttcaagaacccatctaggcacccgctttgcctgatcataagacaaagcgtgattagtgtaacaccttgcctctgttccagttaaagggaatccaaattgttccaagacagccttttctgcagatctgaatgccaattatgtaccaggtactgtgctggttagatgatggagaccaaaacagacatagtctcaagtcttatggagctaacaatcatccggctgcttccctgtcaacgctccctcagcgccctgactccggaagaactgcagggccgcgagcccagctcccgcagcgcccactacagccccagccacgaagccgctcagaaaacgacgggaaccccggaggcgggaagcgatactcttgatagccatcttgcccgaggtaccggccttttaccacggcgcatgcgcgcgcatgccggcccccgccatccccccgtcaccccacgcctcaccgcccgccaagctgagggcctcgcacgccccctggtgacaaaccgggatgcctagcgcatccccgcttcatccctggtccactggacggggcgatggatggggaatatgatgtctagagggcttagtggtatgctatatatagtcatgagaagaaaat

SEQ ID NO: 11697 - RNA, 2517 nt, Homo sapiens
  source 1..2517: mol_type = other RNA
ctgaatagctgggactacaggtgtgcaccaccacgcccagctaatttttgtatttttttgtaaagatagggtttcattatgttgcccaggctggtctcaaactcctgggctcaagcgatccacccacctcgatttcccaaagtgctgagattataggcctgagccaccatgcctggctgcagatccttcataggtttcttaatcttaagaacaaaaagctcacctggaaagcaagaacacatcaatttggcagtatctggtcactaaaagaactgtatctctggaggcaagcatgggctctaataaaccccacaaagtattgccgtctaattcccaaatattcctgactgtctctttccacagagctaaggagggttcaattcaaagaacattaaagtccctttggcttgcatagcagacgagaaaccagactcttcttgccaagcatgcctcaggcccacaaatacccatggaaataggtatatatttctgagtaaaaagccaccatccatgtcagaaaagatttgaatctacctcagctgtctttcttctcttagatctgtctgcctcatactttgtggatgactactttggaaaagtgaaactcaggtaagacactaagctctctaagcctcaattttctcacaggtaaaatggggatagtgtatttacctcagagagtcattgtgagacaacacatgtaaagcactgagcctagtatatagaacacatttaatgagcagaaactagttgctgagtgcttctacgtagacagaagtagagaaacgagcagattcatgagaggagaaaaaagaaacaaatatatagtgcatgtggacaggaactacacagaggatttctaaaagctgcctccaagaccaattcaggtcctagagggaaaaatgtacaacattgagttctgagaaggctgggcagatacatcacagacaatgcatggtttggaggcatgaaactaaacaaatgccttcccaatactctacatccacagggatacaaatgcagtgtcatctgtgggcagtcttcctgttaacttgacacaagatcagccctccatctgcaggtgtcaaagctcccttaataattagttcctgagtcaaatataatactgacaaaaacattgtagatctttcatcttttgggggaatttttagtcataaatttaggattccactgtttctttaaagcaaagccactagtagctgagggtgatggtgtgtgcctgtagtcccagctgctcagggggcagaggcaggaggattgcttaagcccagaagtttgaggctatagtgagctatgattccaccactgcactccagcctggatgacacggcgagaccacatctcttaaagagaaaaactttttaaaaagcaaaaagcaaagccactaaaatatgttagcctaaagagggcatgcctgcttcattacagacggtatgacacatcttgagataaaaactaggatggctttcttatctgggttcctgactgctccttagctttgagttcttctagcttcttctcatagcgactcataaagtaatcatctggttcaatctctgcattcttcaagttttccatgatcttttccagtctgagcactgatcgggctccttcaatctttcttgtactcaagtacaaggtgaactcctggaaatccaggagcttacaggtgtccacagagcagatattccggatatcactagttctatccaaatgaggaaaaaacaccagtcctgacaacttctctaggtcctggaggctcacttggaattcagttaactggggctggaagccgatggcttcattgggtaccacaaaggcccctagcgccagtggttcggtagatactgagcttctgcgggccaggattaccttataaaggtgtgaggggactgccacgttgtcctcgccaatcacctggtaactaactattttctttccatcgcctctagtctgaggtaaggtcaaaggcccagataccacccaaacatcttcaaacctttctgtcagctctcgacagtacatttctattctgttccaatatccagaattattatcaaaatcctgaggcacaatgttagaaaggtaaaaggtttcagccatggctttacttgaaaatttgttatttcctgctggagccatgtgtcctcgtgaccacccacttccaacataatcttcattgaaggcactgaaggttggagggatattgggatcaggcttaaatttacaatgctttctgtctgcatcacctctgttccagttaaagggaatccaaattgttccaagacagccttttctgcagatccatccggctgcttccctgtcaacgctccctcagcgccctgactccggaagaactgcagggccgcgagcccagctcccgcagcgcccactacagccccagccacgaagccgctcagaaaacgacgggaaccccggaggcgggaagcgatactcttgatagccatcttgcccgaggtaccggccttttaccac

SEQ ID NO: 11698 - RNA, 4627 nt, Homo sapiens
  source 1..4627: mol_type = other RNA
ctgaatagctgggactacaggtgtgcaccaccacgcccagctaatttttgtatttttttgtaaagatagggtttcattatgttgcccaggctggtctcaaactcctgggctcaagcgatccacccacctcgatttcccaaagtgctgagattataggcctgagccaccatgcctggctgcagatccttcataggtttcttaatcttaagaacaaaaagctcacctggaaagcaagaacacatcaatttggcagtatctggtcactaaaagaactgtatctctggaggcaagcatgggctctaataaaccccacaaagtattgccgtctaattcccaaatattcctgactgtctctttccacagagctaaggagggttcaattcaaagaacattaaagtccctttggcttgcatagcagacgagaaaccagactcttcttgccaagcatgcctcaggcccacaaatacccatggaaataggtatatatttctgagtaaaaagccaccatccatgtcagaaaagatttgaatctacctcagctgtctttcttctcttagatctgtctgcctcatactttgtggatgactactttggaaaagtgaaactcaggtaagacactaagctctctaagcctcaattttctcacaggtaaaatggggatagtgtatttacctcagagagtcattgtgagacaacacatgtaaagcactgagcctagtatatagaacacatttaatgagcagaaactagttgctgagtgcttctacgtagacagaagtagagaaacgagcagattcatgagaggagaaaaaagaaacaaatatatagtgcatgtggacaggaactacacagaggatttctaaaagctgcctccaagaccaattcaggtcctagagggaaaaatgtacaacattgagttctgagaaggctgggcagatacatcacagacaatgcatggtttggaggcatgaaactaaacaaatgccttcccaatactctacatccacagggatacaaatgcagtgtcatctgtgggcagtcttcctgttaacttgacacaagatcagccctccatctgcaggtgtcaaagctcccttaataattagttcctgagtcaaatataatactgacaaaaacattgtagatctttcatcttttgggggaatttttagtcataaatttaggattccactgtttctttaaagcaaagccactagtagctgagggtgatggtgtgtgcctgtagtcccagctgctcagggggcagaggcaggaggattgcttaagcccagaagtttgaggctatagtgagctatgattccaccactgcactccagcctggatgacacggcgagaccacatctcttaaagagaaaaactttttaaaaagcaaaaagcaaagccactaaaatatgttagcctaaagagggcatgcctgcttcattacagacggtatgacacatcttgagataaaaactaggatggctttcttatctgggttcctgactgctccttagctttgagttcttctagcttcttctcatagcgactcataaagtaatcatctggttcaatctctgcattcttcaagttttccatgatcttttccagtctgagcactgatcgggctccttcaatctttcttgtactcaagtacaaggtgaactcctggaaatccaggagcttacaggtgtccacagagcagatattccggatatcactagttctatccaaatgaggaaaaaacaccagtcctgacaacttctctaggtcctggaggctcacttggaattcagttaactggggctggaagccgatggcttcattgggtaccacaaaggcccctagcgccagtggttcggtagatactgagcttctgcgggccaggattaccttataaaggtgtgaggggactgccacgttgtcctcgccaatcacctggtaactaactattttctttccatcgcctctagtctgaggtaaggtcaaaggcccagataccacccaaacatcttcaaacctttctgtcagctctcgacagtacatttctattctgttccaatatccagaattattatcaaaatcctgaggcacaatgttagaaaggtaaaaggtttcagccatggctttacttgaaaatttgttatttcctgctggagccatgtgtcctcgtgaccacccacttccaacataatcttcattgaaggcactgaaggttggagggatattgggatcaggcttaaatttacaatgctttctgtctgcatcacctgaagaaaaacacacaaaatggatatgttatcagtagacaaatgtccctcaagattctctaagcaaggcaagctggttgctactggctggtgtctctccaagcagctagtattagggattgcatgcatgtctcaagttcctgggatagttcagatacttcatctgaatttagaaagtactagtctaggaaagaatgcttttcatacagtgtagctatctcatataattttgactctggcctttccagttaaagaaaaactcctctgaatagtattttaagtaaaaacaatcaccaatcaaaacactaaactatataaaaagcttggctactaaataaactcttgttttttaaaaaagactcccatgtattgtattttgtacgattgtatttgacaagtttatgtgtactgaaataatggatatatatagacacaaaacaatttgttctaggcaagcacagccttggggagaggagtgtctctgatatcttgcttactgcctctcgaaccatgacaaaataaacatttaagttatgagctccacccagaaatttctaaaacagaatatctgggtaccacataggagagaagaaatctcagattttatttattttctgacacctccagaatggtttgtcacagagaacattagcaaatcctaacactacctattgcactatcgtgaggtgagactttcttaaactacaaaagttatgacaacaaatgaaacatactcagactgttattcaaagaagtgtaaaatggagaacaatgaagtcactgattccaaggtgatttcattcagccaagaaaaatttagtatcagatcccaaagtttacagtaaagtatcatatatgtagctttttagaatcactttataaagaataatacagaaaaatttatcattagtaaatttctaagtgtcattaccattggaatcacttccttctacagctagttatctttggctggtgcttactgccctggaaaagcaatttgtaggaatttccaaagacctaaaaagataccttccttgagaaaagatataaatttactgctgtaaggtgtctagcagtattcccagtggagaaccgtattaaaccatgctcagggattaaggttccctgatctcctctcgatgcacagatttgggctgtaagtctgcatgatagccagtttttgactttaccttctctggaacaaactttttatcttccttttgacctttctccgttcagtgccaagacaaccttccatgtagtcccataggtgaaggttgagagagagaagaaacaatgatgctaggagtgtaaacttgaagaatctacctagaaaccaatttgacattaattatcaagatctggcaattctacaggaccctatcaagacataaggacacatgaataaactgacacacctgcttacttctccagcatcatttcacatcaccttccccctcattcatctactggcactcttttagttccctaaaagaacaaaactcctgtccacattgggggcctccgaagatgcaaatgttcctttcttcctagaatgctcttctccatatcccatggcacattcaaccccttgcctaagtaatttccgttcactcttcagtccacttttccagagaagccttactaatcaaaatcaggttcttgtgttataatctctcatcacacttttttttttttttgagacacattctccctctgttgcctaagctggagtgtggtgctgcgatcttggctcactgcaacccccacctcctgggctcaagagatcctcccatctcagtcccccaagtagctggaaccacagaggtgcaccaccacgcccagctaatttttgtattttttgtagaaacgcggttttgccatgttggccaggctcatctcaaactcctgagctcaaacgcctcagcctcccaaagtactgggattacaggtgtgagccaccacgcccagcctctcatcaaactttttactgttccttaattatactacactaacttgcaatcacctcctttggaaaaattattgtaattatacatctaaaattatttgtttgatgggtcaacccactctcccaactcaaagtgtcactggggtagagatcctctactctggtcacacataggtccccaagggttaccacagtgccagacacatagcaggcacataaatatttgttaaggtaaaactgaatggtgctcattgctgtaatatttatgacagagcctcccaactagtgtgtcaagatatgggtattttcagccctgagacagctggaaagggtctggctttctggctgccaggcagggttgatttaaccagtaagttatataaatata

SEQ ID NO: 11699 - RNA, 4538 nt, Homo sapiens
  source 1..4538: mol_type = other RNA
ctgaatagctgggactacaggtgtgcaccaccacgcccagctaatttttgtatttttttgtaaagatagggtttcattatgttgcccaggctggtctcaaactcctgggctcaagcgatccacccacctcgatttcccaaagtgctgagattataggcctgagccaccatgcctggctgcagatccttcataggtttcttaatcttaagaacaaaaagctcacctggaaagcaagaacacatcaatttggcagtatctggtcactaaaagaactgtatctctggaggcaagcatgggctctaataaaccccacaaagtattgccgtctaattcccaaatattcctgactgtctctttccacagagctaaggagggttcaattcaaagaacattaaagtccctttggcttgcatagcagacgagaaaccagactcttcttgccaagcatgcctcaggcccacaaatacccatggaaataggtatatatttctgagtaaaaagccaccatccatgtcagaaaagatttgaatctacctcagctgtctttcttctcttagatctgtctgcctcatactttgtggatgactactttggaaaagtgaaactcaggtaagacactaagctctctaagcctcaattttctcacaggtaaaatggggatagtgtatttacctcagagagtcattgtgagacaacacatgtaaagcactgagcctagtatatagaacacatttaatgagcagaaactagttgctgagtgcttctacgtagacagaagtagagaaacgagcagattcatgagaggagaaaaaagaaacaaatatatagtgcatgtggacaggaactacacagaggatttctaaaagctgcctccaagaccaattcaggtcctagagggaaaaatgtacaacattgagttctgagaaggctgggcagatacatcacagacaatgcatggtttggaggcatgaaactaaacaaatgccttcccaatactctacatccacagggatacaaatgcagtgtcatctgtgggcagtcttcctgttaacttgacacaagatcagccctccatctgcaggtgtcaaagctcccttaataattagttcctgagtcaaatataatactgacaaaaacattgtagatctttcatcttttgggggaatttttagtcataaatttaggattccactgtttctttaaagcaaagccactagtagctgagggtgatggtgtgtgcctgtagtcccagctgctcagggggcagaggcaggaggattgcttaagcccagaagtttgaggctatagtgagctatgattccaccactgcactccagcctggatgacacggcgagaccacatctcttaaagagaaaaactttttaaaaagcaaaaagcaaagccactaaaatatgttagcctaaagagggcatgcctgcttcattacagacggtatgacacatcttgagataaaaactaggatggctttcttatctgggttcctgactgctccttagctttgagttcttctagcttcttctcatagcgactcataaagtaatcatctggttcaatctctgcattcttcaagttttccatgatcttttccagtctgagcactgatcgggctccttcaatctttcttgtactcaagtacaaggtgaactcctggaaatccaggagcttacaggtgtccacagagcagatattccggatatcactagttctatccaaatgaggaaaaaacaccagtcctgacaacttctctaggtcctggaggctcacttggaattcagttaactggggctggaagccgatggcttcattgggtaccacaaaggcccctagcgccagtggttcggtagatactgagcttctgcgggccaggattaccttataaaggtgtgaggggactgccacgttgtcctcgccaatcacctggtaactaactattttctttccatcgcctctagtctgaggtaaggtcaaaggcccagataccacccaaacatcttcaaacctttctgtcagctctcgacagtacatttctattctgttccaatatccagaattattatcaaaatcctgaggcacaatgttagaaaggtaaaaggtttcagccatggctttacttgaaaatttgttatttcctgctggagccatgtgtcctcgtgaccacccacttccaacataatcttcattgaaggcactgaaggttggagggatattgggatcaggcttaaatttacaatgctttctgtctgcatcacctgaagaaaaacacacaaaatggatatgttatcagtagacaaatgtccctcaagattctctaagcaaggcaagctggttgctactggctggtgtctctccaagcagctagtattagggattgcatgcatgtctcaagttcctgggatagttcagatacttcatctgaatttagaaagtactagtctaggaaagaatgcttttcatacagtgtagctatctcatataattttgactctggcctttccagttaaagaaaaactcctctgaatagtattttaagtaaaaacaatcaccaatcaaaacactaaactatataaaaagcttggctactaaataaactcttgttttttaaaaaagactcccatgtattgtattttgtacgattgtatttgacaagtttatgtgtactgaaataatggatatatatagacacaaaacaatttgttctaggcaagcacagccttggggagaggagtgtctctgatatcttgcttactgcctctcgaaccatgacaaaataaacatttaagttatgagctccacccagaaatttctaaaacagaatatctgggtaccacataggagagaagaaatctcagattttatttattttctgacacctccagaatggtttgtcacagagaacattagcaaatcctaacactacctattgcactatcgtgaggtgagactttcttaaactacaaaagttatgacaacaaatgaaacatactcagactgttattcaaagaagtgtaaaatggagaacaatgaagtcactgattccaaggtgatttcattcagccaagaaaaatttagtatcagatcccaaagtttacagtaaagtatcatatatgtagctttttagaatcactttataaagaataatacagaaaaatttatcattagtaaatttctaagtgtcattaccattggaatcacttccttctacagctagttatctttggctggtgcttactgccctggaaaagcaatttgtaggaatttccaaagacctaaaaagataccttccttgagaaaagatataaatttactgctgtaaggtgtctagcagtattcccagtggagaaccgtattaaaccatgctcagggattaaggttccctgatctcctctcgatgcacagatttgggctgtaagtctgcatgatagccagtttttgactttaccttctctggaacaaactttttatcttccttttgacctttctccgttcagtgccaagacaaccttccatgtagtcccataggtgaaggttgagagagagaagaaacaatgatgctaggagtgtaaacttgaagaatctacctgcttacttctccagcatcatttcacatcaccttccccctcattcatctactggcactcttttagttccctaaaagaacaaaactcctgtccacattgggggcctccgaagatgcaaatgttcctttcttcctagaatgctcttctccatatcccatggcacattcaaccccttgcctaagtaatttccgttcactcttcagtccacttttccagagaagccttactaatcaaaatcaggttcttgtgttataatctctcatcacacttttttttttttttgagacacattctccctctgttgcctaagctggagtgtggtgctgcgatcttggctcactgcaacccccacctcctgggctcaagagatcctcccatctcagtcccccaagtagctggaaccacagaggtgcaccaccacgcccagctaatttttgtattttttgtagaaacgcggttttgccatgttggccaggctcatctcaaactcctgagctcaaacgcctcagcctcccaaagtactgggattacaggtgtgagccaccacgcccagcctctcatcaaactttttactgttccttaattatactacactaacttgcaatcacctcctttggaaaaattattgtaattatacatctaaaattatttgtttgatgggtcaacccactctcccaactcaaagtgtcactggggtagagatcctctactctggtcacacataggtccccaagggttaccacagtgccagacacatagcaggcacataaatatttgttaaggtaaaactgaatggtgctcattgctgtaatatttatgacagagcctcccaactagtgtgtcaagatatgggtattttcagccctgagacagctggaaagggtctggctttctggctgccaggcagggttgatttaaccagtaagttatataaatata

SEQ ID NO: 11700 - RNA, 5840 nt, Homo sapiens
  source 1..5840: mol_type = other RNA
ctgaatagctgggactacaggtgtgcaccaccacgcccagctaatttttgtatttttttgtaaagatagggtttcattatgttgcccaggctggtctcaaactcctgggctcaagcgatccacccacctcgatttcccaaagtgctgagattataggcctgagccaccatgcctggctgcagatccttcataggtttcttaatcttaagaacaaaaagctcacctggaaagcaagaacacatcaatttggcagtatctggtcactaaaagaactgtatctctggaggcaagcatgggctctaataaaccccacaaagtattgccgtctaattcccaaatattcctgactgtctctttccacagagctaaggagggttcaattcaaagaacattaaagtccctttggcttgcatagcagacgagaaaccagactcttcttgccaagcatgcctcaggcccacaaatacccatggaaataggtatatatttctgagtaaaaagccaccatccatgtcagaaaagatttgaatctacctcagctgtctttcttctcttagatctgtctgcctcatactttgtggatgactactttggaaaagtgaaactcaggtaagacactaagctctctaagcctcaattttctcacaggtaaaatggggatagtgtatttacctcagagagtcattgtgagacaacacatgtaaagcactgagcctagtatatagaacacatttaatgagcagaaactagttgctgagtgcttctacgtagacagaagtagagaaacgagcagattcatgagaggagaaaaaagaaacaaatatatagtgcatgtggacaggaactacacagaggatttctaaaagctgcctccaagaccaattcaggtcctagagggaaaaatgtacaacattgagttctgagaaggctgggcagatacatcacagacaatgcatggtttggaggcatgaaactaaacaaatgccttcccaatactctacatccacagggatacaaatgcagtgtcatctgtgggcagtcttcctgttaacttgacacaagatcagccctccatctgcaggtgtcaaagctcccttaataattagttcctgagtcaaatataatactgacaaaaacattgtagatctttcatcttttgggggaatttttagtcataaatttaggattccactgtttctttaaagcaaagccactagtagctgagggtgatggtgtgtgcctgtagtcccagctgctcagggggcagaggcaggaggattgcttaagcccagaagtttgaggctatagtgagctatgattccaccactgcactccagcctggatgacacggcgagaccacatctcttaaagagaaaaactttttaaaaagcaaaaagcaaagccactaaaatatgttagcctaaagagggcatgcctgcttcattacagacggtatgacacatcttgagataaaaactaggatggctttcttatctgggttcctgactgctccttagctttgagttcttctagcttcttctcatagcgactcataaagtaatcatctggttcaatctctgcattcttcaagttttccatgatcttttccagtctgagcactgatcgggctccttcaatctttcttgtactcaagtacaaggtgaactcctggaaatccaggagcttacaggtgtccacagagcagatattccggatatcactagttctatccaaatgaggaaaaaacaccagtcctgacaacttctctaggtcctggaggctcacttggaattcagttaactggggctggaagccgatggcttcattgggtaccacaaaggcccctagcgccagtggttcggtagatactgagcttctgcgggccaggattaccttataaaggtgtgaggggactgccacgttgtcctcgccaatcacctggtaactaactattttctttccatcgcctctagtctgaggtaaggtcaaaggcccagataccacccaaacatcttcaaacctttctgtcagctctcgacagtacatttctattctgttccaatatccagaattattatcaaaatcctgaggcacaatgttagaaaggtaaaaggtttcagccatggctttacttgaaaatttgttatttcctgctggagccatgtgtcctcgtgaccacccacttccaacataatcttcattgaaggcactgaaggttggagggatattgggatcaggcttaaatttacaatgctttctgtctgcatcacctgaagaaaaacacacaaaatggatatgttatcagtagacaaatgtccctcaagattctctaagcaaggcaagctggttgctactggctggtgtctctccaagcagctagtattagggattgcatgcatgtctcaagttcctgggatagttcagatacttcatctgaatttagaaagtactagtctaggaaagaatgcttttcatacagtgtagctatctcatataattttgactctggcctttccagttaaagaaaaactcctctgaatagtattttaagtaaaaacaatcaccaatcaaaacactaaactatataaaaagcttggctactaaataaactcttgttttttaaaaaagactcccatgtattgtattttgtacgattgtatttgacaagtttatgtgtactgaaataatggatatatatagacacaaaacaatttgttctaggcaagcacagccttggggagaggagtgtctctgatatcttgcttactgcctctcgaaccatgacaaaataaacatttaagttatgagctccacccagaaatttctaaaacagaatatctgggtaccacataggagagaagaaatctcagattttatttattttctgacacctccagaatggtttgtcacagagaacattagcaaatcctaacactacctattgcactatcgtgaggtgagactttcttaaactacaaaagttatgacaacaaatgaaacatactcagactgttattcaaagaagtgtaaaatggagaacaatgaagtcactgattccaaggtgatttcattcagccaagaaaaatttagtatcagatcccaaagtttacagtaaagtatcatatatgtagctttttagaatcactttataaagaataatacagaaaaatttatcattagtaaatttctaagtgtcattaccattggaatcacttccttctacagctagttatctttggctggtgcttactgccctggaaaagcaatttgtaggaatttccaaagacctaaaaagataccttccttgagaaaagatataaatttactgctgtaaggtgtctagcagtattcccagtggagaaccgtattaaaccatgctcagggattaaggttccctgatctcctctcgatgcacagatttgggctgtaagtctgcatgatagccagtttttgactttaccttctctggaacaaactttttatcttccttttgacctttctccgttcagtgccaagacaaccttccatgtagtccctgtaatcccagctactcaggaggctgaggcaggagggtcacttgaacccagaaattcaagaccagcctaggcaacatagcaaaaatccatctcaaaaaaaaaggtaaaaaaaatacagatatacactttttatatactaacattttctgtttcagcaggaagattctatctgaataactcagtccatcattactgaaaacagaagaccttttacattaaaatcaagtaaaacacaggtacattgctccctattttcaaataatattaattggctctattttattgcctcaaaagtacacagctcacaagacttattatacaatataaaatgcccaggttttcttatatgcttgataaagttttcacttacatcagtttctgtctaacaccaagtacattccaagcctcctgttattctgctggttgctgtgcactctagaatggcacacactaactttaatatcagcattttaatatgcatagccatagcacacattttaaagcaaaggagaatatgtggaacacacagcaaattaaaaagcaaataacaaaagggaacaaaacaactgtgacaaaaggtaatatccttaataaataaaagaacttttacaaataaattcaaaagagaataccccaactgaaataggtaaagaataacttaccaaaaaagactaattcacagcatgttaaccctcattgataatcaataaacacaagtaaaatgagcattaaattggtaaagctcagtaatgctcaccataggtgaaggttgagagagagaagaaacaatgatgctaggagtgtaaacttgaagaatctacctagaaaccaatttgacattaattatcaagatctggcaattctacaggaccctatcaagacataaggacacatgaataaactgacacacctgcttacttctccagcatcatttcacatcaccttccccctcattcatctactggcactcttttagttccctaaaagaacaaaactcctgtccacattgggggcctccgaagatgcaaatgttcctttcttcctagaatgctcttctccatatcccatggcacattcaaccccttgcctaagtaatttccgttcactcttcagtccacttttccagagaagccttactaatcaaaatcaggttcttgtgttataatctctcatcacacttttttttttttttgagacacattctccctctgttgcctaagctggagtgtggtgctgcgatcttggctcactgcaacccccacctcctgggctcaagagatcctcccatctcagtcccccaagtagctggaaccacagaggtgcaccaccacgcccagctaatttttgtattttttgtagaaacgcggttttgccatgttggccaggctcatctcaaactcctgagctcaaacgcctcagcctcccaaagtactgggattacaggtgtgagccaccacgcccagcctctcatcaaactttttactgttccttaattatactacactaacttgcaatcacctcctttggaaaaattattgtaattatacatctaaaattatttgtttgatgggtcaacccactctcccaactcaaagtgtcactggggtagagatcctctactctggtcacacataggtccccaagggttaccacagtgccagacacatagcaggcacataaatatttgttaaggtaaaactgaatggtgctcattgctgtaatatttatgacagagcctcccaactagtgtgtcaagatatgggtattttcagccctgagacagctggaaagggtctggctttctggctgccaggcagggttgatttaaccagtaagttatataaatataattttctacatgtgctatgatatgaaaaaggttgagaatattaataatcatccctgttttaaatttggagacatctttcataaatactgttacttcagtttttttatccaaccacctacccattatcttgcttttggaaatatgttcaagaacccatctaggcacccgctttgcctgatcataagacaaagcgtgattagtgtaacaccttgcctctgttccagttaaagggaatccaaattgttccaagacagccttttctgcagatccatccggctgcttccctgtcaacgctccctcagcgccctgactccggaagaactgcagggccgcgagcccagctcccgcagcgcccactacagccccagccacgaagccgctcagaaaacgacgggaaccccggaggcgggaagcgatactcttgatagccatcttgcccgaggtaccggcctttt

SEQ ID NO: 11701 - RNA, 2679 nt, Homo sapiens
  source 1..2679: mol_type = other RNA
ctgaatagctgggactacaggtgtgcaccaccacgcccagctaatttttgtatttttttgtaaagatagggtttcattatgttgcccaggctggtctcaaactcctgggctcaagcgatccacccacctcgatttcccaaagtgctgagattataggcctgagccaccatgcctggctgcagatccttcataggtttcttaatcttaagaacaaaaagctcacctggaaagcaagaacacatcaatttggcagtatctggtcactaaaagaactgtatctctggaggcaagcatgggctctaataaaccccacaaagtattgccgtctaattcccaaatattcctgactgtctctttccacagagctaaggagggttcaattcaaagaacattaaagtccctttggcttgcatagcagacgagaaaccagactcttcttgccaagcatgcctcaggcccacaaatacccatggaaataggtatatatttctgagtaaaaagccaccatccatgtcagaaaagatttgaatctacctcagctgtctttcttctcttagatctgtctgcctcatactttgtggatgactactttggaaaagtgaaactcaggtaagacactaagctctctaagcctcaattttctcacaggtaaaatggggatagtgtatttacctcagagagtcattgtgagacaacacatgtaaagcactgagcctagtatatagaacacatttaatgagcagaaactagttgctgagtgcttctacgtagacagaagtagagaaacgagcagattcatgagaggagaaaaaagaaacaaatatatagtgcatgtggacaggaactacacagaggatttctaaaagctgcctccaagaccaattcaggtcctagagggaaaaatgtacaacattgagttctgagaaggctgggcagatacatcacagacaatgcatggtttggaggcatgaaactaaacaaatgccttcccaatactctacatccacagggatacaaatgcagtgtcatctgtgggcagtcttcctgttaacttgacacaagatcagccctccatctgcaggtgtcaaagctcccttaataattagttcctgagtcaaatataatactgacaaaaacattgtagatctttcatcttttgggggaatttttagtcataaatttaggattccactgtttctttaaagcaaagccactagtagctgagggtgatggtgtgtgcctgtagtcccagctgctcagggggcagaggcaggaggattgcttaagcccagaagtttgaggctatagtgagctatgattccaccactgcactccagcctggatgacacggcgagaccacatctcttaaagagaaaaactttttaaaaagcaaaaagcaaagccactaaaatatgttagcctaaagagggcatgcctgcttcattacagacggtatgacacatcttgagataaaaactaggatggctttcttatctgggttcctgactgctccttagctttgagttcttctagcttcttctcatagcgactcataaagtaatcatctggttcaatctctgcattcttcaagttttccatgatcttttccagtctgagcactgatcgggctccttcaatctttcttgtactcaagtacaaggtgaactcctggaaatccaggagcttacaggtgtccacagagcagatattccggatatcactagttctatccaaatgaggaaaaaacaccagtcctgacaacttctctaggtcctggaggctcacttggaattcagttaactggggctggaagccgatggcttcattgggtaccacaaaggcccctagcgccagtggttcggtagatactgagcttctgcgggccaggattaccttataaaggtgtgaggggactgccacgttgtcctcgccaatcacctggtaactaactattttctttccatcgcctctagtctgaggtaaggtcaaaggcccagataccacccaaacatcttcaaacctttctgtcagctctcgacagtacatttctattctgttccaatatccagaattattatcaaaatcctgaggcacaatgttagaaaggtaaaaggtttcagccatggctttacttgaaaatttgttatttcctgctggagccatgtgtcctcgtgaccacccacttccaacataatcttcattgaaggcactgaaggttggagggatattgggatcaggcttaaatttacaatgctttctgtctgcatcacctgcttacttctccagcatcatttcacatcaccttccccctcattcatctactggcactcttttagttcccttgcctctgttccagttaaagggaatccaaattgttccaagacagccttttctgcagatctgaatgccaattatgtaccaggtactgtgctggttagatgatggagaccaaaacagacatagtctcaagtcttatggagctaacaatcatccggctgcttccctgtcaacgctccctcagcgccctgactccggaagaactgcagggccgcgagcccagctcccgcagcgcccactacagccccagccacgaagccgctcagaaaacgacgggaaccccggaggcgggaagcgatactcttgatagccatcttgcccgaggtaccggccttttaccac

SEQ ID NO: 11702 - RNA, 3042 nt, Homo sapiens
  source 1..3042: mol_type = other RNA
ctgaatagctgggactacaggtgtgcaccaccacgcccagctaatttttgtatttttttgtaaagatagggtttcattatgttgcccaggctggtctcaaactcctgggctcaagcgatccacccacctcgatttcccaaagtgctgagattataggcctgagccaccatgcctggctgcagatccttcataggtttcttaatcttaagaacaaaaagctcacctggaaagcaagaacacatcaatttggcagtatctggtcactaaaagaactgtatctctggaggcaagcatgggctctaataaaccccacaaagtattgccgtctaattcccaaatattcctgactgtctctttccacagagctaaggagggttcaattcaaagaacattaaagtccctttggcttgcatagcagacgagaaaccagactcttcttgccaagcatgcctcaggcccacaaatacccatggaaataggtatatatttctgagtaaaaagccaccatccatgtcagaaaagatttgaatctacctcagctgtctttcttctcttagatctgtctgcctcatactttgtggatgactactttggaaaagtgaaactcaggtaagacactaagctctctaagcctcaattttctcacaggtaaaatggggatagtgtatttacctcagagagtcattgtgagacaacacatgtaaagcactgagcctagtatatagaacacatttaatgagcagaaactagttgctgagtgcttctacgtagacagaagtagagaaacgagcagattcatgagaggagaaaaaagaaacaaatatatagtgcatgtggacaggaactacacagaggatttctaaaagctgcctccaagaccaattcaggtcctagagggaaaaatgtacaacattgagttctgagaaggctgggcagatacatcacagacaatgcatggtttggaggcatgaaactaaacaaatgccttcccaatactctacatccacagggatacaaatgcagtgtcatctgtgggcagtcttcctgttaacttgacacaagatcagccctccatctgcaggtgtcaaagctcccttaataattagttcctgagtcaaatataatactgacaaaaacattgtagatctttcatcttttgggggaatttttagtcataaatttaggattccactgtttctttaaagcaaagccactagtagctgagggtgatggtgtgtgcctgtagtcccagctgctcagggggcagaggcaggaggattgcttaagcccagaagtttgaggctatagtgagctatgattccaccactgcactccagcctggatgacacggcgagaccacatctcttaaagagaaaaactttttaaaaagcaaaaagcaaagccactaaaatatgttagcctaaagagggcatgcctgcttcattacagacggtatgacacatcttgagataaaaactaggatggctttcttatctgggttcctgactgctccttagctttgagttcttctagcttcttctcatagcgactcataaagtaatcatctggttcaatctctgcattcttcaagttttccatgatcttttccagtctgagcactgatcgggctccttcaatctttcttgtactcaagtacaaggtgaactcctggaaatccaggagcttacaggtgtccacagagcagatattccggatatcactagttctatccaaatgaggaaaaaacaccagtcctgacaacttctctaggtcctggaggctcacttggaattcagttaactggggctggaagccgatggcttcattgggtaccacaaaggcccctagcgccagtggttcggtagatactgagcttctgcgggccaggattaccttataaaggtgtgaggggactgccacgttgtcctcgccaatcacctggtaactaactattttctttccatcgcctctagtctgaggtaaggtcaaaggcccagataccacccaaacatcttcaaacctttctgtcagctctcgacagtacatttctattctgttccaatatccagaattattatcaaaatcctgaggcacaatgttagaaaggtaaaaggtttcagccatggctttacttgaaaatttgttatttcctgctggagccatgtgtcctcgtgaccacccacttccaacataatcttcattgaaggcactgaaggttggagggatattgggatcaggcttaaatttacaatgctttctgtctgcatcacctgtaatcccagctactcaggaggctgaggcaggagggtcacttgaacccagaaattcaagaccagccataggtgaaggttgagagagagaagaaacaatgatgctaggagtgtaaacttgaagaatctacccattatcttgcttttggaaatatgttcaagaacccatctaggcacccgctttgcctgatcataagacaaagcgtgattagtgtaacaccttgcctctgttccagttaaagggaatccaaattgttccaagacagccttttctgcagatctgaatgccaattatgtaccaggtactgtgctggttagatgatggagaccaaaacagacatagtctcaagtcttatggagctaacaatcatccggctgcttccctgtcaacgctccctcagcgccctgactccggaagaactgcagggccgcgagcccagctcccgcagcgcccactacagccccagccacgaagccgctcagaaaacgacgggaaccccggaggcgggaagcgatactcttgatagccatcttgcccgaggtaccggccttttaccacggcgcatgcgcgcgcatgccggcccccgccatccccccgtcaccccacgcctcaccgcccgccaagctgagggcctcgcacgccccctggtgacaaaccgggatgcctagcgcatccccgcttcatccctggtccactggacggggcgatggatggggaatatgatgtctagagggcttagtggtatgctatatatagtcatgagaagaaaat

SEQ ID NO: 11703 - RNA, 2735 nt, Homo sapiens
  source 1..2735: mol_type = other RNA
ctgaatagctgggactacaggtgtgcaccaccacgcccagctaatttttgtatttttttgtaaagatagggtttcattatgttgcccaggctggtctcaaactcctgggctcaagcgatccacccacctcgatttcccaaagtgctgagattataggcctgagccaccatgcctggctgcagatccttcataggtttcttaatcttaagaacaaaaagctcacctggaaagcaagaacacatcaatttggcagtatctggtcactaaaagaactgtatctctggaggcaagcatgggctctaataaaccccacaaagtattgccgtctaattcccaaatattcctgactgtctctttccacagagctaaggagggttcaattcaaagaacattaaagtccctttggcttgcatagcagacgagaaaccagactcttcttgccaagcatgcctcaggcccacaaatacccatggaaataggtatatatttctgagtaaaaagccaccatccatgtcagaaaagatttgaatctacctcagctgtctttcttctcttagatctgtctgcctcatactttgtggatgactactttggaaaagtgaaactcaggtaagacactaagctctctaagcctcaattttctcacaggtaaaatggggatagtgtatttacctcagagagtcattgtgagacaacacatgtaaagcactgagcctagtatatagaacacatttaatgagcagaaactagttgctgagtgcttctacgtagacagaagtagagaaacgagcagattcatgagaggagaaaaaagaaacaaatatatagtgcatgtggacaggaactacacagaggatttctaaaagctgcctccaagaccaattcaggtcctagagggaaaaatgtacaacattgagttctgagaaggctgggcagatacatcacagacaatgcatggtttggaggcatgaaactaaacaaatgccttcccaatactctacatccacagggatacaaatgcagtgtcatctgtgggcagtcttcctgttaacttgacacaagatcagccctccatctgcaggtgtcaaagctcccttaataattagttcctgagtcaaatataatactgacaaaaacattgtagatctttcatcttttgggggaatttttagtcataaatttaggattccactgtttctttaaagcaaagccactagtagctgagggtgatggtgtgtgcctgtagtcccagctgctcagggggcagaggcaggaggattgcttaagcccagaagtttgaggctatagtgagctatgattccaccactgcactccagcctggatgacacggcgagaccacatctcttaaagagaaaaactttttaaaaagcaaaaagcaaagccactaaaatatgttagcctaaagagggcatgcctgcttcattacagacggtatgacacatcttgagataaaaactaggatggctttcttatctgggttcctgactgctccttagctttgagttcttctagcttcttctcatagcgactcataaagtaatcatctggttcaatctctgcattcttcaagttttccatgatcttttccagtctgagcactgatcgggctccttcaatctttcttgtactcaagtacaaggtgaactcctggaaatccaggagcttacaggtgtccacagagcagatattccggatatcactagttctatccaaatgaggaaaaaacaccagtcctgacaacttctctaggtcctggaggctcacttggaattcagttaactggggctggaagccgatggcttcattgggtaccacaaaggcccctagcgccagtggttcggtagatactgagcttctgcgggccaggattaccttataaaggtgtgaggggactgccacgttgtcctcgccaatcacctggtaactaactattttctttccatcgcctctagtctgaggtaaggtcaaaggcccagataccacccaaacatcttcaaacctttctgtcagctctcgacagtacatttctattctgttccaatatccagaattattatcaaaatcctgaggcacaatgttagaaaggtaaaaggtttcagccatggctttacttgaaaatttgttatttcctgctggagccatgtgtcctcgtgaccacccacttccaacataatcttcattgaaggcactgaaggttggagggatattgggatcaggcttaaatttacaatgctttctgtctgcatcacctgtaatcccagctactcaggaggctgaggcaggagggtcacttgaacccagaaattcaagaccagccataggtgaaggttgagagagagaagaaacaatgatgctaggagtgtaaacttgaagaatctacctctgttccagttaaagggaatccaaattgttccaagacagccttttctgcagatctgaatgccaattatgtaccaggtactgtgctggttagatgatggagaccaaaacagacatagtctcaagtcttatggagctaacaatcatccggctgcttccctgtcaacgctccctcagcgccctgactccggaagaactgcagggccgcgagcccagctcccgcagcgcccactacagccccagccacgaagccgctcagaaaacgacgggaaccccggaggcgggaagcgatactcttgatagccatcttgcccgaggtaccggccttttaccac

SEQ ID NO: 11704 - RNA, 2678 nt, Homo sapiens
  source 1..2678: mol_type = other RNA
ctgaatagctgggactacaggtgtgcaccaccacgcccagctaatttttgtatttttttgtaaagatagggtttcattatgttgcccaggctggtctcaaactcctgggctcaagcgatccacccacctcgatttcccaaagtgctgagattataggcctgagccaccatgcctggctgcagatccttcataggtttcttaatcttaagaacaaaaagctcacctggaaagcaagaacacatcaatttggcagtatctggtcactaaaagaactgtatctctggaggcaagcatgggctctaataaaccccacaaagtattgccgtctaattcccaaatattcctgactgtctctttccacagagctaaggagggttcaattcaaagaacattaaagtccctttggcttgcatagcagacgagaaaccagactcttcttgccaagcatgcctcaggcccacaaatacccatggaaataggtatatatttctgagtaaaaagccaccatccatgtcagaaaagatttgaatctacctcagctgtctttcttctcttagatctgtctgcctcatactttgtggatgactactttggaaaagtgaaactcaggtaagacactaagctctctaagcctcaattttctcacaggtaaaatggggatagtgtatttacctcagagagtcattgtgagacaacacatgtaaagcactgagcctagtatatagaacacatttaatgagcagaaactagttgctgagtgcttctacgtagacagaagtagagaaacgagcagattcatgagaggagaaaaaagaaacaaatatatagtgcatgtggacaggaactacacagaggatttctaaaagctgcctccaagaccaattcaggtcctagagggaaaaatgtacaacattgagttctgagaaggctgggcagatacatcacagacaatgcatggtttggaggcatgaaactaaacaaatgccttcccaatactctacatccacagggatacaaatgcagtgtcatctgtgggcagtcttcctgttaacttgacacaagatcagccctccatctgcaggtgtcaaagctcccttaataattagttcctgagtcaaatataatactgacaaaaacattgtagatctttcatcttttgggggaatttttagtcataaatttaggattccactgtttctttaaagcaaagccactagtagctgagggtgatggtgtgtgcctgtagtcccagctgctcagggggcagaggcaggaggattgcttaagcccagaagtttgaggctatagtgagctatgattccaccactgcactccagcctggatgacacggcgagaccacatctcttaaagagaaaaactttttaaaaagcaaaaagcaaagccactaaaatatgttagcctaaagagggcatgcctgcttcattacagacggtatgacacatcttgagataaaaactaggatggctttcttatctgggttcctgactgctccttagctttgagttcttctagcttcttctcatagcgactcataaagtaatcatctggttcaatctctgcattcttcaagttttccatgatcttttccagtctgagcactgatcgggctccttcaatctttcttgtactcaagtacaaggtgaactcctggaaatccaggagcttacaggtgtccacagagcagatattccggatatcactagttctatccaaatgaggaaaaaacaccagtcctgacaacttctctaggtcctggaggctcacttggaattcagttaactggggctggaagccgatggcttcattgggtaccacaaaggcccctagcgccagtggttcggtagatactgagcttctgcgggccaggattaccttataaaggtgtgaggggactgccacgttgtcctcgccaatcacctggtaactaactattttctttccatcgcctctagtctgaggtaaggtcaaaggcccagataccacccaaacatcttcaaacctttctgtcagctctcgacagtacatttctattctgttccaatatccagaattattatcaaaatcctgaggcacaatgttagaaaggtaaaaggtttcagccatggctttacttgaaaatttgttatttcctgctggagccatgtgtcctcgtgaccacccacttccaacataatcttcattgaaggcactgaaggttggagggatattgggatcaggcttaaatttacaatgctttctgtctgcatcacctgtaatcccagctactcaggaggctgaggcaggagggtcacttgaacccagaaattcaagaccagcccattatcttgcttttggaaatatgttcaagaacccatctaggcacccgctttgcctgatcataagacaaagcgtgattagtgtaacaccttgcctctgttccagttaaagggaatccaaattgttccaagacagccttttctgcagatccatccggctgcttccctgtcaacgctccctcagcgccctgactccggaagaactgcagggccgcgagcccagctcccgcagcgcccactacagccccagccacgaagccgctcagaaaacgacgggaaccccggaggcgggaagcgatactcttgatagccatcttgcccgaggtaccggccttttaccac

SEQ ID NO: 11705 - RNA, 4575 nt, Homo sapiens
  source 1..4575: mol_type = other RNA
ctgaatagctgggactacaggtgtgcaccaccacgcccagctaatttttgtatttttttgtaaagatagggtttcattatgttgcccaggctggtctcaaactcctgggctcaagcgatccacccacctcgatttcccaaagtgctgagattataggcctgagccaccatgcctggctgcagatccttcataggtttcttaatcttaagaacaaaaagctcacctggaaagcaagaacacatcaatttggcagtatctggtcactaaaagaactgtatctctggaggcaagcatgggctctaataaaccccacaaagtattgccgtctaattcccaaatattcctgactgtctctttccacagagctaaggagggttcaattcaaagaacattaaagtccctttggcttgcatagcagacgagaaaccagactcttcttgccaagcatgcctcaggcccacaaatacccatggaaataggtatatatttctgagtaaaaagccaccatccatgtcagaaaagatttgaatctacctcagctgtctttcttctcttagatctgtctgcctcatactttgtggatgactactttggaaaagtgaaactcaggtaagacactaagctctctaagcctcaattttctcacaggtaaaatggggatagtgtatttacctcagagagtcattgtgagacaacacatgtaaagcactgagcctagtatatagaacacatttaatgagcagaaactagttgctgagtgcttctacgtagacagaagtagagaaacgagcagattcatgagaggagaaaaaagaaacaaatatatagtgcatgtggacaggaactacacagaggatttctaaaagctgcctccaagaccaattcaggtcctagagggaaaaatgtacaacattgagttctgagaaggctgggcagatacatcacagacaatgcatggtttggaggcatgaaactaaacaaatgccttcccaatactctacatccacagggatacaaatgcagtgtcatctgtgggcagtcttcctgttaacttgacacaagatcagccctccatctgcaggtgtcaaagctcccttaataattagttcctgagtcaaatataatactgacaaaaacattgtagatctttcatcttttgggggaatttttagtcataaatttaggattccactgtttctttaaagcaaagccactagtagctgagggtgatggtgtgtgcctgtagtcccagctgctcagggggcagaggcaggaggattgcttaagcccagaagtttgaggctatagtgagctatgattccaccactgcactccagcctggatgacacggcgagaccacatctcttaaagagaaaaactttttaaaaagcaaaaagcaaagccactaaaatatgttagcctaaagagggcatgcctgcttcattacagacggtatgacacatcttgagataaaaactaggatggctttcttatctgggttcctgactgctccttagctttgagttcttctagcttcttctcatagcgactcataaagtaatcatctggttcaatctctgcattcttcaagttttccatgatcttttccagtctgagcactgatcgggctccttcaatctttcttgtactcaagtacaaggtgaactcctggaaatccaggagcttacaggtgtccacagagcagatattccggatatcactagttctatccaaatgaggaaaaaacaccagtcctgacaacttctctaggtcctggaggctcacttggaattcagttaactggggctggaagccgatggcttcattgggtaccacaaaggcccctagcgccagtggttcggtagatactgagcttctgcgggccaggattaccttataaaggtgtgaggggactgccacgttgtcctcgccaatcacctggtaactaactattttctttccatcgcctctagtctgaggtaaggtcaaaggcccagataccacccaaacatcttcaaacctttctgtcagctctcgacagtacatttctattctgttccaatatccagaattattatcaaaatcctgaggcacaatgttagaaaggtaaaaggtttcagccatggctttacttgaaaatttgttatttcctgctggagccatgtgtcctcgtgaccacccacttccaacataatcttcattgaaggcactgaaggttggagggatattgggatcaggcttaaatttacaatgctttctgtctgcatcacctgtaatcccagctactcaggaggctgaggcaggagggtcacttgaacccagaaattcaagaccagcctaggcaacatagcaaaaatccatctcaaaaaaaaaggtaaaaaaaatacagatatacactttttatatactaacattttctgtttcagcaggaagattctatctgaataactcagtccatcattactgaaaacagaagaccttttacattaaaatcaagtaaaacacaggtacattgctccctattttcaaataatattaattggctctattttattgcctcaaaagtacacagctcacaagacttattatacaatataaaatgcccaggttttcttatatgcttgataaagttttcacttacatcagtttctgtctaacaccaagtacattccaagcctcctgttattctgctggttgctgtgcactctagaatggcacacactaactttaatatcagcattttaatatgcatagccatagcacacattttaaagcaaaggagaatatgtggaacacacagcaaattaaaaagcaaataacaaaagggaacaaaacaactgtgacaaaaggtaatatccttaataaataaaagaacttttacaaataaattcaaaagagaataccccaactgaaataggtaaagaataacttaccaaaaaagactaattcacagcatgttaaccctcattgataatcaataaacacaagtaaaatgagcattaaattggtaaagctcagtaatgctcaccataggtgaaggttgagagagagaagaaacaatgatgctaggagtgtaaacttgaagaatctacctagaaaccaatttgacattaattatcaagatctggcaattctacaggaccctatcaagacataaggacacatgaataaactgacacacctgcttacttctccagcatcatttcacatcaccttccccctcattcatctactggcactcttttagttccctaaaagaacaaaactcctgtccacattgggggcctccgaagatgcaaatgttcctttcttcctagaatgctcttctccatatcccatggcacattcaaccccttgcctaagtaatttccgttcactcttcagtccacttttccagagaagccttactaatcaaaatcaggttcttgtgttataatctctcatcacacttttttttttttttgagacacattctccctctgttgcctaagctggagtgtggtgctgcgatcttggctcactgcaacccccacctcctgggctcaagagatcctcccatctcagtcccccaagtagctggaaccacagaggtgcaccaccacgcccagctaatttttgtattttttgtagaaacgcggttttgccatgttggccaggctcatctcaaactcctgagctcaaacgcctcagcctcccaaagtactgggattacaggtgtgagccaccacgcccagcctctcatcaaactttttactgttccttaattatactacactaacttgcaatcacctcctttggaaaaattattgtaattatacatctaaaattatttgtttgatgggtcaacccactctcccaactcaaagtgtcactggggtagagatcctctactctggtcacacataggtccccaagggttaccacagtgccagacacatagcaggcacataaatatttgttaaggtaaaactgaatggtgctcattgctgtaatatttatgacagagcctcccaactagtgtgtcaagatatgggtattttcagccctgagacagctggaaagggtctggctttctggctgccaggcagggttgatttaaccagtaagttatataaatataattttctacatgtgctatgatatgaaaaaggttgagaatattaataatcatccctgttttaaatttggagacatctttcataaatactgttacttcagtttttttatccaaccacctacccattatcttgcttttggaaatatgttcaagaacccatctaggcacccgctttgcctgatcataagacaaagcgtgattagtgtaacaccttgcctctgttccagttaaagggaatccaaattgttccaagacagccttttctgcagatccatccggctgcttccctgtcaacgctccctcagcgccctgactccggaagaactgcagggccgcgagcccagctcccgcagcgcccactacagccccagccacgaagccgctcagaaaacgacgggaaccccggaggcgggaagcgatactcttgatagccatcttgcccgaggtaccggcctttt

SEQ ID NO: 11706 - RNA, 2532 nt, Homo sapiens
  source 1..2532: mol_type = other RNA
ctgaatagctgggactacaggtgtgcaccaccacgcccagctaatttttgtatttttttgtaaagatagggtttcattatgttgcccaggctggtctcaaactcctgggctcaagcgatccacccacctcgatttcccaaagtgctgagattataggcctgagccaccatgcctggctgcagatccttcataggtttcttaatcttaagaacaaaaagctcacctggaaagcaagaacacatcaatttggcagtatctggtcactaaaagaactgtatctctggaggcaagcatgggctctaataaaccccacaaagtattgccgtctaattcccaaatattcctgactgtctctttccacagagctaaggagggttcaattcaaagaacattaaagtccctttggcttgcatagcagacgagaaaccagactcttcttgccaagcatgcctcaggcccacaaatacccatggaaataggtatatatttctgagtaaaaagccaccatccatgtcagaaaagatttgaatctacctcagctgtctttcttctcttagatctgtctgcctcatactttgtggatgactactttggaaaagtgaaactcaggtaagacactaagctctctaagcctcaattttctcacaggtaaaatggggatagtgtatttacctcagagagtcattgtgagacaacacatgtaaagcactgagcctagtatatagaacacatttaatgagcagaaactagttgctgagtgcttctacgtagacagaagtagagaaacgagcagattcatgagaggagaaaaaagaaacaaatatatagtgcatgtggacaggaactacacagaggatttctaaaagctgcctccaagaccaattcaggtcctagagggaaaaatgtacaacattgagttctgagaaggctgggcagatacatcacagacaatgcatggtttggaggcatgaaactaaacaaatgccttcccaatactctacatccacagggatacaaatgcagtgtcatctgtgggcagtcttcctgttaacttgacacaagatcagccctccatctgcaggtgtcaaagctcccttaataattagttcctgagtcaaatataatactgacaaaaacattgtagatctttcatcttttgggggaatttttagtcataaatttaggattccactgtttctttaaagcaaagccactagtagctgagggtgatggtgtgtgcctgtagtcccagctgctcagggggcagaggcaggaggattgcttaagcccagaagtttgaggctatagtgagctatgattccaccactgcactccagcctggatgacacggcgagaccacatctcttaaagagaaaaactttttaaaaagcaaaaagcaaagccactaaaatatgttagcctaaagagggcatgcctgcttcattacagacggtatgacacatcttgagataaaaactaggatggctttcttatctgggttcctgactgctccttagctttgagttcttctagcttcttctcatagcgactcataaagtaatcatctggttcaatctctgcattcttcaagttttccatgatcttttccagtctgagcactgatcgggctccttcaatctttcttgtactcaagtacaaggtgaactcctggaaatccaggagcttacaggtgtccacagagcagatattccggatatcactagttctatccaaatgaggaaaaaacaccagtcctgacaacttctctaggtcctggaggctcacttggaattcagttaactggggctggaagccgatggcttcattgggtaccacaaaggcccctagcgccagtggttcggtagatactgagcttctgcgggccaggattaccttataaaggtgtgaggggactgccacgttgtcctcgccaatcacctggtaactaactattttctttccatcgcctctagtctgaggtaaggtcaaaggcccagataccacccaaacatcttcaaacctttctgtcagctctcgacagtacatttctattctgttccaatatccagaattattatcaaaatcctgaggcacaatgttagaaaggtaaaaggtttcagccatggctttacttgaaaatttgttatttcctgctggagccatgtgtcctcgtgaccacccacttccaacataatcttcattgaaggcactgaaggttggagggatattgggatcaggcttaaatttacaatgctttctgtctgcatcaccttctctggaacaaactttttatcttccttttgacctttctccgttcagtgccaagacaaccttccatgtagtccccattatcttgcttttggaaatatgttcaagaacccatctaggcacccgctttgcctgatcataagacaaagcgtgattagtgtaacaccttgcctctgttccagttaaagggaatccaaattgttccaagacagccttttctgcagatccatccggctgcttccctgtcaacgctccctcagcgcc

SEQ ID NO: 11707 - RNA, 2773 nt, Homo sapiens
  source 1..2773: mol_type = other RNA
ctgaatagctgggactacaggtgtgcaccaccacgcccagctaatttttgtatttttttgtaaagatagggtttcattatgttgcccaggctggtctcaaactcctgggctcaagcgatccacccacctcgatttcccaaagtgctgagattataggcctgagccaccatgcctggctgcagatccttcataggtttcttaatcttaagaacaaaaagctcacctggaaagcaagaacacatcaatttggcagtatctggtcactaaaagaactgtatctctggaggcaagcatgggctctaataaaccccacaaagtattgccgtctaattcccaaatattcctgactgtctctttccacagagctaaggagggttcaattcaaagaacattaaagtccctttggcttgcatagcagacgagaaaccagactcttcttgccaagcatgcctcaggcccacaaatacccatggaaataggtatatatttctgagtaaaaagccaccatccatgtcagaaaagatttgaatctacctcagctgtctttcttctcttagatctgtctgcctcatactttgtggatgactactttggaaaagtgaaactcaggtaagacactaagctctctaagcctcaattttctcacaggtaaaatggggatagtgtatttacctcagagagtcattgtgagacaacacatgtaaagcactgagcctagtatatagaacacatttaatgagcagaaactagttgctgagtgcttctacgtagacagaagtagagaaacgagcagattcatgagaggagaaaaaagaaacaaatatatagtgcatgtggacaggaactacacagaggatttctaaaagctgcctccaagaccaattcaggtcctagagggaaaaatgtacaacattgagttctgagaaggctgggcagatacatcacagacaatgcatggtttggaggcatgaaactaaacaaatgccttcccaatactctacatccacagggatacaaatgcagtgtcatctgtgggcagtcttcctgttaacttgacacaagatcagccctccatctgcaggtgtcaaagctcccttaataattagttcctgagtcaaatataatactgacaaaaacattgtagatctttcatcttttgggggaatttttagtcataaatttaggattccactgtttctttaaagcaaagccactagtagctgagggtgatggtgtgtgcctgtagtcccagctgctcagggggcagaggcaggaggattgcttaagcccagaagtttgaggctatagtgagctatgattccaccactgcactccagcctggatgacacggcgagaccacatctcttaaagagaaaaactttttaaaaagcaaaaagcaaagccactaaaatatgttagcctaaagagggcatgcctgcttcattacagacggtatgacacatcttgagataaaaactaggatggctttcttatctgggttcctgactgctccttagctttgagttcttctagcttcttctcatagcgactcataaagtaatcatctggttcaatctctgcattcttcaagttttccatgatcttttccagtctgagcactgatcgggctccttcaatctttcttgtactcaagtacaaggtgaactcctggaaatccaggagcttacaggtgtccacagagcagatattccggatatcactagttctatccaaatgaggaaaaaacaccagtcctgacaacttctctaggtcctggaggctcacttggaattcagttaactggggctggaagccgatggcttcattgggtaccacaaaggcccctagcgccagtggttcggtagatactgagcttctgcgggccaggattaccttataaaggtgtgaggggactgccacgttgtcctcgccaatcacctggtaactaactattttctttccatcgcctctagtctgaggtaaggtcaaaggcccagataccacccaaacatcttcaaacctttctgtcagctctcgacagtacatttctattctgttccaatatccagaattattatcaaaatcctgaggcacaatgttagaaaggtaaaaggtttcagccatggctttacttgaaaatttgttatttcctgctggagccatgtgtcctcgtgaccacccacttccaacataatcttcattgaaggcactgaaggttggagggatattgggatcaggcttaaatttacaatgctttctgtctgcatcaccttctctggaacaaactttttatcttccttttgacctttctccgttcagtgccaagacaaccttccatgtagtccccattatcttgcttttggaaatatgttcaagaacccatctaggcacccgctttgcctgatcataagacaaagcgtgattagtgtaacaccttgcctctgttccagttaaagggaatccaaattgttccaagacagccttttctgcagatctgaatgccaattatgtaccaggtactgtgctggttagatgatggagaccaaaacagacatagtctcaagtcttatggagctaacaatcatccggctgcttccctgtcaacgctccctcagcgccctgactccggaagaactgcagggccgcgagcccagctcccgcagcgcccactacagccccagccacgaagccgctcagaaaacgacgggaaccccggaggcgggaagcgatactcttgatagccatcttgcccgaggtaccggccttttaccac

SEQ ID NO: 11708 - RNA, 2817 nt, Homo sapiens
  source 1..2817: mol_type = other RNA
ctgaatagctgggactacaggtgtgcaccaccacgcccagctaatttttgtatttttttgtaaagatagggtttcattatgttgcccaggctggtctcaaactcctgggctcaagcgatccacccacctcgatttcccaaagtgctgagattataggcctgagccaccatgcctggctgcagatccttcataggtttcttaatcttaagaacaaaaagctcacctggaaagcaagaacacatcaatttggcagtatctggtcactaaaagaactgtatctctggaggcaagcatgggctctaataaaccccacaaagtattgccgtctaattcccaaatattcctgactgtctctttccacagagctaaggagggttcaattcaaagaacattaaagtccctttggcttgcatagcagacgagaaaccagactcttcttgccaagcatgcctcaggcccacaaatacccatggaaataggtatatatttctgagtaaaaagccaccatccatgtcagaaaagatttgaatctacctcagctgtctttcttctcttagatctgtctgcctcatactttgtggatgactactttggaaaagtgaaactcaggtaagacactaagctctctaagcctcaattttctcacaggtaaaatggggatagtgtatttacctcagagagtcattgtgagacaacacatgtaaagcactgagcctagtatatagaacacatttaatgagcagaaactagttgctgagtgcttctacgtagacagaagtagagaaacgagcagattcatgagaggagaaaaaagaaacaaatatatagtgcatgtggacaggaactacacagaggatttctaaaagctgcctccaagaccaattcaggtcctagagggaaaaatgtacaacattgagttctgagaaggctgggcagatacatcacagacaatgcatggtttggaggcatgaaactaaacaaatgccttcccaatactctacatccacagggatacaaatgcagtgtcatctgtgggcagtcttcctgttaacttgacacaagatcagccctccatctgcaggtgtcaaagctcccttaataattagttcctgagtcaaatataatactgacaaaaacattgtagatctttcatcttttgggggaatttttagtcataaatttaggattccactgtttctttaaagcaaagccactagtagctgagggtgatggtgtgtgcctgtagtcccagctgctcagggggcagaggcaggaggattgcttaagcccagaagtttgaggctatagtgagctatgattccaccactgcactccagcctggatgacacggcgagaccacatctcttaaagagaaaaactttttaaaaagcaaaaagcaaagccactaaaatatgttagcctaaagagggcatgcctgcttcattacagacggtatgacacatcttgagataaaaactaggatggctttcttatctgggttcctgactgctccttagctttgagttcttctagcttcttctcatagcgactcataaagtaatcatctggttcaatctctgcattcttcaagttttccatgatcttttccagtctgagcactgatcgggctccttcaatctttcttgtactcaagtacaaggtgaactcctggaaatccaggagcttacaggtgtccacagagcagatattccggatatcactagttctatccaaatgaggaaaaaacaccagtcctgacaacttctctaggtcctggaggctcacttggaattcagttaactggggctggaagccgatggcttcattgggtaccacaaaggcccctagcgccagtggttcggtagatactgagcttctgcgggccaggattaccttataaaggtgtgaggggactgccacgttgtcctcgccaatcacctggtaactaactattttctttccatcgcctctagtctgaggtaaggtcaaaggcccagataccacccaaacatcttcaaacctttctgtcagctctcgacagtacatttctattctgttccaatatccagaattattatcaaaatcctgaggcacaatgttagaaaggtaaaaggtttcagccatggctttacttgaaaatttgttatttcctgctggagccatgtgtcctcgtgaccacccacttccaacataatcttcattgaaggcactgaaggttggagggatattgggatcaggcttaaatttacaatgctttctgtctgcatcaccttctctggaacaaactttttatcttccttttgacctttctccgttcagtgccaagacaaccttccatgtagtccctgtaatcccagctactcaggaggctgaggcaggagggtcacttgaacccagaaattcaagaccagccataggtgaaggttgagagagagaagaaacaatgatgctaggagtgtaaacttgaagaatctacccattatcttgcttttggaaatatgttcaagaacccatctaggcacccgctttgcctgatcataagacaaagcgtgattagtgtaacaccttgcctctgttccagttaaagggaatccaaattgttccaagacagccttttctgcagatccatccggctgcttccctgtcaacgctccctcagcgccctgactccggaagaactgcagggccgcgagcccagctcccgcagcgcccactacagccccagccacgaagccgctcagaaaacgacgggaaccccggaggcgggaagcgatactcttgatagccatcttgcccgaggtaccggccttttaccac

SEQ ID NO: 11709 - RNA, 4650 nt, Homo sapiens
  source 1..4650: mol_type = other RNA
ctgaatagctgggactacaggtgtgcaccaccacgcccagctaatttttgtatttttttgtaaagatagggtttcattatgttgcccaggctggtctcaaactcctgggctcaagcgatccacccacctcgatttcccaaagtgctgagattataggcctgagccaccatgcctggctgcagatccttcataggtttcttaatcttaagaacaaaaagctcacctggaaagcaagaacacatcaatttggcagtatctggtcactaaaagaactgtatctctggaggcaagcatgggctctaataaaccccacaaagtattgccgtctaattcccaaatattcctgactgtctctttccacagagctaaggagggttcaattcaaagaacattaaagtccctttggcttgcatagcagacgagaaaccagactcttcttgccaagcatgcctcaggcccacaaatacccatggaaataggtatatatttctgagtaaaaagccaccatccatgtcagaaaagatttgaatctacctcagctgtctttcttctcttagatctgtctgcctcatactttgtggatgactactttggaaaagtgaaactcaggtaagacactaagctctctaagcctcaattttctcacaggtaaaatggggatagtgtatttacctcagagagtcattgtgagacaacacatgtaaagcactgagcctagtatatagaacacatttaatgagcagaaactagttgctgagtgcttctacgtagacagaagtagagaaacgagcagattcatgagaggagaaaaaagaaacaaatatatagtgcatgtggacaggaactacacagaggatttctaaaagctgcctccaagaccaattcaggtcctagagggaaaaatgtacaacattgagttctgagaaggctgggcagatacatcacagacaatgcatggtttggaggcatgaaactaaacaaatgccttcccaatactctacatccacagggatacaaatgcagtgtcatctgtgggcagtcttcctgttaacttgacacaagatcagccctccatctgcaggtgtcaaagctcccttaataattagttcctgagtcaaatataatactgacaaaaacattgtagatctttcatcttttgggggaatttttagtcataaatttaggattccactgtttctttaaagcaaagccactagtagctgagggtgatggtgtgtgcctgtagtcccagctgctcagggggcagaggcaggaggattgcttaagcccagaagtttgaggctatagtgagctatgattccaccactgcactccagcctggatgacacggcgagaccacatctcttaaagagaaaaactttttaaaaagcaaaaagcaaagccactaaaatatgttagcctaaagagggcatgcctgcttcattacagacggtatgacacatcttgagataaaaactaggatggctttcttatctgggttcctgactgctccttagctttgagttcttctagcttcttctcatagcgactcataaagtaatcatctggttcaatctctgcattcttcaagttttccatgatcttttccagtctgagcactgatcgggctccttcaatctttcttgtactcaagtacaaggtgaactcctggaaatccaggagcttacaggtgtccacagagcagatattccggatatcactagttctatccaaatgaggaaaaaacaccagtcctgacaacttctctaggtcctggaggctcacttggaattcagttaactggggctggaagccgatggcttcattgggtaccacaaaggcccctagcgccagtggttcggtagatactgagcttctgcgggccaggattaccttataaaggtgtgaggggactgccacgttgtcctcgccaatcacctggtaactaactattttctttccatcgcctctagtctgaggtaaggtcaaaggcccagataccacccaaacatcttcaaacctttctgtcagctctcgacagtacatttctattctgttccaatatccagaattattatcaaaatcctgaggcacaatgttagaaaggtaaaaggtttcagccatggctttacttgaaaatttgttatttcctgctggagccatgtgtcctcgtgaccacccacttccaacataatcttcattgaaggcactgaaggttggagggatattgggatcaggcttaaatttacaatgctttctgtctgcatcaccttctctggaacaaactttttatcttccttttgacctttctccgttcagtgccaagacaaccttccatgtagtccctgtaatcccagctactcaggaggctgaggcaggagggtcacttgaacccagaaattcaagaccagcctaggcaacatagcaaaaatccatctcaaaaaaaaaggtaaaaaaaatacagatatacactttttatatactaacattttctgtttcagcaggaagattctatctgaataactcagtccatcattactgaaaacagaagaccttttacattaaaatcaagtaaaacacaggtacattgctccctattttcaaataatattaattggctctattttattgcctcaaaagtacacagctcacaagacttattatacaatataaaatgcccaggttttcttatatgcttgataaagttttcacttacatcagtttctgtctaacaccaagtacattccaagcctcctgttattctgctggttgctgtgcactctagaatggcacacactaactttaatatcagcattttaatatgcatagccatagcacacattttaaagcaaaggagaatatgtggaacacacagcaaattaaaaagcaaataacaaaagggaacaaaacaactgtgacaaaaggtaatatccttaataaataaaagaacttttacaaataaattcaaaagagaataccccaactgaaataggtaaagaataacttaccaaaaaagactaattcacagcatgttaaccctcattgataatcaataaacacaagtaaaatgagcattaaattggtaaagctcagtaatgctcaccataggtgaaggttgagagagagaagaaacaatgatgctaggagtgtaaacttgaagaatctacctagaaaccaatttgacattaattatcaagatctggcaattctacaggaccctatcaagacataaggacacatgaataaactgacacacctgcttacttctccagcatcatttcacatcaccttccccctcattcatctactggcactcttttagttccctaaaagaacaaaactcctgtccacattgggggcctccgaagatgcaaatgttcctttcttcctagaatgctcttctccatatcccatggcacattcaaccccttgcctaagtaatttccgttcactcttcagtccacttttccagagaagccttactaatcaaaatcaggttcttgtgttataatctctcatcacacttttttttttttttgagacacattctccctctgttgcctaagctggagtgtggtgctgcgatcttggctcactgcaacccccacctcctgggctcaagagatcctcccatctcagtcccccaagtagctggaaccacagaggtgcaccaccacgcccagctaatttttgtattttttgtagaaacgcggttttgccatgttggccaggctcatctcaaactcctgagctcaaacgcctcagcctcccaaagtactgggattacaggtgtgagccaccacgcccagcctctcatcaaactttttactgttccttaattatactacactaacttgcaatcacctcctttggaaaaattattgtaattatacatctaaaattatttgtttgatgggtcaacccactctcccaactcaaagtgtcactggggtagagatcctctactctggtcacacataggtccccaagggttaccacagtgccagacacatagcaggcacataaatatttgttaaggtaaaactgaatggtgctcattgctgtaatatttatgacagagcctcccaactagtgtgtcaagatatgggtattttcagccctgagacagctggaaagggtctggctttctggctgccaggcagggttgatttaaccagtaagttatataaatataattttctacatgtgctatgatatgaaaaaggttgagaatattaataatcatccctgttttaaatttggagacatctttcataaatactgttacttcagtttttttatccaaccacctacccattatcttgcttttggaaatatgttcaagaacccatctaggcacccgctttgcctgatcataagacaaagcgtgattagtgtaacaccttgcctctgttccagttaaagggaatccaaattgttccaagacagccttttctgcagatccatccggctgcttccctgtcaacgctccctcagcgccctgactccggaagaactgcagggccgcgagcccagctcccgcagcgcccactacagccccagccacgaagccgctcagaaaacgacgggaaccccggaggcgggaagcgatactcttgatagccatcttgcccgaggtaccggcctttt

SEQ ID NO: 11710 - RNA, 2451 nt, Homo sapiens
  source 1..2451: mol_type = other RNA
ctgaatagctgggactacaggtgtgcaccaccacgcccagctaatttttgtatttttttgtaaagatagggtttcattatgttgcccaggctggtctcaaactcctgggctcaagcgatccacccacctcgatttcccaaagtgctgagattataggcctgagccaccatgcctggctgcagatccttcataggtttcttaatcttaagaacaaaaagctcacctggaaagcaagaacacatcaatttggcagtatctggtcactaaaagaactgtatctctggaggcaagcatgggctctaataaaccccacaaagtattgccgtctaattcccaaatattcctgactgtctctttccacagagctaaggagggttcaattcaaagaacattaaagtccctttggcttgcatagcagacgagaaaccagactcttcttgccaagcatgcctcaggcccacaaatacccatggaaataggtatatatttctgagtaaaaagccaccatccatgtcagaaaagatttgaatctacctcagctgtctttcttctcttagatctgtctgcctcatactttgtggatgactactttggaaaagtgaaactcaggtaagacactaagctctctaagcctcaattttctcacaggtaaaatggggatagtgtatttacctcagagagtcattgtgagacaacacatgtaaagcactgagcctagtatatagaacacatttaatgagcagaaactagttgctgagtgcttctacgtagacagaagtagagaaacgagcagattcatgagaggagaaaaaagaaacaaatatatagtgcatgtggacaggaactacacagaggatttctaaaagctgcctccaagaccaattcaggtcctagagggaaaaatgtacaacattgagttctgagaaggctgggcagatacatcacagacaatgcatggtttggaggcatgaaactaaacaaatgccttcccaatactctacatccacagggatacaaatgcagtgtcatctgtgggcagtcttcctgttaacttgacacaagatcagccctccatctgcaggtgtcaaagctcccttaataattagttcctgagtcaaatataatactgacaaaaacattgtagatctttcatcttttgggggaatttttagtcataaatttaggattccactgtttctttaaagcaaagccactagtagctgagggtgatggtgtgtgcctgtagtcccagctgctcagggggcagaggcaggaggattgcttaagcccagaagtttgaggctatagtgagctatgattccaccactgcactccagcctggatgacacggcgagaccacatctcttaaagagaaaaactttttaaaaagcaaaaagcaaagccactaaaatatgttagcctaaagagggcatgcctgcttcattacagacggtatgacacatcttgagataaaaactaggatggctttcttatctgggttcctgactgctccttagctttgagttcttctagcttcttctcatagcgactcataaagtaatcatctggttcaatctctgcattcttcaagttttccatgatcttttccagtctgagcactgatcgggctccttcaatctttcttgtactcaagtacaaggtgaactcctggaaatccaggagcttacaggtgtccacagagcagatattccggatatcactagttctatccaaatgaggaaaaaacaccagtcctgacaacttctctaggtcctggaggctcacttggaattcagttaactggggctggaagccgatggcttcattgggtaccacaaaggcccctagcgccagtggttcggtagatactgagcttctgcgggccaggattaccttataaaggtgtgaggggactgccacgttgtcctcgccaatcacctggtaactaactattttctttccatcgcctctagtctgaggtaaggtcaaaggcccagataccacccaaacatcttcaaacctttctgtcagctctcgacagtacatttctattctgttccaatatccagaattattatcaaaatcctgaggcacaatgttagaaaggtaaaaggtttcagccatggctttacttgaaaatttgttatttcctgctggagccatgtgtcctcgtgaccacccacttccaacataatcttcattgaaggcactgaaggttggagggatattgggatcaggcttaaatttacaatgctttctgtctgcatcaccttctctggaacaaactttttatcttccttttgacctttctccgttcagtgccaagacaaccttccatgtagtcccttgcctctgttccagttaaagggaatccaaattgttccaagacagccttttctgcagatccatccggctgcttccctgtcaacgctccctcagcgccctgactcc

SEQ ID NO: 11711 - RNA, 2522 nt, Homo sapiens
  source 1..2522: mol_type = other RNA
ctgaatagctgggactacaggtgtgcaccaccacgcccagctaatttttgtatttttttgtaaagatagggtttcattatgttgcccaggctggtctcaaactcctgggctcaagcgatccacccacctcgatttcccaaagtgctgagattataggcctgagccaccatgcctggctgcagatccttcataggtttcttaatcttaagaacaaaaagctcacctggaaagcaagaacacatcaatttggcagtatctggtcactaaaagaactgtatctctggaggcaagcatgggctctaataaaccccacaaagtattgccgtctaattcccaaatattcctgactgtctctttccacagagctaaggagggttcaattcaaagaacattaaagtccctttggcttgcatagcagacgagaaaccagactcttcttgccaagcatgcctcaggcccacaaatacccatggaaataggtatatatttctgagtaaaaagccaccatccatgtcagaaaagatttgaatctacctcagctgtctttcttctcttagatctgtctgcctcatactttgtggatgactactttggaaaagtgaaactcaggtaagacactaagctctctaagcctcaattttctcacaggtaaaatggggatagtgtatttacctcagagagtcattgtgagacaacacatgtaaagcactgagcctagtatatagaacacatttaatgagcagaaactagttgctgagtgcttctacgtagacagaagtagagaaacgagcagattcatgagaggagaaaaaagaaacaaatatatagtgcatgtggacaggaactacacagaggatttctaaaagctgcctccaagaccaattcaggtcctagagggaaaaatgtacaacattgagttctgagaaggctgggcagatacatcacagacaatgcatggtttggaggcatgaaactaaacaaatgccttcccaatactctacatccacagggatacaaatgcagtgtcatctgtgggcagtcttcctgttaacttgacacaagatcagccctccatctgcaggtgtcaaagctcccttaataattagttcctgagtcaaatataatactgacaaaaacattgtagatctttcatcttttgggggaatttttagtcataaatttaggattccactgtttctttaaagcaaagccactagtagctgagggtgatggtgtgtgcctgtagtcccagctgctcagggggcagaggcaggaggattgcttaagcccagaagtttgaggctatagtgagctatgattccaccactgcactccagcctggatgacacggcgagaccacatctcttaaagagaaaaactttttaaaaagcaaaaagcaaagccactaaaatatgttagcctaaagagggcatgcctgcttcattacagacggtatgacacatcttgagataaaaactaggatggctttcttatctgggttcctgactgctccttagctttgagttcttctagcttcttctcatagcgactcataaagtaatcatctggttcaatctctgcattcttcaagttttccatgatcttttccagtctgagcactgatcgggctccttcaatctttcttgtactcaagtacaaggtgaactcctggaaatccaggagcttacaggtgtccacagagcagatattccggatatcactagttctatccaaatgaggaaaaaacaccagtcctgacaacttctctaggtcctggaggctcacttggaattcagttaactggggctggaagccgatggcttcattgggtaccacaaaggcccctagcgccagtggttcggtagatactgagcttctgcgggccaggattaccttataaaggtgtgaggggactgccacgttgtcctcgccaatcacctggtaactaactattttctttccatcgcctctagtctgaggtaaggtcaaaggcccagataccacccaaacatcttcaaacctttctgtcagctctcgacagtacatttctattctgttccaatatccagaattattatcaaaatcctgaggcacaatgttagaaaggtaaaaggtttcagccatggctttacttgaaaatttgttatttcctgctggagccatgtgtcctcgtgaccacccacttccaacataatcttcattgaaggcactgaaggttggagggatattgggatcaggcttaaatttacaatgctttctgtctgcatcaccttgcctctgttccagttaaagggaatccaaattgttccaagacagccttttctgcagatccatccggctgcttccctgtcaacgctccctcagcgccctgactccggaagaactgcagggccgcgagcccagctcccgcagcgcccactacagccccagccacgaagccgctcagaaaacgacgggaaccccggaggcgggaagcgatactcttgatagccatcttgcccgaggtaccggccttttaccac

SEQ ID NO: 11712 - RNA, 3084 nt, Homo sapiens
  source 1..3084: mol_type = other RNA
ctgaatagctgggactacaggtgtgcaccaccacgcccagctaatttttgtatttttttgtaaagatagggtttcattatgttgcccaggctggtctcaaactcctgggctcaagcgatccacccacctcgatttcccaaagtgctgagattataggcctgagccaccatgcctggctgcagatccttcataggtttcttaatcttaagaacaaaaagctcacctggaaagcaagaacacatcaatttggcagtatctggtcactaaaagaactgtatctctggaggcaagcatgggctctaataaaccccacaaagtattgccgtctaattcccaaatattcctgactgtctctttccacagagctaaggagggttcaattcaaagaacattaaagtccctttggcttgcatagcagacgagaaaccagactcttcttgccaagcatgcctcaggcccacaaatacccatggaaataggtatatatttctgagtaaaaagccaccatccatgtcagaaaagatttgaatctacctcagctgtctttcttctcttagatctgtctgcctcatactttgtggatgactactttggaaaagtgaaactcaggtaagacactaagctctctaagcctcaattttctcacaggtaaaatggggatagtgtatttacctcagagagtcattgtgagacaacacatgtaaagcactgagcctagtatatagaacacatttaatgagcagaaactagttgctgagtgcttctacgtagacagaagtagagaaacgagcagattcatgagaggagaaaaaagaaacaaatatatagtgcatgtggacaggaactacacagaggatttctaaaagctgcctccaagaccaattcaggtcctagagggaaaaatgtacaacattgagttctgagaaggctgggcagatacatcacagacaatgcatggtttggaggcatgaaactaaacaaatgccttcccaatactctacatccacagggatacaaatgcagtgtcatctgtgggcagtcttcctgttaacttgacacaagatcagccctccatctgcaggtgtcaaagctcccttaataattagttcctgagtcaaatataatactgacaaaaacattgtagatctttcatcttttgggggaatttttagtcataaatttaggattccactgtttctttaaagcaaagccactagtagctgagggtgatggtgtgtgcctgtagtcccagctgctcagggggcagaggcaggaggattgcttaagcccagaagtttgaggctatagtgagctatgattccaccactgcactccagcctggatgacacggcgagaccacatctcttaaagagaaaaactttttaaaaagcaaaaagcaaagccactaaaatatgttagcctaaagagggcatgcctgcttcattacagacggtatgacacatcttgagataaaaactaggatggctttcttatctgggttcctgactgctccttagctttgagttcttctagcttcttctcatagcgactcataaagtaatcatctggttcaatctctgcattcttcaagttttccatgatcttttccagtctgagcactgatcgggctccttcaatctttcttgtactcaagtacaaggtgaactcctggaaatccaggagcttacaggtgtccacagagcagatattccggatatcactagttctatccaaatgaggaaaaaacaccagtcctgacaacttctctaggtcctggaggctcacttggaattcagttaactggggctggaagccgatggcttcattgggtaccacaaaggcccctagcgccagtggttcggtagatactgagcttctgcgggccaggattaccttataaaggtgtgaggggactgccacgttgtcctcgccaatcacctgtaatcccagcactttgggacgccaaggcgggcagatcacttgaggtcaggagttcaagaccagcctggccaacatggtgaaaccccatctctactaaaaaaaaatacaaaaattagctgggtgtggtggcaggcgcctgtaatcccagctacttgggaggctgaagcagaagaattgcttgaacccaggaggcagagggtgcagtgagccgagattgcaccactgcactccagcctggccgacagagcaagactccacctcaaaaaataaaaataaaataatgccaacccaaagatcaggggtcacagtctctgttctgtttgtaggacaaaggacaaaggaatgccatgagtgagtcctggttttttaatagacaagaaaagctgtcattttctcttcatctcataatcagaacttctggtgctccaaacattcaaaggtcaaaactgcaggcttgggtactcccagctctggtaactaactattttctttccatcgcctctagtctgaggtaaggtcaaaggcccagataccacccaaacatcttcaaacctttctgtcagctctcgacagtacatttctattctgttccaatatccagaattattatcaaaatcctgaggcacaatgttagaaaggtaaaaggtttcagccatggctttacttgaaaatttgttatttcctgctggagccatgtgtcctcgtgaccacccacttccaacataatcttcattgaaggcactgaaggttggagggatattgggatcaggcttaaatttacaatgctttctgtctgcatcacccattatcttgcttttggaaatatgttcaagaacccatctaggcacccgctttgcctgatcataagacaaagcgtgattagtgtaacaccttgcctctgttccagttaaagggaatccaaattgttccaagacagccttttctgcagatccatccggctgcttccctgtcaacgctccctcagcgccctgactccggaagaactgcagggccgcgagcccagctcccgcagcgcccactacagccccagccacgaagccgctcagaaaacgacgggaaccccggaggcgggaagcgatactcttgatagccatcttgcccgaggtaccggccttttaccac

SEQ ID NO: 11713 - RNA, 3118 nt, Homo sapiens
  source 1..3118: mol_type = other RNA
ctgaatagctgggactacaggtgtgcaccaccacgcccggctaactttcgtatttttagtaaagacggggtttcaccacattggccaggatggtctcggtctcttgacctcgtgatccaccagcctgggcctcctactcactttttaagtagactctttacttattattgagttttaagagctatttgtatttttttttacccaagtcttttatcagatatgtgtttgcaaatattttctcccagtctttggcttatcttttcattctcttaacagtgtctttcacagagcataagtttttaattttcatgaagccaactaattctttttttaatgattcatgcttttgctgttatatctaaaaagtcatcgccaaacccaaggtcacctagattttctcctatattatcttctagcagtttatattagtacttttgtattttacatctagattcatttttttacatgtggatgtccagttatttcagcaccatttgttgaaaagagtaaactttctccattaaattgcttttgctcctttgtctaagatcaattgaccatttttgtgtaggtttgtttctggttctctattctactccactgatttctctattattttaacaataccatactgtcttgattactgtagctttatagtaggaagaagttggatagcagcactcctccaactttgttcttcttcaatattttattggctattctgagtcttttgcctttgcacataaacattagaatcatcttatcaatgtccacaaagttatttgctgggatcttgattgggattgcattgaatctacagatcaaactggggaaaactaacatcttaacaatattgagtctttctattcatgaacatggaaaatcttcccattcatttacagcttctttgatttctttcctcagagtgttgtcattttcctcatagagatcttgtacatatttaattaggtttatatgtaagtattttttggtgtttcctctgtccctctgccttttccagtagaagcttccttttgtgttcctgctatattatctttgccctccttctgtccatggacagaaggacatttttgctcctccttaggtccatgactcaagctgcttttgacagaaaataaattctggctctgtgatttcttttcatttgaatgttttatcttgaatgatacattgttcatctgaataccttttaccagattctttattttagcttcatacagggagaattccaaatcccaggtcctgttgtgcttcatagattccatctgttctttaaaatgcttcagatcctgcgctaaacagggagaaattctgaagcagaacttgagctccaagttcgagaagctgtcttttttcgagatgtccagtaaaaactgcatagtgagggtcatctcatcattcccttcctgctcctttacctccagcagcctttgcacttctctgcgggactccttccccagccggctttggtcctctttcaccaggtaagacatggcatgaaaaaagtcctggaagctgatgtggcggaagctgtagaacttcttgatggcaagtcccaattggtagtcgttactactcaggaaagcggcaagcctggggccatctaaattatgtttcctgagctcagcttcttcaaataggaacctctggtgctgaatcccttcagctgctagggagcacagactcctcaggaccctgtgccgggaaagctcggagcagcccccatcatcatcgggcggcagaaaggtggagacgtaagccatgaagatgtcagtgctgtttctaggtgtctctaagacaactttgcctctctccatctgcccctgcagccaggagcagaccacccagcaaatgcctggaacctgacacgctttgtagagaatgtcatttttctgtacaatgtcgaaggcacggtcagcttgcttctcatccgtgaaataggagctgaagtacctcgccctctcctcctcagagaagcctaggatatggacatgacgtgcttgtttcagcaagggctccagattcctcaaagccaggggccgggtggtgatgagaagggagcacgtggggagtgtatgtctcctaattagaaggtgcagcaggctctccttgggactcaaacccctcttcttcaacttttcttcaaagggcctctgcagctcatcaaagccatccaggatgaacaggagccgctctggctgcctcagaatctctgtgacaggggcttgattgtccccgcagcaccagaaaaggagctgctccagtttgctctccagcagcaggaccacttctttgcagcttacataaaagacataatcaaaccggcctgggtacagagtaccggtggcccagtccaacaccatttttctggcgagagttgtctttccagtgccagccgacccctgtagcacaactaaggatggggccagtgagggcttttcccctgaatcaaatagagcctccaccgtgacagactccagctcctgctccgggaaggggcaggcaagtgattctgggctctctgagctgggcttggccaccaggagcacctggttgtatctgccattgactcctgcttcctgccattcctctaggcagcgcacatgctctcggtatacttctctgtaatcatgcagacaaatatggctgagctggtccacaagttccaacaggttcatgaccttcaagcccttgaggacaactttcacagcctccttttctccatactttgaaatcagtaattctgccaggtccaccggaatcaggccctccaactcccctctggccagtgggggctggccctcagacagggtcatatcccgtaagtagaactttaacttcttgaaatcgttctcctcaaggtcactcaaggcccagagcaatgcctcccggggctttctggccttggccatggccatggtgatctgggggaaggatcaagtccagaccagaagaccagtgacctggagaaagaggcaaaaggagaggtccactgctgagaggcccaccctgctttctgggggcttggccaagttatagagcggaggccagggagagacgagatacatgtgcaaagctccaagaaagacaagcagat

SEQ ID NO: 11714 - RNA, 2284 nt, Homo sapiens
  source 1..2284: mol_type = other RNA
ctgaatagctgggactacaggtgtgcaccaccacgcctggctaatttttgtatttttagtagagacaaggtttcaccatgttggccaggctggtcttgaactcctgatctcaagtgatccaccctccttggcccccaaagtgctgggattacaggcatgagccaccacacccagctaacttcagtttttgatgagacagaaatgggaaaatgtagactggtttactactttatcttatgatacaatgttattgtagtataatatactatagactacccattaaagaaccaggaaggatattccgctagccttaagaagtaaatattgaatataaatataactttctacctcatctataacatattgatacattttattacaaagaaactcacacataaatgatttgtcctatttatcataataggccaccaatcactaggagccaagcttcatcagcttaagtcctaggtagcatgtctcaatgcatacatatttatatgttattaaccgtgtttcttttctttttttcgagacagagtgtccaggctggaggtgatctcggcttaccgcaacctccgcctccgggttcaagtgattctgccgcctcagccttcctgggtagctgggattacaggcacgcatcaccacgcccggctacttttgtatttttagtagagatagggtttctccgtgttggtcaggctggtctcgaactcccaacctcaggtgatccgcccgcctcagcctcccaaagtgctgggattacaggcatgagccaccatgcctggctattaaccttgtttctaacttcagcattgcacatctccttagtaaagcagtagccattaacaagtcaggtccaacaaccattttcctctggtcctcaagcagagactcagagccagttacacataaactatttcattataacatgaaaatagcaagccttgggctattgcaaaaggcttttcaaatgttgacctctaacttggagaaaatagagggaagcagaaatatagggtgctaatttgtgctataacctggtctcatgtcgtggtatattcccagttgcaacattttaaatttataagtgagaaagtaaaacaaagcttcatatctgtgaaagtgaaaaattgtccagaagtcttctattcaaagaccaattagctttttcttcccaataacttatcagaaagaaatgggtacttagaaacctaaggggttctttaaataggagtcagaaaaaatatataaaaataaaaaacaaagcaagaaagaacattgtataaaaataaaatgttctttaaagatgactgccctctcttgaaagatgagtgctatattaaaagggtagatgtatctctataactcatcgtgtttatatgtaaattctctggcagatataaacccatctttgtcttcatcttctttatcaaaaatatcctccaccaaagcatcatgatgactttcattcaccaccgcaccatgtttttcaaactccttctttaaatatgctttaacctcatctttagagagtttccagtcatcattaagatccatttcttggaatgattcatgggatcttggtccatttcgaatctccaggagatcaatattaaatatcagtgtactttctgggggaattttaccatttcagatctagacagagatgtgacatgcgctaggttgttgataaaactggtatctttccaaaagaggcatgcaagcatgtactaaaagacttttccttcttttccatagcccagagcaggaggaatgatgagctttctcttctctcctacacacattcctttcaagccctggtcccaacctttgagagcctccaggatgcccagggtaaaccaaatgggctgaccattgttatgtttgtgagtggagtgaaataaggagccgtccttttctaagtagccttcatagtggaccaacatcaaatcccctcctttggtcttgcgatggcagatgaatggcttctggagaacttcaattttcacttctggttcagggatcaaagccccaatcaaagaagtgacgaacagagtcaagaccgcgttccacaagaaaagcctcatgttgctgaagcaaggaaagaagtccctacaaaagcagcgaaaggtccctcgacttcatagatttaagaacgtagttcaaggcttacggacaagggcttcagacaagttcaggactcccccttcttagaagacgtggcacatttaccaccaactcttttctcaagggtcacgaacctacctttaaagagttaagc

SEQ ID NO: 11715 - RNA, 2192 nt, Homo sapiens
  source 1..2192: mol_type = other RNA
ctgaatagctgggactacaggtgtgcaccaccacgcctggctaatttttgtatttttagtagagacaaggtttcaccatgttggccaggctggtcttgaactcctgatctcaagtgatccaccctccttggcccccaaagtgctgggattacaggcatgagccaccacacccagctaacttcagtttttgatgagacagaaatgggaaaatgtagactggtttactactttatcttatgatacaatgttattgtagtataatatactatagactacccattaaagaaccaggaaggatattccgctagccttaagaagtaaatattgaatataaatataactttctacctcatctataacatattgatacattttattacaaagaaactcacacataaatgatttgtcctatttatcataataggccaccaatcactaggagccaagcttcatcagcttaagtcctaggtagcatgtctcaatgcatacatatttatatgttattaaccgtgtttcttttctttttttcgagacagagtgtccaggctggaggtgatctcggcttaccgcaacctccgcctccgggttcaagtgattctgccgcctcagccttcctgggtagctgggattacaggcacgcatcaccacgcccggctacttttgtatttttagtagagatagggtttctccgtgttggtcaggctggtctcgaactcccaacctcaggtgatccgcccgcctcagcctcccaaagtgctgggattacaggcatgagccaccatgcctggctattaaccttgtttctaacttcagcattgcacatctccttagtaaagcagtagccattaacaagtcaggtccaacaaccattttcctctggtcctcaagcagagactcagagccagttacacataaactatttcattataacatgaaaatagcaagccttgggctattgcaaaaggcttttcaaatgttgacctctaacttggagaaaatagagggaagcagaaatatagggtgctaatttgtgctataacctggtctcatgtcgtggtatattcccagttgcaacattttaaatttataagtgagaaagtaaaacaaagcttcatatctgtgaaagtgaaaaattgtccagaagtcttctattcaaagaccaattagctttttcttcccaataacttatcagaaagaaatgggtacttagaaacctaaggggttctttaaataggagtcagaaaaaatatataaaaataaaaaacaaagcaagaaagaacattgtataaaaataaaatgttctttaaagatgactgccctctcttgaaagatgagtgctatattaaaagggtagatgtatctctataactcatcgtgtttatatgtaaattctctggcagatataaacccatctttgtcttcatcttctttatcaaaaatatcctccaccaaagcatcatgatgactttcattcaccaccgcaccatgtttttcaaactccttctttaaatatgctttaacctcatctttagagagtttccagtcatcattaagatccatttcttggaatgattcatgggatcttggtccatttcgaatctccaggagatcaatattaaatatcagtgtactttctgggggaattttaccttttccttcttttccatagcccagagcaggaggaatgatgagctttctcttctctcctacacacattcctttcaagccctggtcccaacctttgagagcctccaggatgcccagggtaaaccaaatgggctgaccattgttatgtttgtgagtggagtgaaataaggagccgtccttttctaagtagccttcatagtggaccaacatcaaatcccctcctttggtcttgcgatggcagatgaatggcttctggagaacttcaattttcacttctggttcagggatcaaagccccaatcaaagaagtgacgaacagagtcaagaccgcgttccacaagaaaagcctcatgttgctgaagcaaggaaagaagtccctacaaaagcagcgaaaggtccctcgacttcatagatttaagaacgtagttcaaggcttacggacaagggcttcagacaagttcaggactcccccttcttagaagacgtggcacatttaccaccaactcttttctcaagggtcacgaacctacctttaaagagttaagc

SEQ ID NO: 11716 - RNA, 2040 nt, Homo sapiens
  source 1..2040: mol_type = other RNA
ctgaatagctgggactacaggtgtgcaccaccacgcctggctaatttttgtatttttagtagagacaaggtttcaccatgttggccaggctggtcttgaactcctgatctcaagtgatccaccctccttggcccccaaagtgctgggattacaggcatgagccaccacacccagctaacttcagtttttgatgagacagaaatgggaaaatgtagactggtttactactttatcttatgatacaatgttattgtagtataatatactatagactacccattaaagaaccaggaaggatattccgctagccttaagaagtaaatattgaatataaatataactttctacctcatctataacatattgatacattttattacaaagaaactcacacataaatgatttgtcctatttatcataataggccaccaatcactaggagccaagcttcatcagcttaagtcctaggtagcatgtctcaatgcatacatatttatatgttattaaccgtgtttcttttctttttttcgagacagagtgtccaggctggaggtgatctcggcttaccgcaacctccgcctccgggttcaagtgattctgccgcctcagccttcctgggtagctgggattacaggcacgcatcaccacgcccggctacttttgtatttttagtagagatagggtttctccgtgttggtcaggctggtctcgaactcccaacctcaggtgatccgcccgcctcagcctcccaaagtgctgggattacaggcatgagccaccatgcctggctattaaccttgtttctaacttcagcattgcacatctccttagtaaagcagtagccattaacaagtcaggtccaacaaccattttcctctggtcctcaagcagagactcagagccagttacacataaactatttcattataacatgaaaatagcaagccttgggctattgcaaaaggcttttcaaatgttgacctctaacttggagaaaatagagggaagcagaaatatagggtgctaatttgtgctataacctggtctcatgtcgtggtatattcccagttgcaacattttaaatttataagtgagaaagtaaaacaaagcttcatatctgtgaaagtgaaaaattgtccagaagtcttctattcaaagaccaattagctttttcttcccaataacttatcagaaagaaatgggtacttagaaacctaaggggttctttaaataggagtcagaaaaaatatataaaaataaaaaacaaagcaagaaagaacattgtataaaaataaaatgttctttaaagatgactgccctctcttgaaagatgagtgctatattaaaagggtagatgtatctctataactcatcgtgtttatatgtaaattctctggcagatataaacccatctttgtcttcatcttctttatcaaaaatatcctccaccaaagcatcatgatgactttcattcaccaccgcaccatgtttttcaaactccttctttaaatatgctttaacctcatctttagagagtttccagtcatcattaagatccatttcttggaatgattcatgggatcttggtccatttcgaatctccaggagatcaatattaaatatcagtgtactttctgggggaattttacgtggagtgaaataaggagccgtccttttctaagtagccttcatagtggaccaacatcaaatcccctcctttggtcttgcgatggcagatgaatggcttctggagaacttcaattttcacttctggttcagggatcaaagccccaatcaaagaagtgacgaacagagtcaagaccgcgttccacaagaaaagcctcatgttgctgaagcaaggaaagaagtccctacaaaagcagcgaaaggtccctcgacttcatagatttaagaacgtagttcaaggcttacggacaagggcttcagacaagttcaggactcccccttcttagaagacgtggcacatttaccaccaactcttttctcaagggtcacgaacctacctttaaagagttaagc

SEQ ID NO: 11717 - RNA, 15519 nt, Homo sapiens
  source 1..15519: mol_type = other RNA
ctgaatagctgggactacaggtgtgcaccaccacgtccagctaattttttgtatttttagtagagatggggtttcaccatgttggccaggctggtctcaaactcctgaccttgtgatctgcccaccttggcctcccaaagtgctgggattacaggtgtgagccaccatgcccagcctatttttttatttattttttgaagggacagggtctcgctgtgttgccagagttggtcttgaacttcctgggctcaactgatcctcctgcctcagccttccaaaatgctggtattacaggtgtgtggcactgcacctggccagctttattttaaggcactaataataaagggtatgaaaaaagctaggaataagtcagatctttccagaaataaaagacaattttaaaaaacatcagttaacctgtctggcctatttcaacatctaaagaggatagagaatgtaaaagttttcatgcctacctgattcagctcttttccattctcccaaacacttatttccatgtctcagatttacatttcctcaaaaggcagtagagatttggaaacaacaacaacaacaacaacaacaacaacaaaaccaccccaaaacaagcaagcctagtttgtagcctagtctcatgattaatgaattccctaatgctggcatttagcccacatactgagaggccggaactgtaacaaggtgctcttttctagtgttgtaaggggaaaatgtataaggaaaattaatttttcataatcaggtaaatataatttgttaatagcaaaacaagaaattccggagagaaaaaagatttactctgaaacaccagttccagcaggatttccctacaccttccaacgtattctactttgccatgagaaaaaaactaaataaataaaatggggttcaagtcagttaggcgagcaaacaccaaaaaacgagtgatttcattgtggaggtaggcatgatggggcaggatttccctcaagtggaaatgcttcctgtgcacacacacgtatacatgcacacacaaacctgtacactcacactaatttcaaaagcatggatgtggggaaagccctgccagcatgactagacatgaggagttagcccatctgcctgtatctctacacaggctctgacgtacattccacacccatagacagtcatgcacgagagccagcctggcttgcacacagactgagaatcagatctggagactcctagagctgctgcttctacaggaattattagtaactgcaggattatacttcctgttgatgtgcagggtttttatcttgctcttctttccagacatctccccttttcaagagtactaaatcttgatttagtggagggactaatcttgattcttcgatgggcatgacttagaacaggagctacaggaattaaaactagcaacaatagggcccctttgggattggggtgaagaagtatttcaggatttaaacagtttctgtgggtggggcggggggaaagcagagttcttggtggaagtggatgacctctgtgaaggagatgaaaatgcctccaagtccagaaatcaatataaacaaacaaacaaacaaacaaaaatgaacataacttaaaggggcttcaactaaatatcactgcaactgagtttgttgactcaagaaattctgctctgacgcagggaattgaaatataagaactgataatatttcttcttcagaaggctaagctgggagtgccatggcgggtattgagggtgggatagagacaagaggcttgaggctcaggttttgctcctagggtttcttgcctgattttgaagggaagggtgctagagcaaatggatcagcagctggcagctccgtagtcctggaggaaagggatgtgatagaaacagacccagctatcgactgcttgttggtttgtgaaacaattttgtaggcagcaatgggctgggcttctggacttggctcgtcttctgggctatagtgacgggaatacttggataaggactgggggcggaatggtttgccagccatggggcctgagacagcttctttctggagctgaggtcctttgtttctgtcattagaatgacccccagattccaggcaggatcccctgggagagatgctgtccagatggtctgctgcttgtacagaatgggacaggaggttagactgttgcacaaaaccagctgtggaatactgagcttggacagaggtgtacacagctctctcacggcccgcgggcagggggacatcacctgtctgactgaggagaccggtctgtgcaggcagctcctgggaggtgcattggataactgttaactcctccatgcttttcttcttagtgaaaggagctctcaaaaacacgtctgactcctctggctgggaaggagccatactgctcttggagacaaatggggctttggagaaaatgtccatgtcatcatttggaacccttgagctcctgaagggagctatggcaaaaacatctggctcactgagcccatcagtggctggctgtgtgaaggcttgaaactggttctttcttccaccttgcactgtctttgcttgctcaggagagacttctggtggagcgaatggaacggctcctcccagcttccccggggggggtctgcagctctcatcttcttcttcagactccataaggagaggccgagacccactgcagtccagcatgtctccttcaaggtcagtcccttcctcttcgctgctgtggaatgagctgttgcttgaagggccatctctggccaagtagtcagattctaagttgttctgagtctttgtgccaggtactctggaggggtctggatacagcggaaggcctttaacacccagtgattctttaaagtgctctacagttattacaggacagggattggactccctctggagatctagaaaagcataaaatgcagaattaatgtgtaggtcaattcaactctatttggaacatttaatggtcaacccgcggcaaaaacattgtgggaccaaataatagatgttgaaaatgcaacaggaaaaacataaaaataaaagtcaggcaaggaaactgcacacaaactggaacacaatcaaccactgtctcacgttttggaacatgataggcacgacgtacaggaaaggagatgaagatgttaggcacacagacattcagcgtaactatgcaatgctcctacacacagggccaggcacggacacctgctctacctggcactggctcattatggaatgaaaacaaacccagtcattcatctccacatataccatgacagttttggattatgtagaaacactgtctggggatgactcaattcagaatctggcatgtggtcatccgcgccacatgcagagggacaaactctctgaaaagaagcagaatgtggctgcttgataaatgcaagtttacttgatgacttacatcacaagcactactcaaagagcatacgagtgcccaaaatataaatactgaaggtaccttctgaggggagcatacagcatcaaaatcagaccaaataaatcaccttcagctggagttgccccagaattttgttttcagtcttctaagttcataaagatctcctctgcttaaatgaatctgccataaagttctttaagcagaaggagtaaaatgcatgggccattacagaagcattagcaaactccaatatactagtctatttctatctaggtagaggtgcctcagggtgctctggcttttaaaatcaaatagacaattatcagaatgcaagagagcttaccttccaagaaatattagcaggttagaagtatgtcattgggcacatgttagcaagagggcaggaaaaaggcatatgtaactaagcaagaagaatccagagaaagggtggttgggggtaaaggtatcatttcatcatgggctcagtaaagagatactactggagtttcccaacccaccaggataagaatattagatacaatgatttggagccatagatgacccagaacctctgtagagatggaactcaatgatccccttcccatactgaccctctcccctcctatgcaaaccattagctagcagaaatttctgccaaaaattatcccctgctaaagtttctgcatgaattaagcacacagaccacagcagaagaggcattaaaatcagtttattgggaaaccagtcacttagagacattacattgtaaagagaatgtagagagaggtctgaacattttataagatactgtacaaaaatactatgtttctctgaatcctataactttttagcagtgcttctttttaaacagttctgaccttaaatattgttttcagaaacagaacaaaaatgtgtttgtcctccatttttattttcctttctaacagtttgaatgcgttcagtgaattccagattggggcgttaagttaaattctgtactggtgccaaatggctttcagaatagtatttgaagaataagattttgaaaagaataaatttttccttgtattataattttagtatgtgcagctacatggtgatacgaaagcatcagtcagtggacaggaaataaacagaataccttcttccttgcgatttatgtggacagacataatcctaatttctcaggcaagtaaattgatattagatttgtctcagtgataccaagatgataatttctgggaggaaattcaaataaaagggagaaaaataagttttccaaaataaggtttgcagagccttaaagaaggacaagagggccctaaaactccttgaaccaccttcctcacatagtatcagttggacaaagttttcagttgccaaaacaaaagcacaatttctcatcttccaaaactaccttgaaagttgatgttattaagcttgttctgcaggagagcaaaatatctcttagggaaaaaaaatggaaaacttagtcaagccagtgaccaactctggcatcatacaggtcaataatccaatgaacactagtttgaacagagtcagtgttttttggaaatttaaactgaattcagttaaaacaatttgtgcacagagactggcaaaaaagcagctatctattgaaccaggggcactttggatgcctgaagtgctagattacattttgagaactaggaagtaccaaggggtgtgtgtatgtgcccatattcagggttggagaggatggaagaacatgtctaacccatcaaaattatttgttaaaaagtgggtttttggtcgagaacccatttggaaaaccttccaactcagagcatattctatgaccttcatgatgagtactgggaaaatcagacttaaaattccaacaactttgaataatttacaaaaacagtcacaaaaacaccagaatatcaagtttgaagggaaaattagtctcctgtccttcaaaacaaggacaagagctatttcctatctttctttcagcatcaacaggctttgtaggaatggaaaagtacatttaaagggttgtcctgagaaggccaagtcccttaacctttctattcttgttagaggaggtacagtgtggctgaggcggagagcaaccacactttgcaactctccaggcctggcactctgaagggcaaagaaatgccagagaatatgggggaagcccagacctccacattcccttaaggaattctggtggtggcagcaccagaaacaaggtagtcgagagaaggataaattccaaatatactagaaacagaaggtaaccattaaatcttgttggcagataaaagtctttttttgagtatgtgaatgtgttcttacagggaaaatgtgttttcagggtgaacagttcctttatatgaaggtagcattgtgtcaacaagaaaacgtgtttgaagcagtctctttactagcattgaaggatttatactaacctaaccacatgccttgacccagttcctttggtaaccaatggcacgtcatagcagataccctgtggccatagagctcagtaaacactgcctgttgtacctcaggggctaaagcccagggcctggcttcatagtctgcacagggtcttacttatcatagagcctaacgtagggttttgttataattccctcaaactggatcatgcctctttttattttggtttcacacataaaattaagcaagaagtcaaaacatacttctttttcttgctctgatgtaggactgtgtgccaggttaggcacgttgacactttcaatatgggtaactccatattagtctattttgaggctccaaattatgtagatttcagcaagaactcacatgcttcagggaagagaaggagttcctaaaatacctgacaacttggcaactatcctcaccagctccctattcacttccaaagcaacccaaagtgctgaatcatttaggatgggtttcccctggaaactccatctgattgacatagtgagggccatcagaatgctccctacagaattaaaatctgaagacttaaatgtcaggctggatattccttaatgaaatacatcacacaacaccagaagtttacttttcctcataccaaaaactgaaagaacggttacagggagtatcaaagatatgattcttgccaaaaacagaaaacgaagacttggagcattgagaagaagccttctcacatatagttagtaaacagaaagcaaaatatcccttcacaagaacttggaaatgcagcagcaattgaaacgtaaaattttagaaccaaactggggaaatcaagagacgtacatcaaactaataattaccatgaccttctagctcacataacaaaattaagcatttggttccaccatatattaggtagctgcattaaaacccacgactgggaaatgagggacctcatggaagccaaaaatggccagctgtgcctctcaggccaatgaggcaattaaatgagtgagttttctcactggggataaaattattcttgccaacacaaaatgtttaattaagttggcctgggtatattagggattaagttagaggagggaagctgcaaacctgcgctccattttacaaccctgagtctggtcatatccagtgtaggctggcaggcgtcttattctccttgagactaaaacaggggttttactctctcaggtagccatgattcattaatatgtcctcagtgtgtagctatacttttcttgtgcccaggtacttattgtcactcaatactgtgattaaatcctttctgcaaaaaagtgggttttcagctcaggaaaagagcaacttattttaagttatttacatctctaaacatcatgctcccatttgaacagataaaagtctttattcccctgtatgtttacataagaaagttctttacagacttttttttatacaatacttgtgcagcaatgttcaaatttcacgtttttactgcataagatatcttcatgtacaactgtatgctttgtcttcttgggaaggacgcgttaaagacctatgataaacacacatccacatgacaaaggagagtgcaatagggcagagtagaatactcacaggaaaagagtaaattcaggtcactacatcaaagtgtgaaccaagaacgtgtctttaattctagcaactaccaccatttggtaacttctttgcataggttagcattacccaaggagcctccctatcccgtattagtgaaaggaaatctgggagaagcaaaagaggtttcttgttatagatttcctagcactcattctgatttaagaaatctaagcacatccaacttcagaaacattactaatgtggaaaaagaaaaggctgactttgtgttgataaaattatagcctttagagaggaataaagatagctttgcagtatctggagtgtttcaggaaagcttccattctaaatattcatgtgatagtttttctgttctgccaggcagcctctaatttgcttaacccggcacactgggcaatcctgtcattttcatcccaaagctcaaagttagtggctatgggagcctgataatcttgcagacagagaaggttaaggactctgggaaatcacagaaaaaccttatcaagagagactttattttggcccaaggtatctatagcatgtatttatttagctgagtgcagatccctccacatcataggctgtcagccccaaagatcccttcattcccacagcactgctgaaggcagaactgttcctaacctggggaaggttatattggttgatcaattatctgtcaggagagtaggaaataagtaatcaaaacaaccaaaagtattaataataaaacaaatattacatcttgagaaagtagttcgtttcttgggtttgtttttccacaagtattagcaatccaagttgtgtaattctaattcaggaagagcgaagtccaatatcaaataacactgaacaaagtgacaacttctttcagaggtgttttaatacccatatctttcaatgttttaaaccattctaaagactaaggaatcacagaagtttccttattcagaaaattacagaaattaagtcttaatcatgttcactttctattataaggtcctctctgagaattttttgtggattatcctttttactgtcttcaacagtaaccactcttcatcttacagggttgaatttgctttctggaaatggctaaatgttactcagaaccaagagtagtagaaaaagtagacaaagaaagaatatacttccaggtgctttctcaaagtgatactaattaaataatatagctgattttcttataccttattaccttccttgatattatttctaaggagaggagtttcaaaaataactttaaggatggcagcatcattagaataagtattaacttcttaagtaaaactagatgacattgaggggaacaacacttaattagatgtcaaaattctgatatgtctgctaaagaaatcattaattataataattataatcatacttagaagtgtccacttaagccttatctcctctgaggtatgtatttttgaaaacattgggactcatttgaatgttgtaaagggaaaaatcaatttgtcatgttttctgctatagttactcctcttacatagctggaataaaagcaaatcagaaacatatgcttatagtatttgcccgttttaaactggtagatgcctgattatacatttaaaaagaaatcttctgataccattttattagaataggtaggtgtgtgtccacgcatgtgtttctgtaatacttaaaaaggaaaatctctaagattatgatttaggcttctattcagataatcaagaaagagcaagttagtaaaagcccattataattctttaaaatgtaaacactgctaccgtaatagcaggaactacagaagataactgaagaacatcaggattatataaatccttcatagcccttctcaatataataatatatacttaggaccctatacttctataatcttaaagaccatctagtccaaacccatcgtataactctaaggaacagcaactctgagaggtgaagtgcctgctgaaggtcactcagccagtggctggcaagggccaggatgagatcccaggtggcctgtcctgcccaggcctcttctcccccgaccctgttcaatccagctcaggtcccacacctgtaaaatgaagaggatggtggactagaggatggtctcaaaggtccctttgtagctcaggctatgattccacaggtaccaggacactatgctcaactcaaataaactctttcagctcagggatgatgctctaaaccaaggaaggctccgtttaccaaagcactcatatgtgttccttaacagaaaaatagttctcccctttgaggaggccttactctaaataagcccaagacaatttcttgtcattatctcccttaggcttctactgccgtctctggcttctagtctgctcattttcattaactgcctccattaagctttactgagccaaatgactagataatatatttcaatgtaattatgggtaatatatgaaaagaacaatttagagatacctaatttctaaactgtactcttcatagtttcaattaaattgagaaactagatatttcattatatttctaacatgtatatacgaaaaaaatcaaatatgaaaacatagaactcaaacattattcttatttaaaaataaacatttccttcattaatttatacattctttctatgtccaggaaagagaatacaattctgacctgcagcaattttcctgtccataaaggggtaaaccaagtcctattttcactgctatccaaccacagagagcccttcgtggatatcttttgctttttaatcctcggcaggaagcttgtgcctctctcagttttggaaatggtctgttattcaactagaggcctttacctagctcatcttgtttcagccagcacgggaagtatttaaagacagaaggaaggctggaagattcagacttttcctccaatgcctttcaaaggctactcgcacattcctagggtcaaaccttgccctccagaatgcagtgttttataggctgttgttgctgttaaacttttttcccccataaagtgcaaatgtgaggaagaagaaacaaaagtactagatagcaaaacaagcaaatggacttggaattttatttgtacagatctgattaactaagagtttcccttttgatgatggacaatggcactagaggaaaagaacaggagtggggttctctgtgcccacttcttttcaaaagggtgattttataaaagtgctttccacataaggaaataaaatacactttaatgagtaagtacatatagagagggtgaccatgaggcatgttgtcatgttagtgcaggggcctttatttattttatgaacaatatcctaaagttaataaagaactatgctttattatttttttttaatctaggaagccaaggaaaaccagctgaacatattccattggctgcagccttcaatttaaacatcagaaagaaaggtaagctgggcacacccagattgtgtccagcttgtcagcacacttatttctgattatctgaaaataaacaacatgcttattctagagacagaggacctgctgaaagcttatagcacacaagtctattcaaaatgattccatatgttacactgtaggattgttgtgtagttatacaagggaaagaaatcaaaaccctgtacagacacctgatatcagacttgaaatgccaagtggaaacagaactattcagcatcttcatttatacacaatttacaatatttgattcaaaataaaaatcacaagaaaaatacatctgtttctgctacaattccttcccctccccatcctccccccacccccgccccagtgaaaagtcttctaataaaaggtatcatattaccaccgtcttgttttggtctaattctgagatcccacttggaacagttaacatgaaaaggaatggcaatacttgggatttatataacgtacacattgtatccaaggatctcaaatacttgcagtcacgtctccagatctgagaaatcacggttcaatggaagccagaaagctggacgaatgctgggcaggttgcatggggtgtaaaatcccttggctaagtctatgatcaaacaaggtcaaagttggttggctagagctgggctcaatttctcttctcaaatatatactaccagtcagtaagttttaccctttcttaaaccacacacccatctccaggctactgcctagagttaagaccaactgaagtagccatgtcctcatgataatgcatcaggataaaaagcaaaaacagggaaatacattcatcagcatctggccaaaggagacgggggttgggagaattgatctgggaggccattcctagcaagaacgagacaaaagtgtcaattcactagtttcagttacagttaagcttttggtggagttgattccagcagaggtgaagctcatggcatctagtgcttgatttaagataatgctattgaagaagggtaatgagaaaacacagcaaactaacaaggaggaactggccaaggaatatctggagggccaaagtgattttctttccttatcatttctacaggagaaggcaaggggtaggagaaaagggctggagggccccttatttgcagatttttttaaaaaaatcatttttttcataactccgtaatgaaaatgtattttacggtatgaaggttacagaactgcatctgctactgggtcacggctacaggtctatgagctgatccaccagcagtaaagacctggctaggttgggaagactggactcagagctcccactgctgtttctagagtgcccaccttgtgggtttttggttatcaatacaggaatagggtcaaactcatcttcagccaccttgtccgagccctcagggacatcaaaacctgagatgagattactatcttctgcagctttatggactggagcagagattgctgtgggggcaaactcttccagaaggtcagtagtagggttagagagcagagagcaatcaagcagggaatcttccccggtgagagaatctgtgcgattcgaggtcacagattccgtctgagatgggaggcgctggggaactgggggctccagtcctggtatgagactctcaacagcaacatcagctttttcaattacagcatcagaagtgctaccaaaaggatctgtcataggcaagaggtcagggagcagaagagaagtgtcaggagatttgagtccctcaattagtttttctggtgcatcaggtacttgaagaggaatgaaaggatcagacacgcttagaagcgggaggccagagtccacagtctgcccacccttccttttttcagcagttccagcagaaaatgaggtcgtagcaaaagcatcaccttgggttgattgaaagcctgggatcaaactctcagctgagcctccaagcttctcgggatgtttgccttccccaagcttggcaaagtccttgtttagcagttcttcagctgtgagtttggagaaattatcgtcatcaaagggattccacgtagacccttctgaaggattataaacgttttgttgagaggtccgaggagagcctgatggagtggtggttgcagacttggacttattgagactggcctcagctgcagctgcctggagcagctgggttgatttgctggcagggaccccaaagactgcactgtgggttacgtcactgagaatacgcctgtgcccagcacgttgggttttgggggatgagggtggagtgagagatccaactttctgcccctggacggcaggaggtggggttgtctgaacctttggctgttgtcttactggggcttgaatcgctggctcctgggcaggggctggctgtggggctgcagctggctgtggctggggctgctgtcctgctgccatagtgggcttttgctgcaaggcagcctgctgagtcatcagctgttgttgatgcagggctgtggccagctgttgctgttgctgttgttgttgctgctgctgctgctgctggtagaaattctgcattagctgctgttgagagcctccttgggacaccacagggaactgagcaattgctggtttctgggttgctggatgtactgcctgaaactgctgagtctgggcctgctgctgctggtaaaacgtgcctgccggctgctgctgtgctggcggtggctgttgctgctgctgttgctgcttgaggaagagttgctgctggtgctggggtgtggcctgggcctgagcgggcagaccctgggcctgagtagaaggcgtctgctgtggagtgggaggagcctgtggctgcttggcctgagtttgcggcagaggctggctgggtggggcttggggttttggttggggaacactggctaaaaggccaggctgattgctggatcctgcagcctgaggtgggggctgaacagtggccctcttccggggtgtcagcgctggctggatgggaaggattcctgggttcggctgagtctgcccagctttaggcctctggcggggtgcaattgaagtctctgtggtgggaatgggatctgtcagtctggcctttggctgggtcttttttgcagctgcctcactggctttcactggttcaggaagctttgcaggaatgggagagttctgtacatttggaattgggcactctttcttgagtagcttaaatgagaagtaggacacctggtaaatatccggccttttgtcagggtctggttccaacatatacctaattaggcagtgcatgtcttgagaatatcgagaattatcaggaattgtgaagtttccatcacaaattgccacctgactttccccaaatggcaaagtgaagtagcataatttatacaacaaacatccaagagcccaaatgtctgccttcgtagtgatgattttgccactgtacaggttgaccatttctggtgctcgataggacagcgttgtgtatttcttaatctcatcttctactgcattgactccctcagtttgtggattctggaatttgttggtggcgcttccaaagtcacacaggacatagtggcctcggtcatgcaagaggatgttttcaaccttcaggtcccggtggataataggagttttgcactgatgcaggcgggcaacagcttcacaggtatcacaaaatatctggagcacttcattctctgtaaagcctgtttgcaggcgctggttcatcaggtttaccacctggccacctctacaaaagtccatcagaatgagcacttcccatacatcaccgctactcacgttgttgatactagaatcaatgtaacccacaatattcttgtgccctgaaagatccctcattatctggatttctctcttgcacacctggagatcatgctcattgttgacaaacatgcgtttcaaggcacatttcatcccattgcttgtcctcaccagaaatacaatagcaaatccaccttccgccaacacctcgtccactgtgacctgctgtcgcccgatgccgaagactcttccgatgtagccactgcccaggcccgaggtgctgccccctcctccgctggagccggagcccaggccagagccgccctgctctcgccgggagtcgaaaaacttcttcatcttgcgaatagggagcagcaaagcaaaataccgatggtttctagattttttttttttttttttttttttaagaaaagagatccaaggatttcttctcagatttcacctcggagaggagccacccgaatccggccgtgggggtgggggctgagggaggatgcctataggaatatgcgtgtcaatcgcgcagcgggtcccctcctcctccagaaagcgattcgtgtaagtttaaacttgagacggctcggcggccggcgccctgctaccagccccgcgacattgtcacggccgccgggccggcctgcgacgcagagaagaggcggcgctgcagcgagagccggggccgcgctcggctcccgcccgcccgccagctgatcccgggagcgccgggcggagact

SEQ ID NO: 11718 - RNA, 15401 nt, Homo sapiens
  source 1..15401: mol_type = other RNA
ctgaatagctgggactacaggtgtgcaccaccacgtccagctaattttttgtatttttagtagagatggggtttcaccatgttggccaggctggtctcaaactcctgaccttgtgatctgcccaccttggcctcccaaagtgctgggattacaggtgtgagccaccatgcccagcctatttttttatttattttttgaagggacagggtctcgctgtgttgccagagttggtcttgaacttcctgggctcaactgatcctcctgcctcagccttccaaaatgctggtattacaggtgtgtggcactgcacctggccagctttattttaaggcactaataataaagggtatgaaaaaagctaggaataagtcagatctttccagaaataaaagacaattttaaaaaacatcagttaacctgtctggcctatttcaacatctaaagaggatagagaatgtaaaagttttcatgcctacctgattcagctcttttccattctcccaaacacttatttccatgtctcagatttacatttcctcaaaaggcagtagagatttggaaacaacaacaacaacaacaacaacaacaacaaaaccaccccaaaacaagcaagcctagtttgtagcctagtctcatgattaatgaattccctaatgctggcatttagcccacatactgagaggccggaactgtaacaaggtgctcttttctagtgttgtaaggggaaaatgtataaggaaaattaatttttcataatcaggtaaatataatttgttaatagcaaaacaagaaattccggagagaaaaaagatttactctgaaacaccagttccagcaggatttccctacaccttccaacgtattctactttgccatgagaaaaaaactaaataaataaaatggggttcaagtcagttaggcgagcaaacaccaaaaaacgagtgatttcattgtggaggtaggcatgatggggcaggatttccctcaagtggaaatgcttcctgtgcacacacacgtatacatgcacacacaaacctgtacactcacactaatttcaaaagcatggatgtggggaaagccctgccagcatgactagacatgaggagttagcccatctgcctgtatctctacacaggctctgacgtacattccacacccatagacagtcatgcacgagagccagcctggcttgcacacagactgagaatcagatctggagactcctagagctgctgcttctacaggaattattagtaactgcaggattatacttcctgttgatgtgcagggtttttatcttgctcttctttccagacatctccccttttcaagagtactaaatcttgatttagtggagggactaatcttgattcttcgatgggcatgacttagaacaggagctacaggaattaaaactagcaacaatagggcccctttgggattggggtgaagaagtatttcaggatttaaacagtttctgtgggtggggcggggggaaagcagagttcttggtggaagtggatgacctctgtgaaggagatgaaaatgcctccaagtccagaaatcaatataaacaaacaaacaaacaaacaaaaatgaacataacttaaaggggcttcaactaaatatcactgcaactgagtttgttgactcaagaaattctgctctgacgcagggaattgaaatataagaactgataatatttcttcttcagaaggctaagctgggagtgccatggcgggtattgagggtgggatagagacaagaggcttgaggctcaggttttgctcctagggtttcttgcctgattttgaagggaagggtgctagagcaaatggatcagcagctggcagctccgtagtcctggaggaaagggatgtgatagaaacagacccagctatcgactgcttgttggtttgtgaaacaattttgtaggcagcaatgggctgggcttctggacttggctcgtcttctgggctatagtgacgggaatacttggataaggactgggggcggaatggtttgccagccatggggcctgagacagcttctttctggagctgaggtcctttgtttctgtcattagaatgacccccagattccaggcaggatcccctgggagagatgctgtccagatggtctgctgcttgtacagaatgggacaggaggttagactgttgcacaaaaccagctgtggaatactgagcttggacagaggtgtacacagctctctcacggcccgcgggcagggggacatcacctgtctgactgaggagaccggtctgtgcaggcagctcctgggaggtgcattggataactgttaactcctccatgcttttcttcttagtgaaaggagctctcaaaaacacgtctgactcctctggctgggaaggagccatactgctcttggagacaaatggggctttggagaaaatgtccatgtcatcatttggaacccttgagctcctgaagggagctatggcaaaaacatctggctcactgagcccatcagtggctggctgtgtgaaggcttgaaactggttctttcttccaccttgcactgtctttgcttgctcaggagagacttctggtggagcgaatggaacggctcctcccagcttccccggggggggtctgcagctctcatcttcttcttcagactccataaggagaggccgagacccactgcagtccagcatgtctccttcaaggtcagtcccttcctcttcgctgctgtggaatgagctgttgcttgaagggccatctctggccaagtagtcagattctaagttgttctgagtctttgtgccaggtactctggaggggtctggatacagcggaaggcctttaacacccagtgattctttaaagtgctctacagttattacaggacagggattggactccctctggagatctagaaaagcataaaatgcagaattaatgtgtaggtcaattcaactctatttggaacatttaatggtcaacccgcggcaaaaacattgtgggaccaaataatagatgttgaaaatgcaacaggaaaaacataaaaataaaagtcaggcaaggaaactgcacacaaactggaacacaatcaaccactgtctcacgttttggaacatgataggcacgacgtacaggaaaggagatgaagatgttaggcacacagacattcagcgtaactatgcaatgctcctacacacagggccaggcacggacacctgctctacctggcactggctcattatggaatgaaaacaaacccagtcattcatctccacatataccatgacagttttggattatgtagaaacactgtctggggatgactcaattcagaatctggcatgtggtcatccgcgccacatgcagagggacaaactctctgaaaagaagcagaatgtggctgcttgataaatgcaagtttacttgatgacttacatcacaagcactactcaaagagcatacgagtgcccaaaatataaatactgaaggtaccttctgaggggagcatacagcatcaaaatcagaccaaataaatcaccttcagctggagttgccccagaattttgttttcagtcttctaagttcataaagatctcctctgcttaaatgaatctgccataaagttctttaagcagaaggagtaaaatgcatgggccattacagaagcattagcaaactccaatatactagtctatttctatctaggtagaggtgcctcagggtgctctggcttttaaaatcaaatagacaattatcagaatgcaagagagcttaccttccaagaaatattagcaggttagaagtatgtcattgggcacatgttagcaagagggcaggaaaaaggcatatgtaactaagcaagaagaatccagagaaagggtggttgggggtaaaggtatcatttcatcatgggctcagtaaagagatactactggagtttcccaacccaccaggataagaatattagatacaatgatttggagccatagatgacccagaacctctgtagagatggaactcaatgatccccttcccatactgaccctctcccctcctatgcaaaccattagctagcagaaatttctgccaaaaattatcccctgctaaagtttctgcatgaattaagcacacagaccacagcagaagaggcattaaaatcagtttattgggaaaccagtcacttagagacattacattgtaaagagaatgtagagagaggtctgaacattttataagatactgtacaaaaatactatgtttctctgaatcctataactttttagcagtgcttctttttaaacagttctgaccttaaatattgttttcagaaacagaacaaaaatgtgtttgtcctccatttttattttcctttctaacagtttgaatgcgttcagtgaattccagattggggcgttaagttaaattctgtactggtgccaaatggctttcagaatagtatttgaagaataagattttgaaaagaataaatttttccttgtattataattttagtatgtgcagctacatggtgatacgaaagcatcagtcagtggacaggaaataaacagaataccttcttccttgcgatttatgtggacagacataatcctaatttctcaggcaagtaaattgatattagatttgtctcagtgataccaagatgataatttctgggaggaaattcaaataaaagggagaaaaataagttttccaaaataaggtttgcagagccttaaagaaggacaagagggccctaaaactccttgaaccaccttcctcacatagtatcagttggacaaagttttcagttgccaaaacaaaagcacaatttctcatcttccaaaactaccttgaaagttgatgttattaagcttgttctgcaggagagcaaaatatctcttagggaaaaaaaatggaaaacttagtcaagccagtgaccaactctggcatcatacaggtcaataatccaatgaacactagtttgaacagagtcagtgttttttggaaatttaaactgaattcagttaaaacaatttgtgcacagagactggcaaaaaagcagctatctattgaaccaggggcactttggatgcctgaagtgctagattacattttgagaactaggaagtaccaaggggtgtgtgtatgtgcccatattcagggttggagaggatggaagaacatgtctaacccatcaaaattatttgttaaaaagtgggtttttggtcgagaacccatttggaaaaccttccaactcagagcatattctatgaccttcatgatgagtactgggaaaatcagacttaaaattccaacaactttgaataatttacaaaaacagtcacaaaaacaccagaatatcaagtttgaagggaaaattagtctcctgtccttcaaaacaaggacaagagctatttcctatctttctttcagcatcaacaggctttgtaggaatggaaaagtacatttaaagggttgtcctgagaaggccaagtcccttaacctttctattcttgttagaggaggtacagtgtggctgaggcggagagcaaccacactttgcaactctccaggcctggcactctgaagggcaaagaaatgccagagaatatgggggaagcccagacctccacattcccttaaggaattctggtggtggcagcaccagaaacaaggtagtcgagagaaggataaattccaaatatactagaaacagaaggtaaccattaaatcttgttggcagataaaagtctttttttgagtatgtgaatgtgttcttacagggaaaatgtgttttcagggtgaacagttcctttatatgaaggtagcattgtgtcaacaagaaaacgtgtttgaagcagtctctttactagcattgaaggatttatactaacctaaccacatgccttgacccagttcctttggtaaccaatggcacgtcatagcagataccctgtggccatagagctcagtaaacactgcctgttgtacctcaggggctaaagcccagggcctggcttcatagtctgcacagggtcttacttatcatagagcctaacgtagggttttgttataattccctcaaactggatcatgcctctttttattttggtttcacacataaaattaagcaagaagtcaaaacatacttctttttcttgctctgatgtaggactgtgtgccaggttaggcacgttgacactttcaatatgggtaactccatattagtctattttgaggctccaaattatgtagatttcagcaagaactcacatgcttcagggaagagaaggagttcctaaaatacctgacaacttggcaactatcctcaccagctccctattcacttccaaagcaacccaaagtgctgaatcatttaggatgggtttcccctggaaactccatctgattgacatagtgagggccatcagaatgctccctacagaattaaaatctgaagacttaaatgtcaggctggatattccttaatgaaatacatcacacaacaccagaagtttacttttcctcataccaaaaactgaaagaacggttacagggagtatcaaagatatgattcttgccaaaaacagaaaacgaagacttggagcattgagaagaagccttctcacatatagttagtaaacagaaagcaaaatatcccttcacaagaacttggaaatgcagcagcaattgaaacgtaaaattttagaaccaaactggggaaatcaagagacgtacatcaaactaataattaccatgaccttctagctcacataacaaaattaagcatttggttccaccatatattaggtagctgcattaaaacccacgactgggaaatgagggacctcatggaagccaaaaatggccagctgtgcctctcaggccaatgaggcaattaaatgagtgagttttctcactggggataaaattattcttgccaacacaaaatgtttaattaagttggcctgggtatattagggattaagttagaggagggaagctgcaaacctgcgctccattttacaaccctgagtctggtcatatccagtgtaggctggcaggcgtcttattctccttgagactaaaacaggggttttactctctcaggtagccatgattcattaatatgtcctcagtgtgtagctatacttttcttgtgcccaggtacttattgtcactcaatactgtgattaaatcctttctgcaaaaaagtgggttttcagctcaggaaaagagcaacttattttaagttatttacatctctaaacatcatgctcccatttgaacagataaaagtctttattcccctgtatgtttacataagaaagttctttacagacttttttttatacaatacttgtgcagcaatgttcaaatttcacgtttttactgcataagatatcttcatgtacaactgtatgctttgtcttcttgggaaggacgcgttaaagacctatgataaacacacatccacatgacaaaggagagtgcaatagggcagagtagaatactcacaggaaaagagtaaattcaggtcactacatcaaagtgtgaaccaagaacgtgtctttaattctagcaactaccaccatttggtaacttctttgcataggttagcattacccaaggagcctccctatcccgtattagtgaaaggaaatctgggagaagcaaaagaggtttcttgttatagatttcctagcactcattctgatttaagaaatctaagcacatccaacttcagaaacattactaatgtggaaaaagaaaaggctgactttgtgttgataaaattatagcctttagagaggaataaagatagctttgcagtatctggagtgtttcaggaaagcttccattctaaatattcatgtgatagtttttctgttctgccaggcagcctctaatttgcttaacccggcacactgggcaatcctgtcattttcatcccaaagctcaaagttagtggctatgggagcctgataatcttgcagacagagaaggttaaggactctgggaaatcacagaaaaaccttatcaagagagactttattttggcccaaggtatctatagcatgtatttatttagctgagtgcagatccctccacatcataggctgtcagccccaaagatcccttcattcccacagcactgctgaaggcagaactgttcctaacctggggaaggttatattggttgatcaattatctgtcaggagagtaggaaataagtaatcaaaacaaccaaaagtattaataataaaacaaatattacatcttgagaaagtagttcgtttcttgggtttgtttttccacaagtattagcaatccaagttgtgtaattctaattcaggaagagcgaagtccaatatcaaataacactgaacaaagtgacaacttctttcagaggtgttttaatacccatatctttcaatgttttaaaccattctaaagactaaggaatcacagaagtttccttattcagaaaattacagaaattaagtcttaatcatgttcactttctattataaggtcctctctgagaattttttgtggattatcctttttactgtcttcaacagtaaccactcttcatcttacagggttgaatttgctttctggaaatggctaaatgttactcagaaccaagagtagtagaaaaagtagacaaagaaagaatatacttccaggtgctttctcaaagtgatactaattaaataatatagctgattttcttataccttattaccttccttgatattatttctaaggagaggagtttcaaaaataactttaaggatggcagcatcattagaataagtattaacttcttaagtaaaactagatgacattgaggggaacaacacttaattagatgtcaaaattctgatatgtctgctaaagaaatcattaattataataattataatcatacttagaagtgtccacttaagccttatctcctctgaggtatgtatttttgaaaacattgggactcatttgaatgttgtaaagggaaaaatcaatttgtcatgttttctgctatagttactcctcttacatagctggaataaaagcaaatcagaaacatatgcttatagtatttgcccgttttaaactggtagatgcctgattatacatttaaaaagaaatcttctgataccattttattagaataggtaggtgtgtgtccacgcatgtgtttctgtaatacttaaaaaggaaaatctctaagattatgatttaggcttctattcagataatcaagaaagagcaagttagtaaaagcccattataattctttaaaatgtaaacactgctaccgtaatagcaggaactacagaagataactgaagaacatcaggattatataaatccttcatagcccttctcaatataataatatatacttaggaccctatacttctataatcttaaagaccatctagtccaaacccatcgtataactctaaggaacagcaactctgagaggtgaagtgcctgctgaaggtcactcagccagtggctggcaagggccaggatgagatcccaggtggcctgtcctgcccaggcctcttctcccccgaccctgttcaatccagctcaggtcccacacctgtaaaatgaagaggatggtggactagaggatggtctcaaaggtccctttgtagctcaggctatgattccacaggtaccaggacactatgctcaactcaaataaactctttcagctcagggatgatgctctaaaccaaggaaggctccgtttaccaaagcactcatatgtgttccttaacagaaaaatagttctcccctttgaggaggccttactctaaataagcccaagacaatttcttgtcattatctcccttaggcttctactgccgtctctggcttctagtctgctcattttcattaactgcctccattaagctttactgagccaaatgactagataatatatttcaatgtaattatgggtaatatatgaaaagaacaatttagagatacctaatttctaaactgtactcttcatagtttcaattaaattgagaaactagatatttcattatatttctaacatgtatatacgaaaaaaatcaaatatgaaaacatagaactcaaacattattcttatttaaaaataaacatttccttcattaatttatacattctttctatgtccaggaaagagaatacaattctgacctgcagcaattttcctgtccataaaggggtaaaccaagtcctattttcactgctatccaaccacagagagcccttcgtggatatcttttgctttttaatcctcggcaggaagcttgtgcctctctcagttttggaaatggtctgttattcaactagaggcctttacctagctcatcttgtttcagccagcacgggaagtatttaaagacagaaggaaggctggaagattcagacttttcctccaatgcctttcaaaggctactcgcacattcctagggtcaaaccttgccctccagaatgcagtgttttataggctgttgttgctgttaaacttttttcccccataaagtgcaaatgtgaggaagaagaaacaaaagtactagatagcaaaacaagcaaatggacttggaattttatttgtacagatctgattaactaagagtttcccttttgatgatggacaatggcactagaggaaaagaacaggagtggggttctctgtgcccacttcttttcaaaagggtgattttataaaagtgctttccacataaggaaataaaatacactttaatgagtaagtacatatagagagggtgaccatgaggcatgttgtcatgttagtgcaggggcctttatttattttatgaacaatatcctaaagttaataaagaactatgctttattatttttttttaatctaggaagccaaggaaaaccagctgaacatattccattggctgcagccttcaatttaaacatcagaaagaaaggtaagctgggcacacccagattgtgtccagcttgtcagcacacttatttctgattatctgaaaataaacaacatgcttattctagagacagaggacctgctgaaagcttatagcacacaagtctattcaaaatgattccatatgttacactgtaggattgttgtgtagttatacaagggaaagaaatcaaaaccctgtacagacacctgatatcagacttgaaatgccaagtggaaacagaactattcagcatcttcatttatacacaatttacaatatttgattcaaaataaaaatcacaagaaaaatacatctgtttctgctacaattccttcccctccccatcctccccccacccccgccccagtgaaaagtcttctaataaaaggtatcatattaccaccgtcttgttttggtctaattctgagatcccacttggaacagttaacatgaaaaggaatggcaatacttgggatttatataacgtacacattgtatccaaggatctcaaatacttgcagtcacgtctccagatctgagaaatcacggttcaatggaagccagaaagctggacgaatgctgggcaggttgcatggggtgtaaaatcccttggctaagtctatgatcaaacaaggtcaaagttggttggctagagctgggctcaatttctcttctcaaatatatactaccagtcagtaagttttaccctttcttaaaccacacacccatctccaggctactgcctagagttaagaccaactgaagtagccatgtcctcatgataatgcatcaggataaaaagcaaaaacagggaaatacattcatcagcatctggccaaaggagacgggggttgggagaattgatctgggaggccattcctagcaagaacgagacaaaagtgtcaattcactagtttcagttacagttaagcttttggtggagttgattccagcagaggtgaagctcatggcatctagtgcttgatttaagataatgctattgaagaagggtaatgagaaaacacagcaaactaacaaggaggaactggccaaggaatatctggagggccaaagtgattttctttccttatcatttctacaggagaaggcaaggggtaggagaaaagggctggagggccccttatttgcagatttttttaaaaaaatcatttttttcataactccgtaatgaaaatgtattttacggtatgaaggttacagaactgcatctgctactgggtcacggctacaggtctatgagctgatccaccagcagtaaagacctggctaggttgggaagactggactcagagctcccactgctgtttctagagtgcccaccttgtgggtttttggttatcaatacaggaatagggtcaaactcatcttcagccaccttgtccgagccctcagggacatcaaaacctgagatgagattactatcttctgtgcgattcgaggtcacagattccgtctgagatgggaggcgctggggaactgggggctccagtcctggtatgagactctcaacagcaacatcagctttttcaattacagcatcagaagtgctaccaaaaggatctgtcataggcaagaggtcagggagcagaagagaagtgtcaggagatttgagtccctcaattagtttttctggtgcatcaggtacttgaagaggaatgaaaggatcagacacgcttagaagcgggaggccagagtccacagtctgcccacccttccttttttcagcagttccagcagaaaatgaggtcgtagcaaaagcatcaccttgggttgattgaaagcctgggatcaaactctcagctgagcctccaagcttctcgggatgtttgccttccccaagcttggcaaagtccttgtttagcagttcttcagctgtgagtttggagaaattatcgtcatcaaagggattccacgtagacccttctgaaggattataaacgttttgttgagaggtccgaggagagcctgatggagtggtggttgcagacttggacttattgagactggcctcagctgcagctgcctggagcagctgggttgatttgctggcagggaccccaaagactgcactgtgggttacgtcactgagaatacgcctgtgcccagcacgttgggttttgggggatgagggtggagtgagagatccaactttctgcccctggacggcaggaggtggggttgtctgaacctttggctgttgtcttactggggcttgaatcgctggctcctgggcaggggctggctgtggggctgcagctggctgtggctggggctgctgtcctgctgccatagtgggcttttgctgcaaggcagcctgctgagtcatcagctgttgttgatgcagggctgtggccagctgttgctgttgctgttgttgttgctgctgctgctgctgctggtagaaattctgcattagctgctgttgagagcctccttgggacaccacagggaactgagcaattgctggtttctgggttgctggatgtactgcctgaaactgctgagtctgggcctgctgctgctggtaaaacgtgcctgccggctgctgctgtgctggcggtggctgttgctgctgctgttgctgcttgaggaagagttgctgctggtgctggggtgtggcctgggcctgagcgggcagaccctgggcctgagtagaaggcgtctgctgtggagtgggaggagcctgtggctgcttggcctgagtttgcggcagaggctggctgggtggggcttggggttttggttggggaacactggctaaaaggccaggctgattgctggatcctgcagcctgaggtgggggctgaacagtggccctcttccggggtgtcagcgctggctggatgggaaggattcctgggttcggctgagtctgcccagctttaggcctctggcggggtgcaattgaagtctctgtggtgggaatgggatctgtcagtctggcctttggctgggtcttttttgcagctgcctcactggctttcactggttcaggaagctttgcaggaatgggagagttctgtacatttggaattgggcactctttcttgagtagcttaaatgagaagtaggacacctggtaaatatccggccttttgtcagggtctggttccaacatatacctaattaggcagtgcatgtcttgagaatatcgagaattatcaggaattgtgaagtttccatcacaaattgccacctgactttccccaaatggcaaagtgaagtagcataatttatacaacaaacatccaagagcccaaatgtctgccttcgtagtgatgattttgccactgtacaggttgaccatttctggtgctcgataggacagcgttgtgtatttcttaatctcatcttctactgcattgactccctcagtttgtggattctggaatttgttggtggcgcttccaaagtcacacaggacatagtggcctcggtcatgcaagaggatgttttcaaccttcaggtcccggtggataataggagttttgcactgatgcaggcgggcaacagcttcacaggtatcacaaaatatctggagcacttcattctctgtaaagcctgtttgcaggcgctggttcatcaggtttaccacctggccacctctacaaaagtccatcagaatgagcacttcccatacatcaccgctactcacgttgttgatactagaatcaatgtaacccacaatattcttgtgccctgaaagatccctcattatctggatttctctcttgcacacctggagatcatgctcattgttgacaaacatgcgtttcaaggcacatttcatcccattgcttgtcctcaccagaaatacaatagcaaatccaccttccgccaacacctcgtccactgtgacctgctgtcgcccgatgccgaagactcttccgatgtagccactgcccaggcccgaggtgctgccccctcctccgctggagccggagcccaggccagagccgccctgctctcgccgggagtcgaaaaacttcttcatcttgcgaatagggagcagcaaagcaaaataccgatggtttctagattttttttttttttttttttttttaagaaaagagatccaaggatttcttctcagatttcacctcggagaggagccacccgaatccggccgtgggggtgggggctgagggaggatgcctataggaatatgcgtgtcaatcgcgcagcgggtcccctcctcctccagaaagcgattcgtgtaagtttaaacttgagacggctcggcggccggcgccctgctaccagccccgcgacattgtcacggccgccgggccggcctgcgacgcagagaagaggcggcgctgcagcgagagccggggccgcgctcggctcccgcccgcccgccagctgatcccgggagcgccgggcggagac

SEQ ID NO: 11719 - RNA, 1756 nt, Homo sapiens
  source 1..1756: mol_type = other RNA
ctgaatagctgggactacaggtgtgcaccaccacgtgtggctatttttgtaaaacagcagagatggcgtttccccatgttggccaggctggtctcaaactcctgatctcaggtgatccacccacctcggcctcccaaaatgctgggtattcttcagttttctgaagtgcacactgatttccctgttcaataagtatcaggaagcagcatgtagtacagaggtttactaactctgtgaatgggaagatcacttggctacccagtgctctcttataaacataagtacaagagtgtttcatgaaatccgtttttaaaatgaacatctctgtgtgccacagttcctaggactggggcaaggacacagtgtcaagtcttgttttgaggatgagtctctgaagagacagaattcctgccagaatgcgcacagaacataagtcagccaagtgtgtcgtgccagggatactttgactttggtttgctgctgctgctagggatattgggagggttatcctttccaggttgtaggagagggttgtgggtaaaggtctgtcgtaaaggacccctggctgctagctccaactgattccgcatgcgttgttcacgctctcgcagctgacgcgtcatttcagcatttttccagccttttttgaagctctctaggaagccttcccgtggaggtaatttgtccaggtcatgtacaacacgctgggggattttaagtacagtgcgtactgctggaatccggagacaggatacttggaccagggaaaacaaattggaggagagccagtacataaacactgccgtggggaaatgcatggttatgggcaaggttatcaggggcatcattctgatgacatttctcatccactgaaggtcagaactttgcacacctgtctcagcacctagctcaagaacagcccacattgtagcagtgactgccagtggtaatatgtagatgggatcggataccgtgagatcctggaaccaccagaggccacctgtctgcaggctgggcacaggaaggttggccatctctctcaaagcaatgaagaaggagatgaagattggggcctgagtcacagggagaatgagaggtttatagagtttaataccatgttttttctggtaaagtgccatctccgaggaagccttgtaatactcaatatggtctcctgctaacttggcctctctgattcgactggaaaacttctggatctctggcaagtgattgtggatcctggctgcctctcgctggcccgtcacgatgagaggaaaaatcaggcagcgggcaaagactgtacatgcagcaatggccccccaccaaggtaggcccagatcaacatgcataaattccagtaaattctggatcagtcccactggggtgtatgaccccagccccagttcagcgaagctctgctctgcagcagtttggactacatctgcagtctctccagaagccacctcaggtactgctgtgggtgagggagttgcagcaacaacaggaggggcctgaacctggacttctgcaaaagagatagcagaggtactgaggctgcgggggccggaagccgcaaggaagaggtagtgtgggcgacagcagcacggggctgctgggaataggagccgtgtggtcagcggtttcccaagccattgcgagggccctgcgacgctgtggacccgacgcccggactgtagcaagcgcagaagctcccggcgtccgcacattagtcccatcgccattttgcccggaagag

SEQ ID NO: 11720 - RNA, 635 nt, Homo sapiens
  source 1..635: mol_type = other RNA
ctgaatagctgggactacaggtgtgcaccaccactccccgctaatttttgtgtttttagtagagacgagattttgccatattggccaggctggtctcgaactcctgacctcaagtgatcctcccgcgtcggcctcccaaagtgctgggattacaggcgtgagccaccgtgcccagcctcgcaaaatgttttaataggtacatgcacgttttcctgagaagctaatccatataattaagttttcaaaagaagtgtgccacaacaggttaagaatcattgttctggtcactgcttacaactcaagtccctcaacacgtagtggcctgtgtgttctgctttgtctgaatcttctcgtctaaatttccttattaaattttcaaggcccaggttaaatggcatcttactctttgagatcttccaccaccctgtgtcctatcatttgttttctcttaagtttctttgcaaacgcactctgcacaccatatctagcaagtgttagttcccttccgtaactggattttttactctttgaggacgatggcagagtctccgttcgactcccaaaatacagggtcaagtactgcggccttcggacatttccgtctccggatcctgatagtctcggttactttcgcg

SEQ ID NO: 11721 - RNA, 1488 nt, Homo sapiens
  source 1..1488: mol_type = other RNA
ctgaatagctgggactacaggtgtgcaccaccatacctggctaatttttgtattttctgtatagatggggtcttgccatgttgcccaggctggtctcaaacttgtggcctcaagggatcctcccacctcagcctcccaaagcactgggattgcaggttcacaccaccatatccaggtcctgggggtcccttttataaggacattaatcctatttatgaaggttctacacttatgacttgcttacctcccaaagaccccacctcataaaaccatcacgttgggagttaggacttcaacatatgaatttggggggttggcacaaacgtttggttcattacaagaatagaggccttcccccaatacggctgcttttacctggagaatcctccaagtcacaaggtgaccttgtgcagggcacttctcatcttcgagcctctgtttcctctctgacagtgggggacctgggctgacattggctggagccaccatgacttaatggggaagtccccgcggccctgggactcatctgaggtcattaagcactgtcagggtcacctgtccgaagctggatttttcctaaacttcatttgcttttctctcctttcttttgccctggatactctcatctccctcaatttttctttcctttttcccttctcactacccacctccaatttcaaaatgtgcaaatagcagagcatcccagtggagttgccacggcaacagaagctggttttccctttccaaatgatgggccccttggaagcctctctcccctttgcctccttggtgaccagagctcaaggaagaaagcaaggtgtgtgggcaccccgaactggagggtccctttcttgtgcttgcaaggtgcccaggtcgtagagactgaggggccaggacaggggaggccatggagccagtttttgtttgctggggctgccataagaaagtatcaaaaactgggtggttttatcagaaacattctctcaccgttgtgggggcggacgcctgtgattagggtgtcccagggctggtttctcctgaggcctctcctcctggcttgcaggtggctgtcgtcatcctcactcggtttcttcctgtctgtccaggtttcctcttcttacaacacacctctccttcactgggatccagagttaaaatgaggatttgcatgggagcaggtgggcgagtcctagagataaggaaaaccccccacagaatccgtgtcttccaccacatagccgtggccaggagttcacaggcgtcccagggcaccgagcagaggatgcttggggctcgtccagacagggccagcactggatgaaccaggatgaggtcgggctgtgttcggggagccggcatctgggcactgggcagttgtgccatcagctcaggttctggtgcttagatcagctccagtttactagactctagactgtgtcctgctgcccagttgactactcccgtgggggaatcccaaaggatccaaaa

SEQ ID NO: 11722 - RNA, 649 nt, Homo sapiens
  source 1..649: mol_type = other RNA
ctgaatagctgggactacaggtgtgcaccaccatacctggctaatttttgtatttttagtagagacggggtttcgccatgttgatcaagctgatcttgaaatcctgacctcacacaatctgcccacctcagcctcccgaagtgctaggattacaggcatgagccaccgcattcggccaaccattctgagttcacttttttcatctcacaatggacaaatccaaccccagtctggaaggcaggagaccatggatacagttcccagggagtctccagagcagagagcaggatgcagaatggtgaagagtggattctgagacataaatggaaaatgcttataaggaatttgtttttgtaaactcttttcaatacgacctcacttctctggtcaaaagcaatccagagacttccctctcttctcttcctcttccctgactgccagtgggtggatggtttcctctctgtctgcgataagcactgcagaggactctcggagtttgtcctcactcctgatgccacacaccttttcttggcactttatctcgtcccaggggaagattcctgcagaaatttccttctctgtaatctcttgacagatggctctgctggcaagaacctcaatccttaggagtgcattaataggcttttat

SEQ ID NO: 11723 - RNA, 5709 nt, Homo sapiens
  source 1..5709: mol_type = other RNA
ctgaatagctgggactacaggtgtgcaccaccatgactggataaattttttttttgtattttttgtagagacggggtttcaccatgttgcccaggctggtctcaaacttctgagctcagggcaatctgcctgcctcagcctccccaagtgctgggacaactctttagcagtcatgaagaagccaaagttatcataacaagcagagttgtttctggcctctgtggatactgtcaacgaggggacaattttagctaccgttgaataaggagacacctctgtattgtaacaaattttaaaaatatcatttatgctaattctcataatctttggcctgaataaaaattagagacctacaggcacaactacagagaagcagaaattaaagcctgtatattgtattcattctaaagtttctcttttctgagatgtttttcggaaacagtattcttccaagatggatacatggaaagagaattagatatgcagtttttaaacatgatgagtgattggtactgtggagtatcatttgctccgtaaaattattccctcttttttggggatccatgttccaagacatgactctcatttgagaagtgtcctctcccaggctcaccaacttggcttccacggcatcccctttccccgaatcttagaaagggctatttaaagccagagcttctgtacccagaagatttgaaggttaaagcagaggaaccagaaagtgtttccttgttgctattctttacacacactataaaaagctttcatcagaaaggggaagggagaaaaaggatcccatgcaaataatctctggaaaaaaaattaaacttgttctaaaaatgagaaagaaacttatactttataaatgagcaatgttctaggcaaagagtggggttctgcctactctgctctctgattcctgcttagctccaggtaacaagttaaatagctacagcttgcatttacaggatattcgagtctcggaggctcaagtacagcatctccttagactttacaacctcccaggagaccatgggtacattttacagacgaggcaactaaggcacctggagagaaaaagtcagatgactttacaaacccaaagtggagccaggatggtaatttggtcttaggacttgctgagtgctgcctcctggccagagctgcctcaggctgcagagaacagacgtttccccagcaaggactccagcccaggaaaaggtcttctccggctgatgactgatggggattctccaggctttctctgttccctgccactgtttatttctggaaaggtggttcatcaacatctgctgacagtatctgtttgttttcgccatcttcccagaatggaagaaattacttgatgtgatcttgtgaacagatcaactaaggaagcaggctgcatgaaacacaagccttcaaaagcagtgttccttgagctaaaagttttgttcaagaaggaggaaaaatgggagtagatgatggaaacttcctttcctagggttttgttccctcggataaaaaacacacaaatgtttctcacaaagaaacctgcagtggccaatggcccacgttgaaaactttctttgtaactgcgatgtgccaagtatttgattaaatttctgctgtagataaccctgcaggtacatccttctcgggtcttctgtattacgagtcctttgaggccaagaccaagtgttctctctttgtcatatttcccatgacatccaggagagagttgcacagggttctcggctaacaggcaaacggagagaaagctggcattggacatgtaaagaattaaatggagtagctagcattcatcacaaatgatgggcgcccacctgccttgtgggagggaactcggggtgcttttcctatctgggattctaggagcttgtgaattggggctcattttgatcatctaaagggagcatgatgatgccactttcagaaggaagtgggtgaagagctgtggctttaggtacagactgcccaggcaggcttgctgtctatccaacacactgaatgtttgtgtcgcctcaaaatccatgttaaaatccttaccacgaatgtgaggaaattaggaggtggggcctgtggggggtgactaggtcatgagggtacagcccttaagaaggggattagtgcccttataaaagaggcctgagagttctccagctgtcttgctgccacatgaggatacagagggaggtcagcagtctgcaacctgggagagagccctgaccaggattccagcctcccaccatgctggtgccttgatcttggctctccaacgtccagaactgtgagaagtgagtggctgtccccagtccatgctgctttgctatggcagcctggatggactgaggcacctgctgcccagcacccactctccacaggtgagggcagcccctcagtgtacagaccccgtgcagctgcgtcatccctgccaggatgcaggcacctctgtggtgccaggggtactcagagagcctcagggaggctgcacagccacctcgggcctgttaccactgtccaggaaggggcctgggccaggaggatgagggagaaaaggagaaaccaggctgctaattcctgagtctgtagttggctatgaagcagaggggagcaaaactcaaccaaacacttctgcaccctggagttcagcaggggcagctggtaggtccttaagagcaacattagccttctggaaatggacttccaaggcagcttagaatctgagaagtgagctcacaaaggcctttttttgttttagttaacattagaataataaaaaagaccattttgcctcacccagcaactggagaaaaaggaccctaagaagatggttctttaagagaaaagactttaagaatggtttccgaaaagaatttttatttctttttacttgtttctttcttccactcctatgcattttgattcatttaaataattaaagtagacttattaaatctgctgtaaatccactgggcactcctggctggcccatcctcttcctttctcccctggggctcagcaaacactccctggagtagggacctcatgcgtactttttaaatggccaatttcctgcttttgcagggtttcctcatgtcctctgagctttcttgccttttaagggataaaatatttaccacttgcattgtccctgacaacaaatatttcctggtcccctaactccttaaataaagcaaccttgcatgcctgtttatctgctgaaatactctggagtcaagaaatataatgagctgtttctgcaatagaagtgtctatcagcagccttgtagcccagtgattgtgacactgcacacctcggcccagataaaaggtccacaaaagcaaccccttcagggtcaagaccccctcaacctatcccaattgccagctctgttttttcatagaattgtgcaacatttgctgccttataggaaacacctggctccagggagcagtcacagttttcttctagggttctccttcctgtaagactagttcttgaaactgtcttaggtcatgacttcttgaacttctggttgtccaccacctcgtccatctcccatcacctctgcaaatccacactagcagaaagaaaagtggtatggaattcttccacaagcacctggctccttctataccccagagacgcagccgcccacccacccaggagccacaccaagcacatgctcaggagacgtccctccatgctggctcctgcagctaggctgaaaagtccaggctccaagaccacctgactcaacatccccatggtgtcactgacatcaggaagctgcacaggtcacacatcctctaaaaagcctctgagaggcaagctacctcaaaaacatatgctggctccagcctagcggctcctaaagaatttgagagagaaagcacagcatgctctttttctgcagttctcaggtactcccaaagcccggtgcttttctccctcccgtgtgtagctcccctgctgtacatgtgctgggatcgagtatttcagatgcacagcctggggaaggctgtctggttttcagacagcccctttgatttacgatcctgtggttaaatcagtgcaggattttggagaaagaccaattccatttgcttacgagtctgatcctgaggctctggcatctctaacgaccttggcaatcatttgcttttaattaccatttgattccatccctgaaagaatgagcctggcttctacccctccaactgcatagttctgaagaatctcggcagaggattatggctgctctgacgctaaacttgattcaggcaaagcatcttctttcagggttactttacgctgtcttgacttttttataatgaagagtagccagttccatcctgaatgaaccctcccagcacacctgaatctcttcaaacgtcacttatttgccaaaggactctggacctcacagcaaagctgtataaagcttagaaaaacaagttgacttaaagtttctatttttacacggtgtcctgtttctagaggggctgaggctcgtggtttgaaactcaatttagcatttaaactaattttcagcttggtctctatggaccagcaattagggaagtagaagagttcaaaggaggaggttccagcctctcctgggcaggcgtgtacggtctttgaagacgttctcccagcctttcttcctgtctccgctggcggccacagacagctcggacaacctgctgtggctgggcccgcgtgggcacacagtgcccagtctttctggtgcccgggtctggaaagacaccaatggctgagtccattttgttccttctcagagctgtcctggggaaggatctgaaaacttcctgaagactccgctgcacacttggcattctgcagagggggctggtaactggagggccggtagaacatcctctgggtggcatcagtgtgaatgtcaccaaggaagagctcctcgaccaggtggtcgaggttgtggtgaaggtactgcttctccacccggatgagctgaagttcatgcatggcaaagttcacggccttggtgcactcacagccgttctcctctcgccagaggtcataggccacgtcctgcacccagggacccccgtctgcgaggaagcccgggcatgtgcggttcacctgctggccgagcttctcggccaccgcctctgtgtggcagatcacctggacgttgtgcagctggtagtcggcttccgtgccccctcggatgatccaggaggcctggcggaggcggatcttgccccggatgatgagagtataagtgggatttgtgcaccggttgctgccataataaaattggtaggccttgaaggtgttattgtggtagaatctgtaggaccttgtgatgaactctgggcctgaccttacttcacagcctgtggagacccagtggccctcgattgtaggtggcatctgcactgtgatccttgcaccattgtggagatgtttgagcatgtgatggcactgtgactccttaaaagccctccaggcacttttctctaaggacctaggatgagacctgctgtctggatgaaggagggcagaaccctctcccagcccgtgaagcaggagggccgggaacaggtatctgagcaggaggcggcgcggccaggacatttccagtcctgctctggggcctcccgcacgccgcgctccgatttggtgcccgggcaact

SEQ ID NO: 11724 - RNA, 4674 nt, Homo sapiens
  source 1..4674: mol_type = other RNA
ctgaatagctgggactacaggtgtgcaccaccatgactggctaattttttgtatttttagtagagacggggtttctactgtctactgtgttagccaggatggtctcaatctcctgaccctgtgatccgcccaccttggcctcccaaagtgctgggtgtttttaatttcaaattccacttgttctttgctgacatataggaaagcagttgacttccgtgtattaactttgtatcgtacaaccccactataatcctttattagttccagaagtcttttttgttgcttctttcagattttcattacctgctttttctttaaaaactttgttatactgattgaaaaagcaagaaaatttctaacaggcacaatggacagtgcattagctttctagggctgccactacaaagccccacagactgggcgaagtcaacaacagacatttgttctctcacagcccggaaggctggaaggccaaggtcatagtctcagcagggctggctttggaccttggcttgcagacgccgttctctctcagttgtcacagggtcaagcctctctacgtatgtgtgtcctgatctcatcttctaatatggacaccagtaatactggattagggtgcaccctgacgacttcattgacccttaatcaactttaggaccccatctccaaacacagtcacattctgaagtatggggggttagggcttcaacatacaaatttgctggtggcggctgtgaggcggggagcgcaattcagcctataataagtatattctttaaatggcaaaagtatgtgcaaaagcagtcatttactccttaattggaacgttatcctactacactgggagcttgtaccatttgaaaacattaagccatatgggaaaaatgtagaaaagaacatggaatacacggatttgtcccatgggaaaagcatgcttagtgtaaccccgtatctaggagacgtgaagggaactttttccttctcacttgtcttctatccttgaccagaacggtgtctgtggcactcatcacatcgcaggttagacaggctttctgagccggcctggaaatggaatcaccacacagaatattacgtctgtgggaagatgtgttcagagtcaatggagatctgacctgtggggctggaaggtgatttgtgggatgacgaggacctgcctgctgagatcctggtgcgcagctccattataaggtgtgtgaaaaccagagaccacgcagctctcaggaacacaaatgcgtggagaacaaatgcccagtgagagaccaccactatacaaacacgaacgagacccccagaaatggcacccaggaacccacgtctggcttcatagacttatgtgtttactggggaaccgaatggacccgcccacatgtgctgcacccaggcggcctcttctggcatctctcagtgggatgtgctgcacccaggcggcctcttccggcatctctcggtgggatgtgctgcacccaggcggcctcttcccgcatctctcggtgggatgtgctgcacccaggcggcctcttcccgcatctctcggtgggatgtgctgcacccaggcggcctcttcccgcatctctcggtgggatgtgctgcacccaggcggcctcttcccgcatctctcggtgggatgtgctgcacccaggcggcctcttccggcatctctcggtgggatgtgctgcacccaggcggcctcttccggcatctctcggtgggatgtgctgcacccaggcggcctcttccggcatctctcggtgggatgtgctgcacccaggcggcctcttccggcatctctcggtgggatgtgctgcacccaggcggcctcttcccgcatctctcggtgggatgtgctgcacccaggcggcctcttcccgcatctctcggtgggatgtgctgcacccaggcggcctcttccggcatctctcggtgggatgtgctgcacccaggcggcctcttcccgcatctctcggtgggatgtgctgcacccaggcggcctcttccggcatctctcggtgggatgtgctgcacccaggcggcctcttcccgcatctctcggtgggatgtgctgcacccaggcggcctcttccggcatctctcggtgggatgtgctgcacccaggcggcctcttccggcatctctcggtgggatgtgctgcacccaggcggcctcttccggcatctctcggtgggatgtgctgcacccaggcggcctcttccggcatctctcggtgggatgtgctgcacccagatgttctcatcccacgtctctcagtaggatgtgctgtacataggtggtctattcccgtgtctctcggtgggatgtgctgcacagaggtgacctcttcctgcatctctcggtgggatgtactccacccaggtgttctcttcccacgtctctcagttggatgtgctgcgcacagccggtctattctcgtgtctcttggtgggatgtcttacacccaggtggtctattcccgtgtctctcggtgggatgtgccgcacccaggtggtctattcccgtgtctctcagtgggatgtgttacatccaggtggtctcttcccacatctctcagtgggatgtgctgcacccaggtggcctcttcccgcatctctcagtgggatgtggtccacccaggtggtctcttctcgtgtctctcagtaggatgtgccgcagacaggtggtctattcccgtgtctctcagtgggatgtgctgcacccaggtggtctcttcccgtgtctctcagcggggtcctctcacagtctcacaggtgagcggagttgcactgcagggaccagagctgatgggactctcatggcagatgatcctgcagccaccaagagcttaacatggggctgtcatgggacagacgtctgtcaaaggctcagcatgtttctggctcactttctcagaggtcactttctttggtggattttggacggccagcgtctggggttccctctttccttggccacttggaacaggaggaaaaagtctctgcagcaccttctccacaaacactgcaggccagctgctcaggatgctgcgtcaggaggattactggagaaccagcccggacaacatagtgagatccgatctcttcacgggcggctgcaatagttttcattaagcactggtaaacacacccagcgggatgcgagcagcccaggggcttccggagaggccggcactgccccgacgggggcgggacctcagagcagcccactcagttctcggagtcagtttctcaccaaaacaaggctgggctaaaacacgctgagaggtcattgggaaggccgttcagcaagctgctgacccctccggcttctgtacctgctgtcccctccggcttcctgtctgctgtcctctctggcttcttgtctgctgtcccctccagcctccgtgcctgctgacccctccggcttcctgtctgctgtcccctccggcttccgtgcctgctgtcccctccggcttccgtgcctgctgtcctctccggcttcctgtctgctctgttctcacaggcacaagggtcccctacctccgtgtctactgcacccagcggacaggaccagcggcagtgaccagcttgtgactccatcagaaccttgcatgtgatcggtcacctggctgggtcctcacggtgctgccgcccactttacagatgagccacctgagcattagtagagtgagctctgaggcagcagcccagcaggactgacctcggtggccatccccatcgagacctaggcctgctgtgcactgaggcgccagccgtcagggatgggcacattgggcatccaccacctcctcggcccacttccctctccagctgtacaccaagcacgactctctcccaacctgcaagcagccgagactgcagctgcccccatgtctgagcagctcctgcaaccctcctccagccgtcgcagtaccgcatctcttcatccccacgtgctctggccttgccatccctgcacctgcccttccctgctggggccgaccctcaccccccaacctcaccatgcaccaacactcccgcaggacctggctggcacggcgcctcttcctttgccaggattctctaaacctccctgttccatgaggctgattccttccttcttctctcccctccttcgttcattcattcagtcattcacttgggaagcgctcctgagcacgttgtccttccttgaagatgggaaaagaggtgccaactcctgttctggaggaaggattctaccacatctgagtagaaaatgtcaaagccacatgtgtcaatgaacacagccccacttctcctgcagcacagcaatgactcctgtccagttctgcacacagtcccacacacggggccagaatgaaagtcggccccaacagagtcaccaggcacccaaccagaccaacgccatgctgtaagaagaaaaaggggcctctttccaatggaaacaaatctgagccagcatcttcagctctgggactccaagggagaggcaggtatcacaggcaagttgcagggtacagctgggagatgcacacaccacacaaggacacacacagacacgcatgtacaaacacgccacacgcagacacgtgtatgcaggcacacaacacacaggcgcacatgcatacacaggcgcacatgcatgcatagacacacagga

SEQ ID NO: 11725 - RNA, 4677 nt, Homo sapiens
  source 1..4677: mol_type = other RNA
ctgaatagctgggactacaggtgtgcaccaccatgactggctaattttttgtatttttagtagagacggggtttctactgtctactgtgttagccaggatggtctcaatctcctgaccctgtgatccgcccaccttggcctcccaaagtgctgggtgtttttaatttcaaattccacttgttctttgctgacatataggaaagcagttgacttccgtgtattaactttgtatcgtacaaccccactataatcctttattagttccagaagtcttttttgttgcttctttcagattttcattacctgctttttctttaaaaactttgttatactgattgaaaaagcaagaaaatttctaacaggcacaatggacagtgcattagctttctagggctgccactacaaagccccacagactgggcgaagtcaacaacagacatttgttctctcacagcccggaaggctggaaggccaaggtcatagtctcagcagggctggctttggaccttggcttgcagacgccgttctctctcagttgtcacagggtcaagcctctctacgtatgtgtgtcctgatctcatcttctaatatggacaccagtaatactggattagggtgcaccctgacgacttcattgacccttaatcaactttaggaccccatctccaaacacagtcacattctgaagtatggggggttagggcttcaacatacaaatttgctggtggcggctgtgaggcggggagcgcaattcagcctataataagtatattctttaaatggcaaaagtatgtgcaaaagcagtcatttactccttaattggaacgttatcctactacactgggagcttgtaccatttgaaaacattaagccatatgggaaaaatgtagaaaagaacatggaatacacggatttgtcccatgggaaaagcatgcttagtgtaaccccgtatctaggagacgtgaagggaactttttccttctcacttgtcttctatccttgaccagaacggtgtctgtggcactcatcacatcgcaggttagacaggctttctgagccggcctggaaatggaatcaccacacagaatattacgtctgtgggaagatgtgttcagagtcaatggagatctgacctgtggggctggaaggtgatttgtgggatgacgaggacctgcctgctgagatcctggtgcgcagctccattataaggtgtgtgaaaaccagagaccacgcagctctcaggaacacaaatgcgtggagaacaaatgcccagtgagagaccaccactatacaaacacgaacgagacccccagaaatggcacccaggaacccacgtctggcttcatagacttatgtgtttactggggaaccgaatggacccgcccacatgtgctgcacccaggcggcctcttctggcatctctcagtgggatgtgctgcacccaggcggcctcttccggcatctctcggtgggatgtgctgcacccaggcggcctcttcccgcatctctcggtgggatgtgctgcacccaggcggcctcttcccgcatctctcggtgggatgtgctgcacccaggcggcctcttcccgcatctctcggtgggatgtgctgcacccaggcggcctcttcccgcatctctcggtgggatgtgctgcacccaggcggcctcttccggcatctctcggtgggatgtgctgcacccaggcggcctcttccggcatctctcggtgggatgtgctgcacccaggcggcctcttccggcatctctcggtgggatgtgctgcacccaggcggcctcttccggcatctctcggtgggatgtgctgcacccaggcggcctcttcccgcatctctcggtgggatgtgctgcacccaggcggcctcttcccgcatctctcggtgggatgtgctgcacccaggcggcctcttccggcatctctcggtgggatgtgctgcacccaggcggcctcttcccgcatctctcggtgggatgtgctgcacccaggcggcctcttccggcatctctcggtgggatgtgctgcacccaggcggcctcttcccgcatctctcggtgggatgtgctgcacccaggcggcctcttccggcatctctcggtgggatgtgctgcacccaggcggcctcttccggcatctctcggtgggatgtgctgcacccaggcggcctcttccggcatctctcggtgggatgtgctgcacccaggcggcctcttccggcatctctcggtgggatgtgctgcacccagatgttctcatcccacgtctctcagtaggatgtgctgtacataggtggtctattcccgtgtctctcggtgggatgtgctgcacagaggtgacctcttcctgcatctctcggtgggatgtactccacccaggtgttctcttcccacgtctctcagttggatgtgctgcgcacagccggtctattctcgtgtctcttggtgggatgtcttacacccaggtggtctattcccgtgtctctcggtgggatgtgccgcacccaggtggtctattcccgtgtctctcagtgggatgtgttacatccaggtggtctcttcccacatctctcagtgggatgtgctgcacccaggtggcctcttcccgcatctctcagtgggatgtggtccacccaggtggtctcttctcgtgtctctcagtaggatgtgccgcagacaggtggtctattcccgtgtctctcagtgggatgtgctgcacccaggtggtctcttcccgtgtctctcagcggggtcctctcacagtctcacaggtgagcggagttgcactgcagggaccagagctgatgggactctcatggcagatgatcctgcagccaccaagagcttaacatggggctgtcatgggacagacgtctgtcaaaggctcagcatgtttctggctcactttctcagaggtcactttctttggtggattttggacggccagcgtctggggttccctctttccttggccacttggaacaggaggaaaaagtctctgcagcaccttctccacaaacactgcaggccagctgctcaggatgctgcgtcaggaggattactggagaaccagcccggacaacatagtgagatccgatctcttcacgggcggctgcaatagttttcattaagcactggtaaacacacccagcgggatgcgagcagcccaggggcttccggagaggccggcactgccccgacgggggcgggacctcagagcagcccactcagttctcggagtcagtttctcaccaaaacaaggctgggctaaaacacgctgagaggtcattgggaaggccgttcagcaagctgctgctgacccctccggcttctgtacctgctgtcccctccggcttcctgtctgctgtcctctctggcttcttgtctgctgtcccctccagcctccgtgcctgctgacccctccggcttcctgtctgctgtcccctccggcttccgtgcctgctgtcccctccggcttccgtgcctgctgtcctctccggcttcctgtctgctctgttctcacaggcacaagggtcccctacctccgtgtctactgcacccagcggacaggaccagcggcagtgaccagcttgtgactccatcagaaccttgcatgtgatcggtcacctggctgggtcctcacggtgctgccgcccactttacagatgagccacctgagcattagtagagtgagctctgaggcagcagcccagcaggactgacctcggtggccatccccatcgagacctaggcctgctgtgcactgaggcgccagccgtcagggatgggcacattgggcatccaccacctcctcggcccacttccctctccagctgtacaccaagcacgactctctcccaacctgcaagcagccgagactgcagctgcccccatgtctgagcagctcctgcaaccctcctccagccgtcgcagtaccgcatctcttcatccccacgtgctctggccttgccatccctgcacctgcccttccctgctggggccgaccctcaccccccaacctcaccatgcaccaacactcccgcaggacctggctggcacggcgcctcttcctttgccaggattctctaaacctccctgttccatgaggctgattccttccttcttctctcccctccttcgttcattcattcagtcattcacttgggaagcgctcctgagcacgttgtccttccttgaagatgggaaaagaggtgccaactcctgttctggaggaaggattctaccacatctgagtagaaaatgtcaaagccacatgtgtcaatgaacacagccccacttctcctgcagcacagcaatgactcctgtccagttctgcacacagtcccacacacggggccagaatgaaagtcggccccaacagagtcaccaggcacccaaccagaccaacgccatgctgtaagaagaaaaaggggcctctttccaatggaaacaaatctgagccagcatcttcagctctgggactccaagggagaggcaggtatcacaggcaagttgcagggtacagctgggagatgcacacaccacacaaggacacacacagacacgcatgtacaaacacgccacacgcagacacgtgtatgcaggcacacaacacacaggcgcacatgcatacacaggcgcacatgcatgcatagacacacagga

SEQ ID NO: 11726 - RNA, 4652 nt, Homo sapiens
  source 1..4652: mol_type = other RNA
ctgaatagctgggactacaggtgtgcaccaccatgactggctaattttttgtatttttagtagagacggggtttctactgtctactgtgttagccaggatggtctcaatctcctgaccctgtgatccgcccaccttggcctcccaaagtgctgggtgtttttaatttcaaattccacttgttctttgctgacatataggaaagcagttgacttccgtgtattaactttgtatcgtacaaccccactataatcctttattagttccagaagtcttttttgttgcttctttcagattttcattacctgctttttctttaaaaactttgttatactgattgaaaaagcaagaaaatttctaacaggcacaatggacagtgcattagctttctagggctgccactacaaagccccacagactgggcgaagtcaacaacagacatttgttctctcacagcccggaaggctggaaggccaaggtcatagtctcagcagggctggctttggaccttggcttgcagacgccgttctctctcagttgtcacagggtcaagcctctctacgtatgtgtgtcctgatctcatcttctaatatggacaccagtaatactggattagggtgcaccctgacgacttcattgacccttaatcaactttaggaccccatctccaaacacagtcacattctgaagtatggggggttagggcttcaacatacaaatttgctggtggcggctgtgaggcggggagcgcaattcagcctataataagtatattctttaaatggcaaaagtatgtgcaaaagcagtcatttactccttaattggaacgttatcctactacactgggagcttgtaccatttgaaaacattaagccatatgggaaaaatgtagaaaagaacatggaatacacggatttgtcccatgggaaaagcatgcttagtgtaaccccgtatctaggagacgtgaagggaactttttccttctcacttgtcttctatccttgaccagaacggtgtctgtggcactcatcacatcgcaggttagacaggctttctgagccggcctggaaatggaatcaccacacagaatattacgtctgtgggaagatgtgttcagagtcaatggagatctgacctgtggggctggaaggtgatttgtgggatgacgaggacctgcctgctgagatcctggtgcgcagctccattataaggtgtgtgaaaaccagagaccacgcagctctcaggaacacaaatgcgtggagaacaaatgcccagtgagagaccaccactatacaaacacgaacgagacccccagaaatggcacccaggaacccacgtctggcttcatagacttatgtgtttactggggaaccgaatggacccgcccacatgtgctgcacccaggcggcctcttctggcatctctcagtgggatgtgctgcacccaggcggcctcttccggcatctctcggtgggatgtgctgcacccaggcggcctcttcccgcatctctcggtgggatgtgctgcacccaggcggcctcttcccgcatctctcggtgggatgtgctgcacccaggcggcctcttcccgcatctctcggtgggatgtgctgcacccaggcggcctcttcccgcatctctcggtgggatgtgctgcacccaggcggcctcttccggcatctctcggtgggatgtgctgcacccaggcggcctcttccggcatctctcggtgggatgtgctgcacccaggcggcctcttccggcatctctcggtgggatgtgctgcacccaggcggcctcttccggcatctctcggtgggatgtgctgcacccaggcggcctcttcccgcatctctcggtgggatgtgctgcacccaggcggcctcttcccgcatctctcggtgggatgtgctgcacccaggcggcctcttccggcatctctcggtgggatgtgctgcacccaggcggcctcttcccgcatctctcggtgggatgtgctgcacccaggcggcctcttccggcatctctcggtgggatgtgctgcacccaggcggcctcttcccgcatctctcggtgggatgtgctgcacccaggcggcctcttccggcatctctcggtgggatgtgctgcacccaggcggcctcttccggcatctctcggtgggatgtgctgcacccaggcggcctcttccggcatctctcggtgggatgtgctgcacccaggcggcctcttccggcatctctcggtgggatgtgctgcacccagatgttctcatcccacgtctctcagtaggatgtgctgtacataggtggtctattcccgtgtctctcggtgggatgtgctgcacagaggtgacctcttcctgcatctctcggtgggatgtactccacccaggtgttctcttcccacgtctctcagttggatgtgctgcgcacagccggtctattctcgtgtctcttggtgggatgtcttacacccaggtggtctattcccgtgtctctcggtgggatgtgccgcacccaggtggtctattcccgtgtctctcagtgggatgtgttacatccaggtggtctcttcccacatctctcagtgggatgtgctgcacccaggtggcctcttcccgcatctctcagtgggatgtggtccacccaggtggtctcttctcgtgtctctcagtaggatgtgccgcagacaggtggtctattcccgtgtctctcagtgggatgtgctgcacccaggtggtctcttcccgtgtctctcagcggggtcctctcacagtctcacaggtgagcggagttgcactgcagggaccagagctgatgggactctcatggcagatgatcctgcagccaccaagagcttaacatggggctgtcatgggacagacgtctgtcaaaggctcagcatgtttctggctcactttctcagaggtcactttctttggtggattttggacggccagcgtctggggttccctctttccttggccacttggaacaggaggaaaaagtctctgcagcaccttctccacaaacactgcaggccagctgctcaggatgctgcgtcaggaggattactggagaaccagcccggacaacatagtgagatccgatctcttcacgggcggctgcaatagttttcattaagcactggtaaacacacccagcgggatgcgagcagcccaggggcttccggagaggccggcactgccccgacgggggcgggacctcagagcagcccactcagttctcggagtcagtttctcaccaaaacaaggctgggctaaaacacgctgagaggtcattgggaaggccgttcagcaagctgctgctgtcccctccggcttcctgtctgctgtcctctctggcttcttgtctgctgtcccctccagcctccgtgcctgctgacccctccggcttcctgtctgctgtcccctccggcttccgtgcctgctgtcccctccggcttccgtgcctgctgtcctctccggcttcctgtctgctctgttctcacaggcacaagggtcccctacctccgtgtctactgcacccagcggacaggaccagcggcagtgaccagcttgtgactccatcagaaccttgcatgtgatcggtcacctggctgggtcctcacggtgctgccgcccactttacagatgagccacctgagcattagtagagtgagctctgaggcagcagcccagcaggactgacctcggtggccatccccatcgagacctaggcctgctgtgcactgaggcgccagccgtcagggatgggcacattgggcatccaccacctcctcggcccacttccctctccagctgtacaccaagcacgactctctcccaacctgcaagcagccgagactgcagctgcccccatgtctgagcagctcctgcaaccctcctccagccgtcgcagtaccgcatctcttcatccccacgtgctctggccttgccatccctgcacctgcccttccctgctggggccgaccctcaccccccaacctcaccatgcaccaacactcccgcaggacctggctggcacggcgcctcttcctttgccaggattctctaaacctccctgttccatgaggctgattccttccttcttctctcccctccttcgttcattcattcagtcattcacttgggaagcgctcctgagcacgttgtccttccttgaagatgggaaaagaggtgccaactcctgttctggaggaaggattctaccacatctgagtagaaaatgtcaaagccacatgtgtcaatgaacacagccccacttctcctgcagcacagcaatgactcctgtccagttctgcacacagtcccacacacggggccagaatgaaagtcggccccaacagagtcaccaggcacccaaccagaccaacgccatgctgtaagaagaaaaaggggcctctttccaatggaaacaaatctgagccagcatcttcagctctgggactccaagggagaggcaggtatcacaggcaagttgcagggtacagctgggagatgcacacaccacacaaggacacacacagacacgcatgtacaaacacgccacacgcagacacgtgtatgcaggcacacaacacacaggcgcacatgcatacacaggcgcacatgcatgcatagacacacagga

SEQ ID NO: 11727 - RNA, 4649 nt, Homo sapiens
  source 1..4649: mol_type = other RNA
ctgaatagctgggactacaggtgtgcaccaccatgactggctaattttttgtatttttagtagagacggggtttctactgtctactgtgttagccaggatggtctcaatctcctgaccctgtgatccgcccaccttggcctcccaaagtgctgggtgtttttaatttcaaattccacttgttctttgctgacatataggaaagcagttgacttccgtgtattaactttgtatcgtacaaccccactataatcctttattagttccagaagtcttttttgttgcttctttcagattttcattacctgctttttctttaaaaactttgttatactgattgaaaaagcaagaaaatttctaacaggcacaatggacagtgcattagctttctagggctgccactacaaagccccacagactgggcgaagtcaacaacagacatttgttctctcacagcccggaaggctggaaggccaaggtcatagtctcagcagggctggctttggaccttggcttgcagacgccgttctctctcagttgtcacagggtcaagcctctctacgtatgtgtgtcctgatctcatcttctaatatggacaccagtaatactggattagggtgcaccctgacgacttcattgacccttaatcaactttaggaccccatctccaaacacagtcacattctgaagtatggggggttagggcttcaacatacaaatttgctggtggcggctgtgaggcggggagcgcaattcagcctataataagtatattctttaaatggcaaaagtatgtgcaaaagcagtcatttactccttaattggaacgttatcctactacactgggagcttgtaccatttgaaaacattaagccatatgggaaaaatgtagaaaagaacatggaatacacggatttgtcccatgggaaaagcatgcttagtgtaaccccgtatctaggagacgtgaagggaactttttccttctcacttgtcttctatccttgaccagaacggtgtctgtggcactcatcacatcgcaggttagacaggctttctgagccggcctggaaatggaatcaccacacagaatattacgtctgtgggaagatgtgttcagagtcaatggagatctgacctgtggggctggaaggtgatttgtgggatgacgaggacctgcctgctgagatcctggtgcgcagctccattataaggtgtgtgaaaaccagagaccacgcagctctcaggaacacaaatgcgtggagaacaaatgcccagtgagagaccaccactatacaaacacgaacgagacccccagaaatggcacccaggaacccacgtctggcttcatagacttatgtgtttactggggaaccgaatggacccgcccacatgtgctgcacccaggcggcctcttctggcatctctcagtgggatgtgctgcacccaggcggcctcttccggcatctctcggtgggatgtgctgcacccaggcggcctcttcccgcatctctcggtgggatgtgctgcacccaggcggcctcttcccgcatctctcggtgggatgtgctgcacccaggcggcctcttcccgcatctctcggtgggatgtgctgcacccaggcggcctcttcccgcatctctcggtgggatgtgctgcacccaggcggcctcttccggcatctctcggtgggatgtgctgcacccaggcggcctcttccggcatctctcggtgggatgtgctgcacccaggcggcctcttccggcatctctcggtgggatgtgctgcacccaggcggcctcttccggcatctctcggtgggatgtgctgcacccaggcggcctcttcccgcatctctcggtgggatgtgctgcacccaggcggcctcttcccgcatctctcggtgggatgtgctgcacccaggcggcctcttccggcatctctcggtgggatgtgctgcacccaggcggcctcttcccgcatctctcggtgggatgtgctgcacccaggcggcctcttccggcatctctcggtgggatgtgctgcacccaggcggcctcttcccgcatctctcggtgggatgtgctgcacccaggcggcctcttccggcatctctcggtgggatgtgctgcacccaggcggcctcttccggcatctctcggtgggatgtgctgcacccaggcggcctcttccggcatctctcggtgggatgtgctgcacccaggcggcctcttccggcatctctcggtgggatgtgctgcacccagatgttctcatcccacgtctctcagtaggatgtgctgtacataggtggtctattcccgtgtctctcggtgggatgtgctgcacagaggtgacctcttcctgcatctctcggtgggatgtactccacccaggtgttctcttcccacgtctctcagttggatgtgctgcgcacagccggtctattctcgtgtctcttggtgggatgtcttacacccaggtggtctattcccgtgtctctcggtgggatgtgccgcacccaggtggtctattcccgtgtctctcagtgggatgtgttacatccaggtggtctcttcccacatctctcagtgggatgtgctgcacccaggtggcctcttcccgcatctctcagtgggatgtggtccacccaggtggtctcttctcgtgtctctcagtaggatgtgccgcagacaggtggtctattcccgtgtctctcagtgggatgtgctgcacccaggtggtctcttcccgtgtctctcagcggggtcctctcacagtctcacaggtgagcggagttgcactgcagggaccagagctgatgggactctcatggcagatgatcctgcagccaccaagagcttaacatggggctgtcatgggacagacgtctgtcaaaggctcagcatgtttctggctcactttctcagaggtcactttctttggtggattttggacggccagcgtctggggttccctctttccttggccacttggaacaggaggaaaaagtctctgcagcaccttctccacaaacactgcaggccagctgctcaggatgctgcgtcaggaggattactggagaaccagcccggacaacatagtgagatccgatctcttcacgggcggctgcaatagttttcattaagcactggtaaacacacccagcgggatgcgagcagcccaggggcttccggagaggccggcactgccccgacgggggcgggacctcagagcagcccactcagttctcggagtcagtttctcaccaaaacaaggctgggctaaaacacgctgagaggtcattgggaaggccgttcagcaagctgctgtcccctccggcttcctgtctgctgtcctctctggcttcttgtctgctgtcccctccagcctccgtgcctgctgacccctccggcttcctgtctgctgtcccctccggcttccgtgcctgctgtcccctccggcttccgtgcctgctgtcctctccggcttcctgtctgctctgttctcacaggcacaagggtcccctacctccgtgtctactgcacccagcggacaggaccagcggcagtgaccagcttgtgactccatcagaaccttgcatgtgatcggtcacctggctgggtcctcacggtgctgccgcccactttacagatgagccacctgagcattagtagagtgagctctgaggcagcagcccagcaggactgacctcggtggccatccccatcgagacctaggcctgctgtgcactgaggcgccagccgtcagggatgggcacattgggcatccaccacctcctcggcccacttccctctccagctgtacaccaagcacgactctctcccaacctgcaagcagccgagactgcagctgcccccatgtctgagcagctcctgcaaccctcctccagccgtcgcagtaccgcatctcttcatccccacgtgctctggccttgccatccctgcacctgcccttccctgctggggccgaccctcaccccccaacctcaccatgcaccaacactcccgcaggacctggctggcacggcgcctcttcctttgccaggattctctaaacctccctgttccatgaggctgattccttccttcttctctcccctccttcgttcattcattcagtcattcacttgggaagcgctcctgagcacgttgtccttccttgaagatgggaaaagaggtgccaactcctgttctggaggaaggattctaccacatctgagtagaaaatgtcaaagccacatgtgtcaatgaacacagccccacttctcctgcagcacagcaatgactcctgtccagttctgcacacagtcccacacacggggccagaatgaaagtcggccccaacagagtcaccaggcacccaaccagaccaacgccatgctgtaagaagaaaaaggggcctctttccaatggaaacaaatctgagccagcatcttcagctctgggactccaagggagaggcaggtatcacaggcaagttgcagggtacagctgggagatgcacacaccacacaaggacacacacagacacgcatgtacaaacacgccacacgcagacacgtgtatgcaggcacacaacacacaggcgcacatgcatacacaggcgcacatgcatgcatagacacacagga

SEQ ID NO: 11728 - RNA, 4707 nt, Homo sapiens
  source 1..4707: mol_type = other RNA
ctgaatagctgggactacaggtgtgcaccaccatgactggctaattttttgtatttttagtagagacggggtttctactgtctactgtgttagccaggatggtctcaatctcctgaccctgtgatccgcccaccttggcctcccaaagtgctgggtgtttttaatttcaaattccacttgttctttgctgacatataggaaagcagttgacttccgtgtattaactttgtatcgtacaaccccactataatcctttattagttccagaagtcttttttgttgcttctttcagattttcattacctgctttttctttaaaaactttgttatactgattgaaaaagcaagaaaatttctaacaggcacaatggacagtgcattagctttctagggctgccactacaaagccccacagactgggcgaagtcaacaacagacatttgttctctcacagcccggaaggctggaaggccaaggtcatagtctcagcagggctggctttggaccttggcttgcagacgccgttctctctcagttgtcacagggtcaagcctctctacgtatgtgtgtcctgatctcatcttctaatatggacaccagtaatactggattagggtgcaccctgacgacttcattgacccttaatcaactttaggaccccatctccaaacacagtcacattctgaagtatggggggttagggcttcaacatacaaatttgctggtggcggctgtgaggcggggagcgcaattcagcctataataagtatattctttaaatggcaaaagtatgtgcaaaagcagtcatttactccttaattggaacgttatcctactacactgggagcttgtaccatttgaaaacattaagccatatgggaaaaatgtagaaaagaacatggaatacacggatttgtcccatgggaaaagcatgcttagtgtaaccccgtatctaggagacgtgaagggaactttttccttctcacttgtcttctatccttgaccagaacggtgtctgtggcactcatcacatcgcaggttagacaggctttctgagccggcctggaaatggaatcaccacacagaatattacgtctgtgggaagatgtgttcagagtcaatggagatctgacctgtggggctggaaggtgatttgtgggatgacgaggacctgcctgctgagatcctggtgcgcagctccattataaggtgtgtgaaaaccagagaccacgcagctctcaggaacacaaatgcgtggagaacaaatgcccagtgagagaccaccactatacaaacacgaacgagacccccagaaatggcacccaggaacccacgtctggcttcatagacttatgtgtttactggggaaccgaatggacccgcccacatgtgctgcacccaggcggcctcttctggcatctctcagtgggatgtgctgcacccaggcggcctcttccggcatctctcggtgggatgtgctgcacccaggcggcctcttcccgcatctctcggtgggatgtgctgcacccaggcggcctcttcccgcatctctcggtgggatgtgctgcacccaggcggcctcttcccgcatctctcggtgggatgtgctgcacccaggcggcctcttcccgcatctctcggtgggatgtgctgcacccaggcggcctcttccggcatctctcggtgggatgtgctgcacccaggcggcctcttccggcatctctcggtgggatgtgctgcacccaggcggcctcttccggcatctctcggtgggatgtgctgcacccaggcggcctcttccggcatctctcggtgggatgtgctgcacccaggcggcctcttcccgcatctctcggtgggatgtgctgcacccaggcggcctcttcccgcatctctcggtgggatgtgctgcacccaggcggcctcttccggcatctctcggtgggatgtgctgcacccaggcggcctcttcccgcatctctcggtgggatgtgctgcacccaggcggcctcttccggcatctctcggtgggatgtgctgcacccaggcggcctcttcccgcatctctcggtgggatgtgctgcacccaggcggcctcttccggcatctctcggtgggatgtgctgcacccaggcggcctcttccggcatctctcggtgggatgtgctgcacccaggcggcctcttccggcatctctcggtgggatgtgctgcacccaggcggcctcttccggcatctctcggtgggatgtgctgcacccagatgttctcatcccacgtctctcagtaggatgtgctgtacataggtggtctattcccgtgtctctcggtgggatgtgctgcacagaggtgacctcttcctgcatctctcggtgggatgtactccacccaggtgttctcttcccacgtctctcagttggatgtgctgcgcacagccggtctattctcgtgtctcttggtgggatgtcttacacccaggtggtctattcccgtgtctctcggtgggatgtgccgcacccaggtggtctattcccgtgtctctcagtgggatgtgttacatccaggtggtctcttcccacatctctcagtgggatgtgctgcacccaggtggcctcttcccgcatctctcagtgggatgtggtccacccaggtggtctcttctcgtgtctctcagtaggatgtgccgcagacaggtggtctattcccgtgtctctcagtgggatgtgctgcacccaggtggtctcttcccgtgtctctcagcggggtcctctcacagtctcacaggtgagcggagttgcactgcagggaccagagctgatgggactctcatggcagatgatcctgcagccaccaagagcttaacatggggctgtcatgggacagacgtctgtcaaaggctcagcatgtttctggctcactttctcagaggtcactttctttggtggattttggacggccagcgtctggggttccctctttccttggccacttggaacaggaggaaaaagtctctgcagcaccttctccacaaacactgcaggccagctgctcaggatgctgcgtcaggaggattactggagaaccagcccggacaacatagtgagatccgatctcttcacgggcggctgcaatagttttcattaagcactggtaaacacacccagcgggatgcgagcagcccaggggcttccggagaggccggcactgccccgacgggggcgggacctcagagcagcccactcagttctcggagtcagtttctcaccaaaacaaggctgggctaaaacacgctgagaggtcattgggaaggccgttcagcaagctgctttatgaaaatcaggagacaccagataaactacaccttttactccaatattgttattttttccactttcattaaacattggctttttccttagataggtcctgaattcagcccaaagaacttgcaacccataagggattccacaccgacaagccccgtgttgtttgcacgggcaggttacgctcactgaggaacgctatcaaagatgtggaacccagaacccgggaagcagctgtacctcctgcacccacgccgcctggcccggaccacgagggagccacggctgccccattgtggcctcctggaccccacttcttccctgcgccagccacgaaggaccatgtggtccttttcgggtgctgtggtttctcgtcccacaccctgacgcagtgatgcctgctcacctgctgacccctccggcttctgtacctgctgtcccctccggcttcctgtctgctgtcctctctggcttcttgtctgctgtcccctccagcctccgtgcctgctgacccctccggcttcctgtctgctgtcccctccggcttccgtgcctgctgtcccctccggcttccgtgcctgctgtcctctccggcttcctgtctgctctgttctcacaggcacaagggtcccctacctccgtgtctactgcacccagcggacaggaccagcggcagtgaccagcttgtgactccatcagaaccttgcatgtgatcggtcacctggctgggtcctcacggtgctgccgcccactttacagatgagccacctggctggcacggcgcctcttcctttgccaggattctctaaacctccctgttccatgaggctgattccttccttcttctctcccctccttcgttcattcattcagtcattcacttgggaagcgctcctgagcacgttgtccttccttgaagatgggaaaagaggtgccaactcctgttctggaggaaggattctaccacatctgagtagaaaatgtcaaagccacatgtgtcaatgaacacagccccacttctcctgcagcacagcaatgactcctgtccagttctgcacacagtcccacacacggggccagaatgaaagtcggccccaacagagtcaccaggcacccaaccagaccaacgccatgctgtaagaagaaaaaggggcctctttccaatggaaacaaatctgagccagcatcttcagctctgggactccaagggagaggcaggtatcacaggcaagttgcagggtacagctgggagatgcacacaccacacaaggacacacacagacacgcatgtacaaacacgccacacgcagacacgtgtatgcaggcacacaacacacaggcgcacatgcatacacaggcgcacatgcatgcatagacacacagga

SEQ ID NO: 11729 - RNA, 691 nt, Homo sapiens
  source 1..691: mol_type = other RNA
ctgaatagctgggactacaggtgtgcaccaccatgccaggctaagttttgtatttttagtagagatggggtttcactatgttgcccaggctggtctcgaacttctgacctcaggtgatctgcctgcctcagcctcccaaagtgctgaaattacaggcatgagccaccgcgcctggcctccaaaagaattttccaaaatggtgattctcccattaagacaaacggtcatgggaacgtaggcaagccactctgaattctctccaagaccttccactgtggcctgttgcgcatctgcagaatcctgcagcagattgggaatcaggggccatttcaaacacgtgttattaagtcaggagcccagtatgcactaagtgtcgtgggagcacagccagccagtgtgaccccacgctgggggcaaggagccttgcaccaggactacacagcctgagttccttcttgacttgaccactttgtcttggacctgtggtttgccttttcttactgtcagtgtcttcaccttgctgacaccttgatcttggacttcccagcctccagaactgtgagaaataaatttttgttgtttaatccatccagtctgtgatattttgttatggcagctgaagcagtcaggaaaggatcctccccatctctgcagaagcctgaccatccccctagagggcctgggaggaagt

SEQ ID NO: 11730 - RNA, 6500 nt, Homo sapiens
  source 1..6500: mol_type = other RNA
ctgaatagctgggactacaggtgtgcaccaccatgcccagctaatttttgtatttttagtagagacggggtttcaccatgttggccaggatggtctcaatctcttgacctcatgatccatctgcctcggcctcccaaagtgctgggattacaggcatgagccaccacacccggctggctatttcttaaaaaagaaaaagaaaaaaaaagtacaaacatgtgcttcacaggagaacaaaatttcgtgaagatgaaacactccctaaataagattgtgtggcagaagaagatgaagaatagaaacatgaacacaatttccaagatggaaaggatctggaagactggtcccatccatatatgttgtctttcttgcatttgaatgataagcattgtgatgcagattgcccagcctgcagattagtgcctagcacaccaaaggcattcaacaatatttattgaacaaacaaatgaatctcctctgcccacaagtttgtacagctgtggagaccacctaccaaaaagtccctagaagcctaagatggttgggcttctttgatacctgttttgatagctgttaacagctgaaaccactaggttaacagcttaaaccactaggttccccagatgaagagattaaatcaacattaatatttggtccatattctaatatccaggtaaatatatagaccatgaactgctggttttgaaagtcctcagactttggtctttttagttctgaactgaaatctcaaaattcaagaaaaaaggcatcagtactcaaaaaatcttatattttatgctatatattagattctgttgttattaaataatgatacatacgaatacctcagtctgttgatatctattgaatctgttgaacctggcaagacctactttaacattaaggactaaatctctaaaattaatcatgcatgtgaccttggacaagccccattcctgtagtggcataatgagaataccggactagatcaatggttctcaaactttgctgcctgttagaatcactttgggagctttaaaaaaatcttgatgtgcaggctgcaccccagaccaatttaatcaggctttctggacacacgaactgggcatcataggttataaatcaccttcaggtgataccaatgaacagcctgcagtgaaaactactggattaggggccctctaaagttccttgctcttctcaaagctgggattctttagttccaaaaaggtgagatgacctctcctggaactagaatttctctccttaatatgtagtctatctttttcaaccaacttggattaaactgcctaagcactccgatatatcacacattcatgcccaaactgctcttcagcaatgctggggcttggaggttctggcttctgataatgcagggtttaaggaactagatttttgctactggtcaaaagctcccacttagtccctgagggtgtatgcaccaggagtatgtgacggaaagtttttctgctcctgtaattttgtcagaccttcagatgggtttgcctaaaggaccaagtagaaaagtgtacatattcaccattctcccttctcctttctcctatacacacgtgctttgaaaacagaaataggcaaagtgctttacctattcagtttccttcccctgctttgcttttctaatgtgaaatcatgtctcctattgccaggagaggagtttcttgaacttgtccatgacaagctggatgattaagttaattaactgttctgaattggtaagggcaagagtattcatacttaacaggctcccacagtactgtgcttagaacgacttgcccatcctccccaatacccctgcccctgcaatgtaagaggttcttacattagtgcatgagagtaggagagcagggtccagaggcttgatttattgacagccatcaaatgccaggtactttgtatcaccttgtttcaacctaggatgctggagctgtccctgttttacaatgaagaaaacctggcctctgagaggccccctgatttgcctaaaggcatacagttggtcaatggaaatgcctagatttgaacccaggtgtaagtgagcaaaatttcactctgctgagcacatcgtgaatgaggaacagataaagcaagaacatggctgggagagagagttcatttctattatctgttcacctacacttaaattaggaagcaggagagtgtacccaaaagctcagagagaggacagccaactaactgtgcagcagttcagaaagaagtttcaggacttcctgaaagacaggagcaggccattcaactccttccctcctttttccttcacattctaactcaacacaaccctaggctcaggaaccagcgcacccctccttccatctacccttttatagtcagtccacaatccttattccaaaaataaatcctcctgatgagatgatgagaggcaacaaaaagcaaagctaaaaagttttatgcttttgttatgggacattatttggacagaattattatcatgtttttacaaatttccctaaaacaaataattctggatatacccaaattactccagcctcctggcccaatatgtttttgcaattacttggcactccaactctatgcaacttaaattagttaacagtcaccaagttatttttaggccatagcaacacacacactctactatacctagcttgttatttgtactccttaggaacaaaatttgcctttgtactggcactatcatttcctttcaatcaatatcaataaaaacattctaccatatttatggagtgcttaccatgtatgtgtataaagttctgaacactttacacacattaattcatttatttcagaaactaacactttgagatagctattgttatatcctctttttgttaatgaggtaactaaggaactgaaggattcagttccttccccaagggcacatacctagttagaggggagccaaggctagcattcaggctgactagatccgaagttctgccttgatttctccatcatttgctacaaggctaatgtttgacattttagccttggatgttaaccagaggctcagaataacaacagcacgtttatgaatgtagatatgtctttatttcaggtattttttaaaatcctcataacatctctgagagaaaaggggagacttttattcccttccccaccccacccccgaaaaaagggcagaaacagaatatttttcacaggtctctgatttctgagcctagccatccactttgtcatagaactctattgccaataagagtatatttcagaattcttttcaactagggaaaagtgtgcaatgtatggtgctcaattctaaggagtgatgaagttttatagtataaaggcctaactgcctgcatgatcaaatcctccccatggatcatccttttaaaccatttccctcttcttctcacattcccccagtaaaggcctttggtacagagcagtcctataaagattgtagcagttggtcattccttgttttacaacagcatagagcaagtagaggcatgggctctgacataccagggaggaagggggacacacagaccccaaggaggcacctggagccctcctactcccagggagggaagctcctctgtagacctgactgccagtcagtcacagagggattcgaagttgaaaagcacttaaaaatgggtacatgacactcaagtgtttacgagtgaaaatgttcatagtatactataaaatatttccagctttattgaatttgaaacattaatttacacattaaacatacttaaatacattaaaacattatctatatttttaaatatttcaacagaaaagagaaagcaaataggaaaaatataattgtttaatctggttgataggtgtatggatgttcattacacacttttctgcttttctatatgcttgaaaatgtttataataacatttttgaaggcatatactgtctttaagaaaaaggggcagtagactatttcttcctacctaagtaaatgacaaattatttccctggacccagctttactgaaaagaaagggagcctgaaaaactttatagcaaaaacggtagctctcgttatggatggtctagaattgttcaactttcttactcagtttgactagaaagcaagttttagttgattaaaaatcagctttgagtaaaacaatataattctttcaaagacctcacaaatccctaaatatttattcatttggatcattttcaccaggttgaagagaagcacaggtctgatgccatttattctttagaagatgagactaaaacatagattctagcataggtcacaacagggagggcactgtaaattagaacagtaacttaatcccaggggctgccatgcctctgatcggtttcttcccaacctgacacagcattactaaaatggcaagttagcagccgctctacttgacagacagcaccaaaaatggagagtatggcatggagacagggggacaaggatcttggacagggagggtagcaaccagtgtttacaaacataaaccagagcatcagatgggccagccataaattacccaagattgtactgaaatctctgaaaataaactaacaagcctttagaagtttcctccttatgttctaactatgcccccctcccaccaacttccctgcaaaaattactccttccgaaatggtaccactaccactcttgctgaaacacaatcttatcaccaagggaggggattactcaaataaatctgagaggagaagccagaccagaatggtctgcttgacccactcaagaatctgagagaagtctgctggtcatgcctttggggaatgcccaccccgtctttcaccacagtggtgctatggtattaatctctggtttaccaagttgaaaggataacgaagggcattctaatattgacccattcctttcccttcttttccatcttggtcccaattttaggccattctcccaaaagataccaaaatgataatgataattataaagtagaatatagaccccttcactcctgaactacatattttcaatgaaattcccagatatttgaagaaaaggcccccaaaactacaaataatctaacctctaccaccagagcatcttccaagtcgactgccgcggtgtctcaccaactcgaaaatgacgaggcctcgcagtggctgcccagggcgcccagtggtgaggtcagcagtgtgtcctgccccgccccattgaggcaatcttactctgacactgaggaagaagtctaggctgtccagaatctcagctgcatccacaggaaagggagagaggatcctcactttcacaagtagcacccaggagattcatttctcaatgactgatgggtcacccctatccacaactccacccactgcaaaatagagagtagggtctgcaactccttgtaatcatccccatgattaggaggtctaggatcatcttgatccgtgttgtttcctctcttcagatcatgaagacacaaaagacttgctttttatcatgaacacctttcaacaccagaggttctttgccttctctcttcagggactcgaggactatgtgaagtggctgggagggcatcactcggcttggttcattggtattctcatcataaactataatttctttggaaaagatcctcttgaaagagtccttgccttccctacaggaaatcaagtctaggacagtgatcttgccctgctgcagtctccgccggctgatcttatcggcacagttaatgtggacagctccttggatgtgactcttgttgtactccatgaagggcctgcagtcaatgatgacagggccctgactcggcaggtgactcttgctgcatttggtcatcttctttgccaagtcattggggtagattattttgatgctggctagctgcttgggggtccctgacacagggctgcccaccccacttgatggacttagagagcctgtattctcattattgttgaccatctggttagcagggcaggtggtagaggttccgatggcagtggtggtggtgccagcggcaatggcttgggtttgggcctgattgtccttgtcgtaggttgccacagtgcagcagctggcactgctgcatccacaattcagcgagcgggcagagccgctggatgagggcatatacgtcagattcgcagccttgagggacacaacggtggtggcgatgacaggagggtggctgttactgcctgggttggcagagccaaggtaactagagtctaaacaaaggttgagatcctgaggtcggacgggcctagatagtgccactactaccctgtcgtctaaaggagacggaggcatgaggaggctgaaaactggcaattcaagaagaactcaagacagtttcataaataagtgtattcctccaccatctggcgctcctcttcagctatggactcgcacattcagcccccattcactcggcttcattgatctccagcagcaacatagttac

SEQ ID NO: 11731 - RNA, 12706 nt, Homo sapiens
  source 1..12706: mol_type = other RNA
ctgaatagctgggactacaggtgtgcaccaccatgcccggctaagttttgtatttttagtagagacgggggtttcaccatgttggccaggctggtctcaaactcctgacctcaaatgatccacccgccctggcctcccaaagtgccaccgctcccggcctgtgtatggtatttttctatggcatgtaattttctgtacacaccctctttctttcttaggcttttttgtcagcagcccaagatggaaaaggcagctttatgtcaaggttcgccaaagacagtcaagagctgtgaaagccaaatgttcacatttaactttttttaaagtatttattactcggcatcaatgtatttcttaatcattatcctgagtggacttttaagtaggaagaaaatggtgtgttcattactccaaagctgaaacacagttggggttgtgtaaggtgacagcaggtgagttggtaaaagagttagcagaagtgacggctttcgtttcctcaactactggattcaccagtaagccacatgagacctcagtcacaatcggtaattcaaaggtagatttaaatataaatatcctgttatttctgacacctttactgaggtataattgatgtatgataaactgcatatatttaaagtgtacaatttgttaagttttgccatatggctacacttgtgaaccataaccacaatcaagagagtaaacacatatatcagccccagaagtttccctttgcccttttgtaatcatttcccctcgcccaccccattccaggcaaccaatgatgtgcttgcattattatagattagtttgcattttatagttttacataaatgtaattatacattttgtacacataaactgctggcgggaatgtcaaaaggtacaattaacttgaaaaagacttttagcagttccttaaaaatttaaatatacacttatcatatgatttagccatcccagtcctaggtatttgcccaagagaaatgaaagcttatgtccacataaagacttgtaaatgaatgctcatagcagctttacataatagcccaaaactggaaccaacaaatgtccatcaacaggtgaatggtataaacaaactgttatattctataccatgcagcactactcagcgataaaaaataatgaatgattgatacataaaacaacatggaagaacctcaaagaagccagggcatctgggtctggagatttcttttatcaggagattttaaattatgaatttaattctttaatggttataggatattcagattatttcatcttggttgagttttaatagtttgtggttttcaagaatcagattatttcttctaagttgtcatgtgtataagccgaaagttacagtatttcctcattatctttttaatgactgcctgatttatagtgatactcttcatttcattcttgataataatgatttgtgttttttctttttgtcagtctttctacaggtttatggattttcttgattgttttttgaagaaccagttttttgtttatgtatttttctatttgcagtttcattgatttctgcttttggttatttcctttcttttgcctgctttgggcttattttgctattctttttcttgtttcttgtggtgggaacttaggttattgtgctgagacctttcctcatttctaatatgctatcttcctaggtattccctgggatgtaggagacagctcttggagacacatggggttggctatctggcttttggagagactttgtctaccacaagaatagagtaaaagcagactctttcaggaagggaagaggatggctgcctctttcatctttataagtagggaaaattaattttccctgtcccttgcctatgcagtatttggccacttacatagccaaaatcccatgagtttcttatcaggttgctctgggggatatggacgagtgcaaaggtgggcaggtgcacttgtttaccctgagtaataagaaatctatctctgactctgaacatcttatgtgcatactcaagataagaaaaataaagatgaatattaaaaagcaaactttttatgagtggatactggtttatcaaatactttttctggatctactgaaatattatttttctcctttcattctgttaatgtgttgaatcatattgattgatttgcaactatcacaccaacctcactttttcaggaagaaacccaacttgattgtgattattctgtgtgtgtaggggtgtgtgtgtgtgtgtgtatgtgtgtagtttagtttgctagtattttgtttgggatttttgcattgatgttggggggaatgaaataggtccctttctcataaagtttttgccaggttttggtatctaggttttctggcatcataaaatgagttggggagggttcctgcatttctactgctctttgtaagaatttaagattgtctttccattgacgaatcaatccatctaggcttgttgtttcactatggaaaagcaaataaagtaactataggttccacttctttagcagatagggaactactcgaattttctattttttcatttgtcaattttggctcttccatagtttaaagaatttattcacttcatctaaaatttccaactaattggcatgaagttgtgcacatattttgtcagatgactctaggatttgtaatatcctttcattcctgatattggttgtttgtgtttcttcctttttcagtctaccagacacttatcaattatcttttcaaagaatcaacttttggcttagttgatccactttatcttcattttctactccattaattcttgttctttattatttcctttattttcttcaggtttaatttgctattcttagaatattttaactactaggttcattttcaatcttttttttttaatgtgcgtttaagactataaatttccttctaagcatggctttaggcgtctaccataagttttgacatgtagcactttcactactcagttcaaatatattctaattttcattgtaatttattgtctgatccatgagttatttaaaagtgtatttcttaatttatgaacttaatagaatttttctatttttgaaattattattgatttctaagtgaatgatacatggccaaagaatatattccattcctatgacttggaatatggtcagttttgataaatattctatctgcatttgaaaataatgtgtattttgcagttgttgggtattctgtttcatatatgccaattaggttaagttttaaagtattattccaatctttacatatttacgtatttttgcatggctgctgttctgttactgagtatattaaaatctgggaatgcagacttgtcttttctcattttagttctgttcatttctgcttatatatttgaggctatattgttaaatcattaaaatattagacctgttgaaactttctggtgaatcaaatcttttatcattacaaattgtctctctttgtaatacttttcaccttaaggtctacattgaataatgttgcaatagccaccatagtcccctgccctatcgtttttgttttttgtatttcatattataatttttccattcttgtttacttcaaacctttgtattcctatacttaagacatctcttgcataaaggtactttgtgggttttctttcttttcactttgatgatctttgcatttaattggtacactgtctattcatatgaatgttgtaactgatatttaaacctcctaatctactgtttgatttctatttgtcctatttgttctatattttctctacctttttgccttattattccactttagccctgtattagctttgtagttctacgattgttttattttgctttttgctgttcttttagtggttaccctatagatgacacagcagtcttatttatactttaatcttctttctgataattctgaccttagaattcctgcaccaaatttgtatattattgtcacattttaacattatttattttaacctcgaagactattttatatagttaatattcacttaaactgtatatatatatttttaaattactgttcattcctacctttatctctaacctttttctgggatctttttccttctgtctgaagaataccctttactatcacctttaatgacaatctgctattaaatttgttgcgtttgaaagtgtctttgccttcattcttaagaattgtttttggggaaaggctgggtattgaattctaaaattgcagatattttctttcagtaacctgaaaatatcatgccattgatttctgcttcccatattttctgttgagaagttagctgtcagtttaataaaattgtgcctcctttaaaagtaatgtcttttatcattgtctggctcctttaatgattttctttttgtgttttattttttcttaggatgtgctaagttgtaattttgtttttatttatcatgctttgatcttgcaggtcttcatgtcttaaaaacttggagaattctcagtcattatctcctcacaggttgcttctgccatattctctcttctcctggaaatccagttacgtgtatgttagatcttctcaagttaactctatgtctcttatactctctactatattttctattcttttgtctcttagtttttcacatctggtatttacttctgacataacttctagttcactaattcttacttcactgtatgcactttctatcaaatctattcactgaatcctttttttttttttttctttttgagatggagtctcgctctgtcgcccaggctggagtgcagtggcatgatcttggctcactgaaacctctgcctcccgggttcaagtgattctcctgcctcagcctcctgagtagctgggactacaggcacccaccaccacacccggttatttttttttttatttttactacagatggggtttcattgtgttagccaggatggtctcgatctcctgacctcatgatccacccgcctcagcctcccaaagtgctgggattacaggcgtgagccaccgcgcccggcctattcactgaattcttaaacttgattaatgtacttttaagttggggacttgttgattgattcttctatatagtttctgattttctgctgaaattctcaatcttgtgttttagatctttaaacacactaaacatagtaattttagaccctgtgttgtatagctcattatctgggtcccctgtggctctgtcccatcatctgtcgcttctttcggattttcatcatgttgtcttgtttcctcagataccttaaataactttccaacactaaacatgaaaagttataaaaataactcaaaagatcagtccagagaggatttacatttgctctgggtagcggctgcagcaaagggtcacctgaatccagttttgggaagtgagaagatcctaactgcatctggtttttcttcacccttacaatttggatatggtccttggggtcacaacccaatgtatggtcagttaactaggattcctttcccctcccctacttccttggagagtcttggtctccagtttttgtccctctaactcagcagcaaggctgttataagtgttacttagcgtctcagactctcaaccaccttatcctgaattggcatgtctcctataagaaaagcagcccaaatgctgagctcaggtctctaagtttcattctgtcttagatcttagtgatgttattcttcactgtcttttggttctctaatgcctttaagcagattttaaaatactattttgcctggcattgctagttctctgaaatagttggtatgaatgcaccactaaaagttagaagtagaaaagtaggttttagggaaaattcagtaacgttagtgttagtccaaactgcaccattttgtaagctccccgctattttgcagaccttgatcaaagtaaaacatttcacaggggttcgggcagtgagaaacatgctgcctaaccacctgaccacaaggcggaaaaaggcccaacctaagaaatatccctatcatatcttgctgggcaaagttccaaggaatactatgatgacatcccaccacaacaagggccagaaccacctcatcatgggagcatcttatcaatatcctgccgagcagcaagccatactgcccagacccctctcacccatgcctataagtacgcccagcctgtaagcagcggtgggctctggcattaagctggtcccccacttctgtaggttttatgctagacataaagtctgcatttgctgtcaagctgccctctgtgtgtctttctttaactctcaccttcccttcaaaatctaacagtcagtttttaatataccaagtgaagataccaaataagtgatatatataggttcagtgtaagaagagaggttgggttaggtacatatatttgatcatcatcaatttattgatgatatttcaagtcttgaagtagatgagattatctatggtgattgcagaaacacaaaggggggcctagaatcaattgttgagaaattctaaaatttagaggtcaggtagaagaggagaggcagcaaagatgtttgaggagttgctaggaagataagaagaaaacaaagataatgtagtgtcaggaaagttcaaaagaaaacacaaaagctgcttcaaggaatggtcaaatgtgtcaattactactagctggtttgacaataaaaaggtcaatagtgaccttaataaaaactttttttttttttaatttgggagagtcatggagatgggatccagattggaatgatttgacaagtaaatgaaagagaaaacctggctatgaatgaaatggagatatgggagcactttgaggaggatgcaaggttaagcgaaggcatagcttgacattattatcacagtgaaaatctctaaacaacttaaaattcacattatttgggggacagtagtccaataaataatatctatcaatggaattttatgctgtcattaaaagtgataattatggctgggcacggtggctcacgcctgtaatcccagcactttgggaggctgaggcgggcggagcatgaggtcaagagttcgagaccagcctggccaacatggtgaaactctgtctctactaaaaatacaaaaattagccggcgtggtggcatgcgcctttaatcccagctactcaggaggctgagccaggagaatcgcttgaacccagaaggcggaggttgcagtgagctgagatcgtgccactgcaccccagcctgggtgacagagcgagattccatctcggaaaaaaaaaaaagctgataattacaagtacttttaacgacatgagaaaatatttctacatgacaaagatataaaggtgtacagctagcaaatctcaatcatgtaaattaaatcataagtctgagatgtaaactcagagtaatacaaaatcctatcttagtaactgtactatattacctccaaaaaaagaataacatacaaatctcttgaattcattaactgaaaattggtccaaaaagtttatcctttaacattgttagagtgaactcgtccacatactaaataaatggaatactaataacaacttaactggtacatttcatataatttgaatgatttctaaggagaatacattattataaatctagggggctcctactgatttcattggaaattaagtaagaattagaggaaactgatctctcaactgatgtggattcattattaatcccccttacatgtatctgtaaaacgttcctaagcaagaagagaatgaaaataaaattcagatcgtattataaaaattttcttccatctccttctgactttagttcatataccttaagacactagtaactggtagtcctgttgggtaaatcatttttcagaagcagtaaattcagttgaaagaaatacataatgagtcagatatatgctttagtagtcatatgcagattaccctaacattgctcttcctgtgaatattcacatgatgaatgggatgaaccccgctcctttcacatatattagaaggatatttgaaaaggaaggaaaatattttattaaaagttttttaaagtttatgaattgaagtctatgaaaacaaactacttgatacaaaaacattcagatattagatgtcaaaataaatcagcacatttgaaaatactataaattatatttcaaacaaatatatacacattatgttaaccttcaacaggatccattatcactacttagaacactgatatgtttatctcttaagtatgtaaaaattacatagctgttaactttgtatggcaattcacctataacacatttaagaaagcattacaaaattcattatatgataattctacaaaagttttctcacatttaccaaagcctactaaagtccagagggcacaaatattggccaaatagttcttttatcttagacataaagatgtttttgctgttttttagaaccattaagatggctaagagaaccaactttacggagcttagctgttctcaggcatctgaatgggggtgtggagaagtcctcaagttacaagaatcacagttacttttttaggatgaaaaaataaaaacattgcatttgatgacattacagtcaaaatgagctctaatacaaatgtatgtggagaggttttgaagaataaatcggatatcccaggggaggttctgctgcttgtaccgtaagatttcttaaaagtagtggatgagcttgtatactataacgttcttcatcatcgtttgtggcataaagtaattcccatgaaagattggcccactgacctctaacagcttcaggatttaactttcccacttggatcaataattcttgaaggctaagcactctcccagtgtaaattcccatattagaatcataccccagagaaaacaagtatggcttttcttgtaaaattgcttccttccacttttcatcagataccaaaccaatgtaccagtcacgttcatattcttcaaggtacttaatcagttctctaaagtcttctattggacctaaacttgctttatcaatcattagtttcagagtatacctgaatgctttcagtgctagttgaaacagttctggcttttctgtgagccagtccaaagcaacagaccaaggcaaaacaccaccgtaaactctcaatatatgaccaggactaggagccatattgtctattccaaataaactaaaataacaagtcattactgtatgaacataaaagtcttttaaaactttgtccttggcaatttcttccagtacatttgaggccttctcttctgaatgataacattccaactgccttagaacaaattggtaccagtcttctggaaataacgagctcatctccttcattttggaactgggcatacagctagtcctccactctgcgggtaagcatactaagtgagaatgtgaacaactgaactccatgagaggaatatatggcatgtcctcttgttttcctttgtcaacagcagggtatcctaatagaactgctttgtaaagatcgttttcaggaacagtgcctgtagaatgatcaccaaccctctgtgattctactgatcctggaataaacaaatttgtacctggcaaatctttcaactgatgtttttcttctattacttttttgatagttggctcatcatcaaaaatattatcatcagaccagtcattaaaagtttctgaatttaaactgtctatgtcttctggggatttgggaggtggcaaagtgttcaaagcaggcaacattagaggtgctttccctttattttcagtgttgtgaacattctctttcatgccaggccttttggagcagtattgaacaagtatccacacaagtactttaatgaggtcacctttaaattcttttaagttttcatgagaatcaattatgcctgatagaacattcctggcatcagaatacaatttcacaggcaaaacagtacagggtgtcaagacatttccaaagtgttcattaagggaacatactcttgtgtattcttgctcaaaagcatcttcaaaaacttcatcaactctgcgagcttctgcagtatgacaggatgtttcctgcaattctaaccccttaatgttaatagagcagtaagtatagccacattccagaatcattatccacattaaacgatcctgaaaacggcccaagtaatgagatccaggtaggaggagacctaaacttccagctgccattgcagtctgcagtacagcagtcaacctgggcaccatttggtagtagtacactgtatctgcacacacacaggctgtggtgcctgctgctcctggccaactctgaataggtcggggaaaccccaccaagaacacaggaagggtgaaaagagggagtaagggagaagagagtagtgtagaaaaaactatgatgaccaacacgaatggagaaaagacaatgttgagtatacataaagtggcagttgtttttcgacgttgttttttctctgtccatgatgtcaaaagcacagtcacggcaaactgcaatttagagatgaactgaatcaaacgatcacgtatgataccaaccagtaagagtctgagtcctgtatccaggcttctgttccaccatatgtctgtactggagatcaagtgtactgttgatacaatgactgtctccaataaagcattttctgtattctgccataccattctaaaggctcttgtgaatccaatacagacagacactgagtggagcccttgtaaggaactgtccaatgaaagaaatgctatcatggcaaaaggtgatactaaagttagcaaaatccgtctgacaataccaatcttcatgagcctagtttgcttctcaaagaatacagtcacagtttgcacatccttcggataaaagggatttcggaaaattccaatgatatatacgctttgaatttctctaagtatccacagtattataagtaatatcatcaaaccatagcccacaatagcctgggaattgcttttagaaatctgtgagaagccagcaaagtgatgaagcaagctagtttctaaaagagccaagactaatataatgatgtagaaaaggcattccttccatgaaaaatgtttttccggaccactgggtaaatccttagatttggttccaattttgtgacccatatcacttaagttcagactcagcaagaaaccaaatccagtcatgaaaagaaccacaccaacagtgcttggaatgaaatatgatgctatagctgttccagcagacatgatgaacattactaataaccgtaagtgggttgacatagatgagcctccaaggccgaactctaaaacctgctccattgcccataagagaagtgcatcgggtgggggcagagtcccaagtgcccacagaaagggtaaaaatacaaacaagatgtgtaaaatctgattcatgtgttctagagctggcatatttaccacaaacctgtgtgccagatccacagaaacaaagaaaaaaatataaagaggtctcataagaggaataatttcataagtatcctgtgtttggaaagtcgcagtctctgtagctgtgtttacaattaaagaatattctgctatacatagtgtcatccatccaaagaagaatagtagagcagtgcctcctgtactgccatacagcaaggttattctatttgggagcagataccatgttccaagaccacacgctaatccagcaagaatagaatgaaaaactgtattggctacatatttcttgccaggaatgagaaatttgacagtctcagcaccagtacaactggtaaattcatgctcatcctcctctgctaagatatccgtggttagtattctttctactgttgttgatttgtttttggcgtataaacttgtgaactggatgacaaatgcagtaaaaagcattaatccacctgaaagtgctgctgtataatagtctttcaggatgcctaactggtataaaagtgttccgactccaccccaaacccatggcattagaaaaagaataatttgattaacatatatgtaaggaggggcacaatagcctaatttgaatcgagggcctccaagaacagtctgtggaaagcgcttcagaaagaagtcctgcttgtaatcattcagtagaggcacatctggactcatcctcactcgggattattctgaaagtcacatgcttttctgtaacacagcagtttctcaagtcacccgagggaagagaagacgcgaaggcatcccagggaccgcatttttgcaggtaaactcgggctgggcgctcccgccgggaggttggttagtgcccgaatgcggaggcagaaaagctgcggcggccgaataacgagctcaccgcggccccgcccgggccagctctcggtttccatggctaacgtctactccggcggccgccacccggagctgaacggagcgcgtgcgcgttcggggacctcgtcggcgcctggctggcctcgctgccccggtctgtgctcgctcccgaggcgggccctgccgtaaagcaggcttggcctagaggaagcagggaaatagcgcgcttcgttcgcgccaggactaggccaacatctgcctggccggggacgacgggagtcgctcgtgctctggtctcgcactgggcctagcagaagcagcagcggggaaagccgagacgccctgaacgttcccttgggccgggcctttacgc

SEQ ID NO: 11732 - RNA, 6718 nt, Homo sapiens
  source 1..6718: mol_type = other RNA
ctgaatagctgggactacaggtgtgcaccaccatgcccggctaattttgttattttttgcagagatgaggtctccctatgttgcctaggctaagattctgcatttctaccaagctcccaggtgctgttactggcccgggaccgtaatcttgagtgtctaaggtctagaaagcctcttgcacccagaagtgacccagccatggatcctgtatcagactgcttgttctgacttagaattcagaaaatacactccctgcaatataaacccctggttctgcaaactgcccttcccaggaaaggcaaccgtccctgctaacctcctccccaggaaacacacacagtcaccattgcctgtcagagtgaagactatcacagaggtgacagggctcagtccaaccccgtgaaacccccagtgaggagccacagtggtttgcttctctggcctctccactgtctctcctagcaccattttcctggctgttctgttgttttataaaccggttccttgcaggtttcaggtatgctgtctctccagctgcagagtgagccccacggcaggggccgtgtgcccaccacctcaatgttaggttttgttgggtgggttgaatatggcttgaaataaggacccacctccagcagctcagtggtagaaggggttgtggctttaggatttactttgtggcttggtcactcctcaaggggctgtgaagctgtcattttcccacaagccttggccctcatgtcattgcatgctcagcctattcccagcaggcatggaaaccactcttggtgtctccagacaaactacggaaaggcagccctgtgggaacagcaggtattcctgggatccgcggtgagactccagctggaggagtgcaggagggttcaggccacgggcccagcagctactggttgccacctggcctcctgctcagctcccccactccacccagggtatcattttagactccagcacccattttattgcaaagccacttactcctccagccctgcctcggtgcctggaatctgcacatgctgccaagggctgaggccagaacagttttccaaacctctctgaccatggaaccgtaccctgaccctttctaatagagcatctcatggtcccagtgttctatggaacacactttggggaaggagcttgaatggtgacttagaaatgatctcagagtatgtgatgggtcattgtcaaagaaccgacatctaaaattctcctagaataacaaattagctaacactggaggtttattaggtgctaggcactgttctaaacaccttataagaattctgcgttcacaggccaggcatgctggctcatgcctgtaatcccagcactttgggaggctgagacggggggatcacctgaggtcaggagtttgagaccagcctggccaacatggtgaaaccccatctctactaaaaatacaaacagtaaccgggcgtggtgatgcttgcctataatcccaggtacgcgagaggctgaggcgggagaatcacttgtacccaggaggcagaggtcgcagtgagccgagatcgtgccactgcactccagcctgggcaacaagagtgaaactctgtctcaaaagaaaaaaaaaaaaaaagaagtatgcattcactactcacaacaaccctatgaagggagagttattattcccattttacagatgaaaaaatcaaggcacagagaccttaagaaactttcctaaggttgccaaagctgtgagaggtggaataggtggatttaacaccagccacactgctacagatggaaggggagagcagagactctccgccccagctgcacctgaagttacctgggagaaaaactatgaagcccagaccaaacaaaacagaagctttgtgggtgggccccaggcctgtgaatgttcctggattattgcaacgtgcagccagcgttgagagtgagcaggcttgagcaggggttggcaaaccgtgaccctcaggccaaatctgccccactgcctggttttgcgcagttggcaagcaaagagcagtttttgcacttttaaatggttttagaaaattaaactaataatattttatggccaggtgcggtggctcacacctgtaatcccagcattttgggaggctgaggcgggcggatcacctgaggtcagaagtttgagaccagcctggccaacatggtaaaaccttatctctactaaaaatacaaaaattaaccaggtgtggtggcacatgcctgtagtcacagctacttgggaggctgaggcaggagaattgcttgaacctgggatgaagaggttgcagtgagctgagactgagccactgcattccagcctgggcagcagagcaaaactccatctccaaaaaaaaaaaaaaggaaagagagaataatattttgtgacatgtgaaaagtatacagaattcacatgtgtgtccagaaatagttttcctggagcatagccatgaattcatttacacactctctgtggctgcttcgagctacggcagagctgagtagctggtggagatcagatggcttgcaaatcctaaaatgtttatttggctcctcacagtaaaagtttgctaaaccctggattagaggaaactggcttctgtatgagcaaaataaatttaagatagacctaaggaagaacttcctggcagagaggttggttagacacttgagagggctttgggattcccagctctggagttaagaggttccatccacccatccctctttggaaatgtcaaatagagatagctagggcaaagagacgggccttgaatttccaaccatggaactaccctggcaaccagtggcagttctatgggcattttagctttgtcctgaccctctgtgttctccatggctgatgtcctaggaccatctaacagctgtcccccagccatagtaatgctgggctttcttccggcggtactccttagggttctagccccacagagccagcacagtcccgagtcaccacttaatgtgaggcacacacagcatgtgtgggttgtctggtctcaagtacgaagctgctggcagatctgcctttttacatttttaagtgttttatatttttggagtctcactctgtcgcccaggctggagtgcaatggcgtgatcttggctcaccgcaacctccgcctcctgggttcaagtgattctcccgcctgagcctcctgagtagctgggattacaggcacctgccaccatgcctggctaatttttgtatttttagtagagatggggtttcaccatgttggtcaggctgttctcgaacgccttacttcaagtgatctgcctacctcggcctcccagagtgctgggatgtcagacatgagccctcgtgcccagccttaatttttgtatatttggtagagaccgggttttgccatgttggccaggctggtctcaaactcctgacctgaggtggtccgcccacctcagcctcccaaagtgctgggattacaggcatgagccattgtgtctagccatatctgcctttcagctagcctgctttgatctcccagttcccctgccctccctgctccctccccacaaggttcccatgcccatcaaacttggatagggagagaacaagcatatttaatttcttctagatctgcctgctttccttggtgcctgacccctgaccccgactgatttttccaacgcagtaaacatctctggcatcttatgggcgtgatccaggccagtgaggaatttggccaggaaagtcttttgtcatttgcaacctggttcgccctggaacagagggttggccaggagtgagatgccaagtggggggatttaaatggttctcctgaagtgacccctgaagccagatctgctgggacagatgtcctgggtgggcattgtgagtctggcctgttaggggcagttagcttcagatagcacctcaatttcaggtgagcctcaacttcccagtgggctctgctgcaaaaatgtggggtggggttccagggatggttttgtggtcctggaaatcactaaacagtatgcaaagtgggtaaacatgggcaatatgtgtggggtttttttggattccatgcttgcatcagaacccctgggggggaagtgctccagaaaactgtaaagtgcctgtccaggactggatgatcaggaccacagggacataaaggccaacatgattcttttccccaaacacttcttatcccaggatatcagctactagaccacagggatcaacctgcccaacttattcctgcaagcaagtatgtgcttaagttgtattttgttttgtttttaaacatgatacacctttatccagggaaggcagagaacagtcaagttattccagccacagaggaagggaataccagggtgtgagcctctcttgccaaaagccttagagaatctggaagaaattcttggctgtggagcagcaagaacgtgggccttggagctggacagccttggcccaggttcatgtccttgctctgccatgtacttcccaggacctctcagtgggtccctgggccagcagcctcgcgttccctgggagcttgttagagcacagagcccactgagtcagatgtgcttttttttttttttttttttgagatggagtttcactcttgtcccccaggctggagtgcagtggcacgatctctgctcactgcaacctctgcctcccaagttcaagcgattctggtgcctcagcctccgagtagctgggattacaggtgtgcaccaccgcgcctggcctaatttttgtatttttaatagagacggggtttccccatgttggccaggctggtctcgaactcctgacctcaggtgagccacccgccttggcctcccaaagtgctgggattacaagcgtgagccgccgcgcccggccagatgtacatttttaactggacctccaggtgactcttagcatgttcaggtttgaggagcactgacctgggaccctgggcaagtcgagtcaaataactccagcgtgcctcacggtcctcaacctgtcgcatggtgataatgcctacttgaaaaggtcgttgtgataattcaatgagataatgtattccagcacttagcacagtgcctggtacataggagatgttccatattcatctcctgatggtggaccttctttcgggaagtttaaatttcttttccactctcaaaaacgcctcttggttttgaacttgaagctgttgcagtgctggagtcggacagtagagggcactctcggcattgccatcgcggagagcaagacacgcgggatggaggctgcgtgggtccggacttcgtgtgtgcaggtgctgcgggccggctcctgggcacccacccagctcattcgccgagcggctcccctcctggggttgagtgtcctgggcctgagtctgcagcctcagccatctgttccccaacttgatctcccactgctagttacaaacaaatcgcccggcttgtgcaaacctcctgggctcagtccccagtcccgcggggccgctagacgttgatgaaggatccctggtcgccgttggccgtctcgggctccacacagcgccctttcctccgtgtaaccctgcggttccggtggaatttggcatagcagcgcagcccttccacacacatgcagtcatcgaagcatttgttgttgaggcctcggttgtggggtgtgcagagatgctcccgcaggtcgcagcaagtccctggcaggcagtcttggtgatggtcgcatggttccccttcggctggtgatgtttcgttaccatcactggagagtttaccgcggtgtttctctttcttctttgcagagggccaaccatcaggttttaagtcttcataatcggtccagtcgaacaaggccatgtccagcgtgggcatcacctccccgtcagacctgggctgtgcctgctggggccgcagggaggtgacgggcaggatcagggactcttctgtggcaggtgctgcctcaaaggtggtgagaaagaacatggtgggcgccaggctggtggaggattcctccatggctgcatccagcacctgggcttcggagagctctgccttcttcatcagggagctgggacctcggaccaaggctcggccttggtgcagcctcaacctgtccctgcgtctcttgtgctccctgctgcgtttcctggtcctctcccaacctggaggtcggttctccttctcggggtagggcaatgccagtcccaggagcaggtccttgtcctgcagcaggcctgcaggactctgctcaggcagcagcccctcagcctctggcagcctggaggcctgcctggtggcggtgaccacagccccatcctgggcctggctgggcaggcctgggccccactccttcttgcccgggccccgccggcggtggtggctggcctgaggcgtccacagcgctgggcctgggaggtcaatgtgattctcagggaggttccgggcaggggtcccaggtgcaagggcgcctgccaggctcagctccaggggcagcaggaggacgaggaacagcatgggagcggtgtggatggcaggcccagccattggctcctccctgtccggccggcgggtagggggaggaggggctcggggccgagcgcccgcgggagccgagcgcagccgagggcgagccgcggaacggggccggcgtggagaggtgcgcgggcagccggaggatgtgcccgggctgagcgggact

SEQ ID NO: 11733 - RNA, 977 nt, Homo sapiens
  source 1..977: mol_type = other RNA
ctgaatagctgggactacaggtgtgcaccaccatgcccggctaatttttgtatattttgtagagatggggtttcgccatgttgcccaggctggtcttgaactcctgagctcaagccatccacccacctcagcctcccaaaatgctgggattacaggcatgagccactgcgcccagccaagacagcattttagatcattccaaacactgctaggggaattttcgtgaggctgaaagtgaagggtttaccagagtacctgatgaaggcaaaggggaagtgctcttgaatccaactgctcaacttcacctcgtataagtgaaaacagagactgcagaacaagctttggcgcctctggctgctcattagcatttacttcagcagcttcttcatcatcaacagcatatgtgactgcgcttagtactttttcttgcattaaaggtgcaatatctcctgaaaaaagtcctggtggtatcttcttagcagtcccttttttgcttcttggacttctttttccaggaatttttttgtcctttcccaagaaggcctgttcatctctggaggcttcacaaagggtgttttgcaagttctcacctgcagccacctcgcagctcaatgtgcagctttcattattattgagactgtcctgctcagacacttggggctttcccatcgcactgtcactgctggtcagatgctcatgcccgtccccgtcaagctgattttcattttcatctgatgcagaaggcagacaggtcacactcctttccacgctgtcaccaggatgacatccatcttgtggttctatttgcagataatatgtaggagtatcgctgtcatccattagagcatcctttggtgaaccatttaaagttacattaaagaccttccatgtctgggaatcggaggcgcaaggagggctaccgctgggcgccgggtctgtttccagccccactcggcgacatggcggccgacgtgctg

SEQ ID NO: 11734 - RNA, 19767 nt, Homo sapiens
  source 1..19767: mol_type = other RNA
ctgaatagctgggactacaggtgtgcaccaccatgcctggctaatttttgtattttttgtagagacaaggttttgccatgttgcccaggttggtcttgaactcatgagctcaagcgatcggcccaacacagcctcccagagtgctgggattccaagtgtgagccaccacaccccgcccatttcattcttatttggtgagattgtcacagacttggctgaaacttaacaagaaactgtttacagcaacaaaggaagcaattaaagttaacatgatcattcaactgtgccattcatcatgcacttattgacatgctcaaaataggggaatgttaagtaaggaaatgaagtgggaacaggaacaagggagctaagccaagaggacttccagggacttgaacaaaaacaattcccaaccacatactacttttcaagcattttgaaactcttcttttcctttagtgatgttttcagtaacaaacttgcaagtgttcttggtggttaaaaaacaaaacaaaactacaagtatcagctgagaaagacaaagaaaaaactaagaatttaaattagataattccatttaaagtttccaattcctcgtttaggtggagttggaacattagaactcaggggtggtttggatattaacaaggtactcctgcctcctcagaagctacagtcttttctgcagctctcttatgtacctctcatcaaaataatttcagtcccacatttctcggataaaaccacatctgtggttttatccagcaaccatttcacagtcgactggcacgtgttctccaatttcagttccaaacacacaacacagaatcacacttttctttattaaagggacccaagtgatttttaagctgtattcttcctgctagagaatgaattgagtagcatccttctctaatttcctacaataaaatttcctatgtgatatactgcatatatattatatctgatatatgttttgattatttttctttatggaagcaaatacagaatttccttgtcagatcactctgatgattataatctgctactttgattatgcatcagtgaaatgtccaccaagcagttgaaaacactgatgtacatgtattctaaaacttactaaataatgggccagtaagataccagtatctttctagaacgtttagaaagagatcttagttgccagagaaaactcagatacaacatgagcctctaaacacatacactctagtctacaaatatgagacttttcaactcaacaataagtgggccgaaaacaatatagggcgtatgacctagactccctgggtgctgctcagcagctgcttcagcatcaaattgtgttcatcccattttctaatctaaccaagcacttggaactaaagggctgtatgtgagcccaagaaactgatatattaaatatttttcaccacatatgacatctttcattcagtactgcctgttagtcaattactgtggattctttcagggttcatcaatgcatgtgtggctcgatggtttaggaataaatatattctggctcaatgctttccactgaaatgaaaggtcacaacttctatgttccctatcaaatgtgtaaagcaaaaacacaacaaacgaaaacaagaaagtagagttgtttgttgattatatacagtcatgtgctgcataaaaacgattccatcaatgatggaccacatataccatgatggtcccataagattataccatatttttactgtaccttttctatgtctaaaatgtttggatacagaaatacttaccattgtgttacaactgcctacagtattcagtacagtaacatgctgtacaggtttgtagcccaggagcaacaggctggaccatatagcctaggtaggtagtaggccgtgccatctaggtttgtgttaagtacactctgtgatgttcacacaatgacaaaatcacctaaggatgcatttctctgaatgtctccctcatcattaagtggggcatgactgtatttttttttctctttaaggaaataagaccctactgtaatacaagtcggcagaatctaactgttactaataattaatgtaatccacaagtcaaagttttttcatgcatcaccaaaaaaaaaaaaaaaagtaatttgcatgtgtttgcatccgtttctgtattcaaagaaggtatgtagagtctccacccatcatgtctccagtgacaattttttttttttttttgaggcggagttttgctcttctcgcccaggctggagtgcaatgacacaatcttggctcactgcaaagtctgcctccctgggtcaagcaattctgcctcagcctccctagtaactgggactacaggtgcgtgccatcacgcccagctactttttgtatttttggtagagacagggtttcaccatgttggccaggctggtctcaaactcctaccctcaagtgatccacccacctcggcctcccaaagtgctgggattacaagcgtgagccaccgcgcctggcctccagtgaaaaatttaaaaaggatacaagctcatacttgacgaagtattcaactatgtagtaaaatcaccatgattttatcctgatttgcaccttgagaattaaaatagtcacttgattagaagggaattatcaaataaccaaaggaaaaacattttgctgggctgttacagagataatcctgaatatttggaaaggggaattagaatgatctcttactttaagaatttctgaaccaaacaccgcatgttctcactcataggtgggaattgaacaaagagaacacatggacacagtaaggggaacatcacactctggggactgttgtggggtggggggaggggggcgggatagcattaggagatatacctaatgctaaatgacgagttagtgggtgcagcacacgagcatggcacatgtatacatatgtaactaacctgcacattgtgcacatgtaccctaaaacttaaagtataataataatttaaaaaaaaaaaaagaatttctgggccaggtgcggtggctcacgcctgtaatcctagcactttgggaagccaaggtgggtggatcacaaggtcaagagttcaagaccaacctggccaacatggtgaaaccccatctctactaagaatacaaaaattagccaggcgcggtggtgtgtgcctataatcccagctactcgggaggctgaggcagaatcgcttgaactcggaaaatggaggttgcagtgagccgagatcacaccactgcactcccgcctgagcgacagagcaagacgccgtcttgaaaaaaaaaaaaaaaatttctgagttggggtgagaaatctccctgagtatttctaggctcttcgctcatgtttttgagggcttcacttgataatgaccatgggaagaatctggggtgcaaagttccacgtgcattagccgaaattattcattcaactagaaagacaattttgcatccactaatacataaaaatcagaaaggagaattgggaaaaagcatattcttagaataacatttagcatccaccaaagtgaaggacataggtttctggcacagttgaaaccttagttggaaaaccaaaccttggcacagtgccaattatttatcttttgatcaggacatttgaaataggcagagaccaccaaaaaaggacaaagtattgaaaagtagctgctcattttttactgccaatattcctgaactttaaagaatatcacacctaatcaaccgcaatagaattgggcattcagacttgattcttagatgaatttccaataatttttaaatcattgatctggcttggtaaatagctctccaaacttctacagctaatggaaaaatcacttaacctttactagaagtaacagaaagcattaaagttgaaacctaatgcagcagttctttccagtgagttgaactgccttagcagaaatcttcccattgagatacaggctttatttttattattatatttttggagacagtgtctcactctgtcacccaggctggactcacaactcactgcagcctcaaactcctgggctcaagtgatccttccagctcagcctcctgagtagctacaggcatatgtcaccatacccagctaatttttttcattattttatttaattttattttttagactcgctctgtcgcccaggccagagtgcagtggcgcaatctctgctcactgcaacctctgcctcccgggttcaagcgattctcctgcctcagcctcctgagtagctgggactacaggtgtgcaccaccacgtccagctaattttttgtatttttagtagagatggggtttcaccatgttggccaggctggtctcaaactcctgaccttgtgatctgcccaccttggcctcccaaagtgctgggattacaggtgtgagccaccatgcccagcctatttttttatttattttttgaagggacagggtctcgctgtgttgccagagttggtcttgaacttcctgggctcaactgatcctcctgcctcagccttccaaaatgctggtattacaggtgtgtggcactgcacctggccagctttattttaaggcactaataataaagggtatgaaaaaagctaggaataagtcagatctttccagaaataaaagacaattttaaaaaacatcagttaacctgtctggcctatttcaacatctaaagaggatagagaatgtaaaagttttcatgcctacctgattcagctcttttccattctcccaaacacttatttccatgtctcagatttacatttcctcaaaaggcagtagagatttggaaacaacaacaacaacaacaacaacaacaacaaaaccaccccaaaacaagcaagcctagtttgtagcctagtctcatgattaatgaattccctaatgctggcatttagcccacatactgagaggccggaactgtaacaaggtgctcttttctagtgttgtaaggggaaaatgtataaggaaaattaatttttcataatcaggtaaatataatttgttaatagcaaaacaagaaattccggagagaaaaaagatttactctgaaacaccagttccagcaggatttccctacaccttccaacgtattctactttgccatgagaaaaaaactaaataaataaaatggggttcaagtcagttaggcgagcaaacaccaaaaaacgagtgatttcattgtggaggtaggcatgatggggcaggatttccctcaagtggaaatgcttcctgtgcacacacacgtatacatgcacacacaaacctgtacactcacactaatttcaaaagcatggatgtggggaaagccctgccagcatgactagacatgaggagttagcccatctgcctgtatctctacacaggctctgacgtacattccacacccatagacagtcatgcacgagagccagcctggcttgcacacagactgagaatcagatctggagactcctagagctgctgcttctacaggaattattagtaactgcaggattatacttcctgttgatgtgcagggtttttatcttgctcttctttccagacatctccccttttcaagagtactaaatcttgatttagtggagggactaatcttgattcttcgatgggcatgacttagaacaggagctacaggaattaaaactagcaacaatagggcccctttgggattggggtgaagaagtatttcaggatttaaacagtttctgtgggtggggcggggggaaagcagagttcttggtggaagtggatgacctctgtgaaggagatgaaaatgcctccaagtccagaaatcaatataaacaaacaaacaaacaaacaaaaatgaacataacttaaaggggcttcaactaaatatcactgcaactgagtttgttgactcaagaaattctgctctgacgcagggaattgaaatataagaactgataatatttcttcttcagaaggctaagctgggagtgccatggcgggtattgagggtgggatagagacaagaggcttgaggctcaggttttgctcctagggtttcttgcctgattttgaagggaagggtgctagagcaaatggatcagcagctggcagctccgtagtcctggaggaaagggatgtgatagaaacagacccagctatcgactgcttgttggtttgtgaaacaattttgtaggcagcaatgggctgggcttctggacttggctcgtcttctgggctatagtgacgggaatacttggataaggactgggggcggaatggtttgccagccatggggcctgagacagcttctttctggagctgaggtcctttgtttctgtcattagaatgacccccagattccaggcaggatcccctgggagagatgctgtccagatggtctgctgcttgtacagaatgggacaggaggttagactgttgcacaaaaccagctgtggaatactgagcttggacagaggtgtacacagctctctcacggcccgcgggcagggggacatcacctgtctgactgaggagaccggtctgtgcaggcagctcctgggaggtgcattggataactgttaactcctccatgcttttcttcttagtgaaaggagctctcaaaaacacgtctgactcctctggctgggaaggagccatactgctcttggagacaaatggggctttggagaaaatgtccatgtcatcatttggaacccttgagctcctgaagggagctatggcaaaaacatctggctcactgagcccatcagtggctggctgtgtgaaggcttgaaactggttctttcttccaccttgcactgtctttgcttgctcaggagagacttctggtggagcgaatggaacggctcctcccagcttccccggggggggtctgcagctctcatcttcttcttcagactccataaggagaggccgagacccactgcagtccagcatgtctccttcaaggtcagtcccttcctcttcgctgctgtggaatgagctgttgcttgaagggccatctctggccaagtagtcagattctaagttgttctgagtctttgtgccaggtactctggaggggtctggatacagcggaaggcctttaacacccagtgattctttaaagtgctctacagttattacaggacagggattggactccctctggagatctagaaaagcataaaatgcagaattaatgtgtaggtcaattcaactctatttggaacatttaatggtcaacccgcggcaaaaacattgtgggaccaaataatagatgttgaaaatgcaacaggaaaaacataaaaataaaagtcaggcaaggaaactgcacacaaactggaacacaatcaaccactgtctcacgttttggaacatgataggcacgacgtacaggaaaggagatgaagatgttaggcacacagacattcagcgtaactatgcaatgctcctacacacagggccaggcacggacacctgctctacctggcactggctcattatggaatgaaaacaaacccagtcattcatctccacatataccatgacagttttggattatgtagaaacactgtctggggatgactcaattcagaatctggcatgtggtcatccgcgccacatgcagagggacaaactctctgaaaagaagcagaatgtggctgcttgataaatgcaagtttacttgatgacttacatcacaagcactactcaaagagcatacgagtgcccaaaatataaatactgaaggtaccttctgaggggagcatacagcatcaaaatcagaccaaataaatcaccttcagctggagttgccccagaattttgttttcagtcttctaagttcataaagatctcctctgcttaaatgaatctgccataaagttctttaagcagaaggagtaaaatgcatgggccattacagaagcattagcaaactccaatatactagtctatttctatctaggtagaggtgcctcagggtgctctggcttttaaaatcaaatagacaattatcagaatgcaagagagcttaccttccaagaaatattagcaggttagaagtatgtcattgggcacatgttagcaagagggcaggaaaaaggcatatgtaactaagcaagaagaatccagagaaagggtggttgggggtaaaggtatcatttcatcatgggctcagtaaagagatactactggagtttcccaacccaccaggataagaatattagatacaatgatttggagccatagatgacccagaacctctgtagagatggaactcaatgatccccttcccatactgaccctctcccctcctatgcaaaccattagctagcagaaatttctgccaaaaattatcccctgctaaagtttctgcatgaattaagcacacagaccacagcagaagaggcattaaaatcagtttattgggaaaccagtcacttagagacattacattgtaaagagaatgtagagagaggtctgaacattttataagatactgtacaaaaatactatgtttctctgaatcctataactttttagcagtgcttctttttaaacagttctgaccttaaatattgttttcagaaacagaacaaaaatgtgtttgtcctccatttttattttcctttctaacagtttgaatgcgttcagtgaattccagattggggcgttaagttaaattctgtactggtgccaaatggctttcagaatagtatttgaagaataagattttgaaaagaataaatttttccttgtattataattttagtatgtgcagctacatggtgatacgaaagcatcagtcagtggacaggaaataaacagaataccttcttccttgcgatttatgtggacagacataatcctaatttctcaggcaagtaaattgatattagatttgtctcagtgataccaagatgataatttctgggaggaaattcaaataaaagggagaaaaataagttttccaaaataaggtttgcagagccttaaagaaggacaagagggccctaaaactccttgaaccaccttcctcacatagtatcagttggacaaagttttcagttgccaaaacaaaagcacaatttctcatcttccaaaactaccttgaaagttgatgttattaagcttgttctgcaggagagcaaaatatctcttagggaaaaaaaatggaaaacttagtcaagccagtgaccaactctggcatcatacaggtcaataatccaatgaacactagtttgaacagagtcagtgttttttggaaatttaaactgaattcagttaaaacaatttgtgcacagagactggcaaaaaagcagctatctattgaaccaggggcactttggatgcctgaagtgctagattacattttgagaactaggaagtaccaaggggtgtgtgtatgtgcccatattcagggttggagaggatggaagaacatgtctaacccatcaaaattatttgttaaaaagtgggtttttggtcgagaacccatttggaaaaccttccaactcagagcatattctatgaccttcatgatgagtactgggaaaatcagacttaaaattccaacaactttgaataatttacaaaaacagtcacaaaaacaccagaatatcaagtttgaagggaaaattagtctcctgtccttcaaaacaaggacaagagctatttcctatctttctttcagcatcaacaggctttgtaggaatggaaaagtacatttaaagggttgtcctgagaaggccaagtcccttaacctttctattcttgttagaggaggtacagtgtggctgaggcggagagcaaccacactttgcaactctccaggcctggcactctgaagggcaaagaaatgccagagaatatgggggaagcccagacctccacattcccttaaggaattctggtggtggcagcaccagaaacaaggtagtcgagagaaggataaattccaaatatactagaaacagaaggtaaccattaaatcttgttggcagataaaagtctttttttgagtatgtgaatgtgttcttacagggaaaatgtgttttcagggtgaacagttcctttatatgaaggtagcattgtgtcaacaagaaaacgtgtttgaagcagtctctttactagcattgaaggatttatactaacctaaccacatgccttgacccagttcctttggtaaccaatggcacgtcatagcagataccctgtggccatagagctcagtaaacactgcctgttgtacctcaggggctaaagcccagggcctggcttcatagtctgcacagggtcttacttatcatagagcctaacgtagggttttgttataattccctcaaactggatcatgcctctttttattttggtttcacacataaaattaagcaagaagtcaaaacatacttctttttcttgctctgatgtaggactgtgtgccaggttaggcacgttgacactttcaatatgggtaactccatattagtctattttgaggctccaaattatgtagatttcagcaagaactcacatgcttcagggaagagaaggagttcctaaaatacctgacaacttggcaactatcctcaccagctccctattcacttccaaagcaacccaaagtgctgaatcatttaggatgggtttcccctggaaactccatctgattgacatagtgagggccatcagaatgctccctacagaattaaaatctgaagacttaaatgtcaggctggatattccttaatgaaatacatcacacaacaccagaagtttacttttcctcataccaaaaactgaaagaacggttacagggagtatcaaagatatgattcttgccaaaaacagaaaacgaagacttggagcattgagaagaagccttctcacatatagttagtaaacagaaagcaaaatatcccttcacaagaacttggaaatgcagcagcaattgaaacgtaaaattttagaaccaaactggggaaatcaagagacgtacatcaaactaataattaccatgaccttctagctcacataacaaaattaagcatttggttccaccatatattaggtagctgcattaaaacccacgactgggaaatgagggacctcatggaagccaaaaatggccagctgtgcctctcaggccaatgaggcaattaaatgagtgagttttctcactggggataaaattattcttgccaacacaaaatgtttaattaagttggcctgggtatattagggattaagttagaggagggaagctgcaaacctgcgctccattttacaaccctgagtctggtcatatccagtgtaggctggcaggcgtcttattctccttgagactaaaacaggggttttactctctcaggtagccatgattcattaatatgtcctcagtgtgtagctatacttttcttgtgcccaggtacttattgtcactcaatactgtgattaaatcctttctgcaaaaaagtgggttttcagctcaggaaaagagcaacttattttaagttatttacatctctaaacatcatgctcccatttgaacagataaaagtctttattcccctgtatgtttacataagaaagttctttacagacttttttttatacaatacttgtgcagcaatgttcaaatttcacgtttttactgcataagatatcttcatgtacaactgtatgctttgtcttcttgggaaggacgcgttaaagacctatgataaacacacatccacatgacaaaggagagtgcaatagggcagagtagaatactcacaggaaaagagtaaattcaggtcactacatcaaagtgtgaaccaagaacgtgtctttaattctagcaactaccaccatttggtaacttctttgcataggttagcattacccaaggagcctccctatcccgtattagtgaaaggaaatctgggagaagcaaaagaggtttcttgttatagatttcctagcactcattctgatttaagaaatctaagcacatccaacttcagaaacattactaatgtggaaaaagaaaaggctgactttgtgttgataaaattatagcctttagagaggaataaagatagctttgcagtatctggagtgtttcaggaaagcttccattctaaatattcatgtgatagtttttctgttctgccaggcagcctctaatttgcttaacccggcacactgggcaatcctgtcattttcatcccaaagctcaaagttagtggctatgggagcctgataatcttgcagacagagaaggttaaggactctgggaaatcacagaaaaaccttatcaagagagactttattttggcccaaggtatctatagcatgtatttatttagctgagtgcagatccctccacatcataggctgtcagccccaaagatcccttcattcccacagcactgctgaaggcagaactgttcctaacctggggaaggttatattggttgatcaattatctgtcaggagagtaggaaataagtaatcaaaacaaccaaaagtattaataataaaacaaatattacatcttgagaaagtagttcgtttcttgggtttgtttttccacaagtattagcaatccaagttgtgtaattctaattcaggaagagcgaagtccaatatcaaataacactgaacaaagtgacaacttctttcagaggtgttttaatacccatatctttcaatgttttaaaccattctaaagactaaggaatcacagaagtttccttattcagaaaattacagaaattaagtcttaatcatgttcactttctattataaggtcctctctgagaattttttgtggattatcctttttactgtcttcaacagtaaccactcttcatcttacagggttgaatttgctttctggaaatggctaaatgttactcagaaccaagagtagtagaaaaagtagacaaagaaagaatatacttccaggtgctttctcaaagtgatactaattaaataatatagctgattttcttataccttattaccttccttgatattatttctaaggagaggagtttcaaaaataactttaaggatggcagcatcattagaataagtattaacttcttaagtaaaactagatgacattgaggggaacaacacttaattagatgtcaaaattctgatatgtctgctaaagaaatcattaattataataattataatcatacttagaagtgtccacttaagccttatctcctctgaggtatgtatttttgaaaacattgggactcatttgaatgttgtaaagggaaaaatcaatttgtcatgttttctgctatagttactcctcttacatagctggaataaaagcaaatcagaaacatatgcttatagtatttgcccgttttaaactggtagatgcctgattatacatttaaaaagaaatcttctgataccattttattagaataggtaggtgtgtgtccacgcatgtgtttctgtaatacttaaaaaggaaaatctctaagattatgatttaggcttctattcagataatcaagaaagagcaagttagtaaaagcccattataattctttaaaatgtaaacactgctaccgtaatagcaggaactacagaagataactgaagaacatcaggattatataaatccttcatagcccttctcaatataataatatatacttaggaccctatacttctataatcttaaagaccatctagtccaaacccatcgtataactctaaggaacagcaactctgagaggtgaagtgcctgctgaaggtcactcagccagtggctggcaagggccaggatgagatcccaggtggcctgtcctgcccaggcctcttctcccccgaccctgttcaatccagctcaggtcccacacctgtaaaatgaagaggatggtggactagaggatggtctcaaaggtccctttgtagctcaggctatgattccacaggtaccaggacactatgctcaactcaaataaactctttcagctcagggatgatgctctaaaccaaggaaggctccgtttaccaaagcactcatatgtgttccttaacagaaaaatagttctcccctttgaggaggccttactctaaataagcccaagacaatttcttgtcattatctcccttaggcttctactgccgtctctggcttctagtctgctcattttcattaactgcctccattaagctttactgagccaaatgactagataatatatttcaatgtaattatgggtaatatatgaaaagaacaatttagagatacctaatttctaaactgtactcttcatagtttcaattaaattgagaaactagatatttcattatatttctaacatgtatatacgaaaaaaatcaaatatgaaaacatagaactcaaacattattcttatttaaaaataaacatttccttcattaatttatacattctttctatgtccaggaaagagaatacaattctgacctgcagcaattttcctgtccataaaggggtaaaccaagtcctattttcactgctatccaaccacagagagcccttcgtggatatcttttgctttttaatcctcggcaggaagcttgtgcctctctcagttttggaaatggtctgttattcaactagaggcctttacctagctcatcttgtttcagccagcacgggaagtatttaaagacagaaggaaggctggaagattcagacttttcctccaatgcctttcaaaggctactcgcacattcctagggtcaaaccttgccctccagaatgcagtgttttataggctgttgttgctgttaaacttttttcccccataaagtgcaaatgtgaggaagaagaaacaaaagtactagatagcaaaacaagcaaatggacttggaattttatttgtacagatctgattaactaagagtttcccttttgatgatggacaatggcactagaggaaaagaacaggagtggggttctctgtgcccacttcttttcaaaagggtgattttataaaagtgctttccacataaggaaataaaatacactttaatgagtaagtacatatagagagggtgaccatgaggcatgttgtcatgttagtgcaggggcctttatttattttatgaacaatatcctaaagttaataaagaactatgctttattatttttttttaatctaggaagccaaggaaaaccagctgaacatattccattggctgcagccttcaatttaaacatcagaaagaaaggtaagctgggcacacccagattgtgtccagcttgtcagcacacttatttctgattatctgaaaataaacaacatgcttattctagagacagaggacctgctgaaagcttatagcacacaagtctattcaaaatgattccatatgttacactgtaggattgttgtgtagttatacaagggaaagaaatcaaaaccctgtacagacacctgatatcagacttgaaatgccaagtggaaacagaactattcagcatcttcatttatacacaatttacaatatttgattcaaaataaaaatcacaagaaaaatacatctgtttctgctacaattccttcccctccccatcctccccccacccccgccccagtgaaaagtcttctaataaaaggtatcatattaccaccgtcttgttttggtctaattctgagatcccacttggaacagttaacatgaaaaggaatggcaatacttgggatttatataacgtacacattgtatccaaggatctcaaatacttgcagtcacgtctccagatctgagaaatcacggttcaatggaagccagaaagctggacgaatgctgggcaggttgcatggggtgtaaaatcccttggctaagtctatgatcaaacaaggtcaaagttggttggctagagctgggctcaatttctcttctcaaatatatactaccagtcagtaagttttaccctttcttaaaccacacacccatctccaggctactgcctagagttaagaccaactgaagtagccatgtcctcatgataatgcatcaggataaaaagcaaaaacagggaaatacattcatcagcatctggccaaaggagacgggggttgggagaattgatctgggaggccattcctagcaagaacgagacaaaagtgtcaattcactagtttcagttacagttaagcttttggtggagttgattccagcagaggtgaagctcatggcatctagtgcttgatttaagataatgctattgaagaagggtaatgagaaaacacagcaaactaacaaggaggaactggccaaggaatatctggagggccaaagtgattttctttccttatcatttctacaggagaaggcaaggggtaggagaaaagggctggagggccccttatttgcagatttttttaaaaaaatcatttttttcataactccgtaatgaaaatgtattttacggtatgaaggttacagaactgcatctgctactgggtcacggctacaggtctatgagctgatccaccagcagtaaagacctggctaggttgggaagactggactcagagctcccactgctgtttctagagtgcccaccttgtgggtttttggttatcaatacaggaatagggtcaaactcatcttcagccaccttgtccgagccctcagggacatcaaaacctgagatgagattactatcttctgcagctttatggactggagcagagattgctgtgggggcaaactcttccagaaggtcagtagtagggttagagagcagagagcaatcaagcagggaatcttccccggtgagagaatctgtgcgattcgaggtcacagattccgtctgagatgggaggcgctggggaactgggggctccagtcctggtatgagactctcaacagcaacatcagctttttcaattacagcatcagaagtgctaccaaaaggatctgtcataggcaagaggtcagggagcagaagagaagtgtcaggagatttgagtccctcaattagtttttctggtgcatcaggtacttgaagaggaatgaaaggatcagacacgcttagaagcgggaggccagagtccacagtctgcccacccttccttttttcagcagttccagcagaaaatgaggtcgtagcaaaagcatcaccttgggttgattgaaagcctgggatcaaactctcagctgagcctccaagcttctcgggatgtttgccttccccaagcttggcaaagtccttgtttagcagttcttcagctgtgagtttggagaaattatcgtcatcaaagggattccacgtagacccttctgaaggattataaacgttttgttgagaggtccgaggagagcctgatggagtggtggttgcagacttggacttattgagactggcctcagctgcagctgcctggagcagctgggttgatttgctggcagggaccccaaagactgcactgtgggttacgtcactgagaatacgcctgtgcccagcacgttgggttttgggggatgagggtggagtgagagatccaactttctgcccctggacggcaggaggtggggttgtctgaacctttggctgttgtcttactggggcttgaatcgctggctcctgggcaggggctggctgtggggctgcagctggctgtggctggggctgctgtcctgctgccatagtgggcttttgctgcaaggcagcctgctgagtcatcagctgttgttgatgcagggctgtggccagctgttgctgttgctgttgttgttgctgctgctgctgctgctggtagaaattctgcattagctgctgttgagagcctccttgggacaccacagggaactgagcaattgctggtttctgggttgctggatgtactgcctgaaactgctgagtctgggcctgctgctgctggtaaaacgtgcctgccggctgctgctgtgctggcggtggctgttgctgctgctgttgctgcttgaggaagagttgctgctggtgctggggtgtggcctgggcctgagcgggcagaccctgggcctgagtagaaggcgtctgctgtggagtgggaggagcctgtggctgcttggcctgagtttgcggcagaggctggctgggtggggcttggggttttggttggggaacactggctaaaaggccaggctgattgctggatcctgcagcctgaggtgggggctgaacagtggccctcttccggggtgtcagcgctggctggatgggaaggattcctgggttcggctgagtctgcccagctttaggcctctggcggggtgcaattgaagtctctgtggtgggaatgggatctgtcagtctggcctttggctgggtcttttttgcagctgcctcactggctttcactggttcaggaagctttgcaggaatgggagagttctgtacatttggaattgggcactctttcttgagtagcttaaatgagaagtaggacacctggtaaatatccggccttttgtcagggtctggttccaacatatacctaattaggcagtgcatgtcttgagaatatcgagaattatcaggaattgtgaagtttccatcacaaattgccacctgactttccccaaatggcaaagtgaagtagcataatttatacaacaaacatccaagagcccaaatgtctgccttcgtagtgatgattttgccactgtacaggttgaccatttctggtgctcgataggacagcgttgtgtatttcttaatctcatcttctactgcattgactccctcagtttgtggattctggaatttgttggtggcgcttccaaagtcacacaggacatagtggcctcggtcatgcaagaggatgttttcaaccttcaggtcccggtggataataggagttttgcactgatgcaggcgggcaacagcttcacaggtatcacaaaatatctggagcacttcattctctgtaaagcctgtttgcaggcgctggttcatcaggtttaccacctggccacctctacaaaagtccatcagaatgagcacttcccatacatcaccgctactcacgttgttgatactagaatcaatgtaacccacaatattcttgtgccctgaaagatccctcattatctggatttctctcttgcacacctggagatcatgctcattgttgacaaacatgcgtttcaaggcacatttcatcccattgcttgtcctcaccagaaatacaatagcaaatccaccttccgccaacacctcgtccactgtgacctgctgtcgcccgatgccgaagactcttccgatgtagccactgcccaggcccgaggtgctgccccctcctccgctggagccggagcccaggccagagccgccctgctctcgccgggagtcgaaaaacttcttcatcttgcgaatagggagcagcaaagcaaaataccgatggtttctagattttttttttttttttttttttttaagaaaagagatccaaggatttcttctcagatttcacctcggagaggagccacccgaatccggccgtgggggtgggggctgagggaggatgcctataggaatatgcgtgtcaatcgcgcagcgggtcccctcctcctccagaaagcgattcgtgtaagtttaaacttgagacggctcggcggccggcgccctgctaccagccccgcgacattgtcacggccgccgggccggcctgcgacgcagagaagaggcggcgctgcagcgagagccggggccgcgctcggctcccgcccgcccgccagctgatcccgggagcgccgggcggagact

SEQ ID NO: 11735 - RNA, 19649 nt, Homo sapiens
  source 1..19649: mol_type = other RNA
ctgaatagctgggactacaggtgtgcaccaccatgcctggctaatttttgtattttttgtagagacaaggttttgccatgttgcccaggttggtcttgaactcatgagctcaagcgatcggcccaacacagcctcccagagtgctgggattccaagtgtgagccaccacaccccgcccatttcattcttatttggtgagattgtcacagacttggctgaaacttaacaagaaactgtttacagcaacaaaggaagcaattaaagttaacatgatcattcaactgtgccattcatcatgcacttattgacatgctcaaaataggggaatgttaagtaaggaaatgaagtgggaacaggaacaagggagctaagccaagaggacttccagggacttgaacaaaaacaattcccaaccacatactacttttcaagcattttgaaactcttcttttcctttagtgatgttttcagtaacaaacttgcaagtgttcttggtggttaaaaaacaaaacaaaactacaagtatcagctgagaaagacaaagaaaaaactaagaatttaaattagataattccatttaaagtttccaattcctcgtttaggtggagttggaacattagaactcaggggtggtttggatattaacaaggtactcctgcctcctcagaagctacagtcttttctgcagctctcttatgtacctctcatcaaaataatttcagtcccacatttctcggataaaaccacatctgtggttttatccagcaaccatttcacagtcgactggcacgtgttctccaatttcagttccaaacacacaacacagaatcacacttttctttattaaagggacccaagtgatttttaagctgtattcttcctgctagagaatgaattgagtagcatccttctctaatttcctacaataaaatttcctatgtgatatactgcatatatattatatctgatatatgttttgattatttttctttatggaagcaaatacagaatttccttgtcagatcactctgatgattataatctgctactttgattatgcatcagtgaaatgtccaccaagcagttgaaaacactgatgtacatgtattctaaaacttactaaataatgggccagtaagataccagtatctttctagaacgtttagaaagagatcttagttgccagagaaaactcagatacaacatgagcctctaaacacatacactctagtctacaaatatgagacttttcaactcaacaataagtgggccgaaaacaatatagggcgtatgacctagactccctgggtgctgctcagcagctgcttcagcatcaaattgtgttcatcccattttctaatctaaccaagcacttggaactaaagggctgtatgtgagcccaagaaactgatatattaaatatttttcaccacatatgacatctttcattcagtactgcctgttagtcaattactgtggattctttcagggttcatcaatgcatgtgtggctcgatggtttaggaataaatatattctggctcaatgctttccactgaaatgaaaggtcacaacttctatgttccctatcaaatgtgtaaagcaaaaacacaacaaacgaaaacaagaaagtagagttgtttgttgattatatacagtcatgtgctgcataaaaacgattccatcaatgatggaccacatataccatgatggtcccataagattataccatatttttactgtaccttttctatgtctaaaatgtttggatacagaaatacttaccattgtgttacaactgcctacagtattcagtacagtaacatgctgtacaggtttgtagcccaggagcaacaggctggaccatatagcctaggtaggtagtaggccgtgccatctaggtttgtgttaagtacactctgtgatgttcacacaatgacaaaatcacctaaggatgcatttctctgaatgtctccctcatcattaagtggggcatgactgtatttttttttctctttaaggaaataagaccctactgtaatacaagtcggcagaatctaactgttactaataattaatgtaatccacaagtcaaagttttttcatgcatcaccaaaaaaaaaaaaaaaagtaatttgcatgtgtttgcatccgtttctgtattcaaagaaggtatgtagagtctccacccatcatgtctccagtgacaattttttttttttttttgaggcggagttttgctcttctcgcccaggctggagtgcaatgacacaatcttggctcactgcaaagtctgcctccctgggtcaagcaattctgcctcagcctccctagtaactgggactacaggtgcgtgccatcacgcccagctactttttgtatttttggtagagacagggtttcaccatgttggccaggctggtctcaaactcctaccctcaagtgatccacccacctcggcctcccaaagtgctgggattacaagcgtgagccaccgcgcctggcctccagtgaaaaatttaaaaaggatacaagctcatacttgacgaagtattcaactatgtagtaaaatcaccatgattttatcctgatttgcaccttgagaattaaaatagtcacttgattagaagggaattatcaaataaccaaaggaaaaacattttgctgggctgttacagagataatcctgaatatttggaaaggggaattagaatgatctcttactttaagaatttctgaaccaaacaccgcatgttctcactcataggtgggaattgaacaaagagaacacatggacacagtaaggggaacatcacactctggggactgttgtggggtggggggaggggggcgggatagcattaggagatatacctaatgctaaatgacgagttagtgggtgcagcacacgagcatggcacatgtatacatatgtaactaacctgcacattgtgcacatgtaccctaaaacttaaagtataataataatttaaaaaaaaaaaaagaatttctgggccaggtgcggtggctcacgcctgtaatcctagcactttgggaagccaaggtgggtggatcacaaggtcaagagttcaagaccaacctggccaacatggtgaaaccccatctctactaagaatacaaaaattagccaggcgcggtggtgtgtgcctataatcccagctactcgggaggctgaggcagaatcgcttgaactcggaaaatggaggttgcagtgagccgagatcacaccactgcactcccgcctgagcgacagagcaagacgccgtcttgaaaaaaaaaaaaaaaatttctgagttggggtgagaaatctccctgagtatttctaggctcttcgctcatgtttttgagggcttcacttgataatgaccatgggaagaatctggggtgcaaagttccacgtgcattagccgaaattattcattcaactagaaagacaattttgcatccactaatacataaaaatcagaaaggagaattgggaaaaagcatattcttagaataacatttagcatccaccaaagtgaaggacataggtttctggcacagttgaaaccttagttggaaaaccaaaccttggcacagtgccaattatttatcttttgatcaggacatttgaaataggcagagaccaccaaaaaaggacaaagtattgaaaagtagctgctcattttttactgccaatattcctgaactttaaagaatatcacacctaatcaaccgcaatagaattgggcattcagacttgattcttagatgaatttccaataatttttaaatcattgatctggcttggtaaatagctctccaaacttctacagctaatggaaaaatcacttaacctttactagaagtaacagaaagcattaaagttgaaacctaatgcagcagttctttccagtgagttgaactgccttagcagaaatcttcccattgagatacaggctttatttttattattatatttttggagacagtgtctcactctgtcacccaggctggactcacaactcactgcagcctcaaactcctgggctcaagtgatccttccagctcagcctcctgagtagctacaggcatatgtcaccatacccagctaatttttttcattattttatttaattttattttttagactcgctctgtcgcccaggccagagtgcagtggcgcaatctctgctcactgcaacctctgcctcccgggttcaagcgattctcctgcctcagcctcctgagtagctgggactacaggtgtgcaccaccacgtccagctaattttttgtatttttagtagagatggggtttcaccatgttggccaggctggtctcaaactcctgaccttgtgatctgcccaccttggcctcccaaagtgctgggattacaggtgtgagccaccatgcccagcctatttttttatttattttttgaagggacagggtctcgctgtgttgccagagttggtcttgaacttcctgggctcaactgatcctcctgcctcagccttccaaaatgctggtattacaggtgtgtggcactgcacctggccagctttattttaaggcactaataataaagggtatgaaaaaagctaggaataagtcagatctttccagaaataaaagacaattttaaaaaacatcagttaacctgtctggcctatttcaacatctaaagaggatagagaatgtaaaagttttcatgcctacctgattcagctcttttccattctcccaaacacttatttccatgtctcagatttacatttcctcaaaaggcagtagagatttggaaacaacaacaacaacaacaacaacaacaacaaaaccaccccaaaacaagcaagcctagtttgtagcctagtctcatgattaatgaattccctaatgctggcatttagcccacatactgagaggccggaactgtaacaaggtgctcttttctagtgttgtaaggggaaaatgtataaggaaaattaatttttcataatcaggtaaatataatttgttaatagcaaaacaagaaattccggagagaaaaaagatttactctgaaacaccagttccagcaggatttccctacaccttccaacgtattctactttgccatgagaaaaaaactaaataaataaaatggggttcaagtcagttaggcgagcaaacaccaaaaaacgagtgatttcattgtggaggtaggcatgatggggcaggatttccctcaagtggaaatgcttcctgtgcacacacacgtatacatgcacacacaaacctgtacactcacactaatttcaaaagcatggatgtggggaaagccctgccagcatgactagacatgaggagttagcccatctgcctgtatctctacacaggctctgacgtacattccacacccatagacagtcatgcacgagagccagcctggcttgcacacagactgagaatcagatctggagactcctagagctgctgcttctacaggaattattagtaactgcaggattatacttcctgttgatgtgcagggtttttatcttgctcttctttccagacatctccccttttcaagagtactaaatcttgatttagtggagggactaatcttgattcttcgatgggcatgacttagaacaggagctacaggaattaaaactagcaacaatagggcccctttgggattggggtgaagaagtatttcaggatttaaacagtttctgtgggtggggcggggggaaagcagagttcttggtggaagtggatgacctctgtgaaggagatgaaaatgcctccaagtccagaaatcaatataaacaaacaaacaaacaaacaaaaatgaacataacttaaaggggcttcaactaaatatcactgcaactgagtttgttgactcaagaaattctgctctgacgcagggaattgaaatataagaactgataatatttcttcttcagaaggctaagctgggagtgccatggcgggtattgagggtgggatagagacaagaggcttgaggctcaggttttgctcctagggtttcttgcctgattttgaagggaagggtgctagagcaaatggatcagcagctggcagctccgtagtcctggaggaaagggatgtgatagaaacagacccagctatcgactgcttgttggtttgtgaaacaattttgtaggcagcaatgggctgggcttctggacttggctcgtcttctgggctatagtgacgggaatacttggataaggactgggggcggaatggtttgccagccatggggcctgagacagcttctttctggagctgaggtcctttgtttctgtcattagaatgacccccagattccaggcaggatcccctgggagagatgctgtccagatggtctgctgcttgtacagaatgggacaggaggttagactgttgcacaaaaccagctgtggaatactgagcttggacagaggtgtacacagctctctcacggcccgcgggcagggggacatcacctgtctgactgaggagaccggtctgtgcaggcagctcctgggaggtgcattggataactgttaactcctccatgcttttcttcttagtgaaaggagctctcaaaaacacgtctgactcctctggctgggaaggagccatactgctcttggagacaaatggggctttggagaaaatgtccatgtcatcatttggaacccttgagctcctgaagggagctatggcaaaaacatctggctcactgagcccatcagtggctggctgtgtgaaggcttgaaactggttctttcttccaccttgcactgtctttgcttgctcaggagagacttctggtggagcgaatggaacggctcctcccagcttccccggggggggtctgcagctctcatcttcttcttcagactccataaggagaggccgagacccactgcagtccagcatgtctccttcaaggtcagtcccttcctcttcgctgctgtggaatgagctgttgcttgaagggccatctctggccaagtagtcagattctaagttgttctgagtctttgtgccaggtactctggaggggtctggatacagcggaaggcctttaacacccagtgattctttaaagtgctctacagttattacaggacagggattggactccctctggagatctagaaaagcataaaatgcagaattaatgtgtaggtcaattcaactctatttggaacatttaatggtcaacccgcggcaaaaacattgtgggaccaaataatagatgttgaaaatgcaacaggaaaaacataaaaataaaagtcaggcaaggaaactgcacacaaactggaacacaatcaaccactgtctcacgttttggaacatgataggcacgacgtacaggaaaggagatgaagatgttaggcacacagacattcagcgtaactatgcaatgctcctacacacagggccaggcacggacacctgctctacctggcactggctcattatggaatgaaaacaaacccagtcattcatctccacatataccatgacagttttggattatgtagaaacactgtctggggatgactcaattcagaatctggcatgtggtcatccgcgccacatgcagagggacaaactctctgaaaagaagcagaatgtggctgcttgataaatgcaagtttacttgatgacttacatcacaagcactactcaaagagcatacgagtgcccaaaatataaatactgaaggtaccttctgaggggagcatacagcatcaaaatcagaccaaataaatcaccttcagctggagttgccccagaattttgttttcagtcttctaagttcataaagatctcctctgcttaaatgaatctgccataaagttctttaagcagaaggagtaaaatgcatgggccattacagaagcattagcaaactccaatatactagtctatttctatctaggtagaggtgcctcagggtgctctggcttttaaaatcaaatagacaattatcagaatgcaagagagcttaccttccaagaaatattagcaggttagaagtatgtcattgggcacatgttagcaagagggcaggaaaaaggcatatgtaactaagcaagaagaatccagagaaagggtggttgggggtaaaggtatcatttcatcatgggctcagtaaagagatactactggagtttcccaacccaccaggataagaatattagatacaatgatttggagccatagatgacccagaacctctgtagagatggaactcaatgatccccttcccatactgaccctctcccctcctatgcaaaccattagctagcagaaatttctgccaaaaattatcccctgctaaagtttctgcatgaattaagcacacagaccacagcagaagaggcattaaaatcagtttattgggaaaccagtcacttagagacattacattgtaaagagaatgtagagagaggtctgaacattttataagatactgtacaaaaatactatgtttctctgaatcctataactttttagcagtgcttctttttaaacagttctgaccttaaatattgttttcagaaacagaacaaaaatgtgtttgtcctccatttttattttcctttctaacagtttgaatgcgttcagtgaattccagattggggcgttaagttaaattctgtactggtgccaaatggctttcagaatagtatttgaagaataagattttgaaaagaataaatttttccttgtattataattttagtatgtgcagctacatggtgatacgaaagcatcagtcagtggacaggaaataaacagaataccttcttccttgcgatttatgtggacagacataatcctaatttctcaggcaagtaaattgatattagatttgtctcagtgataccaagatgataatttctgggaggaaattcaaataaaagggagaaaaataagttttccaaaataaggtttgcagagccttaaagaaggacaagagggccctaaaactccttgaaccaccttcctcacatagtatcagttggacaaagttttcagttgccaaaacaaaagcacaatttctcatcttccaaaactaccttgaaagttgatgttattaagcttgttctgcaggagagcaaaatatctcttagggaaaaaaaatggaaaacttagtcaagccagtgaccaactctggcatcatacaggtcaataatccaatgaacactagtttgaacagagtcagtgttttttggaaatttaaactgaattcagttaaaacaatttgtgcacagagactggcaaaaaagcagctatctattgaaccaggggcactttggatgcctgaagtgctagattacattttgagaactaggaagtaccaaggggtgtgtgtatgtgcccatattcagggttggagaggatggaagaacatgtctaacccatcaaaattatttgttaaaaagtgggtttttggtcgagaacccatttggaaaaccttccaactcagagcatattctatgaccttcatgatgagtactgggaaaatcagacttaaaattccaacaactttgaataatttacaaaaacagtcacaaaaacaccagaatatcaagtttgaagggaaaattagtctcctgtccttcaaaacaaggacaagagctatttcctatctttctttcagcatcaacaggctttgtaggaatggaaaagtacatttaaagggttgtcctgagaaggccaagtcccttaacctttctattcttgttagaggaggtacagtgtggctgaggcggagagcaaccacactttgcaactctccaggcctggcactctgaagggcaaagaaatgccagagaatatgggggaagcccagacctccacattcccttaaggaattctggtggtggcagcaccagaaacaaggtagtcgagagaaggataaattccaaatatactagaaacagaaggtaaccattaaatcttgttggcagataaaagtctttttttgagtatgtgaatgtgttcttacagggaaaatgtgttttcagggtgaacagttcctttatatgaaggtagcattgtgtcaacaagaaaacgtgtttgaagcagtctctttactagcattgaaggatttatactaacctaaccacatgccttgacccagttcctttggtaaccaatggcacgtcatagcagataccctgtggccatagagctcagtaaacactgcctgttgtacctcaggggctaaagcccagggcctggcttcatagtctgcacagggtcttacttatcatagagcctaacgtagggttttgttataattccctcaaactggatcatgcctctttttattttggtttcacacataaaattaagcaagaagtcaaaacatacttctttttcttgctctgatgtaggactgtgtgccaggttaggcacgttgacactttcaatatgggtaactccatattagtctattttgaggctccaaattatgtagatttcagcaagaactcacatgcttcagggaagagaaggagttcctaaaatacctgacaacttggcaactatcctcaccagctccctattcacttccaaagcaacccaaagtgctgaatcatttaggatgggtttcccctggaaactccatctgattgacatagtgagggccatcagaatgctccctacagaattaaaatctgaagacttaaatgtcaggctggatattccttaatgaaatacatcacacaacaccagaagtttacttttcctcataccaaaaactgaaagaacggttacagggagtatcaaagatatgattcttgccaaaaacagaaaacgaagacttggagcattgagaagaagccttctcacatatagttagtaaacagaaagcaaaatatcccttcacaagaacttggaaatgcagcagcaattgaaacgtaaaattttagaaccaaactggggaaatcaagagacgtacatcaaactaataattaccatgaccttctagctcacataacaaaattaagcatttggttccaccatatattaggtagctgcattaaaacccacgactgggaaatgagggacctcatggaagccaaaaatggccagctgtgcctctcaggccaatgaggcaattaaatgagtgagttttctcactggggataaaattattcttgccaacacaaaatgtttaattaagttggcctgggtatattagggattaagttagaggagggaagctgcaaacctgcgctccattttacaaccctgagtctggtcatatccagtgtaggctggcaggcgtcttattctccttgagactaaaacaggggttttactctctcaggtagccatgattcattaatatgtcctcagtgtgtagctatacttttcttgtgcccaggtacttattgtcactcaatactgtgattaaatcctttctgcaaaaaagtgggttttcagctcaggaaaagagcaacttattttaagttatttacatctctaaacatcatgctcccatttgaacagataaaagtctttattcccctgtatgtttacataagaaagttctttacagacttttttttatacaatacttgtgcagcaatgttcaaatttcacgtttttactgcataagatatcttcatgtacaactgtatgctttgtcttcttgggaaggacgcgttaaagacctatgataaacacacatccacatgacaaaggagagtgcaatagggcagagtagaatactcacaggaaaagagtaaattcaggtcactacatcaaagtgtgaaccaagaacgtgtctttaattctagcaactaccaccatttggtaacttctttgcataggttagcattacccaaggagcctccctatcccgtattagtgaaaggaaatctgggagaagcaaaagaggtttcttgttatagatttcctagcactcattctgatttaagaaatctaagcacatccaacttcagaaacattactaatgtggaaaaagaaaaggctgactttgtgttgataaaattatagcctttagagaggaataaagatagctttgcagtatctggagtgtttcaggaaagcttccattctaaatattcatgtgatagtttttctgttctgccaggcagcctctaatttgcttaacccggcacactgggcaatcctgtcattttcatcccaaagctcaaagttagtggctatgggagcctgataatcttgcagacagagaaggttaaggactctgggaaatcacagaaaaaccttatcaagagagactttattttggcccaaggtatctatagcatgtatttatttagctgagtgcagatccctccacatcataggctgtcagccccaaagatcccttcattcccacagcactgctgaaggcagaactgttcctaacctggggaaggttatattggttgatcaattatctgtcaggagagtaggaaataagtaatcaaaacaaccaaaagtattaataataaaacaaatattacatcttgagaaagtagttcgtttcttgggtttgtttttccacaagtattagcaatccaagttgtgtaattctaattcaggaagagcgaagtccaatatcaaataacactgaacaaagtgacaacttctttcagaggtgttttaatacccatatctttcaatgttttaaaccattctaaagactaaggaatcacagaagtttccttattcagaaaattacagaaattaagtcttaatcatgttcactttctattataaggtcctctctgagaattttttgtggattatcctttttactgtcttcaacagtaaccactcttcatcttacagggttgaatttgctttctggaaatggctaaatgttactcagaaccaagagtagtagaaaaagtagacaaagaaagaatatacttccaggtgctttctcaaagtgatactaattaaataatatagctgattttcttataccttattaccttccttgatattatttctaaggagaggagtttcaaaaataactttaaggatggcagcatcattagaataagtattaacttcttaagtaaaactagatgacattgaggggaacaacacttaattagatgtcaaaattctgatatgtctgctaaagaaatcattaattataataattataatcatacttagaagtgtccacttaagccttatctcctctgaggtatgtatttttgaaaacattgggactcatttgaatgttgtaaagggaaaaatcaatttgtcatgttttctgctatagttactcctcttacatagctggaataaaagcaaatcagaaacatatgcttatagtatttgcccgttttaaactggtagatgcctgattatacatttaaaaagaaatcttctgataccattttattagaataggtaggtgtgtgtccacgcatgtgtttctgtaatacttaaaaaggaaaatctctaagattatgatttaggcttctattcagataatcaagaaagagcaagttagtaaaagcccattataattctttaaaatgtaaacactgctaccgtaatagcaggaactacagaagataactgaagaacatcaggattatataaatccttcatagcccttctcaatataataatatatacttaggaccctatacttctataatcttaaagaccatctagtccaaacccatcgtataactctaaggaacagcaactctgagaggtgaagtgcctgctgaaggtcactcagccagtggctggcaagggccaggatgagatcccaggtggcctgtcctgcccaggcctcttctcccccgaccctgttcaatccagctcaggtcccacacctgtaaaatgaagaggatggtggactagaggatggtctcaaaggtccctttgtagctcaggctatgattccacaggtaccaggacactatgctcaactcaaataaactctttcagctcagggatgatgctctaaaccaaggaaggctccgtttaccaaagcactcatatgtgttccttaacagaaaaatagttctcccctttgaggaggccttactctaaataagcccaagacaatttcttgtcattatctcccttaggcttctactgccgtctctggcttctagtctgctcattttcattaactgcctccattaagctttactgagccaaatgactagataatatatttcaatgtaattatgggtaatatatgaaaagaacaatttagagatacctaatttctaaactgtactcttcatagtttcaattaaattgagaaactagatatttcattatatttctaacatgtatatacgaaaaaaatcaaatatgaaaacatagaactcaaacattattcttatttaaaaataaacatttccttcattaatttatacattctttctatgtccaggaaagagaatacaattctgacctgcagcaattttcctgtccataaaggggtaaaccaagtcctattttcactgctatccaaccacagagagcccttcgtggatatcttttgctttttaatcctcggcaggaagcttgtgcctctctcagttttggaaatggtctgttattcaactagaggcctttacctagctcatcttgtttcagccagcacgggaagtatttaaagacagaaggaaggctggaagattcagacttttcctccaatgcctttcaaaggctactcgcacattcctagggtcaaaccttgccctccagaatgcagtgttttataggctgttgttgctgttaaacttttttcccccataaagtgcaaatgtgaggaagaagaaacaaaagtactagatagcaaaacaagcaaatggacttggaattttatttgtacagatctgattaactaagagtttcccttttgatgatggacaatggcactagaggaaaagaacaggagtggggttctctgtgcccacttcttttcaaaagggtgattttataaaagtgctttccacataaggaaataaaatacactttaatgagtaagtacatatagagagggtgaccatgaggcatgttgtcatgttagtgcaggggcctttatttattttatgaacaatatcctaaagttaataaagaactatgctttattatttttttttaatctaggaagccaaggaaaaccagctgaacatattccattggctgcagccttcaatttaaacatcagaaagaaaggtaagctgggcacacccagattgtgtccagcttgtcagcacacttatttctgattatctgaaaataaacaacatgcttattctagagacagaggacctgctgaaagcttatagcacacaagtctattcaaaatgattccatatgttacactgtaggattgttgtgtagttatacaagggaaagaaatcaaaaccctgtacagacacctgatatcagacttgaaatgccaagtggaaacagaactattcagcatcttcatttatacacaatttacaatatttgattcaaaataaaaatcacaagaaaaatacatctgtttctgctacaattccttcccctccccatcctccccccacccccgccccagtgaaaagtcttctaataaaaggtatcatattaccaccgtcttgttttggtctaattctgagatcccacttggaacagttaacatgaaaaggaatggcaatacttgggatttatataacgtacacattgtatccaaggatctcaaatacttgcagtcacgtctccagatctgagaaatcacggttcaatggaagccagaaagctggacgaatgctgggcaggttgcatggggtgtaaaatcccttggctaagtctatgatcaaacaaggtcaaagttggttggctagagctgggctcaatttctcttctcaaatatatactaccagtcagtaagttttaccctttcttaaaccacacacccatctccaggctactgcctagagttaagaccaactgaagtagccatgtcctcatgataatgcatcaggataaaaagcaaaaacagggaaatacattcatcagcatctggccaaaggagacgggggttgggagaattgatctgggaggccattcctagcaagaacgagacaaaagtgtcaattcactagtttcagttacagttaagcttttggtggagttgattccagcagaggtgaagctcatggcatctagtgcttgatttaagataatgctattgaagaagggtaatgagaaaacacagcaaactaacaaggaggaactggccaaggaatatctggagggccaaagtgattttctttccttatcatttctacaggagaaggcaaggggtaggagaaaagggctggagggccccttatttgcagatttttttaaaaaaatcatttttttcataactccgtaatgaaaatgtattttacggtatgaaggttacagaactgcatctgctactgggtcacggctacaggtctatgagctgatccaccagcagtaaagacctggctaggttgggaagactggactcagagctcccactgctgtttctagagtgcccaccttgtgggtttttggttatcaatacaggaatagggtcaaactcatcttcagccaccttgtccgagccctcagggacatcaaaacctgagatgagattactatcttctgtgcgattcgaggtcacagattccgtctgagatgggaggcgctggggaactgggggctccagtcctggtatgagactctcaacagcaacatcagctttttcaattacagcatcagaagtgctaccaaaaggatctgtcataggcaagaggtcagggagcagaagagaagtgtcaggagatttgagtccctcaattagtttttctggtgcatcaggtacttgaagaggaatgaaaggatcagacacgcttagaagcgggaggccagagtccacagtctgcccacccttccttttttcagcagttccagcagaaaatgaggtcgtagcaaaagcatcaccttgggttgattgaaagcctgggatcaaactctcagctgagcctccaagcttctcgggatgtttgccttccccaagcttggcaaagtccttgtttagcagttcttcagctgtgagtttggagaaattatcgtcatcaaagggattccacgtagacccttctgaaggattataaacgttttgttgagaggtccgaggagagcctgatggagtggtggttgcagacttggacttattgagactggcctcagctgcagctgcctggagcagctgggttgatttgctggcagggaccccaaagactgcactgtgggttacgtcactgagaatacgcctgtgcccagcacgttgggttttgggggatgagggtggagtgagagatccaactttctgcccctggacggcaggaggtggggttgtctgaacctttggctgttgtcttactggggcttgaatcgctggctcctgggcaggggctggctgtggggctgcagctggctgtggctggggctgctgtcctgctgccatagtgggcttttgctgcaaggcagcctgctgagtcatcagctgttgttgatgcagggctgtggccagctgttgctgttgctgttgttgttgctgctgctgctgctgctggtagaaattctgcattagctgctgttgagagcctccttgggacaccacagggaactgagcaattgctggtttctgggttgctggatgtactgcctgaaactgctgagtctgggcctgctgctgctggtaaaacgtgcctgccggctgctgctgtgctggcggtggctgttgctgctgctgttgctgcttgaggaagagttgctgctggtgctggggtgtggcctgggcctgagcgggcagaccctgggcctgagtagaaggcgtctgctgtggagtgggaggagcctgtggctgcttggcctgagtttgcggcagaggctggctgggtggggcttggggttttggttggggaacactggctaaaaggccaggctgattgctggatcctgcagcctgaggtgggggctgaacagtggccctcttccggggtgtcagcgctggctggatgggaaggattcctgggttcggctgagtctgcccagctttaggcctctggcggggtgcaattgaagtctctgtggtgggaatgggatctgtcagtctggcctttggctgggtcttttttgcagctgcctcactggctttcactggttcaggaagctttgcaggaatgggagagttctgtacatttggaattgggcactctttcttgagtagcttaaatgagaagtaggacacctggtaaatatccggccttttgtcagggtctggttccaacatatacctaattaggcagtgcatgtcttgagaatatcgagaattatcaggaattgtgaagtttccatcacaaattgccacctgactttccccaaatggcaaagtgaagtagcataatttatacaacaaacatccaagagcccaaatgtctgccttcgtagtgatgattttgccactgtacaggttgaccatttctggtgctcgataggacagcgttgtgtatttcttaatctcatcttctactgcattgactccctcagtttgtggattctggaatttgttggtggcgcttccaaagtcacacaggacatagtggcctcggtcatgcaagaggatgttttcaaccttcaggtcccggtggataataggagttttgcactgatgcaggcgggcaacagcttcacaggtatcacaaaatatctggagcacttcattctctgtaaagcctgtttgcaggcgctggttcatcaggtttaccacctggccacctctacaaaagtccatcagaatgagcacttcccatacatcaccgctactcacgttgttgatactagaatcaatgtaacccacaatattcttgtgccctgaaagatccctcattatctggatttctctcttgcacacctggagatcatgctcattgttgacaaacatgcgtttcaaggcacatttcatcccattgcttgtcctcaccagaaatacaatagcaaatccaccttccgccaacacctcgtccactgtgacctgctgtcgcccgatgccgaagactcttccgatgtagccactgcccaggcccgaggtgctgccccctcctccgctggagccggagcccaggccagagccgccctgctctcgccgggagtcgaaaaacttcttcatcttgcgaatagggagcagcaaagcaaaataccgatggtttctagattttttttttttttttttttttttaagaaaagagatccaaggatttcttctcagatttcacctcggagaggagccacccgaatccggccgtgggggtgggggctgagggaggatgcctataggaatatgcgtgtcaatcgcgcagcgggtcccctcctcctccagaaagcgattcgtgtaagtttaaacttgagacggctcggcggccggcgccctgctaccagccccgcgacattgtcacggccgccgggccggcctgcgacgcagagaagaggcggcgctgcagcgagagccggggccgcgctcggctcccgcccgcccgccagctgatcccgggagcgccgggcggagac

SEQ ID NO: 11736 - RNA, 4704 nt, Homo sapiens
  source 1..4704: mol_type = other RNA
ctgaatagctgggactacaggtgtgcaccaccatgcctggctaatttttgtattttttgtagagacaaggttttgccatgttgcccaggttggtcttgaactcatgagctcaagcgatcggcccaacacagcctcccagagtgctgggattccaagtgtgagccaccacaccccgcccatttcattcttatttggtgagattgtcacagacttggctgaaacttaacaagaaactgtttacagcaacaaaggaagcaattaaagttaacatgatcattcaactgtgccattcatcatgcacttattgacatgctcaaaataggggaatgttaagtaaggaaatgaagtgggaacaggaacaagggagctaagccaagaggacttccagggacttgaacaaaaacaattcccaaccacatactacttttcaagcattttgaaactcttcttttcctttagtgatgttttcagtaacaaacttgcaagtgttcttggtggttaaaaaacaaaacaaaactacaagtatcagctgagaaagacaaagaaaaaactaagaatttaaattagataattccatttaaagtttccaattcctcgtttaggtggagttggaacattagaactcaggggtggtttggatattaacaaggtactcctgcctcctcagaagctacagtcttttctgcagctctcttatgtacctctcatcaaaataatttcagtcccacatttctcggataaaaccacatctgtggttttatccagcaaccatttcacagtcgactggcacgtgttctccaatttcagttccaaacacacaacacagaatcacacttttctttattaaagggacccaagtgatttttaagctgtattcttcctgctagagaatgaattgagtagcatccttctctaatttcctacaataaaatttcctatgtgatatactgcatatatattatatctgatatatgttttgattatttttctttatggaagcaaatacagaatttccttgtcagatcactctgatgattataatctgctactttgattatgcatcagtgaaatgtccaccaagcagttgaaaacactgatgtacatgtattctaaaacttactaaataatgggccagtaagataccagtatctttctagaacgtttagaaagagatcttagttgccagagaaaactcagatacaacatgagcctctaaacacatacactctagtctacaaatatgagacttttcaactcaacaataagtgggccgaaaacaatatagggcgtatgacctagactccctgggtgctgctcagcagctgcttcagcatcaaattgtgttcatcccattttctaatctaaccaagcacttggaactaaagggctgtatgtgagcccaagaaactgatatattaaatatttttcaccacatatgacatctttcattcagtactgcctgttagtcaattactgtggattctttcagggttcatcaatgcatgtgtggctcgatggtttaggaataaatatattctggctcaatgctttccactgaaatgaaaggtcacaacttctatgttccctatcaaatgtgtaaagcaaaaacacaacaaacgaaaacaagaaagtagagttgtttgttgattatatacagtcatgtgctgcataaaaacgattccatcaatgatggaccacatataccatgatggtcccataagattataccatatttttactgtaccttttctatgtctaaaatgtttggatacagaaatacttaccattgtgttacaactgcctacagtattcagtacagtaacatgctgtacaggtttgtagcccaggagcaacaggctggaccatatagcctaggtaggtagtaggccgtgccatctaggtttgtgttaagtacactctgtgatgttcacacaatgacaaaatcacctaaggatgcatttctctgaatgtctccctcatcattaagtggggcatgactgtatttttttttctctttaaggaaataagaccctactgtaatacaagtcggcagaatctaactgttactaataattaatgtaatccacaagtcaaagttttttcatgcatcaccaaaaaaaaaaaaaaaagtaatttgcatgtgtttgcatccgtttctgtattcaaagaaggtatgtagagtctccacccatcatgtctccagtgacaattttttttttttttttgaggcggagttttgctcttctcgcccaggctggagtgcaatgacacaatcttggctcactgcaaagtctgcctccctgggtcaagcaattctgcctcagctgcagctgcctggagcagctgggttgatttgctggcagggaccccaaagactgcactgtgggttacgtcactgagaatacgcctgtgcccagcacgttgggttttgggggatgagggtggagtgagagatccaactttctgcccctggacggcaggaggtggggttgtctgaacctttggctgttgtcttactggggcttgaatcgctggctcctgggcaggggctggctgtggggctgcagctggctgtggctggggctgctgtcctgctgccatagtgggcttttgctgcaaggcagcctgctgagtcatcagctgttgttgatgcagggctgtggccagctgttgctgttgctgttgttgttgctgctgctgctgctgctggtagaaattctgcattagctgctgttgagagcctccttgggacaccacagggaactgagcaattgctggtttctgggttgctggatgtactgcctgaaactgctgagtctgggcctgctgctgctggtaaaacgtgcctgccggctgctgctgtgctggcggtggctgttgctgctgctgttgctgcttgaggaagagttgctgctggtgctggggtgtggcctgggcctgagcgggcagaccctgggcctgagtagaaggcgtctgctgtggagtgggaggagcctgtggctgcttggcctgagtttgcggcagaggctggctgggtggggcttggggttttggttggggaacactggctaaaaggccaggctgattgctggatcctgcagcctgaggtgggggctgaacagtggccctcttccggggtgtcagcgctggctggatgggaaggattcctgggttcggctgagtctgcccagctttaggcctctggcggggtgcaattgaagtctctgtggtgggaatgggatctgtcagtctggcctttggctgggtcttttttgcagctgcctcactggctttcactggttcaggaagctttgcaggaatgggagagttctgtacatttggaattgggcactctttcttgagtagcttaaatgagaagtaggacacctggtaaatatccggccttttgtcagggtctggttccaacatatacctaattaggcagtgcatgtcttgagaatatcgagaattatcaggaattgtgaagtttccatcacaaattgccacctgactttccccaaatggcaaagtgaagtagcataatttatacaacaaacatccaagagcccaaatgtctgccttcgtagtgatgattttgccactgtacaggttgaccatttctggtgctcgataggacagcgttgtgtatttcttaatctcatcttctactgcattgactccctcagtttgtggattctggaatttgttggtggcgcttccaaagtcacacaggacatagtggcctcggtcatgcaagaggatgttttcaaccttcaggtcccggtggataataggagttttgcactgatgcaggcgggcaacagcttcacaggtatcacaaaatatctggagcacttcattctctgtaaagcctgtttgcaggcgctggttcatcaggtttaccacctggccacctctacaaaagtccatcagaatgagcacttcccatacatcaccgctactcacgttgttgatactagaatcaatgtaacccacaatattcttgtgccctgaaagatccctcattatctggatttctctcttgcacacctggagatcatgctcattgttgacaaacatgcgtttcaaggcacatttcatcccattgcttgtcctcaccagaaatacaatagcaaatccaccttccgccaacacctcgtccactgtgacctgctgtcgcccgatgccgaagactcttccgatgtagccactgcccaggcccgaggtgctgccccctcctccgctggagccggagcccaggccagagccgccctgctctcgccgggagtcgaaaaacttcttcatcttgcgaatagggagcagcaaagcaaaataccgatggtttctagattttttttttttttttttttttttaagaaaagagatccaaggatttcttctcagatttcacctcggagaggagccacccgaatccggccgtgggggtgggggctgagggaggatgcctataggaatatgcgtgtcaatcgcgcagcgggtcccctcctcctccagaaagcgattcgtgtaagtttaaacttgagacggctcggcggccggcgccctgctaccagccccgcgacattgtcacggccgccgggccggcctgcgacgcagagaagaggcggcgctgcagcgagagccggggccgcgctcggctcccgcccgcccgccagctgatcccgggagcgccgggcggagact

SEQ ID NO: 11737 - RNA, 2204 nt, Homo sapiens
  source 1..2204: mol_type = other RNA
ctgaatagctgggactacaggtgtgcaccaccatggccagctaattttttttgttgtttttttgtttgtttttaagatggagtcttgctcttgttgtccaggctggagtgcaatggcatgatttcggctcactgcaatctctgcctcctgggttcaagcgatcctcctgcctcagcctcccaagtagctgaggttataggtgcccaccaccacgcccagctaattttttttttttttttttttgagacggagcctcgctctttcgcccaagctagagtgcagtggcgtgatcttggctcactgcaagctttgcctcccaggttcacgccattctcctgcctcagcctcccgagtagctggtactacaggtgcccgccaccaagcccagctaatttctgtattttttagtagagacggggtttcaccgtgttagccaggatgatctggatctcctgagctggtgatccgccctcctcggcttcccaaagtgctgggattacaggcgtgagccaccgtgcctggcctggatatgttaacataataatttaagataaaatgaatgagttaatcagcagattagacggaagggagtaatttgatgagggggtaaaagaaaatggtgaggatatggagaaggaattcgtggtgaaactggacacaattgttgagggatttccagagctgatgaacgttgtggacctgtggcttacaccaaacagggtgggtgtgagctcggcacagctaggacgcgctggtgagaccaaggaacaccaaagtcagtgaggagatcttagtgtctcccggagagagccgaccgaggctggcgcatgtctgaatgcgagcctggccataggctgagcccggctgccgccacccctgggcttctggaaccctgggcttggccgagcgtgggtgtctcccctgggagccccagagccctggacgatggaggccgggacctgggcaggcgcgggaggccttgggctggggcctgcgcccctcctctgagggctgcctgccgggctctgccctgccctgcccttccctcccctctcttcccctcccctctcctctctttccctcacctcccctctctttgcctcccctcccctcccctcccctcttcccctcccctcccctctcttcccctcccctcccctctcttcccctcccctcccctctcttcccctcccctcccctcttcccctcccctcccctcccctctctccccctcccctcccctctcttcccctcccctcccctctcttcccctcccctgccctccgtggcgggggcggggctgcgggcgggggaggccggggtcgtaagccgggagcgctgcgcgcccagccaggaaggggcagcgggggcgaccctcagttttccgggccgggccacgcgatggggtcgcgcgcgagctcggaggcctcccggggtttcgcagcggccgccgggtcacacccaggcgcagagttgctcgtcctcgtcggggcgccccggggggcggcggggtccgggggtcccagcgggcggaggcagcagcgggcggaggcgccgggctaggcgggcgcggacggccgaggcgagcaccagcagcggcggcagcgagagaagcccgaacacgatgagcgccgcggagccgcggtctgagaacagcgcgcggcaccggggacccggagcggggtggaccctcgagtggcacaggaatcccaggtagacgacggcggccgcgggcaggagcaccagcaggaaggctgcggcgggcagcaggaggtgcagcaggagcccggccagcagccggccgggcagcagcgggggccccgaccaccctgggcacgtcagggctgaggcctggtggtcgggaggtccccggggcagcatgggcgctgtgtcggaagcaccacctcccccctcctcctcctccgtctccctcccctgctcactcatgctcctgccactgcaggcctgtggcccgggcggtgctcaatgcagagtggtgctctccagggctgccctggaagacctttaaccccgccccacgttgcagccagtccacatcccccagccagaccgtggaccctggctagggaggtcctgccctgatgtctgtcccagagccacacccccacctcagtttcccctctgccaggcagctgcagctccagcagcgccagtctccagccccagccagctcctggtgctct

SEQ ID NO: 11738 - RNA, 3136 nt, Homo sapiens
  source 1..3136: mol_type = other RNA
ctgaatagctgggactacaggtgtgcaccaccatgtctggctacttacaaacaaatttttttagagacagggtctccctgtgttgcccagtctggtcttgaactcctgggctcaagtgatccttctgcttcagtctccagagtcactgggattacaggtatgagtcactgaacctggctacgtttttaaaaagtttctttgctttattaaattcctcttcaagacttaacagaacaatggaagctcatcataatcagggaaacaagaagaaaagagaatcactcaggctcctttctggcgggggagtggagaggctgggaaacacaatgacagtgaaccatgggaagcagggggcatggccactggatctgaaagggaccggctaacagtcactaaatgtccaaggcctgggcttgagcaatagcctcaggtatctccatcacttacacagcactcattcgttcagtgagatgtcatttattaagcagttacaatgctgcaggtgctgtgcaggagactggacatacaaaagaagaatttgacccagaccttccccctctggggtctcataatcttgtagggggaagggaatacaaatacaaattagcgaagaatgatagcagtatcttaggacactgtaactgtgtgctacgggacccaaggactggagagccatcccttcgtgaaggtcagggaagagctgggtggtggagagagctgagcctgtgtggacccctgatgcatgctctgatgctgagggagtacagtagagatggacactgatagtgacagaagagtttggccccaaagcagaagcggcatcctgcaccgactccccttagaatgaatgagtacgcacaagaaaacaaccacaggcatcgccgcccttcagtggatctctttgctggagaattgacagagtgcgtgtcgcgcctgagtgagccggtaaattctctccttaaggattcttctcttggtagcggtctcactctgctcttgaagcagccaggaatagcgatttttttcctgtagtatctgcatcatggctttctgcaaggagtcaccattctctcggagcataaaatactgaattataaatgggatctggttggcgagacgtttgctggtttccaagaagtaggcattcaggtggatgcctatttcagtaaaggaggaaaccgaagactcattactgggaaaatgagagttcaacttcatattctgtgaaggcgtccccagagggttaaaaatctcttctcggactttcttcagaacaacactgtaaatctgatcttgacaaaaaaccatctgctccattctgaactgaagttggatcatgttttctgcctttgctgtgtgtttcacttttatgtcttcaatcgtgctctgaacagtttggttaaggttgaaaaattcgccaaaatgttttttggccacgttaatgaaagcttgctggataatttccatggctttctggagcatgctaagggcgggctccaccagctgctggatgtactgatgcacgatgatctcaaatgtcttgtagttgacaaatcccagaagctccttgcctcgatactgcttttcatatttttcaacttcttcgtggataatatttttaactttttgggtattagttgcaagtatgcctacccagtttttaaaatcctctctgattttgttgtataaacgggtctcattctcccttacaacttcttctccttctactaacttttcgatgtcctgattaaacatcttgattttctcaattagaaagaacatcttgtcggcctcctggctggggatgtcagccccgcaacgccgcagctcctcggtcgccttctggtggctctcccttatttgtccttctaacaacgggagcgatttttggatatgcatgatgagttcagtggtaagtctttctgccagtcggggaaccgtggctgacccctcctccaggagaactctgaaatatggatgtgtttgaaagaatgtaatttctttcttggttgcctctgccaagctcagcctgtttgtgatctcctgctggccccggcacttcacaatcatgtagcccttcttgagggggtacgtgaggttccgcaccacattcatgacgcttttctcagtgcccctgtccattagatctggtttggtcaggataccgatggtcctgtccccttccgggtccacctcatgggccatgctcagcgcctccgtggtggcaatgtccacgttacagggaaccaccaccaagttgatcgtctgctgcctctggatgtacttcttgatgagagccttgatctgcagtccgatgtctcggggctggttgtccacagccaccctggtgatgccgggaaggtcaatgatggtcaggtctggaacctcaggggaggtgatctccaggctgatgagctcatggctgatgccccggccattcccggccatgacgttctgggctttgtgtatctctttctccacctggccagggtcctgaagctctagctcggtgttccggtagctgatccttccggcccatgcctcacagggctgctttttcagtttcagcaccagcggacacctggttacgattccgctgcctctgggaagcgcgactcctgacagtgcctccagcacagagctcttgcccgagctctggtccccgatgacggcgatggctggcagggccaggtcctgctccacacccagagcccgcagggagtcgatgaggtcaatgcaggggcgcaccttctgctcgtactggctgtacaggttgttctcgggccccattgcccttggttggctcctgtttcctggtggtggctgattgttcaaagtgagaaagttgaagtccttggcgaggaaagcagcgtccttctctgccccctgccagtttggaggaaacatcatttgtggtggcactgtgccgaatggcggtggctgttgctggaaggaattcatttcttttttcaggtattttcgagaagaaaattgacttctcctccggtagggccaaggcttgtgggccttagacatgtgctgtctccctgtcagagctgggggatgctttctctgctacttggcacctccgatcttcctgacaagctcgctgcacgttcaggatggagaaatcatc

SEQ ID NO: 11739 - RNA, 2547 nt, Homo sapiens
  source 1..2547: mol_type = other RNA
ctgaatagctgggactacaggtgtgcaccacctacgcccagctaatatttttttgtatttttagtagagacagggtttcaccgtgttagccaggatggccttgatctcctgacctcgtgatcggcccgcctcggcctcccaaagtgttgggattacaggcgtgagccactgtgcccggccaaattttactatttttatttgctttttcccctagatttgactacatggatagttttagaagcttgagttcctaagataattccatagctacactggctcctacaatgtgactgagtgaggttagggaaatatccttggggattctgaacaactagacccttagaaacttaaaaataacaggtgctttcattaggatccttctaacatggaaaaaatacagccattgtccattaaaatacaatccaatttgggtactcttcaggttttctaagttctccatctgaataataagactaggccaccatcttttctggcaacccagcctacagccactgccatcttcctaactagcagcctcctaagctgcactaaaactgggattaacacaactgaagataacatttttgacctttcttcctagaagtcaaagggctcttcaggtaggaaaggtcaggaggttttgcatcaagcttgccttcacactcactattagtagaagggctgtgaaatctacccatcacacacctgtattcagtgtttgagtgtacttacccatcaacacacaaggaagttagagtaaattaacaagtcactctggaccaagcccctcaaaacagaggcaaatttggtgaaccaaggtcattcactgcctgtggtaaaaacctcagttcacctaagtcctttcctgaaaaaccacattaatctgattcaagaggcacctctggccagcacagagcacagaaggaaagcataacttcagggtaggggaatgccacatggaatttagaagttgcagtttagtctacagcaaaagatggcaccatcgctaatatttacagctggaaagagcgctggctggaccacactcctggagcatctttactaatgcagcttaacagcagttgcccagatgtcgttgctggggagcgggggaaggacccatccttggggaacgaagttgcctttgggatgatcggatggcaccaggtactgatcccaatcatgcctgatctggatgagcgctggcagggagtgctcggcttggagataatactgtcggaaaggctccaagaggtgagcaagtgggaactcatctggatccccaaacaacttggactcaatttcacgtttctgaagtaaaattttctctttttcttttctttgtttcttttctaattctcttttcctctcttcctcttgttctccttctagcataactctgagggctctctcttcagcttcatacagttcagagcgctttttaatgagttttctcagtcgctgaagatgatgcgtaaaagtctcatctgctgaggctggaggacagacccctttcctcgctgcagcctctttcctcagtttcctcaatttctccaaagcccgtagaatgtccaccattcttttggtatctgcttgttttttcctcacttcagatagtacgccatcagcggctgctttgagttcctgctcccgcttcttctcctccacctcctgcacacacttcaccctccagcggtcaatctcctgctcgcgttccactgcccgcgcggcctctgcctcccgctcggcctcgcgttcccgggccctctcgcgaagccgcagccggcggcgccggaccctctccagcctcctccgcgcctcgcccacataggcagcctgggtcaacggctgtagccgctcggccagttccgcgcgcagcggcgcggtctgggagtacagcaggacccaggccgcgccgtcggcttcggcctcgcgcagggcctggctcaggccgcgcagccgccgcaccaggcgcagagcccggagcaatcgcgcgcgcacttcgccaaggctgggcccggcatgcgtgcgctggggcaccggacagcctgcccgccgcggggtcccgaacaccgcctccagccactgccggtcgcgcaggcgttggagggccgcatccccgagcacgtcggccggcggcggcggcgcctcaggccaccgcgggctccagggcggccccgggccgggaggcggtggccgcggccgctcgccggcgtcggtccccgggaagggccgacactggggcggcggaggaggcagcggcggtggtggcaccgggtagaaggcgccagcgccgcctccgccgcgggaggcctccgcggaggctcggggctgcagagccagcggaggctgaaggaagggggcggaggcccccggaaaagggccgggccgctgggggagaggcggcgggaaagccggggagggcagcggcggtggcggacagccgaaaggagcaggaggcggcggctgcgggggcggtgggcctgggcgaccctggccgaagaatggtggcagggccatgttcacgacggagatgctttgagaagt

SEQ ID NO: 11740 - RNA, 4390 nt, Homo sapiens
  source 1..4390: mol_type = other RNA
ctgaatagctgggactacaggtgtgcaccacgacgcccagttatctagtttactcttacccaagtataaatgatatgaaacaatctgagactagtcagtcaactgtccttggtaagatctccttcttgacagccatgtggattctatcacaccctttataatttacagcaatcttcagtggttaaagcaaaactgtacatctataaaggaattcaagagaagtgcaggaaaaggatgacaaaaggtaaatccctagctaccaccagaatgttatctatctaaaactgccaacttacgaataggtaaaacttatggtaaaattataaaggtgagcacaacaggaactggaatctattctgaagggcaatataatgtacttccaagaattctagatttttttttttttttggagacagtttcactcgtcacccaggcttgagtgcagtggcacaatcttggctcactgcaacctccacctcccaagttcaagtgattcttgtgcctcagcctcccaagtagctgagattacaggtgcccaccaccacacctggctaatttttatgttttttgtagagacagggtttcgccatgttgaccaggctggtctcaaacgcctgacctcaagtgatctgcctgccttggcctcccaaagtgctgggattacaggcatgagcgaccatgcccggctaattctagatttaatagagtaaagagaaagtacttttgttacagaccactggttctagtcctagacccagaatgtcaatacagtagccactagccacttgtgcctatgtaaatttaaaataaaatactttctagtcacactagctatatttcaagggcttaacagccacatgtggttagtggctaccacactggacagcaaaagtctacaaaatatccatcgtcacagaaagttctattagacagcactgttctagacaaaataagcatgtaggtggcatctgaataccccttaaatacatctggcccttgtttttgattctaccaacctagccacttacagcgaagcactagaaatgaaaacatgtggtttatagtgctctttttttcccctatttccttatttctgaaggtatatatccctgatagaaatgtcctttttaaaaaattacataattggccaggcgtggtggctcacgcctgtaatcccagcactttgggaggccgaggcaggtagatcacctgacgtcgggagttcaagaccagcctgtccagcatggagaaaccctgtctctactaaaaacacaaaataagctgggcatggtggcgcatgcttgtaatcccagctacttgagaggctgagtcaggagaatcgcttgaacctggaaggcggaggttgcggtgagcagcgatcacgccattgcactccagcctgggcaacaagagtgaaattatctcaaaaaaataaaaataaaaaagttacagaatcacattttaaaccaccagaagtgcttgggtataactgacctagaacatggcagttactcatctgtgccaacacagaccttaatataggaggcatagaaatgagaaaaattggccggacgtggtggctcacacctgtaatcctagaactttgggaggccaaggtgggtggatcacgaggtcaggagtccaagaccagtctggccaacatggtgaaacaccatctccactaaaaatacaaaaattagccaggcgtggtggcgggtgcctgtaatcccagctactcaggaggctgaggcaggagaatcacttgcaactggaaggcggaggttgcagtgagattgcaccactgtactcagcctgggcgaaaagggcgaaactccgtctcagaaaaaataaatgagaaaaattttaaacctgaaaaaaaattaaacctaagttactactgggctgattacttctgggttaaataataagatttctgaatttgaaaaccaggcagggcctggtggctcacgcctgtaatcccagcactttggggagccaaggcaagtggacggattgcttgagctcaggagtttgagaccagcctgggaccacatggcaaaactccatctctacaaaaaaattagctgggcatggtggcgaacacctgtagtcccagctacttgggaagctgaagtgagagaatcgcttgagcctgggaaatagaggttgcagccagccgagatcgcaccactgcactccagccttggcgacacagcgtgaccatgtctcaaaaaacaaactaaacgccacaactagccaagatggaaggttgaacacatttctgtatctatcttaatatgtttcctgtatcatttccaggatgccaaaaaaaaaaaaaatcaactctctagccttcacttcaggtctttctcattagtccagaattgtccccttgtaagctacttgctacactgtccctgaataccactaactttatacagtcaccaagtcctctgctacaaggcctttcaaagtctgaaatctttaaaggatttccaggatgcatttttaaattccccaccagaactcagactaggacttcaaatatgaattacagcaagctttccacatttctataaataaaaataagactcatatgttataaattgctttcaggccttaaaacacctatctaatcgtccctatcacctttgagaccatggattcacatcttctcagtcttctcactgtcccacaaagatacagttctcagctgcaccagcatagatttattttctcattattctttatgacttaccttgtgctcaccatctccataaaatctccaaggactactctaaatgtgtatggcacagactatgcatgaaataattcagtatgtaattatacactgttacacatcacaaaactatgaccacaggcattcctctgtccatgtctggcataaatgctgcagttctcaatctgagcaaagaaactaagagtcaattagtgaagtgttattctagttgaggcagtcctagaaaaccaagtaaacaatctagcaccatgactggttaacactgctgcactgacatttagggctgctgcactgacatttagggctcctgcactttttaatcattaaaatttgtgcatcagtcatgaaatcaagcacagtcaaaaagtcatgatctgtggttttctttttaattatctttagtcttgtgatcacacataattttaaaatttgtgtatatctccgttactttaatccttttaagttggcaaaagcaccattcccaatcaaatacacagttctacagttttgtttctgaatggctgtttaaagacaatcctaaattataacttagtttgacttagattgtaaagaattcaagagtgaagtttaacttgctactattttaaaagcatgtgaccttatagatctgtaagatgtgagaggtgttgaataatctttaatattacacataaaccacactaaaatgcctttcaataagtaaaagaaaccattttaaatacagggaattataattagattggcatagttaaggccaaaactatagacattgctaccttatttatcttcaacccttgcctttaagaggcaaatgaacatgaacacaaaacacaggtgaatcttgcttggttctaagacagtgaagcaatttccccagtatttaaatatattcacataaccagttatataaatctaaatataaaaccaatctccagtaagttttaagatggcactcaccatctttgtgaaaagttgaacattactaacgaagtctaatcatatctttaaaaggggtaaacagtgataccatttactgaattggagttactattaaaattcaaaaactgaacatattcatttaaccacaagccagtcttagttttaaatcaggactgcccaacaaaatattctgtcagtcattcatgatctgaattctggtgtatgagatctattaaaggatggtacacataaaaaagtcatgagacatttctgttttgtaataaataaggcagtggccaattattactcattagtagcttttttgagataagctattaagtctgccctttcttccttcttcttaatgccgacaaagatcatttttgttccagggatgtacttcttgggattctccaaatactccatcagtgtatcctctccccagatgatgcctttgttcttattggcggctgtgtaagagtatccaggggcctgacctgtcttccgcccaaagagaccatggagatttggcccagtcttgtgcttgcctcccttttcaacggtgtggcactgggaacacttcataataaaaatcttcttgcctttctcaacatcacccatatttaattctctttttagtcgctggcacaacgaacactcccgctccgaagccggacgtccccactctct

SEQ ID NO: 11741 - RNA, 2945 nt, Homo sapiens
  source 1..2945: mol_type = other RNA
ctgaatagctgggactacaggtgtgcaccactacacctggctaattttttatatttttagtagagatggggtttcaccatatgggccaggctggtcttgaactcttgaccaggtgatctgcctgcctcagcctcccaaagtgctgggattacaggcatgagccaccgcacccagtcaaactcttttatctttagtaagggtagaggaccattgaccaggtgatctgcctgcctcagcctcccaaagtgctgggattacaggcatgagccaccgcacccagtcaaactcttttatctttagtaagggtagaggaccagtcaaagcctttgccacattcttcacatttgtagaaattctcttccgcatgaattctcctatgtgtagtaaagtatgagtactggttataaggtttgccacattttttacatttgtagtgttattctccaatatgaattatcttatgtatagtaagggttgaagattggttaaaagctttgccacattcttcacatttgtagggtgtctctccagtatgaattttcttatgtttagtaaggtttgaggaccagttataagctttgccacattcttcacatttgtagggtttctctccagtatgaactctcttatgtctagtaagagttgaggactggttaaaagcttttccacattcttcacatttgtagggtttctctccagtatgagttatcttatgattagtaaggtttgaggatttttaaaaagctttgccacattcttcacatttgtagggtttctctccagtatgaattatcttatgtctagtaatttgtgaggaacagttaaaagctttgccactttcttcatgtttgtagggtctctctccagtatgaatcatcttatgtgtagtaaggtatgagaattggtagaaatctttgccacattctaaacatttgtagggtttctctccattatgaattctcttatgtttagtaagggttgagaatacattaaaggctttgccacattcttcacacttgtagggtctctctccagtatgaattatcttatgtttagtaagggttgagaatacactaaaggctttgccacattcttcacatttgtagggtttctcaccagtatgaattctcttatgtgtagtaaggcgtgagtaccagttaaaagctttgccacattcctcacatttgtagcgtttctctacagtatgaatcatcttatgtgtagtaagataagataatcggtagaaagctttgccacattcttcacatttgtagggtttctctccagtgtgaattctcttatgtgtagtaaggtaaatgaatcggtagaaagctttgccacattcttcacatttgtagggtttctctccagtatgaatcaacttatgtgcagtaaggtaggagtaacagttaaaagctttgccacattcttcacatttgtagggtttctctccagtatgaattatcttatgtgtagtaaggtatgagaatctgaagaaagctttgccacattctccacatttgtagggtttctctccagaatgaattttcatgagtagtaaggtttgaggactgtttaaaagctttgccacattcctcacatttgtagggtttctcttcagtatgaattatcttatgtctagtaagggttgcgaatacattaaaggctttgccacattattcacatttgtagggtttctctccagtatgaattatcttatgtctggtaaggtgtgagtaccaattaaaagctttgccacattcctcacatttgtagggtttctctccagtatgaattatcttatgtttagtaaggtatgagaattggcagaaagctttgccacatccttcacatttgtagggtttctctccagcatgaattgtcttatgtttagtaaggtgtgaggactgtttaaaatctttgccacatttttcacatttgtagtgtttctctccagcatgaattaccttatgtctagtaagagttgtggagtggttaaaaccttttccacattcttcatgtttgtaggatttgtctccagtatgaattctcttgtgtctagtaagggttgagaaccatttaaaggctttgccacattcttcacattggtaagaattctctctaatatgaattattttatgttgacctaggtgtaaaagcatgcaaaatgatttgccacattttttacatttgaaaggtttctttccagtatgtcttgtcttatgtgtatttgaatttaaaaatttatgaaagactttcacatatttatcacattgaaatattttgctctgggtagttgtcaaatactcttttagttcattataaccttctttttgcacattacactcattcacacttttacagccttttcttaactgtaaatctttatgtccataatttccatattctctcagtatcactttttggaaagaatcttttatgcccggctgtggccaaaggtcctgggcaaaatgagaatatgtaactgggggtgtggctaccatactgtgtctcttcatattccagggatcttttccttgctccagacaggtgatcagatctggcttagagacatcaatacccaagaacaccaggtttctgaagttctctaacatcactttcctatacaaatcttgctgagcagtgtccaggcattgccactcctcctgagagaattctatgaccacatccctaaatgtcaacggccccttttcaaaataagagtactccagaagattcctctcagccccagggtatccacttgcccccttgacaggatacactccatacctcaggtcgtccatttctaggcttccagggtgtcccggcgtcttagctgtggattcccaatacctgcaggtcacaggaccagaggctgggcctctaggagcagaggacacagagcagtgaagacgagacccggagttccagcggcagccaaagac

SEQ ID NO: 11742 - RNA, 5494 nt, Homo sapiens
  source 1..5494: mol_type = other RNA
ctgaatagctgggactacaggtgtgcaccactatgcctagctcatcttttttttttttttttttttcctttaaaagatatggagtctcgctattttgcccaggctggtcttgaactcctggactcaagcaatccacctgcctcagcctcccagagtgttgggattacaggtgtgagccactgtgcccggcctgaattatcttcttattgtaaaatttcctttaatgcttaatagttgatgtatattaagtgctaactaaatgttcactgataaacattaatcagatgctgctaaatattgtctttctttattcacagatgatagtcaatgggcacaacatataagtagttacaatgaaatgagaagcaatatagcagtcaggctatatgcatgatttaacaacaaaattatcacttccttttaatttagaataagggacaatttaaaaagcatctcttggccctatcatttctgttccagtagttagtgttcatatgtgaatactaagtttgacattcctttctcccatagaaccattttggtgatttggatggtggccactacactgctttctgcaagaattcagtcacccaggcctgatatagctttgataacacacgagtcagtgagattccagatacttctgttcaaaatgctatggatctcctgttctatagctgccagcccttttccataccaatacaaaagcgttaagagccaggaaaatggtgtttcctgaacactgcaaaacaagcagtcagcatctggtggtagagttttgcttggtcattaaactcttagaacttacttgcatcattaacatttttatgccttgtgggcatgttatacaacctttcatcttaagataaatctgtcgtccagaagatgggtcttggttcactaaaaaaggcagtgtgaatataatgcaatgctaatggatgcaggccttcaaaacactgcaattatatagtgagttcaggtttcaaaattcagtgtttatcagaaaatatctcataatcatatatattcaacaaattattttccaaagatactcatgaagctaaacaaaaataatttttgttcaaatggctcgatgagtttaagaatatgatttgaatatatttgatataataatttagccaagaagtggtctcttagactaattgtaaaacatgaaaagttgtcagcttcacaatttgaaccccatcctttcatcttctccctgagagcctgctaatggtggtctctttctgaagcacttttagaatcttatttttatatggagtgttttactgactatatatatagcaactgagtccctcggttaaataaattataagctcctttaaccctcttaatacatcactctgtaaagatgtagtttataatgcagttcactttgcaatcatgcctgactcccggcatttttactttaatatttagaatgaatattctcaatatgtgagaatactagtcttgaaagaatgactctgggtgttattatatagcacgtgtgtatataaaatctatggttttactgtcctatatttgataatacaatattaaagacagaacacccacagggttataaattatttttctcattaagattttaatgtagctgtaaatgaaattctcgttttaaaaaaattaaagtttccatttttttttttagaataaagatttagtgcacaaatacagcccaaagccaacagaaaaattgctttgccctgtcatttccctaagaaagcactgaagttaactcaaaataggctgaaagaaaaaaagcaatcctctgagttctaggtttcacaaaaggaccacgtgttaaactatgtacatcgatttgatgtgcaagtatgcaataaatatgtacacatacattcctatctgctttacatcattctagagtattcatagtatatcaagatgggatttagaaatgtgaaaaggccataacagtgaaaaggaaaaaaaaaagataacaatagtttttagaccagtcgaataataatgcttagctagttaattattttaactttggagcagactaaaaaagttgttttgaaataaatggtacctgtaagtgatgattactgcaatacttgttaaatgttatttgtcagcactgaccggaattatatagtgctagtaacacagctcccactgtcctagaattcctctaaatggccagctatagctaccattatcctgataagcatttcaagagttgtgttgctgagccttttaaaagataactagtttataacctatgtctccttatgtggctacatcagttactcgtggtcccaatgaagtataaaagaggatataagctgctgaagatttcacagaagaaacggagatatcagaaacttcatgatcatcaaacttaaaccaccgttgtcttgctgcatttttacaataggctgtgtagtggcctccatccagcccaccgtagtgatttgaaacagaaaacaaattatatttcttcaaattgttctttggaccaataacatactgtgacaagtcaagattttctaacgggaagtccacagatgtctgtaatttttgtttccacctgccatcgtaggaaaaacgtttcagatgcactaaaagcacaggtggtaacttccagatttctatcttttttagagaatcccgtcgagctctgcaatgactgcagtaaaatctgttgttatctgtgagtttttcttctttggaaaataatctaaggcaatcctgtaatgtacatttacttgtggatgctagtggtagagacaaatacatgaaggcctcaaatgtcctagactttttgtgacatgtgaggcactgtactgtagatttgaattgaccctgaaaaagtgcaacaataatagactcattgagctgcttgtgtttctgccaggcatgttctgcagctttaaagtcatcgagatgatcattattttcttctttatatctcttccgattatcagctttatttagatcttcatggagaccatccattaggaacagaagcaattcttgtgaatcttgctgactgtatcctgcaaactggtcattgatcttcccaatggtgattttaaagtcctttggactgatatatctatactgtcctgtccacagggctttcatgattataccaaattcttctgccacttcacctttatgccccaacaaatttgacctgttaatatcatcctgataacagtttcggttgaaataatcagccaaatgtggagcgttacataggcactgcaatattgagttcatataacaagtatttcctaagttacgaagtccagtaagagctggtccagaacctccaaaaacaggattgaggttccgaatctgagaagcagaaagccttgagatctcagctttaggataacatgttggcttgttttcccgattaactgttggagttactgttggcttcctcttctcttcctcttgaatagcctgggttatatctggggaggagtaggagcgcttcagtttggaaggttccctatcccgctcagcaggaatctgtggcttggctttatgagttggaggggtggaaggaggtgcagatgaaggagccatttccggtgggtacatatgaacagtgttggtgggtgaatgataataacgaaaggttccagtgattgggtcaagaaacttggcccagcctgaaggcagtcctggtacgatcctccccatttcttcacttcgtgctcttgtcaaaggttctcgttgagccttgcctgaacctgaatcccctgtcacagatgtatggggcacatctcctgttgactttttctgtatttctggggttggacaccttttccccctatcttctacagatttcttggcatcagaagtttcatgttcacttttactttgtctttttactcctgttatttctttgcccctctttgctgaggtttctttatcttctttcttggcctgttcactttctttcttctccatttcttcttttgctttttgttgcttctctgtaatttcattttcttcagcttcttgtttctttttggctttttgttcttgttcttccttcctcagtttctctttctgttcctcttgctgcctttcccgaagttctttttcttgtttgtttttttccattagaagagcagtttctgcatgaatacgagccttttcttcatctgttaacatgagagttggagaaaaaactactggcttggtggaacgatcaggaataacttttccactctgaggagattgttgctcatggtttgtactttcagattttattctatgctcttcaggcaatttgactgctggttttttagtacgatcaatctgtggaacattctttatactaggcactggctgaattatgggtgaaacatcagatttagaagcagcaactggttcaactggagttgatatattcagtggtcccattctctcattttgaccacttatcaattctatattttcatctacttctatagatgcaggtggcgtctgggcagcaggtttagaaggaattgattcttccaatgagggataagtaaaatccaatgagatagacacctcttcattctggcgtcgtgggggtggagtgaccttagcatttgttgtatactggggataacaaaggagccagttttcatagcctccctctaaaaccaaaggctcattgcgcaggacagttttactttcccacttgaaaagtgcatctttcagactccggagagttgttccaatctgtaaatctttggcagaactaaaccagtcaagaagtaccacatactccacattccccctcttcttccatgtgtctttagaatcatctggcaggtgtgcttcaatccaactagcagtgactcctggactgatggcttcttcaggaacactgagagaatgtaaaatacaggaatcctgataatcctgcattcttcgagcatccattataatcaagctgatgtttttatccgtcatcattgtgtatagttcctttgctgtgattgctcctttctctttggtctcacatttttcattcttttcaccattgctcttttgggttttgtctttggaatccaaaacattctccaaagagcctttagccaatgtgccaccatcctctcttcctgtttcctgccttttttgttgtagccgctgtgcttcctcctgcctgtctttttcctcaagttttttccggacttcagcttcttcatatctcttagtgcttattttctctggtttaacttctgtcttcttattaaggtcttttagtgaagaactgaggtagagttctttaggaactgaagccacagcaggcatgatgaattatctttacttttccactttcacaatggatgctatatttccttacaagtgcttctttccgtgacgccgggcgcgcttcactaacgccagccttctcgccaaatgcccatctcccaagaactcgagggagaattagccttggctaccaggacggaagccagcccagctc

SEQ ID NO: 11743 - RNA, 5812 nt, Homo sapiens
  source 1..5812: mol_type = other RNA
ctgaatagctgggactacaggtgtgcaccactatgcctagctcatcttttttttttttttttttttcctttaaaagatatggagtctcgctattttgcccaggctggtcttgaactcctggactcaagcaatccacctgcctcagcctcccagagtgttgggattacaggtgtgagccactgtgcccggcctgaattatcttcttattgtaaaatttcctttaatgcttaatagttgatgtatattaagtgctaactaaatgttcactgataaacattaatcagatgctgctaaatattgtctttctttattcacagatgatagtcaatgggcacaacatataagtagttacaatgaaatgagaagcaatatagcagtcaggctatatgcatgatttaacaacaaaattatcacttccttttaatttagaataagggacaatttaaaaagcatctcttggccctatcatttctgttccagtagttagtgttcatatgtgaatactaagtttgacattcctttctcccatagaaccattttggtgatttggatggtggccactacactgctttctgcaagaattcagtcacccaggcctgatatagctttgataacacacgagtcagtgagattccagatacttctgttcaaaatgctatggatctcctgttctatagctgccagcccttttccataccaatacaaaagcgttaagagccaggaaaatggtgtttcctgaacactgcaaaacaagcagtcagcatctggtggtagagttttgcttggtcattaaactcttagaacttacttgcatcattaacatttttatgccttgtgggcatgttatacaacctttcatcttaagataaatctgtcgtccagaagatgggtcttggttcactaaaaaaggcagtgtgaatataatgcaatgctaatggatgcaggccttcaaaacactgcaattatatagtgagttcaggtttcaaaattcagtgtttatcagaaaatatctcataatcatatatattcaacaaattattttccaaagatactcatgaagctaaacaaaaataatttttgttcaaatggctcgatgagtttaagaatatgatttgaatatatttgatataataatttagccaagaagtggtctcttagactaattgtaaaacatgaaaagttgtcagcttcacaatttgaaccccatcctttcatcttctccctgagagcctgctaatggtggtctctttctgaagcacttttagaatcttatttttatatggagtgttttactgactatatatatagcaactgagtccctcggttaaataaattataagctcctttaaccctcttaatacatcactctgtaaagatgtagtttataatgcagttcactttgcaatcatgcctgactcccggcatttttactttaatatttagaatgaatattctcaatatgtgagaatactagtcttgaaagaatgactctgggtgttattatatagcacgtgtgtatataaaatctatggttttactgtcctatatttgataatacaatattaaagacagaacacccacagggttataaattatttttctcattaagattttaatgtagctgtaaatgaaattctcgttttaaaaaaattaaagtttccatttttttttttagaataaagatttagtgcacaaatacagcccaaagccaacagaaaaattgctttgccctgtcatttccctaagaaagcactgaagttaactcaaaataggctgaaagaaaaaaagcaatcctctgagttctaggtttcacaaaaggaccacgtgttaaactatgtacatcgatttgatgtgcaagtatgcaataaatatgtacacatacattcctatctgctttacatcattctagagtattcatagtatatcaagatgggatttagaaatgtgaaaaggccataacagtgaaaaggaaaaaaaaaagataacaatagtttttagaccagtcgaataataatgcttagctagttaattattttaactttggagcagactaaaaaagttgttttgaaataaatggtacctgtaagtgatgattactgcaatacttgttaaatgttatttgtcagcactgaccggaattatatagtgctagtaacacagctcccactgtcctagaattcctctaaatggccagctatagctaccattatcctgataagcatttcaagagttgtgttgctgagccttttaaaagataactagtttataacctatgtctccttatgtggctacatcagttactcgtggtcccaatgaagtataaaagaggatataagctgctgaagatttcacagaagaaacggagatatcagaaacttcatgatcatcaaacttaaaccaccgttgtcttgctgcatttttacaataggctgtgtagtggcctccatccagcccaccgtagtgatttgaaacagaaaacaaattatatttcttcaaattgttctttggaccaataacatactgtgacaagtcaagattttctaacgggaagtccacagatgtctgtaatttttgtttccacctgccatcgtaggaaaaacgtttcagatgcactaaaagcacaggtggtaacttccagatttctatcttttttagagaatcccgtcgagctctgcaatgactgcagtaaaatctgttgttatctgtgagtttttcttctttggaaaataatctaaggcaatcctgtaatgtacatttacttgtggatgctagtggtagagacaaatacatgaaggcctcaaatgtcctagactttttgtgacatgtgaggcactgtactgtagatttgaattgaccctgaaaaagtgcaacaataatagactcattgagctgcttgtgtttctgccaggcatgttctgcagctttaaagtcatcgagatgatcattattttcttctttatatctcttccgattatcagctttatttagatcttcatggagaccatccattaggaacagaagcaattcttgtgaatcttgctgactgtatcctgcaaactggtcattgatcttcccaatggtgattttaaagtcctttggactgatatatctatactgtcctgtccacagggctttcatgattataccaaattcttctgccacttcacctttatgccccaacaaatttgacctgttaatatcatcctgataacagtttcggttgaaataatcagccaaatgtggagcgttacataggcactgcaatattgagttcatataacaagtatttcctaagttacgaagtccagtaagagctggtccagaacctccaaaaacaggattgaggttccgaatctgagaagcagaaagccttgagatctcagctttaggataacatgttggcttgttttcccgattaactgttggagttactgttggcttcctcttctcttcctcttgaatagcctgggttatatctggggaggagtaggagcgcttcagtttggaaggttccctatcccgctcagcaggaatctgtggcttggctttatgagttggaggggtggaaggaggtgcagatgaaggagccatttccggtgggtacatatgaacagtgttggtgggtgaatgataataacgaaaggttccagtgattgggtcaagaaacttggcccagcctgaaggcagtcctggtacgatcctccccatttcttcacttcgtgctcttgtcaaaggttctcgttgagctttatttctttcggtatcgtctgtatcctctctaaaagttcctgtccttagaattccactttctggttgtcctttaatcttaaatggcttgcctgaacctgaatcccctgtcacagatgtatggggcacatctcctgttgactttttctgtatttctggggttggacaccttttccccctatcttctacagatttcttggcatcagaagtttcatgttcacttttactttgtctttttactcctgttatttctttgcccctctttgctgaggtttctttatcttctttcttggcctgttcactttctttcttctccatttcttcttttgctttttgttgcttctctgtaatttcattttcttcagcttcttgtttctttttggctttttgttcttgttcttccttcctcagtttctctttctgttcctcttgctgcctttcccgaagttctttttcttgtttgtttttttccattagaagagcagtttctgcatgaatacgagccttttcttcatctgttaacatgagagttggagaaaaaactactggcttggtggaacgatcaggaataacttttccactctgaggagattgttgctcatggtttgtactttcagattttattctatgctcttcaggcaatttgactgctggttttttagtacgatcaatctgtggaacattctttatactaggcactggctgaattatgggtgaaacatcagatttagaagcagcaactggttcaactggagttgatatattcagtggtcccattctctcattttgaccacttatcaattctatattttcatctacttctatagatgcaggtggcgtctgggcagcaggtttagaaggaattgattcttccaatgagggataagtaaaatccaatgagatagacacctcttcattctggcgtcgtgggggtggagtgaccttagcatttgttgtatactggggataacaaaggagccagttttcatagcctccctctaaaaccaaaggctcattgcgcaggacagttttactttcccacttgaaaagtgcatctttcagactccggagagttgttccaatctgtaaatctttggcagaactaaaccagtcaagaagtaccacatactccacattccccctcttcttccatgtgtctttagaatcatctggcaggtgtgcttcaatccaactagcagtgactcctggactgatggcttcttcaggaacactgagagaatgtaaaatacaggaatcctgataatcctgcattcttcgagcatccattataatcaagctgatgtttttatccgtcatcattgtgtatagttcctttgctgtgattgctcctttctctttggtctcacatttttcattcttttcaccattgctcttttgggttttgtctttggaatccaaaacattctccaaagagcctttagccaatgtgccaccatcctctcttcctgtttcctgccttttttgttgtagccgctgtgcttcctcctgcctgtctttttcctcaagttttttccggacttcagcttcttcatatcttaatttaaggctttcagagagtctttcagcttcttcgacagcttttttgatgtttccaggtccaagtattgaatggaaataatcctgctgttgcttgaaatcaggtctttttttgataagattataaacagtcacgtatttcatatatagtacataggccctttcctcatcacgatctaatctgcattcttctgctgtcttaaagatcttcagggcactgtgcacataactcttagtgcttattttctctggtttaacttctgtcttcttattaaggtcttttagtgaagaactgaggtagagttctttaggaactgaagccacagcaggcatgatgaattatctttacttttccactttcacaatggatgctatatttccttacaagtgcttctttccgtgacgccgggcgcgcttcactaacgccagccttctcgccaaatgcccatctcccaagaactcgagggagaattagccttggctaccaggacggaagccagcccagctc

SEQ ID NO: 11744 - RNA, 5952 nt, Homo sapiens
  source 1..5952: mol_type = other RNA
ctgaatagctgggactacaggtgtgcaccactatgcctagctcatcttttttttttttttttttttcctttaaaagatatggagtctcgctattttgcccaggctggtcttgaactcctggactcaagcaatccacctgcctcagcctcccagagtgttgggattacaggtgtgagccactgtgcccggcctgaattatcttcttattgtaaaatttcctttaatgcttaatagttgatgtatattaagtgctaactaaatgttcactgataaacattaatcagatgctgctaaatattgtctttctttattcacagatgatagtcaatgggcacaacatataagtagttacaatgaaatgagaagcaatatagcagtcaggctatatgcatgatttaacaacaaaattatcacttccttttaatttagaataagggacaatttaaaaagcatctcttggccctatcatttctgttccagtagttagtgttcatatgtgaatactaagtttgacattcctttctcccatagaaccattttggtgatttggatggtggccactacactgctttctgcaagaattcagtcacccaggcctgatatagctttgataacacacgagtcagtgagattccagatacttctgttcaaaatgctatggatctcctgttctatagctgccagcccttttccataccaatacaaaagcgttaagagccaggaaaatggtgtttcctgaacactgcaaaacaagcagtcagcatctggtggtagagttttgcttggtcattaaactcttagaacttacttgcatcattaacatttttatgccttgtgggcatgttatacaacctttcatcttaagataaatctgtcgtccagaagatgggtcttggttcactaaaaaaggcagtgtgaatataatgcaatgctaatggatgcaggccttcaaaacactgcaattatatagtgagttcaggtttcaaaattcagtgtttatcagaaaatatctcataatcatatatattcaacaaattattttccaaagatactcatgaagctaaacaaaaataatttttgttcaaatggctcgatgagtttaagaatatgatttgaatatatttgatataataatttagccaagaagtggtctcttagactaattgtaaaacatgaaaagttgtcagcttcacaatttgaaccccatcctttcatcttctccctgagagcctgctaatggtggtctctttctgaagcacttttagaatcttatttttatatggagtgttttactgactatatatatagcaactgagtccctcggttaaataaattataagctcctttaaccctcttaatacatcactctgtaaagatgtagtttataatgcagttcactttgcaatcatgcctgactcccggcatttttactttaatatttagaatgaatattctcaatatgtgagaatactagtcttgaaagaatgactctgggtgttattatatagcacgtgtgtatataaaatctatggttttactgtcctatatttgataatacaatattaaagacagaacacccacagggttataaattatttttctcattaagattttaatgtagctgtaaatgaaattctcgttttaaaaaaattaaagtttccatttttttttttagaataaagatttagtgcacaaatacagcccaaagccaacagaaaaattgctttgccctgtcatttccctaagaaagcactgaagttaactcaaaataggctgaaagaaaaaaagcaatcctctgagttctaggtttcacaaaaggaccacgtgttaaactatgtacatcgatttgatgtgcaagtatgcaataaatatgtacacatacattcctatctgctttacatcattctagagtattcatagtatatcaagatgggatttagaaatgtgaaaaggccataacagtgaaaaggaaaaaaaaaagataacaatagtttttagaccagtcgaataataatgcttagctagttaattattttaactttggagcagactaaaaaagttgttttgaaataaatggtacctgtaagtgatgattactgcaatacttgttaaatgttatttgtcagcactgaccggaattatatagtgctagtaacacagctcccactgtcctagaattcctctaaatggccagctatagctaccattatcctgataagcatttcaagagttgtgttgctgagccttttaaaagataactagtttataacctatgtctccttatgtggctacatcagttactcgtggtcccaatgaagtataaaagaggatataagctgctgaagatttcacagaagaaacggagatatcagaaacttcatgatcatcaaacttaaaccaccgttgtcttgctgcatttttacaataggctgtgtagtggcctccatccagcccaccgtagtgatttgaaacagaaaacaaattatatttcttcaaattgttctttggaccaataacatactgtgacaagtcaagattttctaacgggaagtccacagatgtctgtaatttttgtttccacctgccatcgtaggaaaaacgtttcagatgcactaaaagcacaggtggtaacttccagatttctatcttttttagagaatcccgtcgagctctgcaatgactgcagtaaaatctgttgttatctgtgagtttttcttctttggaaaataatctaaggcaatcctgtaatgtacatttacttgtggatgctagtggtagagacaaatacatgaaggcctcaaatgtcctagactttttgtgacatgtgaggcactgtactgtagatttgaattgaccctgaaaaagtgcaacaataatagactcattgagctgcttgtgtttctgccaggcatgttctgcagctttaaagtcatcgagatgatcattattttcttctttatatctcttccgattatcagctttatttagatcttcatggagaccatccattaggaacagaagcaattcttgtgaatcttgctgactgtatcctgcaaactggtcattgatcttcccaatggtgattttaaagtcctttggactgatatatctatactgtcctgtccacagggctttcatgattataccaaattcttctgccacttcacctttatgccccaacaaatttgacctgttaatatcatcctgataacagtttcggttgaaataatcagccaaatgtggagcgttacataggcactgcaatattgagttcatataacaagtatttcctaagttacgaagtccagtaagagctggtccagaacctccaaaaacaggattgaggttccgaatctgagaagcagaaagccttgagatctcagctttaggataacatgttggcttgttttcccgattaactgttggagttactgttggcttcctcttctcttcctcttgaatagcctgggttatatctggggaggagtaggagcgcttcagtttggaaggttccctatcccgctcagcaggaatctgtggcttggctttatgagttggaggggtggaaggaggtgcagatgaaggagccatttccggtgggtacatatgaacagtgttggtgggtgaatgataataacgaaaggttccagtgattgggtcaagaaacttggcccagcctgaaggcagtcctggtacgatcctccccatttcttcacttcgtgctcttgtcaaaggttctcgttgagctttatttctttcggtatcgtctgtatcctctctaaaagttcctgtccttagaattccactttctggttgtcctttaatcttaaatggcttgcctgaacctgaatcccctgtcacagatgtatggggcacatctcctgttgactttttctgtatttctggggttggacaccttttccccctatcttctacagatttcttggcatcagaagtttcatgttcacttttactttgtctttttactcctgttatttctttgcccctctttgctgaggtttctttatcttctttcttggcctgttcactttctttcttctccatttcttcttttgctttttgttgcttctctgtaatttcattttcttcagcttcttgtttctttttggctttttgttcttgttcttccttcctcagtttctctttctgttcctcttgctgcctttcccgaagttctttttcttgtttgtttttttccattagaagagcagtttctgcatgaatacgagccttttcttcatctgttaacatgagagttggagaaaaaactactggcttggtggaacgatcaggaataacttttccactctgaggagattgttgctcatggtttgtactttcagattttattctatgctcttcaggcaatttgactgctggttttttagtacgatcaatctgtggaacattctttatactaggcactggctgaattatgggtgaaacatcagatttagaagcagcaactggttcaactggagttgatatattcagtggtcccattctctcattttgaccacttatcaattctatattttcatctacttctatagatgcaggtggcgtctgggcagcaggtttagaaggaattgattcttccaatgagggataagtaaaatccaatgagatagacacctcttcattctggcgtcgtgggggtggagtgaccttagcatttgttgtatactggggataacaaaggagccagttttcatagcctccctctaaaaccaaaggctcattgcgcaggacagttttactttcccacttgaaaagtgcatctttcagactccggagagttgttccaatctgtaaatctttggcagaactaaaccagtcaagaagtaccacatactccacattccccctcttcttccatgtgtctttagaatcatctggcaggtgtgcttcaatccaactagcagtgactcctggactgatggcttcttcaggaacactgagagaatgtaaaatacaggaatcctgataatcctgcattcttcgagcatccattataatcaagctgatgtttttatccgtcatcattgtgtatagttcctttgctgtgattgctcctttctctttggtctcacatttttcattcttttcaccattgctcttttgggttttgtctttggaatccaaaacattctccaaagagcctttagccaatgtgccaccatcctctcttcctgtttcctgccttttttgttgtagccgctgtgcttcctcctgcctgtctttttcctcaagttttttccggacttcagcttcttcatatcttaatttaaggctttcagagagtctttcagcttcttcgacagcttttttgatgtttccaggtccaagtattgaatggaaataatcctgctgttgcttgaaatcaggtctttttttgataagattataaacagtcacgtatttcatatatagtacataggccctttcctcatcacgatctaatctgcattcttctgctgtcttaaagatcttcagggcactgtgcacataactcttagtgcttattttctctggtttaacttctgtcttcttattaaggtcttttagtgaagaactgaggtagagttctttaggaactgaagccacagcaggcatgatgaattatctttacttttccactttcacaatggatgctatatttccttacaagtgcttctttcctttaggagttgtcccactcctctccgcggacagagcttgtctccggggtaaccagcagctggtggaaggaaaggcgttcatcgttcacagcggacgacttcccagagaacaggtgctagggcccaagacccgcactcaccgtgacgccgggcgcgcttcactaacgccagccttctcgccaaatgcccatctcccaagaactcgagggagaattagccttggctaccaggacggaagccagcccagctc

SEQ ID NO: 11745 - RNA, 2324 nt, Homo sapiens
  source 1..2324: mol_type = other RNA
ctgaatagctgggactacaggtgtgcaccattgtacttggctctcacaatttttaaatataaaagtacttatatttatccataataaacagctatcataaatcaataagaaaaaagcaaccactactgaaaatgtgcaaaggatataaacaggtgattcacagaaggacaaagaaaagtgacccacaaacatctcaaaagatgctcaatctcattagtgagagagaagtgcaaattacaacaatgaaatagctatcatttctcaccttcataagactggcaaaaattcaaaagattcttctttttcttttttttttgaggcagggtctggctctgtcgcccaggctggagtgcagtggcacaatcttggctcactgcaacttccgcctcccaggctcaagccatcctcctatctcagccttctgagtggctgggactacaggcatgcaccaccacacccagctaatttttgtatttattgtagagacgaggtttcaccatgttggccaggctggtcttgaactcatgagctcaagctatccaccagccttggcctcccagaatgctgggattacagatgtgaagcactgtgcccaggctcaaaagattattctatcttgcattgaccaaaggatggaaaaagaggcactcatactgtatgactggggctgtaaagtgaaatcaaagttttttaagcgggaaatttggtactctttaatataatttaaaatgtacatatcctttgagggattccatttctttattttattttatttttttttttttttttgaggcagagttttgctcctgttgtccaggctggaatgcagtggcgcgatctttctcaccgcaactcctgcctcccaggttcaagtgattctcctgcctcagcctcccaagtagctgggattacaggtgtgagccaccacacctggcctgagggatttcatttctaaaaattttattttacagaaaaacttgaacatgtttacaaaaatataatagcaaaaatttaaaatgaataagcatatagtatgcttaaaaagaggatgtcaaggccaggcacagtggctcatgcctgtaatcccagcactttggcaggccgaggtagacagatcacaaggtcaggagatcgagaccatcctggctaacatggtgaaaccccatctctactaaaaatacacacacaaaaaaaattagccgggcgtggtggtgggtgcctgtagtcccagctactcgggaggctgaggcaggagaatggcatgaacccggaaggcagagcttgcagtgagctgagatcgcgccactgcgctccagcctgggtggcagagtaagactccatctcaaaaaaaaaaaaaaaaaagaggatgtcaataactatgaaatgcatagaaaagaatacaactgaatgcacatcaaattgttgatggcagtttctctaagcaagggcatgggatgaggtgcaggctgtggtgaagatgaacttttctttttttacttttggtttggtttaagtatacattcctgtatttattgtgtaattaataaatggaaagatccatagatgaataactgccttgtaacgtcagacattctttaatggaatgaacatgtggcacatggatctttgggagtttgggttggattttggggatgttaaggtctcctatcaatcttagttaacatgtcacagcttctggtccctgacttagatcacctctgtgtaccctcagcctactgaggaaaaaggcaggaatcacctctgtgtcattgaagcggtgaggctccaggcatgggttccacctgaccacctggggagacggcatgaagtccaaaaatggataaatggatgttcttgtaaagttgaatccatgaatgccatcttctggaaacactataatctgtacatccttttgggctgcagtcatcacttgctgttcatagatgtcaaggttctggttcatgagctccaaggcctcttggcggctgatgagagccagagggttcagactcaggatggatggatgctcatacacggcagccacataatattcagcctcgtgatggtcagccacgctctcctccccggtgtgggctcccagggcaaccacgtaacagccgcagaggaaaagagcaagcttacttctggctccagacataatgcagaccacaaatctgctcttagcgcgccttccgccctgaatatgcgcatgcgccattctccctttacagccccgaaaacgctccagctggccgactcggagacaatggcgagaggcctcagagttcggcttcttacctgctttgcataggcagcaatctcct

SEQ ID NO: 11746 - RNA, 2008 nt, Homo sapiens
  source 1..2008: mol_type = other RNA
ctgaatagctgggactacaggtgtgcaccgccacactccacagctgatgttttaataaagtgccactgagtatcagactgatcaaactgaaaacatcccagaacttcagaccaggttaagggggccaatgagaagatcatgaaaagtgacatcagatgaaagctgagatctgtgaaagtttcaaatcagtttttccaagtaagtccacagaccatttgataggctaagcccagttctttacacaatgtagcagccatcatgtctgagtactaattgttctcttcccactggtttttgtgaaattttctgttctgttaccttttaaagattctagcaagtttttgactgtttcaattgcaaacttattgcttttcttcttggtaaaggactttctgtttggagcagatggtagcaatagggataccagcccccagggccgattacttgatatggaaggtcgatctgtatcttcctgttgtaaaatccaggcactttctcgggccaaatctacaaatttttgcagctggctttgacttacatttttgcttatgttgagagaagtttcaaatggattctgaatgtacagaggagaagaatcaggtttgttttgctcccttccctgtcgaatatttatggaatttttatcgaaagcaaaattgccaaaatactcaaaaaattccttcagtagtaattctaatgtttctgtgttctgtgaaggtttaattctactcaagtcacgaacaaatgtgcagttgttgccttctattacacatttatcttctgcatctgctagggtttttaaggaatctagtgttggaagaatagggggtgatcttctctggagaaaaaagatgaccatcattgtaagggagaaatttgtaatccatgcaccaggaatactacttgttagtgaatgtgctcgagcccagcaccgtacactgaacaccaaggctctcactcttgagtctagggcaccatatatataaaggagttcggaacttgtcaaggcaatcctattgttcgtagtcaaatcacactgaaatccggaggcctggtgtgagaacctcacgagcggacaccgggcatttaatattttttgcacacccacacagccagggccaaagtggtcaaggcactctcctaacacagacaggatcttctgagttgcaattctttctgaaggaacatttttcacttgaaattccatcagaaaatttcctgagatcttgtgagcgctgaggtttctggtttcatctagatccaaaaacatgtccaaatcacatcctaacttcccaaaagtgttgactgaggagccaaagggtctgactatgcagtctggaaaatacgcggcggccatgtcttcaataagagaacaggtgagatatcggagcttagtgttctcctctgttagctggaactccttcaagagagtgttcagctgatcgtctatactttctgcataacaaagtaattcaaaaagctgcttgtttgaacgtggcaactgattacttgaccgtacgcgtgaccgttcagaagtctggtttttcaacttcagattgaagaaacgtgatctgaatggaattgcagtctccatggccgtgcttggagtatgagtcccattctgcagtgaacctatgctttccttttggcaaaattctacgacagcatagagaccaaagctttcatagaagaaatgattattaataggtccaaattgggataaatatttaagaaacttgttttcactgattttctctgggcaatgtattaaaacagtccgctgtgcctgttctcgtctttcattttgcatctcagagaatctccttttgggaatcttgtcttcaaagcctgtctccacgctccctgaaggctgctcgtctctcctaaggtctttggccacagttcctgggcaactcaaaagcctgacgataggccgctggactcgagttcttctccgggcacacaggttcaaacgggtcaagagccccacgccgggaaccgccattgc

SEQ ID NO: 11747 - RNA, 6550 nt, Homo sapiens
  source 1..6550: mol_type = other RNA
ctgaatagctgggactacaggtgtgcactaccatgcctggctccttttttttattttttgtagagacagggtctccctatgttgctcaggctggtctcgaattctgggctcaagcaatcctctcaccttggcctcccaaagtgctgggattacaggtgtgagccaccacacccggctgccaacaccactttcgattttgggataatctgggtgcacagtgatcagaagcttacctaccccacgttgcataaaaaaaagtatgaatttaaaaattccaagagtaaactaccctatgaaaacctctggcagtgctgatgaaaacacatttctggtagtgatatgtcttggtccctctggtctcacagaatgtgtagtcctgagaaaaaataaacctggactcttggtaaaatatttgaataattaactgctttgctcattggttgtaactggcaagtcattctctttactacattaaagtctgcactttcattttacagacagtcctacagttcaactccaacatcagggactgagtcgtacacaggaagatcactgagtaggttctgtggagacgcagtcggcccatatgcacgtcaccactcggctcccagctcaggtgcagaccaacggcgaccacttgctccactttgctctgtgacagcagacgaggtaaggcatgttgcagatacatgctgaatatagggatgcctgtacacaaaactgcactcatgctgtgataacacgcaaaaggtcacacactggaagagccttgcccaacgaacgatagactaacaggccagaggcggggaaagcttctcggagtcccactatcttctttgtttttattgctcctacttacttatgtgatacctttttagtagaatgactagttttctaaacagaacctgtaatgacaggctcacatttcttcctcaactcccacctccaaagccactccattcaaagaactgctggtgaggtgctggggagtcaatccgtcgtagaggggaagcgttctacccctccagatccttctgcagacaggagggtgtctgcattcggcggagtccaagagtgcggtgaggacacagtggcaaaggaataatgccattccttgaggcagcgctgggctagtagagacctgtgaggaagtaatgtgtcctgtggggatttcagggtaatttaatcagcagcacttcagcagggtagaaagcaagggcggggaaaaataatgaagtcagcactcagctaccaggagctcctctgttcaatctaacggggagatatgaccccagagcagggcttccctccctccacccggctcccacttccagccaggtaattctgtgtcgtgggggctgttgggcaccatccctggcctccctccacgagtgcccacagtactgccctcctccccacctgtgacaaaaatgtctccagacattgccaaatgttccctggggggcaaaattgcccctgttgagcaccactgccctagatgaactggaaaagttggtttgtgaatatgtgagcttagttgtttctaacacagggctgaaaaacaagagaaggggacaaaggctgctttcatataaaaatgtactgtagtaatcagtaagaaaaagaaacaacattggctaagtcacgaataggcatttcaccatatgtacatgataaatggccaatcaaaataaggaatggggctcattctgctggaaattaaatacattcaaacaagaacagagatccattagcaaaatgtttaaaaataatatcacagggttaccaggggtatgacaaaaatggacacttccatacacactaggtgaatatattggtgaaaatagttcagataaacatacaaccatgtatgtaaaagtatttatcatcaatgcattatttgtagtagcaaaaacaacaagcagccttggaaaccagttaatgtcctcagcagggaattaataatattattgtatattcatgaaattgacaccatgtggccacacaaatgcattacacaggcctctatgtaacataggatattcattagagaattgtttttcaagaggacaaagtactttcatttttgcctagaaaatgggggaagacaaaaatgcgcttctctctaggttgtgtgattttaggttatcctaagtttcatccttacgtgctcctgaattatctgaaatatcgtatctttaaaaacagtaacaacaatagtaacaagagctctgtaattcctacccttccaacctcaggagcccacccacccctatccgagccgacccctgactgcccctgccattgctccctgctgagttgcagacattgacttcttgccaagcctcaggccttgctcacatcgacacctcacagtgaccctgagaggcagatgctgtgaccccatttcacagatgaagggcctgagccacagaggaggaagactgcctcagccacgccgctagtaagtggtagttcccaactctagagtcccaaaagaattctgtcctacttatgaaaagtatatccaataagcagtacctccctgtgtttacaacttatctgctgatcccaaggatgggaaaagctgcactcagaaacttgcaaattgtgcaactgttccccacgattcccttggggccagtgccgactgaggcatctccaggaggccccagttgggcttggggacatgctgagaggtgacagcactgctctcaagtcatatcctctgcttctgcaaaagctgtggagctcacccatcaatagcagctccatgccgggcgcagtggctcacgcctgtaatcccagcactttcggaggctcaggcgggcagatcatctgaggtcaggagtccgtgaccagcctggccaacatggtgaaaccccgtctctactaaaagtacaaaaacttagctgggtgtggtggtgtacgcctgtgatcccagctactcaggaggctgaggcaggagaattgcttgaacccaggagggggaggttgcagtgagctgagatcacgccattgcactccagcctgagcaacagagcaagactccatcgcaaaaaaaaaaaaaaaaaaaaaaggctctagcattgccagatcccaggccctgtggaaggtatttccctccctcttttgtccttgcttgtctcagagcccttttcacagtctcttgtgtgcttctttccctgttaggaccaatctttacaactccagcaagcgcagcaaataagatgcagaactgggggagatgcaacgtatgactcaattcccttgagccgaaaacactcacttattaacaatatttttttcttttttttgagacagagtctcacaaaaacaggcacacgcccccacacccggctaatttttgtatttttagtatagatggggtttcaccatattggtcaggctggtctgaactcctgccttcaggtgatccacctgcctcagccttccaaagtgctgggattacaggcataagccaccacgccccaccaatgaaatgttttctaaaggtgttttcatcccttttgtgatctcctaaactcccaaggtgtatcacacacttcgctgggctctgggcaaacaaaacttagacaaggtccctgattctagaaaccctcggtcgagggaaccacaaaccaaccagagtggagggcagggagaggtcctaggttgggagctgggagcctggagcacgtgccaggtgctctgcagcccagcttcattatggaggctcaagcgctgtgaatttccaaaaacagtgaacacacccctagctgattgaaatacaaaaaacatattccacagccaaatgaaaatgacttttggatcctccacctaatttgggtgtttatgccgcctcgcccctcttttggcctggacaattgaaatatatctgctctcaggggagacgcccacggtgtcagggctggagttggcaagagacagggggaagaggactagacctggagtcagagatgaagttcttgtctgggatctgtcactaagtctcagcggggacccaggaagtcactccacctctcatagttcctcatccacaaagtggaaatacaagcaagtttaattctccatcgtaaggttggagctcctgtctgtgaaaggactggaaatgtaaaatgcgctcttcaagtacaaaggcagagaggatccataaacaggcacaggctgccctttggtataaactgttcacattaaatctatgttatgttgctcaagagttaaaataagctcaaaggagaggctgattccaatgtcaacccagggaagacagacactgaaattccaaactgagttaccaaaaacaatagatggatgagacatgcagacatgccacaatccggcacatcagagttcgatgtagtcctgctgcaaacacatggaatccgagaagtccaatgcaaacggaatagatttcttgggatctaatatttttcaaattgcctgaccagcttaccttctaggaaaacttatttaagggaggcaaataatttggggagatgagtataagaggtagtaggaggaagctaagggaaatcaccactacatattgcaggaatgtattagaaggcaaatatggcccaaagaaaaagctccactgaaaaaaacattgaatactgaccacagaattagcaccttgctcccaggtcaataaagtgaaccaaaaaaattacaaagaccttgctcaatcctgaggttcgtgaggaatataggagagttgtgtgttcacgtgactcctgaaaacaaagagcagtactattcgaagggcatgatgtcttgatcttaggatcaaatattctagaccttgagccggagaatctgcattacagtaggaaaaatggggagtgctttatgcctgtggattcaggacacaccagcaacctacacgtgtagcattctctaagtcataatgaccattctcatctcccactgagggcaggtgtaagactcttctcttgcagtgctctgatagaaagctgggtttcttcttcttctctataaatcatagggaaaccaaatatttgtacctgttacagccccaaagctgaaagcaataaagaataaacacatacagcaagctacgaggtgcgtctgtttaggaattgcctcaacgttgggtttctattgatagaacaggggaggaggttgcctctgaccttcctgaggctcccactgtaccctggctgagtagcccacagttaattttaagtggcaaaagaaatgagaacaaattcctccaggaagagaaattagatttctgctaaaacagtgctctccatagggtatatgagcacattcgactaccactggaaaataacctgagggcaggcacatggtgcccactgttagaaatcgtgcagttagattagaatggaagagtgtctgagtttttagataattttacacgtcaggatatggctaacaggtcacgttcagggcctatgcttgatactgtcgaaatacaaacaaaaataactgcctagagagaatattcacgtcctaaaagagaaaatgttgtatctgggtggaagaatgatttaactcctgaaactcgagaacacagaacaacaacaaaaataatttccttgaacatattcaactagaatggcaaggcattttcctacataaaacattagaatgttcccattactccaaaggaatccaataaataattttacagtgaaagagcctggatcaaaactggaagtgacaccggcccccgatgaacacaagtcacaggtccctgtgcaggtcccagggctgagtcatccaagaactccaccaccaccgtgagcccggcctccggtttcatctttcccgaatgggactggctggaggggccaagctgctttacagaagagttccatctggtaagcccgggtggtgagcgaagccaaagatgacaacacgagaaggggtcaaagccaaggtttcctcacgctgcctttgtcttcttcctgcagcctggcccgatggctgaagctgggtcccaggaggcgagttcttcagcggggcctcctcacccaggctggagcaagtccgctgcacccgtcaagcggggaagagctcgggcgggctttctccatagcaatactttgctatggggtcccggtaggtgttctcatgctgcacgctctgagatgaggtcctgcatttggccaggcacaactcaaagtgatcttcgactgccatgaagaggttctggaatgccacggctgcccggttgaggaagcgctccaggagaagttgctgcttgaaggtgctgctgaggaagtagacgagcgacagcccgaagaccagggcgagcacccacctcttccgcagaagccggcgccacaccatggccgccaggttcaccatcccggcgcggacgtggggcgcggcggccggggcgcggaacgcggcaggcccgggtcccgggcggcatggcccctacgcgcccggcagccccatccctccaggcaggcgccggccccgccgcccgcagcccagtctgctcccggcagccttgggcgcagccccacgtgac

SEQ ID NO: 11748 - RNA, 6859 nt, Homo sapiens
  source 1..6859: mol_type = other RNA
ctgaatagctgggactacaggtgtgcactaccatgcctggctccttttttttattttttgtagagacagggtctccctatgttgctcaggctggtctcgaattctgggctcaagcaatcctctcaccttggcctcccaaagtgctgggattacaggtgtgagccaccacacccggctgccaacaccactttcgattttgggataatctgggtgcacagtgatcagaagcttacctaccccacgttgcataaaaaaaagtatgaatttaaaaattccaagagtaaactaccctatgaaaacctctggcagtgctgatgaaaacacatttctggtagtgatatgtcttggtccctctggtctcacagaatgtgtagtcctgagaaaaaataaacctggactcttggtaaaatatttgaataattaactgctttgctcattggttgtaactggcaagtcattctctttactacattaaagtctgcactttcattttacagacagtcctacagttcaactccaacatcagggactgagtcgtacacaggaagatcactgagtaggttctgtggagacgcagtcggcccatatgcacgtcaccactcggctcccagctcaggtgcagaccaacggcgaccacttgctccactttgctctgtgacagcagacgaggtaaggcatgttgcagatacatgctgaatatagggatgcctgtacacaaaactgcactcatgctgtgataacacgcaaaaggtcacacactggaagagccttgcccaacgaacgatagactaacaggccagaggcggggaaagcttctcggagtcccactatcttctttgtttttattgctcctacttacttatgtgatacctttttagtagaatgactagttttctaaacagaacctgtaatgacaggctcacatttcttcctcaactcccacctccaaagccactccattcaaagaactgctggtgaggtgctggggagtcaatccgtcgtagaggggaagcgttctacccctccagatccttctgcagacaggagggtgtctgcattcggcggagtccaagagtgcggtgaggacacagtggcaaaggaataatgccattccttgaggcagcgctgggctagtagagacctgtgaggaagtaatgtgtcctgtggggatttcagggtaatttaatcagcagcacttcagcagggtagaaagcaagggcggggaaaaataatgaagtcagcactcagctaccaggagctcctctgttcaatctaacggggagatatgaccccagagcagggcttccctccctccacccggctcccacttccagccaggtaattctgtgtcgtgggggctgttgggcaccatccctggcctccctccacgagtgcccacagtactgccctcctccccacctgtgacaaaaatgtctccagacattgccaaatgttccctggggggcaaaattgcccctgttgagcaccactgccctagatgaactggaaaagttggtttgtgaatatgtgagcttagttgtttctaacacagggctgaaaaacaagagaaggggacaaaggctgctttcatataaaaatgtactgtagtaatcagtaagaaaaagaaacaacattggctaagtcacgaataggcatttcaccatatgtacatgataaatggccaatcaaaataaggaatggggctcattctgctggaaattaaatacattcaaacaagaacagagatccattagcaaaatgtttaaaaataatatcacagggttaccaggggtatgacaaaaatggacacttccatacacactaggtgaatatattggtgaaaatagttcagataaacatacaaccatgtatgtaaaagtatttatcatcaatgcattatttgtagtagcaaaaacaacaagcagccttggaaaccagttaatgtcctcagcagggaattaataatattattgtatattcatgaaattgacaccatgtggccacacaaatgcattacacaggcctctatgtaacataggatattcattagagaattgtttttcaagaggacaaagtactttcatttttgcctagaaaatgggggaagacaaaaatgcgcttctctctaggttgtgtgattttaggttatcctaagtttcatccttacgtgctcctgaattatctgaaatatcgtatctttaaaaacagtaacaacaatagtaacaagagctctgtaattcctacccttccaacctcaggagcccacccacccctatccgagccgacccctgactgcccctgccattgctccctgctgagttgcagacattgacttcttgccaagcctcaggccttgctcacatcgacacctcacagtgaccctgagaggcagatgctgtgaccccatttcacagatgaagggcctgagccacagaggaggaagactgcctcagccacgccgctagtaagtggtagttcccaactctagagtcccaaaagaattctgtcctacttatgaaaagtatatccaataagcagtacctccctgtgtttacaacttatctgctgatcccaaggatgggaaaagctgcactcagaaacttgcaaattgtgcaactgttccccacgattcccttggggccagtgccgactgaggcatctccaggaggccccagttgggcttggggacatgctgagaggtgacagcactgctctcaagtcatatcctctgcttctgcaaaagctgtggagctcacccatcaatagcagctccatgccgggcgcagtggctcacgcctgtaatcccagcactttcggaggctcaggcgggcagatcatctgaggtcaggagtccgtgaccagcctggccaacatggtgaaaccccgtctctactaaaagtacaaaaacttagctgggtgtggtggtgtacgcctgtgatcccagctactcaggaggctgaggcaggagaattgcttgaacccaggagggggaggttgcagtgagctgagatcacgccattgcactccagcctgagcaacagagcaagactccatcgcaaaaaaaaaaaaaaaaaaaaaaggctctagcattgccagatcccaggccctgtggaaggtatttccctccctcttttgtccttgcttgtctcagagcccttttcacagtctcttgtgtgcttctttccctgttaggaccaatctttacaactccagcaagcgcagcaaataagatgcagaactgggggagatgcaacgtatgactcaattcccttgagccgaaaacactcacttattaacaatatttttttcttttttttgagacagagtctcacaaaaacaggcacacgcccccacacccggctaatttttgtatttttagtatagatggggtttcaccatattggtcaggctggtctgaactcctgccttcaggtgatccacctgcctcagccttccaaagtgctgggattacaggcataagccaccacgccccaccaatgaaatgttttctaaaggtgttttcatcccttttgtgatctcctaaactcccaaggtgtatcacacacttcgctgggctctgggcaaacaaaacttagacaaggtccctgattctagaaaccctcggtcgagggaaccacaaaccaaccagagtggagggcagggagaggtcctaggttgggagctgggagcctggagcacgtgccaggtgctctgcagcccagcttcattatggaggctcaagcgctgtgaatttccaaaaacagtgaacacacccctagctgattgaaatacaaaaaacatattccacagccaaatgaaaatgacttttggatcctccacctaatttgggtgtttatgccgcctcgcccctcttttggcctggacaattgaaatatatctgctctcaggggagacgcccacggtgtcagggctggagttggcaagagacagggggaagaggactagacctggagtcagagatgaagttcttgtctgggatctgtcactaagtctcagcggggacccaggaagtcactccacctctcatagttcctcatccacaaagtggaaatacaagcaagtttaattctccatcgtaaggttggagctcctgtctgtgaaaggactggaaatgtaaaatgcgctcttcaagtacaaaggcagagaggatccataaacaggcacaggctgccctttggtataaactgttcacattaaatctatgttatgttgctcaagagttaaaataagctcaaaggagaggctgattccaatgtcaacccagggaagacagacactgaaattccaaactgagttaccaaaaacaatagatggatgagacatgcagacatgccacaatccggcacatcagagttcgatgtagtcctgctgcaaacacatggaatccgagaagtccaatgcaaacggaatagatttcttgggatctaatatttttcaaattgcctgaccagcttaccttctaggaaaacttatttaagggaggcaaataatttggggagatgagtataagaggtagtaggaggaagctaagggaaatcaccactacatattgcaggaatgtattagaaggcaaatatggcccaaagaaaaagctccactgaaaaaaacattgaatactgaccacagaattagcaccttgctcccaggtcaataaagtgaaccaaaaaaattacaaagaccttgctcaatcctgaggttcgtgaggaatataggagagttgtgtgttcacgtgactcctgaaaacaaagagcagtactattcgaagggcatgatgtcttgatcttaggatcaaatattctagaccttgagccggagaatctgcattacagtaggaaaaatggggagtgctttatgcctgtggattcaggacacaccagcaacctacacgtgtagcattctctaagtcataatgaccattctcatctcccactgagggcaggtgtaagactcttctcttgcagtgctctgatagaaagctgggtttcttcttcttctctataaatcatagggaaaccaaatatttgtacctgttacagccccaaagctgaaagcaataaagaataaacacatacagcaagctacgaggtgcgtctgtttaggaattgcctcaacgttgggtttctattgatagaacaggggaggaggttgcctctgaccttcctgaggctcccactgtaccctggctgagtagcccacagttaattttaagtggcaaaagaaatgagaacaaattcctccaggaagagaaattagatttctgctaaaacagtgctctccatagggtatatgagcacattcgactaccactggaaaataacctgagggcaggcacatggtgcccactgttagaaatcgtgcagttagattagaatggaagagtgtctgagtttttagataattttacacgtcaggatatggctaacaggtcacgttcagggcctatgcttgatactgtcgaaatacaaacaaaaataactgcctagagagaatattcacgtcctaaaagagaaaatgttgtatctgggtggaagaatgatttaactcctgaaactcgagaacacagaacaacaacaaaaataatttccttgaacatattcaactagaatggcaaggcattttcctacataaaacattagaatgttcccattactccaaaggaatccaataaataattttacagtgaaagagcctggatcaaaactggaagtgacaccggcccccgatgaacacaagtcacaggtccctgtgcaggtcccagggctgagtcatccaagaactccaccaccaccgtgagcccggcctccggtttcatctttcccgaatgggactggctggaggggccaagctgctttacagaagagttccatctggtaagcccgggtggtgagcgaagccaaagatgacaacacgagaaggggtcaaagccaaggtttcctcacgctgcctttgtcttcttcctgcagcctggcccgatggctgaagctgggtcccaggaggcgagttcttcagcggggcctcctcacccaggctggagcaagtccgctgcacccgtcaagcggggaagagctcgggcgggctttctccatagcaatactttgctatggggtcccggtaggtgttctcatgctgcacgctctgagatgaggtcctgcatttggccaggcacaactcaaagtgatcttcgactgccatgaagaggttctggaatgccacggctgcccggttgaggaagcgctccaggagaagttgcttgttgggctgcaggcagcaggagacacagtactcataggcgctgcagcagccgttgggccagcagccatcacagcagtactgcttcgtgctagggacgttgacattacagcagccatttaccagcaaatccttcctctcgcaaacgtagccgagttcatccgtgatgaggtgcttcccttgaatggagttgcggcactgattgctcggacgactgctattgcccaagttaaactgcactttccacgggatgggctgattatggtcatgaacctggaggagattcctatctctcactgccctctcctcctgcttgaaggtgctgctgaggaagtagacgagcgacagcccgaagaccagggcgagcacccacctcttccgcagaagccggcgccacaccatggccgccaggttcaccatcccggcgcggacgtggggcgcggcggccggggcgcggaacgcggcaggcccgggtcccgggcggcatggcccctacgcgcccggcagccccatccctccaggcaggcgccggccccgccgcccgcagcccagtctgctcccggcagccttgggcgcagccccacgtgac

SEQ ID NO: 11749 - RNA, 6702 nt, Homo sapiens
  source 1..6702: mol_type = other RNA
ctgaatagctgggactacaggtgtgcactaccatgcctggctccttttttttattttttgtagagacagggtctccctatgttgctcaggctggtctcgaattctgggctcaagcaatcctctcaccttggcctcccaaagtgctgggattacaggtgtgagccaccacacccggctgccaacaccactttcgattttgggataatctgggtgcacagtgatcagaagcttacctaccccacgttgcataaaaaaaagtatgaatttaaaaattccaagagtaaactaccctatgaaaacctctggcagtgctgatgaaaacacatttctggtagtgatatgtcttggtccctctggtctcacagaatgtgtagtcctgagaaaaaataaacctggactcttggtaaaatatttgaataattaactgctttgctcattggttgtaactggcaagtcattctctttactacattaaagtctgcactttcattttacagacagtcctacagttcaactccaacatcagggactgagtcgtacacaggaagatcactgagtaggttctgtggagacgcagtcggcccatatgcacgtcaccactcggctcccagctcaggtgcagaccaacggcgaccacttgctccactttgctctgtgacagcagacgaggtaaggcatgttgcagatacatgctgaatatagggatgcctgtacacaaaactgcactcatgctgtgataacacgcaaaaggtcacacactggaagagccttgcccaacgaacgatagactaacaggccagaggcggggaaagcttctcggagtcccactatcttctttgtttttattgctcctacttacttatgtgatacctttttagtagaatgactagttttctaaacagaacctgtaatgacaggctcacatttcttcctcaactcccacctccaaagccactccattcaaagaactgctggtgaggtgctggggagtcaatccgtcgtagaggggaagcgttctacccctccagatccttctgcagacaggagggtgtctgcattcggcggagtccaagagtgcggtgaggacacagtggcaaaggaataatgccattccttgaggcagcgctgggctagtagagacctgtgaggaagtaatgtgtcctgtggggatttcagggtaatttaatcagcagcacttcagcagggtagaaagcaagggcggggaaaaataatgaagtcagcactcagctaccaggagctcctctgttcaatctaacggggagatatgaccccagagcagggcttccctccctccacccggctcccacttccagccaggtaattctgtgtcgtgggggctgttgggcaccatccctggcctccctccacgagtgcccacagtactgccctcctccccacctgtgacaaaaatgtctccagacattgccaaatgttccctggggggcaaaattgcccctgttgagcaccactgccctagatgaactggaaaagttggtttgtgaatatgtgagcttagttgtttctaacacagggctgaaaaacaagagaaggggacaaaggctgctttcatataaaaatgtactgtagtaatcagtaagaaaaagaaacaacattggctaagtcacgaataggcatttcaccatatgtacatgataaatggccaatcaaaataaggaatggggctcattctgctggaaattaaatacattcaaacaagaacagagatccattagcaaaatgtttaaaaataatatcacagggttaccaggggtatgacaaaaatggacacttccatacacactaggtgaatatattggtgaaaatagttcagataaacatacaaccatgtatgtaaaagtatttatcatcaatgcattatttgtagtagcaaaaacaacaagcagccttggaaaccagttaatgtcctcagcagggaattaataatattattgtatattcatgaaattgacaccatgtggccacacaaatgcattacacaggcctctatgtaacataggatattcattagagaattgtttttcaagaggacaaagtactttcatttttgcctagaaaatgggggaagacaaaaatgcgcttctctctaggttgtgtgattttaggttatcctaagtttcatccttacgtgctcctgaattatctgaaatatcgtatctttaaaaacagtaacaacaatagtaacaagagctctgtaattcctacccttccaacctcaggagcccacccacccctatccgagccgacccctgactgcccctgccattgctccctgctgagttgcagacattgacttcttgccaagcctcaggccttgctcacatcgacacctcacagtgaccctgagaggcagatgctgtgaccccatttcacagatgaagggcctgagccacagaggaggaagactgcctcagccacgccgctagtaagtggtagttcccaactctagagtcccaaaagaattctgtcctacttatgaaaagtatatccaataagcagtacctccctgtgtttacaacttatctgctgatcccaaggatgggaaaagctgcactcagaaacttgcaaattgtgcaactgttccccacgattcccttggggccagtgccgactgaggcatctccaggaggccccagttgggcttggggacatgctgagaggtgacagcactgctctcaagtcatatcctctgcttctgcaaaagctgtggagctcacccatcaatagcagctccatgccgggcgcagtggctcacgcctgtaatcccagcactttcggaggctcaggcgggcagatcatctgaggtcaggagtccgtgaccagcctggccaacatggtgaaaccccgtctctactaaaagtacaaaaacttagctgggtgtggtggtgtacgcctgtgatcccagctactcaggaggctgaggcaggagaattgcttgaacccaggagggggaggttgcagtgagctgagatcacgccattgcactccagcctgagcaacagagcaagactccatcgcaaaaaaaaaaaaaaaaaaaaaaggctctagcattgccagatcccaggccctgtggaaggtatttccctccctcttttgtccttgcttgtctcagagcccttttcacagtctcttgtgtgcttctttccctgttaggaccaatctttacaactccagcaagcgcagcaaataagatgcagaactgggggagatgcaacgtatgactcaattcccttgagccgaaaacactcacttattaacaatatttttttcttttttttgagacagagtctcacaaaaacaggcacacgcccccacacccggctaatttttgtatttttagtatagatggggtttcaccatattggtcaggctggtctgaactcctgccttcaggtgatccacctgcctcagccttccaaagtgctgggattacaggcataagccaccacgccccaccaatgaaatgttttctaaaggtgttttcatcccttttgtgatctcctaaactcccaaggtgtatcacacacttcgctgggctctgggcaaacaaaacttagacaaggtccctgattctagaaaccctcggtcgagggaaccacaaaccaaccagagtggagggcagggagaggtcctaggttgggagctgggagcctggagcacgtgccaggtgctctgcagcccagcttcattatggaggctcaagcgctgtgaatttccaaaaacagtgaacacacccctagctgattgaaatacaaaaaacatattccacagccaaatgaaaatgacttttggatcctccacctaatttgggtgtttatgccgcctcgcccctcttttggcctggacaattgaaatatatctgctctcaggggagacgcccacggtgtcagggctggagttggcaagagacagggggaagaggactagacctggagtcagagatgaagttcttgtctgggatctgtcactaagtctcagcggggacccaggaagtcactccacctctcatagttcctcatccacaaagtggaaatacaagcaagtttaattctccatcgtaaggttggagctcctgtctgtgaaaggactggaaatgtaaaatgcgctcttcaagtacaaaggcagagaggatccataaacaggcacaggctgccctttggtataaactgttcacattaaatctatgttatgttgctcaagagttaaaataagctcaaaggagaggctgattccaatgtcaacccagggaagacagacactgaaattccaaactgagttaccaaaaacaatagatggatgagacatgcagacatgccacaatccggcacatcagagttcgatgtagtcctgctgcaaacacatggaatccgagaagtccaatgcaaacggaatagatttcttgggatctaatatttttcaaattgcctgaccagcttaccttctaggaaaacttatttaagggaggcaaataatttggggagatgagtataagaggtagtaggaggaagctaagggaaatcaccactacatattgcaggaatgtattagaaggcaaatatggcccaaagaaaaagctccactgaaaaaaacattgaatactgaccacagaattagcaccttgctcccaggtcaataaagtgaaccaaaaaaattacaaagaccttgctcaatcctgaggttcgtgaggaatataggagagttgtgtgttcacgtgactcctgaaaacaaagagcagtactattcgaagggcatgatgtcttgatcttaggatcaaatattctagaccttgagccggagaatctgcattacagtaggaaaaatggggagtgctttatgcctgtggattcaggacacaccagcaacctacacgtgtagcattctctaagtcataatgaccattctcatctcccactgagggcaggtgtaagactcttctcttgcagtgctctgatagaaagctgggtttcttcttcttctctataaatcatagggaaaccaaatatttgtacctgttacagccccaaagctgaaagcaataaagaataaacacatacagcaagctacgaggtgcgtctgtttaggaattgcctcaacgttgggtttctattgatagaacaggggaggaggttgcctctgaccttcctgaggctcccactgtaccctggctgagtagcccacagttaattttaagtggcaaaagaaatgagaacaaattcctccaggaagagaaattagatttctgctaaaacagtgctctccatagggtatatgagcacattcgactaccactggaaaataacctgagggcaggcacatggtgcccactgttagaaatcgtgcagttagattagaatggaagagtgtctgagtttttagataattttacacgtcaggatatggctaacaggtcacgttcagggcctatgcttgatactgtcgaaatacaaacaaaaataactgcctagagagaatattcacgtcctaaaagagaaaatgttgtatctgggtggaagaatgatttaactcctgaaactcgagaacacagaacaacaacaaaaataatttccttgaacatattcaactagaatggcaaggcattttcctacataaaacattagaatgttcccattactccaaaggaatccaataaataattttacagtgaaagagcctggatcaaaactggaagtgacaccggcccccgatgaacacaagtcacaggtccctgtgcaggtcccagggctgagtcatccaagaactccaccaccaccgtgagcccggcctccggtttcatctttcccgaatgggactggctggaggggccaagctgctttacagaagagttccatctggtaagcccgggtggtgagcgaagccaaagatgacaacacgagaaggggtcaaagccaaggtttcctcacgctgcctttgtcttcttcctgcagcctggcccgatggctgaagctgggtcccaggaggcgagttcttcagcggggcctcctcacccaggctggagcaagtccgctgcacccgtcaagcggggaagagctcgggcgggctttctccatagcaatactttgctatggggtcccggtaggtgttctcatgctgcacgctctgagatgaggtcctgcatttggccaggcacaactcaaagtgatcttcgactgccatgaagaggttctggaatgccacggctgcccggttgaggaagcgctccaggagaagttgcttgttgggctgcaggcagcaggagacacagtactcataggcgctgcagcagccgttgggccagcagccatcacagcagtactgcttcgtgctagggacgttgacattacagcagccatttaccagcaaatccttcctctcgcaaacgtagcctgcttgaaggtgctgctgaggaagtagacgagcgacagcccgaagaccagggcgagcacccacctcttccgcagaagccggcgccacaccatggccgccaggttcaccatcccggcgcggacgtggggcgcggcggccggggcgcggaacgcggcaggcccgggtcccgggcggcatggcccctacgcgcccggcagccccatccctccaggcaggcgccggccccgccgcccgcagcccagtctgctcccggcagccttgggcgcagccccacgtgac

SEQ ID NO: 11750 - RNA, 6436 nt, Homo sapiens
  source 1..6436: mol_type = other RNA
ctgaatagctgggactacaggtgtgcactaccatgcctggctccttttttttattttttgtagagacagggtctccctatgttgctcaggctggtctcgaattctgggctcaagcaatcctctcaccttggcctcccaaagtgctgggattacaggtgtgagccaccacacccggctgccaacaccactttcgattttgggataatctgggtgcacagtgatcagaagcttacctaccccacgttgcataaaaaaaagtatgaatttaaaaattccaagagtaaactaccctatgaaaacctctggcagtgctgatgaaaacacatttctggtagtgatatgtcttggtccctctggtctcacagaatgtgtagtcctgagaaaaaataaacctggactcttggtaaaatatttgaataattaactgctttgctcattggttgtaactggcaagtcattctctttactacattaaagtctgcactttcattttacagacagtcctacagttcaactccaacatcagggactgagtcgtacacaggaagatcactgagtaggttctgtggagacgcagtcggcccatatgcacgtcaccactcggctcccagctcaggtgcagaccaacggcgaccacttgctccactttgctctgtgacagcagacgaggtaaggcatgttgcagatacatgctgaatatagggatgcctgtacacaaaactgcactcatgctgtgataacacgcaaaaggtcacacactggaagagccttgcccaacgaacgatagactaacaggccagaggcggggaaagcttctcggagtcccactatcttctttgtttttattgctcctacttacttatgtgatacctttttagtagaatgactagttttctaaacagaacctgtaatgacaggctcacatttcttcctcaactcccacctccaaagccactccattcaaagaactgctggtgaggtgctggggagtcaatccgtcgtagaggggaagcgttctacccctccagatccttctgcagacaggagggtgtctgcattcggcggagtccaagagtgcggtgaggacacagtggcaaaggaataatgccattccttgaggcagcgctgggctagtagagacctgtgaggaagtaatgtgtcctgtggggatttcagggtaatttaatcagcagcacttcagcagggtagaaagcaagggcggggaaaaataatgaagtcagcactcagctaccaggagctcctctgttcaatctaacggggagatatgaccccagagcagggcttccctccctccacccggctcccacttccagccaggtaattctgtgtcgtgggggctgttgggcaccatccctggcctccctccacgagtgcccacagtactgccctcctccccacctgtgacaaaaatgtctccagacattgccaaatgttccctggggggcaaaattgcccctgttgagcaccactgccctagatgaactggaaaagttggtttgtgaatatgtgagcttagttgtttctaacacagggctgaaaaacaagagaaggggacaaaggctgctttcatataaaaatgtactgtagtaatcagtaagaaaaagaaacaacattggctaagtcacgaataggcatttcaccatatgtacatgataaatggccaatcaaaataaggaatggggctcattctgctggaaattaaatacattcaaacaagaacagagatccattagcaaaatgtttaaaaataatatcacagggttaccaggggtatgacaaaaatggacacttccatacacactaggtgaatatattggtgaaaatagttcagataaacatacaaccatgtatgtaaaagtatttatcatcaatgcattatttgtagtagcaaaaacaacaagcagccttggaaaccagttaatgtcctcagcagggaattaataatattattgtatattcatgaaattgacaccatgtggccacacaaatgcattacacaggcctctatgtaacataggatattcattagagaattgtttttcaagaggacaaagtactttcatttttgcctagaaaatgggggaagacaaaaatgcgcttctctctaggttgtgtgattttaggttatcctaagtttcatccttacgtgctcctgaattatctgaaatatcgtatctttaaaaacagtaacaacaatagtaacaagagctctgtaattcctacccttccaacctcaggagcccacccacccctatccgagccgacccctgactgcccctgccattgctccctgctgagttgcagacattgacttcttgccaagcctcaggccttgctcacatcgacacctcacagtgaccctgagaggcagatgctgtgaccccatttcacagatgaagggcctgagccacagaggaggaagactgcctcagccacgccgctagtaagtggtagttcccaactctagagtcccaaaagaattctgtcctacttatgaaaagtatatccaataagcagtacctccctgtgtttacaacttatctgctgatcccaaggatgggaaaagctgcactcagaaacttgcaaattgtgcaactgttccccacgattcccttggggccagtgccgactgaggcatctccaggaggccccagttgggcttggggacatgctgagaggtgacagcactgctctcaagtcatatcctctgcttctgcaaaagctgtggagctcacccatcaatagcagctccatgccgggcgcagtggctcacgcctgtaatcccagcactttcggaggctcaggcgggcagatcatctgaggtcaggagtccgtgaccagcctggccaacatggtgaaaccccgtctctactaaaagtacaaaaacttagctgggtgtggtggtgtacgcctgtgatcccagctactcaggaggctgaggcaggagaattgcttgaacccaggagggggaggttgcagtgagctgagatcacgccattgcactccagcctgagcaacagagcaagactccatcgcaaaaaaaaaaaaaaaaaaaaaaggctctagcattgccagatcccaggccctgtggaaggtatttccctccctcttttgtccttgcttgtctcagagcccttttcacagtctcttgtgtgcttctttccctgttaggaccaatctttacaactccagcaagcgcagcaaataagatgcagaactgggggagatgcaacgtatgactcaattcccttgagccgaaaacactcacttattaacaatatttttttcttttttttgagacagagtctcacaaaaacaggcacacgcccccacacccggctaatttttgtatttttagtatagatggggtttcaccatattggtcaggctggtctgaactcctgccttcaggtgatccacctgcctcagccttccaaagtgctgggattacaggcataagccaccacgccccaccaatgaaatgttttctaaaggtgttttcatcccttttgtgatctcctaaactcccaaggtgtatcacacacttcgctgggctctgggcaaacaaaacttagacaaggtccctgattctagaaaccctcggtcgagggaaccacaaaccaaccagagtggagggcagggagaggtcctaggttgggagctgggagcctggagcacgtgccaggtgctctgcagcccagcttcattatggaggctcaagcgctgtgaatttccaaaaacagtgaacacacccctagctgattgaaatacaaaaaacatattccacagccaaatgaaaatgacttttggatcctccacctaatttgggtgtttatgccgcctcgcccctcttttggcctggacaattgaaatatatctgctctcaggggagacgcccacggtgtcagggctggagttggcaagagacagggggaagaggactagacctggagtcagagatgaagttcttgtctgggatctgtcactaagtctcagcggggacccaggaagtcactccacctctcatagttcctcatccacaaagtggaaatacaagcaagtttaattctccatcgtaaggttggagctcctgtctgtgaaaggactggaaatgtaaaatgcgctcttcaagtacaaaggcagagaggatccataaacaggcacaggctgccctttggtataaactgttcacattaaatctatgttatgttgctcaagagttaaaataagctcaaaggagaggctgattccaatgtcaacccagggaagacagacactgaaattccaaactgagttaccaaaaacaatagatggatgagacatgcagacatgccacaatccggcacatcagagttcgatgtagtcctgctgcaaacacatggaatccgagaagtccaatgcaaacggaatagatttcttgggatctaatatttttcaaattgcctgaccagcttaccttctaggaaaacttatttaagggaggcaaataatttggggagatgagtataagaggtagtaggaggaagctaagggaaatcaccactacatattgcaggaatgtattagaaggcaaatatggcccaaagaaaaagctccactgaaaaaaacattgaatactgaccacagaattagcaccttgctcccaggtcaataaagtgaaccaaaaaaattacaaagaccttgctcaatcctgaggttcgtgaggaatataggagagttgtgtgttcacgtgactcctgaaaacaaagagcagtactattcgaagggcatgatgtcttgatcttaggatcaaatattctagaccttgagccggagaatctgcattacagtaggaaaaatggggagtgctttatgcctgtggattcaggacacaccagcaacctacacgtgtagcattctctaagtcataatgaccattctcatctcccactgagggcaggtgtaagactcttctcttgcagtgctctgatagaaagctgggtttcttcttcttctctataaatcatagggaaaccaaatatttgtacctgttacagccccaaagctgaaagcaataaagaataaacacatacagcaagctacgaggtgcgtctgtttaggaattgcctcaacgttgggtttctattgatagaacaggggaggaggttgcctctgaccttcctgaggctcccactgtaccctggctgagtagcccacagttaattttaagtggcaaaagaaatgagaacaaattcctccaggaagagaaattagatttctgctaaaacagtgctctccatagggtatatgagcacattcgactaccactggaaaataacctgagggcaggcacatggtgcccactgttagaaatcgtgcagttagattagaatggaagagtgtctgagtttttagataattttacacgtcaggatatggctaacaggtcacgttcagggcctatgcttgatactgtcgaaatacaaacaaaaataactgcctagagagaatattcacgtcctaaaagagaaaatgttgtatctgggtggaagaatgatttaactcctgaaactcgagaacacagaacaacaacaaaaataatttccttgaacatattcaactagaatggcaaggcattttcctacataaaacattagaatgttcccattactccaaaggaatccaataaataattttacagtgaaagagcctggatcaaaactggaagtgacaccggcccccgatgaacacaagtcacaggtccctgtgcaggtcccagggctgagtcatccaagaactccaccaccaccgtgagcccggcctccggtttcatctttcccgaatgggactggctggaggggccaagctgctttacagaagagttccatctggtaagcccgggtggtgagcgaagccaaagatgacaacacgagaaggggtcaaagccaaggtttcctcacgctgcctttgtcttcttcctgcagcctggcccgatggctgaagctgggtcccaggaggcgagttcttcagcggggcctcctcacccaggctggagcaagtccgctgcacccgtcaagcggggaagagctcgggcgggctttctccatagcaatactttgctatggggtcccggtaggtgttctcatgctgcacgctctgcttgaaggtgctgctgaggaagtagacgagcgacagcccgaagaccagggcgagcacccacctcttccgcagaagccggcgccacaccatggccgccaggttcaccatcccggcgcggacgtggggcgcggcggccggggcgcggaacgcggcaggcccgggtcccgggcggcatggcccctacgcgcccggcagccccatccctccaggcaggcgccggccccgccgcccgcagcccagtctgctcccggcagccttgggcgcagccccacgtgac

SEQ ID NO: 11751 - RNA, 9390 nt, Homo sapiens
  source 1..9390: mol_type = other RNA
ctgaatagctgggactacaggtgtgcagcaccatgcctggctagttttttaaaatttaataattattttttttattatactttaagttctgggttacatgtgcagaacatgtagttttgttacataggtatacacatgccatggtggtttgctgcacccaccaacctgtcacctacattaggtatttctcctaatgttatccctcccttagccccccaccccccacaggccctggtgtgtgatgttaccctccctgtgtccatgtgttctcattgtttaactcccacttatgagtgagaacatgcgttgtttggttttctgatcttgtgatagtttgctgagaatgatggtttccggctttatccatgtccctgcaaaggacatgaactcatccttttttatggctgcatagtattccatggtatacatgtgccacattttcttaatccagtctatcattgacgggcatttgggttggtttcaaatctttgctattgtgaatagtgcagcaataaacatacgtgtgcatgtgtctttattgtagaatgatttataatcttttgggtatatgcccaatagtgggattgctgggtcaaatggtatttccagttctagatccttgaggagtcgtcacactgacttccacaatggtcggactaatttgcactcccaccaacagtgtaaaagcgttccaatttttccacaacctctccagcatctattgtttcctgatttttaatgatcgccattctaactggcatgagatggtatctcactgtggttttgattttcatttctctaatgactagtgatgatgagcattttttcatatgtctgttggctgcataaatgtcttcttttgagaagtatctgttcatatcctttgcccattttttgatggggttgtttgcttttttcttgtaaatttgtttaagttctttgtagattctggatattagccctttgtcagatggatatattgcaaaaatgttctcccattctgtaggttgcctgttcactctgatgatagtttattttgctgtgcagaagctctttaattagaacccatttgtcaattttggcttttgttgccattgcttttggtgttttagacatgaagtctttgcccatgcctatgtcctgaatggtattgcccaggttttcttctaggatttttatggtcctaggtcttacgtttaagtctttgttccatcttgagttgatttttgtataaggtgtaaggaaagggtccagttacagttttctgcatatggctagcccgttttcccaacaccatttattaaatagggaatcttttccccattgcttgtgtgtgtcaggtttgtcaaagatcagatggtggtagacgtgtggtgttatttctgaggcctccattctgttccattcgtctgcatatctgtttttgtaccagtgccatgctgttttggttactgtaggcttgtagtaaagtttgaagtcaggtagtgtgatgcctccagctttgttcttcttgcccaggattgtcttggctaggtgggctcttttttggttccatatgaatcttaaagtagttttttccaattctgtgaagaaagttagtggtagcttgatggggatagcattgaatctataaatcagtttgggcaacaaggccattgtcatgatattgattcttcctatccatgagcatggaatgtttttccatttgtttgtgtcctctcttatttccttgagcagtgctttgtattttattttcttagtagcaattgtgaatgggagttcactcatgatttggctctttgtctattattggtatataggaatgcttgtgatttttgcacaccgattttgtatcctgagactttgctgaagttgcttatcagcttaaggagattttgggatgagacgatggggttttctaaatatacaatcatgtcatctgcaaacagagacaatttgacttcctctcttcctatttgaatatgctttattgctttctcttgcctgattgccctggccagaacttccaatactatgttgaataggagtggtgagagagggcatccttgccttgtgctggtcttcaaaggaaatgcttccagcttttgcccattcagtatgctattggctgtgggtttgtcataaataacctcttattatattgagatacattccatcaatacctagtttattgagggtttttagcatgaaaggctgttgaattttgttgaaggccttttttgtatctattgagataatcatgtggtttttgccgttggttctgtttatgtgatggattatgtttattgatttgcatatgttgaaccagccttgcatcccagggaagaagctgacttgatcgtggtggataagctttttgatatgctgctggattcggtttgccagtattttattgaggattttcgcatcgatgttcatcagggatattggcctaaaattctctttttttgttgtgtctctgccaggctttggtatcaggatgatgttagcctcataaaatgagttagggaggattcccttttcttctattgattggaatagtttcagaaggaatggtaccagcacctctttgtacctttcgtagaatttggctgtgaatccgtctggtcctggactttttttggttggtaggctattaattattgcctcaatttcagaacctgttactggtttattcagagattcaacttcttcctggtttagtcttgggagggtgtatgtgtcgaggaatttatccatttcttctagattttctagtttatttgtgtagaggtgtttatagtattcgctgatggtagtttgtatttctgtgggatcagtggtgatatcccctttatcattttttattgcatctatttgactcttctctcttttcttcttttttagccttgctaacggtctatcaattttgttgatcttttcaaaaaactagctcctggattcactgattttttgaagggtttgttgagtctctatctccttcagttctgctctgatcttagttatttcttgccttctgctagcttttgaatttgtttggtcttgcttctctagttcttttaattgtgatgttagggtgttgattttagatcactcctgctttcacttgtgggcatttagtgctataaatttccctctacatactgctttaaacatgtcctagagattctggtacattgtgtctttgttctcgttggttccaaagaacatctttatttctgccttcatttcgttatttacccagtagtcattcaggaacaggttgttcagtttccatgcagttgtgcagttgagtgagattcttgatcctgagttctaatttgattgcattgtggtctgagacggtttgttgtgatttctgttcttttgcatttgctgaagagtgctttacttccaattatgtggtcaattttggaataagtgtgatgtggtgctgacaagaatgtatattctgttgatttggggtggagagttctgtcgatgtctattaggtctgcttggtccagagctgagttcaagtcctggatatctttgttaattttctgtcttgttgatctgtctaatattgacagtggggtgttaaagtcacccattaatattgtgtgggagtctaaatctctttgtagaacttgctttatgaatctgggtgctcctgtattgggtgcatatatatttaggatagttagctgttcttgttgaattgatccctttaccattatgtaatgaccttctttgtctcttttgatctttgttggtttaaagtctgttttatcagagactaggattgcaacccctgcttttttctgctttccatttgcttggtaaatcttcctacatccttttattctgagcctatgtgtgtctttgcacatgagatgggtctcctgaatatagctcactgatgggtcttgactgtttattcaatttgccagtctgtgtcttttaattggggcatttatcccatttacatttaaggttaatattgttatgtgggaatttgatcctgtcattatgatgctagctggttatttcatccattaattgatgcagtttcttcatagtgttgatggtctttaccatttggcatgtttttgcagtggctggtactggttgttcctgtccattttagtgcttacttcaggagctcttgtaaggcaggcctggtggtgacaaaatctctcagcatttgcttgtctgtaaaggattttatttctccttcacttaagaagcttagtttggctggatatgagattctgggttgaaaattcttttctttaagaatgttgaatattggcccccattctcttctggcttgtagggtttctgcccagaggtccgctgttaatctgatgggcttccctttgtgggtaacctgacctttctctctggctgcccttaacagtttttccttcatttcaaccttggtgaatctgacaattatgtgtcttggggttgctcttcttgaggagtatctttgtggtgttctctgtatttcctgaatttgaatgttggccttccttgctaggttggggaagctctcctggataatatcctgaagagtgttttcaaacttggttctgttctccccatcactttcaggtacaccaatcaaacatagatttggtcttttcacatagtctcatatttcttggaggctttgttcatttcttttcactcttttttctctaatcttgtcctctcgctttatttcattaatttgatcttcagttactgatatcctttcttccacttgatcgaattggctattgaagcttgtgtatgcttcacgaagttcccgtactgtggttttcagctccatcaggtcatttaagctcttctctacactggttattctagttagccatttgtctaaccttttttcaagatttttagcttccttgcgacgcattagaacatgctcctttagcttggagaagtttgttattaccgaccttctgaagcctacttctgtcaacttgtcaaactcattctctgtccagttttgttcccttgctggcaaggagttgtgttcctttggaggagaagaggcattctggtttttggaattttcagcctttctggtctggtttctccccatctttgtggttttacctacctttggtctctgatgttggtgtcctatggatggggttttggtgtagatgtcctttttttgatgttgatgctattcctttctgttagttttccttctaatagacaggccccttagctgcaggtctgttggagtttgctggaggtccactccagaccctgtttgcctgggtgtcaccagtggaggctgcagaacagcaaatattgctgcctgatccttactgtggaagcttcgttccagtggggcatctacctctctgaggtgtctttcggcgcctactgggagatgtctcccagtcaggctacacgggggtcagggacccacttgaggaggcagtctgtctattatcggagcttgaacgcggtgctgggagaaccactgctctcttcagagctgtcaggcagggacgtttaagtctggagaagctgtctgctgccttttgttcagatatgccctgcccctggaggtggaatctacagagacagtaggccttgctgagctgtggtgggctctgcccagtttgagcttccctgctgctttgtttacactgtgagcatagaaccgcctactcaagcctcagcaatggcggacacctctaccccgccaagctcccacgtcccaggtcgatttcagactgctggcgctagcagtgagcaaggctctgtgggcgtgggacccactgaaccaggcatgggaggggatttcgtggtctgccagttgcgaagactgtgggaaaagagcagtatttgggcaggagtgtacccctcctccaggtatagtcactcacggcttcccttggctaggaaagggaaatcccccgaccccttggcgcttcccaggtgaggcgatgccccaccttgcttcggctaaccctctgtgggctacacccactgtccagccagtcccagtgagacgaaccaggtactttagttgaaaatgcagaaatcacccatcttctgtgtccatcctgctgggagctgtagactggagctgttcctattcggccatcttcaatttatttttatttttattttttgtggagacagggtctcactttgttgcccaggctggtcttgaactcctgggctcaagcagtcctcctgcctctgcctccaaagtgctagaactaaaggcatgagccaccatgcccagccctcttgaatgttttatagttttcgttatacaagtcttatacttattttgttaaatttattcctaagtatttaattctctttggtgatattgtgaacacaattttctttatttcatttttggagttttctgaacagaaaaatacaattgattttctgtatattgatctagcctgtgaccttgctgaacttgattaattctattacactatgattttttgttgtggttagacccttacacaatcaaatgaggttaaaaaaaattgtcagagtggccccagaccaacaacaggatgacagtagcctttgcccatacagagataaaatttagtttttgcagtcctttcccatagagattgtatggcagtagccaattctatggcctactgccatacaacctgaactgaagtccagaaagtttaggtgactgggccacagagctaattactggtggagccaagaagagaaattatatccctacctccttgcccactaagctccccattccagtgggctgctttctggtccttttccatgattgggctttagtagctgtcatttcctccagtgtccaagagtattttcttggccttccagtaaagctccccaagttgtctgtgttccgcctcaactgctaacttgcctacctgataaacattttgaaaagcaatctaaattctagaaattgtctctcctgcaaacaaactacagattccatttaaagcatttccttgagtccagaaagttctgagattttcctgttttggactagacttccaaagggcttcatcttaaattgtatgtatttattgacctaattgtttactgatctttagaatttagagtttaggttgggaggtcaaaatcataactttctcaatttttttggcaaactgatatgatggctggaaatcatccagaaaaagtagagatcattatattttcttgaatattcattcaagtttcaatttaatacttaaacattcattttcgaataaaaatactatgtcttgtactagggatacaaagacttggttattcttgttggagtaatgattctcctctatctggggaggtcatcctctgcagttggggactgaaggactgggagatgggagattgaaacttaaagaggtaaaggtatgtcttggaataaaactagttatcagtcaccaccagaccatcatggcggctagaattccagaaacggtgaatagaagttcatcttctattttgtcttcatggaatatatcactctggtaaacagctggttctaaatatgatggttagactttcaaggtcttcattttttagatgtaattcttcaaggagggtgtctagaaaccgtgtaaacaccataccttcctgagaatgtttctgaatgccaagaattggggtcagtaatgacagcaacaccatagcaattaaagtccattccgcaggtttgtgtataatatttctatttgttaacctgaaagttcgaacaagatttttaagttgtgtgtaaatatctcccaatgtaatctgaagaggaaccagaagcccaggcaacactttactcaacttttcaagtacgatgcgttttctaatctggttctgggaacttgagtctatcagtggaaaggtggaatcatgctcttctgagtcttgtgatttggtggtttcttcacccaaaacataccgtcctctgtaaaactccctgatcctcagatttaacttttcagtttcttttttcaaattctcgtaacttggcagtggtttaatggctgtacctgagcccctaaaaggtaaagactcatccaagctgttctgagattccctccaggcagggaaatgactatctggatctgagattatgtcatcttcatcaagttcttctttaaccagagaggcttcgggtttcagacacacagaagcataattctggccatacaaaaacctcaatgtttcttctgtcttccactcaatcaaagtctccttcaaaactttaagtaagtttctctttccaacttcaggacacacctgcactgaactagacactgacctagacacttggtttgatttggcaaattttctcttaaaatgctctgcacttttcttacttatgcctactagagttatttctgacctactgtattcactttcagaattttctgacgcttttaatctttcaggcaaagtgctatttgaagaactctgagtatttactttctgtaaaggaagttcacatgtagcatctttctcctgactatctaatttgcaatcgcctaactgctcagtgacatctactactgtctgttctttgtctttgtgtttggagttagctttgtgaccagctttctttttcattatgcttttttggtgcagctgtggtctaatatttgttgaatttggtctgtttcctggtagaatggaggaaacaaagtcttgctcattgtcactgctactatcactgtgagtgctagaagaactagattcatattgcttttcaaagtggctaggattgtcgatatctgatgttttaatggctttactgcataactgtacttcttctccagaatggccactttgttcttcctttagcagttgaaaatcaggatgcctctcttcttctcgaacccatactggagttttgggaatttgtgcttcaaaaaacttagatgcttgataacaaaaattgctgcaaaaagactttctttcagtaatatcatagactttattggttttggtagaaattttatatttctgttttggtacaattcccagcttcttctgacataaaggataaccacagagtttgacaatagaacgttcatccacgacatcactgtagtgagcaggtgtaatgaacctcccacactccattaggaactcttctgtaatattctcctctaaaagctgttcaacaatatgtagagcttttctctcaaattcaatcttctttctcacagctgcttctagttcagctttccttttagaagcatcttcttgtttcaaagtacttgtctgtttagtacctgcggcttttcgagagcagcggggagccccggccttgcggccggcagaagacggcccagcgaagtccgccatgggggagagtagtct

SEQ ID NO: 11752 - RNA, 158 nt, Homo sapiens
  source 1..158: mol_type = other RNA
ctgaatagctgggactacaggtgtgcatcaccactcagctaatttttttgattctttaatagagacaaggtttttccatgttgctcagcatggtctcaaactcctgggcaataagagcaaaactccatctcaaaaaaaaagaaaaaagaaaaaaaatg

SEQ ID NO: 11753 - RNA, 2566 nt, Homo sapiens
  source 1..2566: mol_type = other RNA
ctgaatagctgggactacaggtgtgcatcatcatgtctggttaatttttatttatttattaattattattattatttttggacagagtcttgctctgttgcccaggctggagtacagtggtgtgatctcggctcactgcaagctctgcttcccgggttcatgccattctcccgcctcagcctccccagtagctgggactacaggcacccaccaccaagcctggctaattttgtttttgtatttttagtagagatgggctttcaccatgttagccgggatggtctcgatctcctgaccttgtgatccacccgccttggcctcccaaagtgctgggattacaggcataagccaccgcgcccggcctattatcatgattttttgtagagatgaggtttcactaagttgcccaggctggtcttgaactcttgggctcaagtgatccctccacctcagcctcccaaagtgctaagattacaggcataagacacctcatgtggacaagtacatgttgttttccttgcttggattgttcttttctgatctttttccccttgaaaatgtctactggctgttaaatgtctttggaaactctcaagtaatattgtggctacagttcccctagcactttgtttatttattttttattttttttatttttttgagatggagtttcgctcttgttgcccaggctggagtgtgatggtgtgatctcagcttactgcaacctctgcctcccgggttcaagtgattctcctgcctcagccttccgagtagctgggattacaggcatgcgccaccatgcctggcctatttttctttgtatttttagtagagactgagtttctccatgttggtcaggctggtcttgaactcccgacctcaggtcatctgcctgccttggcctcccaaagtgctgggattacaggtgtgagccaccacgcctggcctgtttatattttttaataagtattttgggttatgcctccaggaaggtgactacatttaatctttttgcagcaatctgaatcccagtactttcagacatatagtgtatgctctataaaaatttgtggaatgaataattgaaagtgagtagggaaagacttgagtggattttgtcttagagcagtatcatccacgtggtccccaacatatatgatggaataacttcttttaggactcgatggtggccataggtatctctttgttttgggcatgaacaagctcctttcccattttgagaaagtgaaatttaatgtctatctttaaatatgggtactatcttacccttattgaattaaaatcctttctgattgtcctagccgtctcttcagtttcctcatggccaacttcatttcctgattcctcagcgtgtaaattataggattgagcaaaggggagatgacagtgaaggtgacagagatggcagtgtctgtggggagggcagtgaagggccgggcatagacatagatgcagggcacgaaatgcagggtcaccacggtgatgtgggaggtgcaggtggagatggctttcctcctgccttccccagtgtgagacctcagcatcatcaagatgaccgtgtaagatatgaggagaaagaagaatacaaaccaactgactaacccattatttgaaatcatcaggagctccagagtgaaggtgtcagtgcaggcaagtttgaggacctgggggacatcgcagtagaaagtgtcaagaacattgggtccacagaaagggagtgggagcaatagagaaatctgcgctatggagtggacaaagccccccacccaggaagccacgatgaggcctgtgcatcgccccctactcatgatggtcatatagtgcaggggcttggagatggctatatagcggtcaaacgccatcacagagagagaaaaaacgtctgctccccccagaaggtggaagaagaacatttgagtgacacagccactgaaggagatggtttttgtctctgatagaagatctatcaggaccttaggagctgtgatggaggaaaagcagatgtcaagaatagacaggttgcggagcaggaagtacatgggcgtatgaaggtgagattcacaggtaactgtaaccatgatgaggaagtttcccattagagttgtcatgtacaccaaaaacaggaaggtaaataagacctggctcagttctcgggactgagtaattcccaggaaggtaaattctttcactctggtgtaatttctctgatccattgaatcacagatcctttatcaggttcatcttgtgtctgcaagtcagtatgccaccactggatgaaagattacccaggtttttgattcagtcatcccaggagacaaagttctctcactgctgctgctcttttctttgcttcttaagagtcttgacttccataggaacattctacacatttgcagcatttctcaaaattcagcacaaacagcttttcagtttcagaagttcataggcactaatactaactgctggtttaatctttaagtgggaaattgatcctcttatgatgcctcagctgcattttagaagaagtaggtactggggaaattct

SEQ ID NO: 11754 - RNA, 1207 nt, Homo sapiens
  source 1..1207: mol_type = other RNA
ctgaatagctgggactacaggtgtgccaccatgccctgctgcatacagaagtcttaattaaaaaaaatacattggtagaataatattaaagtattactaagcttgatttttctatacattttgaatttaaaaactttattaatgcatccccgagttaatgaatatttttctgttgattcaatttactgattactttgaaaagttctgactttgagtagccaacatatcacatatcataatcagaatattttcctagaagcaaaaaagcaaaatagattttccattgcaagtagaaaaaaataacgatgttctaattttcaagatttcaagttccttttcatattaaactagatatcagtgttaatgaaaatagaaggaacactgaagtaattccaaagcatgtggctttgtaatacatagcagtcccttggtatccataggggattggttccaggacctcccgtggataccgaaatctgcgaatgctcaagtctctcatataaaatagtgtagtatttgcaaataacctatgtgtatcctcccatatactttaagtcatttctagattacttataatatctaatataatgtaagtgctatgtaagtagttgttatcctgtgttgttcagggaataatgacaagaaagagaagtttgttcatgtgtagtacagatgtatttttttcccctaatattttcagtctgaggttggttgaatccatggatgtaaaacccatggatatgaaggactgactgtattttctaatgttaaaatatattgactgtcttaactacatctaccataagtcatttttcatatcagtttgtattcctggagcacacattaactgatgttgtaggggagtggtccagcagcatgcatcataaggaaaaatcactagggcattgaaaactcttccatgtatcatccctttctacggggtgctgtccaaagaaatctggatgtactgcaaaatagaaaggcctcaaggcattgactgcttcagctcccgataaagctcttgaaaagggaaaccagtgtggaaatatcttctctagacataacctcctcataggtctcaggtggcaaaacatttctgaatatatatgtacgtcaacttcgaggcatccattaattgagttctggcaagggtccgacgcgagggctttgtccgactagttccacctcccacccagtacaccagaag

SEQ ID NO: 11755 - RNA, 1521 nt, Homo sapiens
  source 1..1521: mol_type = other RNA
ctgaatagctgggactacaggtgtgccaccatgccctgctgcatacagaagtcttaattaaaaaaaatacattggtagaataatattaaagtattactaagcttgatttttctatacattttgaatttaaaaactttattaatgcatccccgagttaatgaatatttttctgttgattcaatttactgattactttgaaaagttctgactttgagtagccaacatatcacatatcataatcagaatattttcctagaagcaaaaaagcaaaatagattttccattgcaagtagaaaaaaataacgatgttctaattttcaagatttcaagttccttttcatattaaactagatatcagtgttaatgaaaatagaaggaacactgaagtaattccaaagcatgtggctttgtaatacatagcagtcccttggtatccataggggattggttccaggacctcccgtggataccgaaatctgcgaatgctcaagtctctcatataaaatagtgtagtatttgcaaataacctatgtgtatcctcccatatactttaagtcatttctagattacttataatatctaatataatgtaagtgctatgtaagtagttgttatcctgtgttgttcagggaataatgacaagaaagagaagtttgttcatgtgtagtacagatgtatttttttcccctaatattttcagtctgaggttggttgaatccatggatgtaaaacccatggatatgaaggactgactgtattttctaatgttaaaatatattgactgtcttaactacatctaccataagtcatttttcatatcagtttgtattcctggagcacacattaactgatgttgtaggggagtggtccagcagcatgcatcataaggaaaaatcactagggcattgaaaactcttccatgtatcatccctttctacggggtgctgtccaaagaaatctggatgtactgcaaaatagaaaggcctcaaggcattgactgcttcagctcccgataaagctcttgaaaagggaaaccagtgtggaaatatcttctctagacataacctcctcataggtctcaggtggcaaaacatttctgaatatatatgtacgtcaacttcgaggcatccattaattgagttctggcaagggtccgacgcgagggctttgtccgactagttccacctcccacccagtacaccagaagggaggacagtcgctccgcccgcagggctgttcggacgcgcatgcgcactggggcgtcagctggccaaccagcgcgcgacgcacggccaggcgctcccacctgccctcgccccggtgggcgacaggctttgacgggctcctagccgcagtgccctctgagcccccaaccctgaattctcagctgggccctcccggctccacctgcccccaacaccctccccgctccggcggcggcagggcgctcgaggcaagcccgggcagggggacgagctgcaggtgacgccctggttggctggagcgtgccaggccttcccc

SEQ ID NO: 11756 - RNA, 1329 nt, Homo sapiens
  source 1..1329: mol_type = other RNA
ctgaatagctgggactacaggtgtgccaccatgccctgctgcatacagaagtcttaattaaaaaaaatacattggtagaataatattaaagtattactaagcttgatttttctatacattttgaatttaaaaactttattaatgcatccccgagttaatgaatatttttctgttgattcaatttactgattactttgaaaagttctgactttgagtagccaacatatcacatatcataatcagaatattttcctagaagcaaaaaagcaaaatagattttccattgcaagtagaaaaaaataacgatgttctaattttcaagatttcaagttccttttcatattaaactagatatcagtgttaatgaaaatagaaggaacactgaagtaattccaaagcatgtggctttgtaatacatagcagtcccttggtatccataggggattggttccaggacctcccgtggataccgaaatctgcgaatgctcaagtctctcatataaaatagtgtagtatttgcaaataacctatgtgtatcctcccatatactttaagtcatttctagattacttataatatctaatataatgtaagtgctatgtaagtagttgttatcctgtgttgttcagggaataatgacaagaaagagaagtttgttcatgtgtagtacagatgtatttttttcccctaatattttcagtctgaggttggttgaatccatggatgtaaaacccatggatatgaaggactgactgtattttctaatgttaaaatatattgactgtcttaactacatctaccataagtcatttttcatatcagtttgtattcctggagcacacattaactgatgttgtaggggagtggtccagcagcatgcatcataaggaaaaatcactagggcattgaaaactcttccatgtatcatccctttctacggggtgctgtccaaagaaatctggatgtactgcaaaatagaaaggcctcaaggcattgactgcttcagctcccgataaagctcttgaaaagggaaaccagtgtggaaatatcttctctagacataacctcctcataggtctcaggtggcaaaacatttctgaatatatatgtacgtcaacttcgaggcatccattaattgcggccgccctgaggggtctcggcgcgctcggctgagagctttaggaggcgcgagcgagcactccgactaggccggagggactcggaaaatgatggtccggcaggtggtgggtcctgacccaagggcctgcaaggaacggagaagggcaaccgagcacgcgctggatcttggggaagaaggggaaagggact

SEQ ID NO: 11757 - RNA, 1993 nt, Homo sapiens
  source 1..1993: mol_type = other RNA
ctgaatagctgggactacaggtgtgccaccatgccctgctgcatacagaagtcttaattaaaaaaaatacattggtagaataatattaaagtattactaagcttgatttttctatacattttgaatttaaaaactttattaatgcatccccgagttaatgaatatttttctgttgattcaatttactgattactttgaaaagttctgactttgagtagccaacatatcacatatcataatcagaatattttcctagaagcaaaaaagcaaaatagattttccattgcaagtagaaaaaaataacgatgttctaattttcaagatttcaagttccttttcatattaaactagatatcagtgttaatgaaaatagaaggaacactgaagtaattccaaagcatgtggctttgtaatacatagcagtcccttggtatccataggggattggttccaggacctcccgtggataccgaaatctgcgaatgctcaagtctctcatataaaatagtgtagtatttgcaaataacctatgtgtatcctcccatatactttaagtcatttctagattacttataatatctaatataatgtaagtgctatgtaagtagttgttatcctgtgttgttcagggaataatgacaagaaagagaagtttgttcatgtgtagtacagatgtatttttttcccctaatattttcagtctgaggttggttgaatccatggatgtaaaacccatggatatgaaggactgactgtattttctaatgttaaaatatattgactgtcttaactacatctaccataagtcatttttcatatcagtttgtattcctggagcacacattaactgatgttgtaggggagtggtccagcagcatgcatcataaggaaaaatcactagggcattgaaaactcttccatgtatcatccctttctacggggtgctgtccaaagaaatctggatgtactgcaaaatagaaaggcctcaaggcattgactgcttcagctcccgataaagctcttgaaaagggaaaccagtgtggaaatatcttctctagacataacctcctcataggtctcaggtggcaaaacatttctgaatatatatgtacgtcaacttcgaggcatccattaattgcggccgccctgaggggtctcggcgcgctcggctgagagctttaggaggcgcgagcgagcactccgactaggccggagggactcggaaaatgatggtccggcaggtggtgggtcctgacccaagggcctgcaaggaacggagaagggcaaccgagcacgcgctggatcttggggaagaaggggaaagggactgctggaggaggcgcgcatgcgccgtgcggtccttcgccccgggcgccctggcagggggcgaggctctgcggaactcccggagctggcgccagggaacaagtctcagtggagagcctcgaattttaaaagtctcatttaagtatttcttttggttttccttgtataaatatagctaacttttaaacatttcttttccggcttgtgttgtttgctttggacccttcagcacctatttttaaacgttaagcattccccagtcagcatgaaagttttactgttagttttattttgttcctataattttgattccccccagaaactgccacagatgaaatcaagccaatagaattgaaagcaaagatcacctggtggccatgaagccgaccatccttaggcagaaactccttacctgaggaatttagaggtaactagacttccctgttacctaaagccagcatctggtaccagacttcttccctccaaatttaaaagtaactagaatttctatgcatctccgtaatgcacgcatgtcaaaactcattgtgcaccccttgccatctgctccatgccccaatcaacccctgtcccctaccatccagatactttattaccctcacatacttgcacaggagttacatatgccactagtacaaagtcctcagaa

SEQ ID NO: 11758 - RNA, 6660 nt, Homo sapiens
  source 1..6660: mol_type = other RNA
ctgaatagctgggactacaggtgtgcgcacatgccaggctaatttttgtatttttagtagagacggggtttcaccatgttggccgggatggtctcgatctcttgacctcatgatctacccgccttggcctcccaaagtgctgagattacaggcgtgagccaccgtgcctggccaggccccttctcttttaatggagacagggtcttgcactatcacccaggctggagtgcagtggcataatcatacctcattgcagcctcagactcctgggttcaagcaatcctcctgcctcagcctcccaagtagctgagactacaggcacgagccaccacacccagctaatttttaagttttcttgtagagacagggtctcactatgttgtctaggctggtcttgaactcttggcctcaagtaatcctcctgcctcagcctcccaaagtgttgggattgcagatatgagccactggcctggccttcagcagttctttttgtgaagtaaaacttgtatgttggaaagagtagattttattggtctacccttttctcactgtagctgctggcagccctgtgccatatctggactctagttgtcagtatctgagttggacactattcctgctccctcttgtttcttacatatcagacttcttacttgaatgaaacctgatctttcctaatcctcacttttttcttttttaaaaagcagtttctccactgctaaatgttagtcattgaggtggggccaattttaatcataagccttaataagatttttctaagaaatgtgaaatagaacaattttcatctaattccatttacttttagatgaatggcattgtgaatgccattcttttaatgaatttcaagagaattctctggttttctgtgtaattccagatgagtcactgtaactctagaagattaaccttccagccaacctattttcctttcccttgtctctctcatcctcttttccttccttctttcctttctcttcttttatctccaaggttaatcaggaaaaatagcttttgacaggggaaaaaactcaataactagctatttttgacctcctgatcaggaactttagttgaagcgtaaatctaaagaaacattttctctgaaatatattattaagggcaatggagataaattaatagtagatgtggttcccagaaaatataatcaaaattcaaagattttttttgtttctgtaactggaactaaatcaaatgattactagtgttaatagtagataacttgtttttattgttggtgcatattagtataactgtggggtaggtcggggagagggtaagggaatagatcactcagatgtattttagataagctatttagcctttgatggaatcataaatacagtgaatacaatcctttgcattgttaaggaggttttttgtttttaaatggtgggtcaaggagctagtttacaggcttactgtgatttaagcaaatgtgaaaagtgaaaccttaattttatcaaaagaaatttctgtaaatggtatgtctccttagaatacccaaatcataattttatttgtacacactgttaggggctcatctcatgtaggcagagtataaagtattaccttttggaattaaaagccactgactgttataaagtataacaacacacatcaggttttaaaaagccttgaatggcccttgtcttaaaaagaaattaggagccaggtgcggtggcacgtgcctgtaatcccagctccttgggaggctaagacaggaggattccttgagccctggagtttgagtccagcctgggtgacatagcaagaccctgtcttaaaagaaaaatgggaagaaagacaaggtaacatgaagaaagaagagatacctagtatgatggagctgcaaatttcatggcagttcatgcagtcggtcaagaggaggattttgttttgtagtttgcagatgagcatttctaaagcattttcccttgctgtatttttttgtattataaattacattggacttcatatatataatttttttttacattatatgtctcttgtatgttttgaaactcttgtatttatgatatagcttatatgatttttttgccttggtatacattttaaaatatgaatttaaaaaatttttgtaaaaataaaattcacaaaattgttttgaaaaacatttttggattgtttcattctttgcttgtcatttatctgttgattagaccactaaagtgaaggattcaagctaaatacatcaacctttctatttaggctttatcagctatatgtaaattcaattctatcaaaattttctgagtgcctcctcagtgtgtctctctgatggttcctgcccggtatggctggcatgaagaagatccacggacttgcgaatgctaacgcggggcttggggatgggtttggagggtttgttttcaaagctttctggaagtgtggaggagtgtcccccttttcttgcttgtagtgctagctggtaagcgacttcgaatgcctgtcccagggttaggatgatttcataggctaaattcacatcaaaggcagtaaacacatgacagtagtggtgattagacttcaaatcttttgtgatataggcaaatgttgagaggtcttctgggtcctgggcagcacaggagatattacgaatttcatgctcagcaattatgttcttatttgttgcatcaataaatttgactcctttatatgagacagaaagaataatagtagggaccttcttcatttgctctgtagacttctgacagttagcccgcatttttgcacaagcatcttgggttgattctgtccccctaagctcttttatcagcatagaacctaaataaaaagctttgtaatcacacgactggaagataagcttttctgggtgatgctgccagtactgtaccggggtagaggctgtggcttcattcggaggtcgcaaggtaatggaaggttctccccagtctcctgtattatgaacctgatggatcgctgagaaaggaaatcctgcgttctgattcgtccatatttcacagacagacgactgctgagccatctgcctctccagttttgatcggggaatatcatcaaagtagttttcatttcttctcctccttgcatcgccctgcatgataatgtgaggaacgtctagggagccaccagtggtgtaagtgctttggctaagtgatggagacaactgaggaggagtgtgattaccactgggttccctgagggtgatggaccgagggggcttctgtgggggatcgtcgtgcagcctgtctcccagagatgccaaaatacgtttcctgtggccaatcaaattgatttttaaaacattaataagttcaacctcccagatttttttcaacaggtccatcgaagtgtagccattaattagaaaggctttggtgtagtcgcccagttcaatggaatccagccactcagctacagaggtgggatggtagccatcatgcccaatgggtctcatctttggaaggagctggattgcctgtagaattctttgtctgtgcccagaattaaggattccaatttccaacaaatcctgatcttccataacattgcttcccataaactgcacattgtcaaatccattagccatcaggtggttctcgtactgaggtagcccaatgctttccaaccattgtcccactgtttggacagggcatctgggtcttgtggtctcaccattcatctctttaagttcgttgttgattccaacatctatggaactcattattttgtcaatttcttcccattccgatgtgaaggatggtgttctttcagaattccctttagaactgtgttcagcagtggaagattcactccagttaactcttgatgttttctcattggaaggataggcaatgagatcagaatcagatttagagacactttttgacaaatgcatgtcgatcaaggctttaggcaatgaccttattctccccagagtacaggctctctccacaaatccccctgcgttcataacccactggtccccattccgagatccactcctggttgatcttgtgccaacaatggtatggttttcgagttggttgctttttttgtgaaaaattgttctactgaccactttgggtttaattttctttaccaaaggttctgagttattttctattggagactgcttgaaaggcaaaggactgtttgccaaactgacttcatcttgtcctttttcacattgttctcttttcccatagagatgaaatggattttcaggggactcacaggctggagaggatccatggagcaggcctgcaaattgcccaggatcatattcttttgggggatcattgtcatcctgtcgggagaggtcatctgtatggttagttccctcattcttgacttctgtggttcccacagaagaggtgggtggactagcaggaggactggcagtaaagcttgtgcaccctgtagatgtgttgatttcaaaatattcttggttgtgattcattcggtgaaaatccagagaagacacaatggatgttcgctgtttaggctggggtcgaatgacttttacaatatttttgagggcagtatcaggggatggaggtgaacaatcaggtgttgggcctgttgagctgtttctatggttactagttcctggagtagtaactgctacctcagaggcattatcagttcttggggaaggtgcccttgcaatttctaaggagcaaggtttctttgtaacagctgtgtccatgagatcacacagaaagttctcattttctgaaggaaatgtatccagagaagcagatggtacaatttccatagtgtaatttctcttctttggataggactcctgggcaagcatggggaagccaaggttcctacatccattacacggagttaatgcttcccaaagtcctgatggcccacacgtattttcatcatcatcctcttcttccacttctcctggtgacaaattgattgtagatgaggttcttacactctggcttccatttttcccaagttcttcctctgaaatcttgctcaaattatctaagtagtggtctgatattgtgtggcacaagtcttcaaacgaataatccttttcttgacagagttttatttcatccaagagttttgataattctccagtgacggtttcacttttggtcttttgggaaggagactcaacaggagatgaaatgtgtgtttcttgtgttgcatcttcctgtacaggctcttcgaggactgtagatcttcccacgccttctaaatactcttgtaagagtgttgcaatctggagagatttctgagatggatgttctttcagaatgtccaagacagttctacctaagctatcctttatgttggcatcaattcctgtttctaacagaactcgtacaacatccacctttccaaacaaagctgcttcatgaagtgcactccccttttctgtttgacagctcacatccattcctgcctccagcagcacctgcacgactgctttgtggccattgcgcgcagcaaggtgaagtggcgtgtgcttgcgagtgttgcagctcattaagttaggatgtgcactgatgatcatttttaccactctaagccgtccgtagagtgccgccaagtccaaaggtgtttccagcttgctatttctaattgtcgggtcagtgagctcttctaggagaacagcaactacttctgagtgtccatattgagctgcacagtgtagggcagtttcattttcattgttctgttcattgaccctggaatgtgatggtccatgatgaataagaatcttcacaatttccacatctcctttccaggcagccaggtgaataggaaaataccctttgttgtctgctacatttgttgatgcctcatactgaagtagtttgagaactatgtccttatgtccatttaaggctgcgtggtgtaaagcagtgtaacccgaactgtctgtgcagttcacattggggcctcgccagatgcttagcagattagacaggggcaggggtccggatccaccgcccaggatccctcctttcctgccagacaggagtttctccaccagagccacatttccagtgcgagcagcttccagcagctcctggtccttccccatagtctctcaccgactcccccacagagtccttgcccccctcgggtcctcctccccacccacccccactccccaaaatccagggccctcttcgccccaccctaaaataatgcaagagcttcagcacggagagctccctgcagccccaggcagggagcacgactctctcctcctcttcggggcgcagcttttacaatggggatcagaccatgtcttgaaagaggggctggccgagctgggagccgcgacgcgcccccacagccactcccctgaattcccaaggcctcgttcccgcgggtgcggcgtgagggggtggggactcgggggtgcttttgaggagcgggaggagggtggtgaggactgaggtcggaggaggaggaggaggcggcagagagagtcctagctggagcgggagcgcagggaacacccgcggtggcagcagcggcccgcgcgccctcgcgcccgacccgggctcgcctcggcttcctcggcggttacgcgggggcggcgtccgcggcggggaggagcgcggcggcggc

SEQ ID NO: 11759 - RNA, 1854 nt, Homo sapiens
  source 1..1854: mol_type = other RNA
ctgaatagctgggactacaggtgtgcgccaccacacctggctaatttttgtatttttagtagagacagggtttcaccatgctggccaggctggtctcgaactcccaacctcaggcgatccatctgcctcagcctcccaaagtgctgggattaaaggcgtgagccactgtgcccagccttttttttttttttttttttccgagacaagagtctcactctgttgcccaggctggagcacagcggtgcaatcttggctcactacaacctccacctcctgggtttaggcgattctcctgcctcagcctcccaaatagctgggattacaggcacatgccaccacacctggctaatttttgtatttttagtagcgacggggtttcgccatgttggccaggctggtctcgaactcctgacctcaggcgatccacttcccgacctcaggtgatccgcctgcctcggcctctaaaagtgctgcaattacaggcataagccactgtgcctggccctatcccttttaattttctaagtgaccagtaataaacaatgatttgtttattactaggtagcaggagaaaaactttttagtcacttttccagctaagaatttcatttaaagatacctatgacatatcttgtggtactaagaatattagagaactggaaatccagtttttttgtggttttttaagaaagagaatctgactccattgcccagcttggagagcagtggtgcaatagctggggctacaggcgtgagccaccacaccaggcctggaaacccagttttaatttgtgaactacaaatggttggcaactgattccttaattgttattgcaggagtaggcccaacatgagtccatatgtagcccttctctggtctggtgggaactgtgggaaatggtgatgaccgtgacttgaaatactcagaaggtgcatgacaaacaaattccaagtattccatcttccttggaagatcttcctctggccctatgatataggaggcgggatcaaattggtctctggggctagagagggtaggaatgagccacgtcagtgctgcactcttctcgcaatactggtcctggataaaacctctgatttgagcatagtagggctttccatcttgttcatcaatcacagaaacaacatcaccaatttggtaatatactcccttgtagaagattgattctgcagtgattatagtggaaactgactcaggagctttgatgggatttttcaatttaaatatatgtcttctcccttttcctttggtggagactttcttttcagcagccggagcagatttgtatttagtgtttctgagccgagcagacctcctgtgaatttcctgcttactctgcttgccgcccccgcccccgttgctctgcggaggggtggcggaggtgctggcgaaggtcgccgcgccgaagccgccgccgccgctgcccccagtccctccagccgcccccgagcctgcgcccccgctgcccgcgccgccccggccagtgcaatgatggcagaggatctccccctgcgctcccttcttccacatggaggacgacgtggtcttgcatacgctgcaggtgggcttcaggcccagcggcatggtggccggctcgggcggcccccgcgggcgcagagacacgggaatggcggacggtagcccggccgccccctggtcggcccgccactcccggcgataggaagagcggtgagagcgtcggcacggagctgccggtgaaaggaccaggccgctggcgctgccccgtggaggcgggaagcgggttccgccggctccgcaggcggaggccaggattccctggcccgaggcactgggaagcaggactgggaaag

SEQ ID NO: 11760 - RNA, 1888 nt, Homo sapiens
  source 1..1888: mol_type = other RNA
ctgaatagctgggactacaggtgtgcgccaccacacctggctaatttttgtatttttagtagagacagggtttcaccatgctggccaggctggtctcgaactcccaacctcaggcgatccatctgcctcagcctcccaaagtgctgggattaaaggcgtgagccactgtgcccagccttttttttttttttttttttccgagacaagagtctcactctgttgcccaggctggagcacagcggtgcaatcttggctcactacaacctccacctcctgggtttaggcgattctcctgcctcagcctcccaaatagctgggattacaggcacatgccaccacacctggctaatttttgtatttttagtagcgacggggtttcgccatgttggccaggctggtctcgaactcctgacctcaggcgatccacttcccgacctcaggtgatccgcctgcctcggcctctaaaagtgctgcaattacaggcataagccactgtgcctggccctatcccttttaattttctaagtgaccagtaataaacaatgatttgtttattactaggtagcaggagaaaaactttttagtcacttttccagctaagaatttcatttaaagatacctatgacatatcttgtggtactaagaatattagagaactggaaatccagtttttttgtggttttttaagaaagagaatctgactccattgcccagcttggagagcagtggtgcaatagctggggctacaggcgtgagccaccacaccaggcctggaaacccagttttaatttgtgaactacaaatggttggcaactgattccttaattgttattgcaggagtaggcccaacatgagtccatatgtagcccttctctggtctggtgggaactgtgggaaatggtgatgaccgtgacttgaaatactcagaaggtgcatgacaaacaaattccaagtattccatcttccttggaagatcttcctctggccctatgatataggaggcgggatcaaattggtctctggggctagagagggtaggaatgagccacgtcagtgctgcactcttctcgcaatactggtcctggataaaacctctgatttgagcatagtagggctttccatcttgttcatcaatcacagaaacaacatcaccaatttggtaatatactcccttgtagaagattgattctgcagtgattatagtggaaactgactcaggagctttgatgggatttttcaatttaaatatatgtcttctcccttttcctttggtggagactttcttttcagcagccggagcagatttgtatttagtgtttctgagccgagcagacctcctgtgaatttcctgcttactctgcttgccgcccccgcccccgttgctctgcggaggggtggcggaggtgctggcgaaggtcgccgcgccgaagccgccgccgccgctgcccccagtccctccagccgcccccgagcctgcgcccccgctgcccgcgccgccccggccagtgcaatgatggcagaggatctccccctgcgctcccttcttccacatggaggacgacgtggtcttgcatacgctgcaggtgggcttcaggcccagcggcatggtggccggctcgggcggcccccgcgggcgcagagacacgggaatggcggacggtagcccggccgccccctggtcggcccgccactcccggcgataggaagagcggtgagagcgtcggcacggagctgccggtgaaaggaccaggccgctggcgctgccccgtggaggcgggaagcgggttccgccggctccgcaggcggaggccaggattccctggcccgaggcactgggaagcaggactgggaaagggatctggccggggtgggggggacgcggagactt

SEQ ID NO: 11761 - RNA, 3463 nt, Homo sapiens
  source 1..3463: mol_type = other RNA
ctgaatagctgggactacaggtgtgcgccaccacacctggctaatttttgtatttttagtagagacagggtttcaccatgctggccaggctggtctcgaactcccaacctcaggcgatccatctgcctcagcctcccaaagtgctgggattaaaggcgtgagccactgtgcccagccttttttttttttttttttttccgagacaagagtctcactctgttgcccaggctggagcacagcggtgcaatcttggctcactacaacctccacctcctgggtttaggcgattctcctgcctcagcctcccaaatagctgggattacaggcacatgccaccacacctggctaatttttgtatttttagtagcgacggggtttcgccatgttggccaggctggtctcgaactcctgacctcaggcgatccacttcccgacctcaggtgatccgcctgcctcggcctctaaaagtgctgcaattacaggcataagccactgtgcctggccctatcccttttaattttctaagtgaccagtaataaacaatgatttgtttattactaggtagcaggagaaaaactttttagtcacttttccagctaagaatttcatttaaagatacctatgacatatcttgtggtactaagaatattagagaactggaaatccagtttttttgtggttttttaagaaagagaatctgactccattgcccagcttggagagcagtggtgcaatagctggggctacaggcgtgagccaccacaccaggcctggaaacccagttttaatttgtgaactacaaatggttggcaactgattccttaattgttattgcaggagtaggcccaacatgagtccatatgtagcccttctctggtctggtgggaactgtgggaaatggtgatgaccgtgacttgaaatactcagaaggtgcatgacaaacaaattccaagtattccatcttccttggaagatcttcctctggccctatgatataggaggcgggatcaaattggtctctggggctagagagggtaggaatgagccacgtcagtgctgcactcttctcgcaatactggtcctggataaaacctctgatttgagcatagtagggctttccatcttgttcatcaatcacagaaacaacatcaccaatttggtaatatactcccttgtagaagattgattctgcagtgattatagtggaaactgactcaggagctttgatgggctatgaaaatacaaaaaacattagcacattcatagtatgtatgtgtctacaggcattttcccagccctatgagagttctgcaatttgagaagtactaaaatgtattgtttggtgacaagaactgcaataaaaagataaatgattttctgaatgttgtggcaaagcagtctatttccactgcaatttctgctactattagcttaaaaattgctgagacaaaggacaaccttctgattatgctgctgagatctaatgcaaagtcctctcagagcttcactacacataaacattccagttataaaaatgtacctgctctaatagcctgagcatgacagaatgcaagtaacagaaaatgtacagatgaatacaaagtgaaaaagtgtctcctcaaagacatttcccaactcaactatggaactagccataatactcaacataggttttctagcaagctgaaactaaggctttagaaactttgagagttcttagtaatttgctaccatccaaccatttttgagatctctactaaagcttcaatacatacttttatgccacaacatagaaagtaggcctccccagatgtgtcttgcttagtaccattgaagaaaggttgcagagaaacgataatgaaataattgctgagaacacggtataccatacttaaaaggaaaaaaatgtgcatatgtgatacaaatatcaataacatgttttgtgtaatcaacaaatgcctcacttaactataaaaatcttaaataaattagaagcaactagtctgaataagaaaatactttggggaagggaacatcacacactggggcctgtcggagatgggggccaaggggagggagagcattaggacaaatatctaatgcatgcggggcttaaaacctagatgatgggttgataggtgcagcaaaccaccatggcacgtatacctatgtaacaaacctgcacattctgcacatgtatcccagaacttaaagtaaaattaaaaaaaattcattaaattaaattaaaaaaaaaaaaagaaaatagtctgccatctgcataagtctactgcagggtccctttgtgttttagaaataaatatggccaacttcagaaacgtctttacgggtaagtgaaacattcctgttctgaaagaaaagaatatcatactgagacttaaaaaaatagtccataatgcactgtccactgtgtttgaacattatcccttgtttataaaaactgagaatttaattgcaataaaaatatgctttcaactacttccagcacaggtctttcaacaatctcttttcttagagcagaagaggagataaggcttagcaaaatttttgactcatattcatcaaatacatcatcatcataagtcagtaagatacattttctggggctttaataacaaataaatatgcaaatgatgagttctagtgttaatatttacttagatttttaaagaatgaaaaaaaaaagttttcttagtgtacctggccatatcaagaaccataatctctcctcttcctttccatagagaaccccaaaaaatgggctcaaggttgatgtttcttttaaacccatattttatattttccaggggaaaaaataaaagatttttcaatttaaatatatgtcttctcccttttcctttggtggagactttcttttcagcagccggagcagatttgtatttagtgtttctgagccgagcagacctcctgtgaatttcctgcttactctgcttgccgcccccgcccccgttgctctgcggaggggtggcggaggtgctggcgaaggtcgccgcgccgaagccgccgccgccgctgcccccagtccctccagccgcccccgagcctgcgcccccgctgcccgcgccgccccggccagtgcaatgatggcagaggatctccccctgcgctcccttcttccacatggaggacgacgtggtcttgcatacgctgcaggtgggcttcaggcccagcggcatggtggccggctcgggcggcccccgcgggcgcagagacacgggaatggcggacggtagcccggccgccccctggtcggcccgccactcccggcgataggaagagcggtgagagcgtcggcacggagctgccggtgaaaggaccaggccgctggcgctgccccgtggaggcgggaagcgggttccgccggctccgcaggcggaggccaggattccctggcccgaggcactgggaagcaggactgggaaag

SEQ ID NO: 11762 - RNA, 2176 nt, Homo sapiens
  source 1..2176: mol_type = other RNA
ctgaatagctgggactacaggtgtgcgccaccacacctggctaattttttgtgtttagtagagatggggttttaccatgtaagtcaggctggtctcgaactcctgacctcaggtgctccacctgccccagcctcccaaagtgctgggattacaggcgtgagccactgtgcccggccgggacttcttaaaagaaaactggagaccgggcgtggtggctcacgcctgtaattccagcactttgggagtctaaggcgggcggatcatgaggtcaggagatcgagaccatcctggctaacgcggtgaaactccatctctattaaaaatacaaaaaattagccgggcatagtggtgggcacctgtaatcccagctacttgggaggctgaagcaggagaatggcgtgaacccaggaggtggagcttgcagtgagaggagattgtgccactgcactccggcctgggagacagagcaagactgtctcaaaaaagaaaaaaaaaaaaagaaaaaaaaaaaaaaagaaaactggagagtccccatcccatttggtttctggacaagggagaacgctgccacagtgggtactggggacctcaaccacagctggaggtggggacctgggtcccaggattggggtgatgggaagacaggacacaggtgggctgtgaggcctgcacctgtggacccaggtggtcctcccaagatgtgatcaatccatgactgctgggctcgagcccactatgctttggatggacaagggatgggaacacagcataggctggctcatggcgccttctttattgtccaccccagccccccttccctgcagccccctccaaatgacaaaactacccacatcccatggcccacccccaaagcggcgggattcagagctgcgagaacactggaagctccccctctgacagcagcggcgacaccttgggtgcaagcggggccggatccgcgggggcgtcggggcgcggcggcccggccgcgggggccgcgggggcgccggggcggtggtcctccaggtgcagggtcatggcgggccgcgaggccgtggagaaggcgcactgcatgcacgagtagcggccgcgtgtgtgctcccacacgatgcggctcggggccgcgtgccctgagggcgcgtcggagccgccctggggtcttcgggggctgctgccagcaccttggctctttttccagacggcggcgctggaagccggcggcccgggtgcagcggccaggaaggggcgcaggcgcggggggcttaggccaaagggcgcagggttcaagtagggcaggaacggtccggtgggggcaggggcgggggtcgtgaagggttccagcagcgggaacggcaggcccggcgctgatgcggggtcaacctccggggggcgctccggcgcgggcggctctcggtccagggccgggggtggcggcggggctgggctctgcgcatgctccgcgcaaacatgcaggtgcttgaagagcgagcggtgcgtgcggaagcgcaggaggcagttctcacacttgaagtagcgattgggtttgtagtgcagtttgctgtgagccaccagctcctgcatgctggggaaggtctcggtgcagctcagggctgagcagcggaagagcttgccttccagggactgtgtgggcgggcagtgggttcgcagatgctgtgccaggtcacggacgctgggaaaactgaggcagcagccagggctggagcaagggatttgcttccctggaggtgggcgtcgtctgggaggccgcaggtcctcgctggtcccggagactatgctggtcaggccagggctgggtccggggccaggctggcagctgtctggggctggggaggagccctgctgcatccctccagcccctccacgttcccacactggcggtgtggctgcctgctcagggcctggctcctccgacatggaggaggaaggggctgcagctggcacagccggggacaacacctccttgtcggtctcactggagctgggctctgcagtggccagcatgtctgggatgggccctgagggtttctcctccatcttcgacacggctcggcctcttgtttctgcggctccggcggctgcagcttaggcggcggccaccctctgggcagtgcgagttcgcgctcacgtcagcgccattttccacctctcagctctc

SEQ ID NO: 11763 - RNA, 3512 nt, Homo sapiens
  source 1..3512: mol_type = other RNA
ctgaatagctgggactacaggtgtgcgccaccacgcccagctaatttttgtgtttttagtagagatggggtttcaccatgttggccaggatggtctcaatttattgacctcatgatccacccacctcggcctccgaaagtgctgggattacaggcataagccaccacacccagcctgtgggaactatttattggatttcaaaacaccctctgcctcattaatccactaagctttctcagcaaaaagctgtttaaataaataatgggaacatctaatttaaaacagtttttctaattatagaccagtacacgaagaagagcttaacttatccaagtatagtctagtttgggtccataatggagctgaaggctcagaggacattcagggccattacactgcaggaaaacaaggaataagggatgtagaaatgacctaagaaaagcacgaagtggaatgtatactggaggcaagttaatgaaagctaataaatacaaagtgctgggaaaaatctaaaagcaaaatagctattgtaacttgcaatgcattaaaaacaactttaaaaccaaaaagtcttgataaggaaactctatagtggggtctcagttaaatgctgatgatttttaatgctcagataacattaagtggaatattaacttctgcatccgacaccatctgaattttctcacacactactacacttgttcacttttcaatcaagttccactttctgaacttgttcaaaacctcatttgaaatatatccagctactgcttttcccctttcacctagcacagggcagttacctggcaaagctctattctggccaagtcactgggactgagtagaacccacgttagcagctctggacctgaacaggagctggcccaacatcacagtgaccacccacaaagagacaagccctcctggatttttttcagcatttcttatactgactacagtagtgatgattaaagttatctgccctacagactccactgaatttgaagctgtatttattgtacagatgggggaaatgtgttttattgtgtcagttatattaatttttatcaatgtgattagatacatattttggcctattaatcttattcattatattcttagtctgagatgggttttaattctgactaacagcagctacttaagagtccaatcatacaaaatcaggagagtattaccctttctacagctaagcgagtcagtaatacagcagcaactaatactggccattaataacgtccagagagcacattagcaaaccttgtactcccagtgactgtcaggagacttgaaaataactactattctcttccaaagtagaatagcgtttttctagatagtgaaggaaatgatagtcatagttggtctgaactccaagatcctactcctcaaaacagcaccgaagcaggggttcgggatgcctgctaagagcatttccacagttcaagtctcttcagaaccttagggaccttcgtgtctagcttcacacacccacctccacatatgaaccagcctaccacacttcacatctgggtacactggccattagcaacaatgcagtctcatgcagcagcacattaaaatcaaacgggtggcaatcgttcaccaccctcagagtgttgggagactttcacatttcatcatccttataatccacaaacagaaacatgaagggatgcaagtgagttcagcattcactcgtttggtgcactcaagtgctgagagaatgcagaatttacagtgtcacagaggaaaaaagccatctgaaataattgtaaaaatggttaagtgtggtatttaaatgttggttccctcctcttcatacaagtggaagaaaagaaggggctagggtacccactgggccatgaggttaaccccttagcacaggcaatgaagaacatccaatgccacagattctgcaggaggagaaatcccaagggtatacagtattcctgagaaagatcccagatttttctgaatcagtcttaatctgattttgttttggctacacagttatgctgttatacctttgacatacataaaaatggtcattttatttcaatccagacagctcagcattgtacaaatgatggcagaaagatccatttgttcagactcagcttgctttgtttttaatacatcgtcattcttcttgatgacataaataatggctccttcctgaaaggacagctcatcttccttgtcttttgtatagtcataaattgccacaaccttttccaagtaagaacgtggagcccacggtgggtcctcttcagcataaggatcactatactcaaccacagcagcttcctcctcttcgtaatcttctggaggaggaggaggtgggggagactcatcaaagactggttcttccacaggtggcggtggaggtggtgtatctgaaactggattctggctataaaaaggtcctccattcatctgattctgaaggcttgtttgtgaagtaatggaaggagggcgtctatagggcaacgagccccctattgttgggggagtatggcgagaggcaggcctattcatgctgtagaactgtacaggatgacctggaaagacactgggaggagatggagtaggaacagcaataggaacccccacactaccacttccactgttctctcgactgctgctccgactacttgggtggctccctccactactcccactgctgccaagtgtccctttccctgacatagggggactagggggcttctgagttggaggtgttgtacgcggcagcccacccatcttcatgttctgggtactcacctttactccatgtccaatatcatctagaattgtatagtcaataggttttctaatataacgaactggtcgttcaaggttggctggagcaataatcttatgtgtccttgaagtgtttttattggtagtcaaaataccaatttctcttcttgcaactttctctttatgaatatcaactgtttgtgaaatatgattgattgaagattccatccttcgtagctgggatgcctggatatccagcatctgcaggacattgttggccaaggtgtttatcagataggcaacacttgctaaggattgggtggtgtaggctttggtttcttctagggctctctgcttatctgctgactgtagtcccagactactgagagactgaggcaggatgatcacttgagcacaggagttcaaggctgcagtgagctatgatcacaccactgcattccagcctgcatgacataccaagaccccatctctgtatgtagttgttctcgcagtaatcggccacccgttccagatttgtgtagctgtcgaagagggcccggcggccccccgggatttcctcttccagcagcatctgcagctccgccatcttcacatcctcctcctcctcctcctcatacaggtcgcagagggagcggcggccgcagcgccaaggaaacccaggaccgggagaggaggagcggcggcgacggcggcggtaactcggaagg

SEQ ID NO: 11764 - RNA, 3388 nt, Homo sapiens
  source 1..3388: mol_type = other RNA
ctgaatagctgggactacaggtgtgcgccaccacgcccagctaatttttgtgtttttagtagagatggggtttcaccatgttggccaggatggtctcaatttattgacctcatgatccacccacctcggcctccgaaagtgctgggattacaggcataagccaccacacccagcctgtgggaactatttattggatttcaaaacaccctctgcctcattaatccactaagctttctcagcaaaaagctgtttaaataaataatgggaacatctaatttaaaacagtttttctaattatagaccagtacacgaagaagagcttaacttatccaagtatagtctagtttgggtccataatggagctgaaggctcagaggacattcagggccattacactgcaggaaaacaaggaataagggatgtagaaatgacctaagaaaagcacgaagtggaatgtatactggaggcaagttaatgaaagctaataaatacaaagtgctgggaaaaatctaaaagcaaaatagctattgtaacttgcaatgcattaaaaacaactttaaaaccaaaaagtcttgataaggaaactctatagtggggtctcagttaaatgctgatgatttttaatgctcagataacattaagtggaatattaacttctgcatccgacaccatctgaattttctcacacactactacacttgttcacttttcaatcaagttccactttctgaacttgttcaaaacctcatttgaaatatatccagctactgcttttcccctttcacctagcacagggcagttacctggcaaagctctattctggccaagtcactgggactgagtagaacccacgttagcagctctggacctgaacaggagctggcccaacatcacagtgaccacccacaaagagacaagccctcctggatttttttcagcatttcttatactgactacagtagtgatgattaaagttatctgccctacagactccactgaatttgaagctgtatttattgtacagatgggggaaatgtgttttattgtgtcagttatattaatttttatcaatgtgattagatacatattttggcctattaatcttattcattatattcttagtctgagatgggttttaattctgactaacagcagctacttaagagtccaatcatacaaaatcaggagagtattaccctttctacagctaagcgagtcagtaatacagcagcaactaatactggccattaataacgtccagagagcacattagcaaaccttgtactcccagtgactgtcaggagacttgaaaataactactattctcttccaaagtagaatagcgtttttctagatagtgaaggaaatgatagtcatagttggtctgaactccaagatcctactcctcaaaacagcaccgaagcaggggttcgggatgcctgctaagagcatttccacagttcaagtctcttcagaaccttagggaccttcgtgtctagcttcacacacccacctccacatatgaaccagcctaccacacttcacatctgggtacactggccattagcaacaatgcagtctcatgcagcagcacattaaaatcaaacgggtggcaatcgttcaccaccctcagagtgttgggagactttcacatttcatcatccttataatccacaaacagaaacatgaagggatgcaagtgagttcagcattcactcgtttggtgcactcaagtgctgagagaatgcagaatttacagtgtcacagaggaaaaaagccatctgaaataattgtaaaaatggttaagtgtggtatttaaatgttggttccctcctcttcatacaagtggaagaaaagaaggggctagggtacccactgggccatgaggttaaccccttagcacaggcaatgaagaacatccaatgccacagattctgcaggaggagaaatcccaagggtatacagtattcctgagaaagatcccagatttttctgaatcagtcttaatctgattttgttttggctacacagttatgctgttatacctttgacatacataaaaatggtcattttatttcaatccagacagctcagcattgtacaaatgatggcagaaagatccatttgttcagactcagcttgctttgtttttaatacatcgtcattcttcttgatgacataaataatggctccttcctgaaaggacagctcatcttccttgtcttttgtatagtcataaattgccacaaccttttccaagtaagaacgtggagcccacggtgggtcctcttcagcataaggatcactatactcaaccacagcagcttcctcctcttcgtaatcttctggaggaggaggaggtgggggagactcatcaaagactggttcttccacaggtggcggtggaggtggtgtatctgaaactggattctggctataaaaaggtcctccattcatctgattctgaaggcttgtttgtgaagtaatggaaggagggcgtctatagggcaacgagccccctattgttgggggagtatggcgagaggcaggcctattcatgctgtagaactgtacaggatgacctggaaagacactgggaggagatggagtaggaacagcaataggaacccccacactaccacttccactgttctctcgactgctgctccgactacttgggtggctccctccactactcccactgctgccaagtgtccctttccctgacatagggggactagggggcttctgagttggaggtgttgtacgcggcagcccacccatcttcatgttctgggtactcacctttactccatgtccaatatcatctagaattgtatagtcaataggttttctaatataacgaactggtcgttcaaggttggctggagcaataatcttatgtgtccttgaagtgtttttattggtagtcaaaataccaatttctcttcttgcaactttctctttatgaatatcaactgtttgtgaaatatgattgattgaagattccatccttcgtagctgggatgcctggatatccagcatctgcaggacattgttggccaaggtgtttatcagataggcaacacttgctaaggattgggtggtgtaggctttggtttcttctagggctctctgcttatctgctgactgtatgtagttgttctcgcagtaatcggccacccgttccagatttgtgtagctgtcgaagagggcccggcggccccccgggatttcctcttccagcagcatctgcagctccgccatcttcacatcctcctcctcctcctcctcatacaggtcgcagagggagcggcggccgcagcgccaaggaaacccaggaccgggagaggaggagcggcggcgacggcggcggtaactcggaagg

SEQ ID NO: 11765 - RNA, 4073 nt, Homo sapiens
  source 1..4073: mol_type = other RNA
ctgaatagctgggactacaggtgtgcgccaccacgcccagctaatttttgtgtttttagtagagatggggtttcaccatgttggccaggatggtctcaatttattgacctcatgatccacccacctcggcctccgaaagtgctgggattacaggcataagccaccacacccagcctgtgggaactatttattggatttcaaaacaccctctgcctcattaatccactaagctttctcagcaaaaagctgtttaaataaataatgggaacatctaatttaaaacagtttttctaattatagaccagtacacgaagaagagcttaacttatccaagtatagtctagtttgggtccataatggagctgaaggctcagaggacattcagggccattacactgcaggaaaacaaggaataagggatgtagaaatgacctaagaaaagcacgaagtggaatgtatactggaggcaagttaatgaaagctaataaatacaaagtgctgggaaaaatctaaaagcaaaatagctattgtaacttgcaatgcattaaaaacaactttaaaaccaaaaagtcttgataaggaaactctatagtggggtctcagttaaatgctgatgatttttaatgctcagataacattaagtggaatattaacttctgcatccgacaccatctgaattttctcacacactactacacttgttcacttttcaatcaagttccactttctgaacttgttcaaaacctcatttgaaatatatccagctactgcttttcccctttcacctagcacagggcagttacctggcaaagctctattctggccaagtcactgggactgagtagaacccacgttagcagctctggacctgaacaggagctggcccaacatcacagtgaccacccacaaagagacaagccctcctggatttttttcagcatttcttatactgactacagtagtgatgattaaagttatctgccctacagactccactgaatttgaagctgtatttattgtacagatgggggaaatgtgttttattgtgtcagttatattaatttttatcaatgtgattagatacatattttggcctattaatcttattcattatattcttagtctgagatgggttttaattctgactaacagcagctacttaagagtccaatcatacaaaatcaggagagtattaccctttctacagctaagcgagtcagtaatacagcagcaactaatactggccattaataacgtccagagagcacattagcaaaccttgtactcccagtgactgtcaggagacttgaaaataactactattctcttccaaagtagaatagcgtttttctagatagtgaaggaaatgatagtcatagttggtctgaactccaagatcctactcctcaaaacagcaccgaagcaggggttcgggatgcctgctaagagcatttccacagttcaagtctcttcagaaccttagggaccttcgtgtctagcttcacacacccacctccacatatgaaccagcctaccacacttcacatctgggtacactggccattagcaacaatgcagtctcatgcagcagcacattaaaatcaaacgggtggcaatcgttcaccaccctcagagtgttgggagactttcacatttcatcatccttataatccacaaacagaaacatgaagggatgcaagtgagttcagcattcactcgtttggtgcactcaagtgctgagagaatgcagaatttacagtgtcacagaggaaaaaagccatctgaaataattgtaaaaatggttaagtgtggtatttaaatgttggttccctcctcttcatacaagtggaagaaaagaaggggctagggtacccactgggccatgaggttaaccccttagcacaggcaatgaagaacatccaatgccacagattctgcaggaggagaaatcccaagggtatacagtattcctgagaaagatcccagatttttctgaatcagtcttaatctgattttgttttggctacacagttatgctgttatacctttgacatacataaaaatggtcattttatttcaatccagacagctcagcattgtacaaatgatggcagaaagatccatttgttcagactcagcttgctttgtttttaatacatcgtcattcttcttgatgacataaataatggctccttcctgaaaggacagctcatcttccttgtcttttgtatagtcataaattgccacaaccttttccaagtaagaacgtggagcccacggtgggtcctcttcagcataaggatcactatactcaaccacagcagcttcctcctcttcgtaatcttctggaggaggaggaggtgggggagactcatcaaagactggttcttccacaggtggcggtggaggtggtgtatctgaaactggattctggctataaaaaggtcctccattcatctgattctgaaggcttgtttgtgaagtaatggaaggagggcgtctatagggcaacgagccccctattgttgggggagtatggcgagaggcaggcctattcatgctgtagaactgtacaggatgacctggaaagacactgggaggagatggagtaggaacagcaataggaacccccacactaccacttccactgttctctcgactgctgctccgactacttgggtggctccctccactactcccactgctgctgtaagttcgatttctttgattcacagaagctgtcctcacagggctctgctgcgagggagccatattacgggttgggctaggtacgtaatcatttggtaccactggaggacgcactggctccagtgtgcgatagggggagtgccgcccaagtgtccctttccctgacatagggggactagggggcttctgagttggaggtgttgtacgcggcagcccacccatcttcatgttctgggtactcaccttaaatctaagcaaccactttactccatgtccaatatcatctagaattgtatagtcaataggttttctaatataacgaactggtcgttcaaggttggctggagcaataatcttatgtgtccttgaagtgtttttattggtagtcaaaataccaatttctcttcttgcaactttctctttatgaatatcaactgtttgtgaaatatgattgattgaagattccatccttcgtagctgggatgcctggatatccagcatctgcaggacattgttggccaaggtgtttatcagataggcaacacttgctaaggattgggtggtgtaggctttggtttcttctagggctctctgcttatctgctgactgtatgtagttgttctcgcagtaatcggccacccgttccagatttgtgtagctgtcgaagagggcccggcggccccccgggatttcctcttccagcagcatctgcagctccgccatcttcacatcctcctcctcctcctcctcatacaggtcgcagagggagcggcggccgcagcgccaaggaaacccaggaccgggagaggaggagcggcggcgacggcggcggtaactcggaaggagcgagaaacagccccagcgcgcgacaggggagggggcgacgggggcggggcgcgagccgacggactccgaggacggtcaccgcggcgacggccggccgggcgcgcgcacgcgcgctcccttccctccgcccccgggagcccgaaaaagattcccaccctcgcccgcgccgccggcccctcccccacttccggcgtctcctagcgacggcgggggtaggggccgggatgcgcgcgggagttggtggtgcagttaacccttccgccgcccgcccgccgctggagcggctggagaagcccccacctcccggcggcctttgttagcccggcgggaacacaccaccctgctcagctggcttcctgccggctccctccgggactcatctcggctccgtccccatggaggtcatcggcctagggaacttctcgaggcttttctccctctgctgctgacgggaggccgaaggagggcacagcctccactcttgggaccctcctctgtgaaagatcacacctcaacag

SEQ ID NO: 11766 - RNA, 3367 nt, Homo sapiens
  source 1..3367: mol_type = other RNA
ctgaatagctgggactacaggtgtgcgccaccacgcccagctaatttttgtgtttttagtagagatggggtttcaccatgttggccaggatggtctcaatttattgacctcatgatccacccacctcggcctccgaaagtgctgggattacaggcataagccaccacacccagcctgtgggaactatttattggatttcaaaacaccctctgcctcattaatccactaagctttctcagcaaaaagctgtttaaataaataatgggaacatctaatttaaaacagtttttctaattatagaccagtacacgaagaagagcttaacttatccaagtatagtctagtttgggtccataatggagctgaaggctcagaggacattcagggccattacactgcaggaaaacaaggaataagggatgtagaaatgacctaagaaaagcacgaagtggaatgtatactggaggcaagttaatgaaagctaataaatacaaagtgctgggaaaaatctaaaagcaaaatagctattgtaacttgcaatgcattaaaaacaactttaaaaccaaaaagtcttgataaggaaactctatagtggggtctcagttaaatgctgatgatttttaatgctcagataacattaagtggaatattaacttctgcatccgacaccatctgaattttctcacacactactacacttgttcacttttcaatcaagttccactttctgaacttgttcaaaacctcatttgaaatatatccagctactgcttttcccctttcacctagcacagggcagttacctggcaaagctctattctggccaagtcactgggactgagtagaacccacgttagcagctctggacctgaacaggagctggcccaacatcacagtgaccacccacaaagagacaagccctcctggatttttttcagcatttcttatactgactacagtagtgatgattaaagttatctgccctacagactccactgaatttgaagctgtatttattgtacagatgggggaaatgtgttttattgtgtcagttatattaatttttatcaatgtgattagatacatattttggcctattaatcttattcattatattcttagtctgagatgggttttaattctgactaacagcagctacttaagagtccaatcatacaaaatcaggagagtattaccctttctacagctaagcgagtcagtaatacagcagcaactaatactggccattaataacgtccagagagcacattagcaaaccttgtactcccagtgactgtcaggagacttgaaaataactactattctcttccaaagtagaatagcgtttttctagatagtgaaggaaatgatagtcatagttggtctgaactccaagatcctactcctcaaaacagcaccgaagcaggggttcgggatgcctgctaagagcatttccacagttcaagtctcttcagaaccttagggaccttcgtgtctagcttcacacacccacctccacatatgaaccagcctaccacacttcacatctgggtacactggccattagcaacaatgcagtctcatgcagcagcacattaaaatcaaacgggtggcaatcgttcaccaccctcagagtgttgggagactttcacatttcatcatccttataatccacaaacagaaacatgaagggatgcaagtgagttcagcattcactcgtttggtgcactcaagtgctgagagaatgcagaatttacagtgtcacagaggaaaaaagccatctgaaataattgtaaaaatggttaagtgtggtatttaaatgttggttccctcctcttcatacaagtggaagaaaagaaggggctagggtacccactgggccatgaggttaaccccttagcacaggcaatgaagaacatccaatgccacagattctgcaggaggagaaatcccaagggtatacagtattcctgagaaagatcccagatttttctgaatcagtcttaatctgattttgttttggctacacagttatgctgttatacctttgacatacataaaaatggtcattttatttcaatccagacagctcagcattgtacaaatgatggcagaaagatccatttgttcagactcagcttgctttgtttttaatacatcgtcattcttcttgatgacataaataatggctccttcctgaaaggacagctcatcttccttgtcttttgtatagtcataaattgccacaaccttttccaagtaagaacgtggagcccacggtgggtcctcttcagcataaggatcactatactcaaccacagcagcttcctcctcttcgtaatcttctggaggaggaggaggtgggggagactcatcaaagactggttcttccacaggtggcggtggaggtggtgtatctgaaactggattctggctataaaaaggtcctccattcatctgattctgaaggcttgtttgtgaagtaatggaaggagggcgtctatagggcaacgagccccctattgttgggggagtatggcgagaggcaggcctattcatgctgtagaactgtacaggatgacctggaaagacactgggaggagatggagtaggaacagcaataggaacccccacactaccacttccactgttctctcgactgctgctccgactacttgggtggctccctccactactcccactgctgctgtaagttcgatttctttgattcacagaagctgtcctcacagggctctgctgcgagggagccatattacgggttgggctaggtacgtaatcatttggtaccactggaggacgcactggctccagtgtgcgatagggggagtgccgcccaagtgtccctttccctgacatagggggactagggggcttctgagttggaggtgttgtacgcggcagcccacccatcttcatgttctgggtactcacctttactccatgtccaatatcatctagaattgtatagtcaataggttttctaatataacgaactggtcgttcaaggttggctggagcaataatcttatgtgtccttgaagtgtttttattggtagtcaaaataccaatttctcttcttgcaactttctctttatgaatatcaactgtctgtatgtagttgttctcgcagtaatcggccacccgttccagatttgtgtagctgtcgaagagggcccggcggccccccgggatttcctcttccagcagcatctgcagctccgccatcttcacatcctcctcctcctcctcctcatacaggtcgcagagggagcggcggccgcagcgccaaggaaacccaggaccgggagaggaggagcggcggcgacggcggcggtaactcggaagg

SEQ ID NO: 11767 - RNA, 3535 nt, Homo sapiens
  source 1..3535: mol_type = other RNA
ctgaatagctgggactacaggtgtgcgccaccacgcccagctaatttttgtgtttttagtagagatggggtttcaccatgttggccaggatggtctcaatttattgacctcatgatccacccacctcggcctccgaaagtgctgggattacaggcataagccaccacacccagcctgtgggaactatttattggatttcaaaacaccctctgcctcattaatccactaagctttctcagcaaaaagctgtttaaataaataatgggaacatctaatttaaaacagtttttctaattatagaccagtacacgaagaagagcttaacttatccaagtatagtctagtttgggtccataatggagctgaaggctcagaggacattcagggccattacactgcaggaaaacaaggaataagggatgtagaaatgacctaagaaaagcacgaagtggaatgtatactggaggcaagttaatgaaagctaataaatacaaagtgctgggaaaaatctaaaagcaaaatagctattgtaacttgcaatgcattaaaaacaactttaaaaccaaaaagtcttgataaggaaactctatagtggggtctcagttaaatgctgatgatttttaatgctcagataacattaagtggaatattaacttctgcatccgacaccatctgaattttctcacacactactacacttgttcacttttcaatcaagttccactttctgaacttgttcaaaacctcatttgaaatatatccagctactgcttttcccctttcacctagcacagggcagttacctggcaaagctctattctggccaagtcactgggactgagtagaacccacgttagcagctctggacctgaacaggagctggcccaacatcacagtgaccacccacaaagagacaagccctcctggatttttttcagcatttcttatactgactacagtagtgatgattaaagttatctgccctacagactccactgaatttgaagctgtatttattgtacagatgggggaaatgtgttttattgtgtcagttatattaatttttatcaatgtgattagatacatattttggcctattaatcttattcattatattcttagtctgagatgggttttaattctgactaacagcagctacttaagagtccaatcatacaaaatcaggagagtattaccctttctacagctaagcgagtcagtaatacagcagcaactaatactggccattaataacgtccagagagcacattagcaaaccttgtactcccagtgactgtcaggagacttgaaaataactactattctcttccaaagtagaatagcgtttttctagatagtgaaggaaatgatagtcatagttggtctgaactccaagatcctactcctcaaaacagcaccgaagcaggggttcgggatgcctgctaagagcatttccacagttcaagtctcttcagaaccttagggaccttcgtgtctagcttcacacacccacctccacatatgaaccagcctaccacacttcacatctgggtacactggccattagcaacaatgcagtctcatgcagcagcacattaaaatcaaacgggtggcaatcgttcaccaccctcagagtgttgggagactttcacatttcatcatccttataatccacaaacagaaacatgaagggatgcaagtgagttcagcattcactcgtttggtgcactcaagtgctgagagaatgcagaatttacagtgtcacagaggaaaaaagccatctgaaataattgtaaaaatggttaagtgtggtatttaaatgttggttccctcctcttcatacaagtggaagaaaagaaggggctagggtacccactgggccatgaggttaaccccttagcacaggcaatgaagaacatccaatgccacagattctgcaggaggagaaatcccaagggtatacagtattcctgagaaagatcccagatttttctgaatcagtcttaatctgattttgttttggctacacagttatgctgttatacctttgacatacataaaaatggtcattttatttcaatccagacagctcagcattgtacaaatgatggcagaaagatccatttgttcagactcagcttgctttgtttttaatacatcgtcattcttcttgatgacataaataatggctccttcctgaaaggacagctcatcttccttgtcttttgtatagtcataaattgccacaaccttttccaagtaagaacgtggagcccacggtgggtcctcttcagcataaggatcactatactcaaccacagcagcttcctcctcttcgtaatcttctggaggaggaggaggtgggggagactcatcaaagactggttcttccacaggtggcggtggaggtggtgtatctgaaactggattctggctataaaaaggtcctccattcatctgattctgaaggcttgtttgtgaagtaatggaaggagggcgtctatagggcaacgagccccctattgttgggggagtatggcgagaggcaggcctattcatgctgtagaactgtacaggatgacctggaaagacactgggaggagatggagtaggaacagcaataggaacccccacactaccacttccactgttctctcgactgctgctccgactacttgggtggctccctccactactcccactgctgctgtaagttcgatttctttgattcacagaagctgtcctcacagggctctgctgcgagggagccatattacgggttgggctaggtacgtaatcatttggtaccactggaggacgcactggctccagtgtgcgatagggggagtgccgcccaagtgtccctttccctgacatagggggactagggggcttctgagttggaggtgttgtacgcggcagcccacccatcttcatgttctgggtactcacctttactccatgtccaatatcatctagaattgtatagtcaataggttttctaatataacgaactggtcgttcaaggttggctggagcaataatcttatgtgtccttgaagtgtttttattggtagtcaaaataccaatttctcttcttgcaactttctctttatgaatatcaactgtttgtgaaatatgattgattgaagattccatccttcgtagctgggatgcctggatatccagcatctgcaggacattgttggccaaggtgtttatcagataggcaacacttgctaaggattgggtggtgtaggctttggtttcttctagggctctctgcttatctgctgactgtatgtagttgttctcgcagtaatcggccacccgttccagatttgtgtagctgtcgaagagggcccggcggccccccgggatttcctcttccagcagcatctgcagctccgccatcttcacatcctcctcctcctcctcctcatacaggtcgcagagggagcggcggccgcagcgccaaggaaacccaggaccgggagaggaggagcggcggcgacggcggcggtaactcggaagg

SEQ ID NO: 11768 - RNA, 3532 nt, Homo sapiens
  source 1..3532: mol_type = other RNA
ctgaatagctgggactacaggtgtgcgccaccacgcccagctaatttttgtgtttttagtagagatggggtttcaccatgttggccaggatggtctcaatttattgacctcatgatccacccacctcggcctccgaaagtgctgggattacaggcataagccaccacacccagcctgtgggaactatttattggatttcaaaacaccctctgcctcattaatccactaagctttctcagcaaaaagctgtttaaataaataatgggaacatctaatttaaaacagtttttctaattatagaccagtacacgaagaagagcttaacttatccaagtatagtctagtttgggtccataatggagctgaaggctcagaggacattcagggccattacactgcaggaaaacaaggaataagggatgtagaaatgacctaagaaaagcacgaagtggaatgtatactggaggcaagttaatgaaagctaataaatacaaagtgctgggaaaaatctaaaagcaaaatagctattgtaacttgcaatgcattaaaaacaactttaaaaccaaaaagtcttgataaggaaactctatagtggggtctcagttaaatgctgatgatttttaatgctcagataacattaagtggaatattaacttctgcatccgacaccatctgaattttctcacacactactacacttgttcacttttcaatcaagttccactttctgaacttgttcaaaacctcatttgaaatatatccagctactgcttttcccctttcacctagcacagggcagttacctggcaaagctctattctggccaagtcactgggactgagtagaacccacgttagcagctctggacctgaacaggagctggcccaacatcacagtgaccacccacaaagagacaagccctcctggatttttttcagcatttcttatactgactacagtagtgatgattaaagttatctgccctacagactccactgaatttgaagctgtatttattgtacagatgggggaaatgtgttttattgtgtcagttatattaatttttatcaatgtgattagatacatattttggcctattaatcttattcattatattcttagtctgagatgggttttaattctgactaacagcagctacttaagagtccaatcatacaaaatcaggagagtattaccctttctacagctaagcgagtcagtaatacagcagcaactaatactggccattaataacgtccagagagcacattagcaaaccttgtactcccagtgactgtcaggagacttgaaaataactactattctcttccaaagtagaatagcgtttttctagatagtgaaggaaatgatagtcatagttggtctgaactccaagatcctactcctcaaaacagcaccgaagcaggggttcgggatgcctgctaagagcatttccacagttcaagtctcttcagaaccttagggaccttcgtgtctagcttcacacacccacctccacatatgaaccagcctaccacacttcacatctgggtacactggccattagcaacaatgcagtctcatgcagcagcacattaaaatcaaacgggtggcaatcgttcaccaccctcagagtgttgggagactttcacatttcatcatccttataatccacaaacagaaacatgaagggatgcaagtgagttcagcattcactcgtttggtgcactcaagtgctgagagaatgcagaatttacagtgtcacagaggaaaaaagccatctgaaataattgtaaaaatggttaagtgtggtatttaaatgttggttccctcctcttcatacaagtggaagaaaagaaggggctagggtacccactgggccatgaggttaaccccttagcacaggcaatgaagaacatccaatgccacagattctgcaggaggagaaatcccaagggtatacagtattcctgagaaagatcccagatttttctgaatcagtcttaatctgattttgttttggctacacagttatgctgttatacctttgacatacataaaaatggtcattttatttcaatccagacagctcagcattgtacaaatgatggcagaaagatccatttgttcagactcagcttgctttgtttttaatacatcgtcattcttcttgatgacataaataatggctccttcctgaaaggacagctcatcttccttgtcttttgtatagtcataaattgccacaaccttttccaagtaagaacgtggagcccacggtgggtcctcttcagcataaggatcactatactcaaccacagcagcttcctcctcttcgtaatcttctggaggaggaggaggtgggggagactcatcaaagactggttcttccacaggtggcggtggaggtggtgtatctgaaactggattctggctataaaaaggtcctccattcatctgattctgaaggcttgtttgtgaagtaatggaaggagggcgtctatagggcaacgagccccctattgttgggggagtatggcgagaggcaggcctattcatgctgtagaactgtacaggatgacctggaaagacactgggaggagatggagtaggaacagcaataggaacccccacactaccacttccactgttctctcgactgctgctccgactacttgggtggctccctccactactcccactgctgtaagttcgatttctttgattcacagaagctgtcctcacagggctctgctgcgagggagccatattacgggttgggctaggtacgtaatcatttggtaccactggaggacgcactggctccagtgtgcgatagggggagtgccgcccaagtgtccctttccctgacatagggggactagggggcttctgagttggaggtgttgtacgcggcagcccacccatcttcatgttctgggtactcacctttactccatgtccaatatcatctagaattgtatagtcaataggttttctaatataacgaactggtcgttcaaggttggctggagcaataatcttatgtgtccttgaagtgtttttattggtagtcaaaataccaatttctcttcttgcaactttctctttatgaatatcaactgtttgtgaaatatgattgattgaagattccatccttcgtagctgggatgcctggatatccagcatctgcaggacattgttggccaaggtgtttatcagataggcaacacttgctaaggattgggtggtgtaggctttggtttcttctagggctctctgcttatctgctgactgtatgtagttgttctcgcagtaatcggccacccgttccagatttgtgtagctgtcgaagagggcccggcggccccccgggatttcctcttccagcagcatctgcagctccgccatcttcacatcctcctcctcctcctcctcatacaggtcgcagagggagcggcggccgcagcgccaaggaaacccaggaccgggagaggaggagcggcggcgacggcggcggtaactcggaagg

SEQ ID NO: 11769 - RNA, 3815 nt, Homo sapiens
  source 1..3815: mol_type = other RNA
ctgaatagctgggactacaggtgtgcgccaccacgcccagctaatttttgtgtttttagtagagatggggtttcaccatgttggccaggatggtctcaatttattgacctcatgatccacccacctcggcctccgaaagtgctgggattacaggcataagccaccacacccagcctgtgggaactatttattggatttcaaaacaccctctgcctcattaatccactaagctttctcagcaaaaagctgtttaaataaataatgggaacatctaatttaaaacagtttttctaattatagaccagtacacgaagaagagcttaacttatccaagtatagtctagtttgggtccataatggagctgaaggctcagaggacattcagggccattacactgcaggaaaacaaggaataagggatgtagaaatgacctaagaaaagcacgaagtggaatgtatactggaggcaagttaatgaaagctaataaatacaaagtgctgggaaaaatctaaaagcaaaatagctattgtaacttgcaatgcattaaaaacaactttaaaaccaaaaagtcttgataaggaaactctatagtggggtctcagttaaatgctgatgatttttaatgctcagataacattaagtggaatattaacttctgcatccgacaccatctgaattttctcacacactactacacttgttcacttttcaatcaagttccactttctgaacttgttcaaaacctcatttgaaatatatccagctactgcttttcccctttcacctagcacagggcagttacctggcaaagctctattctggccaagtcactgggactgagtagaacccacgttagcagctctggacctgaacaggagctggcccaacatcacagtgaccacccacaaagagacaagccctcctggatttttttcagcatttcttatactgactacagtagtgatgattaaagttatctgccctacagactccactgaatttgaagctgtatttattgtacagatgggggaaatgtgttttattgtgtcagttatattaatttttatcaatgtgattagatacatattttggcctattaatcttattcattatattcttagtctgagatgggttttaattctgactaacagcagctacttaagagtccaatcatacaaaatcaggagagtattaccctttctacagctaagcgagtcagtaatacagcagcaactaatactggccattaataacgtccagagagcacattagcaaaccttgtactcccagtgactgtcaggagacttgaaaataactactattctcttccaaagtagaatagcgtttttctagatagtgaaggaaatgatagtcatagttggtctgaactccaagatcctactcctcaaaacagcaccgaagcaggggttcgggatgcctgctaagagcatttccacagttcaagtctcttcagaaccttagggaccttcgtgtctagcttcacacacccacctccacatatgaaccagcctaccacacttcacatctgggtacactggccattagcaacaatgcagtctcatgcagcagcacattaaaatcaaacgggtggcaatcgttcaccaccctcagagtgttgggagactttcacatttcatcatccttataatccacaaacagaaacatgaagggatgcaagtgagttcagcattcactcgtttggtgcactcaagtgctgagagaatgcagaatttacagtgtcacagaggaaaaaagccatctgaaataattgtaaaaatggttaagtgtggtatttaaatgttggttccctcctcttcatacaagtggaagaaaagaaggggctagggtacccactgggccatgaggttaaccccttagcacaggcaatgaagaacatccaatgccacagattctgcaggaggagaaatcccaagggtatacagtattcctgagaaagatcccagatttttctgaatcagtcttaatctgattttgttttggctacacagttatgctgttatacctttgacatacataaaaatggtcattttatttcaatccagacagctcagcattgtacaaatgatggcagaaagatccatttgttcagactcagcttgctttgtttttaatacatcgtcattcttcttgatgacataaataatggctccttcctgaaaggacagctcatcttccttgtcttttgtatagtcataaattgccacaaccttttccaagtaagaacgtggagcccacggtgggtcctcttcagcataaggatcactatactcaaccacagcagcttcctcctcttcgtaatcttctggaggaggaggaggtgggggagactcatcaaagactggttcttccacaggtggcggtggaggtggtgtatctgaaactggattctggctataaaaaggtcctccattcatctgattctgaaggcttgtttgtgaagtaatggaaggagggcgtctatagggcaacgagccccctattgttgggggagtatggcgagaggcaggcctattcatgctgtagaactgtacaggatgacctgtagggggagtggaagaaacaacagggggagttggagaagtgaagccatcagcaagggtctgggcacccccagcagcagcgtctggggcagtggaggaagggacagtagcaggaacaagaggagcaggggcagatgcagaagtagcaggaaggggaggagtgccagcagagccagcaggggctggaaagacactgggaggagatggagtaggaacagcaataggaacccccacactaccacttccactgttctctcgactgctgctccgactacttgggtggctccctccactactcccactgctgctgtaagttcgatttctttgattcacagaagctgtcctcacagggctctgctgcgagggagccatattacgggttgggctaggtacgtaatcatttggtaccactggaggacgcactggctccagtgtgcgatagggggagtgccgcccaagtgtccctttccctgacatagggggactagggggcttctgagttggaggtgttgtacgcggcagcccacccatcttcatgttctgggtactcaccatgactgaggatttggaaccaacaatccaatcaataatacaggtgtccatatgcctgggctcttccaatcaaatctaccttaaatctaagcaaccactttactccatgtccaatatcatctagaattgtatagtcaataggttttctaatataacgaactggtcgttcaaggttggctggagcaataatcttatgtgtccttgaagtgtttttattggtagtcaaaataccaatttctcttcttgcaactttctctttatgaatatcaactgtttgtgaaatatgattgattgaagattccatccttcgtagctgggatgcctggatatccagcatctgcaggacattgttggccaaggtgtttatcagataggcaacacttgctaaggattgggtggtgtaggctttggtttcttctagggctctctgcttatctgctgactgtatgtagttgttctcgcagtaatcggccacccgttccagatttgtgtagctgtcgaagagggcccggcggccccccgggatttcctcttccagcagcatctgcagctccgccatcttcacatcctcctcctcctcctcctcatacaggtcgcagagggagcggcggccgcagcgccaaggaaacccaggaccgggagaggaggagcggcggcgacggcggcggtaactcggaagg

SEQ ID NO: 11770 - RNA, 3622 nt, Homo sapiens
  source 1..3622: mol_type = other RNA
ctgaatagctgggactacaggtgtgcgccaccacgcccagctaatttttgtgtttttagtagagatggggtttcaccatgttggccaggatggtctcaatttattgacctcatgatccacccacctcggcctccgaaagtgctgggattacaggcataagccaccacacccagcctgtgggaactatttattggatttcaaaacaccctctgcctcattaatccactaagctttctcagcaaaaagctgtttaaataaataatgggaacatctaatttaaaacagtttttctaattatagaccagtacacgaagaagagcttaacttatccaagtatagtctagtttgggtccataatggagctgaaggctcagaggacattcagggccattacactgcaggaaaacaaggaataagggatgtagaaatgacctaagaaaagcacgaagtggaatgtatactggaggcaagttaatgaaagctaataaatacaaagtgctgggaaaaatctaaaagcaaaatagctattgtaacttgcaatgcattaaaaacaactttaaaaccaaaaagtcttgataaggaaactctatagtggggtctcagttaaatgctgatgatttttaatgctcagataacattaagtggaatattaacttctgcatccgacaccatctgaattttctcacacactactacacttgttcacttttcaatcaagttccactttctgaacttgttcaaaacctcatttgaaatatatccagctactgcttttcccctttcacctagcacagggcagttacctggcaaagctctattctggccaagtcactgggactgagtagaacccacgttagcagctctggacctgaacaggagctggcccaacatcacagtgaccacccacaaagagacaagccctcctggatttttttcagcatttcttatactgactacagtagtgatgattaaagttatctgccctacagactccactgaatttgaagctgtatttattgtacagatgggggaaatgtgttttattgtgtcagttatattaatttttatcaatgtgattagatacatattttggcctattaatcttattcattatattcttagtctgagatgggttttaattctgactaacagcagctacttaagagtccaatcatacaaaatcaggagagtattaccctttctacagctaagcgagtcagtaatacagcagcaactaatactggccattaataacgtccagagagcacattagcaaaccttgtactcccagtgactgtcaggagacttgaaaataactactattctcttccaaagtagaatagcgtttttctagatagtgaaggaaatgatagtcatagttggtctgaactccaagatcctactcctcaaaacagcaccgaagcaggggttcgggatgcctgctaagagcatttccacagttcaagtctcttcagaaccttagggaccttcgtgtctagcttcacacacccacctccacatatgaaccagcctaccacacttcacatctgggtacactggccattagcaacaatgcagtctcatgcagcagcacattaaaatcaaacgggtggcaatcgttcaccaccctcagagtgttgggagactttcacatttcatcatccttataatccacaaacagaaacatgaagggatgcaagtgagttcagcattcactcgtttggtgcactcaagtgctgagagaatgcagaatttacagtgtcacagaggaaaaaagccatctgaaataattgtaaaaatggttaagtgtggtatttaaatgttggttccctcctcttcatacaagtggaagaaaagaaggggctagggtacccactgggccatgaggttaaccccttagcacaggcaatgaagaacatccaatgccacagattctgcaggaggagaaatcccaagggtatacagtattcctgagaaagatcccagatttttctgaatcagtcttaatctgattttgttttggctacacagttatgctgttatacctttgacatacataaaaatggtcattttatttcaatccagacagctcagcattgtacaaatgatggcagaaagatccatttgttcagactcagcttgctttgtttttaatacatcgtcattcttcttgatgacataaataatggctccttcctgaaaggacagctcatcttccttgtcttttgtatagtcataaattgccacaaccttttccaagtaagaacgtggagcccacggtgggtcctcttcagcataaggatcactatactcaaccacagcagcttcctcctcttcgtaatcttctggaggaggaggaggtgggggagactcatcaaagactggttcttccacaggtggcggtggaggtggtgtatctgaaatattttcttggactctggccacaaatcccattaaaggtaactgaggagttacctgtaggatggagggaggaggaggagcaagagatactggattctggctataaaaaggtcctccattcatctgattctgaaggcttgtttgtgaagtaatggaaggagggcgtctatagggcaacgagccccctattgttgggggagtatggcgagaggcaggcctattcatgctgtagaactgtacaggatgacctggaaagacactgggaggagatggagtaggaacagcaataggaacccccacactaccacttccactgttctctcgactgctgctccgactacttgggtggctccctccactactcccactgctgctgtaagttcgatttctttgattcacagaagctgtcctcacagggctctgctgcgagggagccatattacgggttgggctaggtacgtaatcatttggtaccactggaggacgcactggctccagtgtgcgatagggggagtgccgcccaagtgtccctttccctgacatagggggactagggggcttctgagttggaggtgttgtacgcggcagcccacccatcttcatgttctgggtactcacctttactccatgtccaatatcatctagaattgtatagtcaataggttttctaatataacgaactggtcgttcaaggttggctggagcaataatcttatgtgtccttgaagtgtttttattggtagtcaaaataccaatttctcttcttgcaactttctctttatgaatatcaactgtttgtgaaatatgattgattgaagattccatccttcgtagctgggatgcctggatatccagcatctgcaggacattgttggccaaggtgtttatcagataggcaacacttgctaaggattgggtggtgtaggctttggtttcttctagggctctctgcttatctgctgactgtatgtagttgttctcgcagtaatcggccacccgttccagatttgtgtagctgtcgaagagggcccggcggccccccgggatttcctcttccagcagcatctgcagctccgccatcttcacatcctcctcctcctcctcctcatacaggtcgcagagggagcggcggccgcagcgccaaggaaacccaggaccgggagaggaggagcggcggcgacggcggcggtaactcggaagg

SEQ ID NO: 11771 - RNA, 3619 nt, Homo sapiens
  source 1..3619: mol_type = other RNA
ctgaatagctgggactacaggtgtgcgccaccacgcccagctaatttttgtgtttttagtagagatggggtttcaccatgttggccaggatggtctcaatttattgacctcatgatccacccacctcggcctccgaaagtgctgggattacaggcataagccaccacacccagcctgtgggaactatttattggatttcaaaacaccctctgcctcattaatccactaagctttctcagcaaaaagctgtttaaataaataatgggaacatctaatttaaaacagtttttctaattatagaccagtacacgaagaagagcttaacttatccaagtatagtctagtttgggtccataatggagctgaaggctcagaggacattcagggccattacactgcaggaaaacaaggaataagggatgtagaaatgacctaagaaaagcacgaagtggaatgtatactggaggcaagttaatgaaagctaataaatacaaagtgctgggaaaaatctaaaagcaaaatagctattgtaacttgcaatgcattaaaaacaactttaaaaccaaaaagtcttgataaggaaactctatagtggggtctcagttaaatgctgatgatttttaatgctcagataacattaagtggaatattaacttctgcatccgacaccatctgaattttctcacacactactacacttgttcacttttcaatcaagttccactttctgaacttgttcaaaacctcatttgaaatatatccagctactgcttttcccctttcacctagcacagggcagttacctggcaaagctctattctggccaagtcactgggactgagtagaacccacgttagcagctctggacctgaacaggagctggcccaacatcacagtgaccacccacaaagagacaagccctcctggatttttttcagcatttcttatactgactacagtagtgatgattaaagttatctgccctacagactccactgaatttgaagctgtatttattgtacagatgggggaaatgtgttttattgtgtcagttatattaatttttatcaatgtgattagatacatattttggcctattaatcttattcattatattcttagtctgagatgggttttaattctgactaacagcagctacttaagagtccaatcatacaaaatcaggagagtattaccctttctacagctaagcgagtcagtaatacagcagcaactaatactggccattaataacgtccagagagcacattagcaaaccttgtactcccagtgactgtcaggagacttgaaaataactactattctcttccaaagtagaatagcgtttttctagatagtgaaggaaatgatagtcatagttggtctgaactccaagatcctactcctcaaaacagcaccgaagcaggggttcgggatgcctgctaagagcatttccacagttcaagtctcttcagaaccttagggaccttcgtgtctagcttcacacacccacctccacatatgaaccagcctaccacacttcacatctgggtacactggccattagcaacaatgcagtctcatgcagcagcacattaaaatcaaacgggtggcaatcgttcaccaccctcagagtgttgggagactttcacatttcatcatccttataatccacaaacagaaacatgaagggatgcaagtgagttcagcattcactcgtttggtgcactcaagtgctgagagaatgcagaatttacagtgtcacagaggaaaaaagccatctgaaataattgtaaaaatggttaagtgtggtatttaaatgttggttccctcctcttcatacaagtggaagaaaagaaggggctagggtacccactgggccatgaggttaaccccttagcacaggcaatgaagaacatccaatgccacagattctgcaggaggagaaatcccaagggtatacagtattcctgagaaagatcccagatttttctgaatcagtcttaatctgattttgttttggctacacagttatgctgttatacctttgacatacataaaaatggtcattttatttcaatccagacagctcagcattgtacaaatgatggcagaaagatccatttgttcagactcagcttgctttgtttttaatacatcgtcattcttcttgatgacataaataatggctccttcctgaaaggacagctcatcttccttgtcttttgtatagtcataaattgccacaaccttttccaagtaagaacgtggagcccacggtgggtcctcttcagcataaggatcactatactcaaccacagcagcttcctcctcttcgtaatcttctggaggaggaggaggtgggggagactcatcaaagactggttcttccacaggtggcggtggaggtggtgtatctgaaatattttcttggactctggccacaaatcccattaaaggtaactgaggagttacctgtaggatggagggaggaggaggagcaagagatactggattctggctataaaaaggtcctccattcatctgattctgaaggcttgtttgtgaagtaatggaaggagggcgtctatagggcaacgagccccctattgttgggggagtatggcgagaggcaggcctattcatgctgtagaactgtacaggatgacctggaaagacactgggaggagatggagtaggaacagcaataggaacccccacactaccacttccactgttctctcgactgctgctccgactacttgggtggctccctccactactcccactgctgtaagttcgatttctttgattcacagaagctgtcctcacagggctctgctgcgagggagccatattacgggttgggctaggtacgtaatcatttggtaccactggaggacgcactggctccagtgtgcgatagggggagtgccgcccaagtgtccctttccctgacatagggggactagggggcttctgagttggaggtgttgtacgcggcagcccacccatcttcatgttctgggtactcacctttactccatgtccaatatcatctagaattgtatagtcaataggttttctaatataacgaactggtcgttcaaggttggctggagcaataatcttatgtgtccttgaagtgtttttattggtagtcaaaataccaatttctcttcttgcaactttctctttatgaatatcaactgtttgtgaaatatgattgattgaagattccatccttcgtagctgggatgcctggatatccagcatctgcaggacattgttggccaaggtgtttatcagataggcaacacttgctaaggattgggtggtgtaggctttggtttcttctagggctctctgcttatctgctgactgtatgtagttgttctcgcagtaatcggccacccgttccagatttgtgtagctgtcgaagagggcccggcggccccccgggatttcctcttccagcagcatctgcagctccgccatcttcacatcctcctcctcctcctcctcatacaggtcgcagagggagcggcggccgcagcgccaaggaaacccaggaccgggagaggaggagcggcggcgacggcggcggtaactcggaagg

SEQ ID NO: 11772 - RNA, 3823 nt, Homo sapiens
  source 1..3823: mol_type = other RNA
ctgaatagctgggactacaggtgtgcgccaccacgcccagctaatttttgtgtttttagtagagatggggtttcaccatgttggccaggatggtctcaatttattgacctcatgatccacccacctcggcctccgaaagtgctgggattacaggcataagccaccacacccagcctgtgggaactatttattggatttcaaaacaccctctgcctcattaatccactaagctttctcagcaaaaagctgtttaaataaataatgggaacatctaatttaaaacagtttttctaattatagaccagtacacgaagaagagcttaacttatccaagtatagtctagtttgggtccataatggagctgaaggctcagaggacattcagggccattacactgcaggaaaacaaggaataagggatgtagaaatgacctaagaaaagcacgaagtggaatgtatactggaggcaagttaatgaaagctaataaatacaaagtgctgggaaaaatctaaaagcaaaatagctattgtaacttgcaatgcattaaaaacaactttaaaaccaaaaagtcttgataaggaaactctatagtggggtctcagttaaatgctgatgatttttaatgctcagataacattaagtggaatattaacttctgcatccgacaccatctgaattttctcacacactactacacttgttcacttttcaatcaagttccactttctgaacttgttcaaaacctcatttgaaatatatccagctactgcttttcccctttcacctagcacagggcagttacctggcaaagctctattctggccaagtcactgggactgagtagaacccacgttagcagctctggacctgaacaggagctggcccaacatcacagtgaccacccacaaagagacaagccctcctggatttttttcagcatttcttatactgactacagtagtgatgattaaagttatctgccctacagactccactgaatttgaagctgtatttattgtacagatgggggaaatgtgttttattgtgtcagttatattaatttttatcaatgtgattagatacatattttggcctattaatcttattcattatattcttagtctgagatgggttttaattctgactaacagcagctacttaagagtccaatcatacaaaatcaggagagtattaccctttctacagctaagcgagtcagtaatacagcagcaactaatactggccattaataacgtccagagagcacattagcaaaccttgtactcccagtgactgtcaggagacttgaaaataactactattctcttccaaagtagaatagcgtttttctagatagtgaaggaaatgatagtcatagttggtctgaactccaagatcctactcctcaaaacagcaccgaagcaggggttcgggatgcctgctaagagcatttccacagttcaagtctcttcagaaccttagggaccttcgtgtctagcttcacacacccacctccacatatgaaccagcctaccacacttcacatctgggtacactggccattagcaacaatgcagtctcatgcagcagcacattaaaatcaaacgggtggcaatcgttcaccaccctcagagtgttgggagactttcacatttcatcatccttataatccacaaacagaaacatgaagggatgcaagtgagttcagcattcactcgtttggtgcactcaagtgctgagagaatgcagaatttacagtgtcacagaggaaaaaagccatctgaaataattgtaaaaatggttaagtgtggtatttaaatgttggttccctcctcttcatacaagtggaagaaaagaaggggctagggtacccactgggccatgaggttaaccccttagcacaggcaatgaagaacatccaatgccacagattctgcaggaggagaaatcccaagggtatacagtattcctgagaaagatcccagatttttctgaatcagtcttaatctgattttgttttggctacacagttatgctgttatacctttgacatacataaaaatggtcattttatttcaatccagacagctcagcattgtacaaatgatggcagaaagatccatttgttcagactcagcttgctttgtttttaatacatcgtcattcttcttgatgacataaataatggctccttcctgaaaggacagctcatcttccttgtcttttgtatagtcataaattgccacaaccttttccaagtaagaacgtggagcccacggtgggtcctcttcagcataaggatcactatactcaaccacagcagcttcctcctcttcgtaatcttctggaggaggaggaggtgggggagactcatcaaagactggttcttccacaggtggcggtggaggtggtgtatctgaaatattttcttggactctggccacaaatcccattaaaggtaactgaggagttacctgtaggatggagggaggaggaggagcaagagatactggattctggctataaaaaggtcctccattcatctgattctgaaggcttgtttgtgaagtaatggaaggagggcgtctatagggcaacgagccccctattgttgggggagtatggcgagaggcaggcctattcatgctgtagaactgtacaggatgacctgtagggggagtggaagaaacaacagggggagttggagaagtgaagccatcagcaagggtctgggcacccccagcagcagcgtctggggcagtggaggaagggacagtagcaggaacaagaggagcaggggcagatgcagaagtagcaggaaggggaggagtgccagcagagccagcaggggctggaaagacactgggaggagatggagtaggaacagcaataggaacccccacactaccacttccactgttctctcgactgctgctccgactacttgggtggctccctccactactcccactgctgctgtaagttcgatttctttgattcacagaagctgtcctcacagggctctgctgcgagggagccatattacgggttgggctaggtacgtaatcatttggtaccactggaggacgcactggctccagtgtgcgatagggggagtgccgcccaagtgtccctttccctgacatagggggactagggggcttctgagttggaggtgttgtacgcggcagcccacccatcttcatgttctgggtactcaccttaaatctaagcaaccactttactccatgtccaatatcatctagaattgtatagtcaataggttttctaatataacgaactggtcgttcaaggttggctggagcaataatcttatgtgtccttgaagtgtttttattggtagtcaaaataccaatttctcttcttgcaactttctctttatgaatatcaactgtttgtgaaatatgattgattgaagattccatccttcgtagctgggatgcctggatatccagcatctgcaggacattgttggccaaggtgtttatcagataggcaacacttgctaaggattgggtggtgtaggctttggtttcttctagggctctctgcttatctgctgactgtatgtagttgttctcgcagtaatcggccacccgttccagatttgtgtagctgtcgaagagggcccggcggccccccgggatttcctcttccagcagcatctgcagctccgccatcttcacatcctcctcctcctcctcctcatacaggtcgcagagggagcggcggccgcagcgccaaggaaacccaggaccgggagaggaggagcggcggcgacggcggcggtaactcggaagg

SEQ ID NO: 11773 - RNA, 3820 nt, Homo sapiens
  source 1..3820: mol_type = other RNA
ctgaatagctgggactacaggtgtgcgccaccacgcccagctaatttttgtgtttttagtagagatggggtttcaccatgttggccaggatggtctcaatttattgacctcatgatccacccacctcggcctccgaaagtgctgggattacaggcataagccaccacacccagcctgtgggaactatttattggatttcaaaacaccctctgcctcattaatccactaagctttctcagcaaaaagctgtttaaataaataatgggaacatctaatttaaaacagtttttctaattatagaccagtacacgaagaagagcttaacttatccaagtatagtctagtttgggtccataatggagctgaaggctcagaggacattcagggccattacactgcaggaaaacaaggaataagggatgtagaaatgacctaagaaaagcacgaagtggaatgtatactggaggcaagttaatgaaagctaataaatacaaagtgctgggaaaaatctaaaagcaaaatagctattgtaacttgcaatgcattaaaaacaactttaaaaccaaaaagtcttgataaggaaactctatagtggggtctcagttaaatgctgatgatttttaatgctcagataacattaagtggaatattaacttctgcatccgacaccatctgaattttctcacacactactacacttgttcacttttcaatcaagttccactttctgaacttgttcaaaacctcatttgaaatatatccagctactgcttttcccctttcacctagcacagggcagttacctggcaaagctctattctggccaagtcactgggactgagtagaacccacgttagcagctctggacctgaacaggagctggcccaacatcacagtgaccacccacaaagagacaagccctcctggatttttttcagcatttcttatactgactacagtagtgatgattaaagttatctgccctacagactccactgaatttgaagctgtatttattgtacagatgggggaaatgtgttttattgtgtcagttatattaatttttatcaatgtgattagatacatattttggcctattaatcttattcattatattcttagtctgagatgggttttaattctgactaacagcagctacttaagagtccaatcatacaaaatcaggagagtattaccctttctacagctaagcgagtcagtaatacagcagcaactaatactggccattaataacgtccagagagcacattagcaaaccttgtactcccagtgactgtcaggagacttgaaaataactactattctcttccaaagtagaatagcgtttttctagatagtgaaggaaatgatagtcatagttggtctgaactccaagatcctactcctcaaaacagcaccgaagcaggggttcgggatgcctgctaagagcatttccacagttcaagtctcttcagaaccttagggaccttcgtgtctagcttcacacacccacctccacatatgaaccagcctaccacacttcacatctgggtacactggccattagcaacaatgcagtctcatgcagcagcacattaaaatcaaacgggtggcaatcgttcaccaccctcagagtgttgggagactttcacatttcatcatccttataatccacaaacagaaacatgaagggatgcaagtgagttcagcattcactcgtttggtgcactcaagtgctgagagaatgcagaatttacagtgtcacagaggaaaaaagccatctgaaataattgtaaaaatggttaagtgtggtatttaaatgttggttccctcctcttcatacaagtggaagaaaagaaggggctagggtacccactgggccatgaggttaaccccttagcacaggcaatgaagaacatccaatgccacagattctgcaggaggagaaatcccaagggtatacagtattcctgagaaagatcccagatttttctgaatcagtcttaatctgattttgttttggctacacagttatgctgttatacctttgacatacataaaaatggtcattttatttcaatccagacagctcagcattgtacaaatgatggcagaaagatccatttgttcagactcagcttgctttgtttttaatacatcgtcattcttcttgatgacataaataatggctccttcctgaaaggacagctcatcttccttgtcttttgtatagtcataaattgccacaaccttttccaagtaagaacgtggagcccacggtgggtcctcttcagcataaggatcactatactcaaccacagcagcttcctcctcttcgtaatcttctggaggaggaggaggtgggggagactcatcaaagactggttcttccacaggtggcggtggaggtggtgtatctgaaatattttcttggactctggccacaaatcccattaaaggtaactgaggagttacctgtaggatggagggaggaggaggagcaagagatactggattctggctataaaaaggtcctccattcatctgattctgaaggcttgtttgtgaagtaatggaaggagggcgtctatagggcaacgagccccctattgttgggggagtatggcgagaggcaggcctattcatgctgtagaactgtacaggatgacctgtagggggagtggaagaaacaacagggggagttggagaagtgaagccatcagcaagggtctgggcacccccagcagcagcgtctggggcagtggaggaagggacagtagcaggaacaagaggagcaggggcagatgcagaagtagcaggaaggggaggagtgccagcagagccagcaggggctggaaagacactgggaggagatggagtaggaacagcaataggaacccccacactaccacttccactgttctctcgactgctgctccgactacttgggtggctccctccactactcccactgctgtaagttcgatttctttgattcacagaagctgtcctcacagggctctgctgcgagggagccatattacgggttgggctaggtacgtaatcatttggtaccactggaggacgcactggctccagtgtgcgatagggggagtgccgcccaagtgtccctttccctgacatagggggactagggggcttctgagttggaggtgttgtacgcggcagcccacccatcttcatgttctgggtactcaccttaaatctaagcaaccactttactccatgtccaatatcatctagaattgtatagtcaataggttttctaatataacgaactggtcgttcaaggttggctggagcaataatcttatgtgtccttgaagtgtttttattggtagtcaaaataccaatttctcttcttgcaactttctctttatgaatatcaactgtttgtgaaatatgattgattgaagattccatccttcgtagctgggatgcctggatatccagcatctgcaggacattgttggccaaggtgtttatcagataggcaacacttgctaaggattgggtggtgtaggctttggtttcttctagggctctctgcttatctgctgactgtatgtagttgttctcgcagtaatcggccacccgttccagatttgtgtagctgtcgaagagggcccggcggccccccgggatttcctcttccagcagcatctgcagctccgccatcttcacatcctcctcctcctcctcctcatacaggtcgcagagggagcggcggccgcagcgccaaggaaacccaggaccgggagaggaggagcggcggcgacggcggcggtaactcggaagg

SEQ ID NO: 11774 - RNA, 3806 nt, Homo sapiens
  source 1..3806: mol_type = other RNA
ctgaatagctgggactacaggtgtgcgccaccacgcccagctaatttttgtgtttttagtagagatggggtttcaccatgttggccaggatggtctcaatttattgacctcatgatccacccacctcggcctccgaaagtgctgggattacaggcataagccaccacacccagcctgtgggaactatttattggatttcaaaacaccctctgcctcattaatccactaagctttctcagcaaaaagctgtttaaataaataatgggaacatctaatttaaaacagtttttctaattatagaccagtacacgaagaagagcttaacttatccaagtatagtctagtttgggtccataatggagctgaaggctcagaggacattcagggccattacactgcaggaaaacaaggaataagggatgtagaaatgacctaagaaaagcacgaagtggaatgtatactggaggcaagttaatgaaagctaataaatacaaagtgctgggaaaaatctaaaagcaaaatagctattgtaacttgcaatgcattaaaaacaactttaaaaccaaaaagtcttgataaggaaactctatagtggggtctcagttaaatgctgatgatttttaatgctcagataacattaagtggaatattaacttctgcatccgacaccatctgaattttctcacacactactacacttgttcacttttcaatcaagttccactttctgaacttgttcaaaacctcatttgaaatatatccagctactgcttttcccctttcacctagcacagggcagttacctggcaaagctctattctggccaagtcactgggactgagtagaacccacgttagcagctctggacctgaacaggagctggcccaacatcacagtgaccacccacaaagagacaagccctcctggatttttttcagcatttcttatactgactacagtagtgatgattaaagttatctgccctacagactccactgaatttgaagctgtatttattgtacagatgggggaaatgtgttttattgtgtcagttatattaatttttatcaatgtgattagatacatattttggcctattaatcttattcattatattcttagtctgagatgggttttaattctgactaacagcagctacttaagagtccaatcatacaaaatcaggagagtattaccctttctacagctaagcgagtcagtaatacagcagcaactaatactggccattaataacgtccagagagcacattagcaaaccttgtactcccagtgactgtcaggagacttgaaaataactactattctcttccaaagtagaatagcgtttttctagatagtgaaggaaatgatagtcatagttggtctgaactccaagatcctactcctcaaaacagcaccgaagcaggggttcgggatgcctgctaagagcatttccacagttcaagtctcttcagaaccttagggaccttcgtgtctagcttcacacacccacctccacatatgaaccagcctaccacacttcacatctgggtacactggccattagcaacaatgcagtctcatgcagcagcacattaaaatcaaacgggtggcaatcgttcaccaccctcagagtgttgggagactttcacatttcatcatccttataatccacaaacagaaacatgaagggatgcaagtgagttcagcattcactcgtttggtgcactcaagtgctgagagaatgcagaatttacagtgtcacagaggaaaaaagccatctgaaataattgtaaaaatggttaagtgtggtatttaaatgttggttccctcctcttcatacaagtggaagaaaagaaggggctagggtacccactgggccatgaggttaaccccttagcacaggcaatgaagaacatccaatgccacagattctgcaggaggagaaatcccaagggtatacagtattcctgagaaagatcccagatttttctgaatcagtcttaatctgattttgttttggctacacagttatgctgttatacctttgacatacataaaaatggtcattttatttcaatccagacagctcagcattgtacaaatgatggcagaaagatccatttgttcagactcagcttgctttgtttttaatactggggaataaaccaaaaaaaaaagtgtaatttttatcatttgtatccttcattctactttactggagtggaatccccagggccttcagataatctgggaagacctgactattcctgtgaggcaagcacagccctgctgagctttactcagaataatgcatgatagactcaacgtaattcccaggaaaaagcccagtcactccattcataactccctcataccaaccatcgtcattcttcttgatgacataaataatggctccttcctgaaaggacagctcatcttccttgtcttttgtatagtcataaattgccacaaccttttccaagtaagaacgtggagcccacggtgggtcctcttcagcataaggatcactatactcaaccacagcagcttcctcctcttcgtaatcttctggaggaggaggaggtgggggagactcatcaaagactggttcttccacaggtggcggtggaggtggtgtatctgaaacatgtccacaatagccatggtgtctaatatttgttcttgccctctctggattctggctataaaaaggtcctccattcatctgattctgaaggcttgtttgtgaagtaatggaaggagggcgtctatagggcaacgagccccctattgttgggggagtatggcgagaggcaggcctattcatgctgtagaactgtacaggatgacctggaaagacactgggaggagatggagtaggaacagcaataggaacccccacactaccacttccactgttctctcgactgctgctccgactacttgggtggctccctccactactcccactgctgctgtaagttcgatttctttgattcacagaagctgtcctcacagggctctgctgcgagggagccatattacgggttgggctaggtacgtaatcatttggtaccactggaggacgcactggctccagtgtgcgatagggggagtgccgcccaagtgtccctttccctgacatagggggactagggggcttctgagttggaggtgttgtacgcggcagcccacccatcttcatgttctgggtactcacctttactccatgtccaatatcatctagaattgtatagtcaataggttttctaatataacgaactggtcgttcaaggttggctggagcaataatcttatgtgtccttgaagtgtttttattggtagtcaaaataccaatttctcttcttgcaactttctctttatgaatatcaactgtttgtgaaatatgattgattgaagattccatccttcgtagctgggatgcctggatatccagcatctgcaggacattgttggccaaggtgtttatcagataggcaacacttgctaaggattgggtggtgtaggctttggtttcttctagggctctctgcttatctgctgactgtatgtagttgttctcgcagtaatcggccacccgttccagatttgtgtagctgtcgaagagggcccggcggccccccgggatttcctcttccagcagcatctgcagctccgccatcttcacatcctcctcctcctcctcctcatacaggtcgcagagggagcggcggccgcagcgccaaggaaacccaggaccgggagaggaggagcggcggcgacggcggcggtaactcggaagg

SEQ ID NO: 11775 - RNA, 3860 nt, Homo sapiens
  source 1..3860: mol_type = other RNA
ctgaatagctgggactacaggtgtgcgccaccacgcccagctaatttttgtgtttttagtagagatggggtttcaccatgttggccaggatggtctcaatttattgacctcatgatccacccacctcggcctccgaaagtgctgggattacaggcataagccaccacacccagcctgtgggaactatttattggatttcaaaacaccctctgcctcattaatccactaagctttctcagcaaaaagctgtttaaataaataatgggaacatctaatttaaaacagtttttctaattatagaccagtacacgaagaagagcttaacttatccaagtatagtctagtttgggtccataatggagctgaaggctcagaggacattcagggccattacactgcaggaaaacaaggaataagggatgtagaaatgacctaagaaaagcacgaagtggaatgtatactggaggcaagttaatgaaagctaataaatacaaagtgctgggaaaaatctaaaagcaaaatagctattgtaacttgcaatgcattaaaaacaactttaaaaccaaaaagtcttgataaggaaactctatagtggggtctcagttaaatgctgatgatttttaatgctcagataacattaagtggaatattaacttctgcatccgacaccatctgaattttctcacacactactacacttgttcacttttcaatcaagttccactttctgaacttgttcaaaacctcatttgaaatatatccagctactgcttttcccctttcacctagcacagggcagttacctggcaaagctctattctggccaagtcactgggactgagtagaacccacgttagcagctctggacctgaacaggagctggcccaacatcacagtgaccacccacaaagagacaagccctcctggatttttttcagcatttcttatactgactacagtagtgatgattaaagttatctgccctacagactccactgaatttgaagctgtatttattgtacagatgggggaaatgtgttttattgtgtcagttatattaatttttatcaatgtgattagatacatattttggcctattaatcttattcattatattcttagtctgagatgggttttaattctgactaacagcagctacttaagagtccaatcatacaaaatcaggagagtattaccctttctacagctaagcgagtcagtaatacagcagcaactaatactggccattaataacgtccagagagcacattagcaaaccttgtactcccagtgactgtcaggagacttgaaaataactactattctcttccaaagtagaatagcgtttttctagatagtgaaggaaatgatagtcatagttggtctgaactccaagatcctactcctcaaaacagcaccgaagcaggggttcgggatgcctgctaagagcatttccacagttcaagtctcttcagaaccttagggaccttcgtgtctagcttcacacacccacctccacatatgaaccagcctaccacacttcacatctgggtacactggccattagcaacaatgcagtctcatgcagcagcacattaaaatcaaacgggtggcaatcgttcaccaccctcagagtgttgggagactttcacatttcatcatccttataatccacaaacagaaacatgaagggatgcaagtgagttcagcattcactcgtttggtgcactcaagtgctgagagaatgcagaatttacagtgtcacagaggaaaaaagccatctgaaataattgtaaaaatggttaagtgtggtatttaaatgttggttccctcctcttcatacaagtggaagaaaagaaggggctagggtacccactgggccatgaggttaaccccttagcacaggcaatgaagaacatccaatgccacagattctgcaggaggagaaatcccaagggtatacagtattcctgagaaagatcccagatttttctgaatcagtcttaatctgattttgttttggctacacagttatgctgttatacctttgacatacataaaaatggtcattttatttcaatccagacagctcagcattgtacaaatgatggcagaaagatccatttgttcagactcagcttgctttgtttttaatactggggaataaaccaaaaaaaaaagtgtaatttttatcatttgtatccttcattctactttactggagtggaatccccagggccttcagataatctgggaagacctgactattcctgtgaggcaagcacagccctgctgagctttactcagaataatgcatgatagactcaacgtaattcccaggaaaaagcccagtcactccattcataactccctcataccaaccatcgtcattcttcttgatgacataaataatggctccttcctgaaaggacagctcatcttccttgtcttttgtatagtcataaattgccacaaccttttccaagtaagaacgtggagcccacggtgggtcctcttcagcataaggatcactatactcaaccacagcagcttcctcctcttcgtaatcttctggaggaggaggaggtgggggagactcatcaaagactggttcttccacaggtggcggtggaggtggtgtatctgaaacatgtccacaatagccatggtgtctaatatttgttcttgccctctctggattctggctataaaaaggtcctccattcatctgattctgaaggcttgtttgtgaagtaatggaaggagggcgtctatagggcaacgagccccctattgttgggggagtatggcgagaggcaggcctattcatgctgtagaactgtacaggatgacctgtagggggagtggaagaaacaacagggggagttggagaagtgaagccatcagcaagggtctgggcacccccagcagcagcgtctggggcagtggaggaagggacagtagcaggaacaagaggagcaggggcagatgcagaagtagcaggaaggggaggagtgccagcagagccagcaggggctggaaagacactgggaggagatggagtaggaacagcaataggaacccccacactaccacttccactgttctctcgactgctgctccgactacttgggtggctccctccactactcccactgctgccaagtgtccctttccctgacatagggggactagggggcttctgagttggaggtgttgtacgcggcagcccacccatcttcatgttctgggtactcaccttaaatctaagcaaccactttactccatgtccaatatcatctagaattgtatagtcaataggttttctaatataacgaactggtcgttcaaggttggctggagcaataatcttatgtgtccttgaagtgtttttattggtagtcaaaataccaatttctcttcttgcaactttctctttatgaatatcaactgtttgtgaaatatgattgattgaagattccatccttcgtagctgggatgcctggatatccagcatctgcaggacattgttggccaaggtgtttatcagataggcaacacttgctaaggattgggtggtgtaggctttggtttcttctagggctctctgcttatctgctgactgtatgtagttgttctcgcagtaatcggccacccgttccagatttgtgtagctgtcgaagagggcccggcggccccccgggatttcctcttccagcagcatctgcagctccgccatcttcacatcctcctcctcctcctcctcatacaggtcgcagagggagcggcggccgcagcgccaaggaaacccaggaccgggagaggaggagcggcggcgacggcggcggtaactcggaagg

SEQ ID NO: 11776 - RNA, 3489 nt, Homo sapiens
  source 1..3489: mol_type = other RNA
ctgaatagctgggactacaggtgtgcgccaccacgcccagctaatttttgtgtttttagtagagatggggtttcaccatgttggccaggatggtctcaatttattgacctcatgatccacccacctcggcctccgaaagtgctgggattacaggcataagccaccacacccagcctgtgggaactatttattggatttcaaaacaccctctgcctcattaatccactaagctttctcagcaaaaagctgtttaaataaataatgggaacatctaatttaaaacagtttttctaattatagaccagtacacgaagaagagcttaacttatccaagtatagtctagtttgggtccataatggagctgaaggctcagaggacattcagggccattacactgcaggaaaacaaggaataagggatgtagaaatgacctaagaaaagcacgaagtggaatgtatactggaggcaagttaatgaaagctaataaatacaaagtgctgggaaaaatctaaaagcaaaatagctattgtaacttgcaatgcattaaaaacaactttaaaaccaaaaagtcttgataaggaaactctatagtggggtctcagttaaatgctgatgatttttaatgctcagataacattaagtggaatattaacttctgcatccgacaccatctgaattttctcacacactactacacttgttcacttttcaatcaagttccactttctgaacttgttcaaaacctcatttgaaatatatccagctactgcttttcccctttcacctagcacagggcagttacctggcaaagctctattctggccaagtcactgggactgagtagaacccacgttagcagctctggacctgaacaggagctggcccaacatcacagtgaccacccacaaagagacaagccctcctggatttttttcagcatttcttatactgactacagtagtgatgattaaagttatctgccctacagactccactgaatttgaagctgtatttattgtacagatgggggaaatgtgttttattgtgtcagttatattaatttttatcaatgtgattagatacatattttggcctattaatcttattcattatattcttagtctgagatgggttttaattctgactaacagcagctacttaagagtccaatcatacaaaatcaggagagtattaccctttctacagctaagcgagtcagtaatacagcagcaactaatactggccattaataacgtccagagagcacattagcaaaccttgtactcccagtgactgtcaggagacttgaaaataactactattctcttccaaagtagaatagcgtttttctagatagtgaaggaaatgatagtcatagttggtctgaactccaagatcctactcctcaaaacagcaccgaagcaggggttcgggatgcctgctaagagcatttccacagttcaagtctcttcagaaccttagggaccttcgtgtctagcttcacacacccacctccacatatgaaccagcctaccacacttcacatctgggtacactggccattagcaacaatgcagtctcatgcagcagcacattaaaatcaaacgggtggcaatcgttcaccaccctcagagtgttgggagactttcacatttcatcatccttataatccacaaacagaaacatgaagggatgcaagtgagttcagcattcactcgtttggtgcactcaagtgctgagagaatgcagaatttacagtgtcacagaggaaaaaagccatctgaaataattgtaaaaatggttaagtgtggtatttaaatgttggttccctcctcttcatacaagtggaagaaaagaaggggctagggtacccactgggccatgaggttaaccccttagcacaggcaatgaagaacatccaatgccacagattctgcaggaggagaaatcccaagggtatacagtattcctgagaaagatcccagatttttctgaatcagtcttaatctgattttgttttggctacacagttatgctgttatacctttgacatacataaaaatggtcattttatttcaatccagacagctcagcattgtacaaatgatggcagaaagatccatttgttcagactcagcttgctttgtttttaatactggggaataaaccaaaaaaaaaagtgtaatttttatcatttgtatccttcattctactttactggagtggaatccccagggccttcagataatctgggaagacctgactattcctgtgaggcaagcacagccctgctgagctttactcagaataatgcatgatagactcaacgtaattcccaggaaaaagcccagtcactccattcataactccctcataccaaccatcgtcattcttcttgatgacataaataatggctccttcctgaaaggacagctcatcttccttgtcttttgtatagtcataaattgccacaaccttttccaagtaagaacgtggagcccacggtgggtcctcttcagcataaggatcactatactcaaccacagcagcttcctcctcttcgtaatcttctggaggaggaggaggtgggggagactcatcaaagactggttcttccacaggtggcggtggaggtggtgtatctgaaactggattctggctataaaaaggtcctccattcatctgattctgaaggcttgtttgtgaagtaatggaaggagggcgtctatagggcaacgagccccctattgttgggggagtatggcgagaggcaggcctattcatgctgtagaactgtacaggatgacccaagtgtccctttccctgacatagggggactagggggcttctgagttggaggtgttgtacgcggcagcccacccatcttcatgttctgggtactcacctttactccatgtccaatatcatctagaattgtatagtcaataggttttctaatataacgaactggtcgttcaaggttggctggagcaataatcttatgtgtccttgaagtgtttttattggtagtcaaaataccaatttctcttcttgcaactttctctttatgaatatcaactgtttgtgaaatatgattgattgaagattccatccttcgtagctgggatgcctggatatccagcatctgcaggacattgttggccaaggtgtttatcagataggcaacacttgctaaggattgggtggtgtaggctttggtttcttctagggctctctgcttatctgctgactgtatgtagttgttctcgcagtaatcggccacccgttccagatttgtgtagctgtcgaagagggcccggcggccccccgggatttcctcttccagcagcatctgcagctccgccatcttcacatcctcctcctcctcctcctcatacaggtcgcagagggagcggcggccgcagcgccaaggaaacccaggaccgggagaggaggagcggcggcgacggcggcggtaactcggaagg

SEQ ID NO: 11777 - RNA, 3611 nt, Homo sapiens
  source 1..3611: mol_type = other RNA
ctgaatagctgggactacaggtgtgcgccaccacgcccagctaatttttgtgtttttagtagagatggggtttcaccatgttggccaggatggtctcaatttattgacctcatgatccacccacctcggcctccgaaagtgctgggattacaggcataagccaccacacccagcctgtgggaactatttattggatttcaaaacaccctctgcctcattaatccactaagctttctcagcaaaaagctgtttaaataaataatgggaacatctaatttaaaacagtttttctaattatagaccagtacacgaagaagagcttaacttatccaagtatagtctagtttgggtccataatggagctgaaggctcagaggacattcagggccattacactgcaggaaaacaaggaataagggatgtagaaatgacctaagaaaagcacgaagtggaatgtatactggaggcaagttaatgaaagctaataaatacaaagtgctgggaaaaatctaaaagcaaaatagctattgtaacttgcaatgcattaaaaacaactttaaaaccaaaaagtcttgataaggaaactctatagtggggtctcagttaaatgctgatgatttttaatgctcagataacattaagtggaatattaacttctgcatccgacaccatctgaattttctcacacactactacacttgttcacttttcaatcaagttccactttctgaacttgttcaaaacctcatttgaaatatatccagctactgcttttcccctttcacctagcacagggcagttacctggcaaagctctattctggccaagtcactgggactgagtagaacccacgttagcagctctggacctgaacaggagctggcccaacatcacagtgaccacccacaaagagacaagccctcctggatttttttcagcatttcttatactgactacagtagtgatgattaaagttatctgccctacagactccactgaatttgaagctgtatttattgtacagatgggggaaatgtgttttattgtgtcagttatattaatttttatcaatgtgattagatacatattttggcctattaatcttattcattatattcttagtctgagatgggttttaattctgactaacagcagctacttaagagtccaatcatacaaaatcaggagagtattaccctttctacagctaagcgagtcagtaatacagcagcaactaatactggccattaataacgtccagagagcacattagcaaaccttgtactcccagtgactgtcaggagacttgaaaataactactattctcttccaaagtagaatagcgtttttctagatagtgaaggaaatgatagtcatagttggtctgaactccaagatcctactcctcaaaacagcaccgaagcaggggttcgggatgcctgctaagagcatttccacagttcaagtctcttcagaaccttagggaccttcgtgtctagcttcacacacccacctccacatatgaaccagcctaccacacttcacatctgggtacactggccattagcaacaatgcagtctcatgcagcagcacattaaaatcaaacgggtggcaatcgttcaccaccctcagagtgttgggagactttcacatttcatcatccttataatccacaaacagaaacatgaagggatgcaagtgagttcagcattcactcgtttggtgcactcaagtgctgagagaatgcagaatttacagtgtcacagaggaaaaaagccatctgaaataattgtaaaaatggttaagtgtggtatttaaatgttggttccctcctcttcatacaagtggaagaaaagaaggggctagggtacccactgggccatgaggttaaccccttagcacaggcaatgaagaacatccaatgccacagattctgcaggaggagaaatcccaagggtatacagtattcctgagaaagatcccagatttttctgaatcagtcttaatctgattttgttttggctacacagttatgctgttatacctttgacatacataaaaatggtcattttatttcaatccagacagctcagcattgtacaaatgatggcagaaagatccatttgttcagactcagcttgctttgtttttaatactggggaataaaccaaaaaaaaaagtgtaatttttatcatttgtatccttcattctactttactggagtggaatccccagggccttcagataatctgggaagacctgactattcctgtgaggcaagcacagccctgctgagctttactcagaataatgcatgatagactcaacgtaattcccaggaaaaagcccagtcactccattcataactccctcataccaaccatcgtcattcttcttgatgacataaataatggctccttcctgaaaggacagctcatcttccttgtcttttgtatagtcataaattgccacaaccttttccaagtaagaacgtggagcccacggtgggtcctcttcagcataaggatcactatactcaaccacagcagcttcctcctcttcgtaatcttctggaggaggaggaggtgggggagactcatcaaagactggttcttccacaggtggcggtggaggtggtgtatctgaaactggattctggctataaaaaggtcctccattcatctgattctgaaggcttgtttgtgaagtaatggaaggagggcgtctatagggcaacgagccccctattgttgggggagtatggcgagaggcaggcctattcatgctgtagaactgtacaggatgacctggaaagacactgggaggagatggagtaggaacagcaataggaacccccacactaccacttccactgttctctcgactgctgctccgactacttgggtggctccctccactactcccactgccaagtgtccctttccctgacatagggggactagggggcttctgagttggaggtgttgtacgcggcagcccacccatcttcatgttctgggtactcacctttactccatgtccaatatcatctagaattgtatagtcaataggttttctaatataacgaactggtcgttcaaggttggctggagcaataatcttatgtgtccttgaagtgtttttattggtagtcaaaataccaatttctcttcttgcaactttctctttatgaatatcaactgtttgtgaaatatgattgattgaagattccatccttcgtagctgggatgcctggatatccagcatctgcaggacattgttggccaaggtgtttatcagataggcaacacttgctaaggattgggtggtgtaggctttggtttcttctagggctctctgcttatctgctgactgtatgtagttgttctcgcagtaatcggccacccgttccagatttgtgtagctgtcgaagagggcccggcggccccccgggatttcctcttccagcagcatctgcagctccgccatcttcacatcctcctcctcctcctcctcatacaggtcgcagagggagcggcggccgcagcgccaaggaaacccaggaccgggagaggaggagcggcggcgacggcggcggtaactcggaagg

SEQ ID NO: 11778 - RNA, 4152 nt, Homo sapiens
  source 1..4152: mol_type = other RNA
ctgaatagctgggactacaggtgtgcgccaccacgcccagctaatttttgtgtttttagtagagatggggtttcaccatgttggccaggatggtctcaatttattgacctcatgatccacccacctcggcctccgaaagtgctgggattacaggcataagccaccacacccagcctgtgggaactatttattggatttcaaaacaccctctgcctcattaatccactaagctttctcagcaaaaagctgtttaaataaataatgggaacatctaatttaaaacagtttttctaattatagaccagtacacgaagaagagcttaacttatccaagtatagtctagtttgggtccataatggagctgaaggctcagaggacattcagggccattacactgcaggaaaacaaggaataagggatgtagaaatgacctaagaaaagcacgaagtggaatgtatactggaggcaagttaatgaaagctaataaatacaaagtgctgggaaaaatctaaaagcaaaatagctattgtaacttgcaatgcattaaaaacaactttaaaaccaaaaagtcttgataaggaaactctatagtggggtctcagttaaatgctgatgatttttaatgctcagataacattaagtggaatattaacttctgcatccgacaccatctgaattttctcacacactactacacttgttcacttttcaatcaagttccactttctgaacttgttcaaaacctcatttgaaatatatccagctactgcttttcccctttcacctagcacagggcagttacctggcaaagctctattctggccaagtcactgggactgagtagaacccacgttagcagctctggacctgaacaggagctggcccaacatcacagtgaccacccacaaagagacaagccctcctggatttttttcagcatttcttatactgactacagtagtgatgattaaagttatctgccctacagactccactgaatttgaagctgtatttattgtacagatgggggaaatgtgttttattgtgtcagttatattaatttttatcaatgtgattagatacatattttggcctattaatcttattcattatattcttagtctgagatgggttttaattctgactaacagcagctacttaagagtccaatcatacaaaatcaggagagtattaccctttctacagctaagcgagtcagtaatacagcagcaactaatactggccattaataacgtccagagagcacattagcaaaccttgtactcccagtgactgtcaggagacttgaaaataactactattctcttccaaagtagaatagcgtttttctagatagtgaaggaaatgatagtcatagttggtctgaactccaagatcctactcctcaaaacagcaccgaagcaggggttcgggatgcctgctaagagcatttccacagttcaagtctcttcagaaccttagggaccttcgtgtctagcttcacacacccacctccacatatgaaccagcctaccacacttcacatctgggtacactggccattagcaacaatgcagtctcatgcagcagcacattaaaatcaaacgggtggcaatcgttcaccaccctcagagtgttgggagactttcacatttcatcatccttataatccacaaacagaaacatgaagggatgcaagtgagttcagcattcactcgtttggtgcactcaagtgctgagagaatgcagaatttacagtgtcacagaggaaaaaagccatctgaaataattgtaaaaatggttaagtgtggtatttaaatgttggttccctcctcttcatacaagtggaagaaaagaaggggctagggtacccactgggccatgaggttaaccccttagcacaggcaatgaagaacatccaatgccacagattctgcaggaggagaaatcccaagggtatacagtattcctgagaaagatcccagatttttctgaatcagtcttaatctgattttgttttggctacacagttatgctgttatacctttgacatacataaaaatggtcattttatttcaatccagacagctcagcattgtacaaatgatggcagaaagatccatttgttcagactcagcttgctttgtttttaatactggggaataaaccaaaaaaaaaagtgtaatttttatcatttgtatccttcattctactttactggagtggaatccccagggccttcagataatctgggaagacctgactattcctgtgaggcaagcacagccctgctgagctttactcagaataatgcatgatagactcaacgtaattcccaggaaaaagcccagtcactccattcataactccctcataccaaccatcgtcattcttcttgatgacataaataatggctccttcctgaaaggacagctcatcttccttgtcttttgtatagtcataaattgccacaaccttttccaagtaagaacgtggagcccacggtgggtcctcttcagcataaggatcactatactcaaccacagcagcttcctcctcttcgtaatcttctggaggaggaggaggtgggggagactcatcaaagactggttcttccacaggtggcggtggaggtggtgtatctgaaactggattctggctataaaaaggtcctccattcatctgattctgaaggcttgtttgtgaagtaatggaaggagggcgtctatagggcaacgagccccctattgttgggggagtatggcgagaggcaggcctattcatgctgtagaactgtacaggatgacctggaaagacactgggaggagatggagtaggaacagcaataggaacccccacactaccacttccactgttctctcgactgctgctccgactacttgggtggctccctccactactcccactgctgccaagtgtccctttccctgacatagggggactagggggcttctgagttggaggtgttgtacgcggcagcccacccatcttcatgttctgggtactcaccttaaatctaagcaaccactttactccatgtccaatatcatctagaattgtatagtcaataggttttctaatataacgaactggtcgttcaaggttggctggagcaataatcttatgtgtccttgaagtgtttttattggtagtcaaaataccaatttctcttcttgcaactttctctttatgaatatcaactgtttgtgaaatatgattgattgaagattccatccttcgtagctgggatgcctggatatccagcatctgcaggacattgttggccaaggtgtttatcagataggcaacacttgctaaggattgggtggtgtaggctttggtttcttctagggctctctgcttatctgctgactgtatgtagttgttctcgcagtaatcggccacccgttccagatttgtgtagctgtcgaagagggcccggcggccccccgggatttcctcttccagcagcatctgcagctccgccatcttcacatcctcctcctcctcctcctcatacaggtcgcagagggagcggcggccgcagcgccaaggaaacccaggaccgggagaggaggagcggcggcgacggcggcggtaactcggaaggagcgagaaacagccccagcgcgcgacaggggagggggcgacgggggcggggcgcgagccgacggactccgaggacggtcaccgcggcgacggccggccgggcgcgcgcacgcgcgctcccttccctccgcccccgggagcccgaaaaagattcccaccctcgcccgcgccgccggcccctcccccacttccggcgtctcctagcgacggcgggggtaggggccgggatgcgcgcgggagttggtggtgcagttaacccttccgccgcccgcccgccgctggagcggctggagaagcccccacctcccggcggcctttgttagcccggcgggaacacaccaccctgctcagctggcttcctgccggctccctccgggactcatctcggctccgtccccatggaggtcatcggcctagggaacttctcgaggcttttctccctctgctgctgacgggaggccgaaggagggcacagcctccactcttgggaccctcctctgtgaaagatcacacctcaacag

SEQ ID NO: 11779 - RNA, 3446 nt, Homo sapiens
  source 1..3446: mol_type = other RNA
ctgaatagctgggactacaggtgtgcgccaccacgcccagctaatttttgtgtttttagtagagatggggtttcaccatgttggccaggatggtctcaatttattgacctcatgatccacccacctcggcctccgaaagtgctgggattacaggcataagccaccacacccagcctgtgggaactatttattggatttcaaaacaccctctgcctcattaatccactaagctttctcagcaaaaagctgtttaaataaataatgggaacatctaatttaaaacagtttttctaattatagaccagtacacgaagaagagcttaacttatccaagtatagtctagtttgggtccataatggagctgaaggctcagaggacattcagggccattacactgcaggaaaacaaggaataagggatgtagaaatgacctaagaaaagcacgaagtggaatgtatactggaggcaagttaatgaaagctaataaatacaaagtgctgggaaaaatctaaaagcaaaatagctattgtaacttgcaatgcattaaaaacaactttaaaaccaaaaagtcttgataaggaaactctatagtggggtctcagttaaatgctgatgatttttaatgctcagataacattaagtggaatattaacttctgcatccgacaccatctgaattttctcacacactactacacttgttcacttttcaatcaagttccactttctgaacttgttcaaaacctcatttgaaatatatccagctactgcttttcccctttcacctagcacagggcagttacctggcaaagctctattctggccaagtcactgggactgagtagaacccacgttagcagctctggacctgaacaggagctggcccaacatcacagtgaccacccacaaagagacaagccctcctggatttttttcagcatttcttatactgactacagtagtgatgattaaagttatctgccctacagactccactgaatttgaagctgtatttattgtacagatgggggaaatgtgttttattgtgtcagttatattaatttttatcaatgtgattagatacatattttggcctattaatcttattcattatattcttagtctgagatgggttttaattctgactaacagcagctacttaagagtccaatcatacaaaatcaggagagtattaccctttctacagctaagcgagtcagtaatacagcagcaactaatactggccattaataacgtccagagagcacattagcaaaccttgtactcccagtgactgtcaggagacttgaaaataactactattctcttccaaagtagaatagcgtttttctagatagtgaaggaaatgatagtcatagttggtctgaactccaagatcctactcctcaaaacagcaccgaagcaggggttcgggatgcctgctaagagcatttccacagttcaagtctcttcagaaccttagggaccttcgtgtctagcttcacacacccacctccacatatgaaccagcctaccacacttcacatctgggtacactggccattagcaacaatgcagtctcatgcagcagcacattaaaatcaaacgggtggcaatcgttcaccaccctcagagtgttgggagactttcacatttcatcatccttataatccacaaacagaaacatgaagggatgcaagtgagttcagcattcactcgtttggtgcactcaagtgctgagagaatgcagaatttacagtgtcacagaggaaaaaagccatctgaaataattgtaaaaatggttaagtgtggtatttaaatgttggttccctcctcttcatacaagtggaagaaaagaaggggctagggtacccactgggccatgaggttaaccccttagcacaggcaatgaagaacatccaatgccacagattctgcaggaggagaaatcccaagggtatacagtattcctgagaaagatcccagatttttctgaatcagtcttaatctgattttgttttggctacacagttatgctgttatacctttgacatacataaaaatggtcattttatttcaatccagacagctcagcattgtacaaatgatggcagaaagatccatttgttcagactcagcttgctttgtttttaatactggggaataaaccaaaaaaaaaagtgtaatttttatcatttgtatccttcattctactttactggagtggaatccccagggccttcagataatctgggaagacctgactattcctgtgaggcaagcacagccctgctgagctttactcagaataatgcatgatagactcaacgtaattcccaggaaaaagcccagtcactccattcataactccctcataccaaccatcgtcattcttcttgatgacataaataatggctccttcctgaaaggacagctcatcttccttgtcttttgtatagtcataaattgccacaaccttttccaagtaagaacgtggagcccacggtgggtcctcttcagcataaggatcactatactcaaccacagcagcttcctcctcttcgtaatcttctggaggaggaggaggtgggggagactcatcaaagactggttcttccacaggtggcggtggaggtggtgtatctgaaactggattctggctataaaaaggtcctccattcatctgattctgaaggcttgtttgtgaagtaatggaaggagggcgtctatagggcaacgagccccctattgttgggggagtatggcgagaggcaggcctattcatgctgtagaactgtacaggatgacctggaaagacactgggaggagatggagtaggaacagcaataggaacccccacactaccacttccactgttctctcgactgctgctccgactacttgggtggctccctccactactcccactgctgccaagtgtccctttccctgacatagggggactagggggcttctgagttggaggtgttgtacgcggcagcccacccatcttcatgttctgggtactcacctttactccatgtccaatatcatctagaattgtatagtcaataggttttctaatataacgaactggtcgttcaaggttggctggagcaataatcttatgtgtccttgaagtgtttttattggtagtcaaaataccaatttctcttcttgcaactttctctttatgaatatcaactgtctgtatgtagttgttctcgcagtaatcggccacccgttccagatttgtgtagctgtcgaagagggcccggcggccccccgggatttcctcttccagcagcatctgcagctccgccatcttcacatcctcctcctcctcctcctcatacaggtcgcagagggagcggcggccgcagcgccaaggaaacccaggaccgggagaggaggagcggcggcgacggcggcggtaactcggaagg

SEQ ID NO: 11780 - RNA, 3614 nt, Homo sapiens
  source 1..3614: mol_type = other RNA
ctgaatagctgggactacaggtgtgcgccaccacgcccagctaatttttgtgtttttagtagagatggggtttcaccatgttggccaggatggtctcaatttattgacctcatgatccacccacctcggcctccgaaagtgctgggattacaggcataagccaccacacccagcctgtgggaactatttattggatttcaaaacaccctctgcctcattaatccactaagctttctcagcaaaaagctgtttaaataaataatgggaacatctaatttaaaacagtttttctaattatagaccagtacacgaagaagagcttaacttatccaagtatagtctagtttgggtccataatggagctgaaggctcagaggacattcagggccattacactgcaggaaaacaaggaataagggatgtagaaatgacctaagaaaagcacgaagtggaatgtatactggaggcaagttaatgaaagctaataaatacaaagtgctgggaaaaatctaaaagcaaaatagctattgtaacttgcaatgcattaaaaacaactttaaaaccaaaaagtcttgataaggaaactctatagtggggtctcagttaaatgctgatgatttttaatgctcagataacattaagtggaatattaacttctgcatccgacaccatctgaattttctcacacactactacacttgttcacttttcaatcaagttccactttctgaacttgttcaaaacctcatttgaaatatatccagctactgcttttcccctttcacctagcacagggcagttacctggcaaagctctattctggccaagtcactgggactgagtagaacccacgttagcagctctggacctgaacaggagctggcccaacatcacagtgaccacccacaaagagacaagccctcctggatttttttcagcatttcttatactgactacagtagtgatgattaaagttatctgccctacagactccactgaatttgaagctgtatttattgtacagatgggggaaatgtgttttattgtgtcagttatattaatttttatcaatgtgattagatacatattttggcctattaatcttattcattatattcttagtctgagatgggttttaattctgactaacagcagctacttaagagtccaatcatacaaaatcaggagagtattaccctttctacagctaagcgagtcagtaatacagcagcaactaatactggccattaataacgtccagagagcacattagcaaaccttgtactcccagtgactgtcaggagacttgaaaataactactattctcttccaaagtagaatagcgtttttctagatagtgaaggaaatgatagtcatagttggtctgaactccaagatcctactcctcaaaacagcaccgaagcaggggttcgggatgcctgctaagagcatttccacagttcaagtctcttcagaaccttagggaccttcgtgtctagcttcacacacccacctccacatatgaaccagcctaccacacttcacatctgggtacactggccattagcaacaatgcagtctcatgcagcagcacattaaaatcaaacgggtggcaatcgttcaccaccctcagagtgttgggagactttcacatttcatcatccttataatccacaaacagaaacatgaagggatgcaagtgagttcagcattcactcgtttggtgcactcaagtgctgagagaatgcagaatttacagtgtcacagaggaaaaaagccatctgaaataattgtaaaaatggttaagtgtggtatttaaatgttggttccctcctcttcatacaagtggaagaaaagaaggggctagggtacccactgggccatgaggttaaccccttagcacaggcaatgaagaacatccaatgccacagattctgcaggaggagaaatcccaagggtatacagtattcctgagaaagatcccagatttttctgaatcagtcttaatctgattttgttttggctacacagttatgctgttatacctttgacatacataaaaatggtcattttatttcaatccagacagctcagcattgtacaaatgatggcagaaagatccatttgttcagactcagcttgctttgtttttaatactggggaataaaccaaaaaaaaaagtgtaatttttatcatttgtatccttcattctactttactggagtggaatccccagggccttcagataatctgggaagacctgactattcctgtgaggcaagcacagccctgctgagctttactcagaataatgcatgatagactcaacgtaattcccaggaaaaagcccagtcactccattcataactccctcataccaaccatcgtcattcttcttgatgacataaataatggctccttcctgaaaggacagctcatcttccttgtcttttgtatagtcataaattgccacaaccttttccaagtaagaacgtggagcccacggtgggtcctcttcagcataaggatcactatactcaaccacagcagcttcctcctcttcgtaatcttctggaggaggaggaggtgggggagactcatcaaagactggttcttccacaggtggcggtggaggtggtgtatctgaaactggattctggctataaaaaggtcctccattcatctgattctgaaggcttgtttgtgaagtaatggaaggagggcgtctatagggcaacgagccccctattgttgggggagtatggcgagaggcaggcctattcatgctgtagaactgtacaggatgacctggaaagacactgggaggagatggagtaggaacagcaataggaacccccacactaccacttccactgttctctcgactgctgctccgactacttgggtggctccctccactactcccactgctgccaagtgtccctttccctgacatagggggactagggggcttctgagttggaggtgttgtacgcggcagcccacccatcttcatgttctgggtactcacctttactccatgtccaatatcatctagaattgtatagtcaataggttttctaatataacgaactggtcgttcaaggttggctggagcaataatcttatgtgtccttgaagtgtttttattggtagtcaaaataccaatttctcttcttgcaactttctctttatgaatatcaactgtttgtgaaatatgattgattgaagattccatccttcgtagctgggatgcctggatatccagcatctgcaggacattgttggccaaggtgtttatcagataggcaacacttgctaaggattgggtggtgtaggctttggtttcttctagggctctctgcttatctgctgactgtatgtagttgttctcgcagtaatcggccacccgttccagatttgtgtagctgtcgaagagggcccggcggccccccgggatttcctcttccagcagcatctgcagctccgccatcttcacatcctcctcctcctcctcctcatacaggtcgcagagggagcggcggccgcagcgccaaggaaacccaggaccgggagaggaggagcggcggcgacggcggcggtaactcggaagg

SEQ ID NO: 11781 - RNA, 3668 nt, Homo sapiens
  source 1..3668: mol_type = other RNA
ctgaatagctgggactacaggtgtgcgccaccacgcccagctaatttttgtgtttttagtagagatggggtttcaccatgttggccaggatggtctcaatttattgacctcatgatccacccacctcggcctccgaaagtgctgggattacaggcataagccaccacacccagcctgtgggaactatttattggatttcaaaacaccctctgcctcattaatccactaagctttctcagcaaaaagctgtttaaataaataatgggaacatctaatttaaaacagtttttctaattatagaccagtacacgaagaagagcttaacttatccaagtatagtctagtttgggtccataatggagctgaaggctcagaggacattcagggccattacactgcaggaaaacaaggaataagggatgtagaaatgacctaagaaaagcacgaagtggaatgtatactggaggcaagttaatgaaagctaataaatacaaagtgctgggaaaaatctaaaagcaaaatagctattgtaacttgcaatgcattaaaaacaactttaaaaccaaaaagtcttgataaggaaactctatagtggggtctcagttaaatgctgatgatttttaatgctcagataacattaagtggaatattaacttctgcatccgacaccatctgaattttctcacacactactacacttgttcacttttcaatcaagttccactttctgaacttgttcaaaacctcatttgaaatatatccagctactgcttttcccctttcacctagcacagggcagttacctggcaaagctctattctggccaagtcactgggactgagtagaacccacgttagcagctctggacctgaacaggagctggcccaacatcacagtgaccacccacaaagagacaagccctcctggatttttttcagcatttcttatactgactacagtagtgatgattaaagttatctgccctacagactccactgaatttgaagctgtatttattgtacagatgggggaaatgtgttttattgtgtcagttatattaatttttatcaatgtgattagatacatattttggcctattaatcttattcattatattcttagtctgagatgggttttaattctgactaacagcagctacttaagagtccaatcatacaaaatcaggagagtattaccctttctacagctaagcgagtcagtaatacagcagcaactaatactggccattaataacgtccagagagcacattagcaaaccttgtactcccagtgactgtcaggagacttgaaaataactactattctcttccaaagtagaatagcgtttttctagatagtgaaggaaatgatagtcatagttggtctgaactccaagatcctactcctcaaaacagcaccgaagcaggggttcgggatgcctgctaagagcatttccacagttcaagtctcttcagaaccttagggaccttcgtgtctagcttcacacacccacctccacatatgaaccagcctaccacacttcacatctgggtacactggccattagcaacaatgcagtctcatgcagcagcacattaaaatcaaacgggtggcaatcgttcaccaccctcagagtgttgggagactttcacatttcatcatccttataatccacaaacagaaacatgaagggatgcaagtgagttcagcattcactcgtttggtgcactcaagtgctgagagaatgcagaatttacagtgtcacagaggaaaaaagccatctgaaataattgtaaaaatggttaagtgtggtatttaaatgttggttccctcctcttcatacaagtggaagaaaagaaggggctagggtacccactgggccatgaggttaaccccttagcacaggcaatgaagaacatccaatgccacagattctgcaggaggagaaatcccaagggtatacagtattcctgagaaagatcccagatttttctgaatcagtcttaatctgattttgttttggctacacagttatgctgttatacctttgacatacataaaaatggtcattttatttcaatccagacagctcagcattgtacaaatgatggcagaaagatccatttgttcagactcagcttgctttgtttttaatactggggaataaaccaaaaaaaaaagtgtaatttttatcatttgtatccttcattctactttactggagtggaatccccagggccttcagataatctgggaagacctgactattcctgtgaggcaagcacagccctgctgagctttactcagaataatgcatgatagactcaacgtaattcccaggaaaaagcccagtcactccattcataactccctcataccaaccatcgtcattcttcttgatgacataaataatggctccttcctgaaaggacagctcatcttccttgtcttttgtatagtcataaattgccacaaccttttccaagtaagaacgtggagcccacggtgggtcctcttcagcataaggatcactatactcaaccacagcagcttcctcctcttcgtaatcttctggaggaggaggaggtgggggagactcatcaaagactggttcttccacaggtggcggtggaggtggtgtatctgaaactggattctggctataaaaaggtcctccattcatctgattctgaaggcttgtttgtgaagtaatggaaggagggcgtctatagggcaacgagccccctattgttgggggagtatggcgagaggcaggcctattcatgctgtagaactgtacaggatgacctggaaagacactgggaggagatggagtaggaacagcaataggaacccccacactaccacttccactgttctctcgactgctgctccgactacttgggtggctccctccactactcccactgctgctgtaagttcgatttctttgattcacagaagctgtcctcacagggctctgctgcgagggagccatattacgggttgggctaggtacgtaatcatttggtaccactggaggacgcactggctccagtgtgcgatagggggagtgccgcccaagtgtccctttccctgacatagggggactagggggcttctgagttggaggtgttgtacgcggcagcccacccatcttcatgttctgggtactcaccatgactgaggatttggaaccaacaatccaatcaataatacaggtgtccatatgcctgggctcttccaatcaaatctttactccatgtccaatatcatctagaattgtatagtcaataggttttctaatataacgaactggtcgttcaaggttggctggagcaataatcttatgtgtccttgaagtgtttttattggtagtcaaaataccaatttctcttcttgcaactttctctttatgaatatcaactgtctgtatgtagttgttctcgcagtaatcggccacccgttccagatttgtgtagctgtcgaagagggcccggcggccccccgggatttcctcttccagcagcatctgcagctccgccatcttcacatcctcctcctcctcctcctcatacaggtcgcagagggagcggcggccgcagcgccaaggaaacccaggaccgggagaggaggagcggcggcgacggcggcggtaactcggaagg

SEQ ID NO: 11782 - RNA, 3832 nt, Homo sapiens
  source 1..3832: mol_type = other RNA
ctgaatagctgggactacaggtgtgcgccaccacgcccagctaatttttgtgtttttagtagagatggggtttcaccatgttggccaggatggtctcaatttattgacctcatgatccacccacctcggcctccgaaagtgctgggattacaggcataagccaccacacccagcctgtgggaactatttattggatttcaaaacaccctctgcctcattaatccactaagctttctcagcaaaaagctgtttaaataaataatgggaacatctaatttaaaacagtttttctaattatagaccagtacacgaagaagagcttaacttatccaagtatagtctagtttgggtccataatggagctgaaggctcagaggacattcagggccattacactgcaggaaaacaaggaataagggatgtagaaatgacctaagaaaagcacgaagtggaatgtatactggaggcaagttaatgaaagctaataaatacaaagtgctgggaaaaatctaaaagcaaaatagctattgtaacttgcaatgcattaaaaacaactttaaaaccaaaaagtcttgataaggaaactctatagtggggtctcagttaaatgctgatgatttttaatgctcagataacattaagtggaatattaacttctgcatccgacaccatctgaattttctcacacactactacacttgttcacttttcaatcaagttccactttctgaacttgttcaaaacctcatttgaaatatatccagctactgcttttcccctttcacctagcacagggcagttacctggcaaagctctattctggccaagtcactgggactgagtagaacccacgttagcagctctggacctgaacaggagctggcccaacatcacagtgaccacccacaaagagacaagccctcctggatttttttcagcatttcttatactgactacagtagtgatgattaaagttatctgccctacagactccactgaatttgaagctgtatttattgtacagatgggggaaatgtgttttattgtgtcagttatattaatttttatcaatgtgattagatacatattttggcctattaatcttattcattatattcttagtctgagatgggttttaattctgactaacagcagctacttaagagtccaatcatacaaaatcaggagagtattaccctttctacagctaagcgagtcagtaatacagcagcaactaatactggccattaataacgtccagagagcacattagcaaaccttgtactcccagtgactgtcaggagacttgaaaataactactattctcttccaaagtagaatagcgtttttctagatagtgaaggaaatgatagtcatagttggtctgaactccaagatcctactcctcaaaacagcaccgaagcaggggttcgggatgcctgctaagagcatttccacagttcaagtctcttcagaaccttagggaccttcgtgtctagcttcacacacccacctccacatatgaaccagcctaccacacttcacatctgggtacactggccattagcaacaatgcagtctcatgcagcagcacattaaaatcaaacgggtggcaatcgttcaccaccctcagagtgttgggagactttcacatttcatcatccttataatccacaaacagaaacatgaagggatgcaagtgagttcagcattcactcgtttggtgcactcaagtgctgagagaatgcagaatttacagtgtcacagaggaaaaaagccatctgaaataattgtaaaaatggttaagtgtggtatttaaatgttggttccctcctcttcatacaagtggaagaaaagaaggggctagggtacccactgggccatgaggttaaccccttagcacaggcaatgaagaacatccaatgccacagattctgcaggaggagaaatcccaagggtatacagtattcctgagaaagatcccagatttttctgaatcagtcttaatctgattttgttttggctacacagttatgctgttatacctttgacatacataaaaatggtcattttatttcaatccagacagctcagcattgtacaaatgatggcagaaagatccatttgttcagactcagcttgctttgtttttaatactggggaataaaccaaaaaaaaaagtgtaatttttatcatttgtatccttcattctactttactggagtggaatccccagggccttcagataatctgggaagacctgactattcctgtgaggcaagcacagccctgctgagctttactcagaataatgcatgatagactcaacgtaattcccaggaaaaagcccagtcactccattcataactccctcataccaaccatcgtcattcttcttgatgacataaataatggctccttcctgaaaggacagctcatcttccttgtcttttgtatagtcataaattgccacaaccttttccaagtaagaacgtggagcccacggtgggtcctcttcagcataaggatcactatactcaaccacagcagcttcctcctcttcgtaatcttctggaggaggaggaggtgggggagactcatcaaagactggttcttccacaggtggcggtggaggtggtgtatctgaaactggattctggctataaaaaggtcctccattcatctgattctgaaggcttgtttgtgaagtaatggaaggagggcgtctatagggcaacgagccccctattgttgggggagtatggcgagaggcaggcctattcatgctgtagaactgtacaggatgacctggaaagacactgggaggagatggagtaggaacagcaataggaacccccacactaccacttccactgttctctcgactgctgctccgactacttgggtggctccctccactactcccactgctgctgtaagttcgatttctttgattcacagaagctgtcctcacagggctctgctgcgagggagccatattacgggttgggctaggtacgtaatcatttggtaccactggaggacgcactggctccagtgtgcgatagggggagtgccgcccaagtgtccctttccctgacatagggggactagggggcttctgagttggaggtgttgtacgcggcagcccacccatcttcatgttctgggtactcaccatgactgaggatttggaaccaacaatccaatcaataatacaggtgtccatatgcctgggctcttccaatcaaatctttactccatgtccaatatcatctagaattgtatagtcaataggttttctaatataacgaactggtcgttcaaggttggctggagcaataatcttatgtgtccttgaagtgtttttattggtagtcaaaataccaatttctcttcttgcaactttctctttatgaatatcaactgtttgtgaaatatgattgattgaagattccatccttcgtagctgggatgcctggatatccagcatctgcaggacattgttggccaaggtgtttatcagataggcaacacttgctaaggattgggtggtgtaggctttggtttcttctagggctctctgcttatctgctgtatgtagttgttctcgcagtaatcggccacccgttccagatttgtgtagctgtcgaagagggcccggcggccccccgggatttcctcttccagcagcatctgcagctccgccatcttcacatcctcctcctcctcctcctcatacaggtcgcagagggagcggcggccgcagcgccaaggaaacccaggaccgggagaggaggagcggcggcgacggcggcggtaactcggaagg

SEQ ID NO: 11783 - RNA, 4299 nt, Homo sapiens
  source 1..4299: mol_type = other RNA
ctgaatagctgggactacaggtgtgcgccaccacgcccagctaatttttgtgtttttagtagagatggggtttcaccatgttggccaggatggtctcaatttattgacctcatgatccacccacctcggcctccgaaagtgctgggattacaggcataagccaccacacccagcctgtgggaactatttattggatttcaaaacaccctctgcctcattaatccactaagctttctcagcaaaaagctgtttaaataaataatgggaacatctaatttaaaacagtttttctaattatagaccagtacacgaagaagagcttaacttatccaagtatagtctagtttgggtccataatggagctgaaggctcagaggacattcagggccattacactgcaggaaaacaaggaataagggatgtagaaatgacctaagaaaagcacgaagtggaatgtatactggaggcaagttaatgaaagctaataaatacaaagtgctgggaaaaatctaaaagcaaaatagctattgtaacttgcaatgcattaaaaacaactttaaaaccaaaaagtcttgataaggaaactctatagtggggtctcagttaaatgctgatgatttttaatgctcagataacattaagtggaatattaacttctgcatccgacaccatctgaattttctcacacactactacacttgttcacttttcaatcaagttccactttctgaacttgttcaaaacctcatttgaaatatatccagctactgcttttcccctttcacctagcacagggcagttacctggcaaagctctattctggccaagtcactgggactgagtagaacccacgttagcagctctggacctgaacaggagctggcccaacatcacagtgaccacccacaaagagacaagccctcctggatttttttcagcatttcttatactgactacagtagtgatgattaaagttatctgccctacagactccactgaatttgaagctgtatttattgtacagatgggggaaatgtgttttattgtgtcagttatattaatttttatcaatgtgattagatacatattttggcctattaatcttattcattatattcttagtctgagatgggttttaattctgactaacagcagctacttaagagtccaatcatacaaaatcaggagagtattaccctttctacagctaagcgagtcagtaatacagcagcaactaatactggccattaataacgtccagagagcacattagcaaaccttgtactcccagtgactgtcaggagacttgaaaataactactattctcttccaaagtagaatagcgtttttctagatagtgaaggaaatgatagtcatagttggtctgaactccaagatcctactcctcaaaacagcaccgaagcaggggttcgggatgcctgctaagagcatttccacagttcaagtctcttcagaaccttagggaccttcgtgtctagcttcacacacccacctccacatatgaaccagcctaccacacttcacatctgggtacactggccattagcaacaatgcagtctcatgcagcagcacattaaaatcaaacgggtggcaatcgttcaccaccctcagagtgttgggagactttcacatttcatcatccttataatccacaaacagaaacatgaagggatgcaagtgagttcagcattcactcgtttggtgcactcaagtgctgagagaatgcagaatttacagtgtcacagaggaaaaaagccatctgaaataattgtaaaaatggttaagtgtggtatttaaatgttggttccctcctcttcatacaagtggaagaaaagaaggggctagggtacccactgggccatgaggttaaccccttagcacaggcaatgaagaacatccaatgccacagattctgcaggaggagaaatcccaagggtatacagtattcctgagaaagatcccagatttttctgaatcagtcttaatctgattttgttttggctacacagttatgctgttatacctttgacatacataaaaatggtcattttatttcaatccagacagctcagcattgtacaaatgatggcagaaagatccatttgttcagactcagcttgctttgtttttaatactggggaataaaccaaaaaaaaaagtgtaatttttatcatttgtatccttcattctactttactggagtggaatccccagggccttcagataatctgggaagacctgactattcctgtgaggcaagcacagccctgctgagctttactcagaataatgcatgatagactcaacgtaattcccaggaaaaagcccagtcactccattcataactccctcataccaaccatcgtcattcttcttgatgacataaataatggctccttcctgaaaggacagctcatcttccttgtcttttgtatagtcataaattgccacaaccttttccaagtaagaacgtggagcccacggtgggtcctcttcagcataaggatcactatactcaaccacagcagcttcctcctcttcgtaatcttctggaggaggaggaggtgggggagactcatcaaagactggttcttccacaggtggcggtggaggtggtgtatctgaaactggattctggctataaaaaggtcctccattcatctgattctgaaggcttgtttgtgaagtaatggaaggagggcgtctatagggcaacgagccccctattgttgggggagtatggcgagaggcaggcctattcatgctgtagaactgtacaggatgacctggaaagacactgggaggagatggagtaggaacagcaataggaacccccacactaccacttccactgttctctcgactgctgctccgactacttgggtggctccctccactactcccactgctgctgtaagttcgatttctttgattcacagaagctgtcctcacagggctctgctgcgagggagccatattacgggttgggctaggtacgtaatcatttggtaccactggaggacgcactggctccagtgtgcgatagggggagtgccgcccaagtgtccctttccctgacatagggggactagggggcttctgagttggaggtgttgtacgcggcagcccacccatcttcatgttctgggtactcaccttaaatctaagcaaccactttactccatgtccaatatcatctagaattgtatagtcaataggttttctaatataacgaactggtcgttcaaggttggctggagcaataatcttatgtgtccttgaagtgtttttattggtagtcaaaataccaatttctcttcttgcaactttctctttatgaatatcaactgtttgtgaaatatgattgattgaagattccatccttcgtagctgggatgcctggatatccagcatctgcaggacattgttggccaaggtgtttatcagataggcaacacttgctaaggattgggtggtgtaggctttggtttcttctagggctctctgcttatctgctgactgtatgtagttgttctcgcagtaatcggccacccgttccagatttgtgtagctgtcgaagagggcccggcggccccccgggatttcctcttccagcagcatctgcagctccgccatcttcacatcctcctcctcctcctcctcatacaggtcgcagagggagcggcggccgcagcgccaaggaaacccaggaccgggagaggaggagcggcggcgacggcggcggtaactcggaaggagcgagaaacagccccagcgcgcgacaggggagggggcgacgggggcggggcgcgagccgacggactccgaggacggtcaccgcggcgacggccggccgggcgcgcgcacgcgcgctcccttccctccgcccccgggagcccgaaaaagattcccaccctcgcccgcgccgccggcccctcccccacttccggcgtctcctagcgacggcgggggtaggggccgggatgcgcgcgggagttggtggtgcagttaacccttccgccgcccgcccgccgctggagcggctggagaagcccccacctcccggcggcctttgttagcccggcgggaacacaccaccctgctcagctggcttcctgccggctccctccgggactcatctcggctccgtccccatggaggtcatcggcctagggaacttctcgaggcttttctccctctgctgctgacgggaggccgaaggagggcacagcctccactcttgggaccctcctctgtgaaagatcacacctcaacag

SEQ ID NO: 11784 - RNA, 3958 nt, Homo sapiens
  source 1..3958: mol_type = other RNA
ctgaatagctgggactacaggtgtgcgccaccacgcccagctaatttttgtgtttttagtagagatggggtttcaccatgttggccaggatggtctcaatttattgacctcatgatccacccacctcggcctccgaaagtgctgggattacaggcataagccaccacacccagcctgtgggaactatttattggatttcaaaacaccctctgcctcattaatccactaagctttctcagcaaaaagctgtttaaataaataatgggaacatctaatttaaaacagtttttctaattatagaccagtacacgaagaagagcttaacttatccaagtatagtctagtttgggtccataatggagctgaaggctcagaggacattcagggccattacactgcaggaaaacaaggaataagggatgtagaaatgacctaagaaaagcacgaagtggaatgtatactggaggcaagttaatgaaagctaataaatacaaagtgctgggaaaaatctaaaagcaaaatagctattgtaacttgcaatgcattaaaaacaactttaaaaccaaaaagtcttgataaggaaactctatagtggggtctcagttaaatgctgatgatttttaatgctcagataacattaagtggaatattaacttctgcatccgacaccatctgaattttctcacacactactacacttgttcacttttcaatcaagttccactttctgaacttgttcaaaacctcatttgaaatatatccagctactgcttttcccctttcacctagcacagggcagttacctggcaaagctctattctggccaagtcactgggactgagtagaacccacgttagcagctctggacctgaacaggagctggcccaacatcacagtgaccacccacaaagagacaagccctcctggatttttttcagcatttcttatactgactacagtagtgatgattaaagttatctgccctacagactccactgaatttgaagctgtatttattgtacagatgggggaaatgtgttttattgtgtcagttatattaatttttatcaatgtgattagatacatattttggcctattaatcttattcattatattcttagtctgagatgggttttaattctgactaacagcagctacttaagagtccaatcatacaaaatcaggagagtattaccctttctacagctaagcgagtcagtaatacagcagcaactaatactggccattaataacgtccagagagcacattagcaaaccttgtactcccagtgactgtcaggagacttgaaaataactactattctcttccaaagtagaatagcgtttttctagatagtgaaggaaatgatagtcatagttggtctgaactccaagatcctactcctcaaaacagcaccgaagcaggggttcgggatgcctgctaagagcatttccacagttcaagtctcttcagaaccttagggaccttcgtgtctagcttcacacacccacctccacatatgaaccagcctaccacacttcacatctgggtacactggccattagcaacaatgcagtctcatgcagcagcacattaaaatcaaacgggtggcaatcgttcaccaccctcagagtgttgggagactttcacatttcatcatccttataatccacaaacagaaacatgaagggatgcaagtgagttcagcattcactcgtttggtgcactcaagtgctgagagaatgcagaatttacagtgtcacagaggaaaaaagccatctgaaataattgtaaaaatggttaagtgtggtatttaaatgttggttccctcctcttcatacaagtggaagaaaagaaggggctagggtacccactgggccatgaggttaaccccttagcacaggcaatgaagaacatccaatgccacagattctgcaggaggagaaatcccaagggtatacagtattcctgagaaagatcccagatttttctgaatcagtcttaatctgattttgttttggctacacagttatgctgttatacctttgacatacataaaaatggtcattttatttcaatccagacagctcagcattgtacaaatgatggcagaaagatccatttgttcagactcagcttgctttgtttttaatactggggaataaaccaaaaaaaaaagtgtaatttttatcatttgtatccttcattctactttactggagtggaatccccagggccttcagataatctgggaagacctgactattcctgtgaggcaagcacagccctgctgagctttactcagaataatgcatgatagactcaacgtaattcccaggaaaaagcccagtcactccattcataactccctcataccaaccatcgtcattcttcttgatgacataaataatggctccttcctgaaaggacagctcatcttccttgtcttttgtatagtcataaattgccacaaccttttccaagtaagaacgtggagcccacggtgggtcctcttcagcataaggatcactatactcaaccacagcagcttcctcctcttcgtaatcttctggaggaggaggaggtgggggagactcatcaaagactggttcttccacaggtggcggtggaggtggtgtatctgaaactggattctggctataaaaaggtcctccattcatctgattctgaaggcttgtttgtgaagtaatggaaggagggcgtctatagggcaacgagccccctattgttgggggagtatggcgagaggcaggcctattcatgctgtagaactgtacaggatgacctggaaagacactgggaggagatggagtaggaacagcaataggaacccccacactaccacttccactgttctctcgactgctgctccgactacttgggtggctccctccactactcccactgctgctgtaagttcgatttctttgattcacagaagctgtcctcacagggctctgctgcgagggagccatattacgggttgggctaggtacgtaatcatttggtaccactggaggacgcactggctccagtgtgcgatagggggagtgccgcccaagtgtccctttccctgacatagggggactagggggcttctgagttggaggtgttgtacgcggcagcccacccatcttcatgttctgggtactcacctttactccatgtccaatatcatctagaattgtatagtcaataggttttctaatataacgaactggtcgttcaaggttggctggagcaataatcttatgtgtccttgaagtgtttttattggtagtcaaaataccaatttctcttcttgcaactttctctttatgaatatcaactgtctcattcaatctcaaactgcaattgtttccaaatttggtcacaaaagtcgactcaagatcaacgcctctaatttgcctaagtatagatattttaagtaaataacttttaaaaaacatctataataataaaggtaatctaacaacggtataatttgcattcttgccatcatactaccacacggggttgaactgcagtattgcttgtgaaatatgattgattgaagattccatccttcgtagctgggatgcctggatatccagcatctgcaggacattgttggccaaggtgtttatcagataggcaacacttgctaaggattgggtggtgtaggctttggtttcttctagggctctctgcttatctgctgtatgtagttgttctcgcagtaatcggccacccgttccagatttgtgtagctgtcgaagagggcccggcggccccccgggatttcctcttccagcagcatctgcagctccgccatcttcacatcctcctcctcctcctcctcatacaggtcgcagagggagcggcggccgcagcgccaaggaaacccaggaccgggagaggaggagcggcggcgacggcggcggtaactcggaagg

SEQ ID NO: 11785 - RNA, 3837 nt, Homo sapiens
  source 1..3837: mol_type = other RNA
ctgaatagctgggactacaggtgtgcgccaccacgcccagctaatttttgtgtttttagtagagatggggtttcaccatgttggccaggatggtctcaatttattgacctcatgatccacccacctcggcctccgaaagtgctgggattacaggcataagccaccacacccagcctgtgggaactatttattggatttcaaaacaccctctgcctcattaatccactaagctttctcagcaaaaagctgtttaaataaataatgggaacatctaatttaaaacagtttttctaattatagaccagtacacgaagaagagcttaacttatccaagtatagtctagtttgggtccataatggagctgaaggctcagaggacattcagggccattacactgcaggaaaacaaggaataagggatgtagaaatgacctaagaaaagcacgaagtggaatgtatactggaggcaagttaatgaaagctaataaatacaaagtgctgggaaaaatctaaaagcaaaatagctattgtaacttgcaatgcattaaaaacaactttaaaaccaaaaagtcttgataaggaaactctatagtggggtctcagttaaatgctgatgatttttaatgctcagataacattaagtggaatattaacttctgcatccgacaccatctgaattttctcacacactactacacttgttcacttttcaatcaagttccactttctgaacttgttcaaaacctcatttgaaatatatccagctactgcttttcccctttcacctagcacagggcagttacctggcaaagctctattctggccaagtcactgggactgagtagaacccacgttagcagctctggacctgaacaggagctggcccaacatcacagtgaccacccacaaagagacaagccctcctggatttttttcagcatttcttatactgactacagtagtgatgattaaagttatctgccctacagactccactgaatttgaagctgtatttattgtacagatgggggaaatgtgttttattgtgtcagttatattaatttttatcaatgtgattagatacatattttggcctattaatcttattcattatattcttagtctgagatgggttttaattctgactaacagcagctacttaagagtccaatcatacaaaatcaggagagtattaccctttctacagctaagcgagtcagtaatacagcagcaactaatactggccattaataacgtccagagagcacattagcaaaccttgtactcccagtgactgtcaggagacttgaaaataactactattctcttccaaagtagaatagcgtttttctagatagtgaaggaaatgatagtcatagttggtctgaactccaagatcctactcctcaaaacagcaccgaagcaggggttcgggatgcctgctaagagcatttccacagttcaagtctcttcagaaccttagggaccttcgtgtctagcttcacacacccacctccacatatgaaccagcctaccacacttcacatctgggtacactggccattagcaacaatgcagtctcatgcagcagcacattaaaatcaaacgggtggcaatcgttcaccaccctcagagtgttgggagactttcacatttcatcatccttataatccacaaacagaaacatgaagggatgcaagtgagttcagcattcactcgtttggtgcactcaagtgctgagagaatgcagaatttacagtgtcacagaggaaaaaagccatctgaaataattgtaaaaatggttaagtgtggtatttaaatgttggttccctcctcttcatacaagtggaagaaaagaaggggctagggtacccactgggccatgaggttaaccccttagcacaggcaatgaagaacatccaatgccacagattctgcaggaggagaaatcccaagggtatacagtattcctgagaaagatcccagatttttctgaatcagtcttaatctgattttgttttggctacacagttatgctgttatacctttgacatacataaaaatggtcattttatttcaatccagacagctcagcattgtacaaatgatggcagaaagatccatttgttcagactcagcttgctttgtttttaatactggggaataaaccaaaaaaaaaagtgtaatttttatcatttgtatccttcattctactttactggagtggaatccccagggccttcagataatctgggaagacctgactattcctgtgaggcaagcacagccctgctgagctttactcagaataatgcatgatagactcaacgtaattcccaggaaaaagcccagtcactccattcataactccctcataccaaccatcgtcattcttcttgatgacataaataatggctccttcctgaaaggacagctcatcttccttgtcttttgtatagtcataaattgccacaaccttttccaagtaagaacgtggagcccacggtgggtcctcttcagcataaggatcactatactcaaccacagcagcttcctcctcttcgtaatcttctggaggaggaggaggtgggggagactcatcaaagactggttcttccacaggtggcggtggaggtggtgtatctgaaactggattctggctataaaaaggtcctccattcatctgattctgaaggcttgtttgtgaagtaatggaaggagggcgtctatagggcaacgagccccctattgttgggggagtatggcgagaggcaggcctattcatgctgtagaactgtacaggatgacctggaaagacactgggaggagatggagtaggaacagcaataggaacccccacactaccacttccactgttctctcgactgctgctccgactacttgggtggctccctccactactcccactgctgctgtaagttcgatttctttgattcacagaagctgtcctcacagggctctgctgcgagggagccatattacgggttgggctaggtacgtaatcatttggtaccactggaggacgcactggctccagtgtgcgatagggggagtgccgcccaagtgtccctttccctgacatagggggactagggggcttctgagttggaggtgttgtacgcggcagcccacccatcttcatgttctgggtactcacctttactccatgtccaatatcatctagaattgtatagtcaataggttttctaatataacgaactggtcgttcaaggttggctggagcaataatcttatgtgtccttgaagtgtttttattggtagtcaaaataccaatttctcttcttgcaactttctctttatgaatatcaactgtctcattcaatctcaaactgcaattgtttccaaatttggtcacaaaagtcgactcaagatcaacgcctctaatttgcttgtgaaatatgattgattgaagattccatccttcgtagctgggatgcctggatatccagcatctgcaggacattgttggccaaggtgtttatcagataggcaacacttgctaaggattgggtggtgtaggctttggtttcttctagggctctctgcttatctgctgactgtatgtagttgttctcgcagtaatcggccacccgttccagatttgtgtagctgtcgaagagggcccggcggccccccgggatttcctcttccagcagcatctgcagctccgccatcttcacatcctcctcctcctcctcctcatacaggtcgcagagggagcggcggccgcagcgccaaggaaacccaggaccgggagaggaggagcggcggcgacggcggcggtaactcggaagg

SEQ ID NO: 11786 - RNA, 3833 nt, Homo sapiens
  source 1..3833: mol_type = other RNA
ctgaatagctgggactacaggtgtgcgccaccacgcccagctaatttttgtgtttttagtagagatggggtttcaccatgttggccaggatggtctcaatttattgacctcatgatccacccacctcggcctccgaaagtgctgggattacaggcataagccaccacacccagcctgtgggaactatttattggatttcaaaacaccctctgcctcattaatccactaagctttctcagcaaaaagctgtttaaataaataatgggaacatctaatttaaaacagtttttctaattatagaccagtacacgaagaagagcttaacttatccaagtatagtctagtttgggtccataatggagctgaaggctcagaggacattcagggccattacactgcaggaaaacaaggaataagggatgtagaaatgacctaagaaaagcacgaagtggaatgtatactggaggcaagttaatgaaagctaataaatacaaagtgctgggaaaaatctaaaagcaaaatagctattgtaacttgcaatgcattaaaaacaactttaaaaccaaaaagtcttgataaggaaactctatagtggggtctcagttaaatgctgatgatttttaatgctcagataacattaagtggaatattaacttctgcatccgacaccatctgaattttctcacacactactacacttgttcacttttcaatcaagttccactttctgaacttgttcaaaacctcatttgaaatatatccagctactgcttttcccctttcacctagcacagggcagttacctggcaaagctctattctggccaagtcactgggactgagtagaacccacgttagcagctctggacctgaacaggagctggcccaacatcacagtgaccacccacaaagagacaagccctcctggatttttttcagcatttcttatactgactacagtagtgatgattaaagttatctgccctacagactccactgaatttgaagctgtatttattgtacagatgggggaaatgtgttttattgtgtcagttatattaatttttatcaatgtgattagatacatattttggcctattaatcttattcattatattcttagtctgagatgggttttaattctgactaacagcagctacttaagagtccaatcatacaaaatcaggagagtattaccctttctacagctaagcgagtcagtaatacagcagcaactaatactggccattaataacgtccagagagcacattagcaaaccttgtactcccagtgactgtcaggagacttgaaaataactactattctcttccaaagtagaatagcgtttttctagatagtgaaggaaatgatagtcatagttggtctgaactccaagatcctactcctcaaaacagcaccgaagcaggggttcgggatgcctgctaagagcatttccacagttcaagtctcttcagaaccttagggaccttcgtgtctagcttcacacacccacctccacatatgaaccagcctaccacacttcacatctgggtacactggccattagcaacaatgcagtctcatgcagcagcacattaaaatcaaacgggtggcaatcgttcaccaccctcagagtgttgggagactttcacatttcatcatccttataatccacaaacagaaacatgaagggatgcaagtgagttcagcattcactcgtttggtgcactcaagtgctgagagaatgcagaatttacagtgtcacagaggaaaaaagccatctgaaataattgtaaaaatggttaagtgtggtatttaaatgttggttccctcctcttcatacaagtggaagaaaagaaggggctagggtacccactgggccatgaggttaaccccttagcacaggcaatgaagaacatccaatgccacagattctgcaggaggagaaatcccaagggtatacagtattcctgagaaagatcccagatttttctgaatcagtcttaatctgattttgttttggctacacagttatgctgttatacctttgacatacataaaaatggtcattttatttcaatccagacagctcagcattgtacaaatgatggcagaaagatccatttgttcagactcagcttgctttgtttttaatactggggaataaaccaaaaaaaaaagtgtaatttttatcatttgtatccttcattctactttactggagtggaatccccagggccttcagataatctgggaagacctgactattcctgtgaggcaagcacagccctgctgagctttactcagaataatgcatgatagactcaacgtaattcccaggaaaaagcccagtcactccattcataactccctcataccaaccatcgtcattcttcttgatgacataaataatggctccttcctgaaaggacagctcatcttccttgtcttttgtatagtcataaattgccacaaccttttccaagtaagaacgtggagcccacggtgggtcctcttcagcataaggatcactatactcaaccacagcagcttcctcctcttcgtaatcttctggaggaggaggaggtgggggagactcatcaaagactggttcttccacaggtggcggtggaggtggtgtatctgaaactggattctggctataaaaaggtcctccattcatctgattctgaaggcttgtttgtgaagtaatggaaggagggcgtctatagggcaacgagccccctattgttgggggagtatggcgagaggcaggcctattcatgctgtagaactgtacaggatgacctggaaagacactgggaggagatggagtaggaacagcaataggaacccccacactaccacttccactgttctctcgactgctgctccgactacttgggtggctccctccactactcccactgctgctgtaagttcgatttctttgattcacagaagctgtcctcacagggctctgctgcgagggagccatattacgggttgggctaggtacgtaatcatttggtaccactggaggacgcactggctccagtgtgcgatagggggagtgccgcccaagtgtccctttccctgacatagggggactagggggcttctgagttggaggtgttgtacgcggcagcccacccatcttcatgttctgggtactcacctttactccatgtccaatatcatctagaattgtatagtcaataggttttctaatataacgaactggtcgttcaaggttggctggagcaataatcttatgtgtccttgaagtgtttttattggtagtcaaaataccaatttctcttcttgcaactttctctttatgaatatcaactgtctcattcaatctcaaactgcaattgtttccaaatttggtcacaaaagtcgactcaagatcaacgcctctaatttgcttgtgaaatatgattgattgaagattccatccttcgtagctgggatgcctggatatccagcatctgcaggacattgttggccaaggtgtttatcagataggcaacacttgctaaggattgggtggtgtaggctttggtttcttctagggctctctgcttatctgctgtatgtagttgttctcgcagtaatcggccacccgttccagatttgtgtagctgtcgaagagggcccggcggccccccgggatttcctcttccagcagcatctgcagctccgccatcttcacatcctcctcctcctcctcctcatacaggtcgcagagggagcggcggccgcagcgccaaggaaacccaggaccgggagaggaggagcggcggcgacggcggcggtaactcggaagg

SEQ ID NO: 11787 - RNA, 3593 nt, Homo sapiens
  source 1..3593: mol_type = other RNA
ctgaatagctgggactacaggtgtgcgccaccacgcccagctaatttttgtgtttttagtagagatggggtttcaccatgttggccaggatggtctcaatttattgacctcatgatccacccacctcggcctccgaaagtgctgggattacaggcataagccaccacacccagcctgtgggaactatttattggatttcaaaacaccctctgcctcattaatccactaagctttctcagcaaaaagctgtttaaataaataatgggaacatctaatttaaaacagtttttctaattatagaccagtacacgaagaagagcttaacttatccaagtatagtctagtttgggtccataatggagctgaaggctcagaggacattcagggccattacactgcaggaaaacaaggaataagggatgtagaaatgacctaagaaaagcacgaagtggaatgtatactggaggcaagttaatgaaagctaataaatacaaagtgctgggaaaaatctaaaagcaaaatagctattgtaacttgcaatgcattaaaaacaactttaaaaccaaaaagtcttgataaggaaactctatagtggggtctcagttaaatgctgatgatttttaatgctcagataacattaagtggaatattaacttctgcatccgacaccatctgaattttctcacacactactacacttgttcacttttcaatcaagttccactttctgaacttgttcaaaacctcatttgaaatatatccagctactgcttttcccctttcacctagcacagggcagttacctggcaaagctctattctggccaagtcactgggactgagtagaacccacgttagcagctctggacctgaacaggagctggcccaacatcacagtgaccacccacaaagagacaagccctcctggatttttttcagcatttcttatactgactacagtagtgatgattaaagttatctgccctacagactccactgaatttgaagctgtatttattgtacagatgggggaaatgtgttttattgtgtcagttatattaatttttatcaatgtgattagatacatattttggcctattaatcttattcattatattcttagtctgagatgggttttaattctgactaacagcagctacttaagagtccaatcatacaaaatcaggagagtattaccctttctacagctaagcgagtcagtaatacagcagcaactaatactggccattaataacgtccagagagcacattagcaaaccttgtactcccagtgactgtcaggagacttgaaaataactactattctcttccaaagtagaatagcgtttttctagatagtgaaggaaatgatagtcatagttggtctgaactccaagatcctactcctcaaaacagcaccgaagcaggggttcgggatgcctgctaagagcatttccacagttcaagtctcttcagaaccttagggaccttcgtgtctagcttcacacacccacctccacatatgaaccagcctaccacacttcacatctgggtacactggccattagcaacaatgcagtctcatgcagcagcacattaaaatcaaacgggtggcaatcgttcaccaccctcagagtgttgggagactttcacatttcatcatccttataatccacaaacagaaacatgaagggatgcaagtgagttcagcattcactcgtttggtgcactcaagtgctgagagaatgcagaatttacagtgtcacagaggaaaaaagccatctgaaataattgtaaaaatggttaagtgtggtatttaaatgttggttccctcctcttcatacaagtggaagaaaagaaggggctagggtacccactgggccatgaggttaaccccttagcacaggcaatgaagaacatccaatgccacagattctgcaggaggagaaatcccaagggtatacagtattcctgagaaagatcccagatttttctgaatcagtcttaatctgattttgttttggctacacagttatgctgttatacctttgacatacataaaaatggtcattttatttcaatccagacagctcagcattgtacaaatgatggcagaaagatccatttgttcagactcagcttgctttgtttttaatactggggaataaaccaaaaaaaaaagtgtaatttttatcatttgtatccttcattctactttactggagtggaatccccagggccttcagataatctgggaagacctgactattcctgtgaggcaagcacagccctgctgagctttactcagaataatgcatgatagactcaacgtaattcccaggaaaaagcccagtcactccattcataactccctcataccaaccatcgtcattcttcttgatgacataaataatggctccttcctgaaaggacagctcatcttccttgtcttttgtatagtcataaattgccacaaccttttccaagtaagaacgtggagcccacggtgggtcctcttcagcataaggatcactatactcaaccacagcagcttcctcctcttcgtaatcttctggaggaggaggaggtgggggagactcatcaaagactggttcttccacaggtggcggtggaggtggtgtatctgaaactggattctggctataaaaaggtcctccattcatctgattctgaaggcttgtttgtgaagtaatggaaggagggcgtctatagggcaacgagccccctattgttgggggagtatggcgagaggcaggcctattcatgctgtagaactgtacaggatgacctggaaagacactgggaggagatggagtaggaacagcaataggaacccccacactaccacttccactgttctctcgactgctgctccgactacttgggtggctccctccactactcccactgctgctgtaagttcgatttctttgattcacagaagctgtcctcacagggctctgctgcgagggagccatattacgggttgggctaggtacgtaatcatttggtaccactggaggacgcactggctccagtgtgcgatagggggagtgccgcccaagtgtccctttccctgacatagggggactagggggcttctgagttggaggtgttgtacgcggcagcccacccatcttcatgttctgggtactcacctttactccatgtccaatatcatctagaattgtatagtcaataggttttctaatataacgaactggtcgttcaaggttggctggagcaataatcttatgtgtccttgaagtgtttttattggtagtcaaaataccaatttctcttcttgcaactttctctttatgaatatcaactgtctgtatgtagttgttctcgcagtaatcggccacccgttccagatttgtgtagctgtcgaagagggcccggcggccccccgggatttcctcttccagcagcatctgcagctccgccatcttcacatcctcctcctcctcctcctcatacaggtcgcagagggagcggcggccgcagcgccaaggaaacccaggaccgggagaggaggagcggcggcgacggcggcggtaactcggaagg

SEQ ID NO: 11788 - RNA, 3885 nt, Homo sapiens
  source 1..3885: mol_type = other RNA
ctgaatagctgggactacaggtgtgcgccaccacgcccagctaatttttgtgtttttagtagagatggggtttcaccatgttggccaggatggtctcaatttattgacctcatgatccacccacctcggcctccgaaagtgctgggattacaggcataagccaccacacccagcctgtgggaactatttattggatttcaaaacaccctctgcctcattaatccactaagctttctcagcaaaaagctgtttaaataaataatgggaacatctaatttaaaacagtttttctaattatagaccagtacacgaagaagagcttaacttatccaagtatagtctagtttgggtccataatggagctgaaggctcagaggacattcagggccattacactgcaggaaaacaaggaataagggatgtagaaatgacctaagaaaagcacgaagtggaatgtatactggaggcaagttaatgaaagctaataaatacaaagtgctgggaaaaatctaaaagcaaaatagctattgtaacttgcaatgcattaaaaacaactttaaaaccaaaaagtcttgataaggaaactctatagtggggtctcagttaaatgctgatgatttttaatgctcagataacattaagtggaatattaacttctgcatccgacaccatctgaattttctcacacactactacacttgttcacttttcaatcaagttccactttctgaacttgttcaaaacctcatttgaaatatatccagctactgcttttcccctttcacctagcacagggcagttacctggcaaagctctattctggccaagtcactgggactgagtagaacccacgttagcagctctggacctgaacaggagctggcccaacatcacagtgaccacccacaaagagacaagccctcctggatttttttcagcatttcttatactgactacagtagtgatgattaaagttatctgccctacagactccactgaatttgaagctgtatttattgtacagatgggggaaatgtgttttattgtgtcagttatattaatttttatcaatgtgattagatacatattttggcctattaatcttattcattatattcttagtctgagatgggttttaattctgactaacagcagctacttaagagtccaatcatacaaaatcaggagagtattaccctttctacagctaagcgagtcagtaatacagcagcaactaatactggccattaataacgtccagagagcacattagcaaaccttgtactcccagtgactgtcaggagacttgaaaataactactattctcttccaaagtagaatagcgtttttctagatagtgaaggaaatgatagtcatagttggtctgaactccaagatcctactcctcaaaacagcaccgaagcaggggttcgggatgcctgctaagagcatttccacagttcaagtctcttcagaaccttagggaccttcgtgtctagcttcacacacccacctccacatatgaaccagcctaccacacttcacatctgggtacactggccattagcaacaatgcagtctcatgcagcagcacattaaaatcaaacgggtggcaatcgttcaccaccctcagagtgttgggagactttcacatttcatcatccttataatccacaaacagaaacatgaagggatgcaagtgagttcagcattcactcgtttggtgcactcaagtgctgagagaatgcagaatttacagtgtcacagaggaaaaaagccatctgaaataattgtaaaaatggttaagtgtggtatttaaatgttggttccctcctcttcatacaagtggaagaaaagaaggggctagggtacccactgggccatgaggttaaccccttagcacaggcaatgaagaacatccaatgccacagattctgcaggaggagaaatcccaagggtatacagtattcctgagaaagatcccagatttttctgaatcagtcttaatctgattttgttttggctacacagttatgctgttatacctttgacatacataaaaatggtcattttatttcaatccagacagctcagcattgtacaaatgatggcagaaagatccatttgttcagactcagcttgctttgtttttaatactggggaataaaccaaaaaaaaaagtgtaatttttatcatttgtatccttcattctactttactggagtggaatccccagggccttcagataatctgggaagacctgactattcctgtgaggcaagcacagccctgctgagctttactcagaataatgcatgatagactcaacgtaattcccaggaaaaagcccagtcactccattcataactccctcataccaaccatcgtcattcttcttgatgacataaataatggctccttcctgaaaggacagctcatcttccttgtcttttgtatagtcataaattgccacaaccttttccaagtaagaacgtggagcccacggtgggtcctcttcagcataaggatcactatactcaaccacagcagcttcctcctcttcgtaatcttctggaggaggaggaggtgggggagactcatcaaagactggttcttccacaggtggcggtggaggtggtgtatctgaaactggattctggctataaaaaggtcctccattcatctgattctgaaggcttgtttgtgaagtaatggaaggagggcgtctatagggcaacgagccccctattgttgggggagtatggcgagaggcaggcctattcatgctgtagaactgtacaggatgacctggaaagacactgggaggagatggagtaggaacagcaataggaacccccacactaccacttccactgttctctcgactgctgctccgactacttgggtggctccctccactactcccactgctgctgtaagttcgatttctttgattcacagaagctgtcctcacagggctctgctgcgagggagccatattacgggttgggctaggtacgtaatcatttggtaccactggaggacgcactggctccagtgtgcgatagggggagtgccgcccaagtgtccctttccctgacatagggggactagggggcttctgagttggaggtgttgtacgcggcagcccacccatcttcatgttctgggtactcacctttactccatgtccaatatcatctagaattgtatagtcaataggttttctaatataacgaactggtcgttcaaggttggctggagcaataatcttatgtgtccttgaagtgtttttattggtagtcaaaataccaatttctcttcttgcaactttctctttatgaatatcaactgtttgtgaaatatgattgattgaagattccatccttcgtagctgggatgcctggatatccagcatctgcaggacattgttggccaaggtgtttatcagataggcaacacttgctaaggattgggtggtgtaggctttggtttcttctagggctctctgcttatctgctgactgtagtcccagactactgagagactgaggcaggatgatcacttgagcacaggagttcaaggctgcagtgagctatgatcacaccactgcattccagcctgcatgacataccaagaccccatctctgtatgtagttgttctcgcagtaatcggccacccgttccagatttgtgtagctgtcgaagagggcccggcggccccccgggatttcctcttccagcagcatctgcagctccgccatcttcacatcctcctcctcctcctcctcatacaggtcgcagagggagcggcggccgcagcgccaaggaaacccaggaccgggagaggaggagcggcggcgacggcggcggtaactcggaagg

SEQ ID NO: 11789 - RNA, 3761 nt, Homo sapiens
  source 1..3761: mol_type = other RNA
ctgaatagctgggactacaggtgtgcgccaccacgcccagctaatttttgtgtttttagtagagatggggtttcaccatgttggccaggatggtctcaatttattgacctcatgatccacccacctcggcctccgaaagtgctgggattacaggcataagccaccacacccagcctgtgggaactatttattggatttcaaaacaccctctgcctcattaatccactaagctttctcagcaaaaagctgtttaaataaataatgggaacatctaatttaaaacagtttttctaattatagaccagtacacgaagaagagcttaacttatccaagtatagtctagtttgggtccataatggagctgaaggctcagaggacattcagggccattacactgcaggaaaacaaggaataagggatgtagaaatgacctaagaaaagcacgaagtggaatgtatactggaggcaagttaatgaaagctaataaatacaaagtgctgggaaaaatctaaaagcaaaatagctattgtaacttgcaatgcattaaaaacaactttaaaaccaaaaagtcttgataaggaaactctatagtggggtctcagttaaatgctgatgatttttaatgctcagataacattaagtggaatattaacttctgcatccgacaccatctgaattttctcacacactactacacttgttcacttttcaatcaagttccactttctgaacttgttcaaaacctcatttgaaatatatccagctactgcttttcccctttcacctagcacagggcagttacctggcaaagctctattctggccaagtcactgggactgagtagaacccacgttagcagctctggacctgaacaggagctggcccaacatcacagtgaccacccacaaagagacaagccctcctggatttttttcagcatttcttatactgactacagtagtgatgattaaagttatctgccctacagactccactgaatttgaagctgtatttattgtacagatgggggaaatgtgttttattgtgtcagttatattaatttttatcaatgtgattagatacatattttggcctattaatcttattcattatattcttagtctgagatgggttttaattctgactaacagcagctacttaagagtccaatcatacaaaatcaggagagtattaccctttctacagctaagcgagtcagtaatacagcagcaactaatactggccattaataacgtccagagagcacattagcaaaccttgtactcccagtgactgtcaggagacttgaaaataactactattctcttccaaagtagaatagcgtttttctagatagtgaaggaaatgatagtcatagttggtctgaactccaagatcctactcctcaaaacagcaccgaagcaggggttcgggatgcctgctaagagcatttccacagttcaagtctcttcagaaccttagggaccttcgtgtctagcttcacacacccacctccacatatgaaccagcctaccacacttcacatctgggtacactggccattagcaacaatgcagtctcatgcagcagcacattaaaatcaaacgggtggcaatcgttcaccaccctcagagtgttgggagactttcacatttcatcatccttataatccacaaacagaaacatgaagggatgcaagtgagttcagcattcactcgtttggtgcactcaagtgctgagagaatgcagaatttacagtgtcacagaggaaaaaagccatctgaaataattgtaaaaatggttaagtgtggtatttaaatgttggttccctcctcttcatacaagtggaagaaaagaaggggctagggtacccactgggccatgaggttaaccccttagcacaggcaatgaagaacatccaatgccacagattctgcaggaggagaaatcccaagggtatacagtattcctgagaaagatcccagatttttctgaatcagtcttaatctgattttgttttggctacacagttatgctgttatacctttgacatacataaaaatggtcattttatttcaatccagacagctcagcattgtacaaatgatggcagaaagatccatttgttcagactcagcttgctttgtttttaatactggggaataaaccaaaaaaaaaagtgtaatttttatcatttgtatccttcattctactttactggagtggaatccccagggccttcagataatctgggaagacctgactattcctgtgaggcaagcacagccctgctgagctttactcagaataatgcatgatagactcaacgtaattcccaggaaaaagcccagtcactccattcataactccctcataccaaccatcgtcattcttcttgatgacataaataatggctccttcctgaaaggacagctcatcttccttgtcttttgtatagtcataaattgccacaaccttttccaagtaagaacgtggagcccacggtgggtcctcttcagcataaggatcactatactcaaccacagcagcttcctcctcttcgtaatcttctggaggaggaggaggtgggggagactcatcaaagactggttcttccacaggtggcggtggaggtggtgtatctgaaactggattctggctataaaaaggtcctccattcatctgattctgaaggcttgtttgtgaagtaatggaaggagggcgtctatagggcaacgagccccctattgttgggggagtatggcgagaggcaggcctattcatgctgtagaactgtacaggatgacctggaaagacactgggaggagatggagtaggaacagcaataggaacccccacactaccacttccactgttctctcgactgctgctccgactacttgggtggctccctccactactcccactgctgctgtaagttcgatttctttgattcacagaagctgtcctcacagggctctgctgcgagggagccatattacgggttgggctaggtacgtaatcatttggtaccactggaggacgcactggctccagtgtgcgatagggggagtgccgcccaagtgtccctttccctgacatagggggactagggggcttctgagttggaggtgttgtacgcggcagcccacccatcttcatgttctgggtactcacctttactccatgtccaatatcatctagaattgtatagtcaataggttttctaatataacgaactggtcgttcaaggttggctggagcaataatcttatgtgtccttgaagtgtttttattggtagtcaaaataccaatttctcttcttgcaactttctctttatgaatatcaactgtttgtgaaatatgattgattgaagattccatccttcgtagctgggatgcctggatatccagcatctgcaggacattgttggccaaggtgtttatcagataggcaacacttgctaaggattgggtggtgtaggctttggtttcttctagggctctctgcttatctgctgactgtatgtagttgttctcgcagtaatcggccacccgttccagatttgtgtagctgtcgaagagggcccggcggccccccgggatttcctcttccagcagcatctgcagctccgccatcttcacatcctcctcctcctcctcctcatacaggtcgcagagggagcggcggccgcagcgccaaggaaacccaggaccgggagaggaggagcggcggcgacggcggcggtaactcggaagg

SEQ ID NO: 11790 - RNA, 3757 nt, Homo sapiens
  source 1..3757: mol_type = other RNA
ctgaatagctgggactacaggtgtgcgccaccacgcccagctaatttttgtgtttttagtagagatggggtttcaccatgttggccaggatggtctcaatttattgacctcatgatccacccacctcggcctccgaaagtgctgggattacaggcataagccaccacacccagcctgtgggaactatttattggatttcaaaacaccctctgcctcattaatccactaagctttctcagcaaaaagctgtttaaataaataatgggaacatctaatttaaaacagtttttctaattatagaccagtacacgaagaagagcttaacttatccaagtatagtctagtttgggtccataatggagctgaaggctcagaggacattcagggccattacactgcaggaaaacaaggaataagggatgtagaaatgacctaagaaaagcacgaagtggaatgtatactggaggcaagttaatgaaagctaataaatacaaagtgctgggaaaaatctaaaagcaaaatagctattgtaacttgcaatgcattaaaaacaactttaaaaccaaaaagtcttgataaggaaactctatagtggggtctcagttaaatgctgatgatttttaatgctcagataacattaagtggaatattaacttctgcatccgacaccatctgaattttctcacacactactacacttgttcacttttcaatcaagttccactttctgaacttgttcaaaacctcatttgaaatatatccagctactgcttttcccctttcacctagcacagggcagttacctggcaaagctctattctggccaagtcactgggactgagtagaacccacgttagcagctctggacctgaacaggagctggcccaacatcacagtgaccacccacaaagagacaagccctcctggatttttttcagcatttcttatactgactacagtagtgatgattaaagttatctgccctacagactccactgaatttgaagctgtatttattgtacagatgggggaaatgtgttttattgtgtcagttatattaatttttatcaatgtgattagatacatattttggcctattaatcttattcattatattcttagtctgagatgggttttaattctgactaacagcagctacttaagagtccaatcatacaaaatcaggagagtattaccctttctacagctaagcgagtcagtaatacagcagcaactaatactggccattaataacgtccagagagcacattagcaaaccttgtactcccagtgactgtcaggagacttgaaaataactactattctcttccaaagtagaatagcgtttttctagatagtgaaggaaatgatagtcatagttggtctgaactccaagatcctactcctcaaaacagcaccgaagcaggggttcgggatgcctgctaagagcatttccacagttcaagtctcttcagaaccttagggaccttcgtgtctagcttcacacacccacctccacatatgaaccagcctaccacacttcacatctgggtacactggccattagcaacaatgcagtctcatgcagcagcacattaaaatcaaacgggtggcaatcgttcaccaccctcagagtgttgggagactttcacatttcatcatccttataatccacaaacagaaacatgaagggatgcaagtgagttcagcattcactcgtttggtgcactcaagtgctgagagaatgcagaatttacagtgtcacagaggaaaaaagccatctgaaataattgtaaaaatggttaagtgtggtatttaaatgttggttccctcctcttcatacaagtggaagaaaagaaggggctagggtacccactgggccatgaggttaaccccttagcacaggcaatgaagaacatccaatgccacagattctgcaggaggagaaatcccaagggtatacagtattcctgagaaagatcccagatttttctgaatcagtcttaatctgattttgttttggctacacagttatgctgttatacctttgacatacataaaaatggtcattttatttcaatccagacagctcagcattgtacaaatgatggcagaaagatccatttgttcagactcagcttgctttgtttttaatactggggaataaaccaaaaaaaaaagtgtaatttttatcatttgtatccttcattctactttactggagtggaatccccagggccttcagataatctgggaagacctgactattcctgtgaggcaagcacagccctgctgagctttactcagaataatgcatgatagactcaacgtaattcccaggaaaaagcccagtcactccattcataactccctcataccaaccatcgtcattcttcttgatgacataaataatggctccttcctgaaaggacagctcatcttccttgtcttttgtatagtcataaattgccacaaccttttccaagtaagaacgtggagcccacggtgggtcctcttcagcataaggatcactatactcaaccacagcagcttcctcctcttcgtaatcttctggaggaggaggaggtgggggagactcatcaaagactggttcttccacaggtggcggtggaggtggtgtatctgaaactggattctggctataaaaaggtcctccattcatctgattctgaaggcttgtttgtgaagtaatggaaggagggcgtctatagggcaacgagccccctattgttgggggagtatggcgagaggcaggcctattcatgctgtagaactgtacaggatgacctggaaagacactgggaggagatggagtaggaacagcaataggaacccccacactaccacttccactgttctctcgactgctgctccgactacttgggtggctccctccactactcccactgctgctgtaagttcgatttctttgattcacagaagctgtcctcacagggctctgctgcgagggagccatattacgggttgggctaggtacgtaatcatttggtaccactggaggacgcactggctccagtgtgcgatagggggagtgccgcccaagtgtccctttccctgacatagggggactagggggcttctgagttggaggtgttgtacgcggcagcccacccatcttcatgttctgggtactcacctttactccatgtccaatatcatctagaattgtatagtcaataggttttctaatataacgaactggtcgttcaaggttggctggagcaataatcttatgtgtccttgaagtgtttttattggtagtcaaaataccaatttctcttcttgcaactttctctttatgaatatcaactgtttgtgaaatatgattgattgaagattccatccttcgtagctgggatgcctggatatccagcatctgcaggacattgttggccaaggtgtttatcagataggcaacacttgctaaggattgggtggtgtaggctttggtttcttctagggctctctgcttatctgctgtatgtagttgttctcgcagtaatcggccacccgttccagatttgtgtagctgtcgaagagggcccggcggccccccgggatttcctcttccagcagcatctgcagctccgccatcttcacatcctcctcctcctcctcctcatacaggtcgcagagggagcggcggccgcagcgccaaggaaacccaggaccgggagaggaggagcggcggcgacggcggcggtaactcggaagg

SEQ ID NO: 11791 - RNA, 3584 nt, Homo sapiens
  source 1..3584: mol_type = other RNA
ctgaatagctgggactacaggtgtgcgccaccacgcccagctaatttttgtgtttttagtagagatggggtttcaccatgttggccaggatggtctcaatttattgacctcatgatccacccacctcggcctccgaaagtgctgggattacaggcataagccaccacacccagcctgtgggaactatttattggatttcaaaacaccctctgcctcattaatccactaagctttctcagcaaaaagctgtttaaataaataatgggaacatctaatttaaaacagtttttctaattatagaccagtacacgaagaagagcttaacttatccaagtatagtctagtttgggtccataatggagctgaaggctcagaggacattcagggccattacactgcaggaaaacaaggaataagggatgtagaaatgacctaagaaaagcacgaagtggaatgtatactggaggcaagttaatgaaagctaataaatacaaagtgctgggaaaaatctaaaagcaaaatagctattgtaacttgcaatgcattaaaaacaactttaaaaccaaaaagtcttgataaggaaactctatagtggggtctcagttaaatgctgatgatttttaatgctcagataacattaagtggaatattaacttctgcatccgacaccatctgaattttctcacacactactacacttgttcacttttcaatcaagttccactttctgaacttgttcaaaacctcatttgaaatatatccagctactgcttttcccctttcacctagcacagggcagttacctggcaaagctctattctggccaagtcactgggactgagtagaacccacgttagcagctctggacctgaacaggagctggcccaacatcacagtgaccacccacaaagagacaagccctcctggatttttttcagcatttcttatactgactacagtagtgatgattaaagttatctgccctacagactccactgaatttgaagctgtatttattgtacagatgggggaaatgtgttttattgtgtcagttatattaatttttatcaatgtgattagatacatattttggcctattaatcttattcattatattcttagtctgagatgggttttaattctgactaacagcagctacttaagagtccaatcatacaaaatcaggagagtattaccctttctacagctaagcgagtcagtaatacagcagcaactaatactggccattaataacgtccagagagcacattagcaaaccttgtactcccagtgactgtcaggagacttgaaaataactactattctcttccaaagtagaatagcgtttttctagatagtgaaggaaatgatagtcatagttggtctgaactccaagatcctactcctcaaaacagcaccgaagcaggggttcgggatgcctgctaagagcatttccacagttcaagtctcttcagaaccttagggaccttcgtgtctagcttcacacacccacctccacatatgaaccagcctaccacacttcacatctgggtacactggccattagcaacaatgcagtctcatgcagcagcacattaaaatcaaacgggtggcaatcgttcaccaccctcagagtgttgggagactttcacatttcatcatccttataatccacaaacagaaacatgaagggatgcaagtgagttcagcattcactcgtttggtgcactcaagtgctgagagaatgcagaatttacagtgtcacagaggaaaaaagccatctgaaataattgtaaaaatggttaagtgtggtatttaaatgttggttccctcctcttcatacaagtggaagaaaagaaggggctagggtacccactgggccatgaggttaaccccttagcacaggcaatgaagaacatccaatgccacagattctgcaggaggagaaatcccaagggtatacagtattcctgagaaagatcccagatttttctgaatcagtcttaatctgattttgttttggctacacagttatgctgttatacctttgacatacataaaaatggtcattttatttcaatccagacagctcagcattgtacaaatgatggcagaaagatccatttgttcagactcagcttgctttgtttttaatactggggaataaaccaaaaaaaaaagtgtaatttttatcatttgtatccttcattctactttactggagtggaatccccagggccttcagataatctgggaagacctgactattcctgtgaggcaagcacagccctgctgagctttactcagaataatgcatgatagactcaacgtaattcccaggaaaaagcccagtcactccattcataactccctcataccaaccatcgtcattcttcttgatgacataaataatggctccttcctgaaaggacagctcatcttccttgtcttttgtatagtcataaattgccacaaccttttccaagtaagaacgtggagcccacggtgggtcctcttcagcataaggatcactatactcaaccacagcagcttcctcctcttcgtaatcttctggaggaggaggaggtgggggagactcatcaaagactggttcttccacaggtggcggtggaggtggtgtatctgaaactggattctggctataaaaaggtcctccattcatctgattctgaaggcttgtttgtgaagtaatggaaggagggcgtctatagggcaacgagccccctattgttgggggagtatggcgagaggcaggcctattcatgctgtagaactgtacaggatgacctggaaagacactgggaggagatggagtaggaacagcaataggaacccccacactaccacttccactgttctctcgactgctgctccgactacttgggtggctccctccactactcccactgctgctgtaagttcgatttctttgattcacagaagctgtcctcacagggctctgctgcgagggagccatattacgggttgggctaggtacgtaatcatttggtaccactggaggacgcactggctccagtgtgcgatagggggagtgccgcccaagtgtccctttccctgacatagggggactagggggcttctgagttggaggtgttgtacgcggcagcccacccatcttcatgttctgggtactcacttgtgaaatatgattgattgaagattccatccttcgtagctgggatgcctggatatccagcatctgcaggacattgttggccaaggtgtttatcagataggcaacacttgctaaggattgggtggtgtaggctttggtttcttctagggctctctgcttatctgctgactgtatgtagttgttctcgcagtaatcggccacccgttccagatttgtgtagctgtcgaagagggcccggcggccccccgggatttcctcttccagcagcatctgcagctccgccatcttcacatcctcctcctcctcctcctcatacaggtcgcagagggagcggcggccgcagcgccaaggaaacccaggaccgggagaggaggagcggcggcgacggcggcggtaactcggaagg

SEQ ID NO: 11792 - RNA, 3833 nt, Homo sapiens
  source 1..3833: mol_type = other RNA
ctgaatagctgggactacaggtgtgcgccaccacgcccagctaatttttgtgtttttagtagagatggggtttcaccatgttggccaggatggtctcaatttattgacctcatgatccacccacctcggcctccgaaagtgctgggattacaggcataagccaccacacccagcctgtgggaactatttattggatttcaaaacaccctctgcctcattaatccactaagctttctcagcaaaaagctgtttaaataaataatgggaacatctaatttaaaacagtttttctaattatagaccagtacacgaagaagagcttaacttatccaagtatagtctagtttgggtccataatggagctgaaggctcagaggacattcagggccattacactgcaggaaaacaaggaataagggatgtagaaatgacctaagaaaagcacgaagtggaatgtatactggaggcaagttaatgaaagctaataaatacaaagtgctgggaaaaatctaaaagcaaaatagctattgtaacttgcaatgcattaaaaacaactttaaaaccaaaaagtcttgataaggaaactctatagtggggtctcagttaaatgctgatgatttttaatgctcagataacattaagtggaatattaacttctgcatccgacaccatctgaattttctcacacactactacacttgttcacttttcaatcaagttccactttctgaacttgttcaaaacctcatttgaaatatatccagctactgcttttcccctttcacctagcacagggcagttacctggcaaagctctattctggccaagtcactgggactgagtagaacccacgttagcagctctggacctgaacaggagctggcccaacatcacagtgaccacccacaaagagacaagccctcctggatttttttcagcatttcttatactgactacagtagtgatgattaaagttatctgccctacagactccactgaatttgaagctgtatttattgtacagatgggggaaatgtgttttattgtgtcagttatattaatttttatcaatgtgattagatacatattttggcctattaatcttattcattatattcttagtctgagatgggttttaattctgactaacagcagctacttaagagtccaatcatacaaaatcaggagagtattaccctttctacagctaagcgagtcagtaatacagcagcaactaatactggccattaataacgtccagagagcacattagcaaaccttgtactcccagtgactgtcaggagacttgaaaataactactattctcttccaaagtagaatagcgtttttctagatagtgaaggaaatgatagtcatagttggtctgaactccaagatcctactcctcaaaacagcaccgaagcaggggttcgggatgcctgctaagagcatttccacagttcaagtctcttcagaaccttagggaccttcgtgtctagcttcacacacccacctccacatatgaaccagcctaccacacttcacatctgggtacactggccattagcaacaatgcagtctcatgcagcagcacattaaaatcaaacgggtggcaatcgttcaccaccctcagagtgttgggagactttcacatttcatcatccttataatccacaaacagaaacatgaagggatgcaagtgagttcagcattcactcgtttggtgcactcaagtgctgagagaatgcagaatttacagtgtcacagaggaaaaaagccatctgaaataattgtaaaaatggttaagtgtggtatttaaatgttggttccctcctcttcatacaagtggaagaaaagaaggggctagggtacccactgggccatgaggttaaccccttagcacaggcaatgaagaacatccaatgccacagattctgcaggaggagaaatcccaagggtatacagtattcctgagaaagatcccagatttttctgaatcagtcttaatctgattttgttttggctacacagttatgctgttatacctttgacatacataaaaatggtcattttatttcaatccagacagctcagcattgtacaaatgatggcagaaagatccatttgttcagactcagcttgctttgtttttaatactggggaataaaccaaaaaaaaaagtgtaatttttatcatttgtatccttcattctactttactggagtggaatccccagggccttcagataatctgggaagacctgactattcctgtgaggcaagcacagccctgctgagctttactcagaataatgcatgatagactcaacgtaattcccaggaaaaagcccagtcactccattcataactccctcataccaaccatcgtcattcttcttgatgacataaataatggctccttcctgaaaggacagctcatcttccttgtcttttgtatagtcataaattgccacaaccttttccaagtaagaacgtggagcccacggtgggtcctcttcagcataaggatcactatactcaaccacagcagcttcctcctcttcgtaatcttctggaggaggaggaggtgggggagactcatcaaagactggttcttccacaggtggcggtggaggtggtgtatctgaaactggattctggctataaaaaggtcctccattcatctgattctgaaggcttgtttgtgaagtaatggaaggagggcgtctatagggcaacgagccccctattgttgggggagtatggcgagaggcaggcctattcatgctgtagaactgtacaggatgacctggaaagacactgggaggagatggagtaggaacagcaataggaacccccacactaccacttccactgttctctcgactgctgctccgactacttgggtggctccctccactactcccactgctgtaagttcgatttctttgattcacagaagctgtcctcacagggctctgctgcgagggagccatattacgggttgggctaggtacgtaatcatttggtaccactggaggacgcactggctccagtgtgcgatagggggagtgccgcccaagtgtccctttccctgacatagggggactagggggcttctgagttggaggtgttgtacgcggcagcccacccatcttcatgttctgggtactcaccatgactgaggatttggaaccaacaatccaatcaataatacaggtgtccatatgcctgggctcttccaatcaaatctttactccatgtccaatatcatctagaattgtatagtcaataggttttctaatataacgaactggtcgttcaaggttggctggagcaataatcttatgtgtccttgaagtgtttttattggtagtcaaaataccaatttctcttcttgcaactttctctttatgaatatcaactgtttgtgaaatatgattgattgaagattccatccttcgtagctgggatgcctggatatccagcatctgcaggacattgttggccaaggtgtttatcagataggcaacacttgctaaggattgggtggtgtaggctttggtttcttctagggctctctgcttatctgctgactgtatgtagttgttctcgcagtaatcggccacccgttccagatttgtgtagctgtcgaagagggcccggcggccccccgggatttcctcttccagcagcatctgcagctccgccatcttcacatcctcctcctcctcctcctcatacaggtcgcagagggagcggcggccgcagcgccaaggaaacccaggaccgggagaggaggagcggcggcgacggcggcggtaactcggaagg

SEQ ID NO: 11793 - RNA, 4296 nt, Homo sapiens
  source 1..4296: mol_type = other RNA
ctgaatagctgggactacaggtgtgcgccaccacgcccagctaatttttgtgtttttagtagagatggggtttcaccatgttggccaggatggtctcaatttattgacctcatgatccacccacctcggcctccgaaagtgctgggattacaggcataagccaccacacccagcctgtgggaactatttattggatttcaaaacaccctctgcctcattaatccactaagctttctcagcaaaaagctgtttaaataaataatgggaacatctaatttaaaacagtttttctaattatagaccagtacacgaagaagagcttaacttatccaagtatagtctagtttgggtccataatggagctgaaggctcagaggacattcagggccattacactgcaggaaaacaaggaataagggatgtagaaatgacctaagaaaagcacgaagtggaatgtatactggaggcaagttaatgaaagctaataaatacaaagtgctgggaaaaatctaaaagcaaaatagctattgtaacttgcaatgcattaaaaacaactttaaaaccaaaaagtcttgataaggaaactctatagtggggtctcagttaaatgctgatgatttttaatgctcagataacattaagtggaatattaacttctgcatccgacaccatctgaattttctcacacactactacacttgttcacttttcaatcaagttccactttctgaacttgttcaaaacctcatttgaaatatatccagctactgcttttcccctttcacctagcacagggcagttacctggcaaagctctattctggccaagtcactgggactgagtagaacccacgttagcagctctggacctgaacaggagctggcccaacatcacagtgaccacccacaaagagacaagccctcctggatttttttcagcatttcttatactgactacagtagtgatgattaaagttatctgccctacagactccactgaatttgaagctgtatttattgtacagatgggggaaatgtgttttattgtgtcagttatattaatttttatcaatgtgattagatacatattttggcctattaatcttattcattatattcttagtctgagatgggttttaattctgactaacagcagctacttaagagtccaatcatacaaaatcaggagagtattaccctttctacagctaagcgagtcagtaatacagcagcaactaatactggccattaataacgtccagagagcacattagcaaaccttgtactcccagtgactgtcaggagacttgaaaataactactattctcttccaaagtagaatagcgtttttctagatagtgaaggaaatgatagtcatagttggtctgaactccaagatcctactcctcaaaacagcaccgaagcaggggttcgggatgcctgctaagagcatttccacagttcaagtctcttcagaaccttagggaccttcgtgtctagcttcacacacccacctccacatatgaaccagcctaccacacttcacatctgggtacactggccattagcaacaatgcagtctcatgcagcagcacattaaaatcaaacgggtggcaatcgttcaccaccctcagagtgttgggagactttcacatttcatcatccttataatccacaaacagaaacatgaagggatgcaagtgagttcagcattcactcgtttggtgcactcaagtgctgagagaatgcagaatttacagtgtcacagaggaaaaaagccatctgaaataattgtaaaaatggttaagtgtggtatttaaatgttggttccctcctcttcatacaagtggaagaaaagaaggggctagggtacccactgggccatgaggttaaccccttagcacaggcaatgaagaacatccaatgccacagattctgcaggaggagaaatcccaagggtatacagtattcctgagaaagatcccagatttttctgaatcagtcttaatctgattttgttttggctacacagttatgctgttatacctttgacatacataaaaatggtcattttatttcaatccagacagctcagcattgtacaaatgatggcagaaagatccatttgttcagactcagcttgctttgtttttaatactggggaataaaccaaaaaaaaaagtgtaatttttatcatttgtatccttcattctactttactggagtggaatccccagggccttcagataatctgggaagacctgactattcctgtgaggcaagcacagccctgctgagctttactcagaataatgcatgatagactcaacgtaattcccaggaaaaagcccagtcactccattcataactccctcataccaaccatcgtcattcttcttgatgacataaataatggctccttcctgaaaggacagctcatcttccttgtcttttgtatagtcataaattgccacaaccttttccaagtaagaacgtggagcccacggtgggtcctcttcagcataaggatcactatactcaaccacagcagcttcctcctcttcgtaatcttctggaggaggaggaggtgggggagactcatcaaagactggttcttccacaggtggcggtggaggtggtgtatctgaaactggattctggctataaaaaggtcctccattcatctgattctgaaggcttgtttgtgaagtaatggaaggagggcgtctatagggcaacgagccccctattgttgggggagtatggcgagaggcaggcctattcatgctgtagaactgtacaggatgacctggaaagacactgggaggagatggagtaggaacagcaataggaacccccacactaccacttccactgttctctcgactgctgctccgactacttgggtggctccctccactactcccactgctgtaagttcgatttctttgattcacagaagctgtcctcacagggctctgctgcgagggagccatattacgggttgggctaggtacgtaatcatttggtaccactggaggacgcactggctccagtgtgcgatagggggagtgccgcccaagtgtccctttccctgacatagggggactagggggcttctgagttggaggtgttgtacgcggcagcccacccatcttcatgttctgggtactcaccttaaatctaagcaaccactttactccatgtccaatatcatctagaattgtatagtcaataggttttctaatataacgaactggtcgttcaaggttggctggagcaataatcttatgtgtccttgaagtgtttttattggtagtcaaaataccaatttctcttcttgcaactttctctttatgaatatcaactgtttgtgaaatatgattgattgaagattccatccttcgtagctgggatgcctggatatccagcatctgcaggacattgttggccaaggtgtttatcagataggcaacacttgctaaggattgggtggtgtaggctttggtttcttctagggctctctgcttatctgctgactgtatgtagttgttctcgcagtaatcggccacccgttccagatttgtgtagctgtcgaagagggcccggcggccccccgggatttcctcttccagcagcatctgcagctccgccatcttcacatcctcctcctcctcctcctcatacaggtcgcagagggagcggcggccgcagcgccaaggaaacccaggaccgggagaggaggagcggcggcgacggcggcggtaactcggaaggagcgagaaacagccccagcgcgcgacaggggagggggcgacgggggcggggcgcgagccgacggactccgaggacggtcaccgcggcgacggccggccgggcgcgcgcacgcgcgctcccttccctccgcccccgggagcccgaaaaagattcccaccctcgcccgcgccgccggcccctcccccacttccggcgtctcctagcgacggcgggggtaggggccgggatgcgcgcgggagttggtggtgcagttaacccttccgccgcccgcccgccgctggagcggctggagaagcccccacctcccggcggcctttgttagcccggcgggaacacaccaccctgctcagctggcttcctgccggctccctccgggactcatctcggctccgtccccatggaggtcatcggcctagggaacttctcgaggcttttctccctctgctgctgacgggaggccgaaggagggcacagcctccactcttgggaccctcctctgtgaaagatcacacctcaacag

SEQ ID NO: 11794 - RNA, 3758 nt, Homo sapiens
  source 1..3758: mol_type = other RNA
ctgaatagctgggactacaggtgtgcgccaccacgcccagctaatttttgtgtttttagtagagatggggtttcaccatgttggccaggatggtctcaatttattgacctcatgatccacccacctcggcctccgaaagtgctgggattacaggcataagccaccacacccagcctgtgggaactatttattggatttcaaaacaccctctgcctcattaatccactaagctttctcagcaaaaagctgtttaaataaataatgggaacatctaatttaaaacagtttttctaattatagaccagtacacgaagaagagcttaacttatccaagtatagtctagtttgggtccataatggagctgaaggctcagaggacattcagggccattacactgcaggaaaacaaggaataagggatgtagaaatgacctaagaaaagcacgaagtggaatgtatactggaggcaagttaatgaaagctaataaatacaaagtgctgggaaaaatctaaaagcaaaatagctattgtaacttgcaatgcattaaaaacaactttaaaaccaaaaagtcttgataaggaaactctatagtggggtctcagttaaatgctgatgatttttaatgctcagataacattaagtggaatattaacttctgcatccgacaccatctgaattttctcacacactactacacttgttcacttttcaatcaagttccactttctgaacttgttcaaaacctcatttgaaatatatccagctactgcttttcccctttcacctagcacagggcagttacctggcaaagctctattctggccaagtcactgggactgagtagaacccacgttagcagctctggacctgaacaggagctggcccaacatcacagtgaccacccacaaagagacaagccctcctggatttttttcagcatttcttatactgactacagtagtgatgattaaagttatctgccctacagactccactgaatttgaagctgtatttattgtacagatgggggaaatgtgttttattgtgtcagttatattaatttttatcaatgtgattagatacatattttggcctattaatcttattcattatattcttagtctgagatgggttttaattctgactaacagcagctacttaagagtccaatcatacaaaatcaggagagtattaccctttctacagctaagcgagtcagtaatacagcagcaactaatactggccattaataacgtccagagagcacattagcaaaccttgtactcccagtgactgtcaggagacttgaaaataactactattctcttccaaagtagaatagcgtttttctagatagtgaaggaaatgatagtcatagttggtctgaactccaagatcctactcctcaaaacagcaccgaagcaggggttcgggatgcctgctaagagcatttccacagttcaagtctcttcagaaccttagggaccttcgtgtctagcttcacacacccacctccacatatgaaccagcctaccacacttcacatctgggtacactggccattagcaacaatgcagtctcatgcagcagcacattaaaatcaaacgggtggcaatcgttcaccaccctcagagtgttgggagactttcacatttcatcatccttataatccacaaacagaaacatgaagggatgcaagtgagttcagcattcactcgtttggtgcactcaagtgctgagagaatgcagaatttacagtgtcacagaggaaaaaagccatctgaaataattgtaaaaatggttaagtgtggtatttaaatgttggttccctcctcttcatacaagtggaagaaaagaaggggctagggtacccactgggccatgaggttaaccccttagcacaggcaatgaagaacatccaatgccacagattctgcaggaggagaaatcccaagggtatacagtattcctgagaaagatcccagatttttctgaatcagtcttaatctgattttgttttggctacacagttatgctgttatacctttgacatacataaaaatggtcattttatttcaatccagacagctcagcattgtacaaatgatggcagaaagatccatttgttcagactcagcttgctttgtttttaatactggggaataaaccaaaaaaaaaagtgtaatttttatcatttgtatccttcattctactttactggagtggaatccccagggccttcagataatctgggaagacctgactattcctgtgaggcaagcacagccctgctgagctttactcagaataatgcatgatagactcaacgtaattcccaggaaaaagcccagtcactccattcataactccctcataccaaccatcgtcattcttcttgatgacataaataatggctccttcctgaaaggacagctcatcttccttgtcttttgtatagtcataaattgccacaaccttttccaagtaagaacgtggagcccacggtgggtcctcttcagcataaggatcactatactcaaccacagcagcttcctcctcttcgtaatcttctggaggaggaggaggtgggggagactcatcaaagactggttcttccacaggtggcggtggaggtggtgtatctgaaactggattctggctataaaaaggtcctccattcatctgattctgaaggcttgtttgtgaagtaatggaaggagggcgtctatagggcaacgagccccctattgttgggggagtatggcgagaggcaggcctattcatgctgtagaactgtacaggatgacctggaaagacactgggaggagatggagtaggaacagcaataggaacccccacactaccacttccactgttctctcgactgctgctccgactacttgggtggctccctccactactcccactgctgtaagttcgatttctttgattcacagaagctgtcctcacagggctctgctgcgagggagccatattacgggttgggctaggtacgtaatcatttggtaccactggaggacgcactggctccagtgtgcgatagggggagtgccgcccaagtgtccctttccctgacatagggggactagggggcttctgagttggaggtgttgtacgcggcagcccacccatcttcatgttctgggtactcacctttactccatgtccaatatcatctagaattgtatagtcaataggttttctaatataacgaactggtcgttcaaggttggctggagcaataatcttatgtgtccttgaagtgtttttattggtagtcaaaataccaatttctcttcttgcaactttctctttatgaatatcaactgtttgtgaaatatgattgattgaagattccatccttcgtagctgggatgcctggatatccagcatctgcaggacattgttggccaaggtgtttatcagataggcaacacttgctaaggattgggtggtgtaggctttggtttcttctagggctctctgcttatctgctgactgtatgtagttgttctcgcagtaatcggccacccgttccagatttgtgtagctgtcgaagagggcccggcggccccccgggatttcctcttccagcagcatctgcagctccgccatcttcacatcctcctcctcctcctcctcatacaggtcgcagagggagcggcggccgcagcgccaaggaaacccaggaccgggagaggaggagcggcggcgacggcggcggtaactcggaagg

SEQ ID NO: 11795 - RNA, 3581 nt, Homo sapiens
  source 1..3581: mol_type = other RNA
ctgaatagctgggactacaggtgtgcgccaccacgcccagctaatttttgtgtttttagtagagatggggtttcaccatgttggccaggatggtctcaatttattgacctcatgatccacccacctcggcctccgaaagtgctgggattacaggcataagccaccacacccagcctgtgggaactatttattggatttcaaaacaccctctgcctcattaatccactaagctttctcagcaaaaagctgtttaaataaataatgggaacatctaatttaaaacagtttttctaattatagaccagtacacgaagaagagcttaacttatccaagtatagtctagtttgggtccataatggagctgaaggctcagaggacattcagggccattacactgcaggaaaacaaggaataagggatgtagaaatgacctaagaaaagcacgaagtggaatgtatactggaggcaagttaatgaaagctaataaatacaaagtgctgggaaaaatctaaaagcaaaatagctattgtaacttgcaatgcattaaaaacaactttaaaaccaaaaagtcttgataaggaaactctatagtggggtctcagttaaatgctgatgatttttaatgctcagataacattaagtggaatattaacttctgcatccgacaccatctgaattttctcacacactactacacttgttcacttttcaatcaagttccactttctgaacttgttcaaaacctcatttgaaatatatccagctactgcttttcccctttcacctagcacagggcagttacctggcaaagctctattctggccaagtcactgggactgagtagaacccacgttagcagctctggacctgaacaggagctggcccaacatcacagtgaccacccacaaagagacaagccctcctggatttttttcagcatttcttatactgactacagtagtgatgattaaagttatctgccctacagactccactgaatttgaagctgtatttattgtacagatgggggaaatgtgttttattgtgtcagttatattaatttttatcaatgtgattagatacatattttggcctattaatcttattcattatattcttagtctgagatgggttttaattctgactaacagcagctacttaagagtccaatcatacaaaatcaggagagtattaccctttctacagctaagcgagtcagtaatacagcagcaactaatactggccattaataacgtccagagagcacattagcaaaccttgtactcccagtgactgtcaggagacttgaaaataactactattctcttccaaagtagaatagcgtttttctagatagtgaaggaaatgatagtcatagttggtctgaactccaagatcctactcctcaaaacagcaccgaagcaggggttcgggatgcctgctaagagcatttccacagttcaagtctcttcagaaccttagggaccttcgtgtctagcttcacacacccacctccacatatgaaccagcctaccacacttcacatctgggtacactggccattagcaacaatgcagtctcatgcagcagcacattaaaatcaaacgggtggcaatcgttcaccaccctcagagtgttgggagactttcacatttcatcatccttataatccacaaacagaaacatgaagggatgcaagtgagttcagcattcactcgtttggtgcactcaagtgctgagagaatgcagaatttacagtgtcacagaggaaaaaagccatctgaaataattgtaaaaatggttaagtgtggtatttaaatgttggttccctcctcttcatacaagtggaagaaaagaaggggctagggtacccactgggccatgaggttaaccccttagcacaggcaatgaagaacatccaatgccacagattctgcaggaggagaaatcccaagggtatacagtattcctgagaaagatcccagatttttctgaatcagtcttaatctgattttgttttggctacacagttatgctgttatacctttgacatacataaaaatggtcattttatttcaatccagacagctcagcattgtacaaatgatggcagaaagatccatttgttcagactcagcttgctttgtttttaatactggggaataaaccaaaaaaaaaagtgtaatttttatcatttgtatccttcattctactttactggagtggaatccccagggccttcagataatctgggaagacctgactattcctgtgaggcaagcacagccctgctgagctttactcagaataatgcatgatagactcaacgtaattcccaggaaaaagcccagtcactccattcataactccctcataccaaccatcgtcattcttcttgatgacataaataatggctccttcctgaaaggacagctcatcttccttgtcttttgtatagtcataaattgccacaaccttttccaagtaagaacgtggagcccacggtgggtcctcttcagcataaggatcactatactcaaccacagcagcttcctcctcttcgtaatcttctggaggaggaggaggtgggggagactcatcaaagactggttcttccacaggtggcggtggaggtggtgtatctgaaactggattctggctataaaaaggtcctccattcatctgattctgaaggcttgtttgtgaagtaatggaaggagggcgtctatagggcaacgagccccctattgttgggggagtatggcgagaggcaggcctattcatgctgtagaactgtacaggatgacctggaaagacactgggaggagatggagtaggaacagcaataggaacccccacactaccacttccactgttctctcgactgctgctccgactacttgggtggctccctccactactcccactgctgtaagttcgatttctttgattcacagaagctgtcctcacagggctctgctgcgagggagccatattacgggttgggctaggtacgtaatcatttggtaccactggaggacgcactggctccagtgtgcgatagggggagtgccgcccaagtgtccctttccctgacatagggggactagggggcttctgagttggaggtgttgtacgcggcagcccacccatcttcatgttctgggtactcacttgtgaaatatgattgattgaagattccatccttcgtagctgggatgcctggatatccagcatctgcaggacattgttggccaaggtgtttatcagataggcaacacttgctaaggattgggtggtgtaggctttggtttcttctagggctctctgcttatctgctgactgtatgtagttgttctcgcagtaatcggccacccgttccagatttgtgtagctgtcgaagagggcccggcggccccccgggatttcctcttccagcagcatctgcagctccgccatcttcacatcctcctcctcctcctcctcatacaggtcgcagagggagcggcggccgcagcgccaaggaaacccaggaccgggagaggaggagcggcggcgacggcggcggtaactcggaagg

SEQ ID NO: 11796 - RNA, 3166 nt, Homo sapiens
  source 1..3166: mol_type = other RNA
ctgaatagctgggactacaggtgtgcgccaccacgcccagctaatttttgtgtttttagtagagatggggtttcaccatgttggccaggatggtctcaatttattgacctcatgatccacccacctcggcctccgaaagtgctgggattacaggcataagccaccacacccagcctgtgggaactatttattggatttcaaaacaccctctgcctcattaatccactaagctttctcagcaaaaagctgtttaaataaataatgggaacatctaatttaaaacagtttttctaattatagaccagtacacgaagaagagcttaacttatccaagtatagtctagtttgggtccataatggagctgaaggctcagaggacattcagggccattacactgcaggaaaacaaggaataagggatgtagaaatgacctaagaaaagcacgaagtggaatgtatactggaggcaagttaatgaaagctaataaatacaaagtgctgggaaaaatctaaaagcaaaatagctattgtaacttgcaatgcattaaaaacaactttaaaaccaaaaagtcttgataaggaaactctatagtggggtctcagttaaatgctgatgatttttaatgctcagataacattaagtggaatattaacttctgcatccgacaccatctgaattttctcacacactactacacttgttcacttttcaatcaagttccactttctgaacttgttcaaaacctcatttgaaatatatccagctactgcttttcccctttcacctagcacagggcagttacctggcaaagctctattctggccaagtcactgggactgagtagaacccacgttagcagctctggacctgaacaggagctggcccaacatcacagtgaccacccacaaagagacaagccctcctggatttttttcagcatttcttatactgactacagtagtgatgattaaagttatctgccctacagactccactgaatttgaagctgtatttattgtacagatgggggaaatgtgttttattgtgtcagttatattaatttttatcaatgtgattagatacatattttggcctattaatcttattcattatattcttagtctgagatgggttttaattctgactaacagcagctacttaagagtccaatcatacaaaatcaggagagtattaccctttctacagctaagcgagtcagtaatacagcagcaactaatactggccattaataacgtccagagagcacattagcaaaccttgtactcccagtgactgtcaggagacttgaaaataactactattctcttccaaagtagaatagcgtttttctagatagtgaaggaaatgatagtcatagttggtctgaactccaagatcctactcctcaaaacagcaccgaagcaggggttcgggatgcctgctaagagcatttccacagttcaagtctcttcagaaccttagggaccttcgtgtctagcttcacacacccacctccacatatgaaccagcctaccacacttcacatctgggtacactggccattagcaacaatgcagtctcatgcagcagcacattaaaatcaaacgggtggcaatcgttcaccaccctcagagtgttgggagactttcacatttcatcatccttataatccacaaacagaaacatgaagggatgcaagtgagttcagcattcactcgtttggtgcactcaagtgctgagagaatgcagaatttacagtgtcacagaggaaaaaagccatctgaaataattgtaaaaatggttaagtgtggtatttaaatgttggttccctcctcttcatacaagtggaagaaaagaaggggctagggtacccactgggccatgaggttaaccccttagcacaggcaatgaagaacatccaatgccacagattctgcaggaggagaaatcccaagggtatacagtattcctgagaaagatcccagatttttctgaatcagtcttaatctgattttgttttggctacacagttatgctgttatacctttgacatacataaaaatggtcattttatttcaatccagacagctcagcattgtacaaatgatggcagaaagatccatttgttcagactcagcttgctttgtttttaatactggggaataaaccaaaaaaaaaagtgtaatttttatcatttgtatccttcattctactttactggagtggaatccccagggccttcagataatctgggaagacctgactattcctgtgaggcaagcacagccctgctgagctttactcagaataatgcatgatagactcaacgtaattcccaggaaaaagcccagtcactccattcataactccctcataccaaccatcgtcattcttcttgatgacataaataatggctccttcctgaaaggacagctcatcttccttgtcttttgtatagtcataaattgccacaaccttttccaagtaagaacgtggagcccacggtgggtcctcttcagcataaggatcactatactcaaccacagcagcttcctcctcttcgtaatcttctggaggaggaggaggtgggggagactcatcaaagactggttcttccacaggtggcggtggaggtggtgtatctgaaactggattctggctataaaaaggtcctccattcatctgattctgaaggcttgtttgtgaagtaatggaaggagggcgtctatagggcaacgagccccctattgttgggggagtatggcgagaggcaggcctattcatgctgtagaactgtacaggatgacctggatatccagcatctgcaggacattgttggccaaggtgtttatcagataggcaacacttgctaaggattgggtggtgtaggctttggtttcttctagggctctctgcttatctgctgactgtatgtagttgttctcgcagtaatcggccacccgttccagatttgtgtagctgtcgaagagggcccggcggccccccgggatttcctcttccagcagcatctgcagctccgccatcttcacatcctcctcctcctcctcctcatacaggtcgcagagggagcggcggccgcagcgccaaggaaacccaggaccgggagaggaggagcggcggcgacggcggcggtaactcggaagg

SEQ ID NO: 11797 - RNA, 3636 nt, Homo sapiens
  source 1..3636: mol_type = other RNA
ctgaatagctgggactacaggtgtgcgccaccacgcccagctaatttttgtgtttttagtagagatggggtttcaccatgttggccaggatggtctcaatttattgacctcatgatccacccacctcggcctccgaaagtgctgggattacaggcataagccaccacacccagcctgtgggaactatttattggatttcaaaacaccctctgcctcattaatccactaagctttctcagcaaaaagctgtttaaataaataatgggaacatctaatttaaaacagtttttctaattatagaccagtacacgaagaagagcttaacttatccaagtatagtctagtttgggtccataatggagctgaaggctcagaggacattcagggccattacactgcaggaaaacaaggaataagggatgtagaaatgacctaagaaaagcacgaagtggaatgtatactggaggcaagttaatgaaagctaataaatacaaagtgctgggaaaaatctaaaagcaaaatagctattgtaacttgcaatgcattaaaaacaactttaaaaccaaaaagtcttgataaggaaactctatagtggggtctcagttaaatgctgatgatttttaatgctcagataacattaagtggaatattaacttctgcatccgacaccatctgaattttctcacacactactacacttgttcacttttcaatcaagttccactttctgaacttgttcaaaacctcatttgaaatatatccagctactgcttttcccctttcacctagcacagggcagttacctggcaaagctctattctggccaagtcactgggactgagtagaacccacgttagcagctctggacctgaacaggagctggcccaacatcacagtgaccacccacaaagagacaagccctcctggatttttttcagcatttcttatactgactacagtagtgatgattaaagttatctgccctacagactccactgaatttgaagctgtatttattgtacagatgggggaaatgtgttttattgtgtcagttatattaatttttatcaatgtgattagatacatattttggcctattaatcttattcattatattcttagtctgagatgggttttaattctgactaacagcagctacttaagagtccaatcatacaaaatcaggagagtattaccctttctacagctaagcgagtcagtaatacagcagcaactaatactggccattaataacgtccagagagcacattagcaaaccttgtactcccagtgactgtcaggagacttgaaaataactactattctcttccaaagtagaatagcgtttttctagatagtgaaggaaatgatagtcatagttggtctgaactccaagatcctactcctcaaaacagcaccgaagcaggggttcgggatgcctgctaagagcatttccacagttcaagtctcttcagaaccttagggaccttcgtgtctagcttcacacacccacctccacatatgaaccagcctaccacacttcacatctgggtacactggccattagcaacaatgcagtctcatgcagcagcacattaaaatcaaacgggtggcaatcgttcaccaccctcagagtgttgggagactttcacatttcatcatccttataatccacaaacagaaacatgaagggatgcaagtgagttcagcattcactcgtttggtgcactcaagtgctgagagaatgcagaatttacagtgtcacagaggaaaaaagccatctgaaataattgtaaaaatggttaagtgtggtatttaaatgttggttccctcctcttcatacaagtggaagaaaagaaggggctagggtacccactgggccatgaggttaaccccttagcacaggcaatgaagaacatccaatgccacagattctgcaggaggagaaatcccaagggtatacagtattcctgagaaagatcccagatttttctgaatcagtcttaatctgattttgttttggctacacagttatgctgttatacctttgacatacataaaaatggtcattttatttcaatccagacagctcagcattgtacaaatgatggcagaaagatccatttgttcagactcagcttgctttgtttttaatactggggaataaaccaaaaaaaaaagtgtaatttttatcatttgtatccttcattctactttactggagtggaatccccagggccttcagataatctgggaagacctgactattcctgtgaggcaagcacagccctgctgagctttactcagaataatgcatgatagactcaacgtaattcccaggaaaaagcccagtcactccattcataactccctcataccaaccatcgtcattcttcttgatgacataaataatggctccttcctgaaaggacagctcatcttccttgtcttttgtatagtcataaattgccacaaccttttccaagtaagaacgtggagcccacggtgggtcctcttcagcataaggatcactatactcaaccacagcagcttcctcctcttcgtaatcttctggaggaggaggaggtgggggagactcatcaaagactggttcttccacaggtggcggtggaggtggtgtatctgaaactggattctggctataaaaaggtcctccattcatctgattctgaaggcttgtttgtgaagtaatggaaggagggcgtctatagggcaacgagccccctattgttgggggagtatggcgagaggcaggcctattcatgctgtagaactgtacaggatgacctgtaagttcgatttctttgattcacagaagctgtcctcacagggctctgctgcgagggagccatattacgggttgggctaggtacgtaatcatttggtaccactggaggacgcactggctccagtgtgcgatagggggagtgccgcccaagtgtccctttccctgacatagggggactagggggcttctgagttggaggtgttgtacgcggcagcccacccatcttcatgttctgggtactcacctttactccatgtccaatatcatctagaattgtatagtcaataggttttctaatataacgaactggtcgttcaaggttggctggagcaataatcttatgtgtccttgaagtgtttttattggtagtcaaaataccaatttctcttcttgcaactttctctttatgaatatcaactgtttgtgaaatatgattgattgaagattccatccttcgtagctgggatgcctggatatccagcatctgcaggacattgttggccaaggtgtttatcagataggcaacacttgctaaggattgggtggtgtaggctttggtttcttctagggctctctgcttatctgctgactgtatgtagttgttctcgcagtaatcggccacccgttccagatttgtgtagctgtcgaagagggcccggcggccccccgggatttcctcttccagcagcatctgcagctccgccatcttcacatcctcctcctcctcctcctcatacaggtcgcagagggagcggcggccgcagcgccaaggaaacccaggaccgggagaggaggagcggcggcgacggcggcggtaactcggaagg

SEQ ID NO: 11798 - RNA, 4408 nt, Homo sapiens
  source 1..4408: mol_type = other RNA
ctgaatagctgggactacaggtgtgcgccaccacgcccagctaatttttgtgtttttagtagagatggggtttcaccatgttggccaggatggtctcaatttattgacctcatgatccacccacctcggcctccgaaagtgctgggattacaggcataagccaccacacccagcctgtgggaactatttattggatttcaaaacaccctctgcctcattaatccactaagctttctcagcaaaaagctgtttaaataaataatgggaacatctaatttaaaacagtttttctaattatagaccagtacacgaagaagagcttaacttatccaagtatagtctagtttgggtccataatggagctgaaggctcagaggacattcagggccattacactgcaggaaaacaaggaataagggatgtagaaatgacctaagaaaagcacgaagtggaatgtatactggaggcaagttaatgaaagctaataaatacaaagtgctgggaaaaatctaaaagcaaaatagctattgtaacttgcaatgcattaaaaacaactttaaaaccaaaaagtcttgataaggaaactctatagtggggtctcagttaaatgctgatgatttttaatgctcagataacattaagtggaatattaacttctgcatccgacaccatctgaattttctcacacactactacacttgttcacttttcaatcaagttccactttctgaacttgttcaaaacctcatttgaaatatatccagctactgcttttcccctttcacctagcacagggcagttacctggcaaagctctattctggccaagtcactgggactgagtagaacccacgttagcagctctggacctgaacaggagctggcccaacatcacagtgaccacccacaaagagacaagccctcctggatttttttcagcatttcttatactgactacagtagtgatgattaaagttatctgccctacagactccactgaatttgaagctgtatttattgtacagatgggggaaatgtgttttattgtgtcagttatattaatttttatcaatgtgattagatacatattttggcctattaatcttattcattatattcttagtctgagatgggttttaattctgactaacagcagctacttaagagtccaatcatacaaaatcaggagagtattaccctttctacagctaagcgagtcagtaatacagcagcaactaatactggccattaataacgtccagagagcacattagcaaaccttgtactcccagtgactgtcaggagacttgaaaataactactattctcttccaaagtagaatagcgtttttctagatagtgaaggaaatgatagtcatagttggtctgaactccaagatcctactcctcaaaacagcaccgaagcaggggttcgggatgcctgctaagagcatttccacagttcaagtctcttcagaaccttagggaccttcgtgtctagcttcacacacccacctccacatatgaaccagcctaccacacttcacatctgggtacactggccattagcaacaatgcagtctcatgcagcagcacattaaaatcaaacgggtggcaatcgttcaccaccctcagagtgttgggagactttcacatttcatcatccttataatccacaaacagaaacatgaagggatgcaagtgagttcagcattcactcgtttggtgcactcaagtgctgagagaatgcagaatttacagtgtcacagaggaaaaaagccatctgaaataattgtaaaaatggttaagtgtggtatttaaatgttggttccctcctcttcatacaagtggaagaaaagaaggggctagggtacccactgggccatgaggttaaccccttagcacaggcaatgaagaacatccaatgccacagattctgcaggaggagaaatcccaagggtatacagtattcctgagaaagatcccagatttttctgaatcagtcttaatctgattttgttttggctacacagttatgctgttatacctttgacatacataaaaatggtcattttatttcaatccagacagctcagcattgtacaaatgatggcagaaagatccatttgttcagactcagcttgctttgtttttaatactggggaataaaccaaaaaaaaaagtgtaatttttatcatttgtatccttcattctactttactggagtggaatccccagggccttcagataatctgggaagacctgactattcctgtgaggcaagcacagccctgctgagctttactcagaataatgcatgatagactcaacgtaattcccaggaaaaagcccagtcactccattcataactccctcataccaaccatcgtcattcttcttgatgacataaataatggctccttcctgaaaggacagctcatcttccttgtcttttgtatagtcataaattgccacaaccttttccaagtaagaacgtggagcccacggtgggtcctcttcagcataaggatcactatactcaaccacagcagcttcctcctcttcgtaatcttctggaggaggaggaggtgggggagactcatcaaagactggttcttccacaggtggcggtggaggtggtgtatctgaaactggattctggctataaaaaggtcctccattcatctgattctgaaggcttgtttgtgaagtaatggaaggagggcgtctatagggcaacgagccccctattgttgggggagtatggcgagaggcaggcctattcatgctgtagaactgtacaggatgacctgtagggggagtggaagaaacaacagggggagttggagaagtgaagccatcagcaagggtctgggcacccccagcagcagcgtctggggcagtggaggaagggacagtagcaggaacaagaggagcaggggcagatgcagaagtagcaggaaggggaggagtgccagcagagccagcaggggctggaaagacactgggaggagatggagtaggaacagcaataggaacccccacactaccacttccactgttctctcgactgctgctccgactacttgggtggctccctccactactcccactgccaagtgtccctttccctgacatagggggactagggggcttctgagttggaggtgttgtacgcggcagcccacccatcttcatgttctgggtactcaccttaaatctaagcaaccactttactccatgtccaatatcatctagaattgtatagtcaataggttttctaatataacgaactggtcgttcaaggttggctggagcaataatcttatgtgtccttgaagtgtttttattggtagtcaaaataccaatttctcttcttgcaactttctctttatgaatatcaactgtctcattcaatctcaaactgcaattgtttccaaatttggtcacaaaagtcgactcaagatcaacgcctctaatttgcttgtgaaatatgattgattgaagattccatccttcgtagctgggatgcctggatatccagcatctgcaggacattgttggccaaggtgtttatcagataggcaacacttgctaaggattgggtggtgtaggctttggtttcttctagggctctctgcttatctgctgactgtatgtagttgttctcgcagtaatcggccacccgttccagatttgtgtagctgtcgaagagggcccggcggccccccgggatttcctcttccagcagcatctgcagctccgccatcttcacatcctcctcctcctcctcctcatacaggtcgcagagggagcggcggccgcagcgccaaggaaacccaggaccgggagaggaggagcggcggcgacggcggcggtaactcggaaggagcgagaaacagccccagcgcgcgacaggggagggggcgacgggggcggggcgcgagccgacggactccgaggacggtcaccgcggcgacggccggccgggcgcgcgcacgcgcgctcccttccctccgcccccgggagcccgaaaaagattcccaccctcgcccgcgccgccggcccctcccccacttccggcgtctcctagcgacggcgggggtaggggccgggatgcgcgcgggagttggtggtgcagttaacccttccgccgcccgcccgccgctggagcggctggagaagcccccacctcccggcggcctttgttagcccggcgggaacacaccaccctgctcagctggcttcctgccggctccctccgggactcatctcggctccgtccccatggaggtcatcggcctagggaacttctcgaggcttttctccctctgctgctgacgggaggccgaaggagggcacagcctccactcttgggaccctcctctgtgaaagatcacacctcaacag

SEQ ID NO: 11799 - RNA, 3812 nt, Homo sapiens
  source 1..3812: mol_type = other RNA
ctgaatagctgggactacaggtgtgcgccaccacgcccagctaatttttgtgtttttagtagagatggggtttcaccatgttggccaggatggtctcaatttattgacctcatgatccacccacctcggcctccgaaagtgctgggattacaggcataagccaccacacccagcctgtgggaactatttattggatttcaaaacaccctctgcctcattaatccactaagctttctcagcaaaaagctgtttaaataaataatgggaacatctaatttaaaacagtttttctaattatagaccagtacacgaagaagagcttaacttatccaagtatagtctagtttgggtccataatggagctgaaggctcagaggacattcagggccattacactgcaggaaaacaaggaataagggatgtagaaatgacctaagaaaagcacgaagtggaatgtatactggaggcaagttaatgaaagctaataaatacaaagtgctgggaaaaatctaaaagcaaaatagctattgtaacttgcaatgcattaaaaacaactttaaaaccaaaaagtcttgataaggaaactctatagtggggtctcagttaaatgctgatgatttttaatgctcagataacattaagtggaatattaacttctgcatccgacaccatctgaattttctcacacactactacacttgttcacttttcaatcaagttccactttctgaacttgttcaaaacctcatttgaaatatatccagctactgcttttcccctttcacctagcacagggcagttacctggcaaagctctattctggccaagtcactgggactgagtagaacccacgttagcagctctggacctgaacaggagctggcccaacatcacagtgaccacccacaaagagacaagccctcctggatttttttcagcatttcttatactgactacagtagtgatgattaaagttatctgccctacagactccactgaatttgaagctgtatttattgtacagatgggggaaatgtgttttattgtgtcagttatattaatttttatcaatgtgattagatacatattttggcctattaatcttattcattatattcttagtctgagatgggttttaattctgactaacagcagctacttaagagtccaatcatacaaaatcaggagagtattaccctttctacagctaagcgagtcagtaatacagcagcaactaatactggccattaataacgtccagagagcacattagcaaaccttgtactcccagtgactgtcaggagacttgaaaataactactattctcttccaaagtagaatagcgtttttctagatagtgaaggaaatgatagtcatagttggtctgaactccaagatcctactcctcaaaacagcaccgaagcaggggttcgggatgcctgctaagagcatttccacagttcaagtctcttcagaaccttagggaccttcgtgtctagcttcacacacccacctccacatatgaaccagcctaccacacttcacatctgggtacactggccattagcaacaatgcagtctcatgcagcagcacattaaaatcaaacgggtggcaatcgttcaccaccctcagagtgttgggagactttcacatttcatcatccttataatccacaaacagaaacatgaagggatgcaagtgagttcagcattcactcgtttggtgcactcaagtgctgagagaatgcagaatttacagtgtcacagaggaaaaaagccatctgaaataattgtaaaaatggttaagtgtggtatttaaatgttggttccctcctcttcatacaagtggaagaaaagaaggggctagggtacccactgggccatgaggttaaccccttagcacaggcaatgaagaacatccaatgccacagattctgcaggaggagaaatcccaagggtatacagtattcctgagaaagatcccagatttttctgaatcagtcttaatctgattttgttttggctacacagttatgctgttatacctttgacatacataaaaatggtcattttatttcaatccagacagctcagcattgtacaaatgatggcagaaagatccatttgttcagactcagcttgctttgtttttaatactggggaataaaccaaaaaaaaaagtgtaatttttatcatttgtatccttcattctactttactggagtggaatccccagggccttcagataatctgggaagacctgactattcctgtgaggcaagcacagccctgctgagctttactcagaataatgcatgatagactcaacgtaattcccaggaaaaagcccagtcactccattcataactccctcataccaaccatcgtcattcttcttgatgacataaataatggctccttcctgaaaggacagctcatcttccttgtcttttgtatagtcataaattgccacaaccttttccaagtaagaacgtggagcccacggtgggtcctcttcagcataaggatcactatactcaaccacagcagcttcctcctcttcgtaatcttctggaggaggaggaggtgggggagactcatcaaagactggttcttccacaggtggcggtggaggtggtgtatctgaaactggattctggctataaaaaggtcctccattcatctgattctgaaggcttgtttgtgaagtaatggaaggagggcgtctatagggcaacgagccccctattgttgggggagtatggcgagaggcaggcctattcatgctgtagaactgtacaggatgacctgtagggggagtggaagaaacaacagggggagttggagaagtgaagccatcagcaagggtctgggcacccccagcagcagcgtctggggcagtggaggaagggacagtagcaggaacaagaggagcaggggcagatgcagaagtagcaggaaggggaggagtgccagcagagccagcaggggctggaaagacactgggaggagatggagtaggaacagcaataggaacccccacactaccacttccactgttctctcgactgctgctccgactacttgggtggctccctccactactcccactgccaagtgtccctttccctgacatagggggactagggggcttctgagttggaggtgttgtacgcggcagcccacccatcttcatgttctgggtactcaccttaaatctaagcaaccactttactccatgtccaatatcatctagaattgtatagtcaataggttttctaatataacgaactggtcgttcaaggttggctggagcaataatcttatgtgtccttgaagtgtttttattggtagtcaaaataccaatttctcttcttgcaactttctctttatgaatatcaactgtttgtgaaatatgattgattgaagattccatccttcgtagctgggatgcctggatatccagcatctgcaggacattgttggccaaggtgtttatcagataggcaacacttgctaaggattgggtggtgtaggctttggtttcttctagggctctctgcttatctgctgactgtatgtagttgttctcgcagtaatcggccacccgttccagatttgtgtagctgtcgaagagggcccggcggccccccgggatttcctcttccagcagcatctgcagctccgccatcttcacatcctcctcctcctcctcctcatacaggtcgcagagggagcggcggccgcagcgccaaggaaacccaggaccgggagaggaggagcggcggcgacggcggcggtaactcggaagg

SEQ ID NO: 11800 - RNA, 3808 nt, Homo sapiens
  source 1..3808: mol_type = other RNA
ctgaatagctgggactacaggtgtgcgccaccacgcccagctaatttttgtgtttttagtagagatggggtttcaccatgttggccaggatggtctcaatttattgacctcatgatccacccacctcggcctccgaaagtgctgggattacaggcataagccaccacacccagcctgtgggaactatttattggatttcaaaacaccctctgcctcattaatccactaagctttctcagcaaaaagctgtttaaataaataatgggaacatctaatttaaaacagtttttctaattatagaccagtacacgaagaagagcttaacttatccaagtatagtctagtttgggtccataatggagctgaaggctcagaggacattcagggccattacactgcaggaaaacaaggaataagggatgtagaaatgacctaagaaaagcacgaagtggaatgtatactggaggcaagttaatgaaagctaataaatacaaagtgctgggaaaaatctaaaagcaaaatagctattgtaacttgcaatgcattaaaaacaactttaaaaccaaaaagtcttgataaggaaactctatagtggggtctcagttaaatgctgatgatttttaatgctcagataacattaagtggaatattaacttctgcatccgacaccatctgaattttctcacacactactacacttgttcacttttcaatcaagttccactttctgaacttgttcaaaacctcatttgaaatatatccagctactgcttttcccctttcacctagcacagggcagttacctggcaaagctctattctggccaagtcactgggactgagtagaacccacgttagcagctctggacctgaacaggagctggcccaacatcacagtgaccacccacaaagagacaagccctcctggatttttttcagcatttcttatactgactacagtagtgatgattaaagttatctgccctacagactccactgaatttgaagctgtatttattgtacagatgggggaaatgtgttttattgtgtcagttatattaatttttatcaatgtgattagatacatattttggcctattaatcttattcattatattcttagtctgagatgggttttaattctgactaacagcagctacttaagagtccaatcatacaaaatcaggagagtattaccctttctacagctaagcgagtcagtaatacagcagcaactaatactggccattaataacgtccagagagcacattagcaaaccttgtactcccagtgactgtcaggagacttgaaaataactactattctcttccaaagtagaatagcgtttttctagatagtgaaggaaatgatagtcatagttggtctgaactccaagatcctactcctcaaaacagcaccgaagcaggggttcgggatgcctgctaagagcatttccacagttcaagtctcttcagaaccttagggaccttcgtgtctagcttcacacacccacctccacatatgaaccagcctaccacacttcacatctgggtacactggccattagcaacaatgcagtctcatgcagcagcacattaaaatcaaacgggtggcaatcgttcaccaccctcagagtgttgggagactttcacatttcatcatccttataatccacaaacagaaacatgaagggatgcaagtgagttcagcattcactcgtttggtgcactcaagtgctgagagaatgcagaatttacagtgtcacagaggaaaaaagccatctgaaataattgtaaaaatggttaagtgtggtatttaaatgttggttccctcctcttcatacaagtggaagaaaagaaggggctagggtacccactgggccatgaggttaaccccttagcacaggcaatgaagaacatccaatgccacagattctgcaggaggagaaatcccaagggtatacagtattcctgagaaagatcccagatttttctgaatcagtcttaatctgattttgttttggctacacagttatgctgttatacctttgacatacataaaaatggtcattttatttcaatccagacagctcagcattgtacaaatgatggcagaaagatccatttgttcagactcagcttgctttgtttttaatactggggaataaaccaaaaaaaaaagtgtaatttttatcatttgtatccttcattctactttactggagtggaatccccagggccttcagataatctgggaagacctgactattcctgtgaggcaagcacagccctgctgagctttactcagaataatgcatgatagactcaacgtaattcccaggaaaaagcccagtcactccattcataactccctcataccaaccatcgtcattcttcttgatgacataaataatggctccttcctgaaaggacagctcatcttccttgtcttttgtatagtcataaattgccacaaccttttccaagtaagaacgtggagcccacggtgggtcctcttcagcataaggatcactatactcaaccacagcagcttcctcctcttcgtaatcttctggaggaggaggaggtgggggagactcatcaaagactggttcttccacaggtggcggtggaggtggtgtatctgaaactggattctggctataaaaaggtcctccattcatctgattctgaaggcttgtttgtgaagtaatggaaggagggcgtctatagggcaacgagccccctattgttgggggagtatggcgagaggcaggcctattcatgctgtagaactgtacaggatgacctgtagggggagtggaagaaacaacagggggagttggagaagtgaagccatcagcaagggtctgggcacccccagcagcagcgtctggggcagtggaggaagggacagtagcaggaacaagaggagcaggggcagatgcagaagtagcaggaaggggaggagtgccagcagagccagcaggggctggaaagacactgggaggagatggagtaggaacagcaataggaacccccacactaccacttccactgttctctcgactgctgctccgactacttgggtggctccctccactactcccactgccaagtgtccctttccctgacatagggggactagggggcttctgagttggaggtgttgtacgcggcagcccacccatcttcatgttctgggtactcaccttaaatctaagcaaccactttactccatgtccaatatcatctagaattgtatagtcaataggttttctaatataacgaactggtcgttcaaggttggctggagcaataatcttatgtgtccttgaagtgtttttattggtagtcaaaataccaatttctcttcttgcaactttctctttatgaatatcaactgtttgtgaaatatgattgattgaagattccatccttcgtagctgggatgcctggatatccagcatctgcaggacattgttggccaaggtgtttatcagataggcaacacttgctaaggattgggtggtgtaggctttggtttcttctagggctctctgcttatctgctgtatgtagttgttctcgcagtaatcggccacccgttccagatttgtgtagctgtcgaagagggcccggcggccccccgggatttcctcttccagcagcatctgcagctccgccatcttcacatcctcctcctcctcctcctcatacaggtcgcagagggagcggcggccgcagcgccaaggaaacccaggaccgggagaggaggagcggcggcgacggcggcggtaactcggaagg

SEQ ID NO: 11801 - RNA, 3794 nt, Homo sapiens
  source 1..3794: mol_type = other RNA
ctgaatagctgggactacaggtgtgcgccaccacgcccagctaatttttgtgtttttagtagagatggggtttcaccatgttggccaggatggtctcaatttattgacctcatgatccacccacctcggcctccgaaagtgctgggattacaggcataagccaccacacccagcctgtgggaactatttattggatttcaaaacaccctctgcctcattaatccactaagctttctcagcaaaaagctgtttaaataaataatgggaacatctaatttaaaacagtttttctaattatagaccagtacacgaagaagagcttaacttatccaagtatagtctagtttgggtccataatggagctgaaggctcagaggacattcagggccattacactgcaggaaaacaaggaataagggatgtagaaatgacctaagaaaagcacgaagtggaatgtatactggaggcaagttaatgaaagctaataaatacaaagtgctgggaaaaatctaaaagcaaaatagctattgtaacttgcaatgcattaaaaacaactttaaaaccaaaaagtcttgataaggaaactctatagtggggtctcagttaaatgctgatgatttttaatgctcagataacattaagtggaatattaacttctgcatccgacaccatctgaattttctcacacactactacacttgttcacttttcaatcaagttccactttctgaacttgttcaaaacctcatttgaaatatatccagctactgcttttcccctttcacctagcacagggcagttacctggcaaagctctattctggccaagtcactgggactgagtagaacccacgttagcagctctggacctgaacaggagctggcccaacatcacagtgaccacccacaaagagacaagccctcctggatttttttcagcatttcttatactgactacagtagtgatgattaaagttatctgccctacagactccactgaatttgaagctgtatttattgtacagatgggggaaatgtgttttattgtgtcagttatattaatttttatcaatgtgattagatacatattttggcctattaatcttattcattatattcttagtctgagatgggttttaattctgactaacagcagctacttaagagtccaatcatacaaaatcaggagagtattaccctttctacagctaagcgagtcagtaatacagcagcaactaatactggccattaataacgtccagagagcacattagcaaaccttgtactcccagtgactgtcaggagacttgaaaataactactattctcttccaaagtagaatagcgtttttctagatagtgaaggaaatgatagtcatagttggtctgaactccaagatcctactcctcaaaacagcaccgaagcaggggttcgggatgcctgctaagagcatttccacagttcaagtctcttcagaaccttagggaccttcgtgtctagcttcacacacccacctccacatatgaaccagcctaccacacttcacatctgggtacactggccattagcaacaatgcagtctcatgcagcagcacattaaaatcaaacgggtggcaatcgttcaccaccctcagagtgttgggagactttcacatttcatcatccttataatccacaaacagaaacatgaagggatgcaagtgagttcagcattcactcgtttggtgcactcaagtgctgagagaatgcagaatttacagtgtcacagaggaaaaaagccatctgaaataattgtaaaaatggttaagtgtggtatttaaatgttggttccctcctcttcatacaagtggaagaaaagaaggggctagggtacccactgggccatgaggttaaccccttagcacaggcaatgaagaacatccaatgccacagattctgcaggaggagaaatcccaagggtatacagtattcctgagaaagatcccagatttttctgaatcagtcttaatctgattttgttttggctacacagttatgctgttatacctttgacatacataaaaatggtcattttatttcaatccagacagctcagcattgtacaaatgatggcagaaagatccatttgttcagactcagcttgctttgtttttaatactggggaataaaccaaaaaaaaaagtgtaatttttatcatttgtatccttcattctactttactggagtggaatccccagggccttcagataatctgggaagacctgactattcctgtgaggcaagcacagccctgctgagctttactcagaataatgcatgatagactcaacgtaattcccaggaaaaagcccagtcactccattcataactccctcataccaaccatcgtcattcttcttgatgacataaataatggctccttcctgaaaggacagctcatcttccttgtcttttgtatagtcataaattgccacaaccttttccaagtaagaacgtggagcccacggtgggtcctcttcagcataaggatcactatactcaaccacagcagcttcctcctcttcgtaatcttctggaggaggaggaggtgggggagactcatcaaagactggttcttccacaggtggcggtggaggtggtgtatctgaaactggattctggctataaaaaggtcctccattcatctgattctgaaggcttgtttgtgaagtaatggaaggagggcgtctatagggcaacgagccccctattgttgggggagtatggcgagaggcaggcctattcatgctgtagaactgtacaggatgacctgtagggggagtggaagaaacaacagggggagttggagaagtgaagccatcagcaagggtctgggcacccccagcagcagcgtctggggcagtggaggaagggacagtagcaggaacaagaggagcaggggcagatgcagaagtagcaggaaggggaggagtgccagcagagccagcaggggctggaaagacactgggaggagatggagtaggaacagcaataggaacccccacactaccacttccactgttctctcgactgctgctccgactacttgggtggctccctccactactcccactgccaagtgtccctttccctgacatagggggactagggggcttctgagttggaggtgttgtacgcggcagcccacccatcttcatgttctgggtactcacctttactccatgtccaatatcatctagaattgtatagtcaataggttttctaatataacgaactggtcgttcaaggttggctggagcaataatcttatgtgtccttgaagtgtttttattggtagtcaaaataccaatttctcttcttgcaactttctctttatgaatatcaactgtttgtgaaatatgattgattgaagattccatccttcgtagctgggatgcctggatatccagcatctgcaggacattgttggccaaggtgtttatcagataggcaacacttgctaaggattgggtggtgtaggctttggtttcttctagggctctctgcttatctgctgactgtatgtagttgttctcgcagtaatcggccacccgttccagatttgtgtagctgtcgaagagggcccggcggccccccgggatttcctcttccagcagcatctgcagctccgccatcttcacatcctcctcctcctcctcctcatacaggtcgcagagggagcggcggccgcagcgccaaggaaacccaggaccgggagaggaggagcggcggcgacggcggcggtaactcggaagg

SEQ ID NO: 11802 - RNA, 3901 nt, Homo sapiens
  source 1..3901: mol_type = other RNA
ctgaatagctgggactacaggtgtgcgccaccacgcccagctaatttttgtgtttttagtagagatggggtttcaccatgttggccaggatggtctcaatttattgacctcatgatccacccacctcggcctccgaaagtgctgggattacaggcataagccaccacacccagcctgtgggaactatttattggatttcaaaacaccctctgcctcattaatccactaagctttctcagcaaaaagctgtttaaataaataatgggaacatctaatttaaaacagtttttctaattatagaccagtacacgaagaagagcttaacttatccaagtatagtctagtttgggtccataatggagctgaaggctcagaggacattcagggccattacactgcaggaaaacaaggaataagggatgtagaaatgacctaagaaaagcacgaagtggaatgtatactggaggcaagttaatgaaagctaataaatacaaagtgctgggaaaaatctaaaagcaaaatagctattgtaacttgcaatgcattaaaaacaactttaaaaccaaaaagtcttgataaggaaactctatagtggggtctcagttaaatgctgatgatttttaatgctcagataacattaagtggaatattaacttctgcatccgacaccatctgaattttctcacacactactacacttgttcacttttcaatcaagttccactttctgaacttgttcaaaacctcatttgaaatatatccagctactgcttttcccctttcacctagcacagggcagttacctggcaaagctctattctggccaagtcactgggactgagtagaacccacgttagcagctctggacctgaacaggagctggcccaacatcacagtgaccacccacaaagagacaagccctcctggatttttttcagcatttcttatactgactacagtagtgatgattaaagttatctgccctacagactccactgaatttgaagctgtatttattgtacagatgggggaaatgtgttttattgtgtcagttatattaatttttatcaatgtgattagatacatattttggcctattaatcttattcattatattcttagtctgagatgggttttaattctgactaacagcagctacttaagagtccaatcatacaaaatcaggagagtattaccctttctacagctaagcgagtcagtaatacagcagcaactaatactggccattaataacgtccagagagcacattagcaaaccttgtactcccagtgactgtcaggagacttgaaaataactactattctcttccaaagtagaatagcgtttttctagatagtgaaggaaatgatagtcatagttggtctgaactccaagatcctactcctcaaaacagcaccgaagcaggggttcgggatgcctgctaagagcatttccacagttcaagtctcttcagaaccttagggaccttcgtgtctagcttcacacacccacctccacatatgaaccagcctaccacacttcacatctgggtacactggccattagcaacaatgcagtctcatgcagcagcacattaaaatcaaacgggtggcaatcgttcaccaccctcagagtgttgggagactttcacatttcatcatccttataatccacaaacagaaacatgaagggatgcaagtgagttcagcattcactcgtttggtgcactcaagtgctgagagaatgcagaatttacagtgtcacagaggaaaaaagccatctgaaataattgtaaaaatggttaagtgtggtatttaaatgttggttccctcctcttcatacaagtggaagaaaagaaggggctagggtacccactgggccatgaggttaaccccttagcacaggcaatgaagaacatccaatgccacagattctgcaggaggagaaatcccaagggtatacagtattcctgagaaagatcccagatttttctgaatcagtcttaatctgattttgttttggctacacagttatgctgttatacctttgacatacataaaaatggtcattttatttcaatccagacagctcagcattgtacaaatgatggcagaaagatccatttgttcagactcagcttgctttgtttttaatactggggaataaaccaaaaaaaaaagtgtaatttttatcatttgtatccttcattctactttactggagtggaatccccagggccttcagataatctgggaagacctgactattcctgtgaggcaagcacagccctgctgagctttactcagaataatgcatgatagactcaacgtaattcccaggaaaaagcccagtcactccattcataactccctcataccaaccatcgtcattcttcttgatgacataaataatggctccttcctgaaaggacagctcatcttccttgtcttttgtatagtcataaattgccacaaccttttccaagtaagaacgtggagcccacggtgggtcctcttcagcataaggatcactatactcaaccacagcagcttcctcctcttcgtaatcttctggaggaggaggaggtgggggagactcatcaaagactggttcttccacaggtggcggtggaggtggtgtatctgaaactggattctggctataaaaaggtcctccattcatctgattctgaaggcttgtttgtgaagtaatggaaggagggcgtctatagggcaacgagccccctattgttgggggagtatggcgagaggcaggcctattcatgctgtagaactgtacaggatgacctgtagggggagtggaagaaacaacagggggagttggagaagtgaagccatcagcaagggtctgggcacccccagcagcagcgtctggggcagtggaggaagggacagtagcaggaacaagaggagcaggggcagatgcagaagtagcaggaaggggaggagtgccagcagagccagcaggggctggaaagacactgggaggagatggagtaggaacagcaataggaacccccacactaccacttccactgttctctcgactgctgctccgactacttgggtggctccctccactactcccactgctgccaagtgtccctttccctgacatagggggactagggggcttctgagttggaggtgttgtacgcggcagcccacccatcttcatgttctgggtactcaccttaaatctaagcaaccactttactccatgtccaatatcatctagaattgtatagtcaataggttttctaatataacgaactggtcgttcaaggttggctggagcaataatcttatgtgtccttgaagtgtttttattggtagtcaaaataccaatttctcttcttgcaactttctctttatgaatatcaactgtataataaaagctgccagcattacagatagcctgtgtttattattaagggttcctcataggcaaataggaaaatattgtggtctcacttgtgaaatatgattgattgaagattccatccttcgtagctgggatgcctggatatccagcatctgcaggacattgttggccaaggtgtttatcagataggcaacacttgctaaggattgggtggtgtaggctttggtttcttctagggctctctgcttatctgctgactgtatgtagttgttctcgcagtaatcggccacccgttccagatttgtgtagctgtcgaagagggcccggcggccccccgggatttcctcttccagcagcatctgcagctccgccatcttcacatcctcctcctcctcctcctcatacaggtcgcagagggagcggcggccgcagcgccaaggaaacccaggaccgggagaggaggagcggcggcgacggcggcggtaactcggaagg

SEQ ID NO: 11803 - RNA, 3647 nt, Homo sapiens
  source 1..3647: mol_type = other RNA
ctgaatagctgggactacaggtgtgcgccaccacgcccagctaatttttgtgtttttagtagagatggggtttcaccatgttggccaggatggtctcaatttattgacctcatgatccacccacctcggcctccgaaagtgctgggattacaggcataagccaccacacccagcctgtgggaactatttattggatttcaaaacaccctctgcctcattaatccactaagctttctcagcaaaaagctgtttaaataaataatgggaacatctaatttaaaacagtttttctaattatagaccagtacacgaagaagagcttaacttatccaagtatagtctagtttgggtccataatggagctgaaggctcagaggacattcagggccattacactgcaggaaaacaaggaataagggatgtagaaatgacctaagaaaagcacgaagtggaatgtatactggaggcaagttaatgaaagctaataaatacaaagtgctgggaaaaatctaaaagcaaaatagctattgtaacttgcaatgcattaaaaacaactttaaaaccaaaaagtcttgataaggaaactctatagtggggtctcagttaaatgctgatgatttttaatgctcagataacattaagtggaatattaacttctgcatccgacaccatctgaattttctcacacactactacacttgttcacttttcaatcaagttccactttctgaacttgttcaaaacctcatttgaaatatatccagctactgcttttcccctttcacctagcacagggcagttacctggcaaagctctattctggccaagtcactgggactgagtagaacccacgttagcagctctggacctgaacaggagctggcccaacatcacagtgaccacccacaaagagacaagccctcctggatttttttcagcatttcttatactgactacagtagtgatgattaaagttatctgccctacagactccactgaatttgaagctgtatttattgtacagatgggggaaatgtgttttattgtgtcagttatattaatttttatcaatgtgattagatacatattttggcctattaatcttattcattatattcttagtctgagatgggttttaattctgactaacagcagctacttaagagtccaatcatacaaaatcaggagagtattaccctttctacagctaagcgagtcagtaatacagcagcaactaatactggccattaataacgtccagagagcacattagcaaaccttgtactcccagtgactgtcaggagacttgaaaataactactattctcttccaaagtagaatagcgtttttctagatagtgaaggaaatgatagtcatagttggtctgaactccaagatcctactcctcaaaacagcaccgaagcaggggttcgggatgcctgctaagagcatttccacagttcaagtctcttcagaaccttagggaccttcgtgtctagcttcacacacccacctccacatatgaaccagcctaccacacttcacatctgggtacactggccattagcaacaatgcagtctcatgcagcagcacattaaaatcaaacgggtggcaatcgttcaccaccctcagagtgttgggagactttcacatttcatcatccttataatccacaaacagaaacatgaagggatgcaagtgagttcagcattcactcgtttggtgcactcaagtgctgagagaatgcagaatttacagtgtcacagaggaaaaaagccatctgaaataattgtaaaaatggttaagtgtggtatttaaatgttggttccctcctcttcatacaagtggaagaaaagaaggggctagggtacccactgggccatgaggttaaccccttagcacaggcaatgaagaacatccaatgccacagattctgcaggaggagaaatcccaagggtatacagtattcctgagaaagatcccagatttttctgaatcagtcttaatctgattttgttttggctacacagttatgctgttatacctttgacatacataaaaatggtcattttatttcaatccagacagctcagcattgtacaaatgatggcagaaagatccatttgttcagactcagcttgctttgtttttaatactggggaataaaccaaaaaaaaaagtgtaatttttatcatttgtatccttcattctactttactggagtggaatccccagggccttcagataatctgggaagacctgactattcctgtgaggcaagcacagccctgctgagctttactcagaataatgcatgatagactcaacgtaattcccaggaaaaagcccagtcactccattcataactccctcataccaaccatcgtcattcttcttgatgacataaataatggctccttcctgaaaggacagctcatcttccttgtcttttgtatagtcataaattgccacaaccttttccaagtaagaacgtggagcccacggtgggtcctcttcagcataaggatcactatactcaaccacagcagcttcctcctcttcgtaatcttctggaggaggaggaggtgggggagactcatcaaagactggttcttccacaggtggcggtggaggtggtgtatctgaaactggattctggctataaaaaggtcctccattcatctgattctgaaggcttgtttgtgaagtaatggaaggagggcgtctatagggcaacgagccccctattgttgggggagtatggcgagaggcaggcctattcatgctgtagaactgtacaggatgacctgtagggggagtggaagaaacaacagggggagttggagaagtgaagccatcagcaagggtctgggcacccccagcagcagcgtctggggcagtggaggaagggacagtagcaggaacaagaggagcaggggcagatgcagaagtagcaggaaggggaggagtgccagcagagccagcaggggctggaaagacactgggaggagatggagtaggaacagcaataggaacccccacactaccacttccactgttctctcgactgctgctccgactacttgggtggctccctccactactcccactgctgccaagtgtccctttccctgacatagggggactagggggcttctgagttggaggtgttgtacgcggcagcccacccatcttcatgttctgggtactcaccttaaatctaagcaaccactttactccatgtccaatatcatctagaattgtatagtcaataggttttctaatataacgaactggtcgttcaaggttggctggagcaataatcttatgtgtccttgaagtgtttttattggtagtcaaaataccaatttctcttcttgcaactttctctttatgaatatcaactgtctgtatgtagttgttctcgcagtaatcggccacccgttccagatttgtgtagctgtcgaagagggcccggcggccccccgggatttcctcttccagcagcatctgcagctccgccatcttcacatcctcctcctcctcctcctcatacaggtcgcagagggagcggcggccgcagcgccaaggaaacccaggaccgggagaggaggagcggcggcgacggcggcggtaactcggaagg

SEQ ID NO: 11804 - RNA, 3939 nt, Homo sapiens
  source 1..3939: mol_type = other RNA
ctgaatagctgggactacaggtgtgcgccaccacgcccagctaatttttgtgtttttagtagagatggggtttcaccatgttggccaggatggtctcaatttattgacctcatgatccacccacctcggcctccgaaagtgctgggattacaggcataagccaccacacccagcctgtgggaactatttattggatttcaaaacaccctctgcctcattaatccactaagctttctcagcaaaaagctgtttaaataaataatgggaacatctaatttaaaacagtttttctaattatagaccagtacacgaagaagagcttaacttatccaagtatagtctagtttgggtccataatggagctgaaggctcagaggacattcagggccattacactgcaggaaaacaaggaataagggatgtagaaatgacctaagaaaagcacgaagtggaatgtatactggaggcaagttaatgaaagctaataaatacaaagtgctgggaaaaatctaaaagcaaaatagctattgtaacttgcaatgcattaaaaacaactttaaaaccaaaaagtcttgataaggaaactctatagtggggtctcagttaaatgctgatgatttttaatgctcagataacattaagtggaatattaacttctgcatccgacaccatctgaattttctcacacactactacacttgttcacttttcaatcaagttccactttctgaacttgttcaaaacctcatttgaaatatatccagctactgcttttcccctttcacctagcacagggcagttacctggcaaagctctattctggccaagtcactgggactgagtagaacccacgttagcagctctggacctgaacaggagctggcccaacatcacagtgaccacccacaaagagacaagccctcctggatttttttcagcatttcttatactgactacagtagtgatgattaaagttatctgccctacagactccactgaatttgaagctgtatttattgtacagatgggggaaatgtgttttattgtgtcagttatattaatttttatcaatgtgattagatacatattttggcctattaatcttattcattatattcttagtctgagatgggttttaattctgactaacagcagctacttaagagtccaatcatacaaaatcaggagagtattaccctttctacagctaagcgagtcagtaatacagcagcaactaatactggccattaataacgtccagagagcacattagcaaaccttgtactcccagtgactgtcaggagacttgaaaataactactattctcttccaaagtagaatagcgtttttctagatagtgaaggaaatgatagtcatagttggtctgaactccaagatcctactcctcaaaacagcaccgaagcaggggttcgggatgcctgctaagagcatttccacagttcaagtctcttcagaaccttagggaccttcgtgtctagcttcacacacccacctccacatatgaaccagcctaccacacttcacatctgggtacactggccattagcaacaatgcagtctcatgcagcagcacattaaaatcaaacgggtggcaatcgttcaccaccctcagagtgttgggagactttcacatttcatcatccttataatccacaaacagaaacatgaagggatgcaagtgagttcagcattcactcgtttggtgcactcaagtgctgagagaatgcagaatttacagtgtcacagaggaaaaaagccatctgaaataattgtaaaaatggttaagtgtggtatttaaatgttggttccctcctcttcatacaagtggaagaaaagaaggggctagggtacccactgggccatgaggttaaccccttagcacaggcaatgaagaacatccaatgccacagattctgcaggaggagaaatcccaagggtatacagtattcctgagaaagatcccagatttttctgaatcagtcttaatctgattttgttttggctacacagttatgctgttatacctttgacatacataaaaatggtcattttatttcaatccagacagctcagcattgtacaaatgatggcagaaagatccatttgttcagactcagcttgctttgtttttaatactggggaataaaccaaaaaaaaaagtgtaatttttatcatttgtatccttcattctactttactggagtggaatccccagggccttcagataatctgggaagacctgactattcctgtgaggcaagcacagccctgctgagctttactcagaataatgcatgatagactcaacgtaattcccaggaaaaagcccagtcactccattcataactccctcataccaaccatcgtcattcttcttgatgacataaataatggctccttcctgaaaggacagctcatcttccttgtcttttgtatagtcataaattgccacaaccttttccaagtaagaacgtggagcccacggtgggtcctcttcagcataaggatcactatactcaaccacagcagcttcctcctcttcgtaatcttctggaggaggaggaggtgggggagactcatcaaagactggttcttccacaggtggcggtggaggtggtgtatctgaaactggattctggctataaaaaggtcctccattcatctgattctgaaggcttgtttgtgaagtaatggaaggagggcgtctatagggcaacgagccccctattgttgggggagtatggcgagaggcaggcctattcatgctgtagaactgtacaggatgacctgtagggggagtggaagaaacaacagggggagttggagaagtgaagccatcagcaagggtctgggcacccccagcagcagcgtctggggcagtggaggaagggacagtagcaggaacaagaggagcaggggcagatgcagaagtagcaggaaggggaggagtgccagcagagccagcaggggctggaaagacactgggaggagatggagtaggaacagcaataggaacccccacactaccacttccactgttctctcgactgctgctccgactacttgggtggctccctccactactcccactgctgccaagtgtccctttccctgacatagggggactagggggcttctgagttggaggtgttgtacgcggcagcccacccatcttcatgttctgggtactcaccttaaatctaagcaaccactttactccatgtccaatatcatctagaattgtatagtcaataggttttctaatataacgaactggtcgttcaaggttggctggagcaataatcttatgtgtccttgaagtgtttttattggtagtcaaaataccaatttctcttcttgcaactttctctttatgaatatcaactgtttgtgaaatatgattgattgaagattccatccttcgtagctgggatgcctggatatccagcatctgcaggacattgttggccaaggtgtttatcagataggcaacacttgctaaggattgggtggtgtaggctttggtttcttctagggctctctgcttatctgctgactgtagtcccagactactgagagactgaggcaggatgatcacttgagcacaggagttcaaggctgcagtgagctatgatcacaccactgcattccagcctgcatgacataccaagaccccatctctgtatgtagttgttctcgcagtaatcggccacccgttccagatttgtgtagctgtcgaagagggcccggcggccccccgggatttcctcttccagcagcatctgcagctccgccatcttcacatcctcctcctcctcctcctcatacaggtcgcagagggagcggcggccgcagcgccaaggaaacccaggaccgggagaggaggagcggcggcgacggcggcggtaactcggaagg

SEQ ID NO: 11805 - RNA, 3815 nt, Homo sapiens
  source 1..3815: mol_type = other RNA
ctgaatagctgggactacaggtgtgcgccaccacgcccagctaatttttgtgtttttagtagagatggggtttcaccatgttggccaggatggtctcaatttattgacctcatgatccacccacctcggcctccgaaagtgctgggattacaggcataagccaccacacccagcctgtgggaactatttattggatttcaaaacaccctctgcctcattaatccactaagctttctcagcaaaaagctgtttaaataaataatgggaacatctaatttaaaacagtttttctaattatagaccagtacacgaagaagagcttaacttatccaagtatagtctagtttgggtccataatggagctgaaggctcagaggacattcagggccattacactgcaggaaaacaaggaataagggatgtagaaatgacctaagaaaagcacgaagtggaatgtatactggaggcaagttaatgaaagctaataaatacaaagtgctgggaaaaatctaaaagcaaaatagctattgtaacttgcaatgcattaaaaacaactttaaaaccaaaaagtcttgataaggaaactctatagtggggtctcagttaaatgctgatgatttttaatgctcagataacattaagtggaatattaacttctgcatccgacaccatctgaattttctcacacactactacacttgttcacttttcaatcaagttccactttctgaacttgttcaaaacctcatttgaaatatatccagctactgcttttcccctttcacctagcacagggcagttacctggcaaagctctattctggccaagtcactgggactgagtagaacccacgttagcagctctggacctgaacaggagctggcccaacatcacagtgaccacccacaaagagacaagccctcctggatttttttcagcatttcttatactgactacagtagtgatgattaaagttatctgccctacagactccactgaatttgaagctgtatttattgtacagatgggggaaatgtgttttattgtgtcagttatattaatttttatcaatgtgattagatacatattttggcctattaatcttattcattatattcttagtctgagatgggttttaattctgactaacagcagctacttaagagtccaatcatacaaaatcaggagagtattaccctttctacagctaagcgagtcagtaatacagcagcaactaatactggccattaataacgtccagagagcacattagcaaaccttgtactcccagtgactgtcaggagacttgaaaataactactattctcttccaaagtagaatagcgtttttctagatagtgaaggaaatgatagtcatagttggtctgaactccaagatcctactcctcaaaacagcaccgaagcaggggttcgggatgcctgctaagagcatttccacagttcaagtctcttcagaaccttagggaccttcgtgtctagcttcacacacccacctccacatatgaaccagcctaccacacttcacatctgggtacactggccattagcaacaatgcagtctcatgcagcagcacattaaaatcaaacgggtggcaatcgttcaccaccctcagagtgttgggagactttcacatttcatcatccttataatccacaaacagaaacatgaagggatgcaagtgagttcagcattcactcgtttggtgcactcaagtgctgagagaatgcagaatttacagtgtcacagaggaaaaaagccatctgaaataattgtaaaaatggttaagtgtggtatttaaatgttggttccctcctcttcatacaagtggaagaaaagaaggggctagggtacccactgggccatgaggttaaccccttagcacaggcaatgaagaacatccaatgccacagattctgcaggaggagaaatcccaagggtatacagtattcctgagaaagatcccagatttttctgaatcagtcttaatctgattttgttttggctacacagttatgctgttatacctttgacatacataaaaatggtcattttatttcaatccagacagctcagcattgtacaaatgatggcagaaagatccatttgttcagactcagcttgctttgtttttaatactggggaataaaccaaaaaaaaaagtgtaatttttatcatttgtatccttcattctactttactggagtggaatccccagggccttcagataatctgggaagacctgactattcctgtgaggcaagcacagccctgctgagctttactcagaataatgcatgatagactcaacgtaattcccaggaaaaagcccagtcactccattcataactccctcataccaaccatcgtcattcttcttgatgacataaataatggctccttcctgaaaggacagctcatcttccttgtcttttgtatagtcataaattgccacaaccttttccaagtaagaacgtggagcccacggtgggtcctcttcagcataaggatcactatactcaaccacagcagcttcctcctcttcgtaatcttctggaggaggaggaggtgggggagactcatcaaagactggttcttccacaggtggcggtggaggtggtgtatctgaaactggattctggctataaaaaggtcctccattcatctgattctgaaggcttgtttgtgaagtaatggaaggagggcgtctatagggcaacgagccccctattgttgggggagtatggcgagaggcaggcctattcatgctgtagaactgtacaggatgacctgtagggggagtggaagaaacaacagggggagttggagaagtgaagccatcagcaagggtctgggcacccccagcagcagcgtctggggcagtggaggaagggacagtagcaggaacaagaggagcaggggcagatgcagaagtagcaggaaggggaggagtgccagcagagccagcaggggctggaaagacactgggaggagatggagtaggaacagcaataggaacccccacactaccacttccactgttctctcgactgctgctccgactacttgggtggctccctccactactcccactgctgccaagtgtccctttccctgacatagggggactagggggcttctgagttggaggtgttgtacgcggcagcccacccatcttcatgttctgggtactcaccttaaatctaagcaaccactttactccatgtccaatatcatctagaattgtatagtcaataggttttctaatataacgaactggtcgttcaaggttggctggagcaataatcttatgtgtccttgaagtgtttttattggtagtcaaaataccaatttctcttcttgcaactttctctttatgaatatcaactgtttgtgaaatatgattgattgaagattccatccttcgtagctgggatgcctggatatccagcatctgcaggacattgttggccaaggtgtttatcagataggcaacacttgctaaggattgggtggtgtaggctttggtttcttctagggctctctgcttatctgctgactgtatgtagttgttctcgcagtaatcggccacccgttccagatttgtgtagctgtcgaagagggcccggcggccccccgggatttcctcttccagcagcatctgcagctccgccatcttcacatcctcctcctcctcctcctcatacaggtcgcagagggagcggcggccgcagcgccaaggaaacccaggaccgggagaggaggagcggcggcgacggcggcggtaactcggaagg

SEQ ID NO: 11806 - RNA, 3927 nt, Homo sapiens
  source 1..3927: mol_type = other RNA
ctgaatagctgggactacaggtgtgcgccaccacgcccagctaatttttgtgtttttagtagagatggggtttcaccatgttggccaggatggtctcaatttattgacctcatgatccacccacctcggcctccgaaagtgctgggattacaggcataagccaccacacccagcctgtgggaactatttattggatttcaaaacaccctctgcctcattaatccactaagctttctcagcaaaaagctgtttaaataaataatgggaacatctaatttaaaacagtttttctaattatagaccagtacacgaagaagagcttaacttatccaagtatagtctagtttgggtccataatggagctgaaggctcagaggacattcagggccattacactgcaggaaaacaaggaataagggatgtagaaatgacctaagaaaagcacgaagtggaatgtatactggaggcaagttaatgaaagctaataaatacaaagtgctgggaaaaatctaaaagcaaaatagctattgtaacttgcaatgcattaaaaacaactttaaaaccaaaaagtcttgataaggaaactctatagtggggtctcagttaaatgctgatgatttttaatgctcagataacattaagtggaatattaacttctgcatccgacaccatctgaattttctcacacactactacacttgttcacttttcaatcaagttccactttctgaacttgttcaaaacctcatttgaaatatatccagctactgcttttcccctttcacctagcacagggcagttacctggcaaagctctattctggccaagtcactgggactgagtagaacccacgttagcagctctggacctgaacaggagctggcccaacatcacagtgaccacccacaaagagacaagccctcctggatttttttcagcatttcttatactgactacagtagtgatgattaaagttatctgccctacagactccactgaatttgaagctgtatttattgtacagatgggggaaatgtgttttattgtgtcagttatattaatttttatcaatgtgattagatacatattttggcctattaatcttattcattatattcttagtctgagatgggttttaattctgactaacagcagctacttaagagtccaatcatacaaaatcaggagagtattaccctttctacagctaagcgagtcagtaatacagcagcaactaatactggccattaataacgtccagagagcacattagcaaaccttgtactcccagtgactgtcaggagacttgaaaataactactattctcttccaaagtagaatagcgtttttctagatagtgaaggaaatgatagtcatagttggtctgaactccaagatcctactcctcaaaacagcaccgaagcaggggttcgggatgcctgctaagagcatttccacagttcaagtctcttcagaaccttagggaccttcgtgtctagcttcacacacccacctccacatatgaaccagcctaccacacttcacatctgggtacactggccattagcaacaatgcagtctcatgcagcagcacattaaaatcaaacgggtggcaatcgttcaccaccctcagagtgttgggagactttcacatttcatcatccttataatccacaaacagaaacatgaagggatgcaagtgagttcagcattcactcgtttggtgcactcaagtgctgagagaatgcagaatttacagtgtcacagaggaaaaaagccatctgaaataattgtaaaaatggttaagtgtggtatttaaatgttggttccctcctcttcatacaagtggaagaaaagaaggggctagggtacccactgggccatgaggttaaccccttagcacaggcaatgaagaacatccaatgccacagattctgcaggaggagaaatcccaagggtatacagtattcctgagaaagatcccagatttttctgaatcagtcttaatctgattttgttttggctacacagttatgctgttatacctttgacatacataaaaatggtcattttatttcaatccagacagctcagcattgtacaaatgatggcagaaagatccatttgttcagactcagcttgctttgtttttaatactggggaataaaccaaaaaaaaaagtgtaatttttatcatttgtatccttcattctactttactggagtggaatccccagggccttcagataatctgggaagacctgactattcctgtgaggcaagcacagccctgctgagctttactcagaataatgcatgatagactcaacgtaattcccaggaaaaagcccagtcactccattcataactccctcataccaaccatcgtcattcttcttgatgacataaataatggctccttcctgaaaggacagctcatcttccttgtcttttgtatagtcataaattgccacaaccttttccaagtaagaacgtggagcccacggtgggtcctcttcagcataaggatcactatactcaaccacagcagcttcctcctcttcgtaatcttctggaggaggaggaggtgggggagactcatcaaagactggttcttccacaggtggcggtggaggtggtgtatctgaaactggattctggctataaaaaggtcctccattcatctgattctgaaggcttgtttgtgaagtaatggaaggagggcgtctatagggcaacgagccccctattgttgggggagtatggcgagaggcaggcctattcatgctgtagaactgtacaggatgacctgtagggggagtggaagaaacaacagggggagttggagaagtgaagccatcagcaagggtctgggcacccccagcagcagcgtctggggcagtggaggaagggacagtagcaggaacaagaggagcaggggcagatgcagaagtagcaggaaggggaggagtgccagcagagccagcaggggctggaaagacactgggaggagatggagtaggaacagcaataggaacccccacactaccacttccactgttctctcgactgctgctccgactacttgggtggctccctccactactcccactgctgccaagtgtccctttccctgacatagggggactagggggcttctgagttggaggtgttgtacgcggcagcccacccatcttcatgttctgggtactcaccttaaatctaagcaaccactttactccatgtccaatatcatctagaattgtatagtcaataggttttctaatataacgaactggtcgttcaaggttggctggagcaataatcttatgtgtccttgaagtgtttttattggtagtcaaaataccaatttctcttcttgcaactttctctttatgaatatcaactgtttgtgaaatatgattgattgaagattccatccttcgtagctgggatgcctggatatccagcatctgcaggacattgttggccaaggtgtttatcagataggcaacacttgctaaggattgggtggtgtaggctttggtttcttctagggctctctgcttatctgctgacttccttcttacagctgatgtgttcattcaggcagtaatatggtatcatacacactggtgatacacatgcctattagtcccatatattcccaagctgcagaaatattttcctctgtatgtagttgttctcgcagtaatcggccacccgttccagatttgtgtagctgtcgaagagggcccggcggccccccgggatttcctcttccagcagcatctgcagctccgccatcttcacatcctcctcctcctcctcctcatacaggtcgcagagggagcggcggccgcagcgccaaggaaacccaggaccgggagaggaggagcggcggcgacggcggcggtaactcggaagg

SEQ ID NO: 11807 - RNA, 3811 nt, Homo sapiens
  source 1..3811: mol_type = other RNA
ctgaatagctgggactacaggtgtgcgccaccacgcccagctaatttttgtgtttttagtagagatggggtttcaccatgttggccaggatggtctcaatttattgacctcatgatccacccacctcggcctccgaaagtgctgggattacaggcataagccaccacacccagcctgtgggaactatttattggatttcaaaacaccctctgcctcattaatccactaagctttctcagcaaaaagctgtttaaataaataatgggaacatctaatttaaaacagtttttctaattatagaccagtacacgaagaagagcttaacttatccaagtatagtctagtttgggtccataatggagctgaaggctcagaggacattcagggccattacactgcaggaaaacaaggaataagggatgtagaaatgacctaagaaaagcacgaagtggaatgtatactggaggcaagttaatgaaagctaataaatacaaagtgctgggaaaaatctaaaagcaaaatagctattgtaacttgcaatgcattaaaaacaactttaaaaccaaaaagtcttgataaggaaactctatagtggggtctcagttaaatgctgatgatttttaatgctcagataacattaagtggaatattaacttctgcatccgacaccatctgaattttctcacacactactacacttgttcacttttcaatcaagttccactttctgaacttgttcaaaacctcatttgaaatatatccagctactgcttttcccctttcacctagcacagggcagttacctggcaaagctctattctggccaagtcactgggactgagtagaacccacgttagcagctctggacctgaacaggagctggcccaacatcacagtgaccacccacaaagagacaagccctcctggatttttttcagcatttcttatactgactacagtagtgatgattaaagttatctgccctacagactccactgaatttgaagctgtatttattgtacagatgggggaaatgtgttttattgtgtcagttatattaatttttatcaatgtgattagatacatattttggcctattaatcttattcattatattcttagtctgagatgggttttaattctgactaacagcagctacttaagagtccaatcatacaaaatcaggagagtattaccctttctacagctaagcgagtcagtaatacagcagcaactaatactggccattaataacgtccagagagcacattagcaaaccttgtactcccagtgactgtcaggagacttgaaaataactactattctcttccaaagtagaatagcgtttttctagatagtgaaggaaatgatagtcatagttggtctgaactccaagatcctactcctcaaaacagcaccgaagcaggggttcgggatgcctgctaagagcatttccacagttcaagtctcttcagaaccttagggaccttcgtgtctagcttcacacacccacctccacatatgaaccagcctaccacacttcacatctgggtacactggccattagcaacaatgcagtctcatgcagcagcacattaaaatcaaacgggtggcaatcgttcaccaccctcagagtgttgggagactttcacatttcatcatccttataatccacaaacagaaacatgaagggatgcaagtgagttcagcattcactcgtttggtgcactcaagtgctgagagaatgcagaatttacagtgtcacagaggaaaaaagccatctgaaataattgtaaaaatggttaagtgtggtatttaaatgttggttccctcctcttcatacaagtggaagaaaagaaggggctagggtacccactgggccatgaggttaaccccttagcacaggcaatgaagaacatccaatgccacagattctgcaggaggagaaatcccaagggtatacagtattcctgagaaagatcccagatttttctgaatcagtcttaatctgattttgttttggctacacagttatgctgttatacctttgacatacataaaaatggtcattttatttcaatccagacagctcagcattgtacaaatgatggcagaaagatccatttgttcagactcagcttgctttgtttttaatactggggaataaaccaaaaaaaaaagtgtaatttttatcatttgtatccttcattctactttactggagtggaatccccagggccttcagataatctgggaagacctgactattcctgtgaggcaagcacagccctgctgagctttactcagaataatgcatgatagactcaacgtaattcccaggaaaaagcccagtcactccattcataactccctcataccaaccatcgtcattcttcttgatgacataaataatggctccttcctgaaaggacagctcatcttccttgtcttttgtatagtcataaattgccacaaccttttccaagtaagaacgtggagcccacggtgggtcctcttcagcataaggatcactatactcaaccacagcagcttcctcctcttcgtaatcttctggaggaggaggaggtgggggagactcatcaaagactggttcttccacaggtggcggtggaggtggtgtatctgaaactggattctggctataaaaaggtcctccattcatctgattctgaaggcttgtttgtgaagtaatggaaggagggcgtctatagggcaacgagccccctattgttgggggagtatggcgagaggcaggcctattcatgctgtagaactgtacaggatgacctgtagggggagtggaagaaacaacagggggagttggagaagtgaagccatcagcaagggtctgggcacccccagcagcagcgtctggggcagtggaggaagggacagtagcaggaacaagaggagcaggggcagatgcagaagtagcaggaaggggaggagtgccagcagagccagcaggggctggaaagacactgggaggagatggagtaggaacagcaataggaacccccacactaccacttccactgttctctcgactgctgctccgactacttgggtggctccctccactactcccactgctgccaagtgtccctttccctgacatagggggactagggggcttctgagttggaggtgttgtacgcggcagcccacccatcttcatgttctgggtactcaccttaaatctaagcaaccactttactccatgtccaatatcatctagaattgtatagtcaataggttttctaatataacgaactggtcgttcaaggttggctggagcaataatcttatgtgtccttgaagtgtttttattggtagtcaaaataccaatttctcttcttgcaactttctctttatgaatatcaactgtttgtgaaatatgattgattgaagattccatccttcgtagctgggatgcctggatatccagcatctgcaggacattgttggccaaggtgtttatcagataggcaacacttgctaaggattgggtggtgtaggctttggtttcttctagggctctctgcttatctgctgtatgtagttgttctcgcagtaatcggccacccgttccagatttgtgtagctgtcgaagagggcccggcggccccccgggatttcctcttccagcagcatctgcagctccgccatcttcacatcctcctcctcctcctcctcatacaggtcgcagagggagcggcggccgcagcgccaaggaaacccaggaccgggagaggaggagcggcggcgacggcggcggtaactcggaagg

SEQ ID NO: 11808 - RNA, 3629 nt, Homo sapiens
  source 1..3629: mol_type = other RNA
ctgaatagctgggactacaggtgtgcgccaccacgcccagctaatttttgtgtttttagtagagatggggtttcaccatgttggccaggatggtctcaatttattgacctcatgatccacccacctcggcctccgaaagtgctgggattacaggcataagccaccacacccagcctgtgggaactatttattggatttcaaaacaccctctgcctcattaatccactaagctttctcagcaaaaagctgtttaaataaataatgggaacatctaatttaaaacagtttttctaattatagaccagtacacgaagaagagcttaacttatccaagtatagtctagtttgggtccataatggagctgaaggctcagaggacattcagggccattacactgcaggaaaacaaggaataagggatgtagaaatgacctaagaaaagcacgaagtggaatgtatactggaggcaagttaatgaaagctaataaatacaaagtgctgggaaaaatctaaaagcaaaatagctattgtaacttgcaatgcattaaaaacaactttaaaaccaaaaagtcttgataaggaaactctatagtggggtctcagttaaatgctgatgatttttaatgctcagataacattaagtggaatattaacttctgcatccgacaccatctgaattttctcacacactactacacttgttcacttttcaatcaagttccactttctgaacttgttcaaaacctcatttgaaatatatccagctactgcttttcccctttcacctagcacagggcagttacctggcaaagctctattctggccaagtcactgggactgagtagaacccacgttagcagctctggacctgaacaggagctggcccaacatcacagtgaccacccacaaagagacaagccctcctggatttttttcagcatttcttatactgactacagtagtgatgattaaagttatctgccctacagactccactgaatttgaagctgtatttattgtacagatgggggaaatgtgttttattgtgtcagttatattaatttttatcaatgtgattagatacatattttggcctattaatcttattcattatattcttagtctgagatgggttttaattctgactaacagcagctacttaagagtccaatcatacaaaatcaggagagtattaccctttctacagctaagcgagtcagtaatacagcagcaactaatactggccattaataacgtccagagagcacattagcaaaccttgtactcccagtgactgtcaggagacttgaaaataactactattctcttccaaagtagaatagcgtttttctagatagtgaaggaaatgatagtcatagttggtctgaactccaagatcctactcctcaaaacagcaccgaagcaggggttcgggatgcctgctaagagcatttccacagttcaagtctcttcagaaccttagggaccttcgtgtctagcttcacacacccacctccacatatgaaccagcctaccacacttcacatctgggtacactggccattagcaacaatgcagtctcatgcagcagcacattaaaatcaaacgggtggcaatcgttcaccaccctcagagtgttgggagactttcacatttcatcatccttataatccacaaacagaaacatgaagggatgcaagtgagttcagcattcactcgtttggtgcactcaagtgctgagagaatgcagaatttacagtgtcacagaggaaaaaagccatctgaaataattgtaaaaatggttaagtgtggtatttaaatgttggttccctcctcttcatacaagtggaagaaaagaaggggctagggtacccactgggccatgaggttaaccccttagcacaggcaatgaagaacatccaatgccacagattctgcaggaggagaaatcccaagggtatacagtattcctgagaaagatcccagatttttctgaatcagtcttaatctgattttgttttggctacacagttatgctgttatacctttgacatacataaaaatggtcattttatttcaatccagacagctcagcattgtacaaatgatggcagaaagatccatttgttcagactcagcttgctttgtttttaatactggggaataaaccaaaaaaaaaagtgtaatttttatcatttgtatccttcattctactttactggagtggaatccccagggccttcagataatctgggaagacctgactattcctgtgaggcaagcacagccctgctgagctttactcagaataatgcatgatagactcaacgtaattcccaggaaaaagcccagtcactccattcataactccctcataccaaccatcgtcattcttcttgatgacataaataatggctccttcctgaaaggacagctcatcttccttgtcttttgtatagtcataaattgccacaaccttttccaagtaagaacgtggagcccacggtgggtcctcttcagcataaggatcactatactcaaccacagcagcttcctcctcttcgtaatcttctggaggaggaggaggtgggggagactcatcaaagactggttcttccacaggtggcggtggaggtggtgtatctgaaactggattctggctataaaaaggtcctccattcatctgattctgaaggcttgtttgtgaagtaatggaaggagggcgtctatagggcaacgagccccctattgttgggggagtatggcgagaggcaggcctattcatgctgtagaactgtacaggatgacctgtagggggagtggaagaaacaacagggggagttggagaagtgaagccatcagcaagggtctgggcacccccagcagcagcgtctggggcagtggaggaagggacagtagcaggaacaagaggagcaggggcagatgcagaagtagcaggaaggggaggagtgccagcagagccagcaggggctggaaagacactgggaggagatggagtaggaacagcaataggaacccccacactaccacttccactgttctctcgactgctgctccgactacttgggtggctccctccactactcccactgctgccaagtgtccctttccctgacatagggggactagggggcttctgagttggaggtgttgtacgcggcagcccacccatcttcatgttctgggtactcacctttactccatgtccaatatcatctagaattgtatagtcaataggttttctaatataacgaactggtcgttcaaggttggctggagcaataatcttatgtgtccttgaagtgtttttattggtagtcaaaataccaatttctcttcttgcaactttctctttatgaatatcaactgtctgtatgtagttgttctcgcagtaatcggccacccgttccagatttgtgtagctgtcgaagagggcccggcggccccccgggatttcctcttccagcagcatctgcagctccgccatcttcacatcctcctcctcctcctcctcatacaggtcgcagagggagcggcggccgcagcgccaaggaaacccaggaccgggagaggaggagcggcggcgacggcggcggtaactcggaagg

SEQ ID NO: 11809 - RNA, 3797 nt, Homo sapiens
  source 1..3797: mol_type = other RNA
ctgaatagctgggactacaggtgtgcgccaccacgcccagctaatttttgtgtttttagtagagatggggtttcaccatgttggccaggatggtctcaatttattgacctcatgatccacccacctcggcctccgaaagtgctgggattacaggcataagccaccacacccagcctgtgggaactatttattggatttcaaaacaccctctgcctcattaatccactaagctttctcagcaaaaagctgtttaaataaataatgggaacatctaatttaaaacagtttttctaattatagaccagtacacgaagaagagcttaacttatccaagtatagtctagtttgggtccataatggagctgaaggctcagaggacattcagggccattacactgcaggaaaacaaggaataagggatgtagaaatgacctaagaaaagcacgaagtggaatgtatactggaggcaagttaatgaaagctaataaatacaaagtgctgggaaaaatctaaaagcaaaatagctattgtaacttgcaatgcattaaaaacaactttaaaaccaaaaagtcttgataaggaaactctatagtggggtctcagttaaatgctgatgatttttaatgctcagataacattaagtggaatattaacttctgcatccgacaccatctgaattttctcacacactactacacttgttcacttttcaatcaagttccactttctgaacttgttcaaaacctcatttgaaatatatccagctactgcttttcccctttcacctagcacagggcagttacctggcaaagctctattctggccaagtcactgggactgagtagaacccacgttagcagctctggacctgaacaggagctggcccaacatcacagtgaccacccacaaagagacaagccctcctggatttttttcagcatttcttatactgactacagtagtgatgattaaagttatctgccctacagactccactgaatttgaagctgtatttattgtacagatgggggaaatgtgttttattgtgtcagttatattaatttttatcaatgtgattagatacatattttggcctattaatcttattcattatattcttagtctgagatgggttttaattctgactaacagcagctacttaagagtccaatcatacaaaatcaggagagtattaccctttctacagctaagcgagtcagtaatacagcagcaactaatactggccattaataacgtccagagagcacattagcaaaccttgtactcccagtgactgtcaggagacttgaaaataactactattctcttccaaagtagaatagcgtttttctagatagtgaaggaaatgatagtcatagttggtctgaactccaagatcctactcctcaaaacagcaccgaagcaggggttcgggatgcctgctaagagcatttccacagttcaagtctcttcagaaccttagggaccttcgtgtctagcttcacacacccacctccacatatgaaccagcctaccacacttcacatctgggtacactggccattagcaacaatgcagtctcatgcagcagcacattaaaatcaaacgggtggcaatcgttcaccaccctcagagtgttgggagactttcacatttcatcatccttataatccacaaacagaaacatgaagggatgcaagtgagttcagcattcactcgtttggtgcactcaagtgctgagagaatgcagaatttacagtgtcacagaggaaaaaagccatctgaaataattgtaaaaatggttaagtgtggtatttaaatgttggttccctcctcttcatacaagtggaagaaaagaaggggctagggtacccactgggccatgaggttaaccccttagcacaggcaatgaagaacatccaatgccacagattctgcaggaggagaaatcccaagggtatacagtattcctgagaaagatcccagatttttctgaatcagtcttaatctgattttgttttggctacacagttatgctgttatacctttgacatacataaaaatggtcattttatttcaatccagacagctcagcattgtacaaatgatggcagaaagatccatttgttcagactcagcttgctttgtttttaatactggggaataaaccaaaaaaaaaagtgtaatttttatcatttgtatccttcattctactttactggagtggaatccccagggccttcagataatctgggaagacctgactattcctgtgaggcaagcacagccctgctgagctttactcagaataatgcatgatagactcaacgtaattcccaggaaaaagcccagtcactccattcataactccctcataccaaccatcgtcattcttcttgatgacataaataatggctccttcctgaaaggacagctcatcttccttgtcttttgtatagtcataaattgccacaaccttttccaagtaagaacgtggagcccacggtgggtcctcttcagcataaggatcactatactcaaccacagcagcttcctcctcttcgtaatcttctggaggaggaggaggtgggggagactcatcaaagactggttcttccacaggtggcggtggaggtggtgtatctgaaactggattctggctataaaaaggtcctccattcatctgattctgaaggcttgtttgtgaagtaatggaaggagggcgtctatagggcaacgagccccctattgttgggggagtatggcgagaggcaggcctattcatgctgtagaactgtacaggatgacctgtagggggagtggaagaaacaacagggggagttggagaagtgaagccatcagcaagggtctgggcacccccagcagcagcgtctggggcagtggaggaagggacagtagcaggaacaagaggagcaggggcagatgcagaagtagcaggaaggggaggagtgccagcagagccagcaggggctggaaagacactgggaggagatggagtaggaacagcaataggaacccccacactaccacttccactgttctctcgactgctgctccgactacttgggtggctccctccactactcccactgctgccaagtgtccctttccctgacatagggggactagggggcttctgagttggaggtgttgtacgcggcagcccacccatcttcatgttctgggtactcacctttactccatgtccaatatcatctagaattgtatagtcaataggttttctaatataacgaactggtcgttcaaggttggctggagcaataatcttatgtgtccttgaagtgtttttattggtagtcaaaataccaatttctcttcttgcaactttctctttatgaatatcaactgtttgtgaaatatgattgattgaagattccatccttcgtagctgggatgcctggatatccagcatctgcaggacattgttggccaaggtgtttatcagataggcaacacttgctaaggattgggtggtgtaggctttggtttcttctagggctctctgcttatctgctgactgtatgtagttgttctcgcagtaatcggccacccgttccagatttgtgtagctgtcgaagagggcccggcggccccccgggatttcctcttccagcagcatctgcagctccgccatcttcacatcctcctcctcctcctcctcatacaggtcgcagagggagcggcggccgcagcgccaaggaaacccaggaccgggagaggaggagcggcggcgacggcggcggtaactcggaagg

SEQ ID NO: 11810 - RNA, 3620 nt, Homo sapiens
  source 1..3620: mol_type = other RNA
ctgaatagctgggactacaggtgtgcgccaccacgcccagctaatttttgtgtttttagtagagatggggtttcaccatgttggccaggatggtctcaatttattgacctcatgatccacccacctcggcctccgaaagtgctgggattacaggcataagccaccacacccagcctgtgggaactatttattggatttcaaaacaccctctgcctcattaatccactaagctttctcagcaaaaagctgtttaaataaataatgggaacatctaatttaaaacagtttttctaattatagaccagtacacgaagaagagcttaacttatccaagtatagtctagtttgggtccataatggagctgaaggctcagaggacattcagggccattacactgcaggaaaacaaggaataagggatgtagaaatgacctaagaaaagcacgaagtggaatgtatactggaggcaagttaatgaaagctaataaatacaaagtgctgggaaaaatctaaaagcaaaatagctattgtaacttgcaatgcattaaaaacaactttaaaaccaaaaagtcttgataaggaaactctatagtggggtctcagttaaatgctgatgatttttaatgctcagataacattaagtggaatattaacttctgcatccgacaccatctgaattttctcacacactactacacttgttcacttttcaatcaagttccactttctgaacttgttcaaaacctcatttgaaatatatccagctactgcttttcccctttcacctagcacagggcagttacctggcaaagctctattctggccaagtcactgggactgagtagaacccacgttagcagctctggacctgaacaggagctggcccaacatcacagtgaccacccacaaagagacaagccctcctggatttttttcagcatttcttatactgactacagtagtgatgattaaagttatctgccctacagactccactgaatttgaagctgtatttattgtacagatgggggaaatgtgttttattgtgtcagttatattaatttttatcaatgtgattagatacatattttggcctattaatcttattcattatattcttagtctgagatgggttttaattctgactaacagcagctacttaagagtccaatcatacaaaatcaggagagtattaccctttctacagctaagcgagtcagtaatacagcagcaactaatactggccattaataacgtccagagagcacattagcaaaccttgtactcccagtgactgtcaggagacttgaaaataactactattctcttccaaagtagaatagcgtttttctagatagtgaaggaaatgatagtcatagttggtctgaactccaagatcctactcctcaaaacagcaccgaagcaggggttcgggatgcctgctaagagcatttccacagttcaagtctcttcagaaccttagggaccttcgtgtctagcttcacacacccacctccacatatgaaccagcctaccacacttcacatctgggtacactggccattagcaacaatgcagtctcatgcagcagcacattaaaatcaaacgggtggcaatcgttcaccaccctcagagtgttgggagactttcacatttcatcatccttataatccacaaacagaaacatgaagggatgcaagtgagttcagcattcactcgtttggtgcactcaagtgctgagagaatgcagaatttacagtgtcacagaggaaaaaagccatctgaaataattgtaaaaatggttaagtgtggtatttaaatgttggttccctcctcttcatacaagtggaagaaaagaaggggctagggtacccactgggccatgaggttaaccccttagcacaggcaatgaagaacatccaatgccacagattctgcaggaggagaaatcccaagggtatacagtattcctgagaaagatcccagatttttctgaatcagtcttaatctgattttgttttggctacacagttatgctgttatacctttgacatacataaaaatggtcattttatttcaatccagacagctcagcattgtacaaatgatggcagaaagatccatttgttcagactcagcttgctttgtttttaatactggggaataaaccaaaaaaaaaagtgtaatttttatcatttgtatccttcattctactttactggagtggaatccccagggccttcagataatctgggaagacctgactattcctgtgaggcaagcacagccctgctgagctttactcagaataatgcatgatagactcaacgtaattcccaggaaaaagcccagtcactccattcataactccctcataccaaccatcgtcattcttcttgatgacataaataatggctccttcctgaaaggacagctcatcttccttgtcttttgtatagtcataaattgccacaaccttttccaagtaagaacgtggagcccacggtgggtcctcttcagcataaggatcactatactcaaccacagcagcttcctcctcttcgtaatcttctggaggaggaggaggtgggggagactcatcaaagactggttcttccacaggtggcggtggaggtggtgtatctgaaactggattctggctataaaaaggtcctccattcatctgattctgaaggcttgtttgtgaagtaatggaaggagggcgtctatagggcaacgagccccctattgttgggggagtatggcgagaggcaggcctattcatgctgtagaactgtacaggatgacctgtagggggagtggaagaaacaacagggggagttggagaagtgaagccatcagcaagggtctgggcacccccagcagcagcgtctggggcagtggaggaagggacagtagcaggaacaagaggagcaggggcagatgcagaagtagcaggaaggggaggagtgccagcagagccagcaggggctggaaagacactgggaggagatggagtaggaacagcaataggaacccccacactaccacttccactgttctctcgactgctgctccgactacttgggtggctccctccactactcccactgctgccaagtgtccctttccctgacatagggggactagggggcttctgagttggaggtgttgtacgcggcagcccacccatcttcatgttctgggtactcacttgtgaaatatgattgattgaagattccatccttcgtagctgggatgcctggatatccagcatctgcaggacattgttggccaaggtgtttatcagataggcaacacttgctaaggattgggtggtgtaggctttggtttcttctagggctctctgcttatctgctgactgtatgtagttgttctcgcagtaatcggccacccgttccagatttgtgtagctgtcgaagagggcccggcggccccccgggatttcctcttccagcagcatctgcagctccgccatcttcacatcctcctcctcctcctcctcatacaggtcgcagagggagcggcggccgcagcgccaaggaaacccaggaccgggagaggaggagcggcggcgacggcggcggtaactcggaagg

SEQ ID NO: 11811 - RNA, 4038 nt, Homo sapiens
  source 1..4038: mol_type = other RNA
ctgaatagctgggactacaggtgtgcgccaccacgcccagctaatttttgtgtttttagtagagatggggtttcaccatgttggccaggatggtctcaatttattgacctcatgatccacccacctcggcctccgaaagtgctgggattacaggcataagccaccacacccagcctgtgggaactatttattggatttcaaaacaccctctgcctcattaatccactaagctttctcagcaaaaagctgtttaaataaataatgggaacatctaatttaaaacagtttttctaattatagaccagtacacgaagaagagcttaacttatccaagtatagtctagtttgggtccataatggagctgaaggctcagaggacattcagggccattacactgcaggaaaacaaggaataagggatgtagaaatgacctaagaaaagcacgaagtggaatgtatactggaggcaagttaatgaaagctaataaatacaaagtgctgggaaaaatctaaaagcaaaatagctattgtaacttgcaatgcattaaaaacaactttaaaaccaaaaagtcttgataaggaaactctatagtggggtctcagttaaatgctgatgatttttaatgctcagataacattaagtggaatattaacttctgcatccgacaccatctgaattttctcacacactactacacttgttcacttttcaatcaagttccactttctgaacttgttcaaaacctcatttgaaatatatccagctactgcttttcccctttcacctagcacagggcagttacctggcaaagctctattctggccaagtcactgggactgagtagaacccacgttagcagctctggacctgaacaggagctggcccaacatcacagtgaccacccacaaagagacaagccctcctggatttttttcagcatttcttatactgactacagtagtgatgattaaagttatctgccctacagactccactgaatttgaagctgtatttattgtacagatgggggaaatgtgttttattgtgtcagttatattaatttttatcaatgtgattagatacatattttggcctattaatcttattcattatattcttagtctgagatgggttttaattctgactaacagcagctacttaagagtccaatcatacaaaatcaggagagtattaccctttctacagctaagcgagtcagtaatacagcagcaactaatactggccattaataacgtccagagagcacattagcaaaccttgtactcccagtgactgtcaggagacttgaaaataactactattctcttccaaagtagaatagcgtttttctagatagtgaaggaaatgatagtcatagttggtctgaactccaagatcctactcctcaaaacagcaccgaagcaggggttcgggatgcctgctaagagcatttccacagttcaagtctcttcagaaccttagggaccttcgtgtctagcttcacacacccacctccacatatgaaccagcctaccacacttcacatctgggtacactggccattagcaacaatgcagtctcatgcagcagcacattaaaatcaaacgggtggcaatcgttcaccaccctcagagtgttgggagactttcacatttcatcatccttataatccacaaacagaaacatgaagggatgcaagtgagttcagcattcactcgtttggtgcactcaagtgctgagagaatgcagaatttacagtgtcacagaggaaaaaagccatctgaaataattgtaaaaatggttaagtgtggtatttaaatgttggttccctcctcttcatacaagtggaagaaaagaaggggctagggtacccactgggccatgaggttaaccccttagcacaggcaatgaagaacatccaatgccacagattctgcaggaggagaaatcccaagggtatacagtattcctgagaaagatcccagatttttctgaatcagtcttaatctgattttgttttggctacacagttatgctgttatacctttgacatacataaaaatggtcattttatttcaatccagacagctcagcattgtacaaatgatggcagaaagatccatttgttcagactcagcttgctttgtttttaatactggggaataaaccaaaaaaaaaagtgtaatttttatcatttgtatccttcattctactttactggagtggaatccccagggccttcagataatctgggaagacctgactattcctgtgaggcaagcacagccctgctgagctttactcagaataatgcatgatagactcaacgtaattcccaggaaaaagcccagtcactccattcataactccctcataccaaccatcgtcattcttcttgatgacataaataatggctccttcctgaaaggacagctcatcttccttgtcttttgtatagtcataaattgccacaaccttttccaagtaagaacgtggagcccacggtgggtcctcttcagcataaggatcactatactcaaccacagcagcttcctcctcttcgtaatcttctggaggaggaggaggtgggggagactcatcaaagactggttcttccacaggtggcggtggaggtggtgtatctgaaactggattctggctataaaaaggtcctccattcatctgattctgaaggcttgtttgtgaagtaatggaaggagggcgtctatagggcaacgagccccctattgttgggggagtatggcgagaggcaggcctattcatgctgtagaactgtacaggatgacctgtagggggagtggaagaaacaacagggggagttggagaagtgaagccatcagcaagggtctgggcacccccagcagcagcgtctggggcagtggaggaagggacagtagcaggaacaagaggagcaggggcagatgcagaagtagcaggaaggggaggagtgccagcagagccagcaggggctggaaagacactgggaggagatggagtaggaacagcaataggaacccccacactaccacttccactgttctctcgactgctgctccgactacttgggtggctccctccactactcccactgctgctgtaagttcgatttctttgattcacagaagctgtcctcacagggctctgctgcgagggagccatattacgggttgggctaggtacgtaatcatttggtaccactggaggacgcactggctccagtgtgcgatagggggagtgccgcccaagtgtccctttccctgacatagggggactagggggcttctgagttggaggtgttgtacgcggcagcccacccatcttcatgttctgggtactcaccttaaatctaagcaaccactttactccatgtccaatatcatctagaattgtatagtcaataggttttctaatataacgaactggtcgttcaaggttggctggagcaataatcttatgtgtccttgaagtgtttttattggtagtcaaaataccaatttctcttcttgcaactttctctttatgaatatcaactgtctcattcaatctcaaactgcaattgtttccaaatttggtcacaaaagtcgactcaagatcaacgcctctaatttgcttgtgaaatatgattgattgaagattccatccttcgtagctgggatgcctggatatccagcatctgcaggacattgttggccaaggtgtttatcagataggcaacacttgctaaggattgggtggtgtaggctttggtttcttctagggctctctgcttatctgctgactgtatgtagttgttctcgcagtaatcggccacccgttccagatttgtgtagctgtcgaagagggcccggcggccccccgggatttcctcttccagcagcatctgcagctccgccatcttcacatcctcctcctcctcctcctcatacaggtcgcagagggagcggcggccgcagcgccaaggaaacccaggaccgggagaggaggagcggcggcgacggcggcggtaactcggaagg

SEQ ID NO: 11812 - RNA, 3794 nt, Homo sapiens
  source 1..3794: mol_type = other RNA
ctgaatagctgggactacaggtgtgcgccaccacgcccagctaatttttgtgtttttagtagagatggggtttcaccatgttggccaggatggtctcaatttattgacctcatgatccacccacctcggcctccgaaagtgctgggattacaggcataagccaccacacccagcctgtgggaactatttattggatttcaaaacaccctctgcctcattaatccactaagctttctcagcaaaaagctgtttaaataaataatgggaacatctaatttaaaacagtttttctaattatagaccagtacacgaagaagagcttaacttatccaagtatagtctagtttgggtccataatggagctgaaggctcagaggacattcagggccattacactgcaggaaaacaaggaataagggatgtagaaatgacctaagaaaagcacgaagtggaatgtatactggaggcaagttaatgaaagctaataaatacaaagtgctgggaaaaatctaaaagcaaaatagctattgtaacttgcaatgcattaaaaacaactttaaaaccaaaaagtcttgataaggaaactctatagtggggtctcagttaaatgctgatgatttttaatgctcagataacattaagtggaatattaacttctgcatccgacaccatctgaattttctcacacactactacacttgttcacttttcaatcaagttccactttctgaacttgttcaaaacctcatttgaaatatatccagctactgcttttcccctttcacctagcacagggcagttacctggcaaagctctattctggccaagtcactgggactgagtagaacccacgttagcagctctggacctgaacaggagctggcccaacatcacagtgaccacccacaaagagacaagccctcctggatttttttcagcatttcttatactgactacagtagtgatgattaaagttatctgccctacagactccactgaatttgaagctgtatttattgtacagatgggggaaatgtgttttattgtgtcagttatattaatttttatcaatgtgattagatacatattttggcctattaatcttattcattatattcttagtctgagatgggttttaattctgactaacagcagctacttaagagtccaatcatacaaaatcaggagagtattaccctttctacagctaagcgagtcagtaatacagcagcaactaatactggccattaataacgtccagagagcacattagcaaaccttgtactcccagtgactgtcaggagacttgaaaataactactattctcttccaaagtagaatagcgtttttctagatagtgaaggaaatgatagtcatagttggtctgaactccaagatcctactcctcaaaacagcaccgaagcaggggttcgggatgcctgctaagagcatttccacagttcaagtctcttcagaaccttagggaccttcgtgtctagcttcacacacccacctccacatatgaaccagcctaccacacttcacatctgggtacactggccattagcaacaatgcagtctcatgcagcagcacattaaaatcaaacgggtggcaatcgttcaccaccctcagagtgttgggagactttcacatttcatcatccttataatccacaaacagaaacatgaagggatgcaagtgagttcagcattcactcgtttggtgcactcaagtgctgagagaatgcagaatttacagtgtcacagaggaaaaaagccatctgaaataattgtaaaaatggttaagtgtggtatttaaatgttggttccctcctcttcatacaagtggaagaaaagaaggggctagggtacccactgggccatgaggttaaccccttagcacaggcaatgaagaacatccaatgccacagattctgcaggaggagaaatcccaagggtatacagtattcctgagaaagatcccagatttttctgaatcagtcttaatctgattttgttttggctacacagttatgctgttatacctttgacatacataaaaatggtcattttatttcaatccagacagctcagcattgtacaaatgatggcagaaagatccatttgttcagactcagcttgctttgtttttaatactggggaataaaccaaaaaaaaaagtgtaatttttatcatttgtatccttcattctactttactggagtggaatccccagggccttcagataatctgggaagacctgactattcctgtgaggcaagcacagccctgctgagctttactcagaataatgcatgatagactcaacgtaattcccaggaaaaagcccagtcactccattcataactccctcataccaaccatcgtcattcttcttgatgacataaataatggctccttcctgaaaggacagctcatcttccttgtcttttgtatagtcataaattgccacaaccttttccaagtaagaacgtggagcccacggtgggtcctcttcagcataaggatcactatactcaaccacagcagcttcctcctcttcgtaatcttctggaggaggaggaggtgggggagactcatcaaagactggttcttccacaggtggcggtggaggtggtgtatctgaaactggattctggctataaaaaggtcctccattcatctgattctgaaggcttgtttgtgaagtaatggaaggagggcgtctatagggcaacgagccccctattgttgggggagtatggcgagaggcaggcctattcatgctgtagaactgtacaggatgacctgtagggggagtggaagaaacaacagggggagttggagaagtgaagccatcagcaagggtctgggcacccccagcagcagcgtctggggcagtggaggaagggacagtagcaggaacaagaggagcaggggcagatgcagaagtagcaggaaggggaggagtgccagcagagccagcaggggctggaaagacactgggaggagatggagtaggaacagcaataggaacccccacactaccacttccactgttctctcgactgctgctccgactacttgggtggctccctccactactcccactgctgctgtaagttcgatttctttgattcacagaagctgtcctcacagggctctgctgcgagggagccatattacgggttgggctaggtacgtaatcatttggtaccactggaggacgcactggctccagtgtgcgatagggggagtgccgcccaagtgtccctttccctgacatagggggactagggggcttctgagttggaggtgttgtacgcggcagcccacccatcttcatgttctgggtactcaccttaaatctaagcaaccactttactccatgtccaatatcatctagaattgtatagtcaataggttttctaatataacgaactggtcgttcaaggttggctggagcaataatcttatgtgtccttgaagtgtttttattggtagtcaaaataccaatttctcttcttgcaactttctctttatgaatatcaactgtctgtatgtagttgttctcgcagtaatcggccacccgttccagatttgtgtagctgtcgaagagggcccggcggccccccgggatttcctcttccagcagcatctgcagctccgccatcttcacatcctcctcctcctcctcctcatacaggtcgcagagggagcggcggccgcagcgccaaggaaacccaggaccgggagaggaggagcggcggcgacggcggcggtaactcggaagg

SEQ ID NO: 11813 - RNA, 3962 nt, Homo sapiens
  source 1..3962: mol_type = other RNA
ctgaatagctgggactacaggtgtgcgccaccacgcccagctaatttttgtgtttttagtagagatggggtttcaccatgttggccaggatggtctcaatttattgacctcatgatccacccacctcggcctccgaaagtgctgggattacaggcataagccaccacacccagcctgtgggaactatttattggatttcaaaacaccctctgcctcattaatccactaagctttctcagcaaaaagctgtttaaataaataatgggaacatctaatttaaaacagtttttctaattatagaccagtacacgaagaagagcttaacttatccaagtatagtctagtttgggtccataatggagctgaaggctcagaggacattcagggccattacactgcaggaaaacaaggaataagggatgtagaaatgacctaagaaaagcacgaagtggaatgtatactggaggcaagttaatgaaagctaataaatacaaagtgctgggaaaaatctaaaagcaaaatagctattgtaacttgcaatgcattaaaaacaactttaaaaccaaaaagtcttgataaggaaactctatagtggggtctcagttaaatgctgatgatttttaatgctcagataacattaagtggaatattaacttctgcatccgacaccatctgaattttctcacacactactacacttgttcacttttcaatcaagttccactttctgaacttgttcaaaacctcatttgaaatatatccagctactgcttttcccctttcacctagcacagggcagttacctggcaaagctctattctggccaagtcactgggactgagtagaacccacgttagcagctctggacctgaacaggagctggcccaacatcacagtgaccacccacaaagagacaagccctcctggatttttttcagcatttcttatactgactacagtagtgatgattaaagttatctgccctacagactccactgaatttgaagctgtatttattgtacagatgggggaaatgtgttttattgtgtcagttatattaatttttatcaatgtgattagatacatattttggcctattaatcttattcattatattcttagtctgagatgggttttaattctgactaacagcagctacttaagagtccaatcatacaaaatcaggagagtattaccctttctacagctaagcgagtcagtaatacagcagcaactaatactggccattaataacgtccagagagcacattagcaaaccttgtactcccagtgactgtcaggagacttgaaaataactactattctcttccaaagtagaatagcgtttttctagatagtgaaggaaatgatagtcatagttggtctgaactccaagatcctactcctcaaaacagcaccgaagcaggggttcgggatgcctgctaagagcatttccacagttcaagtctcttcagaaccttagggaccttcgtgtctagcttcacacacccacctccacatatgaaccagcctaccacacttcacatctgggtacactggccattagcaacaatgcagtctcatgcagcagcacattaaaatcaaacgggtggcaatcgttcaccaccctcagagtgttgggagactttcacatttcatcatccttataatccacaaacagaaacatgaagggatgcaagtgagttcagcattcactcgtttggtgcactcaagtgctgagagaatgcagaatttacagtgtcacagaggaaaaaagccatctgaaataattgtaaaaatggttaagtgtggtatttaaatgttggttccctcctcttcatacaagtggaagaaaagaaggggctagggtacccactgggccatgaggttaaccccttagcacaggcaatgaagaacatccaatgccacagattctgcaggaggagaaatcccaagggtatacagtattcctgagaaagatcccagatttttctgaatcagtcttaatctgattttgttttggctacacagttatgctgttatacctttgacatacataaaaatggtcattttatttcaatccagacagctcagcattgtacaaatgatggcagaaagatccatttgttcagactcagcttgctttgtttttaatactggggaataaaccaaaaaaaaaagtgtaatttttatcatttgtatccttcattctactttactggagtggaatccccagggccttcagataatctgggaagacctgactattcctgtgaggcaagcacagccctgctgagctttactcagaataatgcatgatagactcaacgtaattcccaggaaaaagcccagtcactccattcataactccctcataccaaccatcgtcattcttcttgatgacataaataatggctccttcctgaaaggacagctcatcttccttgtcttttgtatagtcataaattgccacaaccttttccaagtaagaacgtggagcccacggtgggtcctcttcagcataaggatcactatactcaaccacagcagcttcctcctcttcgtaatcttctggaggaggaggaggtgggggagactcatcaaagactggttcttccacaggtggcggtggaggtggtgtatctgaaactggattctggctataaaaaggtcctccattcatctgattctgaaggcttgtttgtgaagtaatggaaggagggcgtctatagggcaacgagccccctattgttgggggagtatggcgagaggcaggcctattcatgctgtagaactgtacaggatgacctgtagggggagtggaagaaacaacagggggagttggagaagtgaagccatcagcaagggtctgggcacccccagcagcagcgtctggggcagtggaggaagggacagtagcaggaacaagaggagcaggggcagatgcagaagtagcaggaaggggaggagtgccagcagagccagcaggggctggaaagacactgggaggagatggagtaggaacagcaataggaacccccacactaccacttccactgttctctcgactgctgctccgactacttgggtggctccctccactactcccactgctgctgtaagttcgatttctttgattcacagaagctgtcctcacagggctctgctgcgagggagccatattacgggttgggctaggtacgtaatcatttggtaccactggaggacgcactggctccagtgtgcgatagggggagtgccgcccaagtgtccctttccctgacatagggggactagggggcttctgagttggaggtgttgtacgcggcagcccacccatcttcatgttctgggtactcaccttaaatctaagcaaccactttactccatgtccaatatcatctagaattgtatagtcaataggttttctaatataacgaactggtcgttcaaggttggctggagcaataatcttatgtgtccttgaagtgtttttattggtagtcaaaataccaatttctcttcttgcaactttctctttatgaatatcaactgtttgtgaaatatgattgattgaagattccatccttcgtagctgggatgcctggatatccagcatctgcaggacattgttggccaaggtgtttatcagataggcaacacttgctaaggattgggtggtgtaggctttggtttcttctagggctctctgcttatctgctgactgtatgtagttgttctcgcagtaatcggccacccgttccagatttgtgtagctgtcgaagagggcccggcggccccccgggatttcctcttccagcagcatctgcagctccgccatcttcacatcctcctcctcctcctcctcatacaggtcgcagagggagcggcggccgcagcgccaaggaaacccaggaccgggagaggaggagcggcggcgacggcggcggtaactcggaagg

SEQ ID NO: 11814 - RNA, 3958 nt, Homo sapiens
  source 1..3958: mol_type = other RNA
ctgaatagctgggactacaggtgtgcgccaccacgcccagctaatttttgtgtttttagtagagatggggtttcaccatgttggccaggatggtctcaatttattgacctcatgatccacccacctcggcctccgaaagtgctgggattacaggcataagccaccacacccagcctgtgggaactatttattggatttcaaaacaccctctgcctcattaatccactaagctttctcagcaaaaagctgtttaaataaataatgggaacatctaatttaaaacagtttttctaattatagaccagtacacgaagaagagcttaacttatccaagtatagtctagtttgggtccataatggagctgaaggctcagaggacattcagggccattacactgcaggaaaacaaggaataagggatgtagaaatgacctaagaaaagcacgaagtggaatgtatactggaggcaagttaatgaaagctaataaatacaaagtgctgggaaaaatctaaaagcaaaatagctattgtaacttgcaatgcattaaaaacaactttaaaaccaaaaagtcttgataaggaaactctatagtggggtctcagttaaatgctgatgatttttaatgctcagataacattaagtggaatattaacttctgcatccgacaccatctgaattttctcacacactactacacttgttcacttttcaatcaagttccactttctgaacttgttcaaaacctcatttgaaatatatccagctactgcttttcccctttcacctagcacagggcagttacctggcaaagctctattctggccaagtcactgggactgagtagaacccacgttagcagctctggacctgaacaggagctggcccaacatcacagtgaccacccacaaagagacaagccctcctggatttttttcagcatttcttatactgactacagtagtgatgattaaagttatctgccctacagactccactgaatttgaagctgtatttattgtacagatgggggaaatgtgttttattgtgtcagttatattaatttttatcaatgtgattagatacatattttggcctattaatcttattcattatattcttagtctgagatgggttttaattctgactaacagcagctacttaagagtccaatcatacaaaatcaggagagtattaccctttctacagctaagcgagtcagtaatacagcagcaactaatactggccattaataacgtccagagagcacattagcaaaccttgtactcccagtgactgtcaggagacttgaaaataactactattctcttccaaagtagaatagcgtttttctagatagtgaaggaaatgatagtcatagttggtctgaactccaagatcctactcctcaaaacagcaccgaagcaggggttcgggatgcctgctaagagcatttccacagttcaagtctcttcagaaccttagggaccttcgtgtctagcttcacacacccacctccacatatgaaccagcctaccacacttcacatctgggtacactggccattagcaacaatgcagtctcatgcagcagcacattaaaatcaaacgggtggcaatcgttcaccaccctcagagtgttgggagactttcacatttcatcatccttataatccacaaacagaaacatgaagggatgcaagtgagttcagcattcactcgtttggtgcactcaagtgctgagagaatgcagaatttacagtgtcacagaggaaaaaagccatctgaaataattgtaaaaatggttaagtgtggtatttaaatgttggttccctcctcttcatacaagtggaagaaaagaaggggctagggtacccactgggccatgaggttaaccccttagcacaggcaatgaagaacatccaatgccacagattctgcaggaggagaaatcccaagggtatacagtattcctgagaaagatcccagatttttctgaatcagtcttaatctgattttgttttggctacacagttatgctgttatacctttgacatacataaaaatggtcattttatttcaatccagacagctcagcattgtacaaatgatggcagaaagatccatttgttcagactcagcttgctttgtttttaatactggggaataaaccaaaaaaaaaagtgtaatttttatcatttgtatccttcattctactttactggagtggaatccccagggccttcagataatctgggaagacctgactattcctgtgaggcaagcacagccctgctgagctttactcagaataatgcatgatagactcaacgtaattcccaggaaaaagcccagtcactccattcataactccctcataccaaccatcgtcattcttcttgatgacataaataatggctccttcctgaaaggacagctcatcttccttgtcttttgtatagtcataaattgccacaaccttttccaagtaagaacgtggagcccacggtgggtcctcttcagcataaggatcactatactcaaccacagcagcttcctcctcttcgtaatcttctggaggaggaggaggtgggggagactcatcaaagactggttcttccacaggtggcggtggaggtggtgtatctgaaactggattctggctataaaaaggtcctccattcatctgattctgaaggcttgtttgtgaagtaatggaaggagggcgtctatagggcaacgagccccctattgttgggggagtatggcgagaggcaggcctattcatgctgtagaactgtacaggatgacctgtagggggagtggaagaaacaacagggggagttggagaagtgaagccatcagcaagggtctgggcacccccagcagcagcgtctggggcagtggaggaagggacagtagcaggaacaagaggagcaggggcagatgcagaagtagcaggaaggggaggagtgccagcagagccagcaggggctggaaagacactgggaggagatggagtaggaacagcaataggaacccccacactaccacttccactgttctctcgactgctgctccgactacttgggtggctccctccactactcccactgctgctgtaagttcgatttctttgattcacagaagctgtcctcacagggctctgctgcgagggagccatattacgggttgggctaggtacgtaatcatttggtaccactggaggacgcactggctccagtgtgcgatagggggagtgccgcccaagtgtccctttccctgacatagggggactagggggcttctgagttggaggtgttgtacgcggcagcccacccatcttcatgttctgggtactcaccttaaatctaagcaaccactttactccatgtccaatatcatctagaattgtatagtcaataggttttctaatataacgaactggtcgttcaaggttggctggagcaataatcttatgtgtccttgaagtgtttttattggtagtcaaaataccaatttctcttcttgcaactttctctttatgaatatcaactgtttgtgaaatatgattgattgaagattccatccttcgtagctgggatgcctggatatccagcatctgcaggacattgttggccaaggtgtttatcagataggcaacacttgctaaggattgggtggtgtaggctttggtttcttctagggctctctgcttatctgctgtatgtagttgttctcgcagtaatcggccacccgttccagatttgtgtagctgtcgaagagggcccggcggccccccgggatttcctcttccagcagcatctgcagctccgccatcttcacatcctcctcctcctcctcctcatacaggtcgcagagggagcggcggccgcagcgccaaggaaacccaggaccgggagaggaggagcggcggcgacggcggcggtaactcggaagg

SEQ ID NO: 11815 - RNA, 3944 nt, Homo sapiens
  source 1..3944: mol_type = other RNA
ctgaatagctgggactacaggtgtgcgccaccacgcccagctaatttttgtgtttttagtagagatggggtttcaccatgttggccaggatggtctcaatttattgacctcatgatccacccacctcggcctccgaaagtgctgggattacaggcataagccaccacacccagcctgtgggaactatttattggatttcaaaacaccctctgcctcattaatccactaagctttctcagcaaaaagctgtttaaataaataatgggaacatctaatttaaaacagtttttctaattatagaccagtacacgaagaagagcttaacttatccaagtatagtctagtttgggtccataatggagctgaaggctcagaggacattcagggccattacactgcaggaaaacaaggaataagggatgtagaaatgacctaagaaaagcacgaagtggaatgtatactggaggcaagttaatgaaagctaataaatacaaagtgctgggaaaaatctaaaagcaaaatagctattgtaacttgcaatgcattaaaaacaactttaaaaccaaaaagtcttgataaggaaactctatagtggggtctcagttaaatgctgatgatttttaatgctcagataacattaagtggaatattaacttctgcatccgacaccatctgaattttctcacacactactacacttgttcacttttcaatcaagttccactttctgaacttgttcaaaacctcatttgaaatatatccagctactgcttttcccctttcacctagcacagggcagttacctggcaaagctctattctggccaagtcactgggactgagtagaacccacgttagcagctctggacctgaacaggagctggcccaacatcacagtgaccacccacaaagagacaagccctcctggatttttttcagcatttcttatactgactacagtagtgatgattaaagttatctgccctacagactccactgaatttgaagctgtatttattgtacagatgggggaaatgtgttttattgtgtcagttatattaatttttatcaatgtgattagatacatattttggcctattaatcttattcattatattcttagtctgagatgggttttaattctgactaacagcagctacttaagagtccaatcatacaaaatcaggagagtattaccctttctacagctaagcgagtcagtaatacagcagcaactaatactggccattaataacgtccagagagcacattagcaaaccttgtactcccagtgactgtcaggagacttgaaaataactactattctcttccaaagtagaatagcgtttttctagatagtgaaggaaatgatagtcatagttggtctgaactccaagatcctactcctcaaaacagcaccgaagcaggggttcgggatgcctgctaagagcatttccacagttcaagtctcttcagaaccttagggaccttcgtgtctagcttcacacacccacctccacatatgaaccagcctaccacacttcacatctgggtacactggccattagcaacaatgcagtctcatgcagcagcacattaaaatcaaacgggtggcaatcgttcaccaccctcagagtgttgggagactttcacatttcatcatccttataatccacaaacagaaacatgaagggatgcaagtgagttcagcattcactcgtttggtgcactcaagtgctgagagaatgcagaatttacagtgtcacagaggaaaaaagccatctgaaataattgtaaaaatggttaagtgtggtatttaaatgttggttccctcctcttcatacaagtggaagaaaagaaggggctagggtacccactgggccatgaggttaaccccttagcacaggcaatgaagaacatccaatgccacagattctgcaggaggagaaatcccaagggtatacagtattcctgagaaagatcccagatttttctgaatcagtcttaatctgattttgttttggctacacagttatgctgttatacctttgacatacataaaaatggtcattttatttcaatccagacagctcagcattgtacaaatgatggcagaaagatccatttgttcagactcagcttgctttgtttttaatactggggaataaaccaaaaaaaaaagtgtaatttttatcatttgtatccttcattctactttactggagtggaatccccagggccttcagataatctgggaagacctgactattcctgtgaggcaagcacagccctgctgagctttactcagaataatgcatgatagactcaacgtaattcccaggaaaaagcccagtcactccattcataactccctcataccaaccatcgtcattcttcttgatgacataaataatggctccttcctgaaaggacagctcatcttccttgtcttttgtatagtcataaattgccacaaccttttccaagtaagaacgtggagcccacggtgggtcctcttcagcataaggatcactatactcaaccacagcagcttcctcctcttcgtaatcttctggaggaggaggaggtgggggagactcatcaaagactggttcttccacaggtggcggtggaggtggtgtatctgaaactggattctggctataaaaaggtcctccattcatctgattctgaaggcttgtttgtgaagtaatggaaggagggcgtctatagggcaacgagccccctattgttgggggagtatggcgagaggcaggcctattcatgctgtagaactgtacaggatgacctgtagggggagtggaagaaacaacagggggagttggagaagtgaagccatcagcaagggtctgggcacccccagcagcagcgtctggggcagtggaggaagggacagtagcaggaacaagaggagcaggggcagatgcagaagtagcaggaaggggaggagtgccagcagagccagcaggggctggaaagacactgggaggagatggagtaggaacagcaataggaacccccacactaccacttccactgttctctcgactgctgctccgactacttgggtggctccctccactactcccactgctgctgtaagttcgatttctttgattcacagaagctgtcctcacagggctctgctgcgagggagccatattacgggttgggctaggtacgtaatcatttggtaccactggaggacgcactggctccagtgtgcgatagggggagtgccgcccaagtgtccctttccctgacatagggggactagggggcttctgagttggaggtgttgtacgcggcagcccacccatcttcatgttctgggtactcacctttactccatgtccaatatcatctagaattgtatagtcaataggttttctaatataacgaactggtcgttcaaggttggctggagcaataatcttatgtgtccttgaagtgtttttattggtagtcaaaataccaatttctcttcttgcaactttctctttatgaatatcaactgtttgtgaaatatgattgattgaagattccatccttcgtagctgggatgcctggatatccagcatctgcaggacattgttggccaaggtgtttatcagataggcaacacttgctaaggattgggtggtgtaggctttggtttcttctagggctctctgcttatctgctgactgtatgtagttgttctcgcagtaatcggccacccgttccagatttgtgtagctgtcgaagagggcccggcggccccccgggatttcctcttccagcagcatctgcagctccgccatcttcacatcctcctcctcctcctcctcatacaggtcgcagagggagcggcggccgcagcgccaaggaaacccaggaccgggagaggaggagcggcggcgacggcggcggtaactcggaagg

SEQ ID NO: 11816 - RNA, 3959 nt, Homo sapiens
  source 1..3959: mol_type = other RNA
ctgaatagctgggactacaggtgtgcgccaccacgcccagctaatttttgtgtttttagtagagatggggtttcaccatgttggccaggatggtctcaatttattgacctcatgatccacccacctcggcctccgaaagtgctgggattacaggcataagccaccacacccagcctgtgggaactatttattggatttcaaaacaccctctgcctcattaatccactaagctttctcagcaaaaagctgtttaaataaataatgggaacatctaatttaaaacagtttttctaattatagaccagtacacgaagaagagcttaacttatccaagtatagtctagtttgggtccataatggagctgaaggctcagaggacattcagggccattacactgcaggaaaacaaggaataagggatgtagaaatgacctaagaaaagcacgaagtggaatgtatactggaggcaagttaatgaaagctaataaatacaaagtgctgggaaaaatctaaaagcaaaatagctattgtaacttgcaatgcattaaaaacaactttaaaaccaaaaagtcttgataaggaaactctatagtggggtctcagttaaatgctgatgatttttaatgctcagataacattaagtggaatattaacttctgcatccgacaccatctgaattttctcacacactactacacttgttcacttttcaatcaagttccactttctgaacttgttcaaaacctcatttgaaatatatccagctactgcttttcccctttcacctagcacagggcagttacctggcaaagctctattctggccaagtcactgggactgagtagaacccacgttagcagctctggacctgaacaggagctggcccaacatcacagtgaccacccacaaagagacaagccctcctggatttttttcagcatttcttatactgactacagtagtgatgattaaagttatctgccctacagactccactgaatttgaagctgtatttattgtacagatgggggaaatgtgttttattgtgtcagttatattaatttttatcaatgtgattagatacatattttggcctattaatcttattcattatattcttagtctgagatgggttttaattctgactaacagcagctacttaagagtccaatcatacaaaatcaggagagtattaccctttctacagctaagcgagtcagtaatacagcagcaactaatactggccattaataacgtccagagagcacattagcaaaccttgtactcccagtgactgtcaggagacttgaaaataactactattctcttccaaagtagaatagcgtttttctagatagtgaaggaaatgatagtcatagttggtctgaactccaagatcctactcctcaaaacagcaccgaagcaggggttcgggatgcctgctaagagcatttccacagttcaagtctcttcagaaccttagggaccttcgtgtctagcttcacacacccacctccacatatgaaccagcctaccacacttcacatctgggtacactggccattagcaacaatgcagtctcatgcagcagcacattaaaatcaaacgggtggcaatcgttcaccaccctcagagtgttgggagactttcacatttcatcatccttataatccacaaacagaaacatgaagggatgcaagtgagttcagcattcactcgtttggtgcactcaagtgctgagagaatgcagaatttacagtgtcacagaggaaaaaagccatctgaaataattgtaaaaatggttaagtgtggtatttaaatgttggttccctcctcttcatacaagtggaagaaaagaaggggctagggtacccactgggccatgaggttaaccccttagcacaggcaatgaagaacatccaatgccacagattctgcaggaggagaaatcccaagggtatacagtattcctgagaaagatcccagatttttctgaatcagtcttaatctgattttgttttggctacacagttatgctgttatacctttgacatacataaaaatggtcattttatttcaatccagacagctcagcattgtacaaatgatggcagaaagatccatttgttcagactcagcttgctttgtttttaatactggggaataaaccaaaaaaaaaagtgtaatttttatcatttgtatccttcattctactttactggagtggaatccccagggccttcagataatctgggaagacctgactattcctgtgaggcaagcacagccctgctgagctttactcagaataatgcatgatagactcaacgtaattcccaggaaaaagcccagtcactccattcataactccctcataccaaccatcgtcattcttcttgatgacataaataatggctccttcctgaaaggacagctcatcttccttgtcttttgtatagtcataaattgccacaaccttttccaagtaagaacgtggagcccacggtgggtcctcttcagcataaggatcactatactcaaccacagcagcttcctcctcttcgtaatcttctggaggaggaggaggtgggggagactcatcaaagactggttcttccacaggtggcggtggaggtggtgtatctgaaactggattctggctataaaaaggtcctccattcatctgattctgaaggcttgtttgtgaagtaatggaaggagggcgtctatagggcaacgagccccctattgttgggggagtatggcgagaggcaggcctattcatgctgtagaactgtacaggatgacctgtagggggagtggaagaaacaacagggggagttggagaagtgaagccatcagcaagggtctgggcacccccagcagcagcgtctggggcagtggaggaagggacagtagcaggaacaagaggagcaggggcagatgcagaagtagcaggaaggggaggagtgccagcagagccagcaggggctggaaagacactgggaggagatggagtaggaacagcaataggaacccccacactaccacttccactgttctctcgactgctgctccgactacttgggtggctccctccactactcccactgctgtaagttcgatttctttgattcacagaagctgtcctcacagggctctgctgcgagggagccatattacgggttgggctaggtacgtaatcatttggtaccactggaggacgcactggctccagtgtgcgatagggggagtgccgcccaagtgtccctttccctgacatagggggactagggggcttctgagttggaggtgttgtacgcggcagcccacccatcttcatgttctgggtactcaccttaaatctaagcaaccactttactccatgtccaatatcatctagaattgtatagtcaataggttttctaatataacgaactggtcgttcaaggttggctggagcaataatcttatgtgtccttgaagtgtttttattggtagtcaaaataccaatttctcttcttgcaactttctctttatgaatatcaactgtttgtgaaatatgattgattgaagattccatccttcgtagctgggatgcctggatatccagcatctgcaggacattgttggccaaggtgtttatcagataggcaacacttgctaaggattgggtggtgtaggctttggtttcttctagggctctctgcttatctgctgactgtatgtagttgttctcgcagtaatcggccacccgttccagatttgtgtagctgtcgaagagggcccggcggccccccgggatttcctcttccagcagcatctgcagctccgccatcttcacatcctcctcctcctcctcctcatacaggtcgcagagggagcggcggccgcagcgccaaggaaacccaggaccgggagaggaggagcggcggcgacggcggcggtaactcggaagg

SEQ ID NO: 11817 - RNA, 3214 nt, Homo sapiens
  source 1..3214: mol_type = other RNA
ctgaatagctgggactacaggtgtgcgccaccacgcccagctaatttttgtgtttttagtagagatggggtttcaccatgttggccaggatggtctcaatttattgacctcatgatccacccacctcggcctccgaaagtgctgggattacaggcataagccaccacacccagcctgtgggaactatttattggatttcaaaacaccctctgcctcattaatccactaagctttctcagcaaaaagctgtttaaataaataatgggaacatctaatttaaaacagtttttctaattatagaccagtacacgaagaagagcttaacttatccaagtatagtctagtttgggtccataatggagctgaaggctcagaggacattcagggccattacactgcaggaaaacaaggaataagggatgtagaaatgacctaagaaaagcacgaagtggaatgtatactggaggcaagttaatgaaagctaataaatacaaagtgctgggaaaaatctaaaagcaaaatagctattgtaacttgcaatgcattaaaaacaactttaaaaccaaaaagtcttgataaggaaactctatagtggggtctcagttaaatgctgatgatttttaatgctcagataacattaagtggaatattaacttctgcatccgacaccatctgaattttctcacacactactacacttgttcacttttcaatcaagttccactttctgaacttgttcaaaacctcatttgaaatatatccagctactgcttttcccctttcacctagcacagggcagttacctggcaaagctctattctggccaagtcactgggactgagtagaacccacgttagcagctctggacctgaacaggagctggcccaacatcacagtgaccacccacaaagagacaagccctcctggatttttttcagcatttcttatactgactacagtagtgatgattaaagttatctgccctacagactccactgaatttgaagctgtatttattgtacagatgggggaaatgtgttttattgtgtcagttatattaatttttatcaatgtgattagatacatattttggcctattaatcttattcattatattcttagtctgagatgggttttaattctgactaacagcagctacttaagagtccaatcatacaaaatcaggagagtattaccctttctacagctaagcgagtcagtaatacagcagcaactaatactggccattaataacgtccagagagcacattagcaaaccttgtactcccagtgactgtcaggagacttgaaaataactactattctcttccaaagtagaatagcgtttttctagatagtgaaggaaatgatagtcatagttggtctgaactccaagatcctactcctcaaaacagcaccgaagcaggggttcgggatgcctgctaagagcatttccacagttcaagtctcttcagaaccttagggaccttcgtgtctagcttcacacacccacctccacatatgaaccagcctaccacacttcacatctgggtacactggccattagcaacaatgcagtctcatgcagcagcacattaaaatcaaacgggtggcaatcgttcaccaccctcagagtgttgggagactttcacatttcatcatccttataatccacaaacagaaacatgaagggatgcaagtgagttcagcattcactcgtttggtgcactcaagtgctgagagaatgcagaatttacagtgtcacagaggaaaaaagccatctgaaataattgtaaaaatggttaagtgtggtatttaaatgttggttccctcctcttcatacaagtggaagaaaagaaggggctagggtacccactgggccatgaggttaaccccttagcacaggcaatgaagaacatccaatgccacagattctgcaggaggagaaatcccaagggtatacagtattcctgagaaagatcccagatttttctgaatcagtcttaatctgattttgttttggctacacagttatgctgttatacctttgacatacataaaaatggtcattttatttcaatccagacagctcagcattgtacaaatgatggcagaaagatccatttgttcagactcagcttgctttgtttttaatactggggaataaaccaaaaaaaaaagtgtaatttttatcatttgtatccttcattctactttactggagtggaatccccagggccttcagataatctgggaagacctgactattcctgtgaggcaagcacagccctgctgagctttactcagaataatgcatgatagactcaacgtaattcccaggaaaaagcccagtcactccattcataactccctcataccaaccatcgtcattcttcttgatgacataaataatggctccttcctgaaaggacagctcatcttccttgtcttttgtatagtcataaattgccacaaccttttccaagtaagaacgtggagcccacggtgggtcctcttcagcataaggatcactatactcaaccacagcagcttcctcctcttcgtaatcttctggaggaggaggaggtgggggagactcatcaaagactggttcttccacaggtggcggtggaggtggtgtatctgaaactggattctggctataaaaaggtcctccattcatctgattctgaaggcttgtttgtgaagtaatggaaggagggcgtctatagggcaacgagccccctattgttgggggagtatggcgagaggcaggcctattcatgctgtagaactgtacaggatgacttgtgaaatatgattgattgaagattccatccttcgtagctgggatgcctggatatccagcatctgcaggacattgttggccaaggtgtttatcagataggcaacacttgctaaggattgggtggtgtaggctttggtttcttctagggctctctgcttatctgctgactgtatgtagttgttctcgcagtaatcggccacccgttccagatttgtgtagctgtcgaagagggcccggcggccccccgggatttcctcttccagcagcatctgcagctccgccatcttcacatcctcctcctcctcctcctcatacaggtcgcagagggagcggcggccgcagcgccaaggaaacccaggaccgggagaggaggagcggcggcgacggcggcggtaactcggaagg

SEQ ID NO: 11818 - RNA, 4081 nt, Homo sapiens
  source 1..4081: mol_type = other RNA
ctgaatagctgggactacaggtgtgcgccaccacgcccagctaatttttgtgtttttagtagagatggggtttcaccatgttggccaggatggtctcaatttattgacctcatgatccacccacctcggcctccgaaagtgctgggattacaggcataagccaccacacccagcctgtgggaactatttattggatttcaaaacaccctctgcctcattaatccactaagctttctcagcaaaaagctgtttaaataaataatgggaacatctaatttaaaacagtttttctaattatagaccagtacacgaagaagagcttaacttatccaagtatagtctagtttgggtccataatggagctgaaggctcagaggacattcagggccattacactgcaggaaaacaaggaataagggatgtagaaatgacctaagaaaagcacgaagtggaatgtatactggaggcaagttaatgaaagctaataaatacaaagtgctgggaaaaatctaaaagcaaaatagctattgtaacttgcaatgcattaaaaacaactttaaaaccaaaaagtcttgataaggaaactctatagtggggtctcagttaaatgctgatgatttttaatgctcagataacattaagtggaatattaacttctgcatccgacaccatctgaattttctcacacactactacacttgttcacttttcaatcaagttccactttctgaacttgttcaaaacctcatttgaaatatatccagctactgcttttcccctttcacctagcacagggcagttacctggcaaagctctattctggccaagtcactgggactgagtagaacccacgttagcagctctggacctgaacaggagctggcccaacatcacagtgaccacccacaaagagacaagccctcctggatttttttcagcatttcttatactgactacagtagtgatgattaaagttatctgccctacagactccactgaatttgaagctgtatttattgtacagatgggggaaatgtgttttattgtgtcagttatattaatttttatcaatgtgattagatacatattttggcctattaatcttattcattatattcttagtctgagatgggttttaattctgactaacagcagctacttaagagtccaatcatacaaaatcaggagagtattaccctttctacagctaagcgagtcagtaatacagcagcaactaatactggccattaataacgtccagagagcacattagcaaaccttgtactcccagtgactgtcaggagacttgaaaataactactattctcttccaaagtagaatagcgtttttctagatagtgaaggaaatgatagtcatagttggtctgaactccaagatcctactcctcaaaacagcaccgaagcaggggttcgggatgcctgctaagagcatttccacagttcaagtctcttcagaaccttagggaccttcgtgtctagcttcacacacccacctccacatatgaaccagcctaccacacttcacatctgggtacactggccattagcaacaatgcagtctcatgcagcagcacattaaaatcaaacgggtggcaatcgttcaccaccctcagagtgttgggagactttcacatttcatcatccttataatccacaaacagaaacatgaagggatgcaagtgagttcagcattcactcgtttggtgcactcaagtgctgagagaatgcagaatttacagtgtcacagaggaaaaaagccatctgaaataattgtaaaaatggttaagtgtggtatttaaatgttggttccctcctcttcatacaagtggaagaaaagaaggggctagggtacccactgggccatgaggttaaccccttagcacaggcaatgaagaacatccaatgccacagattctgcaggaggagaaatcccaagggtatacagtattcctgagaaagatcccagatttttctgaatcagtcttaatctgattttgttttggctacacagttatgctgttatacctttgacatacataaaaatggtcattttatttcaatccagacagctcagcattgtacaaatgatggcagaaagatccatttgttcagactcagcttgctttgtttttaatactggggaataaaccaaaaaaaaaagtgtaatttttatcatttgtatccttcattctactttactggagtggaatccccagggccttcagataatctgggaagacctgactattcctgtgaggcaagcacagccctgctgagctttactcagaataatgcatgatagactcaacgtaattcccaggaaaaagcccagtcactccattcataactccctcataccaaccatcgtcattcttcttgatgacataaataatggctccttcctgaaaggacagctcatcttccttgtcttttgtatagtcataaattgccacaaccttttccaagtaagaacgtggagcccacggtgggtcctcttcagcataaggatcactatactcaaccacagcagcttcctcctcttcgtaatcttctggaggaggaggaggtgggggagactcatcaaagactggttcttccacaggtggcggtggaggtggtgtatctgaaactttaataaggtggtcgaaattaattcagataccacatcattttcttttcggaccttgtaagatttcatctgacaagaacgtctgtgagccagaatatactgtctttcttggagttgagctggattctggctataaaaaggtcctccattcatctgattctgaaggcttgtttgtgaagtaatggaaggagggcgtctatagggcaacgagccccctattgttgggggagtatggcgagaggcaggcctattcatgctgtagaactgtacaggatgacctgtagggggagtggaagaaacaacagggggagttggagaagtgaagccatcagcaagggtctgggcacccccagcagcagcgtctggggcagtggaggaagggacagtagcaggaacaagaggagcaggggcagatgcagaagtagcaggaaggggaggagtgccagcagagccagcaggggctggaaagacactgggaggagatggagtaggaacagcaataggaacccccacactaccacttccactgttctctcgactgctgctccgactacttgggtggctccctccactactcccactgctgctgtaagttcgatttctttgattcacagaagctgtcctcacagggctctgctgcgagggagccatattacgggttgggctaggtacgtaatcatttggtaccactggaggacgcactggctccagtgtgcgatagggggagtgccgcccaagtgtccctttccctgacatagggggactagggggcttctgagttggaggtgttgtacgcggcagcccacccatcttcatgttctgggtactcaccttaaatctaagcaaccactttactccatgtccaatatcatctagaattgtatagtcaataggttttctaatataacgaactggtcgttcaaggttggctggagcaataatcttatgtgtccttgaagtgtttttattggtagtcaaaataccaatttctcttcttgcaactttctctttatgaatatcaactgtttgtgaaatatgattgattgaagattccatccttcgtagctgggatgcctggatatccagcatctgcaggacattgttggccaaggtgtttatcagataggcaacacttgctaaggattgggtggtgtaggctttggtttcttctagggctctctgcttatctgctgactgtatgtagttgttctcgcagtaatcggccacccgttccagatttgtgtagctgtcgaagagggcccggcggccccccgggatttcctcttccagcagcatctgcagctccgccatcttcacatcctcctcctcctcctcctcatacaggtcgcagagggagcggcggccgcagcgccaaggaaacccaggaccgggagaggaggagcggcggcgacggcggcggtaactcggaagg

SEQ ID NO: 11819 - RNA, 3947 nt, Homo sapiens
  source 1..3947: mol_type = other RNA
ctgaatagctgggactacaggtgtgcgccaccacgcccagctaatttttgtgtttttagtagagatggggtttcaccatgttggccaggatggtctcaatttattgacctcatgatccacccacctcggcctccgaaagtgctgggattacaggcataagccaccacacccagcctgtgggaactatttattggatttcaaaacaccctctgcctcattaatccactaagctttctcagcaaaaagctgtttaaataaataatgggaacatctaatttaaaacagtttttctaattatagaccagtacacgaagaagagcttaacttatccaagtatagtctagtttgggtccataatggagctgaaggctcagaggacattcagggccattacactgcaggaaaacaaggaataagggatgtagaaatgacctaagaaaagcacgaagtggaatgtatactggaggcaagttaatgaaagctaataaatacaaagtgctgggaaaaatctaaaagcaaaatagctattgtaacttgcaatgcattaaaaacaactttaaaaccaaaaagtcttgataaggaaactctatagtggggtctcagttaaatgctgatgatttttaatgctcagataacattaagtggaatattaacttctgcatccgacaccatctgaattttctcacacactactacacttgttcacttttcaatcaagttccactttctgaacttgttcaaaacctcatttgaaatatatccagctactgcttttcccctttcacctagcacagggcagttacctggcaaagctctattctggccaagtcactgggactgagtagaacccacgttagcagctctggacctgaacaggagctggcccaacatcacagtgaccacccacaaagagacaagccctcctggatttttttcagcatttcttatactgactacagtagtgatgattaaagttatctgccctacagactccactgaatttgaagctgtatttattgtacagatgggggaaatgtgttttattgtgtcagttatattaatttttatcaatgtgattagatacatattttggcctattaatcttattcattatattcttagtctgagatgggttttaattctgactaacagcagctacttaagagtccaatcatacaaaatcaggagagtattaccctttctacagctaagcgagtcagtaatacagcagcaactaatactggccattaataacgtccagagagcacattagcaaaccttgtactcccagtgactgtcaggagacttgaaaataactactattctcttccaaagtagaatagcgtttttctagatagtgaaggaaatgatagtcatagttggtctgaactccaagatcctactcctcaaaacagcaccgaagcaggggttcgggatgcctgctaagagcatttccacagttcaagtctcttcagaaccttagggaccttcgtgtctagcttcacacacccacctccacatatgaaccagcctaccacacttcacatctgggtacactggccattagcaacaatgcagtctcatgcagcagcacattaaaatcaaacgggtggcaatcgttcaccaccctcagagtgttgggagactttcacatttcatcatccttataatccacaaacagaaacatgaagggatgcaagtgagttcagcattcactcgtttggtgcactcaagtgctgagagaatgcagaatttacagtgtcacagaggaaaaaagccatctgaaataattgtaaaaatggttaagtgtggtatttaaatgttggttccctcctcttcatacaagtggaagaaaagaaggggctagggtacccactgggccatgaggttaaccccttagcacaggcaatgaagaacatccaatgccacagattctgcaggaggagaaatcccaagggtatacagtattcctgagaaagatcccagatttttctgaatcagtcttaatctgattttgttttggctacacagttatgctgttatacctttgacatacataaaaatggtcattttatttcaatccagacagctcagcattgtacaaatgatggcagaaagatccatttgttcagactcagcttgctttgtttttaatactggggaataaaccaaaaaaaaaagtgtaatttttatcatttgtatccttcattctactttactggagtggaatccccagggccttcagataatctgggaagacctgactattcctgtgaggcaagcacagccctgctgagctttactcagaataatgcatgatagactcaacgtaattcccaggaaaaagcccagtcactccattcataactccctcataccaaccatcgtcattcttcttgatgacataaataatggctccttcctgaaaggacagctcatcttccttgtcttttgtatagtcataaattgccacaaccttttccaagtaagaacgtggagcccacggtgggtcctcttcagcataaggatcactatactcaaccacagcagcttcctcctcttcgtaatcttctggaggaggaggaggtgggggagactcatcaaagactggttcttccacaggtggcggtggaggtggtgtatctgaaatattttcttggactctggccacaaatcccattaaaggtaactgaggagttacctgtaggatggagggaggaggaggagcaagagatacatgtccacaatagccatggtgtctaatatttgttcttgccctctctggattctggctataaaaaggtcctccattcatctgattctgaaggcttgtttgtgaagtaatggaaggagggcgtctatagggcaacgagccccctattgttgggggagtatggcgagaggcaggcctattcatgctgtagaactgtacaggatgacctgtagggggagtggaagaaacaacagggggagttggagaagtgaagccatcagcaagggtctgggcacccccagcagcagcgtctggggcagtggaggaagggacagtagcaggaacaagaggagcaggggcagatgcagaagtagcaggaaggggaggagtgccagcagagccagcaggggctggaaagacactgggaggagatggagtaggaacagcaataggaacccccacactaccacttccactgttctctcgactgctgctccgactacttgggtggctccctccactactcccactgctgccaagtgtccctttccctgacatagggggactagggggcttctgagttggaggtgttgtacgcggcagcccacccatcttcatgttctgggtactcaccttaaatctaagcaaccactttactccatgtccaatatcatctagaattgtatagtcaataggttttctaatataacgaactggtcgttcaaggttggctggagcaataatcttatgtgtccttgaagtgtttttattggtagtcaaaataccaatttctcttcttgcaactttctctttatgaatatcaactgtttgtgaaatatgattgattgaagattccatccttcgtagctgggatgcctggatatccagcatctgcaggacattgttggccaaggtgtttatcagataggcaacacttgctaaggattgggtggtgtaggctttggtttcttctagggctctctgcttatctgctgactgtatgtagttgttctcgcagtaatcggccacccgttccagatttgtgtagctgtcgaagagggcccggcggccccccgggatttcctcttccagcagcatctgcagctccgccatcttcacatcctcctcctcctcctcctcatacaggtcgcagagggagcggcggccgcagcgccaaggaaacccaggaccgggagaggaggagcggcggcgacggcggcggtaactcggaagg

SEQ ID NO: 11820 - RNA, 3387 nt, Homo sapiens
  source 1..3387: mol_type = other RNA
ctgaatagctgggactacaggtgtgcgccaccacgcccagctaatttttgtgtttttagtagagatggggtttcaccatgttggccaggatggtctcaatttattgacctcatgatccacccacctcggcctccgaaagtgctgggattacaggcataagccaccacacccagcctgtgggaactatttattggatttcaaaacaccctctgcctcattaatccactaagctttctcagcaaaaagctgtttaaataaataatgggaacatctaatttaaaacagtttttctaattatagaccagtacacgaagaagagcttaacttatccaagtatagtctagtttgggtccataatggagctgaaggctcagaggacattcagggccattacactgcaggaaaacaaggaataagggatgtagaaatgacctaagaaaagcacgaagtggaatgtatactggaggcaagttaatgaaagctaataaatacaaagtgctgggaaaaatctaaaagcaaaatagctattgtaacttgcaatgcattaaaaacaactttaaaaccaaaaagtcttgataaggaaactctatagtggggtctcagttaaatgctgatgatttttaatgctcagataacattaagtggaatattaacttctgcatccgacaccatctgaattttctcacacactactacacttgttcacttttcaatcaagttccactttctgaacttgttcaaaacctcatttgaaatatatccagctactgcttttcccctttcacctagcacagggcagttacctggcaaagctctattctggccaagtcactgggactgagtagaacccacgttagcagctctggacctgaacaggagctggcccaacatcacagtgaccacccacaaagagacaagccctcctggatttttttcagcatttcttatactgactacagtagtgatgattaaagttatctgccctacagactccactgaatttgaagctgtatttattgtacagatgggggaaatgtgttttattgtgtcagttatattaatttttatcaatgtgattagatacatattttggcctattaatcttattcattatattcttagtctgagatgggttttaattctgactaacagcagctacttaagagtccaatcatacaaaatcaggagagtattaccctttctacagctaagcgagtcagtaatacagcagcaactaatactggccattaataacgtccagagagcacattagcaaaccttgtactcccagtgactgtcaggagacttgaaaataactactattctcttccaaagtagaatagcgtttttctagatagtgaaggaaatgatagtcatagttggtctgaactccaagatcctactcctcaaaacagcaccgaagcaggggttcgggatgcctgctaagagcatttccacagttcaagtctcttcagaaccttagggaccttcgtgtctagcttcacacacccacctccacatatgaaccagcctaccacacttcacatctgggtacactggccattagcaacaatgcagtctcatgcagcagcacattaaaatcaaacgggtggcaatcgttcaccaccctcagagtgttgggagactttcacatttcatcatccttataatccacaaacagaaacatgaagggatgcaagtgagttcagcattcactcgtttggtgcactcaagtgctgagagaatgcagaatttacagtgtcacagaggaaaaaagccatctgaaataattgtaaaaatggttaagtgtggtatttaaatgttggttccctcctcttcatacaagtggaagaaaagaaggggctagggtacccactgggccatgaggttaaccccttagcacaggcaatgaagaacatccaatgccacagattctgcaggaggagaaatcccaagggtatacagtattcctgagaaagatcccagatttttctgaatcagtcttaatctgattttgttttggctacacagttatgctgttatacctttgacatacataaaaatggtcattttatttcaatccagacagctcagcattgtacaaatgatggcagaaagatccatttgttcagactcagcttgctttgtttttaatactggggaataaaccaaaaaaaaaagtgtaatttttatcatttgtatccttcattctactttactggagtggaatccccagggccttcagataatctgggaagacctgactattcctgtgaggcaagcacagccctgctgagctttactcagaataatgcatgatagactcaacgtaattcccaggaaaaagcccagtcactccattcataactccctcataccaaccatcgtcattcttcttgatgacataaataatggctccttcctgaaaggacagctcatcttccttgtcttttgtatagtcataaattgccacaaccttttccaagtaagaacgtggagcccacggtgggtcctcttcagcataaggatcactatactcaaccacagcagcttcctcctcttcgtaatcttctggaggaggaggaggtgggggagactcatcaaagactggttcttccacaggtggcggtggaggtggtgtatctgaaatattttcttggactctggccacaaatcccattaaaggtaactgaggagttacctgtaggatggagggaggaggaggagcaagagatactggattctggctataaaaaggtcctccattcatctgattctgaaggcttgtttgtgaagtaatggaaggagggcgtctatagggcaacgagccccctattgttgggggagtatggcgagaggcaggcctattcatgctgtagaactgtacaggatgacataataaaagctgccagcattacagatagcctgtgtttattattaagggttcctcataggcaaataggaaaatattgtggtctcacttgtgaaatatgattgattgaagattccatccttcgtagctgggatgcctggatatccagcatctgcaggacattgttggccaaggtgtttatcagataggcaacacttgctaaggattgggtggtgtaggctttggtttcttctagggctctctgcttatctgctgactgtatgtagttgttctcgcagtaatcggccacccgttccagatttgtgtagctgtcgaagagggcccggcggccccccgggatttcctcttccagcagcatctgcagctccgccatcttcacatcctcctcctcctcctcctcatacaggtcgcagagggagcggcggccgcagcgccaaggaaacccaggaccgggagaggaggagcggcggcgacggcggcggtaactcggaagg

SEQ ID NO: 11821 - RNA, 4236 nt, Homo sapiens
  source 1..4236: mol_type = other RNA
ctgaatagctgggactacaggtgtgcgccaccacgcccagctaatttttgtgtttttagtagagatggggtttcaccatgttggccaggatggtctcaatttattgacctcatgatccacccacctcggcctccgaaagtgctgggattacaggcataagccaccacacccagcctgtgggaactatttattggatttcaaaacaccctctgcctcattaatccactaagctttctcagcaaaaagctgtttaaataaataatgggaacatctaatttaaaacagtttttctaattatagaccagtacacgaagaagagcttaacttatccaagtatagtctagtttgggtccataatggagctgaaggctcagaggacattcagggccattacactgcaggaaaacaaggaataagggatgtagaaatgacctaagaaaagcacgaagtggaatgtatactggaggcaagttaatgaaagctaataaatacaaagtgctgggaaaaatctaaaagcaaaatagctattgtaacttgcaatgcattaaaaacaactttaaaaccaaaaagtcttgataaggaaactctatagtggggtctcagttaaatgctgatgatttttaatgctcagataacattaagtggaatattaacttctgcatccgacaccatctgaattttctcacacactactacacttgttcacttttcaatcaagttccactttctgaacttgttcaaaacctcatttgaaatatatccagctactgcttttcccctttcacctagcacagggcagttacctggcaaagctctattctggccaagtcactgggactgagtagaacccacgttagcagctctggacctgaacaggagctggcccaacatcacagtgaccacccacaaagagacaagccctcctggatttttttcagcatttcttatactgactacagtagtgatgattaaagttatctgccctacagactccactgaatttgaagctgtatttattgtacagatgggggaaatgtgttttattgtgtcagttatattaatttttatcaatgtgattagatacatattttggcctattaatcttattcattatattcttagtctgagatgggttttaattctgactaacagcagctacttaagagtccaatcatacaaaatcaggagagtattaccctttctacagctaagcgagtcagtaatacagcagcaactaatactggccattaataacgtccagagagcacattagcaaaccttgtactcccagtgactgtcaggagacttgaaaataactactattctcttccaaagtagaatagcgtttttctagatagtgaaggaaatgatagtcatagttggtctgaactccaagatcctactcctcaaaacagcaccgaagcaggggttcgggatgcctgctaagagcatttccacagttcaagtctcttcagaaccttagggaccttcgtgtctagcttcacacacccacctccacatatgaaccagcctaccacacttcacatctgggtacactggccattagcaacaatgcagtctcatgcagcagcacattaaaatcaaacgggtggcaatcgttcaccaccctcagagtgttgggagactttcacatttcatcatccttataatccacaaacagaaacatgaagggatgcaagtgagttcagcattcactcgtttggtgcactcaagtgctgagagaatgcagaatttacagtgtcacagaggaaaaaagccatctgaaataattgtaaaaatggttaagtgtggtatttaaatgttggttccctcctcttcatacaagtggaagaaaagaaggggctagggtacccactgggccatgaggttaaccccttagcacaggcaatgaagaacatccaatgccacagattctgcaggaggagaaatcccaagggtatacagtattcctgagaaagatcccagatttttctgaatcagtcttaatctgattttgttttggctacacagttatgctgttatacctttgacatacataaaaatggtcattttatttcaatccagacagctcagcattgtacaaatgatggcagaaagatccatttgttcagactcagcttgctttgtttttaatactggggaataaaccaaaaaaaaaagtgtaatttttatcatttgtatccttcattctactttactggagtggaatccccagggccttcagataatctgggaagacctgactattcctgtgaggcaagcacagccctgctgagctttactcagaataatgcatgatagactcaacgtaattcccaggaaaaagcccagtcactccattcataactccctcataccaaccatcgtcattcttcttgatgacataaataatggctccttcctgaaaggacagctcatcttccttgtcttttgtatagtcataaattgccacaaccttttccaagtaagaacgtggagcccacggtgggtcctcttcagcataaggatcactatactcaaccacagcagcttcctcctcttcgtaatcttctggaggaggaggaggtgggggagactcatcaaagactggttcttccacaggtggcggtggaggtggtgtatctgaaatattttcttggactctggccacaaatcccattaaaggtaactgaggagttacctgtaggatggagggaggaggaggagcaagagatactggattctggctataaaaaggtcctccattcatctgattctgaaggcttgtttgtgaagtaatggaaggagggcgtctatagggcaacgagccccctattgttgggggagtatggcgagaggcaggcctattcatgctgtagaactgtacaggatgacctggaaagacactgggaggagatggagtaggaacagcaataggaacccccacactaccacttccactgttctctcgactgctgctccgactacttgggtggctccctccactactcccactgccaagtgtccctttccctgacatagggggactagggggcttctgagttggaggtgttgtacgcggcagcccacccatcttcatgttctgggtactcaccttaaatctaagcaaccactttactccatgtccaatatcatctagaattgtatagtcaataggttttctaatataacgaactggtcgttcaaggttggctggagcaataatcttatgtgtccttgaagtgtttttattggtagtcaaaataccaatttctcttcttgcaactttctctttatgaatatcaactgtttgtgaaatatgattgattgaagattccatccttcgtagctgggatgcctggatatccagcatctgcaggacattgttggccaaggtgtttatcagataggcaacacttgctaaggattgggtggtgtaggctttggtttcttctagggctctctgcttatctgctgactgtatgtagttgttctcgcagtaatcggccacccgttccagatttgtgtagctgtcgaagagggcccggcggccccccgggatttcctcttccagcagcatctgcagctccgccatcttcacatcctcctcctcctcctcctcatacaggtcgcagagggagcggcggccgcagcgccaaggaaacccaggaccgggagaggaggagcggcggcgacggcggcggtaactcggaaggagcgagaaacagccccagcgcgcgacaggggagggggcgacgggggcggggcgcgagccgacggactccgaggacggtcaccgcggcgacggccggccgggcgcgcgcacgcgcgctcccttccctccgcccccgggagcccgaaaaagattcccaccctcgcccgcgccgccggcccctcccccacttccggcgtctcctagcgacggcgggggtaggggccgggatgcgcgcgggagttggtggtgcagttaacccttccgccgcccgcccgccgctggagcggctggagaagcccccacctcccggcggcctttgttagcccggcgggaacacaccaccctgctcagctggcttcctgccggctccctccgggactcatctcggctccgtccccatggaggtcatcggcctagggaacttctcgaggcttttctccctctgctgctgacgggaggccgaaggagggcacagcctccactcttgggaccctcctctgtgaaagatcacacctcaacag

SEQ ID NO: 11822 - RNA, 3774 nt, Homo sapiens
  source 1..3774: mol_type = other RNA
ctgaatagctgggactacaggtgtgcgccaccacgcccagctaatttttgtgtttttagtagagatggggtttcaccatgttggccaggatggtctcaatttattgacctcatgatccacccacctcggcctccgaaagtgctgggattacaggcataagccaccacacccagcctgtgggaactatttattggatttcaaaacaccctctgcctcattaatccactaagctttctcagcaaaaagctgtttaaataaataatgggaacatctaatttaaaacagtttttctaattatagaccagtacacgaagaagagcttaacttatccaagtatagtctagtttgggtccataatggagctgaaggctcagaggacattcagggccattacactgcaggaaaacaaggaataagggatgtagaaatgacctaagaaaagcacgaagtggaatgtatactggaggcaagttaatgaaagctaataaatacaaagtgctgggaaaaatctaaaagcaaaatagctattgtaacttgcaatgcattaaaaacaactttaaaaccaaaaagtcttgataaggaaactctatagtggggtctcagttaaatgctgatgatttttaatgctcagataacattaagtggaatattaacttctgcatccgacaccatctgaattttctcacacactactacacttgttcacttttcaatcaagttccactttctgaacttgttcaaaacctcatttgaaatatatccagctactgcttttcccctttcacctagcacagggcagttacctggcaaagctctattctggccaagtcactgggactgagtagaacccacgttagcagctctggacctgaacaggagctggcccaacatcacagtgaccacccacaaagagacaagccctcctggatttttttcagcatttcttatactgactacagtagtgatgattaaagttatctgccctacagactccactgaatttgaagctgtatttattgtacagatgggggaaatgtgttttattgtgtcagttatattaatttttatcaatgtgattagatacatattttggcctattaatcttattcattatattcttagtctgagatgggttttaattctgactaacagcagctacttaagagtccaatcatacaaaatcaggagagtattaccctttctacagctaagcgagtcagtaatacagcagcaactaatactggccattaataacgtccagagagcacattagcaaaccttgtactcccagtgactgtcaggagacttgaaaataactactattctcttccaaagtagaatagcgtttttctagatagtgaaggaaatgatagtcatagttggtctgaactccaagatcctactcctcaaaacagcaccgaagcaggggttcgggatgcctgctaagagcatttccacagttcaagtctcttcagaaccttagggaccttcgtgtctagcttcacacacccacctccacatatgaaccagcctaccacacttcacatctgggtacactggccattagcaacaatgcagtctcatgcagcagcacattaaaatcaaacgggtggcaatcgttcaccaccctcagagtgttgggagactttcacatttcatcatccttataatccacaaacagaaacatgaagggatgcaagtgagttcagcattcactcgtttggtgcactcaagtgctgagagaatgcagaatttacagtgtcacagaggaaaaaagccatctgaaataattgtaaaaatggttaagtgtggtatttaaatgttggttccctcctcttcatacaagtggaagaaaagaaggggctagggtacccactgggccatgaggttaaccccttagcacaggcaatgaagaacatccaatgccacagattctgcaggaggagaaatcccaagggtatacagtattcctgagaaagatcccagatttttctgaatcagtcttaatctgattttgttttggctacacagttatgctgttatacctttgacatacataaaaatggtcattttatttcaatccagacagctcagcattgtacaaatgatggcagaaagatccatttgttcagactcagcttgctttgtttttaatactggggaataaaccaaaaaaaaaagtgtaatttttatcatttgtatccttcattctactttactggagtggaatccccagggccttcagataatctgggaagacctgactattcctgtgaggcaagcacagccctgctgagctttactcagaataatgcatgatagactcaacgtaattcccaggaaaaagcccagtcactccattcataactccctcataccaaccatcgtcattcttcttgatgacataaataatggctccttcctgaaaggacagctcatcttccttgtcttttgtatagtcataaattgccacaaccttttccaagtaagaacgtggagcccacggtgggtcctcttcagcataaggatcactatactcaaccacagcagcttcctcctcttcgtaatcttctggaggaggaggaggtgggggagactcatcaaagactggttcttccacaggtggcggtggaggtggtgtatctgaaatattttcttggactctggccacaaatcccattaaaggtaactgaggagttacctgtaggatggagggaggaggaggagcaagagatactggattctggctataaaaaggtcctccattcatctgattctgaaggcttgtttgtgaagtaatggaaggagggcgtctatagggcaacgagccccctattgttgggggagtatggcgagaggcaggcctattcatgctgtagaactgtacaggatgacctggaaagacactgggaggagatggagtaggaacagcaataggaacccccacactaccacttccactgttctctcgactgctgctccgactacttgggtggctccctccactactcccactgccaagtgtccctttccctgacatagggggactagggggcttctgagttggaggtgttgtacgcggcagcccacccatcttcatgttctgggtactcacctttactccatgtccaatatcatctagaattgtatagtcaataggttttctaatataacgaactggtcgttcaaggttggctggagcaataatcttatgtgtccttgaagtgtttttattggtagtcaaaataccaatttctcttcttgcaactttctctttatgaatatcaactgtctcattcaatctcaaactgcaattgtttccaaatttggtcacaaaagtcgactcaagatcaacgcctctaatttgcttgtgaaatatgattgattgaagattccatccttcgtagctgggatgcctggatatccagcatctgcaggacattgttggccaaggtgtttatcagataggcaacacttgctaaggattgggtggtgtaggctttggtttcttctagggctctctgcttatctgctgactgtatgtagttgttctcgcagtaatcggccacccgttccagatttgtgtagctgtcgaagagggcccggcggccccccgggatttcctcttccagcagcatctgcagctccgccatcttcacatcctcctcctcctcctcctcatacaggtcgcagagggagcggcggccgcagcgccaaggaaacccaggaccgggagaggaggagcggcggcgacggcggcggtaactcggaagg

SEQ ID NO: 11823 - RNA, 3698 nt, Homo sapiens
  source 1..3698: mol_type = other RNA
ctgaatagctgggactacaggtgtgcgccaccacgcccagctaatttttgtgtttttagtagagatggggtttcaccatgttggccaggatggtctcaatttattgacctcatgatccacccacctcggcctccgaaagtgctgggattacaggcataagccaccacacccagcctgtgggaactatttattggatttcaaaacaccctctgcctcattaatccactaagctttctcagcaaaaagctgtttaaataaataatgggaacatctaatttaaaacagtttttctaattatagaccagtacacgaagaagagcttaacttatccaagtatagtctagtttgggtccataatggagctgaaggctcagaggacattcagggccattacactgcaggaaaacaaggaataagggatgtagaaatgacctaagaaaagcacgaagtggaatgtatactggaggcaagttaatgaaagctaataaatacaaagtgctgggaaaaatctaaaagcaaaatagctattgtaacttgcaatgcattaaaaacaactttaaaaccaaaaagtcttgataaggaaactctatagtggggtctcagttaaatgctgatgatttttaatgctcagataacattaagtggaatattaacttctgcatccgacaccatctgaattttctcacacactactacacttgttcacttttcaatcaagttccactttctgaacttgttcaaaacctcatttgaaatatatccagctactgcttttcccctttcacctagcacagggcagttacctggcaaagctctattctggccaagtcactgggactgagtagaacccacgttagcagctctggacctgaacaggagctggcccaacatcacagtgaccacccacaaagagacaagccctcctggatttttttcagcatttcttatactgactacagtagtgatgattaaagttatctgccctacagactccactgaatttgaagctgtatttattgtacagatgggggaaatgtgttttattgtgtcagttatattaatttttatcaatgtgattagatacatattttggcctattaatcttattcattatattcttagtctgagatgggttttaattctgactaacagcagctacttaagagtccaatcatacaaaatcaggagagtattaccctttctacagctaagcgagtcagtaatacagcagcaactaatactggccattaataacgtccagagagcacattagcaaaccttgtactcccagtgactgtcaggagacttgaaaataactactattctcttccaaagtagaatagcgtttttctagatagtgaaggaaatgatagtcatagttggtctgaactccaagatcctactcctcaaaacagcaccgaagcaggggttcgggatgcctgctaagagcatttccacagttcaagtctcttcagaaccttagggaccttcgtgtctagcttcacacacccacctccacatatgaaccagcctaccacacttcacatctgggtacactggccattagcaacaatgcagtctcatgcagcagcacattaaaatcaaacgggtggcaatcgttcaccaccctcagagtgttgggagactttcacatttcatcatccttataatccacaaacagaaacatgaagggatgcaagtgagttcagcattcactcgtttggtgcactcaagtgctgagagaatgcagaatttacagtgtcacagaggaaaaaagccatctgaaataattgtaaaaatggttaagtgtggtatttaaatgttggttccctcctcttcatacaagtggaagaaaagaaggggctagggtacccactgggccatgaggttaaccccttagcacaggcaatgaagaacatccaatgccacagattctgcaggaggagaaatcccaagggtatacagtattcctgagaaagatcccagatttttctgaatcagtcttaatctgattttgttttggctacacagttatgctgttatacctttgacatacataaaaatggtcattttatttcaatccagacagctcagcattgtacaaatgatggcagaaagatccatttgttcagactcagcttgctttgtttttaatactggggaataaaccaaaaaaaaaagtgtaatttttatcatttgtatccttcattctactttactggagtggaatccccagggccttcagataatctgggaagacctgactattcctgtgaggcaagcacagccctgctgagctttactcagaataatgcatgatagactcaacgtaattcccaggaaaaagcccagtcactccattcataactccctcataccaaccatcgtcattcttcttgatgacataaataatggctccttcctgaaaggacagctcatcttccttgtcttttgtatagtcataaattgccacaaccttttccaagtaagaacgtggagcccacggtgggtcctcttcagcataaggatcactatactcaaccacagcagcttcctcctcttcgtaatcttctggaggaggaggaggtgggggagactcatcaaagactggttcttccacaggtggcggtggaggtggtgtatctgaaatattttcttggactctggccacaaatcccattaaaggtaactgaggagttacctgtaggatggagggaggaggaggagcaagagatactggattctggctataaaaaggtcctccattcatctgattctgaaggcttgtttgtgaagtaatggaaggagggcgtctatagggcaacgagccccctattgttgggggagtatggcgagaggcaggcctattcatgctgtagaactgtacaggatgacctggaaagacactgggaggagatggagtaggaacagcaataggaacccccacactaccacttccactgttctctcgactgctgctccgactacttgggtggctccctccactactcccactgccaagtgtccctttccctgacatagggggactagggggcttctgagttggaggtgttgtacgcggcagcccacccatcttcatgttctgggtactcacctttactccatgtccaatatcatctagaattgtatagtcaataggttttctaatataacgaactggtcgttcaaggttggctggagcaataatcttatgtgtccttgaagtgtttttattggtagtcaaaataccaatttctcttcttgcaactttctctttatgaatatcaactgtttgtgaaatatgattgattgaagattccatccttcgtagctgggatgcctggatatccagcatctgcaggacattgttggccaaggtgtttatcagataggcaacacttgctaaggattgggtggtgtaggctttggtttcttctagggctctctgcttatctgctgactgtatgtagttgttctcgcagtaatcggccacccgttccagatttgtgtagctgtcgaagagggcccggcggccccccgggatttcctcttccagcagcatctgcagctccgccatcttcacatcctcctcctcctcctcctcatacaggtcgcagagggagcggcggccgcagcgccaaggaaacccaggaccgggagaggaggagcggcggcgacggcggcggtaactcggaagg

SEQ ID NO: 11824 - RNA, 3694 nt, Homo sapiens
  source 1..3694: mol_type = other RNA
ctgaatagctgggactacaggtgtgcgccaccacgcccagctaatttttgtgtttttagtagagatggggtttcaccatgttggccaggatggtctcaatttattgacctcatgatccacccacctcggcctccgaaagtgctgggattacaggcataagccaccacacccagcctgtgggaactatttattggatttcaaaacaccctctgcctcattaatccactaagctttctcagcaaaaagctgtttaaataaataatgggaacatctaatttaaaacagtttttctaattatagaccagtacacgaagaagagcttaacttatccaagtatagtctagtttgggtccataatggagctgaaggctcagaggacattcagggccattacactgcaggaaaacaaggaataagggatgtagaaatgacctaagaaaagcacgaagtggaatgtatactggaggcaagttaatgaaagctaataaatacaaagtgctgggaaaaatctaaaagcaaaatagctattgtaacttgcaatgcattaaaaacaactttaaaaccaaaaagtcttgataaggaaactctatagtggggtctcagttaaatgctgatgatttttaatgctcagataacattaagtggaatattaacttctgcatccgacaccatctgaattttctcacacactactacacttgttcacttttcaatcaagttccactttctgaacttgttcaaaacctcatttgaaatatatccagctactgcttttcccctttcacctagcacagggcagttacctggcaaagctctattctggccaagtcactgggactgagtagaacccacgttagcagctctggacctgaacaggagctggcccaacatcacagtgaccacccacaaagagacaagccctcctggatttttttcagcatttcttatactgactacagtagtgatgattaaagttatctgccctacagactccactgaatttgaagctgtatttattgtacagatgggggaaatgtgttttattgtgtcagttatattaatttttatcaatgtgattagatacatattttggcctattaatcttattcattatattcttagtctgagatgggttttaattctgactaacagcagctacttaagagtccaatcatacaaaatcaggagagtattaccctttctacagctaagcgagtcagtaatacagcagcaactaatactggccattaataacgtccagagagcacattagcaaaccttgtactcccagtgactgtcaggagacttgaaaataactactattctcttccaaagtagaatagcgtttttctagatagtgaaggaaatgatagtcatagttggtctgaactccaagatcctactcctcaaaacagcaccgaagcaggggttcgggatgcctgctaagagcatttccacagttcaagtctcttcagaaccttagggaccttcgtgtctagcttcacacacccacctccacatatgaaccagcctaccacacttcacatctgggtacactggccattagcaacaatgcagtctcatgcagcagcacattaaaatcaaacgggtggcaatcgttcaccaccctcagagtgttgggagactttcacatttcatcatccttataatccacaaacagaaacatgaagggatgcaagtgagttcagcattcactcgtttggtgcactcaagtgctgagagaatgcagaatttacagtgtcacagaggaaaaaagccatctgaaataattgtaaaaatggttaagtgtggtatttaaatgttggttccctcctcttcatacaagtggaagaaaagaaggggctagggtacccactgggccatgaggttaaccccttagcacaggcaatgaagaacatccaatgccacagattctgcaggaggagaaatcccaagggtatacagtattcctgagaaagatcccagatttttctgaatcagtcttaatctgattttgttttggctacacagttatgctgttatacctttgacatacataaaaatggtcattttatttcaatccagacagctcagcattgtacaaatgatggcagaaagatccatttgttcagactcagcttgctttgtttttaatactggggaataaaccaaaaaaaaaagtgtaatttttatcatttgtatccttcattctactttactggagtggaatccccagggccttcagataatctgggaagacctgactattcctgtgaggcaagcacagccctgctgagctttactcagaataatgcatgatagactcaacgtaattcccaggaaaaagcccagtcactccattcataactccctcataccaaccatcgtcattcttcttgatgacataaataatggctccttcctgaaaggacagctcatcttccttgtcttttgtatagtcataaattgccacaaccttttccaagtaagaacgtggagcccacggtgggtcctcttcagcataaggatcactatactcaaccacagcagcttcctcctcttcgtaatcttctggaggaggaggaggtgggggagactcatcaaagactggttcttccacaggtggcggtggaggtggtgtatctgaaatattttcttggactctggccacaaatcccattaaaggtaactgaggagttacctgtaggatggagggaggaggaggagcaagagatactggattctggctataaaaaggtcctccattcatctgattctgaaggcttgtttgtgaagtaatggaaggagggcgtctatagggcaacgagccccctattgttgggggagtatggcgagaggcaggcctattcatgctgtagaactgtacaggatgacctggaaagacactgggaggagatggagtaggaacagcaataggaacccccacactaccacttccactgttctctcgactgctgctccgactacttgggtggctccctccactactcccactgccaagtgtccctttccctgacatagggggactagggggcttctgagttggaggtgttgtacgcggcagcccacccatcttcatgttctgggtactcacctttactccatgtccaatatcatctagaattgtatagtcaataggttttctaatataacgaactggtcgttcaaggttggctggagcaataatcttatgtgtccttgaagtgtttttattggtagtcaaaataccaatttctcttcttgcaactttctctttatgaatatcaactgtttgtgaaatatgattgattgaagattccatccttcgtagctgggatgcctggatatccagcatctgcaggacattgttggccaaggtgtttatcagataggcaacacttgctaaggattgggtggtgtaggctttggtttcttctagggctctctgcttatctgctgtatgtagttgttctcgcagtaatcggccacccgttccagatttgtgtagctgtcgaagagggcccggcggccccccgggatttcctcttccagcagcatctgcagctccgccatcttcacatcctcctcctcctcctcctcatacaggtcgcagagggagcggcggccgcagcgccaaggaaacccaggaccgggagaggaggagcggcggcgacggcggcggtaactcggaagg

SEQ ID NO: 11825 - RNA, 3825 nt, Homo sapiens
  source 1..3825: mol_type = other RNA
ctgaatagctgggactacaggtgtgcgccaccacgcccagctaatttttgtgtttttagtagagatggggtttcaccatgttggccaggatggtctcaatttattgacctcatgatccacccacctcggcctccgaaagtgctgggattacaggcataagccaccacacccagcctgtgggaactatttattggatttcaaaacaccctctgcctcattaatccactaagctttctcagcaaaaagctgtttaaataaataatgggaacatctaatttaaaacagtttttctaattatagaccagtacacgaagaagagcttaacttatccaagtatagtctagtttgggtccataatggagctgaaggctcagaggacattcagggccattacactgcaggaaaacaaggaataagggatgtagaaatgacctaagaaaagcacgaagtggaatgtatactggaggcaagttaatgaaagctaataaatacaaagtgctgggaaaaatctaaaagcaaaatagctattgtaacttgcaatgcattaaaaacaactttaaaaccaaaaagtcttgataaggaaactctatagtggggtctcagttaaatgctgatgatttttaatgctcagataacattaagtggaatattaacttctgcatccgacaccatctgaattttctcacacactactacacttgttcacttttcaatcaagttccactttctgaacttgttcaaaacctcatttgaaatatatccagctactgcttttcccctttcacctagcacagggcagttacctggcaaagctctattctggccaagtcactgggactgagtagaacccacgttagcagctctggacctgaacaggagctggcccaacatcacagtgaccacccacaaagagacaagccctcctggatttttttcagcatttcttatactgactacagtagtgatgattaaagttatctgccctacagactccactgaatttgaagctgtatttattgtacagatgggggaaatgtgttttattgtgtcagttatattaatttttatcaatgtgattagatacatattttggcctattaatcttattcattatattcttagtctgagatgggttttaattctgactaacagcagctacttaagagtccaatcatacaaaatcaggagagtattaccctttctacagctaagcgagtcagtaatacagcagcaactaatactggccattaataacgtccagagagcacattagcaaaccttgtactcccagtgactgtcaggagacttgaaaataactactattctcttccaaagtagaatagcgtttttctagatagtgaaggaaatgatagtcatagttggtctgaactccaagatcctactcctcaaaacagcaccgaagcaggggttcgggatgcctgctaagagcatttccacagttcaagtctcttcagaaccttagggaccttcgtgtctagcttcacacacccacctccacatatgaaccagcctaccacacttcacatctgggtacactggccattagcaacaatgcagtctcatgcagcagcacattaaaatcaaacgggtggcaatcgttcaccaccctcagagtgttgggagactttcacatttcatcatccttataatccacaaacagaaacatgaagggatgcaagtgagttcagcattcactcgtttggtgcactcaagtgctgagagaatgcagaatttacagtgtcacagaggaaaaaagccatctgaaataattgtaaaaatggttaagtgtggtatttaaatgttggttccctcctcttcatacaagtggaagaaaagaaggggctagggtacccactgggccatgaggttaaccccttagcacaggcaatgaagaacatccaatgccacagattctgcaggaggagaaatcccaagggtatacagtattcctgagaaagatcccagatttttctgaatcagtcttaatctgattttgttttggctacacagttatgctgttatacctttgacatacataaaaatggtcattttatttcaatccagacagctcagcattgtacaaatgatggcagaaagatccatttgttcagactcagcttgctttgtttttaatactggggaataaaccaaaaaaaaaagtgtaatttttatcatttgtatccttcattctactttactggagtggaatccccagggccttcagataatctgggaagacctgactattcctgtgaggcaagcacagccctgctgagctttactcagaataatgcatgatagactcaacgtaattcccaggaaaaagcccagtcactccattcataactccctcataccaaccatcgtcattcttcttgatgacataaataatggctccttcctgaaaggacagctcatcttccttgtcttttgtatagtcataaattgccacaaccttttccaagtaagaacgtggagcccacggtgggtcctcttcagcataaggatcactatactcaaccacagcagcttcctcctcttcgtaatcttctggaggaggaggaggtgggggagactcatcaaagactggttcttccacaggtggcggtggaggtggtgtatctgaaatattttcttggactctggccacaaatcccattaaaggtaactgaggagttacctgtaggatggagggaggaggaggagcaagagatactggattctggctataaaaaggtcctccattcatctgattctgaaggcttgtttgtgaagtaatggaaggagggcgtctatagggcaacgagccccctattgttgggggagtatggcgagaggcaggcctattcatgctgtagaactgtacaggatgacctggaaagacactgggaggagatggagtaggaacagcaataggaacccccacactaccacttccactgttctctcgactgctgctccgactacttgggtggctccctccactactcccactgctgccaagtgtccctttccctgacatagggggactagggggcttctgagttggaggtgttgtacgcggcagcccacccatcttcatgttctgggtactcacctttactccatgtccaatatcatctagaattgtatagtcaataggttttctaatataacgaactggtcgttcaaggttggctggagcaataatcttatgtgtccttgaagtgtttttattggtagtcaaaataccaatttctcttcttgcaactttctctttatgaatatcaactgtttgtgaaatatgattgattgaagattccatccttcgtagctgggatgcctggatatccagcatctgcaggacattgttggccaaggtgtttatcagataggcaacacttgctaaggattgggtggtgtaggctttggtttcttctagggctctctgcttatctgctgactgtagtcccagactactgagagactgaggcaggatgatcacttgagcacaggagttcaaggctgcagtgagctatgatcacaccactgcattccagcctgcatgacataccaagaccccatctctgtatgtagttgttctcgcagtaatcggccacccgttccagatttgtgtagctgtcgaagagggcccggcggccccccgggatttcctcttccagcagcatctgcagctccgccatcttcacatcctcctcctcctcctcctcatacaggtcgcagagggagcggcggccgcagcgccaaggaaacccaggaccgggagaggaggagcggcggcgacggcggcggtaactcggaagg

SEQ ID NO: 11826 - RNA, 3701 nt, Homo sapiens
  source 1..3701: mol_type = other RNA
ctgaatagctgggactacaggtgtgcgccaccacgcccagctaatttttgtgtttttagtagagatggggtttcaccatgttggccaggatggtctcaatttattgacctcatgatccacccacctcggcctccgaaagtgctgggattacaggcataagccaccacacccagcctgtgggaactatttattggatttcaaaacaccctctgcctcattaatccactaagctttctcagcaaaaagctgtttaaataaataatgggaacatctaatttaaaacagtttttctaattatagaccagtacacgaagaagagcttaacttatccaagtatagtctagtttgggtccataatggagctgaaggctcagaggacattcagggccattacactgcaggaaaacaaggaataagggatgtagaaatgacctaagaaaagcacgaagtggaatgtatactggaggcaagttaatgaaagctaataaatacaaagtgctgggaaaaatctaaaagcaaaatagctattgtaacttgcaatgcattaaaaacaactttaaaaccaaaaagtcttgataaggaaactctatagtggggtctcagttaaatgctgatgatttttaatgctcagataacattaagtggaatattaacttctgcatccgacaccatctgaattttctcacacactactacacttgttcacttttcaatcaagttccactttctgaacttgttcaaaacctcatttgaaatatatccagctactgcttttcccctttcacctagcacagggcagttacctggcaaagctctattctggccaagtcactgggactgagtagaacccacgttagcagctctggacctgaacaggagctggcccaacatcacagtgaccacccacaaagagacaagccctcctggatttttttcagcatttcttatactgactacagtagtgatgattaaagttatctgccctacagactccactgaatttgaagctgtatttattgtacagatgggggaaatgtgttttattgtgtcagttatattaatttttatcaatgtgattagatacatattttggcctattaatcttattcattatattcttagtctgagatgggttttaattctgactaacagcagctacttaagagtccaatcatacaaaatcaggagagtattaccctttctacagctaagcgagtcagtaatacagcagcaactaatactggccattaataacgtccagagagcacattagcaaaccttgtactcccagtgactgtcaggagacttgaaaataactactattctcttccaaagtagaatagcgtttttctagatagtgaaggaaatgatagtcatagttggtctgaactccaagatcctactcctcaaaacagcaccgaagcaggggttcgggatgcctgctaagagcatttccacagttcaagtctcttcagaaccttagggaccttcgtgtctagcttcacacacccacctccacatatgaaccagcctaccacacttcacatctgggtacactggccattagcaacaatgcagtctcatgcagcagcacattaaaatcaaacgggtggcaatcgttcaccaccctcagagtgttgggagactttcacatttcatcatccttataatccacaaacagaaacatgaagggatgcaagtgagttcagcattcactcgtttggtgcactcaagtgctgagagaatgcagaatttacagtgtcacagaggaaaaaagccatctgaaataattgtaaaaatggttaagtgtggtatttaaatgttggttccctcctcttcatacaagtggaagaaaagaaggggctagggtacccactgggccatgaggttaaccccttagcacaggcaatgaagaacatccaatgccacagattctgcaggaggagaaatcccaagggtatacagtattcctgagaaagatcccagatttttctgaatcagtcttaatctgattttgttttggctacacagttatgctgttatacctttgacatacataaaaatggtcattttatttcaatccagacagctcagcattgtacaaatgatggcagaaagatccatttgttcagactcagcttgctttgtttttaatactggggaataaaccaaaaaaaaaagtgtaatttttatcatttgtatccttcattctactttactggagtggaatccccagggccttcagataatctgggaagacctgactattcctgtgaggcaagcacagccctgctgagctttactcagaataatgcatgatagactcaacgtaattcccaggaaaaagcccagtcactccattcataactccctcataccaaccatcgtcattcttcttgatgacataaataatggctccttcctgaaaggacagctcatcttccttgtcttttgtatagtcataaattgccacaaccttttccaagtaagaacgtggagcccacggtgggtcctcttcagcataaggatcactatactcaaccacagcagcttcctcctcttcgtaatcttctggaggaggaggaggtgggggagactcatcaaagactggttcttccacaggtggcggtggaggtggtgtatctgaaatattttcttggactctggccacaaatcccattaaaggtaactgaggagttacctgtaggatggagggaggaggaggagcaagagatactggattctggctataaaaaggtcctccattcatctgattctgaaggcttgtttgtgaagtaatggaaggagggcgtctatagggcaacgagccccctattgttgggggagtatggcgagaggcaggcctattcatgctgtagaactgtacaggatgacctggaaagacactgggaggagatggagtaggaacagcaataggaacccccacactaccacttccactgttctctcgactgctgctccgactacttgggtggctccctccactactcccactgctgccaagtgtccctttccctgacatagggggactagggggcttctgagttggaggtgttgtacgcggcagcccacccatcttcatgttctgggtactcacctttactccatgtccaatatcatctagaattgtatagtcaataggttttctaatataacgaactggtcgttcaaggttggctggagcaataatcttatgtgtccttgaagtgtttttattggtagtcaaaataccaatttctcttcttgcaactttctctttatgaatatcaactgtttgtgaaatatgattgattgaagattccatccttcgtagctgggatgcctggatatccagcatctgcaggacattgttggccaaggtgtttatcagataggcaacacttgctaaggattgggtggtgtaggctttggtttcttctagggctctctgcttatctgctgactgtatgtagttgttctcgcagtaatcggccacccgttccagatttgtgtagctgtcgaagagggcccggcggccccccgggatttcctcttccagcagcatctgcagctccgccatcttcacatcctcctcctcctcctcctcatacaggtcgcagagggagcggcggccgcagcgccaaggaaacccaggaccgggagaggaggagcggcggcgacggcggcggtaactcggaagg

SEQ ID NO: 11827 - RNA, 3697 nt, Homo sapiens
  source 1..3697: mol_type = other RNA
ctgaatagctgggactacaggtgtgcgccaccacgcccagctaatttttgtgtttttagtagagatggggtttcaccatgttggccaggatggtctcaatttattgacctcatgatccacccacctcggcctccgaaagtgctgggattacaggcataagccaccacacccagcctgtgggaactatttattggatttcaaaacaccctctgcctcattaatccactaagctttctcagcaaaaagctgtttaaataaataatgggaacatctaatttaaaacagtttttctaattatagaccagtacacgaagaagagcttaacttatccaagtatagtctagtttgggtccataatggagctgaaggctcagaggacattcagggccattacactgcaggaaaacaaggaataagggatgtagaaatgacctaagaaaagcacgaagtggaatgtatactggaggcaagttaatgaaagctaataaatacaaagtgctgggaaaaatctaaaagcaaaatagctattgtaacttgcaatgcattaaaaacaactttaaaaccaaaaagtcttgataaggaaactctatagtggggtctcagttaaatgctgatgatttttaatgctcagataacattaagtggaatattaacttctgcatccgacaccatctgaattttctcacacactactacacttgttcacttttcaatcaagttccactttctgaacttgttcaaaacctcatttgaaatatatccagctactgcttttcccctttcacctagcacagggcagttacctggcaaagctctattctggccaagtcactgggactgagtagaacccacgttagcagctctggacctgaacaggagctggcccaacatcacagtgaccacccacaaagagacaagccctcctggatttttttcagcatttcttatactgactacagtagtgatgattaaagttatctgccctacagactccactgaatttgaagctgtatttattgtacagatgggggaaatgtgttttattgtgtcagttatattaatttttatcaatgtgattagatacatattttggcctattaatcttattcattatattcttagtctgagatgggttttaattctgactaacagcagctacttaagagtccaatcatacaaaatcaggagagtattaccctttctacagctaagcgagtcagtaatacagcagcaactaatactggccattaataacgtccagagagcacattagcaaaccttgtactcccagtgactgtcaggagacttgaaaataactactattctcttccaaagtagaatagcgtttttctagatagtgaaggaaatgatagtcatagttggtctgaactccaagatcctactcctcaaaacagcaccgaagcaggggttcgggatgcctgctaagagcatttccacagttcaagtctcttcagaaccttagggaccttcgtgtctagcttcacacacccacctccacatatgaaccagcctaccacacttcacatctgggtacactggccattagcaacaatgcagtctcatgcagcagcacattaaaatcaaacgggtggcaatcgttcaccaccctcagagtgttgggagactttcacatttcatcatccttataatccacaaacagaaacatgaagggatgcaagtgagttcagcattcactcgtttggtgcactcaagtgctgagagaatgcagaatttacagtgtcacagaggaaaaaagccatctgaaataattgtaaaaatggttaagtgtggtatttaaatgttggttccctcctcttcatacaagtggaagaaaagaaggggctagggtacccactgggccatgaggttaaccccttagcacaggcaatgaagaacatccaatgccacagattctgcaggaggagaaatcccaagggtatacagtattcctgagaaagatcccagatttttctgaatcagtcttaatctgattttgttttggctacacagttatgctgttatacctttgacatacataaaaatggtcattttatttcaatccagacagctcagcattgtacaaatgatggcagaaagatccatttgttcagactcagcttgctttgtttttaatactggggaataaaccaaaaaaaaaagtgtaatttttatcatttgtatccttcattctactttactggagtggaatccccagggccttcagataatctgggaagacctgactattcctgtgaggcaagcacagccctgctgagctttactcagaataatgcatgatagactcaacgtaattcccaggaaaaagcccagtcactccattcataactccctcataccaaccatcgtcattcttcttgatgacataaataatggctccttcctgaaaggacagctcatcttccttgtcttttgtatagtcataaattgccacaaccttttccaagtaagaacgtggagcccacggtgggtcctcttcagcataaggatcactatactcaaccacagcagcttcctcctcttcgtaatcttctggaggaggaggaggtgggggagactcatcaaagactggttcttccacaggtggcggtggaggtggtgtatctgaaatattttcttggactctggccacaaatcccattaaaggtaactgaggagttacctgtaggatggagggaggaggaggagcaagagatactggattctggctataaaaaggtcctccattcatctgattctgaaggcttgtttgtgaagtaatggaaggagggcgtctatagggcaacgagccccctattgttgggggagtatggcgagaggcaggcctattcatgctgtagaactgtacaggatgacctggaaagacactgggaggagatggagtaggaacagcaataggaacccccacactaccacttccactgttctctcgactgctgctccgactacttgggtggctccctccactactcccactgctgccaagtgtccctttccctgacatagggggactagggggcttctgagttggaggtgttgtacgcggcagcccacccatcttcatgttctgggtactcacctttactccatgtccaatatcatctagaattgtatagtcaataggttttctaatataacgaactggtcgttcaaggttggctggagcaataatcttatgtgtccttgaagtgtttttattggtagtcaaaataccaatttctcttcttgcaactttctctttatgaatatcaactgtttgtgaaatatgattgattgaagattccatccttcgtagctgggatgcctggatatccagcatctgcaggacattgttggccaaggtgtttatcagataggcaacacttgctaaggattgggtggtgtaggctttggtttcttctagggctctctgcttatctgctgtatgtagttgttctcgcagtaatcggccacccgttccagatttgtgtagctgtcgaagagggcccggcggccccccgggatttcctcttccagcagcatctgcagctccgccatcttcacatcctcctcctcctcctcctcatacaggtcgcagagggagcggcggccgcagcgccaaggaaacccaggaccgggagaggaggagcggcggcgacggcggcggtaactcggaagg

SEQ ID NO: 11828 - RNA, 3524 nt, Homo sapiens
  source 1..3524: mol_type = other RNA
ctgaatagctgggactacaggtgtgcgccaccacgcccagctaatttttgtgtttttagtagagatggggtttcaccatgttggccaggatggtctcaatttattgacctcatgatccacccacctcggcctccgaaagtgctgggattacaggcataagccaccacacccagcctgtgggaactatttattggatttcaaaacaccctctgcctcattaatccactaagctttctcagcaaaaagctgtttaaataaataatgggaacatctaatttaaaacagtttttctaattatagaccagtacacgaagaagagcttaacttatccaagtatagtctagtttgggtccataatggagctgaaggctcagaggacattcagggccattacactgcaggaaaacaaggaataagggatgtagaaatgacctaagaaaagcacgaagtggaatgtatactggaggcaagttaatgaaagctaataaatacaaagtgctgggaaaaatctaaaagcaaaatagctattgtaacttgcaatgcattaaaaacaactttaaaaccaaaaagtcttgataaggaaactctatagtggggtctcagttaaatgctgatgatttttaatgctcagataacattaagtggaatattaacttctgcatccgacaccatctgaattttctcacacactactacacttgttcacttttcaatcaagttccactttctgaacttgttcaaaacctcatttgaaatatatccagctactgcttttcccctttcacctagcacagggcagttacctggcaaagctctattctggccaagtcactgggactgagtagaacccacgttagcagctctggacctgaacaggagctggcccaacatcacagtgaccacccacaaagagacaagccctcctggatttttttcagcatttcttatactgactacagtagtgatgattaaagttatctgccctacagactccactgaatttgaagctgtatttattgtacagatgggggaaatgtgttttattgtgtcagttatattaatttttatcaatgtgattagatacatattttggcctattaatcttattcattatattcttagtctgagatgggttttaattctgactaacagcagctacttaagagtccaatcatacaaaatcaggagagtattaccctttctacagctaagcgagtcagtaatacagcagcaactaatactggccattaataacgtccagagagcacattagcaaaccttgtactcccagtgactgtcaggagacttgaaaataactactattctcttccaaagtagaatagcgtttttctagatagtgaaggaaatgatagtcatagttggtctgaactccaagatcctactcctcaaaacagcaccgaagcaggggttcgggatgcctgctaagagcatttccacagttcaagtctcttcagaaccttagggaccttcgtgtctagcttcacacacccacctccacatatgaaccagcctaccacacttcacatctgggtacactggccattagcaacaatgcagtctcatgcagcagcacattaaaatcaaacgggtggcaatcgttcaccaccctcagagtgttgggagactttcacatttcatcatccttataatccacaaacagaaacatgaagggatgcaagtgagttcagcattcactcgtttggtgcactcaagtgctgagagaatgcagaatttacagtgtcacagaggaaaaaagccatctgaaataattgtaaaaatggttaagtgtggtatttaaatgttggttccctcctcttcatacaagtggaagaaaagaaggggctagggtacccactgggccatgaggttaaccccttagcacaggcaatgaagaacatccaatgccacagattctgcaggaggagaaatcccaagggtatacagtattcctgagaaagatcccagatttttctgaatcagtcttaatctgattttgttttggctacacagttatgctgttatacctttgacatacataaaaatggtcattttatttcaatccagacagctcagcattgtacaaatgatggcagaaagatccatttgttcagactcagcttgctttgtttttaatactggggaataaaccaaaaaaaaaagtgtaatttttatcatttgtatccttcattctactttactggagtggaatccccagggccttcagataatctgggaagacctgactattcctgtgaggcaagcacagccctgctgagctttactcagaataatgcatgatagactcaacgtaattcccaggaaaaagcccagtcactccattcataactccctcataccaaccatcgtcattcttcttgatgacataaataatggctccttcctgaaaggacagctcatcttccttgtcttttgtatagtcataaattgccacaaccttttccaagtaagaacgtggagcccacggtgggtcctcttcagcataaggatcactatactcaaccacagcagcttcctcctcttcgtaatcttctggaggaggaggaggtgggggagactcatcaaagactggttcttccacaggtggcggtggaggtggtgtatctgaaatattttcttggactctggccacaaatcccattaaaggtaactgaggagttacctgtaggatggagggaggaggaggagcaagagatactggattctggctataaaaaggtcctccattcatctgattctgaaggcttgtttgtgaagtaatggaaggagggcgtctatagggcaacgagccccctattgttgggggagtatggcgagaggcaggcctattcatgctgtagaactgtacaggatgacctggaaagacactgggaggagatggagtaggaacagcaataggaacccccacactaccacttccactgttctctcgactgctgctccgactacttgggtggctccctccactactcccactgctgccaagtgtccctttccctgacatagggggactagggggcttctgagttggaggtgttgtacgcggcagcccacccatcttcatgttctgggtactcacttgtgaaatatgattgattgaagattccatccttcgtagctgggatgcctggatatccagcatctgcaggacattgttggccaaggtgtttatcagataggcaacacttgctaaggattgggtggtgtaggctttggtttcttctagggctctctgcttatctgctgactgtatgtagttgttctcgcagtaatcggccacccgttccagatttgtgtagctgtcgaagagggcccggcggccccccgggatttcctcttccagcagcatctgcagctccgccatcttcacatcctcctcctcctcctcctcatacaggtcgcagagggagcggcggccgcagcgccaaggaaacccaggaccgggagaggaggagcggcggcgacggcggcggtaactcggaagg

SEQ ID NO: 11829 - RNA, 4386 nt, Homo sapiens
  source 1..4386: mol_type = other RNA
ctgaatagctgggactacaggtgtgcgccaccacgcccagctaatttttgtgtttttagtagagatggggtttcaccatgttggccaggatggtctcaatttattgacctcatgatccacccacctcggcctccgaaagtgctgggattacaggcataagccaccacacccagcctgtgggaactatttattggatttcaaaacaccctctgcctcattaatccactaagctttctcagcaaaaagctgtttaaataaataatgggaacatctaatttaaaacagtttttctaattatagaccagtacacgaagaagagcttaacttatccaagtatagtctagtttgggtccataatggagctgaaggctcagaggacattcagggccattacactgcaggaaaacaaggaataagggatgtagaaatgacctaagaaaagcacgaagtggaatgtatactggaggcaagttaatgaaagctaataaatacaaagtgctgggaaaaatctaaaagcaaaatagctattgtaacttgcaatgcattaaaaacaactttaaaaccaaaaagtcttgataaggaaactctatagtggggtctcagttaaatgctgatgatttttaatgctcagataacattaagtggaatattaacttctgcatccgacaccatctgaattttctcacacactactacacttgttcacttttcaatcaagttccactttctgaacttgttcaaaacctcatttgaaatatatccagctactgcttttcccctttcacctagcacagggcagttacctggcaaagctctattctggccaagtcactgggactgagtagaacccacgttagcagctctggacctgaacaggagctggcccaacatcacagtgaccacccacaaagagacaagccctcctggatttttttcagcatttcttatactgactacagtagtgatgattaaagttatctgccctacagactccactgaatttgaagctgtatttattgtacagatgggggaaatgtgttttattgtgtcagttatattaatttttatcaatgtgattagatacatattttggcctattaatcttattcattatattcttagtctgagatgggttttaattctgactaacagcagctacttaagagtccaatcatacaaaatcaggagagtattaccctttctacagctaagcgagtcagtaatacagcagcaactaatactggccattaataacgtccagagagcacattagcaaaccttgtactcccagtgactgtcaggagacttgaaaataactactattctcttccaaagtagaatagcgtttttctagatagtgaaggaaatgatagtcatagttggtctgaactccaagatcctactcctcaaaacagcaccgaagcaggggttcgggatgcctgctaagagcatttccacagttcaagtctcttcagaaccttagggaccttcgtgtctagcttcacacacccacctccacatatgaaccagcctaccacacttcacatctgggtacactggccattagcaacaatgcagtctcatgcagcagcacattaaaatcaaacgggtggcaatcgttcaccaccctcagagtgttgggagactttcacatttcatcatccttataatccacaaacagaaacatgaagggatgcaagtgagttcagcattcactcgtttggtgcactcaagtgctgagagaatgcagaatttacagtgtcacagaggaaaaaagccatctgaaataattgtaaaaatggttaagtgtggtatttaaatgttggttccctcctcttcatacaagtggaagaaaagaaggggctagggtacccactgggccatgaggttaaccccttagcacaggcaatgaagaacatccaatgccacagattctgcaggaggagaaatcccaagggtatacagtattcctgagaaagatcccagatttttctgaatcagtcttaatctgattttgttttggctacacagttatgctgttatacctttgacatacataaaaatggtcattttatttcaatccagacagctcagcattgtacaaatgatggcagaaagatccatttgttcagactcagcttgctttgtttttaatactggggaataaaccaaaaaaaaaagtgtaatttttatcatttgtatccttcattctactttactggagtggaatccccagggccttcagataatctgggaagacctgactattcctgtgaggcaagcacagccctgctgagctttactcagaataatgcatgatagactcaacgtaattcccaggaaaaagcccagtcactccattcataactccctcataccaaccatcgtcattcttcttgatgacataaataatggctccttcctgaaaggacagctcatcttccttgtcttttgtatagtcataaattgccacaaccttttccaagtaagaacgtggagcccacggtgggtcctcttcagcataaggatcactatactcaaccacagcagcttcctcctcttcgtaatcttctggaggaggaggaggtgggggagactcatcaaagactggttcttccacaggtggcggtggaggtggtgtatctgaaatattttcttggactctggccacaaatcccattaaaggtaactgaggagttacctgtaggatggagggaggaggaggagcaagagatactggattctggctataaaaaggtcctccattcatctgattctgaaggcttgtttgtgaagtaatggaaggagggcgtctatagggcaacgagccccctattgttgggggagtatggcgagaggcaggcctattcatgctgtagaactgtacaggatgacctggaaagacactgggaggagatggagtaggaacagcaataggaacccccacactaccacttccactgttctctcgactgctgctccgactacttgggtggctccctccactactcccactgctgctgtaagttcgatttctttgattcacagaagctgtcctcacagggctctgctgcgagggagccatattacgggttgggctaggtacgtaatcatttggtaccactggaggacgcactggctccagtgtgcgatagggggagtgccgcccaagtgtccctttccctgacatagggggactagggggcttctgagttggaggtgttgtacgcggcagcccacccatcttcatgttctgggtactcaccttaaatctaagcaaccactttactccatgtccaatatcatctagaattgtatagtcaataggttttctaatataacgaactggtcgttcaaggttggctggagcaataatcttatgtgtccttgaagtgtttttattggtagtcaaaataccaatttctcttcttgcaactttctctttatgaatatcaactgtttgtgaaatatgattgattgaagattccatccttcgtagctgggatgcctggatatccagcatctgcaggacattgttggccaaggtgtttatcagataggcaacacttgctaaggattgggtggtgtaggctttggtttcttctagggctctctgcttatctgctgactgtatgtagttgttctcgcagtaatcggccacccgttccagatttgtgtagctgtcgaagagggcccggcggccccccgggatttcctcttccagcagcatctgcagctccgccatcttcacatcctcctcctcctcctcctcatacaggtcgcagagggagcggcggccgcagcgccaaggaaacccaggaccgggagaggaggagcggcggcgacggcggcggtaactcggaaggagcgagaaacagccccagcgcgcgacaggggagggggcgacgggggcggggcgcgagccgacggactccgaggacggtcaccgcggcgacggccggccgggcgcgcgcacgcgcgctcccttccctccgcccccgggagcccgaaaaagattcccaccctcgcccgcgccgccggcccctcccccacttccggcgtctcctagcgacggcgggggtaggggccgggatgcgcgcgggagttggtggtgcagttaacccttccgccgcccgcccgccgctggagcggctggagaagcccccacctcccggcggcctttgttagcccggcgggaacacaccaccctgctcagctggcttcctgccggctccctccgggactcatctcggctccgtccccatggaggtcatcggcctagggaacttctcgaggcttttctccctctgctgctgacgggaggccgaaggagggcacagcctccactcttgggaccctcctctgtgaaagatcacacctcaacag

SEQ ID NO: 11830 - RNA, 3934 nt, Homo sapiens
  source 1..3934: mol_type = other RNA
ctgaatagctgggactacaggtgtgcgccaccacgcccagctaatttttgtgtttttagtagagatggggtttcaccatgttggccaggatggtctcaatttattgacctcatgatccacccacctcggcctccgaaagtgctgggattacaggcataagccaccacacccagcctgtgggaactatttattggatttcaaaacaccctctgcctcattaatccactaagctttctcagcaaaaagctgtttaaataaataatgggaacatctaatttaaaacagtttttctaattatagaccagtacacgaagaagagcttaacttatccaagtatagtctagtttgggtccataatggagctgaaggctcagaggacattcagggccattacactgcaggaaaacaaggaataagggatgtagaaatgacctaagaaaagcacgaagtggaatgtatactggaggcaagttaatgaaagctaataaatacaaagtgctgggaaaaatctaaaagcaaaatagctattgtaacttgcaatgcattaaaaacaactttaaaaccaaaaagtcttgataaggaaactctatagtggggtctcagttaaatgctgatgatttttaatgctcagataacattaagtggaatattaacttctgcatccgacaccatctgaattttctcacacactactacacttgttcacttttcaatcaagttccactttctgaacttgttcaaaacctcatttgaaatatatccagctactgcttttcccctttcacctagcacagggcagttacctggcaaagctctattctggccaagtcactgggactgagtagaacccacgttagcagctctggacctgaacaggagctggcccaacatcacagtgaccacccacaaagagacaagccctcctggatttttttcagcatttcttatactgactacagtagtgatgattaaagttatctgccctacagactccactgaatttgaagctgtatttattgtacagatgggggaaatgtgttttattgtgtcagttatattaatttttatcaatgtgattagatacatattttggcctattaatcttattcattatattcttagtctgagatgggttttaattctgactaacagcagctacttaagagtccaatcatacaaaatcaggagagtattaccctttctacagctaagcgagtcagtaatacagcagcaactaatactggccattaataacgtccagagagcacattagcaaaccttgtactcccagtgactgtcaggagacttgaaaataactactattctcttccaaagtagaatagcgtttttctagatagtgaaggaaatgatagtcatagttggtctgaactccaagatcctactcctcaaaacagcaccgaagcaggggttcgggatgcctgctaagagcatttccacagttcaagtctcttcagaaccttagggaccttcgtgtctagcttcacacacccacctccacatatgaaccagcctaccacacttcacatctgggtacactggccattagcaacaatgcagtctcatgcagcagcacattaaaatcaaacgggtggcaatcgttcaccaccctcagagtgttgggagactttcacatttcatcatccttataatccacaaacagaaacatgaagggatgcaagtgagttcagcattcactcgtttggtgcactcaagtgctgagagaatgcagaatttacagtgtcacagaggaaaaaagccatctgaaataattgtaaaaatggttaagtgtggtatttaaatgttggttccctcctcttcatacaagtggaagaaaagaaggggctagggtacccactgggccatgaggttaaccccttagcacaggcaatgaagaacatccaatgccacagattctgcaggaggagaaatcccaagggtatacagtattcctgagaaagatcccagatttttctgaatcagtcttaatctgattttgttttggctacacagttatgctgttatacctttgacatacataaaaatggtcattttatttcaatccagacagctcagcattgtacaaatgatggcagaaagatccatttgttcagactcagcttgctttgtttttaatactggggaataaaccaaaaaaaaaagtgtaatttttatcatttgtatccttcattctactttactggagtggaatccccagggccttcagataatctgggaagacctgactattcctgtgaggcaagcacagccctgctgagctttactcagaataatgcatgatagactcaacgtaattcccaggaaaaagcccagtcactccattcataactccctcataccaaccatcgtcattcttcttgatgacataaataatggctccttcctgaaaggacagctcatcttccttgtcttttgtatagtcataaattgccacaaccttttccaagtaagaacgtggagcccacggtgggtcctcttcagcataaggatcactatactcaaccacagcagcttcctcctcttcgtaatcttctggaggaggaggaggtgggggagactcatcaaagactggttcttccacaggtggcggtggaggtggtgtatctgaaatattttcttggactctggccacaaatcccattaaaggtaactgaggagttacctgtaggatggagggaggaggaggagcaagagatactggattctggctataaaaaggtcctccattcatctgattctgaaggcttgtttgtgaagtaatggaaggagggcgtctatagggcaacgagccccctattgttgggggagtatggcgagaggcaggcctattcatgctgtagaactgtacaggatgacctggaaagacactgggaggagatggagtaggaacagcaataggaacccccacactaccacttccactgttctctcgactgctgctccgactacttgggtggctccctccactactcccactgctgctgtaagttcgatttctttgattcacagaagctgtcctcacagggctctgctgcgagggagccatattacgggttgggctaggtacgtaatcatttggtaccactggaggacgcactggctccagtgtgcgatagggggagtgccgcccaagtgtccctttccctgacatagggggactagggggcttctgagttggaggtgttgtacgcggcagcccacccatcttcatgttctgggtactcacctttactccatgtccaatatcatctagaattgtatagtcaataggttttctaatataacgaactggtcgttcaaggttggctggagcaataatcttatgtgtccttgaagtgtttttattggtagtcaaaataccaatttctcttcttgcaactttctctttatgaatatcaactgtataataaaagctgccagcattacagatagcctgtgtttattattaagggttcctcataggcaaataggaaaatattgtggtctcacttgtgaaatatgattgattgaagattccatccttcgtagctgggatgcctggatatccagcatctgcaggacattgttggccaaggtgtttatcagataggcaacacttgctaaggattgggtggtgtaggctttggtttcttctagggctctctgcttatctgctgactgtatgtagttgttctcgcagtaatcggccacccgttccagatttgtgtagctgtcgaagagggcccggcggccccccgggatttcctcttccagcagcatctgcagctccgccatcttcacatcctcctcctcctcctcctcatacaggtcgcagagggagcggcggccgcagcgccaaggaaacccaggaccgggagaggaggagcggcggcgacggcggcggtaactcggaagg

SEQ ID NO: 11831 - RNA, 3924 nt, Homo sapiens
  source 1..3924: mol_type = other RNA
ctgaatagctgggactacaggtgtgcgccaccacgcccagctaatttttgtgtttttagtagagatggggtttcaccatgttggccaggatggtctcaatttattgacctcatgatccacccacctcggcctccgaaagtgctgggattacaggcataagccaccacacccagcctgtgggaactatttattggatttcaaaacaccctctgcctcattaatccactaagctttctcagcaaaaagctgtttaaataaataatgggaacatctaatttaaaacagtttttctaattatagaccagtacacgaagaagagcttaacttatccaagtatagtctagtttgggtccataatggagctgaaggctcagaggacattcagggccattacactgcaggaaaacaaggaataagggatgtagaaatgacctaagaaaagcacgaagtggaatgtatactggaggcaagttaatgaaagctaataaatacaaagtgctgggaaaaatctaaaagcaaaatagctattgtaacttgcaatgcattaaaaacaactttaaaaccaaaaagtcttgataaggaaactctatagtggggtctcagttaaatgctgatgatttttaatgctcagataacattaagtggaatattaacttctgcatccgacaccatctgaattttctcacacactactacacttgttcacttttcaatcaagttccactttctgaacttgttcaaaacctcatttgaaatatatccagctactgcttttcccctttcacctagcacagggcagttacctggcaaagctctattctggccaagtcactgggactgagtagaacccacgttagcagctctggacctgaacaggagctggcccaacatcacagtgaccacccacaaagagacaagccctcctggatttttttcagcatttcttatactgactacagtagtgatgattaaagttatctgccctacagactccactgaatttgaagctgtatttattgtacagatgggggaaatgtgttttattgtgtcagttatattaatttttatcaatgtgattagatacatattttggcctattaatcttattcattatattcttagtctgagatgggttttaattctgactaacagcagctacttaagagtccaatcatacaaaatcaggagagtattaccctttctacagctaagcgagtcagtaatacagcagcaactaatactggccattaataacgtccagagagcacattagcaaaccttgtactcccagtgactgtcaggagacttgaaaataactactattctcttccaaagtagaatagcgtttttctagatagtgaaggaaatgatagtcatagttggtctgaactccaagatcctactcctcaaaacagcaccgaagcaggggttcgggatgcctgctaagagcatttccacagttcaagtctcttcagaaccttagggaccttcgtgtctagcttcacacacccacctccacatatgaaccagcctaccacacttcacatctgggtacactggccattagcaacaatgcagtctcatgcagcagcacattaaaatcaaacgggtggcaatcgttcaccaccctcagagtgttgggagactttcacatttcatcatccttataatccacaaacagaaacatgaagggatgcaagtgagttcagcattcactcgtttggtgcactcaagtgctgagagaatgcagaatttacagtgtcacagaggaaaaaagccatctgaaataattgtaaaaatggttaagtgtggtatttaaatgttggttccctcctcttcatacaagtggaagaaaagaaggggctagggtacccactgggccatgaggttaaccccttagcacaggcaatgaagaacatccaatgccacagattctgcaggaggagaaatcccaagggtatacagtattcctgagaaagatcccagatttttctgaatcagtcttaatctgattttgttttggctacacagttatgctgttatacctttgacatacataaaaatggtcattttatttcaatccagacagctcagcattgtacaaatgatggcagaaagatccatttgttcagactcagcttgctttgtttttaatactggggaataaaccaaaaaaaaaagtgtaatttttatcatttgtatccttcattctactttactggagtggaatccccagggccttcagataatctgggaagacctgactattcctgtgaggcaagcacagccctgctgagctttactcagaataatgcatgatagactcaacgtaattcccaggaaaaagcccagtcactccattcataactccctcataccaaccatcgtcattcttcttgatgacataaataatggctccttcctgaaaggacagctcatcttccttgtcttttgtatagtcataaattgccacaaccttttccaagtaagaacgtggagcccacggtgggtcctcttcagcataaggatcactatactcaaccacagcagcttcctcctcttcgtaatcttctggaggaggaggaggtgggggagactcatcaaagactggttcttccacaggtggcggtggaggtggtgtatctgaaatattttcttggactctggccacaaatcccattaaaggtaactgaggagttacctgtaggatggagggaggaggaggagcaagagatactggattctggctataaaaaggtcctccattcatctgattctgaaggcttgtttgtgaagtaatggaaggagggcgtctatagggcaacgagccccctattgttgggggagtatggcgagaggcaggcctattcatgctgtagaactgtacaggatgacctggaaagacactgggaggagatggagtaggaacagcaataggaacccccacactaccacttccactgttctctcgactgctgctccgactacttgggtggctccctccactactcccactgctgctgtaagttcgatttctttgattcacagaagctgtcctcacagggctctgctgcgagggagccatattacgggttgggctaggtacgtaatcatttggtaccactggaggacgcactggctccagtgtgcgatagggggagtgccgcccaagtgtccctttccctgacatagggggactagggggcttctgagttggaggtgttgtacgcggcagcccacccatcttcatgttctgggtactcacctttactccatgtccaatatcatctagaattgtatagtcaataggttttctaatataacgaactggtcgttcaaggttggctggagcaataatcttatgtgtccttgaagtgtttttattggtagtcaaaataccaatttctcttcttgcaactttctctttatgaatatcaactgtctcattcaatctcaaactgcaattgtttccaaatttggtcacaaaagtcgactcaagatcaacgcctctaatttgcttgtgaaatatgattgattgaagattccatccttcgtagctgggatgcctggatatccagcatctgcaggacattgttggccaaggtgtttatcagataggcaacacttgctaaggattgggtggtgtaggctttggtttcttctagggctctctgcttatctgctgactgtatgtagttgttctcgcagtaatcggccacccgttccagatttgtgtagctgtcgaagagggcccggcggccccccgggatttcctcttccagcagcatctgcagctccgccatcttcacatcctcctcctcctcctcctcatacaggtcgcagagggagcggcggccgcagcgccaaggaaacccaggaccgggagaggaggagcggcggcgacggcggcggtaactcggaagg

SEQ ID NO: 11832 - RNA, 3680 nt, Homo sapiens
  source 1..3680: mol_type = other RNA
ctgaatagctgggactacaggtgtgcgccaccacgcccagctaatttttgtgtttttagtagagatggggtttcaccatgttggccaggatggtctcaatttattgacctcatgatccacccacctcggcctccgaaagtgctgggattacaggcataagccaccacacccagcctgtgggaactatttattggatttcaaaacaccctctgcctcattaatccactaagctttctcagcaaaaagctgtttaaataaataatgggaacatctaatttaaaacagtttttctaattatagaccagtacacgaagaagagcttaacttatccaagtatagtctagtttgggtccataatggagctgaaggctcagaggacattcagggccattacactgcaggaaaacaaggaataagggatgtagaaatgacctaagaaaagcacgaagtggaatgtatactggaggcaagttaatgaaagctaataaatacaaagtgctgggaaaaatctaaaagcaaaatagctattgtaacttgcaatgcattaaaaacaactttaaaaccaaaaagtcttgataaggaaactctatagtggggtctcagttaaatgctgatgatttttaatgctcagataacattaagtggaatattaacttctgcatccgacaccatctgaattttctcacacactactacacttgttcacttttcaatcaagttccactttctgaacttgttcaaaacctcatttgaaatatatccagctactgcttttcccctttcacctagcacagggcagttacctggcaaagctctattctggccaagtcactgggactgagtagaacccacgttagcagctctggacctgaacaggagctggcccaacatcacagtgaccacccacaaagagacaagccctcctggatttttttcagcatttcttatactgactacagtagtgatgattaaagttatctgccctacagactccactgaatttgaagctgtatttattgtacagatgggggaaatgtgttttattgtgtcagttatattaatttttatcaatgtgattagatacatattttggcctattaatcttattcattatattcttagtctgagatgggttttaattctgactaacagcagctacttaagagtccaatcatacaaaatcaggagagtattaccctttctacagctaagcgagtcagtaatacagcagcaactaatactggccattaataacgtccagagagcacattagcaaaccttgtactcccagtgactgtcaggagacttgaaaataactactattctcttccaaagtagaatagcgtttttctagatagtgaaggaaatgatagtcatagttggtctgaactccaagatcctactcctcaaaacagcaccgaagcaggggttcgggatgcctgctaagagcatttccacagttcaagtctcttcagaaccttagggaccttcgtgtctagcttcacacacccacctccacatatgaaccagcctaccacacttcacatctgggtacactggccattagcaacaatgcagtctcatgcagcagcacattaaaatcaaacgggtggcaatcgttcaccaccctcagagtgttgggagactttcacatttcatcatccttataatccacaaacagaaacatgaagggatgcaagtgagttcagcattcactcgtttggtgcactcaagtgctgagagaatgcagaatttacagtgtcacagaggaaaaaagccatctgaaataattgtaaaaatggttaagtgtggtatttaaatgttggttccctcctcttcatacaagtggaagaaaagaaggggctagggtacccactgggccatgaggttaaccccttagcacaggcaatgaagaacatccaatgccacagattctgcaggaggagaaatcccaagggtatacagtattcctgagaaagatcccagatttttctgaatcagtcttaatctgattttgttttggctacacagttatgctgttatacctttgacatacataaaaatggtcattttatttcaatccagacagctcagcattgtacaaatgatggcagaaagatccatttgttcagactcagcttgctttgtttttaatactggggaataaaccaaaaaaaaaagtgtaatttttatcatttgtatccttcattctactttactggagtggaatccccagggccttcagataatctgggaagacctgactattcctgtgaggcaagcacagccctgctgagctttactcagaataatgcatgatagactcaacgtaattcccaggaaaaagcccagtcactccattcataactccctcataccaaccatcgtcattcttcttgatgacataaataatggctccttcctgaaaggacagctcatcttccttgtcttttgtatagtcataaattgccacaaccttttccaagtaagaacgtggagcccacggtgggtcctcttcagcataaggatcactatactcaaccacagcagcttcctcctcttcgtaatcttctggaggaggaggaggtgggggagactcatcaaagactggttcttccacaggtggcggtggaggtggtgtatctgaaatattttcttggactctggccacaaatcccattaaaggtaactgaggagttacctgtaggatggagggaggaggaggagcaagagatactggattctggctataaaaaggtcctccattcatctgattctgaaggcttgtttgtgaagtaatggaaggagggcgtctatagggcaacgagccccctattgttgggggagtatggcgagaggcaggcctattcatgctgtagaactgtacaggatgacctggaaagacactgggaggagatggagtaggaacagcaataggaacccccacactaccacttccactgttctctcgactgctgctccgactacttgggtggctccctccactactcccactgctgctgtaagttcgatttctttgattcacagaagctgtcctcacagggctctgctgcgagggagccatattacgggttgggctaggtacgtaatcatttggtaccactggaggacgcactggctccagtgtgcgatagggggagtgccgcccaagtgtccctttccctgacatagggggactagggggcttctgagttggaggtgttgtacgcggcagcccacccatcttcatgttctgggtactcacctttactccatgtccaatatcatctagaattgtatagtcaataggttttctaatataacgaactggtcgttcaaggttggctggagcaataatcttatgtgtccttgaagtgtttttattggtagtcaaaataccaatttctcttcttgcaactttctctttatgaatatcaactgtctgtatgtagttgttctcgcagtaatcggccacccgttccagatttgtgtagctgtcgaagagggcccggcggccccccgggatttcctcttccagcagcatctgcagctccgccatcttcacatcctcctcctcctcctcctcatacaggtcgcagagggagcggcggccgcagcgccaaggaaacccaggaccgggagaggaggagcggcggcgacggcggcggtaactcggaagg

SEQ ID NO: 11833 - RNA, 3848 nt, Homo sapiens
  source 1..3848: mol_type = other RNA
ctgaatagctgggactacaggtgtgcgccaccacgcccagctaatttttgtgtttttagtagagatggggtttcaccatgttggccaggatggtctcaatttattgacctcatgatccacccacctcggcctccgaaagtgctgggattacaggcataagccaccacacccagcctgtgggaactatttattggatttcaaaacaccctctgcctcattaatccactaagctttctcagcaaaaagctgtttaaataaataatgggaacatctaatttaaaacagtttttctaattatagaccagtacacgaagaagagcttaacttatccaagtatagtctagtttgggtccataatggagctgaaggctcagaggacattcagggccattacactgcaggaaaacaaggaataagggatgtagaaatgacctaagaaaagcacgaagtggaatgtatactggaggcaagttaatgaaagctaataaatacaaagtgctgggaaaaatctaaaagcaaaatagctattgtaacttgcaatgcattaaaaacaactttaaaaccaaaaagtcttgataaggaaactctatagtggggtctcagttaaatgctgatgatttttaatgctcagataacattaagtggaatattaacttctgcatccgacaccatctgaattttctcacacactactacacttgttcacttttcaatcaagttccactttctgaacttgttcaaaacctcatttgaaatatatccagctactgcttttcccctttcacctagcacagggcagttacctggcaaagctctattctggccaagtcactgggactgagtagaacccacgttagcagctctggacctgaacaggagctggcccaacatcacagtgaccacccacaaagagacaagccctcctggatttttttcagcatttcttatactgactacagtagtgatgattaaagttatctgccctacagactccactgaatttgaagctgtatttattgtacagatgggggaaatgtgttttattgtgtcagttatattaatttttatcaatgtgattagatacatattttggcctattaatcttattcattatattcttagtctgagatgggttttaattctgactaacagcagctacttaagagtccaatcatacaaaatcaggagagtattaccctttctacagctaagcgagtcagtaatacagcagcaactaatactggccattaataacgtccagagagcacattagcaaaccttgtactcccagtgactgtcaggagacttgaaaataactactattctcttccaaagtagaatagcgtttttctagatagtgaaggaaatgatagtcatagttggtctgaactccaagatcctactcctcaaaacagcaccgaagcaggggttcgggatgcctgctaagagcatttccacagttcaagtctcttcagaaccttagggaccttcgtgtctagcttcacacacccacctccacatatgaaccagcctaccacacttcacatctgggtacactggccattagcaacaatgcagtctcatgcagcagcacattaaaatcaaacgggtggcaatcgttcaccaccctcagagtgttgggagactttcacatttcatcatccttataatccacaaacagaaacatgaagggatgcaagtgagttcagcattcactcgtttggtgcactcaagtgctgagagaatgcagaatttacagtgtcacagaggaaaaaagccatctgaaataattgtaaaaatggttaagtgtggtatttaaatgttggttccctcctcttcatacaagtggaagaaaagaaggggctagggtacccactgggccatgaggttaaccccttagcacaggcaatgaagaacatccaatgccacagattctgcaggaggagaaatcccaagggtatacagtattcctgagaaagatcccagatttttctgaatcagtcttaatctgattttgttttggctacacagttatgctgttatacctttgacatacataaaaatggtcattttatttcaatccagacagctcagcattgtacaaatgatggcagaaagatccatttgttcagactcagcttgctttgtttttaatactggggaataaaccaaaaaaaaaagtgtaatttttatcatttgtatccttcattctactttactggagtggaatccccagggccttcagataatctgggaagacctgactattcctgtgaggcaagcacagccctgctgagctttactcagaataatgcatgatagactcaacgtaattcccaggaaaaagcccagtcactccattcataactccctcataccaaccatcgtcattcttcttgatgacataaataatggctccttcctgaaaggacagctcatcttccttgtcttttgtatagtcataaattgccacaaccttttccaagtaagaacgtggagcccacggtgggtcctcttcagcataaggatcactatactcaaccacagcagcttcctcctcttcgtaatcttctggaggaggaggaggtgggggagactcatcaaagactggttcttccacaggtggcggtggaggtggtgtatctgaaatattttcttggactctggccacaaatcccattaaaggtaactgaggagttacctgtaggatggagggaggaggaggagcaagagatactggattctggctataaaaaggtcctccattcatctgattctgaaggcttgtttgtgaagtaatggaaggagggcgtctatagggcaacgagccccctattgttgggggagtatggcgagaggcaggcctattcatgctgtagaactgtacaggatgacctggaaagacactgggaggagatggagtaggaacagcaataggaacccccacactaccacttccactgttctctcgactgctgctccgactacttgggtggctccctccactactcccactgctgctgtaagttcgatttctttgattcacagaagctgtcctcacagggctctgctgcgagggagccatattacgggttgggctaggtacgtaatcatttggtaccactggaggacgcactggctccagtgtgcgatagggggagtgccgcccaagtgtccctttccctgacatagggggactagggggcttctgagttggaggtgttgtacgcggcagcccacccatcttcatgttctgggtactcacctttactccatgtccaatatcatctagaattgtatagtcaataggttttctaatataacgaactggtcgttcaaggttggctggagcaataatcttatgtgtccttgaagtgtttttattggtagtcaaaataccaatttctcttcttgcaactttctctttatgaatatcaactgtttgtgaaatatgattgattgaagattccatccttcgtagctgggatgcctggatatccagcatctgcaggacattgttggccaaggtgtttatcagataggcaacacttgctaaggattgggtggtgtaggctttggtttcttctagggctctctgcttatctgctgactgtatgtagttgttctcgcagtaatcggccacccgttccagatttgtgtagctgtcgaagagggcccggcggccccccgggatttcctcttccagcagcatctgcagctccgccatcttcacatcctcctcctcctcctcctcatacaggtcgcagagggagcggcggccgcagcgccaaggaaacccaggaccgggagaggaggagcggcggcgacggcggcggtaactcggaagg

SEQ ID NO: 11834 - RNA, 3844 nt, Homo sapiens
  source 1..3844: mol_type = other RNA
ctgaatagctgggactacaggtgtgcgccaccacgcccagctaatttttgtgtttttagtagagatggggtttcaccatgttggccaggatggtctcaatttattgacctcatgatccacccacctcggcctccgaaagtgctgggattacaggcataagccaccacacccagcctgtgggaactatttattggatttcaaaacaccctctgcctcattaatccactaagctttctcagcaaaaagctgtttaaataaataatgggaacatctaatttaaaacagtttttctaattatagaccagtacacgaagaagagcttaacttatccaagtatagtctagtttgggtccataatggagctgaaggctcagaggacattcagggccattacactgcaggaaaacaaggaataagggatgtagaaatgacctaagaaaagcacgaagtggaatgtatactggaggcaagttaatgaaagctaataaatacaaagtgctgggaaaaatctaaaagcaaaatagctattgtaacttgcaatgcattaaaaacaactttaaaaccaaaaagtcttgataaggaaactctatagtggggtctcagttaaatgctgatgatttttaatgctcagataacattaagtggaatattaacttctgcatccgacaccatctgaattttctcacacactactacacttgttcacttttcaatcaagttccactttctgaacttgttcaaaacctcatttgaaatatatccagctactgcttttcccctttcacctagcacagggcagttacctggcaaagctctattctggccaagtcactgggactgagtagaacccacgttagcagctctggacctgaacaggagctggcccaacatcacagtgaccacccacaaagagacaagccctcctggatttttttcagcatttcttatactgactacagtagtgatgattaaagttatctgccctacagactccactgaatttgaagctgtatttattgtacagatgggggaaatgtgttttattgtgtcagttatattaatttttatcaatgtgattagatacatattttggcctattaatcttattcattatattcttagtctgagatgggttttaattctgactaacagcagctacttaagagtccaatcatacaaaatcaggagagtattaccctttctacagctaagcgagtcagtaatacagcagcaactaatactggccattaataacgtccagagagcacattagcaaaccttgtactcccagtgactgtcaggagacttgaaaataactactattctcttccaaagtagaatagcgtttttctagatagtgaaggaaatgatagtcatagttggtctgaactccaagatcctactcctcaaaacagcaccgaagcaggggttcgggatgcctgctaagagcatttccacagttcaagtctcttcagaaccttagggaccttcgtgtctagcttcacacacccacctccacatatgaaccagcctaccacacttcacatctgggtacactggccattagcaacaatgcagtctcatgcagcagcacattaaaatcaaacgggtggcaatcgttcaccaccctcagagtgttgggagactttcacatttcatcatccttataatccacaaacagaaacatgaagggatgcaagtgagttcagcattcactcgtttggtgcactcaagtgctgagagaatgcagaatttacagtgtcacagaggaaaaaagccatctgaaataattgtaaaaatggttaagtgtggtatttaaatgttggttccctcctcttcatacaagtggaagaaaagaaggggctagggtacccactgggccatgaggttaaccccttagcacaggcaatgaagaacatccaatgccacagattctgcaggaggagaaatcccaagggtatacagtattcctgagaaagatcccagatttttctgaatcagtcttaatctgattttgttttggctacacagttatgctgttatacctttgacatacataaaaatggtcattttatttcaatccagacagctcagcattgtacaaatgatggcagaaagatccatttgttcagactcagcttgctttgtttttaatactggggaataaaccaaaaaaaaaagtgtaatttttatcatttgtatccttcattctactttactggagtggaatccccagggccttcagataatctgggaagacctgactattcctgtgaggcaagcacagccctgctgagctttactcagaataatgcatgatagactcaacgtaattcccaggaaaaagcccagtcactccattcataactccctcataccaaccatcgtcattcttcttgatgacataaataatggctccttcctgaaaggacagctcatcttccttgtcttttgtatagtcataaattgccacaaccttttccaagtaagaacgtggagcccacggtgggtcctcttcagcataaggatcactatactcaaccacagcagcttcctcctcttcgtaatcttctggaggaggaggaggtgggggagactcatcaaagactggttcttccacaggtggcggtggaggtggtgtatctgaaatattttcttggactctggccacaaatcccattaaaggtaactgaggagttacctgtaggatggagggaggaggaggagcaagagatactggattctggctataaaaaggtcctccattcatctgattctgaaggcttgtttgtgaagtaatggaaggagggcgtctatagggcaacgagccccctattgttgggggagtatggcgagaggcaggcctattcatgctgtagaactgtacaggatgacctggaaagacactgggaggagatggagtaggaacagcaataggaacccccacactaccacttccactgttctctcgactgctgctccgactacttgggtggctccctccactactcccactgctgctgtaagttcgatttctttgattcacagaagctgtcctcacagggctctgctgcgagggagccatattacgggttgggctaggtacgtaatcatttggtaccactggaggacgcactggctccagtgtgcgatagggggagtgccgcccaagtgtccctttccctgacatagggggactagggggcttctgagttggaggtgttgtacgcggcagcccacccatcttcatgttctgggtactcacctttactccatgtccaatatcatctagaattgtatagtcaataggttttctaatataacgaactggtcgttcaaggttggctggagcaataatcttatgtgtccttgaagtgtttttattggtagtcaaaataccaatttctcttcttgcaactttctctttatgaatatcaactgtttgtgaaatatgattgattgaagattccatccttcgtagctgggatgcctggatatccagcatctgcaggacattgttggccaaggtgtttatcagataggcaacacttgctaaggattgggtggtgtaggctttggtttcttctagggctctctgcttatctgctgtatgtagttgttctcgcagtaatcggccacccgttccagatttgtgtagctgtcgaagagggcccggcggccccccgggatttcctcttccagcagcatctgcagctccgccatcttcacatcctcctcctcctcctcctcatacaggtcgcagagggagcggcggccgcagcgccaaggaaacccaggaccgggagaggaggagcggcggcgacggcggcggtaactcggaagg

SEQ ID NO: 11835 - RNA, 3939 nt, Homo sapiens
  source 1..3939: mol_type = other RNA
ctgaatagctgggactacaggtgtgcgccaccacgcccagctaatttttgtgtttttagtagagatggggtttcaccatgttggccaggatggtctcaatttattgacctcatgatccacccacctcggcctccgaaagtgctgggattacaggcataagccaccacacccagcctgtgggaactatttattggatttcaaaacaccctctgcctcattaatccactaagctttctcagcaaaaagctgtttaaataaataatgggaacatctaatttaaaacagtttttctaattatagaccagtacacgaagaagagcttaacttatccaagtatagtctagtttgggtccataatggagctgaaggctcagaggacattcagggccattacactgcaggaaaacaaggaataagggatgtagaaatgacctaagaaaagcacgaagtggaatgtatactggaggcaagttaatgaaagctaataaatacaaagtgctgggaaaaatctaaaagcaaaatagctattgtaacttgcaatgcattaaaaacaactttaaaaccaaaaagtcttgataaggaaactctatagtggggtctcagttaaatgctgatgatttttaatgctcagataacattaagtggaatattaacttctgcatccgacaccatctgaattttctcacacactactacacttgttcacttttcaatcaagttccactttctgaacttgttcaaaacctcatttgaaatatatccagctactgcttttcccctttcacctagcacagggcagttacctggcaaagctctattctggccaagtcactgggactgagtagaacccacgttagcagctctggacctgaacaggagctggcccaacatcacagtgaccacccacaaagagacaagccctcctggatttttttcagcatttcttatactgactacagtagtgatgattaaagttatctgccctacagactccactgaatttgaagctgtatttattgtacagatgggggaaatgtgttttattgtgtcagttatattaatttttatcaatgtgattagatacatattttggcctattaatcttattcattatattcttagtctgagatgggttttaattctgactaacagcagctacttaagagtccaatcatacaaaatcaggagagtattaccctttctacagctaagcgagtcagtaatacagcagcaactaatactggccattaataacgtccagagagcacattagcaaaccttgtactcccagtgactgtcaggagacttgaaaataactactattctcttccaaagtagaatagcgtttttctagatagtgaaggaaatgatagtcatagttggtctgaactccaagatcctactcctcaaaacagcaccgaagcaggggttcgggatgcctgctaagagcatttccacagttcaagtctcttcagaaccttagggaccttcgtgtctagcttcacacacccacctccacatatgaaccagcctaccacacttcacatctgggtacactggccattagcaacaatgcagtctcatgcagcagcacattaaaatcaaacgggtggcaatcgttcaccaccctcagagtgttgggagactttcacatttcatcatccttataatccacaaacagaaacatgaagggatgcaagtgagttcagcattcactcgtttggtgcactcaagtgctgagagaatgcagaatttacagtgtcacagaggaaaaaagccatctgaaataattgtaaaaatggttaagtgtggtatttaaatgttggttccctcctcttcatacaagtggaagaaaagaaggggctagggtacccactgggccatgaggttaaccccttagcacaggcaatgaagaacatccaatgccacagattctgcaggaggagaaatcccaagggtatacagtattcctgagaaagatcccagatttttctgaatcagtcttaatctgattttgttttggctacacagttatgctgttatacctttgacatacataaaaatggtcattttatttcaatccagacagctcagcattgtacaaatgatggcagaaagatccatttgttcagactcagcttgctttgtttttaatactggggaataaaccaaaaaaaaaagtgtaatttttatcatttgtatccttcattctactttactggagtggaatccccagggccttcagataatctgggaagacctgactattcctgtgaggcaagcacagccctgctgagctttactcagaataatgcatgatagactcaacgtaattcccaggaaaaagcccagtcactccattcataactccctcataccaaccatcgtcattcttcttgatgacataaataatggctccttcctgaaaggacagctcatcttccttgtcttttgtatagtcataaattgccacaaccttttccaagtaagaacgtggagcccacggtgggtcctcttcagcataaggatcactatactcaaccacagcagcttcctcctcttcgtaatcttctggaggaggaggaggtgggggagactcatcaaagactggttcttccacaggtggcggtggaggtggtgtatctgaaatattttcttggactctggccacaaatcccattaaaggtaactgaggagttacctgtaggatggagggaggaggaggagcaagagatactggattctggctataaaaaggtcctccattcatctgattctgaaggcttgtttgtgaagtaatggaaggagggcgtctatagggcaacgagccccctattgttgggggagtatggcgagaggcaggcctattcatgctgtagaactgtacaggatgacctggaaagacactgggaggagatggagtaggaacagcaataggaacccccacactaccacttccactgttctctcgactgctgctccgactacttgggtggctccctccactactcccactgctgtaagttcgatttctttgattcacagaagctgtcctcacagggctctgctgcgagggagccatattacgggttgggctaggtacgtaatcatttggtaccactggaggacgcactggctccagtgtgcgatagggggagtgccgcccaagtgtccctttccctgacatagggggactagggggcttctgagttggaggtgttgtacgcggcagcccacccatcttcatgttctgggtactcaccttaaatctaagcaaccactttactccatgtccaatatcatctagaattgtatagtcaataggttttctaatataacgaactggtcgttcaaggttggctggagcaataatcttatgtgtccttgaagtgtttttattggtagtcaaaataccaatttctcttcttgcaactttctctttatgaatatcaactgtctcattcaatctcaaactgcaattgtttccaaatttggtcacaaaagtcgactcaagatcaacgcctctaatttgcttgtgaaatatgattgattgaagattccatccttcgtagctgggatgcctggatatccagcatctgcaggacattgttggccaaggtgtttatcagataggcaacacttgctaaggattgggtggtgtaggctttggtttcttctagggctctctgcttatctgctgactgtatgtagttgttctcgcagtaatcggccacccgttccagatttgtgtagctgtcgaagagggcccggcggccccccgggatttcctcttccagcagcatctgcagctccgccatcttcacatcctcctcctcctcctcctcatacaggtcgcagagggagcggcggccgcagcgccaaggaaacccaggaccgggagaggaggagcggcggcgacggcggcggtaactcggaagg

SEQ ID NO: 11836 - RNA, 3921 nt, Homo sapiens
  source 1..3921: mol_type = other RNA
ctgaatagctgggactacaggtgtgcgccaccacgcccagctaatttttgtgtttttagtagagatggggtttcaccatgttggccaggatggtctcaatttattgacctcatgatccacccacctcggcctccgaaagtgctgggattacaggcataagccaccacacccagcctgtgggaactatttattggatttcaaaacaccctctgcctcattaatccactaagctttctcagcaaaaagctgtttaaataaataatgggaacatctaatttaaaacagtttttctaattatagaccagtacacgaagaagagcttaacttatccaagtatagtctagtttgggtccataatggagctgaaggctcagaggacattcagggccattacactgcaggaaaacaaggaataagggatgtagaaatgacctaagaaaagcacgaagtggaatgtatactggaggcaagttaatgaaagctaataaatacaaagtgctgggaaaaatctaaaagcaaaatagctattgtaacttgcaatgcattaaaaacaactttaaaaccaaaaagtcttgataaggaaactctatagtggggtctcagttaaatgctgatgatttttaatgctcagataacattaagtggaatattaacttctgcatccgacaccatctgaattttctcacacactactacacttgttcacttttcaatcaagttccactttctgaacttgttcaaaacctcatttgaaatatatccagctactgcttttcccctttcacctagcacagggcagttacctggcaaagctctattctggccaagtcactgggactgagtagaacccacgttagcagctctggacctgaacaggagctggcccaacatcacagtgaccacccacaaagagacaagccctcctggatttttttcagcatttcttatactgactacagtagtgatgattaaagttatctgccctacagactccactgaatttgaagctgtatttattgtacagatgggggaaatgtgttttattgtgtcagttatattaatttttatcaatgtgattagatacatattttggcctattaatcttattcattatattcttagtctgagatgggttttaattctgactaacagcagctacttaagagtccaatcatacaaaatcaggagagtattaccctttctacagctaagcgagtcagtaatacagcagcaactaatactggccattaataacgtccagagagcacattagcaaaccttgtactcccagtgactgtcaggagacttgaaaataactactattctcttccaaagtagaatagcgtttttctagatagtgaaggaaatgatagtcatagttggtctgaactccaagatcctactcctcaaaacagcaccgaagcaggggttcgggatgcctgctaagagcatttccacagttcaagtctcttcagaaccttagggaccttcgtgtctagcttcacacacccacctccacatatgaaccagcctaccacacttcacatctgggtacactggccattagcaacaatgcagtctcatgcagcagcacattaaaatcaaacgggtggcaatcgttcaccaccctcagagtgttgggagactttcacatttcatcatccttataatccacaaacagaaacatgaagggatgcaagtgagttcagcattcactcgtttggtgcactcaagtgctgagagaatgcagaatttacagtgtcacagaggaaaaaagccatctgaaataattgtaaaaatggttaagtgtggtatttaaatgttggttccctcctcttcatacaagtggaagaaaagaaggggctagggtacccactgggccatgaggttaaccccttagcacaggcaatgaagaacatccaatgccacagattctgcaggaggagaaatcccaagggtatacagtattcctgagaaagatcccagatttttctgaatcagtcttaatctgattttgttttggctacacagttatgctgttatacctttgacatacataaaaatggtcattttatttcaatccagacagctcagcattgtacaaatgatggcagaaagatccatttgttcagactcagcttgctttgtttttaatactggggaataaaccaaaaaaaaaagtgtaatttttatcatttgtatccttcattctactttactggagtggaatccccagggccttcagataatctgggaagacctgactattcctgtgaggcaagcacagccctgctgagctttactcagaataatgcatgatagactcaacgtaattcccaggaaaaagcccagtcactccattcataactccctcataccaaccatcgtcattcttcttgatgacataaataatggctccttcctgaaaggacagctcatcttccttgtcttttgtatagtcataaattgccacaaccttttccaagtaagaacgtggagcccacggtgggtcctcttcagcataaggatcactatactcaaccacagcagcttcctcctcttcgtaatcttctggaggaggaggaggtgggggagactcatcaaagactggttcttccacaggtggcggtggaggtggtgtatctgaaatattttcttggactctggccacaaatcccattaaaggtaactgaggagttacctgtaggatggagggaggaggaggagcaagagatactggattctggctataaaaaggtcctccattcatctgattctgaaggcttgtttgtgaagtaatggaaggagggcgtctatagggcaacgagccccctattgttgggggagtatggcgagaggcaggcctattcatgctgtagaactgtacaggatgacctggaaagacactgggaggagatggagtaggaacagcaataggaacccccacactaccacttccactgttctctcgactgctgctccgactacttgggtggctccctccactactcccactgctgtaagttcgatttctttgattcacagaagctgtcctcacagggctctgctgcgagggagccatattacgggttgggctaggtacgtaatcatttggtaccactggaggacgcactggctccagtgtgcgatagggggagtgccgcccaagtgtccctttccctgacatagggggactagggggcttctgagttggaggtgttgtacgcggcagcccacccatcttcatgttctgggtactcacctttactccatgtccaatatcatctagaattgtatagtcaataggttttctaatataacgaactggtcgttcaaggttggctggagcaataatcttatgtgtccttgaagtgtttttattggtagtcaaaataccaatttctcttcttgcaactttctctttatgaatatcaactgtctcattcaatctcaaactgcaattgtttccaaatttggtcacaaaagtcgactcaagatcaacgcctctaatttgcttgtgaaatatgattgattgaagattccatccttcgtagctgggatgcctggatatccagcatctgcaggacattgttggccaaggtgtttatcagataggcaacacttgctaaggattgggtggtgtaggctttggtttcttctagggctctctgcttatctgctgactgtatgtagttgttctcgcagtaatcggccacccgttccagatttgtgtagctgtcgaagagggcccggcggccccccgggatttcctcttccagcagcatctgcagctccgccatcttcacatcctcctcctcctcctcctcatacaggtcgcagagggagcggcggccgcagcgccaaggaaacccaggaccgggagaggaggagcggcggcgacggcggcggtaactcggaagg

SEQ ID NO: 11837 - RNA, 3677 nt, Homo sapiens
  source 1..3677: mol_type = other RNA
ctgaatagctgggactacaggtgtgcgccaccacgcccagctaatttttgtgtttttagtagagatggggtttcaccatgttggccaggatggtctcaatttattgacctcatgatccacccacctcggcctccgaaagtgctgggattacaggcataagccaccacacccagcctgtgggaactatttattggatttcaaaacaccctctgcctcattaatccactaagctttctcagcaaaaagctgtttaaataaataatgggaacatctaatttaaaacagtttttctaattatagaccagtacacgaagaagagcttaacttatccaagtatagtctagtttgggtccataatggagctgaaggctcagaggacattcagggccattacactgcaggaaaacaaggaataagggatgtagaaatgacctaagaaaagcacgaagtggaatgtatactggaggcaagttaatgaaagctaataaatacaaagtgctgggaaaaatctaaaagcaaaatagctattgtaacttgcaatgcattaaaaacaactttaaaaccaaaaagtcttgataaggaaactctatagtggggtctcagttaaatgctgatgatttttaatgctcagataacattaagtggaatattaacttctgcatccgacaccatctgaattttctcacacactactacacttgttcacttttcaatcaagttccactttctgaacttgttcaaaacctcatttgaaatatatccagctactgcttttcccctttcacctagcacagggcagttacctggcaaagctctattctggccaagtcactgggactgagtagaacccacgttagcagctctggacctgaacaggagctggcccaacatcacagtgaccacccacaaagagacaagccctcctggatttttttcagcatttcttatactgactacagtagtgatgattaaagttatctgccctacagactccactgaatttgaagctgtatttattgtacagatgggggaaatgtgttttattgtgtcagttatattaatttttatcaatgtgattagatacatattttggcctattaatcttattcattatattcttagtctgagatgggttttaattctgactaacagcagctacttaagagtccaatcatacaaaatcaggagagtattaccctttctacagctaagcgagtcagtaatacagcagcaactaatactggccattaataacgtccagagagcacattagcaaaccttgtactcccagtgactgtcaggagacttgaaaataactactattctcttccaaagtagaatagcgtttttctagatagtgaaggaaatgatagtcatagttggtctgaactccaagatcctactcctcaaaacagcaccgaagcaggggttcgggatgcctgctaagagcatttccacagttcaagtctcttcagaaccttagggaccttcgtgtctagcttcacacacccacctccacatatgaaccagcctaccacacttcacatctgggtacactggccattagcaacaatgcagtctcatgcagcagcacattaaaatcaaacgggtggcaatcgttcaccaccctcagagtgttgggagactttcacatttcatcatccttataatccacaaacagaaacatgaagggatgcaagtgagttcagcattcactcgtttggtgcactcaagtgctgagagaatgcagaatttacagtgtcacagaggaaaaaagccatctgaaataattgtaaaaatggttaagtgtggtatttaaatgttggttccctcctcttcatacaagtggaagaaaagaaggggctagggtacccactgggccatgaggttaaccccttagcacaggcaatgaagaacatccaatgccacagattctgcaggaggagaaatcccaagggtatacagtattcctgagaaagatcccagatttttctgaatcagtcttaatctgattttgttttggctacacagttatgctgttatacctttgacatacataaaaatggtcattttatttcaatccagacagctcagcattgtacaaatgatggcagaaagatccatttgttcagactcagcttgctttgtttttaatactggggaataaaccaaaaaaaaaagtgtaatttttatcatttgtatccttcattctactttactggagtggaatccccagggccttcagataatctgggaagacctgactattcctgtgaggcaagcacagccctgctgagctttactcagaataatgcatgatagactcaacgtaattcccaggaaaaagcccagtcactccattcataactccctcataccaaccatcgtcattcttcttgatgacataaataatggctccttcctgaaaggacagctcatcttccttgtcttttgtatagtcataaattgccacaaccttttccaagtaagaacgtggagcccacggtgggtcctcttcagcataaggatcactatactcaaccacagcagcttcctcctcttcgtaatcttctggaggaggaggaggtgggggagactcatcaaagactggttcttccacaggtggcggtggaggtggtgtatctgaaatattttcttggactctggccacaaatcccattaaaggtaactgaggagttacctgtaggatggagggaggaggaggagcaagagatactggattctggctataaaaaggtcctccattcatctgattctgaaggcttgtttgtgaagtaatggaaggagggcgtctatagggcaacgagccccctattgttgggggagtatggcgagaggcaggcctattcatgctgtagaactgtacaggatgacctggaaagacactgggaggagatggagtaggaacagcaataggaacccccacactaccacttccactgttctctcgactgctgctccgactacttgggtggctccctccactactcccactgctgtaagttcgatttctttgattcacagaagctgtcctcacagggctctgctgcgagggagccatattacgggttgggctaggtacgtaatcatttggtaccactggaggacgcactggctccagtgtgcgatagggggagtgccgcccaagtgtccctttccctgacatagggggactagggggcttctgagttggaggtgttgtacgcggcagcccacccatcttcatgttctgggtactcacctttactccatgtccaatatcatctagaattgtatagtcaataggttttctaatataacgaactggtcgttcaaggttggctggagcaataatcttatgtgtccttgaagtgtttttattggtagtcaaaataccaatttctcttcttgcaactttctctttatgaatatcaactgtctgtatgtagttgttctcgcagtaatcggccacccgttccagatttgtgtagctgtcgaagagggcccggcggccccccgggatttcctcttccagcagcatctgcagctccgccatcttcacatcctcctcctcctcctcctcatacaggtcgcagagggagcggcggccgcagcgccaaggaaacccaggaccgggagaggaggagcggcggcgacggcggcggtaactcggaagg

SEQ ID NO: 11838 - RNA, 3845 nt, Homo sapiens
  source 1..3845: mol_type = other RNA
ctgaatagctgggactacaggtgtgcgccaccacgcccagctaatttttgtgtttttagtagagatggggtttcaccatgttggccaggatggtctcaatttattgacctcatgatccacccacctcggcctccgaaagtgctgggattacaggcataagccaccacacccagcctgtgggaactatttattggatttcaaaacaccctctgcctcattaatccactaagctttctcagcaaaaagctgtttaaataaataatgggaacatctaatttaaaacagtttttctaattatagaccagtacacgaagaagagcttaacttatccaagtatagtctagtttgggtccataatggagctgaaggctcagaggacattcagggccattacactgcaggaaaacaaggaataagggatgtagaaatgacctaagaaaagcacgaagtggaatgtatactggaggcaagttaatgaaagctaataaatacaaagtgctgggaaaaatctaaaagcaaaatagctattgtaacttgcaatgcattaaaaacaactttaaaaccaaaaagtcttgataaggaaactctatagtggggtctcagttaaatgctgatgatttttaatgctcagataacattaagtggaatattaacttctgcatccgacaccatctgaattttctcacacactactacacttgttcacttttcaatcaagttccactttctgaacttgttcaaaacctcatttgaaatatatccagctactgcttttcccctttcacctagcacagggcagttacctggcaaagctctattctggccaagtcactgggactgagtagaacccacgttagcagctctggacctgaacaggagctggcccaacatcacagtgaccacccacaaagagacaagccctcctggatttttttcagcatttcttatactgactacagtagtgatgattaaagttatctgccctacagactccactgaatttgaagctgtatttattgtacagatgggggaaatgtgttttattgtgtcagttatattaatttttatcaatgtgattagatacatattttggcctattaatcttattcattatattcttagtctgagatgggttttaattctgactaacagcagctacttaagagtccaatcatacaaaatcaggagagtattaccctttctacagctaagcgagtcagtaatacagcagcaactaatactggccattaataacgtccagagagcacattagcaaaccttgtactcccagtgactgtcaggagacttgaaaataactactattctcttccaaagtagaatagcgtttttctagatagtgaaggaaatgatagtcatagttggtctgaactccaagatcctactcctcaaaacagcaccgaagcaggggttcgggatgcctgctaagagcatttccacagttcaagtctcttcagaaccttagggaccttcgtgtctagcttcacacacccacctccacatatgaaccagcctaccacacttcacatctgggtacactggccattagcaacaatgcagtctcatgcagcagcacattaaaatcaaacgggtggcaatcgttcaccaccctcagagtgttgggagactttcacatttcatcatccttataatccacaaacagaaacatgaagggatgcaagtgagttcagcattcactcgtttggtgcactcaagtgctgagagaatgcagaatttacagtgtcacagaggaaaaaagccatctgaaataattgtaaaaatggttaagtgtggtatttaaatgttggttccctcctcttcatacaagtggaagaaaagaaggggctagggtacccactgggccatgaggttaaccccttagcacaggcaatgaagaacatccaatgccacagattctgcaggaggagaaatcccaagggtatacagtattcctgagaaagatcccagatttttctgaatcagtcttaatctgattttgttttggctacacagttatgctgttatacctttgacatacataaaaatggtcattttatttcaatccagacagctcagcattgtacaaatgatggcagaaagatccatttgttcagactcagcttgctttgtttttaatactggggaataaaccaaaaaaaaaagtgtaatttttatcatttgtatccttcattctactttactggagtggaatccccagggccttcagataatctgggaagacctgactattcctgtgaggcaagcacagccctgctgagctttactcagaataatgcatgatagactcaacgtaattcccaggaaaaagcccagtcactccattcataactccctcataccaaccatcgtcattcttcttgatgacataaataatggctccttcctgaaaggacagctcatcttccttgtcttttgtatagtcataaattgccacaaccttttccaagtaagaacgtggagcccacggtgggtcctcttcagcataaggatcactatactcaaccacagcagcttcctcctcttcgtaatcttctggaggaggaggaggtgggggagactcatcaaagactggttcttccacaggtggcggtggaggtggtgtatctgaaatattttcttggactctggccacaaatcccattaaaggtaactgaggagttacctgtaggatggagggaggaggaggagcaagagatactggattctggctataaaaaggtcctccattcatctgattctgaaggcttgtttgtgaagtaatggaaggagggcgtctatagggcaacgagccccctattgttgggggagtatggcgagaggcaggcctattcatgctgtagaactgtacaggatgacctggaaagacactgggaggagatggagtaggaacagcaataggaacccccacactaccacttccactgttctctcgactgctgctccgactacttgggtggctccctccactactcccactgctgtaagttcgatttctttgattcacagaagctgtcctcacagggctctgctgcgagggagccatattacgggttgggctaggtacgtaatcatttggtaccactggaggacgcactggctccagtgtgcgatagggggagtgccgcccaagtgtccctttccctgacatagggggactagggggcttctgagttggaggtgttgtacgcggcagcccacccatcttcatgttctgggtactcacctttactccatgtccaatatcatctagaattgtatagtcaataggttttctaatataacgaactggtcgttcaaggttggctggagcaataatcttatgtgtccttgaagtgtttttattggtagtcaaaataccaatttctcttcttgcaactttctctttatgaatatcaactgtttgtgaaatatgattgattgaagattccatccttcgtagctgggatgcctggatatccagcatctgcaggacattgttggccaaggtgtttatcagataggcaacacttgctaaggattgggtggtgtaggctttggtttcttctagggctctctgcttatctgctgactgtatgtagttgttctcgcagtaatcggccacccgttccagatttgtgtagctgtcgaagagggcccggcggccccccgggatttcctcttccagcagcatctgcagctccgccatcttcacatcctcctcctcctcctcctcatacaggtcgcagagggagcggcggccgcagcgccaaggaaacccaggaccgggagaggaggagcggcggcgacggcggcggtaactcggaagg

SEQ ID NO: 11839 - RNA, 3841 nt, Homo sapiens
  source 1..3841: mol_type = other RNA
ctgaatagctgggactacaggtgtgcgccaccacgcccagctaatttttgtgtttttagtagagatggggtttcaccatgttggccaggatggtctcaatttattgacctcatgatccacccacctcggcctccgaaagtgctgggattacaggcataagccaccacacccagcctgtgggaactatttattggatttcaaaacaccctctgcctcattaatccactaagctttctcagcaaaaagctgtttaaataaataatgggaacatctaatttaaaacagtttttctaattatagaccagtacacgaagaagagcttaacttatccaagtatagtctagtttgggtccataatggagctgaaggctcagaggacattcagggccattacactgcaggaaaacaaggaataagggatgtagaaatgacctaagaaaagcacgaagtggaatgtatactggaggcaagttaatgaaagctaataaatacaaagtgctgggaaaaatctaaaagcaaaatagctattgtaacttgcaatgcattaaaaacaactttaaaaccaaaaagtcttgataaggaaactctatagtggggtctcagttaaatgctgatgatttttaatgctcagataacattaagtggaatattaacttctgcatccgacaccatctgaattttctcacacactactacacttgttcacttttcaatcaagttccactttctgaacttgttcaaaacctcatttgaaatatatccagctactgcttttcccctttcacctagcacagggcagttacctggcaaagctctattctggccaagtcactgggactgagtagaacccacgttagcagctctggacctgaacaggagctggcccaacatcacagtgaccacccacaaagagacaagccctcctggatttttttcagcatttcttatactgactacagtagtgatgattaaagttatctgccctacagactccactgaatttgaagctgtatttattgtacagatgggggaaatgtgttttattgtgtcagttatattaatttttatcaatgtgattagatacatattttggcctattaatcttattcattatattcttagtctgagatgggttttaattctgactaacagcagctacttaagagtccaatcatacaaaatcaggagagtattaccctttctacagctaagcgagtcagtaatacagcagcaactaatactggccattaataacgtccagagagcacattagcaaaccttgtactcccagtgactgtcaggagacttgaaaataactactattctcttccaaagtagaatagcgtttttctagatagtgaaggaaatgatagtcatagttggtctgaactccaagatcctactcctcaaaacagcaccgaagcaggggttcgggatgcctgctaagagcatttccacagttcaagtctcttcagaaccttagggaccttcgtgtctagcttcacacacccacctccacatatgaaccagcctaccacacttcacatctgggtacactggccattagcaacaatgcagtctcatgcagcagcacattaaaatcaaacgggtggcaatcgttcaccaccctcagagtgttgggagactttcacatttcatcatccttataatccacaaacagaaacatgaagggatgcaagtgagttcagcattcactcgtttggtgcactcaagtgctgagagaatgcagaatttacagtgtcacagaggaaaaaagccatctgaaataattgtaaaaatggttaagtgtggtatttaaatgttggttccctcctcttcatacaagtggaagaaaagaaggggctagggtacccactgggccatgaggttaaccccttagcacaggcaatgaagaacatccaatgccacagattctgcaggaggagaaatcccaagggtatacagtattcctgagaaagatcccagatttttctgaatcagtcttaatctgattttgttttggctacacagttatgctgttatacctttgacatacataaaaatggtcattttatttcaatccagacagctcagcattgtacaaatgatggcagaaagatccatttgttcagactcagcttgctttgtttttaatactggggaataaaccaaaaaaaaaagtgtaatttttatcatttgtatccttcattctactttactggagtggaatccccagggccttcagataatctgggaagacctgactattcctgtgaggcaagcacagccctgctgagctttactcagaataatgcatgatagactcaacgtaattcccaggaaaaagcccagtcactccattcataactccctcataccaaccatcgtcattcttcttgatgacataaataatggctccttcctgaaaggacagctcatcttccttgtcttttgtatagtcataaattgccacaaccttttccaagtaagaacgtggagcccacggtgggtcctcttcagcataaggatcactatactcaaccacagcagcttcctcctcttcgtaatcttctggaggaggaggaggtgggggagactcatcaaagactggttcttccacaggtggcggtggaggtggtgtatctgaaatattttcttggactctggccacaaatcccattaaaggtaactgaggagttacctgtaggatggagggaggaggaggagcaagagatactggattctggctataaaaaggtcctccattcatctgattctgaaggcttgtttgtgaagtaatggaaggagggcgtctatagggcaacgagccccctattgttgggggagtatggcgagaggcaggcctattcatgctgtagaactgtacaggatgacctggaaagacactgggaggagatggagtaggaacagcaataggaacccccacactaccacttccactgttctctcgactgctgctccgactacttgggtggctccctccactactcccactgctgtaagttcgatttctttgattcacagaagctgtcctcacagggctctgctgcgagggagccatattacgggttgggctaggtacgtaatcatttggtaccactggaggacgcactggctccagtgtgcgatagggggagtgccgcccaagtgtccctttccctgacatagggggactagggggcttctgagttggaggtgttgtacgcggcagcccacccatcttcatgttctgggtactcacctttactccatgtccaatatcatctagaattgtatagtcaataggttttctaatataacgaactggtcgttcaaggttggctggagcaataatcttatgtgtccttgaagtgtttttattggtagtcaaaataccaatttctcttcttgcaactttctctttatgaatatcaattgtgaaatatgattgattgaagattccatccttcgtagctgggatgcctggatatccagcatctgcaggacattgttggccaaggtgtttatcagataggcaacacttgctaaggattgggtggtgtaggctttggtttcttctagggctctctgcttatctgctgactgtatgtagttgttctcgcagtaatcggccacccgttccagatttgtgtagctgtcgaagagggcccggcggccccccgggatttcctcttccagcagcatctgcagctccgccatcttcacatcctcctcctcctcctcctcatacaggtcgcagagggagcggcggccgcagcgccaaggaaacccaggaccgggagaggaggagcggcggcgacggcggcggtaactcggaagg

SEQ ID NO: 11840 - RNA, 3723 nt, Homo sapiens
  source 1..3723: mol_type = other RNA
ctgaatagctgggactacaggtgtgcgccaccacgcccagctaatttttgtgtttttagtagagatggggtttcaccatgttggccaggatggtctcaatttattgacctcatgatccacccacctcggcctccgaaagtgctgggattacaggcataagccaccacacccagcctgtgggaactatttattggatttcaaaacaccctctgcctcattaatccactaagctttctcagcaaaaagctgtttaaataaataatgggaacatctaatttaaaacagtttttctaattatagaccagtacacgaagaagagcttaacttatccaagtatagtctagtttgggtccataatggagctgaaggctcagaggacattcagggccattacactgcaggaaaacaaggaataagggatgtagaaatgacctaagaaaagcacgaagtggaatgtatactggaggcaagttaatgaaagctaataaatacaaagtgctgggaaaaatctaaaagcaaaatagctattgtaacttgcaatgcattaaaaacaactttaaaaccaaaaagtcttgataaggaaactctatagtggggtctcagttaaatgctgatgatttttaatgctcagataacattaagtggaatattaacttctgcatccgacaccatctgaattttctcacacactactacacttgttcacttttcaatcaagttccactttctgaacttgttcaaaacctcatttgaaatatatccagctactgcttttcccctttcacctagcacagggcagttacctggcaaagctctattctggccaagtcactgggactgagtagaacccacgttagcagctctggacctgaacaggagctggcccaacatcacagtgaccacccacaaagagacaagccctcctggatttttttcagcatttcttatactgactacagtagtgatgattaaagttatctgccctacagactccactgaatttgaagctgtatttattgtacagatgggggaaatgtgttttattgtgtcagttatattaatttttatcaatgtgattagatacatattttggcctattaatcttattcattatattcttagtctgagatgggttttaattctgactaacagcagctacttaagagtccaatcatacaaaatcaggagagtattaccctttctacagctaagcgagtcagtaatacagcagcaactaatactggccattaataacgtccagagagcacattagcaaaccttgtactcccagtgactgtcaggagacttgaaaataactactattctcttccaaagtagaatagcgtttttctagatagtgaaggaaatgatagtcatagttggtctgaactccaagatcctactcctcaaaacagcaccgaagcaggggttcgggatgcctgctaagagcatttccacagttcaagtctcttcagaaccttagggaccttcgtgtctagcttcacacacccacctccacatatgaaccagcctaccacacttcacatctgggtacactggccattagcaacaatgcagtctcatgcagcagcacattaaaatcaaacgggtggcaatcgttcaccaccctcagagtgttgggagactttcacatttcatcatccttataatccacaaacagaaacatgaagggatgcaagtgagttcagcattcactcgtttggtgcactcaagtgctgagagaatgcagaatttacagtgtcacagaggaaaaaagccatctgaaataattgtaaaaatggttaagtgtggtatttaaatgttggttccctcctcttcatacaagtggaagaaaagaaggggctagggtacccactgggccatgaggttaaccccttagcacaggcaatgaagaacatccaatgccacagattctgcaggaggagaaatcccaagggtatacagtattcctgagaaagatcccagatttttctgaatcagtcttaatctgattttgttttggctacacagttatgctgttatacctttgacatacataaaaatggtcattttatttcaatccagacagctcagcattgtacaaatgatggcagaaagatccatttgttcagactcagcttgctttgtttttaatactggggaataaaccaaaaaaaaaagtgtaatttttatcatttgtatccttcattctactttactggagtggaatccccagggccttcagataatctgggaagacctgactattcctgtgaggcaagcacagccctgctgagctttactcagaataatgcatgatagactcaacgtaattcccaggaaaaagcccagtcactccattcataactccctcataccaaccatcgtcattcttcttgatgacataaataatggctccttcctgaaaggacagctcatcttccttgtcttttgtatagtcataaattgccacaaccttttccaagtaagaacgtggagcccacggtgggtcctcttcagcataaggatcactatactcaaccacagcagcttcctcctcttcgtaatcttctggaggaggaggaggtgggggagactcatcaaagactggttcttccacaggtggcggtggaggtggtgtatctgaaatattttcttggactctggccacaaatcccattaaaggtaactgaggagttacctgtaggatggagggaggaggaggagcaagagatactggattctggctataaaaaggtcctccattcatctgattctgaaggcttgtttgtgaagtaatggaaggagggcgtctatagggcaacgagccccctattgttgggggagtatggcgagaggcaggcctattcatgctgtagaactgtacaggatgacctgtaagttcgatttctttgattcacagaagctgtcctcacagggctctgctgcgagggagccatattacgggttgggctaggtacgtaatcatttggtaccactggaggacgcactggctccagtgtgcgatagggggagtgccgcccaagtgtccctttccctgacatagggggactagggggcttctgagttggaggtgttgtacgcggcagcccacccatcttcatgttctgggtactcacctttactccatgtccaatatcatctagaattgtatagtcaataggttttctaatataacgaactggtcgttcaaggttggctggagcaataatcttatgtgtccttgaagtgtttttattggtagtcaaaataccaatttctcttcttgcaactttctctttatgaatatcaactgtttgtgaaatatgattgattgaagattccatccttcgtagctgggatgcctggatatccagcatctgcaggacattgttggccaaggtgtttatcagataggcaacacttgctaaggattgggtggtgtaggctttggtttcttctagggctctctgcttatctgctgactgtatgtagttgttctcgcagtaatcggccacccgttccagatttgtgtagctgtcgaagagggcccggcggccccccgggatttcctcttccagcagcatctgcagctccgccatcttcacatcctcctcctcctcctcctcatacaggtcgcagagggagcggcggccgcagcgccaaggaaacccaggaccgggagaggaggagcggcggcgacggcggcggtaactcggaagg

SEQ ID NO: 11841 - RNA, 4023 nt, Homo sapiens
  source 1..4023: mol_type = other RNA
ctgaatagctgggactacaggtgtgcgccaccacgcccagctaatttttgtgtttttagtagagatggggtttcaccatgttggccaggatggtctcaatttattgacctcatgatccacccacctcggcctccgaaagtgctgggattacaggcataagccaccacacccagcctgtgggaactatttattggatttcaaaacaccctctgcctcattaatccactaagctttctcagcaaaaagctgtttaaataaataatgggaacatctaatttaaaacagtttttctaattatagaccagtacacgaagaagagcttaacttatccaagtatagtctagtttgggtccataatggagctgaaggctcagaggacattcagggccattacactgcaggaaaacaaggaataagggatgtagaaatgacctaagaaaagcacgaagtggaatgtatactggaggcaagttaatgaaagctaataaatacaaagtgctgggaaaaatctaaaagcaaaatagctattgtaacttgcaatgcattaaaaacaactttaaaaccaaaaagtcttgataaggaaactctatagtggggtctcagttaaatgctgatgatttttaatgctcagataacattaagtggaatattaacttctgcatccgacaccatctgaattttctcacacactactacacttgttcacttttcaatcaagttccactttctgaacttgttcaaaacctcatttgaaatatatccagctactgcttttcccctttcacctagcacagggcagttacctggcaaagctctattctggccaagtcactgggactgagtagaacccacgttagcagctctggacctgaacaggagctggcccaacatcacagtgaccacccacaaagagacaagccctcctggatttttttcagcatttcttatactgactacagtagtgatgattaaagttatctgccctacagactccactgaatttgaagctgtatttattgtacagatgggggaaatgtgttttattgtgtcagttatattaatttttatcaatgtgattagatacatattttggcctattaatcttattcattatattcttagtctgagatgggttttaattctgactaacagcagctacttaagagtccaatcatacaaaatcaggagagtattaccctttctacagctaagcgagtcagtaatacagcagcaactaatactggccattaataacgtccagagagcacattagcaaaccttgtactcccagtgactgtcaggagacttgaaaataactactattctcttccaaagtagaatagcgtttttctagatagtgaaggaaatgatagtcatagttggtctgaactccaagatcctactcctcaaaacagcaccgaagcaggggttcgggatgcctgctaagagcatttccacagttcaagtctcttcagaaccttagggaccttcgtgtctagcttcacacacccacctccacatatgaaccagcctaccacacttcacatctgggtacactggccattagcaacaatgcagtctcatgcagcagcacattaaaatcaaacgggtggcaatcgttcaccaccctcagagtgttgggagactttcacatttcatcatccttataatccacaaacagaaacatgaagggatgcaagtgagttcagcattcactcgtttggtgcactcaagtgctgagagaatgcagaatttacagtgtcacagaggaaaaaagccatctgaaataattgtaaaaatggttaagtgtggtatttaaatgttggttccctcctcttcatacaagtggaagaaaagaaggggctagggtacccactgggccatgaggttaaccccttagcacaggcaatgaagaacatccaatgccacagattctgcaggaggagaaatcccaagggtatacagtattcctgagaaagatcccagatttttctgaatcagtcttaatctgattttgttttggctacacagttatgctgttatacctttgacatacataaaaatggtcattttatttcaatccagacagctcagcattgtacaaatgatggcagaaagatccatttgttcagactcagcttgctttgtttttaatactggggaataaaccaaaaaaaaaagtgtaatttttatcatttgtatccttcattctactttactggagtggaatccccagggccttcagataatctgggaagacctgactattcctgtgaggcaagcacagccctgctgagctttactcagaataatgcatgatagactcaacgtaattcccaggaaaaagcccagtcactccattcataactccctcataccaaccatcgtcattcttcttgatgacataaataatggctccttcctgaaaggacagctcatcttccttgtcttttgtatagtcataaattgccacaaccttttccaagtaagaacgtggagcccacggtgggtcctcttcagcataaggatcactatactcaaccacagcagcttcctcctcttcgtaatcttctggaggaggaggaggtgggggagactcatcaaagactggttcttccacaggtggcggtggaggtggtgtatctgaaatattttcttggactctggccacaaatcccattaaaggtaactgaggagttacctgtaggatggagggaggaggaggagcaagagatactggattctggctataaaaaggtcctccattcatctgattctgaaggcttgtttgtgaagtaatggaaggagggcgtctatagggcaacgagccccctattgttgggggagtatggcgagaggcaggcctattcatgctgtagaactgtacaggatgacctgtagggggagtggaagaaacaacagggggagttggagaagtgaagccatcagcaagggtctgggcacccccagcagcagcgtctggggcagtggaggaagggacagtagcaggaacaagaggagcaggggcagatgcagaagtagcaggaaggggaggagtgccagcagagccagcaggggctggaaagacactgggaggagatggagtaggaacagcaataggaacccccacactaccacttccactgttctctcgactgctgctccgactacttgggtggctccctccactactcccactgccaagtgtccctttccctgacatagggggactagggggcttctgagttggaggtgttgtacgcggcagcccacccatcttcatgttctgggtactcaccttaaatctaagcaaccactttactccatgtccaatatcatctagaattgtatagtcaataggttttctaatataacgaactggtcgttcaaggttggctggagcaataatcttatgtgtccttgaagtgtttttattggtagtcaaaataccaatttctcttcttgcaactttctctttatgaatatcaactgtttgtgaaatatgattgattgaagattccatccttcgtagctgggatgcctggatatccagcatctgcaggacattgttggccaaggtgtttatcagataggcaacacttgctaaggattgggtggtgtaggctttggtttcttctagggctctctgcttatctgctgactgtagtcccagactactgagagactgaggcaggatgatcacttgagcacaggagttcaaggctgcagtgagctatgatcacaccactgcattccagcctgcatgacataccaagaccccatctctgtatgtagttgttctcgcagtaatcggccacccgttccagatttgtgtagctgtcgaagagggcccggcggccccccgggatttcctcttccagcagcatctgcagctccgccatcttcacatcctcctcctcctcctcctcatacaggtcgcagagggagcggcggccgcagcgccaaggaaacccaggaccgggagaggaggagcggcggcgacggcggcggtaactcggaagg

SEQ ID NO: 11842 - RNA, 3899 nt, Homo sapiens
  source 1..3899: mol_type = other RNA
ctgaatagctgggactacaggtgtgcgccaccacgcccagctaatttttgtgtttttagtagagatggggtttcaccatgttggccaggatggtctcaatttattgacctcatgatccacccacctcggcctccgaaagtgctgggattacaggcataagccaccacacccagcctgtgggaactatttattggatttcaaaacaccctctgcctcattaatccactaagctttctcagcaaaaagctgtttaaataaataatgggaacatctaatttaaaacagtttttctaattatagaccagtacacgaagaagagcttaacttatccaagtatagtctagtttgggtccataatggagctgaaggctcagaggacattcagggccattacactgcaggaaaacaaggaataagggatgtagaaatgacctaagaaaagcacgaagtggaatgtatactggaggcaagttaatgaaagctaataaatacaaagtgctgggaaaaatctaaaagcaaaatagctattgtaacttgcaatgcattaaaaacaactttaaaaccaaaaagtcttgataaggaaactctatagtggggtctcagttaaatgctgatgatttttaatgctcagataacattaagtggaatattaacttctgcatccgacaccatctgaattttctcacacactactacacttgttcacttttcaatcaagttccactttctgaacttgttcaaaacctcatttgaaatatatccagctactgcttttcccctttcacctagcacagggcagttacctggcaaagctctattctggccaagtcactgggactgagtagaacccacgttagcagctctggacctgaacaggagctggcccaacatcacagtgaccacccacaaagagacaagccctcctggatttttttcagcatttcttatactgactacagtagtgatgattaaagttatctgccctacagactccactgaatttgaagctgtatttattgtacagatgggggaaatgtgttttattgtgtcagttatattaatttttatcaatgtgattagatacatattttggcctattaatcttattcattatattcttagtctgagatgggttttaattctgactaacagcagctacttaagagtccaatcatacaaaatcaggagagtattaccctttctacagctaagcgagtcagtaatacagcagcaactaatactggccattaataacgtccagagagcacattagcaaaccttgtactcccagtgactgtcaggagacttgaaaataactactattctcttccaaagtagaatagcgtttttctagatagtgaaggaaatgatagtcatagttggtctgaactccaagatcctactcctcaaaacagcaccgaagcaggggttcgggatgcctgctaagagcatttccacagttcaagtctcttcagaaccttagggaccttcgtgtctagcttcacacacccacctccacatatgaaccagcctaccacacttcacatctgggtacactggccattagcaacaatgcagtctcatgcagcagcacattaaaatcaaacgggtggcaatcgttcaccaccctcagagtgttgggagactttcacatttcatcatccttataatccacaaacagaaacatgaagggatgcaagtgagttcagcattcactcgtttggtgcactcaagtgctgagagaatgcagaatttacagtgtcacagaggaaaaaagccatctgaaataattgtaaaaatggttaagtgtggtatttaaatgttggttccctcctcttcatacaagtggaagaaaagaaggggctagggtacccactgggccatgaggttaaccccttagcacaggcaatgaagaacatccaatgccacagattctgcaggaggagaaatcccaagggtatacagtattcctgagaaagatcccagatttttctgaatcagtcttaatctgattttgttttggctacacagttatgctgttatacctttgacatacataaaaatggtcattttatttcaatccagacagctcagcattgtacaaatgatggcagaaagatccatttgttcagactcagcttgctttgtttttaatactggggaataaaccaaaaaaaaaagtgtaatttttatcatttgtatccttcattctactttactggagtggaatccccagggccttcagataatctgggaagacctgactattcctgtgaggcaagcacagccctgctgagctttactcagaataatgcatgatagactcaacgtaattcccaggaaaaagcccagtcactccattcataactccctcataccaaccatcgtcattcttcttgatgacataaataatggctccttcctgaaaggacagctcatcttccttgtcttttgtatagtcataaattgccacaaccttttccaagtaagaacgtggagcccacggtgggtcctcttcagcataaggatcactatactcaaccacagcagcttcctcctcttcgtaatcttctggaggaggaggaggtgggggagactcatcaaagactggttcttccacaggtggcggtggaggtggtgtatctgaaatattttcttggactctggccacaaatcccattaaaggtaactgaggagttacctgtaggatggagggaggaggaggagcaagagatactggattctggctataaaaaggtcctccattcatctgattctgaaggcttgtttgtgaagtaatggaaggagggcgtctatagggcaacgagccccctattgttgggggagtatggcgagaggcaggcctattcatgctgtagaactgtacaggatgacctgtagggggagtggaagaaacaacagggggagttggagaagtgaagccatcagcaagggtctgggcacccccagcagcagcgtctggggcagtggaggaagggacagtagcaggaacaagaggagcaggggcagatgcagaagtagcaggaaggggaggagtgccagcagagccagcaggggctggaaagacactgggaggagatggagtaggaacagcaataggaacccccacactaccacttccactgttctctcgactgctgctccgactacttgggtggctccctccactactcccactgccaagtgtccctttccctgacatagggggactagggggcttctgagttggaggtgttgtacgcggcagcccacccatcttcatgttctgggtactcaccttaaatctaagcaaccactttactccatgtccaatatcatctagaattgtatagtcaataggttttctaatataacgaactggtcgttcaaggttggctggagcaataatcttatgtgtccttgaagtgtttttattggtagtcaaaataccaatttctcttcttgcaactttctctttatgaatatcaactgtttgtgaaatatgattgattgaagattccatccttcgtagctgggatgcctggatatccagcatctgcaggacattgttggccaaggtgtttatcagataggcaacacttgctaaggattgggtggtgtaggctttggtttcttctagggctctctgcttatctgctgactgtatgtagttgttctcgcagtaatcggccacccgttccagatttgtgtagctgtcgaagagggcccggcggccccccgggatttcctcttccagcagcatctgcagctccgccatcttcacatcctcctcctcctcctcctcatacaggtcgcagagggagcggcggccgcagcgccaaggaaacccaggaccgggagaggaggagcggcggcgacggcggcggtaactcggaagg

SEQ ID NO: 11843 - RNA, 3881 nt, Homo sapiens
  source 1..3881: mol_type = other RNA
ctgaatagctgggactacaggtgtgcgccaccacgcccagctaatttttgtgtttttagtagagatggggtttcaccatgttggccaggatggtctcaatttattgacctcatgatccacccacctcggcctccgaaagtgctgggattacaggcataagccaccacacccagcctgtgggaactatttattggatttcaaaacaccctctgcctcattaatccactaagctttctcagcaaaaagctgtttaaataaataatgggaacatctaatttaaaacagtttttctaattatagaccagtacacgaagaagagcttaacttatccaagtatagtctagtttgggtccataatggagctgaaggctcagaggacattcagggccattacactgcaggaaaacaaggaataagggatgtagaaatgacctaagaaaagcacgaagtggaatgtatactggaggcaagttaatgaaagctaataaatacaaagtgctgggaaaaatctaaaagcaaaatagctattgtaacttgcaatgcattaaaaacaactttaaaaccaaaaagtcttgataaggaaactctatagtggggtctcagttaaatgctgatgatttttaatgctcagataacattaagtggaatattaacttctgcatccgacaccatctgaattttctcacacactactacacttgttcacttttcaatcaagttccactttctgaacttgttcaaaacctcatttgaaatatatccagctactgcttttcccctttcacctagcacagggcagttacctggcaaagctctattctggccaagtcactgggactgagtagaacccacgttagcagctctggacctgaacaggagctggcccaacatcacagtgaccacccacaaagagacaagccctcctggatttttttcagcatttcttatactgactacagtagtgatgattaaagttatctgccctacagactccactgaatttgaagctgtatttattgtacagatgggggaaatgtgttttattgtgtcagttatattaatttttatcaatgtgattagatacatattttggcctattaatcttattcattatattcttagtctgagatgggttttaattctgactaacagcagctacttaagagtccaatcatacaaaatcaggagagtattaccctttctacagctaagcgagtcagtaatacagcagcaactaatactggccattaataacgtccagagagcacattagcaaaccttgtactcccagtgactgtcaggagacttgaaaataactactattctcttccaaagtagaatagcgtttttctagatagtgaaggaaatgatagtcatagttggtctgaactccaagatcctactcctcaaaacagcaccgaagcaggggttcgggatgcctgctaagagcatttccacagttcaagtctcttcagaaccttagggaccttcgtgtctagcttcacacacccacctccacatatgaaccagcctaccacacttcacatctgggtacactggccattagcaacaatgcagtctcatgcagcagcacattaaaatcaaacgggtggcaatcgttcaccaccctcagagtgttgggagactttcacatttcatcatccttataatccacaaacagaaacatgaagggatgcaagtgagttcagcattcactcgtttggtgcactcaagtgctgagagaatgcagaatttacagtgtcacagaggaaaaaagccatctgaaataattgtaaaaatggttaagtgtggtatttaaatgttggttccctcctcttcatacaagtggaagaaaagaaggggctagggtacccactgggccatgaggttaaccccttagcacaggcaatgaagaacatccaatgccacagattctgcaggaggagaaatcccaagggtatacagtattcctgagaaagatcccagatttttctgaatcagtcttaatctgattttgttttggctacacagttatgctgttatacctttgacatacataaaaatggtcattttatttcaatccagacagctcagcattgtacaaatgatggcagaaagatccatttgttcagactcagcttgctttgtttttaatactggggaataaaccaaaaaaaaaagtgtaatttttatcatttgtatccttcattctactttactggagtggaatccccagggccttcagataatctgggaagacctgactattcctgtgaggcaagcacagccctgctgagctttactcagaataatgcatgatagactcaacgtaattcccaggaaaaagcccagtcactccattcataactccctcataccaaccatcgtcattcttcttgatgacataaataatggctccttcctgaaaggacagctcatcttccttgtcttttgtatagtcataaattgccacaaccttttccaagtaagaacgtggagcccacggtgggtcctcttcagcataaggatcactatactcaaccacagcagcttcctcctcttcgtaatcttctggaggaggaggaggtgggggagactcatcaaagactggttcttccacaggtggcggtggaggtggtgtatctgaaatattttcttggactctggccacaaatcccattaaaggtaactgaggagttacctgtaggatggagggaggaggaggagcaagagatactggattctggctataaaaaggtcctccattcatctgattctgaaggcttgtttgtgaagtaatggaaggagggcgtctatagggcaacgagccccctattgttgggggagtatggcgagaggcaggcctattcatgctgtagaactgtacaggatgacctgtagggggagtggaagaaacaacagggggagttggagaagtgaagccatcagcaagggtctgggcacccccagcagcagcgtctggggcagtggaggaagggacagtagcaggaacaagaggagcaggggcagatgcagaagtagcaggaaggggaggagtgccagcagagccagcaggggctggaaagacactgggaggagatggagtaggaacagcaataggaacccccacactaccacttccactgttctctcgactgctgctccgactacttgggtggctccctccactactcccactgccaagtgtccctttccctgacatagggggactagggggcttctgagttggaggtgttgtacgcggcagcccacccatcttcatgttctgggtactcacctttactccatgtccaatatcatctagaattgtatagtcaataggttttctaatataacgaactggtcgttcaaggttggctggagcaataatcttatgtgtccttgaagtgtttttattggtagtcaaaataccaatttctcttcttgcaactttctctttatgaatatcaactgtttgtgaaatatgattgattgaagattccatccttcgtagctgggatgcctggatatccagcatctgcaggacattgttggccaaggtgtttatcagataggcaacacttgctaaggattgggtggtgtaggctttggtttcttctagggctctctgcttatctgctgactgtatgtagttgttctcgcagtaatcggccacccgttccagatttgtgtagctgtcgaagagggcccggcggccccccgggatttcctcttccagcagcatctgcagctccgccatcttcacatcctcctcctcctcctcctcatacaggtcgcagagggagcggcggccgcagcgccaaggaaacccaggaccgggagaggaggagcggcggcgacggcggcggtaactcggaagg

SEQ ID NO: 11844 - RNA, 4498 nt, Homo sapiens
  source 1..4498: mol_type = other RNA
ctgaatagctgggactacaggtgtgcgccaccacgcccagctaatttttgtgtttttagtagagatggggtttcaccatgttggccaggatggtctcaatttattgacctcatgatccacccacctcggcctccgaaagtgctgggattacaggcataagccaccacacccagcctgtgggaactatttattggatttcaaaacaccctctgcctcattaatccactaagctttctcagcaaaaagctgtttaaataaataatgggaacatctaatttaaaacagtttttctaattatagaccagtacacgaagaagagcttaacttatccaagtatagtctagtttgggtccataatggagctgaaggctcagaggacattcagggccattacactgcaggaaaacaaggaataagggatgtagaaatgacctaagaaaagcacgaagtggaatgtatactggaggcaagttaatgaaagctaataaatacaaagtgctgggaaaaatctaaaagcaaaatagctattgtaacttgcaatgcattaaaaacaactttaaaaccaaaaagtcttgataaggaaactctatagtggggtctcagttaaatgctgatgatttttaatgctcagataacattaagtggaatattaacttctgcatccgacaccatctgaattttctcacacactactacacttgttcacttttcaatcaagttccactttctgaacttgttcaaaacctcatttgaaatatatccagctactgcttttcccctttcacctagcacagggcagttacctggcaaagctctattctggccaagtcactgggactgagtagaacccacgttagcagctctggacctgaacaggagctggcccaacatcacagtgaccacccacaaagagacaagccctcctggatttttttcagcatttcttatactgactacagtagtgatgattaaagttatctgccctacagactccactgaatttgaagctgtatttattgtacagatgggggaaatgtgttttattgtgtcagttatattaatttttatcaatgtgattagatacatattttggcctattaatcttattcattatattcttagtctgagatgggttttaattctgactaacagcagctacttaagagtccaatcatacaaaatcaggagagtattaccctttctacagctaagcgagtcagtaatacagcagcaactaatactggccattaataacgtccagagagcacattagcaaaccttgtactcccagtgactgtcaggagacttgaaaataactactattctcttccaaagtagaatagcgtttttctagatagtgaaggaaatgatagtcatagttggtctgaactccaagatcctactcctcaaaacagcaccgaagcaggggttcgggatgcctgctaagagcatttccacagttcaagtctcttcagaaccttagggaccttcgtgtctagcttcacacacccacctccacatatgaaccagcctaccacacttcacatctgggtacactggccattagcaacaatgcagtctcatgcagcagcacattaaaatcaaacgggtggcaatcgttcaccaccctcagagtgttgggagactttcacatttcatcatccttataatccacaaacagaaacatgaagggatgcaagtgagttcagcattcactcgtttggtgcactcaagtgctgagagaatgcagaatttacagtgtcacagaggaaaaaagccatctgaaataattgtaaaaatggttaagtgtggtatttaaatgttggttccctcctcttcatacaagtggaagaaaagaaggggctagggtacccactgggccatgaggttaaccccttagcacaggcaatgaagaacatccaatgccacagattctgcaggaggagaaatcccaagggtatacagtattcctgagaaagatcccagatttttctgaatcagtcttaatctgattttgttttggctacacagttatgctgttatacctttgacatacataaaaatggtcattttatttcaatccagacagctcagcattgtacaaatgatggcagaaagatccatttgttcagactcagcttgctttgtttttaatactggggaataaaccaaaaaaaaaagtgtaatttttatcatttgtatccttcattctactttactggagtggaatccccagggccttcagataatctgggaagacctgactattcctgtgaggcaagcacagccctgctgagctttactcagaataatgcatgatagactcaacgtaattcccaggaaaaagcccagtcactccattcataactccctcataccaaccatcgtcattcttcttgatgacataaataatggctccttcctgaaaggacagctcatcttccttgtcttttgtatagtcataaattgccacaaccttttccaagtaagaacgtggagcccacggtgggtcctcttcagcataaggatcactatactcaaccacagcagcttcctcctcttcgtaatcttctggaggaggaggaggtgggggagactcatcaaagactggttcttccacaggtggcggtggaggtggtgtatctgaaatattttcttggactctggccacaaatcccattaaaggtaactgaggagttacctgtaggatggagggaggaggaggagcaagagatactggattctggctataaaaaggtcctccattcatctgattctgaaggcttgtttgtgaagtaatggaaggagggcgtctatagggcaacgagccccctattgttgggggagtatggcgagaggcaggcctattcatgctgtagaactgtacaggatgacctgtagggggagtggaagaaacaacagggggagttggagaagtgaagccatcagcaagggtctgggcacccccagcagcagcgtctggggcagtggaggaagggacagtagcaggaacaagaggagcaggggcagatgcagaagtagcaggaaggggaggagtgccagcagagccagcaggggctggaaagacactgggaggagatggagtaggaacagcaataggaacccccacactaccacttccactgttctctcgactgctgctccgactacttgggtggctccctccactactcccactgctgccaagtgtccctttccctgacatagggggactagggggcttctgagttggaggtgttgtacgcggcagcccacccatcttcatgttctgggtactcaccttaaatctaagcaaccactttactccatgtccaatatcatctagaattgtatagtcaataggttttctaatataacgaactggtcgttcaaggttggctggagcaataatcttatgtgtccttgaagtgtttttattggtagtcaaaataccaatttctcttcttgcaactttctctttatgaatatcaactgtctcattcaatctcaaactgcaattgtttccaaatttggtcacaaaagtcgactcaagatcaacgcctctaatttgcttgtgaaatatgattgattgaagattccatccttcgtagctgggatgcctggatatccagcatctgcaggacattgttggccaaggtgtttatcagataggcaacacttgctaaggattgggtggtgtaggctttggtttcttctagggctctctgcttatctgctgactgtatgtagttgttctcgcagtaatcggccacccgttccagatttgtgtagctgtcgaagagggcccggcggccccccgggatttcctcttccagcagcatctgcagctccgccatcttcacatcctcctcctcctcctcctcatacaggtcgcagagggagcggcggccgcagcgccaaggaaacccaggaccgggagaggaggagcggcggcgacggcggcggtaactcggaaggagcgagaaacagccccagcgcgcgacaggggagggggcgacgggggcggggcgcgagccgacggactccgaggacggtcaccgcggcgacggccggccgggcgcgcgcacgcgcgctcccttccctccgcccccgggagcccgaaaaagattcccaccctcgcccgcgccgccggcccctcccccacttccggcgtctcctagcgacggcgggggtaggggccgggatgcgcgcgggagttggtggtgcagttaacccttccgccgcccgcccgccgctggagcggctggagaagcccccacctcccggcggcctttgttagcccggcgggaacacaccaccctgctcagctggcttcctgccggctccctccgggactcatctcggctccgtccccatggaggtcatcggcctagggaacttctcgaggcttttctccctctgctgctgacgggaggccgaaggagggcacagcctccactcttgggaccctcctctgtgaaagatcacacctcaacag

SEQ ID NO: 11845 - RNA, 3734 nt, Homo sapiens
  source 1..3734: mol_type = other RNA
ctgaatagctgggactacaggtgtgcgccaccacgcccagctaatttttgtgtttttagtagagatggggtttcaccatgttggccaggatggtctcaatttattgacctcatgatccacccacctcggcctccgaaagtgctgggattacaggcataagccaccacacccagcctgtgggaactatttattggatttcaaaacaccctctgcctcattaatccactaagctttctcagcaaaaagctgtttaaataaataatgggaacatctaatttaaaacagtttttctaattatagaccagtacacgaagaagagcttaacttatccaagtatagtctagtttgggtccataatggagctgaaggctcagaggacattcagggccattacactgcaggaaaacaaggaataagggatgtagaaatgacctaagaaaagcacgaagtggaatgtatactggaggcaagttaatgaaagctaataaatacaaagtgctgggaaaaatctaaaagcaaaatagctattgtaacttgcaatgcattaaaaacaactttaaaaccaaaaagtcttgataaggaaactctatagtggggtctcagttaaatgctgatgatttttaatgctcagataacattaagtggaatattaacttctgcatccgacaccatctgaattttctcacacactactacacttgttcacttttcaatcaagttccactttctgaacttgttcaaaacctcatttgaaatatatccagctactgcttttcccctttcacctagcacagggcagttacctggcaaagctctattctggccaagtcactgggactgagtagaacccacgttagcagctctggacctgaacaggagctggcccaacatcacagtgaccacccacaaagagacaagccctcctggatttttttcagcatttcttatactgactacagtagtgatgattaaagttatctgccctacagactccactgaatttgaagctgtatttattgtacagatgggggaaatgtgttttattgtgtcagttatattaatttttatcaatgtgattagatacatattttggcctattaatcttattcattatattcttagtctgagatgggttttaattctgactaacagcagctacttaagagtccaatcatacaaaatcaggagagtattaccctttctacagctaagcgagtcagtaatacagcagcaactaatactggccattaataacgtccagagagcacattagcaaaccttgtactcccagtgactgtcaggagacttgaaaataactactattctcttccaaagtagaatagcgtttttctagatagtgaaggaaatgatagtcatagttggtctgaactccaagatcctactcctcaaaacagcaccgaagcaggggttcgggatgcctgctaagagcatttccacagttcaagtctcttcagaaccttagggaccttcgtgtctagcttcacacacccacctccacatatgaaccagcctaccacacttcacatctgggtacactggccattagcaacaatgcagtctcatgcagcagcacattaaaatcaaacgggtggcaatcgttcaccaccctcagagtgttgggagactttcacatttcatcatccttataatccacaaacagaaacatgaagggatgcaagtgagttcagcattcactcgtttggtgcactcaagtgctgagagaatgcagaatttacagtgtcacagaggaaaaaagccatctgaaataattgtaaaaatggttaagtgtggtatttaaatgttggttccctcctcttcatacaagtggaagaaaagaaggggctagggtacccactgggccatgaggttaaccccttagcacaggcaatgaagaacatccaatgccacagattctgcaggaggagaaatcccaagggtatacagtattcctgagaaagatcccagatttttctgaatcagtcttaatctgattttgttttggctacacagttatgctgttatacctttgacatacataaaaatggtcattttatttcaatccagacagctcagcattgtacaaatgatggcagaaagatccatttgttcagactcagcttgctttgtttttaatactggggaataaaccaaaaaaaaaagtgtaatttttatcatttgtatccttcattctactttactggagtggaatccccagggccttcagataatctgggaagacctgactattcctgtgaggcaagcacagccctgctgagctttactcagaataatgcatgatagactcaacgtaattcccaggaaaaagcccagtcactccattcataactccctcataccaaccatcgtcattcttcttgatgacataaataatggctccttcctgaaaggacagctcatcttccttgtcttttgtatagtcataaattgccacaaccttttccaagtaagaacgtggagcccacggtgggtcctcttcagcataaggatcactatactcaaccacagcagcttcctcctcttcgtaatcttctggaggaggaggaggtgggggagactcatcaaagactggttcttccacaggtggcggtggaggtggtgtatctgaaatattttcttggactctggccacaaatcccattaaaggtaactgaggagttacctgtaggatggagggaggaggaggagcaagagatactggattctggctataaaaaggtcctccattcatctgattctgaaggcttgtttgtgaagtaatggaaggagggcgtctatagggcaacgagccccctattgttgggggagtatggcgagaggcaggcctattcatgctgtagaactgtacaggatgacctgtagggggagtggaagaaacaacagggggagttggagaagtgaagccatcagcaagggtctgggcacccccagcagcagcgtctggggcagtggaggaagggacagtagcaggaacaagaggagcaggggcagatgcagaagtagcaggaaggggaggagtgccagcagagccagcaggggctggaaagacactgggaggagatggagtaggaacagcaataggaacccccacactaccacttccactgttctctcgactgctgctccgactacttgggtggctccctccactactcccactgctgccaagtgtccctttccctgacatagggggactagggggcttctgagttggaggtgttgtacgcggcagcccacccatcttcatgttctgggtactcaccttaaatctaagcaaccactttactccatgtccaatatcatctagaattgtatagtcaataggttttctaatataacgaactggtcgttcaaggttggctggagcaataatcttatgtgtccttgaagtgtttttattggtagtcaaaataccaatttctcttcttgcaactttctctttatgaatatcaactgtctgtatgtagttgttctcgcagtaatcggccacccgttccagatttgtgtagctgtcgaagagggcccggcggccccccgggatttcctcttccagcagcatctgcagctccgccatcttcacatcctcctcctcctcctcctcatacaggtcgcagagggagcggcggccgcagcgccaaggaaacccaggaccgggagaggaggagcggcggcgacggcggcggtaactcggaagg

SEQ ID NO: 11846 - RNA, 4026 nt, Homo sapiens
  source 1..4026: mol_type = other RNA
ctgaatagctgggactacaggtgtgcgccaccacgcccagctaatttttgtgtttttagtagagatggggtttcaccatgttggccaggatggtctcaatttattgacctcatgatccacccacctcggcctccgaaagtgctgggattacaggcataagccaccacacccagcctgtgggaactatttattggatttcaaaacaccctctgcctcattaatccactaagctttctcagcaaaaagctgtttaaataaataatgggaacatctaatttaaaacagtttttctaattatagaccagtacacgaagaagagcttaacttatccaagtatagtctagtttgggtccataatggagctgaaggctcagaggacattcagggccattacactgcaggaaaacaaggaataagggatgtagaaatgacctaagaaaagcacgaagtggaatgtatactggaggcaagttaatgaaagctaataaatacaaagtgctgggaaaaatctaaaagcaaaatagctattgtaacttgcaatgcattaaaaacaactttaaaaccaaaaagtcttgataaggaaactctatagtggggtctcagttaaatgctgatgatttttaatgctcagataacattaagtggaatattaacttctgcatccgacaccatctgaattttctcacacactactacacttgttcacttttcaatcaagttccactttctgaacttgttcaaaacctcatttgaaatatatccagctactgcttttcccctttcacctagcacagggcagttacctggcaaagctctattctggccaagtcactgggactgagtagaacccacgttagcagctctggacctgaacaggagctggcccaacatcacagtgaccacccacaaagagacaagccctcctggatttttttcagcatttcttatactgactacagtagtgatgattaaagttatctgccctacagactccactgaatttgaagctgtatttattgtacagatgggggaaatgtgttttattgtgtcagttatattaatttttatcaatgtgattagatacatattttggcctattaatcttattcattatattcttagtctgagatgggttttaattctgactaacagcagctacttaagagtccaatcatacaaaatcaggagagtattaccctttctacagctaagcgagtcagtaatacagcagcaactaatactggccattaataacgtccagagagcacattagcaaaccttgtactcccagtgactgtcaggagacttgaaaataactactattctcttccaaagtagaatagcgtttttctagatagtgaaggaaatgatagtcatagttggtctgaactccaagatcctactcctcaaaacagcaccgaagcaggggttcgggatgcctgctaagagcatttccacagttcaagtctcttcagaaccttagggaccttcgtgtctagcttcacacacccacctccacatatgaaccagcctaccacacttcacatctgggtacactggccattagcaacaatgcagtctcatgcagcagcacattaaaatcaaacgggtggcaatcgttcaccaccctcagagtgttgggagactttcacatttcatcatccttataatccacaaacagaaacatgaagggatgcaagtgagttcagcattcactcgtttggtgcactcaagtgctgagagaatgcagaatttacagtgtcacagaggaaaaaagccatctgaaataattgtaaaaatggttaagtgtggtatttaaatgttggttccctcctcttcatacaagtggaagaaaagaaggggctagggtacccactgggccatgaggttaaccccttagcacaggcaatgaagaacatccaatgccacagattctgcaggaggagaaatcccaagggtatacagtattcctgagaaagatcccagatttttctgaatcagtcttaatctgattttgttttggctacacagttatgctgttatacctttgacatacataaaaatggtcattttatttcaatccagacagctcagcattgtacaaatgatggcagaaagatccatttgttcagactcagcttgctttgtttttaatactggggaataaaccaaaaaaaaaagtgtaatttttatcatttgtatccttcattctactttactggagtggaatccccagggccttcagataatctgggaagacctgactattcctgtgaggcaagcacagccctgctgagctttactcagaataatgcatgatagactcaacgtaattcccaggaaaaagcccagtcactccattcataactccctcataccaaccatcgtcattcttcttgatgacataaataatggctccttcctgaaaggacagctcatcttccttgtcttttgtatagtcataaattgccacaaccttttccaagtaagaacgtggagcccacggtgggtcctcttcagcataaggatcactatactcaaccacagcagcttcctcctcttcgtaatcttctggaggaggaggaggtgggggagactcatcaaagactggttcttccacaggtggcggtggaggtggtgtatctgaaatattttcttggactctggccacaaatcccattaaaggtaactgaggagttacctgtaggatggagggaggaggaggagcaagagatactggattctggctataaaaaggtcctccattcatctgattctgaaggcttgtttgtgaagtaatggaaggagggcgtctatagggcaacgagccccctattgttgggggagtatggcgagaggcaggcctattcatgctgtagaactgtacaggatgacctgtagggggagtggaagaaacaacagggggagttggagaagtgaagccatcagcaagggtctgggcacccccagcagcagcgtctggggcagtggaggaagggacagtagcaggaacaagaggagcaggggcagatgcagaagtagcaggaaggggaggagtgccagcagagccagcaggggctggaaagacactgggaggagatggagtaggaacagcaataggaacccccacactaccacttccactgttctctcgactgctgctccgactacttgggtggctccctccactactcccactgctgccaagtgtccctttccctgacatagggggactagggggcttctgagttggaggtgttgtacgcggcagcccacccatcttcatgttctgggtactcaccttaaatctaagcaaccactttactccatgtccaatatcatctagaattgtatagtcaataggttttctaatataacgaactggtcgttcaaggttggctggagcaataatcttatgtgtccttgaagtgtttttattggtagtcaaaataccaatttctcttcttgcaactttctctttatgaatatcaactgtttgtgaaatatgattgattgaagattccatccttcgtagctgggatgcctggatatccagcatctgcaggacattgttggccaaggtgtttatcagataggcaacacttgctaaggattgggtggtgtaggctttggtttcttctagggctctctgcttatctgctgactgtagtcccagactactgagagactgaggcaggatgatcacttgagcacaggagttcaaggctgcagtgagctatgatcacaccactgcattccagcctgcatgacataccaagaccccatctctgtatgtagttgttctcgcagtaatcggccacccgttccagatttgtgtagctgtcgaagagggcccggcggccccccgggatttcctcttccagcagcatctgcagctccgccatcttcacatcctcctcctcctcctcctcatacaggtcgcagagggagcggcggccgcagcgccaaggaaacccaggaccgggagaggaggagcggcggcgacggcggcggtaactcggaagg

SEQ ID NO: 11847 - RNA, 3902 nt, Homo sapiens
  source 1..3902: mol_type = other RNA
ctgaatagctgggactacaggtgtgcgccaccacgcccagctaatttttgtgtttttagtagagatggggtttcaccatgttggccaggatggtctcaatttattgacctcatgatccacccacctcggcctccgaaagtgctgggattacaggcataagccaccacacccagcctgtgggaactatttattggatttcaaaacaccctctgcctcattaatccactaagctttctcagcaaaaagctgtttaaataaataatgggaacatctaatttaaaacagtttttctaattatagaccagtacacgaagaagagcttaacttatccaagtatagtctagtttgggtccataatggagctgaaggctcagaggacattcagggccattacactgcaggaaaacaaggaataagggatgtagaaatgacctaagaaaagcacgaagtggaatgtatactggaggcaagttaatgaaagctaataaatacaaagtgctgggaaaaatctaaaagcaaaatagctattgtaacttgcaatgcattaaaaacaactttaaaaccaaaaagtcttgataaggaaactctatagtggggtctcagttaaatgctgatgatttttaatgctcagataacattaagtggaatattaacttctgcatccgacaccatctgaattttctcacacactactacacttgttcacttttcaatcaagttccactttctgaacttgttcaaaacctcatttgaaatatatccagctactgcttttcccctttcacctagcacagggcagttacctggcaaagctctattctggccaagtcactgggactgagtagaacccacgttagcagctctggacctgaacaggagctggcccaacatcacagtgaccacccacaaagagacaagccctcctggatttttttcagcatttcttatactgactacagtagtgatgattaaagttatctgccctacagactccactgaatttgaagctgtatttattgtacagatgggggaaatgtgttttattgtgtcagttatattaatttttatcaatgtgattagatacatattttggcctattaatcttattcattatattcttagtctgagatgggttttaattctgactaacagcagctacttaagagtccaatcatacaaaatcaggagagtattaccctttctacagctaagcgagtcagtaatacagcagcaactaatactggccattaataacgtccagagagcacattagcaaaccttgtactcccagtgactgtcaggagacttgaaaataactactattctcttccaaagtagaatagcgtttttctagatagtgaaggaaatgatagtcatagttggtctgaactccaagatcctactcctcaaaacagcaccgaagcaggggttcgggatgcctgctaagagcatttccacagttcaagtctcttcagaaccttagggaccttcgtgtctagcttcacacacccacctccacatatgaaccagcctaccacacttcacatctgggtacactggccattagcaacaatgcagtctcatgcagcagcacattaaaatcaaacgggtggcaatcgttcaccaccctcagagtgttgggagactttcacatttcatcatccttataatccacaaacagaaacatgaagggatgcaagtgagttcagcattcactcgtttggtgcactcaagtgctgagagaatgcagaatttacagtgtcacagaggaaaaaagccatctgaaataattgtaaaaatggttaagtgtggtatttaaatgttggttccctcctcttcatacaagtggaagaaaagaaggggctagggtacccactgggccatgaggttaaccccttagcacaggcaatgaagaacatccaatgccacagattctgcaggaggagaaatcccaagggtatacagtattcctgagaaagatcccagatttttctgaatcagtcttaatctgattttgttttggctacacagttatgctgttatacctttgacatacataaaaatggtcattttatttcaatccagacagctcagcattgtacaaatgatggcagaaagatccatttgttcagactcagcttgctttgtttttaatactggggaataaaccaaaaaaaaaagtgtaatttttatcatttgtatccttcattctactttactggagtggaatccccagggccttcagataatctgggaagacctgactattcctgtgaggcaagcacagccctgctgagctttactcagaataatgcatgatagactcaacgtaattcccaggaaaaagcccagtcactccattcataactccctcataccaaccatcgtcattcttcttgatgacataaataatggctccttcctgaaaggacagctcatcttccttgtcttttgtatagtcataaattgccacaaccttttccaagtaagaacgtggagcccacggtgggtcctcttcagcataaggatcactatactcaaccacagcagcttcctcctcttcgtaatcttctggaggaggaggaggtgggggagactcatcaaagactggttcttccacaggtggcggtggaggtggtgtatctgaaatattttcttggactctggccacaaatcccattaaaggtaactgaggagttacctgtaggatggagggaggaggaggagcaagagatactggattctggctataaaaaggtcctccattcatctgattctgaaggcttgtttgtgaagtaatggaaggagggcgtctatagggcaacgagccccctattgttgggggagtatggcgagaggcaggcctattcatgctgtagaactgtacaggatgacctgtagggggagtggaagaaacaacagggggagttggagaagtgaagccatcagcaagggtctgggcacccccagcagcagcgtctggggcagtggaggaagggacagtagcaggaacaagaggagcaggggcagatgcagaagtagcaggaaggggaggagtgccagcagagccagcaggggctggaaagacactgggaggagatggagtaggaacagcaataggaacccccacactaccacttccactgttctctcgactgctgctccgactacttgggtggctccctccactactcccactgctgccaagtgtccctttccctgacatagggggactagggggcttctgagttggaggtgttgtacgcggcagcccacccatcttcatgttctgggtactcaccttaaatctaagcaaccactttactccatgtccaatatcatctagaattgtatagtcaataggttttctaatataacgaactggtcgttcaaggttggctggagcaataatcttatgtgtccttgaagtgtttttattggtagtcaaaataccaatttctcttcttgcaactttctctttatgaatatcaactgtttgtgaaatatgattgattgaagattccatccttcgtagctgggatgcctggatatccagcatctgcaggacattgttggccaaggtgtttatcagataggcaacacttgctaaggattgggtggtgtaggctttggtttcttctagggctctctgcttatctgctgactgtatgtagttgttctcgcagtaatcggccacccgttccagatttgtgtagctgtcgaagagggcccggcggccccccgggatttcctcttccagcagcatctgcagctccgccatcttcacatcctcctcctcctcctcctcatacaggtcgcagagggagcggcggccgcagcgccaaggaaacccaggaccgggagaggaggagcggcggcgacggcggcggtaactcggaagg

SEQ ID NO: 11848 - RNA, 3884 nt, Homo sapiens
  source 1..3884: mol_type = other RNA
ctgaatagctgggactacaggtgtgcgccaccacgcccagctaatttttgtgtttttagtagagatggggtttcaccatgttggccaggatggtctcaatttattgacctcatgatccacccacctcggcctccgaaagtgctgggattacaggcataagccaccacacccagcctgtgggaactatttattggatttcaaaacaccctctgcctcattaatccactaagctttctcagcaaaaagctgtttaaataaataatgggaacatctaatttaaaacagtttttctaattatagaccagtacacgaagaagagcttaacttatccaagtatagtctagtttgggtccataatggagctgaaggctcagaggacattcagggccattacactgcaggaaaacaaggaataagggatgtagaaatgacctaagaaaagcacgaagtggaatgtatactggaggcaagttaatgaaagctaataaatacaaagtgctgggaaaaatctaaaagcaaaatagctattgtaacttgcaatgcattaaaaacaactttaaaaccaaaaagtcttgataaggaaactctatagtggggtctcagttaaatgctgatgatttttaatgctcagataacattaagtggaatattaacttctgcatccgacaccatctgaattttctcacacactactacacttgttcacttttcaatcaagttccactttctgaacttgttcaaaacctcatttgaaatatatccagctactgcttttcccctttcacctagcacagggcagttacctggcaaagctctattctggccaagtcactgggactgagtagaacccacgttagcagctctggacctgaacaggagctggcccaacatcacagtgaccacccacaaagagacaagccctcctggatttttttcagcatttcttatactgactacagtagtgatgattaaagttatctgccctacagactccactgaatttgaagctgtatttattgtacagatgggggaaatgtgttttattgtgtcagttatattaatttttatcaatgtgattagatacatattttggcctattaatcttattcattatattcttagtctgagatgggttttaattctgactaacagcagctacttaagagtccaatcatacaaaatcaggagagtattaccctttctacagctaagcgagtcagtaatacagcagcaactaatactggccattaataacgtccagagagcacattagcaaaccttgtactcccagtgactgtcaggagacttgaaaataactactattctcttccaaagtagaatagcgtttttctagatagtgaaggaaatgatagtcatagttggtctgaactccaagatcctactcctcaaaacagcaccgaagcaggggttcgggatgcctgctaagagcatttccacagttcaagtctcttcagaaccttagggaccttcgtgtctagcttcacacacccacctccacatatgaaccagcctaccacacttcacatctgggtacactggccattagcaacaatgcagtctcatgcagcagcacattaaaatcaaacgggtggcaatcgttcaccaccctcagagtgttgggagactttcacatttcatcatccttataatccacaaacagaaacatgaagggatgcaagtgagttcagcattcactcgtttggtgcactcaagtgctgagagaatgcagaatttacagtgtcacagaggaaaaaagccatctgaaataattgtaaaaatggttaagtgtggtatttaaatgttggttccctcctcttcatacaagtggaagaaaagaaggggctagggtacccactgggccatgaggttaaccccttagcacaggcaatgaagaacatccaatgccacagattctgcaggaggagaaatcccaagggtatacagtattcctgagaaagatcccagatttttctgaatcagtcttaatctgattttgttttggctacacagttatgctgttatacctttgacatacataaaaatggtcattttatttcaatccagacagctcagcattgtacaaatgatggcagaaagatccatttgttcagactcagcttgctttgtttttaatactggggaataaaccaaaaaaaaaagtgtaatttttatcatttgtatccttcattctactttactggagtggaatccccagggccttcagataatctgggaagacctgactattcctgtgaggcaagcacagccctgctgagctttactcagaataatgcatgatagactcaacgtaattcccaggaaaaagcccagtcactccattcataactccctcataccaaccatcgtcattcttcttgatgacataaataatggctccttcctgaaaggacagctcatcttccttgtcttttgtatagtcataaattgccacaaccttttccaagtaagaacgtggagcccacggtgggtcctcttcagcataaggatcactatactcaaccacagcagcttcctcctcttcgtaatcttctggaggaggaggaggtgggggagactcatcaaagactggttcttccacaggtggcggtggaggtggtgtatctgaaatattttcttggactctggccacaaatcccattaaaggtaactgaggagttacctgtaggatggagggaggaggaggagcaagagatactggattctggctataaaaaggtcctccattcatctgattctgaaggcttgtttgtgaagtaatggaaggagggcgtctatagggcaacgagccccctattgttgggggagtatggcgagaggcaggcctattcatgctgtagaactgtacaggatgacctgtagggggagtggaagaaacaacagggggagttggagaagtgaagccatcagcaagggtctgggcacccccagcagcagcgtctggggcagtggaggaagggacagtagcaggaacaagaggagcaggggcagatgcagaagtagcaggaaggggaggagtgccagcagagccagcaggggctggaaagacactgggaggagatggagtaggaacagcaataggaacccccacactaccacttccactgttctctcgactgctgctccgactacttgggtggctccctccactactcccactgctgccaagtgtccctttccctgacatagggggactagggggcttctgagttggaggtgttgtacgcggcagcccacccatcttcatgttctgggtactcacctttactccatgtccaatatcatctagaattgtatagtcaataggttttctaatataacgaactggtcgttcaaggttggctggagcaataatcttatgtgtccttgaagtgtttttattggtagtcaaaataccaatttctcttcttgcaactttctctttatgaatatcaactgtttgtgaaatatgattgattgaagattccatccttcgtagctgggatgcctggatatccagcatctgcaggacattgttggccaaggtgtttatcagataggcaacacttgctaaggattgggtggtgtaggctttggtttcttctagggctctctgcttatctgctgactgtatgtagttgttctcgcagtaatcggccacccgttccagatttgtgtagctgtcgaagagggcccggcggccccccgggatttcctcttccagcagcatctgcagctccgccatcttcacatcctcctcctcctcctcctcatacaggtcgcagagggagcggcggccgcagcgccaaggaaacccaggaccgggagaggaggagcggcggcgacggcggcggtaactcggaagg

SEQ ID NO: 11849 - RNA, 4041 nt, Homo sapiens
  source 1..4041: mol_type = other RNA
ctgaatagctgggactacaggtgtgcgccaccacgcccagctaatttttgtgtttttagtagagatggggtttcaccatgttggccaggatggtctcaatttattgacctcatgatccacccacctcggcctccgaaagtgctgggattacaggcataagccaccacacccagcctgtgggaactatttattggatttcaaaacaccctctgcctcattaatccactaagctttctcagcaaaaagctgtttaaataaataatgggaacatctaatttaaaacagtttttctaattatagaccagtacacgaagaagagcttaacttatccaagtatagtctagtttgggtccataatggagctgaaggctcagaggacattcagggccattacactgcaggaaaacaaggaataagggatgtagaaatgacctaagaaaagcacgaagtggaatgtatactggaggcaagttaatgaaagctaataaatacaaagtgctgggaaaaatctaaaagcaaaatagctattgtaacttgcaatgcattaaaaacaactttaaaaccaaaaagtcttgataaggaaactctatagtggggtctcagttaaatgctgatgatttttaatgctcagataacattaagtggaatattaacttctgcatccgacaccatctgaattttctcacacactactacacttgttcacttttcaatcaagttccactttctgaacttgttcaaaacctcatttgaaatatatccagctactgcttttcccctttcacctagcacagggcagttacctggcaaagctctattctggccaagtcactgggactgagtagaacccacgttagcagctctggacctgaacaggagctggcccaacatcacagtgaccacccacaaagagacaagccctcctggatttttttcagcatttcttatactgactacagtagtgatgattaaagttatctgccctacagactccactgaatttgaagctgtatttattgtacagatgggggaaatgtgttttattgtgtcagttatattaatttttatcaatgtgattagatacatattttggcctattaatcttattcattatattcttagtctgagatgggttttaattctgactaacagcagctacttaagagtccaatcatacaaaatcaggagagtattaccctttctacagctaagcgagtcagtaatacagcagcaactaatactggccattaataacgtccagagagcacattagcaaaccttgtactcccagtgactgtcaggagacttgaaaataactactattctcttccaaagtagaatagcgtttttctagatagtgaaggaaatgatagtcatagttggtctgaactccaagatcctactcctcaaaacagcaccgaagcaggggttcgggatgcctgctaagagcatttccacagttcaagtctcttcagaaccttagggaccttcgtgtctagcttcacacacccacctccacatatgaaccagcctaccacacttcacatctgggtacactggccattagcaacaatgcagtctcatgcagcagcacattaaaatcaaacgggtggcaatcgttcaccaccctcagagtgttgggagactttcacatttcatcatccttataatccacaaacagaaacatgaagggatgcaagtgagttcagcattcactcgtttggtgcactcaagtgctgagagaatgcagaatttacagtgtcacagaggaaaaaagccatctgaaataattgtaaaaatggttaagtgtggtatttaaatgttggttccctcctcttcatacaagtggaagaaaagaaggggctagggtacccactgggccatgaggttaaccccttagcacaggcaatgaagaacatccaatgccacagattctgcaggaggagaaatcccaagggtatacagtattcctgagaaagatcccagatttttctgaatcagtcttaatctgattttgttttggctacacagttatgctgttatacctttgacatacataaaaatggtcattttatttcaatccagacagctcagcattgtacaaatgatggcagaaagatccatttgttcagactcagcttgctttgtttttaatactggggaataaaccaaaaaaaaaagtgtaatttttatcatttgtatccttcattctactttactggagtggaatccccagggccttcagataatctgggaagacctgactattcctgtgaggcaagcacagccctgctgagctttactcagaataatgcatgatagactcaacgtaattcccaggaaaaagcccagtcactccattcataactccctcataccaaccatcgtcattcttcttgatgacataaataatggctccttcctgaaaggacagctcatcttccttgtcttttgtatagtcataaattgccacaaccttttccaagtaagaacgtggagcccacggtgggtcctcttcagcataaggatcactatactcaaccacagcagcttcctcctcttcgtaatcttctggaggaggaggaggtgggggagactcatcaaagactggttcttccacaggtggcggtggaggtggtgtatctgaaatattttcttggactctggccacaaatcccattaaaggtaactgaggagttacctgtaggatggagggaggaggaggagcaagagatactggattctggctataaaaaggtcctccattcatctgattctgaaggcttgtttgtgaagtaatggaaggagggcgtctatagggcaacgagccccctattgttgggggagtatggcgagaggcaggcctattcatgctgtagaactgtacaggatgacctgtagggggagtggaagaaacaacagggggagttggagaagtgaagccatcagcaagggtctgggcacccccagcagcagcgtctggggcagtggaggaagggacagtagcaggaacaagaggagcaggggcagatgcagaagtagcaggaaggggaggagtgccagcagagccagcaggggctggaaagacactgggaggagatggagtaggaacagcaataggaacccccacactaccacttccactgttctctcgactgctgctccgactacttgggtggctccctccactactcccactgctgctgtaagttcgatttctttgattcacagaagctgtcctcacagggctctgctgcgagggagccatattacgggttgggctaggtacgtaatcatttggtaccactggaggacgcactggctccagtgtgcgatagggggagtgccgcccaagtgtccctttccctgacatagggggactagggggcttctgagttggaggtgttgtacgcggcagcccacccatcttcatgttctgggtactcaccatgactgaggatttggaaccaacaatccaatcaataatacaggtgtccatatgcctgggctcttccaatcaaatctttactccatgtccaatatcatctagaattgtatagtcaataggttttctaatataacgaactggtcgttcaaggttggctggagcaataatcttatgtgtccttgaagtgtttttattggtagtcaaaataccaatttctcttcttgcaactttctctttatgaatatcaactgtttgtgaaatatgattgattgaagattccatccttcgtagctgggatgcctggatatccagcatctgcaggacattgttggccaaggtgtttatcagataggcaacacttgctaaggattgggtggtgtaggctttggtttcttctagggctctctgcttatctgctgactgtatgtagttgttctcgcagtaatcggccacccgttccagatttgtgtagctgtcgaagagggcccggcggccccccgggatttcctcttccagcagcatctgcagctccgccatcttcacatcctcctcctcctcctcctcatacaggtcgcagagggagcggcggccgc

SEQ ID NO: 11850 - RNA, 4125 nt, Homo sapiens
  source 1..4125: mol_type = other RNA
ctgaatagctgggactacaggtgtgcgccaccacgcccagctaatttttgtgtttttagtagagatggggtttcaccatgttggccaggatggtctcaatttattgacctcatgatccacccacctcggcctccgaaagtgctgggattacaggcataagccaccacacccagcctgtgggaactatttattggatttcaaaacaccctctgcctcattaatccactaagctttctcagcaaaaagctgtttaaataaataatgggaacatctaatttaaaacagtttttctaattatagaccagtacacgaagaagagcttaacttatccaagtatagtctagtttgggtccataatggagctgaaggctcagaggacattcagggccattacactgcaggaaaacaaggaataagggatgtagaaatgacctaagaaaagcacgaagtggaatgtatactggaggcaagttaatgaaagctaataaatacaaagtgctgggaaaaatctaaaagcaaaatagctattgtaacttgcaatgcattaaaaacaactttaaaaccaaaaagtcttgataaggaaactctatagtggggtctcagttaaatgctgatgatttttaatgctcagataacattaagtggaatattaacttctgcatccgacaccatctgaattttctcacacactactacacttgttcacttttcaatcaagttccactttctgaacttgttcaaaacctcatttgaaatatatccagctactgcttttcccctttcacctagcacagggcagttacctggcaaagctctattctggccaagtcactgggactgagtagaacccacgttagcagctctggacctgaacaggagctggcccaacatcacagtgaccacccacaaagagacaagccctcctggatttttttcagcatttcttatactgactacagtagtgatgattaaagttatctgccctacagactccactgaatttgaagctgtatttattgtacagatgggggaaatgtgttttattgtgtcagttatattaatttttatcaatgtgattagatacatattttggcctattaatcttattcattatattcttagtctgagatgggttttaattctgactaacagcagctacttaagagtccaatcatacaaaatcaggagagtattaccctttctacagctaagcgagtcagtaatacagcagcaactaatactggccattaataacgtccagagagcacattagcaaaccttgtactcccagtgactgtcaggagacttgaaaataactactattctcttccaaagtagaatagcgtttttctagatagtgaaggaaatgatagtcatagttggtctgaactccaagatcctactcctcaaaacagcaccgaagcaggggttcgggatgcctgctaagagcatttccacagttcaagtctcttcagaaccttagggaccttcgtgtctagcttcacacacccacctccacatatgaaccagcctaccacacttcacatctgggtacactggccattagcaacaatgcagtctcatgcagcagcacattaaaatcaaacgggtggcaatcgttcaccaccctcagagtgttgggagactttcacatttcatcatccttataatccacaaacagaaacatgaagggatgcaagtgagttcagcattcactcgtttggtgcactcaagtgctgagagaatgcagaatttacagtgtcacagaggaaaaaagccatctgaaataattgtaaaaatggttaagtgtggtatttaaatgttggttccctcctcttcatacaagtggaagaaaagaaggggctagggtacccactgggccatgaggttaaccccttagcacaggcaatgaagaacatccaatgccacagattctgcaggaggagaaatcccaagggtatacagtattcctgagaaagatcccagatttttctgaatcagtcttaatctgattttgttttggctacacagttatgctgttatacctttgacatacataaaaatggtcattttatttcaatccagacagctcagcattgtacaaatgatggcagaaagatccatttgttcagactcagcttgctttgtttttaatactggggaataaaccaaaaaaaaaagtgtaatttttatcatttgtatccttcattctactttactggagtggaatccccagggccttcagataatctgggaagacctgactattcctgtgaggcaagcacagccctgctgagctttactcagaataatgcatgatagactcaacgtaattcccaggaaaaagcccagtcactccattcataactccctcataccaaccatcgtcattcttcttgatgacataaataatggctccttcctgaaaggacagctcatcttccttgtcttttgtatagtcataaattgccacaaccttttccaagtaagaacgtggagcccacggtgggtcctcttcagcataaggatcactatactcaaccacagcagcttcctcctcttcgtaatcttctggaggaggaggaggtgggggagactcatcaaagactggttcttccacaggtggcggtggaggtggtgtatctgaaatattttcttggactctggccacaaatcccattaaaggtaactgaggagttacctgtaggatggagggaggaggaggagcaagagatactggattctggctataaaaaggtcctccattcatctgattctgaaggcttgtttgtgaagtaatggaaggagggcgtctatagggcaacgagccccctattgttgggggagtatggcgagaggcaggcctattcatgctgtagaactgtacaggatgacctgtagggggagtggaagaaacaacagggggagttggagaagtgaagccatcagcaagggtctgggcacccccagcagcagcgtctggggcagtggaggaagggacagtagcaggaacaagaggagcaggggcagatgcagaagtagcaggaaggggaggagtgccagcagagccagcaggggctggaaagacactgggaggagatggagtaggaacagcaataggaacccccacactaccacttccactgttctctcgactgctgctccgactacttgggtggctccctccactactcccactgctgctgtaagttcgatttctttgattcacagaagctgtcctcacagggctctgctgcgagggagccatattacgggttgggctaggtacgtaatcatttggtaccactggaggacgcactggctccagtgtgcgatagggggagtgccgcccaagtgtccctttccctgacatagggggactagggggcttctgagttggaggtgttgtacgcggcagcccacccatcttcatgttctgggtactcaccttaaatctaagcaaccactttactccatgtccaatatcatctagaattgtatagtcaataggttttctaatataacgaactggtcgttcaaggttggctggagcaataatcttatgtgtccttgaagtgtttttattggtagtcaaaataccaatttctcttcttgcaactttctctttatgaatatcaactgtctcattcaatctcaaactgcaattgtttccaaatttggtcacaaaagtcgactcaagatcaacgcctctaatttgcttgtgaaatatgattgattgaagattccatccttcgtagctgggatgcctggatatccagcatctgcaggacattgttggccaaggtgtttatcagataggcaacacttgctaaggattgggtggtgtaggctttggtttcttctagggctctctgcttatctgctgactgtatgtagttgttctcgcagtaatcggccacccgttccagatttgtgtagctgtcgaagagggcccggcggccccccgggatttcctcttccagcagcatctgcagctccgccatcttcacatcctcctcctcctcctcctcatacaggtcgcagagggagcggcggccgcagcgccaaggaaacccaggaccgggagaggaggagcggcggcgacggcggcggtaactcggaagg

SEQ ID NO: 11851 - RNA, 3992 nt, Homo sapiens
  source 1..3992: mol_type = other RNA
ctgaatagctgggactacaggtgtgcgccaccacgcccagctaatttttgtgtttttagtagagatggggtttcaccatgttggccaggatggtctcaatttattgacctcatgatccacccacctcggcctccgaaagtgctgggattacaggcataagccaccacacccagcctgtgggaactatttattggatttcaaaacaccctctgcctcattaatccactaagctttctcagcaaaaagctgtttaaataaataatgggaacatctaatttaaaacagtttttctaattatagaccagtacacgaagaagagcttaacttatccaagtatagtctagtttgggtccataatggagctgaaggctcagaggacattcagggccattacactgcaggaaaacaaggaataagggatgtagaaatgacctaagaaaagcacgaagtggaatgtatactggaggcaagttaatgaaagctaataaatacaaagtgctgggaaaaatctaaaagcaaaatagctattgtaacttgcaatgcattaaaaacaactttaaaaccaaaaagtcttgataaggaaactctatagtggggtctcagttaaatgctgatgatttttaatgctcagataacattaagtggaatattaacttctgcatccgacaccatctgaattttctcacacactactacacttgttcacttttcaatcaagttccactttctgaacttgttcaaaacctcatttgaaatatatccagctactgcttttcccctttcacctagcacagggcagttacctggcaaagctctattctggccaagtcactgggactgagtagaacccacgttagcagctctggacctgaacaggagctggcccaacatcacagtgaccacccacaaagagacaagccctcctggatttttttcagcatttcttatactgactacagtagtgatgattaaagttatctgccctacagactccactgaatttgaagctgtatttattgtacagatgggggaaatgtgttttattgtgtcagttatattaatttttatcaatgtgattagatacatattttggcctattaatcttattcattatattcttagtctgagatgggttttaattctgactaacagcagctacttaagagtccaatcatacaaaatcaggagagtattaccctttctacagctaagcgagtcagtaatacagcagcaactaatactggccattaataacgtccagagagcacattagcaaaccttgtactcccagtgactgtcaggagacttgaaaataactactattctcttccaaagtagaatagcgtttttctagatagtgaaggaaatgatagtcatagttggtctgaactccaagatcctactcctcaaaacagcaccgaagcaggggttcgggatgcctgctaagagcatttccacagttcaagtctcttcagaaccttagggaccttcgtgtctagcttcacacacccacctccacatatgaaccagcctaccacacttcacatctgggtacactggccattagcaacaatgcagtctcatgcagcagcacattaaaatcaaacgggtggcaatcgttcaccaccctcagagtgttgggagactttcacatttcatcatccttataatccacaaacagaaacatgaagggatgcaagtgagttcagcattcactcgtttggtgcactcaagtgctgagagaatgcagaatttacagtgtcacagaggaaaaaagccatctgaaataattgtaaaaatggttaagtgtggtatttaaatgttggttccctcctcttcatacaagtggaagaaaagaaggggctagggtacccactgggccatgaggttaaccccttagcacaggcaatgaagaacatccaatgccacagattctgcaggaggagaaatcccaagggtatacagtattcctgagaaagatcccagatttttctgaatcagtcttaatctgattttgttttggctacacagttatgctgttatacctttgacatacataaaaatggtcattttatttcaatccagacagctcagcattgtacaaatgatggcagaaagatccatttgttcagactcagcttgctttgtttttaatactggggaataaaccaaaaaaaaaagtgtaatttttatcatttgtatccttcattctactttactggagtggaatccccagggccttcagataatctgggaagacctgactattcctgtgaggcaagcacagccctgctgagctttactcagaataatgcatgatagactcaacgtaattcccaggaaaaagcccagtcactccattcataactccctcataccaaccatcgtcattcttcttgatgacataaataatggctccttcctgaaaggacagctcatcttccttgtcttttgtatagtcataaattgccacaaccttttccaagtaagaacgtggagcccacggtgggtcctcttcagcataaggatcactatactcaaccacagcagcttcctcctcttcgtaatcttctggaggaggaggaggtgggggagactcatcaaagactggttcttccacaggtggcggtggaggtggtgtatctgaaatattttcttggactctggccacaaatcccattaaaggtaactgaggagttacctgtaggatggagggaggaggaggagcaagagatactggattctggctataaaaaggtcctccattcatctgattctgaaggcttgtttgtgaagtaatggaaggagggcgtctatagggcaacgagccccctattgttgggggagtatggcgagaggcaggcctattcatgctgtagaactgtacaggatgacctgtagggggagtggaagaaacaacagggggagttggagaagtgaagccatcagcaagggtctgggcacccccagcagcagcgtctggggcagtggaggaagggacagtagcaggaacaagaggagcaggggcagatgcagaagtagcaggaaggggaggagtgccagcagagccagcaggggctggaaagacactgggaggagatggagtaggaacagcaataggaacccccacactaccacttccactgttctctcgactgctgctccgactacttgggtggctccctccactactcccactgctgctgtaagttcgatttctttgattcacagaagctgtcctcacagggctctgctgcgagggagccatattacgggttgggctaggtacgtaatcatttggtaccactggaggacgcactggctccagtgtgcgatagggggagtgccgcccaagtgtccctttccctgacatagggggactagggggcttctgagttggaggtgttgtacgcggcagcccacccatcttcatgttctgggtactcaccttaaatctaagcaaccactttactccatgtccaatatcatctagaattgtatagtcaataggttttctaatataacgaactggtcgttcaaggttggctggagcaataatcttatgtgtccttgaagtgtttttattggtagtcaaaataccaatttctcttcttgcaactttctctttatgaatatcaactgtctcattcaatctcaaactgcaattgtttccaaatttggtcacaaaagtcgactcaagatcaacgcctctaatttgcttgtgaaatatgattgattgaagattccatccttcgtagctgggatgcctggatatccagcatctgcaggacattgttggccaaggtgtttatcagataggcaacacttgctaaggattgggtggtgtaggctttggtttcttctagggctctctgcttatctgctgactttaaaaaccataacttctagcaggacagggtggctcgtgcctggagtcctacctactcaggagactgagacaggaggatcacttcagccctggagtttgagac

SEQ ID NO: 11852 - RNA, 4173 nt, Homo sapiens
  source 1..4173: mol_type = other RNA
ctgaatagctgggactacaggtgtgcgccaccacgcccagctaatttttgtgtttttagtagagatggggtttcaccatgttggccaggatggtctcaatttattgacctcatgatccacccacctcggcctccgaaagtgctgggattacaggcataagccaccacacccagcctgtgggaactatttattggatttcaaaacaccctctgcctcattaatccactaagctttctcagcaaaaagctgtttaaataaataatgggaacatctaatttaaaacagtttttctaattatagaccagtacacgaagaagagcttaacttatccaagtatagtctagtttgggtccataatggagctgaaggctcagaggacattcagggccattacactgcaggaaaacaaggaataagggatgtagaaatgacctaagaaaagcacgaagtggaatgtatactggaggcaagttaatgaaagctaataaatacaaagtgctgggaaaaatctaaaagcaaaatagctattgtaacttgcaatgcattaaaaacaactttaaaaccaaaaagtcttgataaggaaactctatagtggggtctcagttaaatgctgatgatttttaatgctcagataacattaagtggaatattaacttctgcatccgacaccatctgaattttctcacacactactacacttgttcacttttcaatcaagttccactttctgaacttgttcaaaacctcatttgaaatatatccagctactgcttttcccctttcacctagcacagggcagttacctggcaaagctctattctggccaagtcactgggactgagtagaacccacgttagcagctctggacctgaacaggagctggcccaacatcacagtgaccacccacaaagagacaagccctcctggatttttttcagcatttcttatactgactacagtagtgatgattaaagttatctgccctacagactccactgaatttgaagctgtatttattgtacagatgggggaaatgtgttttattgtgtcagttatattaatttttatcaatgtgattagatacatattttggcctattaatcttattcattatattcttagtctgagatgggttttaattctgactaacagcagctacttaagagtccaatcatacaaaatcaggagagtattaccctttctacagctaagcgagtcagtaatacagcagcaactaatactggccattaataacgtccagagagcacattagcaaaccttgtactcccagtgactgtcaggagacttgaaaataactactattctcttccaaagtagaatagcgtttttctagatagtgaaggaaatgatagtcatagttggtctgaactccaagatcctactcctcaaaacagcaccgaagcaggggttcgggatgcctgctaagagcatttccacagttcaagtctcttcagaaccttagggaccttcgtgtctagcttcacacacccacctccacatatgaaccagcctaccacacttcacatctgggtacactggccattagcaacaatgcagtctcatgcagcagcacattaaaatcaaacgggtggcaatcgttcaccaccctcagagtgttgggagactttcacatttcatcatccttataatccacaaacagaaacatgaagggatgcaagtgagttcagcattcactcgtttggtgcactcaagtgctgagagaatgcagaatttacagtgtcacagaggaaaaaagccatctgaaataattgtaaaaatggttaagtgtggtatttaaatgttggttccctcctcttcatacaagtggaagaaaagaaggggctagggtacccactgggccatgaggttaaccccttagcacaggcaatgaagaacatccaatgccacagattctgcaggaggagaaatcccaagggtatacagtattcctgagaaagatcccagatttttctgaatcagtcttaatctgattttgttttggctacacagttatgctgttatacctttgacatacataaaaatggtcattttatttcaatccagacagctcagcattgtacaaatgatggcagaaagatccatttgttcagactcagcttgctttgtttttaatactggggaataaaccaaaaaaaaaagtgtaatttttatcatttgtatccttcattctactttactggagtggaatccccagggccttcagataatctgggaagacctgactattcctgtgaggcaagcacagccctgctgagctttactcagaataatgcatgatagactcaacgtaattcccaggaaaaagcccagtcactccattcataactccctcataccaaccatcgtcattcttcttgatgacataaataatggctccttcctgaaaggacagctcatcttccttgtcttttgtatagtcataaattgccacaaccttttccaagtaagaacgtggagcccacggtgggtcctcttcagcataaggatcactatactcaaccacagcagcttcctcctcttcgtaatcttctggaggaggaggaggtgggggagactcatcaaagactggttcttccacaggtggcggtggaggtggtgtatctgaaatattttcttggactctggccacaaatcccattaaaggtaactgaggagttacctgtaggatggagggaggaggaggagcaagagatactggattctggctataaaaaggtcctccattcatctgattctgaaggcttgtttgtgaagtaatggaaggagggcgtctatagggcaacgagccccctattgttgggggagtatggcgagaggcaggcctattcatgctgtagaactgtacaggatgacctgtagggggagtggaagaaacaacagggggagttggagaagtgaagccatcagcaagggtctgggcacccccagcagcagcgtctggggcagtggaggaagggacagtagcaggaacaagaggagcaggggcagatgcagaagtagcaggaaggggaggagtgccagcagagccagcaggggctggaaagacactgggaggagatggagtaggaacagcaataggaacccccacactaccacttccactgttctctcgactgctgctccgactacttgggtggctccctccactactcccactgctgctgtaagttcgatttctttgattcacagaagctgtcctcacagggctctgctgcgagggagccatattacgggttgggctaggtacgtaatcatttggtaccactggaggacgcactggctccagtgtgcgatagggggagtgccgcccaagtgtccctttccctgacatagggggactagggggcttctgagttggaggtgttgtacgcggcagcccacccatcttcatgttctgggtactcaccttaaatctaagcaaccactttactccatgtccaatatcatctagaattgtatagtcaataggttttctaatataacgaactggtcgttcaaggttggctggagcaataatcttatgtgtccttgaagtgtttttattggtagtcaaaataccaatttctcttcttgcaactttctctttatgaatatcaactgtttgtgaaatatgattgattgaagattccatccttcgtagctgggatgcctggatatccagcatctgcaggacattgttggccaaggtgtttatcagataggcaacacttgctaaggattgggtggtgtaggctttggtttcttctagggctctctgcttatctgctgactgtagtcccagactactgagagactgaggcaggatgatcacttgagcacaggagttcaaggctgcagtgagctatgatcacaccactgcattccagcctgcatgacataccaagaccccatctctgtatgtagttgttctcgcagtaatcggccacccgttccagatttgtgtagctgtcgaagagggcccggcggccccccgggatttcctcttccagcagcatctgcagctccgccatcttcacatcctcctcctcctcctcctcatacaggtcgcagagggagcggcggccgcagcgccaaggaaacccaggaccgggagaggaggagcggcggcgacggcggcggtaactcggaagg

SEQ ID NO: 11853 - RNA, 4049 nt, Homo sapiens
  source 1..4049: mol_type = other RNA
ctgaatagctgggactacaggtgtgcgccaccacgcccagctaatttttgtgtttttagtagagatggggtttcaccatgttggccaggatggtctcaatttattgacctcatgatccacccacctcggcctccgaaagtgctgggattacaggcataagccaccacacccagcctgtgggaactatttattggatttcaaaacaccctctgcctcattaatccactaagctttctcagcaaaaagctgtttaaataaataatgggaacatctaatttaaaacagtttttctaattatagaccagtacacgaagaagagcttaacttatccaagtatagtctagtttgggtccataatggagctgaaggctcagaggacattcagggccattacactgcaggaaaacaaggaataagggatgtagaaatgacctaagaaaagcacgaagtggaatgtatactggaggcaagttaatgaaagctaataaatacaaagtgctgggaaaaatctaaaagcaaaatagctattgtaacttgcaatgcattaaaaacaactttaaaaccaaaaagtcttgataaggaaactctatagtggggtctcagttaaatgctgatgatttttaatgctcagataacattaagtggaatattaacttctgcatccgacaccatctgaattttctcacacactactacacttgttcacttttcaatcaagttccactttctgaacttgttcaaaacctcatttgaaatatatccagctactgcttttcccctttcacctagcacagggcagttacctggcaaagctctattctggccaagtcactgggactgagtagaacccacgttagcagctctggacctgaacaggagctggcccaacatcacagtgaccacccacaaagagacaagccctcctggatttttttcagcatttcttatactgactacagtagtgatgattaaagttatctgccctacagactccactgaatttgaagctgtatttattgtacagatgggggaaatgtgttttattgtgtcagttatattaatttttatcaatgtgattagatacatattttggcctattaatcttattcattatattcttagtctgagatgggttttaattctgactaacagcagctacttaagagtccaatcatacaaaatcaggagagtattaccctttctacagctaagcgagtcagtaatacagcagcaactaatactggccattaataacgtccagagagcacattagcaaaccttgtactcccagtgactgtcaggagacttgaaaataactactattctcttccaaagtagaatagcgtttttctagatagtgaaggaaatgatagtcatagttggtctgaactccaagatcctactcctcaaaacagcaccgaagcaggggttcgggatgcctgctaagagcatttccacagttcaagtctcttcagaaccttagggaccttcgtgtctagcttcacacacccacctccacatatgaaccagcctaccacacttcacatctgggtacactggccattagcaacaatgcagtctcatgcagcagcacattaaaatcaaacgggtggcaatcgttcaccaccctcagagtgttgggagactttcacatttcatcatccttataatccacaaacagaaacatgaagggatgcaagtgagttcagcattcactcgtttggtgcactcaagtgctgagagaatgcagaatttacagtgtcacagaggaaaaaagccatctgaaataattgtaaaaatggttaagtgtggtatttaaatgttggttccctcctcttcatacaagtggaagaaaagaaggggctagggtacccactgggccatgaggttaaccccttagcacaggcaatgaagaacatccaatgccacagattctgcaggaggagaaatcccaagggtatacagtattcctgagaaagatcccagatttttctgaatcagtcttaatctgattttgttttggctacacagttatgctgttatacctttgacatacataaaaatggtcattttatttcaatccagacagctcagcattgtacaaatgatggcagaaagatccatttgttcagactcagcttgctttgtttttaatactggggaataaaccaaaaaaaaaagtgtaatttttatcatttgtatccttcattctactttactggagtggaatccccagggccttcagataatctgggaagacctgactattcctgtgaggcaagcacagccctgctgagctttactcagaataatgcatgatagactcaacgtaattcccaggaaaaagcccagtcactccattcataactccctcataccaaccatcgtcattcttcttgatgacataaataatggctccttcctgaaaggacagctcatcttccttgtcttttgtatagtcataaattgccacaaccttttccaagtaagaacgtggagcccacggtgggtcctcttcagcataaggatcactatactcaaccacagcagcttcctcctcttcgtaatcttctggaggaggaggaggtgggggagactcatcaaagactggttcttccacaggtggcggtggaggtggtgtatctgaaatattttcttggactctggccacaaatcccattaaaggtaactgaggagttacctgtaggatggagggaggaggaggagcaagagatactggattctggctataaaaaggtcctccattcatctgattctgaaggcttgtttgtgaagtaatggaaggagggcgtctatagggcaacgagccccctattgttgggggagtatggcgagaggcaggcctattcatgctgtagaactgtacaggatgacctgtagggggagtggaagaaacaacagggggagttggagaagtgaagccatcagcaagggtctgggcacccccagcagcagcgtctggggcagtggaggaagggacagtagcaggaacaagaggagcaggggcagatgcagaagtagcaggaaggggaggagtgccagcagagccagcaggggctggaaagacactgggaggagatggagtaggaacagcaataggaacccccacactaccacttccactgttctctcgactgctgctccgactacttgggtggctccctccactactcccactgctgctgtaagttcgatttctttgattcacagaagctgtcctcacagggctctgctgcgagggagccatattacgggttgggctaggtacgtaatcatttggtaccactggaggacgcactggctccagtgtgcgatagggggagtgccgcccaagtgtccctttccctgacatagggggactagggggcttctgagttggaggtgttgtacgcggcagcccacccatcttcatgttctgggtactcaccttaaatctaagcaaccactttactccatgtccaatatcatctagaattgtatagtcaataggttttctaatataacgaactggtcgttcaaggttggctggagcaataatcttatgtgtccttgaagtgtttttattggtagtcaaaataccaatttctcttcttgcaactttctctttatgaatatcaactgtttgtgaaatatgattgattgaagattccatccttcgtagctgggatgcctggatatccagcatctgcaggacattgttggccaaggtgtttatcagataggcaacacttgctaaggattgggtggtgtaggctttggtttcttctagggctctctgcttatctgctgactgtatgtagttgttctcgcagtaatcggccacccgttccagatttgtgtagctgtcgaagagggcccggcggccccccgggatttcctcttccagcagcatctgcagctccgccatcttcacatcctcctcctcctcctcctcatacaggtcgcagagggagcggcggccgcagcgccaaggaaacccaggaccgggagaggaggagcggcggcgacggcggcggtaactcggaagg

SEQ ID NO: 11854 - RNA, 4045 nt, Homo sapiens
  source 1..4045: mol_type = other RNA
ctgaatagctgggactacaggtgtgcgccaccacgcccagctaatttttgtgtttttagtagagatggggtttcaccatgttggccaggatggtctcaatttattgacctcatgatccacccacctcggcctccgaaagtgctgggattacaggcataagccaccacacccagcctgtgggaactatttattggatttcaaaacaccctctgcctcattaatccactaagctttctcagcaaaaagctgtttaaataaataatgggaacatctaatttaaaacagtttttctaattatagaccagtacacgaagaagagcttaacttatccaagtatagtctagtttgggtccataatggagctgaaggctcagaggacattcagggccattacactgcaggaaaacaaggaataagggatgtagaaatgacctaagaaaagcacgaagtggaatgtatactggaggcaagttaatgaaagctaataaatacaaagtgctgggaaaaatctaaaagcaaaatagctattgtaacttgcaatgcattaaaaacaactttaaaaccaaaaagtcttgataaggaaactctatagtggggtctcagttaaatgctgatgatttttaatgctcagataacattaagtggaatattaacttctgcatccgacaccatctgaattttctcacacactactacacttgttcacttttcaatcaagttccactttctgaacttgttcaaaacctcatttgaaatatatccagctactgcttttcccctttcacctagcacagggcagttacctggcaaagctctattctggccaagtcactgggactgagtagaacccacgttagcagctctggacctgaacaggagctggcccaacatcacagtgaccacccacaaagagacaagccctcctggatttttttcagcatttcttatactgactacagtagtgatgattaaagttatctgccctacagactccactgaatttgaagctgtatttattgtacagatgggggaaatgtgttttattgtgtcagttatattaatttttatcaatgtgattagatacatattttggcctattaatcttattcattatattcttagtctgagatgggttttaattctgactaacagcagctacttaagagtccaatcatacaaaatcaggagagtattaccctttctacagctaagcgagtcagtaatacagcagcaactaatactggccattaataacgtccagagagcacattagcaaaccttgtactcccagtgactgtcaggagacttgaaaataactactattctcttccaaagtagaatagcgtttttctagatagtgaaggaaatgatagtcatagttggtctgaactccaagatcctactcctcaaaacagcaccgaagcaggggttcgggatgcctgctaagagcatttccacagttcaagtctcttcagaaccttagggaccttcgtgtctagcttcacacacccacctccacatatgaaccagcctaccacacttcacatctgggtacactggccattagcaacaatgcagtctcatgcagcagcacattaaaatcaaacgggtggcaatcgttcaccaccctcagagtgttgggagactttcacatttcatcatccttataatccacaaacagaaacatgaagggatgcaagtgagttcagcattcactcgtttggtgcactcaagtgctgagagaatgcagaatttacagtgtcacagaggaaaaaagccatctgaaataattgtaaaaatggttaagtgtggtatttaaatgttggttccctcctcttcatacaagtggaagaaaagaaggggctagggtacccactgggccatgaggttaaccccttagcacaggcaatgaagaacatccaatgccacagattctgcaggaggagaaatcccaagggtatacagtattcctgagaaagatcccagatttttctgaatcagtcttaatctgattttgttttggctacacagttatgctgttatacctttgacatacataaaaatggtcattttatttcaatccagacagctcagcattgtacaaatgatggcagaaagatccatttgttcagactcagcttgctttgtttttaatactggggaataaaccaaaaaaaaaagtgtaatttttatcatttgtatccttcattctactttactggagtggaatccccagggccttcagataatctgggaagacctgactattcctgtgaggcaagcacagccctgctgagctttactcagaataatgcatgatagactcaacgtaattcccaggaaaaagcccagtcactccattcataactccctcataccaaccatcgtcattcttcttgatgacataaataatggctccttcctgaaaggacagctcatcttccttgtcttttgtatagtcataaattgccacaaccttttccaagtaagaacgtggagcccacggtgggtcctcttcagcataaggatcactatactcaaccacagcagcttcctcctcttcgtaatcttctggaggaggaggaggtgggggagactcatcaaagactggttcttccacaggtggcggtggaggtggtgtatctgaaatattttcttggactctggccacaaatcccattaaaggtaactgaggagttacctgtaggatggagggaggaggaggagcaagagatactggattctggctataaaaaggtcctccattcatctgattctgaaggcttgtttgtgaagtaatggaaggagggcgtctatagggcaacgagccccctattgttgggggagtatggcgagaggcaggcctattcatgctgtagaactgtacaggatgacctgtagggggagtggaagaaacaacagggggagttggagaagtgaagccatcagcaagggtctgggcacccccagcagcagcgtctggggcagtggaggaagggacagtagcaggaacaagaggagcaggggcagatgcagaagtagcaggaaggggaggagtgccagcagagccagcaggggctggaaagacactgggaggagatggagtaggaacagcaataggaacccccacactaccacttccactgttctctcgactgctgctccgactacttgggtggctccctccactactcccactgctgctgtaagttcgatttctttgattcacagaagctgtcctcacagggctctgctgcgagggagccatattacgggttgggctaggtacgtaatcatttggtaccactggaggacgcactggctccagtgtgcgatagggggagtgccgcccaagtgtccctttccctgacatagggggactagggggcttctgagttggaggtgttgtacgcggcagcccacccatcttcatgttctgggtactcaccttaaatctaagcaaccactttactccatgtccaatatcatctagaattgtatagtcaataggttttctaatataacgaactggtcgttcaaggttggctggagcaataatcttatgtgtccttgaagtgtttttattggtagtcaaaataccaatttctcttcttgcaactttctctttatgaatatcaactgtttgtgaaatatgattgattgaagattccatccttcgtagctgggatgcctggatatccagcatctgcaggacattgttggccaaggtgtttatcagataggcaacacttgctaaggattgggtggtgtaggctttggtttcttctagggctctctgcttatctgctgtatgtagttgttctcgcagtaatcggccacccgttccagatttgtgtagctgtcgaagagggcccggcggccccccgggatttcctcttccagcagcatctgcagctccgccatcttcacatcctcctcctcctcctcctcatacaggtcgcagagggagcggcggccgcagcgccaaggaaacccaggaccgggagaggaggagcggcggcgacggcggcggtaactcggaagg

SEQ ID NO: 11855 - RNA, 4031 nt, Homo sapiens
  source 1..4031: mol_type = other RNA
ctgaatagctgggactacaggtgtgcgccaccacgcccagctaatttttgtgtttttagtagagatggggtttcaccatgttggccaggatggtctcaatttattgacctcatgatccacccacctcggcctccgaaagtgctgggattacaggcataagccaccacacccagcctgtgggaactatttattggatttcaaaacaccctctgcctcattaatccactaagctttctcagcaaaaagctgtttaaataaataatgggaacatctaatttaaaacagtttttctaattatagaccagtacacgaagaagagcttaacttatccaagtatagtctagtttgggtccataatggagctgaaggctcagaggacattcagggccattacactgcaggaaaacaaggaataagggatgtagaaatgacctaagaaaagcacgaagtggaatgtatactggaggcaagttaatgaaagctaataaatacaaagtgctgggaaaaatctaaaagcaaaatagctattgtaacttgcaatgcattaaaaacaactttaaaaccaaaaagtcttgataaggaaactctatagtggggtctcagttaaatgctgatgatttttaatgctcagataacattaagtggaatattaacttctgcatccgacaccatctgaattttctcacacactactacacttgttcacttttcaatcaagttccactttctgaacttgttcaaaacctcatttgaaatatatccagctactgcttttcccctttcacctagcacagggcagttacctggcaaagctctattctggccaagtcactgggactgagtagaacccacgttagcagctctggacctgaacaggagctggcccaacatcacagtgaccacccacaaagagacaagccctcctggatttttttcagcatttcttatactgactacagtagtgatgattaaagttatctgccctacagactccactgaatttgaagctgtatttattgtacagatgggggaaatgtgttttattgtgtcagttatattaatttttatcaatgtgattagatacatattttggcctattaatcttattcattatattcttagtctgagatgggttttaattctgactaacagcagctacttaagagtccaatcatacaaaatcaggagagtattaccctttctacagctaagcgagtcagtaatacagcagcaactaatactggccattaataacgtccagagagcacattagcaaaccttgtactcccagtgactgtcaggagacttgaaaataactactattctcttccaaagtagaatagcgtttttctagatagtgaaggaaatgatagtcatagttggtctgaactccaagatcctactcctcaaaacagcaccgaagcaggggttcgggatgcctgctaagagcatttccacagttcaagtctcttcagaaccttagggaccttcgtgtctagcttcacacacccacctccacatatgaaccagcctaccacacttcacatctgggtacactggccattagcaacaatgcagtctcatgcagcagcacattaaaatcaaacgggtggcaatcgttcaccaccctcagagtgttgggagactttcacatttcatcatccttataatccacaaacagaaacatgaagggatgcaagtgagttcagcattcactcgtttggtgcactcaagtgctgagagaatgcagaatttacagtgtcacagaggaaaaaagccatctgaaataattgtaaaaatggttaagtgtggtatttaaatgttggttccctcctcttcatacaagtggaagaaaagaaggggctagggtacccactgggccatgaggttaaccccttagcacaggcaatgaagaacatccaatgccacagattctgcaggaggagaaatcccaagggtatacagtattcctgagaaagatcccagatttttctgaatcagtcttaatctgattttgttttggctacacagttatgctgttatacctttgacatacataaaaatggtcattttatttcaatccagacagctcagcattgtacaaatgatggcagaaagatccatttgttcagactcagcttgctttgtttttaatactggggaataaaccaaaaaaaaaagtgtaatttttatcatttgtatccttcattctactttactggagtggaatccccagggccttcagataatctgggaagacctgactattcctgtgaggcaagcacagccctgctgagctttactcagaataatgcatgatagactcaacgtaattcccaggaaaaagcccagtcactccattcataactccctcataccaaccatcgtcattcttcttgatgacataaataatggctccttcctgaaaggacagctcatcttccttgtcttttgtatagtcataaattgccacaaccttttccaagtaagaacgtggagcccacggtgggtcctcttcagcataaggatcactatactcaaccacagcagcttcctcctcttcgtaatcttctggaggaggaggaggtgggggagactcatcaaagactggttcttccacaggtggcggtggaggtggtgtatctgaaatattttcttggactctggccacaaatcccattaaaggtaactgaggagttacctgtaggatggagggaggaggaggagcaagagatactggattctggctataaaaaggtcctccattcatctgattctgaaggcttgtttgtgaagtaatggaaggagggcgtctatagggcaacgagccccctattgttgggggagtatggcgagaggcaggcctattcatgctgtagaactgtacaggatgacctgtagggggagtggaagaaacaacagggggagttggagaagtgaagccatcagcaagggtctgggcacccccagcagcagcgtctggggcagtggaggaagggacagtagcaggaacaagaggagcaggggcagatgcagaagtagcaggaaggggaggagtgccagcagagccagcaggggctggaaagacactgggaggagatggagtaggaacagcaataggaacccccacactaccacttccactgttctctcgactgctgctccgactacttgggtggctccctccactactcccactgctgctgtaagttcgatttctttgattcacagaagctgtcctcacagggctctgctgcgagggagccatattacgggttgggctaggtacgtaatcatttggtaccactggaggacgcactggctccagtgtgcgatagggggagtgccgcccaagtgtccctttccctgacatagggggactagggggcttctgagttggaggtgttgtacgcggcagcccacccatcttcatgttctgggtactcacctttactccatgtccaatatcatctagaattgtatagtcaataggttttctaatataacgaactggtcgttcaaggttggctggagcaataatcttatgtgtccttgaagtgtttttattggtagtcaaaataccaatttctcttcttgcaactttctctttatgaatatcaactgtttgtgaaatatgattgattgaagattccatccttcgtagctgggatgcctggatatccagcatctgcaggacattgttggccaaggtgtttatcagataggcaacacttgctaaggattgggtggtgtaggctttggtttcttctagggctctctgcttatctgctgactgtatgtagttgttctcgcagtaatcggccacccgttccagatttgtgtagctgtcgaagagggcccggcggccccccgggatttcctcttccagcagcatctgcagctccgccatcttcacatcctcctcctcctcctcctcatacaggtcgcagagggagcggcggccgcagcgccaaggaaacccaggaccgggagaggaggagcggcggcgacggcggcggtaactcggaagg

SEQ ID NO: 11856 - RNA, 4027 nt, Homo sapiens
  source 1..4027: mol_type = other RNA
ctgaatagctgggactacaggtgtgcgccaccacgcccagctaatttttgtgtttttagtagagatggggtttcaccatgttggccaggatggtctcaatttattgacctcatgatccacccacctcggcctccgaaagtgctgggattacaggcataagccaccacacccagcctgtgggaactatttattggatttcaaaacaccctctgcctcattaatccactaagctttctcagcaaaaagctgtttaaataaataatgggaacatctaatttaaaacagtttttctaattatagaccagtacacgaagaagagcttaacttatccaagtatagtctagtttgggtccataatggagctgaaggctcagaggacattcagggccattacactgcaggaaaacaaggaataagggatgtagaaatgacctaagaaaagcacgaagtggaatgtatactggaggcaagttaatgaaagctaataaatacaaagtgctgggaaaaatctaaaagcaaaatagctattgtaacttgcaatgcattaaaaacaactttaaaaccaaaaagtcttgataaggaaactctatagtggggtctcagttaaatgctgatgatttttaatgctcagataacattaagtggaatattaacttctgcatccgacaccatctgaattttctcacacactactacacttgttcacttttcaatcaagttccactttctgaacttgttcaaaacctcatttgaaatatatccagctactgcttttcccctttcacctagcacagggcagttacctggcaaagctctattctggccaagtcactgggactgagtagaacccacgttagcagctctggacctgaacaggagctggcccaacatcacagtgaccacccacaaagagacaagccctcctggatttttttcagcatttcttatactgactacagtagtgatgattaaagttatctgccctacagactccactgaatttgaagctgtatttattgtacagatgggggaaatgtgttttattgtgtcagttatattaatttttatcaatgtgattagatacatattttggcctattaatcttattcattatattcttagtctgagatgggttttaattctgactaacagcagctacttaagagtccaatcatacaaaatcaggagagtattaccctttctacagctaagcgagtcagtaatacagcagcaactaatactggccattaataacgtccagagagcacattagcaaaccttgtactcccagtgactgtcaggagacttgaaaataactactattctcttccaaagtagaatagcgtttttctagatagtgaaggaaatgatagtcatagttggtctgaactccaagatcctactcctcaaaacagcaccgaagcaggggttcgggatgcctgctaagagcatttccacagttcaagtctcttcagaaccttagggaccttcgtgtctagcttcacacacccacctccacatatgaaccagcctaccacacttcacatctgggtacactggccattagcaacaatgcagtctcatgcagcagcacattaaaatcaaacgggtggcaatcgttcaccaccctcagagtgttgggagactttcacatttcatcatccttataatccacaaacagaaacatgaagggatgcaagtgagttcagcattcactcgtttggtgcactcaagtgctgagagaatgcagaatttacagtgtcacagaggaaaaaagccatctgaaataattgtaaaaatggttaagtgtggtatttaaatgttggttccctcctcttcatacaagtggaagaaaagaaggggctagggtacccactgggccatgaggttaaccccttagcacaggcaatgaagaacatccaatgccacagattctgcaggaggagaaatcccaagggtatacagtattcctgagaaagatcccagatttttctgaatcagtcttaatctgattttgttttggctacacagttatgctgttatacctttgacatacataaaaatggtcattttatttcaatccagacagctcagcattgtacaaatgatggcagaaagatccatttgttcagactcagcttgctttgtttttaatactggggaataaaccaaaaaaaaaagtgtaatttttatcatttgtatccttcattctactttactggagtggaatccccagggccttcagataatctgggaagacctgactattcctgtgaggcaagcacagccctgctgagctttactcagaataatgcatgatagactcaacgtaattcccaggaaaaagcccagtcactccattcataactccctcataccaaccatcgtcattcttcttgatgacataaataatggctccttcctgaaaggacagctcatcttccttgtcttttgtatagtcataaattgccacaaccttttccaagtaagaacgtggagcccacggtgggtcctcttcagcataaggatcactatactcaaccacagcagcttcctcctcttcgtaatcttctggaggaggaggaggtgggggagactcatcaaagactggttcttccacaggtggcggtggaggtggtgtatctgaaatattttcttggactctggccacaaatcccattaaaggtaactgaggagttacctgtaggatggagggaggaggaggagcaagagatactggattctggctataaaaaggtcctccattcatctgattctgaaggcttgtttgtgaagtaatggaaggagggcgtctatagggcaacgagccccctattgttgggggagtatggcgagaggcaggcctattcatgctgtagaactgtacaggatgacctgtagggggagtggaagaaacaacagggggagttggagaagtgaagccatcagcaagggtctgggcacccccagcagcagcgtctggggcagtggaggaagggacagtagcaggaacaagaggagcaggggcagatgcagaagtagcaggaaggggaggagtgccagcagagccagcaggggctggaaagacactgggaggagatggagtaggaacagcaataggaacccccacactaccacttccactgttctctcgactgctgctccgactacttgggtggctccctccactactcccactgctgctgtaagttcgatttctttgattcacagaagctgtcctcacagggctctgctgcgagggagccatattacgggttgggctaggtacgtaatcatttggtaccactggaggacgcactggctccagtgtgcgatagggggagtgccgcccaagtgtccctttccctgacatagggggactagggggcttctgagttggaggtgttgtacgcggcagcccacccatcttcatgttctgggtactcacctttactccatgtccaatatcatctagaattgtatagtcaataggttttctaatataacgaactggtcgttcaaggttggctggagcaataatcttatgtgtccttgaagtgtttttattggtagtcaaaataccaatttctcttcttgcaactttctctttatgaatatcaactgtttgtgaaatatgattgattgaagattccatccttcgtagctgggatgcctggatatccagcatctgcaggacattgttggccaaggtgtttatcagataggcaacacttgctaaggattgggtggtgtaggctttggtttcttctagggctctctgcttatctgctgtatgtagttgttctcgcagtaatcggccacccgttccagatttgtgtagctgtcgaagagggcccggcggccccccgggatttcctcttccagcagcatctgcagctccgccatcttcacatcctcctcctcctcctcctcatacaggtcgcagagggagcggcggccgcagcgccaaggaaacccaggaccgggagaggaggagcggcggcgacggcggcggtaactcggaagg

SEQ ID NO: 11857 - RNA, 4046 nt, Homo sapiens
  source 1..4046: mol_type = other RNA
ctgaatagctgggactacaggtgtgcgccaccacgcccagctaatttttgtgtttttagtagagatggggtttcaccatgttggccaggatggtctcaatttattgacctcatgatccacccacctcggcctccgaaagtgctgggattacaggcataagccaccacacccagcctgtgggaactatttattggatttcaaaacaccctctgcctcattaatccactaagctttctcagcaaaaagctgtttaaataaataatgggaacatctaatttaaaacagtttttctaattatagaccagtacacgaagaagagcttaacttatccaagtatagtctagtttgggtccataatggagctgaaggctcagaggacattcagggccattacactgcaggaaaacaaggaataagggatgtagaaatgacctaagaaaagcacgaagtggaatgtatactggaggcaagttaatgaaagctaataaatacaaagtgctgggaaaaatctaaaagcaaaatagctattgtaacttgcaatgcattaaaaacaactttaaaaccaaaaagtcttgataaggaaactctatagtggggtctcagttaaatgctgatgatttttaatgctcagataacattaagtggaatattaacttctgcatccgacaccatctgaattttctcacacactactacacttgttcacttttcaatcaagttccactttctgaacttgttcaaaacctcatttgaaatatatccagctactgcttttcccctttcacctagcacagggcagttacctggcaaagctctattctggccaagtcactgggactgagtagaacccacgttagcagctctggacctgaacaggagctggcccaacatcacagtgaccacccacaaagagacaagccctcctggatttttttcagcatttcttatactgactacagtagtgatgattaaagttatctgccctacagactccactgaatttgaagctgtatttattgtacagatgggggaaatgtgttttattgtgtcagttatattaatttttatcaatgtgattagatacatattttggcctattaatcttattcattatattcttagtctgagatgggttttaattctgactaacagcagctacttaagagtccaatcatacaaaatcaggagagtattaccctttctacagctaagcgagtcagtaatacagcagcaactaatactggccattaataacgtccagagagcacattagcaaaccttgtactcccagtgactgtcaggagacttgaaaataactactattctcttccaaagtagaatagcgtttttctagatagtgaaggaaatgatagtcatagttggtctgaactccaagatcctactcctcaaaacagcaccgaagcaggggttcgggatgcctgctaagagcatttccacagttcaagtctcttcagaaccttagggaccttcgtgtctagcttcacacacccacctccacatatgaaccagcctaccacacttcacatctgggtacactggccattagcaacaatgcagtctcatgcagcagcacattaaaatcaaacgggtggcaatcgttcaccaccctcagagtgttgggagactttcacatttcatcatccttataatccacaaacagaaacatgaagggatgcaagtgagttcagcattcactcgtttggtgcactcaagtgctgagagaatgcagaatttacagtgtcacagaggaaaaaagccatctgaaataattgtaaaaatggttaagtgtggtatttaaatgttggttccctcctcttcatacaagtggaagaaaagaaggggctagggtacccactgggccatgaggttaaccccttagcacaggcaatgaagaacatccaatgccacagattctgcaggaggagaaatcccaagggtatacagtattcctgagaaagatcccagatttttctgaatcagtcttaatctgattttgttttggctacacagttatgctgttatacctttgacatacataaaaatggtcattttatttcaatccagacagctcagcattgtacaaatgatggcagaaagatccatttgttcagactcagcttgctttgtttttaatactggggaataaaccaaaaaaaaaagtgtaatttttatcatttgtatccttcattctactttactggagtggaatccccagggccttcagataatctgggaagacctgactattcctgtgaggcaagcacagccctgctgagctttactcagaataatgcatgatagactcaacgtaattcccaggaaaaagcccagtcactccattcataactccctcataccaaccatcgtcattcttcttgatgacataaataatggctccttcctgaaaggacagctcatcttccttgtcttttgtatagtcataaattgccacaaccttttccaagtaagaacgtggagcccacggtgggtcctcttcagcataaggatcactatactcaaccacagcagcttcctcctcttcgtaatcttctggaggaggaggaggtgggggagactcatcaaagactggttcttccacaggtggcggtggaggtggtgtatctgaaatattttcttggactctggccacaaatcccattaaaggtaactgaggagttacctgtaggatggagggaggaggaggagcaagagatactggattctggctataaaaaggtcctccattcatctgattctgaaggcttgtttgtgaagtaatggaaggagggcgtctatagggcaacgagccccctattgttgggggagtatggcgagaggcaggcctattcatgctgtagaactgtacaggatgacctgtagggggagtggaagaaacaacagggggagttggagaagtgaagccatcagcaagggtctgggcacccccagcagcagcgtctggggcagtggaggaagggacagtagcaggaacaagaggagcaggggcagatgcagaagtagcaggaaggggaggagtgccagcagagccagcaggggctggaaagacactgggaggagatggagtaggaacagcaataggaacccccacactaccacttccactgttctctcgactgctgctccgactacttgggtggctccctccactactcccactgctgtaagttcgatttctttgattcacagaagctgtcctcacagggctctgctgcgagggagccatattacgggttgggctaggtacgtaatcatttggtaccactggaggacgcactggctccagtgtgcgatagggggagtgccgcccaagtgtccctttccctgacatagggggactagggggcttctgagttggaggtgttgtacgcggcagcccacccatcttcatgttctgggtactcaccttaaatctaagcaaccactttactccatgtccaatatcatctagaattgtatagtcaataggttttctaatataacgaactggtcgttcaaggttggctggagcaataatcttatgtgtccttgaagtgtttttattggtagtcaaaataccaatttctcttcttgcaactttctctttatgaatatcaactgtttgtgaaatatgattgattgaagattccatccttcgtagctgggatgcctggatatccagcatctgcaggacattgttggccaaggtgtttatcagataggcaacacttgctaaggattgggtggtgtaggctttggtttcttctagggctctctgcttatctgctgactgtatgtagttgttctcgcagtaatcggccacccgttccagatttgtgtagctgtcgaagagggcccggcggccccccgggatttcctcttccagcagcatctgcagctccgccatcttcacatcctcctcctcctcctcctcatacaggtcgcagagggagcggcggccgcagcgccaaggaaacccaggaccgggagaggaggagcggcggcgacggcggcggtaactcggaagg

SEQ ID NO: 11858 - RNA, 3608 nt, Homo sapiens
  source 1..3608: mol_type = other RNA
ctgaatagctgggactacaggtgtgcgccaccacgcccagctaatttttgtgtttttagtagagatggggtttcaccatgttggccaggatggtctcaatttattgacctcatgatccacccacctcggcctccgaaagtgctgggattacaggcataagccaccacacccagcctgtgggaactatttattggatttcaaaacaccctctgcctcattaatccactaagctttctcagcaaaaagctgtttaaataaataatgggaacatctaatttaaaacagtttttctaattatagaccagtacacgaagaagagcttaacttatccaagtatagtctagtttgggtccataatggagctgaaggctcagaggacattcagggccattacactgcaggaaaacaaggaataagggatgtagaaatgacctaagaaaagcacgaagtggaatgtatactggaggcaagttaatgaaagctaataaatacaaagtgctgggaaaaatctaaaagcaaaatagctattgtaacttgcaatgcattaaaaacaactttaaaaccaaaaagtcttgataaggaaactctatagtggggtctcagttaaatgctgatgatttttaatgctcagataacattaagtggaatattaacttctgcatccgacaccatctgaattttctcacacactactacacttgttcacttttcaatcaagttccactttctgaacttgttcaaaacctcatttgaaatatatccagctactgcttttcccctttcacctagcacagggcagttacctggcaaagctctattctggccaagtcactgggactgagtagaacccacgttagcagctctggacctgaacaggagctggcccaacatcacagtgaccacccacaaagagacaagccctcctggatttttttcagcatttcttatactgactacagtagtgatgattaaagttatctgccctacagactccactgaatttgaagctgtatttattgtacagatgggggaaatgtgttttattgtgtcagttatattaatttttatcaatgtgattagatacatattttggcctattaatcttattcattatattcttagtctgagatgggttttaattctgactaacagcagctacttaagagtccaatcatacaaaatcaggagagtattaccctttctacagctaagcgagtcagtaatacagcagcaactaatactggccattaataacgtccagagagcacattagcaaaccttgtactcccagtgactgtcaggagacttgaaaataactactattctcttccaaagtagaatagcgtttttctagatagtgaaggaaatgatagtcatagttggtctgaactccaagatcctactcctcaaaacagcaccgaagcaggggttcgggatgcctgctaagagcatttccacagttcaagtctcttcagaaccttagggaccttcgtgtctagcttcacacacccacctccacatatgaaccagcctaccacacttcacatctgggtacactggccattagcaacaatgcagtctcatgcagcagcacattaaaatcaaacgggtggcaatcgttcaccaccctcagagtgttgggagactttcacatttcatcatccttataatccacaaacagaaacatgaagggatgcaagtgagttcagcattcactcgtttggtgcactcaagtgctgagagaatgcagaatttacagtgtcacagaggaaaaaagccatctgaaataattgtaaaaatggttaagtgtggtatttaaatgttggttccctcctcttcatacaagtggaagaaaagaaggggctagggtacccactgggccatgaggttaaccccttagcacaggcaatgaagaacatccaatgccacagattctgcaggaggagaaatcccaagggtatacagtattcctgagaaagatcccagatttttctgaatcagtcttaatctgattttgttttggctacacagttatgctgttatacctttgacatacataaaaatggtcattttatttcaatccagacagctcagcattgtacaaatgatggcagaaagatccatttgttcagactcagcttgctttgtttttaatactggggaataaaccaaaaaaaaaagtgtaatttttatcatttgtatccttcattctactttactggagtggaatccccagggccttcagataatctgggaagacctgactattcctgtgaggcaagcacagccctgctgagctttactcagaataatgcatgatagactcaacgtaattcccaggaaaaagcccagtcactccattcataactccctcataccaaccatcgtcattcttcttgatgacataaataatggctccttcctgaaaggacagctcatcttccttgtcttttgtatagtcataaattgccacaaccttttccaagtaagaacgtggagcccacggtgggtcctcttcagcataaggatcactatactcaaccacagcagcttcctcctcttcgtaatcttctggaggaggaggaggtgggggagactcatcaaagactggttcttccacaggtggcggtggaggtggtgtatctggattctggctataaaaaggtcctccattcatctgattctgaaggcttgtttgtgaagtaatggaaggagggcgtctatagggcaacgagccccctattgttgggggagtatggcgagaggcaggcctattcatgctgtagaactgtacaggatgacctggaaagacactgggaggagatggagtaggaacagcaataggaacccccacactaccacttccactgttctctcgactgctgctccgactacttgggtggctccctccactactcccactgctgccaagtgtccctttccctgacatagggggactagggggcttctgagttggaggtgttgtacgcggcagcccacccatcttcatgttctgggtactcacctttactccatgtccaatatcatctagaattgtatagtcaataggttttctaatataacgaactggtcgttcaaggttggctggagcaataatcttatgtgtccttgaagtgtttttattggtagtcaaaataccaatttctcttcttgcaactttctctttatgaatatcaactgtttgtgaaatatgattgattgaagattccatccttcgtagctgggatgcctggatatccagcatctgcaggacattgttggccaaggtgtttatcagataggcaacacttgctaaggattgggtggtgtaggctttggtttcttctagggctctctgcttatctgctgactgtatgtagttgttctcgcagtaatcggccacccgttccagatttgtgtagctgtcgaagagggcccggcggccccccgggatttcctcttccagcagcatctgcagctccgccatcttcacatcctcctcctcctcctcctcatacaggtcgcagagggagcggcggccgcagcgccaaggaaacccaggaccgggagaggaggagcggcggcgacggcggcggtaactcggaagg

SEQ ID NO: 11859 - RNA, 3755 nt, Homo sapiens
  source 1..3755: mol_type = other RNA
ctgaatagctgggactacaggtgtgcgccaccacgcccagctaatttttgtgtttttagtagagatggggtttcaccatgttggccaggatggtctcaatttattgacctcatgatccacccacctcggcctccgaaagtgctgggattacaggcataagccaccacacccagcctgtgggaactatttattggatttcaaaacaccctctgcctcattaatccactaagctttctcagcaaaaagctgtttaaataaataatgggaacatctaatttaaaacagtttttctaattatagaccagtacacgaagaagagcttaacttatccaagtatagtctagtttgggtccataatggagctgaaggctcagaggacattcagggccattacactgcaggaaaacaaggaataagggatgtagaaatgacctaagaaaagcacgaagtggaatgtatactggaggcaagttaatgaaagctaataaatacaaagtgctgggaaaaatctaaaagcaaaatagctattgtaacttgcaatgcattaaaaacaactttaaaaccaaaaagtcttgataaggaaactctatagtggggtctcagttaaatgctgatgatttttaatgctcagataacattaagtggaatattaacttctgcatccgacaccatctgaattttctcacacactactacacttgttcacttttcaatcaagttccactttctgaacttgttcaaaacctcatttgaaatatatccagctactgcttttcccctttcacctagcacagggcagttacctggcaaagctctattctggccaagtcactgggactgagtagaacccacgttagcagctctggacctgaacaggagctggcccaacatcacagtgaccacccacaaagagacaagccctcctggatttttttcagcatttcttatactgactacagtagtgatgattaaagttatctgccctacagactccactgaatttgaagctgtatttattgtacagatgggggaaatgtgttttattgtgtcagttatattaatttttatcaatgtgattagatacatattttggcctattaatcttattcattatattcttagtctgagatgggttttaattctgactaacagcagctacttaagagtccaatcatacaaaatcaggagagtattaccctttctacagctaagcgagtcagtaatacagcagcaactaatactggccattaataacgtccagagagcacattagcaaaccttgtactcccagtgactgtcaggagacttgaaaataactactattctcttccaaagtagaatagcgtttttctagatagtgaaggaaatgatagtcatagttggtctgaactccaagatcctactcctcaaaacagcaccgaagcaggggttcgggatgcctgctaagagcatttccacagttcaagtctcttcagaaccttagggaccttcgtgtctagcttcacacacccacctccacatatgaaccagcctaccacacttcacatctgggtacactggccattagcaacaatgcagtctcatgcagcagcacattaaaatcaaacgggtggcaatcgttcaccaccctcagagtgttgggagactttcacatttcatcatccttataatccacaaacagaaacatgaagggatgcaagtgagttcagcattcactcgtttggtgcactcaagtgctgagagaatgcagaatttacagtgtcacagaggaaaaaagccatctgaaataattgtaaaaatggttaagtgtggtatttaaatgttggttccctcctcttcatacaagtggaagaaaagaaggggctagggtacccactgggccatgaggttaaccccttagcacaggcaatgaagaacatccaatgccacagattctgcaggaggagaaatcccaagggtatacagtattcctgagaaagatcccagatttttctgaatcagtcttaatctgattttgttttggctacacagttatgctgttatacctttgacatacataaaaatggtcattttatttcaatccagacagctcagcattgtacaaatgatggcagaaagatccatttgttcagactcagcttgctttgtttttaatactggggaataaaccaaaaaaaaaagtgtaatttttatcatttgtatccttcattctactttactggagtggaatccccagggccttcagataatctgggaagacctgactattcctgtgaggcaagcacagccctgctgagctttactcagaataatgcatgatagactcaacgtaattcccaggaaaaagcccagtcactccattcataactccctcataccaaccatcgtcattcttcttgatgacataaataatggctccttcctgaaaggacagctcatcttccttgtcttttgtatagtcataaattgccacaaccttttccaagtaagaacgtggagcccacggtgggtcctcttcagcataaggatcactatactcaaccacagcagcttcctcctcttcgtaatcttctggaggaggaggaggtgggggagactcatcaaagactggttcttccacaggtggcggtggaggtggtgtatctggattctggctataaaaaggtcctccattcatctgattctgaaggcttgtttgtgaagtaatggaaggagggcgtctatagggcaacgagccccctattgttgggggagtatggcgagaggcaggcctattcatgctgtagaactgtacaggatgacctggaaagacactgggaggagatggagtaggaacagcaataggaacccccacactaccacttccactgttctctcgactgctgctccgactacttgggtggctccctccactactcccactgctgctgtaagttcgatttctttgattcacagaagctgtcctcacagggctctgctgcgagggagccatattacgggttgggctaggtacgtaatcatttggtaccactggaggacgcactggctccagtgtgcgatagggggagtgccgcccaagtgtccctttccctgacatagggggactagggggcttctgagttggaggtgttgtacgcggcagcccacccatcttcatgttctgggtactcacctttactccatgtccaatatcatctagaattgtatagtcaataggttttctaatataacgaactggtcgttcaaggttggctggagcaataatcttatgtgtccttgaagtgtttttattggtagtcaaaataccaatttctcttcttgcaactttctctttatgaatatcaactgtttgtgaaatatgattgattgaagattccatccttcgtagctgggatgcctggatatccagcatctgcaggacattgttggccaaggtgtttatcagataggcaacacttgctaaggattgggtggtgtaggctttggtttcttctagggctctctgcttatctgctgactgtatgtagttgttctcgcagtaatcggccacccgttccagatttgtgtagctgtcgaagagggcccggcggccccccgggatttcctcttccagcagcatctgcagctccgccatcttcacatcctcctcctcctcctcctcatacaggtcgcagagggagcggcggccgcagcgccaaggaaacccaggaccgggagaggaggagcggcggcgacggcggcggtaactcggaagg

SEQ ID NO: 11860 - RNA, 3751 nt, Homo sapiens
  source 1..3751: mol_type = other RNA
ctgaatagctgggactacaggtgtgcgccaccacgcccagctaatttttgtgtttttagtagagatggggtttcaccatgttggccaggatggtctcaatttattgacctcatgatccacccacctcggcctccgaaagtgctgggattacaggcataagccaccacacccagcctgtgggaactatttattggatttcaaaacaccctctgcctcattaatccactaagctttctcagcaaaaagctgtttaaataaataatgggaacatctaatttaaaacagtttttctaattatagaccagtacacgaagaagagcttaacttatccaagtatagtctagtttgggtccataatggagctgaaggctcagaggacattcagggccattacactgcaggaaaacaaggaataagggatgtagaaatgacctaagaaaagcacgaagtggaatgtatactggaggcaagttaatgaaagctaataaatacaaagtgctgggaaaaatctaaaagcaaaatagctattgtaacttgcaatgcattaaaaacaactttaaaaccaaaaagtcttgataaggaaactctatagtggggtctcagttaaatgctgatgatttttaatgctcagataacattaagtggaatattaacttctgcatccgacaccatctgaattttctcacacactactacacttgttcacttttcaatcaagttccactttctgaacttgttcaaaacctcatttgaaatatatccagctactgcttttcccctttcacctagcacagggcagttacctggcaaagctctattctggccaagtcactgggactgagtagaacccacgttagcagctctggacctgaacaggagctggcccaacatcacagtgaccacccacaaagagacaagccctcctggatttttttcagcatttcttatactgactacagtagtgatgattaaagttatctgccctacagactccactgaatttgaagctgtatttattgtacagatgggggaaatgtgttttattgtgtcagttatattaatttttatcaatgtgattagatacatattttggcctattaatcttattcattatattcttagtctgagatgggttttaattctgactaacagcagctacttaagagtccaatcatacaaaatcaggagagtattaccctttctacagctaagcgagtcagtaatacagcagcaactaatactggccattaataacgtccagagagcacattagcaaaccttgtactcccagtgactgtcaggagacttgaaaataactactattctcttccaaagtagaatagcgtttttctagatagtgaaggaaatgatagtcatagttggtctgaactccaagatcctactcctcaaaacagcaccgaagcaggggttcgggatgcctgctaagagcatttccacagttcaagtctcttcagaaccttagggaccttcgtgtctagcttcacacacccacctccacatatgaaccagcctaccacacttcacatctgggtacactggccattagcaacaatgcagtctcatgcagcagcacattaaaatcaaacgggtggcaatcgttcaccaccctcagagtgttgggagactttcacatttcatcatccttataatccacaaacagaaacatgaagggatgcaagtgagttcagcattcactcgtttggtgcactcaagtgctgagagaatgcagaatttacagtgtcacagaggaaaaaagccatctgaaataattgtaaaaatggttaagtgtggtatttaaatgttggttccctcctcttcatacaagtggaagaaaagaaggggctagggtacccactgggccatgaggttaaccccttagcacaggcaatgaagaacatccaatgccacagattctgcaggaggagaaatcccaagggtatacagtattcctgagaaagatcccagatttttctgaatcagtcttaatctgattttgttttggctacacagttatgctgttatacctttgacatacataaaaatggtcattttatttcaatccagacagctcagcattgtacaaatgatggcagaaagatccatttgttcagactcagcttgctttgtttttaatactggggaataaaccaaaaaaaaaagtgtaatttttatcatttgtatccttcattctactttactggagtggaatccccagggccttcagataatctgggaagacctgactattcctgtgaggcaagcacagccctgctgagctttactcagaataatgcatgatagactcaacgtaattcccaggaaaaagcccagtcactccattcataactccctcataccaaccatcgtcattcttcttgatgacataaataatggctccttcctgaaaggacagctcatcttccttgtcttttgtatagtcataaattgccacaaccttttccaagtaagaacgtggagcccacggtgggtcctcttcagcataaggatcactatactcaaccacagcagcttcctcctcttcgtaatcttctggaggaggaggaggtgggggagactcatcaaagactggttcttccacaggtggcggtggaggtggtgtatctggattctggctataaaaaggtcctccattcatctgattctgaaggcttgtttgtgaagtaatggaaggagggcgtctatagggcaacgagccccctattgttgggggagtatggcgagaggcaggcctattcatgctgtagaactgtacaggatgacctggaaagacactgggaggagatggagtaggaacagcaataggaacccccacactaccacttccactgttctctcgactgctgctccgactacttgggtggctccctccactactcccactgctgctgtaagttcgatttctttgattcacagaagctgtcctcacagggctctgctgcgagggagccatattacgggttgggctaggtacgtaatcatttggtaccactggaggacgcactggctccagtgtgcgatagggggagtgccgcccaagtgtccctttccctgacatagggggactagggggcttctgagttggaggtgttgtacgcggcagcccacccatcttcatgttctgggtactcacctttactccatgtccaatatcatctagaattgtatagtcaataggttttctaatataacgaactggtcgttcaaggttggctggagcaataatcttatgtgtccttgaagtgtttttattggtagtcaaaataccaatttctcttcttgcaactttctctttatgaatatcaactgtttgtgaaatatgattgattgaagattccatccttcgtagctgggatgcctggatatccagcatctgcaggacattgttggccaaggtgtttatcagataggcaacacttgctaaggattgggtggtgtaggctttggtttcttctagggctctctgcttatctgctgtatgtagttgttctcgcagtaatcggccacccgttccagatttgtgtagctgtcgaagagggcccggcggccccccgggatttcctcttccagcagcatctgcagctccgccatcttcacatcctcctcctcctcctcctcatacaggtcgcagagggagcggcggccgcagcgccaaggaaacccaggaccgggagaggaggagcggcggcgacggcggcggtaactcggaagg

SEQ ID NO: 11861 - RNA, 3930 nt, Homo sapiens
  source 1..3930: mol_type = other RNA
ctgaatagctgggactacaggtgtgcgccaccacgcccagctaatttttgtgtttttagtagagatggggtttcaccatgttggccaggatggtctcaatttattgacctcatgatccacccacctcggcctccgaaagtgctgggattacaggcataagccaccacacccagcctgtgggaactatttattggatttcaaaacaccctctgcctcattaatccactaagctttctcagcaaaaagctgtttaaataaataatgggaacatctaatttaaaacagtttttctaattatagaccagtacacgaagaagagcttaacttatccaagtatagtctagtttgggtccataatggagctgaaggctcagaggacattcagggccattacactgcaggaaaacaaggaataagggatgtagaaatgacctaagaaaagcacgaagtggaatgtatactggaggcaagttaatgaaagctaataaatacaaagtgctgggaaaaatctaaaagcaaaatagctattgtaacttgcaatgcattaaaaacaactttaaaaccaaaaagtcttgataaggaaactctatagtggggtctcagttaaatgctgatgatttttaatgctcagataacattaagtggaatattaacttctgcatccgacaccatctgaattttctcacacactactacacttgttcacttttcaatcaagttccactttctgaacttgttcaaaacctcatttgaaatatatccagctactgcttttcccctttcacctagcacagggcagttacctggcaaagctctattctggccaagtcactgggactgagtagaacccacgttagcagctctggacctgaacaggagctggcccaacatcacagtgaccacccacaaagagacaagccctcctggatttttttcagcatttcttatactgactacagtagtgatgattaaagttatctgccctacagactccactgaatttgaagctgtatttattgtacagatgggggaaatgtgttttattgtgtcagttatattaatttttatcaatgtgattagatacatattttggcctattaatcttattcattatattcttagtctgagatgggttttaattctgactaacagcagctacttaagagtccaatcatacaaaatcaggagagtattaccctttctacagctaagcgagtcagtaatacagcagcaactaatactggccattaataacgtccagagagcacattagcaaaccttgtactcccagtgactgtcaggagacttgaaaataactactattctcttccaaagtagaatagcgtttttctagatagtgaaggaaatgatagtcatagttggtctgaactccaagatcctactcctcaaaacagcaccgaagcaggggttcgggatgcctgctaagagcatttccacagttcaagtctcttcagaaccttagggaccttcgtgtctagcttcacacacccacctccacatatgaaccagcctaccacacttcacatctgggtacactggccattagcaacaatgcagtctcatgcagcagcacattaaaatcaaacgggtggcaatcgttcaccaccctcagagtgttgggagactttcacatttcatcatccttataatccacaaacagaaacatgaagggatgcaagtgagttcagcattcactcgtttggtgcactcaagtgctgagagaatgcagaatttacagtgtcacagaggaaaaaagccatctgaaataattgtaaaaatggttaagtgtggtatttaaatgttggttccctcctcttcatacaagtggaagaaaagaaggggctagggtacccactgggccatgaggttaaccccttagcacaggcaatgaagaacatccaatgccacagattctgcaggaggagaaatcccaagggtatacagtattcctgagaaagatcccagatttttctgaatcagtcttaatctgattttgttttggctacacagttatgctgttatacctttgacatacataaaaatggtcattttatttcaatccagacagctcagcattgtacaaatgatggcagaaagatccatttgttcagactcagcttgctttgtttttaatactggggaataaaccaaaaaaaaaagtgtaatttttatcatttgtatccttcattctactttactggagtggaatccccagggccttcagataatctgggaagacctgactattcctgtgaggcaagcacagccctgctgagctttactcagaataatgcatgatagactcaacgtaattcccaggaaaaagcccagtcactccattcataactccctcataccaaccatcgtcattcttcttgatgacataaataatggctccttcctgaaaggacagctcatcttccttgtcttttgtatagtcataaattgccacaaccttttccaagtaagaacgtggagcccacggtgggtcctcttcagcataaggatcactatactcaaccacagcagcttcctcctcttcgtaatcttctggaggaggaggaggtgggggagactcatcaaagactggttcttccacaggtggcggtggaggtggtgtatctggattctggctataaaaaggtcctccattcatctgattctgaaggcttgtttgtgaagtaatggaaggagggcgtctatagggcaacgagccccctattgttgggggagtatggcgagaggcaggcctattcatgctgtagaactgtacaggatgacctgtagggggagtggaagaaacaacagggggagttggagaagtgaagccatcagcaagggtctgggcacccccagcagcagcgtctggggcagtggaggaagggacagtagcaggaacaagaggagcaggggcagatgcagaagtagcaggaaggggaggagtgccagcagagccagcaggggctggaaagacactgggaggagatggagtaggaacagcaataggaacccccacactaccacttccactgttctctcgactgctgctccgactacttgggtggctccctccactactcccactgccaagtgtccctttccctgacatagggggactagggggcttctgagttggaggtgttgtacgcggcagcccacccatcttcatgttctgggtactcaccttaaatctaagcaaccactttactccatgtccaatatcatctagaattgtatagtcaataggttttctaatataacgaactggtcgttcaaggttggctggagcaataatcttatgtgtccttgaagtgtttttattggtagtcaaaataccaatttctcttcttgcaactttctctttatgaatatcaactgtttgtgaaatatgattgattgaagattccatccttcgtagctgggatgcctggatatccagcatctgcaggacattgttggccaaggtgtttatcagataggcaacacttgctaaggattgggtggtgtaggctttggtttcttctagggctctctgcttatctgctgactgtagtcccagactactgagagactgaggcaggatgatcacttgagcacaggagttcaaggctgcagtgagctatgatcacaccactgcattccagcctgcatgacataccaagaccccatctctgtatgtagttgttctcgcagtaatcggccacccgttccagatttgtgtagctgtcgaagagggcccggcggccccccgggatttcctcttccagcagcatctgcagctccgccatcttcacatcctcctcctcctcctcctcatacaggtcgcagagggagcggcggccgcagcgccaaggaaacccaggaccgggagaggaggagcggcggcgacggcggcggtaactcggaagg

SEQ ID NO: 11862 - RNA, 3692 nt, Homo sapiens
  source 1..3692: mol_type = other RNA
ctgaatagctgggactacaggtgtgcgccaccacgcccagctaatttttgtgtttttagtagagatggggtttcaccatgttggccaggatggtctcaatttattgacctcatgatccacccacctcggcctccgaaagtgctgggattacaggcataagccaccacacccagcctgtgggaactatttattggatttcaaaacaccctctgcctcattaatccactaagctttctcagcaaaaagctgtttaaataaataatgggaacatctaatttaaaacagtttttctaattatagaccagtacacgaagaagagcttaacttatccaagtatagtctagtttgggtccataatggagctgaaggctcagaggacattcagggccattacactgcaggaaaacaaggaataagggatgtagaaatgacctaagaaaagcacgaagtggaatgtatactggaggcaagttaatgaaagctaataaatacaaagtgctgggaaaaatctaaaagcaaaatagctattgtaacttgcaatgcattaaaaacaactttaaaaccaaaaagtcttgataaggaaactctatagtggggtctcagttaaatgctgatgatttttaatgctcagataacattaagtggaatattaacttctgcatccgacaccatctgaattttctcacacactactacacttgttcacttttcaatcaagttccactttctgaacttgttcaaaacctcatttgaaatatatccagctactgcttttcccctttcacctagcacagggcagttacctggcaaagctctattctggccaagtcactgggactgagtagaacccacgttagcagctctggacctgaacaggagctggcccaacatcacagtgaccacccacaaagagacaagccctcctggatttttttcagcatttcttatactgactacagtagtgatgattaaagttatctgccctacagactccactgaatttgaagctgtatttattgtacagatgggggaaatgtgttttattgtgtcagttatattaatttttatcaatgtgattagatacatattttggcctattaatcttattcattatattcttagtctgagatgggttttaattctgactaacagcagctacttaagagtccaatcatacaaaatcaggagagtattaccctttctacagctaagcgagtcagtaatacagcagcaactaatactggccattaataacgtccagagagcacattagcaaaccttgtactcccagtgactgtcaggagacttgaaaataactactattctcttccaaagtagaatagcgtttttctagatagtgaaggaaatgatagtcatagttggtctgaactccaagatcctactcctcaaaacagcaccgaagcaggggttcgggatgcctgctaagagcatttccacagttcaagtctcttcagaaccttagggaccttcgtgtctagcttcacacacccacctccacatatgaaccagcctaccacacttcacatctgggtacactggccattagcaacaatgcagtctcatgcagcagcacattaaaatcaaacgggtggcaatcgttcaccaccctcagagtgttgggagactttcacatttcatcatccttataatccacaaacagaaacatgaagggatgcaagtgagttcagcattcactcgtttggtgcactcaagtgctgagagaatgcagaatttacagtgtcacagaggaaaaaagccatctgaaataattgtaaaaatggttaagtgtggtatttaaatgttggttccctcctcttcatacaagtggaagaaaagaaggggctagggtacccactgggccatgaggttaaccccttagcacaggcaatgaagaacatccaatgccacagattctgcaggaggagaaatcccaagggtatacagtattcctgagaaagatcccagatttttctgaatcagtcttaatctgattttgttttggctacacagttatgctgttatacctttgacatacataaaaatggtcattttatttcaatccagacagctcagcattgtacaaatgatggcagaaagatccatttgttcagactcagcttgctttgtttttaatactggggaataaaccaaaaaaaaaagtgtaatttttatcatttgtatccttcattctactttactggagtggaatccccagggccttcagataatctgggaagacctgactattcctgtgaggcaagcacagccctgctgagctttactcagaataatgcatgatagactcaacgtaattcccaggaaaaagcccagtcactccattcataactccctcataccaaccatcgtcattcttcttgatgacataaataatggctccttcctgaaaggacagctcatcttccttgtcttttgtatagtcataaattgccacaaccttttccaagtaagaacgtggagcccacggtgggtcctcttcagcataaggatcactatactcaaccacagcagcttcctcctcttcgtaatcttctggaggaggaggaggtgggggagactcatcaaagactggttcttccacaggtggcggtggaggtggtgtattattttcttggactctggccacaaatcccattaaaggtaactgaggagttacctgtaggatggagggaggaggaggagcaagagatactggattctggctataaaaaggtcctccattcatctgattctgaaggcttgtttgtgaagtaatggaaggagggcgtctatagggcaacgagccccctattgttgggggagtatggcgagaggcaggcctattcatgctgtagaactgtacaggatgacctggaaagacactgggaggagatggagtaggaacagcaataggaacccccacactaccacttccactgttctctcgactgctgctccgactacttgggtggctccctccactactcccactgccaagtgtccctttccctgacatagggggactagggggcttctgagttggaggtgttgtacgcggcagcccacccatcttcatgttctgggtactcacctttactccatgtccaatatcatctagaattgtatagtcaataggttttctaatataacgaactggtcgttcaaggttggctggagcaataatcttatgtgtccttgaagtgtttttattggtagtcaaaataccaatttctcttcttgcaactttctctttatgaatatcaactgtttgtgaaatatgattgattgaagattccatccttcgtagctgggatgcctggatatccagcatctgcaggacattgttggccaaggtgtttatcagataggcaacacttgctaaggattgggtggtgtaggctttggtttcttctagggctctctgcttatctgctgactgtatgtagttgttctcgcagtaatcggccacccgttccagatttgtgtagctgtcgaagagggcccggcggccccccgggatttcctcttccagcagcatctgcagctccgccatcttcacatcctcctcctcctcctcctcatacaggtcgcagagggagcggcggccgcagcgccaaggaaacccaggaccgggagaggaggagcggcggcgacggcggcggtaactcggaagg

SEQ ID NO: 11863 - RNA, 3695 nt, Homo sapiens
  source 1..3695: mol_type = other RNA
ctgaatagctgggactacaggtgtgcgccaccacgcccagctaatttttgtgtttttagtagagatggggtttcaccatgttggccaggatggtctcaatttattgacctcatgatccacccacctcggcctccgaaagtgctgggattacaggcataagccaccacacccagcctgtgggaactatttattggatttcaaaacaccctctgcctcattaatccactaagctttctcagcaaaaagctgtttaaataaataatgggaacatctaatttaaaacagtttttctaattatagaccagtacacgaagaagagcttaacttatccaagtatagtctagtttgggtccataatggagctgaaggctcagaggacattcagggccattacactgcaggaaaacaaggaataagggatgtagaaatgacctaagaaaagcacgaagtggaatgtatactggaggcaagttaatgaaagctaataaatacaaagtgctgggaaaaatctaaaagcaaaatagctattgtaacttgcaatgcattaaaaacaactttaaaaccaaaaagtcttgataaggaaactctatagtggggtctcagttaaatgctgatgatttttaatgctcagataacattaagtggaatattaacttctgcatccgacaccatctgaattttctcacacactactacacttgttcacttttcaatcaagttccactttctgaacttgttcaaaacctcatttgaaatatatccagctactgcttttcccctttcacctagcacagggcagttacctggcaaagctctattctggccaagtcactgggactgagtagaacccacgttagcagctctggacctgaacaggagctggcccaacatcacagtgaccacccacaaagagacaagccctcctggatttttttcagcatttcttatactgactacagtagtgatgattaaagttatctgccctacagactccactgaatttgaagctgtatttattgtacagatgggggaaatgtgttttattgtgtcagttatattaatttttatcaatgtgattagatacatattttggcctattaatcttattcattatattcttagtctgagatgggttttaattctgactaacagcagctacttaagagtccaatcatacaaaatcaggagagtattaccctttctacagctaagcgagtcagtaatacagcagcaactaatactggccattaataacgtccagagagcacattagcaaaccttgtactcccagtgactgtcaggagacttgaaaataactactattctcttccaaagtagaatagcgtttttctagatagtgaaggaaatgatagtcatagttggtctgaactccaagatcctactcctcaaaacagcaccgaagcaggggttcgggatgcctgctaagagcatttccacagttcaagtctcttcagaaccttagggaccttcgtgtctagcttcacacacccacctccacatatgaaccagcctaccacacttcacatctgggtacactggccattagcaacaatgcagtctcatgcagcagcacattaaaatcaaacgggtggcaatcgttcaccaccctcagagtgttgggagactttcacatttcatcatccttataatccacaaacagaaacatgaagggatgcaagtgagttcagcattcactcgtttggtgcactcaagtgctgagagaatgcagaatttacagtgtcacagaggaaaaaagccatctgaaataattgtaaaaatggttaagtgtggtatttaaatgttggttccctcctcttcatacaagtggaagaaaagaaggggctagggtacccactgggccatgaggttaaccccttagcacaggcaatgaagaacatccaatgccacagattctgcaggaggagaaatcccaagggtatacagtattcctgagaaagatcccagatttttctgaatcagtcttaatctgattttgttttggctacacagttatgctgttatacctttgacatacataaaaatggtcattttatttcaatccagacagctcagcattgtacaaatgatggcagaaagatccatttgttcagactcagcttgctttgtttttaatactggggaataaaccaaaaaaaaaagtgtaatttttatcatttgtatccttcattctactttactggagtggaatccccagggccttcagataatctgggaagacctgactattcctgtgaggcaagcacagccctgctgagctttactcagaataatgcatgatagactcaacgtaattcccaggaaaaagcccagtcactccattcataactccctcataccaaccatcgtcattcttcttgatgacataaataatggctccttcctgaaaggacagctcatcttccttgtcttttgtatagtcataaattgccacaaccttttccaagtaagaacgtggagcccacggtgggtcctcttcagcataaggatcactatactcaaccacagcagcttcctcctcttcgtaatcttctggaggaggaggaggtgggggagactcatcaaagactggttcttccacaggtggcggtggaggtggtgtattattttcttggactctggccacaaatcccattaaaggtaactgaggagttacctgtaggatggagggaggaggaggagcaagagatactggattctggctataaaaaggtcctccattcatctgattctgaaggcttgtttgtgaagtaatggaaggagggcgtctatagggcaacgagccccctattgttgggggagtatggcgagaggcaggcctattcatgctgtagaactgtacaggatgacctggaaagacactgggaggagatggagtaggaacagcaataggaacccccacactaccacttccactgttctctcgactgctgctccgactacttgggtggctccctccactactcccactgctgccaagtgtccctttccctgacatagggggactagggggcttctgagttggaggtgttgtacgcggcagcccacccatcttcatgttctgggtactcacctttactccatgtccaatatcatctagaattgtatagtcaataggttttctaatataacgaactggtcgttcaaggttggctggagcaataatcttatgtgtccttgaagtgtttttattggtagtcaaaataccaatttctcttcttgcaactttctctttatgaatatcaactgtttgtgaaatatgattgattgaagattccatccttcgtagctgggatgcctggatatccagcatctgcaggacattgttggccaaggtgtttatcagataggcaacacttgctaaggattgggtggtgtaggctttggtttcttctagggctctctgcttatctgctgactgtatgtagttgttctcgcagtaatcggccacccgttccagatttgtgtagctgtcgaagagggcccggcggccccccgggatttcctcttccagcagcatctgcagctccgccatcttcacatcctcctcctcctcctcctcatacaggtcgcagagggagcggcggccgcagcgccaaggaaacccaggaccgggagaggaggagcggcggcgacggcggcggtaactcggaagg

SEQ ID NO: 11864 - RNA, 3674 nt, Homo sapiens
  source 1..3674: mol_type = other RNA
ctgaatagctgggactacaggtgtgcgccaccacgcccagctaatttttgtgtttttagtagagatggggtttcaccatgttggccaggatggtctcaatttattgacctcatgatccacccacctcggcctccgaaagtgctgggattacaggcataagccaccacacccagcctgtgggaactatttattggatttcaaaacaccctctgcctcattaatccactaagctttctcagcaaaaagctgtttaaataaataatgggaacatctaatttaaaacagtttttctaattatagaccagtacacgaagaagagcttaacttatccaagtatagtctagtttgggtccataatggagctgaaggctcagaggacattcagggccattacactgcaggaaaacaaggaataagggatgtagaaatgacctaagaaaagcacgaagtggaatgtatactggaggcaagttaatgaaagctaataaatacaaagtgctgggaaaaatctaaaagcaaaatagctattgtaacttgcaatgcattaaaaacaactttaaaaccaaaaagtcttgataaggaaactctatagtggggtctcagttaaatgctgatgatttttaatgctcagataacattaagtggaatattaacttctgcatccgacaccatctgaattttctcacacactactacacttgttcacttttcaatcaagttccactttctgaacttgttcaaaacctcatttgaaatatatccagctactgcttttcccctttcacctagcacagggcagttacctggcaaagctctattctggccaagtcactgggactgagtagaacccacgttagcagctctggacctgaacaggagctggcccaacatcacagtgaccacccacaaagagacaagccctcctggatttttttcagcatttcttatactgactacagtagtgatgattaaagttatctgccctacagactccactgaatttgaagctgtatttattgtacagatgggggaaatgtgttttattgtgtcagttatattaatttttatcaatgtgattagatacatattttggcctattaatcttattcattatattcttagtctgagatgggttttaattctgactaacagcagctacttaagagtccaatcatacaaaatcaggagagtattaccctttctacagctaagcgagtcagtaatacagcagcaactaatactggccattaataacgtccagagagcacattagcaaaccttgtactcccagtgactgtcaggagacttgaaaataactactattctcttccaaagtagaatagcgtttttctagatagtgaaggaaatgatagtcatagttggtctgaactccaagatcctactcctcaaaacagcaccgaagcaggggttcgggatgcctgctaagagcatttccacagttcaagtctcttcagaaccttagggaccttcgtgtctagcttcacacacccacctccacatatgaaccagcctaccacacttcacatctgggtacactggccattagcaacaatgcagtctcatgcagcagcacattaaaatcaaacgggtggcaatcgttcaccaccctcagagtgttgggagactttcacatttcatcatccttataatccacaaacagaaacatgaagggatgcaagtgagttcagcattcactcgtttggtgcactcaagtgctgagagaatgcagaatttacagtgtcacagaggaaaaaagccatctgaaataattgtaaaaatggttaagtgtggtatttaaatgttggttccctcctcttcatacaagtggaagaaaagaaggggctagggtacccactgggccatgaggttaaccccttagcacaggcaatgaagaacatccaatgccacagattctgcaggaggagaaatcccaagggtatacagtattcctgagaaagatcccagatttttctgaatcagtcttaatctgattttgttttggctacacagttatgctgttatacctttgacatacataaaaatggtcattttatttcaatccagacagctcagcattgtacaaatgatggcagaaagatccatttgttcagactcagcttgctttgtttttaatactggggaataaaccaaaaaaaaaagtgtaatttttatcatttgtatccttcattctactttactggagtggaatccccagggccttcagataatctgggaagacctgactattcctgtgaggcaagcacagccctgctgagctttactcagaataatgcatgatagactcaacgtaattcccaggaaaaagcccagtcactccattcataactccctcataccaaccatcgtcattcttcttgatgacataaataatggctccttcctgaaaggacagctcatcttccttgtcttttgtatagtcataaattgccacaaccttttccaagtaagaacgtggagcccacggtgggtcctcttcagcataaggatcactatactcaaccacagcagcttcctcctcttcgtaatcttctggaggaggaggaggtgggggagactcatcaaagactggttcttccacaggtggcggtggaggtggtgtattattttcttggactctggccacaaatcccattaaaggtaactgaggagttacctgtaggatggagggaggaggaggagcaagagatactggattctggctataaaaaggtcctccattcatctgattctgaaggcttgtttgtgaagtaatggaaggagggcgtctatagggcaacgagccccctattgttgggggagtatggcgagaggcaggcctattcatgctgtagaactgtacaggatgacctggaaagacactgggaggagatggagtaggaacagcaataggaacccccacactaccacttccactgttctctcgactgctgctccgactacttgggtggctccctccactactcccactgctgctgtaagttcgatttctttgattcacagaagctgtcctcacagggctctgctgcgagggagccatattacgggttgggctaggtacgtaatcatttggtaccactggaggacgcactggctccagtgtgcgatagggggagtgccgcccaagtgtccctttccctgacatagggggactagggggcttctgagttggaggtgttgtacgcggcagcccacccatcttcatgttctgggtactcacctttactccatgtccaatatcatctagaattgtatagtcaataggttttctaatataacgaactggtcgttcaaggttggctggagcaataatcttatgtgtccttgaagtgtttttattggtagtcaaaataccaatttctcttcttgcaactttctctttatgaatatcaactgtctgtatgtagttgttctcgcagtaatcggccacccgttccagatttgtgtagctgtcgaagagggcccggcggccccccgggatttcctcttccagcagcatctgcagctccgccatcttcacatcctcctcctcctcctcctcatacaggtcgcagagggagcggcggccgcagcgccaaggaaacccaggaccgggagaggaggagcggcggcgacggcggcggtaactcggaagg

SEQ ID NO: 11865 - RNA, 3842 nt, Homo sapiens
  source 1..3842: mol_type = other RNA
ctgaatagctgggactacaggtgtgcgccaccacgcccagctaatttttgtgtttttagtagagatggggtttcaccatgttggccaggatggtctcaatttattgacctcatgatccacccacctcggcctccgaaagtgctgggattacaggcataagccaccacacccagcctgtgggaactatttattggatttcaaaacaccctctgcctcattaatccactaagctttctcagcaaaaagctgtttaaataaataatgggaacatctaatttaaaacagtttttctaattatagaccagtacacgaagaagagcttaacttatccaagtatagtctagtttgggtccataatggagctgaaggctcagaggacattcagggccattacactgcaggaaaacaaggaataagggatgtagaaatgacctaagaaaagcacgaagtggaatgtatactggaggcaagttaatgaaagctaataaatacaaagtgctgggaaaaatctaaaagcaaaatagctattgtaacttgcaatgcattaaaaacaactttaaaaccaaaaagtcttgataaggaaactctatagtggggtctcagttaaatgctgatgatttttaatgctcagataacattaagtggaatattaacttctgcatccgacaccatctgaattttctcacacactactacacttgttcacttttcaatcaagttccactttctgaacttgttcaaaacctcatttgaaatatatccagctactgcttttcccctttcacctagcacagggcagttacctggcaaagctctattctggccaagtcactgggactgagtagaacccacgttagcagctctggacctgaacaggagctggcccaacatcacagtgaccacccacaaagagacaagccctcctggatttttttcagcatttcttatactgactacagtagtgatgattaaagttatctgccctacagactccactgaatttgaagctgtatttattgtacagatgggggaaatgtgttttattgtgtcagttatattaatttttatcaatgtgattagatacatattttggcctattaatcttattcattatattcttagtctgagatgggttttaattctgactaacagcagctacttaagagtccaatcatacaaaatcaggagagtattaccctttctacagctaagcgagtcagtaatacagcagcaactaatactggccattaataacgtccagagagcacattagcaaaccttgtactcccagtgactgtcaggagacttgaaaataactactattctcttccaaagtagaatagcgtttttctagatagtgaaggaaatgatagtcatagttggtctgaactccaagatcctactcctcaaaacagcaccgaagcaggggttcgggatgcctgctaagagcatttccacagttcaagtctcttcagaaccttagggaccttcgtgtctagcttcacacacccacctccacatatgaaccagcctaccacacttcacatctgggtacactggccattagcaacaatgcagtctcatgcagcagcacattaaaatcaaacgggtggcaatcgttcaccaccctcagagtgttgggagactttcacatttcatcatccttataatccacaaacagaaacatgaagggatgcaagtgagttcagcattcactcgtttggtgcactcaagtgctgagagaatgcagaatttacagtgtcacagaggaaaaaagccatctgaaataattgtaaaaatggttaagtgtggtatttaaatgttggttccctcctcttcatacaagtggaagaaaagaaggggctagggtacccactgggccatgaggttaaccccttagcacaggcaatgaagaacatccaatgccacagattctgcaggaggagaaatcccaagggtatacagtattcctgagaaagatcccagatttttctgaatcagtcttaatctgattttgttttggctacacagttatgctgttatacctttgacatacataaaaatggtcattttatttcaatccagacagctcagcattgtacaaatgatggcagaaagatccatttgttcagactcagcttgctttgtttttaatactggggaataaaccaaaaaaaaaagtgtaatttttatcatttgtatccttcattctactttactggagtggaatccccagggccttcagataatctgggaagacctgactattcctgtgaggcaagcacagccctgctgagctttactcagaataatgcatgatagactcaacgtaattcccaggaaaaagcccagtcactccattcataactccctcataccaaccatcgtcattcttcttgatgacataaataatggctccttcctgaaaggacagctcatcttccttgtcttttgtatagtcataaattgccacaaccttttccaagtaagaacgtggagcccacggtgggtcctcttcagcataaggatcactatactcaaccacagcagcttcctcctcttcgtaatcttctggaggaggaggaggtgggggagactcatcaaagactggttcttccacaggtggcggtggaggtggtgtattattttcttggactctggccacaaatcccattaaaggtaactgaggagttacctgtaggatggagggaggaggaggagcaagagatactggattctggctataaaaaggtcctccattcatctgattctgaaggcttgtttgtgaagtaatggaaggagggcgtctatagggcaacgagccccctattgttgggggagtatggcgagaggcaggcctattcatgctgtagaactgtacaggatgacctggaaagacactgggaggagatggagtaggaacagcaataggaacccccacactaccacttccactgttctctcgactgctgctccgactacttgggtggctccctccactactcccactgctgctgtaagttcgatttctttgattcacagaagctgtcctcacagggctctgctgcgagggagccatattacgggttgggctaggtacgtaatcatttggtaccactggaggacgcactggctccagtgtgcgatagggggagtgccgcccaagtgtccctttccctgacatagggggactagggggcttctgagttggaggtgttgtacgcggcagcccacccatcttcatgttctgggtactcacctttactccatgtccaatatcatctagaattgtatagtcaataggttttctaatataacgaactggtcgttcaaggttggctggagcaataatcttatgtgtccttgaagtgtttttattggtagtcaaaataccaatttctcttcttgcaactttctctttatgaatatcaactgtttgtgaaatatgattgattgaagattccatccttcgtagctgggatgcctggatatccagcatctgcaggacattgttggccaaggtgtttatcagataggcaacacttgctaaggattgggtggtgtaggctttggtttcttctagggctctctgcttatctgctgactgtatgtagttgttctcgcagtaatcggccacccgttccagatttgtgtagctgtcgaagagggcccggcggccccccgggatttcctcttccagcagcatctgcagctccgccatcttcacatcctcctcctcctcctcctcatacaggtcgcagagggagcggcggccgcagcgccaaggaaacccaggaccgggagaggaggagcggcggcgacggcggcggtaactcggaagg

SEQ ID NO: 11866 - RNA, 3838 nt, Homo sapiens
  source 1..3838: mol_type = other RNA
ctgaatagctgggactacaggtgtgcgccaccacgcccagctaatttttgtgtttttagtagagatggggtttcaccatgttggccaggatggtctcaatttattgacctcatgatccacccacctcggcctccgaaagtgctgggattacaggcataagccaccacacccagcctgtgggaactatttattggatttcaaaacaccctctgcctcattaatccactaagctttctcagcaaaaagctgtttaaataaataatgggaacatctaatttaaaacagtttttctaattatagaccagtacacgaagaagagcttaacttatccaagtatagtctagtttgggtccataatggagctgaaggctcagaggacattcagggccattacactgcaggaaaacaaggaataagggatgtagaaatgacctaagaaaagcacgaagtggaatgtatactggaggcaagttaatgaaagctaataaatacaaagtgctgggaaaaatctaaaagcaaaatagctattgtaacttgcaatgcattaaaaacaactttaaaaccaaaaagtcttgataaggaaactctatagtggggtctcagttaaatgctgatgatttttaatgctcagataacattaagtggaatattaacttctgcatccgacaccatctgaattttctcacacactactacacttgttcacttttcaatcaagttccactttctgaacttgttcaaaacctcatttgaaatatatccagctactgcttttcccctttcacctagcacagggcagttacctggcaaagctctattctggccaagtcactgggactgagtagaacccacgttagcagctctggacctgaacaggagctggcccaacatcacagtgaccacccacaaagagacaagccctcctggatttttttcagcatttcttatactgactacagtagtgatgattaaagttatctgccctacagactccactgaatttgaagctgtatttattgtacagatgggggaaatgtgttttattgtgtcagttatattaatttttatcaatgtgattagatacatattttggcctattaatcttattcattatattcttagtctgagatgggttttaattctgactaacagcagctacttaagagtccaatcatacaaaatcaggagagtattaccctttctacagctaagcgagtcagtaatacagcagcaactaatactggccattaataacgtccagagagcacattagcaaaccttgtactcccagtgactgtcaggagacttgaaaataactactattctcttccaaagtagaatagcgtttttctagatagtgaaggaaatgatagtcatagttggtctgaactccaagatcctactcctcaaaacagcaccgaagcaggggttcgggatgcctgctaagagcatttccacagttcaagtctcttcagaaccttagggaccttcgtgtctagcttcacacacccacctccacatatgaaccagcctaccacacttcacatctgggtacactggccattagcaacaatgcagtctcatgcagcagcacattaaaatcaaacgggtggcaatcgttcaccaccctcagagtgttgggagactttcacatttcatcatccttataatccacaaacagaaacatgaagggatgcaagtgagttcagcattcactcgtttggtgcactcaagtgctgagagaatgcagaatttacagtgtcacagaggaaaaaagccatctgaaataattgtaaaaatggttaagtgtggtatttaaatgttggttccctcctcttcatacaagtggaagaaaagaaggggctagggtacccactgggccatgaggttaaccccttagcacaggcaatgaagaacatccaatgccacagattctgcaggaggagaaatcccaagggtatacagtattcctgagaaagatcccagatttttctgaatcagtcttaatctgattttgttttggctacacagttatgctgttatacctttgacatacataaaaatggtcattttatttcaatccagacagctcagcattgtacaaatgatggcagaaagatccatttgttcagactcagcttgctttgtttttaatactggggaataaaccaaaaaaaaaagtgtaatttttatcatttgtatccttcattctactttactggagtggaatccccagggccttcagataatctgggaagacctgactattcctgtgaggcaagcacagccctgctgagctttactcagaataatgcatgatagactcaacgtaattcccaggaaaaagcccagtcactccattcataactccctcataccaaccatcgtcattcttcttgatgacataaataatggctccttcctgaaaggacagctcatcttccttgtcttttgtatagtcataaattgccacaaccttttccaagtaagaacgtggagcccacggtgggtcctcttcagcataaggatcactatactcaaccacagcagcttcctcctcttcgtaatcttctggaggaggaggaggtgggggagactcatcaaagactggttcttccacaggtggcggtggaggtggtgtattattttcttggactctggccacaaatcccattaaaggtaactgaggagttacctgtaggatggagggaggaggaggagcaagagatactggattctggctataaaaaggtcctccattcatctgattctgaaggcttgtttgtgaagtaatggaaggagggcgtctatagggcaacgagccccctattgttgggggagtatggcgagaggcaggcctattcatgctgtagaactgtacaggatgacctggaaagacactgggaggagatggagtaggaacagcaataggaacccccacactaccacttccactgttctctcgactgctgctccgactacttgggtggctccctccactactcccactgctgctgtaagttcgatttctttgattcacagaagctgtcctcacagggctctgctgcgagggagccatattacgggttgggctaggtacgtaatcatttggtaccactggaggacgcactggctccagtgtgcgatagggggagtgccgcccaagtgtccctttccctgacatagggggactagggggcttctgagttggaggtgttgtacgcggcagcccacccatcttcatgttctgggtactcacctttactccatgtccaatatcatctagaattgtatagtcaataggttttctaatataacgaactggtcgttcaaggttggctggagcaataatcttatgtgtccttgaagtgtttttattggtagtcaaaataccaatttctcttcttgcaactttctctttatgaatatcaactgtttgtgaaatatgattgattgaagattccatccttcgtagctgggatgcctggatatccagcatctgcaggacattgttggccaaggtgtttatcagataggcaacacttgctaaggattgggtggtgtaggctttggtttcttctagggctctctgcttatctgctgtatgtagttgttctcgcagtaatcggccacccgttccagatttgtgtagctgtcgaagagggcccggcggccccccgggatttcctcttccagcagcatctgcagctccgccatcttcacatcctcctcctcctcctcctcatacaggtcgcagagggagcggcggccgcagcgccaaggaaacccaggaccgggagaggaggagcggcggcgacggcggcggtaactcggaagg

SEQ ID NO: 11867 - RNA, 3839 nt, Homo sapiens
  source 1..3839: mol_type = other RNA
ctgaatagctgggactacaggtgtgcgccaccacgcccagctaatttttgtgtttttagtagagatggggtttcaccatgttggccaggatggtctcaatttattgacctcatgatccacccacctcggcctccgaaagtgctgggattacaggcataagccaccacacccagcctgtgggaactatttattggatttcaaaacaccctctgcctcattaatccactaagctttctcagcaaaaagctgtttaaataaataatgggaacatctaatttaaaacagtttttctaattatagaccagtacacgaagaagagcttaacttatccaagtatagtctagtttgggtccataatggagctgaaggctcagaggacattcagggccattacactgcaggaaaacaaggaataagggatgtagaaatgacctaagaaaagcacgaagtggaatgtatactggaggcaagttaatgaaagctaataaatacaaagtgctgggaaaaatctaaaagcaaaatagctattgtaacttgcaatgcattaaaaacaactttaaaaccaaaaagtcttgataaggaaactctatagtggggtctcagttaaatgctgatgatttttaatgctcagataacattaagtggaatattaacttctgcatccgacaccatctgaattttctcacacactactacacttgttcacttttcaatcaagttccactttctgaacttgttcaaaacctcatttgaaatatatccagctactgcttttcccctttcacctagcacagggcagttacctggcaaagctctattctggccaagtcactgggactgagtagaacccacgttagcagctctggacctgaacaggagctggcccaacatcacagtgaccacccacaaagagacaagccctcctggatttttttcagcatttcttatactgactacagtagtgatgattaaagttatctgccctacagactccactgaatttgaagctgtatttattgtacagatgggggaaatgtgttttattgtgtcagttatattaatttttatcaatgtgattagatacatattttggcctattaatcttattcattatattcttagtctgagatgggttttaattctgactaacagcagctacttaagagtccaatcatacaaaatcaggagagtattaccctttctacagctaagcgagtcagtaatacagcagcaactaatactggccattaataacgtccagagagcacattagcaaaccttgtactcccagtgactgtcaggagacttgaaaataactactattctcttccaaagtagaatagcgtttttctagatagtgaaggaaatgatagtcatagttggtctgaactccaagatcctactcctcaaaacagcaccgaagcaggggttcgggatgcctgctaagagcatttccacagttcaagtctcttcagaaccttagggaccttcgtgtctagcttcacacacccacctccacatatgaaccagcctaccacacttcacatctgggtacactggccattagcaacaatgcagtctcatgcagcagcacattaaaatcaaacgggtggcaatcgttcaccaccctcagagtgttgggagactttcacatttcatcatccttataatccacaaacagaaacatgaagggatgcaagtgagttcagcattcactcgtttggtgcactcaagtgctgagagaatgcagaatttacagtgtcacagaggaaaaaagccatctgaaataattgtaaaaatggttaagtgtggtatttaaatgttggttccctcctcttcatacaagtggaagaaaagaaggggctagggtacccactgggccatgaggttaaccccttagcacaggcaatgaagaacatccaatgccacagattctgcaggaggagaaatcccaagggtatacagtattcctgagaaagatcccagatttttctgaatcagtcttaatctgattttgttttggctacacagttatgctgttatacctttgacatacataaaaatggtcattttatttcaatccagacagctcagcattgtacaaatgatggcagaaagatccatttgttcagactcagcttgctttgtttttaatactggggaataaaccaaaaaaaaaagtgtaatttttatcatttgtatccttcattctactttactggagtggaatccccagggccttcagataatctgggaagacctgactattcctgtgaggcaagcacagccctgctgagctttactcagaataatgcatgatagactcaacgtaattcccaggaaaaagcccagtcactccattcataactccctcataccaaccatcgtcattcttcttgatgacataaataatggctccttcctgaaaggacagctcatcttccttgtcttttgtatagtcataaattgccacaaccttttccaagtaagaacgtggagcccacggtgggtcctcttcagcataaggatcactatactcaaccacagcagcttcctcctcttcgtaatcttctggaggaggaggaggtgggggagactcatcaaagactggttcttccacaggtggcggtggaggtggtgtattattttcttggactctggccacaaatcccattaaaggtaactgaggagttacctgtaggatggagggaggaggaggagcaagagatactggattctggctataaaaaggtcctccattcatctgattctgaaggcttgtttgtgaagtaatggaaggagggcgtctatagggcaacgagccccctattgttgggggagtatggcgagaggcaggcctattcatgctgtagaactgtacaggatgacctggaaagacactgggaggagatggagtaggaacagcaataggaacccccacactaccacttccactgttctctcgactgctgctccgactacttgggtggctccctccactactcccactgctgtaagttcgatttctttgattcacagaagctgtcctcacagggctctgctgcgagggagccatattacgggttgggctaggtacgtaatcatttggtaccactggaggacgcactggctccagtgtgcgatagggggagtgccgcccaagtgtccctttccctgacatagggggactagggggcttctgagttggaggtgttgtacgcggcagcccacccatcttcatgttctgggtactcacctttactccatgtccaatatcatctagaattgtatagtcaataggttttctaatataacgaactggtcgttcaaggttggctggagcaataatcttatgtgtccttgaagtgtttttattggtagtcaaaataccaatttctcttcttgcaactttctctttatgaatatcaactgtttgtgaaatatgattgattgaagattccatccttcgtagctgggatgcctggatatccagcatctgcaggacattgttggccaaggtgtttatcagataggcaacacttgctaaggattgggtggtgtaggctttggtttcttctagggctctctgcttatctgctgactgtatgtagttgttctcgcagtaatcggccacccgttccagatttgtgtagctgtcgaagagggcccggcggccccccgggatttcctcttccagcagcatctgcagctccgccatcttcacatcctcctcctcctcctcctcatacaggtcgcagagggagcggcggccgcagcgccaaggaaacccaggaccgggagaggaggagcggcggcgacggcggcggtaactcggaagg

SEQ ID NO: 11868 - RNA, 3896 nt, Homo sapiens
  source 1..3896: mol_type = other RNA
ctgaatagctgggactacaggtgtgcgccaccacgcccagctaatttttgtgtttttagtagagatggggtttcaccatgttggccaggatggtctcaatttattgacctcatgatccacccacctcggcctccgaaagtgctgggattacaggcataagccaccacacccagcctgtgggaactatttattggatttcaaaacaccctctgcctcattaatccactaagctttctcagcaaaaagctgtttaaataaataatgggaacatctaatttaaaacagtttttctaattatagaccagtacacgaagaagagcttaacttatccaagtatagtctagtttgggtccataatggagctgaaggctcagaggacattcagggccattacactgcaggaaaacaaggaataagggatgtagaaatgacctaagaaaagcacgaagtggaatgtatactggaggcaagttaatgaaagctaataaatacaaagtgctgggaaaaatctaaaagcaaaatagctattgtaacttgcaatgcattaaaaacaactttaaaaccaaaaagtcttgataaggaaactctatagtggggtctcagttaaatgctgatgatttttaatgctcagataacattaagtggaatattaacttctgcatccgacaccatctgaattttctcacacactactacacttgttcacttttcaatcaagttccactttctgaacttgttcaaaacctcatttgaaatatatccagctactgcttttcccctttcacctagcacagggcagttacctggcaaagctctattctggccaagtcactgggactgagtagaacccacgttagcagctctggacctgaacaggagctggcccaacatcacagtgaccacccacaaagagacaagccctcctggatttttttcagcatttcttatactgactacagtagtgatgattaaagttatctgccctacagactccactgaatttgaagctgtatttattgtacagatgggggaaatgtgttttattgtgtcagttatattaatttttatcaatgtgattagatacatattttggcctattaatcttattcattatattcttagtctgagatgggttttaattctgactaacagcagctacttaagagtccaatcatacaaaatcaggagagtattaccctttctacagctaagcgagtcagtaatacagcagcaactaatactggccattaataacgtccagagagcacattagcaaaccttgtactcccagtgactgtcaggagacttgaaaataactactattctcttccaaagtagaatagcgtttttctagatagtgaaggaaatgatagtcatagttggtctgaactccaagatcctactcctcaaaacagcaccgaagcaggggttcgggatgcctgctaagagcatttccacagttcaagtctcttcagaaccttagggaccttcgtgtctagcttcacacacccacctccacatatgaaccagcctaccacacttcacatctgggtacactggccattagcaacaatgcagtctcatgcagcagcacattaaaatcaaacgggtggcaatcgttcaccaccctcagagtgttgggagactttcacatttcatcatccttataatccacaaacagaaacatgaagggatgcaagtgagttcagcattcactcgtttggtgcactcaagtgctgagagaatgcagaatttacagtgtcacagaggaaaaaagccatctgaaataattgtaaaaatggttaagtgtggtatttaaatgttggttccctcctcttcatacaagtggaagaaaagaaggggctagggtacccactgggccatgaggttaaccccttagcacaggcaatgaagaacatccaatgccacagattctgcaggaggagaaatcccaagggtatacagtattcctgagaaagatcccagatttttctgaatcagtcttaatctgattttgttttggctacacagttatgctgttatacctttgacatacataaaaatggtcattttatttcaatccagacagctcagcattgtacaaatgatggcagaaagatccatttgttcagactcagcttgctttgtttttaatactggggaataaaccaaaaaaaaaagtgtaatttttatcatttgtatccttcattctactttactggagtggaatccccagggccttcagataatctgggaagacctgactattcctgtgaggcaagcacagccctgctgagctttactcagaataatgcatgatagactcaacgtaattcccaggaaaaagcccagtcactccattcataactccctcataccaaccatcgtcattcttcttgatgacataaataatggctccttcctgaaaggacagctcatcttccttgtcttttgtatagtcataaattgccacaaccttttccaagtaagaacgtggagcccacggtgggtcctcttcagcataaggatcactatactcaaccacagcagcttcctcctcttcgtaatcttctggaggaggaggaggtgggggagactcatcaaagactggttcttccacaggtggcggtggaggtggtgtattattttcttggactctggccacaaatcccattaaaggtaactgaggagttacctgtaggatggagggaggaggaggagcaagagatactggattctggctataaaaaggtcctccattcatctgattctgaaggcttgtttgtgaagtaatggaaggagggcgtctatagggcaacgagccccctattgttgggggagtatggcgagaggcaggcctattcatgctgtagaactgtacaggatgacctgtagggggagtggaagaaacaacagggggagttggagaagtgaagccatcagcaagggtctgggcacccccagcagcagcgtctggggcagtggaggaagggacagtagcaggaacaagaggagcaggggcagatgcagaagtagcaggaaggggaggagtgccagcagagccagcaggggctggaaagacactgggaggagatggagtaggaacagcaataggaacccccacactaccacttccactgttctctcgactgctgctccgactacttgggtggctccctccactactcccactgctgccaagtgtccctttccctgacatagggggactagggggcttctgagttggaggtgttgtacgcggcagcccacccatcttcatgttctgggtactcaccttaaatctaagcaaccactttactccatgtccaatatcatctagaattgtatagtcaataggttttctaatataacgaactggtcgttcaaggttggctggagcaataatcttatgtgtccttgaagtgtttttattggtagtcaaaataccaatttctcttcttgcaactttctctttatgaatatcaactgtttgtgaaatatgattgattgaagattccatccttcgtagctgggatgcctggatatccagcatctgcaggacattgttggccaaggtgtttatcagataggcaacacttgctaaggattgggtggtgtaggctttggtttcttctagggctctctgcttatctgctgactgtatgtagttgttctcgcagtaatcggccacccgttccagatttgtgtagctgtcgaagagggcccggcggccccccgggatttcctcttccagcagcatctgcagctccgccatcttcacatcctcctcctcctcctcctcatacaggtcgcagagggagcggcggccgcagcgccaaggaaacccaggaccgggagaggaggagcggcggcgacggcggcggtaactcggaagg

SEQ ID NO: 11869 - RNA, 4043 nt, Homo sapiens
  source 1..4043: mol_type = other RNA
ctgaatagctgggactacaggtgtgcgccaccacgcccagctaatttttgtgtttttagtagagatggggtttcaccatgttggccaggatggtctcaatttattgacctcatgatccacccacctcggcctccgaaagtgctgggattacaggcataagccaccacacccagcctgtgggaactatttattggatttcaaaacaccctctgcctcattaatccactaagctttctcagcaaaaagctgtttaaataaataatgggaacatctaatttaaaacagtttttctaattatagaccagtacacgaagaagagcttaacttatccaagtatagtctagtttgggtccataatggagctgaaggctcagaggacattcagggccattacactgcaggaaaacaaggaataagggatgtagaaatgacctaagaaaagcacgaagtggaatgtatactggaggcaagttaatgaaagctaataaatacaaagtgctgggaaaaatctaaaagcaaaatagctattgtaacttgcaatgcattaaaaacaactttaaaaccaaaaagtcttgataaggaaactctatagtggggtctcagttaaatgctgatgatttttaatgctcagataacattaagtggaatattaacttctgcatccgacaccatctgaattttctcacacactactacacttgttcacttttcaatcaagttccactttctgaacttgttcaaaacctcatttgaaatatatccagctactgcttttcccctttcacctagcacagggcagttacctggcaaagctctattctggccaagtcactgggactgagtagaacccacgttagcagctctggacctgaacaggagctggcccaacatcacagtgaccacccacaaagagacaagccctcctggatttttttcagcatttcttatactgactacagtagtgatgattaaagttatctgccctacagactccactgaatttgaagctgtatttattgtacagatgggggaaatgtgttttattgtgtcagttatattaatttttatcaatgtgattagatacatattttggcctattaatcttattcattatattcttagtctgagatgggttttaattctgactaacagcagctacttaagagtccaatcatacaaaatcaggagagtattaccctttctacagctaagcgagtcagtaatacagcagcaactaatactggccattaataacgtccagagagcacattagcaaaccttgtactcccagtgactgtcaggagacttgaaaataactactattctcttccaaagtagaatagcgtttttctagatagtgaaggaaatgatagtcatagttggtctgaactccaagatcctactcctcaaaacagcaccgaagcaggggttcgggatgcctgctaagagcatttccacagttcaagtctcttcagaaccttagggaccttcgtgtctagcttcacacacccacctccacatatgaaccagcctaccacacttcacatctgggtacactggccattagcaacaatgcagtctcatgcagcagcacattaaaatcaaacgggtggcaatcgttcaccaccctcagagtgttgggagactttcacatttcatcatccttataatccacaaacagaaacatgaagggatgcaagtgagttcagcattcactcgtttggtgcactcaagtgctgagagaatgcagaatttacagtgtcacagaggaaaaaagccatctgaaataattgtaaaaatggttaagtgtggtatttaaatgttggttccctcctcttcatacaagtggaagaaaagaaggggctagggtacccactgggccatgaggttaaccccttagcacaggcaatgaagaacatccaatgccacagattctgcaggaggagaaatcccaagggtatacagtattcctgagaaagatcccagatttttctgaatcagtcttaatctgattttgttttggctacacagttatgctgttatacctttgacatacataaaaatggtcattttatttcaatccagacagctcagcattgtacaaatgatggcagaaagatccatttgttcagactcagcttgctttgtttttaatactggggaataaaccaaaaaaaaaagtgtaatttttatcatttgtatccttcattctactttactggagtggaatccccagggccttcagataatctgggaagacctgactattcctgtgaggcaagcacagccctgctgagctttactcagaataatgcatgatagactcaacgtaattcccaggaaaaagcccagtcactccattcataactccctcataccaaccatcgtcattcttcttgatgacataaataatggctccttcctgaaaggacagctcatcttccttgtcttttgtatagtcataaattgccacaaccttttccaagtaagaacgtggagcccacggtgggtcctcttcagcataaggatcactatactcaaccacagcagcttcctcctcttcgtaatcttctggaggaggaggaggtgggggagactcatcaaagactggttcttccacaggtggcggtggaggtggtgtattattttcttggactctggccacaaatcccattaaaggtaactgaggagttacctgtaggatggagggaggaggaggagcaagagatactggattctggctataaaaaggtcctccattcatctgattctgaaggcttgtttgtgaagtaatggaaggagggcgtctatagggcaacgagccccctattgttgggggagtatggcgagaggcaggcctattcatgctgtagaactgtacaggatgacctgtagggggagtggaagaaacaacagggggagttggagaagtgaagccatcagcaagggtctgggcacccccagcagcagcgtctggggcagtggaggaagggacagtagcaggaacaagaggagcaggggcagatgcagaagtagcaggaaggggaggagtgccagcagagccagcaggggctggaaagacactgggaggagatggagtaggaacagcaataggaacccccacactaccacttccactgttctctcgactgctgctccgactacttgggtggctccctccactactcccactgctgctgtaagttcgatttctttgattcacagaagctgtcctcacagggctctgctgcgagggagccatattacgggttgggctaggtacgtaatcatttggtaccactggaggacgcactggctccagtgtgcgatagggggagtgccgcccaagtgtccctttccctgacatagggggactagggggcttctgagttggaggtgttgtacgcggcagcccacccatcttcatgttctgggtactcaccttaaatctaagcaaccactttactccatgtccaatatcatctagaattgtatagtcaataggttttctaatataacgaactggtcgttcaaggttggctggagcaataatcttatgtgtccttgaagtgtttttattggtagtcaaaataccaatttctcttcttgcaactttctctttatgaatatcaactgtttgtgaaatatgattgattgaagattccatccttcgtagctgggatgcctggatatccagcatctgcaggacattgttggccaaggtgtttatcagataggcaacacttgctaaggattgggtggtgtaggctttggtttcttctagggctctctgcttatctgctgactgtatgtagttgttctcgcagtaatcggccacccgttccagatttgtgtagctgtcgaagagggcccggcggccccccgggatttcctcttccagcagcatctgcagctccgccatcttcacatcctcctcctcctcctcctcatacaggtcgcagagggagcggcggccgcagcgccaaggaaacccaggaccgggagaggaggagcggcggcgacggcggcggtaactcggaagg

SEQ ID NO: 11870 - RNA, 4682 nt, Homo sapiens
  source 1..4682: mol_type = other RNA
ctgaatagctgggactacaggtgtgcgccaccacgcccagctaatttttgtgtttttagtagagatggggtttcaccatgttggccaggatggtctcaatttattgacctcatgatccacccacctcggcctccgaaagtgctgggattacaggcataagccaccacacccagcctgtgggaactatttattggatttcaaaacaccctctgcctcattaatccactaagctttctcagcaaaaagctgtttaaataaataatgggaacatctaatttaaaacagtttttctaattatagaccagtacacgaagaagagcttaacttatccaagtatagtctagtttgggtccataatggagctgaaggctcagaggacattcagggccattacactgcaggaaaacaaggaataagggatgtagaaatgacctaagaaaagcacgaagtggaatgtatactggaggcaagttaatgaaagctaataaatacaaagtgctgggaaaaatctaaaagcaaaatagctattgtaacttgcaatgcattaaaaacaactttaaaaccaaaaagtcttgataaggaaactctatagtggggtctcagttaaatgctgatgatttttaatgctcagataacattaagtggaatattaacttctgcatccgacaccatctgaattttctcacacactactacacttgttcacttttcaatcaagttccactttctgaacttgttcaaaacctcatttgaaatatatccagctactgcttttcccctttcacctagcacagggcagttacctggcaaagctctattctggccaagtcactgggactgagtagaacccacgttagcagctctggacctgaacaggagctggcccaacatcacagtgaccacccacaaagagacaagccctcctggatttttttcagcatttcttatactgactacagtagtgatgattaaagttatctgccctacagactccactgaatttgaagctgtatttattgtacagatgggggaaatgtgttttattgtgtcagttatattaatttttatcaatgtgattagatacatattttggcctattaatcttattcattatattcttagtctgagatgggttttaattctgactaacagcagctacttaagagtccaatcatacaaaatcaggagagtattaccctttctacagctaagcgagtcagtaatacagcagcaactaatactggccattaataacgtccagagagcacattagcaaaccttgtactcccagtgactgtcaggagacttgaaaataactactattctcttccaaagtagaatagcgtttttctagatagtgaaggaaatgatagtcatagttggtctgaactccaagatcctactcctcaaaacagcaccgaagcaggggttcgggatgcctgctaagagcatttccacagttcaagtctcttcagaaccttagggaccttcgtgtctagcttcacacacccacctccacatatgaaccagcctaccacacttcacatctgggtacactggccattagcaacaatgcagtctcatgcagcagcacattaaaatcaaacgggtggcaatcgttcaccaccctcagagtgttgggagactttcacatttcatcatccttataatccacaaacagaaacatgaagggatgcaagtgagttcagcattcactcgtttggtgcactcaagtgctgagagaatgcagaatttacagtgtcacagaggaaaaaagccatctgaaataattgtaaaaatggttaagtgtggtatttaaatgttggttccctcctcttcatacaagtggaagaaaagaaggggctagggtacccactgggccatgaggttaaccccttagcacaggcaatgaagaacatccaatgccacagattctgcaggaggagaaatcccaagggtatacagtattcctgagaaagatcccagatttttctgaatcagtcttaatctgattttgttttggctacacagttatgctgttatacctttgacatacataaaaatggtcattttatttcaatccagacagctcagcattgtacaaatgatggcagaaagatccatttgttcagactcagcttgctttgtttttaatactggggaataaaccaaaaaaaaaagtgtaatttttatcatttgtatccttcattctactttactggagtggaatccccagggccttcagataatctgggaagacctgactattcctgtgaggcaagcacagccctgctgagctttactcagaataatgcatgatagactcaacgtaattcccaggaaaaagcccagtcactccattcataactccctcataccaaccatcgtcattcttcttgatgacataaataatggctccttcctgaaaggacagctcatcttccttgtcttttgtatagtcataaattgccacaaccttttccaagtaagaacgtggagcccacggtgggtcctcttcagcataaggatcactatactcaaccacagcagcttcctcctcttcgtaatcttctggaggaggaggaggtgggggagactcatcaaagactggttcttccacaggtggcggtggaggtggtgtattattttcttggactctggccacaaatcccattaaaggtaactgaggagttacctgtaggatggagggaggaggaggagcaagagatactttaataaggtggtcgaaattaattcagataccacatcattttcttttcggaccttgtaagatttcatctgacaagaacgtctgtgagccagaatatactgtctttcttggagttgagctggattctggctataaaaaggtcctccattcatctgattctgaaggcttgtttgtgaagtaatggaaggagggcgtctatagggcaacgagccccctattgttgggggagtatggcgagaggcaggcctattcatgctgtagaactgtacaggatgacctgtagggggagtggaagaaacaacagggggagttggagaagtgaagccatcagcaagggtctgggcacccccagcagcagcgtctggggcagtggaggaagggacagtagcaggaacaagaggagcaggggcagatgcagaagtagcaggaaggggaggagtgccagcagagccagcaggggctggaaagacactgggaggagatggagtaggaacagcaataggaacccccacactaccacttccactgttctctcgactgctgctccgactacttgggtggctccctccactactcccactgctgctgtaagttcgatttctttgattcacagaagctgtcctcacagggctctgctgcgagggagccatattacgggttgggctaggtacgtaatcatttggtaccactggaggacgcactggctccagtgtgcgatagggggagtgccgcccaagtgtccctttccctgacatagggggactagggggcttctgagttggaggtgttgtacgcggcagcccacccatcttcatgttctgggtactcaccttaaatctaagcaaccactttactccatgtccaatatcatctagaattgtatagtcaataggttttctaatataacgaactggtcgttcaaggttggctggagcaataatcttatgtgtccttgaagtgtttttattggtagtcaaaataccaatttctcttcttgcaactttctctttatgaatatcaactgtttgtgaaatatgattgattgaagattccatccttcgtagctgggatgcctggatatccagcatctgcaggacattgttggccaaggtgtttatcagataggcaacacttgctaaggattgggtggtgtaggctttggtttcttctagggctctctgcttatctgctgactgtatgtagttgttctcgcagtaatcggccacccgttccagatttgtgtagctgtcgaagagggcccggcggccccccgggatttcctcttccagcagcatctgcagctccgccatcttcacatcctcctcctcctcctcctcatacaggtcgcagagggagcggcggccgcagcgccaaggaaacccaggaccgggagaggaggagcggcggcgacggcggcggtaactcggaaggagcgagaaacagccccagcgcgcgacaggggagggggcgacgggggcggggcgcgagccgacggactccgaggacggtcaccgcggcgacggccggccgggcgcgcgcacgcgcgctcccttccctccgcccccgggagcccgaaaaagattcccaccctcgcccgcgccgccggcccctcccccacttccggcgtctcctagcgacggcgggggtaggggccgggatgcgcgcgggagttggtggtgcagttaacccttccgccgcccgcccgccgctggagcggctggagaagcccccacctcccggcggcctttgttagcccggcgggaacacaccaccctgctcagctggcttcctgccggctccctccgggactcatctcggctccgtccccatggaggtcatcggcctagggaacttctcgaggcttttctccctctgctgctgacgggaggccgaaggagggcacagcctccactcttgggaccctcctctgtgaaagatcacacctcaacag

SEQ ID NO: 11871 - RNA, 3733 nt, Homo sapiens
  source 1..3733: mol_type = other RNA
ctgaatagctgggactacaggtgtgcgccaccacgcccagctaatttttgtgtttttagtagagatggggtttcaccatgttggccaggatggtctcaatttattgacctcatgatccacccacctcggcctccgaaagtgctgggattacaggcataagccaccacacccagcctgtgggaactatttattggatttcaaaacaccctctgcctcattaatccactaagctttctcagcaaaaagctgtttaaataaataatgggaacatctaatttaaaacagtttttctaattatagaccagtacacgaagaagagcttaacttatccaagtatagtctagtttgggtccataatggagctgaaggctcagaggacattcagggccattacactgcaggaaaacaaggaataagggatgtagaaatgacctaagaaaagcacgaagtggaatgtatactggaggcaagttaatgaaagctaataaatacaaagtgctgggaaaaatctaaaagcaaaatagctattgtaacttgcaatgcattaaaaacaactttaaaaccaaaaagtcttgataaggaaactctatagtggggtctcagttaaatgctgatgatttttaatgctcagataacattaagtggaatattaacttctgcatccgacaccatctgaattttctcacacactactacacttgttcacttttcaatcaagttccactttctgaacttgttcaaaacctcatttgaaatatatccagctactgcttttcccctttcacctagcacagggcagttacctggcaaagctctattctggccaagtcactgggactgagtagaacccacgttagcagctctggacctgaacaggagctggcccaacatcacagtgaccacccacaaagagacaagccctcctggatttttttcagcatttcttatactgactacagtagtgatgattaaagttatctgccctacagactccactgaatttgaagctgtatttattgtacagatgggggaaatgtgttttattgtgtcagttatattaatttttatcaatgtgattagatacatattttggcctattaatcttattcattatattcttagtctgagatgggttttaattctgactaacagcagctacttaagagtccaatcatacaaaatcaggagagtattaccctttctacagctaagcgagtcagtaatacagcagcaactaatactggccattaataacgtccagagagcacattagcaaaccttgtactcccagtgactgtcaggagacttgaaaataactactattctcttccaaagtagaatagcgtttttctagatagtgaaggaaatgatagtcatagttggtctgaactccaagatcctactcctcaaaacagcaccgaagcaggggttcgggatgcctgctaagagcatttccacagttcaagtctcttcagaaccttagggaccttcgtgtctagcttcacacacccacctccacatatgaaccagcctaccacacttcacatctgggtacactggccattagcaacaatgcagtctcatgcagcagcacattaaaatcaaacgggtggcaatcgttcaccaccctcagagtgttgggagactttcacatttcatcatccttataatccacaaacagaaacatgaagggatgcaagtgagttcagcattcactcgtttggtgcactcaagtgctgagagaatgcagaatttacagtgtcacagaggaaaaaagccatctgaaataattgtaaaaatggttaagtgtggtatttaaatgttggttccctcctcttcatacaagtggaagaaaagaaggggctagggtacccactgggccatgaggttaaccccttagcacaggcaatgaagaacatccaatgccacagattctgcaggaggagaaatcccaagggtatacagtattcctgagaaagatcccagatttttctgaatcagtcttaatctgattttgttttggctacacagttatgctgttatacctttgacatacataaaaatggtcattttatttcaatccagacagctcagcattgtacaaatgatggcagaaagatccatttgttcagactcagcttgctttgtttttaatactggggaataaaccaaaaaaaaaagtgtaatttttatcatttgtatccttcattctactttactggagtggaatccccagggccttcagataatctgggaagacctgactattcctgtgaggcaagcacagccctgctgagctttactcagaataatgcatgatagactcaacgtaattcccaggaaaaagcccagtcactccattcataactccctcataccaaccatcgtcattcttcttgatgacataaataatggctccttcctgaaaggacagctcatcttccttgtcttttgtatagtcataaattgccacaaccttttccaagtaagaacgtggagcccacggtgggtcctcttcagcataaggatcactatactcaaccacagcagcttcctcctcttcgtaatcttctggattctggctataaaaaggtcctccattcatctgattctgaaggcttgtttgtgaagtaatggaaggagggcgtctatagggcaacgagccccctattgttgggggagtatggcgagaggcaggcctattcatgctgtagaactgtacaggatgacctgtagggggagtggaagaaacaacagggggagttggagaagtgaagccatcagcaagggtctgggcacccccagcagcagcgtctggggcagtggaggaagggacagtagcaggaacaagaggagcaggggcagatgcagaagtagcaggaaggggaggagtgccagcagagccagcaggggctggaaagacactgggaggagatggagtaggaacagcaataggaacccccacactaccacttccactgttctctcgactgctgctccgactacttgggtggctccctccactactcccactgctgccaagtgtccctttccctgacatagggggactagggggcttctgagttggaggtgttgtacgcggcagcccacccatcttcatgttctgggtactcaccttaaatctaagcaaccactttactccatgtccaatatcatctagaattgtatagtcaataggttttctaatataacgaactggtcgttcaaggttggctggagcaataatcttatgtgtccttgaagtgtttttattggtagtcaaaataccaatttctcttcttgcaactttctctttatgaatatcaactgtttgtgaaatatgattgattgaagattccatccttcgtagctgggatgcctggatatccagcatctgcaggacattgttggccaaggtgtttatcagataggcaacacttgctaaggattgggtggtgtaggctttggtttcttctagggctctctgcttatctgctgtatgtagttgttctcgcagtaatcggccacccgttccagatttgtgtagctgtcgaagagggcccggcggccccccgggatttcctcttccagcagcatctgcagctccgccatcttcacatcctcctcctcctcctcctcatacaggtcgcagagggagcggcggccgcagcgccaaggaaacccaggaccgggagaggaggagcggcggcgacggcggcggtaactcggaagg

SEQ ID NO: 11872 - RNA, 3920 nt, Homo sapiens
  source 1..3920: mol_type = other RNA
ctgaatagctgggactacaggtgtgcgccaccacgcccagctaatttttgtgtttttagtagagatggggtttcaccatgttggccaggatggtctcaatttattgacctcatgatccacccacctcggcctccgaaagtgctgggattacaggcataagccaccacacccagcctgtgggaactatttattggatttcaaaacaccctctgcctcattaatccactaagctttctcagcaaaaagctgtttaaataaataatgggaacatctaatttaaaacagtttttctaattatagaccagtacacgaagaagagcttaacttatccaagtatagtctagtttgggtccataatggagctgaaggctcagaggacattcagggccattacactgcaggaaaacaaggaataagggatgtagaaatgacctaagaaaagcacgaagtggaatgtatactggaggcaagttaatgaaagctaataaatacaaagtgctgggaaaaatctaaaagcaaaatagctattgtaacttgcaatgcattaaaaacaactttaaaaccaaaaagtcttgataaggaaactctatagtggggtctcagttaaatgctgatgatttttaatgctcagataacattaagtggaatattaacttctgcatccgacaccatctgaattttctcacacactactacacttgttcacttttcaatcaagttccactttctgaacttgttcaaaacctcatttgaaatatatccagctactgcttttcccctttcacctagcacagggcagttacctggcaaagctctattctggccaagtcactgggactgagtagaacccacgttagcagctctggacctgaacaggagctggcccaacatcacagtgaccacccacaaagagacaagccctcctggatttttttcagcatttcttatactgactacagtagtgatgattaaagttatctgccctacagactccactgaatttgaagctgtatttattgtacagatgggggaaatgtgttttattgtgtcagttatattaatttttatcaatgtgattagatacatattttggcctattaatcttattcattatattcttagtctgagatgggttttaattctgactaacagcagctacttaagagtccaatcatacaaaatcaggagagtattaccctttctacagctaagcgagtcagtaatacagcagcaactaatactggccattaataacgtccagagagcacattagcaaaccttgtactcccagtgactgtcaggagacttgaaaataactactattctcttccaaagtagaatagcgtttttctagatagtgaaggaaatgatagtcatagttggtctgaactccaagatcctactcctcaaaacagcaccgaagcaggggttcgggatgcctgctaagagcatttccacagttcaagtctcttcagaaccttagggaccttcgtgtctagcttcacacacccacctccacatatgaaccagcctaccacacttcacatctgggtacactggccattagcaacaatgcagtctcatgcagcagcacattaaaatcaaacgggtggcaatcgttcaccaccctcagagtgttgggagactttcacatttcatcatccttataatccacaaacagaaacatgaagggatgcaagtgagttcagcattcactcgtttggtgcactcaagtgctgagagaatgcagaatttacagtgtcacagaggaaaaaagccatctgaaataattgtaaaaatggttaagtgtggtatttaaatgttggttccctcctcttcatacaagtggaagaaaagaaggggctagggtacccactgggccatgaggttaaccccttagcacaggcaatgaagaacatccaatgccacagattctgcaggaggagaaatcccaagggtatacagtattcctgagaaagatcccagatttttctgaatcagtcttaatctgattttgttttggctacacagttatgctgttatacctttgacatacataaaaatggtcattttatttcaatccagacagctcagcattgtacaaatgatggcagaaagatccatttgttcagactcagcttgctttgtttttaatactggggaataaaccaaaaaaaaaagtgtaatttttatcatttgtatccttcattctactttactggagtggaatccccagggccttcagataatctgggaagacctgactattcctgtgaggcaagcacagccctgctgagctttactcagaataatgcatgatagactcaacgtaattcccaggaaaaagcccagtcactccattcataactccctcataccaaccatcgtcattcttcttgatgacataaataatggctccttcctgaaaggacagctcatcttccttgtcttttgtatagtcataaattgccacaagtgattccctcagcttggaaggcccttcctttctctcttctctgcctgagaaactcctattcatcattcaaggcaccaagaacgccatgttctctgagaagctttccttttccaagtaagaacgtggagcccacggtgggtcctcttcagcataaggatcactatactcaaccacagcagcttcctcctcttcgtaatcttctggaggaggaggaggtgggggagactcatcaaagactggttcttccacaggtggcggtggaggtggtgtatctgaaactggattctggctataaaaaggtcctccattcatctgattctgaaggcttgtttgtgaagtaatggaaggagggcgtctatagggcaacgagccccctattgttgggggagtatggcgagaggcaggcctattcatgctgtagaactgtacaggatgacctgtagggggagtggaagaaacaacagggggagttggagaagtgaagccatcagcaagggtctgggcacccccagcagcagcgtctggggcagtggaggaagggacagtagcaggaacaagaggagcaggggcagatgcagaagtagcaggaaggggaggagtgccagcagagccagcaggggctggaaagacactgggaggagatggagtaggaacagcaataggaacccccacactaccacttccactgttctctcgactgctgctccgactacttgggtggctccctccactactcccactgctgccaagtgtccctttccctgacatagggggactagggggcttctgagttggaggtgttgtacgcggcagcccacccatcttcatgttctgggtactcaccttaaatctaagcaaccactttactccatgtccaatatcatctagaattgtatagtcaataggttttctaatataacgaactggtcgttcaaggttggctggagcaataatcttatgtgtccttgaagtgtttttattggtagtcaaaataccaatttctcttcttgcaactttctctttatgaatatcaactgtttgtgaaatatgattgattgaagattccatccttcgtagctgggatgcctggatatccagcatctgcaggacattgttggccaaggtgtttatcagataggcaacacttgctaaggattgggtggtgtaggctttggtttcttctagggctctctgcttatctgctgactgtatgtagttgttctcgcagtaatcggccacccgttccagatttgtgtagctgtcgaagagggcccggcggccccccgggatttcctcttccagcagcatctgcagctccgccatcttcacatcctcctcctcctcctcctcatacaggtcgcagagggagcggcggccgcagcgccaaggaaacccaggaccgggagaggaggagcggcggcgacggcggcggtaactcggaagg

SEQ ID NO: 11873 - RNA, 2426 nt, Homo sapiens
  source 1..2426: mol_type = other RNA
ctgaatagctgggactacaggtgtgcgccaccacgcccagctaattttttgtatttttcgtagagacggggtttcaccatattggccaggctggtctcaaactcctgaccttgtgatccgtccgcctcggcctcccaaagttctgggattacaggcatgagccaccgtgcccggcctgagtttctataatttaagcatctttaaggtaaagaaaaattgaaaatgagattacaggcaatttaacgcacaatttaatgaccagttcaatgagctggtttatttgcttgtaaaattattttatctaatgtaaaaatacttggtaaagaaaagttcttaatggggctggaagacaaaaagtctgcatttaaaaaaggttaacaaaatcaataatatatgggtaagcataggcacagaagaataaaaaatttaaaaatgttaaaatcaataataaagccactaataaccacaaaaggaaaactatggttctttttactttgtcaaagttctgcatctgttcccggttggtcagccaggattccatgtcctgggcagtctgaatgacaaatgcttcgtaatctgcaaacatctgtgtaaaacggttagcaaagacctctcggagctgtacattgagctggtagtcccttagttctgcctcttcacaatgcagttttaaatccttgtctttttcacccagagaagcagagaggtccattttttccacagccacaccagtacgcttggccagagcctgcaagcgggctatggtttcattgcccttcagtaactcatacatgctgatgttattagtacagacattgccgttctttttgtcattgaccaagtctttcagaaccatattcttcagtttgctggtactctcactgcaatgtaggctgccctcaggagggatcccaaattgaacaagaacctcagagagttcttggataaaatccactttattggggaactgtggaaattcttcaggcaactcaataaaatggttgtcaatgtccacaaaacacaaattagcctcttgaggaagttctagtttagaacggtcagttccttcttttgactgaaggcccatcagataagggacaggagcatcaagaaaatgtagcagagaagcaggtagaatgggcacataaacatgttgccattgaaatgggaacaaaagtgtggtgatgccttctgccacagtcatcaggcgttgataatcttgtgagtagagaaggatttgcatctctaaaagaacacaggtaaacacctgcaccaggttctctaatcccaggagctcaaatgcctcccgaagggggtaatcagagagggggagttcactgggcccaggcctctggcagatgacaggttcataaacaccataaaatttcagtgacctccctggaggtggaaggggtacttcataaagaatattgtggatatagctttcaagtggcaagggtggtggctgctgtgaggtaacagccttgtaaagctggataaggaatttcttgcaggcctgcatgaatggtaacggtgtgatcaagcatatactttttgaaacatacagggtgtctctgctaatatcataggagttgtatcgctggagtttcaaaagggaagttgtatctccttcatcaagactacttgccaatgagtccatactgcaggaagatgaagcatacacactgctgtaatgctcagcgttgtgcatctggtaaagtgtctgcattgctgtgcagatttgcttacttgtaacttcttcataaaaagtgagaacaaaaccataggtgcgagaaccatcttccctggtaattataaatgagtgaaactgggggtctttattgtccgtttgtgtcctgaaagatagccctttaggcatgcacaacatgttcaccgcatcttgatcaaaagggttccattctatattctgaggatagtgggcgagaactttggatttgaatgttcttctcaaaggactctggtcaaaattttcgcccgccagctcgtcaggctccagcccgctgtccgcgtcgatcccgcacagcacgaagtagtgcgcgaagcggcaggcggccggggaggagcccgagcccgggccgggcgccgcgcagctcccgctcatcccggccgcgctgctccaggggccgccgccgccgccgcccgggaaggctttctgcggaggctgccaccaccgctccggctgtggtctgtgcgcccgccctagggcgacactggcgcgcccatggccgcgcagccgcctctcgccgccgcagcctgcctcctcgctcggcgcgggggaagcggccgcgggctcgcgcgcggcgggtccggagcccggccgggtgggggaggggcgcggggggagtgtcggcctgagaggccctcgcagccgcagctgcgctcgcgagctgagagccgccgcgtct

SEQ ID NO: 11874 - RNA, 2492 nt, Homo sapiens
  source 1..2492: mol_type = other RNA
ctgaatagctgggactacaggtgtgcgccaccacgcccagctaattttttgtatttttcgtagagacggggtttcaccatattggccaggctggtctcaaactcctgaccttgtgatccgtccgcctcggcctcccaaagttctgggattacaggcatgagccaccgtgcccggcctgagtttctataatttaagcatctttaaggtaaagaaaaattgaaaatgagattacaggcaatttaacgcacaatttaatgaccagttcaatgagctggtttatttgcttgtaaaattattttatctaatgtaaaaatacttggtaaagaaaagttcttaatggggctggaagacaaaaagtctgcatttaaaaaaggttaacaaaatcaataatatatgggtaagcataggcacagaagaataaaaaatttaaaaatgttaaaatcaataataaagccactaataaccacaaaaggaaaactatggttctttttactttgtcaaagttctgcatctgttcccggttggtcagccaggattccatgtcctgggcagtctgaatgacaaatgcttcgtaatctgcaaacatctgtgtaaaacggttagcaaagacctctcggagctgtacattgagctggtagtcccttagttctgcctcttcacaatgcagttttaaatccttgtctttttcacccagagaagcagagaggtccattttttccacagccacaccagtacgcttggccagagcctgcaagcgggctatggtttcattgcccttcagtaactcatacatgctgatgttattagtacagacattgccgttctttttgtcattgaccaagtctttcagaaccatattcttcagtttgctggtactctcactgcaatgtaggctgccctcaggagggatcccaaattgaacaagaacctcagagagttcttggataaaatccactttattggggaactgtggaaattcttcaggcaactcaataaaatggttgtcaatgtccacaaaacacaaattagcctcttgaggaagttctagtttagaacggtcagttccttcttttgactgaaggcccatcagataagggacaggagcatcaagaaaatgtagcagagaagcaggtagaatgggcacataaacatgttgccattgaaatgggaacaaaagtgtggtgatgccttctgccacagtcatcaggcgttgataatcttgtgagtagagaaggatttgcatctctaaaagaacacaggtaaacacctgcaccaggttctctaatcccaggagctcaaatgcctcccgaagggggtaatcagagagggggagttcactgggcccaggcctctggcagatgacaggttcataaacaccataaaatttcagtgacctccctggaggtggaaggggtacttcataaagaatattgtggatatagctttcaagtggcaagggtggtggctgctgtgaggtaacagccttgtaaagctggataaggaatttcttgcaggcctgcatgaatggtaacggtgtgatcaagcatatactttttgaaacatacagggtgtctctgctaatatcataggagttgtatcgctggagtttcaaaagggaagttgtatctccttcatcaagactacttgccaatgagtccatactgcaggaagatgaagcatacacactgctgtaatgctcagcgttgtgcatctggtaaagtgtctgcattgctgtgcagatttgcttacttgtaacttcttcataaaaagtgagaacaaaaccataggtgcgagaaccatcttccctggtaattataaatgagtgaaactgggggtctttattgtccgtttgtgtcctgaaagatagccctttaggcatgcacaacatgttcaccgcatcttgatcaaaagggttccattctatattctgaggatagtgggcgagaactttggatttgaatgttcttctcaaaggactctggtcaaaattttcgcctgaagtcgtatttgcagcaccttggctcttgccatgacgatctgcttctagccattggtacaaaaccgccagctcgtcaggctccagcccgctgtccgcgtcgatcccgcacagcacgaagtagtgcgcgaagcggcaggcggccggggaggagcccgagcccgggccgggcgccgcgcagctcccgctcatcccggccgcgctgctccaggggccgccgccgccgccgcccgggaaggctttctgcggaggctgccaccaccgctccggctgtggtctgtgcgcccgccctagggcgacactggcgcgcccatggccgcgcagccgcctctcgccgccgcagcctgcctcctcgctcggcgcgggggaagcggccgcgggctcgcgcgcggcgggtccggagcccggccgggtgggggaggggcgcggggggagtgtcggcctgagaggccctcgcagccgcagctgcgctcgcgagctgagagccgccgcgtct

SEQ ID NO: 11875 - RNA, 1895 nt, Homo sapiens
  source 1..1895: mol_type = other RNA
ctgaatagctgggactacaggtgtgcgccaccacgcccagctaattttttgtatttttcgtagagacggggtttcaccatattggccaggctggtctcaaactcctgaccttgtgatccgtccgcctcggcctcccaaagttctgggattacaggcatgagccaccgtgcccggcctgagtttctataatttaagcatctttaaggtaaagaaaaattgaaaatgagattacaggcaatttaacgcacaatttaatgaccagttcaatgagctggtttatttgcttgtaaaattattttatctaatgtaaaaatacttggtaaagaaaagttcttaatggggctggaagacaaaaagtctgcatttaaaaaaggttaacaaaatcaataatatatgggtaagcataggcacagaagaataaaaaatttaaaaatgttaaaatcaataataaagccactaataaccacaaaaggaaaactatggttctttttactttgtcaaagttctgcatctgttcccggttggtcagccaggattccatgtcctgggcagtctgaatgacaaatgcttcgtaatctgcaaacatctgtgtaaaacggttagcaaagacctctcggagctgtacattgagctggtagtcccttagttctgcctcttcacaatgcagttttaaatccttgtctttttcacccagagaagcagagaggtccattttttccacagccacaccagtacgcttggccagagcctgcaagcgggctatggtttcattgcccttcagtaactcatacatgctgatgttattagtacagacattgccgttctttttgtcattgaccaagtctttcagaaccatattcttcagtttgctggtactctcactgcaatgtaggctgccctcaggagggatcccaaattgaacaagaacctcagagagttcttggataaaatccactttattggggaactgtggaaattcttcaggcaactcaataaaatggttgtcaatgtccacaaaacacaaattagcctcttgaggaagttctagtttagaacggtcagttccttcttttgactgaaggcccatcagataagggacaggagcatcaagaaaatgtagcagagaagcaggtagaatgggcacataaacatgttgccattgaaatgggaacaaaagtgtggtgatgccttctgccacagtcatcaggcgttgataatttgtaacttcttcataaaaagtgagaacaaaaccataggtgcgagaaccatcttccctggtaattataaatgagtgaaactgggggtctttattgtccgtttgtgtcctgaaagatagccctttaggcatgcacaacatgttcaccgcatcttgatcaaaagggttccattctatattctgaggatagtgggcgagaactttggatttgaatgttcttctcaaaggactctggtcaaaattttcgcccgccagctcgtcaggctccagcccgctgtccgcgtcgatcccgcacagcacgaagtagtgcgcgaagcggcaggcggccggggaggagcccgagcccgggccgggcgccgcgcagctcccgctcatcccggccgcgctgctccaggggccgccgccgccgccgcccgggaaggctttctgcggaggctgccaccaccgctccggctgtggtctgtgcgcccgccctagggcgacactggcgcgcccatggccgcgcagccgcctctcgccgccgcagcctgcctcctcgctcggcgcgggggaagcggccgcgggctcgcgcgcggcgggtccggagcccggccgggtgggggaggggcgcggggggagtgtcggcctgagaggccctcgcagccgcagctgcgctcgcgagctgagagccgccgcgtct

SEQ ID NO: 11876 - RNA, 3839 nt, Homo sapiens
  source 1..3839: mol_type = other RNA
ctgaatagctgggactacaggtgtgcgccaccactcccagctaatttttgtatttttagtagagacagggttttgccatgttggtcaggctggtctcggaactcctgacctcaggtgatccacccgcctctgcctcacaaagtgctgggattacaggcatgagctaccgtgcctggcctaaaccttacgcttttgaggttgagtgcaggccttgtgataactaagcgctacttttgacgagccttcaacaagctgcccagtcctctcctcagcagacgcatcaggttgtagttgcatctttacagtggtctttccttttattaaatctatagcagtgaatatagatttgattcaacttttagttacgttctctcaagaatcctaatcaactttcagttagcctcttaagaaagggaaaaaaaggtgctgccagtcatccccaaattatgtttttggctgtgcattctattttctacatagcactgaatctgagtaacagtcatcctggatttatagttggaacagaacagtaacagacctaactgggactcagccagcactagcctcatcttagctgccccttttctctgctttgcagtttactgcttccctgggctagccataacggggttctgggcaggtcagactcttcagcaagacagtgtattaatagtgtgaattagatacactgatgacctgctctgcctagttaagaaactgaattaatcagcagttacaaagcacatactttgttacgtgctaggctttgcctcctggcctctagataattaagacggcccagggaataccagcagagaagtgctaattgtatttgggtgttacaaaagcagacctagacgagctgttcacttaactggtacctgttggtcagaaaaagaatttatttagagattatgatcatgtaaaattacagtactcaacccttctagcaaagtatttttttgaaaaataaactaaatgcctttataaacttgtgttctctcgtcttgagtaacatgtactgtttggcgaggagtaatttttttcttgtgacattccagtcacgacagaggtcatttcagaacagtgagcagtgcaggccctaaccagctcaccctcagagcagcagcaccatcactcgaattttctacaacggaaatgttctatatcttcatcttagcttgactgagaaactgaatgtttaattctcacacttcactaacatgtattaatagtgatgccttcatctgtacgtttgaattttcacttttctccgattaaagtgagaaacaggtcagatgctatccatgagaaataggaaagaatggtgcagtaaagagactcacatttagtgttctctagcccaggaaacataagatgttcttaatccacccacaatttcccttcccttgcaatcatccagagcatgttttttggaaaactaacctattcttccatcagtagaggttgcttggtgcctatttgatcactttcacaagaaaatctgtgcgctctcttcacacgcagcaatagttatttccaactgtcagtcaatcaaaatggacacgcgaattgtccacactattcatagaatccccctggaactcattcatgtgtatccagagtacaggaattccagaacacaaccctctttataggccaggaaacaggcagcaacaacgataagttcatccagctttattgaaacctattacagaagacaatccgaataaaaccactgtctcctgtagaaatctgagttatgttgttttactacaaaagaatataaaacacattaaattacagtgtgaaggaattttaaaaatgaacagtgtatcctcattaaatgtttgcaaagtttcttcctaagcacttacaactagttacagctcttttaaaaattcagatttctacactcagtttaacgggagagacattcacacttaggtacttcagccccaactttcacggactattggaaattagaaggtactttgttgctaagtgaaaaaaatgcacattttttcatatcagggaaaattatactggacttaacagttttaaatgagcaataactcagatatattagagagaaatcacctcttgccttacaaataccaaataaattccctagactcccctccctgtagagaccatcagctcactgtgaaggcttgagcctcagtaggtaaaatttgaggaaaaaaatgagaaatggctaaaagaggcatctgctgcaggaaccttctgtgactgtcaaacattccctcttcaagctcccttttaaaacccagtccattcccaacatcactgaaaatgaaaagaataaacttgctggtcctcatgtcaaggcagtgttttcattgtctcttgatattttatcccatttcctattgacaacatctcccctacccctgaaattatttagaggttccctctatgacaaacccttgcttttttttagctttaggtataacactgacatcttttgaaaaacgtgttagtaaatactcaagttctggcctcatttcctgatgtatgaagcatggaagcagtgctgtcctgtggagattgcttttgcaccaactacacaggaaggtccttgacctctaagcatgcctttagaggttagaattcacagaaaacaaattcaattgtcaaacacctgttcctaattttgtgcaaagcaatacaacatagcacaactccatttgttgtttttcgttgtgctttgtagagacggggtcttgctatgttgcccagtctagtctcaaactcctggcctcaagctatccttcctcctcagcctcccaaagtgttgggattacacgtgtgagccaccatgcctggccccacctccatttattaggctatctcatgcaaacttaaaattaaaaaaataatcccaggccccaatgtagatcatgaacctacttaagactcattatggtaaaaacaaattcttacatttttctgtctttctaaaagtgtagtggttatggctaaagactaatcaacattacagatccaatctgttgtcaaagaacacaatttctgacctggtaacaaaattgttctgataatctgacacatggccaagattctcagacaagaattaaaggcattcttttggattctgtcctttaataactttcagaggcttccagctcagtaaagacactgatcaaatcttggtaaaaatgggctcgtgtgcagactttaggtgatgttcttcagcaaattcaacaggccaaaggagtgtttgtcactgacagagctctcaccactcactggttctgtgccagttttccatagcctcctctcccagcatcgtagtcctgccgatactcatcccgaacctggcccccagatcgcccacggccgtattgcctgccctccttaaagcctgcgtcccagtctgtgcgaatgattcggtcatccagacgcgtcccatttatgtaccgcatggcgttttccgcatctgcgcgtgagtaatattccacaaaacagaatccacatgctgttttcttcattttatccagacccataatgattttctttatgtcaccacttttgctgaagagttcatagatttgttcttcagttgtgtaaaaagaaagatttccaacatataacgtacagcttttcttcagtaatttttcttgttcttcattgtcacccgtttctcagcgttcttgcccagggccttcccgtctcgcggcccggcctccctcacccggaagtgctggtcccggtactggctcagctccacgtaggagtcgctgcgcagcgccttcaggaggccacccgacatagtgcagagaagcggaccacaatgc

SEQ ID NO: 11877 - RNA, 3878 nt, Homo sapiens
  source 1..3878: mol_type = other RNA
ctgaatagctgggactacaggtgtgcgccaccactcccagctaatttttgtatttttagtagagacagggttttgccatgttggtcaggctggtctcggaactcctgacctcaggtgatccacccgcctctgcctcacaaagtgctgggattacaggcatgagctaccgtgcctggcctaaaccttacgcttttgaggttgagtgcaggccttgtgataactaagcgctacttttgacgagccttcaacaagctgcccagtcctctcctcagcagacgcatcaggttgtagttgcatctttacagtggtctttccttttattaaatctatagcagtgaatatagatttgattcaacttttagttacgttctctcaagaatcctaatcaactttcagttagcctcttaagaaagggaaaaaaaggtgctgccagtcatccccaaattatgtttttggctgtgcattctattttctacatagcactgaatctgagtaacagtcatcctggatttatagttggaacagaacagtaacagacctaactgggactcagccagcactagcctcatcttagctgccccttttctctgctttgcagtttactgcttccctgggctagccataacggggttctgggcaggtcagactcttcagcaagacagtgtattaatagtgtgaattagatacactgatgacctgctctgcctagttaagaaactgaattaatcagcagttacaaagcacatactttgttacgtgctaggctttgcctcctggcctctagataattaagacggcccagggaataccagcagagaagtgctaattgtatttgggtgttacaaaagcagacctagacgagctgttcacttaactggtacctgttggtcagaaaaagaatttatttagagattatgatcatgtaaaattacagtactcaacccttctagcaaagtatttttttgaaaaataaactaaatgcctttataaacttgtgttctctcgtcttgagtaacatgtactgtttggcgaggagtaatttttttcttgtgacattccagtcacgacagaggtcatttcagaacagtgagcagtgcaggccctaaccagctcaccctcagagcagcagcaccatcactcgaattttctacaacggaaatgttctatatcttcatcttagcttgactgagaaactgaatgtttaattctcacacttcactaacatgtattaatagtgatgccttcatctgtacgtttgaattttcacttttctccgattaaagtgagaaacaggtcagatgctatccatgagaaataggaaagaatggtgcagtaaagagactcacatttagtgttctctagcccaggaaacataagatgttcttaatccacccacaatttcccttcccttgcaatcatccagagcatgttttttggaaaactaacctattcttccatcagtagaggttgcttggtgcctatttgatcactttcacaagaaaatctgtgcgctctcttcacacgcagcaatagttatttccaactgtcagtcaatcaaaatggacacgcgaattgtccacactattcatagaatccccctggaactcattcatgtgtatccagagtacaggaattccagaacacaaccctctttataggccaggaaacaggcagcaacaacgataagttcatccagctttattgaaacctattacagaagacaatccgaataaaaccactgtctcctgtagaaatctgagttatgttgttttactacaaaagaatataaaacacattaaattacagtgtgaaggaattttaaaaatgaacagtgtatcctcattaaatgtttgcaaagtttcttcctaagcacttacaactagttacagctcttttaaaaattcagatttctacactcagtttaacgggagagacattcacacttaggtacttcagccccaactttcacggactattggaaattagaaggtactttgttgctaagtgaaaaaaatgcacattttttcatatcagggaaaattatactggacttaacagttttaaatgagcaataactcagatatattagagagaaatcacctcttgccttacaaataccaaataaattccctagactcccctccctgtagagaccatcagctcactgtgaaggcttgagcctcagtaggtaaaatttgaggaaaaaaatgagaaatggctaaaagaggcatctgctgcaggaaccttctgtgactgtcaaacattccctcttcaagctcccttttaaaacccagtccattcccaacatcactgaaaatgaaaagaataaacttgctggtcctcatgtcaaggcagtgttttcattgtctcttgatattttatcccatttcctattgacaacatctcccctacccctgaaattatttagaggttccctctatgacaaacccttgcttttttttagctttaggtataacactgacatcttttgaaaaacgtgttagtaaatactcaagttctggcctcatttcctgatgtatgaagcatggaagcagtgctgtcctgtggagattgcttttgcaccaactacacaggaaggtccttgacctctaagcatgcctttagaggttagaattcacagaaaacaaattcaattgtcaaacacctgttcctaattttgtgcaaagcaatacaacatagcacaactccatttgttgtttttcgttgtgctttgtagagacggggtcttgctatgttgcccagtctagtctcaaactcctggcctcaagctatccttcctcctcagcctcccaaagtgttgggattacacgtgtgagccaccatgcctggccccacctccatttattaggctatctcatgcaaacttaaaattaaaaaaataatcccaggccccaatgtagatcatgaacctacttaagactcattatggtaaaaacaaattcttacatttttctgtctttctaaaagtgtagtggttatggctaaagactaatcaacattacagatccaatctgttgtcaaagaacacaatttctgacctggtaacaaaattgttctgataatctgacacatggccaagattctcagacaagaattaaaggcattcttttggattctgtcctttaataactttcagaggcttccagctcagtaaagacactgatcaaatcttggtaaaaatgggctcgtgtgcagactttaggtgatgttcttcagcaaattcaacaggccaaaggagtgtttgtcactgacagagctctcaccactcactggttctgtgccagttttccatagcctcctctcccagcatcgtagtcctgccgatactcatcccgaacctggcccccagatcgcccacggccgtattgcctgccctccttaaagcctgcgtcccagtctgtgcgaatgattcggtcatccagacgcgtcccatttatgtaccgcatggcgttttccgcatctgcgcgtgagtaatattccacaaaacagaatccacatgctgttttcttcattttatccagacccataatgattttctttatgtcaccacttttgctgaagagttcatagatttgttcttcagttgtgtaaaaagaaagatttccaacatataacgtacagcttttcttcagtaatttttcttgttcttcattgtcaccctccgctgatactgaaaagtctactttgaatatctgctgcctcccctttttccacaaaatatactgtgatatagtccggactaaaaatttccctcttctgaaatccagcaattctccgatctttacatccgaacaccctcaaagtgccgagcttggcgggtccacctccccactccgaagcttccccgagggcggagt

SEQ ID NO: 11878 - RNA, 3953 nt, Homo sapiens
  source 1..3953: mol_type = other RNA
ctgaatagctgggactacaggtgtgcgccaccactcccagctaatttttgtatttttagtagagacagggttttgccatgttggtcaggctggtctcggaactcctgacctcaggtgatccacccgcctctgcctcacaaagtgctgggattacaggcatgagctaccgtgcctggcctaaaccttacgcttttgaggttgagtgcaggccttgtgataactaagcgctacttttgacgagccttcaacaagctgcccagtcctctcctcagcagacgcatcaggttgtagttgcatctttacagtggtctttccttttattaaatctatagcagtgaatatagatttgattcaacttttagttacgttctctcaagaatcctaatcaactttcagttagcctcttaagaaagggaaaaaaaggtgctgccagtcatccccaaattatgtttttggctgtgcattctattttctacatagcactgaatctgagtaacagtcatcctggatttatagttggaacagaacagtaacagacctaactgggactcagccagcactagcctcatcttagctgccccttttctctgctttgcagtttactgcttccctgggctagccataacggggttctgggcaggtcagactcttcagcaagacagtgtattaatagtgtgaattagatacactgatgacctgctctgcctagttaagaaactgaattaatcagcagttacaaagcacatactttgttacgtgctaggctttgcctcctggcctctagataattaagacggcccagggaataccagcagagaagtgctaattgtatttgggtgttacaaaagcagacctagacgagctgttcacttaactggtacctgttggtcagaaaaagaatttatttagagattatgatcatgtaaaattacagtactcaacccttctagcaaagtatttttttgaaaaataaactaaatgcctttataaacttgtgttctctcgtcttgagtaacatgtactgtttggcgaggagtaatttttttcttgtgacattccagtcacgacagaggtcatttcagaacagtgagcagtgcaggccctaaccagctcaccctcagagcagcagcaccatcactcgaattttctacaacggaaatgttctatatcttcatcttagcttgactgagaaactgaatgtttaattctcacacttcactaacatgtattaatagtgatgccttcatctgtacgtttgaattttcacttttctccgattaaagtgagaaacaggtcagatgctatccatgagaaataggaaagaatggtgcagtaaagagactcacatttagtgttctctagcccaggaaacataagatgttcttaatccacccacaatttcccttcccttgcaatcatccagagcatgttttttggaaaactaacctattcttccatcagtagaggttgcttggtgcctatttgatcactttcacaagaaaatctgtgcgctctcttcacacgcagcaatagttatttccaactgtcagtcaatcaaaatggacacgcgaattgtccacactattcatagaatccccctggaactcattcatgtgtatccagagtacaggaattccagaacacaaccctctttataggccaggaaacaggcagcaacaacgataagttcatccagctttattgaaacctattacagaagacaatccgaataaaaccactgtctcctgtagaaatctgagttatgttgttttactacaaaagaatataaaacacattaaattacagtgtgaaggaattttaaaaatgaacagtgtatcctcattaaatgtttgcaaagtttcttcctaagcacttacaactagttacagctcttttaaaaattcagatttctacactcagtttaacgggagagacattcacacttaggtacttcagccccaactttcacggactattggaaattagaaggtactttgttgctaagtgaaaaaaatgcacattttttcatatcagggaaaattatactggacttaacagttttaaatgagcaataactcagatatattagagagaaatcacctcttgccttacaaataccaaataaattccctagactcccctccctgtagagaccatcagctcactgtgaaggcttgagcctcagtaggtaaaatttgaggaaaaaaatgagaaatggctaaaagaggcatctgctgcaggaaccttctgtgactgtcaaacattccctcttcaagctcccttttaaaacccagtccattcccaacatcactgaaaatgaaaagaataaacttgctggtcctcatgtcaaggcagtgttttcattgtctcttgatattttatcccatttcctattgacaacatctcccctacccctgaaattatttagaggttccctctatgacaaacccttgcttttttttagctttaggtataacactgacatcttttgaaaaacgtgttagtaaatactcaagttctggcctcatttcctgatgtatgaagcatggaagcagtgctgtcctgtggagattgcttttgcaccaactacacaggaaggtccttgacctctaagcatgcctttagaggttagaattcacagaaaacaaattcaattgtcaaacacctgttcctaattttgtgcaaagcaatacaacatagcacaactccatttgttgtttttcgttgtgctttgtagagacggggtcttgctatgttgcccagtctagtctcaaactcctggcctcaagctatccttcctcctcagcctcccaaagtgttgggattacacgtgtgagccaccatgcctggccccacctccatttattaggctatctcatgcaaacttaaaattaaaaaaataatcccaggccccaatgtagatcatgaacctacttaagactcattatggtaaaaacaaattcttacatttttctgtctttctaaaagtgtagtggttatggctaaagactaatcaacattacagatccaatctgttgtcaaagaacacaatttctgacctggtaacaaaattgttctgataatctgacacatggccaagattctcagacaagaattaaaggcattcttttggattctgtcctttaataactttcagaggcttccagctcagtaaagacactgatcaaatcttggtaaaaatgggctcgtgtgcagactttaggtgatgttcttcagcaaattcaacaggccaaaggagtgtttgtcactgacagagctctcaccactcactggttctgtgccagttttccatagcctcctctcccagcatcgtagtcctgccgatactcatcccgaacctggcccccagatcgcccacggccgtattgcctgccctccttaaagcctgcgtcccagtctgtgcgaatgattcggtcatccagacgcgtcccatttatgtaccgcatggcgttttccgcatctgcgcgtgagtaatattccacaaaacagaatccacatgctgttttcttcattttatccagacccataatgattttctttatgtcaccacttttgctgaagagttcatagatttgttcttcagttgtgtaaaaagaaagatttccaacatataacgtacagcttttcttcagtaatttttcttgttcttcattgtcaccctctcggcactggctggggtacagggagcggctgcgagcgaatgggataagcgagcctccagttccccgtcttccagagcaagtggcttcagtgatatccaagcgcccttccagcacccattccctgcctcgccagcaggcaccggggccccacttggcgtttgcggatttcagctgaatgggaggcgacacaatgagacaagagcaaaccgtttctcagcgttcttgcccagggccttcccgtctcgcggcccggcctccctcacccggaag

SEQ ID NO: 11879 - RNA, 1804 nt, Homo sapiens
  source 1..1804: mol_type = other RNA
ctgaatagctgggactacaggtgtgcgccaccactcctggctgattttgtattttcagtagggacagggtttcaccatgttggccaggctggtctcgaactcctggcctcaagtgatccacccgcctcagcctcccaaagtgctgggattacaggcgtgagcaaccgtgcccagcccataatttggatttttaaaccagaaagttactatggtcaatccaaaataacccaaagaacttgctaaagttatatcaataagcagctttttattgaaggactgaaagaattaaatagaaggcacagtagcactgtaaagctttctcagaacataataatctttttctatgtatgtgtggaacccagactttcttttttgttgttaaaaatgtcttctggacaatcagaaaatctttatttgtcatccttccctttggtctttctgtaaaccatttctcgaaaactggccagaatcttgttctctctctttcgtctctcttcttggttaaaggatgcaagggctctcttctcatcagcactgtagatctggttctcttttcgcagtcgcacagcctccattcggcgatgcctgctaccactcattacataacctgagcattcaaatgatgcaatttcttcacttgtcaagccaatttcacctcttcgtgggatacgttttccagcttttacatattcagccatagctgcaccttcaccaggtaacagagcatggccatagttcaaaggtttatcatcttgagaggtaagtgtttttggagcctctgggccaattaaatctgatggttcttcagcctttgttcgatccttccagggattttccagaaactcttcttgggattctttagagcttgaatcactggactcttttctgctcttcttagacctctttttcttatatttcttcgatctgtgtttcttcttcttttcctttttcttggctttctttgctctccttttgttatcttcatcactggagtctgtttcagaatcagagtcactgtcgctatcttcagaatacttcttatgttttcttttcgatgattttttctttctccttttcttggacctttcttttgaacggctagacttcttctttttttcttcttctgaagtagaagctgaagtagtgcttttctttggctcttcatcctccactggtgtatgttcatcagaatctggttcaggattctttggagaaagtccccatacttcaggagctcccaattctccaattctctctctctcacttaatctcttctgccgcaggctctcctccctctccttgtcgaggaggctaggccaaggcttgtcgctcccgtaggggcgcgagtagctgccgtaatagactgacgaggaggcagaagcgaaggggatgccccggggcgcagagggccgctctctagaacgcgaccgcgagcgtgagcggtaggactggtttcgggagccttggctgaggccacccagctgatgggtgagtccattccggtccccggaccgagagcaagagtgcgagcgagagcggcggccccgcggggagcgggcagatttgctgggcttcggactcttcgacgaactgcgacgtcttccccccgagcccgaggcctccctatccgggctgcgtgagccggacaccggagccatggctactggggggccccagcagccgtgggacaagggggcgctctcgcgagcctaggaagatgtctgttgccttggttcccgggacctgccgctgcggaacagcccaaatctgaggaaaccttggacacagttctgggtacttctgc

SEQ ID NO: 11880 - RNA, 4016 nt, Homo sapiens
  source 1..4016: mol_type = other RNA
ctgaatagctgggactacaggtgtgcgccaccatgcccagctaatttttgtatttttagtagagatggggtttcaccatattggccaggctggtctcaaacttctgacctcgtgatctgcccgcctcagcctcccaaagtgctgggattacaggcctgagccaccatgcctggcctggggttactattaatacaatagtctaggtgagggctgatgaaggcttaaaccaagacaaagaagtggggatgacaagcctttcaatgtttataagtatgccatatagataggatggccacatgatttgtgattcactgagggacacttctcagagtgaaatgggtatgtattaataatgataccaggacaacaggcatgcatttggaagtacaatcaccctgcacattagtcttttctaagttcagcttctagatgtccctcaccagcaccaacaatgctcagcttatttgattgtaacatactgaaaggaaacttgtttttaattttactggaggcaagacaaaaccaacaagcatcaggcatcctcttaactcagatgtcttttctgactcaattcagccagatttgactgctcagcccaactgagcatgcacaagaggagggcaaccatgttctttctttctgcaccacataggatgtgaaccacacatgctggaaagcagggcctccagctttcatttgcagactgggtggctcagacatcaggtcaacattaatggcttcactatgtctccaaaataggacttggcatctctcccagaccctccctcaaggcaggtaacttgtccgtctgtcttgttctctccaatatacttagcgtcaaacgcagtgtctagcacctagcaggagcctgacaaatacttattaaatattggagtgggcgtggtggggctgggcgtggtggctcatgcctgtaatcccagcactttgggaggccgaggagggtggataacctgaggtcaggagatcaaaaccagcctggccaacatggagaaaccctgtgtctgctaaaaatacaaaaattagccggactggtggttcacacctgtaatcccagctacttgggaggctgaggcacaagaatcgcttgaacctgagaggtggaggttgcagtgagctgagatcacaccactgcactccagcctaggcaacagaacaagactgtctcaaaaaaaaaaaaaaaggagtcatggtattttccttgtaagtattccctatgtgtataaaggttggccaaagctcctaccccattcccaatactcaaagatgccatgtcttccagttcactttcattaggttctgggtaagaaacagtcaaattaatcagaatttctggtgatgggcagtcaatatcttcctcaccatgttttcattagcaatgaaatgttgtatgagccaggggagccttcatagctttacactaacacagggcaatgaagacctaatttattctttttttttttttttttttttttgagatggagtctggctctgtcacccaggctggagcacagtggcatgatcccagctcactgcaagctctgcctcctggttcaagcaattctcctgcctcaacctcctgagtagctgggactacaggtgtgcaccaccacatccagctaatttttgtattttgggtagagacagggctttgccatgttggccaggctggtctcgaagtcctgacctcaagtgatctgcacaccttagcctcccaaagtgctgggattacaggcaagagccaccgcgcccagccaaagactcaatttcttgcttgatatagtggagcaacacaaaggaatcttccagctggttaccatccttctcaggatttcttttattttgggcttgcagtagctcaacctctatttccccctgcccctttgaaagttgatttctcctcagaggccctttccaagccagccttggactggctttcttggctttgcttggctattgtgtggtttcaactgagcagactgatatatgatttggatctgtctccctgcccaaatctcatgttgaatttaatccccagtgttggaggaggtgcctggtgggaggtgattggatcatgggggtggatttcctccttgctgttctcatgatagtgagttctcacgagatttggttgtttaaaagtgcatagcacctcccacttctttctttctcctgctccagactcgtaggacaggtctgcttctcttttgccttctgccttgattgtaagtttcctgaggcctccccagtcatgcttcctgtacagcctggggaaccatgagccaattaaacctcttttctttataaattacccagactcgaggctgggcctggtggctcacgcctgtaatcctaaccctttgagaggccaatgtgactggatggcctgagctcaggagctggagaccagcctgggcaacgtggtgaaaccccatctctactaaaatataaaaacttagccaggtgtagtgtgtgcctgtagtcccagctacttgggaggctgaggctggagaattgcttgaacccaggaggtggaggttgcagtgagccatgatcgcaccactgtactccagcctggagacagagcaagactctatctccaaaataaataaataaataaataaataaataaataaaattacccagtctcaggtagttctctgtacacacagacagtaacttttcccacctatttttccaaaaactgctcctgttctcagtcagtcctttcccaaactggagcctccctatagcccaacctgcaaaaattagggactcacttggaagtttattggtggaagtagagaagcaccttgttggaaacaccatcttacctctcccaaggtcacttggctcacagtggaaaaggagcattataagaggtggtagcaagtacacgtatgcaaggaagagcatgttttgcctaggtgtcaggctcccaagaagtgctctcctaggtaactggctatatgaacttgtagaaggtgctcattccagtcctcttgttcccagaggctgtggctcaaggcagctctcatgggtatattcaaattgattggagatgccactggagagggtatcttgtagctgctgcagttgtctatttcaatggcagtgtcattgttcctgtctgctgtgagctggggctttcctgagagctgtgagaaactgccactggtctgctcagccgccagcagcacgaggggctcgctgggctggggggatgacaggaggctgttttcaggtgttgtttctgtggagttggtgggcatcttgggcaccaggcagtgagtgaatttgattctcgggtctttggtggtgatggacaggcctttctgcagaattttcaccaagcggacccagaattgaaacacaatctctgggtgtttttcgtggagcttcagatagtagatcttttcggtcactgtcctaaccctcaggatgcgctggagccggtcgtagattcgtagctccacgtacttcagggggagaagcctgctgaggttgatgactggggcgtcaccaggtgtgctccaggtggtaaatggaccctggggccaggtaacattggccatcaggaggacattggggagtggcagggagggcaccgaggaggtgaccccgaggatcacggtggcagacccttcacagacatctctccagttcccgggcttagtgaccaaaatctcagcagtctctcaaagaatggcttaagacccttctggaaagccttcttcaactggataaagttgctttcaaacaccaccgagttggagaacaaattgaattctggagaatgaatcagttgacaaagaaggccattttccaccccaagttccactccagggcctggttccctgacctcaggtgggaggcccctgattttactcattggttcttggtaagaatgggcttgggaacatttctggggctccacgccgacccagcccaatgccaggatgttgatgtgatctgcccccacctccccagcatttcct

SEQ ID NO: 11881 - RNA, 4043 nt, Homo sapiens
  source 1..4043: mol_type = other RNA
ctgaatagctgggactacaggtgtgcgccaccatgcccagctaatttttgtatttttagtagagatggggtttcaccatattggccaggctggtctcaaacttctgacctcgtgatctgcccgcctcagcctcccaaagtgctgggattacaggcctgagccaccatgcctggcctggggttactattaatacaatagtctaggtgagggctgatgaaggcttaaaccaagacaaagaagtggggatgacaagcctttcaatgtttataagtatgccatatagataggatggccacatgatttgtgattcactgagggacacttctcagagtgaaatgggtatgtattaataatgataccaggacaacaggcatgcatttggaagtacaatcaccctgcacattagtcttttctaagttcagcttctagatgtccctcaccagcaccaacaatgctcagcttatttgattgtaacatactgaaaggaaacttgtttttaattttactggaggcaagacaaaaccaacaagcatcaggcatcctcttaactcagatgtcttttctgactcaattcagccagatttgactgctcagcccaactgagcatgcacaagaggagggcaaccatgttctttctttctgcaccacataggatgtgaaccacacatgctggaaagcagggcctccagctttcatttgcagactgggtggctcagacatcaggtcaacattaatggcttcactatgtctccaaaataggacttggcatctctcccagaccctccctcaaggcaggtaacttgtccgtctgtcttgttctctccaatatacttagcgtcaaacgcagtgtctagcacctagcaggagcctgacaaatacttattaaatattggagtgggcgtggtggggctgggcgtggtggctcatgcctgtaatcccagcactttgggaggccgaggagggtggataacctgaggtcaggagatcaaaaccagcctggccaacatggagaaaccctgtgtctgctaaaaatacaaaaattagccggactggtggttcacacctgtaatcccagctacttgggaggctgaggcacaagaatcgcttgaacctgagaggtggaggttgcagtgagctgagatcacaccactgcactccagcctaggcaacagaacaagactgtctcaaaaaaaaaaaaaaaggagtcatggtattttccttgtaagtattccctatgtgtataaaggttggccaaagctcctaccccattcccaatactcaaagatgccatgtcttccagttcactttcattaggttctgggtaagaaacagtcaaattaatcagaatttctggtgatgggcagtcaatatcttcctcaccatgttttcattagcaatgaaatgttgtatgagccaggggagccttcatagctttacactaacacagggcaatgaagacctaatttattctttttttttttttttttttttttgagatggagtctggctctgtcacccaggctggagcacagtggcatgatcccagctcactgcaagctctgcctcctggttcaagcaattctcctgcctcaacctcctgagtagctgggactacaggtgtgcaccaccacatccagctaatttttgtattttgggtagagacagggctttgccatgttggccaggctggtctcgaagtcctgacctcaagtgatctgcacaccttagcctcccaaagtgctgggattacaggcaagagccaccgcgcccagccaaagactcaatttcttgcttgatatagtggagcaacacaaaggaatcttccagctggttaccatccttctcaggatttcttttattttgggcttgcagtagctcaacctctatttccccctgcccctttgaaagttgatttctcctcagaggccctttccaagccagccttggactggctttcttggctttgcttggctattgtgtggtttcaactgagcagactgatatatgatttggatctgtctccctgcccaaatctcatgttgaatttaatccccagtgttggaggaggtgcctggtgggaggtgattggatcatgggggtggatttcctccttgctgttctcatgatagtgagttctcacgagatttggttgtttaaaagtgcatagcacctcccacttctttctttctcctgctccagactcgtaggacaggtctgcttctcttttgccttctgccttgattgtaagtttcctgaggcctccccagtcatgcttcctgtacagcctggggaaccatgagccaattaaacctcttttctttataaattacccagactcgaggctgggcctggtggctcacgcctgtaatcctaaccctttgagaggccaatgtgactggatggcctgagctcaggagctggagaccagcctgggcaacgtggtgaaaccccatctctactaaaatataaaaacttagccaggtgtagtgtgtgcctgtagtcccagctacttgggaggctgaggctggagaattgcttgaacccaggaggtggaggttgcagtgagccatgatcgcaccactgtactccagcctggagacagagcaagactctatctccaaaataaataaataaataaataaataaataaataaaattacccagtctcaggtagttctctgtacacacagacagtaacttttcccacctatttttccaaaaactgctcctgttctcagtcagtcctttcccaaactggagcctccctatagcccaacctgcaaaaattagggactcacttggaagtttattggtggaagtagagaagcaccttgttggaaacaccatcttacctctcccaaggtcacttggctcacagtggaaaaggagcattataagaggtggtagcaagtacacgtatgcaaggaagagcatgttttgcctaggtgtcaggctcccaagaagtgctctcctaggtaactggctatatgaacttgtagaaggtgctcattccagtcctcttgttcccagaggctgtggctcaaggcagctctcatgggtatattcaaattgattggagatgccactggagagggtatcttgtagctgctgcagttgtctatttcaatggcagtgtcattgttcctgtctgctgtgagctggggctttcctgagagctgtgagaaactgccactggtctgctcagccgccagcagcacgaggggctcgctgggctggggggatgacaggaggctgttttcaggtgttgtttctgtggagttggtgggcatcttgggcaccaggcagtgagtgaatttgattctcgggtctttggtggtgatggacaggcctttctgcagaattttcaccaagcggacccagaattgaaacacaatctctgggtgtttttcgtggagcttcagatagtagatcttttcggtcactgtcctaaccctcaggatgcgctggagccggtcgtagattcgtagctccacgtacttcagggggagaagcctgctgaggttgatgactggggcgtcaccaggtgtgctccaggtggtaaatggaccctggggccaggtaacattggccatcaggaggacattggggagtggcagggagggcaccgaggaggtgaccccgaggatcacggtggcagacccttcacagacatctctccagttcccgggcttagtgacctggaaatcagcctcaggtacatgggtcaaaatctcagcagtctctcaaagaatggcttaagacccttctggaaagccttcttcaactggataaagttgctttcaaacaccaccgagttggagaacaaattgaattctggagaatgaatcagttgacaaagaaggccattttccaccccaagttccactccagggcctggttccctgacctcaggtgggaggcccctgattttactcattggttcttggtaagaatgggcttgggaacatttctggggctccacgccgacccagcccaatgccaggatgttgatgtgatctgcccccacctccccagcatttcct

SEQ ID NO: 11882 - RNA, 3984 nt, Homo sapiens
  source 1..3984: mol_type = other RNA
ctgaatagctgggactacaggtgtgcgccaccatgcccagctaatttttgtatttttagtagagatggggtttcaccatattggccaggctggtctcaaacttctgacctcgtgatctgcccgcctcagcctcccaaagtgctgggattacaggcctgagccaccatgcctggcctggggttactattaatacaatagtctaggtgagggctgatgaaggcttaaaccaagacaaagaagtggggatgacaagcctttcaatgtttataagtatgccatatagataggatggccacatgatttgtgattcactgagggacacttctcagagtgaaatgggtatgtattaataatgataccaggacaacaggcatgcatttggaagtacaatcaccctgcacattagtcttttctaagttcagcttctagatgtccctcaccagcaccaacaatgctcagcttatttgattgtaacatactgaaaggaaacttgtttttaattttactggaggcaagacaaaaccaacaagcatcaggcatcctcttaactcagatgtcttttctgactcaattcagccagatttgactgctcagcccaactgagcatgcacaagaggagggcaaccatgttctttctttctgcaccacataggatgtgaaccacacatgctggaaagcagggcctccagctttcatttgcagactgggtggctcagacatcaggtcaacattaatggcttcactatgtctccaaaataggacttggcatctctcccagaccctccctcaaggcaggtaacttgtccgtctgtcttgttctctccaatatacttagcgtcaaacgcagtgtctagcacctagcaggagcctgacaaatacttattaaatattggagtgggcgtggtggggctgggcgtggtggctcatgcctgtaatcccagcactttgggaggccgaggagggtggataacctgaggtcaggagatcaaaaccagcctggccaacatggagaaaccctgtgtctgctaaaaatacaaaaattagccggactggtggttcacacctgtaatcccagctacttgggaggctgaggcacaagaatcgcttgaacctgagaggtggaggttgcagtgagctgagatcacaccactgcactccagcctaggcaacagaacaagactgtctcaaaaaaaaaaaaaaaggagtcatggtattttccttgtaagtattccctatgtgtataaaggttggccaaagctcctaccccattcccaatactcaaagatgccatgtcttccagttcactttcattaggttctgggtaagaaacagtcaaattaatcagaatttctggtgatgggcagtcaatatcttcctcaccatgttttcattagcaatgaaatgttgtatgagccaggggagccttcatagctttacactaacacagggcaatgaagacctaatttattctttttttttttttttttttttttgagatggagtctggctctgtcacccaggctggagcacagtggcatgatcccagctcactgcaagctctgcctcctggttcaagcaattctcctgcctcaacctcctgagtagctgggactacaggtgtgcaccaccacatccagctaatttttgtattttgggtagagacagggctttgccatgttggccaggctggtctcgaagtcctgacctcaagtgatctgcacaccttagcctcccaaagtgctgggattacaggcaagagccaccgcgcccagccaaagactcaatttcttgcttgatatagtggagcaacacaaaggaatcttccagctggttaccatccttctcaggatttcttttattttgggcttgcagtagctcaacctctatttccccctgcccctttgaaagttgatttctcctcagaggccctttccaagccagccttggactggctttcttggctttgcttggctattgtgtggtttcaactgagcagactgatatatgatttggatctgtctccctgcccaaatctcatgttgaatttaatccccagtgttggaggaggtgcctggtgggaggtgattggatcatgggggtggatttcctccttgctgttctcatgatagtgagttctcacgagatttggttgtttaaaagtgcatagcacctcccacttctttctttctcctgctccagactcgtaggacaggtctgcttctcttttgccttctgccttgattgtaagtttcctgaggcctccccagtcatgcttcctgtacagcctggggaaccatgagccaattaaacctcttttctttataaattacccagactcgaggctgggcctggtggctcacgcctgtaatcctaaccctttgagaggccaatgtgactggatggcctgagctcaggagctggagaccagcctgggcaacgtggtgaaaccccatctctactaaaatataaaaacttagccaggtgtagtgtgtgcctgtagtcccagctacttgggaggctgaggctggagaattgcttgaacccaggaggtggaggttgcagtgagccatgatcgcaccactgtactccagcctggagacagagcaagactctatctccaaaataaataaataaataaataaataaataaataaaattacccagtctcaggtagttctctgtacacacagacagtaacttttcccacctatttttccaaaaactgctcctgttctcagtcagtcctttcccaaactggagcctccctatagcccaacctgcaaaaattagggactcacttggaagtttattggtggaagtagagaagcaccttgttggaaacaccatcttacctctcccaaggtcacttggctcacagtggaaaaggagcattataagaggtggtagcaagtacacgtatgcaaggaagagcatgttttgcctaggtgtcaggctcccaagaagtgctctcctaggtaactggctatatgaacttgtagaaggtgctcattccagtcctcttgttcccagaggctgtggctcaaggcagctctcatgggtatattcaaattgattggagatgccactggagagggtatcttgtagctgctgcagttgtctatttcaatggcagtgtcattgttcctgtctgctgtgagctggggctttcctgagagctgtgagaaactgccactggtctgctcagccgccagcagcacgaggggctcgctgggctggggggatgacaggaggctgttttcaggtgttgtttctgtggagttggtgggcatcttgggcaccaggcagtgagtgaatttgattctcgggtctttggtggtgatggacaggcctttctgcagaattttcaccaagcggacccagaattgaaacacaatctctgggtgtttttcgtggagcttcagatagtagatcttttcggtcactgtcctaaccctcaggatgcgctggagccggtcgtagattcgtagctccacgtacttcagggggagaagcctgctgaggttgatgactggggcgtcaccaggtgtgctccaggtggtaaatggaccctggggccaggtaacattggccatcaggaggacattggggagtggcagggagggcaccgaggaggtgaccccgaggatcacggtggcagacccttcacagacatctctccagttcccgggcttagtgacctggaaatcagcctcaggtacatgggtctggataaagttgctttcaaacaccaccgagttggagaacaaattgaattctggagaatgaatcagttgacaaagaaggccattttccaccccaagttccactccagggcctggttccctgacctcaggtgggaggcccctgattttactcattggttcttggtaagaatgggcttgggaacatttctggggctccacgccgacccagcccaatgccaggatgttgatgtgatctgcccccacctccccagcatttcct

SEQ ID NO: 11883 - RNA, 3957 nt, Homo sapiens
  source 1..3957: mol_type = other RNA
ctgaatagctgggactacaggtgtgcgccaccatgcccagctaatttttgtatttttagtagagatggggtttcaccatattggccaggctggtctcaaacttctgacctcgtgatctgcccgcctcagcctcccaaagtgctgggattacaggcctgagccaccatgcctggcctggggttactattaatacaatagtctaggtgagggctgatgaaggcttaaaccaagacaaagaagtggggatgacaagcctttcaatgtttataagtatgccatatagataggatggccacatgatttgtgattcactgagggacacttctcagagtgaaatgggtatgtattaataatgataccaggacaacaggcatgcatttggaagtacaatcaccctgcacattagtcttttctaagttcagcttctagatgtccctcaccagcaccaacaatgctcagcttatttgattgtaacatactgaaaggaaacttgtttttaattttactggaggcaagacaaaaccaacaagcatcaggcatcctcttaactcagatgtcttttctgactcaattcagccagatttgactgctcagcccaactgagcatgcacaagaggagggcaaccatgttctttctttctgcaccacataggatgtgaaccacacatgctggaaagcagggcctccagctttcatttgcagactgggtggctcagacatcaggtcaacattaatggcttcactatgtctccaaaataggacttggcatctctcccagaccctccctcaaggcaggtaacttgtccgtctgtcttgttctctccaatatacttagcgtcaaacgcagtgtctagcacctagcaggagcctgacaaatacttattaaatattggagtgggcgtggtggggctgggcgtggtggctcatgcctgtaatcccagcactttgggaggccgaggagggtggataacctgaggtcaggagatcaaaaccagcctggccaacatggagaaaccctgtgtctgctaaaaatacaaaaattagccggactggtggttcacacctgtaatcccagctacttgggaggctgaggcacaagaatcgcttgaacctgagaggtggaggttgcagtgagctgagatcacaccactgcactccagcctaggcaacagaacaagactgtctcaaaaaaaaaaaaaaaggagtcatggtattttccttgtaagtattccctatgtgtataaaggttggccaaagctcctaccccattcccaatactcaaagatgccatgtcttccagttcactttcattaggttctgggtaagaaacagtcaaattaatcagaatttctggtgatgggcagtcaatatcttcctcaccatgttttcattagcaatgaaatgttgtatgagccaggggagccttcatagctttacactaacacagggcaatgaagacctaatttattctttttttttttttttttttttttgagatggagtctggctctgtcacccaggctggagcacagtggcatgatcccagctcactgcaagctctgcctcctggttcaagcaattctcctgcctcaacctcctgagtagctgggactacaggtgtgcaccaccacatccagctaatttttgtattttgggtagagacagggctttgccatgttggccaggctggtctcgaagtcctgacctcaagtgatctgcacaccttagcctcccaaagtgctgggattacaggcaagagccaccgcgcccagccaaagactcaatttcttgcttgatatagtggagcaacacaaaggaatcttccagctggttaccatccttctcaggatttcttttattttgggcttgcagtagctcaacctctatttccccctgcccctttgaaagttgatttctcctcagaggccctttccaagccagccttggactggctttcttggctttgcttggctattgtgtggtttcaactgagcagactgatatatgatttggatctgtctccctgcccaaatctcatgttgaatttaatccccagtgttggaggaggtgcctggtgggaggtgattggatcatgggggtggatttcctccttgctgttctcatgatagtgagttctcacgagatttggttgtttaaaagtgcatagcacctcccacttctttctttctcctgctccagactcgtaggacaggtctgcttctcttttgccttctgccttgattgtaagtttcctgaggcctccccagtcatgcttcctgtacagcctggggaaccatgagccaattaaacctcttttctttataaattacccagactcgaggctgggcctggtggctcacgcctgtaatcctaaccctttgagaggccaatgtgactggatggcctgagctcaggagctggagaccagcctgggcaacgtggtgaaaccccatctctactaaaatataaaaacttagccaggtgtagtgtgtgcctgtagtcccagctacttgggaggctgaggctggagaattgcttgaacccaggaggtggaggttgcagtgagccatgatcgcaccactgtactccagcctggagacagagcaagactctatctccaaaataaataaataaataaataaataaataaataaaattacccagtctcaggtagttctctgtacacacagacagtaacttttcccacctatttttccaaaaactgctcctgttctcagtcagtcctttcccaaactggagcctccctatagcccaacctgcaaaaattagggactcacttggaagtttattggtggaagtagagaagcaccttgttggaaacaccatcttacctctcccaaggtcacttggctcacagtggaaaaggagcattataagaggtggtagcaagtacacgtatgcaaggaagagcatgttttgcctaggtgtcaggctcccaagaagtgctctcctaggtaactggctatatgaacttgtagaaggtgctcattccagtcctcttgttcccagaggctgtggctcaaggcagctctcatgggtatattcaaattgattggagatgccactggagagggtatcttgtagctgctgcagttgtctatttcaatggcagtgtcattgttcctgtctgctgtgagctggggctttcctgagagctgtgagaaactgccactggtctgctcagccgccagcagcacgaggggctcgctgggctggggggatgacaggaggctgttttcaggtgttgtttctgtggagttggtgggcatcttgggcaccaggcagtgagtgaatttgattctcgggtctttggtggtgatggacaggcctttctgcagaattttcaccaagcggacccagaattgaaacacaatctctgggtgtttttcgtggagcttcagatagtagatcttttcggtcactgtcctaaccctcaggatgcgctggagccggtcgtagattcgtagctccacgtacttcagggggagaagcctgctgaggttgatgactggggcgtcaccaggtgtgctccaggtggtaaatggaccctggggccaggtaacattggccatcaggaggacattggggagtggcagggagggcaccgaggaggtgaccccgaggatcacggtggcagacccttcacagacatctctccagttcccgggcttagtgacctggataaagttgctttcaaacaccaccgagttggagaacaaattgaattctggagaatgaatcagttgacaaagaaggccattttccaccccaagttccactccagggcctggttccctgacctcaggtgggaggcccctgattttactcattggttcttggtaagaatgggcttgggaacatttctggggctccacgccgacccagcccaatgccaggatgttgatgtgatctgcccccacctccccagcatttcct

SEQ ID NO: 11884 - RNA, 4151 nt, Homo sapiens
  source 1..4151: mol_type = other RNA
ctgaatagctgggactacaggtgtgcgccaccatgcccagctaattttttcgtatttttagtagagatgtactttatatttttagtaaagatggggttttgccatgttggccaggctggtcttgaactcctgacctcaggtgatctgcctaccttggcctcccaaagtgctgggattacaggcatgagccaccatgcctggccaattctttctacttataaaaaattcttatgttcttggtggataaactggttgcataataaaattattttagttcaatggatagattcctgccagattcacccagttgccaattatctgaactgaaacaaataaaaatatcaagtaaatttttatatcaccctccaaaagcttgggaattatattctgccacttaaggctttactggacttactgtccataaaattttctaattacaaagtggaagtctattcaagagtgtttatacgtagaaaagttaggaagacagaaacttgaaaaagactgtcttcagaaaaacctctctgtttccaataggaatataccatggtcataattttatgctcacatgtcacacaaagataggctgttactggagagttattttgtacagttggtatttttaattctccattttttgttcacaaatgtagtcttcattttaatgaagaagagaagtctgtgtttcttccatgttgaactcctctgtccacttctgcaggtcttgtgcattatgcatcgtccataactttgcaaaatacttgagtctctttcttttcgtatttattaatccttccagctcttttgacttgtgagctgctttcttcaaaatttctccaggaacatctgctagtttagccacatttaatccataactccttgctgcaattcctctagttatttggtaaaggaaggtgacaaaatcagggacttgttctgctgcgcctggatccagtttgctttcatcctcactgaccaagaatcccatgtggtaattccccacctggtgtgagtaatttttttctagttcacaaactggcggataatgggtgacaaacagggttaaggatttcacatctctgatgaaatactcaagtgtagcataggcaatggcaattccatcatgagtgctcgtccctcttcctagttcatccaagataaccaaggactgtgatgttgcttttctgattatttctgctgtgtcagtcagttcttccataaatgtactctgtcctttatatatattgtctgcagcacccatccttgtgaaaatgccatccacaatcccaattgtcgcttcttctgcaggaacataggagccaatctgagccatgatggtaatcaatgcaacttgttttatgtaggagctctttccacccatgtttggtccggtaattatcattactctctctgagtcctctgataaatctgtattatttgggacatattgatcctgttctcccagcaacacatcaatcacagggtgccttccattttttattacaatttttctttcttcttgtacagttggtctgcagtaatctccttgcttagcgaccttggccagggagaaaatgcagtcaacagttgctaggtgatgcactgctttacacaaggagtgataatgttcactgaatttctctagaaaatcaagccattcagcactgcagtcaaggactagctgctcccggagctgattcagatgtctgtaattttctacaataaaaggagagtgaaagcggctcacagcttttgtgcttccaacctttacccaatcagttggtatacaagatacagcagagttctttatttctatcataaactcctgtcctgatactgtcacatattgtgcagaaggattttttagtatttttcgtatttcttgcaaatgcattcggatctcgtcaataacaccttgaatttcatccttcctcttttttattaaagggaagtcagaaaggtctttaaataattcagttttatccccaactttggcagcttgttcattgagtatctttaagtaatgctccactggactgaggagttcaggaatttctaaaataacggtccggagcaagtctgactgaatgtgggaattaacagcaggtattattgcttgaaattctgactttaggtgatataaagttttgacaatcaagaagaactcttgggtagaacattttttgtgataaatgctacagagtcccctctctatgtcgggcaatttacgtagatgattttctatctgaccaaacacactagattctgaatggagaacttccgatacagcatcaagccgggcatttatttcccttaatttaaggagtggctgggtcacccacttctttaacttccgtctcccaaatgaagttttagtgtggtctaaaacccacagcaaacttcctttggttttcatatcagtctgattctgtaggatttccagattccttaatgttgttccattaattgtcataaattccattttacttgatagctgtttaaaattctcaggtttggagagcatcttttccaagttgaattctttgaggtattttatgatggcagccaaagagcaaatcacaggcttctctaagttaacaatgccagaaataatttgagaacctttgatgtcaactgtatcttttgcataaaactctgtaactgcctggaaagcatggctgtattcaaaataaatgttatccatcctttcgactcgaattctgtcatcctgcacactaacagatgtggctctgtggatgagcgcctctgtttgctcggacaaggccgaaggaagcagcagctctactggctgcaggcttgacatccgggtttctagctctgaacgagaagcagagtcctggaaactatcaaacacaacctcgcctgtggcaggctgcactcccacaatgccaataaaaatgttgcccttttttttgtccctaacattttccttattttcagagatgcacagaagatagctggtagaagtatcagtcattatctcatcaacatttacagcatcatccagcttgattaggggattcacatcttctccaataagtgtagattttgtataaagggcagtcaatttccgggaaaagagtgaacttctgttgtctccaatggcctttaatgctgcagtttcagtttgcttcacaactcccaccttatatccttttgccaccaggcggcgtacatgaacaaacagtctgtgagtaggtatacttgctgtcataaagttgtgatctaaatggcaataaatattgagctctcgggctgcaatctctgcatcttccccaaagaatctatacttatatccacattccacacacaaaactgcatctttgtgctgctgcttcatttctatgtattgtaattctagcggcgtatagatgcttttggaccgtttgttagctgatttggaagcagttttctgtaaattttcatgacttgtatttgatgatccaaactgactgagatcaaaaagtgttgtgtccttttgattaatttgacgtttcgaatcttcagaagaaactgcattctttgcgtgtagaagactgatatcatcaaaatcagtacattttggcagaactgcaaatctctcctgcagagattctgtctggactctactttgaggaagggcagaatcgcagcagaattctttcaatttttccagagactttgaaacattcctggtcctcagacatttctttggctcagagttgccagacattcccagatcacttcctccttccttttgttggactttctttactttctttttaacaggcccatcattttccaatggtctcttctttcttctgtcaatttctgtagctatgtgcggcggcagctggggcgggaaggcgggagctgggggcgctgggggcgctgcggccgctgcggccgctgcagccgctgcagcgccagggtccacctggtcggctgcacctgtggaggaggaggtggatttcaggcttcccgtagactggaagaatcggctcaaaaccgcttgcctcgcaggggctgagctggaggcagcgaggccgcccgacgcaggcttccggcgagacatggcagggcaaggatggcagcccggcggcagggcctggcgaggagcgcgagcccgcggccgcagttcccaggcgtct

SEQ ID NO: 11885 - RNA, 2999 nt, Homo sapiens
  source 1..2999: mol_type = other RNA
ctgaatagctgggactacaggtgtgcgccaccatgcccagctaattttttgtattttagtagagacggggtttcaccatgttggccaggagggtctcaatctcctgccctcatgatctgcccgccttggcctcccaaagccccctttttaatttttttttgtagagacgaggtctcgctatgttgcccaggctagtctcgaactcctgggctgcagcgatccttctgcctgggcctcccaaagtgctgggattaccagtgaacctccatacccagcccaaatatgcattcttggaattatctgcaattgcccaagaatgtacaagcaactcctgagaataaaccaaaaaagataagaaactccatgagaaaatgggcaatgcacaggaagggaaaccagaaaggctaagtgaaaaaattccccaaattaatgctgatcagatgaatgtatgttaaagcactgcaccactatctacccatgagactggcaaaaattaggtagtctggcaatacaagtgctggcaaggataaggagaaaagggcggcctcaagtaggagggtcagtcaccgttctaaagaaaatctggaaaaccaaagagaaactgacctctgtgacctataggcccatcctgggtacacatgccacacaagcacagaagggaacacacgaaaggatgtttatcgtggcctgtatccggtgccaaggggtcaggggcacccaggtgtcccccactttaggcaatgtgtgtaaactgcaattgacattgtggagtgccacatggcaggtcaaagcaatactgcatttctagaagagtcaatggggctagatcttagcacacattgagtgaaaacagcataagacctattgcacaatagcactatgtacagtaaaagcacatattcacacatgaaacgtggtattttacaaatacattcatattcaaagacatgggtgcttatgggagaggatggtgtaaagaaagggaaaaaagccataaaaccagagaatctttgcatgggactgtattcctgagatcccaaaccaaagggatgaatgtgctgttatgccttaaatgtgtgcaccaggaaatgcaaactagaaagggtggctctgaagggtcctcaggtgaggaagacccccagggctgagaatccaccaccttcatccttcaaaagagtacctcagttgtctgcttacgcttcagccagcatgtgtgagcttggtcatttcctgcaagccaggcaaccacaccagtgtataagcctcaagcaaatgtcactcccaagccccaaatgggactaaggcctctgctgggctaggcgtggtgtaaatcccaggcctggaagctcctacccaaccctcatttgtttcaactcactttcaatatgtgcatagtttcataaagcagacatttccatgaggaaaagaggatggtggtgaaaggggaggggtgaagggacatctccaagtcacagaggctgcaaaactcagcatgacttgtggacggagccacaggccacccagggcaacaacacccacataactcaccaagtggttaacggctctaaaccagggtcaacaggagaggggacaaaagtcactccttgattttgctgcagcttaaagataagttctacctcagcttatgctagcccttatggggcaaaaaagggaaagtcattctccccaagtccaggctgggccgtcaaacagggagtggggtgtcagccccagacctcaatgaggtccccagattccatgcccaggtcagctggcagctccctgcctgaaagctttgtcccatcaaagaagaaggagagcttccgtcccgacagtcccatggcctcctcatagtgggacatgagggtctttagaggggaatctcgagacagtgagacttccagtgtctggtgtttctcctttccctgcacccggagctggagctgttgggacgtctctgtggcctctggagaacttgttagtaccacacagtcaatgatgtcagccactccgagctttagggtcctgggagtggcagtaggtgatagctctgtctctccaaaaagcaaaaggatcctgcttggggacaccccaaggtgggtggccatgtggtccaccacactctgcaggggctccgacatcctgaggggcaatctgaccaggtcagcccggcaacggattttgagtgggaagagtcggggggtctctgggagggtgggcccttccaccaagaccacttcatcctcttggccctgttgctcttgaccctgaggtggcttggggctcagacaggaacggagatcctggaggcgcttgttcacctcacttaacttcttgagtgcccgagtatgcgttctgcttttggtccttggtgaaggtggggacagaggagagttgtccagatccagaaactctgtctttttcttctcttctttatccttagtcctcagctttgtcttccagggagagcctggtgatggggagccctcatggtagagaccactcgaatctgccagctctgcctcttcctcatcccctggagggtagagtttcaggagggatagatcatctgggataaggcgaaggctgcttttaaccttccccgagtacaccggaaccagcggcgcctcccccggatccagcaccagccgccgccgccgcctgaccggctcccgcgggggtcctgcgggccgcctgtcctccccttcgctgtcactgttgctgttatcccgggacgcgaccggccccgggggctccgggggctccacctcaacctcgtccgcggcaccgcgagcggtggcgacctccagaatttcctcatcgctgtcggtgaccaagtccacagacactacgtccagcgtgccccgggatggagaccgctgggcccgaggacgccggccccgaccgccccagccgccccgaccccctcggccggcaccgctacctccggaccagcggccccgcttccccacaggctccgccatggcacactttcctcc

SEQ ID NO: 11886 - RNA, 2720 nt, Homo sapiens
  source 1..2720: mol_type = other RNA
ctgaatagctgggactacaggtgtgcgccaccatgcccagctgatttttatatttttagtagagacagggttttacaatgttggccaggatggtcttgatctcttgacctcatgatccacctgccttggcctcccaaagtgctgggattacaggtgtgagccaccgcatccggccaggaaattacttttaaagcaaataggaggctgggtgcggtggctcacgcctgtaatcccagcactttgggaggccgaggcgggaggatcacctgaggtcgggagttggagaccagcatgaccaaggagaaacaccgtctctactaaaaatacaaaattagccaggtgtgatggcgcatgcctgtaatcccagctactcgggaggctgaggcaggagaagcgcttgaacccaggaagcggaggttgcagcaggccgagatcgccaccattgcactccagcctgggcaacaagagcaaaattccatctcagaaataaataaataaatagtaagaaaacaagtggaagggatgaaacaggctgcacattatttttctttcaattatatgggttgccttaatcatagaatgaagaggaccaagtgaaaaacagccaagtagcaataaagaggaaaacaagcccagagggcagaggagcctggacagtttgcagggcagagcctagcagacctttctggaaaagggagtggggaggctgagggagggtatttgctaccctgaatgtactcactatagcacttgcaagaactaaggtctaatcaatgttccagaactggagtcagacatgagttgtaccctattgcccagcctccccctccatgcctttcccctgcccctacacaccctggctatgctgaactacttgcgatttcccagctataatatgcattacatgatcctgagcaaacacagaggctaccctccttctgtctgggattcccagtcaacttcgggtcccagcgcaggcattccgtcgcctgtggggccatcctagggagacatagttgctccttctcctttgttctcagtgtactttgcctacacctctcttctccattaaaacacttctttcagagttgtgtttgcacgtctgtctttccatcagactctaagctccttgaaggcagaagcctgtgtctatttatccatttatctctgctgcttacaacagtgcctcgcttacagtagatgataaatcaacatttacaggatacaggggcaagtgggatcgggctctccctatcttaattctacgataaggaaaaagaaataagaacggctgagcgctggggttctgtatatcgtctgaagaaattgctaaaatatgacttttgcatctagcatccctggttcaagtgaaaccacaggaacaaactcagaggggcatcagaagtggcccttttgtcctcaaacttcagctgctacgtgaagataaaattaaccccaatcgggctcctccggccaggtgggtatgccatgagctttcctccgccctccagagctgaagcttggactgtctcaagctctatgaagctgcaggacttgacttcaatggagtgggccatccacacagccaggattcttcccctgctaatacagcagcagtgggaccgccttgcagtaggcacagcggagatgtgccctgccaggtccccaggtgagaacacacgaagaggtgccacagaaggaaaggcgccttaagacatcagtcatctccatcaggccacgcagcagcaatcttcaacttctgattacgaggtggaagcagttctgaaaactacgcctgagggggcaaatgggaaggatacccaacaactggtttcagggggttctcagagaggctgtgagcaggtggctacagctgctggcagttcacacacagtcctcctcatgctcagagaccaaaggtgaagaaacaaaggccatgcaatggacttcctctttttgtttaatttatttaagaccacctccttacaacttccagagagaaaatacaaaacaagaaacagacttggtttcaaatgcataaccaggtgctggagtttaaagcattactgataacattgttacagaagaatggcagcttactccagggcacttcagtattcctgaggaataaacatgatttctcttgtcctcccgctgggatgttctcaggtgaagtcactgctcctgctcctgaagcttctctgtctgctcctttcggttctccccacaatcagctctgatgccaggaaagcgaggagccagggagtggtggaaaaggccggctgccggcttcagtgccacacagctgcgcctcttcttgcatggtccctgtgatgacctcactcttgctttggtgcagagatggctcccctactcccatctctccagcagacatgggctggctgcaggcagctgacggtttcagcaggtttttgacatattttccatgtagaagatatggagcctggaaatcatgctgacagttggaataagccattcctaatcccatgccagaaccgaaggctaatggccacattcttcttttaaagaaggtaagtgagaaaacaattcctaatccaaaaccagtacctatcttcacgaccgcatccgccagacaccggtcccacttcctgccgagctccgactcagacatgttccccacccgcgcctccagctttcctctcggccggcccccgcgctccgacccctgaaagtctcgc

SEQ ID NO: 11887 - RNA, 2431 nt, Homo sapiens
  source 1..2431: mol_type = other RNA
ctgaatagctgggactacaggtgtgcgccaccatgcccagctgatttttatatttttagtagagacagggttttacaatgttggccaggatggtcttgatctcttgacctcatgatccacctgccttggcctcccaaagtgctgggattacaggtgtgagccaccgcatccggccaggaaattacttttaaagcaaataggaggctgggtgcggtggctcacgcctgtaatcccagcactttgggaggccgaggcgggaggatcacctgaggtcgggagttggagaccagcatgaccaaggagaaacaccgtctctactaaaaatacaaaattagccaggtgtgatggcgcatgcctgtaatcccagctactcgggaggctgaggcaggagaagcgcttgaacccaggaagcggaggttgcagcaggccgagatcgccaccattgcactccagcctgggcaacaagagcaaaattccatctcagaaataaataaataaatagtaagaaaacaagtggaagggatgaaacaggctgcacattatttttctttcaattatatgggttgccttaatcatagaatgaagaggaccaagtgaaaaacagccaagtagcaataaagaggaaaacaagcccagagggcagaggagcctggacagtttgcagggcagagcctagcagacctttctggaaaagggagtggggaggctgagggagggtatttgctaccctgaatgtactcactatagcacttgcaagaactaaggtctaatcaatgttccagaactggagtcagacatgagttgtaccctattgcccagcctccccctccatgcctttcccctgcccctacacaccctggctatgctgaactacttgcgatttcccagctataatatgcattacatgatcctgagcaaacacagaggctaccctccttctgtctgggattcccagtcaacttcgggtcccagcgcaggcattccgtcgcctgtggggccatcctagggagacatagttgctccttctcctttgttctcagtgtactttgcctacacctctcttctccattaaaacacttctttcagagttgtgtttgcacgtctgtctttccatcagactctaagctccttgaaggcagaagcctgtgtctatttatccatttatctctgctgcttacaacagtgcctcgcttacagtagatgataaatcaacatttacaggatacaggggcaagtgggatcgggctctccctatcttaattctacgataaggaaaaagaaataagaacggctgagcgctggggttctgtatatcgtctgaagaaattgctaaaatatgacttttgcatctagcatccctggttcaagtgaaaccacaggaacaaactcagaggggcatcagaagtggcccttttgtcctcaaacttcagctgctacgtgaagataaaattaaccccaatcgggctcctccggccaggtgggtatgccatgagctttcctccgccctccagagctgaagcttggactgtctcaagctctatgaagctgcaggacttgacttcaatggagtgggccatccacacagccaggattcttcccctgctaatacagcagcagtgggaccgccttgcagtaggcacagcggagatgtgccctgccaggtccccaggtgagaacacacgaagaggtgccacagaaggaaaggcgccttaagacatcagtcatctccatcaggccacgcagcagcaatcttcaacttctgattacgaggtggaagcagttctgaaaactacgcctgagggggcaaatgggaaggatacccaacaactggtttcagggggttctcagagaggctgtgagcaggtggctacagctgctggcagttcacacacagtcctcctcatgctcagagaccaaaggtgaagaaacaaaggccatgcaatggacttcctctttttgtttaatttatttaagaccacctccttacaacttccagagagaaaatacaaaacaagaaacagacttggtttcaaatgcataaccaggtgctggagtttaaagcattactgataacattgttacagaagaatggcagcttactccagggcacttcagtattcctgaggaataaacatgatttctcttgtcctcccgctgggatgttctcaggtgaagtcactgctcctgctctttgacatattttccatgtagaagatatggagcctggaaatcatgctgacagttggaataagccattcctaatcccatgccagaaccgaaggctaatggccacattcttcctatcttcacgaccgcatccgccagacaccggtcccacttcctgccgagctccgactcagacatgttccccacccgcgcctccagctttcctctcggccggcccccgcgctccgacccctgaaagtctcgc

SEQ ID NO: 11888 - RNA, 2664 nt, Homo sapiens
  source 1..2664: mol_type = other RNA
ctgaatagctgggactacaggtgtgcgccaccatgcccagctgatttttatatttttagtagagacagggttttacaatgttggccaggatggtcttgatctcttgacctcatgatccacctgccttggcctcccaaagtgctgggattacaggtgtgagccaccgcatccggccaggaaattacttttaaagcaaataggaggctgggtgcggtggctcacgcctgtaatcccagcactttgggaggccgaggcgggaggatcacctgaggtcgggagttggagaccagcatgaccaaggagaaacaccgtctctactaaaaatacaaaattagccaggtgtgatggcgcatgcctgtaatcccagctactcgggaggctgaggcaggagaagcgcttgaacccaggaagcggaggttgcagcaggccgagatcgccaccattgcactccagcctgggcaacaagagcaaaattccatctcagaaataaataaataaatagtaagaaaacaagtggaagggatgaaacaggctgcacattatttttctttcaattatatgggttgccttaatcatagaatgaagaggaccaagtgaaaaacagccaagtagcaataaagaggaaaacaagcccagagggcagaggagcctggacagtttgcagggcagagcctagcagacctttctggaaaagggagtggggaggctgagggagggtatttgctaccctgaatgtactcactatagcacttgcaagaactaaggtctaatcaatgttccagaactggagtcagacatgagttgtaccctattgcccagcctccccctccatgcctttcccctgcccctacacaccctggctatgctgaactacttgcgatttcccagctataatatgcattacatgatcctgagcaaacacagaggctaccctccttctgtctgggattcccagtcaacttcgggtcccagcgcaggcattccgtcgcctgtggggccatcctagggagacatagttgctccttctcctttgttctcagtgtactttgcctacacctctcttctccattaaaacacttctttcagagttgtgtttgcacgtctgtctttccatcagactctaagctccttgaaggcagaagcctgtgtctatttatccatttatctctgctgcttacaacagtgcctcgcttacagtagatgataaatcaacatttacaggatacaggggcaagtgggatcgggctctccctatcttaattctacgataaggaaaaagaaataagaacggctgagcgctggggttctgtatatcgtctgaagaaattgctaaaatatgacttttgcatctagcatccctggttcaagtgaaaccacaggaacaaactcagaggggcatcagaagtggcccttttgtcctcaaacttcagctgctacgtgaagataaaattaaccccaatcgggctcctccggccaggtgggtatgccatgagctttcctccgccctccagagctgaagcttggactgtctcaagctctatgaagctgcaggacttgacttcaatggagtgggccatccacacagccaggattcttcccctgctaatacagcagcagtgggaccgccttgcagtaggcacagcggagatgtgccctgccaggtccccaggtgagaacacacgaagaggtgccacagaaggaaaggcgccttaagacatcagtcatctccatcaggccacgcagcagcaatcttcaacttctgattacgaggtggaagcagttctgaaaactacgcctgagggggcaaatgggaaggatacccaacaactggtttcagggggttctcagagaggctgtgagcaggtggctacagctgctggcagttcacacacagtcctcctcatgctcagagaccaaaggtgaagaaacaaaggccatgcaatggacttcctctttttgtttaatttatttaagaccacctccttacaacttccagagagaaaatacaaaacaagaaacagacttggtttcaaatgcataaccaggtgctggagtttaaagcattactgataacattgttacagaagaatggcagcttactccagggcacttcagtattcctgaggaataaacatgatttctcttgtcctcccgctgggatgttctcaggtgaagtcactgctcctgctctttgacatattttccatgtagaagatatggagcctggaaatcatgctgacagttggaataagccattcctaatcccatgccagaaccgaaggctaatggccacattcttcttttaaagaaggtaagtgagaaaacaattcctaatccaaaaccagtacagaagttgctgtgcattcaccatggcttcccttcagtctttgccaagccagagtatgaaattatcaagatggaccaggtgtggtggctcatgcctgtaatcctggcacgttgggaggccaaggtaggtggatcgtttggaccctgagttcaagaccagcctgggcaacatggtgaaaccccatctctatcttcacgaccgcatccgccagacaccggtcccacttcctgccgagctccgactcagacatgttccccacccgcgcctccagctttcctctcggccggcccccgcgctccgacccctgaaagtctcgc

SEQ ID NO: 11889 - RNA, 2558 nt, Homo sapiens
  source 1..2558: mol_type = other RNA
ctgaatagctgggactacaggtgtgcgccaccatgcccagctgatttttatatttttagtagagacagggttttacaatgttggccaggatggtcttgatctcttgacctcatgatccacctgccttggcctcccaaagtgctgggattacaggtgtgagccaccgcatccggccaggaaattacttttaaagcaaataggaggctgggtgcggtggctcacgcctgtaatcccagcactttgggaggccgaggcgggaggatcacctgaggtcgggagttggagaccagcatgaccaaggagaaacaccgtctctactaaaaatacaaaattagccaggtgtgatggcgcatgcctgtaatcccagctactcgggaggctgaggcaggagaagcgcttgaacccaggaagcggaggttgcagcaggccgagatcgccaccattgcactccagcctgggcaacaagagcaaaattccatctcagaaataaataaataaatagtaagaaaacaagtggaagggatgaaacaggctgcacattatttttctttcaattatatgggttgccttaatcatagaatgaagaggaccaagtgaaaaacagccaagtagcaataaagaggaaaacaagcccagagggcagaggagcctggacagtttgcagggcagagcctagcagacctttctggaaaagggagtggggaggctgagggagggtatttgctaccctgaatgtactcactatagcacttgcaagaactaaggtctaatcaatgttccagaactggagtcagacatgagttgtaccctattgcccagcctccccctccatgcctttcccctgcccctacacaccctggctatgctgaactacttgcgatttcccagctataatatgcattacatgatcctgagcaaacacagaggctaccctccttctgtctgggattcccagtcaacttcgggtcccagcgcaggcattccgtcgcctgtggggccatcctagggagacatagttgctccttctcctttgttctcagtgtactttgcctacacctctcttctccattaaaacacttctttcagagttgtgtttgcacgtctgtctttccatcagactctaagctccttgaaggcagaagcctgtgtctatttatccatttatctctgctgcttacaacagtgcctcgcttacagtagatgataaatcaacatttacaggatacaggggcaagtgggatcgggctctccctatcttaattctacgataaggaaaaagaaataagaacggctgagcgctggggttctgtatatcgtctgaagaaattgctaaaatatgacttttgcatctagcatccctggttcaagtgaaaccacaggaacaaactcagaggggcatcagaagtggcccttttgtcctcaaacttcagctgctacgtgaagataaaattaaccccaatcgggctcctccggccaggtgggtatgccatgagctttcctccgccctccagagctgaagcttggactgtctcaagctctatgaagctgcaggacttgacttcaatggagtgggccatccacacagccaggattcttcccctgctaatacagcagcagtgggaccgccttgcagtaggcacagcggagatgtgccctgccaggtccccaggtgagaacacacgaagaggtgccacagaaggaaaggcgccttaagacatcagtcatctccatcaggccacgcagcagcaatcttcaacttctgattacgaggtggaagcagttctgaaaactacgcctgagggggcaaatgggaaggatacccaacaactggtttcagggggttctcagagaggctgtgagcaggtggctacagctgctggcagttcacacacagtcctcctcatgctcagagaccaaaggtgaagaaacaaaggccatgcaatggacttcctctttttgtttaatttatttaagaccacctccttacaacttccagagagaaaatacaaaacaagaaacagacttggtttcaaatgcataaccaggtgctggagtttaaagcattactgataacattgttacagaagaatggcagcttactccagggcacttcagtattcctgaggaataaacatgatttctcttgtcctcccgctgggatgttctcaggtgaagtcactgctcctgctctttgacatattttccatgtagaagatatggagcctggaaatcatgctgacagttggaataagccattcctaatcccatgccagaaccgaaggctaatggccacattcttcttttaaagaaggtaagtgagaaaacaattcctaatccaaaaccagtacccttcctgtggctatctggactagacagaggctggaacatctgcagggatttctcgggtggacatcaattaccaggattctatcttcacgaccgcatccgccagacaccggtcccacttcctgccgagctccgactcagacatgttccccacccgcgcctccagctttcctctcggccggcccccgcgctccgacccctgaaagtctcgc

SEQ ID NO: 11890 - RNA, 2479 nt, Homo sapiens
  source 1..2479: mol_type = other RNA
ctgaatagctgggactacaggtgtgcgccaccatgcccagctgatttttatatttttagtagagacagggttttacaatgttggccaggatggtcttgatctcttgacctcatgatccacctgccttggcctcccaaagtgctgggattacaggtgtgagccaccgcatccggccaggaaattacttttaaagcaaataggaggctgggtgcggtggctcacgcctgtaatcccagcactttgggaggccgaggcgggaggatcacctgaggtcgggagttggagaccagcatgaccaaggagaaacaccgtctctactaaaaatacaaaattagccaggtgtgatggcgcatgcctgtaatcccagctactcgggaggctgaggcaggagaagcgcttgaacccaggaagcggaggttgcagcaggccgagatcgccaccattgcactccagcctgggcaacaagagcaaaattccatctcagaaataaataaataaatagtaagaaaacaagtggaagggatgaaacaggctgcacattatttttctttcaattatatgggttgccttaatcatagaatgaagaggaccaagtgaaaaacagccaagtagcaataaagaggaaaacaagcccagagggcagaggagcctggacagtttgcagggcagagcctagcagacctttctggaaaagggagtggggaggctgagggagggtatttgctaccctgaatgtactcactatagcacttgcaagaactaaggtctaatcaatgttccagaactggagtcagacatgagttgtaccctattgcccagcctccccctccatgcctttcccctgcccctacacaccctggctatgctgaactacttgcgatttcccagctataatatgcattacatgatcctgagcaaacacagaggctaccctccttctgtctgggattcccagtcaacttcgggtcccagcgcaggcattccgtcgcctgtggggccatcctagggagacatagttgctccttctcctttgttctcagtgtactttgcctacacctctcttctccattaaaacacttctttcagagttgtgtttgcacgtctgtctttccatcagactctaagctccttgaaggcagaagcctgtgtctatttatccatttatctctgctgcttacaacagtgcctcgcttacagtagatgataaatcaacatttacaggatacaggggcaagtgggatcgggctctccctatcttaattctacgataaggaaaaagaaataagaacggctgagcgctggggttctgtatatcgtctgaagaaattgctaaaatatgacttttgcatctagcatccctggttcaagtgaaaccacaggaacaaactcagaggggcatcagaagtggcccttttgtcctcaaacttcagctgctacgtgaagataaaattaaccccaatcgggctcctccggccaggtgggtatgccatgagctttcctccgccctccagagctgaagcttggactgtctcaagctctatgaagctgcaggacttgacttcaatggagtgggccatccacacagccaggattcttcccctgctaatacagcagcagtgggaccgccttgcagtaggcacagcggagatgtgccctgccaggtccccaggtgagaacacacgaagaggtgccacagaaggaaaggcgccttaagacatcagtcatctccatcaggccacgcagcagcaatcttcaacttctgattacgaggtggaagcagttctgaaaactacgcctgagggggcaaatgggaaggatacccaacaactggtttcagggggttctcagagaggctgtgagcaggtggctacagctgctggcagttcacacacagtcctcctcatgctcagagaccaaaggtgaagaaacaaaggccatgcaatggacttcctctttttgtttaatttatttaagaccacctccttacaacttccagagagaaaatacaaaacaagaaacagacttggtttcaaatgcataaccaggtgctggagtttaaagcattactgataacattgttacagaagaatggcagcttactccagggcacttcagtattcctgaggaataaacatgatttctcttgtcctcccgctgggatgttctcaggtgaagtcactgctcctgctctttgacatattttccatgtagaagatatggagcctggaaatcatgctgacagttggaataagccattcctaatcccatgccagaaccgaaggctaatggccacattcttcttttaaagaaggtaagtgagaaaacaattcctaatccaaaaccagtacctatcttcacgaccgcatccgccagacaccggtcccacttcctgccgagctccgactcagacatgttccccacccgcgcctccagctttcctctcggccggcccccgcgctccgacccctgaaagtctcgc

SEQ ID NO: 11891 - RNA, 4596 nt, Homo sapiens
  source 1..4596: mol_type = other RNA
ctgaatagctgggactacaggtgtgcgtcaccatacctggctaatttttctatttttagtagagaccaggttttgccatgttggccaggctggtctcaaactccaggcctcaagcgacttgcctgcctcagcctcccaaagtgccgggattacaggcatgagccatcgcacccgtcctccagtaccattttaaacaaatacatattgtggactacgcaccaatagaaattaaggtggcaaaaccgtatcattagtaaagtaagtgaaagccttagtctttttgtttattccttattccccaaaggagttactaagtgaaggaattttccagctgcctttatttttttgagacggagtcttgttctgttgcccaggctggagtgcagtggcacgatcttggctcaccacaacctcctcctcctgggttccagcgattctcctgcctcagcctccagagtagctgggactacaggcgcccaccaacatgcccggctaatttgtgtatttacagtagagatggggtttcattatgttggccaggatggtcttgaactcctgacctcaagatcagcctgcctcggcctcccacagtgctgggattacatgcgtgagccactgcgcccggccttccagctgcatttctgaggtcacaagtatggccttaaatgattgccctcaagaacacagcttttgaaggtaatcatatgcaagtaaattacaatcaaatggaactgtatgattattttattattttaatgctaaactgaacagtgaactgaaatcagaggagaaagaaaatcaagctagtggctcactctcaatagtgtcctctaattttattgatgcttcagttttcataaagtgcaataaacaaaataaataaatgaaaaaagctttgaagatttatatacagttttgaggttaagataaattactgactatattcctttcagccttttaactctgtgaaagctgtaacgtacattaaaagcacattgaactaggttaaataatgatctttcccccttagatcaatctagtattaaggagtatataattatgcaagttcattctataacacaaggctagactaaaaggaaaatttttgtgctacagactaaatccagatacagtcaggtgctgagcagtattcctggcttcaaaataggaggtatctgtttcatcatctggctgggggatgaaaggcatagtctgatgctgcagattttcccagtccacatcactgaagagaggatgacgttttagctctcttttcagaatattctggaatacttgttgtggtgtttcatcattgaaagggggaattcctgttagaaattcaaacaagcaaactccaagtgcccaccagtctaccgcaggaccatgggccctgcctagtaacagctcaggtgcaaggtagtctggggttcctagaattcgcccatcatcaacgggggccacccctcttctcacactcttcggagttcggtatggagttcccgacttgatctgatttggggtctgctgatgtggcatacaggatcttcttttttgagtaggggttatagccatgggatatgaaccactgtaggcacacgaaatatccattgcatctaaagaagtcatgttcattctggatggttctgagttattggatgcattaatatgactgttaaaacttcgaaaagcaacagcatttcttttagaggctaacgttttcagcacctccaaaggaggacctaacattttttggttactctcttgtacagcagggttctcgacaccttttggtgaggtcttttcttggcaatctggtgttacaataagtggatcttcaatatttgattcttcaaaagaggattctttgatgcttctatctgaatctaagggctgactttctaatggactttccattatagaaattccaggaaaagatgaatcagagttcatagaaatatttttagaagctctatcatcatcagaacatagaaaactagaacttaagtagtccctcttactattcttttcacagtcttcatcgagttcacacataaggttttttgctatcattggtataggtaatttttctggtgtttgttgtttatcagtaaaagaattgacaatgttctccttattagcacagtcattttgttgacttttgtgcactgatagcttaaggtcctgcacttcaactgttaagcctgtattttgatttgtataacaatttgtcatttcgttatgcttatactctacacaagtttttttattctgtataatttttttacaaggactggagtcaaccaactcaaaatttctttttaaacttcttttcccaaggtgctcttcagatatcccaccagaatccacagcccactgatttgactgatggaaacctaactgacttgtgtcagtgtccatatttatattatttacatccagttctactgcttcccaagaaacttccccagagaagcattttttagcaaggtttacacaagagcgtccagtggtgggaagggcactgctgttatgaatgggagaaagagctaactccagatcctttttattgaaacctttcgtctcaatggcatttgcagattttgcgcataacttttcaactgcattccaactcatcattgttgggcccaatgcttcatcactttcctggcaatctttttcccatttgggactgctgtggcattctgattccacactggatatgaaggtgtgggattgactactggcactggatgtggccagccttttcctagactggagtaaattagaagttagacacttcacaggcattcctgggttggaggcaactgtttcaagacatgattttagtaatttgctagaataaggcgtagtgtccttttgatctacagacatagggcatacgagtccttgagaaagctgtgatgtttcagacagacaggctgaaaggatgtttgcagggtcttgatttttttctgcaattggtgtgttaaatcccaacgagctgataagcgataacacttgtcctggggttcttgaataatcttgtctaggttttgccattgatggtgttgtaaggatatccatcatattaatatctctattcaaagtaacttttgaaaggccaaaatccgtcagtttaatatgaccctcattagaaataagcatattgtccggtttcaagtccctgtggatgattccatgtctgtgaaggtagtctagagccagtgctacttcagaaatatatttcacagccatctcttcatcaaaataaccatatatatgtaggagagacttgacatctcccccaataagatattccattaccaagtagacattgtttgcagactgcagtgaataatacaaatggacaatgaatgggcttttgcttagtgccagtgcatctctctcagcttggacctgatgagtcatatttttgttgatcatgtctgcttttttaacaacctttactgcatacaatttgccgcctttctgccccagatacactttcccgaaggcgccccggctaatgggcttcactatgctgaattcctcaatggagggcggttttggcactgcgatcctattcacgccctcctcagtcgccgcgcctcctccaggctccttcttgcttcccgcggtgggatccatcgctggacagcatacagcggccccgcagacactgcccctccgcgagcagccactcccgccaactgggttcaaagtgaggctccgcccacgccgcgcgcggccgtgacgtcaccccgccgccgcgccccgccctcgtcacctcccctacgcagacgcggacggagggggcgtcgggaaagccccgacttcgcagccttacactcttcgtgggcggcgaccgcggccccactgacatcattcctcatgagggaggaggcacaaacagttctgggccgaccagaaaaaggacgactgggacttgactctgaatcgcaggatttgaagagatttctcctggcttcccaacgaggctggtgggaagcggtcctcctcccatacacgacctcccaccctcgcgaggcgtagaaaccagttctgactgtacagtaaagcgagggccagggctgaggtctggaagctaatgaaagcacagaaagtgtcgaaactggatgagcaggaagcgagtggcctcccctgtcatctgacgttttcccaggatgtaatttgcctgactgaaacagatcaggaccaacagggagagttttcgatttagtgtgaggaaaagagcactaaattgtagcaaaagaccttattgctcaaggcccagtcagaagatttcataaggaagctgtagaaagtcttaagaggaaatcagccgggcgtggtggcgggcacctgtaatcccagctactcgggaggctgaggcaggagaatcgcttgaacccggggagcagaggttgcagtgagccgagatcgcgccactgtacgccagcctgggcgaaagaacgaaactccgtctccaaaaaaaaaaaaaacgaagaaaaagtccaaagagggtaaaggctgttctccccttaaaaaacagctaaagacctttgggggcgctgctccttgtaaatgtcaactact

SEQ ID NO: 11892 - RNA, 4611 nt, Homo sapiens
  source 1..4611: mol_type = other RNA
ctgaatagctgggactacaggtgtgcgtcaccatacctggctaatttttctatttttagtagagaccaggttttgccatgttggccaggctggtctcaaactccaggcctcaagcgacttgcctgcctcagcctcccaaagtgccgggattacaggcatgagccatcgcacccgtcctccagtaccattttaaacaaatacatattgtggactacgcaccaatagaaattaaggtggcaaaaccgtatcattagtaaagtaagtgaaagccttagtctttttgtttattccttattccccaaaggagttactaagtgaaggaattttccagctgcctttatttttttgagacggagtcttgttctgttgcccaggctggagtgcagtggcacgatcttggctcaccacaacctcctcctcctgggttccagcgattctcctgcctcagcctccagagtagctgggactacaggcgcccaccaacatgcccggctaatttgtgtatttacagtagagatggggtttcattatgttggccaggatggtcttgaactcctgacctcaagatcagcctgcctcggcctcccacagtgctgggattacatgcgtgagccactgcgcccggccttccagctgcatttctgaggtcacaagtatggccttaaatgattgccctcaagaacacagcttttgaaggtaatcatatgcaagtaaattacaatcaaatggaactgtatgattattttattattttaatgctaaactgaacagtgaactgaaatcagaggagaaagaaaatcaagctagtggctcactctcaatagtgtcctctaattttattgatgcttcagttttcataaagtgcaataaacaaaataaataaatgaaaaaagctttgaagatttatatacagttttgaggttaagataaattactgactatattcctttcagccttttaactctgtgaaagctgtaacgtacattaaaagcacattgaactaggttaaataatgatctttcccccttagatcaatctagtattaaggagtatataattatgcaagttcattctataacacaaggctagactaaaaggaaaatttttgtgctacagactaaatccagatacagtcaggtgctgagcagtattcctggcttcaaaataggaggtatctgtttcatcatctggctgggggatgaaaggcatagtctgatgctgcagattttcccagtccacatcactgaagagaggatgacgttttagctctcttttcagaatattctggaatacttgttgtggtgtttcatcattgaaagggggaattcctgttagaaattcaaacaagcaaactccaagtgcccaccagtctaccgcaggaccggaagtcagaaatccatgggccctgcctagtaacagctcaggtgcaaggtagtctggggttcctagaattcgcccatcatcaacgggggccacccctcttctcacactcttcggagttcggtatggagttcccgacttgatctgatttggggtctgctgatgtggcatacaggatcttcttttttgagtaggggttatagccatgggatatgaaccactgtaggcacacgaaatatccattgcatctaaagaagtcatgttcattctggatggttctgagttattggatgcattaatatgactgttaaaacttcgaaaagcaacagcatttcttttagaggctaacgttttcagcacctccaaaggaggacctaacattttttggttactctcttgtacagcagggttctcgacaccttttggtgaggtcttttcttggcaatctggtgttacaataagtggatcttcaatatttgattcttcaaaagaggattctttgatgcttctatctgaatctaagggctgactttctaatggactttccattatagaaattccaggaaaagatgaatcagagttcatagaaatatttttagaagctctatcatcatcagaacatagaaaactagaacttaagtagtccctcttactattcttttcacagtcttcatcgagttcacacataaggttttttgctatcattggtataggtaatttttctggtgtttgttgtttatcagtaaaagaattgacaatgttctccttattagcacagtcattttgttgacttttgtgcactgatagcttaaggtcctgcacttcaactgttaagcctgtattttgatttgtataacaatttgtcatttcgttatgcttatactctacacaagtttttttattctgtataatttttttacaaggactggagtcaaccaactcaaaatttctttttaaacttcttttcccaaggtgctcttcagatatcccaccagaatccacagcccactgatttgactgatggaaacctaactgacttgtgtcagtgtccatatttatattatttacatccagttctactgcttcccaagaaacttccccagagaagcattttttagcaaggtttacacaagagcgtccagtggtgggaagggcactgctgttatgaatgggagaaagagctaactccagatcctttttattgaaacctttcgtctcaatggcatttgcagattttgcgcataacttttcaactgcattccaactcatcattgttgggcccaatgcttcatcactttcctggcaatctttttcccatttgggactgctgtggcattctgattccacactggatatgaaggtgtgggattgactactggcactggatgtggccagccttttcctagactggagtaaattagaagttagacacttcacaggcattcctgggttggaggcaactgtttcaagacatgattttagtaatttgctagaataaggcgtagtgtccttttgatctacagacatagggcatacgagtccttgagaaagctgtgatgtttcagacagacaggctgaaaggatgtttgcagggtcttgatttttttctgcaattggtgtgttaaatcccaacgagctgataagcgataacacttgtcctggggttcttgaataatcttgtctaggttttgccattgatggtgttgtaaggatatccatcatattaatatctctattcaaagtaacttttgaaaggccaaaatccgtcagtttaatatgaccctcattagaaataagcatattgtccggtttcaagtccctgtggatgattccatgtctgtgaaggtagtctagagccagtgctacttcagaaatatatttcacagccatctcttcatcaaaataaccatatatatgtaggagagacttgacatctcccccaataagatattccattaccaagtagacattgtttgcagactgcagtgaataatacaaatggacaatgaatgggcttttgcttagtgccagtgcatctctctcagcttggacctgatgagtcatatttttgttgatcatgtctgcttttttaacaacctttactgcatacaatttgccgcctttctgccccagatacactttcccgaaggcgccccggctaatgggcttcactatgctgaattcctcaatggagggcggttttggcactgcgatcctattcacgccctcctcagtcgccgcgcctcctccaggctccttcttgcttcccgcggtgggatccatcgctggacagcatacagcggccccgcagacactgcccctccgcgagcagccactcccgccaactgggttcaaagtgaggctccgcccacgccgcgcgcggccgtgacgtcaccccgccgccgcgccccgccctcgtcacctcccctacgcagacgcggacggagggggcgtcgggaaagccccgacttcgcagccttacactcttcgtgggcggcgaccgcggccccactgacatcattcctcatgagggaggaggcacaaacagttctgggccgaccagaaaaaggacgactgggacttgactctgaatcgcaggatttgaagagatttctcctggcttcccaacgaggctggtgggaagcggtcctcctcccatacacgacctcccaccctcgcgaggcgtagaaaccagttctgactgtacagtaaagcgagggccagggctgaggtctggaagctaatgaaagcacagaaagtgtcgaaactggatgagcaggaagcgagtggcctcccctgtcatctgacgttttcccaggatgtaatttgcctgactgaaacagatcaggaccaacagggagagttttcgatttagtgtgaggaaaagagcactaaattgtagcaaaagaccttattgctcaaggcccagtcagaagatttcataaggaagctgtagaaagtcttaagaggaaatcagccgggcgtggtggcgggcacctgtaatcccagctactcgggaggctgaggcaggagaatcgcttgaacccggggagcagaggttgcagtgagccgagatcgcgccactgtacgccagcctgggcgaaagaacgaaactccgtctccaaaaaaaaaaaaaacgaagaaaaagtccaaagagggtaaaggctgttctccccttaaaaaacagctaaagacctttgggggcgctgctccttgtaaatgtcaactact

SEQ ID NO: 11893 - RNA, 3708 nt, Homo sapiens
  source 1..3708: mol_type = other RNA
ctgaatagctgggactacaggtgtgcgtcaccatacctggctaatttttctatttttagtagagaccaggttttgccatgttggccaggctggtctcaaactccaggcctcaagcgacttgcctgcctcagcctcccaaagtgccgggattacaggcatgagccatcgcacccgtcctccagtaccattttaaacaaatacatattgtggactacgcaccaatagaaattaaggtggcaaaaccgtatcattagtaaagtaagtgaaagccttagtctttttgtttattccttattccccaaaggagttactaagtgaaggaattttccagctgcctttatttttttgagacggagtcttgttctgttgcccaggctggagtgcagtggcacgatcttggctcaccacaacctcctcctcctgggttccagcgattctcctgcctcagcctccagagtagctgggactacaggcgcccaccaacatgcccggctaatttgtgtatttacagtagagatggggtttcattatgttggccaggatggtcttgaactcctgacctcaagatcagcctgcctcggcctcccacagtgctgggattacatgcgtgagccactgcgcccggccttccagctgcatttctgaggtcacaagtatggccttaaatgattgccctcaagaacacagcttttgaaggtaatcatatgcaagtaaattacaatcaaatggaactgtatgattattttattattttaatgctaaactgaacagtgaactgaaatcagaggagaaagaaaatcaagctagtggctcactctcaatagtgtcctctaattttattgatgcttcagttttcataaagtgcaataaacaaaataaataaatgaaaaaagctttgaagatttatatacagttttgaggttaagataaattactgactatattcctttcagccttttaactctgtgaaagctgtaacgtacattaaaagcacattgaactaggttaaataatgatctttcccccttagatcaatctagtattaaggagtatataattatgcaagttcattctataacacaaggctagactaaaaggaaaatttttgtgctacagactaaatccagatacagtcaggtgctgagcagtattcctggcttcaaaataggaggtatctgtttcatcatctggctgggggatgaaaggcatagtctgatgctgcagattttcccagtccacatcactgaagagaggatgacgttttagctctttcattccagctctctttgtatcatcaatggttaaaagtatttctactgcactttgagcattatcagataacttttcttcaccttctggccaagggatatcatgggccctgcctagtaacagctcaggtgcaaggtagtctggggttcctagaattcgcccatcatcaacgggggccacccctcttctcacactcttcggagttcggtatggagttcccgacttgatctgatttggggtctgatgtggcatacaggatcttcttttttgagtaggggttatagccatgggatatgaaccactgtaggcacacgaaatatccattgcatctaaagaagtcatgttcattctggatggttctgagttattggatgcattaatatgactgttaaaacttcgaaaagcaacagcatttcttttagaggctaacgttttcagcacctccaaaggaggacctaacattttttggttactctcttgtacagcagggttctcgacaccttttggtgaggtcttttcttggcaatctggtgttacaataagtggatcttcaatatttgattcttcaaaagaggattctttgatgcttctatctgaatctaagggctgactttctaatggactttccattatagaaattccaggaaaagatgaatcagagttcatagaaatatttttagaagctctatcatcatcagaacatagaaaactagaacttaagtagtccctcttactattcttttcacagtcttcatcgagttcacacataaggttttttgctatcattggtataggtaatttttctggtgtttgttgtttatcagtaaaagaattgacaatgttctccttattagcacagtcattttgttgacttttgtgcactgatagcttaaggtcctgcacttcaactgttaagcctgtattttgatttgtataacaatttgtcatttcgttatgcttatactctacacaagtttttttattctgtataatttttttacaaggactggagtcaaccaactcaaaatttctttttaaacttcttttcccaaggtgctcttcagatatcccaccagaatccacagcccactgatttgactgatggaaacctaactgacttgtgtcagtgtccatatttatattatttacatccagttctactgcttcccaagaaacttccccagagaagcattttttagcaaggtttacacaagagcgtccagtggtgggaagggcactgctgttatgaatgggagaaagagctaactccagatcctttttattgaaacctttcgtctcaatggcatttgcagattttgcgcataacttttcaactgcattccaactcatcattgttgggcccaatgcttcatcactttcctggcaatctttttcccatttgggactgctgtggcattctgattccacactggatatgaaggtgtgggattgactactggcactggatgtggccagccttttcctagactggagtaaattagaagttagacacttcacaggcattcctgggttggaggcaactgtttcaagacatgattttagtaatttgctagaataaggcgtagtgtccttttgatctacagacatagggcatacgagtccttgagaaagctgtgatgtttcagacagacaggctgaaaggatgtttgcagggtcttgatttttttctgcaattggtgtgttaaatcccaacgagctgataagcgataacacttgtcctggggttcttgaataatcttgtctaggttttgccattgatggtgttgtaaggatatccatcatattaatatctctattcaaagtaacttttgaaaggccaaaatccgtcagtttaatatgaccctcattagaaataagcatattgtccggtttcaagtccctgtggatgattccatgtctgtgaaggtagtctagagccagtgctacttcagaaatatatttcacagccatctcttcatcaaaataaccatatatatgtaggagagacttgacatctcccccaataagatattccattaccaagtagacattgtttgcagactgcagtgaataatacaaatggacaatgaatgggcttttgcttagtgccagtgcatctctctcagcttggacctgatgagtcatatttttgttgatcatgtctgcttttttaacaacctttactgcatacaatttgccgcctttctgccccagatacactttcccgaaggcgccccggctaatgggcttcactatgctgaattcctcaatggagggcggttttggcactgcgatcctattcacgccctcctcagtcgccgcgcctcctccaggctccttcttgcttcccgcggtgggatccatcgctggacagcatacagcggccccgcagacactgcccctccgcgagcagccactcccgccaactgggttcaaagt

SEQ ID NO: 11894 - RNA, 4584 nt, Homo sapiens
  source 1..4584: mol_type = other RNA
ctgaatagctgggactacaggtgtgcgtcaccatacctggctaatttttctatttttagtagagaccaggttttgccatgttggccaggctggtctcaaactccaggcctcaagcgacttgcctgcctcagcctcccaaagtgccgggattacaggcatgagccatcgcacccgtcctccagtaccattttaaacaaatacatattgtggactacgcaccaatagaaattaaggtggcaaaaccgtatcattagtaaagtaagtgaaagccttagtctttttgtttattccttattccccaaaggagttactaagtgaaggaattttccagctgcctttatttttttgagacggagtcttgttctgttgcccaggctggagtgcagtggcacgatcttggctcaccacaacctcctcctcctgggttccagcgattctcctgcctcagcctccagagtagctgggactacaggcgcccaccaacatgcccggctaatttgtgtatttacagtagagatggggtttcattatgttggccaggatggtcttgaactcctgacctcaagatcagcctgcctcggcctcccacagtgctgggattacatgcgtgagccactgcgcccggccttccagctgcatttctgaggtcacaagtatggccttaaatgattgccctcaagaacacagcttttgaaggtaatcatatgcaagtaaattacaatcaaatggaactgtatgattattttattattttaatgctaaactgaacagtgaactgaaatcagaggagaaagaaaatcaagctagtggctcactctcaatagtgtcctctaattttattgatgcttcagttttcataaagtgcaataaacaaaataaataaatgaaaaaagctttgaagatttatatacagttttgaggttaagataaattactgactatattcctttcagccttttaactctgtgaaagctgtaacgtacattaaaagcacattgaactaggttaaataatgatctttcccccttagatcaatctagtattaaggagtatataattatgcaagttcattctataacacaaggctagactaaaaggaaaatttttgtgctacagactaaatccagatacagtcaggtgctgagcagtattcctggcttcaaaataggaggtatctgtttcatcatctggctgggggatgaaaggcatagtctgatgctgcagattttcccagtccacatcactgaagagaggatgacgttttagctctttcattccagctctctttgtatcatcaatggttaaaagtatttctactgcactttgagcattatcagataacttttcttcaccttctggccaagggatatcatgggccctgcctagtaacagctcaggtgcaaggtagtctggggttcctagaattcgcccatcatcaacgggggccacccctcttctcacactcttcggagttcggtatggagttcccgacttgatctgatttggggtctgctgatgtggcatacaggatcttcttttttgagtaggggttatagccatgggatatgaaccactgtaggcacacgaaatatccattgcatctaaagaagtcatgttcattctggatggttctgagttattggatgcattaatatgactgttaaaacttcgaaaagcaacagcatttcttttagaggctaacgttttcagcacctccaaaggaggacctaacattttttggttactctcttgtacagcagggttctcgacaccttttggtgaggtcttttcttggcaatctggtgttacaataagtggatcttcaatatttgattcttcaaaagaggattctttgatgcttctatctgaatctaagggctgactttctaatggactttccattatagaaattccaggaaaagatgaatcagagttcatagaaatatttttagaagctctatcatcatcagaacatagaaaactagaacttaagtagtccctcttactattcttttcacagtcttcatcgagttcacacataaggttttttgctatcattggtataggtaatttttctggtgtttgttgtttatcagtaaaagaattgacaatgttctccttattagcacagtcattttgttgacttttgtgcactgatagcttaaggtcctgcacttcaactgttaagcctgtattttgatttgtataacaatttgtcatttcgttatgcttatactctacacaagtttttttattctgtataatttttttacaaggactggagtcaaccaactcaaaatttctttttaaacttcttttcccaaggtgctcttcagatatcccaccagaatccacagcccactgatttgactgatggaaacctaactgacttgtgtcagtgtccatatttatattatttacatccagttctactgcttcccaagaaacttccccagagaagcattttttagcaaggtttacacaagagcgtccagtggtgggaagggcactgctgttatgaatgggagaaagagctaactccagatcctttttattgaaacctttcgtctcaatggcatttgcagattttgcgcataacttttcaactgcattccaactcatcattgttgggcccaatgcttcatcactttcctggcaatctttttcccatttgggactgctgtggcattctgattccacactggatatgaaggtgtgggattgactactggcactggatgtggccagccttttcctagactggagtaaattagaagttagacacttcacaggcattcctgggttggaggcaactgtttcaagacatgattttagtaatttgctagaataaggcgtagtgtccttttgatctacagacatagggcatacgagtccttgagaaagctgtgatgtttcagacagacaggctgaaaggatgtttgcagggtcttgatttttttctgcaattggtgtgttaaatcccaacgagctgataagcgataacacttgtcctggggttcttgaataatcttgtctaggttttgccattgatggtgttgtaaggatatccatcatattaatatctctattcaaagtaacttttgaaaggccaaaatccgtcagtttaatatgaccctcattagaaataagcatattgtccggtttcaagtccctgtggatgattccatgtctgtgaaggtagtctagagccagtgctacttcagaaatatatttcacagccatctcttcatcaaaataaccatatatatgtaggagagacttgacatctcccccaataagatattccattaccaagtagacattgtttgcagactgcagtgaataatacaaatggacaatgaatgggcttttgcttagtgccagtgcatctctctcagcttggacctgatgagtcatatttttgttgatcatgtctgcttttttaacaacctttactgcatacaatttgccgcctttctgccccagatacactttcccgaaggcgccccggctaatgggcttcactatgctgaattcctcaatggagggcggttttggcactgcgatcctattcacgccctcctcagtcgccgcgcctcctccaggctccttcttgcttcccgcggtgggatccatcgctggacagcatacagcggccccgcagacactgcccctccgcgagcagccactcccgccaactgggttcaaagtgaggctccgcccacgccgcgcgcggccgtgacgtcaccccgccgccgcgccccgccctcgtcacctcccctacgcagacgcggacggagggggcgtcgggaaagccccgacttcgcagccttacactcttcgtgggcggcgaccgcggccccactgacatcattcctcatgagggaggaggcacaaacagttctgggccgaccagaaaaaggacgactgggacttgactctgaatcgcaggatttgaagagatttctcctggcttcccaacgaggctggtgggaagcggtcctcctcccatacacgacctcccaccctcgcgaggcgtagaaaccagttctgactgtacagtaaagcgagggccagggctgaggtctggaagctaatgaaagcacagaaagtgtcgaaactggatgagcaggaagcgagtggcctcccctgtcatctgacgttttcccaggatgtaatttgcctgactgaaacagatcaggaccaacagggagagttttcgatttagtgtgaggaaaagagcactaaattgtagcaaaagaccttattgctcaaggcccagtcagaagatttcataaggaagctgtagaaagtcttaagaggaaatcagccgggcgtggtggcgggcacctgtaatcccagctactcgggaggctgaggcaggagaatcgcttgaacccggggagcagaggttgcagtgagccgagatcgcgccactgtacgccagcctgggcgaaagaacgaaactccgtctccaaaaaaaaaaaaaacgaagaaaaagtccaaagagggtaaaggctgttctccccttaaaaaacagctaaagacctttgggggcgctgctccttgtaaatgtcaactact

SEQ ID NO: 11895 - RNA, 3822 nt, Homo sapiens
  source 1..3822: mol_type = other RNA
ctgaatagctgggactacaggtgtgcgtcaccatacctggctaatttttctatttttagtagagaccaggttttgccatgttggccaggctggtctcaaactccaggcctcaagcgacttgcctgcctcagcctcccaaagtgccgggattacaggcatgagccatcgcacccgtcctccagtaccattttaaacaaatacatattgtggactacgcaccaatagaaattaaggtggcaaaaccgtatcattagtaaagtaagtgaaagccttagtctttttgtttattccttattccccaaaggagttactaagtgaaggaattttccagctgcctttatttttttgagacggagtcttgttctgttgcccaggctggagtgcagtggcacgatcttggctcaccacaacctcctcctcctgggttccagcgattctcctgcctcagcctccagagtagctgggactacaggcgcccaccaacatgcccggctaatttgtgtatttacagtagagatggggtttcattatgttggccaggatggtcttgaactcctgacctcaagatcagcctgcctcggcctcccacagtgctgggattacatgcgtgagccactgcgcccggccttccagctgcatttctgaggtcacaagtatggccttaaatgattgccctcaagaacacagcttttgaaggtaatcatatgcaagtaaattacaatcaaatggaactgtatgattattttattattttaatgctaaactgaacagtgaactgaaatcagaggagaaagaaaatcaagctagtggctcactctcaatagtgtcctctaattttattgatgcttcagttttcataaagtgcaataaacaaaataaataaatgaaaaaagctttgaagatttatatacagttttgaggttaagataaattactgactatattcctttcagccttttaactctgtgaaagctgtaacgtacattaaaagcacattgaactaggttaaataatgatctttcccccttagatcaatctagtattaaggagtatataattatgcaagttcattctataacacaaggctagactaaaaggaaaatttttgtgctacagactaaatccagatacagtcaggtgctgagcagtattcctggcttcaaaataggaggtatctgtttcatcatctggctgggggatgaaaggcatagtctgatgctgcagattttcccagtccacatcactgaagagaggatgacgttttagctctttcattccagctctctttgtatcatcaatggttaaaagtatttctactgcactttgagcattatcagataacttttcttcaccttctggccaagggatatctcttttcagaatattctggaatacttgttgtggtgtttcatcattgaaagggggaattcctgttagaaattcaaacaagcaaactccaagtgcccaccagtctaccgcaggaccatgggccctgcctagtaacagctcaggtgcaaggtagtctggggttcctagaattcgcccatcatcaacgggggccacccctcttctcacactcttcggagttcggtatggagttcccgacttgatctgatttggggtctgatgtggcatacaggatcttcttttttgagtaggggttatagccatgggatatgaaccactgtaggcacacgaaatatccattgcatctaaagaagtcatgttcattctggatggttctgagttattggatgcattaatatgactgttaaaacttcgaaaagcaacagcatttcttttagaggctaacgttttcagcacctccaaaggaggacctaacattttttggttactctcttgtacagcagggttctcgacaccttttggtgaggtcttttcttggcaatctggtgttacaataagtggatcttcaatatttgattcttcaaaagaggattctttgatgcttctatctgaatctaagggctgactttctaatggactttccattatagaaattccaggaaaagatgaatcagagttcatagaaatatttttagaagctctatcatcatcagaacatagaaaactagaacttaagtagtccctcttactattcttttcacagtcttcatcgagttcacacataaggttttttgctatcattggtataggtaatttttctggtgtttgttgtttatcagtaaaagaattgacaatgttctccttattagcacagtcattttgttgacttttgtgcactgatagcttaaggtcctgcacttcaactgttaagcctgtattttgatttgtataacaatttgtcatttcgttatgcttatactctacacaagtttttttattctgtataatttttttacaaggactggagtcaaccaactcaaaatttctttttaaacttcttttcccaaggtgctcttcagatatcccaccagaatccacagcccactgatttgactgatggaaacctaactgacttgtgtcagtgtccatatttatattatttacatccagttctactgcttcccaagaaacttccccagagaagcattttttagcaaggtttacacaagagcgtccagtggtgggaagggcactgctgttatgaatgggagaaagagctaactccagatcctttttattgaaacctttcgtctcaatggcatttgcagattttgcgcataacttttcaactgcattccaactcatcattgttgggcccaatgcttcatcactttcctggcaatctttttcccatttgggactgctgtggcattctgattccacactggatatgaaggtgtgggattgactactggcactggatgtggccagccttttcctagactggagtaaattagaagttagacacttcacaggcattcctgggttggaggcaactgtttcaagacatgattttagtaatttgctagaataaggcgtagtgtccttttgatctacagacatagggcatacgagtccttgagaaagctgtgatgtttcagacagacaggctgaaaggatgtttgcagggtcttgatttttttctgcaattggtgtgttaaatcccaacgagctgataagcgataacacttgtcctggggttcttgaataatcttgtctaggttttgccattgatggtgttgtaaggatatccatcatattaatatctctattcaaagtaacttttgaaaggccaaaatccgtcagtttaatatgaccctcattagaaataagcatattgtccggtttcaagtccctgtggatgattccatgtctgtgaaggtagtctagagccagtgctacttcagaaatatatttcacagccatctcttcatcaaaataaccatatatatgtaggagagacttgacatctcccccaataagatattccattaccaagtagacattgtttgcagactgcagtgaataatacaaatggacaatgaatgggcttttgcttagtgccagtgcatctctctcagcttggacctgatgagtcatatttttgttgatcatgtctgcttttttaacaacctttactgcatacaatttgccgcctttctgccccagatacactttcccgaaggcgccccggctaatgggcttcactatgctgaattcctcaatggagggcggttttggcactgcgatcctattcacgccctcctcagtcgccgcgcctcctccaggctccttcttgcttcccgcggtgggatccatcgctggacagcatacagcggccccgcagacactgcccctccgcgagcagccactcccgccaactgggttcaaagt

SEQ ID NO: 11896 - RNA, 3945 nt, Homo sapiens
  source 1..3945: mol_type = other RNA
ctgaatagctgggactacaggtgtgcgtcaccatacctggctaatttttctatttttagtagagaccaggttttgccatgttggccaggctggtctcaaactccaggcctcaagcgacttgcctgcctcagcctcccaaagtgccgggattacaggcatgagccatcgcacccgtcctccagtaccattttaaacaaatacatattgtggactacgcaccaatagaaattaaggtggcaaaaccgtatcattagtaaagtaagtgaaagccttagtctttttgtttattccttattccccaaaggagttactaagtgaaggaattttccagctgcctttatttttttgagacggagtcttgttctgttgcccaggctggagtgcagtggcacgatcttggctcaccacaacctcctcctcctgggttccagcgattctcctgcctcagcctccagagtagctgggactacaggcgcccaccaacatgcccggctaatttgtgtatttacagtagagatggggtttcattatgttggccaggatggtcttgaactcctgacctcaagatcagcctgcctcggcctcccacagtgctgggattacatgcgtgagccactgcgcccggccttccagctgcatttctgaggtcacaagtatggccttaaatgattgccctcaagaacacagcttttgaaggtaatcatatgcaagtaaattacaatcaaatggaactgtatgattattttattattttaatgctaaactgaacagtgaactgaaatcagaggagaaagaaaatcaagctagtggctcactctcaatagtgtcctctaattttattgatgcttcagttttcataaagtgcaataaacaaaataaataaatgaaaaaagctttgaagatttatatacagttttgaggttaagataaattactgactatattcctttcagccttttaactctgtgaaagctgtaacgtacattaaaagcacattgaactaggttaaataatgatctttcccccttagatcaatctagtattaaggagtatataattatgcaagttcattctataacacaaggctagactaaaaggaaaatttttgtgctacagactaaatccagatacagtcaggtgctgagcagtattcctggcttcaaaataggaggtatctgtttcatcatctggctgggggatgaaaggcatagtctgatgctgcagattttcccagtccacatcactgaagagaggatgacgttttagctctttcattccagctctctttgtatcatcaatggttaaaagtatttctactgcactttgagcattatcagataacttttcttcaccttctggccaagggatatctcttttcagaatattctggaatacttgttgtggtgtttcatcattgaaagggggaattcctgttagaaattcaaacaagcaaactccaagtgcccaccagtctaccgcaggaccatgggccctgcctagtaacagctcaggtgcaaggtagtctggggttcctagaattcgcccatcatcaacgggggccacccctcttctcacactcttcggagttcggtatggagttcccgacttgatctgatttggggtctgctgatgtggcatacaggatcttcttttttgagtaggggttatagccatgggatatgaaccactgtaggcacacgaaatatccattgcatctaaagaagtcatgttcattctggatggttctgagttattggatgcattaatatgactgttaaaacttcgaaaagcaacagcatttcttttagaggctaacgttttcagcacctccaaaggaggacctaacattttttggttactctcttgtacagcagggttctcgacaccttttggtgaggtcttttcttggcaatctggtgttacaataagtggatcttcaatatttgattcttcaaaagaggattctttgatgcttctatctgaatctaagggctgactttctaatggactttccattatagaaattccaggaaaagatgaatcagagttcatagaaatatttttagaagctctatcatcatcagaacatagaaaactagaacttaagtagtccctcttactattcttttcacagtcttcatcgagttcacacataaggttttttgctatcattggtataggtaatttttctggtgtttgttgtttatcagtaaaagaattgacaatgttctccttattagcacagtcattttgttgacttttgtgcactgatagcttaaggtcctgcacttcaactgttaagcctgtattttgatttgtataacaatttgtcatttcgttatgcttatactctacacaagtttttttattctgtataatttttttacaaggactggagtcaaccaactcaaaatttctttttaaacttcttttcccaaggtgctcttcagatatcccaccagaatccacagcccactgatttgactgatggaaacctaactgacttgtgtcagtgtccatatttatattatttacatccagttctactgcttcccaagaaacttccccagagaagcattttttagcaaggtttacacaagagcgtccagtggtgggaagggcactgctgttatgaatgggagaaagagctaactccagatcctttttattgaaacctttcgtctcaatggcatttgcagattttgcgcataacttttcaactgcattccaactcatcattgttgggcccaatgcttcatcactttcctggcaatctttttcccatttgggactgctgtggcattctgattccacactggatatgaaggtgtgggattgactactggcactggatgtggccagccttttcctagactggagtaaattagaagttagacacttcacaggcattcctgggttggaggcaactgtttcaagacatgattttagtaatttgctagaataaggcgtagtgtccttttgatctacagacatagggcatacgagtccttgagaaagctgtgatgtttcagacagacaggctgaaaggatgtttgcagggtcttgatttttttctgcaattggtgtgttaaatcccaacgagctgataagcgataacacttgtcctggggttcttgaataatcttgtctaggttttgccattgatggtgttgtaaggatatccatcatattaatatctctattcaaagtaacttttgaaaggccaaaatccgtcagtttaatatgaccctcattagaaataagcatattgtccggtttcaagtccctctactcccagacacttgggaggctaaggcagggggattgcttgagccccagaggtcgaggctgcagtgagccaaggtcaagtcactgcactgcacaacctggatgacaaagtgagaccctgtggatgattccatgtctgtgaaggtagtctagagccagtgctacttcagaaatatatttcacagccatctcttcatcaaaataaccatatatatgtaggagagacttgacatctcccccaataagatattccattaccaagtagacattgtttgcagactgcagtgaataatacaaatggacaatgaatgggcttttgcttagtgccagtgcatctctctcagcttggacctgatgagtcatatttttgttgatcatgtctgcttttttaacaacctttactgcatacaatttgccgcctttctgccccagatacactttcccgaaggcgccccggctaatgggcttcactatgctgaattcctcaatggagggcggttttggcactgcgatcctattcacgccctcctcagtcgccgcgcctcctccaggctccttcttgcttcccgcggtgggatccatcgctggacagcatacagcggccccgcagacactgcccctccgcgagcagccactcccgccaactgggttcaaagt

SEQ ID NO: 11897 - RNA, 3825 nt, Homo sapiens
  source 1..3825: mol_type = other RNA
ctgaatagctgggactacaggtgtgcgtcaccatacctggctaatttttctatttttagtagagaccaggttttgccatgttggccaggctggtctcaaactccaggcctcaagcgacttgcctgcctcagcctcccaaagtgccgggattacaggcatgagccatcgcacccgtcctccagtaccattttaaacaaatacatattgtggactacgcaccaatagaaattaaggtggcaaaaccgtatcattagtaaagtaagtgaaagccttagtctttttgtttattccttattccccaaaggagttactaagtgaaggaattttccagctgcctttatttttttgagacggagtcttgttctgttgcccaggctggagtgcagtggcacgatcttggctcaccacaacctcctcctcctgggttccagcgattctcctgcctcagcctccagagtagctgggactacaggcgcccaccaacatgcccggctaatttgtgtatttacagtagagatggggtttcattatgttggccaggatggtcttgaactcctgacctcaagatcagcctgcctcggcctcccacagtgctgggattacatgcgtgagccactgcgcccggccttccagctgcatttctgaggtcacaagtatggccttaaatgattgccctcaagaacacagcttttgaaggtaatcatatgcaagtaaattacaatcaaatggaactgtatgattattttattattttaatgctaaactgaacagtgaactgaaatcagaggagaaagaaaatcaagctagtggctcactctcaatagtgtcctctaattttattgatgcttcagttttcataaagtgcaataaacaaaataaataaatgaaaaaagctttgaagatttatatacagttttgaggttaagataaattactgactatattcctttcagccttttaactctgtgaaagctgtaacgtacattaaaagcacattgaactaggttaaataatgatctttcccccttagatcaatctagtattaaggagtatataattatgcaagttcattctataacacaaggctagactaaaaggaaaatttttgtgctacagactaaatccagatacagtcaggtgctgagcagtattcctggcttcaaaataggaggtatctgtttcatcatctggctgggggatgaaaggcatagtctgatgctgcagattttcccagtccacatcactgaagagaggatgacgttttagctctttcattccagctctctttgtatcatcaatggttaaaagtatttctactgcactttgagcattatcagataacttttcttcaccttctggccaagggatatctcttttcagaatattctggaatacttgttgtggtgtttcatcattgaaagggggaattcctgttagaaattcaaacaagcaaactccaagtgcccaccagtctaccgcaggaccatgggccctgcctagtaacagctcaggtgcaaggtagtctggggttcctagaattcgcccatcatcaacgggggccacccctcttctcacactcttcggagttcggtatggagttcccgacttgatctgatttggggtctgctgatgtggcatacaggatcttcttttttgagtaggggttatagccatgggatatgaaccactgtaggcacacgaaatatccattgcatctaaagaagtcatgttcattctggatggttctgagttattggatgcattaatatgactgttaaaacttcgaaaagcaacagcatttcttttagaggctaacgttttcagcacctccaaaggaggacctaacattttttggttactctcttgtacagcagggttctcgacaccttttggtgaggtcttttcttggcaatctggtgttacaataagtggatcttcaatatttgattcttcaaaagaggattctttgatgcttctatctgaatctaagggctgactttctaatggactttccattatagaaattccaggaaaagatgaatcagagttcatagaaatatttttagaagctctatcatcatcagaacatagaaaactagaacttaagtagtccctcttactattcttttcacagtcttcatcgagttcacacataaggttttttgctatcattggtataggtaatttttctggtgtttgttgtttatcagtaaaagaattgacaatgttctccttattagcacagtcattttgttgacttttgtgcactgatagcttaaggtcctgcacttcaactgttaagcctgtattttgatttgtataacaatttgtcatttcgttatgcttatactctacacaagtttttttattctgtataatttttttacaaggactggagtcaaccaactcaaaatttctttttaaacttcttttcccaaggtgctcttcagatatcccaccagaatccacagcccactgatttgactgatggaaacctaactgacttgtgtcagtgtccatatttatattatttacatccagttctactgcttcccaagaaacttccccagagaagcattttttagcaaggtttacacaagagcgtccagtggtgggaagggcactgctgttatgaatgggagaaagagctaactccagatcctttttattgaaacctttcgtctcaatggcatttgcagattttgcgcataacttttcaactgcattccaactcatcattgttgggcccaatgcttcatcactttcctggcaatctttttcccatttgggactgctgtggcattctgattccacactggatatgaaggtgtgggattgactactggcactggatgtggccagccttttcctagactggagtaaattagaagttagacacttcacaggcattcctgggttggaggcaactgtttcaagacatgattttagtaatttgctagaataaggcgtagtgtccttttgatctacagacatagggcatacgagtccttgagaaagctgtgatgtttcagacagacaggctgaaaggatgtttgcagggtcttgatttttttctgcaattggtgtgttaaatcccaacgagctgataagcgataacacttgtcctggggttcttgaataatcttgtctaggttttgccattgatggtgttgtaaggatatccatcatattaatatctctattcaaagtaacttttgaaaggccaaaatccgtcagtttaatatgaccctcattagaaataagcatattgtccggtttcaagtccctgtggatgattccatgtctgtgaaggtagtctagagccagtgctacttcagaaatatatttcacagccatctcttcatcaaaataaccatatatatgtaggagagacttgacatctcccccaataagatattccattaccaagtagacattgtttgcagactgcagtgaataatacaaatggacaatgaatgggcttttgcttagtgccagtgcatctctctcagcttggacctgatgagtcatatttttgttgatcatgtctgcttttttaacaacctttactgcatacaatttgccgcctttctgccccagatacactttcccgaaggcgccccggctaatgggcttcactatgctgaattcctcaatggagggcggttttggcactgcgatcctattcacgccctcctcagtcgccgcgcctcctccaggctccttcttgcttcccgcggtgggatccatcgctggacagcatacagcggccccgcagacactgcccctccgcgagcagccactcccgccaactgggttcaaagt

SEQ ID NO: 11898 - RNA, 3837 nt, Homo sapiens
  source 1..3837: mol_type = other RNA
ctgaatagctgggactacaggtgtgcgtcaccatacctggctaatttttctatttttagtagagaccaggttttgccatgttggccaggctggtctcaaactccaggcctcaagcgacttgcctgcctcagcctcccaaagtgccgggattacaggcatgagccatcgcacccgtcctccagtaccattttaaacaaatacatattgtggactacgcaccaatagaaattaaggtggcaaaaccgtatcattagtaaagtaagtgaaagccttagtctttttgtttattccttattccccaaaggagttactaagtgaaggaattttccagctgcctttatttttttgagacggagtcttgttctgttgcccaggctggagtgcagtggcacgatcttggctcaccacaacctcctcctcctgggttccagcgattctcctgcctcagcctccagagtagctgggactacaggcgcccaccaacatgcccggctaatttgtgtatttacagtagagatggggtttcattatgttggccaggatggtcttgaactcctgacctcaagatcagcctgcctcggcctcccacagtgctgggattacatgcgtgagccactgcgcccggccttccagctgcatttctgaggtcacaagtatggccttaaatgattgccctcaagaacacagcttttgaaggtaatcatatgcaagtaaattacaatcaaatggaactgtatgattattttattattttaatgctaaactgaacagtgaactgaaatcagaggagaaagaaaatcaagctagtggctcactctcaatagtgtcctctaattttattgatgcttcagttttcataaagtgcaataaacaaaataaataaatgaaaaaagctttgaagatttatatacagttttgaggttaagataaattactgactatattcctttcagccttttaactctgtgaaagctgtaacgtacattaaaagcacattgaactaggttaaataatgatctttcccccttagatcaatctagtattaaggagtatataattatgcaagttcattctataacacaaggctagactaaaaggaaaatttttgtgctacagactaaatccagatacagtcaggtgctgagcagtattcctggcttcaaaataggaggtatctgtttcatcatctggctgggggatgaaaggcatagtctgatgctgcagattttcccagtccacatcactgaagagaggatgacgttttagctctttcattccagctctctttgtatcatcaatggttaaaagtatttctactgcactttgagcattatcagataacttttcttcaccttctggccaagggatatctcttttcagaatattctggaatacttgttgtggtgtttcatcattgaaagggggaattcctgttagaaattcaaacaagcaaactccaagtgcccaccagtctaccgcaggaccggaagtcagaaatccatgggccctgcctagtaacagctcaggtgcaaggtagtctggggttcctagaattcgcccatcatcaacgggggccacccctcttctcacactcttcggagttcggtatggagttcccgacttgatctgatttggggtctgatgtggcatacaggatcttcttttttgagtaggggttatagccatgggatatgaaccactgtaggcacacgaaatatccattgcatctaaagaagtcatgttcattctggatggttctgagttattggatgcattaatatgactgttaaaacttcgaaaagcaacagcatttcttttagaggctaacgttttcagcacctccaaaggaggacctaacattttttggttactctcttgtacagcagggttctcgacaccttttggtgaggtcttttcttggcaatctggtgttacaataagtggatcttcaatatttgattcttcaaaagaggattctttgatgcttctatctgaatctaagggctgactttctaatggactttccattatagaaattccaggaaaagatgaatcagagttcatagaaatatttttagaagctctatcatcatcagaacatagaaaactagaacttaagtagtccctcttactattcttttcacagtcttcatcgagttcacacataaggttttttgctatcattggtataggtaatttttctggtgtttgttgtttatcagtaaaagaattgacaatgttctccttattagcacagtcattttgttgacttttgtgcactgatagcttaaggtcctgcacttcaactgttaagcctgtattttgatttgtataacaatttgtcatttcgttatgcttatactctacacaagtttttttattctgtataatttttttacaaggactggagtcaaccaactcaaaatttctttttaaacttcttttcccaaggtgctcttcagatatcccaccagaatccacagcccactgatttgactgatggaaacctaactgacttgtgtcagtgtccatatttatattatttacatccagttctactgcttcccaagaaacttccccagagaagcattttttagcaaggtttacacaagagcgtccagtggtgggaagggcactgctgttatgaatgggagaaagagctaactccagatcctttttattgaaacctttcgtctcaatggcatttgcagattttgcgcataacttttcaactgcattccaactcatcattgttgggcccaatgcttcatcactttcctggcaatctttttcccatttgggactgctgtggcattctgattccacactggatatgaaggtgtgggattgactactggcactggatgtggccagccttttcctagactggagtaaattagaagttagacacttcacaggcattcctgggttggaggcaactgtttcaagacatgattttagtaatttgctagaataaggcgtagtgtccttttgatctacagacatagggcatacgagtccttgagaaagctgtgatgtttcagacagacaggctgaaaggatgtttgcagggtcttgatttttttctgcaattggtgtgttaaatcccaacgagctgataagcgataacacttgtcctggggttcttgaataatcttgtctaggttttgccattgatggtgttgtaaggatatccatcatattaatatctctattcaaagtaacttttgaaaggccaaaatccgtcagtttaatatgaccctcattagaaataagcatattgtccggtttcaagtccctgtggatgattccatgtctgtgaaggtagtctagagccagtgctacttcagaaatatatttcacagccatctcttcatcaaaataaccatatatatgtaggagagacttgacatctcccccaataagatattccattaccaagtagacattgtttgcagactgcagtgaataatacaaatggacaatgaatgggcttttgcttagtgccagtgcatctctctcagcttggacctgatgagtcatatttttgttgatcatgtctgcttttttaacaacctttactgcatacaatttgccgcctttctgccccagatacactttcccgaaggcgccccggctaatgggcttcactatgctgaattcctcaatggagggcggttttggcactgcgatcctattcacgccctcctcagtcgccgcgcctcctccaggctccttcttgcttcccgcggtgggatccatcgctggacagcatacagcggccccgcagacactgcccctccgcgagcagccactcccgccaactgggttcaaagt

SEQ ID NO: 11899 - RNA, 2870 nt, Homo sapiens
  source 1..2870: mol_type = other RNA
ctgaatagctgggactacaggtgtgcgtcaccatacctggctaatttttctatttttagtagagaccaggttttgccatgttggccaggctggtctcaaactccaggcctcaagcgacttgcctgcctcagcctcccaaagtgccgggattacaggcatgagccatcgcacccgtcctccagtaccattttaaacaaatacatattgtggactacgcaccaatagaaattaaggtggcaaaaccgtatcattagtaaagtaagtgaaagccttagtctttttgtttattccttattccccaaaggagttactaagtgaaggaattttccagctgcctttatttttttgagacggagtcttgttctgttgcccaggctggagtgcagtggcacgatcttggctcaccacaacctcctcctcctgggttccagcgattctcctgcctcagcctccagagtagctgggactacaggcgcccaccaacatgcccggctaatttgtgtatttacagtagagatggggtttcattatgttggccaggatggtcttgaactcctgacctcaagatcagcctgcctcggcctcccacagtgctgggattacatgcgtgagccactgcgcccggccttccagctgcatttctgaggtcacaagtatggccttaaatgattgccctcaagaacacagcttttgaaggtaatcatatgcaagtaaattacaatcaaatggaactgtatgattattttattattttaatgctaaactgaacagtgaactgaaatcagaggagaaagaaaatcaagctagtggctcactctcaatagtgtcctctaattttattgatgcttcagttttcataaagtgcaataaacaaaataaataaatgaaaaaagctttgaagatttatatacagttttgaggttaagataaattactgactatattcctttcagccttttaactctgtgaaagctgtaacgtacattaaaagcacattgaactaggttaaataatgatctttcccccttagatcaatctagtattaaggagtatataattatgcaagttcattctataacacaaggctagactaaaaggaaaatttttgtgctacagactaaatccagatacagtcaggtgctgagcagtattcctggcttcaaaataggaggtatctgtttcatcatctggctgggggatgaaaggcatagtctgatgctgcagattttcccagtccacatcactgaagagaggatgacgttttagctctttcattccagctctctttgtatcatcaatggttaaaagtatttctactgcactttgagcattatcagataacttttcttcaccttctggccaagggatatctcttttcagaatattctggaatacttgttgtggtgtttcatcattgaaagggggaattcctgttagaaattcaaacaagcaaactccaagtgcccaccagtctaccgcaggaccggaagtcagaaatccatgggccctgcctagtaacagctcaggtgcaaggtagtctggggttcctagaattcgcccatcatcaacgggggccacccctcttctcacactcttcggagttcggtatggagttcccgacttgatctgatttggggtctgctgatgtggcatacaggatcttcttttttgagtaggggttatagccatgggatatgaaccactgtaggcacacgaaatatccattgcatctaaagaagtcatgttcattctggatggttctgagttattggatgcattaatatgactgttaaaacttcgaaaagcaacagcatttcttttagaggctaacgttttcagcacctccaaaggaggacctaacattttttggttactctcttgtacagcagggttctcgacaccttttggtgaggtcttttcttggcaatctggtgttacaataagtggatcttcaatatttgattcttcaaaagaggattctttgatgcttctatctgaatctaagggctgactttctaatggactttccattatagaaattccaggaaaagatgaatcagagttcatagaaatatttttagaagctctatcatcatcagaacatagaaaactagaacttaagtagtccctcttactattcttttcacagtcttcatcgagttcacacataaggttttttgctatcattggtataggtaatttttctggtgtttgttgtttatcagtaaaagaattgacaatgttctccttattagcacagtcattttgttgacttttgtgcactgatagcttaaggtcctgcacttcaactgttaagcctgtattttgatttgtataacaatttgtcatttcgttatgcttatactctacacaagtttttttattctgtataatttttttacaaggactggagtcaaccaactcaaaatttctttttaaacttcttttcccaaggtgctcttcagatatcccaccagaatccacagcccactgatttgactgatggaaacctaactgacttgtgtcagtgtccatatttatattatttacatccagttctactgcttcccaagaaacttccccagagaagcattttttagcaaggtttacacaagagcgtccagtggtgggaagggcactgctgttatgaatgggagaaagagctaactccagatcctttttattgaaacctttcgtctcaatggcatttgcagattttgcgcataacttttcaactgcattccaactcatcattgttgggcccaatgcttcatcactttcatgattttagtaatttgctagaataaggcgtagtgtccttttgatctacagacatagggcatacgagtccttgagaaagctgtgatgtt

SEQ ID NO: 11900 - RNA, 3960 nt, Homo sapiens
  source 1..3960: mol_type = other RNA
ctgaatagctgggactacaggtgtgcgtcaccatacctggctaatttttctatttttagtagagaccaggttttgccatgttggccaggctggtctcaaactccaggcctcaagcgacttgcctgcctcagcctcccaaagtgccgggattacaggcatgagccatcgcacccgtcctccagtaccattttaaacaaatacatattgtggactacgcaccaatagaaattaaggtggcaaaaccgtatcattagtaaagtaagtgaaagccttagtctttttgtttattccttattccccaaaggagttactaagtgaaggaattttccagctgcctttatttttttgagacggagtcttgttctgttgcccaggctggagtgcagtggcacgatcttggctcaccacaacctcctcctcctgggttccagcgattctcctgcctcagcctccagagtagctgggactacaggcgcccaccaacatgcccggctaatttgtgtatttacagtagagatggggtttcattatgttggccaggatggtcttgaactcctgacctcaagatcagcctgcctcggcctcccacagtgctgggattacatgcgtgagccactgcgcccggccttccagctgcatttctgaggtcacaagtatggccttaaatgattgccctcaagaacacagcttttgaaggtaatcatatgcaagtaaattacaatcaaatggaactgtatgattattttattattttaatgctaaactgaacagtgaactgaaatcagaggagaaagaaaatcaagctagtggctcactctcaatagtgtcctctaattttattgatgcttcagttttcataaagtgcaataaacaaaataaataaatgaaaaaagctttgaagatttatatacagttttgaggttaagataaattactgactatattcctttcagccttttaactctgtgaaagctgtaacgtacattaaaagcacattgaactaggttaaataatgatctttcccccttagatcaatctagtattaaggagtatataattatgcaagttcattctataacacaaggctagactaaaaggaaaatttttgtgctacagactaaatccagatacagtcaggtgctgagcagtattcctggcttcaaaataggaggtatctgtttcatcatctggctgggggatgaaaggcatagtctgatgctgcagattttcccagtccacatcactgaagagaggatgacgttttagctctttcattccagctctctttgtatcatcaatggttaaaagtatttctactgcactttgagcattatcagataacttttcttcaccttctggccaagggatatctcttttcagaatattctggaatacttgttgtggtgtttcatcattgaaagggggaattcctgttagaaattcaaacaagcaaactccaagtgcccaccagtctaccgcaggaccggaagtcagaaatccatgggccctgcctagtaacagctcaggtgcaaggtagtctggggttcctagaattcgcccatcatcaacgggggccacccctcttctcacactcttcggagttcggtatggagttcccgacttgatctgatttggggtctgctgatgtggcatacaggatcttcttttttgagtaggggttatagccatgggatatgaaccactgtaggcacacgaaatatccattgcatctaaagaagtcatgttcattctggatggttctgagttattggatgcattaatatgactgttaaaacttcgaaaagcaacagcatttcttttagaggctaacgttttcagcacctccaaaggaggacctaacattttttggttactctcttgtacagcagggttctcgacaccttttggtgaggtcttttcttggcaatctggtgttacaataagtggatcttcaatatttgattcttcaaaagaggattctttgatgcttctatctgaatctaagggctgactttctaatggactttccattatagaaattccaggaaaagatgaatcagagttcatagaaatatttttagaagctctatcatcatcagaacatagaaaactagaacttaagtagtccctcttactattcttttcacagtcttcatcgagttcacacataaggttttttgctatcattggtataggtaatttttctggtgtttgttgtttatcagtaaaagaattgacaatgttctccttattagcacagtcattttgttgacttttgtgcactgatagcttaaggtcctgcacttcaactgttaagcctgtattttgatttgtataacaatttgtcatttcgttatgcttatactctacacaagtttttttattctgtataatttttttacaaggactggagtcaaccaactcaaaatttctttttaaacttcttttcccaaggtgctcttcagatatcccaccagaatccacagcccactgatttgactgatggaaacctaactgacttgtgtcagtgtccatatttatattatttacatccagttctactgcttcccaagaaacttccccagagaagcattttttagcaaggtttacacaagagcgtccagtggtgggaagggcactgctgttatgaatgggagaaagagctaactccagatcctttttattgaaacctttcgtctcaatggcatttgcagattttgcgcataacttttcaactgcattccaactcatcattgttgggcccaatgcttcatcactttcctggcaatctttttcccatttgggactgctgtggcattctgattccacactggatatgaaggtgtgggattgactactggcactggatgtggccagccttttcctagactggagtaaattagaagttagacacttcacaggcattcctgggttggaggcaactgtttcaagacatgattttagtaatttgctagaataaggcgtagtgtccttttgatctacagacatagggcatacgagtccttgagaaagctgtgatgtttcagacagacaggctgaaaggatgtttgcagggtcttgatttttttctgcaattggtgtgttaaatcccaacgagctgataagcgataacacttgtcctggggttcttgaataatcttgtctaggttttgccattgatggtgttgtaaggatatccatcatattaatatctctattcaaagtaacttttgaaaggccaaaatccgtcagtttaatatgaccctcattagaaataagcatattgtccggtttcaagtccctctactcccagacacttgggaggctaaggcagggggattgcttgagccccagaggtcgaggctgcagtgagccaaggtcaagtcactgcactgcacaacctggatgacaaagtgagaccctgtggatgattccatgtctgtgaaggtagtctagagccagtgctacttcagaaatatatttcacagccatctcttcatcaaaataaccatatatatgtaggagagacttgacatctcccccaataagatattccattaccaagtagacattgtttgcagactgcagtgaataatacaaatggacaatgaatgggcttttgcttagtgccagtgcatctctctcagcttggacctgatgagtcatatttttgttgatcatgtctgcttttttaacaacctttactgcatacaatttgccgcctttctgccccagatacactttcccgaaggcgccccggctaatgggcttcactatgctgaattcctcaatggagggcggttttggcactgcgatcctattcacgccctcctcagtcgccgcgcctcctccaggctccttcttgcttcccgcggtgggatccatcgctggacagcatacagcggccccgcagacactgcccctccgcgagcagccactcccgccaactgggttcaaagt

SEQ ID NO: 11901 - RNA, 3840 nt, Homo sapiens
  source 1..3840: mol_type = other RNA
ctgaatagctgggactacaggtgtgcgtcaccatacctggctaatttttctatttttagtagagaccaggttttgccatgttggccaggctggtctcaaactccaggcctcaagcgacttgcctgcctcagcctcccaaagtgccgggattacaggcatgagccatcgcacccgtcctccagtaccattttaaacaaatacatattgtggactacgcaccaatagaaattaaggtggcaaaaccgtatcattagtaaagtaagtgaaagccttagtctttttgtttattccttattccccaaaggagttactaagtgaaggaattttccagctgcctttatttttttgagacggagtcttgttctgttgcccaggctggagtgcagtggcacgatcttggctcaccacaacctcctcctcctgggttccagcgattctcctgcctcagcctccagagtagctgggactacaggcgcccaccaacatgcccggctaatttgtgtatttacagtagagatggggtttcattatgttggccaggatggtcttgaactcctgacctcaagatcagcctgcctcggcctcccacagtgctgggattacatgcgtgagccactgcgcccggccttccagctgcatttctgaggtcacaagtatggccttaaatgattgccctcaagaacacagcttttgaaggtaatcatatgcaagtaaattacaatcaaatggaactgtatgattattttattattttaatgctaaactgaacagtgaactgaaatcagaggagaaagaaaatcaagctagtggctcactctcaatagtgtcctctaattttattgatgcttcagttttcataaagtgcaataaacaaaataaataaatgaaaaaagctttgaagatttatatacagttttgaggttaagataaattactgactatattcctttcagccttttaactctgtgaaagctgtaacgtacattaaaagcacattgaactaggttaaataatgatctttcccccttagatcaatctagtattaaggagtatataattatgcaagttcattctataacacaaggctagactaaaaggaaaatttttgtgctacagactaaatccagatacagtcaggtgctgagcagtattcctggcttcaaaataggaggtatctgtttcatcatctggctgggggatgaaaggcatagtctgatgctgcagattttcccagtccacatcactgaagagaggatgacgttttagctctttcattccagctctctttgtatcatcaatggttaaaagtatttctactgcactttgagcattatcagataacttttcttcaccttctggccaagggatatctcttttcagaatattctggaatacttgttgtggtgtttcatcattgaaagggggaattcctgttagaaattcaaacaagcaaactccaagtgcccaccagtctaccgcaggaccggaagtcagaaatccatgggccctgcctagtaacagctcaggtgcaaggtagtctggggttcctagaattcgcccatcatcaacgggggccacccctcttctcacactcttcggagttcggtatggagttcccgacttgatctgatttggggtctgctgatgtggcatacaggatcttcttttttgagtaggggttatagccatgggatatgaaccactgtaggcacacgaaatatccattgcatctaaagaagtcatgttcattctggatggttctgagttattggatgcattaatatgactgttaaaacttcgaaaagcaacagcatttcttttagaggctaacgttttcagcacctccaaaggaggacctaacattttttggttactctcttgtacagcagggttctcgacaccttttggtgaggtcttttcttggcaatctggtgttacaataagtggatcttcaatatttgattcttcaaaagaggattctttgatgcttctatctgaatctaagggctgactttctaatggactttccattatagaaattccaggaaaagatgaatcagagttcatagaaatatttttagaagctctatcatcatcagaacatagaaaactagaacttaagtagtccctcttactattcttttcacagtcttcatcgagttcacacataaggttttttgctatcattggtataggtaatttttctggtgtttgttgtttatcagtaaaagaattgacaatgttctccttattagcacagtcattttgttgacttttgtgcactgatagcttaaggtcctgcacttcaactgttaagcctgtattttgatttgtataacaatttgtcatttcgttatgcttatactctacacaagtttttttattctgtataatttttttacaaggactggagtcaaccaactcaaaatttctttttaaacttcttttcccaaggtgctcttcagatatcccaccagaatccacagcccactgatttgactgatggaaacctaactgacttgtgtcagtgtccatatttatattatttacatccagttctactgcttcccaagaaacttccccagagaagcattttttagcaaggtttacacaagagcgtccagtggtgggaagggcactgctgttatgaatgggagaaagagctaactccagatcctttttattgaaacctttcgtctcaatggcatttgcagattttgcgcataacttttcaactgcattccaactcatcattgttgggcccaatgcttcatcactttcctggcaatctttttcccatttgggactgctgtggcattctgattccacactggatatgaaggtgtgggattgactactggcactggatgtggccagccttttcctagactggagtaaattagaagttagacacttcacaggcattcctgggttggaggcaactgtttcaagacatgattttagtaatttgctagaataaggcgtagtgtccttttgatctacagacatagggcatacgagtccttgagaaagctgtgatgtttcagacagacaggctgaaaggatgtttgcagggtcttgatttttttctgcaattggtgtgttaaatcccaacgagctgataagcgataacacttgtcctggggttcttgaataatcttgtctaggttttgccattgatggtgttgtaaggatatccatcatattaatatctctattcaaagtaacttttgaaaggccaaaatccgtcagtttaatatgaccctcattagaaataagcatattgtccggtttcaagtccctgtggatgattccatgtctgtgaaggtagtctagagccagtgctacttcagaaatatatttcacagccatctcttcatcaaaataaccatatatatgtaggagagacttgacatctcccccaataagatattccattaccaagtagacattgtttgcagactgcagtgaataatacaaatggacaatgaatgggcttttgcttagtgccagtgcatctctctcagcttggacctgatgagtcatatttttgttgatcatgtctgcttttttaacaacctttactgcatacaatttgccgcctttctgccccagatacactttcccgaaggcgccccggctaatgggcttcactatgctgaattcctcaatggagggcggttttggcactgcgatcctattcacgccctcctcagtcgccgcgcctcctccaggctccttcttgcttcccgcggtgggatccatcgctggacagcatacagcggccccgcagacactgcccctccgcgagcagccactcccgccaactgggttcaaagt

SEQ ID NO: 11902 - RNA, 3683 nt, Homo sapiens
  source 1..3683: mol_type = other RNA
ctgaatagctgggactacaggtgtgcgtcaccatacctggctaatttttctatttttagtagagaccaggttttgccatgttggccaggctggtctcaaactccaggcctcaagcgacttgcctgcctcagcctcccaaagtgccgggattacaggcatgagccatcgcacccgtcctccagtaccattttaaacaaatacatattgtggactacgcaccaatagaaattaaggtggcaaaaccgtatcattagtaaagtaagtgaaagccttagtctttttgtttattccttattccccaaaggagttactaagtgaaggaattttccagctgcctttatttttttgagacggagtcttgttctgttgcccaggctggagtgcagtggcacgatcttggctcaccacaacctcctcctcctgggttccagcgattctcctgcctcagcctccagagtagctgggactacaggcgcccaccaacatgcccggctaatttgtgtatttacagtagagatggggtttcattatgttggccaggatggtcttgaactcctgacctcaagatcagcctgcctcggcctcccacagtgctgggattacatgcgtgagccactgcgcccggccttccagctgcatttctgaggtcacaagtatggccttaaatgattgccctcaagaacacagcttttgaaggtaatcatatgcaagtaaattacaatcaaatggaactgtatgattattttattattttaatgctaaactgaacagtgaactgaaatcagaggagaaagaaaatcaagctagtggctcactctcaatagtgtcctctaattttattgatgcttcagttttcataaagtgcaataaacaaaataaataaatgaaaaaagctttgaagatttatatacagttttgaggttaagataaattactgactatattcctttcagccttttaactctgtgaaagctgtaacgtacattaaaagcacattgaactaggttaaataatgatctttcccccttagatcaatctagtattaaggagtatataattatgcaagttcattctataacacaaggctagactaaaaggaaaatttttgtgctacagactaaatccagatacagtcaggtgctgagcagtattcctggcttcaaaataggaggtatctgtttcatcatctggctgggggatgaaaggcatagtctgatgctgcagattttcccagtccacatcactgaagagaggatgacgttttagctctttcattccagctctctttgtatcatcaatggttaaaagtatttctactgcactttgagcattatcagataacttttcttcaccttctggccaagggatatctcttttcagaatattctggaatacttgttgtggtgtttcatcattgaaagggggaattcctgttagaaattcaaacaagcaaactccaagtgcccaccagtctaccgcaggacctgatgtggcatacaggatcttcttttttgagtaggggttatagccatgggatatgaaccactgtaggcacacgaaatatccattgcatctaaagaagtcatgttcattctggatggttctgagttattggatgcattaatatgactgttaaaacttcgaaaagcaacagcatttcttttagaggctaacgttttcagcacctccaaaggaggacctaacattttttggttactctcttgtacagcagggttctcgacaccttttggtgaggtcttttcttggcaatctggtgttacaataagtggatcttcaatatttgattcttcaaaagaggattctttgatgcttctatctgaatctaagggctgactttctaatggactttccattatagaaattccaggaaaagatgaatcagagttcatagaaatatttttagaagctctatcatcatcagaacatagaaaactagaacttaagtagtccctcttactattcttttcacagtcttcatcgagttcacacataaggttttttgctatcattggtataggtaatttttctggtgtttgttgtttatcagtaaaagaattgacaatgttctccttattagcacagtcattttgttgacttttgtgcactgatagcttaaggtcctgcacttcaactgttaagcctgtattttgatttgtataacaatttgtcatttcgttatgcttatactctacacaagtttttttattctgtataatttttttacaaggactggagtcaaccaactcaaaatttctttttaaacttcttttcccaaggtgctcttcagatatcccaccagaatccacagcccactgatttgactgatggaaacctaactgacttgtgtcagtgtccatatttatattatttacatccagttctactgcttcccaagaaacttccccagagaagcattttttagcaaggtttacacaagagcgtccagtggtgggaagggcactgctgttatgaatgggagaaagagctaactccagatcctttttattgaaacctttcgtctcaatggcatttgcagattttgcgcataacttttcaactgcattccaactcatcattgttgggcccaatgcttcatcactttcctggcaatctttttcccatttgggactgctgtggcattctgattccacactggatatgaaggtgtgggattgactactggcactggatgtggccagccttttcctagactggagtaaattagaagttagacacttcacaggcattcctgggttggaggcaactgtttcaagacatgattttagtaatttgctagaataaggcgtagtgtccttttgatctacagacatagggcatacgagtccttgagaaagctgtgatgtttcagacagacaggctgaaaggatgtttgcagggtcttgatttttttctgcaattggtgtgttaaatcccaacgagctgataagcgataacacttgtcctggggttcttgaataatcttgtctaggttttgccattgatggtgttgtaaggatatccatcatattaatatctctattcaaagtaacttttgaaaggccaaaatccgtcagtttaatatgaccctcattagaaataagcatattgtccggtttcaagtccctgtggatgattccatgtctgtgaaggtagtctagagccagtgctacttcagaaatatatttcacagccatctcttcatcaaaataaccatatatatgtaggagagacttgacatctcccccaataagatattccattaccaagtagacattgtttgcagactgcagtgaataatacaaatggacaatgaatgggcttttgcttagtgccagtgcatctctctcagcttggacctgatgagtcatatttttgttgatcatgtctgcttttttaacaacctttactgcatacaatttgccgcctttctgccccagatacactttcccgaaggcgccccggctaatgggcttcactatgctgaattcctcaatggagggcggttttggcactgcgatcctattcacgccctcctcagtcgccgcgcctcctccaggctccttcttgcttcccgcggtgggatccatcgctggacagcatacagcggccccgcagacactgcccctccgcgagcagccactcccgccaactgggttcaaagt

SEQ ID NO: 11903 - RNA, 4165 nt, Homo sapiens
  source 1..4165: mol_type = other RNA
ctgaatagctgggactacaggtgtggaccaccactccccagctctgcatataatatttttttttttttttttttttttgagacagggtctcactctgtcacccaggctggagtgcagttgcacaattccagctcactgcaacctgcacctcccaggctcaagtgatcctcctatcttagcctcctgagtagctgggactacaggcgcacaccaccacagccagctaattctctgtatttttggtagagacaaggtttcgccatgttgcccaggctggtctcgaactcctgagttcagatgatccacccacctcggtgcatatagtatttttaaaatgtattttgaaaggataatgtgaacaaaagtccaaataatacaaaactagattctaagcagcccacctagttgaacctcttcttggaggcataattatcactggtttctcgtgcatccttagagataattatatgcatatgcaaataagatgttcacacaccacataccttgttttacacaaatggcagtacagtttcaaatatgtttttcatgtaacatttaatttttctatttttagtagagacggggttttaccatgttggccagaatggtcttgatctgacctcgtgatctgcccacctcggcctcccaaagtgctgggattacaggcatgagccatggcacctgacccaccattacttttattttgaatcttgtctgtgtagcaagcagtgcagtgagaaattttgttggcagaggaaaaaaattcctttttgcatcaggtcaagcccccaaactagccaaagaaaagctgtgtaatctattcagaagtactggagatgtgctgcacattagggagaatggagaattactggtcacaacgaatcccggtttctatcacccatagctatgtgaacccagacaatcattaagcaatctgggttggttagatggcttctaagatctctttcaataaaaaagttctaagattcagaattcctgagaagttgcagctaacatacactgtataagattttatacattaaaaacaaacatctcatttggtcttaacccagtaggaagaaaagattaaaatattttgtatttgaaataaacagaccctaatattaattatgaccagggaaataattttaaaacatcccaaaggaaagttctctaacttttaaaatattataaattaatactgcaacaggagctacctcaaatctctcaacaaagatggaatataattaaatagaagaactagcaccagttatcaactatgtgcctgcccttgaactctctgcatttttgtagttctgttttaaagatgaggaaaataagcttcatagataaatgttattttgtctaaggtcatccagtttgcttctccattaaacaatcaattaagatgactattcagtgcacaaactgtaatctgttttattaatacttccaagttttctacatgactctggatttatactttgtatcaattctcttgctggttaagaaaaaaaacaagatttattaaaaactgaccataaataatgtgtaaactaaggagagttttgtctttttccttactgaaggacaaggaatcagtaaagaagttctttgctttgcttaatgaagatcaaaacctggtaattaaatttggctaatataatcattccttttctgacaagacttttttcacctttattcacctgagtaacttacctgtttccaaagacacctaggaaattcagaatgttatatatgcttttccttatttactataatttataggacatgagtggatggattctcttcaatagagaaaatgattttctctaattaaaatgcaccaaattgatgtactaagagattgctttagatgaacacatttatgttcagtgaagattatgtggtcttcaatgacactgcaatataattactaggtacaaaacaaaagcagagatccacacacaatggctcactgtcttcgatgacaacacttttaggatctcatttattcattctttaagtaatttttcttttaaaaaagggataggtggaaaaaatagttgggaaatctttaactaggctaaggtttagacataggtataaattatttattttgtaacattcaaaaaccaaaaaccaccctgacatactgggtggcaagaaaagtcaagatcagattaaacatttgttttgcactaatcacaaaactaataatccaagtcactatcatcaactccagttgatctcagctctgattatgcatcagaacaccctgtgaggtctattaagttcctataccaaatcccaaacactcttgaatcagtctacaaagttgggacctaggtatctgtacattttttaaagttcctcaaaaaattctgcttctaggcaaatgtaatagatattgtgcgttgctcatgtttttcctatcagaaccatgattttaaaaaaactatcctttctgtccccatatatccctcatgtggcctccacttctactctcagctccagtggacctgactgccctaaaggttattctagaccctttgccagtgactggctcagggatggacaggtctaagttactttagagcaatgagacctaaggatatggaaagtgaattctgggaaagctttctcatactaggacagggcccctagaatccagcctgactcttccgctgcatgtaaatgaagatgcacaaggctccaactgctactggcaatcatcccatgaccacgagggtagccagccttaggatgatgccaatgttgtggttgaaaagggggtggggtgtggaggcgggttcccaaggttcttgatgacattactgaatcattggatcagaaacactgcagcacattctgtcaatagatttcatgtattgtgaatcaatatattttcttactgtttttaagtcattttaagttggacttttagtggtcagcatctgaatgttaaagagtggtcccagcacagcattctttaattataacaatctgtatcaagtagaatccacacaaacaccccttcgtacttacataatctgtaaatctgatgtatctttcctattttaacaaaatctttaatttatatcgttataccttactaaagtgttaatgtgcattgcattcacttcattatttactcagagttcttgctgtaggctttgtcttgaatgtgtaggaccattcgtcgtgcatagaagtccctatattcctctggtaactcggccagtgttttcaaggctctgtccagaatttgtgcagctcttgatgctgctgtaggatctttgtttccataggtatctgttttatcatagcattcagatggaaggtgcttccaaaagatattcactcccactccaaactcttcagaaattacattatggaaccataaagcaggaatgaataatacatcaccagcttcaagggaacattcatatcttctagccttggaaaaaagtggatatttagccaagtctgggttatctatattcagtacttctgatttagtacatcataatgagtccatagttgtaatcctggtgaactaattcgaaaaacactggaaaagaactgttcctctttgaagaattctggaaacttaatatctcctttcaacaaaggaaactgctttctgatatctgcaacatcctttctagggtcttctccaagtgaccgtaagtagtatttctcatcctctgaaacaaagaattctttatgtttctcttcagctgccctctggaccaactggtcaaaaggtaaagttctatatacaaagttcttactaatgaagtccatctgtgcaactgcagcaacatgaatctttacttctttcttccctccaacttggcttaggtaatccactgtccatttgcttgtacatggccccaaatcaatcccttccaacacaagaggttttctctgtgggtagaggtgctgcatgaactgctcccgagaaacgccctccagccggggtaccgggaggtgctgcccggccatggttgctcacgcctgccctcttccaggtcttcggaacttcggctctaaagcgttcctcagcgccatccgcccggaaacacgagcgacagagaaaaggtccgcgaggccggcagactccagagtggctgggtccgagcgcggggcgggttgccga

SEQ ID NO: 11904 - RNA, 4013 nt, Homo sapiens
  source 1..4013: mol_type = other RNA
ctgaatagctgggactacaggtgtggaccaccactccccagctctgcatataatatttttttttttttttttttttttgagacagggtctcactctgtcacccaggctggagtgcagttgcacaattccagctcactgcaacctgcacctcccaggctcaagtgatcctcctatcttagcctcctgagtagctgggactacaggcgcacaccaccacagccagctaattctctgtatttttggtagagacaaggtttcgccatgttgcccaggctggtctcgaactcctgagttcagatgatccacccacctcggtgcatatagtatttttaaaatgtattttgaaaggataatgtgaacaaaagtccaaataatacaaaactagattctaagcagcccacctagttgaacctcttcttggaggcataattatcactggtttctcgtgcatccttagagataattatatgcatatgcaaataagatgttcacacaccacataccttgttttacacaaatggcagtacagtttcaaatatgtttttcatgtaacatttaatttttctatttttagtagagacggggttttaccatgttggccagaatggtcttgatctgacctcgtgatctgcccacctcggcctcccaaagtgctgggattacaggcatgagccatggcacctgacccaccattacttttattttgaatcttgtctgtgtagcaagcagtgcagtgagaaattttgttggcagaggaaaaaaattcctttttgcatcaggtcaagcccccaaactagccaaagaaaagctgtgtaatctattcagaagtactggagatgtgctgcacattagggagaatggagaattactggtcacaacgaatcccggtttctatcacccatagctatgtgaacccagacaatcattaagcaatctgggttggttagatggcttctaagatctctttcaataaaaaagttctaagattcagaattcctgagaagttgcagctaacatacactgtataagattttatacattaaaaacaaacatctcatttggtcttaacccagtaggaagaaaagattaaaatattttgtatttgaaataaacagaccctaatattaattatgaccagggaaataattttaaaacatcccaaaggaaagttctctaacttttaaaatattataaattaatactgcaacaggagctacctcaaatctctcaacaaagatggaatataattaaatagaagaactagcaccagttatcaactatgtgcctgcccttgaactctctgcatttttgtagttctgttttaaagatgaggaaaataagcttcatagataaatgttattttgtctaaggtcatccagtttgcttctccattaaacaatcaattaagatgactattcagtgcacaaactgtaatctgttttattaatacttccaagttttctacatgactctggatttatactttgtatcaattctcttgctggttaagaaaaaaaacaagatttattaaaaactgaccataaataatgtgtaaactaaggagagttttgtctttttccttactgaaggacaaggaatcagtaaagaagttctttgctttgcttaatgaagatcaaaacctggtaattaaatttggctaatataatcattccttttctgacaagacttttttcacctttattcacctgagtaacttacctgtttccaaagacacctaggaaattcagaatgttatatatgcttttccttatttactataatttataggacatgagtggatggattctcttcaatagagaaaatgattttctctaattaaaatgcaccaaattgatgtactaagagattgctttagatgaacacatttatgttcagtgaagattatgtggtcttcaatgacactgcaatataattactaggtacaaaacaaaagcagagatccacacacaatggctcactgtcttcgatgacaacacttttaggatctcatttattcattctttaagtaatttttcttttaaaaaagggataggtggaaaaaatagttgggaaatctttaactaggctaaggtttagacataggtataaattatttattttgtaacattcaaaaaccaaaaaccaccctgacatactgggtggcaagaaaagtcaagatcagattaaacatttgttttgcactaatcacaaaactaataatccaagtcactatcatcaactccagttgatctcagctctgattatgcatcagaacaccctgtgaggtctattaagttcctataccaaatcccaaacactcttgaatcagtctacaaagttgggacctaggtatctgtacattttttaaagttcctcaaaaaattctgcttctaggcaaatgtaatagatattgtgcgttgctcatgtttttcctatcagaaccatgattttaaaaaaactatcctttctgtccccatatatccctcatgtggcctccacttctactctcagctccagtggacctgactgccctaaaggttattctagaccctttgccagtgactggctcagggatggacaggtctaagttactttagagcaatgagacctaaggatatggaaagtgaattctgggaaagctttctcatactaggacagggcccctagaatccagcctgactcttccgctgcatgtaaatgaagatgcacaaggctccaactgctactggcaatcatcccatgaccacgagggtagccagccttaggatgatgccaatgttgtggttgaaaagggggtggggtgtggaggcgggttcccaaggttcttgatgacattactgaatcattggatcagaaacactgcagcacattctgtcaatagatttcatgtattgtgaatcaatatattttcttactgtttttaagtcattttaagttggacttttagtggtcagcatctgaatgttaaagagtggtcccagcacagcattctttaattataacaatctgtatcaagtagaatccacacaaacaccccttcgtacttacataatctgtaaatctgatgtatctttcctattttaacaaaatctttaatttatatcgttataccttactaaagtgttaatgtgcattgcattcacttcattatttactcagagttcttgctgtaggctttgtcttgaatgtgtaggaccattcgtcgtgcatagaagtccctatattcctctggtaactcggccagtgttttcaaggctctgtccagaatttgtgcagctcttgatgctgctgtaggatctttgtttccataggtatctgttttatcatagcattcagatggaaggtgcttccaaaagatattcactcccactccaaactcttcagaaattacattatggaaccataaagcaggaatgaataatacatcaccagcttcaagggaacattcatatcttctagccttggaaaaaagtggatatttagccaagtctgggttatctatattcagtacttctgatttagtacatcataatgagtccatagttgtaatcctggtgaactaattcgaaaaacactggaaaagaactgttcctctttgaagaattctggaaacttaatatctcctttcaacaaaggaaactgctttctgatatctgcaacatcctttctagggtcttctccaagtgaccgtaagtagtatttctcatcctctgaaacaaagaattctttatgtttctcttcagctgccctctggaccaactggtcaaaaggtaaagtttaatgaagtccatctgtgcaactgcagcaacatgaatctttacttctttcttccctccaacttggcttaggtaatccactgtccatttgcttgtacatggccccaaatcaatcccttccaacacaagaggttttctctgtgggtagaggtgctgcatgaactgctcccgagaaacgccctccagccggggtaccgggaggtgctgcccggccatggttgctcacgcctgccctct

SEQ ID NO: 11905 - RNA, 3849 nt, Homo sapiens
  source 1..3849: mol_type = other RNA
ctgaatagctgggactacaggtgtggaccaccactccccagctctgcatataatatttttttttttttttttttttttgagacagggtctcactctgtcacccaggctggagtgcagttgcacaattccagctcactgcaacctgcacctcccaggctcaagtgatcctcctatcttagcctcctgagtagctgggactacaggcgcacaccaccacagccagctaattctctgtatttttggtagagacaaggtttcgccatgttgcccaggctggtctcgaactcctgagttcagatgatccacccacctcggtgcatatagtatttttaaaatgtattttgaaaggataatgtgaacaaaagtccaaataatacaaaactagattctaagcagcccacctagttgaacctcttcttggaggcataattatcactggtttctcgtgcatccttagagataattatatgcatatgcaaataagatgttcacacaccacataccttgttttacacaaatggcagtacagtttcaaatatgtttttcatgtaacatttaatttttctatttttagtagagacggggttttaccatgttggccagaatggtcttgatctgacctcgtgatctgcccacctcggcctcccaaagtgctgggattacaggcatgagccatggcacctgacccaccattacttttattttgaatcttgtctgtgtagcaagcagtgcagtgagaaattttgttggcagaggaaaaaaattcctttttgcatcaggtcaagcccccaaactagccaaagaaaagctgtgtaatctattcagaagtactggagatgtgctgcacattagggagaatggagaattactggtcacaacgaatcccggtttctatcacccatagctatgtgaacccagacaatcattaagcaatctgggttggttagatggcttctaagatctctttcaataaaaaagttctaagattcagaattcctgagaagttgcagctaacatacactgtataagattttatacattaaaaacaaacatctcatttggtcttaacccagtaggaagaaaagattaaaatattttgtatttgaaataaacagaccctaatattaattatgaccagggaaataattttaaaacatcccaaaggaaagttctctaacttttaaaatattataaattaatactgcaacaggagctacctcaaatctctcaacaaagatggaatataattaaatagaagaactagcaccagttatcaactatgtgcctgcccttgaactctctgcatttttgtagttctgttttaaagatgaggaaaataagcttcatagataaatgttattttgtctaaggtcatccagtttgcttctccattaaacaatcaattaagatgactattcagtgcacaaactgtaatctgttttattaatacttccaagttttctacatgactctggatttatactttgtatcaattctcttgctggttaagaaaaaaaacaagatttattaaaaactgaccataaataatgtgtaaactaaggagagttttgtctttttccttactgaaggacaaggaatcagtaaagaagttctttgctttgcttaatgaagatcaaaacctggtaattaaatttggctaatataatcattccttttctgacaagacttttttcacctttattcacctgagtaacttacctgtttccaaagacacctaggaaattcagaatgttatatatgcttttccttatttactataatttataggacatgagtggatggattctcttcaatagagaaaatgattttctctaattaaaatgcaccaaattgatgtactaagagattgctttagatgaacacatttatgttcagtgaagattatgtggtcttcaatgacactgcaatataattactaggtacaaaacaaaagcagagatccacacacaatggctcactgtcttcgatgacaacacttttaggatctcatttattcattctttaagtaatttttcttttaaaaaagggataggtggaaaaaatagttgggaaatctttaactaggctaaggtttagacataggtataaattatttattttgtaacattcaaaaaccaaaaaccaccctgacatactgggtggcaagaaaagtcaagatcagattaaacatttgttttgcactaatcacaaaactaataatccaagtcactatcatcaactccagttgatctcagctctgattatgcatcagaacaccctgtgaggtctattaagttcctataccaaatcccaaacactcttgaatcagtctacaaagttgggacctaggtatctgtacattttttaaagttcctcaaaaaattctgcttctaggcaaatgtaatagatattgtgcgttgctcatgtttttcctatcagaaccatgattttaaaaaaactatcctttctgtccccatatatccctcatgtggcctccacttctactctcagctccagtggacctgactgccctaaaggttattctagaccctttgccagtgactggctcagggatggacaggtctaagttactttagagcaatgagacctaaggatatggaaagtgaattctgggaaagctttctcatactaggacagggcccctagaatccagcctgactcttccgctgcatgtaaatgaagatgcacaaggctccaactgctactggcaatcatcccatgaccacgagggtagccagccttaggatgatgccaatgttgtggttgaaaagggggtggggtgtggaggcgggttcccaaggttcttgatgacattactgaatcattggatcagaaacactgcagcacattctgtcaatagatttcatgtattgtgaatcaatatattttcttactgtttttaagtcattttaagttggacttttagtggtcagcatctgaatgttaaagagtggtcccagcacagcattctttaattataacaatctgtatcaagtagaatccacacaaacaccccttcgtacttacataatctgtaaatctgatgtatctttcctattttaacaaaatctttaatttatatcgttataccttactaaagtgttaatgtgcattgcattcacttcattatttactcagagttcttgctgtaggctttgtcttgaatgtgtaggaccattcgtcgtgcatagaagtccctatattcctctggtaactcggccagtgttttcaaggctctgtccagaatttgtgcagctcttgatgctgctgtaggatctttgtttccataggtatctgttttatcatagcattcagatggaaggtgcttccaaaagatattcactcccactccaaactcttcagaaattacattatggaaccataaagcaggaatgaataatacatcaccagcttcaagggaacattcatatcttctagccttggaaaaaagtggatatttagccaagtctgggttatctatattcagtacttctgatttagtacctctgaaacaaagaattctttatgtttctcttcagctgccctctggaccaactggtcaaaaggtaaagttctatatacaaagttcttactaatgaagtccatctgtgcaactgcagcaacatgaatctttacttctttcttccctccaacttggcttaggtaatccactgtccatttgcttgtacatggccccaaatcaatcccttccaacacaagaggttttctctgtgggtagaggtgctgcatgaactgctcccgagaaacgccctccagccggggtaccgggaggtgctgcccggccatggttgctcacgcctgccctct

SEQ ID NO: 11906 - RNA, 4120 nt, Homo sapiens
  source 1..4120: mol_type = other RNA
ctgaatagctgggactacaggtgtggaccaccactccccagctctgcatataatatttttttttttttttttttttttgagacagggtctcactctgtcacccaggctggagtgcagttgcacaattccagctcactgcaacctgcacctcccaggctcaagtgatcctcctatcttagcctcctgagtagctgggactacaggcgcacaccaccacagccagctaattctctgtatttttggtagagacaaggtttcgccatgttgcccaggctggtctcgaactcctgagttcagatgatccacccacctcggtgcatatagtatttttaaaatgtattttgaaaggataatgtgaacaaaagtccaaataatacaaaactagattctaagcagcccacctagttgaacctcttcttggaggcataattatcactggtttctcgtgcatccttagagataattatatgcatatgcaaataagatgttcacacaccacataccttgttttacacaaatggcagtacagtttcaaatatgtttttcatgtaacatttaatttttctatttttagtagagacggggttttaccatgttggccagaatggtcttgatctgacctcgtgatctgcccacctcggcctcccaaagtgctgggattacaggcatgagccatggcacctgacccaccattacttttattttgaatcttgtctgtgtagcaagcagtgcagtgagaaattttgttggcagaggaaaaaaattcctttttgcatcaggtcaagcccccaaactagccaaagaaaagctgtgtaatctattcagaagtactggagatgtgctgcacattagggagaatggagaattactggtcacaacgaatcccggtttctatcacccatagctatgtgaacccagacaatcattaagcaatctgggttggttagatggcttctaagatctctttcaataaaaaagttctaagattcagaattcctgagaagttgcagctaacatacactgtataagattttatacattaaaaacaaacatctcatttggtcttaacccagtaggaagaaaagattaaaatattttgtatttgaaataaacagaccctaatattaattatgaccagggaaataattttaaaacatcccaaaggaaagttctctaacttttaaaatattataaattaatactgcaacaggagctacctcaaatctctcaacaaagatggaatataattaaatagaagaactagcaccagttatcaactatgtgcctgcccttgaactctctgcatttttgtagttctgttttaaagatgaggaaaataagcttcatagataaatgttattttgtctaaggtcatccagtttgcttctccattaaacaatcaattaagatgactattcagtgcacaaactgtaatctgttttattaatacttccaagttttctacatgactctggatttatactttgtatcaattctcttgctggttaagaaaaaaaacaagatttattaaaaactgaccataaataatgtgtaaactaaggagagttttgtctttttccttactgaaggacaaggaatcagtaaagaagttctttgctttgcttaatgaagatcaaaacctggtaattaaatttggctaatataatcattccttttctgacaagacttttttcacctttattcacctgagtaacttacctgtttccaaagacacctaggaaattcagaatgttatatatgcttttccttatttactataatttataggacatgagtggatggattctcttcaatagagaaaatgattttctctaattaaaatgcaccaaattgatgtactaagagattgctttagatgaacacatttatgttcagtgaagattatgtggtcttcaatgacactgcaatataattactaggtacaaaacaaaagcagagatccacacacaatggctcactgtcttcgatgacaacacttttaggatctcatttattcattctttaagtaatttttcttttaaaaaagggataggtggaaaaaatagttgggaaatctttaactaggctaaggtttagacataggtataaattatttattttgtaacattcaaaaaccaaaaaccaccctgacatactgggtggcaagaaaagtcaagatcagattaaacatttgttttgcactaatcacaaaactaataatccaagtcactatcatcaactccagttgatctcagctctgattatgcatcagaacaccctgtgaggtctattaagttcctataccaaatcccaaacactcttgaatcagtctacaaagttgggacctaggtatctgtacattttttaaagttcctcaaaaaattctgcttctaggcaaatgtaatagatattgtgcgttgctcatgtttttcctatcagaaccatgattttaaaaaaactatcctttctgtccccatatatccctcatgtggcctccacttctactctcagctccagtggacctgactgccctaaaggttattctagaccctttgccagtgactggctcagggatggacaggtctaagttactttagagcaatgagacctaaggatatggaaagtgaattctgggaaagctttctcatactaggacagggcccctagaatccagcctgactcttccgctgcatgtaaatgaagatgcacaaggctccaactgctactggcaatcatcccatgaccacgagggtagccagccttaggatgatgccaatgttgtggttgaaaagggggtggggtgtggaggcgggttcccaaggttcttgatgacattactgaatcattggatcagaaacactgcagcacattctgtcaatagatttcatgtattgtgaatcaatatattttcttactgtttttaagtcattttaagttggacttttagtggtcagcatctgaatgttaaagagtggtcccagcacagcattctttaattataacaatctgtatcaagtagaatccacacaaacaccccttcgtacttacataatctgtaaatctgatgtatctttcctattttaacaaaatctttaatttatatcgttataccttactaaagtgttaatgtgcattgcattcacttcattatttactcagagttcttgctgtaggctttgtcttgaatgtgtaggaccattcgtcgtgcatagaagtccctatattcctctggtaactcggccagtgttttcaaggctctgtccagaatttgtgcagctcttgatgctgctgtaggatctttgtttccataggtatctgttttatcatagcattcagatggaaggtgcttccaaaagatattcactcccactccaaactcttcagaaattacattatggaaccataaagcaggaatgaataatacatcaccagcttcaagggaacattcatatcttctagccttggaaaaaagtggatatttagccaagtctgggttatctatattcagtacttctgatttagtaccttttaaatataaatactgggcatctcgaggactgaagagtacaacacgcttttttcctgtcacttgtattaacaaattatccattacatcataatgagtccatagttgtaatcctggtgaactaattcgaaaaacactggaaaagaactgttcctctttgaagaattctggaaacttaatatctcctttcaacaaaggaaactgctttctgatatctgcaacatcctttctagggtcttctccaagtgaccgtaagtagtatttctcatcctctgaaacaaagaattctttatgtttctcttcagctgccctctggaccaactggtcaaaaggtaaagttctatatacaaagttcttactaatgaagtccatctgtgcaactgcagcaacatgaatctttacttctttcttccctccaacttggcttaggtaatccactgtccatttgcttgtacatggccccaaatcaatcccttccaacacaagaggttttctctgtgggtagaggtgctgcatgaactgctcccgagaaacgccctccagccggggtaccgggaggtgctgcccggccatggttgctcacgcctgccctct

SEQ ID NO: 11907 - RNA, 3965 nt, Homo sapiens
  source 1..3965: mol_type = other RNA
ctgaatagctgggactacaggtgtggaccaccactccccagctctgcatataatatttttttttttttttttttttttgagacagggtctcactctgtcacccaggctggagtgcagttgcacaattccagctcactgcaacctgcacctcccaggctcaagtgatcctcctatcttagcctcctgagtagctgggactacaggcgcacaccaccacagccagctaattctctgtatttttggtagagacaaggtttcgccatgttgcccaggctggtctcgaactcctgagttcagatgatccacccacctcggtgcatatagtatttttaaaatgtattttgaaaggataatgtgaacaaaagtccaaataatacaaaactagattctaagcagcccacctagttgaacctcttcttggaggcataattatcactggtttctcgtgcatccttagagataattatatgcatatgcaaataagatgttcacacaccacataccttgttttacacaaatggcagtacagtttcaaatatgtttttcatgtaacatttaatttttctatttttagtagagacggggttttaccatgttggccagaatggtcttgatctgacctcgtgatctgcccacctcggcctcccaaagtgctgggattacaggcatgagccatggcacctgacccaccattacttttattttgaatcttgtctgtgtagcaagcagtgcagtgagaaattttgttggcagaggaaaaaaattcctttttgcatcaggtcaagcccccaaactagccaaagaaaagctgtgtaatctattcagaagtactggagatgtgctgcacattagggagaatggagaattactggtcacaacgaatcccggtttctatcacccatagctatgtgaacccagacaatcattaagcaatctgggttggttagatggcttctaagatctctttcaataaaaaagttctaagattcagaattcctgagaagttgcagctaacatacactgtataagattttatacattaaaaacaaacatctcatttggtcttaacccagtaggaagaaaagattaaaatattttgtatttgaaataaacagaccctaatattaattatgaccagggaaataattttaaaacatcccaaaggaaagttctctaacttttaaaatattataaattaatactgcaacaggagctacctcaaatctctcaacaaagatggaatataattaaatagaagaactagcaccagttatcaactatgtgcctgcccttgaactctctgcatttttgtagttctgttttaaagatgaggaaaataagcttcatagataaatgttattttgtctaaggtcatccagtttgcttctccattaaacaatcaattaagatgactattcagtgcacaaactgtaatctgttttattaatacttccaagttttctacatgactctggatttatactttgtatcaattctcttgctggttaagaaaaaaaacaagatttattaaaaactgaccataaataatgtgtaaactaaggagagttttgtctttttccttactgaaggacaaggaatcagtaaagaagttctttgctttgcttaatgaagatcaaaacctggtaattaaatttggctaatataatcattccttttctgacaagacttttttcacctttattcacctgagtaacttacctgtttccaaagacacctaggaaattcagaatgttatatatgcttttccttatttactataatttataggacatgagtggatggattctcttcaatagagaaaatgattttctctaattaaaatgcaccaaattgatgtactaagagattgctttagatgaacacatttatgttcagtgaagattatgtggtcttcaatgacactgcaatataattactaggtacaaaacaaaagcagagatccacacacaatggctcactgtcttcgatgacaacacttttaggatctcatttattcattctttaagtaatttttcttttaaaaaagggataggtggaaaaaatagttgggaaatctttaactaggctaaggtttagacataggtataaattatttattttgtaacattcaaaaaccaaaaaccaccctgacatactgggtggcaagaaaagtcaagatcagattaaacatttgttttgcactaatcacaaaactaataatccaagtcactatcatcaactccagttgatctcagctctgattatgcatcagaacaccctgtgaggtctattaagttcctataccaaatcccaaacactcttgaatcagtctacaaagttgggacctaggtatctgtacattttttaaagttcctcaaaaaattctgcttctaggcaaatgtaatagatattgtgcgttgctcatgtttttcctatcagaaccatgattttaaaaaaactatcctttctgtccccatatatccctcatgtggcctccacttctactctcagctccagtggacctgactgccctaaaggttattctagaccctttgccagtgactggctcagggatggacaggtctaagttactttagagcaatgagacctaaggatatggaaagtgaattctgggaaagctttctcatactaggacagggcccctagaatccagcctgactcttccgctgcatgtaaatgaagatgcacaaggctccaactgctactggcaatcatcccatgaccacgagggtagccagccttaggatgatgccaatgttgtggttgaaaagggggtggggtgtggaggcgggttcccaaggttcttgatgacattactgaatcattggatcagaaacactgcagcacattctgtcaatagatttcatgtattgtgaatcaatatattttcttactgtttttaagtcattttaagttggacttttagtggtcagcatctgaatgttaaagagtggtcccagcacagcattctttaattataacaatctgtatcaagtagaatccacacaaacaccccttcgtacttacataatctgtaaatctgatgtatctttcctattttaacaaaatctttaatttatatcgttataccttactaaagtgttaatgtgcattgcattcacttcattatttactcagagttcttgctgtaggctttgtcttgaatgtgtaggaccattcgtcgtgcatagaagtccctatattcctctggtaactcggccagtgttttcaaggctctgtccagaatttgtgcagctcttgatgctgctgtaggatctttgtttccataggtatctgttttatcatagcattcagatggaaggtgcttccaaaagatattcactcccactccaaactcttcagaaattacattatggaaccataaagcaggaatgaataatacatcaccagcttcaagggaacattcatatcttctagccttggaaaaaagtggatatttagccaagtctgggttatctatattcagtacttctgatttagtaccttttaaatataaatactgggcatctcgaggactgaagagtacaacacgcttttttcctgtcacttgtattaacaaattatccattacatcataatgagtccatagttgtaatcctggtgaactaattcgaaaaacactggaaaagaactgttcctctttgaagaattctggaaacttaatatctcctttcaacaaaggaaactgctttctgatatctgcaacatcctttctagggtcttctccaagtgaccgtaagtagtatttctcatcctctgaaacaaagaattctttatgtttctcttcagctgccctctggaccaactggtcaaaaggtaaagttctgtgggtagaggtgctgcatgaactgctcccgagaaacgccctccagccggggtaccgggaggtgctgcccggccatggttgctcacgcctgccctct

SEQ ID NO: 11908 - RNA, 4101 nt, Homo sapiens
  source 1..4101: mol_type = other RNA
ctgaatagctgggactacaggtgtggaccaccactccccagctctgcatataatatttttttttttttttttttttttgagacagggtctcactctgtcacccaggctggagtgcagttgcacaattccagctcactgcaacctgcacctcccaggctcaagtgatcctcctatcttagcctcctgagtagctgggactacaggcgcacaccaccacagccagctaattctctgtatttttggtagagacaaggtttcgccatgttgcccaggctggtctcgaactcctgagttcagatgatccacccacctcggtgcatatagtatttttaaaatgtattttgaaaggataatgtgaacaaaagtccaaataatacaaaactagattctaagcagcccacctagttgaacctcttcttggaggcataattatcactggtttctcgtgcatccttagagataattatatgcatatgcaaataagatgttcacacaccacataccttgttttacacaaatggcagtacagtttcaaatatgtttttcatgtaacatttaatttttctatttttagtagagacggggttttaccatgttggccagaatggtcttgatctgacctcgtgatctgcccacctcggcctcccaaagtgctgggattacaggcatgagccatggcacctgacccaccattacttttattttgaatcttgtctgtgtagcaagcagtgcagtgagaaattttgttggcagaggaaaaaaattcctttttgcatcaggtcaagcccccaaactagccaaagaaaagctgtgtaatctattcagaagtactggagatgtgctgcacattagggagaatggagaattactggtcacaacgaatcccggtttctatcacccatagctatgtgaacccagacaatcattaagcaatctgggttggttagatggcttctaagatctctttcaataaaaaagttctaagattcagaattcctgagaagttgcagctaacatacactgtataagattttatacattaaaaacaaacatctcatttggtcttaacccagtaggaagaaaagattaaaatattttgtatttgaaataaacagaccctaatattaattatgaccagggaaataattttaaaacatcccaaaggaaagttctctaacttttaaaatattataaattaatactgcaacaggagctacctcaaatctctcaacaaagatggaatataattaaatagaagaactagcaccagttatcaactatgtgcctgcccttgaactctctgcatttttgtagttctgttttaaagatgaggaaaataagcttcatagataaatgttattttgtctaaggtcatccagtttgcttctccattaaacaatcaattaagatgactattcagtgcacaaactgtaatctgttttattaatacttccaagttttctacatgactctggatttatactttgtatcaattctcttgctggttaagaaaaaaaacaagatttattaaaaactgaccataaataatgtgtaaactaaggagagttttgtctttttccttactgaaggacaaggaatcagtaaagaagttctttgctttgcttaatgaagatcaaaacctggtaattaaatttggctaatataatcattccttttctgacaagacttttttcacctttattcacctgagtaacttacctgtttccaaagacacctaggaaattcagaatgttatatatgcttttccttatttactataatttataggacatgagtggatggattctcttcaatagagaaaatgattttctctaattaaaatgcaccaaattgatgtactaagagattgctttagatgaacacatttatgttcagtgaagattatgtggtcttcaatgacactgcaatataattactaggtacaaaacaaaagcagagatccacacacaatggctcactgtcttcgatgacaacacttttaggatctcatttattcattctttaagtaatttttcttttaaaaaagggataggtggaaaaaatagttgggaaatctttaactaggctaaggtttagacataggtataaattatttattttgtaacattcaaaaaccaaaaaccaccctgacatactgggtggcaagaaaagtcaagatcagattaaacatttgttttgcactaatcacaaaactaataatccaagtcactatcatcaactccagttgatctcagctctgattatgcatcagaacaccctgtgaggtctattaagttcctataccaaatcccaaacactcttgaatcagtctacaaagttgggacctaggtatctgtacattttttaaagttcctcaaaaaattctgcttctaggcaaatgtaatagatattgtgcgttgctcatgtttttcctatcagaaccatgattttaaaaaaactatcctttctgtccccatatatccctcatgtggcctccacttctactctcagctccagtggacctgactgccctaaaggttattctagaccctttgccagtgactggctcagggatggacaggtctaagttactttagagcaatgagacctaaggatatggaaagtgaattctgggaaagctttctcatactaggacagggcccctagaatccagcctgactcttccgctgcatgtaaatgaagatgcacaaggctccaactgctactggcaatcatcccatgaccacgagggtagccagccttaggatgatgccaatgttgtggttgaaaagggggtggggtgtggaggcgggttcccaaggttcttgatgacattactgaatcattggatcagaaacactgcagcacattctgtcaatagatttcatgtattgtgaatcaatatattttcttactgtttttaagtcattttaagttggacttttagtggtcagcatctgaatgttaaagagtggtcccagcacagcattctttaattataacaatctgtatcaagtagaatccacacaaacaccccttcgtacttacataatctgtaaatctgatgtatctttcctattttaacaaaatctttaatttatatcgttataccttactaaagtgttaatgtgcattgcattcacttcattatttactcagagttcttgctgtaggctttgtcttgaatgtgtaggaccattcgtcgtgcatagaagtccctatattcctctggtaactcggccagtgttttcaaggctctgtccagaatttgtgcagctcttgatgctgctgtaggatctttgtttccataggtatctgttttatcatagcattcagatggaaggtgcttccaaaagatattcactcccactccaaactcttcagaaattacattatggaaccataaagcaggaatgaataatacatcaccagcttcaagggaacattcatatcttctagccttggaaaaaagtggatatttagccaagtctgggttatctatattcagtacttctgatttagtaccttttaaatataaatactgggcatctcgaggactgaagagtacaacacgcttttttcctgtcacttgtattaacaaattatccattacatcataatgagtccatagttgtaatcctggtgaactaattcgaaaaacactggaaaagaactgttcctctttgaagaattctggaaacttaatatctcctttcaacaaaggaaactgctttctgatatctgcaacatcctttctagggtcttctccaagtgaccgtaagtagtatttctcatcctctgaaacaaagaattctttatgtttctcttcagctgccctctggaccaactggtcaaaaggtaaagtttaatgaagtccatctgtgcaactgcagcaacatgaatctttacttctttcttccctccaacttggcttaggtaatccactgtccatttgcttgtacatggccccaaatcaatcccttccaacacaagaggttttctctgtgggtagaggtgctgcatgaactgctcccgagaaacgccctccagccggggtaccgggaggtgctgcccggccatggttgctcacgcctgccctct

SEQ ID NO: 11909 - RNA, 4112 nt, Homo sapiens
  source 1..4112: mol_type = other RNA
ctgaatagctgggactacaggtgtggaccaccactccccagctctgcatataatatttttttttttttttttttttttgagacagggtctcactctgtcacccaggctggagtgcagttgcacaattccagctcactgcaacctgcacctcccaggctcaagtgatcctcctatcttagcctcctgagtagctgggactacaggcgcacaccaccacagccagctaattctctgtatttttggtagagacaaggtttcgccatgttgcccaggctggtctcgaactcctgagttcagatgatccacccacctcggtgcatatagtatttttaaaatgtattttgaaaggataatgtgaacaaaagtccaaataatacaaaactagattctaagcagcccacctagttgaacctcttcttggaggcataattatcactggtttctcgtgcatccttagagataattatatgcatatgcaaataagatgttcacacaccacataccttgttttacacaaatggcagtacagtttcaaatatgtttttcatgtaacatttaatttttctatttttagtagagacggggttttaccatgttggccagaatggtcttgatctgacctcgtgatctgcccacctcggcctcccaaagtgctgggattacaggcatgagccatggcacctgacccaccattacttttattttgaatcttgtctgtgtagcaagcagtgcagtgagaaattttgttggcagaggaaaaaaattcctttttgcatcaggtcaagcccccaaactagccaaagaaaagctgtgtaatctattcagaagtactggagatgtgctgcacattagggagaatggagaattactggtcacaacgaatcccggtttctatcacccatagctatgtgaacccagacaatcattaagcaatctgggttggttagatggcttctaagatctctttcaataaaaaagttctaagattcagaattcctgagaagttgcagctaacatacactgtataagattttatacattaaaaacaaacatctcatttggtcttaacccagtaggaagaaaagattaaaatattttgtatttgaaataaacagaccctaatattaattatgaccagggaaataattttaaaacatcccaaaggaaagttctctaacttttaaaatattataaattaatactgcaacaggagctacctcaaatctctcaacaaagatggaatataattaaatagaagaactagcaccagttatcaactatgtgcctgcccttgaactctctgcatttttgtagttctgttttaaagatgaggaaaataagcttcatagataaatgttattttgtctaaggtcatccagtttgcttctccattaaacaatcaattaagatgactattcagtgcacaaactgtaatctgttttattaatacttccaagttttctacatgactctggatttatactttgtatcaattctcttgctggttaagaaaaaaaacaagatttattaaaaactgaccataaataatgtgtaaactaaggagagttttgtctttttccttactgaaggacaaggaatcagtaaagaagttctttgctttgcttaatgaagatcaaaacctggtaattaaatttggctaatataatcattccttttctgacaagacttttttcacctttattcacctgagtaacttacctgtttccaaagacacctaggaaattcagaatgttatatatgcttttccttatttactataatttataggacatgagtggatggattctcttcaatagagaaaatgattttctctaattaaaatgcaccaaattgatgtactaagagattgctttagatgaacacatttatgttcagtgaagattatgtggtcttcaatgacactgcaatataattactaggtacaaaacaaaagcagagatccacacacaatggctcactgtcttcgatgacaacacttttaggatctcatttattcattctttaagtaatttttcttttaaaaaagggataggtggaaaaaatagttgggaaatctttaactaggctaaggtttagacataggtataaattatttattttgtaacattcaaaaaccaaaaaccaccctgacatactgggtggcaagaaaagtcaagatcagattaaacatttgttttgcactaatcacaaaactaataatccaagtcactatcatcaactccagttgatctcagctctgattatgcatcagaacaccctgtgaggtctattaagttcctataccaaatcccaaacactcttgaatcagtctacaaagttgggacctaggtatctgtacattttttaaagttcctcaaaaaattctgcttctaggcaaatgtaatagatattgtgcgttgctcatgtttttcctatcagaaccatgattttaaaaaaactatcctttctgtccccatatatccctcatgtggcctccacttctactctcagctccagtggacctgactgccctaaaggttattctagaccctttgccagtgactggctcagggatggacaggtctaagttactttagagcaatgagacctaaggatatggaaagtgaattctgggaaagctttctcatactaggacagggcccctagaatccagcctgactcttccgctgcatgtaaatgaagatgcacaaggctccaactgctactggcaatcatcccatgaccacgagggtagccagccttaggatgatgccaatgttgtggttgaaaagggggtggggtgtggaggcgggttcccaaggttcttgatgacattactgaatcattggatcagaaacactgcagcacattctgtcaatagatttcatgtattgtgaatcaatatattttcttactgtttttaagtcattttaagttggacttttagtggtcagcatctgaatgttaaagagtggtcccagcacagcattctttaattataacaatctgtatcaagtagaatccacacaaacaccccttcgtacttacataatctgtaaatctgatgtatctttcctattttaacaaaatctttaatttatatcgttataccttactaaagtgttaatgtgcattgcattcacttcattatttactcagagttcttgctgtaggctttgtcttgaatgtgtaggaccattcgtcgtgcatagaagtccctatattcctctggtaactcggccagtgttttcaaggctctgtccagaatttgtgcagctcttgatgctgctgtaggatctttgtttccataggtatctgttttatcatagcattcagatggaaggtgcttccaaaagatattcactcccactccaaactcttcagaaattacattatggaaccataaagcaggaatgaataatacatcaccagcttcaagggaacattcatatcttctagccttggaaaaaagtggatatttagccaagtctgggttatctatattcagtacttctgatttagtaccttttaaatataaatactgggcatctcgaggactgaagagtacaacacgcttttttcctgtcacttgtattaacaaattatccattacatcataatgagtccatagttgtaatcctggtgaactaattcgaaaaacactggaaaagaactgttcctctttgaagaattctggaaacttaatatctcctttcaacaaaggaaactgctttctgatatctgcaacatctaatgaagtccatctgtgcaactgcagcaacatgaatctttacttctttcttccctccaacttggcttaggtaatccactgtccatttgcttgtacatggccccaaatcaatcccttccaacacaagaggttttctctgtgggtagaggtgctgcatgaactgctcccgagaaacgccctccagccggggtaccgggaggtgctgcccggccatggttgctcacgcctgccctcttccaggtcttcggaacttcggctctaaagcgttcctcagcgccatccgcccggaaacacgagcgacagagaaaaggtccgcgaggccggcagactccagagtggctgggtccgagcgcggggcggg

SEQ ID NO: 11910 - RNA, 4738 nt, Homo sapiens
  source 1..4738: mol_type = other RNA
ctgaatagctgggactacaggtgtgggccaccacgcctggctaagttttgtatttttttttaaattgaggaggagtctcgctctgtcacccaggctggggtgcagtggcgtggccttggctcactgcaagctccgcctcccgggttcaggccattctcctgcctcagcctcccgagtagctgggactacaggtgcccgccaacatgtccggctaattttttgtatttttagtagagatggggtttcaccatgttagccaggatggtcttgatctcctgacctcatgatccgcccacctcagcctcccaaagttctgggattacaggcatgagccactgtgcccggcctaattttcgtatttttagtagagagggggtttcaccatgttggtcaggatggtctcgatctactgaccttgtgatctgcccgcctcggcctcccaaagtgctgggaatacaggtgtgagccaccatgcgcagcctgctgttactttcagtggcaaaaccacaattacttctgcacctaccttgtaggggtgttgcttaacacttattgagattgtgcatataaaggagttagcattgttcagataataaatctcggttgtcatcatcattattgtcatcatgctgatacccagtaagtgaatccatgcaatctaaatccttcatccttttctccagttctagcccagggtcccttggccagaacacatggtcaattgtaaacttgagaggatgtactgggacactttgtaggttttgtaggttgctgacatttcttaaactaactgcatttgttttctagcaatgttgcaacaaagtaccacaaatcaggccgagtgtggtggtttacacctgcaatcccagcactttgtgaagccgaggagggcagatctcttgaggccgggagtttgagaccagcctgggcaacatagtgagaccctgtctctacaaatatatatagctgattgcagtggcataggcctgtagtcccaactactcaggaggctgaggcaggaggattgcttgagcccaggagtttgaggtgaggttgcactttagctatgattgcaccactgtactccagcctgggtgacacagtagatcctgtctgtctctaaaagaaaaaaaaatttaaaaattaccatgaactaggtgacttaaacaatagaaatttgttgtcttacagttctggaggttaagagtccgagatcaaggtgttgggccaggtgcagtggcccacgcttgtaatcccagcactttgggaggctgaggtgggcagatcactggaggccaggagtttgagaccagtctggccaacatagtgaaatcccatctctactaaaaacacaaaattagctgggcgtggtggtgggtgcctgtaatcccagctacttgggaggctgaggcaggagaattgcttgaacctgggaggtggaggttgcagtgagccaaaatcatgccactgcatccagccgggatgacagagcaagactccgtctcaaaaaaaaaaaaaaaaaaaaaagatcagttgtcagcagctttgattccttggttccttctgagggctgagagggatagcctgttccacgcctctcctggcttctggtggtctgcaggcagtccctggcattccttggcttgtaggagcatcaccccaatctctgcctccatcttcatgtggcggtctccatgtgtgtgggtgcctgtgtccaaatctccccttttcataaggacgccagtcgtatcagattagggaccaacctaatgaccttactgtaatctaatgacctctgtaaacaccctatcttcaaatatggtcacattctgaggtccttggggttaggacttcaacatatcttttttattttattattattacttttgcagacagggccttgctctgtttcccaggctggagtgcagtggcaggaacatagctcatgcagcctcgacctccttggctcaagaggtcctcctgtctcagcctcccgagtaactaagatgacaggtgcacaccaccacacccaggtaattttttcttttttcatttttattttttgtagggatgagatctcactatgttgttcaggctggtcctgaactcctagcttcaaatgattctccctactcaacctcccaaagtgccagagtttacaggtgtgagccactgcgcctggcctcccacgtatctttttttgggagccacagttcaacccataacactaactttttaagtgccccgggccacctgatctgctgtggctgaccctgcgtgtagaatcatactgggttcagagtcaggcgatgaatgtcacaggaaacacatagattttggagctaggctagggtctgtgttcccaaactacgattgatggaccgtctgcatcagagtccccttgactgggggttgtggggagacaggaagcctgttgggaattgagaaagtaagccccaaccacagtcatagttacaagtggaggtctcaagaccccccaggaggctgaggcttgctggctgactaagcgaacagcacgtgagctaatctcacttgcaaatattttcaaagttcttccacaacacttaggaaacactggctaatacatgggctgtctgtatctacctatctatctatctatctatctacctacctcctctatctctatctatccatccatctatctatcatctatctgttgatcgattgatcaatcgatcgactgacctacctacctatctcatctatctatctatctatctatctatctatcatctatctacttatatgatctatctatcaatcaatcatctatctgtctgtcaatagatagatctatcgatcggttgacctacctacctacctacctatctatcctatctatctatgtatctatctgtatatctatctatctatctatctatctatctatctatctatctatctatctacatatcttatctatccaccctatctacctatcttatcttatcctctctatctatctgtctgtctatctatctatctatctatctatctatctatctatctatctatctacctatgagtgacagatcttgctcagtttcccaaactgctgaagtgcagtggtgcagtcatagctcactgcaaccttgaactcctgggctcaaatgatctgcctgcctcagcctcctgattagctgagactacaggcgtataccaccatgtcttgctaaagtgattttgtgtgtgtgtgtggagatagggtctctgtatgttgcccaggctggtctcaaactcctggcctcaagtgatccttccaccttggcctcccaaaatgctgggatcacaggcttgagcttccacacctggcctttgtcaatactaaaatgagtgtagctacgtctcttgttttcaactactcttattcacatagcaatcctaaaaggctgatcctccaggagggctaatttcaggccagtttgatccttgctattctgatctttttggggaagataaatcctggggaaaatgcacacctttcctttgggtgctcatacactttgttcatctctttatgacacatttatcacgttgtactggaaggatttattccatgtctctgttcccagctagactctgaactcctccagggtaggggatgggatgcatctctgtgtccctagcagccaacagtgatcctggaacatgataaacatccaataactgttctggcctaggacaggggacggccactttgccgatgagcttccccagggctgccttcatatccttgttccgtatgctgtagataaaggggttgagcatggggatgaacaccccacacattagggcggctgccttgtccttctgggaggagctgggggatgtgggctgtaagtacacagcaaagatggtcccataggacagtgacaccacagtgaggtgtaagccacaggtggagaaggctttccacttgccccgagtagaagggatcttaaagactgtccagaaaatgcggatgtacgagagaaggatgcaggagaatgggctggtgcccacgacaatgccaaaagcaaagatcaccagctcgttggtgtgcgtgtctgagccggagagcttcagcaggggcatgaggtcacagaagaagtgggagatttcagagccggcgcagaaggtcagttgagccatgaggcaggtgtgtatgagagactggaggttggtgatcatccatgatgctcccagcagcagcccacagacaggggagcacatgagaaccaagtaacgctgtgggtggacaatggccacgaagcggtcgatggccattactgccaggagaaagctgtccatggtcccgaacaggtggaaggcatacatctgggtgaggcagcccacaaaggggatggctctgctctgagcctggatgttcgctagcatcttggggacggtggtggaggataatagggtgtcaacgagtgagaggttgaagagaaagaagtacatgggtgtgtggaggtgagagtccgtgatgatggccaggataatgagggcatttccaatgatggtgaccaggtatgtggagaggaacattgtgaagaggagggtctgatgctctggcttttctgagagtccctggaggaagaattctgagatttcggtttgcttttctggttccatgtatggtctgtgactgtgatcgctggggttagcctgatgtctatgggaaggattcatatgtgtacccccccgcccccag

SEQ ID NO: 11911 - RNA, 2839 nt, Homo sapiens
  source 1..2839: mol_type = other RNA
ctgaatagctgggactacaggtgtgtaccaccatgcccagctaattgttttccagagacaaggtctcactatgttgcccaggctggtcttgaactcctgagctcaagtgaccttcccaaagtgctgggattacaggtgtgagccctgcacctggccctggtttaataagaaccagagccacaaccctctcagagtgacccagtggagccccagttacctgcctcactctgagagtgaaattaggcagcgagaaaggaaaagccagtttttcaaccagcaggcaactttcccctctcaacagggacactggggacttatgtgccagcccaggctgaactaactactgtgtgacttactgcctcagctaaagcttgcagctcaagaaggaggatgccccttccttcgcgaaccctccgtgggtctggcaggcacccagcctctgtgcatggcctgggaaggaaccactgccctgggttagagaatgccacgtgaacacaagaaaaaggatgcggcaggagttaaccatcctccccttctgtccctccaggaggcagggaggaacatctcaggctgaatgctggccttccccaaatggcccacagggaaaggctggggaaaaggagctggattcactgcccagtacttgtctcatttcccaagactttatccaattctcagccactgagtagggtaccacctgggtcctagtgtgctagatagtttcaggcaggagcctgggagcaagggctgtgctggccctcttggcttatcagggggcttccctggtcatcctccagcagcaactgtcttagcgctgggtggccagcgtcctgggcttgtagacagggacatctttgtcccagagtgcaggctgccccttgataatgtcagctgccttctctgcgatcatgattgtgggggcgttcaggttgccgctgaccatgctaggcatgatggaggcatcgacgaccctgaggttttccaccccgaggacccttgtctgcggatccaccacggcagtgggatcggagggctggcccatcttacaggtgcacgaggggtggtaggcgctgtcggcttttgcccgcacaaaggcatctatctctttatctgactgaatgtggcttcctggctggagctctttccctcggaacggagccagggcttcctgtgcaaaaatttctctggtgagcttcacacacagacggaaatcctcaatatcagtttctgttgacaagtagttgggctggatcacagggtggtcttggggattggcacttctcagtttgagccagcccacactcgtgccccgcatgggccccacatgtacctggtaagcctcctgctgggtggggacccgcccgtggtcaatcacttgggatggcaggaaatggaactggatgtccgggtgggggaccccaggctggctgcggatgaacccacctgtttccagatgggcagtggctccctcccctgtgaatttccagagccactccagaccaatgcagaccttccgcaggggcttctgtgctgaatggagggtgatagggcgggtgcatgcctgctgaatgtagatctccaggtggtcttgcaggttctggccaaccccaggtaggtggcacaccacagggatgcccagtttcttgaggtcatcagcattcccgatgccagagagcatgagcagctgtggagagttgatggcacctccactcagaatcacctccttgctggcataagccctgtggctctggccattcttgacatactccacgcccactgcacgggtgccctcaaatagcaccctgctcacaagcgtctcggcctcggccttgaggttggtgcggctcagtgctgggtgcaggtaggcacaggccgcgctccaccgtttgccttcatggatggtcatgtccatccagccgaagccctcctgctggaagccattcatgtcctcggtgagcgggtagccggcctgctgcgtggcctccaggaatgcgcagtgcagcgggtggttggtcttgccccgggacacccgcagcgggccatcggcgccccggtaccggctggcgcccagctcgtggccctgcgccttgcggaagtagggcaggcagtgcgcgtagtcccagccgcgggcgccctggcgctgccagcgctcgtagtcctcggcgtgcccacggacgtagaccatggcattgagggatgaggagccaccccagacgcggccgcgtggccagtacagcacgcggccgtccaggccccgctgcacctctgtgtggtagcaccagttgtacctgtcgtcgcacaggttggccaccagggccgcgggcatgtggatcttccacgagagccgcttgctccccgcgagcacgtccttgggcccggcctccagcagcagcacgcgctcggcggggtcctccgtgagcctcccagccagcacgcagcccgccgagcccgcgcccaccaccacatagctgtactcgtcccggctctcagagcctgcgctggccagggcccgggcacccagggattgctgctgccccagggctccccgtgccagggctccaggccggcccaggcctcgtaggagacaccacatgcttctatctagtccaagtcctctgatccacggaggggaatgagatgactcacttctccctcacatccagaagtgacaggatacggtgcactctgtgaccggggctggcctacacactctttgtgattgtaggctgggcgcagtggctcacgcctgtaatcccagcactttgggaggccaaggcaggaggattgcttgaggccagaagttcaatatcagcctcagtaacatagcaagaccccattt

SEQ ID NO: 11912 - RNA, 3060 nt, Homo sapiens
  source 1..3060: mol_type = other RNA
ctgaatagctgggactacaggtgtgtaccaccatgcccagctaattgttttccagagacaaggtctcactatgttgcccaggctggtcttgaactcctgagctcaagtgaccttcccaaagtgctgggattacaggtgtgagccctgcacctggccctggtttaataagaaccagagccacaaccctctcagagtgacccagtggagccccagttacctgcctcactctgagagtgaaattaggcagcgagaaaggaaaagccagtttttcaaccagcaggcaactttcccctctcaacagggacactggggacttatgtgccagcccaggctgaactaactactgtgtgacttactgcctcagctaaagcttgcagctcaagaaggaggatgccccttccttcgcgaaccctccgtgggtctggcaggcacccagcctctgtgcatggcctgggaaggaaccactgccctgggttagagaatgccacgtgaacacaagaaaaaggatgcggcaggagttaaccatcctccccttctgtccctccaggaggcagggaggaacatctcaggctgaatgctggccttccccaaatggcccacagggaaaggctggggaaaaggagctggattcactgcccagtacttgtctcatttcccaagactttatccaattctcagccactgagtagggtaccacctgggtcctagtgtgctagatagtttcaggcaggagcctgggagcaagggctgtgctggccctcttggcttatcagggggcttccctggtcatcctccagcagcaactgtcttagcgctgggtggccagcgtcctgggcttgtagacagggacatctttgtcccagagtgcaggctgccccttgataatgtcagctgccttctctgcgatcatgattgtgggggcgttcaggttgccgctgaccatgctaggcatgatggaggcatcgacgaccctgaggttttccaccccgaggacccttgtctgcggatccaccacggcagtgggatcggagggctggcccatcttacaggtgcacgaggggtggtaggcgctgtcggcttttgcccgcacaaaggcatctatctctttatctgactgaatgtggcttcctggctggagctctttccctcggaacggagccagggcttcctgtgcaaaaatttctctggtgagcttcacacacagacggaaatcctcaatatcagtttctgttgacaagtagttgggctggatcacagggtggtcttggggattggcacttctcagtttgagccagcccacactcgtgccccgcatgggccccacatgtacctggtaagcctcctgctgggtggggacccgcccgtggtcaatcacttgggatggcaggaaatggaactggatgtccgggtgggggaccccaggctggctgcggatgaacccacctgtttccagatgggcagtggctccctcccctgtgaatttccagagccactccagaccaatgcagaccttccgcaggggcttctgtgctgaatggagggtgatagggcgggtgcatgcctgctgaatgtagatctccaggtggtcttgcaggttctggccaaccccaggtaggtggcacaccacagggatgcccagtttcttgaggtcatcagcattcccgatgccagagagcatgagcagctgtggagagttgatggcacctccactcagaatcacctccttgctggcataagccctgtggctctggccattcttgacatactccacgcccactgcacgggtgccctcaaatagcaccctgctcacaagcgtctcggcctcggccttgaggttggtgcggctcagtgctgggtgcaggtaggcacaggccgcgctccaccgtttgccttcatggatggtcatgtccatccagccgaagccctcctgctggaagccattcatgtcctcggtgagcgggtagccggcctgctgcgtggcctccaggaatgcgcagtgcagcgggtggttggtcttgccccgggacacccgcagcgggccatcggcgccccggtaccggctggcgcccagctcgtggccctgcgccttgcggaagtagggcaggcagtgcgcgtagtcccagccgcgggcgccctggcgctgccagcgctcgtagtcctcggcgtgcccacggacgtagaccatggcattgagggatgaggagccaccccagacgcggccgcgtggccagtacagcacgcggccgtccaggccccgctgcacctctgtgtggtagcaccagttgtacctgtcgtcgcacaggttggccaccagggccgcgggcatgtggatcttccacgagagccgcttgctccccgcgagcacgtccttgggcccggcctccagcagcagcacgcgctcggcggggtcctccgtgagcctcccagccagcacgcagcccgccgagcccgcgcccaccaccacatagctgtactcgtcccggctctcagagcctgcgctggccagggcccgggcacccagggattgctgctgccccagggctccccgtgccagggctccaggccggcccaggcctcgtaggagacaccacatgcttctatctagtccaagtcctctgatccacggaggggaatgagatgactcacttctccctcacatccagaagtgacaggatacggtgcactctgtgaccggggctggcctacacactctttgtgattgtccggggcgactcggccgagagcccgacagtcgggaccggagcgggaggagcgggtggccgcggcccggcccctgccccgcggcactttaaccggcggcgccggcgccccgcgcgctctctgcgtccggaatggggacgcagcagttccgacccggtcggccccggagccgcgaggctagctgggctccagcggaggcgcgcgaagcccgagggcgggtgcagctgatgcacctggctcactgcatgcacgtgtgcgcgggggtaggcgcgcgccgcggcggcccgtgctccgccagcgctcggacacggcccatccctccgagccccagcaggcgag

SEQ ID NO: 11913 - RNA, 2847 nt, Homo sapiens
  source 1..2847: mol_type = other RNA
ctgaatagctgggactacaggtgtgtaccaccatgcccagctaattgttttccagagacaaggtctcactatgttgcccaggctggtcttgaactcctgagctcaagtgaccttcccaaagtgctgggattacaggtgtgagccctgcacctggccctggtttaataagaaccagagccacaaccctctcagagtgacccagtggagccccagttacctgcctcactctgagagtgaaattaggcagcgagaaaggaaaagccagtttttcaaccagcaggcaactttcccctctcaacagggacactggggacttatgtgccagcccaggctgaactaactactgtgtgacttactgcctcagctaaagcttgcagctcaagaaggaggatgccccttccttcgcgaaccctccgtgggtctggcaggcacccagcctctgtgcatggcctgggaaggaaccactgccctgggttagagaatgccacgtgaacacaagaaaaaggatgcggcaggagttaaccatcctccccttctgtccctccaggaggcagggaggaacatctcaggctgaatgctggccttccccaaatggcccacagggaaaggctggggaaaaggagctggattcactgcccagtacttgtctcatttcccaagactttatccaattctcagccactgagtagggtaccacctgggtcctagtgtgctagatagtttcaggcaggagcctgggagcaagggctgtgctggccctcttggcttatcagggggcttccctggtcatcctccagcagcaactgtcttagcgctgggtggccagcgtcctgggcttgtagacagggacatctttgtcccagagtgcaggctgccccttgataatgtcagctgccttctctgcgatcatgattgtgggggcgttcaggttgccgctgaccatgctaggcatgatggaggcatcgacgaccctgaggttttccaccccgaggacccttgtctgcggatccaccacggcagtgggatcggagggctggcccatcttacaggtgcacgaggggtggtaggcgctgtcggcttttgcccgcacaaaggcatctatctctttatctgactgaatgtggcttcctggctggagctctttccctcggaacggagccagggcttcctgtgcaaaaatttctctggtgagcttcacacacagacggaaatcctcaatatcagtttctgttgacaagtagttgggctggatcacagggtggtcttggggattggcacttctcagtttgagccagcccacactcgtgccccgcatgggccccacatgtacctggtaagcctcctgctgggtggggacccgcccgtggtcaatcacttgggatggcaggaaatggaactggatgtccgggtgggggaccccaggctggctgcggatgaacccacctgtttccagatgggcagtggctccctcccctgtgaatttccagagccactccagaccaatgcagaccttccgcaggggcttctgtgctgaatggagggtgatagggcgggtgcatgcctgctgaatgtagatctccaggtggtcttgcaggttctggccaaccccaggtaggtggcacaccacagggatgcccagtttcttgaggtcatcagcattcccgatgccagagagcatgagcagctgtggagagttgatggcacctccactcagaatcacctccttgctggcataagccctgtggctctggccattcttgacatactccacgcccactgcacgggtgccctcaaatagcaccctgctcacaagcgtctcggcctcggccttgaggttggtgcggctcagtgctgggtgcaggtaggcacaggccgcgctccaccgtttgccttcatggatggtcatgtccatccagccgaagccctcctgctggaagccattcatgtcctcggtgagcgggtagccggcctgctgcgtggcctccaggaatgcgcagtgcagcgggtggttggtcttgccccgggacacccgcagcgggccatcggcgccccggtaccggctggcgcccagctcgtggccctgcgccttgcggaagtagggcaggcagtgcgcgtagtcccagccgcgggcgccctggcgctgccagcgctcgtagtcctcggcgtgcccacggacgtagaccatggcattgagggatgaggagccaccccagacgcggccgcgtggccagtacagcacgcggccgtccaggccccgctgcacctctgtgtggtagcaccagttgtacctgtcgtcgcacaggttggccaccagggccgcgggcatgtggatcttccacgagagccgcttgctccccgcgagcacgtccttgggcccggcctccagcagcagcacgcgctcggcggggtcctccgtgagcctcccagccagcacgcagcccgccgagcccgcgcccaccaccacatagctgtactcgtcccggctctcagagcctgcgctggccagggcccgggcacccagggattgctgctgccccagggctccccgtgccagggctccaggccggcccaggcctcgtaggagacaccacatgcttctatctagtccaagtcctctgatccacggaggggaatgagatgactcacttctccctcacatccagaagtgacaggatacggtgcactctgtgaccggggctggcctacacactctttgtgattgtggaatgaacgcatgttagtgaatggctgcctgctcgctcgtctcagagggactagccctctattttgccctgcagagccaaccaggtggcctttctaaaaccaaaaatggatgaccatttaagc

SEQ ID NO: 11914 - RNA, 3351 nt, Homo sapiens
  source 1..3351: mol_type = other RNA
ctgaatagctgggactacaggtgtgtaccaccatgcccagctaattgttttccagagacaaggtctcactatgttgcccaggctggtcttgaactcctgagctcaagtgaccttcccaaagtgctgggattacaggtgtgagccctgcacctggccctggtttaataagaaccagagccacaaccctctcagagtgacccagtggagccccagttacctgcctcactctgagagtgaaattaggcagcgagaaaggaaaagccagtttttcaaccagcaggcaactttcccctctcaacagggacactggggacttatgtgccagcccaggctgaactaactactgtgtgacttactgcctcagctaaagcttgcagctcaagaaggaggatgccccttccttcgcgaaccctccgtgggtctggcaggcacccagcctctgtgcatggcctgggaaggaaccactgccctgggttagagaatgccacgtgaacacaagaaaaaggatgcggcaggagttaaccatcctccccttctgtccctccaggaggcagggaggaacatctcaggctgaatgctggccttccccaaatggcccacagggaaaggctggggaaaaggagctggattcactgcccagtacttgtctcatttcccaagactttatccaattctcagccactgagtagggtaccacctgggtcctagtgtgctagatagtttcaggcaggagcctgggagcaagggctgtgctggccctcttggcttatcagggggcttccctggtcatcctccagcagcaactgtcttagcgctgggtggccagcgtcctgggcttgtagacagggacatctttgtcccagagtgcaggctgccccttgataatgtcagctgccttctctgcgatcatgattgtgggggcgttcaggttgccgctgaccatgctaggcatgatggaggcatcgacgaccctgaggttttccaccccgaggacccttgtctgcggatccaccacggcagtgggatcggagggctggcccatcttacaggtgcacgaggggtggtaggcgctgtcggcttttgcccgcacaaaggcatctatctctttatctgactgaatgtggcttcctggctggagctctttccctcggaacggagccagggcttcctgtgcaaaaatttctctggtgagcttcacacacagacggaaatcctcaatatcagtttctgttgacaagtagttgggctggatcacagggtggtcttggggattggcacttctcagtttgagccagcccacactcgtgccccgcatgggccccacatgtacctggtaagcctcctgctgggtggggacccgcccgtggtcaatcacttgggatggcaggaaatggaactggatgtccgggtgggggaccccaggctggctgcggatgaacccacctgtttccagatgggcagtggctccctcccctgtgaatttccagagccactccagaccaatgcagaccttccgcaggggcttctgtgctgaatggagggtgatagggcgggtgcatgcctgctgaatgtagatctccaggtggtcttgcaggttctggccaaccccaggtaggtggcacaccacagggatgcccagtttcttgaggtcatcagcattcccgatgccagagagcatgagcagctgtggagagttgatggcacctccactcagaatcacctccttgctggcataagccctgtggctctggccattcttgacatactccacgcccactgcacgggtgccctcaaatagcaccctgctcacaagcgtctcggcctcggccttgaggttggtgcggctcagtgctgggtgcaggtaggcacaggccgcgctccaccgtttgctaccttcatggatggtcatgtccatccagccgaagccctcctgctggaagccattcatgtcctcggtgagcgggtagccggcctgctgcgtggcctccaggaatgcgcagtgcagcgggtggttggtcttgccccgggacacccgcagcgggccatcggcgccccggtaccggctggcgcccagctcgtggccctgcgccttgcggaagtagggcaggcagtgcgcgtagtcccagccgcgggcgccctggcgctgccagcgctcgtagtcctcggcgtgcccacggacgtagaccatggcattgagggatgaggagccaccccagacgcggccgcgtggccagtacagcacgcggccgtccaggccccgctgcacctctgtgtggtagcaccagttgtacctgtcgtcgcacaggttggccaccagggccgcgggcatgtggatcttccacgagagccgcttgctccccgcgagcacgtccttgggcccggcctccagcagcagcacgcgctcggcggggtcctccgtgagcctcccagccagcacgcagcccgccgagcccgcgcccaccaccacatagctgtactcgtcccggctctcagagcctgcgctggccagggcccgggcacccagggattgctgctgccccagggctccccgtgccagggctccaggccggcccaggcctcgtaggagacaccacatgcttctatctagtccaagtcctctgatccacggaggggaatgagatgactcacttctccctcacatccagaagtgacaggatacggtgcactctgtgaccggggctggcctacacactctttgtgattgtcagaaagcctggggtcgggcagcgggcactcctaccgctctaaccccgcgtagctgaaagaattcgctccctcaaaggagtcagtgagcttcggcagtctgcgttccacccgtttcgcttcgcgcggcggggcgattgtgtaaagcgggcccgggtctcggcgtccagcccggccccaaacctccggcccccaggcctctccgggctagcggccgggcggcgctgctgcggggtggtcggggcgcctccgcggctactcacccggggcgactcggccgagagcccgacagtcgggaccggagcgggaggagcgggtggccgcggcccggcccctgccccgcggcactttaaccggcggcgccggcgccccgcgcgctctctgcgtccggaatggggacgcagcagttccgacccggtcggccccggagccgcgaggctagctgggctccagcggaggcgcgcgaagcccgagggcgggtgcagctgatgcacctggctcactgcatgcacgtgtgcgcgggggtaggcgcgcgccgcggcggcccgtgctccgccagcgctcggacacggcccatccctccgagccccagcaggcgagggcgctgcgacctgccccagcctggga

SEQ ID NO: 11915 - RNA, 3689 nt, Homo sapiens
  source 1..3689: mol_type = other RNA
ctgaatagctgggactacaggtgtgtaccaccatgcccagctaattgttttccagagacaaggtctcactatgttgcccaggctggtcttgaactcctgagctcaagtgaccttcccaaagtgctgggattacaggtgtgagccctgcacctggccctggtttaataagaaccagagccacaaccctctcagagtgacccagtggagccccagttacctgcctcactctgagagtgaaattaggcagcgagaaaggaaaagccagtttttcaaccagcaggcaactttcccctctcaacagggacactggggacttatgtgccagcccaggctgaactaactactgtgtgacttactgcctcagctaaagcttgcagctcaagaaggaggatgccccttccttcgcgaaccctccgtgggtctggcaggcacccagcctctgtgcatggcctgggaaggaaccactgccctgggttagagaatgccacgtgaacacaagaaaaaggatgcggcaggagttaaccatcctccccttctgtccctccaggaggcagggaggaacatctcaggctgaatgctggccttccccaaatggcccacagggaaaggctggggaaaaggagctggattcactgcccagtacttgtctcatttcccaagactttatccaattctcagccactgagtagggtaccacctgggtcctagtgtgctagatagtttcaggcaggagcctgggagcaagggctgtgctggccctcttggcttatcagggggcttccctggtcatcctccagcagcaactgtcttagcgctgggtggccagcgtcctgggcttgtagacagggacatctttgtcccagagtgcaggctgccccttgataatgtcagctgccttctctgcgatcatgattgtgggggcgttcaggttgccgctgaccatgctaggcatgatggaggcatcgacgaccctgaggttttccaccccgaggacccttgtctgcggatccaccacggcagtgggatcggagggctggcccatcttacaggtgcacgaggggtggtaggcgctgtcggcttttgcccgcacaaaggcatctatctctttatctgactgaatgtggcttcctggctggagctctttccctcggaacggagccagggcttcctgtgcaaaaatttctctggtgagcttcacacacagacggaaatcctcaatatcagtttctgttgacaagtagttgggctggatcacagggtggtcttggggattggcacttctcagtttgagccagcccacactcgtgccccgcatgggccccacatgtacctggtaagcctcctgctgggtggggacccgcccgtggtcaatcacttgggatggcaggaaatggaactggatgtccgggtgggggaccccaggctggctgcggatgaacccacctgtttccagatgggcagtggctccctcccctgtgaatttccagagccactccagaccaatgcagaccttccgcaggggcttctgtgctgaatggagggtgatagggcgggtgcatgcctgctgaatgtagatctccaggtggtcttgcaggttctggccaaccccaggtaggtggcacaccacagggatgcccagtttcttgaggtcatcagcattcccgatgccagagagcatgagcagctgtggagagttgatggcacctccactcagaatcacctccttgctggcataagccctgtggctctggccattcttgacatactccacgcccactgcacgggtgccctcaaatagcaccctgctcacaagcgtctcggcctcggccttgaggttggtgcggctcagtgctgggtgcaggtaggcacaggccgcgctccaccgtttgctaccttcatggatggtcatgtccatccagccgaagccctcctgctggaagccattcatgtcctcggtgagcgggtagccggcctgctgcgtggcctccaggaatgcgcagtgcagcgggtggttggtcttgccccgggacacccgcagcgggccatcggcgccccggtaccggctggcgcccagctcgtggccctgcgccttgcggaagtagggcaggcagtgcgcgtagtcccagccgcgggcgccctggcgctgccagcgctcgtagtcctcggcgtgcccacggacgtagaccatggcattgagggatgaggagccaccccagacgcggccgcgtggccagtacagcacgcggccgtccaggccccgctgcacctctgtgtggtagcaccagttgtacctgtcgtcgcacaggttggccaccagggccgcgggcatgtggatcttccacgagagccgcttgctccccgcgagcacgtccttgggcccggcctccagcagcagcacgcgctcggcggggtcctccgtgagcctcccagccagcacgcagcccgccgagcccgcgcccaccaccacatagctgtactcgtcccggctctcagagcctgcgctggccagggcccgggcacccagggattgctgctgccccagggctccccgtgccagggctccaggccggcccaggcctcgtaggagacaccacatgcttctatctagtccaagtcctctgatccacggaggggaatgagatgactcacttctccctcacatccagaagtgacaggatacggtgcactctgtgaccggggctggcctacacactctttgtgattgtcattgttcctcagcaccatgggacaaagttcacaatcttgagcttgcagacgaggctgttttcatctgggcttccgcagcaaggcgggtacttgtgtccttgaaaataattctcactgcactcatcctcactccaggagtacccatcagccagcacccatgtgtggttcacctttgcacccagcaggtatttgctgaacaggaagatgactattagagctgaaaatgttctcaagggccacagggcccaaagcaactcagagaggtggaatgaggggctcagggtggcccagtcccaggcaggggtgcggccacaacctcaactgagttccttggtcaggaaacagagcaattctctgaaaatgctacctgcaactccacacgtatgcatgccagagcccaaacccctggctgatccccagtccatgcaagccttaatcaagctggcaggtgggccaggcctggcacacaagtagggcctcagctaaaacagctgcttgacttagtacagcctctcaccagctgacaacacacccctaagttccatacccctctctaggcctccgtcttctcatctgtagaatggagctaattctgcctacaagtttaaatggccctgagttggtcaccacaaccctgtcgtttgcaaaccgagggggctgaagcagcagttccagcctctgtgactccactgttagcccagctgatttttgtgaactttcccccaaacccactgtgtctcaaaggatggtccctgggccacccacccacgaattacgggggcgtgggtggaggctcgttaaatgcagatcccgggcctgacccggacctgccgtctggatctcattttaggcggcgctagagatcccgggccagggaaacttgagaaccgcagctccaaatcgccagtgctgacggcttccgctttgggagccccaggtgttgctgtccgaactcacttggt

SEQ ID NO: 11916 - RNA, 3108 nt, Homo sapiens
  source 1..3108: mol_type = other RNA
ctgaatagctgggactacaggtgtgtaccaccatgcccagctaattgttttccagagacaaggtctcactatgttgcccaggctggtcttgaactcctgagctcaagtgaccttcccaaagtgctgggattacaggtgtgagccctgcacctggccctggtttaataagaaccagagccacaaccctctcagagtgacccagtggagccccagttacctgcctcactctgagagtgaaattaggcagcgagaaaggaaaagccagtttttcaaccagcaggcaactttcccctctcaacagggacactggggacttatgtgccagcccaggctgaactaactactgtgtgacttactgcctcagctaaagcttgcagctcaagaaggaggatgccccttccttcgcgaaccctccgtgggtctggcaggcacccagcctctgtgcatggcctgggaaggaaccactgccctgggttagagaatgccacgtgaacacaagaaaaaggatgcggcaggagttaaccatcctccccttctgtccctccaggaggcagggaggaacatctcaggctgaatgctggccttccccaaatggcccacagggaaaggctggggaaaaggagctggattcactgcccagtacttgtctcatttcccaagactttatccaattctcagccactgagtagggtaccacctgggtcctagtgtgctagatagtttcaggcaggagcctgggagcaagggctgtgctggccctcttggcttatcagggggcttccctggtcatcctccagcagcaactgtcttagcgctgggtggccagcgtcctgggcttgtagacagggacatctttgtcccagagtgcaggctgccccttgataatgtcagctgccttctctgcgatcatgattgtgggggcgttcaggttgccgctgaccatgctaggcatgatggaggcatcgacgaccctgaggttttccaccccgaggacccttgtctgcggatccaccacggcagtgggatcggagggctggcccatcttacaggtgcacgaggggtggtaggcgctgtcggcttttgcccgcacaaaggcatctatctctttatctgactgaatgtggcttcctggctggagctctttccctcggaacggagccagggcttcctgtgcaaaaatttctctggtgagcttcacacacagacggaaatcctcaatatcagtttctgttgacaagtagttgggctggatcacagggtggtcttggggattggcacttctcagtttgagccagcccacactcgtgccccgcatgggccccacatgtacctggtaagcctcctgctgggtggggacccgcccgtggtcaatcacttgggatggcaggaaatggaactggatgtccgggtgggggaccccaggctggctgcggatgaacccacctgtttccagatgggcagtggctccctcccctgtgaatttccagagccactccagaccaatgcagaccttccgcaggggcttctgtgctgaatggagggtgatagggcgggtgcatgcctgctgaatgtagatctccaggtggtcttgcaggttctggccaaccccaggtaggtggcacaccacagggatgcccagtttcttgaggtcatcagcattcccgatgccagagagcatgagcagctgtggagagttgatggcacctccactcagaatcacctccttgctggcataagccctgtggctctggccattcttgacatactccacgcccactgcacgggtgccctcaaatagcaccctgctcacaagcgtctcggcctcggccttgaggttggtgcggctcagtgctgggtgcaggtaggcacaggccgcgctccaccgtttgctaccttcatggatggtcatgtccatccagccgaagccctcctgctggaagccattcatgtcctcggtgagcgggtagccggcctgctgcgtggcctccaggaatgcgcagtgcagcgggtggttggtcttgccccgggacacccgcagcgggccatcggcgccccggtaccggctggcgcccagctcgtggccctgcgccttgcggaagtagggcaggcagtgcgcgtagtcccagccgcgggcgccctggcgctgccagcgctcgtagtcctcggcgtgcccacggacgtagaccatggcattgagggatgaggagccaccccagacgcggccgcgtggccagtacagcacgcggccgtccaggccccgctgcacctctgtgtggtagcaccagttgtacctgtcgtcgcacaggttggccaccagggccgcgggcatgtggatcttccacgagagccgcttgctccccgcgagcacgtccttgggcccggcctccagcagcagcacgcgctcggcggggtcctccgtgagcctcccagccagcacgcagcccgccgagcccgcgcccaccaccacatagctgtactcgtcccggctctcagagcctgcgctggccagggcccgggcacccagggattgctgctgccccagggctccccgtgccagggctccaggccggcccaggcctcgtaggagacaccacatgcttctatctagtccaagtcctctgatccacggaggggaatgagatgactcacttctccctcacatccagaagtgacaggatacggtgcactctgtgaccggggctggcctacacactctttgtgattgtccggggcgactcggccgagagcccgacagtcgggaccggagcgggaggagcgggtggccgcggcccggcccctgccccgcggcactttaaccggcggcgccggcgccccgcgcgctctctgcgtccggaatggggacgcagcagttccgacccggtcggccccggagccgcgaggctagctgggctccagcggaggcgcgcgaagcccgagggcgggtgcagctgatgcacctggctcactgcatgcacgtgtgcgcgggggtaggcgcgcgccgcggcggcccgtgctccgccagcgctcggacacggcccatccctccgagccccagcaggcgagggcgctgcgacctgccccagcctgggagggggccagcgggcccgc

SEQ ID NO: 11917 - RNA, 2850 nt, Homo sapiens
  source 1..2850: mol_type = other RNA
ctgaatagctgggactacaggtgtgtaccaccatgcccagctaattgttttccagagacaaggtctcactatgttgcccaggctggtcttgaactcctgagctcaagtgaccttcccaaagtgctgggattacaggtgtgagccctgcacctggccctggtttaataagaaccagagccacaaccctctcagagtgacccagtggagccccagttacctgcctcactctgagagtgaaattaggcagcgagaaaggaaaagccagtttttcaaccagcaggcaactttcccctctcaacagggacactggggacttatgtgccagcccaggctgaactaactactgtgtgacttactgcctcagctaaagcttgcagctcaagaaggaggatgccccttccttcgcgaaccctccgtgggtctggcaggcacccagcctctgtgcatggcctgggaaggaaccactgccctgggttagagaatgccacgtgaacacaagaaaaaggatgcggcaggagttaaccatcctccccttctgtccctccaggaggcagggaggaacatctcaggctgaatgctggccttccccaaatggcccacagggaaaggctggggaaaaggagctggattcactgcccagtacttgtctcatttcccaagactttatccaattctcagccactgagtagggtaccacctgggtcctagtgtgctagatagtttcaggcaggagcctgggagcaagggctgtgctggccctcttggcttatcagggggcttccctggtcatcctccagcagcaactgtcttagcgctgggtggccagcgtcctgggcttgtagacagggacatctttgtcccagagtgcaggctgccccttgataatgtcagctgccttctctgcgatcatgattgtgggggcgttcaggttgccgctgaccatgctaggcatgatggaggcatcgacgaccctgaggttttccaccccgaggacccttgtctgcggatccaccacggcagtgggatcggagggctggcccatcttacaggtgcacgaggggtggtaggcgctgtcggcttttgcccgcacaaaggcatctatctctttatctgactgaatgtggcttcctggctggagctctttccctcggaacggagccagggcttcctgtgcaaaaatttctctggtgagcttcacacacagacggaaatcctcaatatcagtttctgttgacaagtagttgggctggatcacagggtggtcttggggattggcacttctcagtttgagccagcccacactcgtgccccgcatgggccccacatgtacctggtaagcctcctgctgggtggggacccgcccgtggtcaatcacttgggatggcaggaaatggaactggatgtccgggtgggggaccccaggctggctgcggatgaacccacctgtttccagatgggcagtggctccctcccctgtgaatttccagagccactccagaccaatgcagaccttccgcaggggcttctgtgctgaatggagggtgatagggcgggtgcatgcctgctgaatgtagatctccaggtggtcttgcaggttctggccaaccccaggtaggtggcacaccacagggatgcccagtttcttgaggtcatcagcattcccgatgccagagagcatgagcagctgtggagagttgatggcacctccactcagaatcacctccttgctggcataagccctgtggctctggccattcttgacatactccacgcccactgcacgggtgccctcaaatagcaccctgctcacaagcgtctcggcctcggccttgaggttggtgcggctcagtgctgggtgcaggtaggcacaggccgcgctccaccgtttgctaccttcatggatggtcatgtccatccagccgaagccctcctgctggaagccattcatgtcctcggtgagcgggtagccggcctgctgcgtggcctccaggaatgcgcagtgcagcgggtggttggtcttgccccgggacacccgcagcgggccatcggcgccccggtaccggctggcgcccagctcgtggccctgcgccttgcggaagtagggcaggcagtgcgcgtagtcccagccgcgggcgccctggcgctgccagcgctcgtagtcctcggcgtgcccacggacgtagaccatggcattgagggatgaggagccaccccagacgcggccgcgtggccagtacagcacgcggccgtccaggccccgctgcacctctgtgtggtagcaccagttgtacctgtcgtcgcacaggttggccaccagggccgcgggcatgtggatcttccacgagagccgcttgctccccgcgagcacgtccttgggcccggcctccagcagcagcacgcgctcggcggggtcctccgtgagcctcccagccagcacgcagcccgccgagcccgcgcccaccaccacatagctgtactcgtcccggctctcagagcctgcgctggccagggcccgggcacccagggattgctgctgccccagggctccccgtgccagggctccaggccggcccaggcctcgtaggagacaccacatgcttctatctagtccaagtcctctgatccacggaggggaatgagatgactcacttctccctcacatccagaagtgacaggatacggtgcactctgtgaccggggctggcctacacactctttgtgattgtggaatgaacgcatgttagtgaatggctgcctgctcgctcgtctcagagggactagccctctattttgccctgcagagccaaccaggtggcctttctaaaaccaaaaatggatgaccatttaagc

SEQ ID NO: 11918 - RNA, 2962 nt, Homo sapiens
  source 1..2962: mol_type = other RNA
ctgaatagctgggactacaggtgtgtaccaccatgcccagctaattgttttccagagacaaggtctcactatgttgcccaggctggtcttgaactcctgagctcaagtgaccttcccaaagtgctgggattacaggtgtgagccctgcacctggccctggtttaataagaaccagagccacaaccctctcagagtgacccagtggagccccagttacctgcctcactctgagagtgaaattaggcagcgagaaaggaaaagccagtttttcaaccagcaggcaactttcccctctcaacagggacactggggacttatgtgccagcccaggctgaactaactactgtgtgacttactgcctcagctaaagcttgcagctcaagaaggaggatgccccttccttcgcgaaccctccgtgggtctggcaggcacccagcctctgtgcatggcctgggaaggaaccactgccctgggttagagaatgccacgtgaacacaagaaaaaggatgcggcaggagttaaccatcctccccttctgtccctccaggaggcagggaggaacatctcaggctgaatgctggccttccccaaatggcccacagggaaaggctggggaaaaggagctggattcactgcccagtacttgtctcatttcccaagactttatccaattctcagccactgagtagggtaccacctgggtcctagtgtgctagatagtttcaggcaggagcctgggagcaagggctgtgctggccctcttggcttatcagggggcttccctggtcatcctccagcagcaactgtcttagcgctgggtggccagcgtcctgggcttgtagacagggacatctttgtcccagagtgcaggctgccccttgataatgtcagctgccttctctgcgatcatgattgtgggggcgttcaggttgccgctgaccatgctaggcatgatggaggcatcgacgaccctgaggttttccaccccgaggacccttgtctgcggatccaccacggcagtgggatcggagggctggcccatcttacaggtgcacgaggggtggtaggcgctgtcggcttttgcccgcacaaaggcatctatctctttatctgactgaatgtggcttcctggctggagctctttccctcggaacggagccagggcttcctgtgcaaaaatttctctggtgagcttcacacacagacggaaatcctcaatatcagtttctgttgacaagtagttgggctggatcacagggtggtcttggggattggcacttctcagtttgagccagcccacactcgtgccccgcatgggccccacatgtacctgtgaatttccagagccactccagaccaatgcagaccttccgcaggggcttctgtgctgaatggagggtgatagggcgggtgcatgcctgctgaatgtagatctccaggtggtcttgcaggttctggccaaccccaggtaggtggcacaccacagggatgcccagtttcttgaggtcatcagcattcccgatgccagagagcatgagcagctgtggagagttgatggcacctccactcagaatcacctccttgctggcataagccctgtggctctggccattcttgacatactccacgcccactgcacgggtgccctcaaatagcaccctgctcacaagcgtctcggcctcggccttgaggttggtgcggctcagtgctgggtgcaggtaggcacaggccgcgctccaccgtttgccttcatggatggtcatgtccatccagccgaagccctcctgctggaagccattcatgtcctcggtgagcgggtagccggcctgctgcgtggcctccaggaatgcgcagtgcagcgggtggttggtcttgccccgggacacccgcagcgggccatcggcgccccggtaccggctggcgcccagctcgtggccctgcgccttgcggaagtagggcaggcagtgcgcgtagtcccagccgcgggcgccctggcgctgccagcgctcgtagtcctcggcgtgcccacggacgtagaccatggcattgagggatgaggagccaccccagacgcggccgcgtggccagtacagcacgcggccgtccaggccccgctgcacctctgtgtggtagcaccagttgtacctgtcgtcgcacaggttggccaccagggccgcgggcatgtggatcttccacgagagccgcttgctccccgcgagcacgtccttgggcccggcctccagcagcagcacgcgctcggcggggtcctccgtgagcctcccagccagcacgcagcccgccgagcccgcgcccaccaccacatagctgtactcgtcccggctctcagagcctgcgctggccagggcccgggcacccagggattgctgctgccccagggctccccgtgccagggctccaggccggcccaggcctcgtaggagacaccacatgcttctatctagtccaagtcctctgatccacggaggggaatgagatgactcacttctccctcacatccagaagtgacaggatacggtgcactctgtgaccggggctggcctacacactctttgtgattgtccggggcgactcggccgagagcccgacagtcgggaccggagcgggaggagcgggtggccgcggcccggcccctgccccgcggcactttaaccggcggcgccggcgccccgcgcgctctctgcgtccggaatggggacgcagcagttccgacccggtcggccccggagccgcgaggctagctgggctccagcggaggcgcgcgaagcccgagggcgggtgcagctgatgcacctggctcactgcatgcacgtgtgcgcgggggtaggcgcgcgccgcggcggcccgtgctccgccagcgctcggacacggcccatccctccgagccccagcaggcgagggcgctgcgacctgccccagcctgggagggggccagcgggcccgc

SEQ ID NO: 11919 - RNA, 2965 nt, Homo sapiens
  source 1..2965: mol_type = other RNA
ctgaatagctgggactacaggtgtgtaccaccatgcccagctaattgttttccagagacaaggtctcactatgttgcccaggctggtcttgaactcctgagctcaagtgaccttcccaaagtgctgggattacaggtgtgagccctgcacctggccctggtttaataagaaccagagccacaaccctctcagagtgacccagtggagccccagttacctgcctcactctgagagtgaaattaggcagcgagaaaggaaaagccagtttttcaaccagcaggcaactttcccctctcaacagggacactggggacttatgtgccagcccaggctgaactaactactgtgtgacttactgcctcagctaaagcttgcagctcaagaaggaggatgccccttccttcgcgaaccctccgtgggtctggcaggcacccagcctctgtgcatggcctgggaaggaaccactgccctgggttagagaatgccacgtgaacacaagaaaaaggatgcggcaggagttaaccatcctccccttctgtccctccaggaggcagggaggaacatctcaggctgaatgctggccttccccaaatggcccacagggaaaggctggggaaaaggagctggattcactgcccagtacttgtctcatttcccaagactttatccaattctcagccactgagtagggtaccacctgggtcctagtgtgctagatagtttcaggcaggagcctgggagcaagggctgtgctggccctcttggcttatcagggggcttccctggtcatcctccagcagcaactgtcttagcgctgggtggccagcgtcctgggcttgtagacagggacatctttgtcccagagtgcaggctgccccttgataatgtcagctgccttctctgcgatcatgattgtgggggcgttcaggttgccgctgaccatgctaggcatgatggaggcatcgacgaccctgaggttttccaccccgaggacccttgtctgcggatccaccacggcagtgggatcggagggctggcccatcttacaggtgcacgaggggtggtaggcgctgtcggcttttgcccgcacaaaggcatctatctctttatctgactgaatgtggcttcctggctggagctctttccctcggaacggagccagggcttcctgtgcaaaaatttctctggtgagcttcacacacagacggaaatcctcaatatcagtttctgttgacaagtagttgggctggatcacagggtggtcttggggattggcacttctcagtttgagccagcccacactcgtgccccgcatgggccccacatgtacctgtgaatttccagagccactccagaccaatgcagaccttccgcaggggcttctgtgctgaatggagggtgatagggcgggtgcatgcctgctgaatgtagatctccaggtggtcttgcaggttctggccaaccccaggtaggtggcacaccacagggatgcccagtttcttgaggtcatcagcattcccgatgccagagagcatgagcagctgtggagagttgatggcacctccactcagaatcacctccttgctggcataagccctgtggctctggccattcttgacatactccacgcccactgcacgggtgccctcaaatagcaccctgctcacaagcgtctcggcctcggccttgaggttggtgcggctcagtgctgggtgcaggtaggcacaggccgcgctccaccgtttgctaccttcatggatggtcatgtccatccagccgaagccctcctgctggaagccattcatgtcctcggtgagcgggtagccggcctgctgcgtggcctccaggaatgcgcagtgcagcgggtggttggtcttgccccgggacacccgcagcgggccatcggcgccccggtaccggctggcgcccagctcgtggccctgcgccttgcggaagtagggcaggcagtgcgcgtagtcccagccgcgggcgccctggcgctgccagcgctcgtagtcctcggcgtgcccacggacgtagaccatggcattgagggatgaggagccaccccagacgcggccgcgtggccagtacagcacgcggccgtccaggccccgctgcacctctgtgtggtagcaccagttgtacctgtcgtcgcacaggttggccaccagggccgcgggcatgtggatcttccacgagagccgcttgctccccgcgagcacgtccttgggcccggcctccagcagcagcacgcgctcggcggggtcctccgtgagcctcccagccagcacgcagcccgccgagcccgcgcccaccaccacatagctgtactcgtcccggctctcagagcctgcgctggccagggcccgggcacccagggattgctgctgccccagggctccccgtgccagggctccaggccggcccaggcctcgtaggagacaccacatgcttctatctagtccaagtcctctgatccacggaggggaatgagatgactcacttctccctcacatccagaagtgacaggatacggtgcactctgtgaccggggctggcctacacactctttgtgattgtccggggcgactcggccgagagcccgacagtcgggaccggagcgggaggagcgggtggccgcggcccggcccctgccccgcggcactttaaccggcggcgccggcgccccgcgcgctctctgcgtccggaatggggacgcagcagttccgacccggtcggccccggagccgcgaggctagctgggctccagcggaggcgcgcgaagcccgagggcgggtgcagctgatgcacctggctcactgcatgcacgtgtgcgcgggggtaggcgcgcgccgcggcggcccgtgctccgccagcgctcggacacggcccatccctccgagccccagcaggcgagggcgctgcgacctgccccagcctgggagggggccagcgggcccgc

SEQ ID NO: 11920 - RNA, 2984 nt, Homo sapiens
  source 1..2984: mol_type = other RNA
ctgaatagctgggactacaggtgtgtaccaccatgccccgctaatttctgtattttttgtagagacagggtttcaccatgttgcccaggctgtaattttaacaacatgaccacattccagtaatgacctgaaagggagaagaggtgacgttcccctgccctggcatgcatattataatcctgggtagaggaggggtgtgtagaatgcttaaatcccctcccagtaattctgatcctctgtgatcacacttctcccccatgatctgaaaagaactggtatgaaatgagatgagaagcagatcttgaatattctgtcttcggtttcaaacacaacaatcttgcttgtgcgccatcagtacgttccacccctctgacacactggtataatttgattaatttatcgtgtttattaagctccctagcttctccagttcctcatgtttggagatacattgatgttgatgaggctggagagctggaggaagcaagacagtaatctgtatcccacaccacagctggcactcccttacgcttacctaaggactctaaacatgcaaaaggcagatgtttggggttggaattgacaatatgaaaagctcagtaagaagacgcaaaagtcacagttcccatggtaaccctccttacctcacagagcacaggcccacagggtctgctggaaaggtgatctgagaggtaggacaaggccgactccttggaaccagcaagaaactctcaagcccccgcctagggactaactccccggcctgctgccgctgctgacgtccccccgccacagcaggtcggggaccacatgccgccctcctcgctgggctctcacatcagcactaccagccaggggttactccagggaaagggaagggtgctactcataaaggctgggtccctccctcaggcttctacaggagcccttctgccgaactcctgaacctcctgtgggcttcccaggctgtccgtgcagaatcacctgctcccttacagtattaactcgcgtagttctactgcatatgcacacagtattatatttaggcatttgtgcatctgtgatgcttcctagacagtgaggcccacagaggtatggactgtatcttgcccttttatccctggcctccagaacaggatctgaaggaggacctcaatttcaagatgacctcaaatgaatgaattcaagattctctcttgactcttgaatgtgttcatcaaggacttactagaagatagagaaagatacttaccaggcttgccaagagcatgaaacagagacacagaatggcaaacagaaagggcagaagaatcagtctctgacacaacctggtggggtaggatcaatgcaccaactcaaacttgggctgaacatgaaagccctgcagtggcatcatgccaaccaaccacacaagttcgtggccatgagacctgccttagcagtagcctcaaaaaatggggagatggccaggtacggtggctcacagtgataattccagcaccttgggaggctgagggaggacgatcgctgagtgcaggtgtttgaaaaccagcctgggcaacacagcaagatcccatctctacaaaaaaaataaaaaaataaaaaataaaaaaattagctaggcatgcgcctgtagtcccagctactcaggaggctgaagtggggtaattgcttgagtccaggagttggaagttacagtgagctgtgttcatgccaccgcactccagcctgagtgacagagcaaggctctgtctcttaaaaaaaaaaaaaaaaaaaaagagggatggaaatgttgcttttgttgactggagtatcagttacaagggtatataagtttgtcaaaactaactggactgcacacttaagacctgtgcatttcattgtattaaacatttgatcttgatagaaaataaatgaaaaggaggtatgacagtctgactccattttttgctctttaactgctgacagcttttttttttaagccccatccctcgctcttccccttctgccccacatctgggcaagctgataagaaagtctggatgctctcccgcttggctgcagcagaaggttcaaaccatgtaagcccctgcccacacggaaccctcgcccaaacctaaccgctaatcaccatacaatccccagaccagtctcctttctcctttctcttccctgtctttcattttcagaccagcttgagaagccggccctgctctctccagaaaaccctattatgtggtctcaacgttcaaatcaaattctgggtggagaccatcctggaaatgtggagcggccacaacaaagggcacacacagaggatttggtgccactgcaaactcagtgtctccagcaggacgcggccatcaaataaggacttggcgcagctccatcagcagaggcagagctccctggtttcacgcagggagctgagaatagccctgtactctgcactccggtttgtgtctgccctctcccagtgcccagctctgaagcacggtcttcacacctgggccccgtacttgaggggagcagagaccaactgctgtgcattcagaagcaggtatctggagagcagggaacctagagatatttccaccagggagcacatggggaagccgggactgtttcccctgatggaaggctctctctgaatttgtaaaagaaaggaaataggcttcttcattgagatcgagagctgaagcatcaagagataaaagcaggttttggaaaacataagaaagagttttctaaaatatgtctgaagatggaagaggctactctgaaggtggcagctccctgtccctgggccttcacgtagtttccactggacaactccacactccagggaggccatggaggagattcaagaactcatgatggggccgggcgcggtggctcacgcctgtaatcccagcactttgggaggccgaggcgggcggatcatgaggtcaggagatcaagaccatcttgggcaatatggtgaa

SEQ ID NO: 11921 - RNA, 2011 nt, Homo sapiens
  source 1..2011: mol_type = other RNA
ctgaatagctgggactacaggtgtgtaccaccgtgcctgactaatttccggttttttgtttttttgtttttgtagagacagggtttctccatgttgcctaggctgctactgaactcctaggatcaagcaatctgcccactttggcttcccaaagtgctgggattacaggcatgagccatcacatccggctggggaatacttttaaaaacttaaagcgagtgaagggagtctgattaaagtatgcacaataaaatataaagctgtttagaaggcttaaaggtctcggcagtaacctaatttccccactttcctaactttatactagtaattccaaaacatttcctgatgagaaacttcgatttccctgaaattttatgatcactaatagggaaggactgctgagtcacaataatcactggtggaatggggatttaattagcaacaacagtcaagtcccacccagtaagcacctgagagcttgtgagtcagttgaagacacgtatttactgagtacctgccatgtgtaaggtgctggtgatagagcccaaggaacttggttgctatgcttcaaaggagtggtggactgttttactaagtgggatatggcaggaacttgattgaaacacatactcagaagtagttcacctcattatagcttaaatatgtaacactctgggcttcaggtgattccatttcttcctcagttcagatctggtgctgtcagaagcaaagatgtagttgatggattcataagacagatcccacacctgagactgggtcaaattaaatgtttcagctgccagctggtactcttgagaaaggtgtgttgcaaaaacacccttatcatcagtacagatcacagaaggatgggcaatgctgtaccagaatccgaaatggtgctggtcataagatggaactgtctgacttttgacgtttgaggtcaaacagagttccagtggtatccgatgttgcctcacaaagtccaccagatccagggatcctccctcaccggagttgagaaatgttccatgcccgattctgtcaggaagcagatccaggagtatttgtgtttcttttttttggtttggaatagtagggtctccactgaggtcaaggccaagaactgtaccctcagtagaaaggaagaactcctcggcaagttttacagtctccttggctactaaagggccacctcttctgtcaactgctatcaaatacctaacatcaatgtccaagttttcttgtttggactgttttataccttcaagtatagattccacataagtctttttagtcattccagtagcattttctcttctgggtgtgctccttagttccaggtacttgacgccgtcatctgcaaattcttttatgacatcttttgtgaccattagaatatcttcagggctactagtaagctgatgaatagtttgaaacatctggaaacattcttccaaagttcttttctttcccttgtcaatcacagtcatctgatcgtggattttaagatctggcttctgggctattaatttcttcatggtatgagaactaatggatccattcaagtgggcatgaagttccacttttggcaattcagaatagaagtctgtcttgcaaggctgttgctcttctgcctctatcattttagcaggaaaaaaatgattcttctccactcttattcttagtatgagcaatatgatgtatttcagtcagtaaattgtatggtactgaatttccttcagattgctttacttccacacattttggtaagattagctgtatgtgtagatctgggttcagcttcaccagtgagttgtcttctcatttttctgttccttcaacctctccctctccactagctggtttccctcacaggaccaacacgcatgtgcagtatttgcttccacctcttagagatttctcaactacaaggacttaggcaaggtttcccttttgactggaaggcttgtagaaacgtgacaacccgccttccctaacactcatgtcacag

SEQ ID NO: 11922 - RNA, 2219 nt, Homo sapiens
  source 1..2219: mol_type = other RNA
ctgaatagctgggactacaggtgtgtaccaccgtgcctgactaatttccggttttttgtttttttgtttttgtagagacagggtttctccatgttgcctaggctgctactgaactcctaggatcaagcaatctgcccactttggcttcccaaagtgctgggattacaggcatgagccatcacatccggctggggaatacttttaaaaacttaaagcgagtgaagggagtctgattaaagtatgcacaataaaatataaagctgtttagaaggcttaaaggtctcggcagtaacctaatttccccactttcctaactttatactagtaattccaaaacatttcctgatgagaaacttcgatttccctgaaattttatgatcactaatagggaaggactgctgagtcacaataatcactggtggaatggggatttaattagcaacaacagtcaagtcccacccagtaagcacctgagagcttgtgagtcagttgaagacacgtatttactgagtacctgccatgtgtaaggtgctggtgatagagcccaaggaacttggttgctatgcttcaaaggagtggtggactgttttactaagtgggatatggcaggaacttgattgaaacacatactcagaagtagttcacctcattatagcttaaatatgtaacactctgggcttcaggtgattccatttcttcctcagttcagatctggtgctgtcagaagcaaagatgtagttgatggattcataagacagatcccacacctgagactgggtcaaattaaatgtttcagctgccagctggtactcttgagaaaggtgtgttgcaaaaacacccttatcatcagtacagatcacagaaggatgggcaatgctgtaccagaatccgaaatggtgctggtcataagatggaactgtctgacttttgacgtttgaggtcaaacagagttccagtggtatccgatgttgcctcacaaagtccaccagatccagggatcctccctcaccggagttgagaaatgttccatgcccgattctgtcaggaagcagatccaggagtatttgtgtttcttttttttggtttggaatagtagggtctccactgaggtcaaggccaagaactgtaccctcagtagaaaggaagaactcctcggcaagttttacagtctccttggctactaaagggccacctcttctgtcaactgctatcaaatacctaacatcaatgtccaagttttcttgtttggactgttttataccttcaagtatagattccacataagtctttttagtcattccagtagcattttctcttctgggtgtgctccttagttccaggtacttgacgccgtcatctgcaaattcttttatgacatcttttgtgaccattagaatatcttcagggctactagtaagctgatgaatagtttgaaacatctggaaacattcttccaaagttcttttctttcccttgtcaatcacagtcatctgatcgtggattttaagatctggcttctgggctattaatttcttcatggtatgagaactaatggatccattcaagtgggcatgaagttccacttttggcaattcagaatagaagtctgtcttgcaaggctgttgctcttctgcctctatcattttagcaggaaaaaaatgattcttctccactcttattcttagtatgagcaatatgatgtatttcagtcagtaaattgtatggtactgaatttccttcagattgctttacttccacacattttggtaagattagctgtatgtgtagatctgggttcagcttcacctttttttttttttcttttgagacaggatcttactttgttgcccaggctggagtgcagtgtcacgatcacagcttgctgcagtctcaagcttccagactcaagcgatcctcccacttcagcctccagtgagttgtcttctcatttttctgttccttcaacctctccctctccactagctggtttccctcacaggaccaacacgcatgtgcagtatttgcttccacctcttagagatttctcaactacaaggacttaggcaaggtttcccttttgactggaaggcttgtagaaacgtgacaacccgccttccctaacactcatgtcacagcggtagcggaccgtattctgggacaaatggaactcacgacattccaaagaaaggtcagccgcaagcgaacttagcactggctac

SEQ ID NO: 11923 - RNA, 2092 nt, Homo sapiens
  source 1..2092: mol_type = other RNA
ctgaatagctgggactacaggtgtgtaccaccgtgcctgactaatttccggttttttgtttttttgtttttgtagagacagggtttctccatgttgcctaggctgctactgaactcctaggatcaagcaatctgcccactttggcttcccaaagtgctgggattacaggcatgagccatcacatccggctggggaatacttttaaaaacttaaagcgagtgaagggagtctgattaaagtatgcacaataaaatataaagctgtttagaaggcttaaaggtctcggcagtaacctaatttccccactttcctaactttatactagtaattccaaaacatttcctgatgagaaacttcgatttccctgaaattttatgatcactaatagggaaggactgctgagtcacaataatcactggtggaatggggatttaattagcaacaacagtcaagtcccacccagtaagcacctgagagcttgtgagtcagttgaagacacgtatttactgagtacctgccatgtgtaaggtgctggtgatagagcccaaggaacttggttgctatgcttcaaaggagtggtggactgttttactaagtgggatatggcaggaacttgattgaaacacatactcagaagtagttcacctcattatagcttaaatatgtaacactctgggcttcaggtgattccatttcttcctcagttcagatctggtgctgtcagaagcaaagatgtagttgatggattcataagacagatcccacacctgagactgggtcaaattaaatgtttcagctgccagctggtactcttgagaaaggtgtgttgcaaaaacacccttatcatcagtacagatcacagaaggatgggcaatgctgtaccagaatccgaaatggtgctggtcataagatggaactgtctgacttttgacgtttgaggtcaaacagagttccagtggtatccgatgttgcctcacaaagtccaccagatccagggatcctccctcaccggagttgagaaatgttccatgcccgattctgtcaggaagcagatccaggagtatttgtgtttcttttttttggtttggaatctctgaaagatgcaatgctaacttcagacctgctttcttagcttctaaaagaggttccaagaagtcttttgcttgtcctacagtagggtctccactgaggtcaaggccaagaactgtaccctcagtagaaaggaagaactcctcggcaagttttacagtctccttggctactaaagggccacctcttctgtcaactgctatcaaatacctaacatcaatgtccaagttttcttgtttggactgttttataccttcaagtatagattccacataagtctttttagtcattccagtagcattttctcttctgggtgtgctccttagttccaggtacttgacgccgtcatctgcaaattcttttatgacatcttttgtgaccattagaatatcttcagggctactagtaagctgatgaatagtttgaaacatctggaaacattcttccaaagttcttttctttcccttgtcaatcacagtcatctgatcgtggattttaagatctggcttctgggctattaatttcttcatggtatgagaactaatggatccattcaagtgggcatgaagttccacttttggcaattcagaatagaagtctgtcttgcaaggctgttgctcttctgcctctatcattttagcaggaaaaaaatgattcttctccactcttattcttagtatgagcaatatgatgtatttcagtcagtaaattgtatggtactgaatttccttcagattgctttacttccacacattttggtaagattagctgtatgtgtagatctgggttcagcttcaccagtgagttgtcttctcatttttctgttccttcaacctctccctctccactagctggtttccctcacaggaccaacacgcatgtgcagtatttgcttccacctcttagagatttctcaactacaaggacttaggcaaggtttcccttttgactggaaggcttgtagaaacgtgacaacccgccttccctaacactcatgtcacag

SEQ ID NO: 11924 - RNA, 2181 nt, Homo sapiens
  source 1..2181: mol_type = other RNA
ctgaatagctgggactacaggtgtgtaccaccgtgcctgactaatttccggttttttgtttttttgtttttgtagagacagggtttctccatgttgcctaggctgctactgaactcctaggatcaagcaatctgcccactttggcttcccaaagtgctgggattacaggcatgagccatcacatccggctggggaatacttttaaaaacttaaagcgagtgaagggagtctgattaaagtatgcacaataaaatataaagctgtttagaaggcttaaaggtctcggcagtaacctaatttccccactttcctaactttatactagtaattccaaaacatttcctgatgagaaacttcgatttccctgaaattttatgatcactaatagggaaggactgctgagtcacaataatcactggtggaatggggatttaattagcaacaacagtcaagtcccacccagtaagcacctgagagcttgtgagtcagttgaagacacgtatttactgagtacctgccatgtgtaaggtgctggtgatagagcccaaggaacttggttgctatgcttcaaaggagtggtggactgttttactaagtgggatatggcaggaacttgattgaaacacatactcagaagtagttcacctcattatagcttaaatatgtaacactctgggcttcaggtgattccatttcttcctcagttcagatctggtgctgtcagaagcaaagatgtagttgatggattcataagacagatcccacacctgagactgggtcaaattaaatgtttcagctgccagctggtactcttgagaaaggtgtgttgcaaaaacacccttatcatcagtacagatcacagaaggatgggcaatgctgtaccagaatccgaaatggtgctggtcataagatggaactgtctgacttttgacgtttgaggtcaaacagagttccagtggtatccgatgttgcctcacaaagtccaccagatccagggatcctccctcaccggagttgagaaatgttccatgcccgattctgtcaggaagcagatccaggagtatttgtgtttcttttttttggtttggaatctctgaaagatgcaatgctaacttcagacctgctttcttagcttctaaaagaggttccaagaagtcttttgcttgtcctacagtagggtctccactgaggtcaaggccaagaactgtaccctcagtagaaaggaagaactcctcggcaagttttacagtctccttggctactaaagggccacctcttctgtcaactgctatcaaatacctaacatcaatgtccaagttttcttgtttggactgttttataccttcaagtatagattccacataagtctttttagtcattccagtagcattttctcttctgggtgtgctccttagttccaggtacttgacgccgtcatctgcaaattcttttatgacatcttttgtgaccattagaatatcttcagggctactagtaagctgatgaatagtttgaaacatctggaaacattcttccaaagttcttttctttcccttgtcaatcacagtcatctgatcgtggattttaagatctggcttctgggctattaatttcttcatggtatgagaactaatggatccattcaagtgggcatgaagttccacttttggcaattcagaatagaagtctgtcttgcaaggctgttgctcttctgcctctatcattttagcaggaaaaaaatgattcttctccactcttattcttagtatgagcaatatgatgtatttcagtcagtaaattgtatggtactgaatttccttcagattgctttacttccacacattttggtaagattagctgtatgtgtagatctgggttcagcttcacctttttttttttttcttttgagacaggatcttactttgttgcccaggctggagtgcagtgtcacgatcacagcttgctgcagtctcaagcttccagactcaagcgatcctcccacttcagcctccagtgagttgtcttctcatttttctgttccttcaacctctccctctccactagctggtttccctcacaggaccaacacgcatgtgcagtatttgcttccaccgaggtccgtgaggtgtgtgctaaccaaggggcggctcacaaccgtgacagactgccattcctgagtct

SEQ ID NO: 11925 - RNA, 2300 nt, Homo sapiens
  source 1..2300: mol_type = other RNA
ctgaatagctgggactacaggtgtgtaccaccgtgcctgactaatttccggttttttgtttttttgtttttgtagagacagggtttctccatgttgcctaggctgctactgaactcctaggatcaagcaatctgcccactttggcttcccaaagtgctgggattacaggcatgagccatcacatccggctggggaatacttttaaaaacttaaagcgagtgaagggagtctgattaaagtatgcacaataaaatataaagctgtttagaaggcttaaaggtctcggcagtaacctaatttccccactttcctaactttatactagtaattccaaaacatttcctgatgagaaacttcgatttccctgaaattttatgatcactaatagggaaggactgctgagtcacaataatcactggtggaatggggatttaattagcaacaacagtcaagtcccacccagtaagcacctgagagcttgtgagtcagttgaagacacgtatttactgagtacctgccatgtgtaaggtgctggtgatagagcccaaggaacttggttgctatgcttcaaaggagtggtggactgttttactaagtgggatatggcaggaacttgattgaaacacatactcagaagtagttcacctcattatagcttaaatatgtaacactctgggcttcaggtgattccatttcttcctcagttcagatctggtgctgtcagaagcaaagatgtagttgatggattcataagacagatcccacacctgagactgggtcaaattaaatgtttcagctgccagctggtactcttgagaaaggtgtgttgcaaaaacacccttatcatcagtacagatcacagaaggatgggcaatgctgtaccagaatccgaaatggtgctggtcataagatggaactgtctgacttttgacgtttgaggtcaaacagagttccagtggtatccgatgttgcctcacaaagtccaccagatccagggatcctccctcaccggagttgagaaatgttccatgcccgattctgtcaggaagcagatccaggagtatttgtgtttcttttttttggtttggaatctctgaaagatgcaatgctaacttcagacctgctttcttagcttctaaaagaggttccaagaagtcttttgcttgtcctacagtagggtctccactgaggtcaaggccaagaactgtaccctcagtagaaaggaagaactcctcggcaagttttacagtctccttggctactaaagggccacctcttctgtcaactgctatcaaatacctaacatcaatgtccaagttttcttgtttggactgttttataccttcaagtatagattccacataagtctttttagtcattccagtagcattttctcttctgggtgtgctccttagttccaggtacttgacgccgtcatctgcaaattcttttatgacatcttttgtgaccattagaatatcttcagggctactagtaagctgatgaatagtttgaaacatctggaaacattcttccaaagttcttttctttcccttgtcaatcacagtcatctgatcgtggattttaagatctggcttctgggctattaatttcttcatggtatgagaactaatggatccattcaagtgggcatgaagttccacttttggcaattcagaatagaagtctgtcttgcaaggctgttgctcttctgcctctatcattttagcaggaaaaaaatgattcttctccactcttattcttagtatgagcaatatgatgtatttcagtcagtaaattgtatggtactgaatttccttcagattgctttacttccacacattttggtaagattagctgtatgtgtagatctgggttcagcttcacctttttttttttttcttttgagacaggatcttactttgttgcccaggctggagtgcagtgtcacgatcacagcttgctgcagtctcaagcttccagactcaagcgatcctcccacttcagcctccagtgagttgtcttctcatttttctgttccttcaacctctccctctccactagctggtttccctcacaggaccaacacgcatgtgcagtatttgcttccacctcttagagatttctcaactacaaggacttaggcaaggtttcccttttgactggaaggcttgtagaaacgtgacaacccgccttccctaacactcatgtcacagcggtagcggaccgtattctgggacaaatggaactcacgacattccaaagaaaggtcagccgcaagcgaacttagcactggctac

SEQ ID NO: 11926 - RNA, 2198 nt, Homo sapiens
  source 1..2198: mol_type = other RNA
ctgaatagctgggactacaggtgtgtaccaccgtgcctgactaatttccggttttttgtttttttgtttttgtagagacagggtttctccatgttgcctaggctgctactgaactcctaggatcaagcaatctgcccactttggcttcccaaagtgctgggattacaggcatgagccatcacatccggctggggaatacttttaaaaacttaaagcgagtgaagggagtctgattaaagtatgcacaataaaatataaagctgtttagaaggcttaaaggtctcggcagtaacctaatttccccactttcctaactttatactagtaattccaaaacatttcctgatgagaaacttcgatttccctgaaattttatgatcactaatagggaaggactgctgagtcacaataatcactggtggaatggggatttaattagcaacaacagtcaagtcccacccagtaagcacctgagagcttgtgagtcagttgaagacacgtatttactgagtacctgccatgtgtaaggtgctggtgatagagcccaaggaacttggttgctatgcttcaaaggagtggtggactgttttactaagtgggatatggcaggaacttgattgaaacacatactcagaagtagttcacctcattatagcttaaatatgtaacactctgggcttcaggtgattccatttcttcctcagttcagatctggtgctgtcagaagcaaagatgtagttgatggattcataagacagatcccacacctgagactgggtcaaattaaatgtttcagctgccagctggtactcttgagaaaggtgtgttgcaaaaacacccttatcatcagtacagatcacagaaggatgggcaatgctgtaccagaatccgaaatggtgctggtcataagatggaactgtctgacttttgacgtttgaggtcaaacagagttccagtggtatccgatgttgcctcacaaagtccaccagatccagggatcctccctcaccggagttgagaaatgttccatgcccgattctgtcaggaagcagatccaggagtatttgtgtttcttttttttggtttggaatctctgaaagatgcaatgctaacttcagacctgctttcttagcttctaaaagaggttccaagaagtcttttgcttgtcctacagtagggtctccactgaggtcaaggccaagaactgtaccctcagtagaaaggaagaactcctcggcaagttttacagtctccttggctactaaagggccacctcttctgtcaactgctatcaaatacctaacatcaatgtccaagttttcttgtttggactgttttataccttcaagtatagattccacataagtctttttagtcattccagtagcattttctcttctgggtgtgctccttagttccaggtacttgacgccgtcatctgcaaattcttttatgacatcttttgtgaccattagaatatcttcagggctactagtaagctgatgaatagtttgaaacatctggaaacattcttccaaagttcttttctttcccttgtcaatcacagtcatctgatcgtggattttaagatctggcttctgggctattaatttcttcatggtatgagaactaatggatccattcaagtgggcatgaagttccacttttggcaattcagaatagaagtctgtcttgcaaggctgttgctcttctgcctctatcattttagcaggaaaaaaatgattcttctccactcttattcttagtatgagcaatatgatgtatttcagtcagtaaattgtatggtactgaatttccttcagattgctttacttccacacattttggtaagattagctgtatgtgtagatctgggttcagcttcacctttttttttttttcttttgagacaggatcttactttgttgcccaggctggagtgcagtgtcacgatcacagcttgctgcagtctcaagcttccagactcaagcgatcctcccacttcagcctccagtgagttgtcttctcatttttctgttccttcaacctctccctctccactagctggtttccctcacaggaccaacacgcatgtgcagtatttgcttccacgacattccaaagaaaggtcagccgcaagcgaacttagcactggctacaccctcctcaattctggttggcgagatgcgctcttcccg

SEQ ID NO: 11927 - RNA, 2195 nt, Homo sapiens
  source 1..2195: mol_type = other RNA
ctgaatagctgggactacaggtgtgtaccaccgtgcctgactaatttccggttttttgtttttttgtttttgtagagacagggtttctccatgttgcctaggctgctactgaactcctaggatcaagcaatctgcccactttggcttcccaaagtgctgggattacaggcatgagccatcacatccggctggggaatacttttaaaaacttaaagcgagtgaagggagtctgattaaagtatgcacaataaaatataaagctgtttagaaggcttaaaggtctcggcagtaacctaatttccccactttcctaactttatactagtaattccaaaacatttcctgatgagaaacttcgatttccctgaaattttatgatcactaatagggaaggactgctgagtcacaataatcactggtggaatggggatttaattagcaacaacagtcaagtcccacccagtaagcacctgagagcttgtgagtcagttgaagacacgtatttactgagtacctgccatgtgtaaggtgctggtgatagagcccaaggaacttggttgctatgcttcaaaggagtggtggactgttttactaagtgggatatggcaggaacttgattgaaacacatactcagaagtagttcacctcattatagcttaaatatgtaacactctgggcttcaggtgattccatttcttcctcagttcagatctggtgctgtcagaagcaaagatgtagttgatggattcataagacagatcccacacctgagactgggtcaaattaaatgtttcagctgccagctggtactcttgagaaaggtgtgttgcaaaaacacccttatcatcagtacagatcacagaaggatgggcaatgctgtaccagaatccgaaatggtgctggtcataagatggaactgtctgacttttgacgtttgaggtcaaacagagttccagtggtatccgatgttgcctcacaaagtccaccagatccagggatcctccctcaccggagttgagaaatgttccatgcccgattctgtcaggaagcagatccaggagtatttgtgtttcttttttttggtttggaatctctgaaagatgcaatgctaacttcagacctgctttcttagcttctaaaagaggttccaagaagtcttttgcttgtcctacagtagggtctccactgaggtcaaggccaagaactgtaccctcagtagaaaggaagaactcctcggcaagttttacagtctccttggctactaaagggccacctcttctgtcaactgctatcaaatacctaacatcaatgtccaagttttcttgtttggactgttttataccttcaagtatagattccacataagtctttttagtcattccagtagcattttctcttctgggtgtgctccttagttccaggtacttgacgccgtcatctgcaaattcttttatgacatcttttgtgaccattagaatatcttcagggctactagtaagctgatgaatagtttgaaacatctggaaacattcttccaaagttcttttctttcccttgtcaatcacagtcatctgatcgtggattttaagatctggcttctgggctattaatttcttcatggtatgagaactaatggatccattcaagtgggcatgaagttccacttttggcaattcagaatagaagtctgtcttgcaaggctgttgctcttctgcctctatcattttagcaggaaaaaaatgattcttctccactcttattcttagtatgagcaatatgatgtatttcagtcagtaaattgtatggtactgaatttccttcagattgctttacttccacacattttggtaagattagctgtatgtgtagatctgggttcagcttcacctttttttttttttcttttgagacaggatcttactttgttgcccaggctggagtgcagtgtcacgatcacagcttgctgcagtctcaagcttccagactcaagcgatcctcccacttcagcctcctcttagagatttctcaactacaaggacttaggcaaggtttcccttttgactggaaggcttgtagaaacgtgacaacccgccttccctaacactcatgtcacagcggtagcggaccgtattctgggacaaatggaactcacgacattccaaagaaaggtcagccgcaagcgaacttagcactgg

SEQ ID NO: 11928 - RNA, 1866 nt, Homo sapiens
  source 1..1866: mol_type = other RNA
ctgaatagctgggactacaggtgtgtaccaccgtgcctgactaatttccggttttttgtttttttgtttttgtagagacagggtttctccatgttgcctaggctgctactgaactcctaggatcaagcaatctgcccactttggcttcccaaagtgctgggattacaggcatgagccatcacatccggctggggaatacttttaaaaacttaaagcgagtgaagggagtctgattaaagtatgcacaataaaatataaagctgtttagaaggcttaaaggtctcggcagtaacctaatttccccactttcctaactttatactagtaattccaaaacatttcctgatgagaaacttcgatttccctgaaattttatgatcactaatagggaaggactgctgagtcacaataatcactggtggaatggggatttaattagcaacaacagtcaagtcccacccagtaagcacctgagagcttgtgagtcagttgaagacacgtatttactgagtacctgccatgtgtaaggtgctggtgatagagcccaaggaacttggttgctatgcttcaaaggagtggtggactgttttactaagtgggatatggcaggaacttgattgaaacacatactcagaagtagttcacctcattatagcttaaatatgtaacactctgggcttcaggtgattccatttcttcctcagttcagatctggtgctgtcagaagcaaagatgtagttgatggattcataagacagatcccacacctgagactgggtcaaattaaatgtttcagctgccagctggtactcttgagaaaggtgtgttgcaaaaacacccttatcatcagtacagatcacagaaggatgggcaatgctgtaccagaatccgaaatggtgctggtcataagatggaactgtctgacttttgacgtttgaggtcaaacagagttccagtggtatccgatgttgcctcacaaagtccaccagatccagggatcctccctcaccggagttgagaaatgttccatgcccgattctgtcaggaagcagatccaggagtatttgtgtttcttttttttggtttggaatctctgaaagatgcaatgctaacttcagacctgctttcttagcttctaaaagaggttccaagaagtcttttgcttgtcctacagtagggtctccactgaggtcaaggccaagaactgtaccctcagtagaaaggaagaactcctcggcaagttttacagtctccttggctactaaagggccacctcttctgtcaactgctatcaaatacctaacatcaatgtccaagttttcttgtttggactgttttataccttcaagtatagattccacataagtctttttagtcattccagtagcattttctcttctgggtgtgctccttagttccaggtacttgacgccgtcatctgcaaattcttttatgacatcttttgtgaccattagaatatcttcagggctactagtaagctgatgaatagtttgaaacatctggaaacattcttccaaagttcttttctttcccttgtcaatcacagtcatctgatcgtggattttaagatctggcttctgggctattaatttcttcatggtatgagaactaatggatccattcaagtgggcatgaagttccagtgagttgtcttctcatttttctgttccttcaacctctccctctccactagctggtttccctcacaggaccaacacgcatgtgcagtatttgcttccacctcttagagatttctcaactacaaggacttaggcaaggtttcccttttgactggaaggcttgtagaaacgtgacaacccgccttccctaacactcatgtcacag

SEQ ID NO: 11929 - RNA, 1910 nt, Homo sapiens
  source 1..1910: mol_type = other RNA
ctgaatagctgggactacaggtgtgtaccaccgtgcctgactaatttccggttttttgtttttttgtttttgtagagacagggtttctccatgttgcctaggctgctactgaactcctaggatcaagcaatctgcccactttggcttcccaaagtgctgggattacaggcatgagccatcacatccggctggggaatacttttaaaaacttaaagcgagtgaagggagtctgattaaagtatgcacaataaaatataaagctgtttagaaggcttaaaggtctcggcagtaacctaatttccccactttcctaactttatactagtaattccaaaacatttcctgatgagaaacttcgatttccctgaaattttatgatcactaatagggaaggactgctgagtcacaataatcactggtggaatggggatttaattagcaacaacagtcaagtcccacccagtaagcacctgagagcttgtgagtcagttgaagacacgtatttactgagtacctgccatgtgtaaggtgctggtgatagagcccaaggaacttggttgctatgcttcaaaggagtggtggactgttttactaagtgggatatggcaggaacttgattgaaacacatactcagaagtagttcacctcattatagcttaaatatgtaacactctgggcttcaggtgattccatttcttcctcagttcagatctggtgctgtcagaagcaaagatgtagttgatggattcataagacagatcccacacctgagactgggtcaaattaaatgtttcagctgccagctggtactcttgagaaaggtgtgttgcaaaaacacccttatcatcagtccagtggtatccgatgttgcctcacaaagtccaccagatccagggatcctccctcaccggagttgagaaatgttccatgcccgattctgtcaggaagcagatccaggagtatttgtgtttcttttttttggtttggaatagtagggtctccactgaggtcaaggccaagaactgtaccctcagtagaaaggaagaactcctcggcaagttttacagtctccttggctactaaagggccacctcttctgtcaactgctatcaaatacctaacatcaatgtccaagttttcttgtttggactgttttataccttcaagtatagattccacataagtctttttagtcattccagtagcattttctcttctgggtgtgctccttagttccaggtacttgacgccgtcatctgcaaattcttttatgacatcttttgtgaccattagaatatcttcagggctactagtaagctgatgaatagtttgaaacatctggaaacattcttccaaagttcttttctttcccttgtcaatcacagtcatctgatcgtggattttaagatctggcttctgggctattaatttcttcatggtatgagaactaatggatccattcaagtgggcatgaagttccacttttggcaattcagaatagaagtctgtcttgcaaggctgttgctcttctgcctctatcattttagcaggaaaaaaatgattcttctccactcttattcttagtatgagcaatatgatgtatttcagtcagtaaattgtatggtactgaatttccttcagattgctttacttccacacattttggtaagattagctgtatgtgtagatctgggttcagcttcaccagtgagttgtcttctcatttttctgttccttcaacctctccctctccactagctggtttccctcacaggaccaacacgcatgtgcagtatttgcttccacctcttagagatttctcaactacaaggacttaggcaaggtttcccttttgactggaaggcttgtagaaacgtgacaacccgccttccctaacactcatgtcacag

SEQ ID NO: 11930 - RNA, 6909 nt, Homo sapiens
  source 1..6909: mol_type = other RNA
ctgaatagctgggactacaggtgtgtactgccatgcccaacatgtcttatttctttataactgcacttcttatgtgaccccaaactcagcttaagcatccttttcattgatcaaacttggatcctaaggactatttccaaatatttaaatttattcttaaaggccaagattgactgccattgggaatattcaaaagaatgggggtactggccattcaagcagctcacacaaggagggccccacatgtttatagcacaggctgtatcaacggaataagtacatgggctcacaaggtgactgaaggacccatcatccaagaggatgtgtcagttctgatgtgttttttttaaatcatcatttcaccattatagtaatattacacaaaggcatgaagatgaaacttcaggtgtaacttttttgggggtattactttttaaagtaatggttttattcataggccgcaaatccaactttggctgcagtttttttctttttttttttttgagacggagtctcgctcttgtcacccaggttggagtgcagtggcacaatctcggctcactgcaacctccacctcctgtgtttaaacgattctcctgcttcagcctcctgagtagctggaattacaggccctgccaccacccccccgctaatttttgtctattttttttttttagtagagacggggtttcaccatgttggccagtctggtcttgaactcccgactgacctcagatgaaccacccgcctcagactcccaaagtgtcaggattacaggcgttagccaccgtacctggcctgctcccagtttttacaagatgttaattcccaataatctgagagcaatgtgttaatatgaatattaattcttctaaatgaatattcatccttatttcctacttgtataggtggatgaataaagatccaatagtataatagaaagactattagtaagaatgccggaaggtcagtctcatgcagcctggtgaaataaaacaaacaaacaaacatgaattctagagcttgtgttgtcagtaaccagctgtggggtaagtgtaagatttaatctctctattccttaagtgttcccatccacaaagtaagaaggctggatgaggtgtgtcaatcctagcacattaacctaagtcatcccccaggttgcctagacctgtcaggagcatggccttatgaagatacaaacatgaaatcctgggttggacccctctatagtttctgatcaccaaacacagtaggagcccagtgtaaaacaggttctggatatctcccacgataaacttcccatgtccctggaagagctgtaccattgtagacacactttagcttcaggcaaacaaatttctggtgtacccagaaccattttcttaaaccatttccatgggtttttatttttatctatttattttttgagatggagtcttgctctgttgcccaggctggagggcagtggcgcgatctcagcttactgcaagctccgcctcgcgggttcacgccattctcctgcctcagcctcctgtacaggcacccgccaccacgcccggctaattttttgtatttttagtagagacggggtttcacggtgttagccaggagggtctcaatctcctgaccttgtgatccgcctgcctcggcctcccaaagtgctgggatcataggcgtgagccaccgcacccggctccatgggtttttaaatacagctgtcaactctccttttcctcaagtatgaagtcacatgttaaaagaggctgtccttggctgtgtttgataaagggagttaggcacttgtttcatctgtttcttcctccaggaaataaggttaacaacacaggtggtgaaagcccagcaacctccgattgcacaaggatactgatgccatggctttgcttttcagccacaactgggaataaaactgggagctctgctgaggcaattttgctgctaaaaatgtacaaatgcctaattagagttacaggacctaccagaagatgaggacttacagtaactagccaatactacatttacttaacttctttataaactatcaaactggaaagttactcacaacttttggtctttcaaaattgttgccacctcttgctttgcttccattttgtcagcctgtgctgccagtggcttttagcttctctgggtcagttgttttacattattactccccttcctacaaaggaacgtaaagcttgccctgaaacacccagaaagggttcattctctctctccttctgttatttgcattatcatggtcaacaaatgctttcacaaaaacattccaagccacacacagccctcctcctccttagacattccttccatttcccgaggggggatgggccctggagaggtgggtgattagaccctaacaaagacagggctcatggttatccttaagaggtagaccactgcacagtttagatggccaaattaaaagtacagaatcaaattgctgtttgcagttcttatcactatgaatctaacactgaaattcacatcttcccaaagtacctcaaataacaagaataaaaatgccaagaatgaagttagtctaggctaatctttccgaagtgtaaagaagttataatcccacaattgaacacatttctcagagctttgtatgttctctttccagttcagccaagctcctggggtctagtgtttaaaatactccaattatatcatcttgtgcggactgaaatttttttccaaaagactggaaaagtgactagcgattcaaatatataaaacagtttgtaacttaaaagatagaagtgaagactaccagtacagtaggtaaagctgtgtgcatccacaatacaaaggatcagactccaagatggatggctactacataacaatgcattctgggtttctttgtgatacctggagaaaaaaaaaagcccgactgggttgcactatatttacatgtttactggcttcttcctggctagcaccactcttccccccaacccccaacatttttaagctacttattttaagtcacaggaatattcaatctaagaaaagcatcttattagagtaatataatttcttaaagaagatagcatatttacacacatctaacacatgaaaatactctattttatactaaattccaggttcaaatgaactacaatacaacattttgccttgtctgtagagtgaggattgttccaaatggggcatatgtttggctgcccctgcagtgactcactactgtcagacaagtccaaatcggtcccctagttggggaaggagcaaggtttggactgagagtttctagccagttgggttacacatccactcctttgatgagtgatccttctaggactatggtgaagtcctgaatggtctgcagaattcggataagggagttgacagtcatgcggtctcgcaggagagcgctctcttcatacattcgagtgatggcaggacactcagctaacaatggaatccactgtgggagcaggcgatcccttgttccaaggcaaactaaaatctggaatttgccatccttcccaatgttcctgggtgcagtattaatagcatttacgtagtggcagaaggttttgcaggatgatttctgaataaggacatcatcttcattatctagaatctggtcagttgtttcaaaataagcaaccactttctctatgaagtcccagatgaagacattcttgtgaaagatgcgggcagatttgaacccatggtggaaaacttgctcaagggctgcaaccaggccattttctccacacagcaacacggtgaggcttcctctctctttttcaggtttatgaaaatgtttcacaatattgttcacagcttctccaattccttcttgtatctgcccagcattgggtttgttgttttttcctgtcagtgaagtgatgctcaatctcctagccgtggtgggtgacttctgctggggtggagtccgacactgctttactagatcttcatctgatgctgatgtcatcaactctccaataagaattctctccaggctcccatcatcaatgcctttccccagccaccgcccacatgggaatctgtatgtatgtcctgtgatttcatttctgaccatgacacaatccactagccatttggctaacagtcctgagttatcgtgaccaatctgaacagtggtcagcttccccaagttctggcactcaaaggtcatttcgaggaggtttttgggaatctgcattactcctgtgtctcccagctctcctgatacacagatccaagggtttgatgtgattattgcattgctcagctttttgattgggatgatcactgacctatacggaatcatgatagtggtgaacacactggtgaagcagaaatagtccacagcattgagagaaagaaggtggtaaagaaactgctctctttcttcttcgcaacgtagaaaagcatatcgcttataaagcttcttggtgagtggttggttagaaagcaactgcttaagatgctgggacaagagcttcttttctagagacagtcttatccacgcccgagctcgtccaacatcagtcttgatctcactcatgttttgaatatgcctcatgtcctgaataagagagaccctgagcgttggcaacataactcctgagtcagattttcttctttctggtccgagggcaactggtgattctgcaaggtgctcttgtttctcttctctgtcctgaaattgaattaaatgtgaccacaaagccgacttcccctgcttgacctgcaagccatggctccatatcctctccagcaggtcacaaaggctggcgatcaaggtgttctcctccaggccggtgatgtttgcttctccatggccaagttccaccgcttcatgtcccatcttctccaccaacatgcgctttgtcttcattctacattcttttaataagccttctacgaatttacagttggtctgtgcaataactgcaggagagaggtctgacagtttgggttgcctcaggttttttcctaaacttcgtgcctcttgcatatatttcaggcagcactcagagaaggattttttaggaagtcgtgcaggaggaggtggaccctggtcccactcccagaatgccatggagttctgacagaccaaaagttccccggaaggctccctcaagtcgttgtccagcccaacatgctcagaatgctggcgaaggcgttctttcctgcgctgtgcagtggcactccgacttacccagcgattgttactggttggtcctgttgccaagacatcggactgtaactttggaaagaacccctgctcatatttgccttgaccaattttcatatcaagtagatgtgggtggattgcagtgtgatccattttcatcagtctctgctcaattgattgggctgcttcttttaaagtgctgcatttctgatatatagatgtccgcaaggtgggtgcccttacattatacagccttatcttatcaatccgagtgtcaaagacccgaagcaaaggatctttctcttcccactgagacataattttattatcaataaaggtggcaaacatctgtgtttcaatgaagcgtgaaagaaatggcaggtaaggctcaggctggtcagacagaaaggaagcctcttgaggaagttctagtttagaacggtcagttccttcttttgactgaaggcccatcagataagggacaggagcatcaagaaaatgtagcagagaagcaggtagaatgggcacataaacatgttgccattgaaatgggaacaaaagtgtggtgatgccttctgccacagtcatcaggcgttgataatcttgtgagtagagaaggatttgcatctctaaaagaacacaggtaaacacctgcaccaggttctctaatcccaggagctcaaatgcctcccgaagggggtaatcagagagggggagttcactgggcccaggcctctggcagatgacaggttcataaacaccataaaatttcagtgacctccctggaggtggaaggggtacttcataaagaatattgtggatatagctttcaagtggcaagggtggtggctgctgtgaggtaacagccttgtaaagctggataaggaatttcttgcaggcctgcatgaatggtaacggtgtgatcaagcatatactttttgaaacatacagggtgtctctgctaatatcataggagttgtatcgctggagtttcaaaagggaagttgtatctccttcatcaagactacttgccaatgagtccatactgcaggaagatgaagcatacacactgctgtaatgctcagcgttgtgcatctggtaaagtgtctgcattgctgtgcagatttgcttacttgtaacttcttcataaaaagtgagaacaaaaccataggtgcgagaaccatcttccctggtaattataaatgagtgaaactgggggtctttattgtccgtttgtgtcctgaaagatagccctttaggcatgcacaacatgttcaccgcatcttgatcaaaagggttccattctatattctgaggatagtgggcgagaactttggatttgaatgttcttctcaaaggactctggtcaaaattttcgcctgaagtcgtatttgcagcaccttggctcttgccatgacgatctgcttctagccattggtacaaaaccgccagctcgtcaggctccagcccgctgtccgcgtcgatcccgcacagcacgaagtagtgcgcgaagcggcaggcggccggggaggagcccgagcccgggccgggcgccgcgcagctcccgctcatcccggccgcgctgctccaggggccgccgccgccgccgcccgggaaggctttctgcggaggctgccaccaccgctccggctgtggtctgtgcgcccgccctagggcgacactggcgcgcccat

SEQ ID NO: 11931 - RNA, 7439 nt, Homo sapiens
  source 1..7439: mol_type = other RNA
ctgaatagctgggactacaggtgtgtactgccatgcccaacatgtcttatttctttataactgcacttcttatgtgaccccaaactcagcttaagcatccttttcattgatcaaacttggatcctaaggactatttccaaatatttaaatttattcttaaaggccaagattgactgccattgggaatattcaaaagaatgggggtactggccattcaagcagctcacacaaggagggccccacatgtttatagcacaggctgtatcaacggaataagtacatgggctcacaaggtgactgaaggacccatcatccaagaggatgtgtcagttctgatgtgttttttttaaatcatcatttcaccattatagtaatattacacaaaggcatgaagatgaaacttcaggtgtaacttttttgggggtattactttttaaagtaatggttttattcataggccgcaaatccaactttggctgcagtttttttctttttttttttttgagacggagtctcgctcttgtcacccaggttggagtgcagtggcacaatctcggctcactgcaacctccacctcctgtgtttaaacgattctcctgcttcagcctcctgagtagctggaattacaggccctgccaccacccccccgctaatttttgtctattttttttttttagtagagacggggtttcaccatgttggccagtctggtcttgaactcccgactgacctcagatgaaccacccgcctcagactcccaaagtgtcaggattacaggcgttagccaccgtacctggcctgctcccagtttttacaagatgttaattcccaataatctgagagcaatgtgttaatatgaatattaattcttctaaatgaatattcatccttatttcctacttgtataggtggatgaataaagatccaatagtataatagaaagactattagtaagaatgccggaaggtcagtctcatgcagcctggtgaaataaaacaaacaaacaaacatgaattctagagcttgtgttgtcagtaaccagctgtggggtaagtgtaagatttaatctctctattccttaagtgttcccatccacaaagtaagaaggctggatgaggtgtgtcaatcctagcacattaacctaagtcatcccccaggttgcctagacctgtcaggagcatggccttatgaagatacaaacatgaaatcctgggttggacccctctatagtttctgatcaccaaacacagtaggagcccagtgtaaaacaggttctggatatctcccacgataaacttcccatgtccctggaagagctgtaccattgtagacacactttagcttcaggcaaacaaatttctggtgtacccagaaccattttcttaaaccatttccatgggtttttatttttatctatttattttttgagatggagtcttgctctgttgcccaggctggagggcagtggcgcgatctcagcttactgcaagctccgcctcgcgggttcacgccattctcctgcctcagcctcctgtacaggcacccgccaccacgcccggctaattttttgtatttttagtagagacggggtttcacggtgttagccaggagggtctcaatctcctgaccttgtgatccgcctgcctcggcctcccaaagtgctgggatcataggcgtgagccaccgcacccggctccatgggtttttaaatacagctgtcaactctccttttcctcaagtatgaagtcacatgttaaaagaggctgtccttggctgtgtttgataaagggagttaggcacttgtttcatctgtttcttcctccaggaaataaggttaacaacacaggtggtgaaagcccagcaacctccgattgcacaaggatactgatgccatggctttgcttttcagccacaactgggaataaaactgggagctctgctgaggcaattttgctgctaaaaatgtacaaatgcctaattagagttacaggacctaccagaagatgaggacttacagtaactagccaatactacatttacttaacttctttataaactatcaaactggaaagttactcacaacttttggtctttcaaaattgttgccacctcttgctttgcttccattttgtcagcctgtgctgccagtggcttttagcttctctgggtcagttgttttacattattactccccttcctacaaaggaacgtaaagcttgccctgaaacacccagaaagggttcattctctctctccttctgttatttgcattatcatggtcaacaaatgctttcacaaaaacattccaagccacacacagccctcctcctccttagacattccttccatttcccgaggggggatgggccctggagaggtgggtgattagaccctaacaaagacagggctcatggttatccttaagaggtagaccactgcacagtttagatggccaaattaaaagtacagaatcaaattgctgtttgcagttcttatcactatgaatctaacactgaaattcacatcttcccaaagtacctcaaataacaagaataaaaatgccaagaatgaagttagtctaggctaatctttccgaagtgtaaagaagttataatcccacaattgaacacatttctcagagctttgtatgttctctttccagttcagccaagctcctggggtctagtgtttaaaatactccaattatatcatcttgtgcggactgaaatttttttccaaaagactggaaaagtgactagcgattcaaatatataaaacagtttgtaacttaaaagatagaagtgaagactaccagtacagtaggtaaagctgtgtgcatccacaatacaaaggatcagactccaagatggatggctactacataacaatgcattctgggtttctttgtgatacctggagaaaaaaaaaagcccgactgggttgcactatatttacatgtttactggcttcttcctggctagcaccactcttccccccaacccccaacatttttaagctacttattttaagtcacaggaatattcaatctaagaaaagcatcttattagagtaatataatttcttaaagaagatagcatatttacacacatctaacacatgaaaatactctattttatactaaattccaggttcaaatgaactacaatacaacattttgccttgtctgtagagtgaggattgttccaaatggggcatatgtttggctgcccctgcagtgactcactactgtcagacaagtccaaatcggtcccctagttggggaaggagcaaggtttggactgagagtttctagccagttgggttacacatccactcctttgatgagtgatccttctaggactatggtgaagtcctgaatggtctgcagaattcggataagggagttgacagtcatgcggtctcgcaggagagcgctctcttcatacattcgagtgatggcaggacactcagctaacaatggaatccactgtgggagcaggcgatcccttgttccaaggcaaactaaaatctggaatttgccatccttcccaatgttcctgggtgcagtattaatagcatttacgtagtggcagaaggttttgcaggatgatttctgaataaggacatcatcttcattatctagaatctggtcagttgtttcaaaataagcaaccactttctctatgaagtcccagatgaagacattcttgtgaaagatgcgggcagatttgaacccatggtggaaaacttgctcaagggctgcaaccaggccattttctccacacagcaacacggtgaggcttcctctctctttttcaggtttatgaaaatgtttcacaatattgttcacagcttctccaattccttcttgtatctgcccagcattgggtttgttgttttttcctgtcagtgaagtgatgctcaatctcctagccgtggtgggtgacttctgctggggtggagtccgacactgctttactagatcttcatctgatgctgatgtcatcaactctccaataagaattctctccaggctcccatcatcaatgcctttccccagccaccgcccacatgggaatctgtatgtatgtcctgtgatttcatttctgaccatgacacaatccactagccatttggctaacagtcctgagttatcgtgaccaatctgaacagtggtcagcttccccaagttctggcactcaaaggtcatttcgaggaggtttttgggaatctgcattactcctgtgtctcccagctctcctgatacacagatccaagggtttgatgtgattattgcattgctcagctttttgattgggatgatcactgacctatacggaatcatgatagtggtgaacacactggtgaagcagaaatagtccacagcattgagagaaagaaggtggtaaagaaactgctctctttcttcttcgcaacgtagaaaagcatatcgcttataaagcttcttggtgagtggttggttagaaagcaactgcttaagatgctgggacaagagcttcttttctagagacagtcttatccacgcccgagctcgtccaacatcagtcttgatctcactcatgttttgaatatgcctcatgtcctgaataagagagaccctgagcgttggcaacataactcctgagtcagattttcttctttctggtccgagggcaactggtgattctgcaaggtgctcttgtttctcttctctgtcctgaaattgaattaaatgtgaccacaaagccgacttcccctgcttgacctgcaagccatggctccatatcctctccagcaggtcacaaaggctggcgatcaaggtgttctcctccaggccggtgatgtttgcttctccatggccaagttccaccgcttcatgtcccatcttctccaccaacatgcgctttgtcttcattctacattcttttaataagccttctacgaatttacagttggtctgtgcaataactgcaggagagaggtctgacagtttgggttgcctcaggttttttcctaaacttcgtgcctcttgcatatatttcaggcagcactcagagaaggattttttaggaagtcgtgcaggaggaggtggaccctggtcccactcccagaatgccatggagttctgacagaccaaaagttccccggaaggctccctcaagtcgttgtccagcccaacatgctcagaatgctggcgaaggcgttctttcctgcgctgtgcagtggcactccgacttacccagcgattgttactggttggtcctgttgccaagacatcggactgtaactttggaaagaacccctgctcatatttgccttgaccaattttcatatcaagtagatgtgggtggattgcagtgtgatccattttcatcagtctctgctcaattgattgggctgcttcttttaaagtgctgcatttctgatatatagatgtccgcaaggtgggtgcccttacattatacagccttatcttatcaatccgagtgtcaaagacccgaagcaaaggatctttctcttcccactgagacataattttattatcaataaaggtggcaaacatctgtgtttcaatgaagcgtgaaagaaatggcaggtaaggctcaggctggtcagacagaaaggaagctttgtcaaagttctgcatctgttcccggttggtcagccaggattccatgtcctgggcagtctgaatgacaaatgcttcgtaatctgcaaacatctgtgtaaaacggttagcaaagacctctcggagctgtacattgagctggtagtcccttagttctgcctcttcacaatgcagttttaaatccttgtctttttcacccagagaagcagagaggtccattttttccacagccacaccagtacgcttggccagagcctgcaagcgggctatggtttcattgcccttcagtaactcatacatgctgatgttattagtacagacattgccgttctttttgtcattgaccaagtctttcagaaccatattcttcagtttgctggtactctcactgcaatgtaggctgccctcaggagggatcccaaattgaacaagaacctcagagagttcttggataaaatccactttattggggaactgtggaaattcttcaggcaactcaataaaatggttgtcaatgtccacaaaacacaaattagcctcttgaggaagttctagtttagaacggtcagttccttcttttgactgaaggcccatcagataagggacaggagcatcaagaaaatgtagcagagaagcaggtagaatgggcacataaacatgttgccattgaaatgggaacaaaagtgtggtgatgccttctgccacagtcatcaggcgttgataatcttgtgagtagagaaggatttgcatctctaaaagaacacaggtaaacacctgcaccaggttctctaatcccaggagctcaaatgcctcccgaagggggtaatcagagagggggagttcactgggcccaggcctctggcagatgacaggttcataaacaccataaaatttcagtgacctccctggaggtggaaggggtacttcataaagaatattgtggatatagctttcaagtggcaagggtggtggctgctgtgaggtaacagccttgtaaagctggataaggaatttcttgcaggcctgcatgaatggtaacggtgtgatcaagcatatactttttgaaacatacagggtgtctctgctaatatcataggagttgtatcgctggagtttcaaaagggaagttgtatctccttcatcaagactacttgccaatgagtccatactgcaggaagatgaagcatacacactgctgtaatgctcagcgttgtgcatctggtaaagtgtctgcattgctgtgcagatttgcttacttgtaacttcttcataaaaagtgagaacaaaaccataggtgcgagaaccatcttccctggtaattataaatgagtgaaactgggggtctttattgtccgtttgtgtcctgaaagatagccctttaggcatgcacaacatgttcaccgcatcttgatcaaaagggttccattctatattctgaggatagtgggcgagaactttggatttgaatgttcttctcaaaggactctggtcaaaattttcgcccgccagctcgtcaggctccagcccgctgtccgcgtcgatcccgcacagcacgaagtagtgcgcgaagcggcaggcggccggggaggagcccgagcccgggccgggcgccgcgcagctcccgctcatcccggccgcgctgctccaggggccgccgccgccgccgcccgggaaggctttctgcggaggctgccaccaccgctccggctgtggtctgtgcgcccgccctagggcgacactggcgcgcccatggccgcgcagccgcctctcgccgccgcagcctgcctcctcgctcggcgcgggggaagcg

SEQ ID NO: 11932 - RNA, 7446 nt, Homo sapiens
  source 1..7446: mol_type = other RNA
ctgaatagctgggactacaggtgtgtactgccatgcccaacatgtcttatttctttataactgcacttcttatgtgaccccaaactcagcttaagcatccttttcattgatcaaacttggatcctaaggactatttccaaatatttaaatttattcttaaaggccaagattgactgccattgggaatattcaaaagaatgggggtactggccattcaagcagctcacacaaggagggccccacatgtttatagcacaggctgtatcaacggaataagtacatgggctcacaaggtgactgaaggacccatcatccaagaggatgtgtcagttctgatgtgttttttttaaatcatcatttcaccattatagtaatattacacaaaggcatgaagatgaaacttcaggtgtaacttttttgggggtattactttttaaagtaatggttttattcataggccgcaaatccaactttggctgcagtttttttctttttttttttttgagacggagtctcgctcttgtcacccaggttggagtgcagtggcacaatctcggctcactgcaacctccacctcctgtgtttaaacgattctcctgcttcagcctcctgagtagctggaattacaggccctgccaccacccccccgctaatttttgtctattttttttttttagtagagacggggtttcaccatgttggccagtctggtcttgaactcccgactgacctcagatgaaccacccgcctcagactcccaaagtgtcaggattacaggcgttagccaccgtacctggcctgctcccagtttttacaagatgttaattcccaataatctgagagcaatgtgttaatatgaatattaattcttctaaatgaatattcatccttatttcctacttgtataggtggatgaataaagatccaatagtataatagaaagactattagtaagaatgccggaaggtcagtctcatgcagcctggtgaaataaaacaaacaaacaaacatgaattctagagcttgtgttgtcagtaaccagctgtggggtaagtgtaagatttaatctctctattccttaagtgttcccatccacaaagtaagaaggctggatgaggtgtgtcaatcctagcacattaacctaagtcatcccccaggttgcctagacctgtcaggagcatggccttatgaagatacaaacatgaaatcctgggttggacccctctatagtttctgatcaccaaacacagtaggagcccagtgtaaaacaggttctggatatctcccacgataaacttcccatgtccctggaagagctgtaccattgtagacacactttagcttcaggcaaacaaatttctggtgtacccagaaccattttcttaaaccatttccatgggtttttatttttatctatttattttttgagatggagtcttgctctgttgcccaggctggagggcagtggcgcgatctcagcttactgcaagctccgcctcgcgggttcacgccattctcctgcctcagcctcctgtacaggcacccgccaccacgcccggctaattttttgtatttttagtagagacggggtttcacggtgttagccaggagggtctcaatctcctgaccttgtgatccgcctgcctcggcctcccaaagtgctgggatcataggcgtgagccaccgcacccggctccatgggtttttaaatacagctgtcaactctccttttcctcaagtatgaagtcacatgttaaaagaggctgtccttggctgtgtttgataaagggagttaggcacttgtttcatctgtttcttcctccaggaaataaggttaacaacacaggtggtgaaagcccagcaacctccgattgcacaaggatactgatgccatggctttgcttttcagccacaactgggaataaaactgggagctctgctgaggcaattttgctgctaaaaatgtacaaatgcctaattagagttacaggacctaccagaagatgaggacttacagtaactagccaatactacatttacttaacttctttataaactatcaaactggaaagttactcacaacttttggtctttcaaaattgttgccacctcttgctttgcttccattttgtcagcctgtgctgccagtggcttttagcttctctgggtcagttgttttacattattactccccttcctacaaaggaacgtaaagcttgccctgaaacacccagaaagggttcattctctctctccttctgttatttgcattatcatggtcaacaaatgctttcacaaaaacattccaagccacacacagccctcctcctccttagacattccttccatttcccgaggggggatgggccctggagaggtgggtgattagaccctaacaaagacagggctcatggttatccttaagaggtagaccactgcacagtttagatggccaaattaaaagtacagaatcaaattgctgtttgcagttcttatcactatgaatctaacactgaaattcacatcttcccaaagtacctcaaataacaagaataaaaatgccaagaatgaagttagtctaggctaatctttccgaagtgtaaagaagttataatcccacaattgaacacatttctcagagctttgtatgttctctttccagttcagccaagctcctggggtctagtgtttaaaatactccaattatatcatcttgtgcggactgaaatttttttccaaaagactggaaaagtgactagcgattcaaatatataaaacagtttgtaacttaaaagatagaagtgaagactaccagtacagtaggtaaagctgtgtgcatccacaatacaaaggatcagactccaagatggatggctactacataacaatgcattctgggtttctttgtgatacctggagaaaaaaaaaagcccgactgggttgcactatatttacatgtttactggcttcttcctggctagcaccactcttccccccaacccccaacatttttaagctacttattttaagtcacaggaatattcaatctaagaaaagcatcttattagagtaatataatttcttaaagaagatagcatatttacacacatctaacacatgaaaatactctattttatactaaattccaggttcaaatgaactacaatacaacattttgccttgtctgtagagtgaggattgttccaaatggggcatatgtttggctgcccctgcagtgactcactactgtcagacaagtccaaatcggtcccctagttggggaaggagcaaggtttggactgagagtttctagccagttgggttacacatccactcctttgatgagtgatccttctaggactatggtgaagtcctgaatggtctgcagaattcggataagggagttgacagtcatgcggtctcgcaggagagcgctctcttcatacattcgagtgatggcaggacactcagctaacaatggaatccactgtgggagcaggcgatcccttgttccaaggcaaactaaaatctggaatttgccatccttcccaatgttcctgggtgcagtattaatagcatttacgtagtggcagaaggttttgcaggatgatttctgaataaggacatcatcttcattatctagaatctggtcagttgtttcaaaataagcaaccactttctctatgaagtcccagatgaagacattcttgtgaaagatgcgggcagatttgaacccatggtggaaaacttgctcaagggctgcaaccaggccattttctccacacagcaacacggtgaggcttcctctctctttttcaggtttatgaaaatgtttcacaatattgttcacagcttctccaattccttcttgtatctgcccagcattgggtttgttgttttttcctgtcagtgaagtgatgctcaatctcctagccgtggtgggtgacttctgctggggtggagtccgacactgctttactagatcttcatctgatgctgatgtcatcaactctccaataagaattctctccaggctcccatcatcaatgcctttccccagccaccgcccacatgggaatctgtatgtatgtcctgtgatttcatttctgaccatgacacaatccactagccatttggctaacagtcctgagttatcgtgaccaatctgaacagtggtcagcttccccaagttctggcactcaaaggtcatttcgaggaggtttttgggaatctgcattactcctgtgtctcccagctctcctgatacacagatccaagggtttgatgtgattattgcattgctcagctttttgattgggatgatcactgacctatacggaatcatgatagtggtgaacacactggtgaagcagaaatagtccacagcattgagagaaagaaggtggtaaagaaactgctctctttcttcttcgcaacgtagaaaagcatatcgcttataaagcttcttggtgagtggttggttagaaagcaactgcttaagatgctgggacaagagcttcttttctagagacagtcttatccacgcccgagctcgtccaacatcagtcttgatctcactcatgttttgaatatgcctcatgtcctgaataagagagaccctgagcgttggcaacataactcctgagtcagattttcttctttctggtccgagggcaactggtgattctgcaaggtgctcttgtttctcttctctgtcctgaaattgaattaaatgtgaccacaaagccgacttcccctgcttgacctgcaagccatggctccatatcctctccagcaggtcacaaaggctggcgatcaaggtgttctcctccaggccggtgatgtttgcttctccatggccaagttccaccgcttcatgtcccatcttctccaccaacatgcgctttgtcttcattctacattcttttaataagccttctacgaatttacagttggtctgtgcaataactgcaggagagaggtctgacagtttgggttgcctcaggttttttcctaaacttcgtgcctcttgcatatatttcaggcagcactcagagaaggattttttaggaagtcgtgcaggaggaggtggaccctggtcccactcccagaatgccatggagttctgacagaccaaaagttccccggaaggctccctcaagtcgttgtccagcccaacatgctcagaatgctggcgaaggcgttctttcctgcgctgtgcagtggcactccgacttacccagcgattgttactggttggtcctgttgccaagacatcggactgtaactttggaaagaacccctgctcatatttgccttgaccaattttcatatcaagtagatgtgggtggattgcagtgtgatccattttcatcagtctctgctcaattgattgggctgcttcttttaaagtgctgcatttctgatatatagatgtccgcaaggtgggtgcccttacattatacagccttatcttatcaatccgagtgtcaaagacccgaagcaaaggatctttctcttcccactgagacataattttattatcaataaaggtggcaaacatctgtgtttcaatgaagcgtgaaagaaatggcaggtaaggctcaggctggtcagacagaaaggaagctttgtcaaagttctgcatctgttcccggttggtcagccaggattccatgtcctgggcagtctgaatgacaaatgcttcgtaatctgcaaacatctgtgtaaaacggttagcaaagacctctcggagctgtacattgagctggtagtcccttagttctgcctcttcacaatgcagttttaaatccttgtctttttcacccagagaagcagagaggtccattttttccacagccacaccagtacgcttggccagagcctgcaagcgggctatggtttcattgcccttcagtaactcatacatgctgatgttattagtacagacattgccgttctttttgtcattgaccaagtctttcagaaccatattcttcagtttgctggtactctcactgcaatgtaggctgccctcaggagggatcccaaattgaacaagaacctcagagagttcttggataaaatccactttattggggaactgtggaaattcttcaggcaactcaataaaatggttgtcaatgtccacaaaacacaaattagcctcttgaggaagttctagtttagaacggtcagttccttcttttgactgaaggcccatcagataagggacaggagcatcaagaaaatgtagcagagaagcaggtagaatgggcacataaacatgttgccattgaaatgggaacaaaagtgtggtgatgccttctgccacagtcatcaggcgttgataatcttgtgagtagagaaggatttgcatctctaaaagaacacaggtaaacacctgcaccaggttctctaatcccaggagctcaaatgcctcccgaagggggtaatcagagagggggagttcactgggcccaggcctctggcagatgacaggttcataaacaccataaaatttcagtgacctccctggaggtggaaggggtacttcataaagaatattgtggatatagctttcaagtggcaagggtggtggctgctgtgaggtaacagccttgtaaagctggataaggaatttcttgcaggcctgcatgaatggtaacggtgtgatcaagcatatactttttgaaacatacagggtgtctctgctaatatcataggagttgtatcgctggagtttcaaaagggaagttgtatctccttcatcaagactacttgccaatgagtccatactgcaggaagatgaagcatacacactgctgtaatgctcagcgttgtgcatctggtaaagtgtctgcattgctgtgcagatttgcttacttgtaacttcttcataaaaagtgagaacaaaaccataggtgcgagaaccatcttccctggtaattataaatgagtgaaactgggggtctttattgtccgtttgtgtcctgaaagatagccctttaggcatgcacaacatgttcaccgcatcttgatcaaaagggttccattctatattctgaggatagtgggcgagaactttggatttgaatgttcttctcaaaggactctggtcaaaattttcgcctgaagtcgtatttgcagcaccttggctcttgccatgacgatctgcttctagccattggtacaaaaccgccagctcgtcaggctccagcccgctgtccgcgtcgatcccgcacagcacgaagtagtgcgcgaagcggcaggcggccggggaggagcccgagcccgggccgggcgccgcgcagctcccgctcatcccggccgcgctgctccaggggccgccgccgccgccgcccgggaaggctttctgcggaggctgccaccaccgctccggctgtggtctgtgcgcccgccctagggcgacactggcgcgcccat

SEQ ID NO: 11933 - RNA, 7809 nt, Homo sapiens
  source 1..7809: mol_type = other RNA
ctgaatagctgggactacaggtgtgtactgccatgcccaacatgtcttatttctttataactgcacttcttatgtgaccccaaactcagcttaagcatccttttcattgatcaaacttggatcctaaggactatttccaaatatttaaatttattcttaaaggccaagattgactgccattgggaatattcaaaagaatgggggtactggccattcaagcagctcacacaaggagggccccacatgtttatagcacaggctgtatcaacggaataagtacatgggctcacaaggtgactgaaggacccatcatccaagaggatgtgtcagttctgatgtgttttttttaaatcatcatttcaccattatagtaatattacacaaaggcatgaagatgaaacttcaggtgtaacttttttgggggtattactttttaaagtaatggttttattcataggccgcaaatccaactttggctgcagtttttttctttttttttttttgagacggagtctcgctcttgtcacccaggttggagtgcagtggcacaatctcggctcactgcaacctccacctcctgtgtttaaacgattctcctgcttcagcctcctgagtagctggaattacaggccctgccaccacccccccgctaatttttgtctattttttttttttagtagagacggggtttcaccatgttggccagtctggtcttgaactcccgactgacctcagatgaaccacccgcctcagactcccaaagtgtcaggattacaggcgttagccaccgtacctggcctgctcccagtttttacaagatgttaattcccaataatctgagagcaatgtgttaatatgaatattaattcttctaaatgaatattcatccttatttcctacttgtataggtggatgaataaagatccaatagtataatagaaagactattagtaagaatgccggaaggtcagtctcatgcagcctggtgaaataaaacaaacaaacaaacatgaattctagagcttgtgttgtcagtaaccagctgtggggtaagtgtaagatttaatctctctattccttaagtgttcccatccacaaagtaagaaggctggatgaggtgtgtcaatcctagcacattaacctaagtcatcccccaggttgcctagacctgtcaggagcatggccttatgaagatacaaacatgaaatcctgggttggacccctctatagtttctgatcaccaaacacagtaggagcccagtgtaaaacaggttctggatatctcccacgataaacttcccatgtccctggaagagctgtaccattgtagacacactttagcttcaggcaaacaaatttctggtgtacccagaaccattttcttaaaccatttccatgggtttttatttttatctatttattttttgagatggagtcttgctctgttgcccaggctggagggcagtggcgcgatctcagcttactgcaagctccgcctcgcgggttcacgccattctcctgcctcagcctcctgtacaggcacccgccaccacgcccggctaattttttgtatttttagtagagacggggtttcacggtgttagccaggagggtctcaatctcctgaccttgtgatccgcctgcctcggcctcccaaagtgctgggatcataggcgtgagccaccgcacccggctccatgggtttttaaatacagctgtcaactctccttttcctcaagtatgaagtcacatgttaaaagaggctgtccttggctgtgtttgataaagggagttaggcacttgtttcatctgtttcttcctccaggaaataaggttaacaacacaggtggtgaaagcccagcaacctccgattgcacaaggatactgatgccatggctttgcttttcagccacaactgggaataaaactgggagctctgctgaggcaattttgctgctaaaaatgtacaaatgcctaattagagttacaggacctaccagaagatgaggacttacagtaactagccaatactacatttacttaacttctttataaactatcaaactggaaagttactcacaacttttggtctttcaaaattgttgccacctcttgctttgcttccattttgtcagcctgtgctgccagtggcttttagcttctctgggtcagttgttttacattattactccccttcctacaaaggaacgtaaagcttgccctgaaacacccagaaagggttcattctctctctccttctgttatttgcattatcatggtcaacaaatgctttcacaaaaacattccaagccacacacagccctcctcctccttagacattccttccatttcccgaggggggatgggccctggagaggtgggtgattagaccctaacaaagacagggctcatggttatccttaagaggtagaccactgcacagtttagatggccaaattaaaagtacagaatcaaattgctgtttgcagttcttatcactatgaatctaacactgaaattcacatcttcccaaagtacctcaaataacaagaataaaaatgccaagaatgaagttagtctaggctaatctttccgaagtgtaaagaagttataatcccacaattgaacacatttctcagagctttgtatgttctctttccagttcagccaagctcctggggtctagtgtttaaaatactccaattatatcatcttgtgcggactgaaatttttttccaaaagactggaaaagtgactagcgattcaaatatataaaacagtttgtaacttaaaagatagaagtgaagactaccagtacagtaggtaaagctgtgtgcatccacaatacaaaggatcagactccaagatggatggctactacataacaatgcattctgggtttctttgtgatacctggagaaaaaaaaaagcccgactgggttgcactatatttacatgtttactggcttcttcctggctagcaccactcttccccccaacccccaacatttttaagctacttattttaagtcacaggaatattcaatctaagaaaagcatcttattagagtaatataatttcttaaagaagatagcatatttacacacatctaacacatgaaaatactctattttatactaaattccaggttcaaatgaactacaatacaacattttgccttgtctgtagagtgaggattgttccaaatggggcatatgtttggctgcccctgcagtgactcactactgtcagacaagtccaaatcggtcccctagttggggaaggagcaaggtttggactgagagtttctagccagttgggttacacatccactcctttgatgagtgatccttctaggactatggtgaagtcctgaatggtctgcagaattcggataagggagttgacagtcatgcggtctcgcaggagagcgctctcttcatacattcgagtgatggcaggacactcagctaacaatggaatccactgtgggagcaggcgatcccttgttccaaggcaaactaaaatctggaatttgccatccttcccaatgttcctgggtgcagtattaatagcatttacgtagtggcagaaggttttgcaggatgatttctgaataaggacatcatcttcattatctagaatctggtcagttgtttcaaaataagcaaccactttctctatgaagtcccagatgaagacattcttgtgaaagatgcgggcagatttgaacccatggtggaaaacttgctcaagggctgcaaccaggccattttctccacacagcaacacggtgaggcttcctctctctttttcaggtttatgaaaatgtttcacaatattgttcacagcttctccaattccttcttgtatctgcccagcattgggtttgttgttttttcctgtcagtgaagtgatgctcaatctcctagccgtggtgggtgacttctgctggggtggagtccgacactgctttactagatcttcatctgatgctgatgtcatcaactctccaataagaattctctccaggctcccatcatcaatgcctttccccagccaccgcccacatgggaatctgtatgtatgtcctgtgatttcatttctgaccatgacacaatccactagccatttggctaacagtcctgagttatcgtgaccaatctgaacagtggtcagcttccccaagttctggcactcaaaggtcatttcgaggaggtttttgggaatctgcattactcctgtgtctcccagctctcctgatacacagatccaagggtttgatgtgattattgcattgctcagctttttgattgggatgatcactgacctatacggaatcatgatagtggtgaacacactggtgaagcagaaatagtccacagcattgagagaaagaaggtggtaaagaaactgctctctttcttcttcgcaacgtagaaaagcatatcgcttataaagcttcttggtgagtggttggttagaaagcaactgcttaagatgctgggacaagagcttcttttctagagacagtcttatccacgcccgagctcgtccaacatcagtcttgatctcactcatgttttgaatatgcctcatgtcctgaataagagagaccctgagcgttggcaacataactcctgagtcagattttcttctttctggtccgagggcaactggtgattctgcaaggtgctcttgtttctcttctctgtcctgaaattgaattaaatgtgaccacaaagccgacttcccctgcttgacctgcaagccatggctccatatcctctccagcaggtcacaaaggctggcgatcaaggtgttctcctccaggccggtgatgtttgcttctccatggccaagttccaccgcttcatgtcccatcttctccaccaacatgcgctttgtcttcattctacattcttttaataagccttctacgaatttacagttggtctgtgcaataactgcaggagagaggtctgacagtttgggttgcctcaggttttttcctaaacttcgtgcctcttgcatatatttcaggcagcactcagagaaggattttttaggaagtcgtgcaggaggaggtggaccctggtcccactcccagaatgccatggagttctgacagaccaaaagttccccggaaggctccctcaagtcgttgtccagcccaacatgctcagaatgctggcgaaggcgttctttcctgcgctgtgcagtggcactccgacttacccagcgattgttactggttggtcctgttgccaagacatcggactgtaactttggaaagaacccctgctcatatttgccttgaccaattttcatatcaagtagatgtgggtggattgcagtgtgatccattttcatcagtctctgctcaattgattgggctgcttcttttaaagtgctgcatttctgatatatagatgtccgcaaggtgggtgcccttacattatacagccttatcttatcaatccgagtgtcaaagacccgaagcaaaggatctttctcttcccactgagacataattttattatcaataaaggtggcaaacatctgtgtttcaatgaagcgtgaaagaaatggcaggtaaggctcaggctggtcagacagaaaggaagctttgtcaaagttctgcatctgttcccggttggtcagccaggattccatgtcctgggcagtctgaatgacaaatgcttcgtaatctgcaaacatctgtgtaaaacggttagcaaagacctctcggagctgtacattgagctggtagtcccttagttctgcctcttcacaatgcagttttaaatccttgtctttttcacccagagaagcagagaggtccattttttccacagccacaccagtacgcttggccagagcctgcaagcgggctatggtttcattgcccttcagtaactcatacatgctgatgttattagtacagacattgccgttctttttgtcattgaccaagtctttcagaaccatattcttcagtttgctggtactctcactgcaatgtaggctgccctcaggagggatcccaaattgaacaagaacctcagagagttcttggataaaatccactttattggggaactgtggaaattcttcaggcaactcaataaaatggttgtcaatgtccacaaaacacaaattagcctcttgaggaagttctagtttagaacggtcagttccttcttttgactgaaggcccatcagataagggacaggagcatcaagaaaatgtagcagagaagcaggtagaatgggcacataaacatgttgccattgaaatgggaacaaaagtgtggtgatgccttctgccacagtcatcaggcgttgataatcttgtgagtagagaaggatttgcatctctaaaagaacacaggtaaacacctgcaccaggttctctaatcccaggagctcaaatgcctcccgaagggggtaatcagagagggggagttcactgggcccaggcctctggcagatgacaggttcataaacaccataaaatttcagtgacctccctggaggtggaaggggtacttcataaagaatattgtggatatagctttcaagtggcaagggtggtggctgctgtgaggtaacagccttgtaaagctggataaggaatttcttgcaggcctgcatgaatggtaacggtgtgatcaagcatatactttttgaaacatacagggtgtctctgctaatatcataggagttgtatcgctggagtttcaaaagggaagttgtatctccttcatcaagactacttgccaatgagtccatactgcaggaagatgaagcatacacactgctgtaatgctcagcgttgtgcatctggtaaagtgtctgcattgctgtgcagatttgcttacttgtaacttcttcataaaaagtgagaacaaaaccataggtgcgagaaccatcttccctggtaattataaatgagtgaaactgggggtctttattgtccgtttgtgtcctgaaagatagccctttaggcatgcacaacatgttcaccgcatcttgatcaaaagggttccattctatattctgaggatagtgggcgagaactttggatttgaatgttcttctcaaaggactctggtcaaaattttcgcctgaagtcgtatttgcagcaccttggctcttgccatgacgatctgcttctagccattggtacaaaatgaatttaaactcgggaacagtgtaggcagtgtcaacaaagcgcggtgctgggtcccgagcgtccaaaggtccctgccagctcccagacgcggccaaatccacaggattccaaaaggtgacttggccggcaccgcagagcggcaggcggcgcagagggcagagtccgaccggtccccgccccgcgctcgctccgcacggccaccggctcctccgcggacgctaccccggcgggagccgagctgagtccgactccccgtctcccgaagaggcccgaaagccgcgtcacgtgcggggccgaaacttcgcggccggggccgggtggctggcgggtgggaggcaggcacggcggtcggggggcagcccgcgcgcccggtgactcaccggccgcctccgagtgcggctgcaagcgaaggggccggcgcgccaggcggggtccgtgcccttggggccacccccgcgcctgttattaataacccagcgcctggaggcgaaagccccggtgggcgcagccgcaaagcccgcacgcggaataaataacaatgtcattaaatcgcgcccgagcgccagttcggccagaaagcggcgggagggcgccaccgggagctgacttt

SEQ ID NO: 11934 - RNA, 6682 nt, Homo sapiens
  source 1..6682: mol_type = other RNA
ctgaatagctgggactacaggtgtgtactgccatgcccaacatgtcttatttctttataactgcacttcttatgtgaccccaaactcagcttaagcatccttttcattgatcaaacttggatcctaaggactatttccaaatatttaaatttattcttaaaggccaagattgactgccattgggaatattcaaaagaatgggggtactggccattcaagcagctcacacaaggagggccccacatgtttatagcacaggctgtatcaacggaataagtacatgggctcacaaggtgactgaaggacccatcatccaagaggatgtgtcagttctgatgtgttttttttaaatcatcatttcaccattatagtaatattacacaaaggcatgaagatgaaacttcaggtgtaacttttttgggggtattactttttaaagtaatggttttattcataggccgcaaatccaactttggctgcagtttttttctttttttttttttgagacggagtctcgctcttgtcacccaggttggagtgcagtggcacaatctcggctcactgcaacctccacctcctgtgtttaaacgattctcctgcttcagcctcctgagtagctggaattacaggccctgccaccacccccccgctaatttttgtctattttttttttttagtagagacggggtttcaccatgttggccagtctggtcttgaactcccgactgacctcagatgaaccacccgcctcagactcccaaagtgtcaggattacaggcgttagccaccgtacctggcctgctcccagtttttacaagatgttaattcccaataatctgagagcaatgtgttaatatgaatattaattcttctaaatgaatattcatccttatttcctacttgtataggtggatgaataaagatccaatagtataatagaaagactattagtaagaatgccggaaggtcagtctcatgcagcctggtgaaataaaacaaacaaacaaacatgaattctagagcttgtgttgtcagtaaccagctgtggggtaagtgtaagatttaatctctctattccttaagtgttcccatccacaaagtaagaaggctggatgaggtgtgtcaatcctagcacattaacctaagtcatcccccaggttgcctagacctgtcaggagcatggccttatgaagatacaaacatgaaatcctgggttggacccctctatagtttctgatcaccaaacacagtaggagcccagtgtaaaacaggttctggatatctcccacgataaacttcccatgtccctggaagagctgtaccattgtagacacactttagcttcaggcaaacaaatttctggtgtacccagaaccattttcttaaaccatttccatgggtttttatttttatctatttattttttgagatggagtcttgctctgttgcccaggctggagggcagtggcgcgatctcagcttactgcaagctccgcctcgcgggttcacgccattctcctgcctcagcctcctgtacaggcacccgccaccacgcccggctaattttttgtatttttagtagagacggggtttcacggtgttagccaggagggtctcaatctcctgaccttgtgatccgcctgcctcggcctcccaaagtgctgggatcataggcgtgagccaccgcacccggctccatgggtttttaaatacagctgtcaactctccttttcctcaagtatgaagtcacatgttaaaagaggctgtccttggctgtgtttgataaagggagttaggcacttgtttcatctgtttcttcctccaggaaataaggttaacaacacaggtggtgaaagcccagcaacctccgattgcacaaggatactgatgccatggctttgcttttcagccacaactgggaataaaactgggagctctgctgaggcaattttgctgctaaaaatgtacaaatgcctaattagagttacaggacctaccagaagatgaggacttacagtaactagccaatactacatttacttaacttctttataaactatcaaactggaaagttactcacaacttttggtctttcaaaattgttgccacctcttgctttgcttccattttgtcagcctgtgctgccagtggcttttagcttctctgggtcagttgttttacattattactccccttcctacaaaggaacgtaaagcttgccctgaaacacccagaaagggttcattctctctctccttctgttatttgcattatcatggtcaacaaatgctttcacaaaaacattccaagccacacacagccctcctcctccttagacattccttccatttcccgaggggggatgggccctggagaggtgggtgattagaccctaacaaagacagggctcatggttatccttaagaggtagaccactgcacagtttagatggccaaattaaaagtacagaatcaaattgctgtttgcagttcttatcactatgaatctaacactgaaattcacatcttcccaaagtacctcaaataacaagaataaaaatgccaagaatgaagttagtctaggctaatctttccgaagtgtaaagaagttataatcccacaattgaacacatttctcagagctttgtatgttctctttccagttcagccaagctcctggggtctagtgtttaaaatactccaattatatcatcttgtgcggactgaaatttttttccaaaagactggaaaagtgactagcgattcaaatatataaaacagtttgtaacttaaaagatagaagtgaagactaccagtacagtaggtaaagctgtgtgcatccacaatacaaaggatcagactccaagatggatggctactacataacaatgcattctgggtttctttgtgatacctggagaaaaaaaaaagcccgactgggttgcactatatttacatgtttactggcttcttcctggctagcaccactcttccccccaacccccaacatttttaagctacttattttaagtcacaggaatattcaatctaagaaaagcatcttattagagtaatataatttcttaaagaagatagcatatttacacacatctaacacatgaaaatactctattttatactaaattccaggttcaaatgaactacaatacaacattttgccttgtctgtagagtgaggattgttccaaatggggcatatgtttggctgcccctgcagtgactcactactgtcagacaagtccaaatcggtcccctagttggggaaggagcaaggtttggactgagagtttctagccagttgggttacacatccactcctttgatgagtgatccttctaggactatggtgaagtcctgaatggtctgcagaattcggataagggagttgacagtcatgcggtctcgcaggagagcgctctcttcatacattcgagtgatggcaggacactcagctaacaatggaatccactgtgggagcaggcgatcccttgttccaaggcaaactaaaatctggaatttgccatccttcccaatgttcctgggtgcagtattaatagcatttacgtagtggcagaaggttttgcaggatgatttctgaataaggacatcatcttcattatctagaatctggtcagttgtttcaaaataagcaaccactttctctatgaagtcccagatgaagacattcttgtgaaagatgcgggcagatttgaacccatggtggaaaacttgctcaagggctgcaaccaggccattttctccacacagcaacacggtgaggcttcctctctctttttcaggtttatgaaaatgtttcacaatattgttcacagcttctccaattccttcttgtatctgcccagcattgggtttgttgttttttcctgtcagtgaagtgatgctcaatctcctagccgtggtgggtgacttctgctggggtggagtccgacactgctttactagatcttcatctgatgctgatgtcatcaactctccaataagaattctctccaggctcccatcatcaatgcctttccccagccaccgcccacatgggaatctgtatgtatgtcctgtgatttcatttctgaccatgacacaatccactagccatttggctaacagtcctgagttatcgtgaccaatctgaacagtggtcagcttccccaagttctggcactcaaaggtcatttcgaggaggtttttgggaatctgcattactcctgtgtctcccagctctcctgatacacagatccaagggtttgatgtgattattgcattgctcagctttttgattgggatgatcactgacctatacggaatcatgatagtggtgaacacactggtgaagcagaaatagtccacagcattgagagaaagaaggtggtaaagaaactgctctctttcttcttcgcaacgtagaaaagcatatcgcttataaagcttcttggtgagtggttggttagaaagcaactgcttaagatgctgggacaagagcttcttttctagagacagtcttatccacgcccgagctcgtccaacatcagtcttgatctcactcatgttttgaatatgcctcatgtcctgaataagagagaccctgagcgttggcaacataactcctgagtcagattttcttctttctggtccgagggcaactggtgattctgcaaggtgctcttgtttctcttctctgtcctgaaattgaattaaatgtgaccacaaagccgacttcccctgcttgacctgcaagccatggctccatatcctctccagcaggtcacaaaggctggcgatcaaggtgttctcctccaggccggtgatgtttgcttctccatggccaagttccaccgcttcatgtcccatcttctccaccaacatgcgctttgtcttcattctacattcttttaataagccttctacgaatttacagttggtctgtgcaataactgcaggagagaggtctgacagtttgggttgcctcaggttttttcctaaacttcgtgcctcttgcatatatttcaggcagcactcagagaaggattttttaggaagtcgtgcaggaggaggtggaccctggtcccactcccagaatgccatggagttctgacagaccaaaagttccccggaaggctccctcaagtcgttgtccagcccaacatgctcagaatgctggcgaaggcgttctttcctgcgctgtgcagtggcactccgacttacccagcgattgttactggttggtcctgttgccaagacatcggactgtaactttggaaagaacccctgctcatatttgccttgaccaattttcatatcaagtagatgtgggtggattgcagtgtgatccattttcatcagtctctgctcaattgattgggctgcttcttttaaagtgctgcatttctgatatatagatgtccgcaaggtgggtgcccttacattatacagccttatcttatcaatccgagtgtcaaagacccgaagcaaaggatctttctcttcccactgagacataattttattatcaataaaggtggcaaacatctgtgtttcaatgaagcgtgaaagaaatggcaggtaaggctcaggctggtcagacagaaaggaagctttgtcaaagttctgcatctgttcccggttggtcagccaggattccatgtcctgggcagtctgaatgacaaatgcttcgtaatctgcaaacatctgtgtaaaacggttagcaaagacctctcggagctgtacattgagctggtagtcccttagttctgcctcttcacaatgcagttttaaatccttgtctttttcacccagagaagcagagaggtccattttttccacagccacaccagtacgcttggccagagcctgcaagcgggctatggtttcattgcccttcagtaactcatacatgctgatgttattagtacagacattgccgttctttttgtcattgaccaagtctttcagaaccatattcttcagtttgctggtactctcactgcaatgtaggctgccctcaggagggatcccaaattgaacaagaacctcagagagttcttggataaaatccactttattggggaactgtggaaattcttcaggcaactcaataaaatggttgtcaatgtccacaaaacacaaattagcctcttgaggaagttctagtttagaacggtcagttccttcttttgactgaaggcccatcagataagggacaggagcatcaagaaaatgtagcagagaagcaggtagaatgggcacataaacatgttgccattgaaatgggaacaaaagtgtggtgatgccttctgccacagtcatcaggcgttgataatcttttctctcactcagatgaaatgctcccacaggcaaagatccaaagttgattgcctcaggaagctgcagagtcaacaatttcatttatcccttttcaatgttcgctgagttttgatgtgaacctttactaatccataaagaatgggaagtctacacgtttctggtagtaacagagttctctcactctcattatgatgaagaaaaaatgttttcttaatgacgattatatattatcaggaaaaaagggctatttccattaataaataaatatacccaaatcagccaagttaacacttgtgttccttcctatttctctctgcagtcact

SEQ ID NO: 11935 - RNA, 6915 nt, Homo sapiens
  source 1..6915: mol_type = other RNA
ctgaatagctgggactacaggtgtgtactgccatgcccaacatgtcttatttctttataactgcacttcttatgtgaccccaaactcagcttaagcatccttttcattgatcaaacttggatcctaaggactatttccaaatatttaaatttattcttaaaggccaagattgactgccattgggaatattcaaaagaatgggggtactggccattcaagcagctcacacaaggagggccccacatgtttatagcacaggctgtatcaacggaataagtacatgggctcacaaggtgactgaaggacccatcatccaagaggatgtgtcagttctgatgtgttttttttaaatcatcatttcaccattatagtaatattacacaaaggcatgaagatgaaacttcaggtgtaacttttttgggggtattactttttaaagtaatggttttattcataggccgcaaatccaactttggctgcagtttttttctttttttttttttgagacggagtctcgctcttgtcacccaggttggagtgcagtggcacaatctcggctcactgcaacctccacctcctgtgtttaaacgattctcctgcttcagcctcctgagtagctggaattacaggccctgccaccacccccccgctaatttttgtctattttttttttttagtagagacggggtttcaccatgttggccagtctggtcttgaactcccgactgacctcagatgaaccacccgcctcagactcccaaagtgtcaggattacaggcgttagccaccgtacctggcctgctcccagtttttacaagatgttaattcccaataatctgagagcaatgtgttaatatgaatattaattcttctaaatgaatattcatccttatttcctacttgtataggtggatgaataaagatccaatagtataatagaaagactattagtaagaatgccggaaggtcagtctcatgcagcctggtgaaataaaacaaacaaacaaacatgaattctagagcttgtgttgtcagtaaccagctgtggggtaagtgtaagatttaatctctctattccttaagtgttcccatccacaaagtaagaaggctggatgaggtgtgtcaatcctagcacattaacctaagtcatcccccaggttgcctagacctgtcaggagcatggccttatgaagatacaaacatgaaatcctgggttggacccctctatagtttctgatcaccaaacacagtaggagcccagtgtaaaacaggttctggatatctcccacgataaacttcccatgtccctggaagagctgtaccattgtagacacactttagcttcaggcaaacaaatttctggtgtacccagaaccattttcttaaaccatttccatgggtttttatttttatctatttattttttgagatggagtcttgctctgttgcccaggctggagggcagtggcgcgatctcagcttactgcaagctccgcctcgcgggttcacgccattctcctgcctcagcctcctgtacaggcacccgccaccacgcccggctaattttttgtatttttagtagagacggggtttcacggtgttagccaggagggtctcaatctcctgaccttgtgatccgcctgcctcggcctcccaaagtgctgggatcataggcgtgagccaccgcacccggctccatgggtttttaaatacagctgtcaactctccttttcctcaagtatgaagtcacatgttaaaagaggctgtccttggctgtgtttgataaagggagttaggcacttgtttcatctgtttcttcctccaggaaataaggttaacaacacaggtggtgaaagcccagcaacctccgattgcacaaggatactgatgccatggctttgcttttcagccacaactgggaataaaactgggagctctgctgaggcaattttgctgctaaaaatgtacaaatgcctaattagagttacaggacctaccagaagatgaggacttacagtaactagccaatactacatttacttaacttctttataaactatcaaactggaaagttactcacaacttttggtctttcaaaattgttgccacctcttgctttgcttccattttgtcagcctgtgctgccagtggcttttagcttctctgggtcagttgttttacattattactccccttcctacaaaggaacgtaaagcttgccctgaaacacccagaaagggttcattctctctctccttctgttatttgcattatcatggtcaacaaatgctttcacaaaaacattccaagccacacacagccctcctcctccttagacattccttccatttcccgaggggggatgggccctggagaggtgggtgattagaccctaacaaagacagggctcatggttatccttaagaggtagaccactgcacagtttagatggccaaattaaaagtacagaatcaaattgctgtttgcagttcttatcactatgaatctaacactgaaattcacatcttcccaaagtacctcaaataacaagaataaaaatgccaagaatgaagttagtctaggctaatctttccgaagtgtaaagaagttataatcccacaattgaacacatttctcagagctttgtatgttctctttccagttcagccaagctcctggggtctagtgtttaaaatactccaattatatcatcttgtgcggactgaaatttttttccaaaagactggaaaagtgactagcgattcaaatatataaaacagtttgtaacttaaaagatagaagtgaagactaccagtacagtaggtaaagctgtgtgcatccacaatacaaaggatcagactccaagatggatggctactacataacaatgcattctgggtttctttgtgatacctggagaaaaaaaaaagcccgactgggttgcactatatttacatgtttactggcttcttcctggctagcaccactcttccccccaacccccaacatttttaagctacttattttaagtcacaggaatattcaatctaagaaaagcatcttattagagtaatataatttcttaaagaagatagcatatttacacacatctaacacatgaaaatactctattttatactaaattccaggttcaaatgaactacaatacaacattttgccttgtctgtagagtgaggattgttccaaatggggcatatgtttggctgcccctgcagtgactcactactgtcagacaagtccaaatcggtcccctagttggggaaggagcaaggtttggactgagagtttctagccagttgggttacacatccactcctttgatgagtgatccttctaggactatggtgaagtcctgaatggtctgcagaattcggataagggagttgacagtcatgcggtctcgcaggagagcgctctcttcatacattcgagtgatggcaggacactcagctaacaatggaatccactgtgggagcaggcgatcccttgttccaaggcaaactaaaatctggaatttgccatccttcccaatgttcctgggtgcagtattaatagcatttacgtagtggcagaaggttttgcaggatgatttctgaataaggacatcatcttcattatctagaatctggtcagttgtttcaaaataagcaaccactttctctatgaagtcccagatgaagacattcttgtgaaagatgcgggcagatttgaacccatggtggaaaacttgctcaagggctgcaaccaggccattttctccacacagcaacacggtgaggcttcctctctctttttcaggtttatgaaaatgtttcacaatattgttcacagcttctccaattccttcttgtatctgcccagcattgggtttgttgttttttcctgtcagtgaagtgatgctcaatctcctagccgtggtgggtgacttctgctggggtggagtccgacactgctttactagatcttcatctgatgctgatgtcatcaactctccaataagaattctctccaggctcccatcatcaatgcctttccccagccaccgcccacatgggaatctgtatgtatgtcctgtgatttcatttctgaccatgacacaatccactagccatttggctaacagtcctgagttatcgtgaccaatctgaacagtggtcagcttccccaagttctggcactcaaaggtcatttcgaggaggtttttgggaatctgcattactcctgtgtctcccagctctcctgatacacagatccaagggtttgatgtgattattgcattgctcagctttttgattgggatgatcactgacctatacggaatcatgatagtggtgaacacactggtgaagcagaaatagtccacagcattgagagaaagaaggtggtaaagaaactgctctctttcttcttcgcaacgtagaaaagcatatcgcttataaagcttcttggtgagtggttggttagaaagcaactgcttaagatgctgggacaagagcttcttttctagagacagtcttatccacgcccgagctcgtccaacatcagtcttgatctcactcatgttttgaatatgcctcatgtcctgaataagagagaccctgagcgttggcaacataactcctgagtcagattttcttctttctggtccgagggcaactggtgattctgcaaggtgctcttgtttctcttctctgtcctgaaattgaattaaatgtgaccacaaagccgacttcccctgcttgacctgcaagccatggctccatatcctctccagcaggtcacaaaggctggcgatcaaggtgttctcctccaggccggtgatgtttgcttctccatggccaagttccaccgcttcatgtcccatcttctccaccaacatgcgctttgtcttcattctacattcttttaataagccttctacgaatttacagttggtctgtgcaataactgcaggagagaggtctgacagtttgggttgcctcaggttttttcctaaacttcgtgcctcttgcatatatttcaggcagcactcagagaaggattttttaggaagtcgtgcaggaggaggtggaccctggtcccactcccagaatgccatggagttctgacagaccaaaagttccccggaaggctccctcaagtcgttgtccagcccaacatgctcagaatgctggcgaaggcgttctttcctgcgctgtgcagtggcactccgacttacccagcgattgttactggttggtcctgttgccaagacatcggactgtaactttggaaagaacccctgctcatatttgccttgaccaattttcatatcaagtagatgtgggtggattgcagtgtgatccattttcatcagtctctgctcaattgattgggctgcttcttttaaagtgctgcatttctgatatatagatgtccgcaaggtgggtgcccttacattatacagccttatcttatcaatccgagtgtcaaagacccgaagcaaaggatctttctcttcccactgagacataattttattatcaataaaggtggcaaacatctgtgtttcaatgaagcgtgaaagaaatggcaggtaaggctcaggctggtcagacagaaaggaagctttgtcaaagttctgcatctgttcccggttggtcagccaggattccatgtcctgggcagtctgaatgacaaatgcttcgtaatctgcaaacatctgtgtaaaacggttagcaaagacctctcggagctgtacattgagctggtagtcccttagttctgcctcttcacaatgcagttttaaatccttgtctttttcacccagagaagcagagaggtccattttttccacagccacaccagtacgcttggccagagcctgcaagcgggctatggtttcattgcccttcagtaactcatacatgctgatgttattagtacagacattgccgttctttttgtcattgaccaagtctttcagaaccatattcttcagtttgctggtactctcactgcaatgtaggctgccctcaggagggatcccaaattgaacaagaacctcagagagttcttggataaaatccactttattggggaactgtggaaattcttcaggcaactcaataaaatggttgtcaatgtccacaaaacacaaattagcctcttgaggaagttctagtttagaacggtcagttccttcttttgactgaaggcccatcagataagggacaggagcatcaagaaaatgtagcagagaagcaggtagaatgggcacataaacatgttgccattgaaatgggaacaaaagtgtggtgatgccttctgccacagtcatcaggcgttgataatttgtaacttcttcataaaaagtgagaacaaaaccataggtgcgagaaccatcttccctggtaattataaatgagtgaaactgggggtctttattgtccgtttgtgtcctgaaagatagccctttaggcatgcacaacatgttcaccgcatcttgatcaaaagggttccattctatattctgaggatagtgggcgagaactttggatttgaatgttcttctcaaaggactctggtcaaaattttcgcctgaagtcgtatttgcagcaccttggctcttgccatgacgatctgcttctagccattggtacaaaaccgccagctcgtcaggctccagcccgctgtccgcgtcgatcccgcacagcacgaagtagtgcgcgaagcggcaggcggccggggaggagcccgagcccgggccgggcgccgcgcagctcccgctcatcccggccgcgctgctccaggggccgccgccgccgccgcccgggaaggctttctgcggaggctgccaccaccgctccggctgtggtctgtgcgcccgccctagggcgacactggcgcgcccat

SEQ ID NO: 11936 - RNA, 7451 nt, Homo sapiens
  source 1..7451: mol_type = other RNA
ctgaatagctgggactacaggtgtgtactgccatgcccaacatgtcttatttctttataactgcacttcttatgtgaccccaaactcagcttaagcatccttttcattgatcaaacttggatcctaaggactatttccaaatatttaaatttattcttaaaggccaagattgactgccattgggaatattcaaaagaatgggggtactggccattcaagcagctcacacaaggagggccccacatgtttatagcacaggctgtatcaacggaataagtacatgggctcacaaggtgactgaaggacccatcatccaagaggatgtgtcagttctgatgtgttttttttaaatcatcatttcaccattatagtaatattacacaaaggcatgaagatgaaacttcaggtgtaacttttttgggggtattactttttaaagtaatggttttattcataggccgcaaatccaactttggctgcagtttttttctttttttttttttgagacggagtctcgctcttgtcacccaggttggagtgcagtggcacaatctcggctcactgcaacctccacctcctgtgtttaaacgattctcctgcttcagcctcctgagtagctggaattacaggccctgccaccacccccccgctaatttttgtctattttttttttttagtagagacggggtttcaccatgttggccagtctggtcttgaactcccgactgacctcagatgaaccacccgcctcagactcccaaagtgtcaggattacaggcgttagccaccgtacctggcctgctcccagtttttacaagatgttaattcccaataatctgagagcaatgtgttaatatgaatattaattcttctaaatgaatattcatccttatttcctacttgtataggtggatgaataaagatccaatagtataatagaaagactattagtaagaatgccggaaggtcagtctcatgcagcctggtgaaataaaacaaacaaacaaacatgaattctagagcttgtgttgtcagtaaccagctgtggggtaagtgtaagatttaatctctctattccttaagtgttcccatccacaaagtaagaaggctggatgaggtgtgtcaatcctagcacattaacctaagtcatcccccaggttgcctagacctgtcaggagcatggccttatgaagatacaaacatgaaatcctgggttggacccctctatagtttctgatcaccaaacacagtaggagcccagtgtaaaacaggttctggatatctcccacgataaacttcccatgtccctggaagagctgtaccattgtagacacactttagcttcaggcaaacaaatttctggtgtacccagaaccattttcttaaaccatttccatgggtttttatttttatctatttattttttgagatggagtcttgctctgttgcccaggctggagggcagtggcgcgatctcagcttactgcaagctccgcctcgcgggttcacgccattctcctgcctcagcctcctgtacaggcacccgccaccacgcccggctaattttttgtatttttagtagagacggggtttcacggtgttagccaggagggtctcaatctcctgaccttgtgatccgcctgcctcggcctcccaaagtgctgggatcataggcgtgagccaccgcacccggctccatgggtttttaaatacagctgtcaactctccttttcctcaagtatgaagtcacatgttaaaagaggctgtccttggctgtgtttgataaagggagttaggcacttgtttcatctgtttcttcctccaggaaataaggttaacaacacaggtggtgaaagcccagcaacctccgattgcacaaggatactgatgccatggctttgcttttcagccacaactgggaataaaactgggagctctgctgaggcaattttgctgctaaaaatgtacaaatgcctaattagagttacaggacctaccagaagatgaggacttacagtaactagccaatactacatttacttaacttctttataaactatcaaactggaaagttactcacaacttttggtctttcaaaattgttgccacctcttgctttgcttccattttgtcagcctgtgctgccagtggcttttagcttctctgggtcagttgttttacattattactccccttcctacaaaggaacgtaaagcttgccctgaaacacccagaaagggttcattctctctctccttctgttatttgcattatcatggtcaacaaatgctttcacaaaaacattccaagccacacacagccctcctcctccttagacattccttccatttcccgaggggggatgggccctggagaggtgggtgattagaccctaacaaagacagggctcatggttatccttaagaggtagaccactgcacagtttagatggccaaattaaaagtacagaatcaaattgctgtttgcagttcttatcactatgaatctaacactgaaattcacatcttcccaaagtacctcaaataacaagaataaaaatgccaagaatgaagttagtctaggctaatctttccgaagtgtaaagaagttataatcccacaattgaacacatttctcagagctttgtatgttctctttccagttcagccaagctcctggggtctagtgtttaaaatactccaattatatcatcttgtgcggactgaaatttttttccaaaagactggaaaagtgactagcgattcaaatatataaaacagtttgtaacttaaaagatagaagtgaagactaccagtacagtaggtaaagctgtgtgcatccacaatacaaaggatcagactccaagatggatggctactacataacaatgcattctgggtttctttgtgatacctggagaaaaaaaaaagcccgactgggttgcactatatttacatgtttactggcttcttcctggctagcaccactcttccccccaacccccaacatttttaagctacttattttaagtcacaggaatattcaatctaagaaaagcatcttattagagtaatataatttcttaaagaagatagcatatttacacacatctaacacatgaaaatactctattttatactaaattccaggttcaaatgaactacaatacaacattttgccttgtctgtagagtgaggattgttccaaatggggcatatgtttggctgcccctgcagtgactcactactgtcagacaagtccaaatcggtcccctagttggggaaggagcaaggtttggactgagagtttctagccagttgggttacacatccactcctttgatgagtgatccttctaggactatggtgaagtcctgaatggtctgcagaattcggataagggagttgacagtcatgcggtctcgcaggagagcgctctcttcatacattcgagtgatggcaggacactcagctaacaatggaatccactgtgggagcaggcgatcccttgttccaaggcaaactaaaatctggaatttgccatccttcccaatgttcctgggtgcagtattaatagcatttacgtagtggcagaaggttttgcaggatgatttctgaataaggacatcatcttcattatctagaatctggtcagttgtttcaaaataagcaaccactttctctatgaagtcccagatgaagacattcttgtgaaagatgcgggcagatttgaacccatggtggaaaacttgctcaagggctgcaaccaggccattttctccacacagcaacacggtgaggcttcctctctctttttcaggtttatgaaaatgtttcacaatattgttcacagcttctccaattccttcttgtatctgcccagcattgggtttgttgttttttcctgtcagtgaagtgatgctcaatctcctagccgtggtgggtgacttctgctggggtggagtccgacactgctttactagatcttcatctgatgctgatgtcatcaactctccaataagaattctctccaggctcccatcatcaatgcctttccccagccaccgcccacatgggaatctgtatgtatgtcctgtgatttcatttctgaccatgacacaatccactagccatttggctaacagtcctgagttatcgtgaccaatctgaacagtggtcagcttccccaagttctggcactcaaaggtcatttcgaggaggtttttgggaatctgcattactcctgtgtctcccagctctcctgatacacagatccaagggtttgatgtgattattgcattgctcagctttttgattgggatgatcactgacctatacggaatcatgatagtggtgaacacactggtgaagcagaaatagtccacagcattgagagaaagaaggtggtaaagaaactgctctctttcttcttcgcaacgtagaaaagcatatcgcttataaagcttcttggtgagtggttggttagaaagcaactgcttaagatgctgggacaagagcttcttttctagagacagtcttatccacgcccgagctcgtccaacatcagtcttgatctcactcatgttttgaatatgcctcatgtcctgaataagagagaccctgagcgttggcaacataactcctgagtcagattttcttctttctggtccgagggcaactggtgattctgcaaggtgctcttgtttctcttctctgtcctgaaattgaattaaatgtgaccacaaagccgacttcccctgcttgacctgcaagccatggctccatatcctctccagcaggtcacaaaggctggcgatcaaggtgttctcctccaggccggtgatgtttgcttctccatggccaagttccaccgcttcatgtcccatcttctccaccaacatgcgctttgtcttcattctacattcttttaataagccttctacgaatttacagttggtctgtgcaataactgcaggagagaggtctgacagtttgggttgcctcaggttttttcctaaacttcgtgcctcttgcatatatttctccctcaagtcgttgtccagcccaacatgctcagaatgctggcgaaggcgttctttcctgcgctgtgcagtggcactccgacttacccagcgattgttactggttggtcctgttgccaagacatcggactgtaactttggaaagaacccctgctcatatttgccttgaccaattttcatatcaagtagatgtgggtggattgcagtgtgatccattttcatcagtctctgctcaattgattgggctgcttcttttaaagtgctgcatttctgatatatagatgtccgcaaggtgggtgcccttacattatacagccttatcttatcaatccgagtgtcaaagacccgaagcaaaggatctttctcttcccactgagacataattttattatcaataaaggtggcaaacatctgtgtttcaatgaagcgtgaaagaaatggcaggtaaggctcaggctggtcagacagaaaggaagctttgtcaaagttctgcatctgttcccggttggtcagccaggattccatgtcctgggcagtctgaatgacaaatgcttcgtaatctgcaaacatctgtgtaaaacggttagcaaagacctctcggagctgtacattgagctggtagtcccttagttctgcctcttcacaatgcagttttaaatccttgtctttttcacccagagaagcagagaggtccattttttccacagccacaccagtacgcttggccagagcctgcaagcgggctatggtttcattgcccttcagtaactcatacatgctgatgttattagtacagacattgccgttctttttgtcattgaccaagtctttcagaaccatattcttcagtttgctggtactctcactgcaatgtaggctgccctcaggagggatcccaaattgaacaagaacctcagagagttcttggataaaatccactttattggggaactgtggaaattcttcaggcaactcaataaaatggttgtcaatgtccacaaaacacaaattagcctcttgaggaagttctagtttagaacggtcagttccttcttttgactgaaggcccatcagataagggacaggagcatcaagaaaatgtagcagagaagcaggtagaatgggcacataaacatgttgccattgaaatgggaacaaaagtgtggtgatgccttctgccacagtcatcaggcgttgataatcttgtgagtagagaaggatttgcatctctaaaagaacacaggtaaacacctgcaccaggttctctaatcccaggagctcaaatgcctcccgaagggggtaatcagagagggggagttcactgggcccaggcctctggcagatgacaggttcataaacaccataaaatttcagtgacctccctggaggtggaaggggtacttcataaagaatattgtggatatagctttcaagtggcaagggtggtggctgctgtgaggtaacagccttgtaaagctggataaggaatttcttgcaggcctgcatgaatggtaacggtgtgatcaagcatatactttttgaaacatacagggtgtctctgctaatatcataggagttgtatcgctggagtttcaaaagggaagttgtatctccttcatcaagactacttgccaatgagtccatactgcaggaagatgaagcatacacactgctgtaatgctcagcgttgtgcatctggtaaagtgtctgcattgctgtgcagatttgcttacttgtaacttcttcataaaaagtgagaacaaaaccataggtgcgagaaccatcttccctggtaattataaatgagtgaaactgggggtctttattgtccgtttgtgtcctgaaagatagccctttaggcatgcacaacatgttcaccgcatcttgatcaaaagggttccattctatattctgaggatagtgggcgagaactttggatttgaatgttcttctcaaaggactctggtcaaaattttcgcccgccagctcgtcaggctccagcccgctgtccgcgtcgatcccgcacagcacgaagtagtgcgcgaagcggcaggcggccggggaggagcccgagcccgggccgggcgccgcgcagctcccgctcatcccggccgcgctgctccaggggccgccgccgccgccgcccgggaaggctttctgcggaggctgccaccaccgctccggctgtggtctgtgcgcccgccctagggcgacactggcgcgcccatggccgcgcagccgcctctcgccgccgcagcctgcctcctcgctcggcgcgggggaagcggccgcgggctcgcgcgcggcgggtccggagcccggccgggtgggggaggggcgcggggggagtgtcggcctgagaggccctcgcagccgcagctgcgctcgcgagctgagagccgccgcgtct

SEQ ID NO: 11937 - RNA, 7403 nt, Homo sapiens
  source 1..7403: mol_type = other RNA
ctgaatagctgggactacaggtgtgtactgccatgcccaacatgtcttatttctttataactgcacttcttatgtgaccccaaactcagcttaagcatccttttcattgatcaaacttggatcctaaggactatttccaaatatttaaatttattcttaaaggccaagattgactgccattgggaatattcaaaagaatgggggtactggccattcaagcagctcacacaaggagggccccacatgtttatagcacaggctgtatcaacggaataagtacatgggctcacaaggtgactgaaggacccatcatccaagaggatgtgtcagttctgatgtgttttttttaaatcatcatttcaccattatagtaatattacacaaaggcatgaagatgaaacttcaggtgtaacttttttgggggtattactttttaaagtaatggttttattcataggccgcaaatccaactttggctgcagtttttttctttttttttttttgagacggagtctcgctcttgtcacccaggttggagtgcagtggcacaatctcggctcactgcaacctccacctcctgtgtttaaacgattctcctgcttcagcctcctgagtagctggaattacaggccctgccaccacccccccgctaatttttgtctattttttttttttagtagagacggggtttcaccatgttggccagtctggtcttgaactcccgactgacctcagatgaaccacccgcctcagactcccaaagtgtcaggattacaggcgttagccaccgtacctggcctgctcccagtttttacaagatgttaattcccaataatctgagagcaatgtgttaatatgaatattaattcttctaaatgaatattcatccttatttcctacttgtataggtggatgaataaagatccaatagtataatagaaagactattagtaagaatgccggaaggtcagtctcatgcagcctggtgaaataaaacaaacaaacaaacatgaattctagagcttgtgttgtcagtaaccagctgtggggtaagtgtaagatttaatctctctattccttaagtgttcccatccacaaagtaagaaggctggatgaggtgtgtcaatcctagcacattaacctaagtcatcccccaggttgcctagacctgtcaggagcatggccttatgaagatacaaacatgaaatcctgggttggacccctctatagtttctgatcaccaaacacagtaggagcccagtgtaaaacaggttctggatatctcccacgataaacttcccatgtccctggaagagctgtaccattgtagacacactttagcttcaggcaaacaaatttctggtgtacccagaaccattttcttaaaccatttccatgggtttttatttttatctatttattttttgagatggagtcttgctctgttgcccaggctggagggcagtggcgcgatctcagcttactgcaagctccgcctcgcgggttcacgccattctcctgcctcagcctcctgtacaggcacccgccaccacgcccggctaattttttgtatttttagtagagacggggtttcacggtgttagccaggagggtctcaatctcctgaccttgtgatccgcctgcctcggcctcccaaagtgctgggatcataggcgtgagccaccgcacccggctccatgggtttttaaatacagctgtcaactctccttttcctcaagtatgaagtcacatgttaaaagaggctgtccttggctgtgtttgataaagggagttaggcacttgtttcatctgtttcttcctccaggaaataaggttaacaacacaggtggtgaaagcccagcaacctccgattgcacaaggatactgatgccatggctttgcttttcagccacaactgggaataaaactgggagctctgctgaggcaattttgctgctaaaaatgtacaaatgcctaattagagttacaggacctaccagaagatgaggacttacagtaactagccaatactacatttacttaacttctttataaactatcaaactggaaagttactcacaacttttggtctttcaaaattgttgccacctcttgctttgcttccattttgtcagcctgtgctgccagtggcttttagcttctctgggtcagttgttttacattattactccccttcctacaaaggaacgtaaagcttgccctgaaacacccagaaagggttcattctctctctccttctgttatttgcattatcatggtcaacaaatgctttcacaaaaacattccaagccacacacagccctcctcctccttagacattccttccatttcccgaggggggatgggccctggagaggtgggtgattagaccctaacaaagacagggctcatggttatccttaagaggtagaccactgcacagtttagatggccaaattaaaagtacagaatcaaattgctgtttgcagttcttatcactatgaatctaacactgaaattcacatcttcccaaagtacctcaaataacaagaataaaaatgccaagaatgaagttagtctaggctaatctttccgaagtgtaaagaagttataatcccacaattgaacacatttctcagagctttgtatgttctctttccagttcagccaagctcctggggtctagtgtttaaaatactccaattatatcatcttgtgcggactgaaatttttttccaaaagactggaaaagtgactagcgattcaaatatataaaacagtttgtaacttaaaagatagaagtgaagactaccagtacagtaggtaaagctgtgtgcatccacaatacaaaggatcagactccaagatggatggctactacataacaatgcattctgggtttctttgtgatacctggagaaaaaaaaaagcccgactgggttgcactatatttacatgtttactggcttcttcctggctagcaccactcttccccccaacccccaacatttttaagctacttattttaagtcacaggaatattcaatctaagaaaagcatcttattagagtaatataatttcttaaagaagatagcatatttacacacatctaacacatgaaaatactctattttatactaaattccaggttcaaatgaactacaatacaacattttgccttgtctgtagagtgaggattgttccaaatggggcatatgtttggctgcccctgcagtgactcactactgtcagacaagtccaaatcggtcccctagttggggaaggagcaaggtttggactgagagtttctagccagttgggttacacatccactcctttgatgagtgatccttctaggactatggtgaagtcctgaatggtctgcagaattcggataagggagttgacagtcatgcggtctcgcaggagagcgctctcttcatacattcgagtgatggcaggacactcagctaacaatggaatccactgtgggagcaggcgatcccttgttccaaggcaaactaaaatctggaatttgccatccttcccaatgttcctgggtgcagtattaatagcatttacgtagtggcagaaggttttgcaggatgatttctgaataaggacatcatcttcattatctagaatctggtcagttgtttcaaaataagcaaccactttctctatgaagtcccagatgaagacattcttgtgaaagatgcgggcagatttgaacccatggtggaaaacttgctcaagggctgcaaccaggccattttctccacacagcaacacggtgaggcttcctctctctttttcaggtttatgaaaatgtttcacaatattgttcacagcttctccaattccttcttgtatctgcccagcattgggtttgttgttttttcctgtcagtgaagtgatgctcaatctcctagccgtggtgggtgacttctgctggggtggagtccgacactgctttactagatcttcatctgatgctgatgtcatcaactctccaataagaattctctccaggctcccatcatcaatgcctttccccagccaccgcccacatgggaatctgtatgtatgtcctgtgatttcatttctgaccatgacacaatccactagccatttggctaacagtcctgagttatcgtgaccaatctgaacagtggtcagcttccccaagttctggcactcaaaggtcatttcgaggaggtttttgggaatctgcattactcctgtgtctcccagctctcctgatacacagatccaagggtttgatgtgattattgcattgctcagctttttgattgggatgatcactgacctatacggaatcatgatagtggtgaacacactggtgaagcagaaatagtccacagcattgagagaaagaaggtggtaaagaaactgctctctttcttcttcgcaacgtagaaaagcatatcgcttataaagcttcttggtgagtggttggttagaaagcaactgcttaagatgctgggacaagagcttcttttctagagacagtcttatccacgcccgagctcgtccaacatcagtcttgatctcactcatgttttgaatatgcctcatgtcctgaataagagagaccctgagcgttggcaacataactcctgagtcagattttcttctttctggtccgagggcaactggtgattctgcaaggtgctcttgtttctcttctctgtcctgaaattgaattaaatgtgaccacaaagccgacttcccctgcttgacctgcaagccatggctccatatcctctccagcaggtcacaaaggctggcgatcaaggtgttctcctccaggccggtgatgtttgcttctccatggccaagttccaccgcttcatgtcccatcttctccaccaacatgcgctttgtcttcattctacattcttttaataagccttctacgaatttacagttggtctgtgcaataactgcaggagagaggtctgacagtttgggttgcctcaggttttttcctaaacttcgtgcctcttgcatatatttctccctcaagtcgttgtccagcccaacatgctcagaatgctggcgaaggcgttctttcctgcgctgtgcagtggcactccgacttacccagcgattgttactggttggtcctgttgccaagacatcggactgtaactttggaaagaacccctgctcatatttgccttgaccaattttcatatcaagtagatgtgggtggattgcagtgtgatccattttcatcagtctctgctcaattgattgggctgcttcttttaaagtgctgcatttctgatatatagatgtccgcaaggtgggtgcccttacattatacagccttatcttatcaatccgagtgtcaaagacccgaagcaaaggatctttctcttcccactgagacataattttattatcaataaaggtggcaaacatctgtgtttcaatgaagcgtgaaagaaatggcaggtaaggctcaggctggtcagacagaaaggaagctttgtcaaagttctgcatctgttcccggttggtcagccaggattccatgtcctgggcagtctgaatgacaaatgcttcgtaatctgcaaacatctgtgtaaaacggttagcaaagacctctcggagctgtacattgagctggtagtcccttagttctgcctcttcacaatgcagttttaaatccttgtctttttcacccagagaagcagagaggtccattttttccacagccacaccagtacgcttggccagagcctgcaagcgggctatggtttcattgcccttcagtaactcatacatgctgatgttattagtacagacattgccgttctttttgtcattgaccaagtctttcagaaccatattcttcagtttgctggtactctcactgcaatgtaggctgccctcaggagggatcccaaattgaacaagaacctcagagagttcttggataaaatccactttattggggaactgtggaaattcttcaggcaactcaataaaatggttgtcaatgtccacaaaacacaaattagcctcttgaggaagttctagtttagaacggtcagttccttcttttgactgaaggcccatcagataagggacaggagcatcaagaaaatgtagcagagaagcaggtagaatgggcacataaacatgttgccattgaaatgggaacaaaagtgtggtgatgccttctgccacagtcatcaggcgttgataatcttgtgagtagagaaggatttgcatctctaaaagaacacaggtaaacacctgcaccaggttctctaatcccaggagctcaaatgcctcccgaagggggtaatcagagagggggagttcactgggcccaggcctctggcagatgacaggttcataaacaccataaaatttcagtgacctccctggaggtggaaggggtacttcataaagaatattgtggatatagctttcaagtggcaagggtggtggctgctgtgaggtaacagccttgtaaagctggataaggaatttcttgcaggcctgcatgaatggtaacggtgtgatcaagcatatactttttgaaacatacagggtgtctctgctaatatcataggagttgtatcgctggagtttcaaaagggaagttgtatctccttcatcaagactacttgccaatgagtccatactgcaggaagatgaagcatacacactgctgtaatgctcagcgttgtgcatctggtaaagtgtctgcattgctgtgcagatttgcttacttgtaacttcttcataaaaagtgagaacaaaaccataggtgcgagaaccatcttccctggtaattataaatgagtgaaactgggggtctttattgtccgtttgtgtcctgaaagatagccctttaggcatgcacaacatgttcaccgcatcttgatcaaaagggttccattctatattctgaggatagtgggcgagaactttggatttgaatgttcttctcaaaggactctggtcaaaattttcgcctgaagtcgtatttgcagcaccttggctcttgccatgacgatctgcttctagccattggtacaaaaatcctggctgggcatgttggctcacaactgtaatctcagcacttcgggaggccgaggcaggtgaattgcttgaggtcaggagttcgagaccagcctgatcaacatggtgaaacctcatctctactaaaaatacaaaaattagctgggcatggtggtgggtgcccataatcccagttactcaggaaggccaggcaggagaattactggaacccaagaggtggaggttgtagtgatctgagatcatgccactgcacttcagccggccgcctccgagtgcggctgcaagcgaaggggccggcgcgccaggcggggtccgt

SEQ ID NO: 11938 - RNA, 7335 nt, Homo sapiens
  source 1..7335: mol_type = other RNA
ctgaatagctgggactacaggtgtgtactgccatgcccaacatgtcttatttctttataactgcacttcttatgtgaccccaaactcagcttaagcatccttttcattgatcaaacttggatcctaaggactatttccaaatatttaaatttattcttaaaggccaagattgactgccattgggaatattcaaaagaatgggggtactggccattcaagcagctcacacaaggagggccccacatgtttatagcacaggctgtatcaacggaataagtacatgggctcacaaggtgactgaaggacccatcatccaagaggatgtgtcagttctgatgtgttttttttaaatcatcatttcaccattatagtaatattacacaaaggcatgaagatgaaacttcaggtgtaacttttttgggggtattactttttaaagtaatggttttattcataggccgcaaatccaactttggctgcagtttttttctttttttttttttgagacggagtctcgctcttgtcacccaggttggagtgcagtggcacaatctcggctcactgcaacctccacctcctgtgtttaaacgattctcctgcttcagcctcctgagtagctggaattacaggccctgccaccacccccccgctaatttttgtctattttttttttttagtagagacggggtttcaccatgttggccagtctggtcttgaactcccgactgacctcagatgaaccacccgcctcagactcccaaagtgtcaggattacaggcgttagccaccgtacctggcctgctcccagtttttacaagatgttaattcccaataatctgagagcaatgtgttaatatgaatattaattcttctaaatgaatattcatccttatttcctacttgtataggtggatgaataaagatccaatagtataatagaaagactattagtaagaatgccggaaggtcagtctcatgcagcctggtgaaataaaacaaacaaacaaacatgaattctagagcttgtgttgtcagtaaccagctgtggggtaagtgtaagatttaatctctctattccttaagtgttcccatccacaaagtaagaaggctggatgaggtgtgtcaatcctagcacattaacctaagtcatcccccaggttgcctagacctgtcaggagcatggccttatgaagatacaaacatgaaatcctgggttggacccctctatagtttctgatcaccaaacacagtaggagcccagtgtaaaacaggttctggatatctcccacgataaacttcccatgtccctggaagagctgtaccattgtagacacactttagcttcaggcaaacaaatttctggtgtacccagaaccattttcttaaaccatttccatgggtttttatttttatctatttattttttgagatggagtcttgctctgttgcccaggctggagggcagtggcgcgatctcagcttactgcaagctccgcctcgcgggttcacgccattctcctgcctcagcctcctgtacaggcacccgccaccacgcccggctaattttttgtatttttagtagagacggggtttcacggtgttagccaggagggtctcaatctcctgaccttgtgatccgcctgcctcggcctcccaaagtgctgggatcataggcgtgagccaccgcacccggctccatgggtttttaaatacagctgtcaactctccttttcctcaagtatgaagtcacatgttaaaagaggctgtccttggctgtgtttgataaagggagttaggcacttgtttcatctgtttcttcctccaggaaataaggttaacaacacaggtggtgaaagcccagcaacctccgattgcacaaggatactgatgccatggctttgcttttcagccacaactgggaataaaactgggagctctgctgaggcaattttgctgctaaaaatgtacaaatgcctaattagagttacaggacctaccagaagatgaggacttacagtaactagccaatactacatttacttaacttctttataaactatcaaactggaaagttactcacaacttttggtctttcaaaattgttgccacctcttgctttgcttccattttgtcagcctgtgctgccagtggcttttagcttctctgggtcagttgttttacattattactccccttcctacaaaggaacgtaaagcttgccctgaaacacccagaaagggttcattctctctctccttctgttatttgcattatcatggtcaacaaatgctttcacaaaaacattccaagccacacacagccctcctcctccttagacattccttccatttcccgaggggggatgggccctggagaggtgggtgattagaccctaacaaagacagggctcatggttatccttaagaggtagaccactgcacagtttagatggccaaattaaaagtacagaatcaaattgctgtttgcagttcttatcactatgaatctaacactgaaattcacatcttcccaaagtacctcaaataacaagaataaaaatgccaagaatgaagttagtctaggctaatctttccgaagtgtaaagaagttataatcccacaattgaacacatttctcagagctttgtatgttctctttccagttcagccaagctcctggggtctagtgtttaaaatactccaattatatcatcttgtgcggactgaaatttttttccaaaagactggaaaagtgactagcgattcaaatatataaaacagtttgtaacttaaaagatagaagtgaagactaccagtacagtaggtaaagctgtgtgcatccacaatacaaaggatcagactccaagatggatggctactacataacaatgcattctgggtttctttgtgatacctggagaaaaaaaaaagcccgactgggttgcactatatttacatgtttactggcttcttcctggctagcaccactcttccccccaacccccaacatttttaagctacttattttaagtcacaggaatattcaatctaagaaaagcatcttattagagtaatataatttcttaaagaagatagcatatttacacacatctaacacatgaaaatactctattttatactaaattccaggttcaaatgaactacaatacaacattttgccttgtctgtagagtgaggattgttccaaatggggcatatgtttggctgcccctgcagtgactcactactgtcagacaagtccaaatcggtcccctagttggggaaggagcaaggtttggactgagagtttctagccagttgggttacacatccactcctttgatgagtgatccttctaggactatggtgaagtcctgaatggtctgcagaattcggataagggagttgacagtcatgcggtctcgcaggagagcgctctcttcatacattcgagtgatggcaggacactcagctaacaatggaatccactgtgggagcaggcgatcccttgttccaaggcaaactaaaatctggaatttgccatccttcccaatgttcctgggtgcagtattaatagcatttacgtagtggcagaaggttttgcaggatgatttctgaataaggacatcatcttcattatctagaatctggtcagttgtttcaaaataagcaaccactttctctatgaagtcccagatgaagacattcttgtgaaagatgcgggcagatttgaacccatggtggaaaacttgctcaagggctgcaaccaggccattttctccacacagcaacacggtgaggcttcctctctctttttcaggtttatgaaaatgtttcacaatattgttcacagcttctccaattccttcttgtatctgcccagcattgggtttgttgttttttcctgtcagtgaagtgatgctcaatctcctagccgtggtgggtgacttctgctggggtggagtccgacactgctttactagatcttcatctgatgctgatgtcatcaactctccaataagaattctctccaggctcccatcatcaatgcctttccccagccaccgcccacatgggaatctgtatgtatgtcctgtgatttcatttctgaccatgacacaatccactagccatttggctaacagtcctgagttatcgtgaccaatctgaacagtggtcagcttccccaagttctggcactcaaaggtcatttcgaggaggtttttgggaatctgcattactcctgtgtctcccagctctcctgatacacagatccaagggtttgatgtgattattgcattgctcagctttttgattgggatgatcactgacctatacggaatcatgatagtggtgaacacactggtgaagcagaaatagtccacagcattgagagaaagaaggtggtaaagaaactgctctctttcttcttcgcaacgtagaaaagcatatcgcttataaagcttcttggtgagtggttggttagaaagcaactgcttaagatgctgggacaagagcttcttttctagagacagtcttatccacgcccgagctcgtccaacatcagtcttgatctcactcatgttttgaatatgcctcatgtcctgaataagagagaccctgagcgttggcaacataactcctgagtcagattttcttctttctggtccgagggcaactggtgattctgcaaggtgctcttgtttctcttctctgtcctgaaattgaattaaatgtgaccacaaagccgacttcccctgcttgacctgcaagccatggctccatatcctctccagcaggtcacaaaggctggcgatcaaggtgttctcctccaggccggtgatgtttgcttctccatggccaagttccaccgcttcatgtcccatcttctccaccaacatgcgctttgtcttcattctacattcttttaataagccttctacgaatttacagttggtctgtgcaataactgcaggagagaggtctgacagtttgggttgcctcaggttttttcctaaacttcgtgcctcttgcatatatttctccctcaagtcgttgtccagcccaacatgctcagaatgctggcgaaggcgttctttcctgcgctgtgcagtggcactccgacttacccagcgattgttactggttggtcctgttgccaagacatcggactgtaactttggaaagaacccctgctcatatttgccttgaccaattttcatatcaagtagatgtgggtggattgcagtgtgatccattttcatcagtctctgctcaattgattgggctgcttcttttaaagtgctgcatttctgatatatagatgtccgcaaggtgggtgcccttacattatacagccttatcttatcaatccgagtgtcaaagacccgaagcaaaggatctttctcttcccactgagacataattttattatcaataaaggtggcaaacatctgtgtttcaatgaagcgtgaaagaaatggcaggtaaggctcaggctggtcagacagaaaggaagctttgtcaaagttctgcatctgttcccggttggtcagccaggattccatgtcctgggcagtctgaatgacaaatgcttcgtaatctgcaaacatctgtgtaaaacggttagcaaagacctctcggagctgtacattgagctggtagtcccttagttctgcctcttcacaatgcagttttaaatccttgtctttttcacccagagaagcagagaggtccattttttccacagccacaccagtacgcttggccagagcctgcaagcgggctatggtttcattgcccttcagtaactcatacatgctgatgttattagtacagacattgccgttctttttgtcattgaccaagtctttcagaaccatattcttcagtttgctggtactctcactgcaatgtaggctgccctcaggagggatcccaaattgaacaagaacctcagagagttcttggataaaatccactttattggggaactgtggaaattcttcaggcaactcaataaaatggttgtcaatgtccacaaaacacaaattagcctcttgaggaagttctagtttagaacggtcagttccttcttttgactgaaggcccatcagataagggacaggagcatcaagaaaatgtagcagagaagcaggtagaatgggcacataaacatgttgccattgaaatgggaacaaaagtgtggtgatgccttctgccacagtcatcaggcgttgataatcttgtgagtagagaaggatttgcatctctaaaagaacacaggtaaacacctgcaccaggttctctaatcccaggagctcaaatgcctcccgaagggggtaatcagagagggggagttcactgggcccaggcctctggcagatgacaggttcataaacaccataaaatttcagtgacctccctggaggtggaaggggtacttcataaagaatattgtggatatagctttcaagtggcaagggtggtggctgctgtgaggtaacagccttgtaaagctggataaggaatttcttgcaggcctgcatgaatggtaacggtgtgatcaagcatatactttttgaaacatacagggtgtctctgctaatatcataggagttgtatcgctggagtttcaaaagggaagttgtatctccttcatcaagactacttgccaatgagtccatactgcaggaagatgaagcatacacactgctgtaatgctcagcgttgtgcatctggtaaagtgtctgcattgctgtgcagatttgcttacttgtaacttcttcataaaaagtgagaacaaaaccataggtgcgagaaccatcttccctggtaattataaatgagtgaaactgggggtctttattgtccgtttgtgtcctgaaagatagccctttaggcatgcacaacatgttcaccgcatcttgatcaaaagggttccattctatattctgaggatagtgggcgagaactttggatttgaatgttcttctcaaaggactctggtcaaaattttcgcctgaagtcgtatttgcagcaccttggctcttgccatgacgatctgcttctagccattggtacaaaaccgccagctcgtcaggctccagcccgctgtccgcgtcgatcccgcacagcacgaagtagtgcgcgaagcggcaggcggccggggaggagcccgagcccgggccgggcgccgcgcagctcccgctcatcccggccgcgctgctccaggggccgccgccgccgccgcccgggaaggctttctgcggaggctgccaccaccgctccggctgtggtctgtgcgcccgccctagggcgacactggcgcgcccat

SEQ ID NO: 11939 - RNA, 6694 nt, Homo sapiens
  source 1..6694: mol_type = other RNA
ctgaatagctgggactacaggtgtgtactgccatgcccaacatgtcttatttctttataactgcacttcttatgtgaccccaaactcagcttaagcatccttttcattgatcaaacttggatcctaaggactatttccaaatatttaaatttattcttaaaggccaagattgactgccattgggaatattcaaaagaatgggggtactggccattcaagcagctcacacaaggagggccccacatgtttatagcacaggctgtatcaacggaataagtacatgggctcacaaggtgactgaaggacccatcatccaagaggatgtgtcagttctgatgtgttttttttaaatcatcatttcaccattatagtaatattacacaaaggcatgaagatgaaacttcaggtgtaacttttttgggggtattactttttaaagtaatggttttattcataggccgcaaatccaactttggctgcagtttttttctttttttttttttgagacggagtctcgctcttgtcacccaggttggagtgcagtggcacaatctcggctcactgcaacctccacctcctgtgtttaaacgattctcctgcttcagcctcctgagtagctggaattacaggccctgccaccacccccccgctaatttttgtctattttttttttttagtagagacggggtttcaccatgttggccagtctggtcttgaactcccgactgacctcagatgaaccacccgcctcagactcccaaagtgtcaggattacaggcgttagccaccgtacctggcctgctcccagtttttacaagatgttaattcccaataatctgagagcaatgtgttaatatgaatattaattcttctaaatgaatattcatccttatttcctacttgtataggtggatgaataaagatccaatagtataatagaaagactattagtaagaatgccggaaggtcagtctcatgcagcctggtgaaataaaacaaacaaacaaacatgaattctagagcttgtgttgtcagtaaccagctgtggggtaagtgtaagatttaatctctctattccttaagtgttcccatccacaaagtaagaaggctggatgaggtgtgtcaatcctagcacattaacctaagtcatcccccaggttgcctagacctgtcaggagcatggccttatgaagatacaaacatgaaatcctgggttggacccctctatagtttctgatcaccaaacacagtaggagcccagtgtaaaacaggttctggatatctcccacgataaacttcccatgtccctggaagagctgtaccattgtagacacactttagcttcaggcaaacaaatttctggtgtacccagaaccattttcttaaaccatttccatgggtttttatttttatctatttattttttgagatggagtcttgctctgttgcccaggctggagggcagtggcgcgatctcagcttactgcaagctccgcctcgcgggttcacgccattctcctgcctcagcctcctgtacaggcacccgccaccacgcccggctaattttttgtatttttagtagagacggggtttcacggtgttagccaggagggtctcaatctcctgaccttgtgatccgcctgcctcggcctcccaaagtgctgggatcataggcgtgagccaccgcacccggctccatgggtttttaaatacagctgtcaactctccttttcctcaagtatgaagtcacatgttaaaagaggctgtccttggctgtgtttgataaagggagttaggcacttgtttcatctgtttcttcctccaggaaataaggttaacaacacaggtggtgaaagcccagcaacctccgattgcacaaggatactgatgccatggctttgcttttcagccacaactgggaataaaactgggagctctgctgaggcaattttgctgctaaaaatgtacaaatgcctaattagagttacaggacctaccagaagatgaggacttacagtaactagccaatactacatttacttaacttctttataaactatcaaactggaaagttactcacaacttttggtctttcaaaattgttgccacctcttgctttgcttccattttgtcagcctgtgctgccagtggcttttagcttctctgggtcagttgttttacattattactccccttcctacaaaggaacgtaaagcttgccctgaaacacccagaaagggttcattctctctctccttctgttatttgcattatcatggtcaacaaatgctttcacaaaaacattccaagccacacacagccctcctcctccttagacattccttccatttcccgaggggggatgggccctggagaggtgggtgattagaccctaacaaagacagggctcatggttatccttaagaggtagaccactgcacagtttagatggccaaattaaaagtacagaatcaaattgctgtttgcagttcttatcactatgaatctaacactgaaattcacatcttcccaaagtacctcaaataacaagaataaaaatgccaagaatgaagttagtctaggctaatctttccgaagtgtaaagaagttataatcccacaattgaacacatttctcagagctttgtatgttctctttccagttcagccaagctcctggggtctagtgtttaaaatactccaattatatcatcttgtgcggactgaaatttttttccaaaagactggaaaagtgactagcgattcaaatatataaaacagtttgtaacttaaaagatagaagtgaagactaccagtacagtaggtaaagctgtgtgcatccacaatacaaaggatcagactccaagatggatggctactacataacaatgcattctgggtttctttgtgatacctggagaaaaaaaaaagcccgactgggttgcactatatttacatgtttactggcttcttcctggctagcaccactcttccccccaacccccaacatttttaagctacttattttaagtcacaggaatattcaatctaagaaaagcatcttattagagtaatataatttcttaaagaagatagcatatttacacacatctaacacatgaaaatactctattttatactaaattccaggttcaaatgaactacaatacaacattttgccttgtctgtagagtgaggattgttccaaatggggcatatgtttggctgcccctgcagtgactcactactgtcagacaagtccaaatcggtcccctagttggggaaggagcaaggtttggactgagagtttctagccagttgggttacacatccactcctttgatgagtgatccttctaggactatggtgaagtcctgaatggtctgcagaattcggataagggagttgacagtcatgcggtctcgcaggagagcgctctcttcatacattcgagtgatggcaggacactcagctaacaatggaatccactgtgggagcaggcgatcccttgttccaaggcaaactaaaatctggaatttgccatccttcccaatgttcctgggtgcagtattaatagcatttacgtagtggcagaaggttttgcaggatgatttctgaataaggacatcatcttcattatctagaatctggtcagttgtttcaaaataagcaaccactttctctatgaagtcccagatgaagacattcttgtgaaagatgcgggcagatttgaacccatggtggaaaacttgctcaagggctgcaaccaggccattttctccacacagcaacacggtgaggcttcctctctctttttcaggtttatgaaaatgtttcacaatattgttcacagcttctccaattccttcttgtatctgcccagcattgggtttgttgttttttcctgtcagtgaagtgatgctcaatctcctagccgtggtgggtgacttctgctggggtggagtccgacactgctttactagatcttcatctgatgctgatgtcatcaactctccaataagaattctctccaggctcccatcatcaatgcctttccccagccaccgcccacatgggaatctgtatgtatgtcctgtgatttcatttctgaccatgacacaatccactagccatttggctaacagtcctgagttatcgtgaccaatctgaacagtggtcagcttccccaagttctggcactcaaaggtcatttcgaggaggtttttgggaatctgcattactcctgtgtctcccagctctcctgatacacagatccaagggtttgatgtgattattgcattgctcagctttttgattgggatgatcactgacctatacggaatcatgatagtggtgaacacactggtgaagcagaaatagtccacagcattgagagaaagaaggtggtaaagaaactgctctctttcttcttcgcaacgtagaaaagcatatcgcttataaagcttcttggtgagtggttggttagaaagcaactgcttaagatgctgggacaagagcttcttttctagagacagtcttatccacgcccgagctcgtccaacatcagtcttgatctcactcatgttttgaatatgcctcatgtcctgaataagagagaccctgagcgttggcaacataactcctgagtcagattttcttctttctggtccgagggcaactggtgattctgcaaggtgctcttgtttctcttctctgtcctgaaattgaattaaatgtgaccacaaagccgacttcccctgcttgacctgcaagccatggctccatatcctctccagcaggtcacaaaggctggcgatcaaggtgttctcctccaggccggtgatgtttgcttctccatggccaagttccaccgcttcatgtcccatcttctccaccaacatgcgctttgtcttcattctacattcttttaataagccttctacgaatttacagttggtctgtgcaataactgcaggagagaggtctgacagtttgggttgcctcaggttttttcctaaacttcgtgcctcttgcatatatttctccctcaagtcgttgtccagcccaacatgctcagaatgctggcgaaggcgttctttcctgcgctgtgcagtggcactccgacttacccagcgattgttactggttggtcctgttgccaagacatcggactgtaactttggaaagaacccctgctcatatttgccttgaccaattttcatatcaagtagatgtgggtggattgcagtgtgatccattttcatcagtctctgctcaattgattgggctgcttcttttaaagtgctgcatttctgatatatagatgtccgcaaggtgggtgcccttacattatacagccttatcttatcaatccgagtgtcaaagacccgaagcaaaggatctttctcttcccactgagacataattttattatcaataaaggtggcaaacatctgtgtttcaatgaagcgtgaaagaaatggcaggtaaggctcaggctggtcagacagaaaggaagctttgtcaaagttctgcatctgttcccggttggtcagccaggattccatgtcctgggcagtctgaatgacaaatgcttcgtaatctgcaaacatctgtgtaaaacggttagcaaagacctctcggagctgtacattgagctggtagtcccttagttctgcctcttcacaatgcagttttaaatccttgtctttttcacccagagaagcagagaggtccattttttccacagccacaccagtacgcttggccagagcctgcaagcgggctatggtttcattgcccttcagtaactcatacatgctgatgttattagtacagacattgccgttctttttgtcattgaccaagtctttcagaaccatattcttcagtttgctggtactctcactgcaatgtaggctgccctcaggagggatcccaaattgaacaagaacctcagagagttcttggataaaatccactttattggggaactgtggaaattcttcaggcaactcaataaaatggttgtcaatgtccacaaaacacaaattagcctcttgaggaagttctagtttagaacggtcagttccttcttttgactgaaggcccatcagataagggacaggagcatcaagaaaatgtagcagagaagcaggtagaatgggcacataaacatgttgccattgaaatgggaacaaaagtgtggtgatgccttctgccacagtcatcaggcgttgataatttgtaacttcttcataaaaagtgagaacaaaaccataggtgcgagaaccatcttccctggtaattataaatgagtgaaactgggggtctttattgtccgtttgtgtcctgaaagatagccctttaggcatgcacaacatgttcaccgcatcttgatcaaaagggttccattctatattctgaggatagtgggcgagaactttggatttgaatgttcttctcaaaggactctggtcaaaattttcgcctgaagtcgtatttgcagcaccttggctcttgccatgacgatctgcttctagccattggtacaaaaatcctggctgggcatgttggctcacaactgtaatctcagcacttcgggaggccgaggcaggtgaattgcttgaggtcaggagttcgagaccagcctgatcaacatggtgaaacctcatctctactaaaaatacaaaaat

SEQ ID NO: 11940 - RNA, 7236 nt, Homo sapiens
  source 1..7236: mol_type = other RNA
ctgaatagctgggactacaggtgtgtactgccatgcccaacatgtcttatttctttataactgcacttcttatgtgaccccaaactcagcttaagcatccttttcattgatcaaacttggatcctaaggactatttccaaatatttaaatttattcttaaaggccaagattgactgccattgggaatattcaaaagaatgggggtactggccattcaagcagctcacacaaggagggccccacatgtttatagcacaggctgtatcaacggaataagtacatgggctcacaaggtgactgaaggacccatcatccaagaggatgtgtcagttctgatgtgttttttttaaatcatcatttcaccattatagtaatattacacaaaggcatgaagatgaaacttcaggtgtaacttttttgggggtattactttttaaagtaatggttttattcataggccgcaaatccaactttggctgcagtttttttctttttttttttttgagacggagtctcgctcttgtcacccaggttggagtgcagtggcacaatctcggctcactgcaacctccacctcctgtgtttaaacgattctcctgcttcagcctcctgagtagctggaattacaggccctgccaccacccccccgctaatttttgtctattttttttttttagtagagacggggtttcaccatgttggccagtctggtcttgaactcccgactgacctcagatgaaccacccgcctcagactcccaaagtgtcaggattacaggcgttagccaccgtacctggcctgctcccagtttttacaagatgttaattcccaataatctgagagcaatgtgttaatatgaatattaattcttctaaatgaatattcatccttatttcctacttgtataggtggatgaataaagatccaatagtataatagaaagactattagtaagaatgccggaaggtcagtctcatgcagcctggtgaaataaaacaaacaaacaaacatgaattctagagcttgtgttgtcagtaaccagctgtggggtaagtgtaagatttaatctctctattccttaagtgttcccatccacaaagtaagaaggctggatgaggtgtgtcaatcctagcacattaacctaagtcatcccccaggttgcctagacctgtcaggagcatggccttatgaagatacaaacatgaaatcctgggttggacccctctatagtttctgatcaccaaacacagtaggagcccagtgtaaaacaggttctggatatctcccacgataaacttcccatgtccctggaagagctgtaccattgtagacacactttagcttcaggcaaacaaatttctggtgtacccagaaccattttcttaaaccatttccatgggtttttatttttatctatttattttttgagatggagtcttgctctgttgcccaggctggagggcagtggcgcgatctcagcttactgcaagctccgcctcgcgggttcacgccattctcctgcctcagcctcctgtacaggcacccgccaccacgcccggctaattttttgtatttttagtagagacggggtttcacggtgttagccaggagggtctcaatctcctgaccttgtgatccgcctgcctcggcctcccaaagtgctgggatcataggcgtgagccaccgcacccggctccatgggtttttaaatacagctgtcaactctccttttcctcaagtatgaagtcacatgttaaaagaggctgtccttggctgtgtttgataaagggagttaggcacttgtttcatctgtttcttcctccaggaaataaggttaacaacacaggtggtgaaagcccagcaacctccgattgcacaaggatactgatgccatggctttgcttttcagccacaactgggaataaaactgggagctctgctgaggcaattttgctgctaaaaatgtacaaatgcctaattagagttacaggacctaccagaagatgaggacttacagtaactagccaatactacatttacttaacttctttataaactatcaaactggaaagttactcacaacttttggtctttcaaaattgttgccacctcttgctttgcttccattttgtcagcctgtgctgccagtggcttttagcttctctgggtcagttgttttacattattactccccttcctacaaaggaacgtaaagcttgccctgaaacacccagaaagggttcattctctctctccttctgttatttgcattatcatggtcaacaaatgctttcacaaaaacattccaagccacacacagccctcctcctccttagacattccttccatttcccgaggggggatgggccctggagaggtgggtgattagaccctaacaaagacagggctcatggttatccttaagaggtagaccactgcacagtttagatggccaaattaaaagtacagaatcaaattgctgtttgcagttcttatcactatgaatctaacactgaaattcacatcttcccaaagtacctcaaataacaagaataaaaatgccaagaatgaagttagtctaggctaatctttccgaagtgtaaagaagttataatcccacaattgaacacatttctcagagctttgtatgttctctttccagttcagccaagctcctggggtctagtgtttaaaatactccaattatatcatcttgtgcggactgaaatttttttccaaaagactggaaaagtgactagcgattcaaatatataaaacagtttgtaacttaaaagatagaagtgaagactaccagtacagtaggtaaagctgtgtgcatccacaatacaaaggatcagactccaagatggatggctactacataacaatgcattctgggtttctttgtgatacctggagaaaaaaaaaagcccgactgggttgcactatatttacatgtttactggcttcttcctggctagcaccactcttccccccaacccccaacatttttaagctacttattttaagtcacaggaatattcaatctaagaaaagcatcttattagagtaatataatttcttaaagaagatagcatatttacacacatctaacacatgaaaatactctattttatactaaattccaggttcaaatgaactacaatacaacattttgccttgtctgtagagtgaggattgttccaaatggggcatatgtttggctgcccctgcagtgactcactactgtcagacaagtccaaatcggtcccctagttggggaaggagcaaggtttggactgagagtttctagccagttgggttacacatccactcctttgatgagtgatccttctaggactatggtgaagtcctgaatggtctgcagaattcggataagggagttgacagtcatgcggtctcgcaggagagcgctctcttcatacattcgagtgatggcaggacactcagctaacaatggaatccactgtgggagcaggcgatcccttgttccaaggcaaactaaaatctggaatttgccatccttcccaatgttcctgggtgcagtattaatagcatttacgtagtggcagaaggttttgcaggatgatttctgaataaggacatcatcttcattatctagaatctggtcagttgtttcaaaataagcaaccactttcttgttgttttttcctgtcagtgaagtgatgctcaatctcctagccgtggtgggtgacttctgctggggtggagtccgacactgctttactagatcttcatctgatgctgatgtcatcaactctccaataagaattctctccaggctcccatcatcaatgcctttccccagccaccgcccacatgggaatctgtatgtatgtcctgtgatttcatttctgaccatgacacaatccactagccatttggctaacagtcctgagttatcgtgaccaatctgaacagtggtcagcttccccaagttctggcactcaaaggtcatttcgaggaggtttttgggaatctgcattactcctgtgtctcccagctctcctgatacacagatccaagggtttgatgtgattattgcattgctcagctttttgattgggatgatcactgacctatacggaatcatgatagtggtgaacacactggtgaagcagaaatagtccacagcattgagagaaagaaggtggtaaagaaactgctctctttcttcttcgcaacgtagaaaagcatatcgcttataaagcttcttggtgagtggttggttagaaagcaactgcttaagatgctgggacaagagcttcttttctagagacagtcttatccacgcccgagctcgtccaacatcagtcttgatctcactcatgttttgaatatgcctcatgtcctgaataagagagaccctgagcgttggcaacataactcctgagtcagattttcttctttctggtccgagggcaactggtgattctgcaaggtgctcttgtttctcttctctgtcctgaaattgaattaaatgtgaccacaaagccgacttcccctgcttgacctgcaagccatggctccatatcctctccagcaggtcacaaaggctggcgatcaaggtgttctcctccaggccggtgatgtttgcttctccatggccaagttccaccgcttcatgtcccatcttctccaccaacatgcgctttgtcttcattctacattcttttaataagccttctacgaatttacagttggtctgtgcaataactgcaggagagaggtctgacagtttgggttgcctcaggttttttcctaaacttcgtgcctcttgcatatatttcaggcagcactcagagaaggattttttaggaagtcgtgcaggaggaggtggaccctggtcccactcccagaatgccatggagttctgacagaccaaaagttccccggaaggctccctcaagtcgttgtccagcccaacatgctcagaatgctggcgaaggcgttctttcctgcgctgtgcagtggcactccgacttacccagcgattgttactggttggtcctgttgccaagacatcggactgtaactttggaaagaacccctgctcatatttgccttgaccaattttcatatcaagtagatgtgggtggattgcagtgtgatccattttcatcagtctctgctcaattgattgggctgcttcttttaaagtgctgcatttctgatatatagatgtccgcaaggtgggtgcccttacattatacagccttatcttatcaatccgagtgtcaaagacccgaagcaaaggatctttctcttcccactgagacataattttattatcaataaaggtggcaaacatctgtgtttcaatgaagcgtgaaagaaatggcaggtaaggctcaggctggtcagacagaaaggaagctttgtcaaagttctgcatctgttcccggttggtcagccaggattccatgtcctgggcagtctgaatgacaaatgcttcgtaatctgcaaacatctgtgtaaaacggttagcaaagacctctcggagctgtacattgagctggtagtcccttagttctgcctcttcacaatgcagttttaaatccttgtctttttcacccagagaagcagagaggtccattttttccacagccacaccagtacgcttggccagagcctgcaagcgggctatggtttcattgcccttcagtaactcatacatgctgatgttattagtacagacattgccgttctttttgtcattgaccaagtctttcagaaccatattcttcagtttgctggtactctcactgcaatgtaggctgccctcaggagggatcccaaattgaacaagaacctcagagagttcttggataaaatccactttattggggaactgtggaaattcttcaggcaactcaataaaatggttgtcaatgtccacaaaacacaaattagcctcttgaggaagttctagtttagaacggtcagttccttcttttgactgaaggcccatcagataagggacaggagcatcaagaaaatgtagcagagaagcaggtagaatgggcacataaacatgttgccattgaaatgggaacaaaagtgtggtgatgccttctgccacagtcatcaggcgttgataatcttgtgagtagagaaggatttgcatctctaaaagaacacaggtaaacacctgcaccaggttctctaatcccaggagctcaaatgcctcccgaagggggtaatcagagagggggagttcactgggcccaggcctctggcagatgacaggttcataaacaccataaaatttcagtgacctccctggaggtggaaggggtacttcataaagaatattgtggatatagctttcaagtggcaagggtggtggctgctgtgaggtaacagccttgtaaagctggataaggaatttcttgcaggcctgcatgaatggtaacggtgtgatcaagcatatactttttgaaacatacagggtgtctctgctaatatcataggagttgtatcgctggagtttcaaaagggaagttgtatctccttcatcaagactacttgccaatgagtccatactgcaggaagatgaagcatacacactgctgtaatgctcagcgttgtgcatctggtaaagtgtctgcattgctgtgcagatttgcttacttgtaacttcttcataaaaagtgagaacaaaaccataggtgcgagaaccatcttccctggtaattataaatgagtgaaactgggggtctttattgtccgtttgtgtcctgaaagatagccctttaggcatgcacaacatgttcaccgcatcttgatcaaaagggttccattctatattctgaggatagtgggcgagaactttggatttgaatgttcttctcaaaggactctggtcaaaattttcgcctgaagtcgtatttgcagcaccttggctcttgccatgacgatctgcttctagccattggtacaaaaccgccagctcgtcaggctccagcccgctgtccgcgtcgatcccgcacagcacgaagtagtgcgcgaagcggcaggcggccggggaggagcccgagcccgggccgggcgccgcgcagctcccgctcatcccggccgcgctgctccaggggccgccgccgccgccgcccgggaaggctttctgcggaggctgccaccaccgctccggctgtggtctgtgcgcccgccctagggcgacactggcgcgcccat

SEQ ID NO: 11941 - RNA, 847 nt, Homo sapiens
  source 1..847: mol_type = other RNA
ctgaatagctgggactacaggtgtgtgacaccatgactggctattttattttatttttgtagagatggaatctcacaatattgcccaggctgatctcaaactcttgggctcaagcagtcctctcgcgtcagcctaccaaagtgctgggattacaggcatgagccaccacgcccagccagattacaaaatactttgacatcttttctctacagccctcaaaaggaggcagggcaagcacaattaaatcccattacaaatggggtgactgaagctccattcatggcttgcccagggtcacacaaagaatgaatagcagagccctgagcctgtgtgcttccctctgtgccaggctgctttacccaggcatgggtgcaccttgtgcatgggacatttctcctttgttgtgtcctgagtaccttaagccactcagatattgctcaggtggagtgaggggaaaatgttttcaggttgtattagtcaaaacaaaataccacacactgggcgactttaaaatcatacatttatccctcacagttctggaggcttggaagtccaagttcaaggtggcagctggacgggttcccggtgagggctctcttcctggtttgcagacagccaccttctcttcgcatcctcactctggtaaggggaccacccgctgcagccagcgagacagtggcatgttcttgttacaactcgatctaactcccccagaagaggaggcagggaaggcggacaaaaccattgaacacgagctgcccaactccgccttgcttccccattcctggcgaccactgcttctgtctctgtgaattttgactattctaggcacttcacaaaactggac

SEQ ID NO: 11942 - RNA, 855 nt, Homo sapiens
  source 1..855: mol_type = other RNA
ctgaatagctgggactacaggtgtgtgacaccatgactggctattttattttatttttgtagagatggaatctcacaatattgcccaggctgatctcaaactcttgggctcaagcagtcctctcgcgtcagcctaccaaagtgctgggattacaggcatgagccaccacgcccagccagattacaaaatactttgacatcttttctctacagccctcaaaaggaggcagggcaagcacaattaaatcccattacaaatggggtgactgaagctccattcatggcttgcccagggtcacacaaagaatgaatagcagagccctgagcctgtgtgcttccctctgtgccaggctgctttacccaggcatgggtgcaccttgtgcatgggacatttctcctttgttgtgtcctgagtaccttaagccactcagatattgctcaggtggagtgaggggaaaatgttttcaggttgtattagtcaaaacaaaataccacacactgggcgactttaaaatcatacatttatccctcacagttctggaggcttggaagtccaagttcaaggtggcagctggacgggttcccggtgagggctctcttcctggtttgcagacagccaccttctcttcgcatcctcactctggtaaggggaccacccgctgcagccagcgagacagtggcatgttcttgttacaactcgatctaactcccccagaagaggaggcagggaaggcggacaaaaccattgaacacgagctgcccaactccgccttgcttccccattcctggcgaccactgcttctgtctctgtgaattttgactattctaggcacttcacaaaactggactcatacga

SEQ ID NO: 11943 - RNA, 7703 nt, Homo sapiens
  source 1..7703: mol_type = other RNA
ctgaatagctgggactacaggtgtgtgcaactatgcccagttaatttttgtttttgctttttttttttttttttttttggtagagatggggtttcaccatgttgccaaggctagtctcaaactcctgggttcaaatgatctgcttaccgcagtctcccgaagtgctgggattacaggtgtgagccaccatgcccagggtttcagtgtcaaactctgaatttgaatgacaatgtcaaactgagaaacaggatgaaatgcacaaaagtaatgtgtaaattgagtagctgacatcagttgacagataaaagtaatgacagtatataagcgtcaggtgaatgttcaaggaataggaaacaacattgtcaggacgtctgtttggaaaaaaacccttaaaagtaaaattacatacatcagattttatctagatattaaactgatgctgctgaggcaggaggatcacttgaagacaggtgtttgagaccagcatgggcaacaaaatgagatcccacttctaataaaattaaaaacaaacaaaaaaaagcttatgccagtatacatgtcagtgatctaagctctggctacataattgaatttcttcaatttgacaagtcaaaaaattgcgactgctgcacaggacacctcactgttacttcatgtgcaagtcagagatttgaaaagaggcattagagatgggggaagaaggcaatgtctaaatggaccttttctgtgccaggattcttctttaaaggctttcttttctgaaacgttttgacttgttcatcactgaatgaggaacaatagtgttttaaattcaaattgtcccatgagttgagatttcttttattaggaaatatacaatttataattgtgactttaatttttaaaaattaccttccagaaaatatcccctctcagcatcaagtattggctttgaatttgggtgagcctttacttgctcaaacctccactatcctaatttctttattacattctaattggtattgacagatttgatagattatcatcttttctaaattccacttgtgtaaatcctactttaatattacaaagcaattggcacgagattcaagtaaaataaaagcatggttgataaaaaagaagaccaaaactgttatcattcttcttaagcccgttttaaaattacatgtttagattttttaaaaaattcatgcgattctcctgtttcagcctccacggatgctgcagtgagctgagactatgtcgctgcactccagcctgggcgacagagccaggactctgtcttaaaaaaaaaaaaatcaaatatacagaagagtataaaggggaagtacgattctcctgcctcagcctccctagtagctgggattacaggtgtgtgccaccatgcccagctaatttttttgtatttttaatagagacagggttttgccatcttggtcaagctggtcttgaactcctgggctcaagtgatccgccttcattggcctcccaaagtgctgagattataggcgtgagccaccacacccatcctaaaactaaaattttatgttcagttcctcacactagctattatttcaactgctcaacaaccccatgaggctaaaggctatcacactgggagtgcggataccaagcatcccatcatcacagcaagttcactggacagtgctgctcggtggtaaccacagctgagcacctgcatgtttgtttgtttttttatcagatacatgatttttcaaaaatttttctcccattctgagggttaacttcactttcttaatggtgtcctttaaggcgctaaagttaattttgatgaagtcccatttatctactgtttgcctttgttgcttgtgcttttggtattatgtctaagaaaccattcctaagcccaacatcacaaagatttacttctgttttcttctaagagtttaaactcttatattgaggtctatgatccattttgagttagaatttgtaatgtggtaggaaggtagggatccttttgctgtgcacgtagctaccagttagttgtcccagcaccgtttgttgaaaagaccactccttctctattgatggtattggcatccttgttgaaaacaagttgaccagaaatgtatgggtttatttctggatgttcagttccattcctctgatcgatatgtctatccatatgcctacactgtcttattgtagcttggtagcactttttgaaattggtacgtcttccaactttgttcttttccaaggttttttggctattctgggtcccctgcgtttccctaccaattttaccagtttgtcaatttctgcaaaaaatacagctaggattttgataggaattgttgaatatgtagactaatttgggcagcattgccatcttaccaatattcagtcttccaatccatgaacatggatgtctttccatttatctggatcttaatttctttaaacgtgttggagttttattcttgatgctactgtatataggatttctttattctcattttcagaatgtttgctgttagtagagaaataaaactgatcttgtatcctgcaacctgttgaactcatttattactttttatggattctttagcattttctatatacaactatgtatcaactgtgaatacatatagtttcacttcttttgcagtataaacctcttttctttattagcttatttgatttttagatgttgaacaaaccttgaattcctaacctaactgctgtggctagaacttcaagtacaatgctgaatagaagtagtgccgagtgaacatccttgtccttcttcccaatcttaaggggaaaacattcagccttcagtctatcaccatgaagtataatgttaggtgtgggcttttcatagatgttatatttatcatatctaggaagattccttttattcctaagtttgttgagtgtttttatgaaagagttttggattttatcaaatgctgtaataagacaatctgtgtgggttttgtgctttattaaatatggtacagttgatcctcattattcaaggttatgtatttgtgaatttaccaacttgctaaaatttataaccctcaaattgatatccgtggcacttttgcagtcatttgtggatatgtgtaaatgggtgaaaaatttgagtcacccagtacacatgttcccagctgaggctgaacaagatgatgctctgccttcctgcttcagtctcatagagaaatgactggagggtggaaatggcaggggcaattctgtgtagtacaagaagctctggctccggggccagctggatggggtttgaatttcagctctgacacctgttaggggggtgcctcaggcatgtcacttaacacttctgatacctcactttcacttctgtaaaataaggtagaatttgctaggatgaattaagaattcaagctcataatgtgtgtgagataaacatatgtatacacacatatacacaaatacactttctcctaaaagcagttgttccatatttaattcagtgtttatgggagaatattctgtagaacataattactgtgaataatgagaactgactgtatattagcttatttgatttttagatgttgaaccaaccttgaattcctgggataaattccacttggtcatgatatagaatcctttttataggttgctggattcagtttgctaatatttttgttaatgatttttgtgtttgtattaataaggaatattggcttatagttttcttgtgatgtctagtctagtatcagggtaatactgacctagagtaagttgggaagtgttctttcctctcctacttttagaaacagtgtgcaaaaaattagtgctaattttaatgtttggcagaattcaacaatgcagccatctaggcctgggattttctttgtgagacttttaaaattactaattcagtatttttccttgttaatgccaattgcatttttaaccaacttttaggtagagccaaagataagagtattatctcattaggccagtgaaattcaagaagaaaatacatattatcaaggaagatgctaaatatttgggaaattctgataggcagctatgaaaattatccattatatcttgattcttaacctctatctagctttaacaaacattttatcacttctcatgtggtttcataatcttatgaacaagaaatttcagcctgttctataacagatttatatacaaacctcttaactaaaacttgcagtgaagtccttataatcaaaaactaaagtttgtacattccttgagataatacacagatatgtatctgtatatatttatatatatataaatatatttcactctatctacaaacataacacttatctcagaacctgtcaggaaggcagttgtgtagtggaaaaaatactggaatagatttctggaggtctcagttctggtgccagctctaacttagatgcctttctgtgtttcttccatggataaaattaggttatgcctggtgatcggcaaggttctttctggtgttaaaaatacaatgacttattctacaataatgccattcccattgctcttacttcagagtggtcacaatgaaaatattttgttatatacatataaacatacacacctccatacttcatttgtatagaactattcaaccaattcacaaaatcttagaaagaggaagtctgtaattaaataatgtaatttcaacatctcaaagtcctgaagtttgctatgaaacagttactactattctttctctacatatacaaatttgccttttcacaatgtctcactttatgtaagtgcagtactatttcacaggcatctaaaattatgctaactttcaaaaacaaggaggtcatttttcagaaattctgagcctgtcagagaaactaaatggtatttcatcagttgtctctactggcacattacttctactaaaatgacatgaagcatggtgagcgaaacttgaaataaatgcatctggagtccggctgcaatgacagctatctgctggtgtaacattacttggattaccaggatgtgaatggtaaacaccatggaatgggtcttgcaatgagtgataatgccctgctcctcctgaggtggctgcagaactctggtaaggaccattagacataagacaagtttgaaagcaagtcttccttcccaaacctcgatgcatgtctaatttagcaatgagaggtttcccaacattcacttcctgcttgtcctctacagtatcttccaatcctgagtactgatatgataaacatactgtgaagactagatgttcctttaatttttgcagtgaactgagtctggtatagaggcaatgcttgggaagatcctttgataccaagtagctgccagtttcttcaggtgtgcctttatttgcatcttttggatcaatatctagatcaagtggaaaatcagtaacgtaggcatcacacattattatctccggtggtttgtaaactatacttgtatagatgatcatgacattggaaaactcagctgcaaatcctaattgaatctgaacaccacagtcaaacttaagacacatactttctggaagttcatgagccttggcccactgtagattccgcacaagagattcagcagaatattctgttccctgtattggatcagtaagtgctctcttctcagataaactacttcgaatctctagagcctgtttgcctttggtaaggtgacacttacccatatcttctgcaacttcatccagtaacacagtgattttcttatcttctaataatctgtcttttaaaaatttcataaagattccatttgccaatccagaatgctggatttcaaaagcttctgctccttgacacctgtaatcccagcgactcagaaggctgaggcaggaggatcgcttgagcccaggagcagtgagctatgatggcgcctctgcactccagcctgggtgacagagttaagacccctgctcctaaaaagcaaaaacaaaaagacatcaaacaataaaggaaacttcaacgtaaacatcaaatgttcttacgtggcatatccaaacacaatattggcggtgacttttagtgcatccaagattggaatggtatcatcgtagtcatttcttttcctacacatatccaataagaacacattaagtccagtttctttttcttgcatcaatttcagtatattttgtacacacagacaattttcagacctatatggatttggagcatcaacggggaccatgaagctgttcccaaaattttcataaccatgtcctgcataatataataacccatatactcccttgtctaaaaggagtaaaaactcatccacagcattacgcatctcatattcagtaagatccaacagtgaaaccactttgaagtccagctgtctcagtaagttagtcaattcgtacacatccaccaaaggagctttgagcttggggtgctcccggtaattcatatttcctatcaaaagggcaaccttgtccttcgccaaaggctggtcagttgtttgctctttattatcaggatgaccaagattatttaattcatctatgatgatttctaccttcttgctatcttgactgtctcgatcattatatacatgacaccagtaggttccttggtgttccaaatccacataaggcaccatgtatagctttttggtctcatgtgttaatggtaattcatttttgaaccactggtagtgaggaatagggcttccaacagcaacacactgtaaaaccaatgtgctgcctggcatcagcttttgggaagttggttcaacacagatttgcaacttggattcagagacgccatcaacacttctctggaagctctctgggatgtcgcaaacatccagctgtgaccactggctgaattcaaaggtgaaattgttattaactcgacagacataaaagcctgcatcttttacatgcactgcattaaaaataagctctgatgtatttccatttggaatctctttattcattttgaaccactgatattgaacaaaaggatgtccagttgcccggcaacacagtttcacaaactgtccagccaagactgcctttgactctgggtttacagtaatctttattcctggggggctgagaagctgaagaacttcagtgtgttccatagcctgcaggaaatcactcaattctgtgactgtgcaacctttttcacccattaacttcagcagacacaggctggggcttccttcaggctccagtaccttaagagaacactgctccaggtctaggcaactgaggcggaggcgcccgcgactccccgccagctccgccagtctcctccagccccggccctcgggcgcctgatccaggagctcgctgagcctccgcagcagcggctcccgcaggcggttgagggtcgcgccggccggaggggcgagcagcggccccgtgggggcggccgagggcggcagggcctgtagcgggtcccccaacagcgacatggccctcgccggcgaccccggactgccggggctcccgcccgccccgtcacgggcctcggccccggggcaccttccgctcgcctccgagccgcggaggcaggggcggaagaacaaatctggcagcgcggcacggccctcagaggaggaagctccgctccccgccccaattagacaggtttgccgaggggagcctggcctgctggccgcgccagccgcgcaaaggg

SEQ ID NO: 11944 - RNA, 7736 nt, Homo sapiens
  source 1..7736: mol_type = other RNA
ctgaatagctgggactacaggtgtgtgcaactatgcccagttaatttttgtttttgctttttttttttttttttttttggtagagatggggtttcaccatgttgccaaggctagtctcaaactcctgggttcaaatgatctgcttaccgcagtctcccgaagtgctgggattacaggtgtgagccaccatgcccagggtttcagtgtcaaactctgaatttgaatgacaatgtcaaactgagaaacaggatgaaatgcacaaaagtaatgtgtaaattgagtagctgacatcagttgacagataaaagtaatgacagtatataagcgtcaggtgaatgttcaaggaataggaaacaacattgtcaggacgtctgtttggaaaaaaacccttaaaagtaaaattacatacatcagattttatctagatattaaactgatgctgctgaggcaggaggatcacttgaagacaggtgtttgagaccagcatgggcaacaaaatgagatcccacttctaataaaattaaaaacaaacaaaaaaaagcttatgccagtatacatgtcagtgatctaagctctggctacataattgaatttcttcaatttgacaagtcaaaaaattgcgactgctgcacaggacacctcactgttacttcatgtgcaagtcagagatttgaaaagaggcattagagatgggggaagaaggcaatgtctaaatggaccttttctgtgccaggattcttctttaaaggctttcttttctgaaacgttttgacttgttcatcactgaatgaggaacaatagtgttttaaattcaaattgtcccatgagttgagatttcttttattaggaaatatacaatttataattgtgactttaatttttaaaaattaccttccagaaaatatcccctctcagcatcaagtattggctttgaatttgggtgagcctttacttgctcaaacctccactatcctaatttctttattacattctaattggtattgacagatttgatagattatcatcttttctaaattccacttgtgtaaatcctactttaatattacaaagcaattggcacgagattcaagtaaaataaaagcatggttgataaaaaagaagaccaaaactgttatcattcttcttaagcccgttttaaaattacatgtttagattttttaaaaaattcatgcgattctcctgtttcagcctccacggatgctgcagtgagctgagactatgtcgctgcactccagcctgggcgacagagccaggactctgtcttaaaaaaaaaaaaatcaaatatacagaagagtataaaggggaagtacgattctcctgcctcagcctccctagtagctgggattacaggtgtgtgccaccatgcccagctaatttttttgtatttttaatagagacagggttttgccatcttggtcaagctggtcttgaactcctgggctcaagtgatccgccttcattggcctcccaaagtgctgagattataggcgtgagccaccacacccatcctaaaactaaaattttatgttcagttcctcacactagctattatttcaactgctcaacaaccccatgaggctaaaggctatcacactgggagtgcggataccaagcatcccatcatcacagcaagttcactggacagtgctgctcggtggtaaccacagctgagcacctgcatgtttgtttgtttttttatcagatacatgatttttcaaaaatttttctcccattctgagggttaacttcactttcttaatggtgtcctttaaggcgctaaagttaattttgatgaagtcccatttatctactgtttgcctttgttgcttgtgcttttggtattatgtctaagaaaccattcctaagcccaacatcacaaagatttacttctgttttcttctaagagtttaaactcttatattgaggtctatgatccattttgagttagaatttgtaatgtggtaggaaggtagggatccttttgctgtgcacgtagctaccagttagttgtcccagcaccgtttgttgaaaagaccactccttctctattgatggtattggcatccttgttgaaaacaagttgaccagaaatgtatgggtttatttctggatgttcagttccattcctctgatcgatatgtctatccatatgcctacactgtcttattgtagcttggtagcactttttgaaattggtacgtcttccaactttgttcttttccaaggttttttggctattctgggtcccctgcgtttccctaccaattttaccagtttgtcaatttctgcaaaaaatacagctaggattttgataggaattgttgaatatgtagactaatttgggcagcattgccatcttaccaatattcagtcttccaatccatgaacatggatgtctttccatttatctggatcttaatttctttaaacgtgttggagttttattcttgatgctactgtatataggatttctttattctcattttcagaatgtttgctgttagtagagaaataaaactgatcttgtatcctgcaacctgttgaactcatttattactttttatggattctttagcattttctatatacaactatgtatcaactgtgaatacatatagtttcacttcttttgcagtataaacctcttttctttattagcttatttgatttttagatgttgaacaaaccttgaattcctaacctaactgctgtggctagaacttcaagtacaatgctgaatagaagtagtgccgagtgaacatccttgtccttcttcccaatcttaaggggaaaacattcagccttcagtctatcaccatgaagtataatgttaggtgtgggcttttcatagatgttatatttatcatatctaggaagattccttttattcctaagtttgttgagtgtttttatgaaagagttttggattttatcaaatgctgtaataagacaatctgtgtgggttttgtgctttattaaatatggtacagttgatcctcattattcaaggttatgtatttgtgaatttaccaacttgctaaaatttataaccctcaaattgatatccgtggcacttttgcagtcatttgtggatatgtgtaaatgggtgaaaaatttgagtcacccagtacacatgttcccagctgaggctgaacaagatgatgctctgccttcctgcttcagtctcatagagaaatgactggagggtggaaatggcaggggcaattctgtgtagtacaagaagctctggctccggggccagctggatggggtttgaatttcagctctgacacctgttaggggggtgcctcaggcatgtcacttaacacttctgatacctcactttcacttctgtaaaataaggtagaatttgctaggatgaattaagaattcaagctcataatgtgtgtgagataaacatatgtatacacacatatacacaaatacactttctcctaaaagcagttgttccatatttaattcagtgtttatgggagaatattctgtagaacataattactgtgaataatgagaactgactgtatattagcttatttgatttttagatgttgaaccaaccttgaattcctgggataaattccacttggtcatgatatagaatcctttttataggttgctggattcagtttgctaatatttttgttaatgatttttgtgtttgtattaataaggaatattggcttatagttttcttgtgatgtctagtctagtatcagggtaatactgacctagagtaagttgggaagtgttctttcctctcctacttttagaaacagtgtgcaaaaaattagtgctaattttaatgtttggcagaattcaacaatgcagccatctaggcctgggattttctttgtgagacttttaaaattactaattcagtatttttccttgttaatgccaattgcatttttaaccaacttttaggtagagccaaagataagagtattatctcattaggccagtgaaattcaagaagaaaatacatattatcaaggaagatgctaaatatttgggaaattctgataggcagctatgaaaattatccattatatcttgattcttaacctctatctagctttaacaaacattttatcacttctcatgtggtttcataatcttatgaacaagaaatttcagcctgttctataacagatttatatacaaacctcttaactaaaacttgcagtgaagtccttataatcaaaaactaaagtttgtacattccttgagataatacacagatatgtatctgtatatatttatatatatataaatatatttcactctatctacaaacataacacttatctcagaacctgtcaggaaggcagttgtgtagtggaaaaaatactggaatagatttctggaggtctcagttctggtgccagctctaacttagatgcctttctgtgtttcttccatggataaaattaggttatgcctggtgatcggcaaggttctttctggtgttaaaaatacaatgacttattctacaataatgccattcccattgctcttacttcagagtggtcacaatgaaaatattttgttatatacatataaacatacacacctccatacttcatttgtatagaactattcaaccaattcacaaaatcttagaaagaggaagtctgtaattaaataatgtaatttcaacatctcaaagtcctgaagtttgctatgaaacagttactactattctttctctacatatacaaatttgccttttcacaatgtctcactttatgtaagtgcagtactatttcacaggcatctaaaattatgctaactttcaaaaacaaggaggtcatttttcagaaattctgagcctgtcagagaaactaaatggtatttcatcagttgtctctactggcacattacttctactaaaatgacatgaagcatggtgagcgaaacttgaaataaatgcatctggagtccggctgcaatgacagctatctgctggtgtaacattacttggattaccaggatgtgaatggtaaacaccatggaatgggtcttgcaatgagtgataatgccctgctcctcctgaggtggctgcagaactctggtaaggaccattagacataagacaagtttgaaagcaagtcttccttcccaaacctcgatgcatgtctaatttagcaatgagaggtttcccaacattcacttcctgcttgtcctctacagtatcttccaatcctgagtactgatatgataaacatactgtgaagactagatgttcctttaatttttgcagtgaactgagtctggtatagaggcaatgcttgggaagatcctttgataccaagtagctgccagtttcttcaggtgtgcctttatttgcatcttttggatcaatatctagatcaagtggaaaatcagtaacgtaggcatcacacattattatctccggtggtttgtaaactatacttgtatagatgatcatgacattggaaaactcagctgcaaatcctaattgaatctgaacaccacagtcaaacttaagacacatactttctggaagttcatgagccttggcccactgtagattccgcacaagagattcagcagaatattctgttccctgtattggatcagtaagtgctctcttctcagataaactacttcgaatctctagagcctgtttgcctttggtaaggtgacacttacccatatcttctgcaacttcatccagtaacacagtgattttcttatcttctaataatctgtcttttaaaaatttcataaagattccatttgccaatccagaatgctggatttcaaaagcttctgctccttgacacctgtaatcccagcgactcagaaggctgaggcaggaggatcgcttgagcccaggagcagtgagctatgatggcgcctctgcactccagcctgggtgacagagttaagacccctgctcctaaaaagcaaaaacaaaaagacatcaaacaataaaggaaacttcaacgtaaacatcaaatgttcttacgtggcatatccaaacacaatattggcggtgacttttagtgcatccaagattggaatggtatcatcgtagtcatttcttttcctacacatatccaataagaacacattaagtccagtttctttttcttgcatcaatttcagtatattttgtacacacagacaattttcagacctatatggatttggagcatcaacggggaccatgaagctgttcccaaaattttcataaccatgtcctgcataatataataacccatatactcccttgtctaaaaggagtaaaaactcatccacagcattacgcatctcatattcagtaagatccaacagtgaaaccactttgaagtccagctgtctcagtaagttagtcaattcgtacacatccaccaaaggagctttgagcttggggtgctcccggtaattcatatttcctatcaaaagggcaaccttgtccttcgccaaaggctggtcagttgtttgctctttattatcaggatgaccaagattatttaattcatcttcagtgcactccactgcctcatctgttcttcctatgatgatttctaccttcttgctatcttgactgtctcgatcattatatacatgacaccagtaggttccttggtgttccaaatccacataaggcaccatgtatagctttttggtctcatgtgttaatggtaattcatttttgaaccactggtagtgaggaatagggcttccaacagcaacacactgtaaaaccaatgtgctgcctggcatcagcttttgggaagttggttcaacacagatttgcaacttggattcagagacgccatcaacacttctctggaagctctctgggatgtcgcaaacatccagctgtgaccactggctgaattcaaaggtgaaattgttattaactcgacagacataaaagcctgcatcttttacatgcactgcattaaaaataagctctgatgtatttccatttggaatctctttattcattttgaaccactgatattgaacaaaaggatgtccagttgcccggcaacacagtttcacaaactgtccagccaagactgcctttgactctgggtttacagtaatctttattcctggggggctgagaagctgaagaacttcagtgtgttccatagcctgcaggaaatcactcaattctgtgactgtgcaacctttttcacccattaacttcagcagacacaggctggggcttccttcaggctccagtaccttaagagaacactgctccaggtctaggcaactgaggcggaggcgcccgcgactccccgccagctccgccagtctcctccagccccggccctcgggcgcctgatccaggagctcgctgagcctccgcagcagcggctcccgcaggcggttgagggtcgcgccggccggaggggcgagcagcggccccgtgggggcggccgagggcggcagggcctgtagcgggtcccccaacagcgacatggccctcgccggcgaccccggactgccggggctcccgcccgccccgtcacgggcctcggccccggggcaccttccgctcgcctccgagccgcggaggcaggggcggaagaacaaatctggcagcgcggcacggccctcagaggaggaagctccgctccccgccccaattagacaggtttgccgaggggagcctggcctgctggccgcgccagccgcgcaaaggg

SEQ ID NO: 11945 - RNA, 7650 nt, Homo sapiens
  source 1..7650: mol_type = other RNA
ctgaatagctgggactacaggtgtgtgcaactatgcccagttaatttttgtttttgctttttttttttttttttttttggtagagatggggtttcaccatgttgccaaggctagtctcaaactcctgggttcaaatgatctgcttaccgcagtctcccgaagtgctgggattacaggtgtgagccaccatgcccagggtttcagtgtcaaactctgaatttgaatgacaatgtcaaactgagaaacaggatgaaatgcacaaaagtaatgtgtaaattgagtagctgacatcagttgacagataaaagtaatgacagtatataagcgtcaggtgaatgttcaaggaataggaaacaacattgtcaggacgtctgtttggaaaaaaacccttaaaagtaaaattacatacatcagattttatctagatattaaactgatgctgctgaggcaggaggatcacttgaagacaggtgtttgagaccagcatgggcaacaaaatgagatcccacttctaataaaattaaaaacaaacaaaaaaaagcttatgccagtatacatgtcagtgatctaagctctggctacataattgaatttcttcaatttgacaagtcaaaaaattgcgactgctgcacaggacacctcactgttacttcatgtgcaagtcagagatttgaaaagaggcattagagatgggggaagaaggcaatgtctaaatggaccttttctgtgccaggattcttctttaaaggctttcttttctgaaacgttttgacttgttcatcactgaatgaggaacaatagtgttttaaattcaaattgtcccatgagttgagatttcttttattaggaaatatacaatttataattgtgactttaatttttaaaaattaccttccagaaaatatcccctctcagcatcaagtattggctttgaatttgggtgagcctttacttgctcaaacctccactatcctaatttctttattacattctaattggtattgacagatttgatagattatcatcttttctaaattccacttgtgtaaatcctactttaatattacaaagcaattggcacgagattcaagtaaaataaaagcatggttgataaaaaagaagaccaaaactgttatcattcttcttaagcccgttttaaaattacatgtttagattttttaaaaaattcatgcgattctcctgtttcagcctccacggatgctgcagtgagctgagactatgtcgctgcactccagcctgggcgacagagccaggactctgtcttaaaaaaaaaaaaatcaaatatacagaagagtataaaggggaagtacgattctcctgcctcagcctccctagtagctgggattacaggtgtgtgccaccatgcccagctaatttttttgtatttttaatagagacagggttttgccatcttggtcaagctggtcttgaactcctgggctcaagtgatccgccttcattggcctcccaaagtgctgagattataggcgtgagccaccacacccatcctaaaactaaaattttatgttcagttcctcacactagctattatttcaactgctcaacaaccccatgaggctaaaggctatcacactgggagtgcggataccaagcatcccatcatcacagcaagttcactggacagtgctgctcggtggtaaccacagctgagcacctgcatgtttgtttgtttttttatcagatacatgatttttcaaaaatttttctcccattctgagggttaacttcactttcttaatggtgtcctttaaggcgctaaagttaattttgatgaagtcccatttatctactgtttgcctttgttgcttgtgcttttggtattatgtctaagaaaccattcctaagcccaacatcacaaagatttacttctgttttcttctaagagtttaaactcttatattgaggtctatgatccattttgagttagaatttgtaatgtggtaggaaggtagggatccttttgctgtgcacgtagctaccagttagttgtcccagcaccgtttgttgaaaagaccactccttctctattgatggtattggcatccttgttgaaaacaagttgaccagaaatgtatgggtttatttctggatgttcagttccattcctctgatcgatatgtctatccatatgcctacactgtcttattgtagcttggtagcactttttgaaattggtacgtcttccaactttgttcttttccaaggttttttggctattctgggtcccctgcgtttccctaccaattttaccagtttgtcaatttctgcaaaaaatacagctaggattttgataggaattgttgaatatgtagactaatttgggcagcattgccatcttaccaatattcagtcttccaatccatgaacatggatgtctttccatttatctggatcttaatttctttaaacgtgttggagttttattcttgatgctactgtatataggatttctttattctcattttcagaatgtttgctgttagtagagaaataaaactgatcttgtatcctgcaacctgttgaactcatttattactttttatggattctttagcattttctatatacaactatgtatcaactgtgaatacatatagtttcacttcttttgcagtataaacctcttttctttattagcttatttgatttttagatgttgaacaaaccttgaattcctaacctaactgctgtggctagaacttcaagtacaatgctgaatagaagtagtgccgagtgaacatccttgtccttcttcccaatcttaaggggaaaacattcagccttcagtctatcaccatgaagtataatgttaggtgtgggcttttcatagatgttatatttatcatatctaggaagattccttttattcctaagtttgttgagtgtttttatgaaagagttttggattttatcaaatgctgtaataagacaatctgtgtgggttttgtgctttattaaatatggtacagttgatcctcattattcaaggttatgtatttgtgaatttaccaacttgctaaaatttataaccctcaaattgatatccgtggcacttttgcagtcatttgtggatatgtgtaaatgggtgaaaaatttgagtcacccagtacacatgttcccagctgaggctgaacaagatgatgctctgccttcctgcttcagtctcatagagaaatgactggagggtggaaatggcaggggcaattctgtgtagtacaagaagctctggctccggggccagctggatggggtttgaatttcagctctgacacctgttaggggggtgcctcaggcatgtcacttaacacttctgatacctcactttcacttctgtaaaataaggtagaatttgctaggatgaattaagaattcaagctcataatgtgtgtgagataaacatatgtatacacacatatacacaaatacactttctcctaaaagcagttgttccatatttaattcagtgtttatgggagaatattctgtagaacataattactgtgaataatgagaactgactgtatattagcttatttgatttttagatgttgaaccaaccttgaattcctgggataaattccacttggtcatgatatagaatcctttttataggttgctggattcagtttgctaatatttttgttaatgatttttgtgtttgtattaataaggaatattggcttatagttttcttgtgatgtctagtctagtatcagggtaatactgacctagagtaagttgggaagtgttctttcctctcctacttttagaaacagtgtgcaaaaaattagtgctaattttaatgtttggcagaattcaacaatgcagccatctaggcctgggattttctttgtgagacttttaaaattactaattcagtatttttccttgttaatgccaattgcatttttaaccaacttttaggtagagccaaagataagagtattatctcattaggccagtgaaattcaagaagaaaatacatattatcaaggaagatgctaaatatttgggaaattctgataggcagctatgaaaattatccattatatcttgattcttaacctctatctagctttaacaaacattttatcacttctcatgtggtttcataatcttatgaacaagaaatttcagcctgttctataacagatttatatacaaacctcttaactaaaacttgcagtgaagtccttataatcaaaaactaaagtttgtacattccttgagataatacacagatatgtatctgtatatatttatatatatataaatatatttcactctatctacaaacataacacttatctcagaacctgtcaggaaggcagttgtgtagtggaaaaaatactggaatagatttctggaggtctcagttctggtgccagctctaacttagatgcctttctgtgtttcttccatggataaaattaggttatgcctggtgatcggcaaggttctttctggtgttaaaaatacaatgacttattctacaataatgccattcccattgctcttacttcagagtggtcacaatgaaaatattttgttatatacatataaacatacacacctccatacttcatttgtatagaactattcaaccaattcacaaaatcttagaaagaggaagtctgtaattaaataatgtaatttcaacatctcaaagtcctgaagtttgctatgaaacagttactactattctttctctacatatacaaatttgccttttcacaatgtctcactttatgtaagtgcagtactatttcacaggcatctaaaattatgctaactttcaaaaacaaggaggtcatttttcagaaattctgagcctgtcagagaaactaaatggtatttcatcagttgtctctactggcacattacttctactaaaatgacatgaagcatggtgagcgaaacttgaaataaatgcatctggagtccggctgcaatgacagctatctgctggtgtaacattacttggattaccaggatgtgaatggtaaacaccatggaatgggtcttgcaatgagtgataatgccctgctcctcctgaggtggctgcagaactctggtaaggaccattagacataagacaagtttgaaagcaagtcttccttcccaaacctcgatgcatgtctaatttagcaatgagaggtttcccaacattcacttcctgcttgtcctctacagtatcttccaatcctgagtactgatatgataaacatactgtgaagactagatgttcctttaatttttgcagtgaactgagtctggtatagaggcaatgcttgggaagatcctttgataccaagtagctgccagtttcttcaggtgtgcctttatttgcatcttttggatcaatatctagatcaagtggaaaatcagtaacgtaggcatcacacattattatctccggtggtttgtaaactatacttgtatagatgatcatgacattggaaaactcagctgcaaatcctaattgaatctgaacaccacagtcaaacttaagacacatactttctggaagttcatgagccttggcccactgtagattccgcacaagagattcagcagaatattctgttccctgtattggatcagtaagtgctctcttctcagataaactacttcgaatctctagagcctgtttgcctttggtaaggtgacacttacccatatcttctgcaacttcatccagtaacacagtgattttcttatcttctaataatctgtcttttaaaaatttcataaagattccatttgccaatccagaatgctggatttcaaaagcttctgctccttgacacgtggcatatccaaacacaatattggcggtgacttttagtgcatccaagattggaatggtatcatcgtagtcatttctccaaacatctgcttcggctactcattccatgtctggaagaccaggactgactagtgagcagagatcccaactccatgggtgttggttttgttaattccttttcctacacatatccaataagaacacattaagtccagtttctttttcttgcatcaatttcagtatattttgtacacacagacaattttcagacctatatggatttggagcatcaacggggaccatgaagctgttcccaaaattttcataaccatgtcctgcataatataataacccatatactcccttgtctaaaaggagtaaaaactcatccacagcattacgcatctcatattcagtaagatccaacagtgaaaccactttgaagtccagctgtctcagtaagttagtcaattcgtacacatccaccaaaggagctttgagcttggggtgctcccggtaattcatatttcctatcaaaagggcaaccttgtccttcgccaaaggctggtcagttgtttgctctttattatcaggatgaccaagattatttaattcatcttcagtgcactccactgcctcatctgttcttcctatgatgatttctaccttcttgctatcttgactgtctcgatcattatatacatgacaccagtaggttccttggtgttccaaatccacataaggcaccatgtatagctttttggtctcatgtgttaatggtaattcatttttgaaccactggtagtgaggaatagggcttccaacagcaacacactgtaaaaccaatgtgctgcctggcatcagcttttgggaagttggttcaacacagatttgcaacttggattcagagacgccatcaacacttctctggaagctctctgggatgtcgcaaacatccagctgtgaccactggctgaattcaaaggtgaaattgttattaactcgacagacataaaagcctgcatcttttacatgcactgcattaaaaataagctctgatgtatttccatttggaatctctttattcattttgaaccactgatattgaacaaaaggatgtccagttgcccggcaacacagtttcacaaactgtccagccaagactgcctttgactctgggtttacagtaatctttattcctggggggctgagaagctgaagaacttcagtgtgttccatagcctgcaggaaatcactcaattctgtgactgtgcaacctttttcacccattaacttcagcagacacaggctggggcttccttcaggctccagtaccttaagagaacactgctccaggtctaggcaactgaggcggaggcgcccgcgactccccgccagctccgccagtctcctccagccccggccctcgggcgcctgatccaggagctcgctgagcctccgcagcagcggctcccgcaggcggttgagggtcgcgccggccggaggggcgagcagcggccccgtgggggcggccgagggcggcagggcctgtagcgggtcccccaacagcgacatggccctcgccggcgaccccggactgccggggctcccgcccgccccgtcacgggcctcggccccggggcaccttccgctcgcctccgagccgcggaggcaggggcggaagaacaaatctggcagcgcggcacggccctcagaggaggaagctccgctccccgccccaattagacaggtttgccgaggggagcctggcctgctggccgcgccagccgcgcaaaggg

SEQ ID NO: 11946 - RNA, 7473 nt, Homo sapiens
  source 1..7473: mol_type = other RNA
ctgaatagctgggactacaggtgtgtgcaactatgcccagttaatttttgtttttgctttttttttttttttttttttggtagagatggggtttcaccatgttgccaaggctagtctcaaactcctgggttcaaatgatctgcttaccgcagtctcccgaagtgctgggattacaggtgtgagccaccatgcccagggtttcagtgtcaaactctgaatttgaatgacaatgtcaaactgagaaacaggatgaaatgcacaaaagtaatgtgtaaattgagtagctgacatcagttgacagataaaagtaatgacagtatataagcgtcaggtgaatgttcaaggaataggaaacaacattgtcaggacgtctgtttggaaaaaaacccttaaaagtaaaattacatacatcagattttatctagatattaaactgatgctgctgaggcaggaggatcacttgaagacaggtgtttgagaccagcatgggcaacaaaatgagatcccacttctaataaaattaaaaacaaacaaaaaaaagcttatgccagtatacatgtcagtgatctaagctctggctacataattgaatttcttcaatttgacaagtcaaaaaattgcgactgctgcacaggacacctcactgttacttcatgtgcaagtcagagatttgaaaagaggcattagagatgggggaagaaggcaatgtctaaatggaccttttctgtgccaggattcttctttaaaggctttcttttctgaaacgttttgacttgttcatcactgaatgaggaacaatagtgttttaaattcaaattgtcccatgagttgagatttcttttattaggaaatatacaatttataattgtgactttaatttttaaaaattaccttccagaaaatatcccctctcagcatcaagtattggctttgaatttgggtgagcctttacttgctcaaacctccactatcctaatttctttattacattctaattggtattgacagatttgatagattatcatcttttctaaattccacttgtgtaaatcctactttaatattacaaagcaattggcacgagattcaagtaaaataaaagcatggttgataaaaaagaagaccaaaactgttatcattcttcttaagcccgttttaaaattacatgtttagattttttaaaaaattcatgcgattctcctgtttcagcctccacggatgctgcagtgagctgagactatgtcgctgcactccagcctgggcgacagagccaggactctgtcttaaaaaaaaaaaaatcaaatatacagaagagtataaaggggaagtacgattctcctgcctcagcctccctagtagctgggattacaggtgtgtgccaccatgcccagctaatttttttgtatttttaatagagacagggttttgccatcttggtcaagctggtcttgaactcctgggctcaagtgatccgccttcattggcctcccaaagtgctgagattataggcgtgagccaccacacccatcctaaaactaaaattttatgttcagttcctcacactagctattatttcaactgctcaacaaccccatgaggctaaaggctatcacactgggagtgcggataccaagcatcccatcatcacagcaagttcactggacagtgctgctcggtggtaaccacagctgagcacctgcatgtttgtttgtttttttatcagatacatgatttttcaaaaatttttctcccattctgagggttaacttcactttcttaatggtgtcctttaaggcgctaaagttaattttgatgaagtcccatttatctactgtttgcctttgttgcttgtgcttttggtattatgtctaagaaaccattcctaagcccaacatcacaaagatttacttctgttttcttctaagagtttaaactcttatattgaggtctatgatccattttgagttagaatttgtaatgtggtaggaaggtagggatccttttgctgtgcacgtagctaccagttagttgtcccagcaccgtttgttgaaaagaccactccttctctattgatggtattggcatccttgttgaaaacaagttgaccagaaatgtatgggtttatttctggatgttcagttccattcctctgatcgatatgtctatccatatgcctacactgtcttattgtagcttggtagcactttttgaaattggtacgtcttccaactttgttcttttccaaggttttttggctattctgggtcccctgcgtttccctaccaattttaccagtttgtcaatttctgcaaaaaatacagctaggattttgataggaattgttgaatatgtagactaatttgggcagcattgccatcttaccaatattcagtcttccaatccatgaacatggatgtctttccatttatctggatcttaatttctttaaacgtgttggagttttattcttgatgctactgtatataggatttctttattctcattttcagaatgtttgctgttagtagagaaataaaactgatcttgtatcctgcaacctgttgaactcatttattactttttatggattctttagcattttctatatacaactatgtatcaactgtgaatacatatagtttcacttcttttgcagtataaacctcttttctttattagcttatttgatttttagatgttgaacaaaccttgaattcctaacctaactgctgtggctagaacttcaagtacaatgctgaatagaagtagtgccgagtgaacatccttgtccttcttcccaatcttaaggggaaaacattcagccttcagtctatcaccatgaagtataatgttaggtgtgggcttttcatagatgttatatttatcatatctaggaagattccttttattcctaagtttgttgagtgtttttatgaaagagttttggattttatcaaatgctgtaataagacaatctgtgtgggttttgtgctttattaaatatggtacagttgatcctcattattcaaggttatgtatttgtgaatttaccaacttgctaaaatttataaccctcaaattgatatccgtggcacttttgcagtcatttgtggatatgtgtaaatgggtgaaaaatttgagtcacccagtacacatgttcccagctgaggctgaacaagatgatgctctgccttcctgcttcagtctcatagagaaatgactggagggtggaaatggcaggggcaattctgtgtagtacaagaagctctggctccggggccagctggatggggtttgaatttcagctctgacacctgttaggggggtgcctcaggcatgtcacttaacacttctgatacctcactttcacttctgtaaaataaggtagaatttgctaggatgaattaagaattcaagctcataatgtgtgtgagataaacatatgtatacacacatatacacaaatacactttctcctaaaagcagttgttccatatttaattcagtgtttatgggagaatattctgtagaacataattactgtgaataatgagaactgactgtatattagcttatttgatttttagatgttgaaccaaccttgaattcctgggataaattccacttggtcatgatatagaatcctttttataggttgctggattcagtttgctaatatttttgttaatgatttttgtgtttgtattaataaggaatattggcttatagttttcttgtgatgtctagtctagtatcagggtaatactgacctagagtaagttgggaagtgttctttcctctcctacttttagaaacagtgtgcaaaaaattagtgctaattttaatgtttggcagaattcaacaatgcagccatctaggcctgggattttctttgtgagacttttaaaattactaattcagtatttttccttgttaatgccaattgcatttttaaccaacttttaggtagagccaaagataagagtattatctcattaggccagtgaaattcaagaagaaaatacatattatcaaggaagatgctaaatatttgggaaattctgataggcagctatgaaaattatccattatatcttgattcttaacctctatctagctttaacaaacattttatcacttctcatgtggtttcataatcttatgaacaagaaatttcagcctgttctataacagatttatatacaaacctcttaactaaaacttgcagtgaagtccttataatcaaaaactaaagtttgtacattccttgagataatacacagatatgtatctgtatatatttatatatatataaatatatttcactctatctacaaacataacacttatctcagaacctgtcaggaaggcagttgtgtagtggaaaaaatactggaatagatttctggaggtctcagttctggtgccagctctaacttagatgcctttctgtgtttcttccatggataaaattaggttatgcctggtgatcggcaaggttctttctggtgttaaaaatacaatgacttattctacaataatgccattcccattgctcttacttcagagtggtcacaatgaaaatattttgttatatacatataaacatacacacctccatacttcatttgtatagaactattcaaccaattcacaaaatcttagaaagaggaagtctgtaattaaataatgtaatttcaacatctcaaagtcctgaagtttgctatgaaacagttactactattctttctctacatatacaaatttgccttttcacaatgtctcactttatgtaagtgcagtactatttcacaggcatctaaaattatgctaactttcaaaaacaaggaggtcatttttcagaaattctgagcctgtcagagaaactaaatggtatttcatcagttgtctctactggcacattacttctactaaaatgacatgaagcatggtgagcgaaacttgaaataaatgcatctggagtccggctgcaatgacagctatctgctggtgtaacattacttggattaccaggatgtgaatggtaaacaccatggaatgggtcttgcaatgagtgataatgccctgctcctcctgaggtggctgcagaactctggtaaggaccattagacataagacaagtttgaaagcaagtcttccttcccaaacctcgatgcatgtctaatttagcaatgagaggtttcccaacattcacttcctgcttgtcctctacagtatcttccaatcctgagtactgatatgataaacatactgtgaagactagatgttcctttaatttttgcagtgaactgagtctggtatagaggcaatgcttgggaagatcctttgataccaagtagctgccagtttcttcaggtgtgcctttatttgcatcttttggatcaatatctagatcaagtggaaaatcagtaacgtaggcatcacacattattatctccggtggtttgtaaactatacttgtatagatgatcatgacattggaaaactcagctgcaaatcctaattgaatctgaacaccacagtcaaacttaagacacatactttctggaagttcatgagccttggcccactgtagattccgcacaagagattcagcagaatattctgttccctgtattggatcagtaagtgctctcttctcagataaactacttcgaatctctagagcctgtttgcctttggtaaggtgacacttacccatatcttctgcaacttcatccagtaacacagtgattttcttatcttctaataatctgtcttttaaaaatttcataaagattccatttgccaatccagaatgctggatttcaaaagcttctgctccttgacacgtggcatatccaaacacaatattggcggtgacttttagtgcatccaagattggaatggtatcatcgtagtcatttcttttcctacacatatccaataagaacacattaagtccagtttctttttcttgcatcaatttcagtatattttgtacacacagacaattttcagacctatatggatttggagcatcaacggggaccatgaagctgttcccaaaattttcataaccatgtcctgcataatataataacccatatactcccttgtctaaaaggagtaaaaactcatccacagcattacgcatctcatattcagtaagatccaacagtgaaaccactttgaagtccagctgtctcagtaagttagtcaattcgtacacatccaccaaaggagctttgagcttggggtgctcccggtaattcatatttcctatcaaaagggcaaccttgtccttcgccaaaggctggtcagttgtttgctctttattatcaggatgaccaagattatttaattcatctatgatgatttctaccttcttgctatcttgactgtctcgatcattatatacatgacaccagtaggttccttggtgttccaaatccacataaggcaccatgtatagctttttggtctcatgtgttaatggtaattcatttttgaaccactggtagtgaggaatagggcttccaacagcaacacactgtaaaaccaatgtgctgcctggcatcagcttttgggaagttggttcaacacagatttgcaacttggattcagagacgccatcaacacttctctggaagctctctgggatgtcgcaaacatccagctgtgaccactggctgaattcaaaggtgaaattgttattaactcgacagacataaaagcctgcatcttttacatgcactgcattaaaaataagctctgatgtatttccatttggaatctctttattcattttgaaccactgatattgaacaaaaggatgtccagttgcccggcaacacagtttcacaaactgtccagccaagactgcctttgactctgggtttacagtaatctttattcctggggggctgagaagctgaagaacttcagtgtgttccatagcctgcaggaaatcactcaattctgtgactgtgcaacctttttcacccattaacttcagcagacacaggctggggcttccttcaggctccagtaccttaagagaacactgctccaggtctaggcaactgaggcggaggcgcccgcgactccccgccagctccgccagtctcctccagccccggccctcgggcgcctgatccaggagctcgctgagcctccgcagcagcggctcccgcaggcggttgagggtcgcgccggccggaggggcgagcagcggccccgtgggggcggccgagggcggcagggcctgtagcgggtcccccaacagcgacatggccctcgccggcgaccccggactgccggggctcccgcccgccccgtcacgggcctcggccccggggcaccttccgctcgcctccgagccgcggaggcaggggcggaagaacaaatctggcagcgcggcacggccctcagaggaggaagctccgctccccgccccaattagacaggttt

SEQ ID NO: 11947 - RNA, 7506 nt, Homo sapiens
  source 1..7506: mol_type = other RNA
ctgaatagctgggactacaggtgtgtgcaactatgcccagttaatttttgtttttgctttttttttttttttttttttggtagagatggggtttcaccatgttgccaaggctagtctcaaactcctgggttcaaatgatctgcttaccgcagtctcccgaagtgctgggattacaggtgtgagccaccatgcccagggtttcagtgtcaaactctgaatttgaatgacaatgtcaaactgagaaacaggatgaaatgcacaaaagtaatgtgtaaattgagtagctgacatcagttgacagataaaagtaatgacagtatataagcgtcaggtgaatgttcaaggaataggaaacaacattgtcaggacgtctgtttggaaaaaaacccttaaaagtaaaattacatacatcagattttatctagatattaaactgatgctgctgaggcaggaggatcacttgaagacaggtgtttgagaccagcatgggcaacaaaatgagatcccacttctaataaaattaaaaacaaacaaaaaaaagcttatgccagtatacatgtcagtgatctaagctctggctacataattgaatttcttcaatttgacaagtcaaaaaattgcgactgctgcacaggacacctcactgttacttcatgtgcaagtcagagatttgaaaagaggcattagagatgggggaagaaggcaatgtctaaatggaccttttctgtgccaggattcttctttaaaggctttcttttctgaaacgttttgacttgttcatcactgaatgaggaacaatagtgttttaaattcaaattgtcccatgagttgagatttcttttattaggaaatatacaatttataattgtgactttaatttttaaaaattaccttccagaaaatatcccctctcagcatcaagtattggctttgaatttgggtgagcctttacttgctcaaacctccactatcctaatttctttattacattctaattggtattgacagatttgatagattatcatcttttctaaattccacttgtgtaaatcctactttaatattacaaagcaattggcacgagattcaagtaaaataaaagcatggttgataaaaaagaagaccaaaactgttatcattcttcttaagcccgttttaaaattacatgtttagattttttaaaaaattcatgcgattctcctgtttcagcctccacggatgctgcagtgagctgagactatgtcgctgcactccagcctgggcgacagagccaggactctgtcttaaaaaaaaaaaaatcaaatatacagaagagtataaaggggaagtacgattctcctgcctcagcctccctagtagctgggattacaggtgtgtgccaccatgcccagctaatttttttgtatttttaatagagacagggttttgccatcttggtcaagctggtcttgaactcctgggctcaagtgatccgccttcattggcctcccaaagtgctgagattataggcgtgagccaccacacccatcctaaaactaaaattttatgttcagttcctcacactagctattatttcaactgctcaacaaccccatgaggctaaaggctatcacactgggagtgcggataccaagcatcccatcatcacagcaagttcactggacagtgctgctcggtggtaaccacagctgagcacctgcatgtttgtttgtttttttatcagatacatgatttttcaaaaatttttctcccattctgagggttaacttcactttcttaatggtgtcctttaaggcgctaaagttaattttgatgaagtcccatttatctactgtttgcctttgttgcttgtgcttttggtattatgtctaagaaaccattcctaagcccaacatcacaaagatttacttctgttttcttctaagagtttaaactcttatattgaggtctatgatccattttgagttagaatttgtaatgtggtaggaaggtagggatccttttgctgtgcacgtagctaccagttagttgtcccagcaccgtttgttgaaaagaccactccttctctattgatggtattggcatccttgttgaaaacaagttgaccagaaatgtatgggtttatttctggatgttcagttccattcctctgatcgatatgtctatccatatgcctacactgtcttattgtagcttggtagcactttttgaaattggtacgtcttccaactttgttcttttccaaggttttttggctattctgggtcccctgcgtttccctaccaattttaccagtttgtcaatttctgcaaaaaatacagctaggattttgataggaattgttgaatatgtagactaatttgggcagcattgccatcttaccaatattcagtcttccaatccatgaacatggatgtctttccatttatctggatcttaatttctttaaacgtgttggagttttattcttgatgctactgtatataggatttctttattctcattttcagaatgtttgctgttagtagagaaataaaactgatcttgtatcctgcaacctgttgaactcatttattactttttatggattctttagcattttctatatacaactatgtatcaactgtgaatacatatagtttcacttcttttgcagtataaacctcttttctttattagcttatttgatttttagatgttgaacaaaccttgaattcctaacctaactgctgtggctagaacttcaagtacaatgctgaatagaagtagtgccgagtgaacatccttgtccttcttcccaatcttaaggggaaaacattcagccttcagtctatcaccatgaagtataatgttaggtgtgggcttttcatagatgttatatttatcatatctaggaagattccttttattcctaagtttgttgagtgtttttatgaaagagttttggattttatcaaatgctgtaataagacaatctgtgtgggttttgtgctttattaaatatggtacagttgatcctcattattcaaggttatgtatttgtgaatttaccaacttgctaaaatttataaccctcaaattgatatccgtggcacttttgcagtcatttgtggatatgtgtaaatgggtgaaaaatttgagtcacccagtacacatgttcccagctgaggctgaacaagatgatgctctgccttcctgcttcagtctcatagagaaatgactggagggtggaaatggcaggggcaattctgtgtagtacaagaagctctggctccggggccagctggatggggtttgaatttcagctctgacacctgttaggggggtgcctcaggcatgtcacttaacacttctgatacctcactttcacttctgtaaaataaggtagaatttgctaggatgaattaagaattcaagctcataatgtgtgtgagataaacatatgtatacacacatatacacaaatacactttctcctaaaagcagttgttccatatttaattcagtgtttatgggagaatattctgtagaacataattactgtgaataatgagaactgactgtatattagcttatttgatttttagatgttgaaccaaccttgaattcctgggataaattccacttggtcatgatatagaatcctttttataggttgctggattcagtttgctaatatttttgttaatgatttttgtgtttgtattaataaggaatattggcttatagttttcttgtgatgtctagtctagtatcagggtaatactgacctagagtaagttgggaagtgttctttcctctcctacttttagaaacagtgtgcaaaaaattagtgctaattttaatgtttggcagaattcaacaatgcagccatctaggcctgggattttctttgtgagacttttaaaattactaattcagtatttttccttgttaatgccaattgcatttttaaccaacttttaggtagagccaaagataagagtattatctcattaggccagtgaaattcaagaagaaaatacatattatcaaggaagatgctaaatatttgggaaattctgataggcagctatgaaaattatccattatatcttgattcttaacctctatctagctttaacaaacattttatcacttctcatgtggtttcataatcttatgaacaagaaatttcagcctgttctataacagatttatatacaaacctcttaactaaaacttgcagtgaagtccttataatcaaaaactaaagtttgtacattccttgagataatacacagatatgtatctgtatatatttatatatatataaatatatttcactctatctacaaacataacacttatctcagaacctgtcaggaaggcagttgtgtagtggaaaaaatactggaatagatttctggaggtctcagttctggtgccagctctaacttagatgcctttctgtgtttcttccatggataaaattaggttatgcctggtgatcggcaaggttctttctggtgttaaaaatacaatgacttattctacaataatgccattcccattgctcttacttcagagtggtcacaatgaaaatattttgttatatacatataaacatacacacctccatacttcatttgtatagaactattcaaccaattcacaaaatcttagaaagaggaagtctgtaattaaataatgtaatttcaacatctcaaagtcctgaagtttgctatgaaacagttactactattctttctctacatatacaaatttgccttttcacaatgtctcactttatgtaagtgcagtactatttcacaggcatctaaaattatgctaactttcaaaaacaaggaggtcatttttcagaaattctgagcctgtcagagaaactaaatggtatttcatcagttgtctctactggcacattacttctactaaaatgacatgaagcatggtgagcgaaacttgaaataaatgcatctggagtccggctgcaatgacagctatctgctggtgtaacattacttggattaccaggatgtgaatggtaaacaccatggaatgggtcttgcaatgagtgataatgccctgctcctcctgaggtggctgcagaactctggtaaggaccattagacataagacaagtttgaaagcaagtcttccttcccaaacctcgatgcatgtctaatttagcaatgagaggtttcccaacattcacttcctgcttgtcctctacagtatcttccaatcctgagtactgatatgataaacatactgtgaagactagatgttcctttaatttttgcagtgaactgagtctggtatagaggcaatgcttgggaagatcctttgataccaagtagctgccagtttcttcaggtgtgcctttatttgcatcttttggatcaatatctagatcaagtggaaaatcagtaacgtaggcatcacacattattatctccggtggtttgtaaactatacttgtatagatgatcatgacattggaaaactcagctgcaaatcctaattgaatctgaacaccacagtcaaacttaagacacatactttctggaagttcatgagccttggcccactgtagattccgcacaagagattcagcagaatattctgttccctgtattggatcagtaagtgctctcttctcagataaactacttcgaatctctagagcctgtttgcctttggtaaggtgacacttacccatatcttctgcaacttcatccagtaacacagtgattttcttatcttctaataatctgtcttttaaaaatttcataaagattccatttgccaatccagaatgctggatttcaaaagcttctgctccttgacacgtggcatatccaaacacaatattggcggtgacttttagtgcatccaagattggaatggtatcatcgtagtcatttcttttcctacacatatccaataagaacacattaagtccagtttctttttcttgcatcaatttcagtatattttgtacacacagacaattttcagacctatatggatttggagcatcaacggggaccatgaagctgttcccaaaattttcataaccatgtcctgcataatataataacccatatactcccttgtctaaaaggagtaaaaactcatccacagcattacgcatctcatattcagtaagatccaacagtgaaaccactttgaagtccagctgtctcagtaagttagtcaattcgtacacatccaccaaaggagctttgagcttggggtgctcccggtaattcatatttcctatcaaaagggcaaccttgtccttcgccaaaggctggtcagttgtttgctctttattatcaggatgaccaagattatttaattcatcttcagtgcactccactgcctcatctgttcttcctatgatgatttctaccttcttgctatcttgactgtctcgatcattatatacatgacaccagtaggttccttggtgttccaaatccacataaggcaccatgtatagctttttggtctcatgtgttaatggtaattcatttttgaaccactggtagtgaggaatagggcttccaacagcaacacactgtaaaaccaatgtgctgcctggcatcagcttttgggaagttggttcaacacagatttgcaacttggattcagagacgccatcaacacttctctggaagctctctgggatgtcgcaaacatccagctgtgaccactggctgaattcaaaggtgaaattgttattaactcgacagacataaaagcctgcatcttttacatgcactgcattaaaaataagctctgatgtatttccatttggaatctctttattcattttgaaccactgatattgaacaaaaggatgtccagttgcccggcaacacagtttcacaaactgtccagccaagactgcctttgactctgggtttacagtaatctttattcctggggggctgagaagctgaagaacttcagtgtgttccatagcctgcaggaaatcactcaattctgtgactgtgcaacctttttcacccattaacttcagcagacacaggctggggcttccttcaggctccagtaccttaagagaacactgctccaggtctaggcaactgaggcggaggcgcccgcgactccccgccagctccgccagtctcctccagccccggccctcgggcgcctgatccaggagctcgctgagcctccgcagcagcggctcccgcaggcggttgagggtcgcgccggccggaggggcgagcagcggccccgtgggggcggccgagggcggcagggcctgtagcgggtcccccaacagcgacatggccctcgccggcgaccccggactgccggggctcccgcccgccccgtcacgggcctcggccccggggcaccttccgctcgcctccgagccgcggaggcaggggcggaagaacaaatctggcagcgcggcacggccctcagaggaggaagctccgctccccgccccaattagacaggttt

SEQ ID NO: 11948 - RNA, 2225 nt, Homo sapiens
  source 1..2225: mol_type = other RNA
ctgaatagctgggactacaggtgtgtgccacaacgcccagctaatttattttaaattattttttgtagagacagggtctccctatgttgcccaggctggtctcaaactactaggctcaagtgatcctcccacctcagcttcccaaagtgttgggattacaggtgtgagccactgtgcccagcccaatcccactttttaaaaagtatacccccaaatccatacactggtgaggaagtggagaacgtggaatcctcacacacagaatgtaaaatggtacagctctggagaacattttagcagtttctcaaaatgtttaacgtagctactacacgacccagcaattcaactcccagatatacacctgagagaactgaaaggatatgtccacacaaaaatttgcagaggaacttgtacacacttgttcacagtagcattattcataatagcccaaagtggcaaaaacgcaaatgttcatcaactgatggacaaataaagcatgaacaactgatggacaaataaagtatatcattcagcatataagaaatgaagtgctaatacatgctacaacaggaatagaccttaataacattttgctaaatgaaaaaagccaaacaaaaggtcacatgttgtatgattccatttacataaaaatacctagactaggcaaatccatagagacacaaagatcagtgactgcccagagccagagggagtggtgaatgtgaaatggctactaatgagtacagacttctttttgaggtattgaacatgttatggaatcagatggtggtgatcaatgcataactttgtgaatataccaaaaaccacatgaaaggtacactttaaaagcctgaattttaaggtatgtgaattgtatctccataaacctgtgattttgttaatatacgcttatttgcaaatgaatacatggataatgaggaataatatgaaaggttaatgacaaccttggtgatagggtacaggagactgggagaggaagataagtgttgaggtagaagaagacaaaaaataaaaggctaaaacaataatccagggccagaggccatgagttgggagatggagcaagacgaagtgtacaaagaaatgagcataaatcataaaaatgagggaactagggttgaaaactccagcaagtagtttgtaatgggggagatgaagcaaacctaagtaactgcaatgattcaacggaatttgcagaaaatgcagaagggcgagaaaagcaatgaaaaaatggatcagaagatttaaaattggctctaccccaccaaagttttaaaaagcaagcaagaagaaaattcagttgctcctgggcaagaattcttgggcccagtggggtagaaccaaaccatgataaggagacaccagtgttttgtaagcaagagaatatattaaggagagaaaaggggcatttattgagagaaaaggtctcactgtgattgttctggaataaagtagccccatcggactgcctcaggaactcatggtggaagaggtgccactggaaaatggctaagtcgggatcttccccaagaacaggtctcatcgtccagtggaggccgcagatgagacatagtgtgccaaatcccaaatgcacagggtgccagacaagtctgcgggaggcaggaggactagggaagccttccaggcaaggtgatgcctgagctgagttgtttttcttttgagtttggaacattaatttaatcggaggaaaacaagggacatgaaaagggcaaggaaataagaaaatgagctgagttttgaaggcaatgatcagatgaagtgagagaagaatattccagcagagggagacaaggagactgcagagatttcaaggggccaagagctgttcggtgcagctcagtgaagcacctaaacagaggtgggggaaggagaacaggggtcaaagcccagtattgaagtgttctggataccaagctaaggagaccttattacgaaggtactggggctgctgaagggtttaaatgggagagtgattgtgaacagattaatagtttggaaagatacaggcagaagtaaacctctggatttaaccaaaaaataaaggacagaaccacaatgaagatgttggaaaagatcaggaaaaacactgttaaaagatattcactctcggggccgggcgctgtggctcacgccttaaatcccggcactttggtaggccgaggcgggctgatcacgaggtcagg

SEQ ID NO: 11949 - RNA, 2300 nt, Homo sapiens
  source 1..2300: mol_type = other RNA
ctgaatagctgggactacaggtgtgtgccacatggttggctaatttttgtatttgagacagggtttttgccatgttggccaggctggtctcgaactcctggcctcaagtcatcttgagtggatcacttgaggcatttgggagtgcctcagcctcccaaaacggtgggattacaggcgtgagccactgtgcccggcctgcacatgtctttcttacatgtggactctccaggggatttatgctgttcaagaagcacctgaatcaaactgtgctttaaaaatatttttaaaacattccatgattcttcatagtacaaaaatgagaaatctcccctaaatctctaaagaattccctttttaaactttttgatttcctgaacttgtctgaaggacttaacacagttatatagagtgttctttgtgtaacagtatccatgactttcatttttagctctggtattagatcttcctggacaagagcattactggccatgtgtatgttgctatcacaaataactagtagttaatatttcctaaatcttagcaagagttatgataaatagctgaattccatgaagagaaaagactcatggcatgacaaccagattaggaaagagtgttttccttgtcctgcaggcaaaacagaactgagagatatgagtatcactcatgatgaggacaaaagggctgcgtgctgggaaacatgaggcgaccaacacagagttggtcactatccactggcctgggtttgcaactacagttgtccaaattgtcagaaaactatggactgaatagaaaacaaaaaaggagctcaccaggaccatgatggtgtgtgtggctctggcttcctgggaaggtctgcaggagagtctgttgctgtgattgtgttggacttgctgcttgtgtctgtagaggaagaagaccatggagccactggcccagaccatgaagcccaaactcataaaatcaggggaaaaatataagactgcatgtaatgagctaaatctctttgatgctttgtaagaacagtatccataattgttttttgcactactgtttttgctattcagtgggccattcactaatagaagaacagatgcattcatcaagacatggggggcccagcagaggagacaacagaagtcaataaaccttggggatctaatcttgatctccatccacctgcatatactggggttgagcttaatggcttggaatccattgagaaggcagatggtgctgagggaaactcttgtgcccaccctgtgataataaaagacaaacttacatccagtgtcattcagcaaatatttcaatccaaaagctgccattgtctgaggtatccctttaaagaaaaggaccatggagttagccaaggccagttggctgagaatcaagtccgtgggtctcagcttgtgtccagtgaacaaaattaagttataaaaacaaaggagaaaggaatttcccaggatcccaactccagtctgaatgaggaagctaatccctgattttacttttccaaaagccatttcatcaaaatctaggggatgttgattttcattgaggtctgaagaatcagtagaataaaaaagcagaaagaagtatcttgtcatcagtggagacagaagttttaatgtgtctccaaccatattttctcatcttaaacagaaattaagattgtccctgttcgtgcaaaggcaattgcttgtgtgtccaactgcagagaagcaggtgaatgaatgagggctcaaccgcacaacagatccacaaatcaaacctataaaactcagggcttacacacatgcaacaagtaaatacaagcaaaactagggaaatatataaaaacagaacacagaagagtcaatatcattagagtgatattatactatagtttgcaaaatgtaatcatgacggaaccctgggtaatatggacagggctttttctgtattatttcttatgactgcttgtgagtctacacttatttcaataaaaccttcaattaagtagcctggagatatgaaaagcaaaaataatacaccataaaaccttttccacactaatattttagtaaacaccattgttattgatgcattgaaacaaattttaggccgggtgcagtggctcacacctgtaattccagcacttcgggaggccaagatggagaccatcctggccaacatggtgaaaccctgtctctactaataatacaaaatactaataatacaaaaattagccgggcatggcggcgcgtgctagtcccagctactcgggaggctgaggcaggagaatcgcttgaacctgg

SEQ ID NO: 11950 - RNA, 4259 nt, Homo sapiens
  source 1..4259: mol_type = other RNA
ctgaatagctgggactacaggtgtgtgccaccaaaccaggctaatttttgtatttttagaagagatggggtttcgccatgttggccaggctggtcttgaactcctgacctcaggtgatccacccacctcagcctcccaaaatgctgggattataggcatgaaccactgcgcctggccataatactttattattatttggttctcatggatttcctaggtgtataatcacttacaaataaaagtaattttggcatttctttaaatattataacttatttttcttgtataattggattggccacctgttctaaaacactgtaaaataagatagatagtaatcaatttttttcatgttcctaactttagtaggaatgcttctgtttcttcatcattaggtatgtattagcttttgtttacatgtatataaaattatggccaaataacatctgtctatcctattttagtaactaatttaataattaagaatggatgttgaatatttttgttttagcccagttgtctaagacttccaggaatatacctgtagtgtaataaaattaggtttattgatccattgcaatgagacagactgcgtcccaggggagccatggggtatctcaccaaacaaaggaaaaggcagagttataggatttggggtaagtttaggttaatattaaataaggcagatcgttgataggctcagaggaaagcagggctgtgtgtaaaacggtccatatcaggtctggactgcaaagtggacccagagtcctattttcttgaatactagacagttgagagaggtgtggaatgttgtgtccagataccccttatctgcacttctgtatttgagtataagatgaggctgtgttaggagtcaggaaaagaaaggagccaactgaagttatttagaaagcaaaatcaacagaacttggtgacgctggatgtagtgtgagggaaaatggcgaactgaaatttcacccctctatttatggcttatgtgattgggtagatgaccaggtcttcagctgatatggaatatactataacaacagttggtttagggaagcaagagagagaagaacaggatgatcacttcaatttttgatttgttgggtttctgactgctgcaagactcgagtatagacccacaggtaggtagtaggatgtataagtgcagggatactgctggaggctggggtcacagctatagatacagatgcctaggagtcatgagcatcactgaaggagggcctgcaaagtgagaggagcactgaccagatcaagagaaaaccccaggaagatttccctaaggtttccaggccagtaggatgagcccacagtgaagactacaaatgaacagagagaggtaggaatcaaagcagagacctgccatgtcagagaaactgaggaaaagagttccaaggaggagggagtggtcaactttatcaactgcaggaaatgggctcaggaatggaagacctgaattggtttaacagttggcaggtagacggtgacttttgccagggtacattcaggtaagttggtgaagcagaagaccaaattctgtatgttcagccaataataagtgagacagaaaagtcagcctccaccttacaggaagctgggctgagaagggcaggagacagggcagtaactgctgtggcatcaagctcagggaatgcttttcagcaaaaaagatgtcagtgtttcacttttttcagctagttagaatcaggacctcagcctgatggaattcatttaaaataccaaataaaggtaagtcttctgtagtctttctgtactcacttgagtacttgatctctgtaactcactctgcatcctccttcttgccccttccttagcatgacacacgcacgcgcacgtgcacacacacaccagtatacatttgattatattttaatgatcacgcagacccttttagaaaagatgtctccttgaactgtacccaggagatgtggccatggcacacacaaagctgtagggaaagaccagacgaatcttgagctgagaaggaagggctcagttgcataggtatttaggcagaatgcataaagaaatcctttgttgaaaatatttaggaaagaatggagtttttgaaatataaaatcaataataatttttattttttgttcagcacacatggcaacacagagctgtgaagacagacgtggttagcacaaaccacttgggccagtgaaaccagggcaaactcatggatcatctgcgttcccatcttcaccttggtggcagccctacctctgagattttaaggtctacggaaagtgcaggcttccaggagtgatgaggtggagcattttctcaggttaccaacagccttgacatattcttctcctaagtatttttcatatgtgtttctgtcatgaagtttggccaaacatactgtgtcatctctgaacagaaggtccttggtttccgaccggaacaaacaaaagttgcccgagcagtcagttacgttgcttccaaataggtgctgctgttgacgtaatatcttgtggacgcaagcttccttatctttccgtgtgaccacagcgtgattcggggctctggccaggtggcagttcgcatactcctccacaggtttcctggtaccatcaaggcacagcaactcatagtctttttcattcagattcttagcccatggatcagggttttttcccccagtgttctgtgggacagtctggtgtttcacaaaggccacatctcccttctcaaccagacacctgaaagcgcctgtgtagccgtagtatccctctttgttgttgggttcacacaggtttaggcctgagcccatacacagcttacagagactggagtctttcttagacccaggggcacaaccttcactgaaaaattcatcaaatctgcagtggttgatcttattgtagagcaggcccatggggatgttccagccagcggttctgccaactgccgtatggcaggacttcttgcctttcagattgtcccaggtgaggtcagaagctgatttcttcaccactgctatagcaaaataccctgcctctggtgtatcctcacaattatcgctcttattgtagttttctgccaagacaggcaccagaccacacttgcccgctatgtagacaaaccctccatccaagctcatggcatcagcttctccattcatgatcttggcgatgcagtcttcggtggtctctgctgatacacactctattttccctacactgttaacactccactcatcacacttgagcctctcgtggtggctcagcgcacaccacttcacaggcttgcattcatctgttggggcttctgggcatgtgccttcccgtagattccggatggcagtgacatactcatagcccaggtacatcttggcatccatcctgggggggacttttaaaaacccgtgggcagagtccttaaacagcaggtccttcccatgaggagagctgaatagttggaattcttttgatttgtctttgccaaaatgttcctgggcctggttgagaagctcccagatcaagtcctccttgccgcccatacttcgggccacgacggtatgagaagggacctgggccaagtggcagtccttgtattcatctaccggcttccgggtgttgtccaggcaaagcagctcatactggtccctgtcagccttgtttgccaagttctcaaatatagtcgagtgcttgacaaaggccacatccccagcaccatccttcagacacttgaaggctcccgagtagccgaagtattggttaagggtggagcagccacaccctggacacagttgacacagctgggggaagtccgtcccatccgcacaaggggcacagctgcccgagaagaaattggccactgctttctcaagaggtttacgtggctcaggtaagtcacagtaaagtaagcctatggggatgttccacccagcggacctgcctagacccgtgtggcaggacttcttgcctcgaagctggttcatctggaagccactatccttcttcaccacagcaacagcataatagaaagtctgtggatcctcttttgacccatagaactctgccaccacaggcttcaggttattgggagccaggtaagcatcatacaccaaacctgcatccagtgtcacagcatccgcttcgtttgcccaggacggcgcagaccagcagggctcccacggcgagcctcatcttccgggtgcggcgctgagcagcgagcacagtcggactcgcttctgt

SEQ ID NO: 11951 - RNA, 5400 nt, Homo sapiens
  source 1..5400: mol_type = other RNA
ctgaatagctgggactacaggtgtgtgccaccaaaccaggctaatttttgtatttttagaagagatggggtttcgccatgttggccaggctggtcttgaactcctgacctcaggtgatccacccacctcagcctcccaaaatgctgggattataggcatgaaccactgcgcctggccataatactttattattatttggttctcatggatttcctaggtgtataatcacttacaaataaaagtaattttggcatttctttaaatattataacttatttttcttgtataattggattggccacctgttctaaaacactgtaaaataagatagatagtaatcaatttttttcatgttcctaactttagtaggaatgcttctgtttcttcatcattaggtatgtattagcttttgtttacatgtatataaaattatggccaaataacatctgtctatcctattttagtaactaatttaataattaagaatggatgttgaatatttttgttttagcccagttgtctaagacttccaggaatatacctgtagtgtaataaaattaggtttattgatccattgcaatgagacagactgcgtcccaggggagccatggggtatctcaccaaacaaaggaaaaggcagagttataggatttggggtaagtttaggttaatattaaataaggcagatcgttgataggctcagaggaaagcagggctgtgtgtaaaacggtccatatcaggtctggactgcaaagtggacccagagtcctattttcttgaatactagacagttgagagaggtgtggaatgttgtgtccagataccccttatctgcacttctgtatttgagtataagatgaggctgtgttaggagtcaggaaaagaaaggagccaactgaagttatttagaaagcaaaatcaacagaacttggtgacgctggatgtagtgtgagggaaaatggcgaactgaaatttcacccctctatttatggcttatgtgattgggtagatgaccaggtcttcagctgatatggaatatactataacaacagttggtttagggaagcaagagagagaagaacaggatgatcacttcaatttttgatttgttgggtttctgactgctgcaagactcgagtatagacccacaggtaggtagtaggatgtataagtgcagggatactgctggaggctggggtcacagctatagatacagatgcctaggagtcatgagcatcactgaaggagggcctgcaaagtgagaggagcactgaccagatcaagagaaaaccccaggaagatttccctaaggtttccaggccagtaggatgagcccacagtgaagactacaaatgaacagagagaggtaggaatcaaagcagagacctgccatgtcagagaaactgaggaaaagagttccaaggaggagggagtggtcaactttatcaactgcaggaaatgggctcaggaatggaagacctgaattggtttaacagttggcaggtagacggtgacttttgccagggtacattcaggtaagttggtgaagcagaagaccaaattctgtatgttcagccaataataagtgagacagaaaagtcagcctccaccttacaggaagctgggctgagaagggcaggagacagggcagtaactgctgtggcatcaagctcagggaatgcttttcagcaaaaaagatgtcagtgtttcacttttttcagctagttagaatcaggacctcagcctgatggaattcatttaaaataccaaataaaggtaagtcttctgtagtctttctgtactcacttgagtacttgatctctgtaactcactctgcatcctccttcttgccccttccttagcatgacacacgcacgcgcacgtgcacacacacaccagtatacatttgattatattttaatgatcacgcagacccttttagaaaagatgtctccttgaactgtacccaggagatgtggccatggcacacacaaagctgtagggaaagaccagacgaatcttgagctgagaaggaagggctcagttgcataggtatttaggcagaatgcataaagaaatcctttgttgaaaatatttaggaaagaatggagtttttgaaatataaaatcaataataatttttattttttgttcagcacacatggcaacacagagctgtgaagacagacgtggttagcacaaaccacttgggccagtgaaaccagggcaaactcatggatcatctgcgttcccatcttcaccttggtggcagccctacctctgagattttaaggtctacggaaagtgcaggcttccaggagtgatgaggtggagcattttctcaggttaccaacagccttgacatattcttctcctaagtatttttcatatgtgtttctgtcatgaagtttggccaaacatactgtgtcatctctgaacagaaggtccttggtttccgaccggaacaaacaaaagttgcccgagcagtcagttacgttgcttccaaataggtgctgctgttgacgtaatatcttgtggacgcaagcttccttatctttccgtgtgaccacagcgtgattcggggctctggccaggtggcagttcgcatactcctccacaggtttcctggtaccatcaaggcacagcaactcatagtctttttcattcagattcttagcccatggatcagggttttttcccccagtgttctgtgggacagtctggtgtttcacaaaggccacatctcccttctcaaccagacacctgaaagcgcctgtgtagccgtagtatccctctttgttgttgggttcacacaggtttaggcctgagcccatacacagcttacagagactggagtctttcttagacccaggggcacaaccttcactgaaaaattcatcaaatctgcagtggttgatcttattgtagagcaggcccatggggatgttccagccagcggttctgccaactgccgtatggcaggacttcttgcctttcagattgtcccaggtgaggtcagaagctgatttcttcaccactgctatagcaaaataccctgcctctggtgtatcctcacaattatcgctcttattgtagttttctgccaagacaggcaccagaccacacttgcccgctatgtagacaaaccctccatccaagctcatggcatcagcttctccattcatgatcttggcgatgcagtcttcggtggtctctgctgatacacactctattttccctacactgttaacactccactcatcacacttgagcctctcgtggtggctcagcgcacaccacttcacaggcttgcattcatctgttggggcttctgggcatgtgccttcccgtagattccggatggcagtgacatactcatagcccaggtacatcttggcatccatcctgggggggacttttaaaaacccgtgggcagagtccttaaacagcaggtccttcccatgaggagagctgaatagttggaattcttttgatttgtctttgccaaaatgttcctgggcctggttgagaagctcccagatcaagtcctccttgccgcccatacttcgggccacgacggtatgagaagggacctgggccaagtggcagtccttgtattcatctaccggcttccgggtgttgtccaggcaaagcagctcatactggtccctgtcagccttgtttgccaagttctcaaatatagtcgagtgcttgacaaaggccacatccccagcaccatccttcagacacttgaaggctcccgagtagccgaagtattggttaagggtggagcagccacaccctggacacagttgacacagctgggggaagtccgtcccatccgcacaaggggcacagctgcccgagaagaaattggccactgctttctcaagaggtttacgtggctcaggtaagtcacagtaaagtaagcctatggggatgttccacccagcggacctgcctagacccgtgtggcaggacttcttgcctcgaagctggttcatctggaagccactatccttcttcaccacagcaacagcataatagaaagtctgtggatcctcttttgacccatagaactctgccaccacaggcttcaggttattgggagccaggtaagcatcatacaccaaacctgcatccagtgtcacagcatccgcttcgtttgccgcaatggccctgatgcaatcaaggtaggaggctttcttcacacaagcaacactgggaccatcggatggaatgacgcttttcatatggtcgcggaaactctggcacttagtggcctcatgctccgacactgcacaccatctcacagttttatcagggacagccagacacagcccagccaagtgtaagaagtgaggtgtctggtgtcccccctgtgattttaaaccaaggctctgatggattcttgacttgtccacagtcacacagaagaaagtggcaaaagtagaactagagttgtgactctgccgccatcattcttgcttctccctaggtgccctaaggtgccctaaatcatctgggtctgcaggagagtgccctgaaagccccactggagccgtagtatctctcctggctgttgtaagcccatatgtgggcaggattgcacctgccaccacacagagcacagagaggggaatccggattagacccaggggcacaactgcgactgaagaaatcatcacatttacaggacccggtttgattgtatattaagcccatggggatgttccagcttgcagaagtgccaactgcagtgtggcaggacttcttgcctcaaagagagttccaggtgacatcagcatctgatttcttaaccacagccatgacataatagccttttctctgtgttgtagatcaggtctctacaaattcaaacttggagaagttgggagtcaacatggcagatggaaggtccgtcttgtccttcttaggtgacctcagacacgtccttatcatctaggagcctaaatttttcttcagttaaatggtggcagtggaacccctcctggagtgactctttttggatcctgagtcgcggaaaaatactcatatcccaggtacagcttggcatctatcttaggtgggaccattaaaaacccatgggcagcatcagtaaacagcagatctgtctcatgaggagagccaaagagctgaaattctgacgacttgtcttttccaaaatgttctgtgatggctttaatgtactcaagggaagacgctctctccacgcaggtgacaaggggaccatctgctggaaacacttttttcatattgtctcggaaactggtgcacttcgtggcctcgtgatctgacatggcacaccatcttccagttttctcaggagcagccaggcacagccctccacgtttgacatttccgctcttctgctgcagct

SEQ ID NO: 11952 - RNA, 4432 nt, Homo sapiens
  source 1..4432: mol_type = other RNA
ctgaatagctgggactacaggtgtgtgccaccaaaccaggctaatttttgtatttttagaagagatggggtttcgccatgttggccaggctggtcttgaactcctgacctcaggtgatccacccacctcagcctcccaaaatgctgggattataggcatgaaccactgcgcctggccataatactttattattatttggttctcatggatttcctaggtgtataatcacttacaaataaaagtaattttggcatttctttaaatattataacttatttttcttgtataattggattggccacctgttctaaaacactgtaaaataagatagatagtaatcaatttttttcatgttcctaactttagtaggaatgcttctgtttcttcatcattaggtatgtattagcttttgtttacatgtatataaaattatggccaaataacatctgtctatcctattttagtaactaatttaataattaagaatggatgttgaatatttttgttttagcccagttgtctaagacttccaggaatatacctgtagtgtaataaaattaggtttattgatccattgcaatgagacagactgcgtcccaggggagccatggggtatctcaccaaacaaaggaaaaggcagagttataggatttggggtaagtttaggttaatattaaataaggcagatcgttgataggctcagaggaaagcagggctgtgtgtaaaacggtccatatcaggtctggactgcaaagtggacccagagtcctattttcttgaatactagacagttgagagaggtgtggaatgttgtgtccagataccccttatctgcacttctgtatttgagtataagatgaggctgtgttaggagtcaggaaaagaaaggagccaactgaagttatttagaaagcaaaatcaacagaacttggtgacgctggatgtagtgtgagggaaaatggcgaactgaaatttcacccctctatttatggcttatgtgattgggtagatgaccaggtcttcagctgatatggaatatactataacaacagttggtttagggaagcaagagagagaagaacaggatgatcacttcaatttttgatttgttgggtttctgactgctgcaagactcgagtatagacccacaggtaggtagtaggatgtataagtgcagggatactgctggaggctggggtcacagctatagatacagatgcctaggagtcatgagcatcactgaaggagggcctgcaaagtgagaggagcactgaccagatcaagagaaaaccccaggaagatttccctaaggtttccaggccagtaggatgagcccacagtgaagactacaaatgaacagagagaggtaggaatcaaagcagagacctgccatgtcagagaaactgaggaaaagagttccaaggaggagggagtggtcaactttatcaactgcaggaaatgggctcaggaatggaagacctgaattggtttaacagttggcaggtagacggtgacttttgccagggtacattcaggtaagttggtgaagcagaagaccaaattctgtatgttcagccaataataagtgagacagaaaagtcagcctccaccttacaggaagctgggctgagaagggcaggagacagggcagtaactgctgtggcatcaagctcagggaatgcttttcagcaaaaaagatgtcagtgtttcacttttttcagctagttagaatcaggacctcagcctgatggaattcatttaaaataccaaataaaggtaagtcttctgtagtctttctgtactcacttgagtacttgatctctgtaactcactctgcatcctccttcttgccccttccttagcatgacacacgcacgcgcacgtgcacacacacaccagtatacatttgattatattttaatgatcacgcagacccttttagaaaagatgtctccttgaactgtacccaggagatgtggccatggcacacacaaagctgtagggaaagaccagacgaatcttgagctgagaaggaagggctcagttgcataggtatttaggcagaatgcataaagaaatcctttgttgaaaatatttaggaaagaatggagtttttgaaatataaaatcaataataatttttattttttgttcagcacacatggcaacacagagctgtgaagacagacgtggttagcacaaaccacttgggccagtgaaaccagggcaaactcatggatcatctgcgttcccatcttcaccttggtggcagccctacctctgagattttaaggtctacggaaagtgcaggcttccaggagtgatgaggtggagcattttctcaggttaccaacagccttgacatattcttctcctaagtatttttcatatgtgtttctgtcatgaagtttggccaaacatactgtgtcatctctgaacagaaggtccttggtttccgaccggaacaaacaaaagttgcccgagcagtcagttacgttgcttccaaataggtgctgctgttgacgtaatatcttgtggacgcaagcttccttatctttccgtgtgaccacagcgtgattcggggctctggccaggtggcagttcgcatactcctccacaggtttcctggtaccatcaaggcacagcaactcatagtctttttcattcagattcttagcccatggatcagggttttttcccccagtgttctgtgggacagtctggtgtttcacaaaggccacatctcccttctcaaccagacacctgaaagcgcctgtgtagccgtagtatccctctttgttgttgggttcacacaggtttaggcctgagcccatacacagcttacagagactggagtctttcttagacccaggggcacaaccttcactgaaaaattcatcaaatctgcagtggttgatcttattgtagagcaggcccatggggatgttccagccagcggttctgccaactgccgtatggcaggacttcttgcctttcagattgtcccaggtgaggtcagaagctgatttcttcaccactgctatagcaaaataccctgcctctggtgtatcctcacaattatcgctcttattgtagttttctgccaagacaggcaccagaccacacttgcccgctatgtagacaaaccctccatccaagctcatggcatcagcttctccattcatgatcttggcgatgcagtcttcggtggtctctgctgatacacactctattttccctacactgttaacactccactcatcacacttgagcctctcgtggtggctcagcgcacaccacttcacaggcttgcattcatctgttggggcttctgggcatgtgccttcccgtagattccggatggcagtgacatactcatagcccaggtacatcttggcatccatcctgggggggacttttaaaaacccgtgggcagagtccttaaacagcaggtccttcccatgaggagagctgaatagttggaattcttttgatttgtctttgccaaaatgttcctgggcctggttgagaagctcccagatcaagtcctccttgccgcccatacttcgggccacgacggtatgagaagggacctgggccaagtggcagtccttgtattcatctaccggcttccgggtgttgtccaggcaaagcagctcatactggtccctgtcagccttgtttgccaagttctcaaatatagtcgagtgcttgacaaaggccacatccccagcaccatccttcagacacttgaaggctcccgagtagccgaagtattggttaagggtggagcagccacaccctggacacagttgacacagctgggggaagtccgtcccatccgcacaaggggcacagctgcccgagaagaaattggccactgctttctcaagaggtttacgtggctcaggtaagtcacagtaaagtaagcctatggggatgttccacccagcggacctgcctagacccgtgtggcaggacttcttgcctcgaagctggttcatctggaagccactatccttcttcaccacagcaacagcataatagaaagtctgtggatcctcttttgacccatagaactctgccaccacaggcttcaggttattgggagccaggtaagcatcatacaccaaacctgcatccagtgtcacagcatccgcttcgtttgccgcaatggccctgatgcaatcaaggtaggaggctttcttcacacaagcaacactgggaccatcggatggaatgacgcttttcatatggtcgcggaaactctggcacttagtggcctcatgctccgacactgcacaccatctcacagttttatcagggacagccagacacagccccaggacggcgcagaccagcagggctcccacggcgagcctcatcttccgggtgcggcgctgagcagcgagcacagtcggactcgcttctgt

SEQ ID NO: 11953 - RNA, 3878 nt, Homo sapiens
  source 1..3878: mol_type = other RNA
ctgaatagctgggactacaggtgtgtgccaccacaccaggataatttatgtatttttagtagtgatggggtctcactacattgcccaggctggtctcgaacttctggcctcaagtgatcttcccgcctcagcctctcaaagtgctgggattaccggtgtgagcccctgcatccgacccaaagtctcgttatcttcacctgttgtatggaaagtttgtagccacttgtctgcatccccgattggcttatgtggctggccaggaggatgctgatggtctgagagcttattgcagaaagtgtctgcaggtgcccttagtatgtgtcaggctgagctaagttattctactattcctttttagagctctaatattgtaccctaatccaaaagtgtttggagagaataaaaactacccattctggctgggcacggtggctcacgcctgtaatcccagcactttgggaggccgagatgggcagatcgcttgagctcaggagttggagaccagcctgagccacctggcaagaacctgtctctacaaaaaatacaaaaaagtagccaggcatggtgcccacctgccagtagtcccagctactcgagaggctgaggtgagaggattgcttaagccctggaggttgaggctgcagtgagccatgatcatgccactgcactccagcctgggtgacagagaggccctgtctcaacaaataaacaaatgaaatgaaacaaaacaaaacaaaaatacccatccctaaatagcatccagctctctgtgtgcctttctctttgatagtttatgactagacttccttaatcagctacaaaggaaggcttaaagaaattatggaaatacctagccacaaagaacactttagagtggaggagtcagagagaaggagagtgcgagaggaatggacgtttcctcccttctttttggatgggcttaaatcatggatagtgtctcacattgaatggaagtgggaacaaagcttggacataaaggagatggggtggaaagcagcagtgggagctggaagggaactcttggctggccagcctgcacaaaggggagcagcacatttcacagaaaaatacatttatgcagctggccaggaggatgctgatggtctgagagtgaattgcagaaaatgtgtgcatgtgcccttagcatgggtgaggctgagctaagtgagtctacccttcctttttaaaagctctaatattgtcccctaaccaaaagatatgggaatcttagaatgacatttgcactttcagttatgttagttattacaagcacacaggccttacctactcccagaaagcatgcaaattatcttaccaagagatttcataacataatacagttagaatatattaaaatgagattcataaccgctaaatgtgaggcaaagctaattgtaacaagaacctcaaataaaataggaatctgggttttacctttgtgtttcctagaagccacagcaaaaagataaaataagggaacctacagctcataaaaggtagcagacaattttgactggaatctctttctcctcctctaaagtatgttagagtctctcctatgcatgggtggggtctgtgatgtttgcattggacctgcaaaatcatccagccctgtttcttcatttttcagggatgcagatggagattcagaggtgacagtgatgtgcccaaggacacaggtgtcagaagtgggatttcctttctcacggtaccaaatggccagcttggtttgtcagcctgttgtcttatcccaccatgactgtggtcagatgaaaaaactcggctcttgcttcatctgttccctgcagctgcagtccgtttggatagactcagacttaggggtggacgtgaggcagggctcatgggcagtcctcagctgtggcaatgacacccacacaccaacagctgcatggtgacttagctcccttttgggctccagcggctcctctagctctgagatactgagggttcttccagggaagcctgcactggggcagaagcctctacatgggcctgtgcctaggatggggctaatgtcggccatggtgtcggggaagggcgccaagcccactgggtggggcgatgcaggctgggcagggctgctctttcccagcctccttccagagtgggccgtttgcagagtagctgggctgccttcttgttgtgaggatgtggccacttctgcagtggcgctgaagtacaacgtggaactctgctgtccttcccctcctctctgctgcccacctgtccccttcccctgtgtcccagaaacagcgtcagctccttcctttggggtgccctccccctgcgtggctgctgggttctgggtaggtgcttcatcctgctgatcgctggcaaaagatacgtaacttgaggtttccaatgggtcggcctctgctttagggacaccttcaaacgcagagctgttctctaaggttgaggggtcacgggatgaggatgggagctcttgctgggcagacaaggcctttctctgcaggtagtcctgttgactcaacccccatgcaggtggacaataggcaggactgttatctccaaaggcggcattgatcttagacacatttcctgtttttagggcaagtttcacccacagccagtggtgatgactgaggaaagagtcctccacagcaacctgggtccccagcccagcctctggggggacctgctcaggggtagggggcttccctaaaatggttggttcataacttgccccttggcatgagcctgagctctcggttctcttcccagctagatctgtggcccggggagaatctcttctctctgttttatcacctcctgcaatgccacaggacttccttaggcagccctgccagatgtctgtggattttggatgcagcaggctgtaataaattaccagtgagacactgccaatcagaaatccagacaggaccccagctatggtctgcaggctggtccacgatgccccctggagaaagtcggtggccaacagcaacaggatgatgttctccaacagcatgaccatgtagaacgtgaccatcctatttctagaagggctgtcccagaagctgaggtagcagaggatgtacacggcccccacgagcaggttgaacagcctccagtggcaggtgctgtcgatgatgtcactctgctgggcgacaagccagaatgtcatcaccagccagtgggcacctgcaaccacaaaaacccaaaagtggtaggctttgtagaacagaaccagactcagcacgcgggttcccaacatgcccatcctccagagctgctggcagaagagggcggcccatggcatggccaggtggcctggcttcatgaagcccatgaagcgagtgtaggacaccagtgcccaggagagtgaggaccaggaaaacagggtgctcacccctggcacaatatctgtgaagtctgaggctagaaaaacatatgtctgaagcagcaggtggggcccagtctgcagcagggcctccaagagtcgaagggccgacaggtcggcctcctgcagctgcagccagcctcggtggggagcctccagttccttctgcagactggtcagtgcagcgtcccagtgccgcttccaaacaccaagctgtaggaggtgcagcatcatcaaggagcaatgccctggatgcccgtctgctcggaaccacaggtagctcagggcctggaccaagaacccgggcaggaggacagcaagggccagccacccccacagaagccgtcctgtggtgaagtagtaagccacggtgtaaaggcgcgcgctctgctcggccgcctgcagcagggccgagagccccaggagcctcgcgtgcatcttccgtgccgaccccgcagcctgcgcccgc

SEQ ID NO: 11954 - RNA, 4016 nt, Homo sapiens
  source 1..4016: mol_type = other RNA
ctgaatagctgggactacaggtgtgtgccaccacaccaggataatttatgtatttttagtagtgatggggtctcactacattgcccaggctggtctcgaacttctggcctcaagtgatcttcccgcctcagcctctcaaagtgctgggattaccggtgtgagcccctgcatccgacccaaagtctcgttatcttcacctgttgtatggaaagtttgtagccacttgtctgcatccccgattggcttatgtggctggccaggaggatgctgatggtctgagagcttattgcagaaagtgtctgcaggtgcccttagtatgtgtcaggctgagctaagttattctactattcctttttagagctctaatattgtaccctaatccaaaagtgtttggagagaataaaaactacccattctggctgggcacggtggctcacgcctgtaatcccagcactttgggaggccgagatgggcagatcgcttgagctcaggagttggagaccagcctgagccacctggcaagaacctgtctctacaaaaaatacaaaaaagtagccaggcatggtgcccacctgccagtagtcccagctactcgagaggctgaggtgagaggattgcttaagccctggaggttgaggctgcagtgagccatgatcatgccactgcactccagcctgggtgacagagaggccctgtctcaacaaataaacaaatgaaatgaaacaaaacaaaacaaaaatacccatccctaaatagcatccagctctctgtgtgcctttctctttgatagtttatgactagacttccttaatcagctacaaaggaaggcttaaagaaattatggaaatacctagccacaaagaacactttagagtggaggagtcagagagaaggagagtgcgagaggaatggacgtttcctcccttctttttggatgggcttaaatcatggatagtgtctcacattgaatggaagtgggaacaaagcttggacataaaggagatggggtggaaagcagcagtgggagctggaagggaactcttggctggccagcctgcacaaaggggagcagcacatttcacagaaaaatacatttatgcagctggccaggaggatgctgatggtctgagagtgaattgcagaaaatgtgtgcatgtgcccttagcatgggtgaggctgagctaagtgagtctacccttcctttttaaaagctctaatattgtcccctaaccaaaagatatgggaatcttagaatgacatttgcactttcagttatgttagttattacaagcacacaggccttacctactcccagaaagcatgcaaattatcttaccaagagatttcataacataatacagttagaatatattaaaatgagattcataaccgctaaatgtgaggcaaagctaattgtaacaagaacctcaaataaaataggaatctgggttttacctttgtgtttcctagaagccacagcaaaaagataaaataagggaacctacagctcataaaaggtagcagacaattttgactggaatctctttctcctcctctaaagtatgttagagtctctcctatgcatgggtggggtctgtgatgtttgcattggacctgcaaaatcatccagccctgtttcttcatttttcagggatgcagatggagattcagaggtgacagtgatgtgcccaaggacacaggtgtcagaagtgggatttcctttctcacggtaccaaatggccagcttggtttgtcagcctgttgtcttatcccaccatgactgtggtcagatgaaaaaactcggctcttgcttcatctgttccctgcagctgcagtccgtttggatagactcagacttaggggtggacgtgaggcagggctcatgggcagtcctcagctgtggcaatgacacccacacaccaacagctgcatggtgacttagctcccttttgggctccagcggctcctctagctctgagatactgagggttcttccagggaagcctgcactggggcagaagcctctacatgggcctgtgcctaggatggggctaatgtcggccatggtgtcggggaagggcgccaagcccactgggtggggcgatgcaggctgggcagggctgctctttcccagcctccttccagagtgggccgtttgcagagtagctgggctgccttcttgttgtgaggatgtggccacttctgcagtggcgctgaagtacaacgtggaactctgctgtccttcccctcctctctgctgcccacctgtccccttcccctgtgtcccagaaacagcgtcagctccttcctttggggtgccctccccctgcgtggctgctgggttctgggtaggtgcttcatcctgctgatcgctggcaaaagatacgtaacttgaggtttccaatgggtcggcctctgctttagggacaccttcaaacgcagagctgttctctaaggttgaggggtcacgggatgaggatgggagctcttgctgggcagacaaggcctttctctgcaggtagtcctgttgactcaacccccatgcaggtggacaataggcaggactgttatctccaaaggcggcattgatcttagacacatttcctgtttttagggcaagtttcacccacagccagtggtgatgactgaggaaagagtcctccacagcaacctgggtccccagcccagcctctggggggacctgctcaggggtagggggcttccctaaaatggttggttcataacttgccccttggcatgagcctgagctctcggttctcttcccagctagatctgtggcccggggagaatctcttctctctgttttatcacctcctgcaatgccacaggacttccttaggcagccctgccagatgtctgtggattttggatgcagcaggctgtaataaattaccagtgagacactgccaatcagaaatccagacaggaccccagctatggtctgcaggctggtccacgatgccccctggagaaagtcggtggccaacagcaacaggatgatgttctccaacagcatgaccatgtagaacgtgaccatcctatttctagaagggctgtcccagaagctgaggtagcagaggatgtacacggcccccacgagcaggttgaacagcctccagtggcaggtgctgtcgatgatgtcactctgctgggcgacaagccagaatgtcatcaccagccagtgggcacctgcaaccacaaaaacccaaaagtggtaggctttgtagaacagaaccagactcagcacgcgggttcccaacatgcccatcctccagagctgctggcagaagagggcggcccatggcatggccaggtggcctggcttcatgaagcccatgaagcgagtgtaggacaccagtgcccaggagagtgaggaccaggaaaacagggtgctcacccctggcacaatatctgtgaagtctgaggctagaaaaacatatgtctgaagcagcaggtggggcccagtctgcagcagggcctccaagagtcgaagggccgacaggtcggcctcctgcagctgcagccagcctcggtggggagcctccagttccttctgcagactggtcagtgcagcgtcccagtgcctttagagtttaccttaactttccttttgacaaccttgaactttcactaaagaaaaattgctaaaccaaggtgcatgctaaggatgagataggccttcttctgtcatctcatgctgcatttacaagtggatttgtgggcgcttccaaacaccaagctgtaggaggtgcagcatcatcaaggagcaatgccctggatgcccgtctgctcggaaccacaggtagctcagggcctggaccaagaacccgggcaggaggacagcaagggccagccacccccacagaagccgtcctgtggtgaagtagtaagccacggtgtaaaggcgcgcgctctgctcggccgcctgcagcagggccgagagccccaggagcctcgcgtgcatcttccgtgccgaccccgcagcctgcgcccgc

SEQ ID NO: 11955 - RNA, 53 nt, Homo sapiens
  source 1..53: mol_type = other RNA
ctgaatagctgggactacaggtgtgtgccaccacacccagctaattctatttt

SEQ ID NO: 11956 - RNA, 1028 nt, Homo sapiens
  source 1..1028: mol_type = other RNA
ctgaatagctgggactacaggtgtgtgccaccacacccagctaatttttgtatttttagtagagacagggtttcaccatgttggccaggatggtctcgatcgcttgacctcgtgatccgcctgcctcggactcccagtgctgggattacaggcatgagccaccgtgcccagccaaaccattcttaacaagaaacaacactaaatcttcctttttcttcttgtctcacaggctgttctcaaggaaaaaagaaaaaagaaatttaaggaaaaaaataatgccaaaaggaaaatctacagattcaaaaacctttgggtttctaagttctttttaaagaactgctaggaaattttcttctataaattctggaaaagaaaaacaaaatgctgatgattaccttataatgaattcttctaatgaatttaaaatcttaaagatgaattcaagaaaaacaaaataatttcattattcccttgtatctaacaaaaacctaataatttaacaaagaacacttagtgtattacagactgagtatatcccttatccaaaatgcctgggaccagaagtattttggaatttttggacttccaaatatttgcaatattactagttgagtatctctaattcaaaaatctgaagtgctccaatgaacatttcctttcagtgtcgtgtcagggctcaaagttttgaattttggagcatttcagatttcagattttcagattagggatactcaacccatacatggattattaaacttacacagcagggtcttgataagttcacatccaaaaccaatgtttacaaaaatctgcaggttaggaaatcaacattttcttccttatttaggaagtatctgtcatgatgtctttgaataattttcaatgagtttatttcagtgtgatgatcaatgagatggcaaggaactcatgtcctttttactgatttcctcatttttataaaatgagcgttttcattcttaaatggccttcaatgtcccattctaagtaatactttaatacatcaaatt

SEQ ID NO: 11957 - RNA, 4056 nt, Homo sapiens
  source 1..4056: mol_type = other RNA
ctgaatagctgggactacaggtgtgtgccaccacacccggctaatttttgtatttttagtagagatggggtttcaccatctcgaacttctgacctcatgatccacctgcctcggcctcccaaagtgttgggattacaggcgtgagccaccgcacccagcagaagttttcttttttcaactatctgtatttgattttggtgttaaaatttattctgacttaataaaataaatgagtacagttcatggattgtattacatccatataataaataacactggtattactctttctttaaaagatagaactaagcatgaactcttctgagcctggagcattttcccattatagatctttaatagcttttttgagtttttcaatgttaactatcctaccaagttttctacttcttattgcagttttcataacttaagtttattagaaaagcatccacctcctctttttaaaaaatatgttgattagagttgtatgaggtatctttttatcacttaaaaaatcatattgatatctgtggttatgtctcctttctcattctggatcaggcagtcttacatggagggaaatcttgaaaaatgtagattccacatggccatttattttctaatatggatgacatagcaactcagggaagcagacttctttccaaacattgaaataattaaaaccttgggatttagtgtctaggacacttgcaaggaaatttatatgaaaaaaatgaatattcttgaattaatttgcagagggatagagagaaaagaaattctccttcagtggtctacgcatgaaacatttctgagttatacaacctgtatatagaatagtgtatctagaatagtgtagcaatgctactaatttgctacaagatattttaagcaagactaagaaaatatgaacagtgtactgtacaccagggtgacactacattttgtcaaatagtttacagtgtttcatttacccagtatcaggttcttaaactattccttagcttgcatttttaatataaataactacattttagtaaaatttttggccaaattatccaaatacatttaaaaacactgctttattatttctgcagaggacagtaacaacctctatagccatttacatgtattacaaaaaggtggaaaaatgtagctggtataataaagttcttttaacaatagtgggccatgttgttgttatttttttgtattgttaagacatcaaaagacaatgatgatatttaaagtggaaaagttttctgaatggcattctatatgttgtgtgacatgtgtctgatattcacattttatgttaatttcacatttacaactccaaaatacaaataatgctgattgtatggctcactgtggaatataccagagtatgcctttaagtctcttcacagatattttgtattctgctgttattccatttaatacatttttaaacgtttacatgccagggtgtccatgcttatgtttgagaaagtattttctagaaaagtttgtatcacaattagatcatgatttccattatgatacaacactgtcggttgggcgcgttggctcatgcctgtaatcccaacactttgggaggccaagggcggggggttggggggtatcacgaggtcaggagttcgagaccagcctagccaaagagaccagcctgaccaacatggtgaaaccccatctctactaaaaatacaaaaattagccaggcgtggtggcaggtgcctgtaatcccagctacttgggaggctgaggcaggagaactgcttgaacctgggaggctgaggttacagtgagccgagatagtgccattgcactccagcctgggaaacagagaatacaactcaaaataaataaataaataaaataaaaacacactgttcaaattcattaaaatgataagatttctcctaaggataaattccctacataccggccaggcgcggtggctcacgcctgtaatcccagcactttgggaggacaaggcgggcagatcacaaggtcaggagatcgagaccatcctggctaacacggtgaaaccccgtctctactaaaaatacaaaaaaaaaattagccgggcatggtggtgggcacctgtagtcccagctactcgggaggctgaggcaggagaatggcgtgaacccgggaggcagagcttgcagtaagccgagatcgcgccactgcactccagcctgggtgacaaagtgagattccaactcaaaaaaaaaaaaaaaaaattccctacataccatgaaaccagatattttgctcaagtatttcccacaattattaagttttcattcctgtaggcattcttccgagcatgaattttctgatgtctgctgaggtttggcttctggtagaaagctttcccacattcattgcacccatagggcttctctcctgtgtgagttctccaatgtttattgaggcatgacttctggctgaaggattttccacattctctgcaacgatacggtctttctcctgtgtgcatttttcgatgtacattgaggtatgacttctcaccaaacgatttcccgcattcactgcagacaaagggtctctctcctgtgtgtgttctctgatgttctgtgcggtgtgacttctgggtaaaggctttcccacaaaaaaaacattcaaagggtcttaccccagtgtgaattctctggtgtttgatgagggttgacttatgtgaaaaggctttcccacagtcagtgcagccataaggcttctccccagtgtgacttctctgatgcctaatgaattcagacttgtagcagaaggctttcccacactcactacagacgtggggtttttctgtaggtggaaccctcttccgtttgtacaagagagaatcacttactgctggtttatacataagtgccgggttctgggtgaaagctttctcacagtgactgcaaccccggggcttttctccattaggtcgtctaccatgatttatacgctgaagcaatttcccataagcataacactcatcttgcttttttgcacagtttctcttaaaaccaatcaagtctaaattatggttcaaattctttccacaagggttccagttactagggctctggattgaagaaaaaagatcagtgctcagaagtgatattttcccaaacttattatattcacagcttttctccttgggcaatgttttcttgcttatggctgcgcctggcctcaaaagcatgtcttgccgtcttttcctctggatattaactcgccagatgtcttcccaacagtggcagcccgggcatgctgcctcaccaatccatggtgcttcttcctgctccagtctgaggatcacatctggtttggtgccttcataacccactgagacgaggttgctataggtttccagcatcacatcccggtacagggccctctgagcaggactcagccggtgccactcctcttgggtgaagcccacaaccacatctttgaatgacacaggtatctggtattcgatcattttctgctgttcttgaaaaagatctgacacctatactcttcaaaaatgtcgacttcatggaagatgaacactgagaaactgctcctgattaaaggagactaaagggatgtgtcacctaaaggcagcatatgatcctggattagatcacttagctgcagggccttctgtagatgttgtgaccaaggtcctgtggctctaagggctggcaggagctagagagccctcccgtccagcaaggtggcaggatccaaaggtctgcagggcacccagagaactcagtaaatttgttttctaaccacgggcaaggtcacatccatccccgctgtcacagagtcagaatggatttccagaaaccagcctcactcttgggatgctggcacagatgcgtatgtcattacctttgccagaaagagccccatgcaccctgaaaatcaagacatttcacagaactcgcatttattgattcccacacactcccaatccatcttcttcagagaccgtgccactgactcccgcaaacctctgtccgccaccactgaggccccgcgaggctc

SEQ ID NO: 11958 - RNA, 3944 nt, Homo sapiens
  source 1..3944: mol_type = other RNA
ctgaatagctgggactacaggtgtgtgccaccacacccggctaatttttgtatttttagtagagatggggtttcaccatctcgaacttctgacctcatgatccacctgcctcggcctcccaaagtgttgggattacaggcgtgagccaccgcacccagcagaagttttcttttttcaactatctgtatttgattttggtgttaaaatttattctgacttaataaaataaatgagtacagttcatggattgtattacatccatataataaataacactggtattactctttctttaaaagatagaactaagcatgaactcttctgagcctggagcattttcccattatagatctttaatagcttttttgagtttttcaatgttaactatcctaccaagttttctacttcttattgcagttttcataacttaagtttattagaaaagcatccacctcctctttttaaaaaatatgttgattagagttgtatgaggtatctttttatcacttaaaaaatcatattgatatctgtggttatgtctcctttctcattctggatcaggcagtcttacatggagggaaatcttgaaaaatgtagattccacatggccatttattttctaatatggatgacatagcaactcagggaagcagacttctttccaaacattgaaataattaaaaccttgggatttagtgtctaggacacttgcaaggaaatttatatgaaaaaaatgaatattcttgaattaatttgcagagggatagagagaaaagaaattctccttcagtggtctacgcatgaaacatttctgagttatacaacctgtatatagaatagtgtatctagaatagtgtagcaatgctactaatttgctacaagatattttaagcaagactaagaaaatatgaacagtgtactgtacaccagggtgacactacattttgtcaaatagtttacagtgtttcatttacccagtatcaggttcttaaactattccttagcttgcatttttaatataaataactacattttagtaaaatttttggccaaattatccaaatacatttaaaaacactgctttattatttctgcagaggacagtaacaacctctatagccatttacatgtattacaaaaaggtggaaaaatgtagctggtataataaagttcttttaacaatagtgggccatgttgttgttatttttttgtattgttaagacatcaaaagacaatgatgatatttaaagtggaaaagttttctgaatggcattctatatgttgtgtgacatgtgtctgatattcacattttatgttaatttcacatttacaactccaaaatacaaataatgctgattgtatggctcactgtggaatataccagagtatgcctttaagtctcttcacagatattttgtattctgctgttattccatttaatacatttttaaacgtttacatgccagggtgtccatgcttatgtttgagaaagtattttctagaaaagtttgtatcacaattagatcatgatttccattatgatacaacactgtcggttgggcgcgttggctcatgcctgtaatcccaacactttgggaggccaagggcggggggttggggggtatcacgaggtcaggagttcgagaccagcctagccaaagagaccagcctgaccaacatggtgaaaccccatctctactaaaaatacaaaaattagccaggcgtggtggcaggtgcctgtaatcccagctacttgggaggctgaggcaggagaactgcttgaacctgggaggctgaggttacagtgagccgagatagtgccattgcactccagcctgggaaacagagaatacaactcaaaataaataaataaataaaataaaaacacactgttcaaattcattaaaatgataagatttctcctaaggataaattccctacataccggccaggcgcggtggctcacgcctgtaatcccagcactttgggaggacaaggcgggcagatcacaaggtcaggagatcgagaccatcctggctaacacggtgaaaccccgtctctactaaaaatacaaaaaaaaaattagccgggcatggtggtgggcacctgtagtcccagctactcgggaggctgaggcaggagaatggcgtgaacccgggaggcagagcttgcagtaagccgagatcgcgccactgcactccagcctgggtgacaaagtgagattccaactcaaaaaaaaaaaaaaaaaattccctacataccatgaaaccagatattttgctcaagtatttcccacaattattaagttttcattcctgtaggcattcttccgagcatgaattttctgatgtctgctgaggtttggcttctggtagaaagctttcccacattcattgcacccatagggcttctctcctgtgtgagttctccaatgtttattgaggcatgacttctggctgaaggattttccacattctctgcaacgatacggtctttctcctgtgtgcatttttcgatgtacattgaggtatgacttctcaccaaacgatttcccgcattcactgcagacaaagggtctctctcctgtgtgtgttctctgatgttctgtgcggtgtgacttctgggtaaaggctttcccacaaaaaaaacattcaaagggtcttaccccagtgtgaattctctggtgtttgatgagggttgacttatgtgaaaaggctttcccacagtcagtgcagccataaggcttctccccagtgtgacttctctgatgcctaatgaattcagacttgtagcagaaggctttcccacactcactacagacgtggggtttttctgtaggtggaaccctcttccgtttgtacaagagagaatcacttactgctggtttatacataagtgccgggttctgggtgaaagctttctcacagtgactgcaaccccggggcttttctccattaggtcgtctaccatgatttatacgctgaagcaatttcccataagcataacactcatcttgcttttttgcacagtttctcttaaaaccaatcaagtctaaattatggttcaaattctttccacaagggttccagttactagggctctggattgaagaaaaaagatcagtgctcagaagtgatattttcccaaacttattatattcacagcttttctccttgggcaatgttttcttgcttatggctgcgcctggcctcaaaagcatgtcttgccgtcttttcctctggatattaactcgccagatgtcttcccaacagtggcagcccgggcatgctgcctcaccaatccatggtgcttcttcctgctccagtctgaggatcacatctggtttggtgccttcataacccactgagacgaggttgctataggtttccagcatcacatcccggtacagggccctctgagcaggactcagccggtgccactcctcttgggtgaagcccacaaccacatctttgaatgacacaggtatctggtattcgatcattttctgctgttcttgaaaaagatctgacacctatactcttcaaaaatgtcgacttcatggaagatgaacactgagaaactgctcctgattaaaggagactaaagggatgtgtcacctaaaggcagcatatgatcctggattagatcacttagctgcagggccttctgtagatgttgtgaccaaggtcctgtggctctaagggctggcaggagctagagagccctcccgtccagcaaggtggcaggatccaaaggtctgcagggcacccagagaactcagtaaatttgttttctaaccacgggcaaggtcacatccatccccgctgtcacagagtcagaatggatttccagaaaccagcctcactcttgggatgctggcacagatgcgtatgtcattacctttgccagaaagagccgcggtataaggtcgtcccatcctgaat

SEQ ID NO: 11959 - RNA, 4343 nt, Homo sapiens
  source 1..4343: mol_type = other RNA
ctgaatagctgggactacaggtgtgtgccaccacacccggctaatttttgtatttttagtagagatggggtttcaccatctcgaacttctgacctcatgatccacctgcctcggcctcccaaagtgttgggattacaggcgtgagccaccgcacccagcagaagttttcttttttcaactatctgtatttgattttggtgttaaaatttattctgacttaataaaataaatgagtacagttcatggattgtattacatccatataataaataacactggtattactctttctttaaaagatagaactaagcatgaactcttctgagcctggagcattttcccattatagatctttaatagcttttttgagtttttcaatgttaactatcctaccaagttttctacttcttattgcagttttcataacttaagtttattagaaaagcatccacctcctctttttaaaaaatatgttgattagagttgtatgaggtatctttttatcacttaaaaaatcatattgatatctgtggttatgtctcctttctcattctggatcaggcagtcttacatggagggaaatcttgaaaaatgtagattccacatggccatttattttctaatatggatgacatagcaactcagggaagcagacttctttccaaacattgaaataattaaaaccttgggatttagtgtctaggacacttgcaaggaaatttatatgaaaaaaatgaatattcttgaattaatttgcagagggatagagagaaaagaaattctccttcagtggtctacgcatgaaacatttctgagttatacaacctgtatatagaatagtgtatctagaatagtgtagcaatgctactaatttgctacaagatattttaagcaagactaagaaaatatgaacagtgtactgtacaccagggtgacactacattttgtcaaatagtttacagtgtttcatttacccagtatcaggttcttaaactattccttagcttgcatttttaatataaataactacattttagtaaaatttttggccaaattatccaaatacatttaaaaacactgctttattatttctgcagaggacagtaacaacctctatagccatttacatgtattacaaaaaggtggaaaaatgtagctggtataataaagttcttttaacaatagtgggccatgttgttgttatttttttgtattgttaagacatcaaaagacaatgatgatatttaaagtggaaaagttttctgaatggcattctatatgttgtgtgacatgtgtctgatattcacattttatgttaatttcacatttacaactccaaaatacaaataatgctgattgtatggctcactgtggaatataccagagtatgcctttaagtctcttcacagatattttgtattctgctgttattccatttaatacatttttaaacgtttacatgccagggtgtccatgcttatgtttgagaaagtattttctagaaaagtttgtatcacaattagatcatgatttccattatgatacaacactgtcggttgggcgcgttggctcatgcctgtaatcccaacactttgggaggccaagggcggggggttggggggtatcacgaggtcaggagttcgagaccagcctagccaaagagaccagcctgaccaacatggtgaaaccccatctctactaaaaatacaaaaattagccaggcgtggtggcaggtgcctgtaatcccagctacttgggaggctgaggcaggagaactgcttgaacctgggaggctgaggttacagtgagccgagatagtgccattgcactccagcctgggaaacagagaatacaactcaaaataaataaataaataaaataaaaacacactgttcaaattcattaaaatgataagatttctcctaaggataaattccctacataccggccaggcgcggtggctcacgcctgtaatcccagcactttgggaggacaaggcgggcagatcacaaggtcaggagatcgagaccatcctggctaacacggtgaaaccccgtctctactaaaaatacaaaaaaaaaattagccgggcatggtggtgggcacctgtagtcccagctactcgggaggctgaggcaggagaatggcgtgaacccgggaggcagagcttgcagtaagccgagatcgcgccactgcactccagcctgggtgacaaagtgagattccaactcaaaaaaaaaaaaaaaaaattccctacataccatgaaaccagatattttgctcaagtatttcccacaattattaagttttcattcctgtaggcattcttccgagcatgaattttctgatgtctgctgaggtttggcttctggtagaaagctttcccacattcattgcacccatagggcttctctcctgtgtgagttctccaatgtttattgaggcatgacttctggctgaaggattttccacattctctgcaacgatacggtctttctcctgtgtgcatttttcgatgtacattgaggtatgacttctcaccaaacgatttcccgcattcactgcagacaaagggtctctctcctgtgtgtgttctctgatgttctgtgcggtgtgacttctgggtaaaggctttcccacaaaaaaaacattcaaagggtcttaccccagtgtgaattctctggtgtttgatgagggttgacttatgtgaaaaggctttcccacagtcagtgcagccataaggcttctccccagtgtgacttctctgatgcctaatgaattcagacttgtagcagaaggctttcccacactcactacagacgtggggtttttctgtaggtggaaccctcttccgtttgtacaagagagaatcacttactgctggtttatacataagtgccgggttctgggtgaaagctttctcacagtgactgcaaccccggggcttttctccattaggtcgtctaccatgatttatacgctgaagcaatttcccataagcataacactcatcttgcttttttgcacagtttctcttaaaaccaatcaagtctaaattatggttcaaattctttccacaagggttccagttactagggctctggattgaagaaaaaagatcagtgctcagaagtgatattttcccaaacttattatattcacagcttttctccttgggcaatgttttcttgcttatggctgcgcctggcctcaaaagcatgtcttgccgtcttttcctctggatattaactcgccagatgtcttcccaacagtggcagcccgggcatgctgcctcaccaatccatggtgcttcttcctgctccagtctgaggatcacatctggtttggtgccttcataacccactgagacgaggttgctataggtttccagcatcacatcccggtacagggccctctgagcaggactcagccggtgccactcctcttgggtgaagcccacaaccacatctttgaatgacacaggtatctggtattcgatcattttctgctgttcttgaaaaagatctgacacctatactcttcaaaaatgtcgacttcatggaagatgaacactgagaaactgctcctgattaaaggagactaaagggatgtgtcacctaaaggcagcatatgatcctggattagatcctctcccttcactctgtcttcctggatcttgggccaaccatcctcccttcatttagccatggagagtccctggaaagagtaacgtcttcaggtttggtcttgctcagcttctggctcagggatgaagctatttccttttatgtgggagtctttgctctgacaagaggtatggggtctgagtgattccttcagaagggaattttcatcccaagttcccttctcctggacagtgtctttaacctggcctgcccaggcactcacagctccatctctcaacagtaactcacacttagctgcagggccttctgtagatgttgtgaccaaggtcctgtggctctaagggctggcaggagctagagagccctcccgtccagcaaggtggcaggatccaaaggtctgcagggcacccagagaactcagtaaatttgttttctaaccacgggcaaggtcacatccatccccgctgtcacagagtcagaatggatttccagaaaccagcctcactcttgggatgctggcacagatgcgtatgtcattacctttgccagaaagagccccatgcaccctgaaaatcaagacatttcacagaactcgcatttattgattcccacacactcccaatccatcttcttcagagaccgtgccactgactcccgcaaacctctgtccgccaccactgaggccccgcgaggctc

SEQ ID NO: 11960 - RNA, 3966 nt, Homo sapiens
  source 1..3966: mol_type = other RNA
ctgaatagctgggactacaggtgtgtgccaccacacccggctaatttttgtatttttagtagagatggggtttcaccatctcgaacttctgacctcatgatccacctgcctcggcctcccaaagtgttgggattacaggcgtgagccaccgcacccagcagaagttttcttttttcaactatctgtatttgattttggtgttaaaatttattctgacttaataaaataaatgagtacagttcatggattgtattacatccatataataaataacactggtattactctttctttaaaagatagaactaagcatgaactcttctgagcctggagcattttcccattatagatctttaatagcttttttgagtttttcaatgttaactatcctaccaagttttctacttcttattgcagttttcataacttaagtttattagaaaagcatccacctcctctttttaaaaaatatgttgattagagttgtatgaggtatctttttatcacttaaaaaatcatattgatatctgtggttatgtctcctttctcattctggatcaggcagtcttacatggagggaaatcttgaaaaatgtagattccacatggccatttattttctaatatggatgacatagcaactcagggaagcagacttctttccaaacattgaaataattaaaaccttgggatttagtgtctaggacacttgcaaggaaatttatatgaaaaaaatgaatattcttgaattaatttgcagagggatagagagaaaagaaattctccttcagtggtctacgcatgaaacatttctgagttatacaacctgtatatagaatagtgtatctagaatagtgtagcaatgctactaatttgctacaagatattttaagcaagactaagaaaatatgaacagtgtactgtacaccagggtgacactacattttgtcaaatagtttacagtgtttcatttacccagtatcaggttcttaaactattccttagcttgcatttttaatataaataactacattttagtaaaatttttggccaaattatccaaatacatttaaaaacactgctttattatttctgcagaggacagtaacaacctctatagccatttacatgtattacaaaaaggtggaaaaatgtagctggtataataaagttcttttaacaatagtgggccatgttgttgttatttttttgtattgttaagacatcaaaagacaatgatgatatttaaagtggaaaagttttctgaatggcattctatatgttgtgtgacatgtgtctgatattcacattttatgttaatttcacatttacaactccaaaatacaaataatgctgattgtatggctcactgtggaatataccagagtatgcctttaagtctcttcacagatattttgtattctgctgttattccatttaatacatttttaaacgtttacatgccagggtgtccatgcttatgtttgagaaagtattttctagaaaagtttgtatcacaattagatcatgatttccattatgatacaacactgtcggttgggcgcgttggctcatgcctgtaatcccaacactttgggaggccaagggcggggggttggggggtatcacgaggtcaggagttcgagaccagcctagccaaagagaccagcctgaccaacatggtgaaaccccatctctactaaaaatacaaaaattagccaggcgtggtggcaggtgcctgtaatcccagctacttgggaggctgaggcaggagaactgcttgaacctgggaggctgaggttacagtgagccgagatagtgccattgcactccagcctgggaaacagagaatacaactcaaaataaataaataaataaaataaaaacacactgttcaaattcattaaaatgataagatttctcctaaggataaattccctacataccggccaggcgcggtggctcacgcctgtaatcccagcactttgggaggacaaggcgggcagatcacaaggtcaggagatcgagaccatcctggctaacacggtgaaaccccgtctctactaaaaatacaaaaaaaaaattagccgggcatggtggtgggcacctgtagtcccagctactcgggaggctgaggcaggagaatggcgtgaacccgggaggcagagcttgcagtaagccgagatcgcgccactgcactccagcctgggtgacaaagtgagattccaactcaaaaaaaaaaaaaaaaaattccctacataccatgaaaccagatattttgctcaagtatttcccacaattattaagttttcattcctgtaggcattcttccgagcatgaattttctgatgtctgctgaggtttggcttctggtagaaagctttcccacattcattgcacccatagggcttctctcctgtgtgagttctccaatgtttattgaggcatgacttctggctgaaggattttccacattctctgcaacgatacggtctttctcctgtgtgcatttttcgatgtacattgaggtatgacttctcaccaaacgatttcccgcattcactgcagacaaagggtctctctcctgtgtgtgttctctgatgttctgtgcggtgtgacttctgggtaaaggctttcccacaaaaaaaacattcaaagggtcttaccccagtgtgaattctctggtgtttgatgagggttgacttatgtgaaaaggctttcccacagtcagtgcagccataaggcttctccccagtgtgacttctctgatgcctaatgaattcagacttgtagcagaaggctttcccacactcactacagacgtggggtttttctgtaggtggaaccctcttccgtttgtacaagagagaatcacttactgctggtttatacataagtgccgggttctgggtgaaagctttctcacagtgactgcaaccccggggcttttctccattaggtcgtctaccatgatttatacgctgaagcaatttcccataagcataacactcatcttgcttttttgcacagtttctcttaaaaccaatcaagtctaaattatggttcaaattctttccacaagggttccagttactagggctctggattgaagaaaaaagatcagtgctcagaagtgatattttcccaaacttattatattcacagcttttctccttgggcaatgttttcttgcttatggctgcgcctggcctcaaaagcatgtcttgccgtcttttcctctggatattaactcgccagatgtcttcccaacagtggcagcccgggcatgctgcctcaccaatccatggtgcttcttcctgctccagtctgaggatcacatctggtttggtgccttcataacccactgagacgaggttgctataggtttccagcatcacatcccggtacagggccctctgagcaggactcagccggtgccactcctcttgggtgaagcccacaaccacatctttgaatgacacaggtatctggtattcgatcattttctgctgttcttgaaaaagatctgacacctatactcttcaaaaatgtcgacttcatggaagatgaacactgagaaactgctcctgattaaaggagactaaagggatgtgtcacctaaaggcagcatatgatcctggattagatctcagtaaatttgttttctaaccacgggcaaggtcacatccatccccgctgtcacagagtcagaatggatttccagaaaccagcctcactcttgggatgctggcacagatgcgtatgtcattacctttgccagaaagagccccatgcaccctgaaaatcaagacatttcacagaactcgcatttattgattcccacacactcccaatccatcttcttcagagaccgtgccactgactcccgcaaacctctgtccgccaccactgaggccccgcgaggctcagacgccgaatctcttaacccttcagttcccttgtcatt

SEQ ID NO: 11961 - RNA, 2307 nt, Homo sapiens
  source 1..2307: mol_type = other RNA
ctgaatagctgggactacaggtgtgtgccaccacacccggctaattttttgtatttttagtagagtcggggtttcaccgtgttggccaggctggtctcgaactcctgaccttgtgatccgcccgcctcgggctcccaaagtgttgggattacaggcgtgagccaccgcccccggcccgatggtcagttttatgtgtcaacttggacgggctacagtcccagttattcaaacactcatctagctgtcgccatggaagtgttttgtagatgtgattaaagtccataatcagttgactttagataagggagattatcctacaaaatcgggggattgggtaaaaaactgattcaattagataaatgggcaaaactgaggctcccctgaaggagaaattcctcctagggacagcgcttcagccttccttcttgccctacatgctcgggcacttcaaggaagaataaggggaggaatttcctgggacacacagctggccatttcccagttttccagtgtggggacttgggctcagcgtgaatcacagaggtatccatggtcctagggtttccttgcagacgtggggtccaggacaggaggccatggagtgcgaatgtgggaaccatggcacagaagatactgggtggggcagttctccaaccaggctgagtcacttgaggctttcacaccccaacatctgagcctgggctggtagctccgccctgcacttgctcaggcctgaaggctgaggctgagcttcctgaagcttccagggaagcagggagtctgagggggcactccctccttgaagccccctccccagtgcctgcttcccggagctggggctcaggcgcctgggttcttccccaggactgatgattcaccccggctggggccttttcacttctcctttggggctaaaaatactgggacccaggcatccagctgggccagccttgccacaaattgcacaacgcccctcactcaagttccgctgacgcaggcttgggtgggggcctgagttgctccctgctcagacctgtggagctcagagcctgggcccctccactgctcctctcctaggccaaggaccctggggtctgggctgacatgcgagccgctgggggactctgggcttggctgtggcccctggaaatgaagtcccttcccttagccccagataacccaggggtgctggccccctgcatagacacagagtcccagttaggagctggggatagaagacagctaaaggggactaagagagagaggtcagagtgagagaaataggaccatggggagaaacacattaacaggaacagagaaacaagggaaaaagagacaggatgagagagacacaactgtaatagagacacagaggagtggcacacagagaccacctcccagctggagacagtcaggaaggactgagggagaggggacagccagggctccacacccaggcaagaatgggggagggcctgtggaacagagaagtcatcaacacacacagttcaaagtctaccctaggctaggagggggagcaggaagaaggggcagggacgcaggggcccggcctgcgagctccctgttggcctctgctgccccctgctggctcccgctgcggtgctcaggcaggaagagaggaggctgctgtgtttaggcccaggacgctcttcattccctttgcacaccacccaccaaccactgcctgccccactccctgtcccccacttcacagagtgcccccagggccagcaggtggtgcgggtgtcttgcccgtgaccttgttggcacagtccagcagggcggtgtgaatgtccttggcacaggaaatctgggctttgatgaccgccaggtactgtgggtaggggaggctgtcaggctgcactgcgtcgggcttggtggcaggcacagctccagctggtcacagagtgcatagaactcttccaggcacttgtcaaagcgctgtatgggtccatcactgctcttttgtccattgtcgatgttagtgttctgaatcaagttttgggccgcaaccttcatcaaggtctgtagactctccttcagctgcgggatgagcatcttataacgctgcacaggatcgaagtcctgttgctgttgctgcaggaggccgctctgggcagggcccaccagttgtgctggcggttgcggctgctgctggggacccgggccgccagccgaactaggacccgatacaccagcagctgaggaagccgctgaagcttgctgctgggatgcagccatcttcctcgcgtagaccgccggaagtgcgttacgactgcgtctctc

SEQ ID NO: 11962 - RNA, 2318 nt, Homo sapiens
  source 1..2318: mol_type = other RNA
ctgaatagctgggactacaggtgtgtgccaccacacccggctaattttttgtatttttagtagagtcggggtttcaccgtgttggccaggctggtctcgaactcctgaccttgtgatccgcccgcctcgggctcccaaagtgttgggattacaggcgtgagccaccgcccccggcccgatggtcagttttatgtgtcaacttggacgggctacagtcccagttattcaaacactcatctagctgtcgccatggaagtgttttgtagatgtgattaaagtccataatcagttgactttagataagggagattatcctacaaaatcgggggattgggtaaaaaactgattcaattagataaatgggcaaaactgaggctcccctgaaggagaaattcctcctagggacagcgcttcagccttccttcttgccctacatgctcgggcacttcaaggaagaataaggggaggaatttcctgggacacacagctggccatttcccagttttccagtgtggggacttgggctcagcgtgaatcacagaggtatccatggtcctagggtttccttgcagacgtggggtccaggacaggaggccatggagtgcgaatgtgggaaccatggcacagaagatactgggtggggcagttctccaaccaggctgagtcacttgaggctttcacaccccaacatctgagcctgggctggtagctccgccctgcacttgctcaggcctgaaggctgaggctgagcttcctgaagcttccagggaagcagggagtctgagggggcactccctccttgaagccccctccccagtgcctgcttcccggagctggggctcaggcgcctgggttcttccccaggactgatgattcaccccggctggggccttttcacttctcctttggggctaaaaatactgggacccaggcatccagctgggccagccttgccacaaattgcacaacgcccctcactcaagttccgctgacgcaggcttgggtgggggcctgagttgctccctgctcagacctgtggagctcagagcctgggcccctccactgctcctctcctaggccaaggaccctggggtctgggctgacatgcgagccgctgggggactctgggcttggctgtggcccctggaaatgaagtcccttcccttagccccagataacccaggggtgctggccccctgcatagacacagagtcccagttaggagctggggatagaagacagctaaaggggactaagagagagaggtcagagtgagagaaataggaccatggggagaaacacattaacaggaacagagaaacaagggaaaaagagacaggatgagagagacacaactgtaatagagacacagaggagtggcacacagagaccacctcccagctggagacagtcaggaaggactgagggagaggggacagccagggctccacacccaggcaagaatgggggagggcctgtggaacagagaagtcatcaacacacacagttcaaagtctaccctaggctaggagggggagcaggaagaaggggcagggacgcaggggcccggcctgcgagctccctgttggcctctgctgccccctgctggctcccgctgcggtgctcaggcaggaagagaggaggctgctgtgtttaggcccaggacgctcttcattccctttgcacaccacccaccaaccactgcctgccccactccctgtcccccacttcacagagtgcccccagggccagcaggtggtgcgggtgtcttgcccgtgaccttgttggcacagtccagcagggcggtgtgaatgtccttggcacaggaaatctgggctttgatgaccgccaggtactgtgggtaggggaggctgtcaggctgcactgcgtcgggcttggtggctgtgggcaccaacgttggagagtgcttggcactgtcacaactctgtgacaggcactcatgcgccaggcgcaggcacagctccagctggtcacagagtgcatagaactcttccaggcacttgtcaaagcgctgtatgggtccatcactgctctttctgtagactctccttcagctgcgggatgagcatcttataacgctgcacaggatcgaagtcctgttgctgttgctgcaggaggccgctctgggcagggcccaccagttgtgctggcggttgcggctgctgctggggacccgggccgccagccgaactaggacccgatacaccagcagctgaggaagccgctgaagcttgctgctgggatgcagccatcttcctcgcgtagaccgccggaagtgcgttacgactgcgtctctc

SEQ ID NO: 11963 - RNA, 2377 nt, Homo sapiens
  source 1..2377: mol_type = other RNA
ctgaatagctgggactacaggtgtgtgccaccacacccggctaattttttgtatttttagtagagtcggggtttcaccgtgttggccaggctggtctcgaactcctgaccttgtgatccgcccgcctcgggctcccaaagtgttgggattacaggcgtgagccaccgcccccggcccgatggtcagttttatgtgtcaacttggacgggctacagtcccagttattcaaacactcatctagctgtcgccatggaagtgttttgtagatgtgattaaagtccataatcagttgactttagataagggagattatcctacaaaatcgggggattgggtaaaaaactgattcaattagataaatgggcaaaactgaggctcccctgaaggagaaattcctcctagggacagcgcttcagccttccttcttgccctacatgctcgggcacttcaaggaagaataaggggaggaatttcctgggacacacagctggccatttcccagttttccagtgtggggacttgggctcagcgtgaatcacagaggtatccatggtcctagggtttccttgcagacgtggggtccaggacaggaggccatggagtgcgaatgtgggaaccatggcacagaagatactgggtggggcagttctccaaccaggctgagtcacttgaggctttcacaccccaacatctgagcctgggctggtagctccgccctgcacttgctcaggcctgaaggctgaggctgagcttcctgaagcttccagggaagcagggagtctgagggggcactccctccttgaagccccctccccagtgcctgcttcccggagctggggctcaggcgcctgggttcttccccaggactgatgattcaccccggctggggccttttcacttctcctttggggctaaaaatactgggacccaggcatccagctgggccagccttgccacaaattgcacaacgcccctcactcaagttccgctgacgcaggcttgggtgggggcctgagttgctccctgctcagacctgtggagctcagagcctgggcccctccactgctcctctcctaggccaaggaccctggggtctgggctgacatgcgagccgctgggggactctgggcttggctgtggcccctggaaatgaagtcccttcccttagccccagataacccaggggtgctggccccctgcatagacacagagtcccagttaggagctggggatagaagacagctaaaggggactaagagagagaggtcagagtgagagaaataggaccatggggagaaacacattaacaggaacagagaaacaagggaaaaagagacaggatgagagagacacaactgtaatagagacacagaggagtggcacacagagaccacctcccagctggagacagtcaggaaggactgagggagaggggacagccagggctccacacccaggcaagaatgggggagggcctgtggaacagagaagtcatcaacacacacagttcaaagtctaccctaggctaggagggggagcaggaagaaggggcagggacgcaggggcccggcctgcgagctccctgttggcctctgctgccccctgctggctcccgctgcggtgctcaggcaggaagagaggaggctgctgtgtttaggcccaggacgctcttcattccctttgcacaccacccaccaaccactgcctgccccactccctgtcccccacttcacagagtgcccccagggccagcaggtggtgcgggtgtcttgcccgtgaccttgttggcacagtccagcagggcggtgtgaatgtccttggcacaggaaatctgggctttgatgaccgccaggtactgtgggtaggggaggctgtcaggctgcactgcgtcgggcttggtggctgtgggcaccaacgttggagagtgcttggcactgtcacaactctgtgacaggcactcatgcgccaggcgcaggcacagctccagctggtcacagagtgcatagaactcttccaggcacttgtcaaagcgctgtatgggtccatcactgctcttttgtccattgtcgatgttagtgttctgaatcaagttttgggccgcaaccttcatcaaggtctgtagactctccttcagctgcgggatgagcatcttataacgctgcacaggatcgaagtcctgttgctgttgctgcaggaggccgctctgggcagggcccaccagttgtgctggcggttgcggctgctgctggggacccgggccgccagccgaactaggacccgatacaccagcagctgaggaagccgctgaagcttgctgctgggatgcagccatcttcctcgcgtagaccgccggaagtgcgttacgactgcgtctctc

SEQ ID NO: 11964 - RNA, 2429 nt, Homo sapiens
  source 1..2429: mol_type = other RNA
ctgaatagctgggactacaggtgtgtgccaccacacctggctaatttttgtatttttagtaaagacgaggttttgccacgttggccaggctggtcttgaacttctgacctcaattgatctacccgcctgagcctcccaaagttcttggattacaggcgtgagccattgcgcccggccaagaacagaatattaaccaaacccatcaaatggcagtcattaaatgccaatttttaaataggtgtaaattgatagattttgaagattaacaattacctattgttaatcttcattgcctaatgaagtcattgcctaatgatgattgaatctaattagttttagatttagaatggaaacattctttgctatttatttgctatcatacttattgctaaggaactgctgcaagttactctgtagaggagacttacaacacaatagtactgactattgcaggacagatgttttctgagtaatgtaagattctgatcatcatgccaaaaaacaactcaggtatattacgtgtacaacaacagcacaccatcatttttctcattttcatataatctgtgttctgcagcatcaatagctttattttttttcagatcagattttaattttgagtacttaacactattgttgacgtgcatttcactttcttcatgtttactaagaatatgtgataaatgttgccaatctttgcacccattttcatttttcagttgattttttccttccccaaagagtttgcaatatagacaaaacacagaatcttttgaggttgaataaagtaaccaggatctagtggttttttcaccatttggaagaatccgtgtataataagtttctgaaaacttcctccctgtattatcttttggaaagttaaaatttcttacttgaggcggaacattttcaacaagagtgtcccgttgtttaatattcaaaattcggggccacgtacctggatctgcggaaagcacaactggtacaatggagtcttcaaaatttttctcttccagttgctcttgaaatgtatcagctatggttgacgtggaagaaggaggtaaattcacattctcttggatcagtaatgtatccgtgccacattctactgaaagctgtagctgtgaagtcttttcctttttttctgggattccctctatttttttcaaaagtgtatttgacgatccatataattgtttctcattttcttctctaaaagcattcctttttctattttctgatgctgttaatttttttgattttgtttccatcatctgtttatattcgttaatacaactttggcagcaaaatctcttctgctgacctccaatcaccaggatgttgtttccagtactcttactaggcatgtactctccacagtgttcacagcagttcattattagaccattggccaatctgtacttattaaagcaatggttactgcacagtttatgtgttacattatttacgctgacttcatggcgaatcaggactatgatgagttgcaaattctccattctgaaataagtctcctgccacattcattctaccagggttaaaaggtcttactccagtcttggtctgtggagttaaagatggggtgtacgtttgtatattaacaccaaaattacttgactgaagtcctttagcgacatctcccaagttggtattctatagtgatgttttatatgtaataattatgttcacatcttgcccagcattcacagagcttatacctgtttctaaggttgtaacattagtaataatgtatttcagagtcaattctgtagtgataccactattacccattcctgcatttaccttacttcttgaaagactggaagtggagaaatccaaatcgttggttttgtttttagttccaggaagtccccattcgataaaacaggaagactttttctctgctcctccatttgtttctatgtcctcttcatcatcaataacaattgtctcacttatatttcctttctgagatgccaaatctcttgaagaaggaggaattacagaataatttccttgaggcttttcattttttgatgatgcaaatatgaagtttctttgatcagctattgctggagcagaaattgaaggaggttgtatagattcaataaacacaacatcatcatcatcatcatcatcttccactggtgagttcctagatctactgactaaaggacaagctggatgaccaaatgaatcccctatgtccatgagactagttgccatggccatattccctaataaagcaggagtctgttcagtcaactctaatcctcccactgaacatttttccatgccaatgaacaatggagatatttccttcttaatttctgccaaagcctcacgacataggcttgaaggtgattcctggtcctcggcctccgcctcctcctccggaggctgcgctgctc

SEQ ID NO: 11965 - RNA, 2803 nt, Homo sapiens
  source 1..2803: mol_type = other RNA
ctgaatagctgggactacaggtgtgtgccaccacacctggctaatttttgtatttttagtaaagacgaggttttgccacgttggccaggctggtcttgaacttctgacctcaattgatctacccgcctgagcctcccaaagttcttggattacaggcgtgagccattgcgcccggccaagaacagaatattaaccaaacccatcaaatggcagtcattaaatgccaatttttaaataggtgtaaattgatagattttgaagattaacaattacctattgttaatcttcattgcctaatgaagtcattgcctaatgatgattgaatctaattagttttagatttagaatggaaacattctttgctatttatttgctatcatacttattgctaaggaactgctgcaagttactctgtagaggagacttacaacacaatagtactgactattgcaggacagatgttttctgagtaatgtaagattctgatcatcatgccaaaaaacaactcaggtatattacgtgtacaacaacagcacaccatcatttttctcattttcatataatctgtgttctgcagcatcaatagctttattttttttcagatcagattttaattttgagtacttaacactattgttgacgtgcatttcactttcttcatgtttactaagaatatgtgataaatgttgccaatctttgcacccattttcatttttcagttgattttttccttccccaaagagtttgcaatatagacaaaacacagaatcttttgaggttgaataaagtaaccaggatctagtggttttttcaccatttggaagaatccgtgtataataagtttctgaaaacttcctccctgtattatcttttggaaagttaaaatttcttacttgaggcggaacattttcaacaagagtgtcccgttgtttaatattcaaaattcggggccacgtacctggatctgcggaaagcacaactggtacaatggagtcttcaaaatttttctcttccagttgctcttgaaatgtatcagctatggttgacgtggaagaaggaggtaaattcacattctcttggatcagtaatgtatccgtgccacattctactgaaagctgtagctgtgaagtcttttcctttttttctgggattccctctatttttttcaaaagtgtatttgacgatccatataattgtttctcattttcttctctaaaagcattcctttttctattttctgatgctgttaatttttttgattttgtttccatcatctgtttatattcgttaatacaactttggcagcaaaatctcttctgctgacctccaatcaccaggatgttgtttccagtactcttactaggcatgtactctccacagtgttcacagcagttcattattagaccattggccaatctgtacttattaaagcaatggttactgcacagtttatgtgttacattatttacgctgacttcatggcgaatctctgctaatttactacaaattgtacatcttgacttattaaaaactccttttttaagattccagttgttttcacagggagacaaacaagatgtactataaaattcttggaaggatttgcttgattctactggaagaatgacattagccttctttgtagatgcatcttttttacatattatgcttcgtgtgttttgagtacgtttatgagagaaggaagaaaggcaggtggtagagcaaaagaggtgagctgatccttttcgttgataagctgtctgtcccttctgtaaaggctttttgcaatttgcacaagtgattttagctggtttagtaagttgttgttgggctgtaggctggaaattctgcttacgaagtaaggccactggtgataaagaatccacccctggctgtttctgattactgggaaatgaagctgactgggagatccaagaatcaggactatgatgagttgcaaattctccattctgaaataagtctcctgccacattcattctaccagggttaaaaggtcttactccagtcttggtcttacttcttgaaagactggaagtggagaaatccaaatcgttggttttgtttttagttccaggaagtccccattcgataaaacaggaagactttttctctgctcctccatttgtttctatgtcctcttcatcatcaataacaattgtctcacttatatttcctttctgagatgccaaatctcttgaagaaggaggaattacagaataatttccttgaggcttttcattttttgatgatgcaaatatgaagtttctttgatcagctattgctggagcagaaattgaaggaggttgtatagattcaataaacacaacatcatcatcatcatcatcatcttccactggtgagttcctagatctactgactaaaggacaagctggatgaccaaatgaatcccctatgtccatgagactagttgccatggccatattccctaataaagcaggagtctgttcagtcaactctaatcctcccactgaacatttttccatgccaatgaacaatggagatatttccttcttaatttctgccaaagcctcacgacataggcttgaaggtgattcctggtcctcggcctccgcctcctcctccggaggctgcgctgctcccagccacccccactctcagcggccctggactggaaagacagcggggataagcgtcacccggttctggctgcggctgcgcggaacgaacaagcccaccccgcttcggcgacaagcacaactccgcgaggtccagtcccggcttttcgcgctggtgaggaggc

SEQ ID NO: 11966 - RNA, 1168 nt, Homo sapiens
  source 1..1168: mol_type = other RNA
ctgaatagctgggactacaggtgtgtgccaccacatccagctaatttttgtatttttagtagagacggggtttcaccatgttggccaggatggtctcaacctcttgacctcgtgatccacctgcctcggtctcccaaagtggtgggattacaggcgtgagccactgtgcccagccagaaaagcatttttaatagaattttgatagctcttaactgagatcctaaatcaaggatttagaaatgaggtatcataaagaatagtaagattttaaagctctcaaaattacatatgatacaaataaagattgtaacagtatttaatcattgtttcaaactttattacttaatgaaacagtttctatatactgcttccaattactttaatccttttttctcattaaattttttttgttgttcttcagttgagctgagatacttttaattactttttattaactgcttccagaaaccgtaacaggtgcaggaatagattgatgatatccaagtagaggctgatggcagctaatacgtactcttcaggtgacagtttatgcatcagtgagtgtgtgtcatagatgatgaatccacagaaaagaagggctcctgcagcggctaagaccaactccattatctcactataaaaaaaaaacttcaagaatccctgctccaaatttgctgaaatccttcttagattgtagagtatacacagtcaaaccaaaaaatactgtagtagtcagtatgaaagcttgcagaataatatatacatcatagaaagtaacaacaactgccacagtcagagcttccaacagcgtaaatccaaaaagtaggtacaggttaaggggatacttatgtctgtttaaaatcaacgcaaaaatcaaacccagagatccgagggcaaacagcaaaattaaggcaggactctcatgtacaaatgtccgtacagactcaaagtataaaaaaactgttgaagtcactgtagttaagagaacctgcagagaaagaatgctgtagacttttctcagaaaggccattcggatgtgcacggtggcggaggccacgctgctgccatagttgaagtcgtcctcgatcgaggagcgagggtaccgggggtcggggtcagccatgatggcaacagcacccctaccggtcccggtccactaaccgcaacc

SEQ ID NO: 11967 - RNA, 1165 nt, Homo sapiens
  source 1..1165: mol_type = other RNA
ctgaatagctgggactacaggtgtgtgccaccacatccagctaatttttgtatttttagtagagacggggtttcaccatgttggccaggatggtctcaacctcttgacctcgtgatccacctgcctcggtctcccaaagtggtgggattacaggcgtgagccactgtgcccagccagaaaagcatttttaatagaattttgatagctcttaactgagatcctaaatcaaggatttagaaatgaggtatcataaagaatagtaagattttaaagctctcaaaattacatatgatacaaataaagattgtaacagtatttaatcattgtttcaaactttattacttaatgaaacagtttctatatactgcttccaattactttaatccttttttctcattaaattttttttgttgttcttcagttgagctgagatacttttaattactttttattaactgcttccagaaaccgtaacaggtgcaggaatagattgatgatatccaagtagaggctgatggcagctaatacgtactcttcaggtgacagtttatgcatcagtgagtgtgtgtcatagatgatgaatccacagaaaagaagggctcctgcagcggctaagaccaactccattatctcactataaaaaaaaaacttcaagaatcctgacaggcacaatatccacaaaagagcaaacagccctgctccaaatttgctgaaatccttcttagattgtagagtatacacagtcaaaccaaaaaatactgtagtagtcagtatgaaagcttgcagaataatatatacatcatagaaagtaacaacaactgccacagtcagagcttccaacagcgtaaatccaaaaagtaggtacaggttaaggggatacttatgtctgtttaaaatcaacgcaaaaatcaaacccagagatccgagggcaaacagcaaaattaaggcaggactctcatgtacaaatgtccgtacagactcaaagtataaaaaaactgttgaagtcactgtagttaagagaacccattcggatgtgcacggtggcggaggccacgctgctgccatagttgaagtcgtcctcgatcgaggagcgagggtaccgggggtcggggtcagccatgatggcaacagcacccctaccggtcccggtccactaaccgcaacc

SEQ ID NO: 11968 - RNA, 1203 nt, Homo sapiens
  source 1..1203: mol_type = other RNA
ctgaatagctgggactacaggtgtgtgccaccacatccagctaatttttgtatttttagtagagacggggtttcaccatgttggccaggatggtctcaacctcttgacctcgtgatccacctgcctcggtctcccaaagtggtgggattacaggcgtgagccactgtgcccagccagaaaagcatttttaatagaattttgatagctcttaactgagatcctaaatcaaggatttagaaatgaggtatcataaagaatagtaagattttaaagctctcaaaattacatatgatacaaataaagattgtaacagtatttaatcattgtttcaaactttattacttaatgaaacagtttctatatactgcttccaattactttaatccttttttctcattaaattttttttgttgttcttcagttgagctgagatacttttaattactttttattaactgcttccagaaaccgtaacaggtgcaggaatagattgatgatatccaagtagaggctgatggcagctaatacgtactcttcaggtgacagtttatgcatcagtgagtgtgtgtcatagatgatgaatccacagaaaagaagggctcctgcagcggctaagaccaactccattatctcactataaaaaaaaaacttcaagaatcctgacaggcacaatatccacaaaagagcaaacagccctgctccaaatttgctgaaatccttcttagattgtagagtatacacagtcaaaccaaaaaatactgtagtagtcagtatgaaagcttgcagaataatatatacatcatagaaagtaacaacaactgccacagtcagagcttccaacagcgtaaatccaaaaagtaggtacaggttaaggggatacttatgtctgtttaaaatcaacgcaaaaatcaaacccagagatccgagggcaaacagcaaaattaaggcaggactctcatgtacaaatgtccgtacagactcaaagtataaaaaaactgttgaagtcactgtagttaagagaacctgcagagaaagaatgctgtagacttttctcagaaaggccattcggatgtgcacggtggcggaggccacgctgctgccatagttgaagtcgtcctcgatcgaggagcgagggtaccgggggtcggggtcagccatgatggcaacagcacccctaccggtcccggtccactaaccgcaacc

SEQ ID NO: 11969 - RNA, 1344 nt, Homo sapiens
  source 1..1344: mol_type = other RNA
ctgaatagctgggactacaggtgtgtgccaccacatccagctaatttttgtatttttagtagagacggggtttcaccatgttggccaggatggtctcaacctcttgacctcgtgatccacctgcctcggtctcccaaagtggtgggattacaggcgtgagccactgtgcccagccagaaaagcatttttaatagaattttgatagctcttaactgagatcctaaatcaaggatttagaaatgaggtatcataaagaatagtaagattttaaagctctcaaaattacatatgatacaaataaagattgtaacagtatttaatcattgtttcaaactttattacttaatgaaacagtttctatatactgcttccaattactttaatccttttttctcattaaattttttttgttgttcttcagttgagctgagatacttttaattactttttattaactgcttccagaaaccgtaacaggtgcaggaatagattgatgatatccaagtagaggctgatggcagctaatacgtactcttcaggtgacagtttatgcatcagtgagtgtgtgtcatagatgatgaatccacagaaaagaagggctcctgcagcggctaagaccaactccattatctcactataaaaaaaaaacttcaagaatcctgacaggcacaatatccacaaaagagcaaacagccctgctccaaatttgctgaaatccttcttagattgtagagtatacacagtcaaaccaaaaaatactgtagtagtcagtatgaaagcttgcagaataatatatacatcatagaaagtaacaacaactgccacagtcagagcttccaacagcgtaaatccaaaaagtaggtacaggttaaggggatacttatgtctgtttaaaatcaacgcaaaaatcaaacccagagatccgagggcaaacagcaaaattaaggcaggactctcatgtacaaatgtccgtacagactcaaagtataaaaaaactgttgaagtcactgtagttaagagaacctgcagagaaagaatgctgtagacttttctcagaaaggttggccctttgtagaaaatgttcaccatccctgatctaccagattgccggagatgaaaaaatctgatgatattcagtgtggctgagggtgcagaaggtatcctcatatattgtttgctgaaggtacaatctctctggagaaccattcggatgtgcacggtggcggaggccacgctgctgccatagttgaagtcgtcctcgatcgaggagcgagggtaccgggggtcggggtcagccatgatggcaacagcacccctaccggtcccggtccactaaccgcaacc

SEQ ID NO: 11970 - RNA, 1271 nt, Homo sapiens
  source 1..1271: mol_type = other RNA
ctgaatagctgggactacaggtgtgtgccaccacatccggctaaactttgtattttttagtacagacggtgttttgccatgttgcccaggctggtctcagactcctgagctcaggcaatctgcccacctcggcctcccaaagtactaggattacaggcatgagccaccacacctggccttcagatgctaatctcttacagaaacaccctcacagacacctccagaaataacgtttaatcagatacctgggcattctataagctcagtcaagttgacatgcaaaattaatcactagtcatgaaattcaaagcttaaatgtagttatgatttgtggtaaacttttaggctatacttaatcaatctacattgttttattataaagagatggtaccaccctaatagtttgttgattcatatttctaacccttacatgttgtttaacttaatgttggtaagccagcttcttgctttccaaaaaataaaatacgtcgatgctgcctaactgcaattaaccaacattcttaaagcatttgccaaaatggattgtttatgagaactcatggtgctcagcactcactttcttcaataaaatcaattgaaaaggtctaactgttggtgagtgaagactgtggcggctttagctgccttctgattgcttgggcagatgtgtgtcagcatgctttctcttcttctggggagtgaaggaagtccctttatgtgtgtgcccaggactggctcctgttcctggaataaataccatcatgttgtgcagtcttgcagtttctagtaagtgctgtgcatgattggcatgtccttcagaaagcagcgagcctgagtgtttacaatgctcgtgaggtgcctccctgatagtaagtgctgctctttcttaacattcttttttcctttaaaatttgtttcaatccatgaggtaaaaaataatgacgatatagatagacgaacagttcatgttgtttttcccccaggttcaggttaaaacaaatacttcttcgtaagtaggttggtaccagttcctattgagaggtgacagcttgctggcagccctcgctggctctgggcgcctcctcggccttggcgcccactctggccgcgcttgaggaacccttcagctcaccgctgcactgtgggagcccctttctgggctggccaaggccagagccggctccctcagcttgcggggaggtgaggagggagaggagcggcggcaacggcgcggcgggaaccgaggatgcgcgcggcgcttgccagacaga

SEQ ID NO: 11971 - RNA, 2708 nt, Homo sapiens
  source 1..2708: mol_type = other RNA
ctgaatagctgggactacaggtgtgtgccaccacgcccagctaacttttttgtatttttagtagagatggggtttcaccatgttggtcaggctgatctcgaattcttgacctcaaatgatcccaaataggtgctttttaaaaagggctttaatactgtttaagtagttcaaataggcttcctcactattaatttgcttcagtaaactcttcagcttaactcattatcttaaatttcagaattaatgaggttttactgtaaaagtagaaaagcaaacacttcaaatgataagactccagtatcacccatactaaaaacttagcaataaaactgcagtttgaaaagctactgtacaatgcagcaaggactaggtgtcaatactgctggaagcagagccaggtaaagaacaggaaatctgcacagtattatccctgtggttcttagactcattcgaaatacagaactgcaatctcacaatgaaacaaacatactgcttattaggaggcactacagttaaagctttttagaaaagagagagaagtatttttaaatgtaggcacagtggtgagctgttcaaattcagttaggcgtcaacatcacacattagcagcaagatgcagccacacttcaggtttctgaatgacatgagtacagacaaaattgagcaaataaaaaccaaaacaaccactacattaaccctgagcttccacattcccctttcacatgagactaatgcagaccatcataattcaggaaaatgtggctttcattacggtcaaatctcaacatgtctcccgaagagtttataaaataagttattctaaacatgtacatttagctttggaatgatggagagacacagagatatatgtaaacgtcaagagaatcactccactccacgtctgggtccacacccttccaggctttgtctggaacattatgtggctggtgcctgattccacagtgaggatgcaggagcccaggtggtgatggataaagcattaggagacaatcaagtgtcaggaattggtcaataagaacggcttaaataatgatttaacaaggaagacgagtaaaaaacaatcccatttcatctttagaaagaattaagtcactaaatgatttcttctaagttgttgccatttgcttggatgagatcttgaaggttttccattctttctccacccagttaagaacacattgactagaaatttgtgacaagaatctagtaaaggccttttccctcctgctcctcattatgccaatgcaagaacacttatagcttcctgtgcaaagtatttgacatccatgtcttcatcttgacctaacttctgtagtactggcttcacttctccctgtaaagcattggtatctagaattggtccaatcttttgtagagatttggccacattgaagcgaacatttgctacttggtctcctgccatttttaatacgatgggcagcatttgcttagtagttatttcctgaccacaggcctcagacagtgcattaatgcagaataaagtggtcattctatgcaagtaattaggatcatttgccattactaacactttgggaacaatagtattttgggcccactctgtaccaaacttctgaactagtttcatgaggttgttggtggcagcttctcggatggcgtatacatggtccacgagccaagccatacataaagaattcagcttttcatcaaagaattccacacccagctggcctgccagcagcggcatatactcaatgatggccaggcggaccctccatttggcatcttctgccagctccactatggcaggaaggagagactgagagagctgacggattccaatcacttcatttacacaatccaaattggagatgatattcaaacgaacgtcaggacactcatcctttaactgagctaagaaaagaggtagaagatgttcaatggtattttctttgcccaaaatagtagacaatcccataattacagaagctagagccgatttgacatgttgattggtatcggatactaattcctttatataaggcagaatttgattcataattatggtctctctatcttcaatgggcaagttctcaccaagttcttttactttgtgggcagcagctgcccggacttcagcttcacagtctttaagtaggttctgaaaggcggggatgaggtcatttagggtgattttaggacccatggctttctggagctctgaaaatctgtcagccaccatatagcgaacgcgccaagatttatcttctgctgcttgtcgaagtgtaggcatcaccaaagtctcaaggtcatcctgagacaataactgggcaatactgacacaagcttccacagcaaggaggcgcactgaatccagcagacagtgggcaaagtcaggacctcccactaggccagtgaaatttcccagctgctcagcaagagctaatagtacctcatcttcatcataaattgtatctgtaagaaatggcaacaattcacttcgggtcctttctactccaagtgctagggcaattgttgataacttcttaatactgttgagtcggagctgcacgtcttcattgcggagctcgtcgattaaaaccgcgatcgggtatagcgaatcatctccatctccacccgctgctcctgggccggtcccgagctctgatgcgcccgccatgttctttctcctcctgctgctggtcacc

SEQ ID NO: 11972 - RNA, 3089 nt, Homo sapiens
  source 1..3089: mol_type = other RNA
ctgaatagctgggactacaggtgtgtgccaccacgcccagctaacttttttgtatttttagtagagatggggtttcaccatgttggtcaggctgatctcgaattcttgacctcaaatgatcccaaataggtgctttttaaaaagggctttaatactgtttaagtagttcaaataggcttcctcactattaatttgcttcagtaaactcttcagcttaactcattatcttaaatttcagaattaatgaggttttactgtaaaagtagaaaagcaaacacttcaaatgataagactccagtatcacccatactaaaaacttagcaataaaactgcagtttgaaaagctactgtacaatgcagcaaggactaggtgtcaatactgctggaagcagagccaggtaaagaacaggaaatctgcacagtattatccctgtggttcttagactcattcgaaatacagaactgcaatctcacaatgaaacaaacatactgcttattaggaggcactacagttaaagctttttagaaaagagagagaagtatttttaaatgtaggcacagtggtgagctgttcaaattcagttaggcgtcaacatcacacattagcagcaagatgcagccacacttcaggtttctgaatgacatgagtacagacaaaattgagcaaataaaaaccaaaacaaccactacattaaccctgagcttccacattcccctttcacatgagactaatgcagaccatcataattcaggaaaatgtggctttcattacggtcaaatctcaacatgtctcccgaagagtttataaaataagttattctaaacatgtacatttagctttggaatgatggagagacacagagatatatgtaaacgtcaagagaatcactccactccacgtctgggtccacacccttccaggctttgtctggaacattatgtggctggtgcctgattccacagtgaggatgcaggagcccaggtggtgatggataaagcattaggagacaatcaagtgtcaggaattggtcaataagaacggcttaaataatgatttaacaaggaagacgagtaaaaaacaatcccatttcatctttagaaagaattaagtcactaaatgatttcttctaagttgttgccatttgcttggatgagatcttgaaggttttccattctttctccacccagttaagaacacattgactagaaatttgtgacaagaatctagtaaaggccttttccctcctgctcctcattatgccaatgcaagaacacttatagcttcctgtgcaaagtatttgacatccatgtcttcatcttgacctaacttctgtagtactggcttcacttctccctgtaaagcattggtatctagaattggtccaatcttttgtagagatttggccacattgaagcgaacatttgctacttggtctcctgccatttttaatacgatgggcagcatttgcttagtagttatttcctgaccacaggcctcagacagtgcattaatgcagaataaagtggtcattctatgcaagtaattaggatcatttgccattactaacactttgggaacaatagtattttgggcccactctgtaccaaacttctgaactagtttcatgaggttgttggtggcagcttctcggatggcgtatacatggtccacgagccaagccatacataaagaattcagcttttcatcaaagaattccacacccagctggcctgccagcagcggcatatactcaatgatggccaggcggaccctccatttggcatcttctgccagctccactatggcaggaaggagagactgagagagctgacggattccaatcacttcatttacacaatccaaattggagatgatattcaaacgaacgtcaggacactcatcctttaactgagctaagaaaagaggtagaagatgttcaatggtattttctttgcccaaaatagtagacaatcccataattacagaagctagagccgatttgacatgttgattggtatcggatactaattcctttatataaggcagaatttgattcataattatggtctctctatcttcaatgggcaagttctcaccaagttcttttactttgtgggcagcagctgcccggacttcagcttcacagtctttaagtaggttctgaaaggcggggatgaggtcatttagggtgattttaggacccatggctttctggagctctgaaaatctgtcagccaccatatagcgaacgcgccaagatttatcttctgctgcttgtcgaagtgtaggcatcaccaaagtctcaaggtcatcctgagacaataactgggcaatactgacacaagcttccacagcaaggaggcgcactgaatcctgttcatctgaagctagactagtgaacagtggaacaatttcacttttcacactgtctaattccaaaacttttgcaaattcacccaatttggaagcagcagcacgtcgtaccattggtgtgtcatctgagcacaaggaacggaattgctgtctgatttctgctttaacagcatttgatgccctgggatagcaaacgctgaacaaaccacatgcagatgtgcgagaggtgaaccaatccccacttgctaagcgtttcaccagaggtacaaaataagcttccagagcaacaggagtatgctcctgggagatctgtctcagggactccacagccttgtcacgaacaacagtctcttccacagttgccagattttccaaaggaggcagcagacagtgggcaaagtcaggacctcccactaggccagtgaaatttcccagctgctcagcaagagctaatagtacctcatcttcatcataaattgtatctgtaagaaatggcaacaattcacttcgggtcctttctactccaagtgctagggcaattgttgataacttcttaatactgttgagtcggagctgcacgtcttcattgcggagctcgtcgattaaaaccgcgatcgggtatagcgaatcatctccatctccacccgctgctcctgggccggtcccgagctctgatgcgcccgccatgttctttctcctcctgctgctggtcacc

SEQ ID NO: 11973 - RNA, 2954 nt, Homo sapiens
  source 1..2954: mol_type = other RNA
ctgaatagctgggactacaggtgtgtgccaccacgcccagctaacttttttgtatttttagtagagatggggtttcaccatgttggtcaggctgatctcgaattcttgacctcaaatgatcccaaataggtgctttttaaaaagggctttaatactgtttaagtagttcaaataggcttcctcactattaatttgcttcagtaaactcttcagcttaactcattatcttaaatttcagaattaatgaggttttactgtaaaagtagaaaagcaaacacttcaaatgataagactccagtatcacccatactaaaaacttagcaataaaactgcagtttgaaaagctactgtacaatgcagcaaggactaggtgtcaatactgctggaagcagagccaggtaaagaacaggaaatctgcacagtattatccctgtggttcttagactcattcgaaatacagaactgcaatctcacaatgaaacaaacatactgcttattaggaggcactacagttaaagctttttagaaaagagagagaagtatttttaaatgtaggcacagtggtgagctgttcaaattcagttaggcgtcaacatcacacattagcagcaagatgcagccacacttcaggtttctgaatgacatgagtacagacaaaattgagcaaataaaaaccaaaacaaccactacattaaccctgagcttccacattcccctttcacatgagactaatgcagaccatcataattcaggaaaatgtggctttcattacggtcaaatctcaacatgtctcccgaagagtttataaaataagttattctaaacatgtacatttagctttggaatgatggagagacacagagatatatgtaaacgtcaagagaatcactccactccacgtctgggtccacacccttccaggctttgtctggaacattatgtggctggtgcctgattccacagtgaggatgcaggagcccaggtggtgatggataaagcattaggagacaatcaagtgtcaggaattggtcaataagaacggcttaaataatgatttaacaaggaagacgagtaaaaaacaatcccatttcatctttagaaagaattaagtcactaaatgatttcttctaagttgttgccatttgcttggatgagatcttgaaggttttccattctttctccacccagttaagaacacattgactagaaatttgtgacaagaatctagtaaaggccttttccctcctgctcctcattatgccaatgcaagaacacttatagcttcctgtgcaaagtatttgacatccatgtcttcatcttgacctaacttctgtagtactggcttcacttctccctgtaaagcattggtatctagaattggtccaatcttttgtagagatttggccacattgaagcgaacatttgctacttggtctcctgccatttttaatacgatgggcagcatttgcttagtagttatttcctgaccacaggcctcagacagtgcattaatgcagaataaagtggtcattctatgcaagtaattaggatcatttgccattactaacactttgggaacaatagtattttgggcccactctgtaccaaacttctgaactagtttcatgaggttgttggtggcagcttctcggatggcgtatacatggtccacgagccaagccatacataaagaattcagcttttcatcaaagaattccacacccagctggcctgccagcagcggcatatactcaatgatggccaggcggaccctccatttggcatcttctgccagctccactatggcaggaaggagagactgagagagctgacggattccaatcacttcatttacacaatccaaattggagatgatattcaaacgaacgtcaggacactttatataaggcagaatttgattcataattatggtctctctatcttcaatgggcaagttctcaccaagttcttttactttgtgggcagcagctgcccggacttcagcttcacagtctttaagtaggttctgaaaggcggggatgaggtcatttagggtgattttaggacccatggctttctggagctctgaaaatctgtcagccaccatatagcgaacgcgccaagatttatcttctgctgcttgtcgaagtgtaggcatcaccaaagtctcaaggtcatcctgagacaataactgggcaatactgacacaagcttccacagcaaggaggcgcactgaatcctgttcatctgaagctagactagtgaacagtggaacaatttcacttttcacactgtctaattccaaaacttttgcaaattcacccaatttggaagcagcagcacgtcgtaccattggtgtgtcatctgagcacaaggaacggaattgctgtctgatttctgctttaacagcatttgatgccctgggatagcaaacgctgaacaaaccacatgcagatgtgcgagaggtgaaccaatccccacttgctaagcgtttcaccagaggtacaaaataagcttccagagcaacaggagtatgctcctgggagatctgtctcagggactccacagccttgtcacgaacaacagtctcttccacagttgccagattttccaaaggaggcagcagacagtgggcaaagtcaggacctcccactaggccagtgaaatttcccagctgctcagcaagagctaatagtacctcatcttcatcataaattgtatctgtaagaaatggcaacaattcacttcgggtcctttctactccaagtgctagggcaattgttgataacttcttaatactgttgagtcggagctgcacgtcttcattgcggagctcgtcgattaaaaccgcgatcgggtatagcgaatcatctccatctccacccgctgctcctgggccggtcccgagctctgatgcgcccgccatgttctttctcctcctgctgctggtcacc

SEQ ID NO: 11974 - RNA, 9629 nt, Homo sapiens
  source 1..9629: mol_type = other RNA
ctgaatagctgggactacaggtgtgtgccaccacgcccagctagtttttgtatttttagtagacatggggtttcaccatgttgcccaggctggtcttgaactcttgagctcaggcaatccacccacctctgcctcccgaaaacactgggattacaggcgtgcgccactgcgcctagccctgactgctttttctaacacaattccctgttcttatcagagaaacttatttgtatccttcatattttgaattctgcctagagtaagaggaagtctaaaaagtatccacaccctttatcaacactttcaaaaagtttgcctttaaaaagtaggagatagaaatggtaagttaaaaaatatattttccccagcactttgggaggccgagacgggcagatcacgaggtcaggagatcgagaccatcctggctaatacggtgaaaccctgtctctactaaaaatacaaaaaattagctgggcatggtggcgtgcgcctgtagtcccagctactcgggaggctgaggcaggagaatggcatgaacccaggaggtggagcttgcggtgagcagagatcgtgccactgcactacagcctgggcgacagagcaagactctgtctcaaaaaatatatatatatatatttatatttatttattaaaaatatatttataaaatataaaaaaatatatttttcaatttttttaatctggtatttaaaaaaatgaaaagaatctatgtgtccaacaacagcctaagcaaattatttactttacaactttgaagatattaaaatcatgctttaaaaagtatttattaaaaagttaatgatagaattatttttaagaaatagaccacagctctgttcactaaactagacatcttaaaaaaagacaaaagaaaaaaattatgacataaccattgataaaactttggtgttatgtctttccatattttcaatgcacacacacatatttataacatgcattaaaaagtcataccatattttgtgactgtttaaaattcataatgtatcaaatatatctccacatgtcaatccacacaaatacattttaatgactgcattatattccattttattgactgttactgggaatttaggaattttccagtttttcactagggcatgaaacaggtgaatattgttacttatacatgaaaaatccttttataaaatctcagtttaaaattgctgggttttaaatatttaaaggttataaatattccagctttggacatttattgctttactgtcccaagttttttttggtttgtttttgtttttagacagggtcttactctgtcacccaggctggagtgcagtggtgcacacagctcactgcagactcaaccccactgcagctcaagtgatcctcctaccccagcatccctagtggctgggaccacagattcatgacaccatgggtaattttttttttttggtagagatggggttttgccatgttgcctaggctggtttcaaactcctgggctcaagcaatctactcacctcagcctctcaaagtgctgggattacagatgtgagccaccacacccacccagtaagtttgtactaatttacgcttccattggtagtctaaagcaagtatacgacacacccaccaatacttggtcaactcatcccttttcatattataatacataatggaacagaatatgaacacttgctctacaaaaaataagtctgtgtagtgaatggggtggtggtgagtgggatgagggaagagaggagaaggactaggagagggacataatataaataacattaaactgctgttgtcctaacagtcttagtttctgcacacctgttatggtgcaacattttcctatacctagaagaaaaattaattccatgcatttttactataatggagtctcatgttactcaggctggtctcaaactcctgggctcaagcaatcctcccacgtcagcctccagagcagataggactacaggcacaggccattgcacccacctccttgcaacttttaccttacaatcacttaaatagcttttaagttaaacttccactagaatggtaagtaaaagaaaaggcacaaaatttgctgaagaaccgtaaatatttaactgaacacctacactgggccaagtaataaaacaatgaaaaatttagacaaagttcccaccttaccaaaacttacagtgtagagggcacaatacacaaacaggcaatacagtgtgaaagtgtgacaagtattgttaaagcagatgaaggacacaatacctaaaggataaataggacaggttaaattagggagacagtgaagataaagggaataaccagagataaggcctgaaaaggcaagagtttgagcaaggtcttgtaaaaagattttatcttaactggagaaaaaggccagaagaagattaaacgtgaaatgttatgtgatcaggttagtactttagatggatcaccctgggaagtgtagagaacagttgataggaaagcacaatatataaacaatattattgattgcagtattgttataaaaactctggaggcaaatggatcaaatacattatggtacaagcatataatcaaatactaagcagctattacaaatgaaatagaactacatgcactgacatggaaagatgtttaaaaagatgttggataggctgggggcgatggcctcacaatcccaacaatttgggaggctgaggcaggcggatcacctgaggttaggagtttgagaccagcctgaccaacatggagaaaccctgtctctactaaaaatacaaaattagccaggagtggtggcacatgcctgtaatcccagctacttgggaggctgaggcaggagaattgcttgaacccaggaggcagaggttgctgtgagccgagaacgtgccactgcactccagcctgggaaaaagcaaaactccttctcaaaaaaaaaaaaaaaaaaaaaaaaaagatgtgggataaaaggtataactcaatttttataaaatgtttgtatgtacataaagtctgacagaatgcacattcacctacgatattaattttttaaggcagtagaatccagggtttccttctgtgtagggcagaagttatttacattgttttctcctatgcatgtattagttttattattaaaaaccacaaagtttttgttttgttttgttttgttttttaataggataccatggcagctgcatagaaaacatactaaaggaaagtatgattcaagtcagagaaaccagttaggaggctattgcaataaaatccaggtgagatgctgggcgagactgtgcctgagtctacctcctggtgtacaggatgagtattccttattcaaaacacttgggaccagaactgttttggattttggaatatttgcattatacctactagttgagcatcacaaatctgaaaatccaaaattttaaatgctccaatgagcatttcttttgaaagtcacatcggcgcacaaggtttcaggttttggagcattctgaatttcagattttcagatttgagatgctcaatctgttccaagatcactgggccaaaattagagtgtaaattccagtcctaaccaagcaaagtacaatcccttgctgagtactccttaagatgatctcacccaaggaccacatgcagttgggacgattttcttgagacggagtcttgctctgtcacctaggccggaatgcagtggtgcgatctcggcttaccacaacctctgcctcccgggttcacagcattctcctgcctcagcctcccgagtagctggtactacaggcgcccaccaccacacttggctaattttttgtatttttagtagagacgaggtttcatcatgttagccaggatggtctcaatctcctgacctcgtgatccgcctgcctcggcctcccaaagtgctgggattagaagcgtgagccactgcacccggccagttgggaccattttctaactactgatggctagtgctatacccaccagggctgctaacacctgaaaccacttggtttcacagcatgactgcaggctctcctttccaagctacaaatgaatcccagtagacctaaatacccatcatcttcttacagactgctgggatttaacctatactccctctaaattttgttttcactggtcatagcccctgatctggtcttttttcctctatcaataatgtcattacaatcttctgtattcctcaggccaaagccagaaaccctaaacccctgcccttctggagactctttcatggtgccctctgagattcccttaataaactcccttaatatcctcaactatttccctgaacatttcctttcattaatttaaacttggctgttccctgggaaggaaaaaacacctacctgacaacaatcacatcacaagggggcttattctcatgtattccacatatccacaggttggaagtgggatcagtatcttccttactccctaacactgcttctaaccattgcagcctggagaaaaccactccttcctttgaagttcataccatctagttataccactttctccctctcttccttgctatcttttatttaaatgacctctcctcaatcacatagactttgctacttgctttgctgtcttctccactgatggctctattgataacttggaaggactttcaaatacatagagatcttcttcactaaaacctccttgcagaatttcatccaccttcctcttagcagataatcttaccatgaaacctataatcatatatctatattttactggccaggaacagtagaaatggcatcaaggctacaaagaggttgggataagtagttttgtagctaaatacaatactactgttagcaaaactgaagatctattcataaagaataaaaaatatatatatttggttagtaattagcagtggctgccacacagttcttaggaaacacaaaacattatatagttcacatattctgatcactgcttagtacagttaggtgtaaataaataaacaagtaatttaaaccaacccacccatttttctactcctgaaagaatggtgggagtatccctccgcctcatggcaaacaccaatacttttgtttgtgctctaaacatctacaccccattctcagaagcttatattaaactttattatgctgcatattaaacctcaccatactacattcatcacattagaattcaaacatgttctagtttttcatattttaaacatattatctctttactccaaatctctccagctactaccctttctcctattattcaaacttgtctacatccagtctttacttctttgccctttattgattcctaaagtcagcccaatctagcaaccatcttcattatgtaccactatgttatttccaactacaatcacaaatgatcttcacttggctgtatatgtttacctttttagacttcatctaattggatccctaagtaacactaaaaacatttaccttcaccttcctttttttttttttttttttgagatgaagtcctgctctgtcaccaggctggagtgcagtggtgagatctcatctcactgcaacctctgcctcccaggttcaagtgattcttctgcctcagctcctgagtagctgggactacaggcatgtgccaccacacccggctaatttttgtattttagtagaaccagggtttcaccatgttggccaggatggtctcgatctgaccttgtgatccgcctgcctcagcctctcaaagtgccaggattacaggcgtgaaccaccacacctggccaacttcaccttcctttttgaaacttgtttgtcttggttcagtgaaactccactcttcttgttttcctcttatctctctactatagttcctttaaatgtatgtcttcagggtaggtggcagaccttcccttttcattcttactcaccttccaaagcctgttattgtctctttactgatgtcactacaatttatatctctatctagacacctcctcaattctagaattgcgtaccaacctcttcatctggatgtctcaccatcctctgaggctaacatgaataactacaacagcagctactgccttctttcttccaccgtatgccactccttccatattttgttagaactaatctggtcagtatctgcaagatcaagcagcaaaatctcatgctttacttagcatttaaaattggtaacttcccctctgtctgaaaactttctgtagttccaatgctgaaatgttgggatactctttttgctgttctaaacacttgctttcagtgatcttggttctatcttcatctgctgcttaagcataaaagctcggtcaacattccttttccatactttttttctatgttcctcttcaaatgtgtacatccaacataaaacatttaactgtatatacttctgtttttctacaatatggtgactgcgttgactgtatttatgtagtgctttaaaaaaaatcagtaagagccaggcatggtaactcatgcctggaatcctagcactttgggaggcaaaggcaggaggactgcttgagcccaggagtttcagaccagtctgagcaatgtaggaagagcctgtctctacaaaatatatatttttaaaattagccaggcatggtggcatgcatttgtgatcccaactactgaggagactgtggtggatcacctgagcccaggaggtcgaggttgcaatgagccatgaccacaccactgcattctagcctgagagacagagactctgtctgaaaaattgaaaaaaaaaaagaaaaaatcaattaacatatttttcttggccgggcacagtggctcacgcctgtaatgccaacactttgggacgcctaggtgggtggatcacctgaggtcaggagtttgagaccaacctggccaacatggtgaaaccccgtctctattaaaaatactaaaattagccaggcatggcggtggtgcctgtaatcccagctactcaggaggctgaggcaggagaatcacctgaacctgggaggtggaggttgcagtgagctgagattgtgccactgcactccagcctgggcaacataccgagactccatctcaaaaaacaaacaaaaaaccttatttttctcatgtaggaacatatccagatacaagtagtgcagggctggtacaactatttaaagatttctttgaggaacagggatctctttcttctacttcatcccttggctacagctgtcattttcatgatcacaagatagctctttcagcagcttcaggaatggccaattcatagggacaaagatgaagtgcaaaaagtagaggacaagatagatagttctgatcccagtgatatgtctatttttgaatcagcaagaatgaatgatatggctacccttagctacaagaagtcaaagaagcgttctataaccagagaccttattgttcttggctaagatggaattcattagtaaggaaagatgagctcaaatgtttggttggctgctagcaataccagtctcactgggccagaaaacaacttttataaaaacaccaacaaagcagtaaaatatagtccagattctctgaacacaatggaattaacctagaaaccaacaataaaaagataactgaaaatatacctacctcacatattaaaaatacctaattctaaacagccatggatcaaaaaaagtcataattagtatttacagaaaatgttatattaaaaaaagagccatttgtaaccttaaatcgttcttttagagaacaaagactgagacaaggagcttggaatccaccttaagacaatgaaaacagcaattccacattcataacacttacagggtttctctctcagtatgaattctcttgtgtataataagtgaagagctctgactgaaggcttttccacattgaatacattcatagggtttctctccagtgtgaattctcacatgcctcctaagggaagaggaaacactgaaggctttcctacattccttacattcatagggtttctctccagtgtgagttcttatatgcattctaagggatgagaccccactgaaaactttcccacagtcactgcattcataaacattctctccggtatgaattttcttatgaactttaaggtgagagctcgtgttgaaggcttttccacactcactgcattcatagagtttttctccagtgtgtattctcttgtgcactataaggtaagagcttgtgccaaaggattttccacactgattacattcataaggtttctctccagtgtgagttctcatgtgagccttaagggatgttttttgactgaaagcttttccacattgattacattcatagggtttctctccagtgtgagttcttacatgtctccttaaggttgaggaatcattgaacactttaccacattctttacattcatattgtttctcacccatgtgacttttcttgtataaagtaagattagaaatccttttgaaggcttttccacattgattgcattcatgtttcttttcagtatgagtttgtccttgtttcttaagggatgattgatgacacagcgtttcatctttattacattcacaggcattctgtgccatatgcaaattgttaggtacaggaaacatattatgtgtgaagtgcattccatgtttagaatatgtgtactctttttgtactgtttgatttctctgaaaatgccatagagttgtatcacattcatgactttcatagagcttctcacttatagagtttttcacataattgtttatgattgaattgtgtttcaaacatccaatctctgagtaacatttttggcaatgtttactggtgaaaatgctctgtgaaaaaataagttttgatccaagtttagagttttcctctaattcatgatagtcacggaatagctcctgaggtactgttttctttggggcatatatcatttgcctccaatgtccccctggaatcttatgctgttttctgatcttatggcattcccagtcttctcttaatgtggaggaccaattatgcattgtgagttttatcattttcactgcattggatggttcctcccacaaaattttctgcacagttgattctttggttttaggttgaatcttctggtctggacagatggcttggggaattctctttttcatattccttatctcttcttgatccaatggggagatcacagtaagcctgtacaactgatattccacggaggtgagatttctatagttttccaacatcacatctctgtacagacttctttgagcagaatccagcatcatccactcctcctgagtgaactccacagctacatctttgaaagtcattggttcctgtaaccaggttgtcagaaatacagcaatcatcctttcctcttcagcatttctcagatggaaacaggcagagtcctgtttagttaaagcccatggggaggataggtccataactgccattttatgagtacataagcctgcacagtagagtagagagatcaggatgtttctgttcttgtgtctccaatccagtcacaggagggatgcatttcacccgaagttctccccgtcctcagtgcctgcctccaggcgtccgcggtcccgcccgaggggg

SEQ ID NO: 11975 - RNA, 4533 nt, Homo sapiens
  source 1..4533: mol_type = other RNA
ctgaatagctgggactacaggtgtgtgccaccacgcctggattttgtatttttagtagagatggggtttcgccaggctggcctctaactcctgacctcaggtgatccaccctccttggcctcccaaagtgctgggattacaggcgtgaaccaccgcgcccagcccagcccctctttttctgtatcttcccactggctctgtcattaattcagtgaaattatgtcaagcacctactagatgtcccacgccctgacatatcatgaggcatcatcccaaggtgaacaagacaagtatagcctttaccctcacagttcactgagagatagctgctaagtacgtcaatcattaaacagggaaaaaacatccaggctgccggatgaagaaacatgacgtgtgctttgagggagtagtgcaggctggtggaagtgtgaaagatgtgaggacccaaccaagtgtgacgtgagctgggatctgctggtcaaggaaggaggggtggcgagatggaaggttcaggcagagggagctgtctgggtgaatgcaggaagacaggaaggagcctggcctgggagaaaggctggtgtcaccagagcttcaacagggaggcatcacggctctagaagaggctggggaaggccacgagggtctcattttgcagggtgctggaaggcatgccaaggaatttggtctttggccaagaacaaggcgtgtgccacagtcacgtagtgacacaggtcacatttgctttctgccagcagaagagactggactccagtgcaggggagtgtgcaaggacaggttctggggggtggaggcatctgtggacatcccagggcaggggtgagggccagaacatccctaggtcctgagactacagtttctccacatttagatcagacattctcttccaaggaaggaaaccaagagaggctggtgaaccgtctggtaatgacaagccctcacttttgcagccctcttggctggtccctcagcaggtcttccctatgagcctgcaaaggagacaggcaggaatgagttccatgttcgagatagggaaactgagggccagggagaggcagtgactcgcccgagggcacacggcagaatgcaggcagaggcagagtggccctgggcatcctgagtccagttctgggcactctgcacctcacaggcctggactcagtccttgccaccaccactctcagagtccttctcatggaggggcttcaggcagccgggatccccagcctcttgcccagatgccagctgctcagagtcttctgcagggattccattcgggacacctctgccagcctccatcttctccttcaggttccgtttgaagaaaccaaccttgtacagcactatgaaaatgagcagcagcagcagcagccccccgatgccgctcagcacgtagaggtagagcatctgcttctcatacaccacgtcaaccttcatgacaacctgggccagggaggcgttgctgccatagaggtggaaatgcttgctgctgttgaaggagatggagagggagctgcagaggctgaacatggaagaggcctcgatctctcccaccagctccagagtcccgatcacttggacgaggatctcctgcctgaagacaacagggcagcggaacagggctccggggagacaaggctcagctgcatccgggagcctctccagatcctcatagtggcagggcacgggaggctccatctgcacgctccactggtgtgtgatgggcccctcgctgggaggctgtggcaccccaaccacagcctccagggtgggtatgttgtggtcgtggatggaaggctggatcctcacctggtacatgtgcttgacttggtggatcttggggcctttgggggtgaaactgacatagagtgtggagtcttcttggtcctggatgaggatgttgatggggtacaggatggggatgatggtagtggctgagttgtcctccaggaggtctgagtcctcattgttacaggtcacattggcgtgcaattcaaccgagtccccccaggagctgtttaccagtgtattaaacatcatctgcagagcaaccgagtggcctgctttgaagatgggagagctcacattgcaagataatgccctggacagaagcctggactcttcaggaagctcctcgcagctcacaggtatctggctatggggcttcagcatctccaccttgcggaaggagagtcccggggggaagtgcaggtccagctggacccagtaagcatcttcttccaagttactcaggctcagctccacagagaggctggcaaaagcagttagacgcagggctctggatcttgcaggagagaaggacactctcaagtttgcctcacacttcttgtcctccccacagttcttctcaaaagggatctcccaggtttccgagtgcagggagggtctcaggatgggcggtatgtccttgcccgccctttggtccctcggtgtcccttcctcctcccaaagagagaaattcagggaaacattgatgggggagatgaggtcttgaacacataccgggaaatgaaatgagaagtcagtgcatgacatgctggtggtgacagctatattccttctgagttcatgtctccctcctgggaacaacccccgtcttctggtccggtggccatccagctgcagagtgtaagtgagattggcaaccaggcggccttggaactgggggatgagagacttgatctggaaacagattgtgatattaactccttctttcatcttgttactggttgaataggagcactccacttcatgcactgggatctcagctggagagaaggacatcagggtgaccatatccaccacgggccgggagctcagcacgatcatctggctctcagcccccacagccacatctgccaagccatccccttcaaggtccttcaccccatggatggagcgtccaaaccactgaattcctgagagcacttgggtcccttctatccgctgacttggctggggactaagccccccgtgcctcccattgaagatgtacacagccccctgctcctccagaggggcccccacagccacgtctaccagcccatcgccgttgatgtctgtcagagcagtgatggcttctccaaaccgcccgagtgggtagccggggtccccctgcagctctgagacttcttcaaaccccaactgtcttctctggtagataaacacccggcctcctctctgctccccatagaacagtggggcaccaatcagcagcagctctgtctccccatcttggtccacgtcgacgccacacagctccccaccgaaataagagccaatctgggtcccatggattgtctggacctggctccagtgtcctccgccctgtggctcttggaacagcagcactcggcccatgtgctggtatcgaggggctcccgaggccagcaacgaagtcttttgccgggagggcagccaggtcacggtgtaacccaaatagcctgctctcacttctggtgtcaatggttcattcccaataaatgtgtcatcctgcaggtctgccttcaggtcaagaaagcccccagcccagtccttggctcctactgcccccacgactgcatggcccctgctgaggtcagcactgatgccgctggaggacagctccatgttgaaggaagtcaggtcctgtttgcttgtgccctcaatgacatagatcttcttctgcagctcagtgaatagatctttcagcttctcaaatgtgtccagaattttcacaaactcgctcgcgggttttgatgcaaatttgtggagggtctcctgactctccttggtctgaaaatgctttccaatcccgatgatgtagcggatgatgtctttggccgcatcgatgttgccactgtcagtggcctccccatccgtgatgatgataagcactttggtggcatctggccgggcccccagctcctcccggaacacctctgtcgcgacataattgatggcaccaaaggtattggtcaacagcaacatgtgctttacatgcttcagcagagcatcagggtccttccgtttaacataatctgagaaatcaaattctgttttgtagcttgtggaaaactgaacagcagcaaacaaaatgcttccatctgtggggtctgttgccaaggtcattcccaagtacttggaggtatagttggaacctctcagggtgactggcaggcagtgtcctgtgcccgactggcactgatagaggcttcctgtgctgttcccctcccctggagctcccacgatgaccccgtttccgacctgcaggacgcggtatccaaagtgcctcccggcgcgcggtggggagaagctccgcgcgccccgcacgtccaggttgtagctcgaggccggcgcgaagaaaaagaacccagacagcagcgccatggccatcacagtgatgcaggaatccttcatccttccagcactcgagggacctgtggccccaggggcagcgtcaggaggcccgtgggatttgctggcaacctagacagggtgaaagaggaaaatgat

SEQ ID NO: 11976 - RNA, 4782 nt, Homo sapiens
  source 1..4782: mol_type = other RNA
ctgaatagctgggactacaggtgtgtgccaccacgcctggattttgtatttttagtagagatggggtttcgccaggctggcctctaactcctgacctcaggtgatccaccctccttggcctcccaaagtgctgggattacaggcgtgaaccaccgcgcccagcccagcccctctttttctgtatcttcccactggctctgtcattaattcagtgaaattatgtcaagcacctactagatgtcccacgccctgacatatcatgaggcatcatcccaaggtgaacaagacaagtatagcctttaccctcacagttcactgagagatagctgctaagtacgtcaatcattaaacagggaaaaaacatccaggctgccggatgaagaaacatgacgtgtgctttgagggagtagtgcaggctggtggaagtgtgaaagatgtgaggacccaaccaagtgtgacgtgagctgggatctgctggtcaaggaaggaggggtggcgagatggaaggttcaggcagagggagctgtctgggtgaatgcaggaagacaggaaggagcctggcctgggagaaaggctggtgtcaccagagcttcaacagggaggcatcacggctctagaagaggctggggaaggccacgagggtctcattttgcagggtgctggaaggcatgccaaggaatttggtctttggccaagaacaaggcgtgtgccacagtcacgtagtgacacaggtcacatttgctttctgccagcagaagagactggactccagtgcaggggagtgtgcaaggacaggttctggggggtggaggcatctgtggacatcccagggcaggggtgagggccagaacatccctaggtcctgagactacagtttctccacatttagatcagacattctcttccaaggaaggaaaccaagagaggctggtgaaccgtctggtaatgacaagccctcacttttgcagccctcttggctggtccctcagcaggtcttccctatgagcctgcaaaggagacaggcaggaatgagttccatgttcgagatagggaaactgagggccagggagaggcagtgactcgcccgagggcacacggcagaatgcaggcagaggcagagtggccctgggcatcctgagtccagttctgggcactctgcacctcacaggcctggactcagtccttgccaccaccactctcagagtccttctcatggaggggcttcaggcagccgggatccccagcctcttgcccagatgccagctgctcagagtcttctgcagggattccattcgggacacctctgccagcctccatcttctccttcaggttccgtttgaagaaaccaaccttgtacagcactatgaaaatgagcagcagcagcagcagccccccgatgccgctcagcacgtagaggtagagcatctgcttctcatacaccacgtcaaccttcatgacaacctgggccagggaggcgttgctgccatagaggtggaaatgcttgctgctgttgaaggagatggagagggagctgcagaggctgaacatggaagaggcctcgatctctcccaccagctccagagtcccgatcacttggacgaggatctcctgcctgaagacaacagggcagcggaacagggctccggggagacaaggctcagctgcatccgggagcctctccagatcctcatagtggcagggcacgggaggctccatctgcacgctccactggtgtgtgatgggcccctcgctgggaggctgtggcaccccaaccacagcctccagggtgggtatgttgtggtcgtggatggaaggctggatcctcacctggtacatgtgcttgacttggtggatcttggggcctttgggggtgaaactgacatagagtgtggagtcttcttggtcctggatgaggatgttgatggggtacaggatggggatgatggtagtggctgagttgtcctccaggaggtctgagtcctcattgttacaggtcacattggcgtgcaattcaaccgagtccccccaggagctgtttaccagtgtattaaacatcatctgcagagcaaccgagtggcctgctttgaagatgggagagctcacattgcaagataatgccctggacagaagcctggactcttcaggaagctcctcgcagctcacaggtatctggctatggggcttcagcatctccaccttgcggaaggagagtcccggggggaagtgcaggtccagctggacccagtaagcatcttcttccaagttactcaggctcagctccacagagaggctggcaaaagcagttagacgcagggctctggatcttgcaggagagaaggacactctcaagtttgcctcacacttcttgtcctccccacagttcttctcaaaagggatctcccaggtttccgagtgcagggagggtctcaggatgggcggtatgtccttgcccgccctttggtccctcggtgtcccttcctcctcccaaagagagaaattcagggaaacattgatgggggagatgaggtcttgaacacataccgggaaatgaaatgagaagtcagtgcatgacatgctggtggtgacagctatattccttctgagttcatgtctccctcctgggaacaacccccgtcttctggtccggtggccatccagctgcagagtgtaagtgagattggcaaccaggcggccttggaactgggggatgagagacttgatctggaaacagattgtgatattaactccttctttcatcttgttactggttgaataggagcactccacttcatgcactgggatctcagctggagagaaggacatcagggtgaccatatccaccacgggccgggagctcagcacgatcatctggctctcagcccccacagccacatctgccaagccatccccttcaaggtccttcaccccatggatggagcgtccaaaccactgaattcctgagagcacttgggtcccttctatccgctgacttggctggggactaagccccccgtgcctcccattgaagatgtacacagccccctgctcctccagaggggcccccacagccacgtctaccagcccatcgccgttgatgtctgtcagagcagtgatggcttctccaaaccgcccgagtgggtagccggggtccccctgcagctctgagacttcttcaaaccccaactgtcttctctggtagataaacacccggcctcctctctgctccccatagaacagtggggcaccaatcagcagcagctctgtctccccatcttggtccacgtcgacgccacacagctccccaccgaaataagagccaatctgggtcccatggattgtctggacctggctccagtgtcctccgccctgtggctcttggaacagcagcactcggcccatgtgctggtatcgaggggctcccgaggccagcaacgaagtcttttgccgggagggcagccaggtcacggtgtaacccaaatagcctgctctcacttctggtgtcaatggttcattcccaataaatgtgtcatcctgcaggtctgccttcaggtcaagaaagcccccagcccagtccttggctcctactgcccccacgactgcatggcccctgctgaggtcagcactgatgccgctggaggacagctccatgttgaaggaagtcaggtcctgtttgcttgtgccctcaatgacatagatcttcttctgcagctcagtgaatagatctttcagcttctcaaatgtgtccagaattttcacaaactcgctcgcgggttttgatgcaaatttgtggagggtctcctgactctccttggtctgaaaatgctttccaatcccgatgatgtagcggatgatgtctttggccgcatcgatgttgccactgtcagtggcctccccatccgtgatgatgataagcactttggtggcatctggccgggcccccagctcctcccggaacacctctgtcgcgacataattgatggcaccaaaggtattggtcaacagcaacatgtgctttacatgcttcagcagagcatcagggtccttccgtttaacataatctgagaaatcaaattctgttttgtagcttgtggaaaactgaacagcagcaaactggtacgaagtgttgctgagtttcttcatcacatccttcatgaagtccagaattttctgaaattcatctggctgcaagctcatcgaaccatcaaacagaaataccaggtctacgttgcccttgatacattcctgaaaaccagggcgcccctgcagcatgggaccctgcagattctggcggaagaggtaacacaggccactcagataggtgttctggtcacacgttcgagacagcccagggtcacaggccaaaatgcttccatctgtggggtctgttgccaaggtcattcccaagtacttggaggtatagttggaacctctcagggtgactggcaggcagtgtcctgtgcccgactggcactgatagaggcttcctgtgctgttcccctcccctggagctcccacgatgaccccgtttccgacctgcaggacgcggtatccaaagtgcctcccggcgcgcggtggggagaagctccgcgcgccccgcacgtccaggttgtagctcgaggccggcgcgaagaaaaagaacccagacagcagcgccatggccatcacagtgatgcaggaatccttcatccttccagcactcgagggacctgtggccccaggggcagcgtcaggaggcccgtgggatttgctggcaacctagacagggtgaaagaggaaaatgat

SEQ ID NO: 11977 - RNA, 4567 nt, Homo sapiens
  source 1..4567: mol_type = other RNA
ctgaatagctgggactacaggtgtgtgccaccacgcctggattttgtatttttagtagagatggggtttcgccaggctggcctctaactcctgacctcaggtgatccaccctccttggcctcccaaagtgctgggattacaggcgtgaaccaccgcgcccagcccagcccctctttttctgtatcttcccactggctctgtcattaattcagtgaaattatgtcaagcacctactagatgtcccacgccctgacatatcatgaggcatcatcccaaggtgaacaagacaagtatagcctttaccctcacagttcactgagagatagctgctaagtacgtcaatcattaaacagggaaaaaacatccaggctgccggatgaagaaacatgacgtgtgctttgagggagtagtgcaggctggtggaagtgtgaaagatgtgaggacccaaccaagtgtgacgtgagctgggatctgctggtcaaggaaggaggggtggcgagatggaaggttcaggcagagggagctgtctgggtgaatgcaggaagacaggaaggagcctggcctgggagaaaggctggtgtcaccagagcttcaacagggaggcatcacggctctagaagaggctggggaaggccacgagggtctcattttgcagggtgctggaaggcatgccaaggaatttggtctttggccaagaacaaggcgtgtgccacagtcacgtagtgacacaggtcacatttgctttctgccagcagaagagactggactccagtgcaggggagtgtgcaaggacaggttctggggggtggaggcatctgtggacatcccagggcaggggtgagggccagaacatccctaggtcctgagactacagtttctccacatttagatcagacattctcttccaaggaaggaaaccaagagaggctggtgaaccgtctggtaatgacaagccctcacttttgcagccctcttggctggtccctcagcaggtcttccctatgagcctgcaaaggagacaggcaggaatgagttccatgttcgagatagggaaactgagggccagggagaggcagtgactcgcccgagggcacacggcagaatgcaggcagaggcagagtggccctgggcatcctgagtccagttctgggcactctgcacctcacaggcctggactcagtccttgccaccaccactctcagagtccttctcatggaggggcttcaggcagccgggatccccagcctcttgcccagatgccagctgctcagagtcttctgcagggattccattcgggacacctctgccagcctccatcttctccttcaggttccgtttgaagaaaccaaccttgtacagcactatgaaaatgagcagcagcagcagcagccccccgatgccgctcagcacgtagaggtagagcatctgcttctcatacaccacgtcaaccttcatgacaacctgggccagggaggcgttgctgccatagaggtggaaatgcttgctgctgttgaaggagatggagagggagctgcagaggctgaacatggaagaggcctcgatctctcccaccagctccagagtcccgatcacttggacgaggatctcctgcctgaagacaacagggcagcggaacagggctccggggagacaaggctcagctgcatccgggagcctctccagatcctcatagtggcagggcacgggaggctccatctgcacgctccactggtgtgtgatgggcccctcgctgggaggctgtggcaccccaaccacagcctccagggtgggtatgttgtggtcgtggatggaaggctggatcctcacctggtacatgtgcttgacttggtggatcttggggcctttgggggtgaaactgacatagagtgtggagtcttcttggtcctggatgaggatgttgatggggtacaggatggggatgatggtagtggctgagttgtcctccaggaggtctgagtcctcattgttacaggtcacattggcgtgcaattcaaccgagtccccccaggagctgtttaccagtgtattaaacatcatctgcagagcaaccgagtggcctgctttgaagatgggagagctcacattgcaagataatgccctggacagaagcctggactcttcaggaagctcctcgcagctcacaggtatctggctatggggcttcagcatctccaccttgcggaaggagagtcccggggggaagtgcaggtccagctggacccagtaagcatcttcttccaagttactcaggctcagctccacagagaggctggcaaaagcagttagacgcagggctctggatcttgcaggagagaaggacactctcaagtttgcctcacacttcttgtcctccccacagttcttctcaaaagggatctcccaggtttccgagtgcagggagggtctcaggatgggcggtatgtccttgccctgcgccctttggtccctcggtgtcccttcctcctcccaaagagagaaattcagggaaacattgatgggggagatgaggtcttgaacacataccgggaaatgaaatgagaagtcagtgcatgacatgctggtggtgacagctatattccttctgagttcatgtctccctcctgggaacaacccccgtcttctggtccggtggccatccagctgcagagtgtaagtgagattggcaaccaggcggccttggaactgggggatgagagacttgatctggaaacagattgtgatattaactccttctttcatcttgttactggttgaataggagcactccacttcatgcactgggatctcagctggagagaaggacatcagggtgaccatatccaccacgggccgggagctcagcacgatcatctggctctcagcccccacagccacatctgccaagccatccccttcaaggtccttcaccccatggatggagcgtccaaaccactgaattcctgagagcacttgggtcccttctatccgctgacttggctggggactaagccccccgtgcctcccattgaagatgtacacagccccctgctcctccagaggggcccccacagccacgtctaccagcccatcgccgttgatgtctgtcagagcagtgatggcttctccaaaccgcccgagtgggtagccggggtccccctgcagctctgagacttcttcaaaccccaactgtcttctctggtagataaacacccggcctcctctctgctccccatagaacagtggggcaccaatcagcagcagctctgtctccccatcttggtccacgtcgacgccacacagctccccaccgaaataagagccaatctgggtcccatggattgtctggacctggctccagtgtcctccgccctgtggctcttggaacagcagcactcggcccatgtgctggtatcgaggggctcccgaggccagcaacgaagtcttttgccgggagggcagccaggtcacggtgtaacccaaatagcctgctctcacttctggtgtcaatggttcattcccaataaatgtgtcatcctgcaggtctgccttcaggtcaagaaagcccccagcccagtccttggctcctactgcccccacgactgcatggcccctgctgaggtcagcactgatgccgctggaggacagctccatgttgaaggaagtcaggtcctgtttgcttgtgccctcaatgacatagatcttcttctgcagctcagtgaatagatctttcagcttctcaaatgtgtccagaattttcacaaactcgctcgcgggttttgatgcaaatttgtggagggtctcctgactctccttggtctgaaaatgctttccaatcccgatgatgtagcggatgatgtctttggccgcatcgatgttgccactgtcagtggcctccccatccgtgatgatgataagcactttggtggcatctggccgggcccccagctcctcccggaacacctctgtcgcgacataattgatggcaccaaaggtattggtcaacagcaacatgtgctttacatgcttcagcagagcatcagggtccttccgtttaacataatctgagaaatcaaattctgttttgtagcttgtggaaaactgaacagcagcaaacaaaatgcttccatctgtggggtctgttgccaaggtcattcccaagtacttggaggtatagttggaacctctcagggtgactggcaggcagtgtcctgtgcccgactggcactgatagaggcttcctgtgctgttcccctcccctggagctcccacgatgaccccgtttccgacctgcaggacgcggtatccaaagtgcctcccggcgcgcggtggggagaagctccgcgcgccccgcacgtccaggttgtagctcgaggccggcgcgaagaaaaagaacccagacagcagcgccatggccatcacagtgatgcaggaatccttcatccttccagcactcgagggacctgtggccccaggggcagcgtcaggaggcccgtgggatttgctggcaacctagacagggtgaaagaggaaaatgatcatgccctttggcctcttacagtggtacttt

SEQ ID NO: 11978 - RNA, 4785 nt, Homo sapiens
  source 1..4785: mol_type = other RNA
ctgaatagctgggactacaggtgtgtgccaccacgcctggattttgtatttttagtagagatggggtttcgccaggctggcctctaactcctgacctcaggtgatccaccctccttggcctcccaaagtgctgggattacaggcgtgaaccaccgcgcccagcccagcccctctttttctgtatcttcccactggctctgtcattaattcagtgaaattatgtcaagcacctactagatgtcccacgccctgacatatcatgaggcatcatcccaaggtgaacaagacaagtatagcctttaccctcacagttcactgagagatagctgctaagtacgtcaatcattaaacagggaaaaaacatccaggctgccggatgaagaaacatgacgtgtgctttgagggagtagtgcaggctggtggaagtgtgaaagatgtgaggacccaaccaagtgtgacgtgagctgggatctgctggtcaaggaaggaggggtggcgagatggaaggttcaggcagagggagctgtctgggtgaatgcaggaagacaggaaggagcctggcctgggagaaaggctggtgtcaccagagcttcaacagggaggcatcacggctctagaagaggctggggaaggccacgagggtctcattttgcagggtgctggaaggcatgccaaggaatttggtctttggccaagaacaaggcgtgtgccacagtcacgtagtgacacaggtcacatttgctttctgccagcagaagagactggactccagtgcaggggagtgtgcaaggacaggttctggggggtggaggcatctgtggacatcccagggcaggggtgagggccagaacatccctaggtcctgagactacagtttctccacatttagatcagacattctcttccaaggaaggaaaccaagagaggctggtgaaccgtctggtaatgacaagccctcacttttgcagccctcttggctggtccctcagcaggtcttccctatgagcctgcaaaggagacaggcaggaatgagttccatgttcgagatagggaaactgagggccagggagaggcagtgactcgcccgagggcacacggcagaatgcaggcagaggcagagtggccctgggcatcctgagtccagttctgggcactctgcacctcacaggcctggactcagtccttgccaccaccactctcagagtccttctcatggaggggcttcaggcagccgggatccccagcctcttgcccagatgccagctgctcagagtcttctgcagggattccattcgggacacctctgccagcctccatcttctccttcaggttccgtttgaagaaaccaaccttgtacagcactatgaaaatgagcagcagcagcagcagccccccgatgccgctcagcacgtagaggtagagcatctgcttctcatacaccacgtcaaccttcatgacaacctgggccagggaggcgttgctgccatagaggtggaaatgcttgctgctgttgaaggagatggagagggagctgcagaggctgaacatggaagaggcctcgatctctcccaccagctccagagtcccgatcacttggacgaggatctcctgcctgaagacaacagggcagcggaacagggctccggggagacaaggctcagctgcatccgggagcctctccagatcctcatagtggcagggcacgggaggctccatctgcacgctccactggtgtgtgatgggcccctcgctgggaggctgtggcaccccaaccacagcctccagggtgggtatgttgtggtcgtggatggaaggctggatcctcacctggtacatgtgcttgacttggtggatcttggggcctttgggggtgaaactgacatagagtgtggagtcttcttggtcctggatgaggatgttgatggggtacaggatggggatgatggtagtggctgagttgtcctccaggaggtctgagtcctcattgttacaggtcacattggcgtgcaattcaaccgagtccccccaggagctgtttaccagtgtattaaacatcatctgcagagcaaccgagtggcctgctttgaagatgggagagctcacattgcaagataatgccctggacagaagcctggactcttcaggaagctcctcgcagctcacaggtatctggctatggggcttcagcatctccaccttgcggaaggagagtcccggggggaagtgcaggtccagctggacccagtaagcatcttcttccaagttactcaggctcagctccacagagaggctggcaaaagcagttagacgcagggctctggatcttgcaggagagaaggacactctcaagtttgcctcacacttcttgtcctccccacagttcttctcaaaagggatctcccaggtttccgagtgcagggagggtctcaggatgggcggtatgtccttgccctgcgccctttggtccctcggtgtcccttcctcctcccaaagagagaaattcagggaaacattgatgggggagatgaggtcttgaacacataccgggaaatgaaatgagaagtcagtgcatgacatgctggtggtgacagctatattccttctgagttcatgtctccctcctgggaacaacccccgtcttctggtccggtggccatccagctgcagagtgtaagtgagattggcaaccaggcggccttggaactgggggatgagagacttgatctggaaacagattgtgatattaactccttctttcatcttgttactggttgaataggagcactccacttcatgcactgggatctcagctggagagaaggacatcagggtgaccatatccaccacgggccgggagctcagcacgatcatctggctctcagcccccacagccacatctgccaagccatccccttcaaggtccttcaccccatggatggagcgtccaaaccactgaattcctgagagcacttgggtcccttctatccgctgacttggctggggactaagccccccgtgcctcccattgaagatgtacacagccccctgctcctccagaggggcccccacagccacgtctaccagcccatcgccgttgatgtctgtcagagcagtgatggcttctccaaaccgcccgagtgggtagccggggtccccctgcagctctgagacttcttcaaaccccaactgtcttctctggtagataaacacccggcctcctctctgctccccatagaacagtggggcaccaatcagcagcagctctgtctccccatcttggtccacgtcgacgccacacagctccccaccgaaataagagccaatctgggtcccatggattgtctggacctggctccagtgtcctccgccctgtggctcttggaacagcagcactcggcccatgtgctggtatcgaggggctcccgaggccagcaacgaagtcttttgccgggagggcagccaggtcacggtgtaacccaaatagcctgctctcacttctggtgtcaatggttcattcccaataaatgtgtcatcctgcaggtctgccttcaggtcaagaaagcccccagcccagtccttggctcctactgcccccacgactgcatggcccctgctgaggtcagcactgatgccgctggaggacagctccatgttgaaggaagtcaggtcctgtttgcttgtgccctcaatgacatagatcttcttctgcagctcagtgaatagatctttcagcttctcaaatgtgtccagaattttcacaaactcgctcgcgggttttgatgcaaatttgtggagggtctcctgactctccttggtctgaaaatgctttccaatcccgatgatgtagcggatgatgtctttggccgcatcgatgttgccactgtcagtggcctccccatccgtgatgatgataagcactttggtggcatctggccgggcccccagctcctcccggaacacctctgtcgcgacataattgatggcaccaaaggtattggtcaacagcaacatgtgctttacatgcttcagcagagcatcagggtccttccgtttaacataatctgagaaatcaaattctgttttgtagcttgtggaaaactgaacagcagcaaactggtacgaagtgttgctgagtttcttcatcacatccttcatgaagtccagaattttctgaaattcatctggctgcaagctcatcgaaccatcaaacagaaataccaggtctacgttgcccttgatacattcctgaaaaccagggcgcccctgcagcatgggaccctgcagattctggcggaagaggtaacacaggccactcagataggtgttctggtcacacgttcgagacagcccagggtcacaggccaaaatgcttccatctgtggggtctgttgccaaggtcattcccaagtacttggaggtatagttggaacctctcagggtgactggcaggcagtgtcctgtgcccgactggcactgatagaggcttcctgtgctgttcccctcccctggagctcccacgatgaccccgtttccgacctgcaggacgcggtatccaaagtgcctcccggcgcgcggtggggagaagctccgcgcgccccgcacgtccaggttgtagctcgaggccggcgcgaagaaaaagaacccagacagcagcgccatggccatcacagtgatgcaggaatccttcatccttccagcactcgagggacctgtggccccaggggcagcgtcaggaggcccgtgggatttgctggcaacctagacagggtgaaagaggaaaatgat

SEQ ID NO: 11979 - RNA, 5075 nt, Homo sapiens
  source 1..5075: mol_type = other RNA
ctgaatagctgggactacaggtgtgtgccaccacgcctggattttgtatttttagtagagatggggtttcgccaggctggcctctaactcctgacctcaggtgatccaccctccttggcctcccaaagtgctgggattacaggcgtgaaccaccgcgcccagcccagcccctctttttctgtatcttcccactggctctgtcattaattcagtgaaattatgtcaagcacctactagatgtcccacgccctgacatatcatgaggcatcatcccaaggtgaacaagacaagtatagcctttaccctcacagttcactgagagatagctgctaagtacgtcaatcattaaacagggaaaaaacatccaggctgccggatgaagaaacatgacgtgtgctttgagggagtagtgcaggctggtggaagtgtgaaagatgtgaggacccaaccaagtgtgacgtgagctgggatctgctggtcaaggaaggaggggtggcgagatggaaggttcaggcagagggagctgtctgggtgaatgcaggaagacaggaaggagcctggcctgggagaaaggctggtgtcaccagagcttcaacagggaggcatcacggctctagaagaggctggggaaggccacgagggtctcattttgcagggtgctggaaggcatgccaaggaatttggtctttggccaagaacaaggcgtgtgccacagtcacgtagtgacacaggtcacatttgctttctgccagcagaagagactggactccagtgcaggggagtgtgcaaggacaggttctggggggtggaggcatctgtggacatcccagggcaggggtgagggccagaacatccctaggtcctgagactacagtttctccacatttagatcagacattctcttccaaggaaggaaaccaagagaggctggtgaaccgtctggtaatgacaagccctcacttttgcagccctcttggctggtccctcagcaggtcttccctatgagcctgcaaaggagacaggcaggaatgagttccatgttcgagatagggaaactgagggccagggagaggcagtgactcgcccgagggcacacggcagaatgcaggcagaggcagagtggccctgggcatcctgagtccagttctgggcactctgcacctcacaggcctggactcagtccttgccaccaccactctcagagtccttctcatggaggggcttcaggcagccgggatccccagcctcttgcccagatgccagctgctcagagtcttctgcagggattccattcgggacacctctgccagcctccatcttctccttcaggttccgtttgaagaaaccaaccttgtacagcactatgaaaatgagcagcagcagcagcagccccccgatgccgctcagcacgtagaggtagagcatctgcttctcatacaccacgtcaaccttcatgacaacctgggccagggaggcgttgctgccatagaggtggaaatgcttgctgctgttgaaggagatggagagggagctgcagaggctgaacatggaagaggcctcgatctctcccaccagctccagagtcccgatcacttggacgaggatctcctgcctgaagacaacagggcagcggaacagggctccggggagacaaggctcagctgcatccgggagcctctccagatcctcatagtggcagggcacgggaggctccatctgcacgctccactggtgtgtgatgggcccctcgctgggaggctgtggcaccccaaccacagcctccagggtgggtatgttgtggtcgtggatggaaggctggatcctcacctggtacatgtgcttgacttggtggatcttggggcctttgggggtgaaactgacatagagtgtggagtcttcttggtcctggatgaggatgttgatggggtacaggatggggatgatggtagtggctgagttgtcctccaggaggtctgagtcctcattgttacaggtcacattggcgtgcaattcaaccgagtccccccaggagctgtttaccagtgtattaaacatcatctgcagagcaaccgagtggcctgctttgaagatgggagagctcacattgcaagataatgccctggacagaagcctggactcttcaggaagctcctcgcagctcacaggtatctggctatggggcttcagcatctccaccttgcggaaggagagtcccggggggaagtgcaggtccagctggacccagtaagcatcttcttccaagttactcaggctcagctccacagagaggctggcaaaagcagttagacgcagggctctggatcttgcaggagagaaggacactctcaagtttgcctcacacttcttgtcctccccacagttcttctcaaaagggatctcccaggtttccgagtgcagggagggtctcaggatgggcggtatgtccttgccctgcgccctttggtccctcggtgtcccttcctcctcccaaagagagaaattcagggaaacattgatgggggagatgaggtcttgaacacataccgggaaatgaaatgagaagtcagtgcatgacatgctggtggtgacagctatattccttctgagttcatgtctccctcctgggaacaacccccgtcttctggtccggtggccatccagctgcagagtgtaagtgagattggcaaccaggcggccttggaactgggggatgagagacttgatctggaaacagattgtgatattaactccttctttcatcttgttactggttgaataggagcactccacttcatgcactgggatctcagctggagagaaggacatcagggtgaccatatccaccacgggccgggagctcagcacgatcatctggctctcagcccccacagccacatctgccaagccatccccttcaaggtccttcaccccatggatggagcgtccaaaccactgaattcctgagagcacttgggtcccttctatccgctgacttggctggggactaagccccccgtgcctcccattgaagatgtacacagccccctgctcctccagaggggcccccacagccacgtctaccagcccatcgccgttgatgtctgtcagagcagtgatggcttctccaaaccgcccgagtgggtagccggggtccccctgcagctctgagacttcttcaaaccccaactgtcttctctggtagataaacacccggcctcctctctgctccccatagaacagtggggcaccaatcagcagcagctctgtctccccatcttggtccacgtcgacgccacacagctccccaccgaaataagagccaatctgggtcccatggattgtctggacctggctccagtgtcctccgccctgtggctcttggaacagcagcactcggcccatgtgctggtatcgaggggctcccgaggccagcaacgaagtcttttgccgggagggcagccaggtcacggtgtaacccaaatagcctgctctcacttctggtgtcaatggttcattcccaataaatgtgtcatcctgcaggtctgccttcaggtcaagaaagcccccagcccagtccttggctcctactgcccccacgactgcatggcccctgctgaggtcagcactgatgccgctggaggacagctccatgttgaaggaagtcaggtcctgtttgcttgtgccctcaatgacatagatcttcttctgcagctcagtgaatagatctttcagcttctcaaatgtgtccagaattttcacaaactcgctcgcgggttttgatgcaaatttgtggagggtctcctgactctccttggtctgaaaatgctttccaatcccgatgatgtagcggatgatgtctttggccgcatcgatgttgccactgtcagtggcctccccatccgtgatgatgataagcactttggtggcatctggccgggcccccagctcctcccggaacacctctgtcgcgacataattgatggcaccaaaggtattggtcaacagcaacatgtgctttacatgcttcagcagagcatcagggtccttccgtttaacataatctgagaaatcaaattctgttttgtagcttgtggaaaactgaacagcagcaaactggtacgaagtgttgctgagtttcttcatcacatccttcatgaagtccagaattttctgaaattcatctggctgcaagctcatcgaaccatcaaacagaaataccaggtctacgttgcccttgatacattcctgaaaaccagggcgcccctgcagcatgggaccctgcagattctggcggaagaggtaacacaggccactcagataggtgttctggtcacacgttcgagacagcccagggtcacaggccaaaatgcttccatctgtggggtctgttgccaaggtcattcccaagtacttggaggtatagttggaacctctcagggtgactggcaggcagtgtcctgtgcccgactggcactgatagaggcttcctgtgctgttcccctcccctggagctcccacgatgaccccgtttccgacctgcaggacgcggtatccaaagtgcctcccggcgcgcggtggggagaagctccgcgcgccccgcacgtccaggttgtagctcgaggccggcgctgaggaaggcaagggtcgtcagctgcgaccgagggacccccgcccctgcacgtgcccagcaggtggccgatcccaggcccacccggatgtcgctccccaggccacccgcaccctgcgcttcccctccagggcgttgacttctgggaatatggaaggagcaactcccggcccccctagagctctgaaagctcttcccagggcctgaggatacaacttcccgtttggcctctcgaagaaaaagaacccagacagcagcgccatggccatcacagtgatgcaggaatccttcatccttccagcactcgagggacctgtggccccaggggcagcgtcaggaggcccgtgggatttgctggcaacctagacagggtgaaagaggaaaatgatcatgccctttggcctcttacagtggtactttctcacagaggcaacaggctggtgacact

SEQ ID NO: 11980 - RNA, 4798 nt, Homo sapiens
  source 1..4798: mol_type = other RNA
ctgaatagctgggactacaggtgtgtgccaccacgcctggattttgtatttttagtagagatggggtttcgccaggctggcctctaactcctgacctcaggtgatccaccctccttggcctcccaaagtgctgggattacaggcgtgaaccaccgcgcccagcccagcccctctttttctgtatcttcccactggctctgtcattaattcagtgaaattatgtcaagcacctactagatgtcccacgccctgacatatcatgaggcatcatcccaaggtgaacaagacaagtatagcctttaccctcacagttcactgagagatagctgctaagtacgtcaatcattaaacagggaaaaaacatccaggctgccggatgaagaaacatgacgtgtgctttgagggagtagtgcaggctggtggaagtgtgaaagatgtgaggacccaaccaagtgtgacgtgagctgggatctgctggtcaaggaaggaggggtggcgagatggaaggttcaggcagagggagctgtctgggtgaatgcaggaagacaggaaggagcctggcctgggagaaaggctggtgtcaccagagcttcaacagggaggcatcacggctctagaagaggctggggaaggccacgagggtctcattttgcagggtgctggaaggcatgccaaggaatttggtctttggccaagaacaaggcgtgtgccacagtcacgtagtgacacaggtcacatttgctttctgccagcagaagagactggactccagtgcaggggagtgtgcaaggacaggttctggggggtggaggcatctgtggacatcccagggcaggggtgagggccagaacatccctaggtcctgagactacagtttctccacatttagatcagacattctcttccaaggaaggaaaccaagagaggctggtgaaccgtctggtaatgacaagccctcacttttgcagccctcttggctggtccctcagcaggtcttccctatgagcctgcaaaggagacaggcaggaatgagttccatgttcgagatagggaaactgagggccagggagaggcagtgactcgcccgagggcacacggcagaatgcaggcagaggcagagtggccctgggcatcctgagtccagttctgggcactctgcacctcacaggcctggactcagtccttgccaccaccactctcagagtccttctcatggaggggcttcaggcagccgggatccccagcctcttgcccagatgccagctgctcagagtcttctgcagggattccattcgggacacctctgccagcctccatcttctccttcaggttccgtttgaagaaaccaaccttgtacagcactatgaaaatgagcagcagcagcagcagccccccgatgccgctcagcacgtagaggtagagcatctgcttctcatacaccacgtcaaccttcatgacaacctgggccagggaggcgttgctgccatagaggtggaaatgcttgctgctgttgaaggagatggagagggagctgcagaggctgaacatggaagaggcctcgatctctcccaccagctccagagtcccgatcacttggacgaggatctcctgcctgaagacaacagggcagcggaacagggctccggggagacaaggctcagctgcatccgggagcctctccagatcctcatagtggcagggcacgggaggctccatctgcacgctccactggtgtgtgatgggcccctcgctgggaggctgtggcaccccaaccacagcctccagggtgggtatgttgtggtcgtggatggaaggctggatcctcacctggtacatgtgcttgacttggtggatcttggggcctttgggggtgaaactgacatagagtgtggagtcttcttggtcctggatgaggatgttgatggggtacaggatggggatgatggtagtggctgagttgtcctccaggaggtctgagtcctcattgttacaggtcacattggcgtgcaattcaaccgagtccccccaggagctgtttaccagtgtattaaacatcatctgcagagcaaccgagtggcctgctttgaagatgggagagctcacattgcaagataatgccctggacagaagcctggactcttcaggaagctcctcgcagctcacaggtatctggctatggggcttcagcatctccaccttgcggaaggagagtcccggggggaagtgcaggtccagctggacccagtaagcatcttcttccaagttactcaggctcagctccacagagaggctggcaaaagcagttagacgcagggctctggatcttgcaggagagaaggacactctcaagtttgcctcacacttcttgtcctccccacagttcttctcaaaagggatctcccaggtttccgagtgcagggagggtctcaggatgggcggtatgtccttgccctgcgccctttggtccctcggtgtcccttcctcctcccaaagagagaaattcagggaaacattgatgggggagatgaggtcttgaacacataccgggaaatgaaatgagaagtcagtgcatgacatgctggtggtgacagctatattccttctgagttcatgtctccctcctgggaacaacccccgtcttctggtccggtggccatccagctgcagagtgtaagtgagattggcaaccaggcggccttggaactgggggatgagagacttgatctggaaacagattgtgatattaactccttctttcatcttgttactggttgaataggagcactccacttcatgcactgggatctcagctggagagaaggacatcagggtgaccatatccaccacgggccgggagctcagcacgatcatctggctctcagcccccacagccacatctgccaagccatccccttcaaggtccttcaccccatggatggagcgtccaaaccactgaattcctgagagcacttgggtcccttctatccgctgacttggctggggactaagccccccgtgcctcccattgaagatgtacacagccccctgctcctccagaggggcccccacagccacgtctaccagcccatcgccgttgatgtctgtcagagcagtgatggcttctccaaaccgcccgagtgggtagccggggtccccctgcagctctgagacttcttcaaaccccaactgtcttctctggtagataaacacccggcctcctctctgctccccatagaacagtggggcaccaatcagcagcagctctgtctccccatcttggtccacgtcgacgccacacagctccccaccgaaataagagccaatctgggtcccatggattgtctggacctggctccagtgtcctccgccctgtggctcttggaacagcagcactcggcccatgtgctggtatcgaggggctcccgaggccagcaacgaagtcttttgccgggagggcagccaggtcacggtgtaacccaaatagcctgctctcacttctggtgtcaatggttcattcccaataaatgtgtcatcctgcaggtctgccttcaggtcaagaaagcccccagcccagtccttggctcctactgcccccacgactgcatggcccctgctgaggtcagcactgatgccgctggaggacagctccatgttgaaggaagtcaggtcctgtttgcttgtgccctcaatgacatagatcttcttctgcagctcagtgaatagatctttcagcttctcaaatgtgtccagaattttcacaaactcgctcgcgggttttgatgcaaatttgtggagggtctcctgactctccttggtctgaaaatgctttccaatcccgatgatgtagcggatgatgtctttggccgcatcgatgttgccactgtcagtggcctccccatccgtgatgatgataagcactttggtggcatctggccgggcccccagctcctcccggaacacctctgtcgcgacataattgatggcaccaaaggtattggtcaacagcaacatgtgctttacatgcttcagcagagcatcagggtccttccgtttaacataatctgagaaatcaaattctgttttgtagcttgtggaaaactgaacagcagcaaactggtacgaagtgttgctgagtttcttcatcacatccttcatgaagtccagaattttctgaaattcatctggctgcaagctcatcgaaccatcaaacagaaataccaggtctacgttgcccttgatacattcctgaaaaccagggcgcccctgcagcatgggaccctgcagattctggcggaagaggtaacacaggccactcagataggtgttctggtcacacgttcgagacagcccagggtcacaggccaaaatgcttccatctgtggggtctgttgccaaggtcattcccaagtacttggaggtatagttggaacctctcagggtgactggcaggcagtgtcctgtgcccgactggcactgatagaggcttcctgtgctgttcccctcccctggagctcccacgatgaccctggtgagaaatctcacccgtttccgacctgcaggacgcggtatccaaagtgcctcccggcgcgcggtggggagaagctccgcgcgccccgcacgtccaggttgtagctcgaggccggcgcgaagaaaaagaacccagacagcagcgccatggccatcacagtgatgcaggaatccttcatccttccagcactcgagggacctgtggccccaggggcagcgtcaggaggcccgtgggatttgctggcaacctagacagggtgaaagaggaaaa

SEQ ID NO: 11981 - RNA, 1397 nt, Homo sapiens
  source 1..1397: mol_type = other RNA
ctgaatagctgggactacaggtgtgtgccaccacgcctggctaatttgtgtcttttttagtagacatgggatttcaccatgttggccaggctggtcttgaactcctgacctcaagtgatctccccacctcggcctctcaaagtgctgggattacaggcatgagccactgcgcccggccacggaagtcagtcttcttagaaggaatcacggcactagagaaaatgatgatgggagcgacaccgtatagaaagacactttattacactgcccactcacaccaggccgggacaggagtcactccttagaaccccgagcggctgtccaggctgatggaggaggggaccactcacccgccacagagccagccccctcacatggcttcctccctgaggagcatctcccacactggggcttccaacgatctttgctctgcgtgtgctgaaaggacagcgtccagaatcagcctcagcctggacttctgttaccatgggaggataagcttgtcatgctcacagatgtgcactcctagtgccacgcctctaaacgtcccccagacggcattggggctctcgccggggagcttggctactgtctcgatccccggccaagcaggcctcatggccaactttctcagtgtccacagcagacaaaaatgtccacagccagagctccaaagctctgccggccctggtgccactgccacctctgcgtccggagcctgtggggctcagctctgctgctctggcccaagtctggcctggagtccctggtgccctttgcaagcacggaggcggctggacatccttcgcatcaccagcctctgggcctgcaagcgcttccggagcttttcattttccttcagagtgaggaagagttttttcttcagggaatctaagtccaaaagggcatagctgtgatcagatggctgcttgttgggggtccttctcaggcctgcagggccagtcggccggccaacagcctctgttgcttgcggcctccgtggcgagacctgttttacgtggccttcggcatttgggggcaactgaagctcttcaagtgcagtgtccatgtttctcccaggactgtcctctccggcccccgcctcagggaggaccttttctttctgagaagagctggcatttcctctctcactggcagggtctgtgttctccctcacctgcccgagcacctgggctgtgccaggcagcgtcctgggtgtggggcctgaagcagggaaggcagcccctgccctcatggagattctgtgtggggtcctgaaaggcgaacaccgtgggcacggcattgtgctttaggttcttgcggtttccaaaggcgctgaagcactctggccggaagtgctcggagcagatgaccgtgtgctgcttgggcttgaagtt

SEQ ID NO: 11982 - RNA, 1824 nt, Homo sapiens
  source 1..1824: mol_type = other RNA
ctgaatagctgggactacaggtgtgtgccaccacgcctggctaatttgtgtcttttttagtagacatgggatttcaccatgttggccaggctggtcttgaactcctgacctcaagtgatctccccacctcggcctctcaaagtgctgggattacaggcatgagccactgcgcccggccacggaagtcagtcttcttagaaggaatcacggcactagagaaaatgatgatgggagcgacaccgtatagaaagacactttattacactgcccactcacaccaggccgggacaggagtcactccttagaaccccgagcggctgtccaggctgatggaggaggggaccactcacccgccacagagccagccccctcacatggcttcctccctgaggagcatctcccacactggggcttccaacgatctttgctctgcgtgtgctgaaaggacagcgtccagaatcagcctcagcctggacttctgttaccatgggaggataagcttgtcatgctcacagatgtgcactcctagtgccacgcctctaaacgtcccccagacggcattggggctctcgccggggagcttggctactgtctcgatccccggccaagcaggcctcatggccaactttctcagtgtccacagcagacaaaaatgtccacagccagagctccaaagctctgccggccctggtgccactgccacctctgcgtccggagcctgtggggctcagctctgctgctctggcccaagtctggcctggagtccctggtgccctttgcaagcacggaggcggctggacatccttcgcatcaccagcctctgggcctgcaagcgcttccggagcttttcattttccttcagagtgaggaagagttttttcttcagggaatctaagtccaaaagggcatagctgtgatcagatggctgcttgttgggggtccttctcaggcctgcagggccagtcggccggccaacagcctctgttgcttgcggcctccgtggcgagacctgttttacgtggccttcggcatttgggggcaactgaagctcttcaagtgcagtgtccatgtttctcccaggactgtcctctccggcccccgcctcagggaggaccttttctttctgagaagagctggcatttcctctctcactggcagggtctgtgttctccctcacctgtgtggggtcctgaaaggcgaacaccgtgggcacggcattgtgctttaggttcttgcggtttccaaaggcgctgaagcactctggccggaagtgctcggagcagatgaccgtgtgctgcttgggcttgaagttgccccggccgatgttcagcacccattccttcagcagctccgggcggctgaacggaaaccggtggaaggtgagctgcttcctgcggctgctgtagcggttgcagcactgccgggccgcgcacgacttcggcatctcgagccaggcctggctgcccccaacaaagatggcggcggcggcggggcctgcggagaggggagggaccccattcgccaatgctggtcgcctttcacctccttgctttgagcacccaaccaggacgcatagccactcacaggcttggacaactggaaaccaacggccaacccctcagtgtttttagggctttgaattgtgaataggtctggactcctctgacgtcactggaggtggtactagttggccactggtggtgtcagttcagaggccagacagctcactgcccttaagtttggtcacagggaacccccaaacgtgaagaggcaaaaagggcaactgaaggggagggagattccagttcaggccttgcagaaact

SEQ ID NO: 11983 - RNA, 4357 nt, Homo sapiens
  source 1..4357: mol_type = other RNA
ctgaatagctgggactacaggtgtgtgccaccatccccagctacttttataataaaatttctatgtagagacggagtcttcctacgttgcccaggctggtcttgaactcctgggctcaagcagtcttcctgcctcggcctcccaaagtgctggaattacaggcatgagccaccacactcagccttaaatgaagattttgtaaggaattgagcattcaactaaactcgtttttgtgagatggtcattttgttttaacctaacatggtttagagattattttatgaactctaagcattctggttcctcagttttctcaaagaaagagaactttagcaagtagcaggacaagctaccccacaccaatgccaccaggcgacaatactatgaataagtcaggaggcctcctagaatgcagccaaataggaaactgttccaaacagaatcagtcttgcatacttctgctcagaaggctcctctcgctttggaaactggaatgaggatcaccaacaggatcctcattttacacaggagttatgagagttacatcctctagcagagatgcttggtcattacctgtggtacatgagattaccgagctaaaagggaaaaaaaacgatcttaatgttctcccatgaactcaacttaagctttttatggaggcactgaggccatgcagctccttttccaaaagacacagataaaagccaaataaggtagaggactttggaaattttctctgaaaagttaaattccacataatagtaagactgtttgctgagagaaaactgacaagtaaaaactggtttaagagacagacattcaagacaaactgtattggaaatacaataatgaattttggcctgatagccctcatgctgtcttatagcaaaacactaaaattcatgcaacagagaaattggtgacatgaggactttttctccagacttcctggggaaaaactgtgagaatatacttttttcttctgtttgctttcgaaatgcattctttcttttgctgactttcccaaactttcccagtcgtttctgatgaaaaattcttcaataggaaaagaccaggtaaacttacatgaaagacatcaagtatcttttgagctccttctctctgccagaggagcaatcaactggattacacaaaactaccttcacaactaaaacaggtagaattggaacaggaattagttgtcattaatatactcgtaataaaataaagcttgttctgaaaccacaaggggtggtaagaagagactgtataaaagctactgggttctctagaaaatggatacagtatacagaatgtgagaagatacagaactcacactccagttataaaaatagacatggttctcagacaaaaagcaaatgagtacaaaagaattctccaaacgtgaactatttttaaaagatacatctatataaaacaacaagatgtcatctcagagctccaaagagtagtttgttgaaatggctgaaaaggggagatgaattggagacagataggtcaagaacccagaacagatgtgtcctactcttgtgtttggcagtgtacattggaggtcacaggcagatagactgcttttggtaatacatatataaataataatggctgactggttgatggtgcttgatggatgaatgagaaaacccaggttatcaaataatctcggtagttgaactgttagcttcttcacttgacaatgttgcacatcagaaatgattctaggttttttttacccagaatgatccctgccattcacaactcatgctccacgccccatggtttctattgtgccctaaaagatcagcctagactaatacataaatagaaaataactctggccttgaaatgaggggcagacaagtacttcatgctcagtacttataaatcacaaagaaatgctgaaattaatggtctgtctccttttactacaaaggagatgccatgagttaaagtcatgaaacaaagaaagtcaaaaagatatgggtagcagcacctttccatacccgcctggattttcaaggagcttttcactccttatgcctttcaaacaaaagttcatcagtttgaagaaaaagaaatggctctaaagttaaagagtccccagagaaaactaacagtacatgaaataggccctatgtgggcaaaaggacaagctgcagaaccagttaagacagaagaggcagcccaaggtcttactaaattacagttttagcatagtgtagcacaacatgggcagccctttttccatccaagcaacaattcagcaccatccacgtctggttcaaaagattactgaagtctgggctttcatctttggtaccacctcatgagttattcttggtttgcagtaggttcaaagaaacagaaaagctggtacctttgccttgtctgtgagtacaaacgctgggactctgattgctgcaaccattgaggccaattaaaataatactgtaacacacaggaatgatgcatccaattcctaatttccagataatagcagccatgcccctacagaggcgggatcatccatccccatcgtttaaggccttcggtttgttgtcctcagagtagaatagaacactgtgttcccacggacaaggaactccagatgaacccatggtctacatttggacagaattttaagtaccagatatgccaggcacagaaagaggactgacctgtggccatcatgcttggagaagcttctgttttggcacacaaactagaaacttcttagtgtattctggttttagttccctttcctgagtgaagcagccagggagtgaccaggttccataagccctcaatctgatacttggcattaattctctccatggtcttcttccacccaagctacaattttcccttcccatccagggatggcatcatcatcatggaaaatctcctctttgacagtgccaaactcaggatccagtgctttgaagtgataccggtgatttccttcccgatcaatagctgctttaaaatcctttaacgtcacctcctccaacctctttggtatattgaccatgaagggcgtaagtgaccggtcagtgaaatagagcactttagtacaggtgctgctgacagttggagagctctgtgagtgaggcaactttgagttagggggccaggactcccggtattcactacctacttgagttctgggtgacttgacccgaacctttctttcttgtttcttctgcgtctccataacatgcaggcgctccatgaggctagaaatgccctgctccaagctgtcaatagtgtggtgctgaggatcgtggccactgaagctgttgcgcaggctgcggagagcatctcgaacaagctgcaggtcgctggtccctctgttgctgactgaagtagctccttttcctgccgttggaaggagaaaaccattgctttgagagttgtgactgttgtagttggtcgcctcatctgcctctcttttcatacagtgagccaagaggacatctttgtgttctagctctcgctctagatccacctggtggtaactgacatcagagagtttccggagtgcttcttctaacttggcctggtgctgctgaagaaggcgatccttctgccccagctcttttttatattctcccaagagccggttcctctcatctagcttcctctgcagatccacattctggttgtgcagctcatctttgtccatatttgccctcagtagctcttgtttgagctgaagaacagatgtgtcctgctgagtcaatctctgctgcaaggcatcctttatcccctgtaagtttctggcttcttgtttacatttcagcagttccttctttaagtcctgattctcctccatactctgatccagacgactttggattataatcagttgttcctcgggattgacacctggttcacagagggccaagggcctctcctgttcatcttcaggtaaggatccattgagcagtaaggccctgggactagttcctttcgttaggtccatgctctggctctttcagctctctggacacctgactgctctgcttcaaggtgccttggccccagaagaaaatctgtagtcctgatatcattttctttgcttcctccatttctttttctaaatattcttgttgttccaacagctgttcttcccatgaggtctccagataggttccagggctccctggccgccagtctcgagataatggagaatctgtcccttctgttctgttctctattccttcagcgggaataatcacaaaatctgccttctcttctgactgggttataatggactcgctctttgcactgtggattggactgggtgaagtcaggcatttgacttgcgtccctccca

SEQ ID NO: 11984 - RNA, 4685 nt, Homo sapiens
  source 1..4685: mol_type = other RNA
ctgaatagctgggactacaggtgtgtgccaccatccccagctacttttataataaaatttctatgtagagacggagtcttcctacgttgcccaggctggtcttgaactcctgggctcaagcagtcttcctgcctcggcctcccaaagtgctggaattacaggcatgagccaccacactcagccttaaatgaagattttgtaaggaattgagcattcaactaaactcgtttttgtgagatggtcattttgttttaacctaacatggtttagagattattttatgaactctaagcattctggttcctcagttttctcaaagaaagagaactttagcaagtagcaggacaagctaccccacaccaatgccaccaggcgacaatactatgaataagtcaggaggcctcctagaatgcagccaaataggaaactgttccaaacagaatcagtcttgcatacttctgctcagaaggctcctctcgctttggaaactggaatgaggatcaccaacaggatcctcattttacacaggagttatgagagttacatcctctagcagagatgcttggtcattacctgtggtacatgagattaccgagctaaaagggaaaaaaaacgatcttaatgttctcccatgaactcaacttaagctttttatggaggcactgaggccatgcagctccttttccaaaagacacagataaaagccaaataaggtagaggactttggaaattttctctgaaaagttaaattccacataatagtaagactgtttgctgagagaaaactgacaagtaaaaactggtttaagagacagacattcaagacaaactgtattggaaatacaataatgaattttggcctgatagccctcatgctgtcttatagcaaaacactaaaattcatgcaacagagaaattggtgacatgaggactttttctccagacttcctggggaaaaactgtgagaatatacttttttcttctgtttgctttcgaaatgcattctttcttttgctgactttcccaaactttcccagtcgtttctgatgaaaaattcttcaataggaaaagaccaggtaaacttacatgaaagacatcaagtatcttttgagctccttctctctgccagaggagcaatcaactggattacacaaaactaccttcacaactaaaacaggtagaattggaacaggaattagttgtcattaatatactcgtaataaaataaagcttgttctgaaaccacaaggggtggtaagaagagactgtataaaagctactgggttctctagaaaatggatacagtatacagaatgtgagaagatacagaactcacactccagttataaaaatagacatggttctcagacaaaaagcaaatgagtacaaaagaattctccaaacgtgaactatttttaaaagatacatctatataaaacaacaagatgtcatctcagagctccaaagagtagtttgttgaaatggctgaaaaggggagatgaattggagacagataggtcaagaacccagaacagatgtgtcctactcttgtgtttggcagtgtacattggaggtcacaggcagatagactgcttttggtaatacatatataaataataatggctgactggttgatggtgcttgatggatgaatgagaaaacccaggttatcaaataatctcggtagttgaactgttagcttcttcacttgacaatgttgcacatcagaaatgattctaggttttttttacccagaatgatccctgccattcacaactcatgctccacgccccatggtttctattgtgccctaaaagatcagcctagactaatacataaatagaaaataactctggccttgaaatgaggggcagacaagtacttcatgctcagtacttataaatcacaaagaaatgctgaaattaatggtctgtctccttttactacaaaggagatgccatgagttaaagtcatgaaacaaagaaagtcaaaaagatatgggtagcagcacctttccatacccgcctggattttcaaggagcttttcactccttatgcctttcaaacaaaagttcatcagtttgaagaaaaagaaatggctctaaagttaaagagtccccagagaaaactaacagtacatgaaataggccctatgtgggcaaaaggacaagctgcagaaccagttaagacagaagaggcagcccaaggtcttactaaattacagttttagcatagtgtagcacaacatgggcagccctttttccatccaagcaacaattcagcaccatccacgtctggttcaaaagattactgaagtctgggctttcatctttggtaccacctcatgagttattcttggtttgcagtaggttcaaagaaacagaaaagctggtacctttgccttgtctgtgagtacaaacgctgggactctgattgctgcaaccattgaggccaattaaaataatactgtaacacacaggaatgatgcatccaattcctaatttccagataatagcagccatgcccctacagaggcgggatcatccatccccatcgtttaaggccttcggtttgttgtcctcagagtagaatagaacactgtgttcccacggacaaggaactccagatgaacccatggtctacatttggacagaattttaagtaccagatatgccaggcacagaaagaggactgacctgtggccatcatgcttggagaagcttctgttttggcacacaaactagaaacttcttagtgtattctggttttagttccctttcctgagtgaagcagccagggagtgaccaggttccataagccctcaatctgatacttggcattaattctctccatggtcttcttccacccaagctacaattttcccttcccatccagggatggcatcatcatcatggaaaatctcctctttgacagtgccaaactcaggatccagtgctttgaagtgataccggtgatttccttcccgatcaatagctgctttaaaatcctttaacgtcacctcctccaacctctttggtatattgaccatgaagggcgtaagtgaccggtcagtgaaatagagcactttagtacaggtgctgctgacagttggagagctctgtgagtgaggcaactttgagttagggggccaggactcccggtattcactacctacttgagttctgggtgacttgacccgaacctttctttcttgtttcttctgcgtctccataacatgcaggcgctccatgaggctagaaatgccctgctccaagctgtcaatagtgtggtgctgaggatcgtggccactgaagctgttgcgcaggctgcggagagcatctcgaacaagctgcaggtcgctggtccctctgttgctgactgaagtagctccttttcctgccgttggaaggagaaaaccattgctttgagagttgtgactgttgtagttggtcgcctcatctgcctctcttttcatacagtgagccaagaggacatctttgtgttctagctctcgctctagatccacctggtggtaactgacatcagagagtttccggagtgcttcttctaacttggcctggtgctgctgaagaaggcgatccttctgccccagctcttttttatattctcccaagagccggttcctctcatctagcttcctctgcagatccacattctggttgtgcagctcatctttgtccatatttgccctcagtagctcttgtttgagctgaagaacagatgtgtcctgctgagtcaatctctgctgcaaggcatcctttatcccctgtaagtttctggcttcttgtttacatttcagcagttccttctttaagtcctgattctcctccatactctgatccagacgactttggattataatcagttgttcctcgggattgacacctggttcacagagggccaagggcctctcctgttcatcttcaggtaaggatccattgagcagtaaggcctgtagtcctgatatcattttctttgcttcctccatttctttttctaaatattcttgttgttccaacagctgttcttcccatgaggtctccagataggttccagggctccctggccgccagtctcgagataatggagaatctgtcccttctgttctgttctctattccttcagcgggaataatcacaaaatctgccttctcttctgactgggttataatggactcgctctttgcactgtggattggactgggtgaagtcaggcatttgacttgcgtccctcccatggtccccctcctgtctcgggcttcagcaagcctgcgtccccgggtgaagtgggaggctgagagtcacatcgctcccaaattcaggcatgtctccccgcgctggggctggaaaacgcctccacgggaaggccagctagcaaagctactggcccggctcgcgggagaaagcgggaacggcggcggcggcggcgtctcggccccagcgactgggatgctccaggctctgaagcgcgcagtcccggccgctcagactgtgcagcagcccggccccggcggaagctgcctcccctcgcaggctgccggcccctggccgctgcatcttggcctccgcggacgcacggtgccgggcatcccccctggcgggggcatctcaacccatctcccactgggagggaggctcccggcggcgcaggctgcgcctcgagtc

SEQ ID NO: 11985 - RNA, 5035 nt, Homo sapiens
  source 1..5035: mol_type = other RNA
ctgaatagctgggactacaggtgtgtgccaccatccccagctacttttataataaaatttctatgtagagacggagtcttcctacgttgcccaggctggtcttgaactcctgggctcaagcagtcttcctgcctcggcctcccaaagtgctggaattacaggcatgagccaccacactcagccttaaatgaagattttgtaaggaattgagcattcaactaaactcgtttttgtgagatggtcattttgttttaacctaacatggtttagagattattttatgaactctaagcattctggttcctcagttttctcaaagaaagagaactttagcaagtagcaggacaagctaccccacaccaatgccaccaggcgacaatactatgaataagtcaggaggcctcctagaatgcagccaaataggaaactgttccaaacagaatcagtcttgcatacttctgctcagaaggctcctctcgctttggaaactggaatgaggatcaccaacaggatcctcattttacacaggagttatgagagttacatcctctagcagagatgcttggtcattacctgtggtacatgagattaccgagctaaaagggaaaaaaaacgatcttaatgttctcccatgaactcaacttaagctttttatggaggcactgaggccatgcagctccttttccaaaagacacagataaaagccaaataaggtagaggactttggaaattttctctgaaaagttaaattccacataatagtaagactgtttgctgagagaaaactgacaagtaaaaactggtttaagagacagacattcaagacaaactgtattggaaatacaataatgaattttggcctgatagccctcatgctgtcttatagcaaaacactaaaattcatgcaacagagaaattggtgacatgaggactttttctccagacttcctggggaaaaactgtgagaatatacttttttcttctgtttgctttcgaaatgcattctttcttttgctgactttcccaaactttcccagtcgtttctgatgaaaaattcttcaataggaaaagaccaggtaaacttacatgaaagacatcaagtatcttttgagctccttctctctgccagaggagcaatcaactggattacacaaaactaccttcacaactaaaacaggtagaattggaacaggaattagttgtcattaatatactcgtaataaaataaagcttgttctgaaaccacaaggggtggtaagaagagactgtataaaagctactgggttctctagaaaatggatacagtatacagaatgtgagaagatacagaactcacactccagttataaaaatagacatggttctcagacaaaaagcaaatgagtacaaaagaattctccaaacgtgaactatttttaaaagatacatctatataaaacaacaagatgtcatctcagagctccaaagagtagtttgttgaaatggctgaaaaggggagatgaattggagacagataggtcaagaacccagaacagatgtgtcctactcttgtgtttggcagtgtacattggaggtcacaggcagatagactgcttttggtaatacatatataaataataatggctgactggttgatggtgcttgatggatgaatgagaaaacccaggttatcaaataatctcggtagttgaactgttagcttcttcacttgacaatgttgcacatcagaaatgattctaggttttttttacccagaatgatccctgccattcacaactcatgctccacgccccatggtttctattgtgccctaaaagatcagcctagactaatacataaatagaaaataactctggccttgaaatgaggggcagacaagtacttcatgctcagtacttataaatcacaaagaaatgctgaaattaatggtctgtctccttttactacaaaggagatgccatgagttaaagtcatgaaacaaagaaagtcaaaaagatatgggtagcagcacctttccatacccgcctggattttcaaggagcttttcactccttatgcctttcaaacaaaagttcatcagtttgaagaaaaagaaatggctctaaagttaaagagtccccagagaaaactaacagtacatgaaataggccctatgtgggcaaaaggacaagctgcagaaccagttaagacagaagaggcagcccaaggtcttactaaattacagttttagcatagtgtagcacaacatgggcagccctttttccatccaagcaacaattcagcaccatccacgtctggttcaaaagattactgaagtctgggctttcatctttggtaccacctcatgagttattcttggtttgcagtaggttcaaagaaacagaaaagctggtacctttgccttgtctgtgagtacaaacgctgggactctgattgctgcaaccattgaggccaattaaaataatactgtaacacacaggaatgatgcatccaattcctaatttccagataatagcagccatgcccctacagaggcgggatcatccatccccatcgtttaaggccttcggtttgttgtcctcagagtagaatagaacactgtgttcccacggacaaggaactccagatgaacccatggtctacatttggacagaattttaagtaccagatatgccaggcacagaaagaggactgacctgtggccatcatgcttggagaagcttctgttttggcacacaaactagaaacttcttagtgtattctggttttagttccctttcctgagtgaagcagccagggagtgaccaggttccataagccctcaatctgatacttggcattaattctctccatggtcttcttccacccaagctacaattttcccttcccatccagggatggcatcatcatcatggaaaatctcctctttgacagtgccaaactcaggatccagtgctttgaagtgataccggtgatttccttcccgatcaatagctgctttaaaatcctttaacgtcacctcctccaacctctttggtatattgaccatgaagggcgtaagtgaccggtcagtgaaatagagcactttagtacaggtgctgctgacagttggagagctctgtgagtgaggcaactttgagttagggggccaggactcccggtattcactacctacttgagttctgggtgacttgacccgaacctttctttcttgtttcttctgcgtctccataacatgcaggcgctccatgaggctagaaatgccctgctccaagctgtcaatagtgtggtgctgaggatcgtggccactgaagctgttgcgcaggctgcggagagcatctcgaacaagctgcaggtcgctggtccctctgttgctgactgaagtagctccttttcctgccgttggaaggagaaaaccattgctttgagagttgtgactgttgtagttggtcgcctcatctgcctctcttttcatacagtgagccaagaggacatctttgtgttctagctctcgctctagatccacctggtggtaactgacatcagagagtttccggagtgcttcttctaacttggcctggtgctgctgaagaaggcgatccttctgccccagctcttttttatattctcccaagagccggttcctctcatctagcttcctctgcagatccacattctggttgtgcagctcatctttgtccatatttgccctcagtagctcttgtttgagctgaagaacagatgtgtcctgctgagtcaatctctgctgcaaggcatcctttatcccctgtaagtttctggcttcttgtttacatttcagcagttccttctttaagtcctgattctcctccatactctgatccagacgactttggattataatcagttgttcctcgggattgacacctggttcacagagggccaagggcctctcctgttcatcttcaggtaaggatccattgagcagtaaggcctgtagtcctgatatcattttctttgcttcctccatttctttttctaaatattcttgttgttccaacagctgttcttcccatgaggtctccagataggttccagggctccctggccgccagtctcgagataatggagaatctgtcccttctgttctgttctctattccttcagcgggaataatcacaaaatctgccttctcttctgactgggttataatggactcgctctttgcactgtggattggactgggtgaagtcaggctctgtctatatcgaaagacatcccgtcctgatcgggacatgtcatgacacacatcggccagagcagcagctgctccctgggcaacagcagtggcacagtgtggtcggtgactttgcagaggggctctggagtcccgtccttggttcaccgtcctgctggagccaggtttgaaatgagctgccaaggcaaggaccagcctcatgatagacttcaggtttccatccacaatatctttagccgaagtctggtgcatacgaatctttttagaggccacaaactgtagcactttctccacattattcttcatctcctgttggttaccgggactcagctgtaccccactcagcttttctcctgcaacaatctcgatgagatatgccaggatcaccccatcccggagatcttgtcgcaggtcctgcacaggcttcactgctggcctcttcttcagctgtgcattcacccaggccacataggcctgcagctgttgagaaggctctgttggcagcaaggagttattgaatctcataaccacttgggtccccatcttcaagagtccctagaagagacgaatcagggccatctcttaaatgatgggtccgtctggttcagcatctctgtccccagccctcctgagctcggcctgccagtgctctggctttgccgcggtttcccgctgccatggtgatgcgggggccggccacaagccccgcccgactccagccagccagagccagcccctgccggccttggtcccgcctctggcccgccggatcccgcctcctgcaggcccagaccgcgc

SEQ ID NO: 11986 - RNA, 5337 nt, Homo sapiens
  source 1..5337: mol_type = other RNA
ctgaatagctgggactacaggtgtgtgccaccatccccagctacttttataataaaatttctatgtagagacggagtcttcctacgttgcccaggctggtcttgaactcctgggctcaagcagtcttcctgcctcggcctcccaaagtgctggaattacaggcatgagccaccacactcagccttaaatgaagattttgtaaggaattgagcattcaactaaactcgtttttgtgagatggtcattttgttttaacctaacatggtttagagattattttatgaactctaagcattctggttcctcagttttctcaaagaaagagaactttagcaagtagcaggacaagctaccccacaccaatgccaccaggcgacaatactatgaataagtcaggaggcctcctagaatgcagccaaataggaaactgttccaaacagaatcagtcttgcatacttctgctcagaaggctcctctcgctttggaaactggaatgaggatcaccaacaggatcctcattttacacaggagttatgagagttacatcctctagcagagatgcttggtcattacctgtggtacatgagattaccgagctaaaagggaaaaaaaacgatcttaatgttctcccatgaactcaacttaagctttttatggaggcactgaggccatgcagctccttttccaaaagacacagataaaagccaaataaggtagaggactttggaaattttctctgaaaagttaaattccacataatagtaagactgtttgctgagagaaaactgacaagtaaaaactggtttaagagacagacattcaagacaaactgtattggaaatacaataatgaattttggcctgatagccctcatgctgtcttatagcaaaacactaaaattcatgcaacagagaaattggtgacatgaggactttttctccagacttcctggggaaaaactgtgagaatatacttttttcttctgtttgctttcgaaatgcattctttcttttgctgactttcccaaactttcccagtcgtttctgatgaaaaattcttcaataggaaaagaccaggtaaacttacatgaaagacatcaagtatcttttgagctccttctctctgccagaggagcaatcaactggattacacaaaactaccttcacaactaaaacaggtagaattggaacaggaattagttgtcattaatatactcgtaataaaataaagcttgttctgaaaccacaaggggtggtaagaagagactgtataaaagctactgggttctctagaaaatggatacagtatacagaatgtgagaagatacagaactcacactccagttataaaaatagacatggttctcagacaaaaagcaaatgagtacaaaagaattctccaaacgtgaactatttttaaaagatacatctatataaaacaacaagatgtcatctcagagctccaaagagtagtttgttgaaatggctgaaaaggggagatgaattggagacagataggtcaagaacccagaacagatgtgtcctactcttgtgtttggcagtgtacattggaggtcacaggcagatagactgcttttggtaatacatatataaataataatggctgactggttgatggtgcttgatggatgaatgagaaaacccaggttatcaaataatctcggtagttgaactgttagcttcttcacttgacaatgttgcacatcagaaatgattctaggttttttttacccagaatgatccctgccattcacaactcatgctccacgccccatggtttctattgtgccctaaaagatcagcctagactaatacataaatagaaaataactctggccttgaaatgaggggcagacaagtacttcatgctcagtacttataaatcacaaagaaatgctgaaattaatggtctgtctccttttactacaaaggagatgccatgagttaaagtcatgaaacaaagaaagtcaaaaagatatgggtagcagcacctttccatacccgcctggattttcaaggagcttttcactccttatgcctttcaaacaaaagttcatcagtttgaagaaaaagaaatggctctaaagttaaagagtccccagagaaaactaacagtacatgaaataggccctatgtgggcaaaaggacaagctgcagaaccagttaagacagaagaggcagcccaaggtcttactaaattacagttttagcatagtgtagcacaacatgggcagccctttttccatccaagcaacaattcagcaccatccacgtctggttcaaaagattactgaagtctgggctttcatctttggtaccacctcatgagttattcttggtttgcagtaggttcaaagaaacagaaaagctggtacctttgccttgtctgtgagtacaaacgctgggactctgattgctgcaaccattgaggccaattaaaataatactgtaacacacaggaatgatgcatccaattcctaatttccagataatagcagccatgcccctacagaggcgggatcatccatccccatcgtttaaggccttcggtttgttgtcctcagagtagaatagaacactgtgttcccacggacaaggaactccagatgaacccatggtctacatttggacagaattttaagtaccagatatgccaggcacagaaagaggactgacctgtggccatcatgcttggagaagcttctgttttggcacacaaactagaaacttcttagtgtattctggttttagttccctttcctgagtgaagcagccagggagtgaccaggttccataagccctcaatctgatacttggcattaattctctccatggtcttcttccacccaagctacaattttcccttcccatccagggatggcatcatcatcatggaaaatctcctctttgacagtgccaaactcaggatccagtgctttgaagtgataccggtgatttccttcccgatcaatagctgctttaaaatcctttaacgtcacctcctccaacctctttggtatattgaccatgaagggcgtaagtgaccggtcagtgaaatagagcactttagtacaggtgctgctgacagttggagagctctgtgagtgaggcaactttgagttagggggccaggactcccggtattcactacctacttgagttctgggtgacttgacccgaacctttctttcttgtttcttctgcgtctccataacatgcaggcgctccatgaggctagaaatgccctgctccaagctgtcaatagtgtggtgctgaggatcgtggccactgaagctgttgcgcaggctgcggagagcatctcgaacaagctgcaggtcgctggtccctctgttgctgactgaagtagctccttttcctgccgttggaaggagaaaaccattgctttgagagttgtgactgttgtagttggtcgcctcatctgcctctcttttcatacagtgagccaagaggacatctttgtgttctagctctcgctctagatccacctggtggtaactgacatcagagagtttccggagtgcttcttctaacttggcctggtgctgctgaagaaggcgatccttctgccccagctcttttttatattctcccaagagccggttcctctcatctagcttcctctgcagatccacattctggttgtgcagctcatctttgtccatatttgccctcagtagctcttgtttgagctgaagaacagatgtgtcctgctgagtcaatctctgctgcaaggcatcctttatcccctgtaagtttctggcttcttgtttacatttcagcagttccttctttaagtcctgattctcctccatactctgatccagacgactttggattataatcagttgttcctcgggattgacacctggttcacagagggccaagggcctctcctgttcatcttcaggtaaggatccattgagcagtaaggcctgtagtcctgatatcattttctttgcttcctccatttctttttctaaatattcttgttgttccaacagctgttcttcccatgaggtctccagataggttccagggctccctggccgccagtctcgagataatggagaatctgtcccttctgttctgttctctattccttcagcgggaataatcacaaaatctgccttctcttctgactgggttataatggactcgctctttgcactgtggattggactgggtgaagtcaggctctgtctatatcgaaagacatcccgtcctgatcgggacatgtcatgacacacatcggccagagcagcagctgctccctgggcaacagcagtggcacagtgtggtcggtgactttgcagaggggctctggagtcccgtccttggttcaccgtcctgctggagccaggtttgaaatgagctgccaaggcaaggaccagcctcatgatagacttcaggtttccatccacaatatctttagccgaagtctggtgcatacgaatctttttagaggccacaaactgtagcactttctccacattattcttcatctcctgttggttaccgggactcagctgtaccccactcagcttttctcctgcaacaatctcgatgagatatgccaggatcaccccatcccggagatcttgtcgcaggtcctgcacaggcttcactgctggcctcttcttcagctgtgcattcacccaggccacataggcctgcagctgttgctcattgaagccctcctgcaggacgtccagtaagttccctcgggtcaggcaggctagcattgttcctgctgggggctccccgggcggggtctccagcccggcggccgccgccgcctcctcctcctccctctgcacacaaaggctctcggctcagctcattgggatccctccggagtcccgcatgccacttactggaaacctagactggagccaaactagcggcttgcactgggcatgctcgcacgggggcctccgctggaggggcccggcgcggtcgcggttcctatggaaacaactgggcgcgcactaggttgagcggcgctgccgggctgcccccagccccgctttcctgcgggaaagccgcacggccaggcgggctggcgagggcgcgcgctgcacgcccgcacgcacgcgcacaccccccccccgcccgggccgcagcacgggcgtgtgtgcgtgcgctacacacacacacactcacacggcttttaggcaaacgtgctgctgtatgtgcgcgctgtgtgcatacacacacacacacacatacacacatacacacatacacacacacacgttgacaaacaggcggcccggctggcgtatgcatgcgcttg

SEQ ID NO: 11987 - RNA, 5143 nt, Homo sapiens
  source 1..5143: mol_type = other RNA
ctgaatagctgggactacaggtgtgtgccaccatccccagctacttttataataaaatttctatgtagagacggagtcttcctacgttgcccaggctggtcttgaactcctgggctcaagcagtcttcctgcctcggcctcccaaagtgctggaattacaggcatgagccaccacactcagccttaaatgaagattttgtaaggaattgagcattcaactaaactcgtttttgtgagatggtcattttgttttaacctaacatggtttagagattattttatgaactctaagcattctggttcctcagttttctcaaagaaagagaactttagcaagtagcaggacaagctaccccacaccaatgccaccaggcgacaatactatgaataagtcaggaggcctcctagaatgcagccaaataggaaactgttccaaacagaatcagtcttgcatacttctgctcagaaggctcctctcgctttggaaactggaatgaggatcaccaacaggatcctcattttacacaggagttatgagagttacatcctctagcagagatgcttggtcattacctgtggtacatgagattaccgagctaaaagggaaaaaaaacgatcttaatgttctcccatgaactcaacttaagctttttatggaggcactgaggccatgcagctccttttccaaaagacacagataaaagccaaataaggtagaggactttggaaattttctctgaaaagttaaattccacataatagtaagactgtttgctgagagaaaactgacaagtaaaaactggtttaagagacagacattcaagacaaactgtattggaaatacaataatgaattttggcctgatagccctcatgctgtcttatagcaaaacactaaaattcatgcaacagagaaattggtgacatgaggactttttctccagacttcctggggaaaaactgtgagaatatacttttttcttctgtttgctttcgaaatgcattctttcttttgctgactttcccaaactttcccagtcgtttctgatgaaaaattcttcaataggaaaagaccaggtaaacttacatgaaagacatcaagtatcttttgagctccttctctctgccagaggagcaatcaactggattacacaaaactaccttcacaactaaaacaggtagaattggaacaggaattagttgtcattaatatactcgtaataaaataaagcttgttctgaaaccacaaggggtggtaagaagagactgtataaaagctactgggttctctagaaaatggatacagtatacagaatgtgagaagatacagaactcacactccagttataaaaatagacatggttctcagacaaaaagcaaatgagtacaaaagaattctccaaacgtgaactatttttaaaagatacatctatataaaacaacaagatgtcatctcagagctccaaagagtagtttgttgaaatggctgaaaaggggagatgaattggagacagataggtcaagaacccagaacagatgtgtcctactcttgtgtttggcagtgtacattggaggtcacaggcagatagactgcttttggtaatacatatataaataataatggctgactggttgatggtgcttgatggatgaatgagaaaacccaggttatcaaataatctcggtagttgaactgttagcttcttcacttgacaatgttgcacatcagaaatgattctaggttttttttacccagaatgatccctgccattcacaactcatgctccacgccccatggtttctattgtgccctaaaagatcagcctagactaatacataaatagaaaataactctggccttgaaatgaggggcagacaagtacttcatgctcagtacttataaatcacaaagaaatgctgaaattaatggtctgtctccttttactacaaaggagatgccatgagttaaagtcatgaaacaaagaaagtcaaaaagatatgggtagcagcacctttccatacccgcctggattttcaaggagcttttcactccttatgcctttcaaacaaaagttcatcagtttgaagaaaaagaaatggctctaaagttaaagagtccccagagaaaactaacagtacatgaaataggccctatgtgggcaaaaggacaagctgcagaaccagttaagacagaagaggcagcccaaggtcttactaaattacagttttagcatagtgtagcacaacatgggcagccctttttccatccaagcaacaattcagcaccatccacgtctggttcaaaagattactgaagtctgggctttcatctttggtaccacctcatgagttattcttggtttgcagtaggttcaaagaaacagaaaagctggtacctttgccttgtctgtgagtacaaacgctgggactctgattgctgcaaccattgaggccaattaaaataatactgtaacacacaggaatgatgcatccaattcctaatttccagataatagcagccatgcccctacagaggcgggatcatccatccccatcgtttaaggccttcggtttgttgtcctcagagtagaatagaacactgtgttcccacggacaaggaactccagatgaacccatggtctacatttggacagaattttaagtaccagatatgccaggcacagaaagaggactgacctgtggccatcatgcttggagaagcttctgttttggcacacaaactagaaacttcttagtgtattctggttttagttccctttcctgagtgaagcagccagggagtgaccaggttccataagccctcaatctgatacttggcattaattctctccatggtcttcttccacccaagctacaattttcccttcccatccagggatggcatcatcatcatggaaaatctcctctttgacagtgccaaactcaggatccagtgctttgaagtgataccggtgatttccttcccgatcaatagctgctttaaaatcctttaacgtcacctcctccaacctctttggtatattgaccatgaagggcgtaagtgaccggtcagtgaaatagagcactttagtacaggtgctgctgacagttggagagctctgtgagtgaggcaactttgagttagggggccaggactcccggtattcactacctacttgagttctgggtgacttgacccgaacctttctttcttgtttcttctgcgtctccataacatgcaggcgctccatgaggctagaaatgccctgctccaagctgtcaatagtgtggtgctgaggatcgtggccactgaagctgttgcgcaggctgcggagagcatctcgaacaagctgcaggtcgctggtccctctgttgctgactgaagtagctccttttcctgccgttggaaggagaaaaccattgctttgagagttgtgactgttgtagttggtcgcctcatctgcctctcttttcatacagtgagccaagaggacatctttgtgttctagctctcgctctagatccacctggtggtaactgacatcagagagtttccggagtgcttcttctaacttggcctggtgctgctgaagaaggcgatccttctgccccagctcttttttatattctcccaagagccggttcctctcatctagcttcctctgcagatccacattctggttgtgcagctcatctttgtccatatttgccctcagtagctcttgtttgagctgaagaacagatgtgtcctgctgagtcaatctctgctgcaaggcatcctttatcccctgtaagtttctggcttcttgtttacatttcagcagttccttctttaagtcctgattctcctccatactctgatccagacgactttggattataatcagttgttcctcgggattgacacctggttcacagagggccaagggcctctcctgttcatcttcaggtaaggatccattgagcagtaaggcctgtagtcctgatatcattttctttgcttcctccatttctttttctaaatattcttgttgttccaacagctgttcttcccatgaggtctccagataggttccagggctccctggccgccagtctcgagataatggagaatctgtcccttctgttctgttctctattccttcagcgggaataatcacaaaatctgccttctcttctgactgggttataatggactcgctctttgcactgtggattggactgggtgaagtcaggctggagcagctggattcagacggggacctttgttgcccttcgtactgctgcactagggcccgcacactccagtatggattctcaatttcctcatccatgctgctgttcctctgtctatatcgaaagacatcccgtcctgatcgggacatgtcatgacacacatcggccagagcagcagctgctccctgggcaacagcagtggcacagtgtggtcggtgactttgcagaggggctctggagtcccgtccttggttcaccgtcctgctggagccaggtttgaaatgagctgccaaggcaaggaccagcctcatgatagacttcaggtttccatccacaatatctttagccgaagtctggtgcatacgaatctttttagaggccacaaactgtagcactttctccacattattcttcatctcctgttggttaccgggactcagctgtaccccactcagcttttctcctgcaacaatctcgatgagatatgccaggatcaccccatcccggagatcttgtcgcaggtcctgcacaggcttcactgctggcctcttcttcagctgtgcattcacccaggccacataggcctgcagctgttgagaaggctctgttggcagcaaggagttattgaatctcataaccacttgggtccccatcttcaagagtccctagaagagacgaatcagggccatctcttaaatgatgggtccgtctggttcagcatctctgtccccagccctcctgagctcggcctgccagtgctctggctttgccgcggtttcccgctgccatggtgatgcgggggccggccacaagccccgcccgactccagccagccagagccagcccctgccggccttggtcccgcctctggcccgccggatcccgcctcctgcaggcccagaccgcgc

SEQ ID NO: 11988 - RNA, 5016 nt, Homo sapiens
  source 1..5016: mol_type = other RNA
ctgaatagctgggactacaggtgtgtgccaccatccccagctacttttataataaaatttctatgtagagacggagtcttcctacgttgcccaggctggtcttgaactcctgggctcaagcagtcttcctgcctcggcctcccaaagtgctggaattacaggcatgagccaccacactcagccttaaatgaagattttgtaaggaattgagcattcaactaaactcgtttttgtgagatggtcattttgttttaacctaacatggtttagagattattttatgaactctaagcattctggttcctcagttttctcaaagaaagagaactttagcaagtagcaggacaagctaccccacaccaatgccaccaggcgacaatactatgaataagtcaggaggcctcctagaatgcagccaaataggaaactgttccaaacagaatcagtcttgcatacttctgctcagaaggctcctctcgctttggaaactggaatgaggatcaccaacaggatcctcattttacacaggagttatgagagttacatcctctagcagagatgcttggtcattacctgtggtacatgagattaccgagctaaaagggaaaaaaaacgatcttaatgttctcccatgaactcaacttaagctttttatggaggcactgaggccatgcagctccttttccaaaagacacagataaaagccaaataaggtagaggactttggaaattttctctgaaaagttaaattccacataatagtaagactgtttgctgagagaaaactgacaagtaaaaactggtttaagagacagacattcaagacaaactgtattggaaatacaataatgaattttggcctgatagccctcatgctgtcttatagcaaaacactaaaattcatgcaacagagaaattggtgacatgaggactttttctccagacttcctggggaaaaactgtgagaatatacttttttcttctgtttgctttcgaaatgcattctttcttttgctgactttcccaaactttcccagtcgtttctgatgaaaaattcttcaataggaaaagaccaggtaaacttacatgaaagacatcaagtatcttttgagctccttctctctgccagaggagcaatcaactggattacacaaaactaccttcacaactaaaacaggtagaattggaacaggaattagttgtcattaatatactcgtaataaaataaagcttgttctgaaaccacaaggggtggtaagaagagactgtataaaagctactgggttctctagaaaatggatacagtatacagaatgtgagaagatacagaactcacactccagttataaaaatagacatggttctcagacaaaaagcaaatgagtacaaaagaattctccaaacgtgaactatttttaaaagatacatctatataaaacaacaagatgtcatctcagagctccaaagagtagtttgttgaaatggctgaaaaggggagatgaattggagacagataggtcaagaacccagaacagatgtgtcctactcttgtgtttggcagtgtacattggaggtcacaggcagatagactgcttttggtaatacatatataaataataatggctgactggttgatggtgcttgatggatgaatgagaaaacccaggttatcaaataatctcggtagttgaactgttagcttcttcacttgacaatgttgcacatcagaaatgattctaggttttttttacccagaatgatccctgccattcacaactcatgctccacgccccatggtttctattgtgccctaaaagatcagcctagactaatacataaatagaaaataactctggccttgaaatgaggggcagacaagtacttcatgctcagtacttataaatcacaaagaaatgctgaaattaatggtctgtctccttttactacaaaggagatgccatgagttaaagtcatgaaacaaagaaagtcaaaaagatatgggtagcagcacctttccatacccgcctggattttcaaggagcttttcactccttatgcctttcaaacaaaagttcatcagtttgaagaaaaagaaatggctctaaagttaaagagtccccagagaaaactaacagtacatgaaataggccctatgtgggcaaaaggacaagctgcagaaccagttaagacagaagaggcagcccaaggtcttactaaattacagttttagcatagtgtagcacaacatgggcagccctttttccatccaagcaacaattcagcaccatccacgtctggttcaaaagattactgaagtctgggctttcatctttggtaccacctcatgagttattcttggtttgcagtaggttcaaagaaacagaaaagctggtacctttgccttgtctgtgagtacaaacgctgggactctgattgctgcaaccattgaggccaattaaaataatactgtaacacacaggaatgatgcatccaattcctaatttccagataatagcagccatgcccctacagaggcgggatcatccatccccatcgtttaaggccttcggtttgttgtcctcagagtagaatagaacactgtgttcccacggacaaggaactccagatgaacccatggtctacatttggacagaattttaagtaccagatatgccaggcacagaaagaggactgacctgtggccatcatgcttggagaagcttctgttttggcacacaaactagaaacttcttagtgtattctggttttagttccctttcctgagtgaagcagccagggagtgaccaggttccataagccctcaatctgatacttggcattaattctctccatggtcttcttccacccaagctacaattttcccttcccatccagggatggcatcatcatcatggaaaatctcctctttgacagtgccaaactcaggatccagtgctttgaagtgataccggtgatttccttcccgatcaatagctgctttaaaatcctttaacgtcacctcctccaacctctttggtatattgaccatgaagggcgtaagtgaccggtcagtgaaatagagcactttagtacaggtgctgctgacagttggagagctctgtgagtgaggcaactttgagttagggggccaggactcccggtattcactacctacttgagttctgggtgacttgacccgaacctttctttcttgtttcttctgcgtctccataacatgcaggcgctccatgaggctagaaatgccctgctccaagctgtcaatagtgtggtgctgaggatcgtggccactgaagctgttgcgcaggctgcggagagcatctcgaacaagctgcaggtcgctggtccctctgttgctgactgaagtagctccttttcctgccgttggaaggagaaaaccattgctttgagagttgtgactgttgtagttggtcgcctcatctgcctctcttttcatacagtgagccaagaggacatctttgtgttctagctctcgctctagatccacctggtggtaactgacatcagagagtttccggagtgcttcttctaacttggcctggtgctgctgaagaaggcgatccttctgccccagctcttttttatattctcccaagagccggttcctctcatctagcttcctctgcagatccacattctggttgtgcagctcatctttgtccatatttgccctcagtagctcttgtttgagctgaagaacagatgtgtcctgctgagtcaatctctgctgcaaggcatcctttatcccctgtaagtttctggcttcttgtttacatttcagcagttccttctttaagtcctgattctcctccatactctgatccagacgactttggattataatcagttgttcctcgggattgacacctggttcacagagggccaagggcctctcctgttcatcttcaggtaaggatccattgagcagtaaggcctgtagtcctgatatcattttctttgcttcctccatttctttttctaaatattcttgttgttccaacagctgttcttcccatgaggtctccagataggttccagggctccctggccgccagtctcgagataatggagaatctgtcccttctgttctgttctctattccttcagcgggaataatcacaaaatctgccttctcttctgactgggttataatggactcgctctttgcactgtggattggactgggtgaagtcaggctggagcagctggattcagacggggacctttgttgcccttcgtactgctgcactagggcccgcacactccagtatggattctcaatttcctcatccatgctgctgttcctctgtctatatcgaaagacatcccgtcctgatcgggacatgtcatgacacacatcggccagagcagcagctgctccctgggcaacagcagtggcacagtgtggtcggtgactttgcagaggggctctggagtcccgtccttggttcaccgtcctgctggagccaggtttgaaatgagctgccaaggcaaggaccagcctcatgatagacttcaggtttccatccacaatatctttagccgaagtctggtgcatacgaatctttttagaggccacaaactgtagcactttctccacattattcttcatctcctgttggttaccgggactcagctgtaccccactcagcttttctcctgcaacaatctcgatgagatatgccaggatcaccccatcccggagatcttgtcgcaggtcctgcacaggcttcactgctggcctcttcttcagctgtgcattcacccaggccacataggcctgcagctgttgagaaggctctgttggcagcaaggagttattgaatctcataaccacttgggtccccatcttcaagagtccctcttaaatgatgggtccgtctggttcagcatctctgtccccagccctcctgagctcggcctgccagtgctctggctttgccgcggtttcccgctgccatggtgatgcgggggccg

SEQ ID NO: 11989 - RNA, 5048 nt, Homo sapiens
  source 1..5048: mol_type = other RNA
ctgaatagctgggactacaggtgtgtgccaccatccccagctacttttataataaaatttctatgtagagacggagtcttcctacgttgcccaggctggtcttgaactcctgggctcaagcagtcttcctgcctcggcctcccaaagtgctggaattacaggcatgagccaccacactcagccttaaatgaagattttgtaaggaattgagcattcaactaaactcgtttttgtgagatggtcattttgttttaacctaacatggtttagagattattttatgaactctaagcattctggttcctcagttttctcaaagaaagagaactttagcaagtagcaggacaagctaccccacaccaatgccaccaggcgacaatactatgaataagtcaggaggcctcctagaatgcagccaaataggaaactgttccaaacagaatcagtcttgcatacttctgctcagaaggctcctctcgctttggaaactggaatgaggatcaccaacaggatcctcattttacacaggagttatgagagttacatcctctagcagagatgcttggtcattacctgtggtacatgagattaccgagctaaaagggaaaaaaaacgatcttaatgttctcccatgaactcaacttaagctttttatggaggcactgaggccatgcagctccttttccaaaagacacagataaaagccaaataaggtagaggactttggaaattttctctgaaaagttaaattccacataatagtaagactgtttgctgagagaaaactgacaagtaaaaactggtttaagagacagacattcaagacaaactgtattggaaatacaataatgaattttggcctgatagccctcatgctgtcttatagcaaaacactaaaattcatgcaacagagaaattggtgacatgaggactttttctccagacttcctggggaaaaactgtgagaatatacttttttcttctgtttgctttcgaaatgcattctttcttttgctgactttcccaaactttcccagtcgtttctgatgaaaaattcttcaataggaaaagaccaggtaaacttacatgaaagacatcaagtatcttttgagctccttctctctgccagaggagcaatcaactggattacacaaaactaccttcacaactaaaacaggtagaattggaacaggaattagttgtcattaatatactcgtaataaaataaagcttgttctgaaaccacaaggggtggtaagaagagactgtataaaagctactgggttctctagaaaatggatacagtatacagaatgtgagaagatacagaactcacactccagttataaaaatagacatggttctcagacaaaaagcaaatgagtacaaaagaattctccaaacgtgaactatttttaaaagatacatctatataaaacaacaagatgtcatctcagagctccaaagagtagtttgttgaaatggctgaaaaggggagatgaattggagacagataggtcaagaacccagaacagatgtgtcctactcttgtgtttggcagtgtacattggaggtcacaggcagatagactgcttttggtaatacatatataaataataatggctgactggttgatggtgcttgatggatgaatgagaaaacccaggttatcaaataatctcggtagttgaactgttagcttcttcacttgacaatgttgcacatcagaaatgattctaggttttttttacccagaatgatccctgccattcacaactcatgctccacgccccatggtttctattgtgccctaaaagatcagcctagactaatacataaatagaaaataactctggccttgaaatgaggggcagacaagtacttcatgctcagtacttataaatcacaaagaaatgctgaaattaatggtctgtctccttttactacaaaggagatgccatgagttaaagtcatgaaacaaagaaagtcaaaaagatatgggtagcagcacctttccatacccgcctggattttcaaggagcttttcactccttatgcctttcaaacaaaagttcatcagtttgaagaaaaagaaatggctctaaagttaaagagtccccagagaaaactaacagtacatgaaataggccctatgtgggcaaaaggacaagctgcagaaccagttaagacagaagaggcagcccaaggtcttactaaattacagttttagcatagtgtagcacaacatgggcagccctttttccatccaagcaacaattcagcaccatccacgtctggttcaaaagattactgaagtctgggctttcatctttggtaccacctcatgagttattcttggtttgcagtaggttcaaagaaacagaaaagctggtacctttgccttgtctgtgagtacaaacgctgggactctgattgctgcaaccattgaggccaattaaaataatactgtaacacacaggaatgatgcatccaattcctaatttccagataatagcagccatgcccctacagaggcgggatcatccatccccatcgtttaaggccttcggtttgttgtcctcagagtagaatagaacactgtgttcccacggacaaggaactccagatgaacccatggtctacatttggacagaattttaagtaccagatatgccaggcacagaaagaggactgacctgtggccatcatgcttggagaagcttctgttttggcacacaaactagaaacttcttagtgtattctggttttagttccctttcctgagtgaagcagccagggagtgaccaggttccataagccctcaatctgatacttggcattaattctctccatggtcttcttccacccaagctacaattttcccttcccatccagggatggcatcatcatcatggaaaatctcctctttgacagtgccaaactcaggatccagtgctttgaagtgataccggtgatttccttcccgatcaatagctgctttaaaatcctttaacgtcacctcctccaacctctttggtatattgaccatgaagggcgtaagtgaccggtcagtgaaatagagcactttagtacaggtgctgctgacagttggagagctctgtgagtgaggcaactttgagttagggggccaggactcccggtattcactacctacttgagttctgggtgacttgacccgaacctttctttcttgtttcttctgcgtctccataacatgcaggcgctccatgaggctagaaatgccctgctccaagctgtcaatagtgtggtgctgaggatcgtggccactgaagctgttgcgcaggctgcggagagcatctcgaacaagctgcaggtcgctggtccctctgttgctgactgaagtagctccttttcctgccgttggaaggagaaaaccattgctttgagagttgtgactgttgtagttggtcgcctcatctgcctctcttttcatacagtgagccaagaggacatctttgtgttctagctctcgctctagatccacctggtggtaactgacatcagagagtttccggagtgcttcttctaacttggcctggtgctgctgaagaaggcgatccttctgccccagctcttttttatattctcccaagagccggttcctctcatctagcttcctctgcagatccacattctggttgtgcagctcatctttgtccatatttgccctcagtagctcttgtttgagctgaagaacagatgtgtcctgctgagtcaatctctgctgcaaggcatcctttatcccctgtaagtttctggcttcttgtttacatttcagcagttccttctttaagtcctgattctcctccatactctgatccagacgactttggattataatcagttgttcctcgggattgacacctggttcacagagggccaagggcctctcctgttcatcttcaggtaaggatccattgagcagtaaggcctgtagtcctgatatcattttctttgcttcctccatttctttttctaaatattcttgttgttccaacagctgttcttcccatgaggtctccagataggttccagggctccctggccgccagtctcgagataatggagaatctgtcccttctgttctgttctctattccttcagcgggaataatcacaaaatctgccttctcttctgactgggttataatggactcgctctttgcactgtggattggactgggtgaagtcaggctggagcagctggattcagacggggacctttgttgcccttcgtactgctgcactagggcccgcacactccagtatggattctcaatttcctcatccatgctgctgttcctctgtctatatcgaaagacatcccgtcctgatcgggacatgtcatgacacacatcggccagagcagcagctgctccctgggcaacagcagtggcacagtgtggtcggtgactttgcagaggggctctggagtcccgtccttggttcaccgtcctgctggagccaggtttgaaatgagctgccaaggcaaggaccagcctcatgatagacttcaggtttccatccacaatatctttagccgaagtctggtgcatacgaatctttttagaggccacaaactgtagcactttctccacattattcttcatctcctgttggttaccgggactcagctgtaccccactcagcttttctcctgcaacaatctcgatgagatatgccaggatcaccccatcccggagatcttgtcgcaggtcctgcacaggcttcactgctggcctcttcttcagctgtgcattcacccaggccacataggcctgcagctgttgctcattgaagccctcctgcaggacgtccagtaagttccctcgggtcaggcaggctagcattgttcctgctgggggctccccgggcggggtctccagcccggcggccgccgccgcctcctcctcctccctctgcacacaaaggctctcggctcagctcattgggatccctccggagtcccgcatgccacttactggaaacctagactggagccaaact

SEQ ID NO: 11990 - RNA, 4332 nt, Homo sapiens
  source 1..4332: mol_type = other RNA
ctgaatagctgggactacaggtgtgtgccaccatccccagctacttttataataaaatttctatgtagagacggagtcttcctacgttgcccaggctggtcttgaactcctgggctcaagcagtcttcctgcctcggcctcccaaagtgctggaattacaggcatgagccaccacactcagccttaaatgaagattttgtaaggaattgagcattcaactaaactcgtttttgtgagatggtcattttgttttaacctaacatggtttagagattattttatgaactctaagcattctggttcctcagttttctcaaagaaagagaactttagcaagtagcaggacaagctaccccacaccaatgccaccaggcgacaatactatgaataagtcaggaggcctcctagaatgcagccaaataggaaactgttccaaacagaatcagtcttgcatacttctgctcagaaggctcctctcgctttggaaactggaatgaggatcaccaacaggatcctcattttacacaggagttatgagagttacatcctctagcagagatgcttggtcattacctgtggtacatgagattaccgagctaaaagggaaaaaaaacgatcttaatgttctcccatgaactcaacttaagctttttatggaggcactgaggccatgcagctccttttccaaaagacacagataaaagccaaataaggtagaggactttggaaattttctctgaaaagttaaattccacataatagtaagactgtttgctgagagaaaactgacaagtaaaaactggtttaagagacagacattcaagacaaactgtattggaaatacaataatgaattttggcctgatagccctcatgctgtcttatagcaaaacactaaaattcatgcaacagagaaattggtgacatgaggactttttctccagacttcctggggaaaaactgtgagaatatacttttttcttctgtttgctttcgaaatgcattctttcttttgctgactttcccaaactttcccagtcgtttctgatgaaaaattcttcaataggaaaagaccaggtaaacttacatgaaagacatcaagtatcttttgagctccttctctctgccagaggagcaatcaactggattacacaaaactaccttcacaactaaaacaggtagaattggaacaggaattagttgtcattaatatactcgtaataaaataaagcttgttctgaaaccacaaggggtggtaagaagagactgtataaaagctactgggttctctagaaaatggatacagtatacagaatgtgagaagatacagaactcacactccagttataaaaatagacatggttctcagacaaaaagcaaatgagtacaaaagaattctccaaacgtgaactatttttaaaagatacatctatataaaacaacaagatgtcatctcagagctccaaagagtagtttgttgaaatggctgaaaaggggagatgaattggagacagataggtcaagaacccagaacagatgtgtcctactcttgtgtttggcagtgtacattggaggtcacaggcagatagactgcttttggtaatacatatataaataataatggctgactggttgatggtgcttgatggatgaatgagaaaacccaggttatcaaataatctcggtagttgaactgttagcttcttcacttgacaatgttgcacatcagaaatgattctaggttttttttacccagaatgatccctgccattcacaactcatgctccacgccccatggtttctattgtgccctaaaagatcagcctagactaatacataaatagaaaataactctggccttgaaatgaggggcagacaagtacttcatgctcagtacttataaatcacaaagaaatgctgaaattaatggtctgtctccttttactacaaaggagatgccatgagttaaagtcatgaaacaaagaaagtcaaaaagatatgggtagcagcacctttccatacccgcctggattttcaaggagcttttcactccttatgcctttcaaacaaaagttcatcagtttgaagaaaaagaaatggctctaaagttaaagagtccccagagaaaactaacagtacatgaaataggccctatgtgggcaaaaggacaagctgcagaaccagttaagacagaagaggcagcccaaggtcttactaaattacagttttagcatagtgtagcacaacatgggcagccctttttccatccaagcaacaattcagcaccatccacgtctggttcaaaagattactgaagtctgggctttcatctttggtaccacctcatgagttattcttggtttgcagtaggttcaaagaaacagaaaagctggtacctttgccttgtctgtgagtacaaacgctgggactctgattgctgcaaccattgaggccaattaaaataatactgtaacacacaggaatgatgcatccaattcctaatttccagataatagcagccatgcccctacagaggcgggatcatccatccccatcgtttaaggccttcggtttgttgtcctcagagtagaatagaacactgtgttcccacggacaaggaactccagatgaacccatggtctacatttggacagaattttaagtaccagatatgccaggcacagaaagaggactgacctgtggccatcatgcttggagaagcttctgttttggcacacaaactagaaacttcttagtgtattctggttttagttccctttcctgagtgaagcagccagggagtgaccaggttccataagccctcaatctgatacttggcattaattctctccatggtcttcttccacccaagctacaattttcccttcccatccagggatggcatcatcatcatggaaaatctcctctttgacagtgccaaactcaggatccagtgctttgaagtgataccggtgatttccttcccgatcaatagctgctttaaaatcctttaacgtcacctcctccaacctctttggtatattgaccatgaagggcgtaagtgaccggtcagtgaaatagagcactttagtacaggtgctgctgacagttggagagctctgtgagtgaggcaactttgagttagggggccaggactcccggtattcactacctacttgagttctgggtgacttgacccgaacctttctttcttgtttcttctgcgtctccataacatgcaggcgctccatgaggctagaaatgccctgctccaagctgtcaatagtgtggtgctgaggatcgtggccactgaagctgttgcgcaggctgcggagagcatctcgaacaagctgcaggtcgctggtccctctgttgctgactgaagtagctccttttcctgccgttggaaggagaaaaccattgctttgagagttgtgactgttgtagttggtcgcctcatctgcctctcttttcatacagtgagccaagaggacatctttgtgttctagctctcgctctagatccacctggtggtaactgacatcagagagtttccggagtgcttcttctaacttggcctggtgctgctgaagaaggcgatccttctgccccagctcttttttatattctcccaagagccggttcctctcatctagcttcctctgcagatccacattctggttgtgcagctcatctttgtccatatttgccctcagtagctcttgtttgagctgaagaacagatgtgtcctgctgagtcaatctctgctgcaaggcatcctttatcccctgtaagtttctggcttcttgtttacatttcagcagttccttctttaagtcctgattctcctccatactctgatccagacgactttggattataatcagttgttcctcgggattgacacctggttcacagagggccaagggcctctcctgttcatcttcaggtaaggatccattgagcagtaaggcctgtagtcctgatatcattttctttgcttcctccatttctttttctaaatattcttgttgttccaacagctgttcttcccatgaggtctccagataggttccagggctccctggccgccagtctcgagataatggagaatctgtcccttctgttctgttctctattccttcagcgggaataatcacaaaatctgccttctcttctgactgggttataatggactcgctctttgcactgtggattggactgggtgaagtcaggcttctccactctgagccctcccttggtggacgaggggtcggtcggacaggtcaggcccgcatggggctctggccgctcctcggggtggagactctga

SEQ ID NO: 11991 - RNA, 5126 nt, Homo sapiens
  source 1..5126: mol_type = other RNA
ctgaatagctgggactacaggtgtgtgccaccatccctggctaattcttttatttatttttgagacagggtcttgctctgttgctcaggctggagtacagtggcatgattatggctcactgcagccttgacttcctaggctcaagcgatcctcccaccttagcctccagagtagctgggacaacaggcacacatcaccgtgccaggctaatttaaaacaattttttgtagagacagggtctcactatgttcccagggctcaagcaatcctcctgccttggcctcccaatgttgggactacagacatgaaccaccacacccggccccttgcttttctttacagtttcatcacccatgtgtttcctcctaagaatattgtttagtctcgcctgtttgggggttttatagaaatggaaatatgctacatgtctattctgggacttgcttctttccttctgtagtcagctgtgtatcttttaaaattaccagctcttatgcctcagatctctgtgtttaaggggtctcatttactctcttataaatccccttcaaaaacatcccttaaacatcccaaaaacatccctaaaatgtcatgacacagcaaatcgaccaattcattctgttctcttggatacaggttgtcaaccacatttaggaaagctgtggccagttcctcaccttttcaacctaaatattttcttacatcagagtgacacttttggtagaattaaagatcagagaaatgcattcaaaccttctgcatgataccatcttccaaaaaggtaacatttccaccactacattcttaatgtttctgcatagtcttctacgcttctttctgattttgtctaactgcccatactcccgattcttgtcctcctctacccatgaagtctaaatgtcccattctagagaattgagattttaggtttcacatctttaccttaatctttgaaccatccacatagcttttataccctctaacttcgtatactctccccatgaatgcctatgtgcttagactgcgctttttactcccatgatcctgcagactgttagtaccatttcctaccaaggagaaaggggtatttgaatatctgcatttcatgctcaatagtgtcttcaagatttgaaaattaacaattagctcaaagagctaaacagaatccctccttcctgggatatggatgcacaagaatcatatctattgatcattttcagcttttggaaggccccagtttgcttctgcctatggcgtctaccaggtactgacttccagtgtttacctagtacccaggacacaggctcactctggttcccatagtgatgggtcagtttgccctcccagagattaatgtggtttaaagcagcagagatcaacactggccagggagctaaatggatctgaactacacaaacatccagatctgccttggacagggcttgctccttttcacacaataacaaccctacaaagccaatttccttgaatcagatgggaccttgccactgtgctcctgtggggtaggtggaacccagggttcttattcctgtgacaaagtcccttatgagacagcgagagagtgacagagggagagagtgagagcaagggagagagagggagcacatgagcgtgtatgtgacccggaaggggcacttcaacgcttgtgcctcagtttcctccaatttgtaggagtatacctactagtcagcccactcatctcttcctctgattttcattctctggttcacctattagcctaacctccctaggtggaccagcagttctttgaacaaggattgtgtctttttctatccctggaatacctgatattaagttgaagacataccgtaccaggtactaaaaaaaatactggttgtctaatgtatactgaagcagaacacttcgtccctggctgggggtgtgtgttccagatgtcttacgttccctggtactgctcctgcacagctgttttttaacacttcagggttcagttactctgcctagcactgctgcacctcagtcaccacgtctggcaatccaaatggatcttgccaaccccgggagttctctcgtgaattcttttgtaaacattttataataggagttagcttttgcaaggtcaacaatcacacctacatttgtttttttttacagtcaaattttcgagctttctttcagtggagcctacctatactttgtgaagtgtgtttaatctctgagttatgtacatcaaaagatacttcctagatctttaagaagctctcccaagggaataaaactctgggcaaattggatggtagaagtatttcaccattcatgacaacgtgtttcctttggttgtgttggtatgtttttagtgttaacactggtgaatctagaaagttttcataaactggggcttgataaaggaggttggatttaaactcttacctgaaaaagaaaaaaaaataccaaaaacacatggggataggttggataaatggtgaaagaaacactgagaacaaaagtcattttccccattcactctcatccttggacactttactggaccttccaccctccttctgaagtccagggaaggccacaaacttctcaggcccaaatctgttagcaccagcaggctcagctctaagagccagagccaggtaataagcttagcttcctagcaacccgcacacaagtgttcccgataaaatggattacatactgctgatgaatcccaggtgaatatcatactgacccaacaaaggaattaatttgtacctcctgccacactaaggaggcggactgagagaattctttttgcccatgatccttcctggcattctccctggaacgtcatggtaaaaacaaaatgctccaatgaggtcaaaagtggaggcttcaacttcctattgcctcttggtctggaagcagcagtagagttgggtaaggtacgggtgtttccgtgccagagccaaaatcctcttctctgtcattgtgcagtccacgtcatcatcctgaaggatgacgtccttctttaagaccttcacagcatatacttcatctttgcccttgagttctgccaacatgaccttgccaaagctgcctttgcccaacaccttgatgaagttgaactcatccaggcccaggcgcttggcctggccttgccggacttcgccattctcaccggggctcatcagctggccatcaggagacgatgctgcccggtgctcctctcctcggttgtcaaatgacaaggctttccgaatgttgttctcaagttcttttatttcctggtcacaaggggaggtgggtgctgacttggatcgatcttcctcagatggtgagcttccagaagcaggctgcggggactcggcaccagcaatgagctttttccttctctggccgctgttggtgattttgtctggggtaacgcccaggtcggccagtactttggcgattcctctggcatccactccacagttgggagccacgttggtctcacatcgacggtgaacattcattttgcagactttacactgcaaaccctgccgcaagagtccccagagcagggacccacagtgatcgcagaaggtagggaccttgtagttgtggataccgaacttgtggggcatgttgacgctgaaccgctgggagcccacctggtcgggggtctcctgcttctttaacccagcacactttgtgattatgagctcgtggcaccgcttgtggaccacgcaggtgcagacttgacactggtatccctgctttcctatgacaccccagatgaagtctctgcaatgggagcagtaggtgggctgccgaagataggtggccatgaacttgtggccgttgacctgatggaccctgcgcctgacggccccctgccgcttcctcggccgcatgcgttccctgaacacacgctcttcattgtctttaggggcttcacccgacgaccctgagagatcgatgatcacatacactcttccttctggctccagatcaatccagtcctcgaagtggcggctcccgttctgcagcagctcctcaaactggatggtgcagttggccacgaagtcgtcgtagcctatgggggcatcgtgaaagacagccagctcgatcttgcgtccgttgcacacatcggtgacgaactcgtcgtgccaggccgggctgttggtcttctgcttggtggccgtttggccgatgcgcgagtcgtccacattgagggcaatgtaggggtcgagaaggaaagtctgcggccggggtcccaccgcatggcgcagcgaccaggctgtgggcttcaagctcacggcctcgcagattttgatcttaagaaggccattgaacactaccatggtcggggcggggagtgggggccggggtcactccgtctgccccgagggcaggaatgaagaaccgacggcccggcactccgagccacagggactcttgggtcccctttcgccccaccccgcacactccctacaccttgtggcgttgcgccctggcgcgggcgattctcagccagtgcatgtatttcctcgccgggttcctaacggaaaacagggaggggggagagctgggggatgtccgtgtttggagcaagtctctccccccgaccaccagctgcacctccagaagagaagacgagctgtcggctccgctgcaagccgcgggggctgcctcgccgcctcgctggctctccggctccggactgcgggaaagcgggcgccgcgcccggcgcttacctacctttccgaaacataatcccgggaaatttcgactccgggagggggatggggcggtgggacggggcggggacgagaaccgggggcgcagatttcaacccggatcctcttcgcacactcagcgcctgcctctgaccgcgcggggcgggggggtgaacggagggatgttcagtctatccggagggatgcatgtcgagaggaaatggtcctcctcggagccaaatttttaaaaatccacaagccccacggccagccggggccgccgcctcctgggcgaagcagcgccgcgccggagccggcgatcgggaggcgccaggagcccggaatctcacatccgcgcgggctcggagtccgggcggccgccgatccggctcgggggcgcaggccagcacc

SEQ ID NO: 11992 - RNA, 1869 nt, Homo sapiens
  source 1..1869: mol_type = other RNA
ctgaatagctgggactacaggtgtgtgccaccatgcccagacgcccagctaatgtttgtattttttgtagagatgggggtctcactatgttgcccaggctggcctcaagcaatcctcccacctgagccccgcaaagtactcggattacaggtgtgagtcaccgcgcctggccgggagctttaatttttcctacttgttaacagcgttatggggctggaaggaggctctcagatttccctgccctcctcacatcccccaaccctccctgggcgtgggggtgtcaagcatgagtcaggctgagcctgactctgaagctgttcccagctctttagtctaaacttcaaatcttcaaccctgttccctaatccaacacattccccaaatgaagggactggacagtgagatatcgggaaaccccatgaaaatagatgcataataaaggtgaaaatcatttaaaatgttcccattttttttttttttcaaaacagtcttgctctgtcaccgaggctggagtgcagtggcgtgatcttggctcactgcaacctccgcctcccaggttcaagcaattctcccaccttagcctcccgagtagctgggattacggctgtgagtcaccacacccggctaatttttgtagtttttgtagagacgggttttcaccgtgttggccaggctggtctcgaactcctggcatcaagtgatccgcccacctcagcctcccaaagtgttaggattacaggtgtgagccactgtgcccggcccccagtattttttaagctcaaatgatcccatgtccccaagactgtgacaaactaaataaccaaaaaagtgtggccacggtccaggtggaagggggctgcctggaggtacgttcccatcaaaacctgctcctgggcagggctcacactgctcacagcatcaggggtcagccatcttctcttgaaaccccgtgagttgcaggaggccctgttctgtgctcctcatttcaatcccgggatcagtcaagtctggagccaaggaggcggttcacacgggtcttccctggaaggagagggcgatccgcagcagttcctggcccagctcttgctgcctccctccagggccaaactcagccgacagctcccggaaagtgacgcagacgcggcgggcctcgatgtgtctgcggtggatggcatgcttccactggtgccgtgccgccccggtgaggaccagcagggagcgggcgggtaaggggatggccacctccacctcctggcatagcaccgaccggctgggtgctatcacgctgtccaccaaggcctccggggcagccgacggggccgagcagaggagcaggctcccgggcgcctcccgacacatggacagcacggtgggggacaggaggttgaggctgaccagccgctccccccacagccaggcgtcgtccaggtgggggtcaatggcagagccccgctcggggcagtagtccaggttgcactgctcgacgggccggaagccctccagccccgggtagaggcccatcctccgcaccacctcccggctgaagctggggaggccgcagaagccctcggtctttagcttctgtttccgaaagttgactttggggccatagtcctgcttcctccgtccagactgggagagcttccaggggtcacggtccatgagccgcaccaactcggcttcttcctcccgggtcacaaagtcctcgatcagcatcactccgctgggggcagctcccagggcgggtcactgccgcgctgccgctcgcagatcagacaggtccggatgcccttgcaaccgcattcccgaaggacttcgggggtctcggcggcagccgccgccatcgcgccgtccgcgtggccagtgcgc

SEQ ID NO: 11993 - RNA, 1962 nt, Homo sapiens
  source 1..1962: mol_type = other RNA
ctgaatagctgggactacaggtgtgtgccaccatgcccagacgcccagctaatgtttgtattttttgtagagatgggggtctcactatgttgcccaggctggcctcaagcaatcctcccacctgagccccgcaaagtactcggattacaggtgtgagtcaccgcgcctggccgggagctttaatttttcctacttgttaacagcgttatggggctggaaggaggctctcagatttccctgccctcctcacatcccccaaccctccctgggcgtgggggtgtcaagcatgagtcaggctgagcctgactctgaagctgttcccagctctttagtctaaacttcaaatcttcaaccctgttccctaatccaacacattccccaaatgaagggactggacagtgagatatcgggaaaccccatgaaaatagatgcataataaaggtgaaaatcatttaaaatgttcccattttttttttttttcaaaacagtcttgctctgtcaccgaggctggagtgcagtggcgtgatcttggctcactgcaacctccgcctcccaggttcaagcaattctcccaccttagcctcccgagtagctgggattacggctgtgagtcaccacacccggctaatttttgtagtttttgtagagacgggttttcaccgtgttggccaggctggtctcgaactcctggcatcaagtgatccgcccacctcagcctcccaaagtgttaggattacaggtgtgagccactgtgcccggcccccagtattttttaagctcaaatgatcccatgtccccaagactgtgacaaactaaataaccaaaaaagtgtggccacggtccaggtggaagggggctgcctggaggtacgttcccatcaaaacctgctcctgggcagggctcacactgctcacagcatcaggggtcagccatcttctcttgaaaccccgtgagttgcaggaggccctgttctgtgctcctcatttcaatcccgggatcagtcaagtctggagccaaggaggcggttcacacgggtcttccctggaaggagagggcgatccgcagcagttcctggcccagctcttgctgcctccctccagggccaaactcagccgacagctcccggaaagtgacgcagacgcggcgggcctcgatgtgtctgcggtggatggcatgcttccactggtgccgtgccgccccggtgaggaccagcagggagcgggcgggtaaggggatggccacctccacctcctggcatagcaccgaccggctgggtgctatcacgctgtccaccaaggcctccggggcagccgacggggccgagcagaggagcaggctcccgggcgcctcccgacacatggacagcacggtgggggacaggaggttgaggctgaccagccgctccccccacagccaggcgtcgtccaggtgggggtcaatggcagagccccgctcggggcagtagtccaggttgcactgctcgacgggccggaagccctccagccccgggtagaggcccatcctccgcaccacctcccggctgaagctggggaggccgcagaagccctcggtctttagcttctgtttccgaaagttgactttggggccatagtcctgcttcctccgtccagactgggagagcttccaggggtcacggtccatgagccgcaccaactcggcttcttcctcccgggtcacaaagtcctcgatcagcatcactcctgggaaggggaaggcccagccctcaaagtcagactcctctgtgcccacggcccagccggtgtcggagcagtaaatgaaacggtatgttttcgctgggggcagctcccagggcgggtcactgccgcgctgccgctcgcagatcagacaggtccggatgcccttgcaaccgcattcccgaaggacttcgggggtctcggcggcagccgccgccatcgcgccgtccgcgtggccagtgcgcag

SEQ ID NO: 11994 - RNA, 1952 nt, Homo sapiens
  source 1..1952: mol_type = other RNA
ctgaatagctgggactacaggtgtgtgccaccatgcccagacgcccagctaatgtttgtattttttgtagagatgggggtctcactatgttgcccaggctggcctcaagcaatcctcccacctgagccccgcaaagtactcggattacaggtgtgagtcaccgcgcctggccgggagctttaatttttcctacttgttaacagcgttatggggctggaaggaggctctcagatttccctgccctcctcacatcccccaaccctccctgggcgtgggggtgtcaagcatgagtcaggctgagcctgactctgaagctgttcccagctctttagtctaaacttcaaatcttcaaccctgttccctaatccaacacattccccaaatgaagggactggacagtgagatatcgggaaaccccatgaaaatagatgcataataaaggtgaaaatcatttaaaatgttcccattttttttttttttcaaaacagtcttgctctgtcaccgaggctggagtgcagtggcgtgatcttggctcactgcaacctccgcctcccaggttcaagcaattctcccaccttagcctcccgagtagctgggattacggctgtgagtcaccacacccggctaatttttgtagtttttgtagagacgggttttcaccgtgttggccaggctggtctcgaactcctggcatcaagtgatccgcccacctcagcctcccaaagtgttaggattacaggtgtgagccactgtgcccggcccccagtattttttaagctcaaatgatcccatgtccccaagactgtgacaaactaaataaccaaaaaagtgtggccacggtccaggtggaagggggctgcctggaggtacgttcccatcaaaacctgctcctgggcagggctcacactgctcacagcatcaggggtcagccatcttctcttgaaaccccgtgagttgcaggaggccctgttctgtgctcctcatttcaatcccgggatcagtcaagtctggagccaaggaggcggttcacacgggtcttccctggaaggagagggcgatccgcagcagttcctggcccagctcttgctgcctccctccagggccaaactcagccgacagctcccggaaagtgacgcagacgcggcgggcctcgatgtgtctgcggtggatggcatgcttccactggtgccgtgccgccccggtgaggaccagcagggagcgggcgggtaaggggatggccacctccacctcctggcatagcaccgaccggctgggtgctatcacgctgtccaccaaggcctccggggcagccgacggggccgagcagaggagcaggctcccgggcgcctcccgacacatggacagcacggtgggggacaggaggttgaggctgaccagccgctccccccacagccaggcgtcgtccaggtgggggtcaatggcagagccccgctcggggcagtagtccaggttgcactgctcgacgggccggaagccctccagccccgggtagaggcccatcctccgcaccacctcccggctgaagctggggaggccgcagaagccctcggtctttagcttctgtttccgaaagttgactttggggccatagtcttcctccgtccagactgggagagcttccaggggtcacggtccatgagccgcaccaactcggcttcttcctcccgggtcacaaagtcctcgatcagcatcactcctgggaaggggaaggcccagccctcaaagtcagactcctctgtgcccacggcccagccggtgtcggagcagtaaatgaaacggtatgttttcgctgggggcagctcccagggcgggtcactgccgcgctgccgctcgcagatcagacaggtccggatgcccttgcaaccgcattcccgaaggacttcgggggtctcggcggcagccgccgccatcgcgccgtccgcgtggccagt

SEQ ID NO: 11995 - RNA, 8055 nt, Homo sapiens
  source 1..8055: mol_type = other RNA
ctgaatagctgggactacaggtgtgtgccaccatgcccagctaatttttgtatttttagtagagacggggtttcaccgtgttggccaggatggtctctatctcttgacctcataatccgcccgcctcggcttcccaaagtgctgggattacaggtgtaagccactgtgcctgaccggaaactgtttcttaacatacatcatgcacgtaatcttcgctctcccaagaggcattcacccaagcagacaggcaagcatctatgtgttcaattcgaaatgcaacaatgacagatgtacaactttaccactcttaaagaaactaacatgccatccattattctccatgtgggaaacattcagtaaacttctaaaaccaaacacaggactctggcatatccccacacccccagcagcaggctgtgacaggctttgatctcaatcaaatgccactgtacacagaacataaaaacaggctcaggatgctgcatgtcactctgacatatcacattatttcatattactctgtcacttactcacaaacaaaagtctccactatggcatgattgagagagaaaataattcactttatataaataacagctaagaacaacatactgtgaacagtttccagagtttgaacattcagcacaatcaattcttacttcttgggaaaaaaatatcttacctatcttttctgttacagtatgccttcttggagaaaatattttagtggtaacatcattttctggggcatttggttaattttgaaagatgattatgccacatgaaccaaaaaaaaaaaaaaaaactggcaggaggaggagggtcctaggccattctggaagcaagctgggttttgcattattcagagtcaactattaagctgacttatattagaatggcgacagataagaggcaatgagtgacaccaggacatgcacagcacacagagaatatggtctactcttgtcttccctgcacagattaaacataagaggcttggtagaaagacatggggaaaggtgctatgggggccagcatttggaaagcatatatcccagtgacttgagtatttgctatgcaacctcctggacgagaaactgggaaaaggcacacttccgcccacagttgtggacagcagcagtcacccgtctgaatgctttcattcaatgtgaagatgcagcttgaacaaaagtttctttttgtttgtttgttttctgagatggagtctcgctctgtcacccaggctggagtgcagtggcacgatctcagctcactgcaacctctgcctcctgggttcaggcgattctcctgtctctgcctcccgagtagctgggaatagagggtgagccacaacacccggctaatttttgtatttttagtagagacggggtttcaccatattggccaggctggtcttgaactcctgacctcatgatccgtccgcctcagcctcccaaagtgctgggattacaggtgtgagccaccacgcctggccgaacaaaagttttttaatcttactgatcccatctttccagctgctctgaacagaggggcagggcggggaaagtcatgtcacagactctgcccacagcagccattctgaggtgccttttcagtctcttatcctcttttgagctttcctcttcttaattttttgttttgttttgttttcattgtactcattaatcccctcctcaatttttaacagaattataaaagcaaagtcaaaaggtccttcaggatgactgggaggcttcctaggctaacttttgcatttgaaaatggaaaaaataaattacttgatatttgtgataagactaagatttcttaaaagtctgcacatcaatatattacctggcttaggagggtgagggcacagtatccatctgcaccctctcctcgtattttttaaaaacaggcaaaatatgtaagaaaaggctggtgcacgttggaagacagagcgtgcctgtctatgccagtgctgctgtgccctgcagcctggcagatggagtcggatgctggggcctcatgcccacttaggccaataacatactcaagactctacagcccgttcaccagcaaagtatgccctgaggggcaacactggctgtggaagtgaagacacacaaagcagggactaaaggcaaatggggcttcacgatgcagcgacatgaagacagaactggtgtgggcgccaaaggcaacctgcagggctcacataaaaggaaaataggacagaaagccacgagttccacaagcagaatcatttctggtcttacatctgagggcatttgtagagaaaagtccaaggcaatgtcccctgggtctgagagaaaaatcctacgcaaaagagggcagacaatgcggtgctcgtcttgagggagcctgaccctgaccctgaccctgacgggctggatgcgagaggggctgagtatggctgtattcagtaaggaaactggtagcagacttttctagaaggtggaaagaaaaagcaaagactttcacagatacaaaaattgttttcaaaacaattacctagaaagttcactgcggttgggtggggaataagtgtaatattttcatttcaaatgagccatggtgctactaatggattataaaagaggatggccagttctggtcttccttcccttcccttaacccccgaaccttcctactcctgacattttccctaccctcactgcaacccacccccatcctggcccaaaattaatttgcccagccactgcaccaaaccagccttgacacacaattgttggttggatttcaattaaacaatgcacctaatgcgttggaagagaaggtggggagggcacaaggatgttggcgtaaacctggaggtgtgtggaccttggacagagcttccgccggccagacccagggcagggtgggcatctgcagtgcagcgcaggccgcaggtaaactgaggtaaggaagaacatggtggctctagctggccctgctttccgagacagtgcagcatgtgtgtgctcttgggtgtgggcaccaaaaaactcattttcttccagttgctgctgccattccaccctctgactagaagaatgctctttacagagtccaaaggatcagccacttggtcttcctctgaggtacaaatccaacagagctttaatcccaaagatccagtggccaccagagtacagaagtcagaatcaaatgctcagaatcaaaaggtgtggcactcctgcccagccggcttatcagcagttgtatagacagatcagaaaaaactagcatttattataaaaactgtttttcaaatggggtgatttcctgtccttctccagagatcataattcttcacgtttctgaggaccttctcggcttggttcttttgtcttctctttgtacagtgctcccgtttctttctccttctgaaagcggatctgtagctgtttgatctcttggtcgtagtcctgccactccgggacaatccgcacagctgcttccagtttcggctctttggtcatcggattattacacaaatcaatggtttttgcccttttcttagaggcgtcatcacaccacgtttcacaccaaagccattcttgagggagggatttaattggcacctgatgaatcatgttattgggcagatcctgatatgatactttcgcccggctaaatgactggcccagtaccctgacttccagaacctgtagccgtccatttctcttcggctgtcacagaaaggagtgtaaccataaggagcaccatccaaattgaaatctcttaactctttcagatctgttcgtacaatctgatcagcatccacaaacaggaacttgtcaacaactagtgggaaaagtacatccaggaagaggatcttgtaaccccagatgatacgctgtttttcagtttgttgatgaagccaccggggccatttgtactgaacaagctcatactggaaattgtattcatttgccatgtaaggtataaactccttaaatgtgggggacaagtaattcttcaagaaccagaatttcacaggagtcttggtattcttcagcacggatagcatcattatgcgaagaaatctttcgtagagatgaccagatgcaacggagaaaatattaattatgtcatctttatcttgcttcacttcctcagtcttctgtcctgtaaagccccatttgaaggaatcccaaaatccagattcattctcactcgttccatcactcagcaagtcttcgttcaccatatctgccttcttctgaaccttcactttaataattttgcttttgaagttgttgaggacgataaccacctcatcagcatcagggggagaatcagtgccatcgtggctgtaaattctataaatatcttcagagcgtcccttcctaagtctgaggatccaagctcctgggttggctttcagctgaaagtagcccagattggccataacaatggtgtccacaatgaccgggttggctgaagttcctaaggtaaactgtagtccccgtggaggctggcctgtggtgatgtcgtagcaatgaccttccagtaacaggtattccagctcatactcagcagccactacactgtccacctcttctaaataaatattatcaagatcatatggtgttctgacagattctaccatccagctctcaggtgtgttcaaattcagagtgaacagtggagactgaggcatatccaaaaattttgcgattggacccttagcaaaactattgtctgaagtgaaagaaatctctggttctaagacataacggtaaaagctttttaaaggcatgtcagaaagtttggattggcagttcataaatactctcagattcatgtttatcagctgagccaaaaccaagagcaaaggagcaagtctctgtgcttctctggtgacagggtcaacgacagccacaacatcaaagtatgtctccccttccttcggcctcagtttgattgcactgtgtctgtcttcaaaaaactggtactcgattcttggatctccttttggttgcgctgacagaagagcatccaccttcattaccaagtcgcttgccacatcttcttctacccgaagctgttgaatatgagattttattttctgtcctgaggtttttaagatgatattttcgaggaggtggaaatcgtcttgattaaagagctcactatcctccagtggcccaatgatccttccattgctgatcactgccctctgtcccttcttcagcttcagaacatccctgcagtacacggcatgagacaaaatgaaatccattttggaagactcaaagacctctttaaaaagactgaaatccattcccccaacagagaactccgcaatgtcagctcctgcagccagggcctctgcagccccctccttggccattttggtgatgaagttcttagcagcgttggaagtctgagtttggagagctgcccagattgctctggagatctgagtgttctcatagcttatctctttggcaggattattgatcatgcttattctaacattgttactggatttctgatgtttgatggcatcatacagtaactgccgtccagaagggctatcaaaatccccaacaatccaaaaagttactggcctaataaaagaatcatcatagatttccttggaggacattcctttctttgtcagatagttcatactattggctacagcagcagtcttgccttgggaatccaagatagtaaatctagcataatcatccacaaagaagttattactcgctgttaaatccaggtagtctcgttcagctgtcaaaatcctagaattgattcgtggaacaacatttggctgattcatgatatactctaccacatcttgatcatggggcagttcacccaagtacaccgctctttggaagaaggtggtggtctccaggattttatgcattgtgatggtttctaactcatcagggtctagctgttccctttcaaagggcattccattgaacagcacaacgggcagaggtccaactccagtctgctcatagtagcctcttgcttccttccgattccgatcataagcagaatcaatccccaaaatgctattcacttctacatacggatatttcttctccaggacactgaccacatgttcaactttcactttttctccagtcctcaccttgttatagatatgtgtcagagtctggaaggcatgataatcatccacttcttgggcaacataattatatgctctaagaacagccactccagcatcttgcatcccatcaacatcttcagagtcattaaccacaaagataaaaccaattcttagtggtatatgattactaaggaacatctcagctgtgttcatcaactctgctgtggtctcatgtgcaggatcaactatgaaaaccatattatgtaagtttttcctgatctgccgaataacaccaggaaaggtgggtcgaagcaactcttgtaaactagaaggccacgaattatatctgctatcaacctccaggttgttgacccatgaaatagcaggactccggatgtctacggcatagtctgcctcagagggctggatgttcagcttcaaaacattatgcagagaaaggccttctattcccaatctatgcagaccctccattacccgagcttcattcctcaacacatcaaacagactgaatatatcctgtgtatctaaatccatgtgaagtccattgatgaagagggctgaatctccaggttgtaatcctaaagttcccttgaaatacttctgattctcttccacttcggttctaagttctgagctcacagctgtttttgttattgctctggctttggtaggaaaattctgactaagatccttcatgacaaccaaagccaactcaacaggagaagccaagattcgagcagcagtctggaaactgagatcttgcaactgccaaacctttaaaggtgccatttcattggtgctctctacaagatgctttctgagttctttcaactgtccctccaggtcggggtgcagatctcttaattttccaaagaggaacccctgaacctcatcaataggatcattttcaccaatcactgtggtgtttacctcagttcctttcacctgagtatcatccttggccttgtactcagtgctcttaatggccaattccacgccatagccagagaggtaaacaggctccttcctgggattaaatatataatgtctgaatacataattgattttgcctgcattgctttttgatataagctggcggtgaaaattggaaaattcctcagagccaatctcagagtagaaaatcaccacagggctttcaggattagacgagggatatctgtgatctcctttgaacaataaaggtttgggtctttcagaggctgtcagtagaagagcctcaagggtatcagattcacaagtcttctttccatgcactgaaaaaaacgaattacatccttctggtggaggttcatcagctgctatctgctggaaggcttggattgtagctgagtaagaacgaagggacagacaaaatttaaacaaattctgctggaggggtgacagaaactgaaatgcagcctccaatattgcatgatagtaggaataatcggtaccgtcatgatctgatgatccaatattttgactggcttctacaaaattccaaaatttctcttgactgtcttctgctaaaaactcactggcttctaacaacaatggagtggaaaaccattttgttgtaagagaggttgtaatggcttttgagtcggcctttactgaggagaacagccacagaacagtgagtacaaccagaactcccattttatagcaaactcctgtcaccggcagcgcacccgcggcacacgcaccgctcgcgtctcccttgcagcccatgcccgggccgtggtcagtccgccacagtgccagagacaacgccagggcagggcggggcgaggcggcagcggcagtgcaggctgcgccagtgagaggccgacacgcgcctttcccgcggctcgactcaacacccagcctcgcaaagcaattgcccagctgccggccgccctttt

SEQ ID NO: 11996 - RNA, 6480 nt, Homo sapiens
  source 1..6480: mol_type = other RNA
ctgaatagctgggactacaggtgtgtgccaccatgcccagctaatttttgtatttttagtagagacggggtttcaccgtgttggccaggatggtctctatctcttgacctcataatccgcccgcctcggcttcccaaagtgctgggattacaggtgtaagccactgtgcctgaccggaaactgtttcttaacatacatcatgcacgtaatcttcgctctcccaagaggcattcacccaagcagacaggcaagcatctatgtgttcaattcgaaatgcaacaatgacagatgtacaactttaccactcttaaagaaactaacatgccatccattattctccatgtgggaaacattcagtaaacttctaaaaccaaacacaggactctggcatatccccacacccccagcagcaggctgtgacaggctttgatctcaatcaaatgccactgtacacagaacataaaaacaggctcaggatgctgcatgtcactctgacatatcacattatttcatattactctgtcacttactcacaaacaaaagtctccactatggcatgattgagagagaaaataattcactttatataaataacagctaagaacaacatactgtgaacagtttccagagtttgaacattcagcacaatcaattcttacttcttgggaaaaaaatatcttacctatcttttctgttacagtatgccttcttggagaaaatattttagtggtaacatcattttctggggcatttggttaattttgaaagatgattatgccacatgaaccaaaaaaaaaaaaaaaaactggcaggaggaggagggtcctaggccattctggaagcaagctgggttttgcattattcagagtcaactattaagctgacttatattagaatggcgacagataagaggcaatgagtgacaccaggacatgcacagcacacagagaatatggtctactcttgtcttccctgcacagattaaacataagaggcttggtagaaagacatggggaaaggtgctatgggggccagcatttggaaagcatatatcccagtgacttgagtatttgctatgcaacctcctggacgagaaactgggaaaaggcacacttccgcccacagttgtggacagcagcagtcacccgtctgaatgctttcattcaatgtgaagatgcagcttgaacaaaagtttctttttgtttgtttgttttctgagatggagtctcgctctgtcacccaggctggagtgcagtggcacgatctcagctcactgcaacctctgcctcctgggttcaggcgattctcctgtctctgcctcccgagtagctgggaatagagggtgagccacaacacccggctaatttttgtatttttagtagagacggggtttcaccatattggccaggctggtcttgaactcctgacctcatgatccgtccgcctcagcctcccaaagtgctgggattacaggtgtgagccaccacgcctggccgaacaaaagttttttaatcttactgatcccatctttccagctgctctgaacagaggggcagggcggggaaagtcatgtcacagactctgcccacagcagccattctgaggtgccttttcagtctcttatcctcttttgagctttcctcttcttaattttttgttttgttttgttttcattgtactcattaatcccctcctcaatttttaacagaattataaaagcaaagtcaaaaggtccttcaggatgactgggaggcttcctaggctaacttttgcatttgaaaatggaaaaaataaattacttgatatttgtgataagactaagatttcttaaaagtctgcacatcaatatattacctggcttaggagggtgagggcacagtatccatctgcaccctctcctcgtattttttaaaaacaggcaaaatatgtaagaaaaggctggtgcacgttggaagacagagcgtgcctgtctatgccagtgctgctgtgccctgcagcctggcagatggagtcggatgctggggcctcatgcccacttaggccaataacatactcaagactctacagcccgttcaccagcaaagtatgccctgaggggcaacactggctgtggaagtgaagacacacaaagcagggactaaaggcaaatggggcttcacgatgcagcgacatgaagacagaactggtgtgggcgccaaaggcaacctgcagggctcacataaaaggaaaataggacagaaagccacgagttccacaagcagaatcatttctggtcttacatctgagggcatttgtagagaaaagtccaaggcaatgtcccctgggtctgagagaaaaatcctacgcaaaagagggcagacaatgcggtgctcgtcttgagggagcctgaccctgaccctgaccctgacgggctggatgcgagaggggctgagtatggctgtattcagtaaggaaactggtagcagacttttctagaaggtggaaagaaaaagcaaagactttcacagatacaaaaattgttttcaaaacaattacctagaaagttcactgcggttgggtggggaataagtgtaatattttcatttcaaatgagccatggtgctactaatggattataaaagaggatggccagttctggtcttccttcccttcccttaacccccgaaccttcctactcctgacattttccctaccctcactgcaacccacccccatcctggcccaaaattaatttgcccagccactgcaccaaaccagccttgacacacaattgttggttggatttcaattaaacaatgcacctaatgcgttggaagagaaggtggggagggcacaaggatgttggcgtaaacctggaggtgtgtggaccttggacagagcttccgccggccagacccagggcagggtgggcatctgcagtgcagcgcaggccgcaggtaaactgaggtaaggaagaacatggtggctctagctggccctgctttccgagacagtgcagcatgtgtgtgctcttgggtgtgggcaccaaaaaactcattttcttccagttgctgctgccattccaccctctgactagaagaatgctctttacagagtccaaaggatcagccacttggtcttcctctgaggtacaaatccaacagagctttaatcccaaagatccagtggccaccagagtacagaagtcagaatcaaatgctcagaatcaaaaggtgtggcactcctgcccagccggcttatcagcagttgtatagacagatcagaaaaaactagcatttattataaaaactgtttttcaaatggggtgatttcctgtccttctccagagatcataattcttcacgtttctgaggaccttctcggcttggttcttttgtcttctctttgtacagtgctcccgtttctttctccttctgaaagcggatctgtagctgtttgatctcttggtcgtagtcctgccactccgggacaatccgcacagctgcttccagtttcggctctttggtcatcggattattacacaaatcaatggtttttgcccttttcttagaggcgtcatcacaccacgtttcacaccaaagccattcttgagggagggatttaattggcacctgatgaatcatgttattgggcagatcttgatcaagatttgaaaggctgttagggtcctgactcagaccttggtactgtcccctgagtctgtcaccagcagctattttcctaaacttcttcagatccacaacatatagtgcactgatatgatactttcgcccggctaaatgactggcccagtaccctgacttccagaacctgtagccgtccatttctcttcggctgtcacagaaaggagtgtaaccataaggagcaccatccaaattgaaatctcttaactctttcagatctgttcgtacaatctgatcagcatccacaaacaggaacttgtcaacaactagtgggaaaagtacatccaggaagaggatcttgtaaccccagatgatacgctgtttttcagtttgttgatgaagccaccggggccatttgtactgaacaagctcatactggaaattgtattcatttgccatgtaaggtataaactccttaaatgtgggggacaagtaattcttcaagaaccagaatttcacaggagtcttggtattcttcagcacggatagcatcattatgcgaagaaatctttcgtagagatgaccagatgcaacggagaaaatattaattatgtcatctttatcttgcttcacttcctcagtcttctgtcctgtaaagccccatttgaaggaatcccaaaatccagattcattctcactcgttccatcactcagcaagtcttcgttcaccatatctgccttcttctgaaccttcactttaataattttgcttttgaagttgttgaggacgataaccacctcatcagcatcagggggagaatcagtgccatcgtggctgtaaattctataaatatcttcagagcgtcccttcctaagtctgaggatccaagctcctgggttggctttcagctgaaagtagcccagattggccataacaatggtgtccacaatgaccgggttggctgaagttcctaaggtaaactgtagtccccgtggaggctggcctgtggtgatgtcgtagcaatgaccttccagtaacaggtattccagctcatactcagcagccactacactgtccacctcttctaaataaatattatcaagatcatatggtgttctgacagattctaccatccagctctcaggtgtgttcaaattcagagtgaacagtggagactgaggcatatccaaaaattttgcgattggacccttagcaaaactattgtctgaagtgaaagaaatctctggttctaagacataacggtaaaagctttttaaaggcatgtcagaaagtttggattggcagttcataaatactctcagattcatgtttatcagctgagccaaaaccaagagcaaaggagcaagtctctgtgcttctctggtgacagggtcaacgacagccacaacatcaaagtatgtctccccttccttcggcctcagtttgattgcactgtgtctgtcttcaaaaaactggtactcgattcttggatctccttttggttgcgctgacagaagagcatccaccttcattaccaagtcgcttgccacatcttcttctacccgaagctgttgaatatgagattttattttctgtcctgaggtttttaagatgatattttcgaggaggtggaaatcgtcttgattaaagagctcactatcctccagtggcccaatgatccttccattgctgatcactgccctctgtcccttcttcagcttcagaacatccctgcagtacacggcatgagacaaaatgaaatccattttggaagactcaaagacctctttaaaaagactgaaatccattcccccaacagagaactccgcaatgtcagctcctgcagccagggcctctgcagccccctccttggccattttggtgatgaagttcttagcagcgttggaagtctgagtttggagagctgcccagattgctctggagatctgagtgttctcatagcttatctctttggcaggattattgatcatgcttattctaacattgttactggatttctgatgtttgatggcatcatacagtaactgccgtccagaagggctatcaaaatccccaacaatccaaaaagttactggcctaataaaagaatcatcatagatttccttggaggacattcctttctttgtcagatagttcatactattggctacagcagcagtcttgccttgggaatccaagatagtaaatctagcataatcatccacaaagaagttattactcgctgttaaatccaggtagtctcgttcagctgtcaaaatcctagaattgattcgtggaacaacatttggctgattcatgatatactctaccacatcttgatcatggggcagttcacccaagtacaccgctctttggaagaaggtggtggtctccaggattttatgcattgtgatggtttctaactcatcagggtctagctgttccctttcaaagggcattccattgaacagcacaacgggcagaggtccaactccagtctgctcatagtagcctcttgcttccttccgattccgatcataagcagaatcaatccccaaaatgctattcacttctacatacggatatttcttctccaggacactgaccacatgttcaactttcactttttctccagtcctcaccttgttatagatatgtgtcagagtctggaaggcatgataatcatccacttcttgggcaacataattatatgctctaagaacagccactccagcatcttgcatcccatcaacatcttcagagtcattaaccacaaagataaaaccaattctaggaaaattcccttccattgggaagcaagctgcagccagaaactatttttacatgggctattta

SEQ ID NO: 11997 - RNA, 8189 nt, Homo sapiens
  source 1..8189: mol_type = other RNA
ctgaatagctgggactacaggtgtgtgccaccatgcccagctaatttttgtatttttagtagagacggggtttcaccgtgttggccaggatggtctctatctcttgacctcataatccgcccgcctcggcttcccaaagtgctgggattacaggtgtaagccactgtgcctgaccggaaactgtttcttaacatacatcatgcacgtaatcttcgctctcccaagaggcattcacccaagcagacaggcaagcatctatgtgttcaattcgaaatgcaacaatgacagatgtacaactttaccactcttaaagaaactaacatgccatccattattctccatgtgggaaacattcagtaaacttctaaaaccaaacacaggactctggcatatccccacacccccagcagcaggctgtgacaggctttgatctcaatcaaatgccactgtacacagaacataaaaacaggctcaggatgctgcatgtcactctgacatatcacattatttcatattactctgtcacttactcacaaacaaaagtctccactatggcatgattgagagagaaaataattcactttatataaataacagctaagaacaacatactgtgaacagtttccagagtttgaacattcagcacaatcaattcttacttcttgggaaaaaaatatcttacctatcttttctgttacagtatgccttcttggagaaaatattttagtggtaacatcattttctggggcatttggttaattttgaaagatgattatgccacatgaaccaaaaaaaaaaaaaaaaactggcaggaggaggagggtcctaggccattctggaagcaagctgggttttgcattattcagagtcaactattaagctgacttatattagaatggcgacagataagaggcaatgagtgacaccaggacatgcacagcacacagagaatatggtctactcttgtcttccctgcacagattaaacataagaggcttggtagaaagacatggggaaaggtgctatgggggccagcatttggaaagcatatatcccagtgacttgagtatttgctatgcaacctcctggacgagaaactgggaaaaggcacacttccgcccacagttgtggacagcagcagtcacccgtctgaatgctttcattcaatgtgaagatgcagcttgaacaaaagtttctttttgtttgtttgttttctgagatggagtctcgctctgtcacccaggctggagtgcagtggcacgatctcagctcactgcaacctctgcctcctgggttcaggcgattctcctgtctctgcctcccgagtagctgggaatagagggtgagccacaacacccggctaatttttgtatttttagtagagacggggtttcaccatattggccaggctggtcttgaactcctgacctcatgatccgtccgcctcagcctcccaaagtgctgggattacaggtgtgagccaccacgcctggccgaacaaaagttttttaatcttactgatcccatctttccagctgctctgaacagaggggcagggcggggaaagtcatgtcacagactctgcccacagcagccattctgaggtgccttttcagtctcttatcctcttttgagctttcctcttcttaattttttgttttgttttgttttcattgtactcattaatcccctcctcaatttttaacagaattataaaagcaaagtcaaaaggtccttcaggatgactgggaggcttcctaggctaacttttgcatttgaaaatggaaaaaataaattacttgatatttgtgataagactaagatttcttaaaagtctgcacatcaatatattacctggcttaggagggtgagggcacagtatccatctgcaccctctcctcgtattttttaaaaacaggcaaaatatgtaagaaaaggctggtgcacgttggaagacagagcgtgcctgtctatgccagtgctgctgtgccctgcagcctggcagatggagtcggatgctggggcctcatgcccacttaggccaataacatactcaagactctacagcccgttcaccagcaaagtatgccctgaggggcaacactggctgtggaagtgaagacacacaaagcagggactaaaggcaaatggggcttcacgatgcagcgacatgaagacagaactggtgtgggcgccaaaggcaacctgcagggctcacataaaaggaaaataggacagaaagccacgagttccacaagcagaatcatttctggtcttacatctgagggcatttgtagagaaaagtccaaggcaatgtcccctgggtctgagagaaaaatcctacgcaaaagagggcagacaatgcggtgctcgtcttgagggagcctgaccctgaccctgaccctgacgggctggatgcgagaggggctgagtatggctgtattcagtaaggaaactggtagcagacttttctagaaggtggaaagaaaaagcaaagactttcacagatacaaaaattgttttcaaaacaattacctagaaagttcactgcggttgggtggggaataagtgtaatattttcatttcaaatgagccatggtgctactaatggattataaaagaggatggccagttctggtcttccttcccttcccttaacccccgaaccttcctactcctgacattttccctaccctcactgcaacccacccccatcctggcccaaaattaatttgcccagccactgcaccaaaccagccttgacacacaattgttggttggatttcaattaaacaatgcacctaatgcgttggaagagaaggtggggagggcacaaggatgttggcgtaaacctggaggtgtgtggaccttggacagagcttccgccggccagacccagggcagggtgggcatctgcagtgcagcgcaggccgcaggtaaactgaggtaaggaagaacatggtggctctagctggccctgctttccgagacagtgcagcatgtgtgtgctcttgggtgtgggcaccaaaaaactcattttcttccagttgctgctgccattccaccctctgactagaagaatgctctttacagagtccaaaggatcagccacttggtcttcctctgaggtacaaatccaacagagctttaatcccaaagatccagtggccaccagagtacagaagtcagaatcaaatgctcagaatcaaaaggtgtggcactcctgcccagccggcttatcagcagttgtatagacagatcagaaaaaactagcatttattataaaaactgtttttcaaatggggtgatttcctgtccttctccagagatcataattcttcacgtttctgaggaccttctcggcttggttcttttgtcttctctttgtacagtgctcccgtttctttctccttctgaaagcggatctgtagctgtttgatctcttggtcgtagtcctgccactccgggacaatccgcacagctgcttccagtttcggctctttggtcatcggattattacacaaatcaatggtttttgcccttttcttagaggcgtcatcacaccacgtttcacaccaaagccattcttgagggagggatttaattggcacctgatgaatcatgttattgggcagatcttgatcaagatttgaaaggctgttagggtcctgactcagaccttggtactgtcccctgagtctgtcaccagcagctattttcctaaacttcttcagatccacaacatatagtgcactgatatgatactttcgcccggctaaatgactggcccagtaccctgacttccagaacctgtagccgtccatttctcttcggctgtcacagaaaggagtgtaaccataaggagcaccatccaaattgaaatctcttaactctttcagatctgttcgtacaatctgatcagcatccacaaacaggaacttgtcaacaactagtgggaaaagtacatccaggaagaggatcttgtaaccccagatgatacgctgtttttcagtttgttgatgaagccaccggggccatttgtactgaacaagctcatactggaaattgtattcatttgccatgtaaggtataaactccttaaatgtgggggacaagtaattcttcaagaaccagaatttcacaggagtcttggtattcttcagcacggatagcatcattatgcgaagaaatctttcgtagagatgaccagatgcaacggagaaaatattaattatgtcatctttatcttgcttcacttcctcagtcttctgtcctgtaaagccccatttgaaggaatcccaaaatccagattcattctcactcgttccatcactcagcaagtcttcgttcaccatatctgccttcttctgaaccttcactttaataattttgcttttgaagttgttgaggacgataaccacctcatcagcatcagggggagaatcagtgccatcgtggctgtaaattctataaatatcttcagagcgtcccttcctaagtctgaggatccaagctcctgggttggctttcagctgaaagtagcccagattggccataacaatggtgtccacaatgaccgggttggctgaagttcctaaggtaaactgtagtccccgtggaggctggcctgtggtgatgtcgtagcaatgaccttccagtaacaggtattccagctcatactcagcagccactacactgtccacctcttctaaataaatattatcaagatcatatggtgttctgacagattctaccatccagctctcaggtgtgttcaaattcagagtgaacagtggagactgaggcatatccaaaaattttgcgattggacccttagcaaaactattgtctgaagtgaaagaaatctctggttctaagacataacggtaaaagctttttaaaggcatgtcagaaagtttggattggcagttcataaatactctcagattcatgtttatcagctgagccaaaaccaagagcaaaggagcaagtctctgtgcttctctggtgacagggtcaacgacagccacaacatcaaagtatgtctccccttccttcggcctcagtttgattgcactgtgtctgtcttcaaaaaactggtactcgattcttggatctccttttggttgcgctgacagaagagcatccaccttcattaccaagtcgcttgccacatcttcttctacccgaagctgttgaatatgagattttattttctgtcctgaggtttttaagatgatattttcgaggaggtggaaatcgtcttgattaaagagctcactatcctccagtggcccaatgatccttccattgctgatcactgccctctgtcccttcttcagcttcagaacatccctgcagtacacggcatgagacaaaatgaaatccattttggaagactcaaagacctctttaaaaagactgaaatccattcccccaacagagaactccgcaatgtcagctcctgcagccagggcctctgcagccccctccttggccattttggtgatgaagttcttagcagcgttggaagtctgagtttggagagctgcccagattgctctggagatctgagtgttctcatagcttatctctttggcaggattattgatcatgcttattctaacattgttactggatttctgatgtttgatggcatcatacagtaactgccgtccagaagggctatcaaaatccccaacaatccaaaaagttactggcctaataaaagaatcatcatagatttccttggaggacattcctttctttgtcagatagttcatactattggctacagcagcagtcttgccttgggaatccaagatagtaaatctagcataatcatccacaaagaagttattactcgctgttaaatccaggtagtctcgttcagctgtcaaaatcctagaattgattcgtggaacaacatttggctgattcatgatatactctaccacatcttgatcatggggcagttcacccaagtacaccgctctttggaagaaggtggtggtctccaggattttatgcattgtgatggtttctaactcatcagggtctagctgttccctttcaaagggcattccattgaacagcacaacgggcagaggtccaactccagtctgctcatagtagcctcttgcttccttccgattccgatcataagcagaatcaatccccaaaatgctattcacttctacatacggatatttcttctccaggacactgaccacatgttcaactttcactttttctccagtcctcaccttgttatagatatgtgtcagagtctggaaggcatgataatcatccacttcttgggcaacataattatatgctctaagaacagccactccagcatcttgcatcccatcaacatcttcagagtcattaaccacaaagataaaaccaattcttagtggtatatgattactaaggaacatctcagctgtgttcatcaactctgctgtggtctcatgtgcaggatcaactatgaaaaccatattatgtaagtttttcctgatctgccgaataacaccaggaaaggtgggtcgaagcaactcttgtaaactagaaggccacgaattatatctgctatcaacctccaggttgttgacccatgaaatagcaggactccggatgtctacggcatagtctgcctcagagggctggatgttcagcttcaaaacattatgcagagaaaggccttctattcccaatctatgcagaccctccattacccgagcttcattcctcaacacatcaaacagactgaatatatcctgtgtatctaaatccatgtgaagtccattgatgaagagggctgaatctccaggttgtaatcctaaagttcccttgaaatacttctgattctcttccacttcggttctaagttctgagctcacagctgtttttgttattgctctggctttggtaggaaaattctgactaagatccttcatgacaaccaaagccaactcaacaggagaagccaagattcgagcagcagtctggaaactgagatcttgcaactgccaaacctttaaaggtgccatttcattggtgctctctacaagatgctttctgagttctttcaactgtccctccaggtcggggtgcagatctcttaattttccaaagaggaacccctgaacctcatcaataggatcattttcaccaatcactgtggtgtttacctcagttcctttcacctgagtatcatccttggccttgtactcagtgctcttaatggccaattccacgccatagccagagaggtaaacaggctccttcctgggattaaatatataatgtctgaatacataattgattttgcctgcattgctttttgatataagctggcggtgaaaattggaaaattcctcagagccaatctcagagtagaaaatcaccacagggctttcaggattagacgagggatatctgtgatctcctttgaacaataaaggtttgggtctttcagaggctgtcagtagaagagcctcaagggtatcagattcacaagtcttctttccatgcactgaaaaaaacgaattacatccttctggtggaggttcatcagctgctatctgctggaaggcttggattgtagctgagtaagaacgaagggacagacaaaatttaaacaaattctgctggaggggtgacagaaactgaaatgcagcctccaatattgcatgatagtaggaataatcggtaccgtcatgatctgatgatccaatattttgactggcttctacaaaattccaaaatttctcttgactgtcttctgctaaaaactcactagccaaaggaagactttcccattacttgtgaacactggggtgtacaatctcactctactccacagctggcttctaacaacaatggagtggaaaaccattttgttgtaagagaggttgtaatggcttttgagtcggcctttactgaggagaacagccacagaacagtgagtacaaccagaactcccattttatagcaaactccgctcgcgtctcccttgcagcccatgcccgggccgtggtcagtccgccacagtgccagagacaacgccagggcagggcggggcgaggcggcagcggcagtgcaggctgcgccagtgagaggccgacacgcgcctttcccgcggctcgactcaacacccagcctcgcaaagcaattgcccagct

SEQ ID NO: 11998 - RNA, 8234 nt, Homo sapiens
  source 1..8234: mol_type = other RNA
ctgaatagctgggactacaggtgtgtgccaccatgcccagctaatttttgtatttttagtagagacggggtttcaccgtgttggccaggatggtctctatctcttgacctcataatccgcccgcctcggcttcccaaagtgctgggattacaggtgtaagccactgtgcctgaccggaaactgtttcttaacatacatcatgcacgtaatcttcgctctcccaagaggcattcacccaagcagacaggcaagcatctatgtgttcaattcgaaatgcaacaatgacagatgtacaactttaccactcttaaagaaactaacatgccatccattattctccatgtgggaaacattcagtaaacttctaaaaccaaacacaggactctggcatatccccacacccccagcagcaggctgtgacaggctttgatctcaatcaaatgccactgtacacagaacataaaaacaggctcaggatgctgcatgtcactctgacatatcacattatttcatattactctgtcacttactcacaaacaaaagtctccactatggcatgattgagagagaaaataattcactttatataaataacagctaagaacaacatactgtgaacagtttccagagtttgaacattcagcacaatcaattcttacttcttgggaaaaaaatatcttacctatcttttctgttacagtatgccttcttggagaaaatattttagtggtaacatcattttctggggcatttggttaattttgaaagatgattatgccacatgaaccaaaaaaaaaaaaaaaaactggcaggaggaggagggtcctaggccattctggaagcaagctgggttttgcattattcagagtcaactattaagctgacttatattagaatggcgacagataagaggcaatgagtgacaccaggacatgcacagcacacagagaatatggtctactcttgtcttccctgcacagattaaacataagaggcttggtagaaagacatggggaaaggtgctatgggggccagcatttggaaagcatatatcccagtgacttgagtatttgctatgcaacctcctggacgagaaactgggaaaaggcacacttccgcccacagttgtggacagcagcagtcacccgtctgaatgctttcattcaatgtgaagatgcagcttgaacaaaagtttctttttgtttgtttgttttctgagatggagtctcgctctgtcacccaggctggagtgcagtggcacgatctcagctcactgcaacctctgcctcctgggttcaggcgattctcctgtctctgcctcccgagtagctgggaatagagggtgagccacaacacccggctaatttttgtatttttagtagagacggggtttcaccatattggccaggctggtcttgaactcctgacctcatgatccgtccgcctcagcctcccaaagtgctgggattacaggtgtgagccaccacgcctggccgaacaaaagttttttaatcttactgatcccatctttccagctgctctgaacagaggggcagggcggggaaagtcatgtcacagactctgcccacagcagccattctgaggtgccttttcagtctcttatcctcttttgagctttcctcttcttaattttttgttttgttttgttttcattgtactcattaatcccctcctcaatttttaacagaattataaaagcaaagtcaaaaggtccttcaggatgactgggaggcttcctaggctaacttttgcatttgaaaatggaaaaaataaattacttgatatttgtgataagactaagatttcttaaaagtctgcacatcaatatattacctggcttaggagggtgagggcacagtatccatctgcaccctctcctcgtattttttaaaaacaggcaaaatatgtaagaaaaggctggtgcacgttggaagacagagcgtgcctgtctatgccagtgctgctgtgccctgcagcctggcagatggagtcggatgctggggcctcatgcccacttaggccaataacatactcaagactctacagcccgttcaccagcaaagtatgccctgaggggcaacactggctgtggaagtgaagacacacaaagcagggactaaaggcaaatggggcttcacgatgcagcgacatgaagacagaactggtgtgggcgccaaaggcaacctgcagggctcacataaaaggaaaataggacagaaagccacgagttccacaagcagaatcatttctggtcttacatctgagggcatttgtagagaaaagtccaaggcaatgtcccctgggtctgagagaaaaatcctacgcaaaagagggcagacaatgcggtgctcgtcttgagggagcctgaccctgaccctgaccctgacgggctggatgcgagaggggctgagtatggctgtattcagtaaggaaactggtagcagacttttctagaaggtggaaagaaaaagcaaagactttcacagatacaaaaattgttttcaaaacaattacctagaaagttcactgcggttgggtggggaataagtgtaatattttcatttcaaatgagccatggtgctactaatggattataaaagaggatggccagttctggtcttccttcccttcccttaacccccgaaccttcctactcctgacattttccctaccctcactgcaacccacccccatcctggcccaaaattaatttgcccagccactgcaccaaaccagccttgacacacaattgttggttggatttcaattaaacaatgcacctaatgcgttggaagagaaggtggggagggcacaaggatgttggcgtaaacctggaggtgtgtggaccttggacagagcttccgccggccagacccagggcagggtgggcatctgcagtgcagcgcaggccgcaggtaaactgaggtaaggaagaacatggtggctctagctggccctgctttccgagacagtgcagcatgtgtgtgctcttgggtgtgggcaccaaaaaactcattttcttccagttgctgctgccattccaccctctgactagaagaatgctctttacagagtccaaaggatcagccacttggtcttcctctgaggtacaaatccaacagagctttaatcccaaagatccagtggccaccagagtacagaagtcagaatcaaatgctcagaatcaaaaggtgtggcactcctgcccagccggcttatcagcagttgtatagacagatcagaaaaaactagcatttattataaaaactgtttttcaaatggggtgatttcctgtccttctccagagatcataattcttcacgtttctgaggaccttctcggcttggttcttttgtcttctctttgtacagtgctcccgtttctttctccttctgaaagcggatctgtagctgtttgatctcttggtcgtagtcctgccactccgggacaatccgcacagctgcttccagtttcggctctttggtcatcggattattacacaaatcaatggtttttgcccttttcttagaggcgtcatcacaccacgtttcacaccaaagccattcttgagggagggatttaattggcacctgatgaatcatgttattgggcagatcttgatcaagatttgaaaggctgttagggtcctgactcagaccttggtactgtcccctgagtctgtcaccagcagctattttcctaaacttcttcagatccacaacatatagtgcactgatatgatactttcgcccggctaaatgactggcccagtaccctgacttccagaacctgtagccgtccatttctcttcggctgtcacagaaaggagtgtaaccataaggagcaccatccaaattgaaatctcttaactctttcagatctgttcgtacaatctgatcagcatccacaaacaggaacttgtcaacaactagtgggaaaagtacatccaggaagaggatcttgtaaccccagatgatacgctgtttttcagtttgttgatgaagccaccggggccatttgtactgaacaagctcatactggaaattgtattcatttgccatgtaaggtataaactccttaaatgtgggggacaagtaattcttcaagaaccagaatttcacaggagtcttggtattcttcagcacggatagcatcattatgcgaagaaatctttcgtagagatgaccagatgcaacggagaaaatattaattatgtcatctttatcttgcttcacttcctcagtcttctgtcctgtaaagccccatttgaaggaatcccaaaatccagattcattctcactcgttccatcactcagcaagtcttcgttcaccatatctgccttcttctgaaccttcactttaataattttgcttttgaagttgttgaggacgataaccacctcatcagcatcagggggagaatcagtgccatcgtggctgtaaattctataaatatcttcagagcgtcccttcctaagtctgaggatccaagctcctgggttggctttcagctgaaagtagcccagattggccataacaatggtgtccacaatgaccgggttggctgaagttcctaaggtaaactgtagtccccgtggaggctggcctgtggtgatgtcgtagcaatgaccttccagtaacaggtattccagctcatactcagcagccactacactgtccacctcttctaaataaatattatcaagatcatatggtgttctgacagattctaccatccagctctcaggtgtgttcaaattcagagtgaacagtggagactgaggcatatccaaaaattttgcgattggacccttagcaaaactattgtctgaagtgaaagaaatctctggttctaagacataacggtaaaagctttttaaaggcatgtcagaaagtttggattggcagttcataaatactctcagattcatgtttatcagctgagccaaaaccaagagcaaaggagcaagtctctgtgcttctctggtgacagggtcaacgacagccacaacatcaaagtatgtctccccttccttcggcctcagtttgattgcactgtgtctgtcttcaaaaaactggtactcgattcttggatctccttttggttgcgctgacagaagagcatccaccttcattaccaagtcgcttgccacatcttcttctacccgaagctgttgaatatgagattttattttctgtcctgaggtttttaagatgatattttcgaggaggtggaaatcgtcttgattaaagagctcactatcctccagtggcccaatgatccttccattgctgatcactgccctctgtcccttcttcagcttcagaacatccctgcagtacacggcatgagacaaaatgaaatccattttggaagactcaaagacctctttaaaaagactgaaatccattcccccaacagagaactccgcaatgtcagctcctgcagccagggcctctgcagccccctccttggccattttggtgatgaagttcttagcagcgttggaagtctgagtttggagagctgcccagattgctctggagatctgagtgttctcatagcttatctctttggcaggattattgatcatgcttattctaacattgttactggatttctgatgtttgatggcatcatacagtaactgccgtccagaagggctatcaaaatccccaacaatccaaaaagttactggcctaataaaagaatcatcatagatttccttggaggacattcctttctttgtcagatagttcatactattggctacagcagcagtcttgccttgggaatccaagatagtaaatctagcataatcatccacaaagaagttattactcgctgttaaatccaggtagtctcgttcagctgtcaaaatcctagaattgattcgtggaacaacatttggctgattcatgatatactctaccacatcttgatcatggggcagttcacccaagtacaccgctctttggaagaaggtggtggtctccaggattttatgcattgtgatggtttctaactcatcagggtctagctgttccctttcaaagggcattccattgaacagcacaacgggcagaggtccaactccagtctgctcatagtagcctcttgcttccttccgattccgatcataagcagaatcaatccccaaaatgctattcacttctacatacggatatttcttctccaggacactgaccacatgttcaactttcactttttctccagtcctcaccttgttatagatatgtgtcagagtctggaaggcatgataatcatccacttcttgggcaacataattatatgctctaagaacagccactccagcatcttgcatcccatcaacatcttcagagtcattaaccacaaagataaaaccaattcttagtggtatatgattactaaggaacatctcagctgtgttcatcaactctgctgtggtctcatgtgcaggatcaactatgaaaaccatattatgtaagtttttcctgatctgccgaataacaccaggaaaggtgggtcgaagcaactcttgtaaactagaaggccacgaattatatctgctatcaacctccaggttgttgacccatgaaatagcaggactccggatgtctacggcatagtctgcctcagagggctggatgttcagcttcaaaacattatgcagagaaaggccttctattcccaatctatgcagaccctccattacccgagcttcattcctcaacacatcaaacagactgaatatatcctgtgtatctaaatccatgtgaagtccattgatgaagagggctgaatctccaggttgtaatcctaaagttcccttgaaatacttctgattctcttccacttcggttctaagttctgagctcacagctgtttttgttattgctctggctttggtaggaaaattctgactaagatccttcatgacaaccaaagccaactcaacaggagaagccaagattcgagcagcagtctggaaactgagatcttgcaactgccaaacctttaaaggtgccatttcattggtgctctctacaagatgctttctgagttctttcaactgtccctccaggtcggggtgcagatctcttaattttccaaagaggaacccctgaacctcatcaataggatcattttcaccaatcactgtggtgtttacctcagttcctttcacctgagtatcatccttggccttgtactcagtgctcttaatggccaattccacgccatagccagagaggtaaacaggctccttcctgggattaaatatataatgtctgaatacataattgattttgcctgcattgctttttgatataagctggcggtgaaaattggaaaattcctcagagccaatctcagagtagaaaatcaccacagggctttcaggattagacgagggatatctgtgatctcctttgaacaataaaggtttgggtctttcagaggctgtcagtagaagagcctcaagggtatcagattcacaagtcttctttccatgcactgaaaaaaacgaattacatccttctggtggaggttcatcagctgctatctgctggaaggcttggattgtagctgagtaagaacgaagggacagacaaaatttaaacaaattctgctggaggggtgacagaaactgaaatgcagcctccaatattgcatgatagtaggaataatcggtaccgtcatgatctgatgatccaatattttgactggcttctacaaaattccaaaatttctcttgactgtcttctgctaaaaactcactagccaaaggaagactttcccattacttgtgaacactggggtgtacaatctcactctactccacagctggcttctaacaacaatggagtggaaaaccattttgttgtaagagaggttgtaatggcttttgagtcggcctttactgaggagaacagccacagaacagtgagtacaaccagaactcccattttatagcaaactcctgtcaccggcagcgcacccgcggcacacgcaccgctcgcgtctcccttgcagcccatgcccgggccgtggtcagtccgccacagtgccagagacaacgccagggcagggcggggcgaggcggcagcggcagtgcaggctgcgccagtgagaggccgacacgcgcctttcccgcggctcgactcaacacccagcctcgcaaagcaattgcccagctgccggccgccct

SEQ ID NO: 11999 - RNA, 8149 nt, Homo sapiens
  source 1..8149: mol_type = other RNA
ctgaatagctgggactacaggtgtgtgccaccatgcccagctaatttttgtatttttagtagagacggggtttcaccgtgttggccaggatggtctctatctcttgacctcataatccgcccgcctcggcttcccaaagtgctgggattacaggtgtaagccactgtgcctgaccggaaactgtttcttaacatacatcatgcacgtaatcttcgctctcccaagaggcattcacccaagcagacaggcaagcatctatgtgttcaattcgaaatgcaacaatgacagatgtacaactttaccactcttaaagaaactaacatgccatccattattctccatgtgggaaacattcagtaaacttctaaaaccaaacacaggactctggcatatccccacacccccagcagcaggctgtgacaggctttgatctcaatcaaatgccactgtacacagaacataaaaacaggctcaggatgctgcatgtcactctgacatatcacattatttcatattactctgtcacttactcacaaacaaaagtctccactatggcatgattgagagagaaaataattcactttatataaataacagctaagaacaacatactgtgaacagtttccagagtttgaacattcagcacaatcaattcttacttcttgggaaaaaaatatcttacctatcttttctgttacagtatgccttcttggagaaaatattttagtggtaacatcattttctggggcatttggttaattttgaaagatgattatgccacatgaaccaaaaaaaaaaaaaaaaactggcaggaggaggagggtcctaggccattctggaagcaagctgggttttgcattattcagagtcaactattaagctgacttatattagaatggcgacagataagaggcaatgagtgacaccaggacatgcacagcacacagagaatatggtctactcttgtcttccctgcacagattaaacataagaggcttggtagaaagacatggggaaaggtgctatgggggccagcatttggaaagcatatatcccagtgacttgagtatttgctatgcaacctcctggacgagaaactgggaaaaggcacacttccgcccacagttgtggacagcagcagtcacccgtctgaatgctttcattcaatgtgaagatgcagcttgaacaaaagtttctttttgtttgtttgttttctgagatggagtctcgctctgtcacccaggctggagtgcagtggcacgatctcagctcactgcaacctctgcctcctgggttcaggcgattctcctgtctctgcctcccgagtagctgggaatagagggtgagccacaacacccggctaatttttgtatttttagtagagacggggtttcaccatattggccaggctggtcttgaactcctgacctcatgatccgtccgcctcagcctcccaaagtgctgggattacaggtgtgagccaccacgcctggccgaacaaaagttttttaatcttactgatcccatctttccagctgctctgaacagaggggcagggcggggaaagtcatgtcacagactctgcccacagcagccattctgaggtgccttttcagtctcttatcctcttttgagctttcctcttcttaattttttgttttgttttgttttcattgtactcattaatcccctcctcaatttttaacagaattataaaagcaaagtcaaaaggtccttcaggatgactgggaggcttcctaggctaacttttgcatttgaaaatggaaaaaataaattacttgatatttgtgataagactaagatttcttaaaagtctgcacatcaatatattacctggcttaggagggtgagggcacagtatccatctgcaccctctcctcgtattttttaaaaacaggcaaaatatgtaagaaaaggctggtgcacgttggaagacagagcgtgcctgtctatgccagtgctgctgtgccctgcagcctggcagatggagtcggatgctggggcctcatgcccacttaggccaataacatactcaagactctacagcccgttcaccagcaaagtatgccctgaggggcaacactggctgtggaagtgaagacacacaaagcagggactaaaggcaaatggggcttcacgatgcagcgacatgaagacagaactggtgtgggcgccaaaggcaacctgcagggctcacataaaaggaaaataggacagaaagccacgagttccacaagcagaatcatttctggtcttacatctgagggcatttgtagagaaaagtccaaggcaatgtcccctgggtctgagagaaaaatcctacgcaaaagagggcagacaatgcggtgctcgtcttgagggagcctgaccctgaccctgaccctgacgggctggatgcgagaggggctgagtatggctgtattcagtaaggaaactggtagcagacttttctagaaggtggaaagaaaaagcaaagactttcacagatacaaaaattgttttcaaaacaattacctagaaagttcactgcggttgggtggggaataagtgtaatattttcatttcaaatgagccatggtgctactaatggattataaaagaggatggccagttctggtcttccttcccttcccttaacccccgaaccttcctactcctgacattttccctaccctcactgcaacccacccccatcctggcccaaaattaatttgcccagccactgcaccaaaccagccttgacacacaattgttggttggatttcaattaaacaatgcacctaatgcgttggaagagaaggtggggagggcacaaggatgttggcgtaaacctggaggtgtgtggaccttggacagagcttccgccggccagacccagggcagggtgggcatctgcagtgcagcgcaggccgcaggtaaactgaggtaaggaagaacatggtggctctagctggccctgctttccgagacagtgcagcatgtgtgtgctcttgggtgtgggcaccaaaaaactcattttcttccagttgctgctgccattccaccctctgactagaagaatgctctttacagagtccaaaggatcagccacttggtcttcctctgaggtacaaatccaacagagctttaatcccaaagatccagtggccaccagagtacagaagtcagaatcaaatgctcagaatcaaaaggtgtggcactcctgcccagccggcttatcagcagttgtatagacagatcagaaaaaactagcatttattataaaaactgtttttcaaatggggtgatttcctgtccttctccagagatcataattcttcacgtttctgaggaccttctcggcttggttcttttgtcttctctttgtacagtgctcccgtttctttctccttctgaaagcggatctgtagctgtttgatctcttggtcgtagtcctgccactccgggacaatccgcacagctgcttccagtttcggctctttggtcatcggattattacacaaatcaatggtttttgcccttttcttagaggcgtcatcacaccacgtttcacaccaaagccattcttgagggagggatttaattggcacctgatgaatcatgttattgggcagatcttgatcaagatttgaaaggctgttagggtcctgactcagaccttggtactgtcccctgagtctgtcaccagcagctattttcctaaacttcttcagatccacaacatatagtgcactgatatgatactttcgcccggctaaatgactggcccagtaccctgacttccagaacctgtagccgtccatttctcttcggctgtcacagaaaggagtgtaaccataaggagcaccatccaaattgaaatctcttaactctttcagatctgttcgtacaatctgatcagcatccacaaacaggaacttgtcaacaactagtgggaaaagtacatccaggaagaggatcttgtaaccccagatgatacgctgtttttcagtttgttgatgaagccaccggggccatttgtactgaacaagctcatactggaaattgtattcatttgccatgtaaggtataaactccttaaatgtgggggacaagtaattcttcaagaaccagaatttcacaggagtcttggtattcttcagcacggatagcatcattatgcgaagaaatctttcgtagagatgaccagatgcaacggagaaaatattaattatgtcatctttatcttgcttcacttcctcagtcttctgtcctgtaaagccccatttgaaggaatcccaaaatccagattcattctcactcgttccatcactcagcaagtcttcgttcaccatatctgccttcttctgaaccttcactttaataattttgcttttgaagttgttgaggacgataaccacctcatcagcatcagggggagaatcagtgccatcgtggctgtaaattctataaatatcttcagagcgtcccttcctaagtctgaggatccaagctcctgggttggctttcagctgaaagtagcccagattggccataacaatggtgtccacaatgaccgggttggctgaagttcctaaggtaaactgtagtccccgtggaggctggcctgtggtgatgtcgtagcaatgaccttccagtaacaggtattccagctcatactcagcagccactacactgtccacctcttctaaataaatattatcaagatcatatggtgttctgacagattctaccatccagctctcaggtgtgttcaaattcagagtgaacagtggagactgaggcatatccaaaaattttgcgattggacccttagcaaaactattgtctgaagtgaaagaaatctctggttctaagacataacggtaaaagctttttaaaggcatgtcagaaagtttggattggcagttcataaatactctcagattcatgtttatcagctgagccaaaaccaagagcaaaggagcaagtctctgtgcttctctggtgacagggtcaacgacagccacaacatcaaagtatgtctccccttccttcggcctcagtttgattgcactgtgtctgtcttcaaaaaactggtactcgattcttggatctccttttggttgcgctgacagaagagcatccaccttcattaccaagtcgcttgccacatcttcttctacccgaagctgttgaatatgagattttattttctgtcctgaggtttttaagatgatattttcgaggaggtggaaatcgtcttgattaaagagctcactatcctccagtggcccaatgatccttccattgctgatcactgccctctgtcccttcttcagcttcagaacatccctgcagtacacggcatgagacaaaatgaaatccattttggaagactcaaagacctctttaaaaagactgaaatccattcccccaacagagaactccgcaatgtcagctcctgcagccagggcctctgcagccccctccttggccattttggtgatgaagttcttagcagcgttggaagtctgagtttggagagctgcccagattgctctggagatctgagtgttctcatagcttatctctttggcaggattattgatcatgcttattctaacattgttactggatttctgatgtttgatggcatcatacagtaactgccgtccagaagggctatcaaaatccccaacaatccaaaaagttactggcctaataaaagaatcatcatagatttccttggaggacattcctttctttgtcagatagttcatactattggctacagcagcagtcttgccttgggaatccaagatagtaaatctagcataatcatccacaaagaagttattactcgctgttaaatccaggtagtctcgttcagctgtcaaaatcctagaattgattcgtggaacaacatttggctgattcatgatatactctaccacatcttgatcatggggcagttcacccaagtacaccgctctttggaagaaggtggtggtctccaggattttatgcattgtgatggtttctaactcatcagggtctagctgttccctttcaaagggcattccattgaacagcacaacgggcagaggtccaactccagtctgctcatagtagcctcttgcttccttccgattccgatcataagcagaatcaatccccaaaatgctattcacttctacatacggatatttcttctccaggacactgaccacatgttcaactttcactttttctccagtcctcaccttgttatagatatgtgtcagagtctggaaggcatgataatcatccacttcttgggcaacataattatatgctctaagaacagccactccagcatcttgcatcccatcaacatcttcagagtcattaaccacaaagataaaaccaattcttagtggtatatgattactaaggaacatctcagctgtgttcatcaactctgctgtggtctcatgtgcaggatcaactatgaaaaccatattatgtaagtttttcctgatctgccgaataacaccaggaaaggtgggtcgaagcaactcttgtaaactagaaggccacgaattatatctgctatcaacctccaggttgttgacccatgaaatagcaggactccggatgtctacggcatagtctgcctcagagggctggatgttcagcttcaaaacattatgcagagaaaggccttctattcccaatctatgcagaccctccattacccgagcttcattcctcaacacatcaaacagactgaatatatcctgtgtatctaaatccatgtgaagtccattgatgaagagggctgaatctccaggttgtaatcctaaagttcccttgaaatacttctgattctcttccacttcggttctaagttctgagctcacagctgtttttgttattgctctggctttggtaggaaaattctgactaagatccttcatgacaaccaaagccaactcaacaggagaagccaagattcgagcagcagtctggaaactgagatcttgcaactgccaaacctttaaaggtgccatttcattggtgctctctacaagatgctttctgagttctttcaactgtccctccaggtcggggtgcagatctcttaattttccaaagaggaacccctgaacctcatcaataggatcattttcaccaatcactgtggtgtttacctcagttcctttcacctgagtatcatccttggccttgtactcagtgctcttaatggccaattccacgccatagccagagaggtaaacaggctccttcctgggattaaatatataatgtctgaatacataattgattttgcctgcattgctttttgatataagctggcggtgaaaattggaaaattcctcagagccaatctcagagtagaaaatcaccacagggctttcaggattagacgagggatatctgtgatctcctttgaacaataaaggtttgggtctttcagaggctgtcagtagaagagcctcaagggtatcagattcacaagtcttctttccatgcactgaaaaaaacgaattacatccttctggtggaggttcatcagctgctatctgctggaaggcttggattgtagctgagtaagaacgaagggacagacaaaatttaaacaaattctgctggaggggtgacagaaactgaaatgcagcctccaatattgcatgatagtaggaataatcggtaccgtcatgatctgatgatccaatattttgactggcttctacaaaattccaaaatttctcttgactgtcttctgctaaaaactcactggcttctaacaacaatggagtggaaaaccattttgttgtaagagaggttgtaatggcttttgagtcggcctttactgaggagaacagccacagaacagtgagtacaaccagaactcccattttatagcaaactcccgcggcacacgcaccgctcgcgtctcccttgcagcccatgcccgggccgtggtcagtccgccacagtgccagagacaacgccagggcagggcggggcgaggcggcagcggcagtgcaggctgcgccagtgagaggccgacacgcgcctttcccgcggctcgactcaacacccagcctcgcaaagcaattgcccagctgccggccgccct

SEQ ID NO: 12000 - RNA, 8138 nt, Homo sapiens
  source 1..8138: mol_type = other RNA
ctgaatagctgggactacaggtgtgtgccaccatgcccagctaatttttgtatttttagtagagacggggtttcaccgtgttggccaggatggtctctatctcttgacctcataatccgcccgcctcggcttcccaaagtgctgggattacaggtgtaagccactgtgcctgaccggaaactgtttcttaacatacatcatgcacgtaatcttcgctctcccaagaggcattcacccaagcagacaggcaagcatctatgtgttcaattcgaaatgcaacaatgacagatgtacaactttaccactcttaaagaaactaacatgccatccattattctccatgtgggaaacattcagtaaacttctaaaaccaaacacaggactctggcatatccccacacccccagcagcaggctgtgacaggctttgatctcaatcaaatgccactgtacacagaacataaaaacaggctcaggatgctgcatgtcactctgacatatcacattatttcatattactctgtcacttactcacaaacaaaagtctccactatggcatgattgagagagaaaataattcactttatataaataacagctaagaacaacatactgtgaacagtttccagagtttgaacattcagcacaatcaattcttacttcttgggaaaaaaatatcttacctatcttttctgttacagtatgccttcttggagaaaatattttagtggtaacatcattttctggggcatttggttaattttgaaagatgattatgccacatgaaccaaaaaaaaaaaaaaaaactggcaggaggaggagggtcctaggccattctggaagcaagctgggttttgcattattcagagtcaactattaagctgacttatattagaatggcgacagataagaggcaatgagtgacaccaggacatgcacagcacacagagaatatggtctactcttgtcttccctgcacagattaaacataagaggcttggtagaaagacatggggaaaggtgctatgggggccagcatttggaaagcatatatcccagtgacttgagtatttgctatgcaacctcctggacgagaaactgggaaaaggcacacttccgcccacagttgtggacagcagcagtcacccgtctgaatgctttcattcaatgtgaagatgcagcttgaacaaaagtttctttttgtttgtttgttttctgagatggagtctcgctctgtcacccaggctggagtgcagtggcacgatctcagctcactgcaacctctgcctcctgggttcaggcgattctcctgtctctgcctcccgagtagctgggaatagagggtgagccacaacacccggctaatttttgtatttttagtagagacggggtttcaccatattggccaggctggtcttgaactcctgacctcatgatccgtccgcctcagcctcccaaagtgctgggattacaggtgtgagccaccacgcctggccgaacaaaagttttttaatcttactgatcccatctttccagctgctctgaacagaggggcagggcggggaaagtcatgtcacagactctgcccacagcagccattctgaggtgccttttcagtctcttatcctcttttgagctttcctcttcttaattttttgttttgttttgttttcattgtactcattaatcccctcctcaatttttaacagaattataaaagcaaagtcaaaaggtccttcaggatgactgggaggcttcctaggctaacttttgcatttgaaaatggaaaaaataaattacttgatatttgtgataagactaagatttcttaaaagtctgcacatcaatatattacctggcttaggagggtgagggcacagtatccatctgcaccctctcctcgtattttttaaaaacaggcaaaatatgtaagaaaaggctggtgcacgttggaagacagagcgtgcctgtctatgccagtgctgctgtgccctgcagcctggcagatggagtcggatgctggggcctcatgcccacttaggccaataacatactcaagactctacagcccgttcaccagcaaagtatgccctgaggggcaacactggctgtggaagtgaagacacacaaagcagggactaaaggcaaatggggcttcacgatgcagcgacatgaagacagaactggtgtgggcgccaaaggcaacctgcagggctcacataaaaggaaaataggacagaaagccacgagttccacaagcagaatcatttctggtcttacatctgagggcatttgtagagaaaagtccaaggcaatgtcccctgggtctgagagaaaaatcctacgcaaaagagggcagacaatgcggtgctcgtcttgagggagcctgaccctgaccctgaccctgacgggctggatgcgagaggggctgagtatggctgtattcagtaaggaaactggtagcagacttttctagaaggtggaaagaaaaagcaaagactttcacagatacaaaaattgttttcaaaacaattacctagaaagttcactgcggttgggtggggaataagtgtaatattttcatttcaaatgagccatggtgctactaatggattataaaagaggatggccagttctggtcttccttcccttcccttaacccccgaaccttcctactcctgacattttccctaccctcactgcaacccacccccatcctggcccaaaattaatttgcccagccactgcaccaaaccagccttgacacacaattgttggttggatttcaattaaacaatgcacctaatgcgttggaagagaaggtggggagggcacaaggatgttggcgtaaacctggaggtgtgtggaccttggacagagcttccgccggccagacccagggcagggtgggcatctgcagtgcagcgcaggccgcaggtaaactgaggtaaggaagaacatggtggctctagctggccctgctttccgagacagtgcagcatgtgtgtgctcttgggtgtgggcaccaaaaaactcattttcttccagttgctgctgccattccaccctctgactagaagaatgctctttacagagtccaaaggatcagccacttggtcttcctctgaggtacaaatccaacagagctttaatcccaaagatccagtggccaccagagtacagaagtcagaatcaaatgctcagaatcaaaaggtgtggcactcctgcccagccggcttatcagcagttgtatagacagatcagaaaaaactagcatttattataaaaactgtttttcaaatggggtgatttcctgtccttctccagagatcataattcttcacgtttctgaggaccttctcggcttggttcttttgtcttctctttgtacagtgctcccgtttctttctccttctgaaagcggatctgtagctgtttgatctcttggtcgtagtcctgccactccgggacaatccgcacagctgcttccagtttcggctctttggtcatcggattattacacaaatcaatggtttttgcccttttcttagaggcgtcatcacaccacgtttcacaccaaagccattcttgagggagggatttaattggcacctgatgaatcatgttattgggcagatcttgatcaagatttgaaaggctgttagggtcctgactcagaccttggtactgtcccctgagtctgtcaccagcagctattttcctaaacttcttcagatccacaacatatagtgcactgatatgatactttcgcccggctaaatgactggcccagtaccctgacttccagaacctgtagccgtccatttctcttcggctgtcacagaaaggagtgtaaccataaggagcaccatccaaattgaaatctcttaactctttcagatctgttcgtacaatctgatcagcatccacaaacaggaacttgtcaacaactagtgggaaaagtacatccaggaagaggatcttgtaaccccagatgatacgctgtttttcagtttgttgatgaagccaccggggccatttgtactgaacaagctcatactggaaattgtattcatttgccatgtaaggtataaactccttaaatgtgggggacaagtaattcttcaagaaccagaatttcacaggagtcttggtattcttcagcacggatagcatcattatgcgaagaaatctttcgtagagatgaccagatgcaacggagaaaatattaattatgtcatctttatcttgcttcacttcctcagtcttctgtcctgtaaagccccatttgaaggaatcccaaaatccagattcattctcactcgttccatcactcagcaagtcttcgttcaccatatctgccttcttctgaaccttcactttaataattttgcttttgaagttgttgaggacgataaccacctcatcagcatcagggggagaatcagtgccatcgtggctgtaaattctataaatatcttcagagcgtcccttcctaagtctgaggatccaagctcctgggttggctttcagctgaaagtagcccagattggccataacaatggtgtccacaatgaccgggttggctgaagttcctaaggtaaactgtagtccccgtggaggctggcctgtggtgatgtcgtagcaatgaccttccagtaacaggtattccagctcatactcagcagccactacactgtccacctcttctaaataaatattatcaagatcatatggtgttctgacagattctaccatccagctctcaggtgtgttcaaattcagagtgaacagtggagactgaggcatatccaaaaattttgcgattggacccttagcaaaactattgtctgaagtgaaagaaatctctggttctaagacataacggtaaaagctttttaaaggcatgtcagaaagtttggattggcagttcataaatactctcagattcatgtttatcagctgagccaaaaccaagagcaaaggagcaagtctctgtgcttctctggtgacagggtcaacgacagccacaacatcaaagtatgtctccccttccttcggcctcagtttgattgcactgtgtctgtcttcaaaaaactggtactcgattcttggatctccttttggttgcgctgacagaagagcatccaccttcattaccaagtcgcttgccacatcttcttctacccgaagctgttgaatatgagattttattttctgtcctgaggtttttaagatgatattttcgaggaggtggaaatcgtcttgattaaagagctcactatcctccagtggcccaatgatccttccattgctgatcactgccctctgtcccttcttcagcttcagaacatccctgcagtacacggcatgagacaaaatgaaatccattttggaagactcaaagacctctttaaaaagactgaaatccattcccccaacagagaactccgcaatgtcagctcctgcagccagggcctctgcagccccctccttggccattttggtgatgaagttcttagcagcgttggaagtctgagtttggagagctgcccagattgctctggagatctgagtgttctcatagcttatctctttggcaggattattgatcatgcttattctaacattgttactggatttctgatgtttgatggcatcatacagtaactgccgtccagaagggctatcaaaatccccaacaatccaaaaagttactggcctaataaaagaatcatcatagatttccttggaggacattcctttctttgtcagatagttcatactattggctacagcagcagtcttgccttgggaatccaagatagtaaatctagcataatcatccacaaagaagttattactcgctgttaaatccaggtagtctcgttcagctgtcaaaatcctagaattgattcgtggaacaacatttggctgattcatgatatactctaccacatcttgatcatggggcagttcacccaagtacaccgctctttggaagaaggtggtggtctccaggattttatgcattgtgatggtttctaactcatcagggtctagctgttccctttcaaagggcattccattgaacagcacaacgggcagaggtccaactccagtctgctcatagtagcctcttgcttccttccgattccgatcataagcagaatcaatccccaaaatgctattcacttctacatacggatatttcttctccaggacactgaccacatgttcaactttcactttttctccagtcctcaccttgttatagatatgtgtcagagtctggaaggcatgataatcatccacttcttgggcaacataattatatgctctaagaacagccactccagcatcttgcatcccatcaacatcttcagagtcattaaccacaaagataaaaccaattcttagtggtatatgattactaaggaacatctcagctgtgttcatcaactctgctgtggtctcatgtgcaggatcaactatgaaaaccatattatgtaagtttttcctgatctgccgaataacaccaggaaaggtgggtcgaagcaactcttgtaaactagaaggccacgaattatatctgctatcaacctccaggttgttgacccatgaaatagcaggactccggatgtctacggcatagtctgcctcagagggctggatgttcagcttcaaaacattatgcagagaaaggccttctattcccaatctatgcagaccctccattacccgagcttcattcctcaacacatcaaacagactgaatatatcctgtgtatctaaatccatgtgaagtccattgatgaagagggctgaatctccaggttgtaatcctaaagttcccttgaaatacttctgattctcttccacttcggttctaagttctgagctcacagctgtttttgttattgctctggctttggtaggaaaattctgactaagatccttcatgacaaccaaagccaactcaacaggagaagccaagattcgagcagcagtctggaaactgagatcttgcaactgccaaacctttaaaggtgccatttcattggtgctctctacaagatgctttctgagttctttcaactgtccctccaggtcggggtgcagatctcttaattttccaaagaggaacccctgaacctcatcaataggatcattttcaccaatcactgtggtgtttacctcagttcctttcacctgagtatcatccttggccttgtactcagtgctcttaatggccaattccacgccatagccagagaggtaaacaggctccttcctgggattaaatatataatgtctgaatacataattgattttgcctgcattgctttttgatataagctggcggtgaaaattggaaaattcctcagagccaatctcagagtagaaaatcaccacagggctttcaggattagacgagggatatctgtgatctcctttgaacaataaaggtttgggtctttcagaggctgtcagtagaagagcctcaagggtatcagattcacaagtcttctttccatgcactgaaaaaaacgaattacatccttctggtggaggttcatcagctgctatctgctggaaggcttggattgtagctgagtaagaacgaagggacagacaaaatttaaacaaattctgctggaggggtgacagaaactgaaatgcagcctccaatattgcatgatagtaggaataatcggtaccgtcatgatctgatgatccaatattttgactggcttctacaaaattccaaaatttctcttgactgtcttctgctaaaaactcactggcttctaacaacaatggagtggaaaaccattttgttgtaagagaggttgtaatggcttttgagtcggcctttactgaggagaacagccacagaacagtgagtacaaccagaactcccattttatagcaaactccgctcgcgtctcccttgcagcccatgcccgggccgtggtcagtccgccacagtgccagagacaacgccagggcagggcggggcgaggcggcagcggcagtgcaggctgcgccagtgagaggccgacacgcgcctttcccgcggctcgactcaacacccagcctcgcaaagcaattgcccagctgccggccgccctttta

SEQ ID NO: 12001 - RNA, 8155 nt, Homo sapiens
  source 1..8155: mol_type = other RNA
ctgaatagctgggactacaggtgtgtgccaccatgcccagctaatttttgtatttttagtagagacggggtttcaccgtgttggccaggatggtctctatctcttgacctcataatccgcccgcctcggcttcccaaagtgctgggattacaggtgtaagccactgtgcctgaccggaaactgtttcttaacatacatcatgcacgtaatcttcgctctcccaagaggcattcacccaagcagacaggcaagcatctatgtgttcaattcgaaatgcaacaatgacagatgtacaactttaccactcttaaagaaactaacatgccatccattattctccatgtgggaaacattcagtaaacttctaaaaccaaacacaggactctggcatatccccacacccccagcagcaggctgtgacaggctttgatctcaatcaaatgccactgtacacagaacataaaaacaggctcaggatgctgcatgtcactctgacatatcacattatttcatattactctgtcacttactcacaaacaaaagtctccactatggcatgattgagagagaaaataattcactttatataaataacagctaagaacaacatactgtgaacagtttccagagtttgaacattcagcacaatcaattcttacttcttgggaaaaaaatatcttacctatcttttctgttacagtatgccttcttggagaaaatattttagtggtaacatcattttctggggcatttggttaattttgaaagatgattatgccacatgaaccaaaaaaaaaaaaaaaaactggcaggaggaggagggtcctaggccattctggaagcaagctgggttttgcattattcagagtcaactattaagctgacttatattagaatggcgacagataagaggcaatgagtgacaccaggacatgcacagcacacagagaatatggtctactcttgtcttccctgcacagattaaacataagaggcttggtagaaagacatggggaaaggtgctatgggggccagcatttggaaagcatatatcccagtgacttgagtatttgctatgcaacctcctggacgagaaactgggaaaaggcacacttccgcccacagttgtggacagcagcagtcacccgtctgaatgctttcattcaatgtgaagatgcagcttgaacaaaagtttctttttgtttgtttgttttctgagatggagtctcgctctgtcacccaggctggagtgcagtggcacgatctcagctcactgcaacctctgcctcctgggttcaggcgattctcctgtctctgcctcccgagtagctgggaatagagggtgagccacaacacccggctaatttttgtatttttagtagagacggggtttcaccatattggccaggctggtcttgaactcctgacctcatgatccgtccgcctcagcctcccaaagtgctgggattacaggtgtgagccaccacgcctggccgaacaaaagttttttaatcttactgatcccatctttccagctgctctgaacagaggggcagggcggggaaagtcatgtcacagactctgcccacagcagccattctgaggtgccttttcagtctcttatcctcttttgagctttcctcttcttaattttttgttttgttttgttttcattgtactcattaatcccctcctcaatttttaacagaattataaaagcaaagtcaaaaggtccttcaggatgactgggaggcttcctaggctaacttttgcatttgaaaatggaaaaaataaattacttgatatttgtgataagactaagatttcttaaaagtctgcacatcaatatattacctggcttaggagggtgagggcacagtatccatctgcaccctctcctcgtattttttaaaaacaggcaaaatatgtaagaaaaggctggtgcacgttggaagacagagcgtgcctgtctatgccagtgctgctgtgccctgcagcctggcagatggagtcggatgctggggcctcatgcccacttaggccaataacatactcaagactctacagcccgttcaccagcaaagtatgccctgaggggcaacactggctgtggaagtgaagacacacaaagcagggactaaaggcaaatggggcttcacgatgcagcgacatgaagacagaactggtgtgggcgccaaaggcaacctgcagggctcacataaaaggaaaataggacagaaagccacgagttccacaagcagaatcatttctggtcttacatctgagggcatttgtagagaaaagtccaaggcaatgtcccctgggtctgagagaaaaatcctacgcaaaagagggcagacaatgcggtgctcgtcttgagggagcctgaccctgaccctgaccctgacgggctggatgcgagaggggctgagtatggctgtattcagtaaggaaactggtagcagacttttctagaaggtggaaagaaaaagcaaagactttcacagatacaaaaattgttttcaaaacaattacctagaaagttcactgcggttgggtggggaataagtgtaatattttcatttcaaatgagccatggtgctactaatggattataaaagaggatggccagttctggtcttccttcccttcccttaacccccgaaccttcctactcctgacattttccctaccctcactgcaacccacccccatcctggcccaaaattaatttgcccagccactgcaccaaaccagccttgacacacaattgttggttggatttcaattaaacaatgcacctaatgcgttggaagagaaggtggggagggcacaaggatgttggcgtaaacctggaggtgtgtggaccttggacagagcttccgccggccagacccagggcagggtgggcatctgcagtgcagcgcaggccgcaggtaaactgaggtaaggaagaacatggtggctctagctggccctgctttccgagacagtgcagcatgtgtgtgctcttgggtgtgggcaccaaaaaactcattttcttccagttgctgctgccattccaccctctgactagaagaatgctctttacagagtccaaaggatcagccacttggtcttcctctgaggtacaaatccaacagagctttaatcccaaagatccagtggccaccagagtacagaagtcagaatcaaatgctcagaatcaaaaggtgtggcactcctgcccagccggcttatcagcagttgtatagacagatcagaaaaaactagcatttattataaaaactgtttttcaaatggggtgatttcctgtccttctccagagatcataattcttcacgtttctgaggaccttctcggcttggttcttttgtcttctctttgtacagtgctcccgtttctttctccttctgaaagcggatctgtagctgtttgatctcttggtcgtagtcctgccactccgggacaatccgcacagctgcttccagtttcggctctttggtcatcggattattacacaaatcaatggtttttgcccttttcttagaggcgtcatcacaccacgtttcacaccaaagccattcttgagggagggatttaattggcacctgatgaatcatgttattgggcagatcttgatcaagatttgaaaggctgttagggtcctgactcagaccttggtactgtcccctgagtctgtcaccagcagctattttcctaaacttcttcagatccacaacatatagtgcactgatatgatactttcgcccggctaaatgactggcccagtaccctgacttccagaacctgtagccgtccatttctcttcggctgtcacagaaaggagtgtaaccataaggagcaccatccaaattgaaatctcttaactctttcagatctgttcgtacaatctgatcagcatccacaaacaggaacttgtcaacaactagtgggaaaagtacatccaggaagaggatcttgtaaccccagatgatacgctgtttttcagtttgttgatgaagccaccggggccatttgtactgaacaagctcatactggaaattgtattcatttgccatgtaaggtataaactccttaaatgtgggggacaagtaattcttcaagaaccagaatttcacaggagtcttggtattcttcagcacggatagcatcattatgcgaagaaatctttcgtagagatgaccagatgcaacggagaaaatattaattatgtcatctttatcttgcttcacttcctcagtcttctgtcctgtaaagccccatttgaaggaatcccaaaatccagattcattctcactcgttccatcactcagcaagtcttcgttcaccatatctgccttcttctgaaccttcactttaataattttgcttttgaagttgttgaggacgataaccacctcatcagcatcagggggagaatcagtgccatcgtggctgtaaattctataaatatcttcagagcgtcccttcctaagtctgaggatccaagctcctgggttggctttcagctgaaagtagcccagattggccataacaatggtgtccacaatgaccgggttggctgaagttcctaaggtaaactgtagtccccgtggaggctggcctgtggtgatgtcgtagcaatgaccttccagtaacaggtattccagctcatactcagcagccactacactgtccacctcttctaaataaatattatcaagatcatatggtgttctgacagattctaccatccagctctcaggtgtgttcaaattcagagtgaacagtggagactgaggcatatccaaaaattttgcgattggacccttagcaaaactattgtctgaagtgaaagaaatctctggttctaagacataacggtaaaagctttttaaaggcatgtcagaaagtttggattggcagttcataaatactctcagattcatgtttatcagctgagccaaaaccaagagcaaaggagcaagtctctgtgcttctctggtgacagggtcaacgacagccacaacatcaaagtatgtctccccttccttcggcctcagtttgattgcactgtgtctgtcttcaaaaaactggtactcgattcttggatctccttttggttgcgctgacagaagagcatccaccttcattaccaagtcgcttgccacatcttcttctacccgaagctgttgaatatgagattttattttctgtcctgaggtttttaagatgatattttcgaggaggtggaaatcgtcttgattaaagagctcactatcctccagtggcccaatgatccttccattgctgatcactgccctctgtcccttcttcagcttcagaacatccctgcagtacacggcatgagacaaaatgaaatccattttggaagactcaaagacctctttaaaaagactgaaatccattcccccaacagagaactccgcaatgtcagctcctgcagccagggcctctgcagccccctccttggccattttggtgatgaagttcttagcagcgttggaagtctgagtttggagagctgcccagattgctctggagatctgagtgttctcatagcttatctctttggcaggattattgatcatgcttattctaacattgttactggatttctgatgtttgatggcatcatacagtaactgccgtccagaagggctatcaaaatccccaacaatccaaaaagttactggcctaataaaagaatcatcatagatttccttggaggacattcctttctttgtcagatagttcatactattggctacagcagcagtcttgccttgggaatccaagatagtaaatctagcataatcatccacaaagaagttattactcgctgttaaatccaggtagtctcgttcagctgtcaaaatcctagaattgattcgtggaacaacatttggctgattcatgatatactctaccacatcttgatcatggggcagttcacccaagtacaccgctctttggaagaaggtggtggtctccaggattttatgcattgtgatggtttctaactcatcagggtctagctgttccctttcaaagggcattccattgaacagcacaacgggcagaggtccaactccagtctgctcatagtagcctcttgcttccttccgattccgatcataagcagaatcaatccccaaaatgctattcacttctacatacggatatttcttctccaggacactgaccacatgttcaactttcactttttctccagtcctcaccttgttatagatatgtgtcagagtctggaaggcatgataatcatccacttcttgggcaacataattatatgctctaagaacagccactccagcatcttgcatcccatcaacatcttcagagtcattaaccacaaagataaaaccaattcttagtggtatatgattactaaggaacatctcagctgtgttcatcaactctgctgtggtctcatgtgcaggatcaactatgaaaaccatattatgtaagtttttcctgatctgccgaataacaccaggaaaggtgggtcgaagcaactcttgtaaactagaaggccacgaattatatctgctatcaacctccaggttgttgacccatgaaatagcaggactccggatgtctacggcatagtctgcctcagagggctggatgttcagcttcaaaacattatgcagagaaaggccttctattcccaatctatgcagaccctccattacccgagcttcattcctcaacacatcaaacagactgaatatatcctgtgtatctaaatccatgtgaagtccattgatgaagagggctgaatctccaggttgtaatcctaaagttcccttgaaatacttctgattctcttccacttcggttctaagttctgagctcacagctgtttttgttattgctctggctttggtaggaaaattctgactaagatccttcatgacaaccaaagccaactcaacaggagaagccaagattcgagcagcagtctggaaactgagatcttgcaactgccaaacctttaaaggtgccatttcattggtgctctctacaagatgctttctgagttctttcaactgtccctccaggtcggggtgcagatctcttaattttccaaagaggaacccctgaacctcatcaataggatcattttcaccaatcactgtggtgtttacctcagttcctttcacctgagtatcatccttggccttgtactcagtgctcttaatggccaattccacgccatagccagagaggtaaacaggctccttcctgggattaaatatataatgtctgaatacataattgattttgcctgcattgctttttgatataagctggcggtgaaaattggaaaattcctcagagccaatctcagagtagaaaatcaccacagggctttcaggattagacgagggatatctgtgatctcctttgaacaataaaggtttgggtctttcagaggctgtcagtagaagagcctcaagggtatcagattcacaagtcttctttccatgcactgaaaaaaacgaattacatccttctggtggaggttcatcagctgctatctgctggaaggcttggattgtagctgagtaagaacgaagggacagacaaaatttaaacaaattctgctggaggggtgacagaaactgaaatgcagcctccaatattgcatgatagtaggaataatcggtaccgtcatgatctgatgatccaatattttgactggcttctacaaaattccaaaatttctcttgactgtcttctgctaaaaactcactggcttctaacaacaatggagtggaaaaccattttgttgtaagagaggttgtaatggcttttgagtcggcctttactgaggagaacagccacagaacagtgagtacaaccagaactcccattttatagcaaactcctgtcaccggcagcgcacccgcggcacacgcaccgctcgcgtctcccttgcagcccatgcccgggccgtggtcagtccgccacagtgccagagacaacgccagggcagggcggggcgaggcggcagcggcagtgcaggctgcgccagtgagaggccgacacgcgcctttcccgcggctcgactcaacacccagcctcgcaaagcaattgcccagct

SEQ ID NO: 12002 - RNA, 8336 nt, Homo sapiens
  source 1..8336: mol_type = other RNA
ctgaatagctgggactacaggtgtgtgccaccatgcccagctaatttttgtatttttagtagagacggggtttcaccgtgttggccaggatggtctctatctcttgacctcataatccgcccgcctcggcttcccaaagtgctgggattacaggtgtaagccactgtgcctgaccggaaactgtttcttaacatacatcatgcacgtaatcttcgctctcccaagaggcattcacccaagcagacaggcaagcatctatgtgttcaattcgaaatgcaacaatgacagatgtacaactttaccactcttaaagaaactaacatgccatccattattctccatgtgggaaacattcagtaaacttctaaaaccaaacacaggactctggcatatccccacacccccagcagcaggctgtgacaggctttgatctcaatcaaatgccactgtacacagaacataaaaacaggctcaggatgctgcatgtcactctgacatatcacattatttcatattactctgtcacttactcacaaacaaaagtctccactatggcatgattgagagagaaaataattcactttatataaataacagctaagaacaacatactgtgaacagtttccagagtttgaacattcagcacaatcaattcttacttcttgggaaaaaaatatcttacctatcttttctgttacagtatgccttcttggagaaaatattttagtggtaacatcattttctggggcatttggttaattttgaaagatgattatgccacatgaaccaaaaaaaaaaaaaaaaactggcaggaggaggagggtcctaggccattctggaagcaagctgggttttgcattattcagagtcaactattaagctgacttatattagaatggcgacagataagaggcaatgagtgacaccaggacatgcacagcacacagagaatatggtctactcttgtcttccctgcacagattaaacataagaggcttggtagaaagacatggggaaaggtgctatgggggccagcatttggaaagcatatatcccagtgacttgagtatttgctatgcaacctcctggacgagaaactgggaaaaggcacacttccgcccacagttgtggacagcagcagtcacccgtctgaatgctttcattcaatgtgaagatgcagcttgaacaaaagtttctttttgtttgtttgttttctgagatggagtctcgctctgtcacccaggctggagtgcagtggcacgatctcagctcactgcaacctctgcctcctgggttcaggcgattctcctgtctctgcctcccgagtagctgggaatagagggtgagccacaacacccggctaatttttgtatttttagtagagacggggtttcaccatattggccaggctggtcttgaactcctgacctcatgatccgtccgcctcagcctcccaaagtgctgggattacaggtgtgagccaccacgcctggccgaacaaaagttttttaatcttactgatcccatctttccagctgctctgaacagaggggcagggcggggaaagtcatgtcacagactctgcccacagcagccattctgaggtgccttttcagtctcttatcctcttttgagctttcctcttcttaattttttgttttgttttgttttcattgtactcattaatcccctcctcaatttttaacagaattataaaagcaaagtcaaaaggtccttcaggatgactgggaggcttcctaggctaacttttgcatttgaaaatggaaaaaataaattacttgatatttgtgataagactaagatttcttaaaagtctgcacatcaatatattacctggcttaggagggtgagggcacagtatccatctgcaccctctcctcgtattttttaaaaacaggcaaaatatgtaagaaaaggctggtgcacgttggaagacagagcgtgcctgtctatgccagtgctgctgtgccctgcagcctggcagatggagtcggatgctggggcctcatgcccacttaggccaataacatactcaagactctacagcccgttcaccagcaaagtatgccctgaggggcaacactggctgtggaagtgaagacacacaaagcagggactaaaggcaaatggggcttcacgatgcagcgacatgaagacagaactggtgtgggcgccaaaggcaacctgcagggctcacataaaaggaaaataggacagaaagccacgagttccacaagcagaatcatttctggtcttacatctgagggcatttgtagagaaaagtccaaggcaatgtcccctgggtctgagagaaaaatcctacgcaaaagagggcagacaatgcggtgctcgtcttgagggagcctgaccctgaccctgaccctgacgggctggatgcgagaggggctgagtatggctgtattcagtaaggaaactggtagcagacttttctagaaggtggaaagaaaaagcaaagactttcacagatacaaaaattgttttcaaaacaattacctagaaagttcactgcggttgggtggggaataagtgtaatattttcatttcaaatgagccatggtgctactaatggattataaaagaggatggccagttctggtcttccttcccttcccttaacccccgaaccttcctactcctgacattttccctaccctcactgcaacccacccccatcctggcccaaaattaatttgcccagccactgcaccaaaccagccttgacacacaattgttggttggatttcaattaaacaatgcacctaatgcgttggaagagaaggtggggagggcacaaggatgttggcgtaaacctggaggtgtgtggaccttggacagagcttccgccggccagacccagggcagggtgggcatctgcagtgcagcgcaggccgcaggtaaactgaggtaaggaagaacatggtggctctagctggccctgctttccgagacagtgcagcatgtgtgtgctcttgggtgtgggcaccaaaaaactcattttcttccagttgctgctgccattccaccctctgactagaagaatgctctttacagagtccaaaggatcagccacttggtcttcctctgaggtacaaatccaacagagctttaatcccaaagatccagtggccaccagagtacagaagtcagaatcaaatgctcagaatcaaaaggtgtggcactcctgcccagccggcttatcagcagttgtatagacagatcagaaaaaactagcatttattataaaaactgtttttcaaatggggtgatttcctgtccttctccagagatcataattcttcacgtttctgaggaccttctcggcttggttcttttgtcttctctttgtacagtgctcccgtttctttctccttctgaaagcggatctgtagctgtttgatctcttggtcgtagtcctgccactccgggacaatccgcacagctgcttccagtttcggctctttggtcatcggattattacacaaatcaatggtttttgcccttttcttagaggcgtcatcacaccacgtttcacaccaaagccattcttgagggagggatttaattggcacctgatgaatcatgttattgggcagatcttgatcaagatttgaaaggctgttagggtcctgactcagaccttggtactgtcccctgagtctgtcaccagcagctattttcctaaacttcttcagatccacaacatatagtgcactgatatgatactttcgcccggctaaatgactggcccagtaccctgacttccagaacctgtagccgtccatttctcttcggctgtcacagaaaggagtgtaaccataaggagcaccatccaaattgaaatctcttaactctttcagatctgttcgtacaatctgatcagcatccacaaacaggaacttgtcaacaactagtgggaaaagtacatccaggaagaggatcttgtaaccccagatgatacgctgtttttcagtttgttgatgaagccaccggggccatttgtactgaacaagctcatactggaaattgtattcatttgccatgtaaggtataaactccttaaatgtgggggacaagtaattcttcaagaaccagaatttcacaggagtcttggtattcttcagcacggatagcatcattatgcgaagaaatctttcgtagagatgaccagatgcaacggagaaaatattaattatgtcatctttatcttgcttcacttcctcagtcttctgtcctgtaaagccccatttgaaggaatcccaaaatccagattcattctcactcgttccatcactcagcaagtcttcgttcaccatatctgccttcttctgaaccttcactttaataattttgcttttgaagttgttgaggacgataaccacctcatcagcatcagggggagaatcagtgccatcgtggctgtaaattctataaatatcttcagagcgtcccttcctaagtctgaggatccaagctcctgggttggctttcagctgaaagtagcccagattggccataacaatggtgtccacaatgaccgggttggctgaagttcctaaggtaaactgtagtccccgtggaggctggcctgtggtgatgtcgtagcaatgaccttccagtaacaggtattccagctcatactcagcagccactacactgtccacctcttctaaataaatattatcaagatcatatggtgttctgacagattctaccatccagctctcaggtgtgttcaaattcagagtgaacagtggagactgaggcatatccaaaaattttgcgattggacccttagcaaaactattgtctgaagtgaaagaaatctctggttctaagacataacggtaaaagctttttaaaggcatgtcagaaagtttggattggcagttcataaatactctcagattcatgtttatcagctgagccaaaaccaagagcaaaggagcaagtctctgtgcttctctggtgacagggtcaacgacagccacaacatcaaagtatgtctccccttccttcggcctcagtttgattgcactgtgtctgtcttcaaaaaactggtactcgattcttggatctccttttggttgcgctgacagaagagcatccaccttcattaccaagtcgcttgccacatcttcttctacccgaagctgttgaatatgagattttattttctgtcctgaggtttttaagatgatattttcgaggaggtggaaatcgtcttgattaaagagctcactatcctccagtggcccaatgatccttccattgctgatcactgccctctgtcccttcttcagcttcagaacatccctgcagtacacggcatgagacaaaatgaaatccattttggaagactcaaagacctctttaaaaagactgaaatccattcccccaacagagaactccgcaatgtcagctcctgcagccagggcctctgcagccccctccttggccattttggtgatgaagttcttagcagcgttggaagtctgagtttggagagctgcccagattgctctggagatctgagtgttctcatagcttatctctttggcaggattattgatcatgcttattctaacattgttactggatttctgatgtttgatggcatcatacagtaactgccgtccagaagggctatcaaaatccccaacaatccaaaaagttactggcctaataaaagaatcatcatagatttccttggaggacattcctttctttgtcagatagttcatactattggctacagcagcagtcttgccttgggaatccaagatagtaaatctagcataatcatccacaaagaagttattactcgctgttaaatccaggtagtctcgttcagctgtcaaaatcctagaattgattcgtggaacaacatttggctgattcatgatatactctaccacatcttgatcatggggcagttcacccaagtacaccgctctttggaagaaggtggtggtctccaggattttatgcattgtgatggtttctaactcatcagggtctagctgttccctttcaaagggcattccattgaacagcacaacgggcagaggtccaactccagtctgctcatagtagcctcttgcttccttccgattccgatcataagcagaatcaatccccaaaatgctattcacttctacatacggatatttcttctccaggacactgaccacatgttcaactttcactttttctccagtcctcaccttgttatagatatgtgtcagagtctggaaggcatgataatcatccacttcttgggcaacataattatatgctctaagaacagccactccagcatcttgcatcccatcaacatcttcagagtcattaaccacaaagataaaaccaattcttagtggtatatgattactaaggaacatctcagctgtgttcatcaactctgctgtggtctcatgtgcaggatcaactatgaaaaccatattatgtaagtttttcctgatctgccgaataacaccaggaaaggtgggtcgaagcaactcttgtaaactagaaggccacgaattatatctgctatcaacctccaggttgttgacccatgaaatagcaggactccggatgtctacggcatagtctgcctcagagggctggatgttcagcttcaaaacattatgcagagaaaggccttctattcccaatctatgcagaccctccattacccgagcttcattcctcaacacatcaaacagactgaatatatcctgtgtatctaaatccatgtgaagtccattgatgaagagggctgaatctccaggttgtaatcctaaagttcccttgaaatacttctgattctcttccacttcggttctaagttctgagctcacagctgtttttgttattgctctggctttggtaggaaaattctgactaagatccttcatgacaaccaaagccaactcaacaggagaagccaagattcgagcagcagtctggaaactgagatcttgcaactgccaaacctttaaaggtgccatttcattggtgctctctacaagatgctttctgagttctttcaactgtccctccaggtcggggtgcagatctcttaattttccaaagaggaacccctgaacctcatcaataggatcattttcaccaatcactgtggtgtttacctcagttcctttcacctgagtatcatccttggccttgtactcagtgctcttaatggccaattccacgccatagccagagaggtaaacaggctccttcctgggattaaatatataatgtctgaatacataattgattttgcctgcattgctttttgatataagctggcggtgaaaattggaaaattcctcagagccaatctcagagtagaaaatcaccacagggctttcaggattagacgagggatatctgtgatctcctttgaacaataaaggtttgggtctttcagaggctgtcagtagaagagcctcaagggtatcagattcacaagtcttctttccatgcactgaaaaaaacgaattacatccttctggtggaggttcatcagctgctatctgctggaaggcttggattgtagctgagtaagaacgaagggacagacaaaatttaaacaaattctgctggaggggtgacagaaactgaaatgcagcctccaatattgcatgatagtaggaataatcggtaccgtcatgatctgatgatccaatattttgactggcttctacaaaattccaaaatttctcttgactgtcttctgctaaaaactcactggcttctaacaacaatggagtggaaaaccattttgttgtaagagaggttgtaatggcttttgagtcggcctttactgaggagaacagccacagaacagtgagtacaaccagaactcccattttatagcaaactccttgccaagaagaccactgagggcaactcggggcgctcgcgaataggggaagggataggacaccagagggtaaactgagtcacggtagaggcggaagctcaatgtgacaggggcacagggtcgccttgtgccccaaaccctctctttgtccacgaggcctcctcacgccacccctgggtacctgtcaccggcagcgcacccgcggcacacgcaccgctcgcgtctcccttgcagcccatgcccgggccgtggtcagtccgccacagtgccagagacaacgccagggcagggcggggcgaggcggcagcggcagtgcaggctgcgccagtgagaggccgacacgcgcctttcccgcggctcgactcaacacccagcctcgcaaagcaattgcccagct

SEQ ID NO: 12003 - RNA, 6859 nt, Homo sapiens
  source 1..6859: mol_type = other RNA
ctgaatagctgggactacaggtgtgtgccaccatgcccagctaatttttgtatttttagtagagacggggtttcaccgtgttggccaggatggtctctatctcttgacctcataatccgcccgcctcggcttcccaaagtgctgggattacaggtgtaagccactgtgcctgaccggaaactgtttcttaacatacatcatgcacgtaatcttcgctctcccaagaggcattcacccaagcagacaggcaagcatctatgtgttcaattcgaaatgcaacaatgacagatgtacaactttaccactcttaaagaaactaacatgccatccattattctccatgtgggaaacattcagtaaacttctaaaaccaaacacaggactctggcatatccccacacccccagcagcaggctgtgacaggctttgatctcaatcaaatgccactgtacacagaacataaaaacaggctcaggatgctgcatgtcactctgacatatcacattatttcatattactctgtcacttactcacaaacaaaagtctccactatggcatgattgagagagaaaataattcactttatataaataacagctaagaacaacatactgtgaacagtttccagagtttgaacattcagcacaatcaattcttacttcttgggaaaaaaatatcttacctatcttttctgttacagtatgccttcttggagaaaatattttagtggtaacatcattttctggggcatttggttaattttgaaagatgattatgccacatgaaccaaaaaaaaaaaaaaaaactggcaggaggaggagggtcctaggccattctggaagcaagctgggttttgcattattcagagtcaactattaagctgacttatattagaatggcgacagataagaggcaatgagtgacaccaggacatgcacagcacacagagaatatggtctactcttgtcttccctgcacagattaaacataagaggcttggtagaaagacatggggaaaggtgctatgggggccagcatttggaaagcatatatcccagtgacttgagtatttgctatgcaacctcctggacgagaaactgggaaaaggcacacttccgcccacagttgtggacagcagcagtcacccgtctgaatgctttcattcaatgtgaagatgcagcttgaacaaaagtttctttttgtttgtttgttttctgagatggagtctcgctctgtcacccaggctggagtgcagtggcacgatctcagctcactgcaacctctgcctcctgggttcaggcgattctcctgtctctgcctcccgagtagctgggaatagagggtgagccacaacacccggctaatttttgtatttttagtagagacggggtttcaccatattggccaggctggtcttgaactcctgacctcatgatccgtccgcctcagcctcccaaagtgctgggattacaggtgtgagccaccacgcctggccgaacaaaagttttttaatcttactgatcccatctttccagctgctctgaacagaggggcagggcggggaaagtcatgtcacagactctgcccacagcagccattctgaggtgccttttcagtctcttatcctcttttgagctttcctcttcttaattttttgttttgttttgttttcattgtactcattaatcccctcctcaatttttaacagaattataaaagcaaagtcaaaaggtccttcaggatgactgggaggcttcctaggctaacttttgcatttgaaaatggaaaaaataaattacttgatatttgtgataagactaagatttcttaaaagtctgcacatcaatatattacctggcttaggagggtgagggcacagtatccatctgcaccctctcctcgtattttttaaaaacaggcaaaatatgtaagaaaaggctggtgcacgttggaagacagagcgtgcctgtctatgccagtgctgctgtgccctgcagcctggcagatggagtcggatgctggggcctcatgcccacttaggccaataacatactcaagactctacagcccgttcaccagcaaagtatgccctgaggggcaacactggctgtggaagtgaagacacacaaagcagggactaaaggcaaatggggcttcacgatgcagcgacatgaagacagaactggtgtgggcgccaaaggcaacctgcagggctcacataaaaggaaaataggacagaaagccacgagttccacaagcagaatcatttctggtcttacatctgagggcatttgtagagaaaagtccaaggcaatgtcccctgggtctgagagaaaaatcctacgcaaaagagggcagacaatgcggtgctcgtcttgagggagcctgaccctgaccctgaccctgacgggctggatgcgagaggggctgagtatggctgtattcagtaaggaaactggtagcagacttttctagaaggtggaaagaaaaagcaaagactttcacagatacaaaaattgttttcaaaacaattacctagaaagttcactgcggttgggtggggaataagtgtaatattttcatttcaaatgagccatggtgctactaatggattataaaagaggatggccagttctggtcttccttcccttcccttaacccccgaaccttcctactcctgacattttccctaccctcactgcaacccacccccatcctggcccaaaattaatttgcccagccactgcaccaaaccagccttgacacacaattgttggttggatttcaattaaacaatgcacctaatgcgttggaagagaaggtggggagggcacaaggatgttggcgtaaacctggaggtgtgtggaccttggacagagcttccgccggccagacccagggcagggtgggcatctgcagtgcagcgcaggccgcaggtaaactgaggtaaggaagaacatggtggctctagctggccctgctttccgagacagtgcagcatgtgtgtgctcttgggtgtgggcaccaaaaaactcattttcttccagttgctgctgccattccaccctctgactagaagaatgctctttacagagtccaaaggatcagccacttggtcttcctctgaggtacaaatccaacagagctttaatcccaaagatccagtggccaccagagtacagaagtcagaatcaaatgctcagaatcaaaaggtgtggcactcctgcccagccggcttatcagcagttgtatagacagatcagaaaaaactagcatttattataaaaactgtttttcaaatggggtgatttcctgtccttctccagagatcataattcttcacgtttctgaggaccttctcggcttggttcttttgtcttctctttgtacagtgctcccgtttctttctccttctgaaagcggatctgtagctgtttgatctcttggtcgtagtcctgccactccgggacaatccgcacagctgcttccagtttcggctctttggtcatcggattattacacaaatcaatggtttttgcccttttcttagaggcgtcatcacaccacgtttcacaccaaagccattcttgagggagggatttaattggcacctgatgaatcatgttattgggcagatcttgatcaagatttgaaaggctgttagggtcctgactcagaccttggtactgtcccctgagtctgtcaccagcagctattttcctaaacttcttcagatccacaacatatagtgcactgatatgatactttcgcccggctaaatgactggcccagtaccctgacttccagaacctgtagccgtccatttctcttcggctgtcacagaaaggagtgtaaccataaggagcaccatccaaattgaaatctcttaactctttcagatctgttcgtacaatctgatcagcatccacaaacaggaacttgtcaacaactagtgggaaaagtacatccaggaagaggatcttgtaaccccagatgatacgctgtttttcagtttgttgatgaagccaccggggccatttgtactgaacaagctcatactggaaattgtattcatttgccatgtaaggtataaactccttaaatgtgggggacaagtaattcttcaagaaccagaatttcacaggagtcttggtattcttcagcacggatagcatcattatgcgaagaaatctttcgtagagatgaccagatgcaacggagaaaatattaattatgtcatctttatcttgcttcacttcctcagtcttctgtcctgtaaagccccatttgaaggaatcccaaaatccagattcattctcactcgttccatcactcagcaagtcttcgttcaccatatctgccttcttctgaaccttcactttaataattttgcttttgaagttgttgaggacgataaccacctcatcagcatcagggggagaatcagtgccatcgtggctgtaaattctataaatatcttcagagcgtcccttcctaagtctgaggatccaagctcctgggttggctttcagctgaaagtagcccagattggccataacaatggtgtccacaatgaccgggttggctgaagttcctaaggtaaactgtagtccccgtggaggctggcctgtggtgatgtcgtagcaatgaccttccagtaacaggtattccagctcatactcagcagccactacactgtccacctcttctaaataaatattatcaagatcatatggtgttctgacagattctaccatccagctctcaggtgtgttcaaattcagagtgaacagtggagactgaggcatatccaaaaattttgcgattggacccttagcaaaactattgtctgaagtgaaagaaatctctggttctaagacataacggtaaaagctttttaaaggcatgtcagaaagtttggattggcagttcataaatactctcagattcatgtttatcagctgagccaaaaccaagagcaaaggagcaagtctctgtgcttctctggtgacagggtcaacgacagccacaacatcaaagtatgtctccccttccttcggcctcagtttgattgcactgtgtctgtcttcaaaaaactggtactcgattcttggatctccttttggttgcgctgacagaagagcatccaccttcattaccaagtcgcttgccacatcttcttctacccgaagctgttgaatatgagattttattttctgtcctgaggtttttaagatgatattttcgaggaggtggaaatcgtcttgattaaagagctcactatcctccagtggcccaatgatccttccattgctgatcactgccctctgtcccttcttcagcttcagaacatccctgcagtacacggcatgagacaaaatgaaatccattttggaagactcaaagacctctttaaaaagactgaaatccattcccccaacagagaactccgcaatgtcagctcctgcagccagggcctctgcagccccctccttggccattttggtgatgaagttcttagcagcgttggaagtctgagtttggagagctgcccagattgctctggagatctgagtgttctcatagcttatctctttggcaggattattgatcatgcttattctaacattgttactggatttctgatgtttgatggcatcatacagtaactgccgtccagaagggctatcaaaatccccaacaatccaaaaagttactggcctaataaaagaatcatcatagatttccttggaggacattcctttctttgtcagatagttcatactattggctacagcagcagtcttgccttgggaatccaagatagtaaatctagcataatcatccacaaagaagttattataacaataaatagctggttatgacttcattacacacatctttccttccccagtgagatttcatgggctagtgatgacagttccatcttatttccaggtgtttgctgaagaggcctcagaatctcgaggaaggcacaaggaacaaattgcacctgggcttaacatatttggctcttataaggtattctagcagaaaactgccaactgtccaccaactgaggaacagatatatgtggactatccataaagtggactataaaaaggaatgaaatgctgacatacacaacaacatgcataagccttaacaatatgctaaattaaacaagccaggcacaaaaggcttccaattatatgaaatgtctagaataggcaaatccatagacacagaaagtagattagttgttgccagaggataggggaagggaggaacagagagtgactactaataggtacatggaattctggggaatttttggggggtgatgataatgatgtatcattagacagtggtgatgactgcacaaactttgtggggtttttttcattaaaaaaaccattgaattgtatactttaaaaggttgagttttatggcatatacatcatatcttgatgaagctgctaaaggccttcctaagttctcagagtaaaattcactgagatatttgttgacattatggctgactgactctagaatgaggatgaagaaagagaactgctttatgactagagaagcgaacaatccaggtccattctcatcatctattgtctgtttagttggcatttaaatggcactaaatatttttcaaagttcacagggttttgcccagaagatgttttcttctttaggaggaaactcttgtgaatttagaatctcatattatgaactaaaggtgcaaagagtttacacataaaattttgtcacaatcttgggctatcttctgaacactgcagaagataatcagaatattaaaatctgaaaaatgtaaagattctgaagc

SEQ ID NO: 12004 - RNA, 8146 nt, Homo sapiens
  source 1..8146: mol_type = other RNA
ctgaatagctgggactacaggtgtgtgccaccatgcccagctaatttttgtatttttagtagagacggggtttcaccgtgttggccaggatggtctctatctcttgacctcataatccgcccgcctcggcttcccaaagtgctgggattacaggtgtaagccactgtgcctgaccggaaactgtttcttaacatacatcatgcacgtaatcttcgctctcccaagaggcattcacccaagcagacaggcaagcatctatgtgttcaattcgaaatgcaacaatgacagatgtacaactttaccactcttaaagaaactaacatgccatccattattctccatgtgggaaacattcagtaaacttctaaaaccaaacacaggactctggcatatccccacacccccagcagcaggctgtgacaggctttgatctcaatcaaatgccactgtacacagaacataaaaacaggctcaggatgctgcatgtcactctgacatatcacattatttcatattactctgtcacttactcacaaacaaaagtctccactatggcatgattgagagagaaaataattcactttatataaataacagctaagaacaacatactgtgaacagtttccagagtttgaacattcagcacaatcaattcttacttcttgggaaaaaaatatcttacctatcttttctgttacagtatgccttcttggagaaaatattttagtggtaacatcattttctggggcatttggttaattttgaaagatgattatgccacatgaaccaaaaaaaaaaaaaaaaactggcaggaggaggagggtcctaggccattctggaagcaagctgggttttgcattattcagagtcaactattaagctgacttatattagaatggcgacagataagaggcaatgagtgacaccaggacatgcacagcacacagagaatatggtctactcttgtcttccctgcacagattaaacataagaggcttggtagaaagacatggggaaaggtgctatgggggccagcatttggaaagcatatatcccagtgacttgagtatttgctatgcaacctcctggacgagaaactgggaaaaggcacacttccgcccacagttgtggacagcagcagtcacccgtctgaatgctttcattcaatgtgaagatgcagcttgaacaaaagtttctttttgtttgtttgttttctgagatggagtctcgctctgtcacccaggctggagtgcagtggcacgatctcagctcactgcaacctctgcctcctgggttcaggcgattctcctgtctctgcctcccgagtagctgggaatagagggtgagccacaacacccggctaatttttgtatttttagtagagacggggtttcaccatattggccaggctggtcttgaactcctgacctcatgatccgtccgcctcagcctcccaaagtgctgggattacaggtgtgagccaccacgcctggccgaacaaaagttttttaatcttactgatcccatctttccagctgctctgaacagaggggcagggcggggaaagtcatgtcacagactctgcccacagcagccattctgaggtgccttttcagtctcttatcctcttttgagctttcctcttcttaattttttgttttgttttgttttcattgtactcattaatcccctcctcaatttttaacagaattataaaagcaaagtcaaaaggtccttcaggatgactgggaggcttcctaggctaacttttgcatttgaaaatggaaaaaataaattacttgatatttgtgataagactaagatttcttaaaagtctgcacatcaatatattacctggcttaggagggtgagggcacagtatccatctgcaccctctcctcgtattttttaaaaacaggcaaaatatgtaagaaaaggctggtgcacgttggaagacagagcgtgcctgtctatgccagtgctgctgtgccctgcagcctggcagatggagtcggatgctggggcctcatgcccacttaggccaataacatactcaagactctacagcccgttcaccagcaaagtatgccctgaggggcaacactggctgtggaagtgaagacacacaaagcagggactaaaggcaaatggggcttcacgatgcagcgacatgaagacagaactggtgtgggcgccaaaggcaacctgcagggctcacataaaaggaaaataggacagaaagccacgagttccacaagcagaatcatttctggtcttacatctgagggcatttgtagagaaaagtccaaggcaatgtcccctgggtctgagagaaaaatcctacgcaaaagagggcagacaatgcggtgctcgtcttgagggagcctgaccctgaccctgaccctgacgggctggatgcgagaggggctgagtatggctgtattcagtaaggaaactggtagcagacttttctagaaggtggaaagaaaaagcaaagactttcacagatacaaaaattgttttcaaaacaattacctagaaagttcactgcggttgggtggggaataagtgtaatattttcatttcaaatgagccatggtgctactaatggattataaaagaggatggccagttctggtcttccttcccttcccttaacccccgaaccttcctactcctgacattttccctaccctcactgcaacccacccccatcctggcccaaaattaatttgcccagccactgcaccaaaccagccttgacacacaattgttggttggatttcaattaaacaatgcacctaatgcgttggaagagaaggtggggagggcacaaggatgttggcgtaaacctggaggtgtgtggaccttggacagagcttccgccggccagacccagggcagggtgggcatctgcagtgcagcgcaggccgcaggtaaactgaggtaaggaagaacatggtggctctagctggccctgctttccgagacagtgcagcatgtgtgtgctcttgggtgtgggcaccaaaaaactcattttcttccagttgctgctgccattccaccctctgactagaagaatgctctttacagagtccaaaggatcagccacttggtcttcctctgaggtacaaatccaacagagctttaatcccaaagatccagtggccaccagagtacagaagtcagaatcaaatgctcagaatcaaaaggtgtggcactcctgcccagccggcttatcagcagttgtatagacagatcagaaaaaactagcatttattataaaaactgtttttcaaatggggtgatttcctgtccttctccagagatcataattcttcacgtttctgaggaccttctcggcttggttcttttgtcttctctttgtacagtgctcccgtttctttctccttctgaaagcggatctgtagctgtttgatctcttggtcgtagtcctgccactccgggacaatccgcacagctgcttccagtttcggctctttggtcatcggattattacacaaatcaatggtttttgcccttttcttagaggcgtcatcacaccacgtttcacaccaaagccattcttgagggagggatttaattggcacctgatgaatcatgttattgggcagatcttgatcaagatttgaaaggctgttagggtcctgactcagaccttggtactgtcccctgagtctgtcaccagcagctattttcctaaacttcttcagatccacaacatatagtgcactgatatgatactttcgcccggctaaatgactggcccagtaccctgacttccagaacctgtagccgtccatttctcttcggctgtcacagaaaggagtgtaaccataaggagcaccatccaaattgaaatctcttaactctttcagatctgttcgtacaatctgatcagcatccacaaacaggaacttgtcaacaactagtgggaaaagtacatccaggaagaggatcttgtaaccccagatgatacgctgtttttcagtttgttgatgaagccaccggggccatttgtactgaacaagctcatactggaaattgtattcatttgccatgtaaggtataaactccttaaatgtgggggacaagtaattcttcaagaaccagaatttcacaggagtcttggtattcttcagcacggatagcatcattatgcgaagaaatctttcgtagagatgaccagatgcaacggagaaaatattaattatgtcatctttatcttgcttcacttcctcagtcttctgtcctgtaaagccccatttgaaggaatcccaaaatccagattcattctcactcgttccatcactcagcaagtcttcgttcaccatatctgccttcttctgaaccttcactttaataattttgcttttgaagttgttgaggacgataaccacctcatcagcatcagggggagaatcagtgccatcgtggctgtaaattctataaatatcttcagagcgtcccttcctaagtctgaggatccaagctcctgggttggctttcagctgaaagtagcccagattggccataacaatggtgtccacaatgaccgggttggctgaagttcctaaggtaaactgtagtccccgtggaggctggcctgtggtgatgtcgtagcaatgaccttccagtaacaggtattccagctcatactcagcagccactacactgtccacctcttctaaataaatattatcaagatcatatggtgttctgacagattctaccatccagctctcaggtgtgttcaaattcagagtgaacagtggagactgaggcatatccaaaaattttgcgattggacccttagcaaaactattgtctgaagtgaaagaaatctctggttctaagacataacggtaaaagctttttaaaggcatgtcagaaagtttggattggcagttcataaatactctcagattcatgtttatcagctgagccaaaaccaagagcaaaggagcaagtctctgtgcttctctggtgacagggtcaacgacagccacaacatcaaagtatgtctccccttccttcggcctcagtttgattgcactgtgtctgtcttcaaaaaactggtactcgattcttggatctccttttggttgcgctgacagaagagcatccaccttcattaccaagtcgcttgccacatcttcttctacccgaagctgttgaatatgagattttattttctgtcctgaggtttttaagatgatattttcgaggaggtggaaatcgtcttgattaaagagctcactatcctccagtggcccaatgatccttccattgctgatcactgccctctgtcccttcttcagcttcagaacatccctgcagtacacggcatgagacaaaatgaaatccattttggaagactcaaagacctctttaaaaagactgaaatccattcccccaacagagaactccgcaatgtcagctcctgcagccagggcctctgcagccccctccttggccattttggtgatgaagttcttagcagcgttggaagtctgagtttggagagctgcccagattgctctggagatctgagtgttctcatagcttatctctttggcaggattattgatcatgcttattctaacattgttactggatttctgatgtttgatggcatcatacagtaactgccgtccagaagggctatcaaaatccccaacaatccaaaaagttactggcctaataaaagaatcatctttctttgtcagatagttcatactattggctacagcagcagtcttgccttgggaatccaagatagtaaatctagcataatcatccacaaagaagttattactcgctgttaaatccaggtagtctcgttcagctgtcaaaatcctagaattgattcgtggaacaacatttggctgattcatgatatactctaccacatcttgatcatggggcagttcacccaagtacaccgctctttggaagaaggtggtggtctccaggattttatgcattgtgatggtttctaactcatcagggtctagctgttccctttcaaagggcattccattgaacagcacaacgggcagaggtccaactccagtctgctcatagtagcctcttgcttccttccgattccgatcataagcagaatcaatccccaaaatgctattcacttctacatacggatatttcttctccaggacactgaccacatgttcaactttcactttttctccagtcctcaccttgttatagatatgtgtcagagtctggaaggcatgataatcatccacttcttgggcaacataattatatgctctaagaacagccactccagcatcttgcatcccatcaacatcttcagagtcattaaccacaaagataaaaccaattcttagtggtatatgattactaaggaacatctcagctgtgttcatcaactctgctgtggtctcatgtgcaggatcaactatgaaaaccatattatgtaagtttttcctgatctgccgaataacaccaggaaaggtgggtcgaagcaactcttgtaaactagaaggccacgaattatatctgctatcaacctccaggttgttgacccatgaaatagcaggactccggatgtctacggcatagtctgcctcagagggctggatgttcagcttcaaaacattatgcagagaaaggccttctattcccaatctatgcagaccctccattacccgagcttcattcctcaacacatcaaacagactgaatatatcctgtgtatctaaatccatgtgaagtccattgatgaagagggctgaatctccaggttgtaatcctaaagttcccttgaaatacttctgattctcttccacttcggttctaagttctgagctcacagctgtttttgttattgctctggctttggtaggaaaattctgactaagatccttcatgacaaccaaagccaactcaacaggagaagccaagattcgagcagcagtctggaaactgagatcttgcaactgccaaacctttaaaggtgccatttcattggtgctctctacaagatgctttctgagttctttcaactgtccctccaggtcggggtgcagatctcttaattttccaaagaggaacccctgaacctcatcaataggatcattttcaccaatcactgtggtgtttacctcagttcctttcacctgagtatcatccttggccttgtactcagtgctcttaatggccaattccacgccatagccagagaggtaaacaggctccttcctgggattaaatatataatgtctgaatacataattgattttgcctgcattgctttttgatataagctggcggtgaaaattggaaaattcctcagagccaatctcagagtagaaaatcaccacagggctttcaggattagacgagggatatctgtgatctcctttgaacaataaaggtttgggtctttcagaggctgtcagtagaagagcctcaagggtatcagattcacaagtcttctttccatgcactgaaaaaaacgaattacatccttctggtggaggttcatcagctgctatctgctggaaggcttggattgtagctgagtaagaacgaagggacagacaaaatttaaacaaattctgctggaggggtgacagaaactgaaatgcagcctccaatattgcatgatagtaggaataatcggtaccgtcatgatctgatgatccaatattttgactggcttctacaaaattccaaaatttctcttgactgtcttctgctaaaaactcactggcttctaacaacaatggagtggaaaaccattttgttgtaagagaggttgtaatggcttttgagtcggcctttactgaggagaacagccacagaacagtgagtacaaccagaactcccattttatagcaaactcctgtcaccggcagcgcacccgcggcacacgcaccgctcgcgtctcccttgcagcccatgcccgggccgtggtcagtccgccacagtgccagagacaacgccagggcagggcggggcgaggcggcagcggcagtgcaggctgcgccagtgagaggccgacacgcgcctttcccgcggctcgactcaacacccagcctcgcaaagcaattgcccagctgccggccgccctttt

SEQ ID NO: 12005 - RNA, 3246 nt, Homo sapiens
  source 1..3246: mol_type = other RNA
ctgaatagctgggactacaggtgtgtgccaccatgcccagctaatttttttttttttttgtatttttagtagaggcaggatttcaccatgttggccaggatggtcttgatctcttgacctcgtgatctgcccgccttggcctcccaacgtgctgggattacaggtgtgagccactgcgcctggcctattcaaaacattttctatgtccttttttaagttttgaagttttctccacagaggtattaatttttttgtgaatttctaggtacttttacatttttcattgagaggtacttatcttatgtttcttttattttttattttttattttttattttttttttgagacagagtcttgctctgttgtccaggctggagtgcagtggtgcgacctcagctcactgcaacctccacctcccaggttcaagcaattctccttcctcagcctcccgagtagctgggattacaggtgtgtgccaccatgcctggcttttttttttttttttttttgtatttttagtagagacgggatttcaccatgttagtcaggctggtctcaatctcctgacctcgtgatccgcccgcctcggcctcccaaagtgctgggattacaggcatgagccaccacccccagcccttatgtttctttattactggtgttcagaaatggtattaattttgtaggttgatcatgtggctggaaaatatgctaacttgtcattctaaaagtttgactctttattttgtgagttttgcaagtttatcatctcaccttcaaaaatctgtttttatttcttcctgtgatagtttttacacctcttattatgtctggaccattgtactatatatatatatattattttttcattgtactatattaaaactagtggtgacagtaatttcccctcaaattaggactgaaagtctcattttaaaaaaacccaaattcagcctgggcaacaaggcgaaaccccatctccactaaaaatacaaaaattagccagacatggtggcgcatgtctgtagtctcagctactcagaaggctgaggtgggaggactgtttgagcccaggaggcagaggctgcagtgagccaagatggtgccactgcactccagcctgggtgacagagtgctgtctacaaaaaacaaataacaaacaaaaaatgaaaaattggaaacaaaatgtaagtttataactttctgtcattaaaagtggatgatagtgtactcacttccacaacacatatactaaaatcagaatgatacagagagaaaagtggatgatggtttcttcggtttccttgaaaaaaagtgtttttaaactagataacccagccgggtgcgatggtgcactcctgtattcctagcactttgggaggctgtggcaggtggatggcgttaagtccaggagttggagaccagcctgggcaacatggcaaaacctcgtctctacaaaaaacacaaaaattggccaggctcggtggctcatgtctgtaatcccagcactttgggaggtcaaggcaggcggatcactggaggtcaggagttcaagaccagcctgggcaacgtggtgaaaccccgtctctactaaaaatacaaaagttagccaggcatggtggcacacgcctgtaatcccagctactcaggaggctgacacaggagaatcacttgaaccccaggaggtggaggttgcactgagctgagatcccgccactgcactccaccctgggtgacagtgcgagactcagtctcaaaaaaaaaaaattagccaggtgtggtggcgagcatctgtagtcctagctactcaggaggctgaggtgggaggatcacctgagcccaggaggtcaaggcttttgtgagccgtgactgtaccactgtattccagcctgggtgacagaatgagagctagtttcaaaaaaataaaagtggataacccccaaaaccactgtcctacttttagaaaatccaagatagttttgggaagggaattttggagtctcattggccatgaaagggactaggcaggcttctcagggagacttgtggggctgattacgtagtgcccagctctacttggaaaactctttttgcaacatttacatggaaatcagagacacagacccagatgttgggttaaaatgagacaaaggaaaaaaacagtcatgtacaagaggcaagaagaccacttttctaaatgatctatatttattagtactctggtcagagaaatcccaagtctaccatattggaggttttctggaattccaggctatctgttagactgtaggcttcaaaggcttggcttgtcatattgggccaggtttgtgcaggagataggcctacagctggaccagcaaagatgctgagagaggaaccctgtcctcctacctggtactttgtgggtgagagatactgatacagacagtggaaagaagagctggatatctcattctcatcaggaagattgtacagttctatgatttggaatatgtcataggcatcagagtacaaagcaggaaccgaggccaccagcctctcccactgagtatcttgcatttggaagtcactggtagaactctcagtgaaggtagagttccatgcccaattggaagggtctaagggctgagatggaagggagctgtagaaatctgaaatcacaggagaaaaagcataaggactgggggatgttctgggggaggtgggcacattcttcttggatggaaggatctggtttcgttgctttgctgattgctgctgctgctgcttcttcaatttgaatcgccggttcctgaaccaaacctttactgttgactccggtaggtcgagtctcaaagctagtttctcctgaagatttctatctgggaacatggtctggctaaacagagcttctagctcctcatactgttggtgggtgaaagaagtacgttctttatgccttctccgtattgctgtagtcgcagctactcgggaggctgaggtgggaggatcagttgaacctgggaggttgaggctgcagtaagccgagaccgtgccactgcactccagcttggataacagagtgaaactgggactagctggatcctgtggtggtatcaccttcatgttggaataattcctattgatgaaagggtctggctggggattctctggggccattctgttcctcatggtttctgaaatctgtcacgaatccccttagagtaaccattttcagtcctacgtggtgtgtctctctctggaaatgc

SEQ ID NO: 12006 - RNA, 2062 nt, Homo sapiens
  source 1..2062: mol_type = other RNA
ctgaatagctgggactacaggtgtgtgccaccatgcctggctaatttttgtatttttagtagagacggggtttcatgatgttggccaggctagtcttgaactcctgacctcaggtgatccacctgcctcggcctcccaaagtgctgagattacaggcgagagccaccacgcccggccaccactgccattttcatcacttaacccgaacacattcctctattccctccctttcctgcttggtgatcatcgactcttctgacccaactaggtgacctgctaaaccatctttactgttatttgccagaaaagactggaccagagacgtaaataatacacctcaatatacaacagctcgggcttaatttctaggcagaatttcatttgctggccatcagaagaatatatacatggagcgtgtttggggaggagatggagtaaggagaacacatcttggtggcaggagaacctggtgggaaccgtgctgatttgtttacttggatttgccaactggtccgatggatactgggtctgtttgcacttgagcatccaacatccgctttggtcccaggcctttaaagaagcccccaagggactgctgccgcttctcaggtctcttttggagcttgtccccattctgcagtgagttcgtgtccaccgtggcctgctctgtgcactgggctggttctttggcttcctgcttgttgctcttctgcttgttcatctcggctgctgacttcttgtccttcgaggagccctctttacccttctgtggtgctcctgttggttcaggctctggcggtgtgatagtcttttctgtggagtctgatgtattctcctccgcacctgtggggactgagtcctctttaactgactttttccaaaacagtttgcccagaggcagagaggtgggtcctgatttctccttggtgccttccttcgcaggttcaggggttgtcacggactgtgtgtgccccgatgggttgcatcctttggaattcttgccagccccttgggtctcctgggatgtaaagttggctttgtctgacttaaggtcagctgaagtggtgggtgacttttcagcacccgtgtcttctgggtccttttttgtttcagctttgttaggtgaaaccagagttttaaagaaactcatgatggaattattattctctgctatagctgctgcctgggaatcgtcctttgcagtctccagtccttctgggtccccagggacagagcaatccgcagttccaagttcttgtccttctttttccttgccgtcaactatgtccttccctgcagggacatcatcggactgccctgataagccaggaacctcatccaccttgtcttgatgctctgccctcttggcttcctgttggctgtcacctggcaccttttcctgtcccttgtccagcttgaagaatttgtcaaaaaagctggagtccttgggcttggagggagcttctcctcctgctccccctgtctcaggtgggagaagcgtgggatccctggcggcagagaggaccttgtcttgggccggggcgtgccctggggttttatctgtgtcctgccccggtccagctgccaccggaagtgtccagctctcacttgggtctttgttcgctggagctttattggagctgacatcaagcttcactgatccaagggatgaatctgcggcttggtctccggtacgtcctggtacaggccgagagagcatcaagaaaaaacgagatttagcagctggtgcctcgggtttggcctctttcccaagattctttccgttggcatccgcaacagcacttatctccgttgtctcgggggaagaagtggccacattatccgtcttgacacttattcccaagtcgacttcctctaagtgctgaactgtgtgggtcgacaccaccactggaaccccgttcagagcagacgcgttgtcctggtaagtctctgcttctggttcattctcttggtcttcaactctttggggaacactcatttggttacccattgctcaatcgtggcagaagacacctctccacaggacaccagaagaatgagt

SEQ ID NO: 12007 - RNA, 2178 nt, Homo sapiens
  source 1..2178: mol_type = other RNA
ctgaatagctgggactacaggtgtgtgccaccatgcctggctaatttttgtatttttagtagagacggggtttcatgatgttggccaggctagtcttgaactcctgacctcaggtgatccacctgcctcggcctcccaaagtgctgagattacaggcgagagccaccacgcccggccaccactgccattttcatcacttaacccgaacacattcctctattccctccctttcctgcttggtgatcatcgactcttctgacccaactaggtgacctgctaaaccatctttactgttatttgccagaaaagactggaccagagacgtaaataatacacctcaatatacaacagctcgggcttaatttctaggcagaatttcatttgctggccatcagaagaatatatacatggagcgtgtttggggaggagatggagtaaggagaacacatcttggtggcaggagaacctggtgggaaccgtgctgatttgtttacttggatttgccaactggtccgatggatactgggtctgtttgcacttgagcatccaacatccgctttggtcccaggcctttaaagaagcccccaagggactgctgccgcttctcaggtctcttttggagcttgtccccattctgcagtgagttcgtgtccaccgtggcctgctctgtgcactgggctggttctttggcttcctgcttgttgctcttctgcttgttcatctcggctgctgacttcttgtccttcgaggagccctctttacccttctgtggtgctcctgttggttcaggctctggcggtgtgatagtcttttctgtggagtctgatgtattctcctccgcacctgtggggactgagtcctctttaactgactttttccaaaacagtttgcccagaggcagagaggtgggtcctgatttctccttggtgccttccttcgcaggttcaggggttgtcacggactgtgtgtgccccgatgggttgcatcctttggaattcttgccagccccttgggtctcctgggatgtaaagttggctttgtctgacttaaggtcagctgaagtggtgggtgacttttcagcacccgtgtcttctgggtccttttttgtttcagctttgttaggtgaaaccagagttttaaagaaactcatgatggaattattattctctgctatagctgctgcctgggaatcgtcctttgcagtctccagtccttctgggtccccagggacagagcaatccgcagttccaagttcttgtccttctttttccttgccgtcaactatgtccttccctgcagggacatcatcggactgccctgataagccaggaacctcatccaccttgtcttgatgctctgccctcttggcttcctgttggctgtcacctggcaccttttcctgtcccttgtccagcttgaagaatttgtcaaaaaagctggagtccttgggcttggagggagcttctcctcctgctccccctgtctcaggtgggagaagcgtgggatccctggcggcagagaggaccttgtcttgggccggggcgtgccctggggttttatctgtgtcctgccccggtccagctgccaccggaagtgtccagctctcacttgggtctttgttcgctggagctttattggagctgacatcaagcttcactgatccaagggatgaatctgcggcttggtctccggtacgtcctggtacaggccgagagagcatcaagaaaaaacgagatttagcagctggtgcctcgggtttggcctctttcccaagattctttccgttggcatccgcaacagcacttatctccgttgtctcgggggaagaagtggccacattatccgtcttgacacttattcccaagtcgacttcctctaagtgctgaactgtgtgggtcgacaccaccactggaaccccgttcagagcagacgcgttgtcctggtaagtctctgcttctggttcattctcttggtcttcaactctttggggaacactcatttggttacccattgctcctgctgagcccctgtgggagtatcttcagtcccctcgtgtcacccggagctgctcctgcacagggtcctgggtctccagtgcgtgctgcccagtgcctggctgtcggtggagcctggctccctgcactttgcttccttgtgcagagcctgctggctgaatac

SEQ ID NO: 12008 - RNA, 2266 nt, Homo sapiens
  source 1..2266: mol_type = other RNA
ctgaatagctgggactacaggtgtgtgccaccatgcctggctaatttttgtatttttagtagagacggggtttcatgatgttggccaggctagtcttgaactcctgacctcaggtgatccacctgcctcggcctcccaaagtgctgagattacaggcgagagccaccacgcccggccaccactgccattttcatcacttaacccgaacacattcctctattccctccctttcctgcttggtgatcatcgactcttctgacccaactaggtgacctgctaaaccatctttactgttatttgccagaaaagactggaccagagacgtaaataatacacctcaatatacaacagctcgggcttaatttctaggcagaatttcatttgctggccatcagaagaatatatacatggagcgtgtttggggaggagatggagtaaggagaacacatcttggtggcaggagaacctggtgggaaccgtgctgatttgtttacttggatttgccaactggtccgatggatactgggtctgtttgcacttgagcatccaacatccgctttggtcccaggcctttaaagaagcccccaagggactgctgccgcttctcaggtctcttttggagcttgtccccattctgcagtgagttcgtgtccaccgtggcctgctctgtgcactgggctggttctttggcttcctgcttgttgctcttctgcttgttcatctcggctgctgacttcttgtccttcgaggagccctctttacccttctgtggtgctcctgttggttcaggctctggcggtgtgatagtcttttctgtggagtctgatgtattctcctccgcacctgtggggactgagtcctctttaactgactttttccaaaacagtttgcccagaggcagagaggtgggtcctgatttctccttggtgccttccttcgcaggttcaggggttgtcacggactgtgtgtgccccgatgggttgcatcctttggaattcttgccagccccttgggtctcctgggatgtaaagttggctttgtctgacttaaggtcagctgaagtggtgggtgacttttcagcacccttatgcctaaagaattttctaaaggcgagtcctagcctggggctatccaggtgctttttcttggtgcctctagcctggatctcggatgtcttctgaccagcttgtccatcacagacactttctgctttcgatgccgtgtcttctgggtccttttttgtttcagctttgttaggtgaaaccagagttttaaagaaactcatgatggaattattattctctgctatagctgctgcctgggaatcgtcctttgcagtctccagtccttctgggtccccagggacagagcaatccgcagttccaagttcttgtccttctttttccttgccgtcaactatgtccttccctgcagggacatcatcggactgccctgataagccaggaacctcatccaccttgtcttgatgctctgccctcttggcttcctgttggctgtcacctggcaccttttcctgtcccttgtccagcttgaagaatttgtcaaaaaagctggagtccttgggcttggagggagcttctcctcctgctccccctgtctcaggtgggagaagcgtgggatccctggcggcagagaggaccttgtcttgggccggggcgtgccctggggttttatctgtgtcctgccccggtccagctgccaccggaagtgtccagctctcacttgggtctttgttcgctggagctttattggagctgacatcaagcttcactgatccaagggatgaatctgcggcttggtctccggtacgtcctggtacaggccgagagagcatcaagaaaaaacgagatttagcagctggtgcctcgggtttggcctctttcccaagattctttccgttggcatccgcaacagcacttatctccgttgtctcgggggaagaagtggccacattatccgtcttgacacttattcccaagtcgacttcctctaagtgctgaactgtgtgggtcgacaccaccactggaaccccgttcagagcagacgcgttgtcctggtaagtctctgcttctggttcattctcttggtcttcaactctttggggaacactcatttggttacccattgctcctgctgagcccctgtgggagtatcttcagtcccctcgtgtcacccggagctgctcctgcacagggtcctgggtctccagtgcgtgctgcccagtgcctggctgtcggtggagcct

SEQ ID NO: 12009 - RNA, 2346 nt, Homo sapiens
  source 1..2346: mol_type = other RNA
ctgaatagctgggactacaggtgtgtgccaccatgcctggctaatttttgtatttttagtagagacggggtttcatgatgttggccaggctagtcttgaactcctgacctcaggtgatccacctgcctcggcctcccaaagtgctgagattacaggcgagagccaccacgcccggccaccactgccattttcatcacttaacccgaacacattcctctattccctccctttcctgcttggtgatcatcgactcttctgacccaactaggtgacctgctaaaccatctttactgttatttgccagaaaagactggaccagagacgtaaataatacacctcaatatacaacagctcgggcttaatttctaggcagaatttcatttgctggccatcagaagaatatatacatggagcgtgtttggggaggagatggagtaaggagaacacatcttggtggcaggagaacctggtgggaaccgtgctgatttgtttacttggatttgccaactggtccgatggatactgggtctgtttgcacttgagcatccaacatccgctttggtcccaggcctttaaagaagcccccaagggactgctgccgcttctcaggtctcttttggagcttgtccccattctgcagtgagttcgtgtccaccgtggcctgctctgtgcactgggctggttctttggcttcctgcttgttgctcttctgcttgttcatctcggctgctgacttcttgtccttcgaggagccctctttacccttctgtggtgctcctgttggttcaggctctggcggtgtgatagtcttttctgtggagtctgatgtcatttgtctgagaaacgccatcagagaggttcttggtttgctttcttctcttttgagtttcgcttctgtgggttcaggtgcagcatctccttcgttgaggtccactgtttgtaaggctgattctacttccttggactttataatctctactggtgactcacacaccacattctcctccgcacctgtggggactgagtcctctttaactgactttttccaaaacagtttgcccagaggcagagaggtgggtcctgatttctccttggtgccttccttcgcaggttcaggggttgtcacggactgtgtgtgccccgatgggttgcatcctttggaattcttgccagccccttgggtctcctgggatgtaaagttggctttgtctgacttaaggtcagctgaagtggtgggtgacttttcagcacccgtgtcttctgggtccttttttgtttcagctttgttaggtgaaaccagagttttaaagaaactcatgatggaattattattctctgctatagctgctgcctgggaatcgtcctttgcagtctccagtccttctgggtccccagggacagagcaatccgcagttccaagttcttgtccttctttttccttgccgtcaactatgtccttccctgcagggacatcatcggactgccctgataagccaggaacctcatccaccttgtcttgatgctctgccctcttggcttcctgttggctgtcacctggcaccttttcctgtcccttgtccagcttgaagaatttgtcaaaaaagctggagtccttgggcttggagggagcttctcctcctgctccccctgtctcaggtgggagaagcgtgggatccctggcggcagagaggaccttgtcttgggccggggcgtgccctggggttttatctgtgtcctgccccggtccagctgccaccggaagtgtccagctctcacttgggtctttgttcgctggagctttattggagctgacatcaagcttcactgatccaagggatgaatctgcggcttggtctccggtacgtcctggtacaggccgagagagcatcaagaaaaaacgagatttagcagctggtgcctcgggtttggcctctttcccaagattctttccgttggcatccgcaacagcacttatctccgttgtctcgggggaagaagtggccacattatccgtcttgacacttattcccaagtcgacttcctctaagtgctgaactgtgtgggtcgacaccaccactggaaccccgttcagagcagacgcgttgtcctggtaagtctctgcttctggttcattctcttggtcttcaactctttggggaacactcatttggttacccattgctcctgctgagcccctgtgggagtatcttcagtcccctcgtgtcacccggagctgctcctgcacagggtcctgggtctccagtgcgtgctgcccagtgcctggctgtcggtggagcctggctccctgcactttgcttccttgtgcagagcctgctggctgaatac

SEQ ID NO: 12010 - RNA, 2434 nt, Homo sapiens
  source 1..2434: mol_type = other RNA
ctgaatagctgggactacaggtgtgtgccaccatgcctggctaatttttgtatttttagtagagacggggtttcatgatgttggccaggctagtcttgaactcctgacctcaggtgatccacctgcctcggcctcccaaagtgctgagattacaggcgagagccaccacgcccggccaccactgccattttcatcacttaacccgaacacattcctctattccctccctttcctgcttggtgatcatcgactcttctgacccaactaggtgacctgctaaaccatctttactgttatttgccagaaaagactggaccagagacgtaaataatacacctcaatatacaacagctcgggcttaatttctaggcagaatttcatttgctggccatcagaagaatatatacatggagcgtgtttggggaggagatggagtaaggagaacacatcttggtggcaggagaacctggtgggaaccgtgctgatttgtttacttggatttgccaactggtccgatggatactgggtctgtttgcacttgagcatccaacatccgctttggtcccaggcctttaaagaagcccccaagggactgctgccgcttctcaggtctcttttggagcttgtccccattctgcagtgagttcgtgtccaccgtggcctgctctgtgcactgggctggttctttggcttcctgcttgttgctcttctgcttgttcatctcggctgctgacttcttgtccttcgaggagccctctttacccttctgtggtgctcctgttggttcaggctctggcggtgtgatagtcttttctgtggagtctgatgtcatttgtctgagaaacgccatcagagaggttcttggtttgctttcttctcttttgagtttcgcttctgtgggttcaggtgcagcatctccttcgttgaggtccactgtttgtaaggctgattctacttccttggactttataatctctactggtgactcacacaccacattctcctccgcacctgtggggactgagtcctctttaactgactttttccaaaacagtttgcccagaggcagagaggtgggtcctgatttctccttggtgccttccttcgcaggttcaggggttgtcacggactgtgtgtgccccgatgggttgcatcctttggaattcttgccagccccttgggtctcctgggatgtaaagttggctttgtctgacttaaggtcagctgaagtggtgggtgacttttcagcacccttatgcctaaagaattttctaaaggcgagtcctagcctggggctatccaggtgctttttcttggtgcctctagcctggatctcggatgtcttctgaccagcttgtccatcacagacactttctgctttcgatgccgtgtcttctgggtccttttttgtttcagctttgttaggtgaaaccagagttttaaagaaactcatgatggaattattattctctgctatagctgctgcctgggaatcgtcctttgcagtctccagtccttctgggtccccagggacagagcaatccgcagttccaagttcttgtccttctttttccttgccgtcaactatgtccttccctgcagggacatcatcggactgccctgataagccaggaacctcatccaccttgtcttgatgctctgccctcttggcttcctgttggctgtcacctggcaccttttcctgtcccttgtccagcttgaagaatttgtcaaaaaagctggagtccttgggcttggagggagcttctcctcctgctccccctgtctcaggtgggagaagcgtgggatccctggcggcagagaggaccttgtcttgggccggggcgtgccctggggttttatctgtgtcctgccccggtccagctgccaccggaagtgtccagctctcacttgggtctttgttcgctggagctttattggagctgacatcaagcttcactgatccaagggatgaatctgcggcttggtctccggtacgtcctggtacaggccgagagagcatcaagaaaaaacgagatttagcagctggtgcctcgggtttggcctctttcccaagattctttccgttggcatccgcaacagcacttatctccgttgtctcgggggaagaagtggccacattatccgtcttgacacttattcccaagtcgacttcctctaagtgctgaactgtgtgggtcgacaccaccactggaaccccgttcagagcagacgcgttgtcctggtaagtctctgcttctggttcattctcttggtcttcaactctttggggaacactcatttggttacccattgctcctgctgagcccctgtgggagtatcttcagtcccctcgtgtcacccggagctgctcctgcacagggtcctgggtctccagtgcgtgctgcccagtgcctggctgtcggtggagcct

SEQ ID NO: 12011 - RNA, 2257 nt, Homo sapiens
  source 1..2257: mol_type = other RNA
ctgaatagctgggactacaggtgtgtgccaccatgcctggctaatttttgtatttttagtagagacggggtttcatgatgttggccaggctagtcttgaactcctgacctcaggtgatccacctgcctcggcctcccaaagtgctgagattacaggcgagagccaccacgcccggccaccactgccattttcatcacttaacccgaacacattcctctattccctccctttcctgcttggtgatcatcgactcttctgacccaactaggtgacctgctaaaccatctttactgttatttgccagaaaagactggaccagagacgtaaataatacacctcaatatacaacagctcgggcttaatttctaggcagaatttcatttgctggccatcagaagaatatatacatggagcgtgtttggggaggagatggagtaaggagaacacatcttggtggcaggagaacctggtgggaaccgtgctgatttgtttacttggatttgccaactggtccgatggatactgggtctgtttgcacttgagcatccaacatccgctttggtcccaggcctttaaagaagcccccaagggactgctgccgcttctcaggtctcttttggagcttgtccccattctgcagtgagttcgtgtccaccgtggcctgctctgtgcactgggctggttctttggcttcctgcttgttgctcttctgcttgttcatctcggctgctgacttcttgtccttcgaggagccctctttacccttctgtggtgctcctgttggttcaggctctggcggtgtgatagtcttttctgtggagtctgatgtcatttgtctgagaaacgccatcagagaggttcttggtttgctttcttctcttttgagtttcgcttctgtgggttcaggtgcagcatctccttcgttgaggtccactgtttgtaaggctgattctacttccttggactttataatctctactggtgactcacacaccacctttttccaaaacagtttgcccagaggcagagaggtgggtcctgatttctccttggtgccttccttcgcaggttcaggggttgtcacggactgtgtgtgccccgatgggttgcatcctttggaattcttgccagccccttgggtctcctgggatgtaaagttggctttgtctgacttaaggtcagctgaagtggtgggtgacttttcagcacccgtgtcttctgggtccttttttgtttcagctttgttaggtgaaaccagagttttaaagaaactcatgatggaattattattctctgctatagctgctgcctgggaatcgtcctttgcagtctccagtccttctgggtccccagggacagagcaatccgcagttccaagttcttgtccttctttttccttgccgtcaactatgtccttccctgcagggacatcatcggactgccctgataagccaggaacctcatccaccttgtcttgatgctctgccctcttggcttcctgttggctgtcacctggcaccttttcctgtcccttgtccagcttgaagaatttgtcaaaaaagctggagtccttgggcttggagggagcttctcctcctgctccccctgtctcaggtgggagaagcgtgggatccctggcggcagagaggaccttgtcttgggccggggcgtgccctggggttttatctgtgtcctgccccggtccagctgccaccggaagtgtccagctctcacttgggtctttgttcgctggagctttattggagctgacatcaagcttcactgatccaagggatgaatctgcggcttggtctccggtacgtcctggtacaggccgagagagcatcaagaaaaaacgagatttagcagctggtgcctcgggtttggcctctttcccaagattctttccgttggcatccgcaacagcacttatctccgttgtctcgggggaagaagtggccacattatccgtcttgacacttattcccaagtcgacttcctctaagtgctgaactgtgtgggtcgacaccaccactggaaccccgttcagagcagacgcgttgtcctggtaagtctctgcttctggttcattctcttggtcttcaactctttggggaacactcatttggttacccattgctcctgctgagcccctgtgggagtatcttcagtcccctcgtgtcacccggagctgctcctgcacagggtcctgggtctccagtgcgtgctgcccagtgcctggctgtcggtggagcct

SEQ ID NO: 12012 - RNA, 2392 nt, Homo sapiens
  source 1..2392: mol_type = other RNA
ctgaatagctgggactacaggtgtgtgccaccatgcctggctaatttttgtatttttagtagagacggggtttcatgatgttggccaggctagtcttgaactcctgacctcaggtgatccacctgcctcggcctcccaaagtgctgagattacaggcgagagccaccacgcccggccaccactgccattttcatcacttaacccgaacacattcctctattccctccctttcctgcttggtgatcatcgactcttctgacccaactaggtgacctgctaaaccatctttactgttatttgccagaaaagactggaccagagacgtaaataatacacctcaatatacaacagctcgggcttaatttctaggcagaatttcatttgctggccatcagaagaatatatacatggagcgtgtttggggaggagatggagtaaggagaacacatcttggtggcaggagaacctggtgggaaccgtgctgatttgtttacttggatttgccaactggtccgatggatactgggtctgtttgcacttgagcatccaacatccgctttggtcccaggcctttaaagaagcccccaagggactgctgccgcttctcaggtctcttttggagcttgtccccattctgcagtgagttcgtgtccaccgtggcctgctctgtgcactgggctggttctttggcttcctgcttgttgctcttctgcttgttcatctcggctgctgacttcttgtccttcgaggagccctctttacccttctgtggtgctcctgttggttcaggctctggcggtgtgatagtcttttctgtggagtctgatgtcatttgtctgagaaacgccatcagagaggttcttggtttgctttcttctcttttgagtttcgcttctgtgggttcaggtgcagcatctccttcgttgaggtccactgtttgtaaggctgattctacttccttggactttataatctctactggtgactcacacaccacctttttccaaaacagtttgcccagaggcagagaggtgggtcctgatttctccttggtgccttccttcgcaggttcaggggttgtcacggactgtgtgtgccccgatgggttgcatcctttggaattcttgccagccccttgggtctcctgggatgtaaagttggctttgtctgacttaaggtcagctgaagtggtgggtgacttttcagcacccttatgcctaaagaattttctaaaggcgagtcctagcctggggctatccaggtgctttttcttggtgcctctagcctggatctcggatgtcttctgaccagcttgtccatcacagacactttctgctttcgatgccgtgtcttctgggtccttttttgtttcagctttgttaggtgaaaccagagttttaaagaaactcatgatggaattattattctctgctatagctgctgcctgggaatcgtcctttgcagtctccagtccttctgggtccccagggacagagcaatccgcagttccaagttcttgtccttctttttccttgccgtcaactatgtccttccctgcagggacatcatcggactgccctgataagccaggaacctcatccaccttgtcttgatgctctgccctcttggcttcctgttggctgtcacctggcaccttttcctgtcccttgtccagcttgaagaatttgtcaaaaaagctggagtccttgggcttggagggagcttctcctcctgctccccctgtctcaggtgggagaagcgtgggatccctggcggcagagaggaccttgtcttgggccggggcgtgccctggggttttatctgtgtcctgccccggtccagctgccaccggaagtgtccagctctcacttgggtctttgttcgctggagctttattggagctgacatcaagcttcactgatccaagggatgaatctgcggcttggtctccggtacgtcctggtacaggccgagagagcatcaagaaaaaacgagatttagcagctggtgcctcgggtttggcctctttcccaagattctttccgttggcatccgcaacagcacttatctccgttgtctcgggggaagaagtggccacattatccgtcttgacacttattcccaagtcgacttcctctaagtgctgaactgtgtgggtcgacaccaccactggaaccccgttcagagcagacgcgttgtcctggtaagtctctgcttctggttcattctcttggtcttcaactctttggggaacactcatttggttacccattgctcctgctgagcccctgtgggagtatcttcagtcccctcgtgtcacccggagctgctcctgcacagggtcctgggtctccagtgcgtgctgcccagtgcctggctgtcggtggagcct

SEQ ID NO: 12013 - RNA, 2136 nt, Homo sapiens
  source 1..2136: mol_type = other RNA
ctgaatagctgggactacaggtgtgtgccaccatgcctggctaatttttgtatttttagtagagacggggtttcatgatgttggccaggctagtcttgaactcctgacctcaggtgatccacctgcctcggcctcccaaagtgctgagattacaggcgagagccaccacgcccggccaccactgccattttcatcacttaacccgaacacattcctctattccctccctttcctgcttggtgatcatcgactcttctgacccaactaggtgacctgctaaaccatctttactgttatttgccagaaaagactggaccagagacgtaaataatacacctcaatatacaacagctcgggcttaatttctaggcagaatttcatttgctggccatcagaagaatatatacatggagcgtgtttggggaggagatggagtaaggagaacacatcttggtggcaggagaacctggtgggaaccgtgctgatttgtttacttggatttgccaactggtccgatggatactgggtctgtttgcacttgagcatccaacatccgctttggtcccaggcctttaaagaagcccccaagggactgctgccgcttctcaggtctcttttggagcttgtccccattctgcagtgagttcgtgtccaccgtggcctgctctgtgcactgggctggttctttggcttcctgcttgttgctcttctgcttgttcatctcggctgctgacttcttgtccttcgaggagccctctttacccttctgtggtgctcctgttggttcaggctctggcggtgtgatagtcttttctgtggagtctgatgtctttttccaaaacagtttgcccagaggcagagaggtgggtcctgatttctccttggtgccttccttcgcaggttcaggggttgtcacggactgtgtgtgccccgatgggttgcatcctttggaattcttgccagccccttgggtctcctgggatgtaaagttggctttgtctgacttaaggtcagctgaagtggtgggtgacttttcagcacccgtgtcttctgggtccttttttgtttcagctttgttaggtgaaaccagagttttaaagaaactcatgatggaattattattctctgctatagctgctgcctgggaatcgtcctttgcagtctccagtccttctgggtccccagggacagagcaatccgcagttccaagttcttgtccttctttttccttgccgtcaactatgtccttccctgcagggacatcatcggactgccctgataagccaggaacctcatccaccttgtcttgatgctctgccctcttggcttcctgttggctgtcacctggcaccttttcctgtcccttgtccagcttgaagaatttgtcaaaaaagctggagtccttgggcttggagggagcttctcctcctgctccccctgtctcaggtgggagaagcgtgggatccctggcggcagagaggaccttgtcttgggccggggcgtgccctggggttttatctgtgtcctgccccggtccagctgccaccggaagtgtccagctctcacttgggtctttgttcgctggagctttattggagctgacatcaagcttcactgatccaagggatgaatctgcggcttggtctccggtacgtcctggtacaggccgagagagcatcaagaaaaaacgagatttagcagctggtgcctcgggtttggcctctttcccaagattctttccgttggcatccgcaacagcacttatctccgttgtctcgggggaagaagtggccacattatccgtcttgacacttattcccaagtcgacttcctctaagtgctgaactgtgtgggtcgacaccaccactggaaccccgttcagagcagacgcgttgtcctggtaagtctctgcttctggttcattctcttggtcttcaactctttggggaacactcatttggttacccattgctcctgctgagcccctgtgggagtatcttcagtcccctcgtgtcacccggagctgctcctgcacagggtcctgggtctccagtgcgtgctgcccagtgcctggctgtcggtggagcctggctccctgcactttgcttccttgtgcagagcctgctggctgaatac

SEQ ID NO: 12014 - RNA, 2224 nt, Homo sapiens
  source 1..2224: mol_type = other RNA
ctgaatagctgggactacaggtgtgtgccaccatgcctggctaatttttgtatttttagtagagacggggtttcatgatgttggccaggctagtcttgaactcctgacctcaggtgatccacctgcctcggcctcccaaagtgctgagattacaggcgagagccaccacgcccggccaccactgccattttcatcacttaacccgaacacattcctctattccctccctttcctgcttggtgatcatcgactcttctgacccaactaggtgacctgctaaaccatctttactgttatttgccagaaaagactggaccagagacgtaaataatacacctcaatatacaacagctcgggcttaatttctaggcagaatttcatttgctggccatcagaagaatatatacatggagcgtgtttggggaggagatggagtaaggagaacacatcttggtggcaggagaacctggtgggaaccgtgctgatttgtttacttggatttgccaactggtccgatggatactgggtctgtttgcacttgagcatccaacatccgctttggtcccaggcctttaaagaagcccccaagggactgctgccgcttctcaggtctcttttggagcttgtccccattctgcagtgagttcgtgtccaccgtggcctgctctgtgcactgggctggttctttggcttcctgcttgttgctcttctgcttgttcatctcggctgctgacttcttgtccttcgaggagccctctttacccttctgtggtgctcctgttggttcaggctctggcggtgtgatagtcttttctgtggagtctgatgtctttttccaaaacagtttgcccagaggcagagaggtgggtcctgatttctccttggtgccttccttcgcaggttcaggggttgtcacggactgtgtgtgccccgatgggttgcatcctttggaattcttgccagccccttgggtctcctgggatgtaaagttggctttgtctgacttaaggtcagctgaagtggtgggtgacttttcagcacccttatgcctaaagaattttctaaaggcgagtcctagcctggggctatccaggtgctttttcttggtgcctctagcctggatctcggatgtcttctgaccagcttgtccatcacagacactttctgctttcgatgccgtgtcttctgggtccttttttgtttcagctttgttaggtgaaaccagagttttaaagaaactcatgatggaattattattctctgctatagctgctgcctgggaatcgtcctttgcagtctccagtccttctgggtccccagggacagagcaatccgcagttccaagttcttgtccttctttttccttgccgtcaactatgtccttccctgcagggacatcatcggactgccctgataagccaggaacctcatccaccttgtcttgatgctctgccctcttggcttcctgttggctgtcacctggcaccttttcctgtcccttgtccagcttgaagaatttgtcaaaaaagctggagtccttgggcttggagggagcttctcctcctgctccccctgtctcaggtgggagaagcgtgggatccctggcggcagagaggaccttgtcttgggccggggcgtgccctggggttttatctgtgtcctgccccggtccagctgccaccggaagtgtccagctctcacttgggtctttgttcgctggagctttattggagctgacatcaagcttcactgatccaagggatgaatctgcggcttggtctccggtacgtcctggtacaggccgagagagcatcaagaaaaaacgagatttagcagctggtgcctcgggtttggcctctttcccaagattctttccgttggcatccgcaacagcacttatctccgttgtctcgggggaagaagtggccacattatccgtcttgacacttattcccaagtcgacttcctctaagtgctgaactgtgtgggtcgacaccaccactggaaccccgttcagagcagacgcgttgtcctggtaagtctctgcttctggttcattctcttggtcttcaactctttggggaacactcatttggttacccattgctcctgctgagcccctgtgggagtatcttcagtcccctcgtgtcacccggagctgctcctgcacagggtcctgggtctccagtgcgtgctgcccagtgcctggctgtcggtggagcct

SEQ ID NO: 12015 - RNA, 2332 nt, Homo sapiens
  source 1..2332: mol_type = other RNA
ctgaatagctgggactacaggtgtgtgccaccatgcctggctaatttttgtatttttagtagagacggggtttcatgatgttggccaggctagtcttgaactcctgacctcaggtgatccacctgcctcggcctcccaaagtgctgagattacaggcgagagccaccacgcccggccaccactgccattttcatcacttaacccgaacacattcctctattccctccctttcctgcttggtgatcatcgactcttctgacccaactaggtgacctgctaaaccatctttactgttatttgccagaaaagactggaccagagacgtaaataatacacctcaatatacaacagctcgggcttaatttctaggcagaatttcatttgctggccatcagaagaatatatacatggagcgtgtttggggaggagatggagtaaggagaacacatcttggtggcaggagaacctggtgggaaccgtgctgatttgtttacttggatttgccaactggtccgatggatactgggtctgtttgcacttgagcatccaacatccgctttggtcccaggcctttaaagaagcccccaagggactgctgccgcttctcaggtctcttttggagcttgtccccattctgcagtgagttcgtgtccaccgtggcctgctctgtgcactgggctggttctttggcttcctgcttgttgctcttctgcttgttcatctcggctgctgacttcttgtccttcgaggagccctctttacccttctgtggtgctcctgttggttcaggctctggcggtgtgatagtcttttctgtggagtctgatgtttggcagctggagtctttcccatttatttcttctgagtgggtgatccctccatcccctttcactgaattctcctccgcacctgtggggactgagtcctctttaactgactttttccaaaacagtttgcccagaggcagagaggtgggtcctgatttctccttggtgccttccttcgcaggttcaggggttgtcacggactgtgtgtgccccgatgggttgcatcctttggaattcttgccagccccttgggtctcctgggatgtaaagttggctttgtctgacttaaggtcagctgaagtggtgggtgacttttcagcacccttatgcctaaagaattttctaaaggcgagtcctagcctggggctatccaggtgctttttcttggtgcctctagcctggatctcggatgtcttctgaccagcttgtccatcacagacactttctgctttcgatgccgtgtcttctgggtccttttttgtttcagctttgttaggtgaaaccagagttttaaagaaactcatgatggaattattattctctgctatagctgctgcctgggaatcgtcctttgcagtctccagtccttctgggtccccagggacagagcaatccgcagttccaagttcttgtccttctttttccttgccgtcaactatgtccttccctgcagggacatcatcggactgccctgataagccaggaacctcatccaccttgtcttgatgctctgccctcttggcttcctgttggctgtcacctggcaccttttcctgtcccttgtccagcttgaagaatttgtcaaaaaagctggagtccttgggcttggagggagcttctcctcctgctccccctgtctcaggtgggagaagcgtgggatccctggcggcagagaggaccttgtcttgggccggggcgtgccctggggttttatctgtgtcctgccccggtccagctgccaccggaagtgtccagctctcacttgggtctttgttcgctggagctttattggagctgacatcaagcttcactgatccaagggatgaatctgcggcttggtctccggtacgtcctggtacaggccgagagagcatcaagaaaaaacgagatttagcagctggtgcctcgggtttggcctctttcccaagattctttccgttggcatccgcaacagcacttatctccgttgtctcgggggaagaagtggccacattatccgtcttgacacttattcccaagtcgacttcctctaagtgctgaactgtgtgggtcgacaccaccactggaaccccgttcagagcagacgcgttgtcctggtaagtctctgcttctggttcattctcttggtcttcaactctttggggaacactcatttggttacccattgctcctgctgagcccctgtgggagtatcttcagtcccctcgtgtcacccggagctgctcctgcacagggtcctgggtctccagtgcgtgctgcccagtgcctggctgtcggtggagcct

SEQ ID NO: 12016 - RNA, 2412 nt, Homo sapiens
  source 1..2412: mol_type = other RNA
ctgaatagctgggactacaggtgtgtgccaccatgcctggctaatttttgtatttttagtagagacggggtttcatgatgttggccaggctagtcttgaactcctgacctcaggtgatccacctgcctcggcctcccaaagtgctgagattacaggcgagagccaccacgcccggccaccactgccattttcatcacttaacccgaacacattcctctattccctccctttcctgcttggtgatcatcgactcttctgacccaactaggtgacctgctaaaccatctttactgttatttgccagaaaagactggaccagagacgtaaataatacacctcaatatacaacagctcgggcttaatttctaggcagaatttcatttgctggccatcagaagaatatatacatggagcgtgtttggggaggagatggagtaaggagaacacatcttggtggcaggagaacctggtgggaaccgtgctgatttgtttacttggatttgccaactggtccgatggatactgggtctgtttgcacttgagcatccaacatccgctttggtcccaggcctttaaagaagcccccaagggactgctgccgcttctcaggtctcttttggagcttgtccccattctgcagtgagttcgtgtccaccgtggcctgctctgtgcactgggctggttctttggcttcctgcttgttgctcttctgcttgttcatctcggctgctgacttcttgtccttcgaggagccctctttacccttctgtggtgctcctgttggttcaggctctggcggtgtgatagtcttttctgtggagtctgatgtttggcagctggagtctttcccatttatttcttctgagtgggtgatccctccatcccctttcactgacatttgtctgagaaacgccatcagagaggttcttggtttgctttcttctcttttgagtttcgcttctgtgggttcaggtgcagcatctccttcgttgaggtccactgtttgtaaggctgattctacttccttggactttataatctctactggtgactcacacaccacattctcctccgcacctgtggggactgagtcctctttaactgactttttccaaaacagtttgcccagaggcagagaggtgggtcctgatttctccttggtgccttccttcgcaggttcaggggttgtcacggactgtgtgtgccccgatgggttgcatcctttggaattcttgccagccccttgggtctcctgggatgtaaagttggctttgtctgacttaaggtcagctgaagtggtgggtgacttttcagcacccgtgtcttctgggtccttttttgtttcagctttgttaggtgaaaccagagttttaaagaaactcatgatggaattattattctctgctatagctgctgcctgggaatcgtcctttgcagtctccagtccttctgggtccccagggacagagcaatccgcagttccaagttcttgtccttctttttccttgccgtcaactatgtccttccctgcagggacatcatcggactgccctgataagccaggaacctcatccaccttgtcttgatgctctgccctcttggcttcctgttggctgtcacctggcaccttttcctgtcccttgtccagcttgaagaatttgtcaaaaaagctggagtccttgggcttggagggagcttctcctcctgctccccctgtctcaggtgggagaagcgtgggatccctggcggcagagaggaccttgtcttgggccggggcgtgccctggggttttatctgtgtcctgccccggtccagctgccaccggaagtgtccagctctcacttgggtctttgttcgctggagctttattggagctgacatcaagcttcactgatccaagggatgaatctgcggcttggtctccggtacgtcctggtacaggccgagagagcatcaagaaaaaacgagatttagcagctggtgcctcgggtttggcctctttcccaagattctttccgttggcatccgcaacagcacttatctccgttgtctcgggggaagaagtggccacattatccgtcttgacacttattcccaagtcgacttcctctaagtgctgaactgtgtgggtcgacaccaccactggaaccccgttcagagcagacgcgttgtcctggtaagtctctgcttctggttcattctcttggtcttcaactctttggggaacactcatttggttacccattgctcctgctgagcccctgtgggagtatcttcagtcccctcgtgtcacccggagctgctcctgcacagggtcctgggtctccagtgcgtgctgcccagtgcctggctgtcggtggagcctggctccctgcactttgcttccttgtgcagagcctgctggctgaatac

SEQ ID NO: 12017 - RNA, 2426 nt, Homo sapiens
  source 1..2426: mol_type = other RNA
ctgaatagctgggactacaggtgtgtgccaccatgcctggctaatttttgtatttttagtagagacggggtttcatgatgttggccaggctagtcttgaactcctgacctcaggtgatccacctgcctcggcctcccaaagtgctgagattacaggcgagagccaccacgcccggccaccactgccattttcatcacttaacccgaacacattcctctattccctccctttcctgcttggtgatcatcgactcttctgacccaactaggtgacctgctaaaccatctttactgttatttgccagaaaagactggaccagagacgtaaataatacacctcaatatacaacagctcgggcttaatttctaggcagaatttcatttgctggccatcagaagaatatatacatggagcgtgtttggggaggagatggagtaaggagaacacatcttggtggcaggagaacctggtgggaaccgtgctgatttgtttacttggatttgccaactggtccgatggatactgggtctgtttgcacttgagcatccaacatccgctttggtcccaggcctttaaagaagcccccaagggactgctgccgcttctcaggtctcttttggagcttgtccccattctgcagtgagttcgtgtccaccgtggcctgctctgtgcactgggctggttctttggcttcctgcttgttgctcttctgcttgttcatctcggctgctgacttcttgtccttcgaggagccctctttacccttctgtggtgctcctgttggttcaggctctggcggtgtgatagtcttttctgtggagtctgatgtttggcagctggagtctttcccatttatttcttctgagtgggtgatccctccatcccctttcactgacatttgtctgagaaacgccatcagagaggttcttggtttgctttcttctcttttgagtttcgcttctgtgggttcaggtgcagcatctccttcgttgaggtccactgtttgtaaggctgattctacttccttggactttataatctctactggtgactcacacaccacattctcctccgcacctgtggggactgagtcctctttaactgactttttccaaaacagtttgcccagaggcagagaggtgggtcctgatttctccttggtgccttccttcgcaggttcaggggttgtcacggactgtgtgtgccccgatgggttgcatcctttggaattcttgccagccccttgggtctcctgggatgtaaagttggctttgtctgacttaaggtcagctgaagtggtgggtgacttttcagcacccttatgcctaaagaattttctaaaggcgagtcctagcctggggctatccaggtgctttttcttggtgcctctagcctggatctcggatgtcttctgaccagcttgtccatcacagacactttctgctttcgatgccgtgtcttctgggtccttttttgtttcagctttgttaggtgaaaccagagttttaaagaaactcatgatggaattattattctctgctatagctgctgcctgggaatcgtcctttgcagtctccagtccttctgggtccccagggacagagcaatccgcagttccaagttcttgtccttctttttccttgccgtcaactatgtccttccctgcagggacatcatcggactgccctgataagccaggaacctcatccaccttgtcttgatgctctgccctcttggcttcctgttggctgtcacctggcaccttttcctgtcccttgtccagcttgaagaatttgtcaaaaaagctggagtccttgggcttggagggagcttctcctcctgctccccctgtctcaggtgggagaagcgtgggatccctggcggcagagaggaccttgtcttgggccggggcgtgccctggggttttatctgtgtcctgccccggtccagctgccaccggaagtgtccagctctcacttgggtctttgttcgctggagctttattggagctgacatcaagcttcactgatccaagggatgaatctgcggcttggtctccggtacgtcctggtacaggccgagagagcatcaagaaaaaacgagatttagcagctggtgcctcgggtttggcctctttcccaagattctttccgttggcatccgcaacagcacttatctccgttgtctcgggggaagaagtggccacattatccgtcttgacacttattcccaagtcgacttcctctaagtgctgaactgtgtgggtcgacaccaccactggaaccccgttcagagcagacgcgttgtcctggtaagtctctgcttctggttcattctcttggtcttcaactctttggggaacactcatttggttacccattgctcaatcgtggcagaagacacctctccacaggacaccagaagaa

SEQ ID NO: 12018 - RNA, 2547 nt, Homo sapiens
  source 1..2547: mol_type = other RNA
ctgaatagctgggactacaggtgtgtgccaccatgcctggctaatttttgtatttttagtagagacggggtttcatgatgttggccaggctagtcttgaactcctgacctcaggtgatccacctgcctcggcctcccaaagtgctgagattacaggcgagagccaccacgcccggccaccactgccattttcatcacttaacccgaacacattcctctattccctccctttcctgcttggtgatcatcgactcttctgacccaactaggtgacctgctaaaccatctttactgttatttgccagaaaagactggaccagagacgtaaataatacacctcaatatacaacagctcgggcttaatttctaggcagaatttcatttgctggccatcagaagaatatatacatggagcgtgtttggggaggagatggagtaaggagaacacatcttggtggcaggagaacctggtgggaaccgtgctgatttgtttacttggatttgccaactggtccgatggatactgggtctgtttgcacttgagcatccaacatccgctttggtcccaggcctttaaagaagcccccaagggactgctgccgcttctcaggtctcttttggagcttgtccccattctgcagtgagttcgtgtccaccgtggcctgctctgtgcactgggctggttctttggcttcctgcttgttgctcttctgcttgttcatctcggctgctgacttcttgtccttcgaggagccctctttacccttctgtggtgctcctgttggttcaggctctggcggtgtgatagtcttttctgtggagtctgatgtttggcagctggagtctttcccatttatttcttctgagtgggtgatccctccatcccctttcactgacatttgtctgagaaacgccatcagagaggttcttggtttgctttcttctcttttgagtttcgcttctgtgggttcaggtgcagcatctccttcgttgaggtccactgtttgtaaggctgattctacttccttggactttataatctctactggtgactcacacaccacattctcctccgcacctgtggggactgagtcctctttaactgactttttccaaaacagtttgcccagaggcagagaggtgggtcctgatttctccttggtgccttccttcgcaggttcaggggttgtcacggactgtgtgtgccccgatgggttgcatcctttggaattcttgccagccccttgggtctcctgggatgtaaagttggctttgtctgacttaaggtcagctgaagtggtgggtgacttttcagcacccttatgcctaaagaattttctaaaggcgagtcctagcctggggctatccaggtgctttttcttggtgcctctagcctggatctcggatgtcttctgaccagcttgtccatcacagacactttctgctttcgatgccgtgtcttctgggtccttttttgtttcagctttgttaggtgaaaccagagttttaaagaaactcatgatggaattattattctctgctatagctgctgcctgggaatcgtcctttgcagtctccagtccttctgggtccccagggacagagcaatccgcagttccaagttcttgtccttctttttccttgccgtcaactatgtccttccctgcagggacatcatcggactgccctgataagccaggaacctcatccaccttgtcttgatgctctgccctcttggcttcctgttggctgtcacctggcaccttttcctgtcccttgtccagcttgaagaatttgtcaaaaaagctggagtccttgggcttggagggagcttctcctcctgctccccctgtctcaggtgggagaagcgtgggatccctggcggcagagaggaccttgtcttgggccggggcgtgccctggggttttatctgtgtcctgccccggtccagctgccaccggaagtgtccagctctcacttgggtctttgttcgctggagctttattggagctgacatcaagcttcactgatccaagggatgaatctgcggcttggtctccggtacgtcctggtacaggccgagagagcatcaagaaaaaacgagatttagcagctggtgcctcgggtttggcctctttcccaagattctttccgttggcatccgcaacagcacttatctccgttgtctcgggggaagaagtggccacattatccgtcttgacacttattcccaagtcgacttcctctaagtgctgaactgtgtgggtcgacaccaccactggaaccccgttcagagcagacgcgttgtcctggtaagtctctgcttctggttcattctcttggtcttcaactctttggggaacactcatttggttacccattgctcctgctgagcccctgtgggagtatcttcagtcccctcgtgtcacccggagctgctcctgcacagggtcctgggtctccagtgcgtgctgcccagtgcctggctgtcggtggagcctggctccctgcactttgcttccttgtgcagagcctgctggctgaatac

SEQ ID NO: 12019 - RNA, 2370 nt, Homo sapiens
  source 1..2370: mol_type = other RNA
ctgaatagctgggactacaggtgtgtgccaccatgcctggctaatttttgtatttttagtagagacggggtttcatgatgttggccaggctagtcttgaactcctgacctcaggtgatccacctgcctcggcctcccaaagtgctgagattacaggcgagagccaccacgcccggccaccactgccattttcatcacttaacccgaacacattcctctattccctccctttcctgcttggtgatcatcgactcttctgacccaactaggtgacctgctaaaccatctttactgttatttgccagaaaagactggaccagagacgtaaataatacacctcaatatacaacagctcgggcttaatttctaggcagaatttcatttgctggccatcagaagaatatatacatggagcgtgtttggggaggagatggagtaaggagaacacatcttggtggcaggagaacctggtgggaaccgtgctgatttgtttacttggatttgccaactggtccgatggatactgggtctgtttgcacttgagcatccaacatccgctttggtcccaggcctttaaagaagcccccaagggactgctgccgcttctcaggtctcttttggagcttgtccccattctgcagtgagttcgtgtccaccgtggcctgctctgtgcactgggctggttctttggcttcctgcttgttgctcttctgcttgttcatctcggctgctgacttcttgtccttcgaggagccctctttacccttctgtggtgctcctgttggttcaggctctggcggtgtgatagtcttttctgtggagtctgatgtttggcagctggagtctttcccatttatttcttctgagtgggtgatccctccatcccctttcactgacatttgtctgagaaacgccatcagagaggttcttggtttgctttcttctcttttgagtttcgcttctgtgggttcaggtgcagcatctccttcgttgaggtccactgtttgtaaggctgattctacttccttggactttataatctctactggtgactcacacaccacctttttccaaaacagtttgcccagaggcagagaggtgggtcctgatttctccttggtgccttccttcgcaggttcaggggttgtcacggactgtgtgtgccccgatgggttgcatcctttggaattcttgccagccccttgggtctcctgggatgtaaagttggctttgtctgacttaaggtcagctgaagtggtgggtgacttttcagcacccgtgtcttctgggtccttttttgtttcagctttgttaggtgaaaccagagttttaaagaaactcatgatggaattattattctctgctatagctgctgcctgggaatcgtcctttgcagtctccagtccttctgggtccccagggacagagcaatccgcagttccaagttcttgtccttctttttccttgccgtcaactatgtccttccctgcagggacatcatcggactgccctgataagccaggaacctcatccaccttgtcttgatgctctgccctcttggcttcctgttggctgtcacctggcaccttttcctgtcccttgtccagcttgaagaatttgtcaaaaaagctggagtccttgggcttggagggagcttctcctcctgctccccctgtctcaggtgggagaagcgtgggatccctggcggcagagaggaccttgtcttgggccggggcgtgccctggggttttatctgtgtcctgccccggtccagctgccaccggaagtgtccagctctcacttgggtctttgttcgctggagctttattggagctgacatcaagcttcactgatccaagggatgaatctgcggcttggtctccggtacgtcctggtacaggccgagagagcatcaagaaaaaacgagatttagcagctggtgcctcgggtttggcctctttcccaagattctttccgttggcatccgcaacagcacttatctccgttgtctcgggggaagaagtggccacattatccgtcttgacacttattcccaagtcgacttcctctaagtgctgaactgtgtgggtcgacaccaccactggaaccccgttcagagcagacgcgttgtcctggtaagtctctgcttctggttcattctcttggtcttcaactctttggggaacactcatttggttacccattgctcctgctgagcccctgtgggagtatcttcagtcccctcgtgtcacccggagctgctcctgcacagggtcctgggtctccagtgcgtgctgcccagtgcctggctgtcggtggagcctggctccctgcactttgcttccttgtgcagagcctgctggctgaatac

SEQ ID NO: 12020 - RNA, 2458 nt, Homo sapiens
  source 1..2458: mol_type = other RNA
ctgaatagctgggactacaggtgtgtgccaccatgcctggctaatttttgtatttttagtagagacggggtttcatgatgttggccaggctagtcttgaactcctgacctcaggtgatccacctgcctcggcctcccaaagtgctgagattacaggcgagagccaccacgcccggccaccactgccattttcatcacttaacccgaacacattcctctattccctccctttcctgcttggtgatcatcgactcttctgacccaactaggtgacctgctaaaccatctttactgttatttgccagaaaagactggaccagagacgtaaataatacacctcaatatacaacagctcgggcttaatttctaggcagaatttcatttgctggccatcagaagaatatatacatggagcgtgtttggggaggagatggagtaaggagaacacatcttggtggcaggagaacctggtgggaaccgtgctgatttgtttacttggatttgccaactggtccgatggatactgggtctgtttgcacttgagcatccaacatccgctttggtcccaggcctttaaagaagcccccaagggactgctgccgcttctcaggtctcttttggagcttgtccccattctgcagtgagttcgtgtccaccgtggcctgctctgtgcactgggctggttctttggcttcctgcttgttgctcttctgcttgttcatctcggctgctgacttcttgtccttcgaggagccctctttacccttctgtggtgctcctgttggttcaggctctggcggtgtgatagtcttttctgtggagtctgatgtttggcagctggagtctttcccatttatttcttctgagtgggtgatccctccatcccctttcactgacatttgtctgagaaacgccatcagagaggttcttggtttgctttcttctcttttgagtttcgcttctgtgggttcaggtgcagcatctccttcgttgaggtccactgtttgtaaggctgattctacttccttggactttataatctctactggtgactcacacaccacctttttccaaaacagtttgcccagaggcagagaggtgggtcctgatttctccttggtgccttccttcgcaggttcaggggttgtcacggactgtgtgtgccccgatgggttgcatcctttggaattcttgccagccccttgggtctcctgggatgtaaagttggctttgtctgacttaaggtcagctgaagtggtgggtgacttttcagcacccttatgcctaaagaattttctaaaggcgagtcctagcctggggctatccaggtgctttttcttggtgcctctagcctggatctcggatgtcttctgaccagcttgtccatcacagacactttctgctttcgatgccgtgtcttctgggtccttttttgtttcagctttgttaggtgaaaccagagttttaaagaaactcatgatggaattattattctctgctatagctgctgcctgggaatcgtcctttgcagtctccagtccttctgggtccccagggacagagcaatccgcagttccaagttcttgtccttctttttccttgccgtcaactatgtccttccctgcagggacatcatcggactgccctgataagccaggaacctcatccaccttgtcttgatgctctgccctcttggcttcctgttggctgtcacctggcaccttttcctgtcccttgtccagcttgaagaatttgtcaaaaaagctggagtccttgggcttggagggagcttctcctcctgctccccctgtctcaggtgggagaagcgtgggatccctggcggcagagaggaccttgtcttgggccggggcgtgccctggggttttatctgtgtcctgccccggtccagctgccaccggaagtgtccagctctcacttgggtctttgttcgctggagctttattggagctgacatcaagcttcactgatccaagggatgaatctgcggcttggtctccggtacgtcctggtacaggccgagagagcatcaagaaaaaacgagatttagcagctggtgcctcgggtttggcctctttcccaagattctttccgttggcatccgcaacagcacttatctccgttgtctcgggggaagaagtggccacattatccgtcttgacacttattcccaagtcgacttcctctaagtgctgaactgtgtgggtcgacaccaccactggaaccccgttcagagcagacgcgttgtcctggtaagtctctgcttctggttcattctcttggtcttcaactctttggggaacactcatttggttacccattgctcctgctgagcccctgtgggagtatcttcagtcccctcgtgtcacccggagctgctcctgcacagggtcctgggtctccagtgcgtgctgcccagtgcctggctgtcggtggagcct

SEQ ID NO: 12021 - RNA, 6544 nt, Homo sapiens
  source 1..6544: mol_type = other RNA
ctgaatagctgggactacaggtgtgtgccaccatgcctggctaatttttgtgtttttagtagagatggggtttccccatattggccaggctggtcttgaactcctgacctcaggtgatctacgcacctcagcctcccaaagtgctgggattacagacgtgagccaccacacctggcctggaaattttcaaaaggctaatactgctaagtgttggccaggatgtagaacaactggaacattcatacactgctgatgggagtacaaaatggtagagcgactttggaaagcactttggcagtttcttatacagttaaattttacacagaccatgcaacctaccaatctcgatcctaggtatctacccaagaaaaatggaaaacatacatacacatacatataaggacttgtacatgaatgttaatggcaacattattaataatagccaaaaactggtgacaaccaaatgtctatcaactgatgaatggataaacaaaatgtgatctattcatacagtggaatagtactcagcaatcaaaaggaaaaactactgatacatgctacagcatgaatgaatcttgcaaacatcattttaagtgaaagaaaccagactcggctgcaaactgtctgattccatctacatgacattctgaaatcagatcatcgttttctggaatcaggagcgtgggaaaggactgactataaattagcacaaggaaacattttaggatgatgaaaatatcttcagtgtggtagggacataactatatacaactgttaaaactcgtcaagcagtacacttaagacgggtgaattttttcatattcaagttctgcctcaataaagctgttccaagaatgttaaatatattgagagatatatgcacagaaaaggacgctatacttgtctcttgcggtaggattttgggtgcttttcattttcttgtctttgcttattgaaatcttgtaaaatttccacaatgattatgtagagcttttgtagagagagagaaaaacaacaataaaatgccatgatcataaataattgggttattcaacaaggaatgtattgttcattcaacattgttcattgtaatgaagcccatttagaccgcctccttctcatctatctttcatcagtgacacttctgaggggtgagctgaggaaacgggtgcaaaaaggtacagagcttaatagcaatcctttgtccatccagctctgggcttggctctcgccttgctttttggatgaatacacagtagactaatgataggggggctctcatcttcctttgccaacttcgccctccattccaatgcagatcagctcatgagtcctccaggccccaagagagactcctcagcacagggctgggcagactgtggtttgtggggtgcaggcccggcatccgcctccagctcacattggtctgttgggtgctgcctggtcttggtaaagtcaagaggccattcatcagtggagagccacaatgagggtgaccactcatgccgcacatggcaggacaggacacagagtccctccaggaggccctctgggtggggatgctcagtgtcaacaggcctctggcccttttcccccatcacgcatgccgttcatctccgaacttgccgcttatgaaagggcagtcaccttaggaaacccagccaacctggaggtggaggatggcgtgtcaggaatggtccacaccacttgcccgtgggcgcctaggctgcacaaggccccgtcagggtccaggtgtcagaacataggaatccagtgaggataataaatctataattataaaatagcttcataaaaacatcttgtagaggaaacatacaattttctagccactctagtcaggaagtaaagcccagcagaagcccagagcagctggggtgggcacagggaagtgagacacatcacagctgtcctggaagcctctgttttgtcagccataaagggtaagttgggagagaccctggttcccaacctggggtctctgtcctcaggattcacacaggcactattgtcaggaactacttctagcatctaaaaactccatacattattcacagtagccaaaagatagaaacaacctaagtgtccactgatggatgaatgaacaaaatgaggactatctagacaatgggatattattcagcttttaaaatgaaagaaattctgacacatgccacaacatggatgaaccttgaagacattgtgctaagtgaaagaagccagtcaaaaaggatagtattgtatgattcctcttgtatagaagtacctagagtggccaaattcacagacagaaagtagaatagtagttaccaggggctaggaggagaggggatgcggtgatattgtttatagatacagagttgcagtttgggataataaaaaattctgaaaatagatagtggtaatggttacacaacaatgtgaatatatttaattccagtcctgtacacttaaaaatggccaaaatggtaaattctatattatttatattttaccacatccacaaagaaacgaactccccacatacccacaatgtctcactgcttcattaaagcattgtcatgcctgttatcactcagatctgaatgggcaggtatagcctctgattgattttttagaagaaacaaaaataacagcaaaatatgttaattgtaaccttcagcgagagctgaaggagttttttgggcagttataacctttcaaagcatgacatcttttgggggaagacaaaggggctgtgatggaaaggttggcttgagtgagtactttggtatccctacccgcccccagcctcaaatgctgatcttgtacttggggaggctatgctaaaggagaaacacaccccagaggagacaccaggtggtgtcttcagacaattcccacccagccatagggataggcattttgggtttgagacggccctttctctggcttacttttagagcctggagtcagacttcttcacaacaaatagcccagaaccagctgggaactctctggcccatatgacacatgacactgatacagtaccagaaatgcatggcaccagctaataccactgaggggcaggagggcatactctctctcagaccctcatccatcacccccagaaccaggacaaggtcatgatggctcttggcagcctgctcagcaccagggcaagaacaactcaggctggacattacgagagtaaacacaatagatttctttcccagaccaagagcttgggcaccaggagtgggcattctggttcactgttaggcaaaaaagcctttggggaaattaccagctctcccgtcatccccaccttccttgaaaggcagcatgtggggtgggaagaacaatcagaagacaaattttaatctaaatcctgcccctctgtggccctggaaacttggcccctttgagcttcagtcactttgtgaaatgacaataacattcaatctccttcaacctcattactatggattaaatgagacggtgtctggggacatgcttggagaatgtattgtacaactgcttaggaattttcttctgcccctaaacctggaacttagagtggagcaaacagtaaacagtcactgtgtgtcggttaagggaacagagcctcagagccccgacccctggaaacgtttcttttttgtttactaaatttctagcaacaccgtgttttctacagaggtggggggaaatgtccatttaagtgcaagatgaaggggcctgtgaaaggaccctccaaggcaatcccatgtgctcccgtctcctggaaagaagccacatttcttcaagttgatgcaggggtgttgggggaaagccagagtaaacagggctctcctggtacctccttagagtacacaagtcatttgtgctggggaagagtttagtgtgtgtccttcaggagtctccaaatggcactccggctgcagcttcagttgaccaacttctccctcccaggaagcagggaggagagagaccttgggcaaggctttgtacctgcagccccagtgagcagatgtgtttcccaatgtggaaaatgcataccgtgcttccccttcctcgttgtctatgagtacgtaaaaggacacctcctgtggccctgcagcattacaatgtctgtggcattgtaagttcttgccttggtctgggagtccctcctctgttctctaagctcagacccagagggcaagacctagagtgccctgcaactgaggcagcctccccaaggctcgttctgaagctgccgtcctctgaggacaatggcttcttggaacttcttggaacaaacaagacaaaccaacacattagagccggcagcgggggcacaccgtgttcttctagaaaaggatcaaggggagtggcttcagtaacggaacatgagggactccctcacatggacacaaagcatcaagggacaggccggctttgcttttcgcttcttcctagctgcctaattaggacttactcagttcacagtgttctaccttaccgggccctcttggagccagctggagatgataaaaaccacacaggtattggagtcagatagcttcacatgccatttccacctgagaaacttgggtgagtcacatctctccaggcctcagtttttgcatctgtagaaggaagagaagacaacctatctccaaagcgttgtgacaattcagtgagatgatgtttgtcaagcccaccacacagggcaagttggttccttcccgtcccccgcatttgcctctactgagggtgaaggcagcagagaagacatcaccagcagctgcccaccactgcctggctctggagagggagggaccacgcatcctcacctaaccacaccaggccgctatcgcctgcatgtatctcgtgtccaatcggggccctgaggcagcgtcccgccctccctggaccccctcagatatcccaggctggaatggtgaggggcaggtgggagcagccaggcccttccctgggcaagccgtggtgagccacccgcccattccgcagcgggaggcggccgggcctgggggccccactgctagggcccgactcagagggcagcccggagtcgctgggccgcaccaccacgaagacccgcctgtgcagaagcccgccgggccgctcggagtaggcctccttgtggctccccgacgggcgcgggcagaggcgggcgcggaaggcggcctggaagccgcggcggaagttctcgttgaagtagccgtagatgatggggttggcgctgctgttgaagaaggccagccagtgcgcgaaggggaaggcgtagacggtgaccaggtgcagctgcggcgcgctgagctgcccgtagtcgatgagcagcagcagcgcccagagcggcagccaggacagcgtgaagaacagcgccaccatgaccagcatgtgcaccacgcgcgctctgcgccgcgatgctcgcgggtccgcagcctcctcgcccccgggggccgggcccggggcctggcagagcttgcgcgcgatgcgggcgtacatgaccacgatgagcgccagcggcgccaggtagatgtgcgagaagagcacagtggtgtagaccctgcgcatgcccttctcgggccaggcctcccagcaggagtagagcgggtaggagcggttgcgggcgtccaccatgaagtggtgctcctcacgggtgacggtcagcgtgacggccgagggacacatgatgagcagcgccagggcccagatgacggcgatggtgacgagcgccttccgcagggtcagcttctcgcggaaagggtgcacgatgcagcggaacctttccacagcaatggccaccagtgtgaaaacggaagccgacacagacatgccctgcaccaagccgctcatcttgcatgtggcattgtcgaagggccacccagtgatgaggttgtccacaagggtggtgggcatgcagaagatgcccaccagcaggtcactgacagccaggttgaggatgaacatgttggtgacagtatgcatgtgccggttcttgagcacgatgaaacagaccagggtgttgcccaccatgcagagcaggaagatgagcgcataggccacaatgaacatggccgccacaggggaggtgtgctgatagtaggaggagaaggtgaggtttgtagccggggtggcctcagtgttagtcccattctgacttaggggccaactgctgttgggaggctgggagggctccccctccatgatgcccccagttgcgggctccggcggtctccgatggcgggaggcagcgggccccttcgggccagcgggcagagggacggtctccgggcacttggttgcgggctgcgcccctgcctccgcgctccgcaggtccggtcggtccgggcagaggtgagcagggggcgtgcgctcccaggccccgggccctggccggtttccctcccctcgggctgactggctcccgcgcagcgctgctgcccgcagggctcagccgcccgccgcccctcgcctcccgaccaggggaaggagggggctcgtgaggcgcagtcgtcatggcacccgcgcacct

SEQ ID NO: 12022 - RNA, 7473 nt, Homo sapiens
  source 1..7473: mol_type = other RNA
ctgaatagctgggactacaggtgtgtgccaccatgcctggctaattttttgttttgttttgttttgagaccaagtctcactctggcacctaggctggaatgcagtagtgcaatcttggctcactgcaacgtccacctcctgggctcaagcaattctcctatgtcagcctctcatgtagctgggattacagatgtgcaccaccacacccggctaatttttgtattctttttattagagacggggcttcaccatgttgggcaggctggtctcgaactcctgacttcaagtgatcctcccaccttggtcttccaaagtactgagattacaggcgtgagccaccgcgcctggcctaaaactctgcttcttattgtggcacgtggctgtagattgaggtggaggttctgagatctgcgcgcagtgggggttactgctgagcactggggtcatttcctatggggaaggagggagggagggaggactccacagagggggaagctgaagccagatgtggtggaagcagaggcctgagtgatcctgttggggctccagagctgggatgacctccacagttgtgccaatcaaggcaaggggcagcctttgcttgcctggccccctcacctaacttctcccctcgcttactctattccaggggatggtaaactttttctgtaaagggccagagagtacgagagccctaggatctctgtgcaaatactcagctctgtcactgtactgcaaaagcaactgtggaaaatatgcaaacgaatgagcgcctgggttccaataagtctttatttacaaagacaggaagcaagggtccccttgatttggcccaaaggccttggtcagcgagcctctgctctattctgacagccagaaactcttgctgttccaggaacaggccaaggccacatctgtcctaggactttcacagatactcacagccctcttcctatctccctccatctgaagcgctgcctcctccctgcccacctgtctagatcagcggtgcccgtaagtccggaactcctaccctgcctccattcctctcagtcctcatcaccctatgctggattagctttttccttttttttttgagatggagtctcgttcttgttgcccaggctggagtgcaatggtgcaatattggctcaccgcaacctccgcctcccgggttcaagcgattctcctgccacagcctcctgagtggctgggattacaggcatgcaccaccatgccctgctaattttgtatttttagtagagatggggtttctccatgtcggtcaggctggtctcgaactcccgacctcaggggattggcccgcctcggcctcccaaagtgctgagattacaggtgtgagccaccacgcctggccactctttccttctttattgccggtctctggcactagaatgtcagctccagtgagggcctctgcttgctcccaactggctcccagctactagaatggagcctggtgcagttgatcctcagtacactcagagttgccatgcttctcctctctctgtccacaccgactccagctacaagccattgccactgggggacccaagcctgccactcagcaacacagcgaccagcccaggagtagctccgtgagccaatagatcaggttggggcttatgtaaagcccattttctcctggggtggctctcagccattttgcctccctccaggcaatggcctgccctacagagaaaccaacaagagggacagcagggcctgccaggagatgggaggggcacagccctcagggcacctcccagggttttgtgagctgggatgaatgggtttatagtcctgagtcactccagagggaggattccggattcagcccagcccctgcttcctaaacaactatggggtggggcagggaacactggaaaagaaatgtacgtgtgagcatctgtaagacccggtgacggcagggctggggctgtctctgtcaccactgtgaccccagcatagggtggggcagagagtgggtaactcagtgagttttgtgttttattttttttattttttttttttttgcgggagacgccctaccaaggacactgggtccatgtcccggtgcgggaccacctcagtgagttttttgagtgaaagaataaataaaggatatttttcctaaggttgacatggaccttatttatttatttatttatttatttatttagagatgaagtctcgctctgtcacccaggctggagtataatggcatgatctcggctcactgcaacctccgcctcccgggtccaagagattctcctgcctcagcctcccgagtaggtgggattacaggtgcacaaccaccatgcccagctaatttttgtatttttagtagagacgaggtttcaccatgttgatcaggttggtcttgaactcctgacctcaggtgatccacccaccctggcctcccaaagtgctaggattacaggtgtgagccactgcgcccagtcccaaggactttttaaatatgaaaaaagaatgcatcaacttgaagataatcagcttcatttacaaatttattctaacccctctccccaaattacaaggtacacagaattctagctagcagaacacacgagcagtgaaccatcctctggcctcttgcattttgagaggacgttctttccacttccacacactctggccacccctgacgccgcagtgggggaagtagatggccctgctgcccacgatgactggctgcctgtcagggcagggcagggcagggctgagtgcgaagtctctgagatgtgagagcagcactccatctgggtcaggacagcgctggggtcaggaattggagctcctgcctgtgttcacactcccacctctgttttttttttttgagttgagtctcactctgtcacccaggctggagtgcagtggcgcgatctcagctcactgcaacctccacctcctgggttcaagcaattctcgtgcctcagcctcccgagtagctgggattcaggaatgtgccaacatgcccggctaatttttgtatttttagtagagacggggttttgccatgttggccaggctggtctcgatctcctaacatcatgtgatcagtccaccttggcctctcaaagtgctgggatgacaggcgtgagctggcctgggtcactcccagttttaaacacagcccactcaggacccactcggtcagttccctctgctccagcttctccccctcttccagaaggaactgaaatgctgtttcaggccaggcgcggtggctcacgcctgtaatcccagcactttgggaggccgaggcgggcggattacctgaggtcaggagttcaagatcagcctgggcaacttggagaaaccccgtctccactaaaatacaaaaattagccaggcgtgggtggtgggcacatgtaatcccagctacttcggaagctgaggcaggatcattggttgagcctgggaggtagaagttgcagtgagccgagattgcaccactgcactccgtcagggtgacggagctagactgtctccgaaagaaaagaaaagaaaaaagaagagaaaagaagaaaagaaaagtttcagaacctgtttcttggctttctatctgggcagatcttggtccaggccagttttacctctttagagaagggaggtgaggatggaagtcggggaaagcccggccctcccactttcacctgcagcttcccaaaagcgggcccaggtggaatggtcacccagtttacacaatgctatgatctctggtgtgatctggggctgctctgagaggggatagagagggtctcccactatcaacgccacctctgggatggtctgggcctctgtgtagagatcgtcaccctcccagcctctgctcagccatcgcctctccctcctcactctgcagctggggtaatccaagcctctcactctgcccctactacttcaccaccctgggcagtcagcccctcactggctgtggcatctctggcaagtccctttgcttacccctggccttagtttccccagctcatagggtgactcttgggcctctccccatcagaaccctcccagtttccctcctgattttaataagctctgtacccattgtggagatccacatggtggttcaggtacagcctcaggatgccttcatcaccttgcagctcctctaatgagagagctacagtcggaaggacagactgcaggctactgggacccaccccctcccgcttcagtggcagatcctggaagagaaacccagtagaaaagggtggttcctagactgttcctctcagctagcaggaaggccaaatggcccgcggggttggcaggagtcccagggtactttttttctgagaaagggtctcactctgtcatccaggctggagtgtagtggcgcgatcacggctcgctgcagcctcgacctccagggctcaggtgatcctcctgcctcagcctcccaagtagctgggactacaggcatgcatcaccgcacctggctaattttttattttacttttgtagagatggggtctcactatgttgcccaggctggtcttcagctcctgggctcaaagagatccctcctgccctggtctcccaaagtgctgggattacaggtgtgagccactgcacctggacgccagcgtactcttggggtgaggaggaatagtgggctgaatggcttgaatggtgtgcccccaacagacaagtccacatactaacccccaggacctgtgcttatgacagtttatttggaaaaagtgttttttcagatgtaattaagggtcttgaggtgggatcatcctgaacttaagatgggccctaaatgcaatgacaggtgttcttgtaagagacaaaatagaagagggaaaaggccatgtgaagctgcaggcagagccaaggaaggcctggaatcaccaggagctggaagagggagcgtgtccctgtcagcaccttggtttcagacttctggactccagaactgtgtgaattaaattcctgttggacttaagccatcaagttcaccacccaatggtgatctgttatggcagtccaaggaaattaatcaagcagttaaggccaactgctggcctaattggtaggatgggggtgggaccgggggctatggaggcaggagggtactgctacatgaagacaggctgtcgggtcagtccagagctccgaggaaagaaagcaagagcacacagattaggagacacggatggaagatgaaggatgtgacaattgaatccatgggcttggattcgactgggtccctgagaaatgctactgagcaaggtggggaaggcaagaaaggacatgccacacagtacaagctccagggactctgaggacaggaaaatagggggctgaggctgaaggacaggctggattagccctagttaggatcaaatttcccaccacggaaaggggggttggaggacattcacagaaaagatcctgtagtgccattccagtgggttgtgccatagactcaaggatgagggggttctgttggaatagtccacttcgggtctcaagggaaggtacaatgattccagggattgactgcaggccaggaccttttgtgggtttttttaagatggagttttgctcgttacccaggctggcatgcaattgcgcaatctcggctcactgcaacctctgcctcccgggttcaagcaattctcctgtctcagcctcccaagtagctgggattacaggtgcatgccaccatgcccagctaatttatgtatttttagtagagacggggtttcatcatattggtcaggctggtctcgagctcccgatctcccgacctcccgacttcaaatgacccgcccacctcgaccttccaaagtgctgggattgcaggtgtgagccaccgtgcccagccaggattttttttttttttttgagacacagtcttgctctgtcacccgggctggaatacagtggtacaatcttggcctccacctcccaagttcaagcaattctcctgcctcagcctcccaagtagctaggattacaggcacccaccaccacgcccggttaacttttggttttaagacggtgtcttgctctgttgcccaggctagggtgcaatggtgccatcttggctcaccgcaacctccacctcatgggttcaagcaattctcctgcctcagcctcccgagtagctgggattacaagcgcaccccaccacacccggctaatttttgtatttttagtagagacggagtttcaccatgttggccaggctggtctggaactcctgacctcaagtgatccgcccgcctcggcctcccaaggtgctaggattacaggcgtgagccaccgctcccagccgcaccgtttttttcctccttaagagagcactgatgctcagctagagctgaccttagaaggtgagggggagaaaaggccactgcaacacactgcatttccttacagtggtctgtgccgattgacaaaaagaagaaggtgttccagtgtaacagatgagtgtcccagtaaaggttaacactgatcaggtaaaccgggggtgggggtaacaataacacattgattcagctcaagaccaggttccattttttcatttgccagagtgcccacggtgtcctgctggctgggaccttgcaggtcgtcctggtttggagtgggggataggaggtgaaggatgatggagggggctatgttgcaacgcttcacctgctggtcccagtggcaggtaacggctgctcttatcagcaggggtaaccaaatgccaagttgcatcaagatcctggtggtttccactgggccagcgcaggcaagggtggtgcgggaagaaggccacgttaggtacataggccatgtccaaattcaggttccatccagcaagctcctatttcttggacgcaggcactgcgtgggaagcggaccggccgggattgcagagctgggcgcgcacctcttgcagctctgtgcgcagttcctccagggcgccctgtggcggcgccgcctgcacctgcgcctgcagcgcttccagcgccagcgccaggtggcccacctcgtcccgcagcgcgttccaggcagcacgctgctcctcctccttgtggcgctgctgcgcctggtggcgccagtactccagcactaggcagccgccgcccacgatgaagatggtggcttcgcccagcagctctgcgcccagctcagctgccgcctcctcgttcagcggcttgatgaccgtgccccggaagcccatgatgcgcatcttggtccgcatctccacccagtgatacagttgagccggcgggaggcagatataggtcttgaagaactcgcttcggcgggcggcctccttaatacggttggcaagcggcttgctgacctgccggatgcccaagtatagcagcttcgccatagggaacgcgcccaccaccatcttggcggtctcacagggcacgcgcaaccttgctgact

SEQ ID NO: 12023 - RNA, 8289 nt, Homo sapiens
  source 1..8289: mol_type = other RNA
ctgaatagctgggactacaggtgtgtgccaccatgctggctaatttttatattttttagtagagactaaacaacatggtctcaacatgttgcctagcctggtcttgaacttctgggctcacactatcctcctgccttggccccccaaagtgctgggattacaggcataagccacctcgtctggcccctataagatttatattggtggtttatctgcttatgtgtagactgaagatggtcagagggctctgactcaccgtttcatatatatttctcaaatgcaccatagtaagtggtcccttaacctcaaatgtggcaattactccttaaatatgtgaaagatttggactttgatagtttctgggctttgcttgcatttaaaatagctatctccttcccaaagattattatatattattaaaagtatagcccagagagctatcaagccatctatctaatctacctaatggcaggtatagaaagctcaatcttccaaccaaggcctatttggaaacactggatctcatgtaatggcagtgcaaggccaagtgacaggccctttgttcatgcccccaaggcttggcctagtgctataggactccccagaaagttacctttaatggaatgaagaaatagctcagtcaagggtgttttccaactcaagctccataatgtatatagatttcattataaaaatactattccttaaaaaaatacataactgtaaaatattccatttctacagccactcctattctcacccatatcatcctactcatcttcgactataacgaatgggcacattcctcagtcatggctcaatcatagaatttgagtccatctctcttgctttttcaagcaatgccaactgtgcttaaaaatatgctcccagatccagttgggggtctgcaagtttccttctctcacagtgggaaggactgtgaggagacgactacaagaggtcatgcgctccatgtggcctgtctccctgaaaggcagggtgtaaaattttgcaggcttatatgagaacacagatacgtgtttggttggtagacgggcagaagtaaatcccaacctatgcccactttagcccctttgggccacacctgcaaggttctgcctcaatgctcctgtaatgaaattcacagctctgaagaaggctgggtaggagtggggaagagaatgttgtgttaatacagctttggaatacaacctgcgtttttttttaccaaaaaggacagaaaagaagaacataaacagtgatgctaaggcaaactgtcaaatggcacatcagtactattttttgtcattcattttgttaacatcacaaggcagatacattctgtaaacatatataccatacagtacattaaccataggaaaataaaaagaaagccaccctgtaattcttttctttctgtatttctattctttcactccagaaggactgtctgaagtctagggagaattttatgatttgtgagatgtactttttatttttattttttgtaaaaatgcagtgacttgcaaaaaatagccccaggtgattatgaagaggcaatatgaggagaagacgaccctttatacctcaacctgtaaaaacttagaaaacagacccaaaatagaaaaagtcattaatttcagaaaacatcttgttttcctggttagtaaaagagaacattgaaaaattatttttataaaagttaaggctgtccagatctttgatgcagaaagtctgcagtccccaaaattacatattatattttcatattgaaatcaagttcttttgtgcgacagttccgaccttcttatattatactggaaaggagaggggaagcagaggcttacttgagttatataaaaattatgctggggaagctggtctaaggagccctggtaaaattcccctttgtagtctttattctatacctttctacattcaaacaatcagtattttggtttttgttgaaatgggaattttactaagaagtttgctgaagctatgaaaacacagatacatatctgcattgtgctcctaataaacgacttttctttttccctagaaaatgcaggaaagttttcctggtaataccagaagaaggcctttgtgaagtgaactggtggtagcaggaatcaaacatcccatcttcctcattaattaagttgttttattatacaaataactgtgtgctcttgctgtgttgtactatccaatagaacaaaggatgttttcaggttctatcctaatcactggagttcaatataccttgattaagaaattgaggagcacctgaaagatcgtgtatttatgaagtttctgaaacacctatgtcttacttatgctgagaatctgtggtttcaatagcaaatgtgcatgtggcaaaaatgcaatgtgaaatggctcactttggaatgatttttattgtaaactaatatggcaggagatgaggttatttcttccaggaaaggacctgttagtgagtaaaactctccagtgggtccagggatgagcagagatgactgagcttctagatttcaagtaaataagaaaaagtcctcgatgcttattctgtctatgtccatctgcgttttatattggcagggctaatatttcttacaaaggaagacctggtatagtagttagattttgtctctatgaccatgttccctccctcctcttttgctacccattggttcaactggcattaaataaatggtaattttcaagggtgtgctgtggtcccttgaaatgaaattctgcaggaagtaaagagaaatagtctgtttttacacttggcctcaacattttgctccagagatgatattgtatctctaggaaactctctcttatacttcccctccttttataaaaacttgactttaaccaaaacaaaatattctacttgcttgtagataaaatacatttatcagcaggaaattaaatggaataggtagacgttttaagcaaatacatgtctattaacattttggaaaggaaccaaatcaaattaatagaatttgagtttcctgaaagcttctgaataattctaagattgctcagaaggctcaaggaaactgtgttttaggtttggccataagggcattccctaccttctcttccaccccatcaccaatattaaatgatgtcactgaacactgtcaaatcagttttagaggcaattattatttttttgcttatgcaaggaaaataatatgggtaaaagagatacaagctgaaaaaattccccttagtttgtcttattgcacactaaaagaaagaaaatatttttaagaagtcaagaatacagaagtcattaagatttttcaagatatgtagaattaatctttatcattttaaccattaaagaatcttttattaaatgccattgaaaatctatttgtatacaaatgagatacccccccttttccttttttttttcctcctctttctatttaaaagggaactgattatatgatttttttttttttttttttttttttgagatggagtttcgctctttgttgcccaggctggagtgcacatctcggctcattgcaacccctgcctcccaggttcaagcgattctcctgcctcagtctcccgagtagctgggattacaggcatgcgccatcacgcctggctaattttgtattttttttttagtagagatgggggtttctccatgttggtcaggctggtcttgaactcccgacctcaggtgaaccacccgccgcggacttccaaagtgccgagattacaggtgtgagccgctgcactcggcctgattatattattttaaaggaaagcccaactaatcattagctcaaaaaagatcatggttttgcaatttcattactgattctttaattagtttggttatgtaaccaaataccctgcatttttggagagtgtgataccacacataataaaatttacagagagaatgccaatggcagcaggaaaggcagcatgttcataatcacagctccatgtacactatcatcatgaagggtagttacttgctgctataggtgggattataggtctcatcccatagaagtactggctaagcctgaattccccattatgacaagaaaatgatgggacatatgcaaatatatgcgccatattcaaacacaccttcatttagtgtggctacaaatagctcgaataaaggtaacacatcttacttcagtccattaaatgataagctttactaataaaagtatagagagaactcgaattcatataatttgctaatcattattcccccataatagtaattagtgaagagaatacagataatcattaatcttttagttcttgtgtgtagtgttgtagtaagatgtgcagatcattttctgtatgagtaactagttcacttatgcaaggataggtcccttcagggaattatctgtcctggaagattgattctgtttatcaaccagcaagcttaaaggttctacattctaccatttcactcactaactgtgcttaactttttaaaactcacattgaatagcttgaatctccaagtgagtagaaaagataagctatggtaagctttcagattgtttctttcttaagtaaatcattaaaataacagattgtccaagacattgaaactgttttctccctctatgtaaataggtttatctgcatgccagtttatgtaatgtctaaatgatgcttcagtgaccacgtactcaggaaaatgaagctgagagtagtggaatttataagcatccaaaccaggtttctcgataaaatagcaattttattccattgcagctgctttgatgaacttgagatttagagatatttccctcagttattcaaaaccaagccttggatgaaataatcttcaacagcagaacttagctcctttatttttctcttctttaacgttttctgtttatgtataggtgtaaacaagatgagtataataaaaataaaatgacccattttgtgctcattaaaatgcaattatttcagaaaattaactttgaaaagtaaaaactgatgtttttacctttcctattgaagtaaatataatttcaagccaggagattaaaaaaaagcaatagatttagcactgagcaagcaaaataggtcaaattagacagcttctataataaaattctctcaagactatcttattttttctgatctactttccacagaagttagactggatgtagtatatcatatgttttttcaaaactatatactgtgggacataattttatgaataattcataacaatgctataaatgggcaaataacttaaagttaagataactcttattaaaaccagtaatcatgttatatctttatttcattactatactattgttattttattaaattgtttccctttggttttactacatatgtggctttttgctttgggggagtgctgagaaggtatttcaaaaactgttcattgtgttctagataaaaaatattctttgctcttctggaatctccagaagctaaaaacaaaacaatgccctaagaagctcagctatgtgccacttaatatttgttatgaaattaagtgcttaacattgagaagataggtctttcttaatttttaaaagttttttaaagtttttttttttgaagggcagataaacctacaagttgaagttacctaaaacattctctttctcatggggccagaaagaaaagagtatggatgcaaggctttgtaatcaactggggaggagatgaacagttaatgcattacagcaccatccatgatgaagtgggagcatcatggcaaccattgtaggttggacagactgttttagaaatatggtcactgcaaagatacttctcaagatgatctcctcattgaaaatagattaacatgaccagaaaatatccagaaaaaagaaacaatataaaaatttacatttttttaagagaatagaaacaaggcttgtgaatttgcctaagtttggagatcaattgctactgatgcttcaaacaatgtttgtttcatgtccttagaaattttaaaatggtgcttcttatataaagggttcatcggttaaaccatagaaagagagacaaccgctgatgggcaggttatggaatcagtccctacatttcagctgtgacaagctctgggttcttctacattgacttcatttcagttttaacagaaagaaagccatgaatgcacaatactgtaatctggaagcttatgtaaggcagcaaaaagcatcaccctagatcggacagactaagtaaggtccacttttggctacactagcaaccggctagagccaacagcattttgccacacaagatataaaaacaaagatccacagcaaaggaggcaagtgagaaaccagagacatggcagtgtgtgactacgttacaggaacacactacaaaatgaaacccccagtgccaatgggttcaattccagtcaagtgagttaaggctaccatatcactggctgatacgaagagtccattccaatcgagcaggaaggaagtgattcactcttgaagacacaaggaaaggtttagaggaaaagcaagttcttggagagaatgaagcacacacatgcacgttgtctctcaggtgaggaaaaggaaaaaaaatgagagagatcaaagcaattcaactgcaaggcaaggcaggtgtttgcttccagttcacagtattgcagttagtggtacagtgaggtctacgtgagtggtggagagtacaggctgcccagaagaaaggagaagaaagaagtggtcacatgacaacacagcattgacagcgctttttcttttgggtacctggggctggctctgtagctaggctctcttccttcccttctggggatgagggctctgtggtgtctgagaccggcctcccggacacaagctcagccgcgttcccgtcaatagtggacacgtccgtcactgtcttctccctcaatgacttctcatcatcttcatcaatgaggaccaattcagccttgatggtttcatcatagcctagcacctttttcgtctcctcttcatcctcgatattttggtagcccataaaaatcatggtgacgggctgatccaagtttgcctccggccctgcagcgctgggggcttgggcctgctgccctgggttcccggaagaatggtctttcctagacttatgtaccatttctaacttagcttctttgcagagcatgtgttccttgggatggctgaggctcccatctgcaatcacagtcctttcagacacgtgccctcctcctaagcttgattgtccagccttctgaataagctcttctacatcctttgtgcttaatttgtgcactccattttctactacggtgcctcctgagcgcacctcatacactactttggtaccatcatcatagactttgactcctttctgatggaccccctctgggccaatggtagatgtagagagaatcttggtctctcctgtttgtttgtctttctccacattaatttccatggcgtacacagcagccgctctgctggtcccgtcctgcccaggtgatggttctgctgttcgtgaacagaggattggcaggtcgggaagctgggaggaaatgtaatttactgcatctccatccgtactggagaaacccttctgaaagtccttgaaggatttttctgtttccttcagtttctctaggatgatttgctctttggcagatatctgggactcttcactttctagcgtttgtatttcttgctccagcctctgaatgttatcttcaagttgcttgactctgaactcatcctcttcagactgccgcctcctggcttcctcctcttcggcagttccagcgggtatgccctgcagcagccatttctcccgaagcactttggacttggaatgctgcagcagaagtatctgctcgtcaagctgttgtcgcttgccttctatttcagtctgcctctttcttttttctgctatggcttgcagcctttccttgtgcaattccgcctctgccatcctggagaagggcacacaggcaggggaaagaggaaagaaaaaacacacgctgtagtcacccaaggaaactgatgggcaccccggggggctttgctagaacccgggagaacgcccagggacggctggggatccgctccaggggcggcgggcagagctgtgcgcacggcgggctcgcccgggctcagcctctggcccccgccctcccggccgcctggctgcgccccagcgccgccgctcactgcatctcccggtcgccgccgccgccggccgcgccagccgaggacgtgggac

SEQ ID NO: 12024 - RNA, 7977 nt, Homo sapiens
  source 1..7977: mol_type = other RNA
ctgaatagctgggactacaggtgtgtgccaccatgctggctaatttttatattttttagtagagactaaacaacatggtctcaacatgttgcctagcctggtcttgaacttctgggctcacactatcctcctgccttggccccccaaagtgctgggattacaggcataagccacctcgtctggcccctataagatttatattggtggtttatctgcttatgtgtagactgaagatggtcagagggctctgactcaccgtttcatatatatttctcaaatgcaccatagtaagtggtcccttaacctcaaatgtggcaattactccttaaatatgtgaaagatttggactttgatagtttctgggctttgcttgcatttaaaatagctatctccttcccaaagattattatatattattaaaagtatagcccagagagctatcaagccatctatctaatctacctaatggcaggtatagaaagctcaatcttccaaccaaggcctatttggaaacactggatctcatgtaatggcagtgcaaggccaagtgacaggccctttgttcatgcccccaaggcttggcctagtgctataggactccccagaaagttacctttaatggaatgaagaaatagctcagtcaagggtgttttccaactcaagctccataatgtatatagatttcattataaaaatactattccttaaaaaaatacataactgtaaaatattccatttctacagccactcctattctcacccatatcatcctactcatcttcgactataacgaatgggcacattcctcagtcatggctcaatcatagaatttgagtccatctctcttgctttttcaagcaatgccaactgtgcttaaaaatatgctcccagatccagttgggggtctgcaagtttccttctctcacagtgggaaggactgtgaggagacgactacaagaggtcatgcgctccatgtggcctgtctccctgaaaggcagggtgtaaaattttgcaggcttatatgagaacacagatacgtgtttggttggtagacgggcagaagtaaatcccaacctatgcccactttagcccctttgggccacacctgcaaggttctgcctcaatgctcctgtaatgaaattcacagctctgaagaaggctgggtaggagtggggaagagaatgttgtgttaatacagctttggaatacaacctgcgtttttttttaccaaaaaggacagaaaagaagaacataaacagtgatgctaaggcaaactgtcaaatggcacatcagtactattttttgtcattcattttgttaacatcacaaggcagatacattctgtaaacatatataccatacagtacattaaccataggaaaataaaaagaaagccaccctgtaattcttttctttctgtatttctattctttcactccagaaggactgtctgaagtctagggagaattttatgatttgtgagatgtactttttatttttattttttgtaaaaatgcagtgacttgcaaaaaatagccccaggtgattatgaagaggcaatatgaggagaagacgaccctttatacctcaacctgtaaaaacttagaaaacagacccaaaatagaaaaagtcattaatttcagaaaacatcttgttttcctggttagtaaaagagaacattgaaaaattatttttataaaagttaaggctgtccagatctttgatgcagaaagtctgcagtccccaaaattacatattatattttcatattgaaatcaagttcttttgtgcgacagttccgaccttcttatattatactggaaaggagaggggaagcagaggcttacttgagttatataaaaattatgctggggaagctggtctaaggagccctggtaaaattcccctttgtagtctttattctatacctttctacattcaaacaatcagtattttggtttttgttgaaatgggaattttactaagaagtttgctgaagctatgaaaacacagatacatatctgcattgtgctcctaataaacgacttttctttttccctagaaaatgcaggaaagttttcctggtaataccagaagaaggcctttgtgaagtgaactggtggtagcaggaatcaaacatcccatcttcctcattaattaagttgttttattatacaaataactgtgtgctcttgctgtgttgtactatccaatagaacaaaggatgttttcaggttctatcctaatcactggagttcaatataccttgattaagaaattgaggagcacctgaaagatcgtgtatttatgaagtttctgaaacacctatgtcttacttatgctgagaatctgtggtttcaatagcaaatgtgcatgtggcaaaaatgcaatgtgaaatggctcactttggaatgatttttattgtaaactaatatggcaggagatgaggttatttcttccaggaaaggacctgttagtgagtaaaactctccagtgggtccagggatgagcagagatgactgagcttctagatttcaagtaaataagaaaaagtcctcgatgcttattctgtctatgtccatctgcgttttatattggcagggctaatatttcttacaaaggaagacctggtatagtagttagattttgtctctatgaccatgttccctccctcctcttttgctacccattggttcaactggcattaaataaatggtaattttcaagggtgtgctgtggtcccttgaaatgaaattctgcaggaagtaaagagaaatagtctgtttttacacttggcctcaacattttgctccagagatgatattgtatctctaggaaactctctcttatacttcccctccttttataaaaacttgactttaaccaaaacaaaatattctacttgcttgtagataaaatacatttatcagcaggaaattaaatggaataggtagacgttttaagcaaatacatgtctattaacattttggaaaggaaccaaatcaaattaatagaatttgagtttcctgaaagcttctgaataattctaagattgctcagaaggctcaaggaaactgtgttttaggtttggccataagggcattccctaccttctcttccaccccatcaccaatattaaatgatgtcactgaacactgtcaaatcagttttagaggcaattattatttttttgcttatgcaaggaaaataatatgggtaaaagagatacaagctgaaaaaattccccttagtttgtcttattgcacactaaaagaaagaaaatatttttaagaagtcaagaatacagaagtcattaagatttttcaagatatgtagaattaatctttatcattttaaccattaaagaatcttttattaaatgccattgaaaatctatttgtatacaaatgagatacccccccttttccttttttttttcctcctctttctatttaaaagggaactgattatatgatttttttttttttttttttttttttgagatggagtttcgctctttgttgcccaggctggagtgcacatctcggctcattgcaacccctgcctcccaggttcaagcgattctcctgcctcagtctcccgagtagctgggattacaggcatgcgccatcacgcctggctaattttgtattttttttttagtagagatgggggtttctccatgttggtcaggctggtcttgaactcccgacctcaggtgaaccacccgccgcggacttccaaagtgccgagattacaggtgtgagccgctgcactcggcctgattatattattttaaaggaaagcccaactaatcattagctcaaaaaagatcatggttttgcaatttcattactgattctttaattagtttggttatgtaaccaaataccctgcatttttggagagtgtgataccacacataataaaatttacagagagaatgccaatggcagcaggaaaggcagcatgttcataatcacagctccatgtacactatcatcatgaagggtagttacttgctgctataggtgggattataggtctcatcccatagaagtactggctaagcctgaattccccattatgacaagaaaatgatgggacatatgcaaatatatgcgccatattcaaacacaccttcatttagtgtggctacaaatagctcgaataaaggtaacacatcttacttcagtccattaaatgataagctttactaataaaagtatagagagaactcgaattcatataatttgctaatcattattcccccataatagtaattagtgaagagaatacagataatcattaatcttttagttcttgtgtgtagtgttgtagtaagatgtgcagatcattttctgtatgagtaactagttcacttatgcaaggataggtcccttcagggaattatctgtcctggaagattgattctgtttatcaaccagcaagcttaaaggttctacattctaccatttcactcactaactgtgcttaactttttaaaactcacattgaatagcttgaatctccaagtgagtagaaaagataagctatggtaagctttcagattgtttctttcttaagtaaatcattaaaataacagattgtccaagacattgaaactgttttctccctctatgtaaataggtttatctgcatgccagtttatgtaatgtctaaatgatgcttcagtgaccacgtactcaggaaaatgaagctgagagtagtggaatttataagcatccaaaccaggtttctcgataaaatagcaattttattccattgcagctgctttgatgaacttgagatttagagatatttccctcagttattcaaaaccaagccttggatgaaataatcttcaacagcagaacttagctcctttatttttctcttctttaacgttttctgtttatgtataggtgtaaacaagatgagtataataaaaataaaatgacccattttgtgctcattaaaatgcaattatttcagaaaattaactttgaaaagtaaaaactgatgtttttacctttcctattgaagtaaatataatttcaagccaggagattaaaaaaaagcaatagatttagcactgagcaagcaaaataggtcaaattagacagcttctataataaaattctctcaagactatcttattttttctgatctactttccacagaagttagactggatgtagtatatcatatgttttttcaaaactatatactgtgggacataattttatgaataattcataacaatgctataaatgggcaaataacttaaagttaagataactcttattaaaaccagtaatcatgttatatctttatttcattactatactattgttattttattaaattgtttccctttggttttactacatatgtggctttttgctttgggggagtgctgagaaggtatttcaaaaactgttcattgtgttctagataaaaaatattctttgctcttctggaatctccagaagctaaaaacaaaacaatgccctaagaagctcagctatgtgccacttaatatttgttatgaaattaagtgcttaacattgagaagataggtctttcttaatttttaaaagttttttaaagtttttttttttgaagggcagataaacctacaagttgaagttacctaaaacattctctttctcatggggccagaaagaaaagagtatggatgcaaggctttgtaatcaactggggaggagatgaacagttaatgcattacagcaccatccatgatgaagtgggagcatcatggcaaccattgtaggttggacagactgttttagaaatatggtcactgcaaagatacttctcaagatgatctcctcattgaaaatagattaacatgaccagaaaatatccagaaaaaagaaacaatataaaaatttacatttttttaagagaatagaaacaaggcttgtgaatttgcctaagtttggagatcaattgctactgatgcttcaaacaatgtttgtttcatgtccttagaaattttaaaatggtgcttcttatataaagggttcatcggttaaaccatagaaagagagacaaccgctgatgggcaggttatggaatcagtccctacatttcagctgtgacaagctctgggttcttctacattgacttcatttcagttttaacagaaagaaagccatgaatgcacaatactgtaatctggaagcttatgtaaggcagcaaaaagcatcaccctagatcggacagactaagtaaggtccacttttggctacactagcaaccggctagagccaacagcattttgccacacaagatataaaaacaaagatccacagcaaaggaggcaagtgagaaaccagagacatggcagtgtgtgactacgttacaggaacacactacaaaatgaaacccccagtgccaatgggttcaattccagtcaagtgagttaaggctaccatatcactggctgatacgaagagtccattccaatcgagcaggaaggaagtgattcactcttgaagacacaaggaaaggtttagaggaaaagcaagttcttggagagaatgaagcacacacatgcacgttgtctctcaggtgaggaaaaggaaaaaaaatgagagagatcaaagcaattcaactgcaaggcaaggcaggtgtttgcttccagttcacagtattgcagttagtggtacagtgaggtctacgtgagtggtggagagtacaggctgcccagaagaaaggagaagaaagaagtggtcacatgacaacacagcattgacagcgctttttcttttgggtacctggggctggctctgtagctaggctctcttccttcccttctggggatgagggctctgtggtgtctgagaccggcctcccggacacaagctcagccgcgttcccgtcaatagtggacacgtccgtcactgtcttctccctcaatgacttctcatcatcttcatcaatgaggaccaattcagccttgatggtttcatcatagcctagcacctttttcgtctcctcttcatcctcgatattttggtagcccataaaaatcatggtgacgggctgatccaagtttgcctccggccctgcagcgctgggggcttgggcctgctgccctgggttcccggaagaatggtctttcctagacttatgtaccatttctaacttagcttctttgcagagcatgtgttccttgggatggctgaggctcccatctgcaatcacagtcctttcagacacgtgccctcctcctaagcttgattgtccagccttctgaataagctcttctacatcctttgtgcttaatttgtgcactccattttctactacggtgcctcctgagcgcacctcatacactactttggtaccatcatcatagactttgactcctttctgatggaccccctctgggccaatggtagatgtagagagaatcttggtctctcctgtttgtttgtctttctccacattaatttccatggcgtacacagctccatccgtactggagaaacccttctgaaagtccttgaaggatttttctgtttccttcagtttctctaggatgatttgctctttggcagatatctgggactcttcactttctagcgtttgtatttcttgctccagcctctgaatgttatcttcaagttgcttgactctgaactcatcctcttcagactgccgcctcctggcttcctcctcttcggcagttccagcgggtatgccctgcagcagccatttctcccgaagcactttggacttggaatgctgcagcagaagtatctgctcgtcaagctgttgtcgcttgccttctatttcagtctgcctctttcttttttctgctatggcttgcagcctttccttgtgcaattccgcctctgccatctccatcgcggggctccgcggccgggtgcgctgctgcggggctcaccggcgctgctcgcctctcccggagccgagtgcact

SEQ ID NO: 12025 - RNA, 3824 nt, Homo sapiens
  source 1..3824: mol_type = other RNA
ctgaatagctgggactacaggtgtgtgccaccccgcccagctaatttttgtatttttagtagaggctgggcttcaccacgttggccaggatggtctcgatctcttgaccttgtgatccgcccgcctcggcctcccaaagtgctgggattacaggcgtgagccaccgctcccggcagcacttatgggttttaaatatgagagtgacaacatcaggttattgggcagcaggaggtgggccagttttgaaaggcaggtgaatgaggcagtgagataagttgggaggggctgcaatagttcagaaacaaggtagtgtgcaagtaaatcacaggtggcaccagagatgaagaggaagaggcagtgtgacagctctgttgcatgacacaacatgggaaacgcaggattgagaagagccagaggtgatgatgccattagcagcgtgcatttagtacttatcacaacctatttacattttctatataaacattgatctcattagactgtgatctcctagaggaacaagtcccatgtcattctcattgacaaaatgaacatggcagatacttggtaaatgtttgctagtaagtgaatggaagtcaggcgagttggcttggtgatggcagctggggtgttgatggaaataccgtgcttctttttggacatgatggaatttggggatgtggtctatttgttagatgcagtttctaggaagagattacccaaagaactgaagaacaatgacaaacttatgtgtatgtgagggcaagataaagagtagagagatggtatagttgggtatggagagaatgctgtaactgaactgctcccttcaagatgtcaggtaagattggagagaaaatgcaggatagcatttgtcacaggtagttggaatgtggagggaagactggaaggatgagaaggactgaggtggacctgtgggctgtgttagccggtgaaagttggagggaaagggaaatgggaggcagtagagcatggagttacatatgcaggcactggagtcaggctgttggagttcaaaggctagctcttctgtggatttgttatgtgactttacacgctctctcttgcctcaagttcctcttctgcaaaatgaggttaataataatacctgcataaacacatgcacagcacacagaacagaagctggaatgtgataagcacttcataagcattaattcttcttactgaaactcactagggtcactttgtgcatattatcctatttaatccttagtaactgtataggtaggtgttattatcttcattctgcaaatgagaaaactgaagtgcaaagaagtttcataattttcctcaatccacacagccactatatgatgtgataaagcttacctaagctagagtcttacctgatccatctggtgcccgggctagtgcactttctcctataacactcagcctaagctaggtagatatggcaagaccactggctgaggcaactcagatgtgatcaataggtagtagggaactgtggctgacttgggggcaggggaagcagcatgctggaaagattcatctggtatgtttatagaagagagcaggcagcaggcatggggggctgatgattcagaccagaaatggctgaggaaatggtgaggtctggcaaatgtcagaggagctgtgatagaagaatgagcagaatttatgactgatgcaaataaggtagatatgatggtacgtgacagaaactgactaagaagtctgtatgcagtgggtgcagcttagagtttcaacttgaaagtttcaaacctgggactctaagaaaatagtctgaatggtaatgagaaagttgtcactttagtatctgcttcccttgaagaaaagcacctttagaggaaccaacttggagaatagtgtcgcatcaaagtgggacacttcattatttttagtggcagcatggttctgatgagcacaccgtcggtaacctttacttcactgtcagtccagctctgtcaatcctcctttattaaggaaggaagctgatggatctttcctttctttctttctttctttcttccctggagtaggatgttttctgtacacagttagcatgtgaacttctttttaaaaagaagtttacattttactctaattctcatccataacggagtgtggtgatttgcatttgggcagttaggaaaatcagttctgttgacttcctgttttctatttctggcctcgagcagaacttcccatttgagtgggaccaagaagagcatacaaagctgaaatgttctccagaagttgatttccaatggggataaagtaagttaatggtctgaggtgtttgtctccccttgcccccgaagcttgccctttagttgctcttgtttttaaactacagggaatgaactgagggaagcattttttttttttttttcctgcaggtcagagtcccaaagctttagtgcagggttccaaggactcaggagttcaaaacatgctgcttaggctgagctcttggccagatttggagattccaatgtcttctccctttgacagttcctaagaatattttatttggatccttttctttaggtttttctgtctaaacattttattttacctagtgtgaaggggtgagggagggcagattgtttcctttcttcctcctctccccttccccctcccctctcccttattctctgtttataatttaaaaggatgctcactttcattttctcatttgcttccttcacagcaccctgtgaagctgatattgttatccccctttgacagaaggggaaactgcagtttcagtgaatttcagtgacttagtcaagtcactcagttaacagtgctgagagtgaagccctagtgttctgcctttagatctctttttcccagtaccatactgcttttctggtggaggttgtagtatataggatgatgtcagaaaggagaggctgggaagcctgaaacgatcacatcgacaattgaattgtctgttttttctaataaaatagaaaatgttaactaaatatattgccatgcaattcttcaagcatataggactttgggtccttttttgtgtctcagactttaagatgatgtctcctggggagtcatttactatatgcaaggagaatagctgaaaagtcagggtaggccagcagtatttcatgctttgtacttgggcaatatgggtttttctgttggaggttcagcagaggatggtagcaaagtgacatttaattctcctgcttgccaaatcttggtgaggccaaagtgggtgggggaatcggttgtgagtaggtgttaatgacgagtgtctggaccttgacgtcttctcagtcctcaggcgtttgctgccgtgcctgccctttggtttctgggacggctcgggtcccgtagcgccggcacagctgagattgccaagccgggaagagaccttgctccaggtgtagctgcgttttccccagatcacctgtccttttcccctccgacaaggaagctgtgatttttctctggcctttagaggcaaagtgattccagataagtagattaatgtgtagaatatctcatctgtgttgttccagtgcagccctttcagctttccagagccagttagacttgttatgaggagctaagtgattggctggctctggagctcagtttcatagattatagcccagcgtacgagaagcacgagtcctatagttggcgtaccctgaggcctgccagttcctgccttaatgcatatgtagtcgtaattgagttctgacacggccttggatgtttctgtcctaaatagctgacattgcatcttcaagactgtgtgagtaatc

SEQ ID NO: 12026 - RNA, 4180 nt, Homo sapiens
  source 1..4180: mol_type = other RNA
ctgaatagctgggactacaggtgtgtgccaccttgcccagctaattaaaaagatttttttttttttttttttgtagagatgaggttttgccatgttacccaggctggtcttcaactcctggactcaagcgatccacctgcctcggcctcctaaagtgctgggatttcaggtgtgagccactgtgcccagcccgaagaagctttatctgatctgaacctgatttagataaggaggtcctggactttgttccaatgctgcagagagtgagacttctgtggggagaggagtgtcctttgcatttgggaaagatgtgaactactgtggccagagggtgaactatggtagattgcttctaaagatgggagcagcaatgtttcttcccaagcaacattctcctttgaaatgtgactttgccacccatcgcatcaagaggtaaggtctattctccctccttctgaatctgtccctgtgacttgctttcaccaatagattgtggcagaagtgacagtgtgcaagtatgaatggggtctgccagtaccatgtggagcaaagggaagcatcctcatggatgatgcctgaattcttgatccacagaatagtgagcaataaaatgtttttttctttttaagcagctaagctttgaggtcatttgttacacagcaatagatagctaatacaccatcaaagagttctggggtcatttcaaaacaactcaggaggcaaattgaggagtttctcactaaaagtggggaacttgcacatgcctgtaatcccagctactcggaggctgaggcaggagaatcgcttgcacccaggaggaggaggttgcagtgagtcaagatgacgctactgtactccggcctgggtgacagagtgagactctgtctcaaaaaaaaaaaaaaaaaaaaaaaaagaaaaagtgggcaactcaagcatcaataaaggtattaactgcaatggtttgtagcatgctacgtatatttaaatatgtgggttcaagataattaaattaaaaaatccctggttacctttagaggatattgggacatcaattcattattttgaacattgctaaataaaaaaacaagcatttatcctattttttgtacaacctgtatttcaaggtaaccgaatactgttaaagagaagctatttgcagaataattctgaccaataattatgtaaaaaaaaacctgaatctcatcattttgcaacctctgatgatatcacggatttaggtattgctaaaaccatcaggtgatagatgatcaggctgataacacgtgcacctgctgccaaccttaacataaaaaataatactaaattcccctgtgaagcctgcatgtgccccaaaacccccaaatcaaaacaaacccctcaaaacctgagttaaagcaagcttctagatctaacttctagcttacaaaaaatgagaggaagagaggactataccactaagaaaatgcaaccagaaaattccagattgcaaaaaatgtaataggaccaaaaccctgagttcttcaataaatacatgacaatttatagcttaaaagagacatagggacaggagagccaaatgcagtgtgtggaacttgtttagatcctgatttgaacaaatcaactctaaaaagacttatgagacagtggggagaatgtgaactatgatggggtatctgatggtattaaggaagtattaattttttttttttttagtgtagatatagacttttaaaggtaaaaagaaagaataaagatggagggtgtgataatcctatgaagtgtctgggtttgggtcctgagggcagccaattacatcccagactcactggcaatcaacagtccaagccagggtcccatcagctgaatcctgaggtggggatgcttcagtctttacagaacagggtcaaggaagagtccagaaaccgccgtcattggcttcatgaaaaccgagcacgtctttgagatctttttcaaattctgcctctaagtcaagtcctacctggccaaagtcagaagcattaaatgggatgcccgtaaaaaaggagctttgtggatgacagtaggccttcaagaggaggaactcacatttcagctggtcctgaggctgcatctgcctctccagggtcttagatacatgatggcactgttggcttcctgaagacctcttcatcctgcagaaggtgcaactccacagcatcctcttggcttccacaggggggatgtgacagtcctcatggaagactcgtggacaagtaccgcagcagagaagttgtcccccttgacagcacacctcgcattcatccgagtttttccgcttcagcagctctcctagggtcattccttcacaacgtatattccgtttccagttctttgcgttccttccttttccttcgacttcaaattcatttggtgttaaccaagttccatcctcattccgaatgcacttcactgaggatccgtgtttcattttcttcttatataaaatccctttcgcctcaccacaggtcacggggagcttagaacagtgaaaatccacagtgtcacttttgggttttcctcttcggtgaatatttttctgaaatctcctttttgagcttgaacagatatctttctcctttttcttttctttcaatctggactttcgggcacatttagttcttgccttttggaccctcatcatgacctctgagttccaggttgagtcgtctttcctttgagtcaccttatccaccacttggagcttctcttggatgccatgcccaggtgaggctgccccttgtgtgacccttcgtggtgtactaggcgtcttctgggacctctttccttcattcatttctgaagtgccatcaatgatctcctctgatctcgactttcgggcacattcagttctcgccttttgggcccttgtctctaccgtggagttacaagttgagtcatctttcttttgaggaacctgatccacccttttgagcttcttttggattccgtgtctagatgaggctgtccctcctgggaggctttttttcttatgtctcctttttggagttgaccagatacatctttttcttttctttcctttcttgtctgaaggtgtgctggacacctcctggggctcttctgggtcatttggttctggagaattatctcttatctctggcatagagcccaagggagagtggggcatctcttgagggtcttctttatctcttatttgggggatcaggttgtcactggccacttgcacagtgctagtgaggaggctgggcatctcttctgagtcttcttccgcattcattttggatgttaacttgtcattggtcactgaagtgcttcttccttcctggatgagtgcagggagaggcaggacagggtcagatgggctgggcgactcactcaggatctcatcgctttgctgggaggatgttccaggctcactgactcttggcgcacagggtgaacagcttggttgagggggttgtggtgggggcagcgccagtggggtatggagggagcttccttctgctaggccagttggggcttcaagtaggattggtgtgtctctgctctgccattcataggaagcaccaacacgtttgaagcttctgtaaatcgtcaccagattgggatattcacgcaggttaatttgactgaacaatgtcaccagaagagacaggttaaaagtcctctccagttgggtgagaatgttgtgcaccactctggatacagggatcaaatttctacaggcttccagagattccatgtacattctcttagtgatgatggagttgtctaggaggccttcaaagaagggaaatggcttgtgtatggcataggcgatccccagcttctggtgcatgaagtgctgaaaaagagcctcttccatggctcttgtcatggtgaacatcctgaagcccctccccatcacctggaaagccccttcatgggcatctgaggatcctggcagcaagaacttcttcctttagatctcaaaacaactttgatctgcttgagttgaatgacttttccaccctctttccttggcaggaacaagtgaccctgtcttccgtggcctcgtggggctggctctgctcctcctcccttgactgagagacgtcatggagattgggtggagggaggactgtagagttggtgcacccacgtcagctagttaggcaatttc

SEQ ID NO: 12027 - RNA, 4015 nt, Homo sapiens
  source 1..4015: mol_type = other RNA
ctgaatagctgggactacaggtgtgtgccaccttgcccagctaattaaaaagatttttttttttttttttttgtagagatgaggttttgccatgttacccaggctggtcttcaactcctggactcaagcgatccacctgcctcggcctcctaaagtgctgggatttcaggtgtgagccactgtgcccagcccgaagaagctttatctgatctgaacctgatttagataaggaggtcctggactttgttccaatgctgcagagagtgagacttctgtggggagaggagtgtcctttgcatttgggaaagatgtgaactactgtggccagagggtgaactatggtagattgcttctaaagatgggagcagcaatgtttcttcccaagcaacattctcctttgaaatgtgactttgccacccatcgcatcaagaggtaaggtctattctccctccttctgaatctgtccctgtgacttgctttcaccaatagattgtggcagaagtgacagtgtgcaagtatgaatggggtctgccagtaccatgtggagcaaagggaagcatcctcatggatgatgcctgaattcttgatccacagaatagtgagcaataaaatgtttttttctttttaagcagctaagctttgaggtcatttgttacacagcaatagatagctaatacaccatcaaagagttctggggtcatttcaaaacaactcaggaggcaaattgaggagtttctcactaaaagtggggaacttgcacatgcctgtaatcccagctactcggaggctgaggcaggagaatcgcttgcacccaggaggaggaggttgcagtgagtcaagatgacgctactgtactccggcctgggtgacagagtgagactctgtctcaaaaaaaaaaaaaaaaaaaaaaaaagaaaaagtgggcaactcaagcatcaataaaggtattaactgcaatggtttgtagcatgctacgtatatttaaatatgtgggttcaagataattaaattaaaaaatccctggttacctttagaggatattgggacatcaattcattattttgaacattgctaaataaaaaaacaagcatttatcctattttttgtacaacctgtatttcaaggtaaccgaatactgttaaagagaagctatttgcagaataattctgaccaataattatgtaaaaaaaaacctgaatctcatcattttgcaacctctgatgatatcacggatttaggtattgctaaaaccatcaggtgatagatgatcaggctgataacacgtgcacctgctgccaaccttaacataaaaaataatactaaattcccctgtgaagcctgcatgtgccccaaaacccccaaatcaaaacaaacccctcaaaacctgagttaaagcaagcttctagatctaacttctagcttacaaaaaatgagaggaagagaggactataccactaagaaaatgcaaccagaaaattccagattgcaaaaaatgtaataggaccaaaaccctgagttcttcaataaatacatgacaatttatagcttaaaagagacatagggacaggagagccaaatgcagtgtgtggaacttgtttagatcctgatttgaacaaatcaactctaaaaagacttatgagacagtggggagaatgtgaactatgatggggtatctgatggtattaaggaagtattaattttttttttttttagtgtagatatagacttttaaaggtaaaaagaaagaataaagatggagggtgtgataatcctatgaagtgtctgggtttgggtcctgagggcagccaattacatcccagactcactggcaatcaacagtccaagccagggtcccatcagctgaatcctgaggtggggatgcttcagtctttacagaacagggtcaaggaagagtccagaaaccgccgtcattggcttcatgaaaaccgagcacgtctttgagatctttttcaaattctgcctctaagtcaagtcctacctggccaaagtcagaagccagctggtcctgaggctgcatctgcctctccagggtcttagatacatgatggcactgttggcttcctgaagacctcttcatcctgcagaaggtgcaactccacagcatcctcttggcttccacaggggggatgtgacagtcctcatggaagactcgtggacaagtaccgcagcagagaagttgtcccccttgacagcacacctcgcattcatccgagtttttccgcttcagcagctctcctagggtcattccttcacaacgtatattccgtttccagttctttgcgttccttccttttccttcgacttcaaattcatttggtgttaaccaagttccatcctcattccgaatgcacttcactgaggatccgtgtttcattttcttcttatataaaatccctttcgcctcaccacaggtcacggggagcttagaacagtgaaaatccacagtgtcacttttgggttttcctcttcggtgaatatttttctgaaatctcctttttgagcttgaacagatatctttctcctttttcttttctttcaatctggactttcgggcacatttagttcttgccttttggaccctcatcatgacctctgagttccaggttgagtcgtctttcctttgagtcaccttatccaccacttggagcttctcttggatgccatgcccaggtgaggctgccccttgtgtgacccttcgtggtgtactaggcgtcttctgggacctctttccttcattcatttctgaagtgccatcaatgatctcctctgatctcgactttcgggcacattcagttctcgccttttgggcccttgtctctaccgtggagttacaagttgagtcatctttcttttgaggaacctgatccacccttttgagcttcttttggattccgtgtctagatgaggctgtccctcctgggaggctttttttcttatgtctcctttttggagttgaccagatacatctttttcttttctttcctttcttgtctgaaggtgtgctggacacctcctggggctcttctgggtcatttggttctggagaattatctcttatctctggcatagagcccaagggagagtggggcatctcttgagggtcttctttatctcttatttgggggatcaggttgtcactggccacttgcacagtgctagtgaggaggctgggcatctcttctgagtcttcttccgcattcattttggatgttaacttgtcattggtcactgaagtgcttcttccttcctggatgagtgcagggagaggcaggacagggtcagatgggctgggcgactcactcaggatctcatcgctttgctgggaggatgttccaggctcactgactcttggcgcacagggtgaacagcttggttgagggggttgtggtgggggcagcgccagtggggtatggagggagcttccttctgctaggccagttggggcttcaagtaggattggtgtgtctctgctctgccattcataggaagcaccaacacgtttgaagcttctgtaaatcgtcaccagattgggatattcacgcaggttaatttgactgaacaatgtcaccagaagagacaggttaaaagtcctctccagttgggtgagaatgttgtgcaccactctggatacagggatcaaatttctacaggcttccagagattccatgtacattctcttagtgatgatggagttgtctaggaggccttcaaagaagggaaatggcttgtgtatggcataggcgatccccagcttctggtgcatgaagtgctgaaaaagagcctcttccatggctcttgtcatggtgaacatcctgaagcccctccccatcacctggaaagccccttcatgggcatctgaggatcctggcagcaagaacttcttcctttagatctcaaaacaactttgatctgcttgagttgaatgacttttccaccctctttccttggcaggaacaagtgaccctgtcttccgtggcctcgtggggctggctct

SEQ ID NO: 12028 - RNA, 3958 nt, Homo sapiens
  source 1..3958: mol_type = other RNA
ctgaatagctgggactacaggtgtgtgccaccttgcccagctaattaaaaagatttttttttttttttttttgtagagatgaggttttgccatgttacccaggctggtcttcaactcctggactcaagcgatccacctgcctcggcctcctaaagtgctgggatttcaggtgtgagccactgtgcccagcccgaagaagctttatctgatctgaacctgatttagataaggaggtcctggactttgttccaatgctgcagagagtgagacttctgtggggagaggagtgtcctttgcatttgggaaagatgtgaactactgtggccagagggtgaactatggtagattgcttctaaagatgggagcagcaatgtttcttcccaagcaacattctcctttgaaatgtgactttgccacccatcgcatcaagaggtaaggtctattctccctccttctgaatctgtccctgtgacttgctttcaccaatagattgtggcagaagtgacagtgtgcaagtatgaatggggtctgccagtaccatgtggagcaaagggaagcatcctcatggatgatgcctgaattcttgatccacagaatagtgagcaataaaatgtttttttctttttaagcagctaagctttgaggtcatttgttacacagcaatagatagctaatacaccatcaaagagttctggggtcatttcaaaacaactcaggaggcaaattgaggagtttctcactaaaagtggggaacttgcacatgcctgtaatcccagctactcggaggctgaggcaggagaatcgcttgcacccaggaggaggaggttgcagtgagtcaagatgacgctactgtactccggcctgggtgacagagtgagactctgtctcaaaaaaaaaaaaaaaaaaaaaaaaagaaaaagtgggcaactcaagcatcaataaaggtattaactgcaatggtttgtagcatgctacgtatatttaaatatgtgggttcaagataattaaattaaaaaatccctggttacctttagaggatattgggacatcaattcattattttgaacattgctaaataaaaaaacaagcatttatcctattttttgtacaacctgtatttcaaggtaaccgaatactgttaaagagaagctatttgcagaataattctgaccaataattatgtaaaaaaaaacctgaatctcatcattttgcaacctctgatgatatcacggatttaggtattgctaaaaccatcaggtgatagatgatcaggctgataacacgtgcacctgctgccaaccttaacataaaaaataatactaaattcccctgtgaagcctgcatgtgccccaaaacccccaaatcaaaacaaacccctcaaaacctgagttaaagcaagcttctagatctaacttctagcttacaaaaaatgagaggaagagaggactataccactaagaaaatgcaaccagaaaattccagattgcaaaaaatgtaataggaccaaaaccctgagttcttcaataaatacatgacaatttatagcttaaaagagacatagggacaggagagccaaatgcagtgtgtggaacttgtttagatcctgatttgaacaaatcaactctaaaaagacttatgagacagtggggagaatgtgaactatgatggggtatctgatggtattaaggaagtattaattttttttttttttagtgtagatatagacttttaaaggtaaaaagaaagaataaagatggagggtgtgataatcctatgaagtgtctgggtttgggtcctgagggcagccaattacatcccagactcactggcaatcaacagtccaagccagggtcccatcagctgaatcctgaggtggggatgcttcagtctttacagaacagggtcaaggaagagtccagaaaccgccgtcattggcttcatgaaaaccgagcacgtctttgagatctttttcaaattctgcctctaagtcaagtcctacctggccaaagtcagaagccagctggtcctgaggctgcatctgcctctccagggtcttagatacatgatggcactgttggcttcctgaagacctcttcatcctgcagaaggtgcaactccacagcatcctcttggcttccacaggggggatgtgacagtcctcatggaagactcgtggacaagtaccgcagcagagaagttgtcccccttgacagcacacctcgcattcatccgagtttttccgcttcagcagctctcctagggtcattccttcacaacgtatattccgtttccagttctttgcgttccttccttttccttcgacttcaaattcatttggtgttaaccaagttccatcctcattccgaatgcacttcactgaggatccgtgtttcattttcttcttatataaaatccctttcgcctcaccacaggtcacggggagcttagaacagtgaaaatccacagtgtcacttttgggttttcctcttcggtgaatatttttctgaaatctcctttttgagcttgaacagatatctttctcctttttcttttctttcaatctggactttcgggcacatttagttcttgccttttggaccctcatcatgacctctgagttccaggttgagtcgtctttcctttgagtcaccttatccaccacttggagcttctcttggatgccatgcccaggtgaggctgccccttgtgtgacccttcgtggtgtactaggcgtcttctgggacctctttccttcattcatttctgaagtgccatcaatgatctctcctgggaggctttttttcttatgtctcctttttggagttgaccagatacatctttttcttttctttcctttcttgtctgaaggtgtgctggacacctcctggggctcttctgggtcatttggttctggagaattatctcttatctctggcatagagcccaagggagagtggggcatctcttgagggtcttctttatctcttatttgggggatcaggttgtcactggccacttgcacagtgctagtgaggaggctgggcatctcttctgagtcttcttccgcattcattttggatgttaacttgtcattggtcactgaagtgcttcttccttcctggatgagtgcagggagaggcaggacagggtcagatgggctgggcgactcactcaggatctcatcgctttgctgggaggatgttccaggctcactgactcttggcgcacagggtgaacagcttggttgagggggttgtggtgggggcagcgccagtggggtatggagggagcttccttctgctaggccagttggggcttcaagtaggattggtgtgtctctgctctgccattcataggaagcaccaacacgtttgaagcttctgtaaatcgtcaccagattgggatattcacgcaggttaatttgactgaacaatgtcaccagaagagacaggttaaaagtcctctccagttgggtgagaatgttgtgcaccactctggatacagggatcaaatttctacaggcttccagagattccatgtacattctcttagtgatgatggagttgtctaggaggccttcaaagaagggaaatggcttgtgtatggcataggcgatccccagcttctggtgcatgaagtgctgaaaaagagcctcttccatggctcttgtcatggtgaacatcctgaagcccctccccatcacctggaaagccccttcatgggcatctgaggatcctggcagcaagaacttcttcctttagatctcaaaacaactttgatctgcttgagttgaatgacttttccaccctctttccttggcaggaacaagtgaccctgtcttccgtggcctcgtggggctggctctgctcctcctcccttgactgagagacgtcatggagattgggtggagggaggactgtagagttggtgcacccacgtcagctagttaggcaatttc

SEQ ID NO: 12029 - RNA, 4228 nt, Homo sapiens
  source 1..4228: mol_type = other RNA
ctgaatagctgggactacaggtgtgtgccaccttgcccagctaattaaaaagatttttttttttttttttttgtagagatgaggttttgccatgttacccaggctggtcttcaactcctggactcaagcgatccacctgcctcggcctcctaaagtgctgggatttcaggtgtgagccactgtgcccagcccgaagaagctttatctgatctgaacctgatttagataaggaggtcctggactttgttccaatgctgcagagagtgagacttctgtggggagaggagtgtcctttgcatttgggaaagatgtgaactactgtggccagagggtgaactatggtagattgcttctaaagatgggagcagcaatgtttcttcccaagcaacattctcctttgaaatgtgactttgccacccatcgcatcaagaggtaaggtctattctccctccttctgaatctgtccctgtgacttgctttcaccaatagattgtggcagaagtgacagtgtgcaagtatgaatggggtctgccagtaccatgtggagcaaagggaagcatcctcatggatgatgcctgaattcttgatccacagaatagtgagcaataaaatgtttttttctttttaagcagctaagctttgaggtcatttgttacacagcaatagatagctaatacaccatcaaagagttctggggtcatttcaaaacaactcaggaggcaaattgaggagtttctcactaaaagtggggaacttgcacatgcctgtaatcccagctactcggaggctgaggcaggagaatcgcttgcacccaggaggaggaggttgcagtgagtcaagatgacgctactgtactccggcctgggtgacagagtgagactctgtctcaaaaaaaaaaaaaaaaaaaaaaaaagaaaaagtgggcaactcaagcatcaataaaggtattaactgcaatggtttgtagcatgctacgtatatttaaatatgtgggttcaagataattaaattaaaaaatccctggttacctttagaggatattgggacatcaattcattattttgaacattgctaaataaaaaaacaagcatttatcctattttttgtacaacctgtatttcaaggtaaccgaatactgttaaagagaagctatttgcagaataattctgaccaataattatgtaaaaaaaaacctgaatctcatcattttgcaacctctgatgatatcacggatttaggtattgctaaaaccatcaggtgatagatgatcaggctgataacacgtgcacctgctgccaaccttaacataaaaaataatactaaattcccctgtgaagcctgcatgtgccccaaaacccccaaatcaaaacaaacccctcaaaacctgagttaaagcaagcttctagatctaacttctagcttacaaaaaatgagaggaagagaggactataccactaagaaaatgcaaccagaaaattccagattgcaaaaaatgtaataggaccaaaaccctgagttcttcaataaatacatgacaatttatagcttaaaagagacatagggacaggagagccaaatgcagtgtgtggaacttgtttagatcctgatttgaacaaatcaactctaaaaagacttatgagacagtggggagaatgtgaactatgatggggtatctgatggtattaaggaagtattaattttttttttttttagtgtagatatagacttttaaaggtaaaaagaaagaataaagatggagggtgtgataatcctatgaagtgtctgggtttgggtcctgagggcagccaattacatcccagactcactggcaatcaacagtccaagccagggtcccatcagctgaatcctgaggtggggatgcttcagtctttacagaacagggtcaaggaagagtccagaaaccgccgtcattggcttcatgaaaaccgagcacgtctttgagatctttttcaaattctgcctctaagtcaagtcctacctggccaaagtcagaagccttgtaaaatgttttatggttgcgaaacatcaggcgcatgtctcgcacaaaccatgccaccgtgtacatttccgtaatcagcctttccttaaccaggtccaaccacattgcttcctgaaagggctcaccgtaatctcgaatattaaatgggatgcccgtaaaaaaggagctttgtggatgacagtaggccttcaagaggaggaactcacatttcagctggtcctgaggctgcatctgcctctccagggtcttagatacatgatggcactgttggcttcctgaagacctcttcatcctgcagaaggtgcaactccacagcatcctcttggcttccacaggggggatgtgacagtcctcatggaagactcgtggacaagtaccgcagcagagaagttgtcccccttgacagcacacctcgcattcatccgagtttttccgcttcagcagctctcctagggtcattccttcacaacgtatattccgtttccagttctttgcgttccttccttttccttcgacttcaaattcatttggtgttaaccaagttccatcctcattccgaatgcacttcactgaggatccgtgtttcattttcttcttatataaaatccctttcgcctcaccacaggtcacggggagcttagaacagtgaaaatccacagtgtcacttttgggttttcctcttcggtgaatatttttctgaaatctcctttttgagcttgaacagatatctttctcctttttcttttctttcaatctggactttcgggcacatttagttcttgccttttggaccctcatcatgacctctgagttccaggttgagtcgtctttcctttgagtcaccttatccaccacttggagcttctcttggatgccatgcccaggtgaggctgccccttgtgtgacccttcgtggtgtactaggcgtcttctgggacctctttccttcattcatttctgaagtgccatcaatgatctcctctgatctcgactttcgggcacattcagttctcgccttttgggcccttgtctctaccgtggagttacaagttgagtcatctttcttttgaggaacctgatccacccttttgagcttcttttggattccgtgtctagatgaggctgtccctcctgggaggctttttttcttatgtctcctttttggagttgaccagatacatctttttcttttctttcctttcttgtctgaaggtgtgctggacacctcctggggctcttctgggtcatttggttctggagaattatctcttatctctggcatagagcccaagggagagtggggcatctcttgagggtcttctttatctcttatttgggggatcaggttgtcactggccacttgcacagtgctagtgaggaggctgggcatctcttctgagtcttcttccgcattcattttggatgttaacttgtcattggtcactgaagtgcttcttccttcctggatgagtgcagggagaggcaggacagggtcagatgggctgggcgactcactcaggatctcatcgctttgctgggaggatgttccaggctcactgactcttggcgcacagggtgaacagcttggttgagggggttgtggtgggggcagcgccagtggggtatggagggagcttccttctgctaggccagttggggcttcaagtaggattggtgtgtctctgctctgccattcataggaagcaccaacacgtttgaagcttctgtaaatcgtcaccagattgggatattcacgcaggttaatttgactgaacaatgtcaccagaagagacaggttaaaagtcctctccagttgggtgagaatgttgtgcaccactctggatacagggatcaaatttctacaggcttccagagattccatgtacattctcttagtgatgatggagttgtctaggaggccttcaaagaagggaaatggcttgtgtatggcataggcgatccccagcttctggtgcatgaagtgctgaaaaagagcctcttccatggctcttgtcatggtgaacatcctgaagcccctccccatcacctggaaagccccttcatgggcatctgaggatcctggcagcaagaacttcttcctttagatctcaaaacaactttgatctgcttgagttgaatgacttttccaccctctttccttggcaggaacaagtgaccctgtcttccgtggcctcgtggggctggctct

SEQ ID NO: 12030 - RNA, 4157 nt, Homo sapiens
  source 1..4157: mol_type = other RNA
ctgaatagctgggactacaggtgtgtgccaccttgcccagctaattaaaaagatttttttttttttttttttgtagagatgaggttttgccatgttacccaggctggtcttcaactcctggactcaagcgatccacctgcctcggcctcctaaagtgctgggatttcaggtgtgagccactgtgcccagcccgaagaagctttatctgatctgaacctgatttagataaggaggtcctggactttgttccaatgctgcagagagtgagacttctgtggggagaggagtgtcctttgcatttgggaaagatgtgaactactgtggccagagggtgaactatggtagattgcttctaaagatgggagcagcaatgtttcttcccaagcaacattctcctttgaaatgtgactttgccacccatcgcatcaagaggtaaggtctattctccctccttctgaatctgtccctgtgacttgctttcaccaatagattgtggcagaagtgacagtgtgcaagtatgaatggggtctgccagtaccatgtggagcaaagggaagcatcctcatggatgatgcctgaattcttgatccacagaatagtgagcaataaaatgtttttttctttttaagcagctaagctttgaggtcatttgttacacagcaatagatagctaatacaccatcaaagagttctggggtcatttcaaaacaactcaggaggcaaattgaggagtttctcactaaaagtggggaacttgcacatgcctgtaatcccagctactcggaggctgaggcaggagaatcgcttgcacccaggaggaggaggttgcagtgagtcaagatgacgctactgtactccggcctgggtgacagagtgagactctgtctcaaaaaaaaaaaaaaaaaaaaaaaaagaaaaagtgggcaactcaagcatcaataaaggtattaactgcaatggtttgtagcatgctacgtatatttaaatatgtgggttcaagataattaaattaaaaaatccctggttacctttagaggatattgggacatcaattcattattttgaacattgctaaataaaaaaacaagcatttatcctattttttgtacaacctgtatttcaaggtaaccgaatactgttaaagagaagctatttgcagaataattctgaccaataattatgtaaaaaaaaacctgaatctcatcattttgcaacctctgatgatatcacggatttaggtattgctaaaaccatcaggtgatagatgatcaggctgataacacgtgcacctgctgccaaccttaacataaaaaataatactaaattcccctgtgaagcctgcatgtgccccaaaacccccaaatcaaaacaaacccctcaaaacctgagttaaagcaagcttctagatctaacttctagcttacaaaaaatgagaggaagagaggactataccactaagaaaatgcaaccagaaaattccagattgcaaaaaatgtaataggaccaaaaccctgagttcttcaataaatacatgacaatttatagcttaaaagagacatagggacaggagagccaaatgcagtgtgtggaacttgtttagatcctgatttgaacaaatcaactctaaaaagacttatgagacagtggggagaatgtgaactatgatggggtatctgatggtattaaggaagtattaattttttttttttttagtgtagatatagacttttaaaggtaaaaagaaagaataaagatggagggtgtgataatcctatgaagtgtctgggtttgggtcctgagggcagccaattacatcccagactcactggcaatcaacagtccaagccagggtcccatcagctgaatcctgaggtggggatgcttcagtctttacagaacagggtcaaggaagagtccagaaaccgccgtcattggcttcatgaaaaccgagcacgtctttgagatctttttcaaattctgcctctaagtcaagtcctacctggccaaagtcagaagccttgtaaaatgttttatggttgcgaaacatcaggcgcatgtctcgcacaaaccatgccaccgtgtacatttccgtaatcagcctttccttaaccaggtccaaccacattgcttcctgaaagggctcaccgtaatctcgaatattaaatgggatgcccgtaaaaaaggagctttgtggatgacagtaggccttcaagaggaggaactcacatttcagctggtcctgaggctgcatctgcctctccagggtcttagatacatgatggcactgttggcttcctgaagacctcttcatcctgcagaaggtgcaactccacagcatcctcttggcttccacaggggggatgtgacagtcctcatggaagactcgtggacaagtaccgcagcagagaagttgtcccccttgacagcacacctcgcattcatccgagtttttccgcttcagcagctctcctagggtcattccttcacaacgtatattccgtttccagttctttgcgttccttccttttccttcgacttcaaattcatttggtgttaaccaagttccatcctcattccgaatgcacttcactgaggatccgtgtttcattttcttcttatataaaatccctttcgcctcaccacaggtcacggggagcttagaacagtgaaaatccacagtgtcacttttgggttttcctcttcggtgaatatttttctgaaatctcctttttgagcttgaacagatatctttctcctttttcttttctttcaatctggactttcgggcacatttagttcttgccttttggaccctcatcatgacctctgagttccaggttgagtcgtctttcctttgagtcaccttatccaccacttggagcttctcttggatgccatgcccaggtgaggctgccccttgtgtgacccttcgtggtgtactaggcgtcttctgggacctctttccttcattcatttctgaagtgccatcaatgatctcctctgatctcgactttcgggcacattcagttctcgccttttgggcccttgtctctaccgtggagttacaagttgagtcatctttcttttgaggaacctgatccacccttttgagcttcttttggattccgtgtctagatgaggctgtccctcctgggaggctttttttcttatgtctcctttttggagttgaccagatacatctttttcttttctttcctttcttgtctgaaggtgtgctggacacctcctggggctcttctgggtcatttggttctggagaattatctcttatctctggcatagagcccaagggagagtggggcatctcttgagggtcttctttatctcttatttgggggatcaggttgtcactggccacttgcacagtgctagtgaggaggctgggcatctcttctgagtcttcttccgcattcattttggatgttaacttgtcattggtcactgaagtgcttcttccttcctggatgagtgcagggagaggcaggacagggtcagatgggctgggcgactcactcaggatctcatcgctttgctgggaggatgttccaggctcactgactcttggcgcacagggtgaacagcttggttgagggggttgtggtgggggcagcgccagtggggtatggagggagcttccttctgctaggccagttggggcttcaagtaggattggtgtgtctctgctctgccattcataggaagcaccaacacgtttgaagcttctgtaaatcgtcaccagattgggatattcacgcaggttaatttgactgaacaatgtcaccagaagagacaggttaaaagtcctctccagttgggtgagaatgttgtgcaccactctggatacagggatcaaatttctacaggcttccagagattccatgtacattctcttagtgatgatggagttgtctaggaggccttcaaagaagggaaatggcttgtgtatggcataggcgatccccagcttctggtgcatgaagtgctgaaaaagagcctcttccatggctcttgtcatggtgaacatcctggactttgagtttgtcgttcctgcccctttccaggggctgggacagggatcactcctcaagattgggagagttacagggagatgctagcaggcaaaacaggaagtctgt

SEQ ID NO: 12031 - RNA, 4156 nt, Homo sapiens
  source 1..4156: mol_type = other RNA
ctgaatagctgggactacaggtgtgtgccaccttgcccagctaattaaaaagatttttttttttttttttttgtagagatgaggttttgccatgttacccaggctggtcttcaactcctggactcaagcgatccacctgcctcggcctcctaaagtgctgggatttcaggtgtgagccactgtgcccagcccgaagaagctttatctgatctgaacctgatttagataaggaggtcctggactttgttccaatgctgcagagagtgagacttctgtggggagaggagtgtcctttgcatttgggaaagatgtgaactactgtggccagagggtgaactatggtagattgcttctaaagatgggagcagcaatgtttcttcccaagcaacattctcctttgaaatgtgactttgccacccatcgcatcaagaggtaaggtctattctccctccttctgaatctgtccctgtgacttgctttcaccaatagattgtggcagaagtgacagtgtgcaagtatgaatggggtctgccagtaccatgtggagcaaagggaagcatcctcatggatgatgcctgaattcttgatccacagaatagtgagcaataaaatgtttttttctttttaagcagctaagctttgaggtcatttgttacacagcaatagatagctaatacaccatcaaagagttctggggtcatttcaaaacaactcaggaggcaaattgaggagtttctcactaaaagtggggaacttgcacatgcctgtaatcccagctactcggaggctgaggcaggagaatcgcttgcacccaggaggaggaggttgcagtgagtcaagatgacgctactgtactccggcctgggtgacagagtgagactctgtctcaaaaaaaaaaaaaaaaaaaaaaaaagaaaaagtgggcaactcaagcatcaataaaggtattaactgcaatggtttgtagcatgctacgtatatttaaatatgtgggttcaagataattaaattaaaaaatccctggttacctttagaggatattgggacatcaattcattattttgaacattgctaaataaaaaaacaagcatttatcctattttttgtacaacctgtatttcaaggtaaccgaatactgttaaagagaagctatttgcagaataattctgaccaataattatgtaaaaaaaaacctgaatctcatcattttgcaacctctgatgatatcacggatttaggtattgctaaaaccatcaggtgatagatgatcaggctgataacacgtgcacctgctgccaaccttaacataaaaaataatactaaattcccctgtgaagcctgcatgtgccccaaaacccccaaatcaaaacaaacccctcaaaacctgagttaaagcaagcttctagatctaacttctagcttacaaaaaatgagaggaagagaggactataccactaagaaaatgcaaccagaaaattccagattgcaaaaaatgtaataggaccaaaaccctgagttcttcaataaatacatgacaatttatagcttaaaagagacatagggacaggagagccaaatgcagtgtgtggaacttgtttagatcctgatttgaacaaatcaactctaaaaagacttatgagacagtggggagaatgtgaactatgatggggtatctgatggtattaaggaagtattaattttttttttttttagtgtagatatagacttttaaaggtaaaaagaaagaataaagatggagggtgtgataatcctatgaagtgtctgggtttgggtcctgagggcagccaattacatcccagactcactggcaatcaacagtccaagccagggtcccatcagctgaatcctgaggtggggatgcttcagtctttacagaacagggtcaaggaagagtccagaaaccgccgtcattggcttcatgaaaaccgagcacgtctttgagatctttttcaaattctgcctctaagtcaagtcctacctggccaaagtcagaagccttgtaaaatgttttatggttgcgaaacatcaggcgcatgtctcgcacaaaccatgccaccgtgtacatttccgtaatcagcctttccttaaccaggtccaaccacattgcttcctgaaagggctcaccgtaatctcgaatcagctggtcctgaggctgcatctgcctctccagggtcttagatacatgatggcactgttggcttcctgaagacctcttcatcctgcagaaggtgcaactccacagcatcctcttggcttccacaggggggatgtgacagtcctcatggaagactcgtggacaagtaccgcagcagagaagttgtcccccttgacagcacacctcgcattcatccgagtttttccgcttcagcagctctcctagggtcattccttcacaacgtatattccgtttccagttctttgcgttccttccttttccttcgacttcaaattcatttggtgttaaccaagttccatcctcattccgaatgcacttcactgaggatccgtgtttcattttcttcttatataaaatccctttcgcctcaccacaggtcacggggagcttagaacagtgaaaatccacagtgtcacttttgggttttcctcttcggtgaatatttttctgaaatctcctttttgagcttgaacagatatctttctcctttttcttttctttcaatctggactttcgggcacatttagttcttgccttttggaccctcatcatgacctctgagttccaggttgagtcgtctttcctttgagtcaccttatccaccacttggagcttctcttggatgccatgcccaggtgaggctgccccttgtgtgacccttcgtggtgtactaggcgtcttctgggacctctttccttcattcatttctgaagtgccatcaatgatctcctctgatctcgactttcgggcacattcagttctcgccttttgggcccttgtctctaccgtggagttacaagttgagtcatctttcttttgaggaacctgatccacccttttgagcttcttttggattccgtgtctagatgaggctgtccctcctgggaggctttttttcttatgtctcctttttggagttgaccagatacatctttttcttttctttcctttcttgtctgaaggtgtgctggacacctcctggggctcttctgggtcatttggttctggagaattatctcttatctctggcatagagcccaagggagagtggggcatctcttgagggtcttctttatctcttatttgggggatcaggttgtcactggccacttgcacagtgctagtgaggaggctgggcatctcttctgagtcttcttccgcattcattttggatgttaacttgtcattggtcactgaagtgcttcttccttcctggatgagtgcagggagaggcaggacagggtcagatgggctgggcgactcactcaggatctcatcgctttgctgggaggatgttccaggctcactgactcttggcgcacagggtgaacagcttggttgagggggttgtggtgggggcagcgccagtggggtatggagggagcttccttctgctaggccagttggggcttcaagtaggattggtgtgtctctgctctgccattcataggaagcaccaacacgtttgaagcttctgtaaatcgtcaccagattgggatattcacgcaggttaatttgactgaacaatgtcaccagaagagacaggttaaaagtcctctccagttgggtgagaatgttgtgcaccactctggatacagggatcaaatttctacaggcttccagagattccatgtacattctcttagtgatgatggagttgtctaggaggccttcaaagaagggaaatggcttgtgtatggcataggcgatccccagcttctggtgcatgaagtgctgaaaaagagcctcttccatggctcttgtcatggtgaacatcctgaagcccctccccatcacctggaaagccccttcatgggcatctgaggatcctggcagcaagaacttcttcctttagatctcaaaacaactttgatctgcttgagttgaatgacttttccaccctctttccttggcaggaacaagtgaccctgtcttccgtggcctcgtggggctggctct

SEQ ID NO: 12032 - RNA, 4085 nt, Homo sapiens
  source 1..4085: mol_type = other RNA
ctgaatagctgggactacaggtgtgtgccaccttgcccagctaattaaaaagatttttttttttttttttttgtagagatgaggttttgccatgttacccaggctggtcttcaactcctggactcaagcgatccacctgcctcggcctcctaaagtgctgggatttcaggtgtgagccactgtgcccagcccgaagaagctttatctgatctgaacctgatttagataaggaggtcctggactttgttccaatgctgcagagagtgagacttctgtggggagaggagtgtcctttgcatttgggaaagatgtgaactactgtggccagagggtgaactatggtagattgcttctaaagatgggagcagcaatgtttcttcccaagcaacattctcctttgaaatgtgactttgccacccatcgcatcaagaggtaaggtctattctccctccttctgaatctgtccctgtgacttgctttcaccaatagattgtggcagaagtgacagtgtgcaagtatgaatggggtctgccagtaccatgtggagcaaagggaagcatcctcatggatgatgcctgaattcttgatccacagaatagtgagcaataaaatgtttttttctttttaagcagctaagctttgaggtcatttgttacacagcaatagatagctaatacaccatcaaagagttctggggtcatttcaaaacaactcaggaggcaaattgaggagtttctcactaaaagtggggaacttgcacatgcctgtaatcccagctactcggaggctgaggcaggagaatcgcttgcacccaggaggaggaggttgcagtgagtcaagatgacgctactgtactccggcctgggtgacagagtgagactctgtctcaaaaaaaaaaaaaaaaaaaaaaaaagaaaaagtgggcaactcaagcatcaataaaggtattaactgcaatggtttgtagcatgctacgtatatttaaatatgtgggttcaagataattaaattaaaaaatccctggttacctttagaggatattgggacatcaattcattattttgaacattgctaaataaaaaaacaagcatttatcctattttttgtacaacctgtatttcaaggtaaccgaatactgttaaagagaagctatttgcagaataattctgaccaataattatgtaaaaaaaaacctgaatctcatcattttgcaacctctgatgatatcacggatttaggtattgctaaaaccatcaggtgatagatgatcaggctgataacacgtgcacctgctgccaaccttaacataaaaaataatactaaattcccctgtgaagcctgcatgtgccccaaaacccccaaatcaaaacaaacccctcaaaacctgagttaaagcaagcttctagatctaacttctagcttacaaaaaatgagaggaagagaggactataccactaagaaaatgcaaccagaaaattccagattgcaaaaaatgtaataggaccaaaaccctgagttcttcaataaatacatgacaatttatagcttaaaagagacatagggacaggagagccaaatgcagtgtgtggaacttgtttagatcctgatttgaacaaatcaactctaaaaagacttatgagacagtggggagaatgtgaactatgatggggtatctgatggtattaaggaagtattaattttttttttttttagtgtagatatagacttttaaaggtaaaaagaaagaataaagatggagggtgtgataatcctatgaagtgtctgggtttgggtcctgagggcagccaattacatcccagactcactggcaatcaacagtccaagccagggtcccatcagctgaatcctgaggtggggatgcttcagtctttacagaacagggtcaaggaagagtccagaaaccgccgtcattggcttcatgaaaaccgagcacgtctttgagatctttttcaaattctgcctctaagtcaagtcctacctggccaaagtcagaagccttgtaaaatgttttatggttgcgaaacatcaggcgcatgtctcgcacaaaccatgccaccgtgtacatttccgtaatcagcctttccttaaccaggtccaaccacattgcttcctgaaagggctcaccgtaatctcgaatcagctggtcctgaggctgcatctgcctctccagggtcttagatacatgatggcactgttggcttcctgaagacctcttcatcctgcagaaggtgcaactccacagcatcctcttggcttccacaggggggatgtgacagtcctcatggaagactcgtggacaagtaccgcagcagagaagttgtcccccttgacagcacacctcgcattcatccgagtttttccgcttcagcagctctcctagggtcattccttcacaacgtatattccgtttccagttctttgcgttccttccttttccttcgacttcaaattcatttggtgttaaccaagttccatcctcattccgaatgcacttcactgaggatccgtgtttcattttcttcttatataaaatccctttcgcctcaccacaggtcacggggagcttagaacagtgaaaatccacagtgtcacttttgggttttcctcttcggtgaatatttttctgaaatctcctttttgagcttgaacagatatctttctcctttttcttttctttcaatctggactttcgggcacatttagttcttgccttttggaccctcatcatgacctctgagttccaggttgagtcgtctttcctttgagtcaccttatccaccacttggagcttctcttggatgccatgcccaggtgaggctgccccttgtgtgacccttcgtggtgtactaggcgtcttctgggacctctttccttcattcatttctgaagtgccatcaatgatctcctctgatctcgactttcgggcacattcagttctcgccttttgggcccttgtctctaccgtggagttacaagttgagtcatctttcttttgaggaacctgatccacccttttgagcttcttttggattccgtgtctagatgaggctgtccctcctgggaggctttttttcttatgtctcctttttggagttgaccagatacatctttttcttttctttcctttcttgtctgaaggtgtgctggacacctcctggggctcttctgggtcatttggttctggagaattatctcttatctctggcatagagcccaagggagagtggggcatctcttgagggtcttctttatctcttatttgggggatcaggttgtcactggccacttgcacagtgctagtgaggaggctgggcatctcttctgagtcttcttccgcattcattttggatgttaacttgtcattggtcactgaagtgcttcttccttcctggatgagtgcagggagaggcaggacagggtcagatgggctgggcgactcactcaggatctcatcgctttgctgggaggatgttccaggctcactgactcttggcgcacagggtgaacagcttggttgagggggttgtggtgggggcagcgccagtggggtatggagggagcttccttctgctaggccagttggggcttcaagtaggattggtgtgtctctgctctgccattcataggaagcaccaacacgtttgaagcttctgtaaatcgtcaccagattgggatattcacgcaggttaatttgactgaacaatgtcaccagaagagacaggttaaaagtcctctccagttgggtgagaatgttgtgcaccactctggatacagggatcaaatttctacaggcttccagagattccatgtacattctcttagtgatgatggagttgtctaggaggccttcaaagaagggaaatggcttgtgtatggcataggcgatccccagcttctggtgcatgaagtgctgaaaaagagcctcttccatggctcttgtcatggtgaacatcctggactttgagtttgtcgttcctgcccctttccaggggctgggacagggatcactcctcaagattgggagagttacagggagatgctagcaggcaaaacaggaagtctgt

SEQ ID NO: 12033 - RNA, 4306 nt, Homo sapiens
  source 1..4306: mol_type = other RNA
ctgaatagctgggactacaggtgtgtgccaccttgcccagctaattaaaaagatttttttttttttttttttgtagagatgaggttttgccatgttacccaggctggtcttcaactcctggactcaagcgatccacctgcctcggcctcctaaagtgctgggatttcaggtgtgagccactgtgcccagcccgaagaagctttatctgatctgaacctgatttagataaggaggtcctggactttgttccaatgctgcagagagtgagacttctgtggggagaggagtgtcctttgcatttgggaaagatgtgaactactgtggccagagggtgaactatggtagattgcttctaaagatgggagcagcaatgtttcttcccaagcaacattctcctttgaaatgtgactttgccacccatcgcatcaagaggtaaggtctattctccctccttctgaatctgtccctgtgacttgctttcaccaatagattgtggcagaagtgacagtgtgcaagtatgaatggggtctgccagtaccatgtggagcaaagggaagcatcctcatggatgatgcctgaattcttgatccacagaatagtgagcaataaaatgtttttttctttttaagcagctaagctttgaggtcatttgttacacagcaatagatagctaatacaccatcaaagagttctggggtcatttcaaaacaactcaggaggcaaattgaggagtttctcactaaaagtggggaacttgcacatgcctgtaatcccagctactcggaggctgaggcaggagaatcgcttgcacccaggaggaggaggttgcagtgagtcaagatgacgctactgtactccggcctgggtgacagagtgagactctgtctcaaaaaaaaaaaaaaaaaaaaaaaaagaaaaagtgggcaactcaagcatcaataaaggtattaactgcaatggtttgtagcatgctacgtatatttaaatatgtgggttcaagataattaaattaaaaaatccctggttacctttagaggatattgggacatcaattcattattttgaacattgctaaataaaaaaacaagcatttatcctattttttgtacaacctgtatttcaaggtaaccgaatactgttaaagagaagctatttgcagaataattctgaccaataattatgtaaaaaaaaacctgaatctcatcattttgcaacctctgatgatatcacggatttaggtattgctaaaaccatcaggtgatagatgatcaggctgataacacgtgcacctgctgccaaccttaacataaaaaataatactaaattcccctgtgaagcctgcatgtgccccaaaacccccaaatcaaaacaaacccctcaaaacctgagttaaagcaagcttctagatctaacttctagcttacaaaaaatgagaggaagagaggactataccactaagaaaatgcaaccagaaaattccagattgcaaaaaatgtaataggaccaaaaccctgagttcttcaataaatacatgacaatttatagcttaaaagagacatagggacaggagagccaaatgcagtgtgtggaacttgtttagatcctgatttgaacaaatcaactctaaaaagacttatgagacagtggggagaatgtgaactatgatggggtatctgatggtattaaggaagtattaattttttttttttttagtgtagatatagacttttaaaggtaaaaagaaagaataaagatggagggtgtgataatcctatgaagtgtctgggtttgggtcctgagggcagccaattacatcccagactcactggcaatcaacagtccaagccagggtcccatcagctgaatcctgaggtggggatgcttcagtctttacagaacagggtcaaggaagagtccagaaaccgccgtcattggcttcatgaaaaccgagcacgtctttgagatctttttcaaattctgcctctaagtcaagtcctacctggccaaagtcagaagccttgtaaaatgttttatggttgcgaaacatcaggcgcatgtctcgcacaaaccatgccaccgtgtacatttccgtaatcagcctttccttaaccaggtccaaccacattgcttcctgaaagggctcaccgtaatctcgaatccggtatcccagagcccgtgagcagtggggtggagtttgaaccaggtagtccctctccagagtgtgcagcaaaatccctgctgccccgctccactgctgccacgctgcccttctcttctgttctccagcttcctgagcaaactgcagcaccagctggtcctgaggctgcatctgcctctccagggtcttagatacatgatggcactgttggcttcctgaagacctcttcatcctgcagaaggtgcaactccacagcatcctcttggcttccacaggggggatgtgacagtcctcatggaagactcgtggacaagtaccgcagcagagaagttgtcccccttgacagcacacctcgcattcatccgagtttttccgcttcagcagctctcctagggtcattccttcacaacgtatattccgtttccagttctttgcgttccttccttttccttcgacttcaaattcatttggtgttaaccaagttccatcctcattccgaatgcacttcactgaggatccgtgtttcattttcttcttatataaaatccctttcgcctcaccacaggtcacggggagcttagaacagtgaaaatccacagtgtcacttttgggttttcctcttcggtgaatatttttctgaaatctcctttttgagcttgaacagatatctttctcctttttcttttctttcaatctggactttcgggcacatttagttcttgccttttggaccctcatcatgacctctgagttccaggttgagtcgtctttcctttgagtcaccttatccaccacttggagcttctcttggatgccatgcccaggtgaggctgccccttgtgtgacccttcgtggtgtactaggcgtcttctgggacctctttccttcattcatttctgaagtgccatcaatgatctcctctgatctcgactttcgggcacattcagttctcgccttttgggcccttgtctctaccgtggagttacaagttgagtcatctttcttttgaggaacctgatccacccttttgagcttcttttggattccgtgtctagatgaggctgtccctcctgggaggctttttttcttatgtctcctttttggagttgaccagatacatctttttcttttctttcctttcttgtctgaaggtgtgctggacacctcctggggctcttctgggtcatttggttctggagaattatctcttatctctggcatagagcccaagggagagtggggcatctcttgagggtcttctttatctcttatttgggggatcaggttgtcactggccacttgcacagtgctagtgaggaggctgggcatctcttctgagtcttcttccgcattcattttggatgttaacttgtcattggtcactgaagtgcttcttccttcctggatgagtgcagggagaggcaggacagggtcagatgggctgggcgactcactcaggatctcatcgctttgctgggaggatgttccaggctcactgactcttggcgcacagggtgaacagcttggttgagggggttgtggtgggggcagcgccagtggggtatggagggagcttccttctgctaggccagttggggcttcaagtaggattggtgtgtctctgctctgccattcataggaagcaccaacacgtttgaagcttctgtaaatcgtcaccagattgggatattcacgcaggttaatttgactgaacaatgtcaccagaagagacaggttaaaagtcctctccagttgggtgagaatgttgtgcaccactctggatacagggatcaaatttctacaggcttccagagattccatgtacattctcttagtgatgatggagttgtctaggaggccttcaaagaagggaaatggcttgtgtatggcataggcgatccccagcttctggtgcatgaagtgctgaaaaagagcctcttccatggctcttgtcatggtgaacatcctgaagcccctccccatcacctggaaagccccttcatgggcatctgaggatcctggcagcaagaacttcttcctttagatctcaaaacaactttgatctgcttgagttgaatgacttttccaccctctttccttggcaggaacaagtgaccctgtcttccgtggcctcgtggggctggctct

SEQ ID NO: 12034 - RNA, 4235 nt, Homo sapiens
  source 1..4235: mol_type = other RNA
ctgaatagctgggactacaggtgtgtgccaccttgcccagctaattaaaaagatttttttttttttttttttgtagagatgaggttttgccatgttacccaggctggtcttcaactcctggactcaagcgatccacctgcctcggcctcctaaagtgctgggatttcaggtgtgagccactgtgcccagcccgaagaagctttatctgatctgaacctgatttagataaggaggtcctggactttgttccaatgctgcagagagtgagacttctgtggggagaggagtgtcctttgcatttgggaaagatgtgaactactgtggccagagggtgaactatggtagattgcttctaaagatgggagcagcaatgtttcttcccaagcaacattctcctttgaaatgtgactttgccacccatcgcatcaagaggtaaggtctattctccctccttctgaatctgtccctgtgacttgctttcaccaatagattgtggcagaagtgacagtgtgcaagtatgaatggggtctgccagtaccatgtggagcaaagggaagcatcctcatggatgatgcctgaattcttgatccacagaatagtgagcaataaaatgtttttttctttttaagcagctaagctttgaggtcatttgttacacagcaatagatagctaatacaccatcaaagagttctggggtcatttcaaaacaactcaggaggcaaattgaggagtttctcactaaaagtggggaacttgcacatgcctgtaatcccagctactcggaggctgaggcaggagaatcgcttgcacccaggaggaggaggttgcagtgagtcaagatgacgctactgtactccggcctgggtgacagagtgagactctgtctcaaaaaaaaaaaaaaaaaaaaaaaaagaaaaagtgggcaactcaagcatcaataaaggtattaactgcaatggtttgtagcatgctacgtatatttaaatatgtgggttcaagataattaaattaaaaaatccctggttacctttagaggatattgggacatcaattcattattttgaacattgctaaataaaaaaacaagcatttatcctattttttgtacaacctgtatttcaaggtaaccgaatactgttaaagagaagctatttgcagaataattctgaccaataattatgtaaaaaaaaacctgaatctcatcattttgcaacctctgatgatatcacggatttaggtattgctaaaaccatcaggtgatagatgatcaggctgataacacgtgcacctgctgccaaccttaacataaaaaataatactaaattcccctgtgaagcctgcatgtgccccaaaacccccaaatcaaaacaaacccctcaaaacctgagttaaagcaagcttctagatctaacttctagcttacaaaaaatgagaggaagagaggactataccactaagaaaatgcaaccagaaaattccagattgcaaaaaatgtaataggaccaaaaccctgagttcttcaataaatacatgacaatttatagcttaaaagagacatagggacaggagagccaaatgcagtgtgtggaacttgtttagatcctgatttgaacaaatcaactctaaaaagacttatgagacagtggggagaatgtgaactatgatggggtatctgatggtattaaggaagtattaattttttttttttttagtgtagatatagacttttaaaggtaaaaagaaagaataaagatggagggtgtgataatcctatgaagtgtctgggtttgggtcctgagggcagccaattacatcccagactcactggcaatcaacagtccaagccagggtcccatcagctgaatcctgaggtggggatgcttcagtctttacagaacagggtcaaggaagagtccagaaaccgccgtcattggcttcatgaaaaccgagcacgtctttgagatctttttcaaattctgcctctaagtcaagtcctacctggccaaagtcagaagccttgtaaaatgttttatggttgcgaaacatcaggcgcatgtctcgcacaaaccatgccaccgtgtacatttccgtaatcagcctttccttaaccaggtccaaccacattgcttcctgaaagggctcaccgtaatctcgaatccggtatcccagagcccgtgagcagtggggtggagtttgaaccaggtagtccctctccagagtgtgcagcaaaatccctgctgccccgctccactgctgccacgctgcccttctcttctgttctccagcttcctgagcaaactgcagcaccagctggtcctgaggctgcatctgcctctccagggtcttagatacatgatggcactgttggcttcctgaagacctcttcatcctgcagaaggtgcaactccacagcatcctcttggcttccacaggggggatgtgacagtcctcatggaagactcgtggacaagtaccgcagcagagaagttgtcccccttgacagcacacctcgcattcatccgagtttttccgcttcagcagctctcctagggtcattccttcacaacgtatattccgtttccagttctttgcgttccttccttttccttcgacttcaaattcatttggtgttaaccaagttccatcctcattccgaatgcacttcactgaggatccgtgtttcattttcttcttatataaaatccctttcgcctcaccacaggtcacggggagcttagaacagtgaaaatccacagtgtcacttttgggttttcctcttcggtgaatatttttctgaaatctcctttttgagcttgaacagatatctttctcctttttcttttctttcaatctggactttcgggcacatttagttcttgccttttggaccctcatcatgacctctgagttccaggttgagtcgtctttcctttgagtcaccttatccaccacttggagcttctcttggatgccatgcccaggtgaggctgccccttgtgtgacccttcgtggtgtactaggcgtcttctgggacctctttccttcattcatttctgaagtgccatcaatgatctcctctgatctcgactttcgggcacattcagttctcgccttttgggcccttgtctctaccgtggagttacaagttgagtcatctttcttttgaggaacctgatccacccttttgagcttcttttggattccgtgtctagatgaggctgtccctcctgggaggctttttttcttatgtctcctttttggagttgaccagatacatctttttcttttctttcctttcttgtctgaaggtgtgctggacacctcctggggctcttctgggtcatttggttctggagaattatctcttatctctggcatagagcccaagggagagtggggcatctcttgagggtcttctttatctcttatttgggggatcaggttgtcactggccacttgcacagtgctagtgaggaggctgggcatctcttctgagtcttcttccgcattcattttggatgttaacttgtcattggtcactgaagtgcttcttccttcctggatgagtgcagggagaggcaggacagggtcagatgggctgggcgactcactcaggatctcatcgctttgctgggaggatgttccaggctcactgactcttggcgcacagggtgaacagcttggttgagggggttgtggtgggggcagcgccagtggggtatggagggagcttccttctgctaggccagttggggcttcaagtaggattggtgtgtctctgctctgccattcataggaagcaccaacacgtttgaagcttctgtaaatcgtcaccagattgggatattcacgcaggttaatttgactgaacaatgtcaccagaagagacaggttaaaagtcctctccagttgggtgagaatgttgtgcaccactctggatacagggatcaaatttctacaggcttccagagattccatgtacattctcttagtgatgatggagttgtctaggaggccttcaaagaagggaaatggcttgtgtatggcataggcgatccccagcttctggtgcatgaagtgctgaaaaagagcctcttccatggctcttgtcatggtgaacatcctggactttgagtttgtcgttcctgcccctttccaggggctgggacagggatcactcctcaagattgggagagttacagggagatgctagcaggcaaaacaggaagtctgt

SEQ ID NO: 12035 - RNA, 3840 nt, Homo sapiens
  source 1..3840: mol_type = other RNA
ctgaatagctgggactacaggtgtgtgccaccttgtctggctaaattttttattatttgtagagacagagtctcactgtgttgcccaggctgttctcaaatttctggcctcaagcaatcctcactccttggtctcccagaatgtgttgggattacaggtgtgagccactgtgcccagccttgtattttgatttttaaattaatttatatgaatatttccttttaccctataatgtatcagggcttaatatttttaaacttcattataaaaagttgattacagaaagtggtatcttctagttgggagccatctttgcacatctctctccaactctgcctttagtgatatgtcaataacaaattggccatggcaggagtattttacaccatggaaagtgataaatgcagcaaatcaaggaattcccctcctgttgtcccctcagaaagccagcttcccagcacctcatcaatttcaaatataaaaaaagaatagtaaattttcatgtacacatcactcagcttcagtaattgtcgtctcatagccagtttttcctctcctatcctcaaggtataccaggtacactggaggtgtattctctagcctgatacccagtggcatttgtcttaaagccaaacatttttgtctagaaattatctaaaaaaatgtagatcatgtctagaaagtcaatcccacaaccaagagataggtaaaaatcatgttaggagtgcatttctattaatttactgagatcactgttaagagcagtgattcttgatccatatatcacctgttaagtagtgaccttgctgcctctgtttttgcagtaaatattagctgttgtttattgagctgtattagatactatatgatgtataattatgtatgaattaactatcatttaattctgataatcctagtaaatgtactacaggttgagtattcctaatctggtaatctgaaatttcacatgctccgaaaatcacaaactttttgagtgccaacatgatgctcaaagaaaatgctcattgcagcatttaagatttcagatttttgggttaggaatgttgaactggtataatgcaaatactccaaaatctgaagaaatccaaagtcttaaatacttctggtcccaagcacttcagataaaggatactcaatttgtattcctattttggagataagagatggagacttacaggctgggttggttggattggttgcctgttttttgttgttgttgtagtggaagctaggaatggtttttcacattttttaagtgtacttaagtcttacatggttacatagttacctgtataatagtcttgaatttgcctaaacccacgaagaataacagtatttgctatctggccctttaagaagtttgccaacctaggctggtctaaataatgaaaattttacattaatgaaagtattttcatggatagtattccttttgttcttagaatatttctttgaggtaggcagaatgtatgttttattccagaattactgttttacgcagttttaactttacaaacaaggcaaataatgctcaagagaagttgctatttagtaagcagcaaaataataactctgttgttttcccccgaagtacaaccaaatttaaatactgagtgaggaagcagtaaatatccaatgatatcttgagtttcttaagaatatcaatttagggttttaaaatgttttaaatattttacaaaaaagtactgaaacaactttgtcacttaggactattctcaggaaggagtgctttgttaagaacagagccatgattgacaaagtcagaagctttctagaaagtctttatttttctgttatgaataattgcattttctaattatcccaaatgattttataaattccgtaacttttatatgcctgcctgggatccatgaaataaaagtattccttaccaaaagagaagcatcagatacactgaaaggctcaatgttttatattttcagaaataaaagtgactgtatacccttttattaactatatggtagcttggtaaaatttttatagaatttttaatgatctatggtgttctatgatgaggcaacattccaccaaattagccttccaaaagttgcagtatcatgtataattatgacagcagttttgttttaaaaccagagtcagattgaatgtagcttttttacagctgaaatttatgccttatgtgtattcataaaacattgataacttagtgtcacattatctttactctttggttatactcttcttgaaaagtaaatttacttatcaaatgataaagtttcagggaaagttaaaaaaagttttttttcttaaggcttcatggaatagaattccatgaatcataatgactacgtaagacccttttctggtaatgaaagcatggagtcttaaccaaaaagctaagcagaattgttagatcttttggtttctgtcataatgtactattggaacttcaagtagatatagtacattaatatgaaatactttgaaatacaccatctttaaaaaaaaaggcacttacacaaaaatcatgtaacactaggtaggatgttgaaatgactggtatgcaatattttttaaagccttcatttttggtcagcataagtttcctttaattatttttctgtttccagttggacttcactttgaggcttaacatagcaaagtgagtataaagttctacaatttagtcattgtggatttcaagtcatttatgatgaaaatggaaatgtgtagtttacttaagaaaattttcttcttctgtaacatctaactcgtcatcctcatcatcttctgcttgttgatcctttcttagtcgacaagtggatacctaaaagttgtatcttgaaaataagtttgttgaattttatattctgaaggctagatatgaaaagggcatagctctctagatcagggtttggcaagttgcggcccagccagcctcctgtcctgttccagatacacacttagctgacagtgatctctgaagaggtgactttgaatttgctcttacaatatctaaacgagatgaataatctggtgcatacagagaatttcggaaaacctctaaatcttcatcttcatcaatgttttgtatattctggtaggcagcagtgtagacctctaaagctttgccgtgaaataacatttcgattgtgataaattcagaaaatatagtctttatatccttcattttctgcctttcaaagttgttaatagtttcctccagatgacgacttgttcggctagcatccattgcagctctctgtaattccgtttctgcctgtgaaataacatgtcgatcagatgggtttcgctgacgtgttctttctaactgagttaattgcttagcttctcgattccttgctgtgagtgttgctttgaggtcatcccgtttcattttcacaatggtcccataagttttcaagggttcaactactttggcttcaagtctttcaacctctgcttgtcgataatcctgaagtttggcaaactcatctgcaaagttcatcaggcccagctttaaatgcggggtctctgtagcagcatacgcgttaatttcattcaccaggaggtctgctttgtctctcagcctggcagttttccgcacataggcagcgaagatttggcacagttctccaaaatgcttctccacatttgagacagctgtttgcagttgtttcgtttgagcgttccggttttccagggtgcgcctcatcatgctgcctcgcgcacggccggggaccttgcgggggcccaaggacggggattccaaggcgcctgggcgcgcgctggggcgcaagcagccgccgggagcct

SEQ ID NO: 12036 - RNA, 3800 nt, Homo sapiens
  source 1..3800: mol_type = other RNA
ctgaatagctgggactacaggtgtgtgccaccttgtctggctaaattttttattatttgtagagacagagtctcactgtgttgcccaggctgttctcaaatttctggcctcaagcaatcctcactccttggtctcccagaatgtgttgggattacaggtgtgagccactgtgcccagccttgtattttgatttttaaattaatttatatgaatatttccttttaccctataatgtatcagggcttaatatttttaaacttcattataaaaagttgattacagaaagtggtatcttctagttgggagccatctttgcacatctctctccaactctgcctttagtgatatgtcaataacaaattggccatggcaggagtattttacaccatggaaagtgataaatgcagcaaatcaaggaattcccctcctgttgtcccctcagaaagccagcttcccagcacctcatcaatttcaaatataaaaaaagaatagtaaattttcatgtacacatcactcagcttcagtaattgtcgtctcatagccagtttttcctctcctatcctcaaggtataccaggtacactggaggtgtattctctagcctgatacccagtggcatttgtcttaaagccaaacatttttgtctagaaattatctaaaaaaatgtagatcatgtctagaaagtcaatcccacaaccaagagataggtaaaaatcatgttaggagtgcatttctattaatttactgagatcactgttaagagcagtgattcttgatccatatatcacctgttaagtagtgaccttgctgcctctgtttttgcagtaaatattagctgttgtttattgagctgtattagatactatatgatgtataattatgtatgaattaactatcatttaattctgataatcctagtaaatgtactacaggttgagtattcctaatctggtaatctgaaatttcacatgctccgaaaatcacaaactttttgagtgccaacatgatgctcaaagaaaatgctcattgcagcatttaagatttcagatttttgggttaggaatgttgaactggtataatgcaaatactccaaaatctgaagaaatccaaagtcttaaatacttctggtcccaagcacttcagataaaggatactcaatttgtattcctattttggagataagagatggagacttacaggctgggttggttggattggttgcctgttttttgttgttgttgtagtggaagctaggaatggtttttcacattttttaagtgtacttaagtcttacatggttacatagttacctgtataatagtcttgaatttgcctaaacccacgaagaataacagtatttgctatctggccctttaagaagtttgccaacctaggctggtctaaataatgaaaattttacattaatgaaagtattttcatggatagtattccttttgttcttagaatatttctttgaggtaggcagaatgtatgttttattccagaattactgttttacgcagttttaactttacaaacaaggcaaataatgctcaagagaagttgctatttagtaagcagcaaaataataactctgttgttttcccccgaagtacaaccaaatttaaatactgagtgaggaagcagtaaatatccaatgatatcttgagtttcttaagaatatcaatttagggttttaaaatgttttaaatattttacaaaaaagtactgaaacaactttgtcacttaggactattctcaggaaggagtgctttgttaagaacagagccatgattgacaaagtcagaagctttctagaaagtctttatttttctgttatgaataattgcattttctaattatcccaaatgattttataaattccgtaacttttatatgcctgcctgggatccatgaaataaaagtattccttaccaaaagagaagcatcagatacactgaaaggctcaatgttttatattttcagaaataaaagtgactgtatacccttttattaactatatggtagcttggtaaaatttttatagaatttttaatgatctatggtgttctatgatgaggcaacattccaccaaattagccttccaaaagttgcagtatcatgtataattatgacagcagttttgttttaaaaccagagtcagattgaatgtagcttttttacagctgaaatttatgccttatgtgtattcataaaacattgataacttagtgtcacattatctttactctttggttatactcttcttgaaaagtaaatttacttatcaaatgataaagtttcagggaaagttaaaaaaagttttttttcttaaggcttcatggaatagaattccatgaatcataatgactacgtaagacccttttctggtaatgaaagcatggagtcttaaccaaaaagctaagcagaattgttagatcttttggtttctgtcataatgtactattggaacttcaagtagatatagtacattaatatgaaatactttgaaatacaccatctttaaaaaaaaaggcacttacacaaaaatcatgtaacactaggtaggatgttgaaatgactggtatgcaatattttttaaagccttcatttttggtcagcataagtttcctttaattatttttctgtttccagttggacttcactttgaggcttaacatagcaaagtgagtataaagttctacaatttagtcattgtggatttcaagtcatttatgatgaaaatggaaatgtgtagtttacttaagaaaattttcttcttctgtaacatctaactcgtcatcctcatcatcttctgcttgttgatcctttcttagtcgacaagtggatacctgtcctgttccagatacacacttagctgacagtgatctctgaagaggtgactttgaatttgctcttacaatatctaaacgagatgaataatctggtgcatacagagaatttcggaaaacctctaaatcttcatcttcatcaatgttttgtatattctggtaggcagcagtgtagacctctaaagctttgccgtgaaataacatttcgattgtgataaattcagaaaatatagtctttatatccttcattttctgcctttcaaagttgttaatagtttcctccagatgacgacttgttcggctagcatccattgcagctctctgtaattccgtttctgcctaaagtaacacatccatttttagcaaagagaatatagatttctaatatttcttcttttcactgaaaattcttcaaaattaataacatgtcgatcagatgggtttcgctgacgtgttctttctaactgagttaattgcttagcttctcgattccttgctgtgagtgttgctttgaggtcatcccgtttcattttcacaatggtcccataagttttcaagggttcaactactttggcttcaagtctttcaacctctgcttgtcgataatcctgaagtttggcaaactcatctgcaaagttcatcaggcccagctttaaatgcggggtctctgtagcagcatacgcgttaatttcattcaccaggaggtctgctttgtctctcagcctggcagttttccgcacataggcagcgaagatttggcacagttctccaaaatgcttctccacatttgagacagctgtttgcagttgtttcgtttgagcgttccggttttccagggtgcgcctcatcatgctgcctcgcgcacggccggggaccttgcgggggcccaaggacggggattccaaggcgcctgggcgcgcgctggggcgcaagcagccgccgggagcct

SEQ ID NO: 12037 - RNA, 3726 nt, Homo sapiens
  source 1..3726: mol_type = other RNA
ctgaatagctgggactacaggtgtgtgccaccttgtctggctaaattttttattatttgtagagacagagtctcactgtgttgcccaggctgttctcaaatttctggcctcaagcaatcctcactccttggtctcccagaatgtgttgggattacaggtgtgagccactgtgcccagccttgtattttgatttttaaattaatttatatgaatatttccttttaccctataatgtatcagggcttaatatttttaaacttcattataaaaagttgattacagaaagtggtatcttctagttgggagccatctttgcacatctctctccaactctgcctttagtgatatgtcaataacaaattggccatggcaggagtattttacaccatggaaagtgataaatgcagcaaatcaaggaattcccctcctgttgtcccctcagaaagccagcttcccagcacctcatcaatttcaaatataaaaaaagaatagtaaattttcatgtacacatcactcagcttcagtaattgtcgtctcatagccagtttttcctctcctatcctcaaggtataccaggtacactggaggtgtattctctagcctgatacccagtggcatttgtcttaaagccaaacatttttgtctagaaattatctaaaaaaatgtagatcatgtctagaaagtcaatcccacaaccaagagataggtaaaaatcatgttaggagtgcatttctattaatttactgagatcactgttaagagcagtgattcttgatccatatatcacctgttaagtagtgaccttgctgcctctgtttttgcagtaaatattagctgttgtttattgagctgtattagatactatatgatgtataattatgtatgaattaactatcatttaattctgataatcctagtaaatgtactacaggttgagtattcctaatctggtaatctgaaatttcacatgctccgaaaatcacaaactttttgagtgccaacatgatgctcaaagaaaatgctcattgcagcatttaagatttcagatttttgggttaggaatgttgaactggtataatgcaaatactccaaaatctgaagaaatccaaagtcttaaatacttctggtcccaagcacttcagataaaggatactcaatttgtattcctattttggagataagagatggagacttacaggctgggttggttggattggttgcctgttttttgttgttgttgtagtggaagctaggaatggtttttcacattttttaagtgtacttaagtcttacatggttacatagttacctgtataatagtcttgaatttgcctaaacccacgaagaataacagtatttgctatctggccctttaagaagtttgccaacctaggctggtctaaataatgaaaattttacattaatgaaagtattttcatggatagtattccttttgttcttagaatatttctttgaggtaggcagaatgtatgttttattccagaattactgttttacgcagttttaactttacaaacaaggcaaataatgctcaagagaagttgctatttagtaagcagcaaaataataactctgttgttttcccccgaagtacaaccaaatttaaatactgagtgaggaagcagtaaatatccaatgatatcttgagtttcttaagaatatcaatttagggttttaaaatgttttaaatattttacaaaaaagtactgaaacaactttgtcacttaggactattctcaggaaggagtgctttgttaagaacagagccatgattgacaaagtcagaagctttctagaaagtctttatttttctgttatgaataattgcattttctaattatcccaaatgattttataaattccgtaacttttatatgcctgcctgggatccatgaaataaaagtattccttaccaaaagagaagcatcagatacactgaaaggctcaatgttttatattttcagaaataaaagtgactgtatacccttttattaactatatggtagcttggtaaaatttttatagaatttttaatgatctatggtgttctatgatgaggcaacattccaccaaattagccttccaaaagttgcagtatcatgtataattatgacagcagttttgttttaaaaccagagtcagattgaatgtagcttttttacagctgaaatttatgccttatgtgtattcataaaacattgataacttagtgtcacattatctttactctttggttatactcttcttgaaaagtaaatttacttatcaaatgataaagtttcagggaaagttaaaaaaagttttttttcttaaggcttcatggaatagaattccatgaatcataatgactacgtaagacccttttctggtaatgaaagcatggagtcttaaccaaaaagctaagcagaattgttagatcttttggtttctgtcataatgtactattggaacttcaagtagatatagtacattaatatgaaatactttgaaatacaccatctttaaaaaaaaaggcacttacacaaaaatcatgtaacactaggtaggatgttgaaatgactggtatgcaatattttttaaagccttcatttttggtcagcataagtttcctttaattatttttctgtttccagttggacttcactttgaggcttaacatagcaaagtgagtataaagttctacaatttagtcattgtggatttcaagtcatttatgatgaaaatggaaatgtgtagtttacttaagaaaattttcttcttctgtaacatctaactcgtcatcctcatcatcttctgcttgttgatcctttcttagtcgacaagtggatacctgtcctgttccagatacacacttagctgacagtgatctctgaagaggtgactttgaatttgctcttacaatatctaaacgagatgaataatctggtgcatacagagaatttcggaaaacctctaaatcttcatcttcatcaatgttttgtatattctggtaggcagcagtgtagacctctaaagctttgccgtgaaataacatttcgattgtgataaattcagaaaatatagtctttatatccttcattttctgcctttcaaagttgttaatagtttcctccagatgacgacttgttcggctagcatccattgcagctctctgtaattccgtttctgcctgtgaaataacatgtcgatcagatgggtttcgctgacgtgttctttctaactgagttaattgcttagcttctcgattccttgctgtgagtgttgctttgaggtcatcccgtttcattttcacaatggtcccataagttttcaagggttcaactactttggcttcaagtctttcaacctctgcttgtcgataatcctgaagtttggcaaactcatctgcaaagttcatcaggcccagctttaaatgcggggtctctgtagcagcatacgcgttaatttcattcaccaggaggtctgctttgtctctcagcctggcagttttccgcacataggcagcgaagatttggcacagttctccaaaatgcttctccacatttgagacagctgtttgcagttgtttcgtttgagcgttccggttttccagggtgcgcctcatcatgctgcctcgcgcacggccggggaccttgcgggggcccaaggacggggattccaaggcgcctgggcgcgcgctggggcgcaagcagccgccgggagcct

SEQ ID NO: 12038 - RNA, 3910 nt, Homo sapiens
  source 1..3910: mol_type = other RNA
ctgaatagctgggactacaggtgtgtgccaccttgtctggctaaattttttattatttgtagagacagagtctcactgtgttgcccaggctgttctcaaatttctggcctcaagcaatcctcactccttggtctcccagaatgtgttgggattacaggtgtgagccactgtgcccagccttgtattttgatttttaaattaatttatatgaatatttccttttaccctataatgtatcagggcttaatatttttaaacttcattataaaaagttgattacagaaagtggtatcttctagttgggagccatctttgcacatctctctccaactctgcctttagtgatatgtcaataacaaattggccatggcaggagtattttacaccatggaaagtgataaatgcagcaaatcaaggaattcccctcctgttgtcccctcagaaagccagcttcccagcacctcatcaatttcaaatataaaaaaagaatagtaaattttcatgtacacatcactcagcttcagtaattgtcgtctcatagccagtttttcctctcctatcctcaaggtataccaggtacactggaggtgtattctctagcctgatacccagtggcatttgtcttaaagccaaacatttttgtctagaaattatctaaaaaaatgtagatcatgtctagaaagtcaatcccacaaccaagagataggtaaaaatcatgttaggagtgcatttctattaatttactgagatcactgttaagagcagtgattcttgatccatatatcacctgttaagtagtgaccttgctgcctctgtttttgcagtaaatattagctgttgtttattgagctgtattagatactatatgatgtataattatgtatgaattaactatcatttaattctgataatcctagtaaatgtactacaggttgagtattcctaatctggtaatctgaaatttcacatgctccgaaaatcacaaactttttgagtgccaacatgatgctcaaagaaaatgctcattgcagcatttaagatttcagatttttgggttaggaatgttgaactggtataatgcaaatactccaaaatctgaagaaatccaaagtcttaaatacttctggtcccaagcacttcagataaaggatactcaatttgtattcctattttggagataagagatggagacttacaggctgggttggttggattggttgcctgttttttgttgttgttgtagtggaagctaggaatggtttttcacattttttaagtgtacttaagtcttacatggttacatagttacctgtataatagtcttgaatttgcctaaacccacgaagaataacagtatttgctatctggccctttaagaagtttgccaacctaggctggtctaaataatgaaaattttacattaatgaaagtattttcatggatagtattccttttgttcttagaatatttctttgaggtaggcagaatgtatgttttattccagaattactgttttacgcagttttaactttacaaacaaggcaaataatgctcaagagaagttgctatttagtaagcagcaaaataataactctgttgttttcccccgaagtacaaccaaatttaaatactgagtgaggaagcagtaaatatccaatgatatcttgagtttcttaagaatatcaatttagggttttaaaatgttttaaatattttacaaaaaagtactgaaacaactttgtcacttaggactattctcaggaaggagtgctttgttaagaacagagccatgattgacaaagtcagaagctttctagaaagtctttatttttctgttatgaataattgcattttctaattatcccaaatgattttataaattccgtaacttttatatgcctgcctgggatccatgaaataaaagtattccttaccaaaagagaagcatcagatacactgaaaggctcaatgttttatattttcagaaataaaagtgactgtatacccttttattaactatatggtagcttggtaaaatttttatagaatttttaatgatctatggtgttctatgatgaggcaacattccaccaaattagccttccaaaagttgcagtatcatgtataattatgacagcagttttgttttaaaaccagagtcagattgaatgtagcttttttacagctgaaatttatgccttatgtgtattcataaaacattgataacttagtgtcacattatctttactctttggttatactcttcttgaaaagtaaatttacttatcaaatgataaagtttcagggaaagttaaaaaaagttttttttcttaaggcttcatggaatagaattccatgaatcataatgactacgtaagacccttttctggtaatgaaagcatggagtcttaaccaaaaagctaagcagaattgttagatcttttggtttctgtcataatgtactattggaacttcaagtagatatagtacattaatatgaaatactttgaaatacaccatctttaaaaaaaaaggcacttacacaaaaatcatgtaacactaggtaggatgttgaaatgactggtatgcaatattttttaaagccttcatttttggtcagcataagtttcctttaattatttttctgtttccagttggacttcactttgaggcttaacatagcaaagtgagtataaagttctacaatttagtcattgtggatttcaagtcatttatgatgaaaatggaaatgtgtagtttacttaagaaaattttcttcttctgtaacatctaactcgtcatcctcatcatcttctgcttgttgatcctttcttagtcgacaagtggatacctgtcctgttccagatacacacttagctgacagtgatctctgaagaggtgactttgaatttgctcttacaatatctaaacgagatgaataatctggtgcatacagagaatttcggaaaacctctaaatcttcatcttcatcaatgttttgtatattctggtaggcagcagtgtagacctctaaagctttgccgtgaaataacatttcgattgtgataaattcagaaaatatagtctttatatccttcattttctgcctttcaaagttgttaatagtttcctccagatgacgacttgttcggctagcatccattgcagctctctgtaattccgtttctgcctttggtccaaaggaagaaggaccaagcaactggcgcagccccaaatcgctgctcaagagactcccctcaggaatggaggtgttctggaacctcaaatgctctcaaagagccactcctcatgtggtttctggctgagctgggcagtaacaaccttaaacatttttttaaagacccaaattcaaaggatacaataacatgtcgatcagatgggtttcgctgacgtgttctttctaactgagttaattgcttagcttctcgattccttgctgtgagtgttgctttgaggtcatcccgtttcattttcacaatggtcccataagttttcaagggttcaactactttggcttcaagtctttcaacctctgcttgtcgataatcctgaagtttggcaaactcatctgcaaagttcatcaggcccagctttaaatgcggggtctctgtagcagcatacgcgttaatttcattcaccaggaggtctgctttgtctctcagcctggcagttttccgcacataggcagcgaagatttggcacagttctccaaaatgcttctccacatttgagacagctgtttgcagttgtttcgtttgagcgttccggttttccagggtgcgcctcatcatgctgcctcgcgcacggccggggaccttgcgggggcccaaggacggggattccaaggcgcctgggcgcgcgctggggcgcaagcagccgccgggagcct

SEQ ID NO: 12039 - RNA, 3988 nt, Homo sapiens
  source 1..3988: mol_type = other RNA
ctgaatagctgggactacaggtgtgtgccaccttgtctggctaaattttttattatttgtagagacagagtctcactgtgttgcccaggctgttctcaaatttctggcctcaagcaatcctcactccttggtctcccagaatgtgttgggattacaggtgtgagccactgtgcccagccttgtattttgatttttaaattaatttatatgaatatttccttttaccctataatgtatcagggcttaatatttttaaacttcattataaaaagttgattacagaaagtggtatcttctagttgggagccatctttgcacatctctctccaactctgcctttagtgatatgtcaataacaaattggccatggcaggagtattttacaccatggaaagtgataaatgcagcaaatcaaggaattcccctcctgttgtcccctcagaaagccagcttcccagcacctcatcaatttcaaatataaaaaaagaatagtaaattttcatgtacacatcactcagcttcagtaattgtcgtctcatagccagtttttcctctcctatcctcaaggtataccaggtacactggaggtgtattctctagcctgatacccagtggcatttgtcttaaagccaaacatttttgtctagaaattatctaaaaaaatgtagatcatgtctagaaagtcaatcccacaaccaagagataggtaaaaatcatgttaggagtgcatttctattaatttactgagatcactgttaagagcagtgattcttgatccatatatcacctgttaagtagtgaccttgctgcctctgtttttgcagtaaatattagctgttgtttattgagctgtattagatactatatgatgtataattatgtatgaattaactatcatttaattctgataatcctagtaaatgtactacaggttgagtattcctaatctggtaatctgaaatttcacatgctccgaaaatcacaaactttttgagtgccaacatgatgctcaaagaaaatgctcattgcagcatttaagatttcagatttttgggttaggaatgttgaactggtataatgcaaatactccaaaatctgaagaaatccaaagtcttaaatacttctggtcccaagcacttcagataaaggatactcaatttgtattcctattttggagataagagatggagacttacaggctgggttggttggattggttgcctgttttttgttgttgttgtagtggaagctaggaatggtttttcacattttttaagtgtacttaagtcttacatggttacatagttacctgtataatagtcttgaatttgcctaaacccacgaagaataacagtatttgctatctggccctttaagaagtttgccaacctaggctggtctaaataatgaaaattttacattaatgaaagtattttcatggatagtattccttttgttcttagaatatttctttgaggtaggcagaatgtatgttttattccagaattactgttttacgcagttttaactttacaaacaaggcaaataatgctcaagagaagttgctatttagtaagcagcaaaataataactctgttgttttcccccgaagtacaaccaaatttaaatactgagtgaggaagcagtaaatatccaatgatatcttgagtttcttaagaatatcaatttagggttttaaaatgttttaaatattttacaaaaaagtactgaaacaactttgtcacttaggactattctcaggaaggagtgctttgttaagaacagagccatgattgacaaagtcagaagctttctagaaagtctttatttttctgttatgaataattgcattttctaattatcccaaatgattttataaattccgtaacttttatatgcctgcctgggatccatgaaataaaagtattccttaccaaaagagaagcatcagatacactgaaaggctcaatgttttatattttcagaaataaaagtgactgtatacccttttattaactatatggtagcttggtaaaatttttatagaatttttaatgatctatggtgttctatgatgaggcaacattccaccaaattagccttccaaaagttgcagtatcatgtataattatgacagcagttttgttttaaaaccagagtcagattgaatgtagcttttttacagctgaaatttatgccttatgtgtattcataaaacattgataacttagtgtcacattatctttactctttggttatactcttcttgaaaagtaaatttacttatcaaatgataaagtttcagggaaagttaaaaaaagttttttttcttaaggcttcatggaatagaattccatgaatcataatgactacgtaagacccttttctggtaatgaaagcatggagtcttaaccaaaaagctaagcagaattgttagatcttttggtttctgtcataatgtactattggaacttcaagtagatatagtacattaatatgaaatactttgaaatacaccatctttaaaaaaaaaggcacttacacaaaaatcatgtaacactaggtaggatgttgaaatgactggtatgcaatattttttaaagccttcatttttggtcagcataagtttcctttaattatttttctgtttccagttggacttcactttgaggcttaacatagcaaagtgagtataaagttctacaatttagtcattgtggatttcaagtcatttatgatgaaaatggaaatgtgtagtttacttaagaaaattttcttcttctgtaacatctaactcgtcatcctcatcatcttctgcttgttgatcctttcttagtcgacaagtggatacctgtcctgttccagatacacacttagctgacagtgatctctgaagaggtgactttgaatttgctcttacaatatctaaacgagatgaataatctggtgcatacagagaatttcggaaaacctctaaatcttcatcttcatcaatgttttgtatattctggtaggcagcagtgtagacctctaaagctttgccgtgaaataacatttcgattgtgataaattcagaaaatatagtctttatatccttcattttctgcctttcaaagttgttaatagtttcctccagatgacgacttgttcggctagcatccattgcagctctctgtaattccgtttctgcctttggtccaaaggaagaaggaccaagcaactggcgcagccccaaatcgctgctcaagagactcccctcaggaatggaggtgttctggaacctcaaatgctctcaaagagccactcctcatgtggtttctggctgagctgggcagtaacaaccttgttatagtagacagtcctttctaggtttgtgtccaacttggatcttaattatactcttaagactcctgaggttaactggctggaagtcatgatgtcacatagttgttttatttaataacatgtcgatcagatgggtttcgctgacgtgttctttctaactgagttaattgcttagcttctcgattccttgctgtgagtgttgctttgaggtcatcccgtttcattttcacaatggtcccataagttttcaagggttcaactactttggcttcaagtctttcaacctctgcttgtcgataatcctgaagtttggcaaactcatctgcaaagttcatcaggcccagctttaaatgcggggtctctgtagcagcatacgcgttaatttcattcaccaggaggtctgctttgtctctcagcctggcagttttccgcacataggcagcgaagatttggcacagttctccaaaatgcttctccacatttgagacagctgtttgcagttgtttcgtttgagcgttccggttttccagggtgcgcctcatcatgctgcctcgcgcacggccggggaccttgcgggggcccaaggacggggattccaaggcgcctgggcgcgcgctggggcgcaagcagccgccgggagcct

SEQ ID NO: 12040 - RNA, 3812 nt, Homo sapiens
  source 1..3812: mol_type = other RNA
ctgaatagctgggactacaggtgtgtgccaccttgtctggctaaattttttattatttgtagagacagagtctcactgtgttgcccaggctgttctcaaatttctggcctcaagcaatcctcactccttggtctcccagaatgtgttgggattacaggtgtgagccactgtgcccagccttgtattttgatttttaaattaatttatatgaatatttccttttaccctataatgtatcagggcttaatatttttaaacttcattataaaaagttgattacagaaagtggtatcttctagttgggagccatctttgcacatctctctccaactctgcctttagtgatatgtcaataacaaattggccatggcaggagtattttacaccatggaaagtgataaatgcagcaaatcaaggaattcccctcctgttgtcccctcagaaagccagcttcccagcacctcatcaatttcaaatataaaaaaagaatagtaaattttcatgtacacatcactcagcttcagtaattgtcgtctcatagccagtttttcctctcctatcctcaaggtataccaggtacactggaggtgtattctctagcctgatacccagtggcatttgtcttaaagccaaacatttttgtctagaaattatctaaaaaaatgtagatcatgtctagaaagtcaatcccacaaccaagagataggtaaaaatcatgttaggagtgcatttctattaatttactgagatcactgttaagagcagtgattcttgatccatatatcacctgttaagtagtgaccttgctgcctctgtttttgcagtaaatattagctgttgtttattgagctgtattagatactatatgatgtataattatgtatgaattaactatcatttaattctgataatcctagtaaatgtactacaggttgagtattcctaatctggtaatctgaaatttcacatgctccgaaaatcacaaactttttgagtgccaacatgatgctcaaagaaaatgctcattgcagcatttaagatttcagatttttgggttaggaatgttgaactggtataatgcaaatactccaaaatctgaagaaatccaaagtcttaaatacttctggtcccaagcacttcagataaaggatactcaatttgtattcctattttggagataagagatggagacttacaggctgggttggttggattggttgcctgttttttgttgttgttgtagtggaagctaggaatggtttttcacattttttaagtgtacttaagtcttacatggttacatagttacctgtataatagtcttgaatttgcctaaacccacgaagaataacagtatttgctatctggccctttaagaagtttgccaacctaggctggtctaaataatgaaaattttacattaatgaaagtattttcatggatagtattccttttgttcttagaatatttctttgaggtaggcagaatgtatgttttattccagaattactgttttacgcagttttaactttacaaacaaggcaaataatgctcaagagaagttgctatttagtaagcagcaaaataataactctgttgttttcccccgaagtacaaccaaatttaaatactgagtgaggaagcagtaaatatccaatgatatcttgagtttcttaagaatatcaatttagggttttaaaatgttttaaatattttacaaaaaagtactgaaacaactttgtcacttaggactattctcaggaaggagtgctttgttaagaacagagccatgattgacaaagtcagaagctttctagaaagtctttatttttctgttatgaataattgcattttctaattatcccaaatgattttataaattccgtaacttttatatgcctgcctgggatccatgaaataaaagtattccttaccaaaagagaagcatcagatacactgaaaggctcaatgttttatattttcagaaataaaagtgactgtatacccttttattaactatatggtagcttggtaaaatttttatagaatttttaatgatctatggtgttctatgatgaggcaacattccaccaaattagccttccaaaagttgcagtatcatgtataattatgacagcagttttgttttaaaaccagagtcagattgaatgtagcttttttacagctgaaatttatgccttatgtgtattcataaaacattgataacttagtgtcacattatctttactctttggttatactcttcttgaaaagtaaatttacttatcaaatgataaagtttcagggaaagttaaaaaaagttttttttcttaaggcttcatggaatagaattccatgaatcataatgactacgtaagacccttttctggtaatgaaagcatggagtcttaaccaaaaagctaagcagaattgttagatcttttggtttctgtcataatgtactattggaacttcaagtagatatagtacattaatatgaaatactttgaaatacaccatctttaaaaaaaaaggcacttacacaaaaatcatgtaacactaggtaggatgttgaaatgactggtatgcaatattttttaaagccttcatttttggtcagcataagtttcctttaattatttttctgtttccagttggacttcactttgaggcttaacatagcaaagtgagtataaagttctacaatttagtcattgtggatttcaagtcatttatgatgaaaatggaaatgtgtagtttacttaagaaaattttcttcttctgtaacatctaactcgtcatcctcatcatcttctgcttgttgatcctttcttagtcgacaagtggatacctgtcctgttccagatacacacttagctgacagtgatctctgaagaggtgactttgaatttgctcttacaatatctaaacgagatgaataatctggtgcatacagagaatttcggaaaacctgacactttgggaggccaacgcaggcggatcgcttgagccccaggagttcaagaccagcctgggcaacatggcgaaactccatctctctaaatcttcatcttcatcaatgttttgtatattctggtaggcagcagtgtagacctctaaagctttgccgtgaaataacatttcgattgtgataaattcagaaaatatagtctttatatccttcattttctgcctttcaaagttgttaatagtttcctccagatgacgacttgttcggctagcatccattgcagctctctgtaattccgtttctgcctgtgaaataacatgtcgatcagatgggtttcgctgacgtgttctttctaactgagttaattgcttagcttctcgattccttgctgtgagtgttgctttgaggtcatcccgtttcattttcacaatggtcccataagttttcaagggttcaactactttggcttcaagtctttcaacctctgcttgtcgataatcctgaagtttggcaaactcatctgcaaagttcatcaggcccagctttaaatgcggggtctctgtagcagcatacgcgttaatttcattcaccaggaggtctgctttgtctctcagcctggcagttttccgcacataggcagcgaagatttggcacagttctccaaaatgcttctccacatttgagacagctgtttgcagttgtttcgtttgagcgttccggttttccagggtgcgcctcatcatgctgcctcgcgcacggccggggaccttgcgggggcccaaggacggggattccaaggcgcctgggcgcgcgctggggcgcaagcagccgccgggagcct

SEQ ID NO: 12041 - RNA, 3612 nt, Homo sapiens
  source 1..3612: mol_type = other RNA
ctgaatagctgggactacaggtgtgtgccaccttgtctggctaaattttttattatttgtagagacagagtctcactgtgttgcccaggctgttctcaaatttctggcctcaagcaatcctcactccttggtctcccagaatgtgttgggattacaggtgtgagccactgtgcccagccttgtattttgatttttaaattaatttatatgaatatttccttttaccctataatgtatcagggcttaatatttttaaacttcattataaaaagttgattacagaaagtggtatcttctagttgggagccatctttgcacatctctctccaactctgcctttagtgatatgtcaataacaaattggccatggcaggagtattttacaccatggaaagtgataaatgcagcaaatcaaggaattcccctcctgttgtcccctcagaaagccagcttcccagcacctcatcaatttcaaatataaaaaaagaatagtaaattttcatgtacacatcactcagcttcagtaattgtcgtctcatagccagtttttcctctcctatcctcaaggtataccaggtacactggaggtgtattctctagcctgatacccagtggcatttgtcttaaagccaaacatttttgtctagaaattatctaaaaaaatgtagatcatgtctagaaagtcaatcccacaaccaagagataggtaaaaatcatgttaggagtgcatttctattaatttactgagatcactgttaagagcagtgattcttgatccatatatcacctgttaagtagtgaccttgctgcctctgtttttgcagtaaatattagctgttgtttattgagctgtattagatactatatgatgtataattatgtatgaattaactatcatttaattctgataatcctagtaaatgtactacaggttgagtattcctaatctggtaatctgaaatttcacatgctccgaaaatcacaaactttttgagtgccaacatgatgctcaaagaaaatgctcattgcagcatttaagatttcagatttttgggttaggaatgttgaactggtataatgcaaatactccaaaatctgaagaaatccaaagtcttaaatacttctggtcccaagcacttcagataaaggatactcaatttgtattcctattttggagataagagatggagacttacaggctgggttggttggattggttgcctgttttttgttgttgttgtagtggaagctaggaatggtttttcacattttttaagtgtacttaagtcttacatggttacatagttacctgtataatagtcttgaatttgcctaaacccacgaagaataacagtatttgctatctggccctttaagaagtttgccaacctaggctggtctaaataatgaaaattttacattaatgaaagtattttcatggatagtattccttttgttcttagaatatttctttgaggtaggcagaatgtatgttttattccagaattactgttttacgcagttttaactttacaaacaaggcaaataatgctcaagagaagttgctatttagtaagcagcaaaataataactctgttgttttcccccgaagtacaaccaaatttaaatactgagtgaggaagcagtaaatatccaatgatatcttgagtttcttaagaatatcaatttagggttttaaaatgttttaaatattttacaaaaaagtactgaaacaactttgtcacttaggactattctcaggaaggagtgctttgttaagaacagagccatgattgacaaagtcagaagctttctagaaagtctttatttttctgttatgaataattgcattttctaattatcccaaatgattttataaattccgtaacttttatatgcctgcctgggatccatgaaataaaagtattccttaccaaaagagaagcatcagatacactgaaaggctcaatgttttatattttcagaaataaaagtgactgtatacccttttattaactatatggtagcttggtaaaatttttatagaatttttaatgatctatggtgttctatgatgaggcaacattccaccaaattagccttccaaaagttgcagtatcatgtataattatgacagcagttttgttttaaaaccagagtcagattgaatgtagcttttttacagctgaaatttatgccttatgtgtattcataaaacattgataacttagtgtcacattatctttactctttggttatactcttcttgaaaagtaaatttacttatcaaatgataaagtttcagggaaagttaaaaaaagttttttttcttaaggcttcatggaatagaattccatgaatcataatgactacgtaagacccttttctggtaatgaaagcatggagtcttaaccaaaaagctaagcagaattgttagatcttttggtttctgtcataatgtactattggaacttcaagtagatatagtacattaatatgaaatactttgaaatacaccatctttaaaaaaaaaggcacttacacaaaaatcatgtaacactaggtaggatgttgaaatgactggtatgcaatattttttaaagccttcatttttggtcagcataagtttcctttaattatttttctgtttccagttggacttcactttgaggcttaacatagcaaagtgagtataaagttctacaatttagtcattgtggatttcaagtcatttatgatgaaaatggaaatgtgtagtttacttaagaaaattttcttcttctgtaacatctaactcgtcatcctcatcatcttctgcttgttgatcctttcttagtcgacaagtggatacctgtcctgttccagatacacacttagctgacagtgatctctgaagaggtgactttgaatttgctcttacaatatctaaacgagatgaataatctggtgcatacagagaatttcggaaaacctttatatccttcattttctgcctttcaaagttgttaatagtttcctccagatgacgacttgttcggctagcatccattgcagctctctgtaattccgtttctgcctgtgaaataacatgtcgatcagatgggtttcgctgacgtgttctttctaactgagttaattgcttagcttctcgattccttgctgtgagtgttgctttgaggtcatcccgtttcattttcacaatggtcccataagttttcaagggttcaactactttggcttcaagtctttcaacctctgcttgtcgataatcctgaagtttggcaaactcatctgcaaagttcatcaggcccagctttaaatgcggggtctctgtagcagcatacgcgttaatttcattcaccaggaggtctgctttgtctctcagcctggcagttttccgcacataggcagcgaagatttggcacagttctccaaaatgcttctccacatttgagacagctgtttgcagttgtttcgtttgagcgttccggttttccagggtgcgcctcatcatgctgcctcgcgcacggccggggaccttgcgggggcccaaggacggggattccaaggcgcctgggcgcgcgctggggcgcaagcagccgccgggagcct

SEQ ID NO: 12042 - RNA, 3224 nt, Homo sapiens
  source 1..3224: mol_type = other RNA
ctgaatagctgggactacaggtgtgtgccactgcacccaactagcagagaattcttaacaagcagtcaggatggaactgatggctgtttgggcactttctactttcttcttaaaaggatgatatcacctcttcttctctggtgagagtctgaggatagagacttttttctcaccatgaatgtcaccccagaggtcaagagtcgtgggatgaagtttgctgaggagcagctgctaaagcatggatggactcaaggtgatccccatggggcctcttccacatcccccagctccctgcctaccatctgcccaggggaaagccatcatcctggattacccccccatgtagtccatttaattaaaggaggaaaagctagtttaaagggaaatttgcagaagaaaatttctaactttcccagaaaagggaagaaaggaagaaatttgacagtggataatgaagaagtggtggttgggaggactaggggagggaaaaagagatatgggctctctaccaaaagaatttgaaggaagagatagttcaggctcacacaaaggcaggggactatatggagtggtactagaaagaagtgcgctaggaggtcttctgagaggtacagagtataccccaatgtcaggtgtgtggaatggcaagaggcctgtgtggggggtgccttgtgaggtctcacagcaggcaggagaataagccaaatcgctcactgtcctctgcaggcaaaggcctcggccggaaggagaatggtatcactcaggctctcagggtgacactgaagcaagacactcatggggtaagactgggtggactgaggaaggttagcatgtgtgggagaggggacccttgagggcaggtgaggcaggcactcagagctcatatttattcccctggcaggtaggacatgaccctgccaaggagttcacaaaccactggtggaatgagctcttcaacaagactgcggccaacttggtagtggaaactgggcaggtatgagctcttgatagatgggcacatgaaacagagggcctgggacctgtggcgtaggcagtcatgatatgtcacccattcactggtactgataattctctacaggatggagtacagataaggagcctttctaaggagaccacccgttataatcatcccaagcccaacttgctgtatcagaagtttgtgaaggtattagaggctgtgggtaacagagtccatcctttttctcttccctggtttccctggggcctgaacagttgccttgtatgccttatcaattctcagaactttcctaacatagtgggatcctgtgaccagccttgctgttgcttacttagactgcccagaccctcagcaggaattgagatcttcaggttccgtggatcctgccatctgttaagggagcagcaatagggcgtgggaggtagggtacagtctcttaagtcaggagctgccaaattttgggggggccaggggacatctaattcaaaggacttagaagccagaggagacctgagagattatctggaccatccctgctttgcagatgtggctaaaagggtgaaaagtggtttgctgaagagcccacagctggctagtaatggcaaacaggactggaacccaggacttcaggcctccactttctactgtaccaataggaggaagctaacatgtaatggtcattatgtgctaagggctatacatgttacctagcaaatctttcccatttctctacatctctgttaccatctactaccccacttcgggccatcatcatctcttgcctaatttctttctccagcagcctcctaagaacacctgtagtctcactccccaccccaacctttgtggaggatggacttctccacaaagcatccagtgttctctctaaaacataaatgtcatcatgtcactgggtcttgtttgacctaggatgacacaatccagatttatcggactggcttatatggctctgcatgcctgttcctgccatctccagcctcatctcttcacttttctccaggaccactactttagcctaaccattagcataacagattccaatctgtttcttttctttgaaggtacgacagtcttccatcttcaggttattgcacatgttgctccctctgcttgggacattcttctccctttccccctttaccttctgagtttctcttatcctccagagctcagcttatacatcagttacttttagaagccattctctgaagtctgagttgagtacccttcctctatcacaggcaacacttccatcataattgcctatgtagattccatctgggctgggcccatctcattcttattccactctgaatccccaactccttggcccatagtagactctcaattaatctgattaaatgaaggtactgtgaacaggtactatggtcggggtggagcggggcatctttactgtcagtcactggcacttgtccactgtgaagacctgatgaaccagagcatttcctcttcttgttctgctcaccagccagcttctggatcccagcacctgagggaatgtcgatgctggcaatgggcacagtgagtcccttcaggacactcaggatgctgtggaacggttcccgaacatcgcccttgaagctgaagccaaagatggcatccaccaccagctcatacagttcatcaatcgtcatgggctctgcgggcatttccccaaggaaagggatgtccattttctgacactgggtcaccaatgcagtgaagaggggcttgttaggccttttggggtaatagatggttggctcgtagccaaagagtttgaggtgtcgagcacagaccagaccatctcctccattattccccgggccacagatgaccaggacagtaggggggctcctggacatggacgtggggggatatgccttggcgatggctgtagcacagctcagcccggccagttccataagttggtccacgctgaactggtattcgttaaatagctcctggtccacggcctgggcctcctcctggctcaggtacttcaccaccgtgctcgccatgacctctgagtcccagcggccacccgagttcagccgctgcggtccccaccaggtgggtcccgagcgacaggcgatggtctggcttttgatccgcggcacgcgcgagcccgcaaccagcagcccgaggcccagcagcgcccgcagcctggacatccagctcgcagagcgcgcgcccccggccc

SEQ ID NO: 12043 - RNA, 5638 nt, Homo sapiens
  source 1..5638: mol_type = other RNA
ctgaatagctgggactacaggtgtgtgccactgtgcccagtttttgtaattttccctcagttgaaaaatggacaaatgttagacaaataccttaatctgggtcaagcatagttgaactacgttttgttttttttttccttaccaactctatagttgatacagctcgtcatttttggatccattttgaaatccccagaaatagactcttactctgagtgaaaccacacggttgaactaaaaggttcctgttacatgtccaggggagatgtccatgtgcagctttacatggaatttggggtattaagaatagaactgattctgtttggtcacatttgctattgaaggactctagataccattgccatcttagtcatcaattactaaagttatggccaggtagagagacaaaacttatgtgagctttactttaaaaattcaaatatttatttgatttaactatttcaaaaccactgtgctattgcatagcaatagacacattttactaaaattgggattaaaacactattaagtgcaatagcaattacagatgtactcatataagaaaatcacaaaacttttaacttaaagaacagattaatcaagtgttgcaggtttatataacatataaaagtattcaccttgggtccttttaaataataaacatccatgggtggttagtgtttggacaccaatcattcacatatgatgacaggtagaaaacctgagatgacgcagaaaaactttaaaagtgaccccaggcacactaaacccattaaaagtgaaccccagacaaactaaaatcaattagtaagacaaagcacatcaaagtaaacctttggttaaaatctaacttaaatgcagtttttaaaaaaatttaaaatgtgtcagtttggttacatttattaaataaagttaacaaaggagtaatctcttatcaatgagagctccagagacttaaaaataacggtaaaatttctgtctcctctctttattaacacaggtaattattacttttacttaccatacacaagacaattaagtaactattttaccaaataacatacaagaattctatcagaaatctgaacgccgaaggaaaaaagatagctaaccttcaacaagtagctctccatgtccttaagagcagacctcttttttcttggaatatgttttctgttgagaccttcactatcattaagatttccaacgcaaggtgactctaggactggccttgtagcataagcagtgaatagagatctggatctggtctgctctttctccacagtaagttgcgtactgacctctgctatcatctcattagttctactgagttcatttgacaaggattctctaactttcacttcttctaggtagagttccttatatctttccaattcggttttattaaagtcggcttgcgaagtttttattctggagatttcagattccagatctttgattgtgagttccatctgagtttttattgaagtagtattatcctcccttaactgtactaactgttcatgagatactgctgcttgtttctgcaaggtgagaatggcttcgtttaatttttcttctatctccttccttgctctttcttcaatcaacagtttatgccattcagctttaccacgttctaacatatttctttccatataacttttgaggtttactacttcttgtttcagctgcttcttattcttctgtagtgtttcacattgcttttgtattgctttcatagagaataatgtctgttgaagttgaagaacttcattctctgcatccagatgtagacatcgtgaaggtacagtttcctgtgcttctgtaaggtcaatttcacttctgatttgacccaatttcttctttgaatcctgtgtctcatctaaattaatgtgacaacgtgaggtagcctctgacgtaggttgttgttttaggagatcggtccattcttgttggaattctctcataactacttttcttcctgctttctctttctcacattgatccattctttcttttaaatgattatattcatccatcagctccttgttcttctcttgtagtgaaagaatctgcttttcactctcagcttgaagatttttggcagcagaatgaaactggtcttggatagtactgcttgtcttttcttgactgttagctttcttgtgagcatcatccagttgctgtcgaagcaacatattttcactttgtagttgagataatctctcctctacagattcctgcttggcaatgtatttcttcagtttgctttgttcaatttggtacatttgttcagtttctttcttctgacactgtgtttggctgaggtctctttgcacacgttccaaaatcaaactctctcttccaagagcatctcttgtgttatggagctgaatttgtaggctgttaattttactttcagcattagaaagtttttcagaaagaatctcattcttagcttgtaggccagacatatcaaccttcattttgtcatgtaaacgaacccactcttgtcttgttctctggaaatcaagttttaggtctcttgctgtctgactttgatcacagtcacgtacagcagcagctagtctacaacggtatgattccatttctatttctagtctttcttggttctgtttcccattctccagttcagaattgagtattttgttctcagctgtcagattgttcagctgtccactgtactggagtattgtttctgttaatgtttcctcatttagttttataattttttgaaggttatcattcttttctttcacagcctcaatgtcctcaaaatatttcttttccttttgcttgttctgattttttattgtatctatttccagtctcagcaaggcaatttcttcctgcaacatgcaatcttcatgaaagagatccttttctttctgatgcctatgagaaatctcagaattcattttctttcgagccatttctagttccttttgtttactcgtcagaatctgatcttgtaatattctggcatcctgttcttcagaaagttgcttctgggcatcgtttctctcctgcacaaccagatccaagttatttcttactgtcctcaattccttaacaagtcttctcagattccatttaagttgttgctttgtttcaaccactttcccacactcctcttcttttattcttaactgttcactatctttattatacaacatatcggcatttcttttctcctcattttcttgttttaaggcaagtctcaaatcgtacagctctttctcccattcaattttttgaagttctaactgtaattttgtcttttttgtttcagatagctcattttgtagtacactgaccatattttccatttgtttaagttttactgtaagttggtcacagtgattattcttaagtttcagtaagtgttcacacaaacaaaatgtgtcttggattcttggtaggctagcagaatctttatactccattctaagttgttcaatcagcaacataaaattctcataaacagagtgagacaattcacaatcctctgaggctatttcagatggctccattgagtcagcaaagtcagcctcaggatatatttggtttttgacctcgttcttttcattagatgttttatctgcaggcctgtcatgctctccattttccttcctaggaatctgctgatttagtccatcatcatcattgccaacagtagtaccatcagttagggttcctgataattctgtgctattacttctgtgcttctccatttcttcttcaacatctttatgaagttgaacatcttctttcttcaaagccaggaactcttcttctaatgtgttgacctcattcttaaacttttgcatgtcttgctgtaattcttcatgtagatatacttctgatgttctgtcagaatctggtggtaaagaactcagattttctaatttaggtttcaggcttttatagttgtttgtactgccactgtcactattttggttcatattttttgtcatttgcaaatcaaactcttggtcttctttcatttcaaccataaccacttctgggttccttgctttcttagtgcttgcatcattatgaaagttcttatctgtactaaaaatatgtccaatgcctggtttgttatcattgtcgcagtctaatttattttcatgtaaatgaaacttagaagatgactggcaaacatgttcctgggacccagagtatggatgatagtatggatggatgatatttttgagactgggttctttttgttcaggaaatgtctcgaataccactgagacagatatttcagatgcatcttcttcctcacaaccaggtatgttatttgtcaaattaaagggaatatcctttacatctgttcctcttgtagagttatcaagtagtggctcttcctcaggacaagccggaattttgtatttttcataaatttcaccaaacctctgctttaactcatttatgacgagttttaattggtttttccactctaatttgccttgttcaatccacatttcctcagatttttgcacatgaggaagtactggatatataggtatatcctctctatcgcaatccttagccatttctggttcttgagacgttttctgtggctgcttattttcgcatcctttaagtctttcttgctcttcctctgatgtcagctccgagtcttgttctgcttctttgctctctttgttttctggtagctgtgattggcacaggtcatggagagtatcattccctgagagaagtacaactccagtgtccatcttttctcgttctgttaagttcatctgtcccagttctttggttgctgactgattttcaggcattgatggtgatacagatggacatttatcatcaactttcagattcttggatctctgacaagtctcatcactaagggtcaaattagtaggatgccaatctggattgttattttgaggaagactttcaggtgtctgtttttccttatattcaggaactagttgctgaatgccgcccggctgccttagggattggcgctgcccagcggggtccagcgcagcctcctgccggttttcccaccggtggctcccgccactggctcctggccgccggctgctacccgcgctccgtgggcagggccagtccgggggagcggaccccgagaggcgcggcgggatggcaggcggtgtccaaaagcctctgaaagtcgcagccgggcgcgagtcgctgaccgaccgggaggccccgatctgtcccagccaaggcctcccggcgccatcacccaccaggagtcccgggcgggggcatcgctccctccacgctgtcgcgggcttctgccaggcggtgatctgtgcccaacgccaccaaagggcagcttgtgcccaagagtgggggaaatgcatccttcccggggatctgaaagctccaggtcctcctgccaggagcccacggcctcagatggcgcccaggacgcgcccgcgctggggaagcgccccctgcacctgagcccgaaattgtccccaacaaaccccacacccgcagggctgacgtttggactccggggtgcggtgtcgatgaaatgggcaccgcgtgctttccatgcaaaagacacggagtctggagtttatggaattattgaaggaaa

SEQ ID NO: 12044 - RNA, 5294 nt, Homo sapiens
  source 1..5294: mol_type = other RNA
ctgaatagctgggactacaggtgtgtgccagcatgcctagctaatttttaaacatttgtttagagatgggtctcactatgttgcccaggctggtcttgacctcctgacctctgctgattccccccacctctgcctcccaagtagcgggattacaggtgtgagccactgtgtctgacaagaatttatacttaagcataggagatggttctggaaattctaagaaattctgctctcagtaagagtagaggtttggagctttacctcttggcagtatcccttggaagggagctctgagattaaatgtaatcaaacacttattgagagctttctatggaccaggcactacactagacgctgggaattacagaggcaattacctgtcctatactcaaggtgttaatgatctagtgtcatttttctttaaaaaagaaagcacctgcatttgtcatcttgagcaaatatagtaactctaacctcaaggttcaagtgatttactcaaggtttaaatcatagttgttttggagaaagtaagtgtcagatgcactgtggctgtcagggtcatagtaggcattaaatcaacatggttggtgttcattaaatgtggattgaagataaaatgactgatcttaagtttcatgaggaataggtttgcttcattgaaactggtttttatcttcccaaatagttttcaatcattcctttaaagtactaggttgattaatattgcaaagttgtaatgtaaaatgtgaccttacctctgtctaacctgtattgttcacatgaatgggagtttgactttgggaataaacattgaaaatttgcagggaggacccacccaaatgtatcatgaaatgtgattccaggtatgaaaaaccagtgatactaatttaaaggatcattttgatttaacatgtggtttcaaatttcactttaacaagaactattttattttagaaacatttatccactcagatgcattggttctttcattaacagagttttggaactggcttttcaatctgggaaagccccagtcacacttctggagcaaggcccataatgcagatggttcaaactttttttttgtttggatacggagtctcactctgttgcctaggctggagtgcagtggtgccatctcagctcactgcaacttctgcctcctgggttcaagcgattctcctgcctcagcctcccgaatagctgggactacaggtgcatgccaccacacccggctaattttttgtagtttagtagagacggggtttcaccgtgttgcctaggctggtctcgaactcctgagctcaggcaattcacctgcctcggcctcccaaagtgctaggattacaggcgtgtgccactgtgcccggctggttcaaacttttcatataacccttaggaaattggatgtgacagggagaaaagataggaccttttcagcatttcttaatatgcagaattgccaaatattccaaagatggtctagtgacataaaagtatattacaagtttgtttgagaacatctatatttaaatctaacctttaaacaattttaaattgatatttgttttaaatatgaattgactattgcccctttatcttagctatggtttggggaaacaagcatttttttatttccaaagaaatgttagaatttctatgctgaactgcattttaaaataaaatataatatttagctttaggtattttaattactacaaaggggagagctttgcatctaagcaatacttttcatcaatagatctccagttttctataggcagacggactccctctgtttgataaagaaggaaacaggcacagagaagttaagaccctcccagtgaagactaagccaggctctccatctcccatctgggagaagctgcttcatcctagagggtggtctcactgtcagtttctcttcggtatttatccatgtctgtgaagtcatagtctgactccatctctatcttcacctgtggcaccatgaacactgggttccgtgagtagctgaaagcaggtgaagctggacaggatattttgaagtgcaaggtgatgcttcggtcaagttctgtgtcactgaaggaagaatcagagtgagtaactccaactggaagatctttttctggcaatgcagtggataccgttttggggatctgattggacactttccatgggaatctttataaccgagggaggagggaactggggctcctcatcacagtcctcgtgggcccctttttttctcttcctcttcttgtctgtctcctttttttccttctctgggaggatgttgtcaatccaggccaggtcgtgctgggaaaagatgaaatccagaagccttcgaacgatgatgaggcccaggatcatgaccgggaagatgatggcagccaccgtggatttgaggatccagagcaccgccaggcagaggatctgcaccagggtgaagaggtggatccggcgcagcggcacgtgccgcaggaaggcatggtccggctggtgcttggctggcatcaggaagagcttgcagcgttcccagaactggatgccattcagggaggccacgcccatgtagaggaagactccgtacagcaccggcagggggatacactttaggatgggagccaggaagacagagattcccgtcaggatgaagacgatgatgccggttactctctgttccctgactcccagaaactggggctgctccccaggggcactggtctctgtctccatcttgaggctgtcgatgtgggcgatggagatgaccgtggcagccacgtaccaggggagccccataaaggagcacaaagccatgaggatgcccacccagaacaggtccagatggtagccggcagccttcttcagtttgttctccttccggttgacaatgacggcagtgatctgctggtccatgaagatcaggatggtcaccagcagggcgggcaggatgcttgctgggtatacccaccacgggttcttcccaaagggggccacgaaccagcctcggtcaggccgcgttggcttgatgacactgggcacatgcagcttgggagtttctaggccaaaacaggcatcgattccacagaacatcaggatggagaaaacaatggaaaagtcagccaccagggcccggaccttggtaggaaaatagcggctgaatttgaacttcttcagggtcagggtcatggagtatgtcccaaagaaaaggatgaaggacatgagcgccaggtctgggataaacttgcaggaattcccaagcaggcgcccgccgtagctcagacactccttcttgctcagcagggaccagtccaacgctgtgaggttaaggaggttgtacagagaagcgttggtgtctggtgccaatggggctgaagcattgaacacggttgtattcactgtgtcaggggcgacacactcgcacttgtaggtagtgatgaagtttggcttgaagtccatattgatagggtagtacttgaaggcaccgatcatcttcttgatggcatcgtagatgaagatgaagctgataagggtggagaagccctcctcggtgaagcgggtgatatatttgatgataaagctggcatctgtggccactaggataaggcactggacagctgagtgtaggccaatccagaggcggaactccatgtagtccaggccattgcctttgctgaagtcgaagaggagcttctcaaagatgaggatgggccccgtgctgctgagaatgatgagaggctgtcccgagaagaggcagaacaaggagccagccatggcagtgcccaggaagctctccatcactccctgataattgtcggtggcatcccccagaagcccaccaaaggtgatcgcgttggtgatacagccgaggtagatgaataggatggcagagatggactgaatgtggaagccatcatagaagtcacttgggaaccagggcaacttcctcttgatatccagacacaggccaccgaagaaccttcctgtccagataagttcctccccgatttcatgcatggctggcatctctccatcatccccgctgcttgttccgccggccccgccactgccagccccgccgccactgccaccaccaccaccacctccattgcctcctccaggagctccgccgcctcctcccacagagccattcatctggcccagctctgctagggagaacacagatttcctcttgtcagcagagggcaccttcttggggggctcaatccggatatttgggtcccattctccaggaggaaggacgatgacctcatccagaaattcatcaattcctgcgatcagatcttcccgattgcgggctttgtaggccacgtcactgaagagatcatctaccatgagggttgcaatggcacggccaatttcattgtaggattttgctctcccagaaggtcccagtagtataaacagaaatctggtggggacaggcacctcggtcactcctcccagcatggccgactggatgaggcgcacgaacgcgatgaatggctggtctaggaagtccacctcgcccacgagcacgttggacgcttctgagtccttggggatcttcttcatgaatttgtttttccgctggtctgtgtttggggtgagagaaatgtcattcatgcttctgctctgggcatgacacagacgtccgtaatttgcactctgccgcatccgcaggtcttccgtggagtggtgtagactcgggccagcaccagggctccgggcaggactgcgatttgtggtggagactgacttcccaatgtcagctaaggagcggtggatgggcttcttggtttggtggcggtgcctcctcaggaggacgtaactgaccctctcccggagctctggccgcaggagaccatcctcaatctgcttctcaatgacatcatctatgatctgtggtaaggagccactgtccaaatccagcagcaccgtccccgtctgcaggcaggtacggagctcgaagaggctgtgcagggatagtgtggacacgtggggcttgctccagcgttcgccgccttcctctaccttttcttcaaactttatccacctggctgactccttccactccatctggtctccgtcatgctgcagagtatccatctctgtaaagagggtggggttgggagcctcatcttcctcccccaggatgtcctggagctgctcagcagctggggaccctgctccctggaacagctgagcgctggggtccctggctgtcgatgctgcctctggccccagcctgcttccgctgctgcctccctggctgctacttccacaggtcc

SEQ ID NO: 12045 - RNA, 5867 nt, Homo sapiens
  source 1..5867: mol_type = other RNA
ctgaatagctgggactacaggtgtgtgccagcatgcctagctaatttttaaacatttgtttagagatgggtctcactatgttgcccaggctggtcttgacctcctgacctctgctgattccccccacctctgcctcccaagtagcgggattacaggtgtgagccactgtgtctgacaagaatttatacttaagcataggagatggttctggaaattctaagaaattctgctctcagtaagagtagaggtttggagctttacctcttggcagtatcccttggaagggagctctgagattaaatgtaatcaaacacttattgagagctttctatggaccaggcactacactagacgctgggaattacagaggcaattacctgtcctatactcaaggtgttaatgatctagtgtcatttttctttaaaaaagaaagcacctgcatttgtcatcttgagcaaatatagtaactctaacctcaaggttcaagtgatttactcaaggtttaaatcatagttgttttggagaaagtaagtgtcagatgcactgtggctgtcagggtcatagtaggcattaaatcaacatggttggtgttcattaaatgtggattgaagataaaatgactgatcttaagtttcatgaggaataggtttgcttcattgaaactggtttttatcttcccaaatagttttcaatcattcctttaaagtactaggttgattaatattgcaaagttgtaatgtaaaatgtgaccttacctctgtctaacctgtattgttcacatgaatgggagtttgactttgggaataaacattgaaaatttgcagggaggacccacccaaatgtatcatgaaatgtgattccaggtatgaaaaaccagtgatactaatttaaaggatcattttgatttaacatgtggtttcaaatttcactttaacaagaactattttattttagaaacatttatccactcagatgcattggttctttcattaacagagttttggaactggcttttcaatctgggaaagccccagtcacacttctggagcaaggcccataatgcagatggttcaaactttttttttgtttggatacggagtctcactctgttgcctaggctggagtgcagtggtgccatctcagctcactgcaacttctgcctcctgggttcaagcgattctcctgcctcagcctcccgaatagctgggactacaggtgcatgccaccacacccggctaattttttgtagtttagtagagacggggtttcaccgtgttgcctaggctggtctcgaactcctgagctcaggcaattcacctgcctcggcctcccaaagtgctaggattacaggcgtgtgccactgtgcccggctggttcaaacttttcatataacccttaggaaattggatgtgacagggagaaaagataggaccttttcagcatttcttaatatgcagaattgccaaatattccaaagatggtctagtgacataaaagtatattacaagtttgtttgagaacatctatatttaaatctaacctttaaacaattttaaattgatatttgttttaaatatgaattgactattgcccctttatcttagctatggtttggggaaacaagcatttttttatttccaaagaaatgttagaatttctatgctgaactgcattttaaaataaaatataatatttagctttaggtattttaattactacaaaggggagagctttgcatctaagcaatacttttcatcaatagatctccagttttctataggcagacggactccctctgtttgataaagaaggaaacaggcacagagaagttaagaccctcccagtgaagactaagccaggctctccatctcccatctgggagaagctgcttcatcctagagggtggtctcactgtcagtttctcttcggtatttatccatgtctgtgaagtcatagtctgactccatctctatcttcacctgtggcaccatgaacactgggttccgtgagtagctgaaagcaggtgaagctggacaggatattttgaagtgcaaggtgatgcttcggtcaagttctgtgtcactgaaggaagaatcagagtgagtaactccaactggaagatctttttctggcaatgcagtggataccgttttggggatctgattggacactttccatgggaatctttataaccgagggaggagggaactggggctcctcatcacagtcctcgtgggcccctttttttctcttcctcttcttgtctgtctcctttttttccttctctgggaggatgttgtcaatccaggccaggtcgtgctgggaaaagatgaaatccagaagccttcgaacgatgatgaggcccaggatcatgaccgggaagatgatggcagccaccgtggatttgaggatccagagcaccgccaggcagaggatctgcaccagggtgaagaggtggatccggcgcagcggcacgtgccgcaggaaggcatggtccggctggtgcttggctggcatcaggaagagcttgcagcgttcccagaactggatgccattcagggaggccacgcccatgtagaggaagactccgtacagcaccggcagggggatacactttaggatgggagccaggaagacagagattcccgtcaggatgaagacgatgatgccggttactctctgttccctgactcccagaaactggggctgctccccaggggcactggtctctgtctccatcttgaggctgtcgatgtgggcgatggagatgaccgtggcagccacgtaccaggggagccccataaaggagcacaaagccatgaggatgcccacccagaacaggtccagatggtagccggcagccttcttcagtttgttctccttccggttgacaatgacggcagtgatctgctggtccatgaagatcaggatggtcaccagcagggcgggcaggatgcttgctgggtatacccaccacgggttcttcccaaagggggccacgaaccagcctcggtcaggccgcgttggcttgatgacactgggcacatgcagcttgggagtttctaggccaaaacaggcatcgattccacagaacatcaggatggagaaaacaatggaaaagtcagccaccagggcccggaccttggtaggaaaatagcggctgaatttgaacttcttcagggtcagggtcatggagtatgtcccaaagaaaaggatgaaggacatgagcgccaggtctgggataaacttgcaggaattcccaagcaggcgcccgccgtagctcagacactccttcttgctcagcagggaccagtccaacgctgtgaggttaaggaggttgtacagagaagcgttggtgtctggtgccaatggggctgaagcattgaacacggttgtattcactgtgtcaggggcgacacactcgcacttgtaggtagtgatgaagtttggcttgaagtccatattgatagggtagtacttgaaggcaccgatcatcttcttgatggcatcgtagatgaagatgaagctgataagggtggagaagccctcctcggtgaagcgggtgatatatttgatgataaagctggcatctgtggccactaggataaggcactggacagctgagtgtaggccaatccagaggcggaactccatgtagtccaggccattgcctttgctgaagtcgaagaggagcttctcaaagatgaggatgggccccgtgctgctgagaatgatgagaggctgtcccgagaagaggcagaacaaggagccagccatggcagtgcccaggaagctctccatcactccctgataattgtcggtggcatcccccagaagcccaccaaaggtgatcgcgttggtgatacagccgaggtagatgaataggatggcagagatggactgaatgtggaagccatcatagaagtcacttgggaaccagggcaacttcctcttgatatccagacacaggccaccgaagaaccttcctgtccagataagttcctccccgatttcatgcatggctggcatctctccatcatccccgctgcttgttccgccggccccgccactgccagccccgccgccactgccaccaccaccaccacctccattgcctcctccaggagctccgccgcctcctcccacagagccattcatctggcccagctctgctagggagaacacagatttcctcttgtcagcagagggcaccttcttggggggctcaatccggatatttgggtcccattctccaggaggaaggacgatgacctcatccagaaattcatcaattcctgcgatcagatcttcccgattgcgggctttgtaggccacgtcactgaagagatcatctaccatgagggttgcaatggcacggccaatttcattgtaggattttgctctcccagaaggtcccagtagtataaacagaaatctggtggggacaggcacctcggtcactcctcccagcatggccgactggatgaggcgcacgaacgcgatgaatggctggtctaggaagtccacctcgcccacgagcacgttggacgcttctgagtccttggggatcttcttcatgaatttgtttttccgctggtctgtgtttggggtgagagaaatgtcattcatgcttctgctctgggcatgacacagacgtccgtaatttgcactctgccgcatccgcaggtcttccgtggagtggtgtagactcgggccagcaccagggctccgggcaggactgcgatttgtggtggagactgacttcccaatgtcagctaaggagcggtggatgggcttcttggtttggtggcggtgcctcctcaggaggacgtaactgaccctctcccggagctctggccgcaggagaccatcctcaatctgcttctcaatgacatcatctatgatctgtggtaaggagccactgtccaaatccagcagcaccgtccccgtctgcaggcaggtacggagctcgaagaggctgtgcagggatagtgtggacacgtggggcttgctccagcgttcgccgccttcctctaccttttcttcaaactttatccacctggctgactccttccactccatctggtctccgtcatgctgcagagtatccatctctgtaaagagggtggggttgggagcctcatcttcctcccccaggatgtcctggagctgctcagcagctggggaccgagtcctgctgataagatccatgctgctgtcctggctgcttgccccactccctgggccagtcagttcctgctgtggctggtctggccgcaggccccagtggactttttgcaggcctgaaagatgtcccttctggtcagtttttctttgagggtaagtgggtactggaagcccaatgtggataggagggcattctttctgatccggaaatctcctcctgtggttagtgtggtccagctttcctaccccagccttctcctccttcaccttcatgactttgtgttcttagctctggaaaccaggatccaaatcccagggaggccagaaccacttgctctgttccacagtatgtgcaatttttggcttccagattgtttgtgccaagctttggcaggtggtacaatattggctgccccagattcttgtctgctttagctgtttctgaaccatgtccagggttgagaagggaacatactgtgatggtgtcagcactcttttggtagcagcaactctttatctggaaggttatcttacactcccacctgggtggtcttcagggtactcctggaaacatccatcagctcatgagctcacagctgaattccaaatcctgggatgccccagtgcagtggcctgtggctcctgggccctgactccaattcctttagggtggaccttgc

SEQ ID NO: 12046 - RNA, 2984 nt, Homo sapiens
  source 1..2984: mol_type = other RNA
ctgaatagctgggactacaggtgtgtgccatcacaccctgctaatttttgtattttttgtagaaatggagtttcactatgttgcccaggctgggctcaagtaatctgtccacttcagcctcccaaagtgctgggattacaggcatgagcccaccgcgcctggctatttcttttctgaaagataattttaagaccctattcaatccagactctttttatcatagagcaagatttgattttcaattttttccttcaacctttccaattccttaaaactacagactttcttgcttttaatccttagcttactagttcttggcctatgcagaaatgcaacttctcctcttacacagtatacttattcaatattattactgctattggtcatgcttttcttagttaataatgctaatacgtactgtctttcccagtggtatttctattttaaactctgctataactatggagtaaaactttgggctctcaagaggatttcaaatctcagctgtctgcctggggactttaaaatataaccattttttaaaaacttataaaaatttccaacacaaagtagaatatagtcattacacagattcaacattaacaggatttttgtcacatttccttaatcgattccttgtttctctgctgaatacttcagagcaaatctatcatgtcatttaaaaactctatgtagcacaatatacctctcttaaaagggagggaccatgttcttatataatcaaaatgcaagtagcttatataatctaatagaattaacaataactcttttgtttggggacctctgaagtgaaacaaatcatacagaattttaatactataaaaacattagcactgtaaaaacagcaacatattatacagcctcaaaacagttttaaactgaagtctagtatgttcagaaacgcagggtgctgacccaccatccaactgaagctgagctcaggaatgcctaagacaactcataaaaatacacagcatcaagatcagtctttgtacattatttcaatgaaaaacacatagctgtgtacaaatatacagatctcaaactgtaacactgaaacacaaaatgcaacaaagtggctttataagttttcttcactgagacagaccttctggtgacttctggtgaatctagacatttatgattattaatacataataagcaagagaaatacagattttccaacctcatgatcagtaaattcctttgaaaaatgaatgaaggtatcagagtcatcaaaaggggaaacagttggtaagtttgatggccctgcctacactgtataatgtaagacacacaataagagctataagaaactatagttaaatgttagaagtaaagccaatatcgttttctcagacttctcccagtgattatatacctgatatataaacatcttcaaatgtgaaatagttcaataacacaatgacactttgccagtgtattaatctgatatatattttgaactggaatgatttgtaaagaaataaataagaaaccctaaaaagaaaccattagttccaagtcaaattatgttaatggtctatagaaaaaagtgagtgtgggcaggaaacattggctacatgccaatttttatttcaaagagtaatgttgcacaaataatagttatcattgtcttacacaacaaaaaatcctaaagttaatctcacaaacctaaattagctgaacatggagtaacaaagtcaaagccagtattatcatcagcacattaatttgataaatcaaactacatctttaaaaaaaaaccctgcatctgctgctgtgcagaactgataattacttttcagcatgtaaacgaaaaatcattatacagctctctctcttttttttttttttcctagaaagatgtataccagggaaacacaacagaatttgttacttgttaaatcccacaaaagctacaagggagctgagagttgatggcacttaaggacagtaaaagtctgcacttttaatatttttaatgcccactgatgggctttgtgtcaatactttttaaaatgctttttatttacaatagataaaacagtaaggaaatacaatattatatcatatccccgcacagagatactatatctgtataaatgaatcactagtaaaagagttatttcttatttcaaatgaagtcttatctaggtattaattaggctgtaatctaaatgttgatggtgcctattttcaactcccaaaataaacagaaagagctcatgtatcaagattaattttctttggccgcaatggataccattttctctgggggcagtctttagtttgctttcttttcagtaccatgtcagaggttttcctggaagcagtctctgttggtgtggtttctatctgtgttataaagttctcaggtttagcatctggtttcctatgacaactggaaaagacttcttggtgaatcctctggaggtggataacaggctgcatcctgagaacttgggaaaatccctctccttgttcaattaatgcaggcaaggacagaatttcttgttttgcttttatggttttgatgacacattccaggatctttctgggatactgcttacgttttgtggctatatctactatgatttcatcaaactgatcttcaagtactttgatgtcagaatccataaaacaattatctgaagcttcctgccatgcttgcccattaatgctgatattctcttgcacagctgattcaaaagtccactgcgcatctcgcagagcgggctcccgaatctcctccggcagagcgtccccgagcttttgcacgaagcggccgcacagttgtagcatttcggtcacagcccgcttcgaggtgcagcgcacccgaaagtcttctcggggagtggcggagaccaaggcctggctctctgtgccagccgcgagctccttgtcccatggagggtcaaggaccaccaactcaggagaccccgccatttttcgtcggaact

SEQ ID NO: 12047 - RNA, 3039 nt, Homo sapiens
  source 1..3039: mol_type = other RNA
ctgaatagctgggactacaggtgtgtgccatcacaccctgctaatttttgtattttttgtagaaatggagtttcactatgttgcccaggctgggctcaagtaatctgtccacttcagcctcccaaagtgctgggattacaggcatgagcccaccgcgcctggctatttcttttctgaaagataattttaagaccctattcaatccagactctttttatcatagagcaagatttgattttcaattttttccttcaacctttccaattccttaaaactacagactttcttgcttttaatccttagcttactagttcttggcctatgcagaaatgcaacttctcctcttacacagtatacttattcaatattattactgctattggtcatgcttttcttagttaataatgctaatacgtactgtctttcccagtggtatttctattttaaactctgctataactatggagtaaaactttgggctctcaagaggatttcaaatctcagctgtctgcctggggactttaaaatataaccattttttaaaaacttataaaaatttccaacacaaagtagaatatagtcattacacagattcaacattaacaggatttttgtcacatttccttaatcgattccttgtttctctgctgaatacttcagagcaaatctatcatgtcatttaaaaactctatgtagcacaatatacctctcttaaaagggagggaccatgttcttatataatcaaaatgcaagtagcttatataatctaatagaattaacaataactcttttgtttggggacctctgaagtgaaacaaatcatacagaattttaatactataaaaacattagcactgtaaaaacagcaacatattatacagcctcaaaacagttttaaactgaagtctagtatgttcagaaacgcagggtgctgacccaccatccaactgaagctgagctcaggaatgcctaagacaactcataaaaatacacagcatcaagatcagtctttgtacattatttcaatgaaaaacacatagctgtgtacaaatatacagatctcaaactgtaacactgaaacacaaaatgcaacaaagtggctttataagttttcttcactgagacagaccttctggtgacttctggtgaatctagacatttatgattattaatacataataagcaagagaaatacagattttccaacctcatgatcagtaaattcctttgaaaaatgaatgaaggtatcagagtcatcaaaaggggaaacagttggtaagtttgatggccctgcctacactgtataatgtaagacacacaataagagctataagaaactatagttaaatgttagaagtaaagccaatatcgttttctcagacttctcccagtgattatatacctgatatataaacatcttcaaatgtgaaatagttcaataacacaatgacactttgccagtgtattaatctgatatatattttgaactggaatgatttgtaaagaaataaataagaaaccctaaaaagaaaccattagttccaagtcaaattatgttaatggtctatagaaaaaagtgagtgtgggcaggaaacattggctacatgccaatttttatttcaaagagtaatgttgcacaaataatagttatcattgtcttacacaacaaaaaatcctaaagttaatctcacaaacctaaattagctgaacatggagtaacaaagtcaaagccagtattatcatcagcacattaatttgataaatcaaactacatctttaaaaaaaaaccctgcatctgctgctgtgcagaactgataattacttttcagcatgtaaacgaaaaatcattatacagctctctctcttttttttttttttcctagaaagatgtataccagggaaacacaacagaatttgttacttgttaaatcccacaaaagctacaagggagctgagagttgatggcacttaaggacagtaaaagtctgcacttttaatatttttaatgcccactgatgggctttgtgtcaatactttttaaaatgctttttatttacaatagataaaacagtaaggaaatacaatattatatcatatccccgcacagagatactatatctgtataaatgaatcactagtaaaagagttatttcttatttcaaatgaagtcttatctaggtattaattaggctgtaatctaaatgttgatggtgcctattttcaactcccaaaataaacagaaagagctcatgtatcaagattaattttctttggccgcaatggataccattttctctgggggcagtctttagtttgctttcttttcagtaccatgtcagaggttttcctggaagcagtctctgttggtgtggtttctatctgtgttataaagttctcaggtttagcatctggtttcctatgacaactggaaaagacttcttggtgaatcctctggaggtggataacaggctgcatcctgagaacttgggaaaatccctctccttgttcaattaatgcaggcaaggactggatcagggtcatattttaggtccagtggatgtacaacagggtggtactgcttcagaatttcttgttttgcttttatggttttgatgacacattccaggatctttctgggatactgcttacgttttgtggctatatctactatgatttcatcaaactgatcttcaagtactttgatgtcagaatccataaaacaattatctgaagcttcctgccatgcttgcccattaatgctgatattctcttgcacagctgattcaaaagtccactgcgcatctcgcagagcgggctcccgaatctcctccggcagagcgtccccgagcttttgcacgaagcggccgcacagttgtagcatttcggtcacagcccgcttcgaggtgcagcgcacccgaaagtcttctcggggagtggcggagaccaaggcctggctctctgtgccagccgcgagctccttgtcccatggagggtcaaggaccaccaactcaggagaccccgccatttttcgtcggaact

SEQ ID NO: 12048 - RNA, 3192 nt, Homo sapiens
  source 1..3192: mol_type = other RNA
ctgaatagctgggactacaggtgtgtgccatcacaccctgctaatttttgtattttttgtagaaatggagtttcactatgttgcccaggctgggctcaagtaatctgtccacttcagcctcccaaagtgctgggattacaggcatgagcccaccgcgcctggctatttcttttctgaaagataattttaagaccctattcaatccagactctttttatcatagagcaagatttgattttcaattttttccttcaacctttccaattccttaaaactacagactttcttgcttttaatccttagcttactagttcttggcctatgcagaaatgcaacttctcctcttacacagtatacttattcaatattattactgctattggtcatgcttttcttagttaataatgctaatacgtactgtctttcccagtggtatttctattttaaactctgctataactatggagtaaaactttgggctctcaagaggatttcaaatctcagctgtctgcctggggactttaaaatataaccattttttaaaaacttataaaaatttccaacacaaagtagaatatagtcattacacagattcaacattaacaggatttttgtcacatttccttaatcgattccttgtttctctgctgaatacttcagagcaaatctatcatgtcatttaaaaactctatgtagcacaatatacctctcttaaaagggagggaccatgttcttatataatcaaaatgcaagtagcttatataatctaatagaattaacaataactcttttgtttggggacctctgaagtgaaacaaatcatacagaattttaatactataaaaacattagcactgtaaaaacagcaacatattatacagcctcaaaacagttttaaactgaagtctagtatgttcagaaacgcagggtgctgacccaccatccaactgaagctgagctcaggaatgcctaagacaactcataaaaatacacagcatcaagatcagtctttgtacattatttcaatgaaaaacacatagctgtgtacaaatatacagatctcaaactgtaacactgaaacacaaaatgcaacaaagtggctttataagttttcttcactgagacagaccttctggtgacttctggtgaatctagacatttatgattattaatacataataagcaagagaaatacagattttccaacctcatgatcagtaaattcctttgaaaaatgaatgaaggtatcagagtcatcaaaaggggaaacagttggtaagtttgatggccctgcctacactgtataatgtaagacacacaataagagctataagaaactatagttaaatgttagaagtaaagccaatatcgttttctcagacttctcccagtgattatatacctgatatataaacatcttcaaatgtgaaatagttcaataacacaatgacactttgccagtgtattaatctgatatatattttgaactggaatgatttgtaaagaaataaataagaaaccctaaaaagaaaccattagttccaagtcaaattatgttaatggtctatagaaaaaagtgagtgtgggcaggaaacattggctacatgccaatttttatttcaaagagtaatgttgcacaaataatagttatcattgtcttacacaacaaaaaatcctaaagttaatctcacaaacctaaattagctgaacatggagtaacaaagtcaaagccagtattatcatcagcacattaatttgataaatcaaactacatctttaaaaaaaaaccctgcatctgctgctgtgcagaactgataattacttttcagcatgtaaacgaaaaatcattatacagctctctctcttttttttttttttcctagaaagatgtataccagggaaacacaacagaatttgttacttgttaaatcccacaaaagctacaagggagctgagagttgatggcacttaaggacagtaaaagtctgcacttttaatatttttaatgcccactgatgggctttgtgtcaatactttttaaaatgctttttatttacaatagataaaacagtaaggaaatacaatattatatcatatccccgcacagagatactatatctgtataaatgaatcactagtaaaagagttatttcttatttcaaatgaagtcttatctaggtattaattaggctgtaatctaaatgttgatggtgcctattttcaactcccaaaataaacagaaagagctcatgtatcaagattaattttctttggccgcaatggataccattttctctgggggcagtctttagtttgctttcttttcagtaccatgtcagaggttttcctggaagcagtctctgttggtgtggtttctatctgtgttataaagttctcaggtttagcatctggtttcctatgacaactggaaaagacttcttggtgaatcctctggaggtggataacaggctgcatcctgagaacttgggaaaatccctctccttgttcaattaatgcaggcaaggacttcatggcttcactgatctcctttgctactgtttcccctctgcatttcaaattttccatatgaggggctcgaagtaataaaaaccatatatgacaaatccacagccaacatcatgttgaatggggaaaagttgaaagcattcccgttgagaactggatcagggtcatattttaggtccagtggatgtacaacagggtggtactgcttcagaatttcttgttttgcttttatggttttgatgacacattccaggatctttctgggatactgcttacgttttgtggctatatctactatgatttcatcaaactgatcttcaagtactttgatgtcagaatccataaaacaattatctgaagcttcctgccatgcttgcccattaatgctgatattctcttgcacagctgattcaaaagtccactgcgcatctcgcagagcgggctcccgaatctcctccggcagagcgtccccgagcttttgcacgaagcggccgcacagttgtagcatttcggtcacagcccgcttcgaggtgcagcgcacccgaaagtcttctcggggagtggcggagaccaaggcctggctctctgtgccagccgcgagctccttgtcccatggagggtcaaggaccaccaactcaggagaccccgccatttttcgtcggaact

SEQ ID NO: 12049 - RNA, 3107 nt, Homo sapiens
  source 1..3107: mol_type = other RNA
ctgaatagctgggactacaggtgtgtgccatcacaccctgctaatttttgtattttttgtagaaatggagtttcactatgttgcccaggctgggctcaagtaatctgtccacttcagcctcccaaagtgctgggattacaggcatgagcccaccgcgcctggctatttcttttctgaaagataattttaagaccctattcaatccagactctttttatcatagagcaagatttgattttcaattttttccttcaacctttccaattccttaaaactacagactttcttgcttttaatccttagcttactagttcttggcctatgcagaaatgcaacttctcctcttacacagtatacttattcaatattattactgctattggtcatgcttttcttagttaataatgctaatacgtactgtctttcccagtggtatttctattttaaactctgctataactatggagtaaaactttgggctctcaagaggatttcaaatctcagctgtctgcctggggactttaaaatataaccattttttaaaaacttataaaaatttccaacacaaagtagaatatagtcattacacagattcaacattaacaggatttttgtcacatttccttaatcgattccttgtttctctgctgaatacttcagagcaaatctatcatgtcatttaaaaactctatgtagcacaatatacctctcttaaaagggagggaccatgttcttatataatcaaaatgcaagtagcttatataatctaatagaattaacaataactcttttgtttggggacctctgaagtgaaacaaatcatacagaattttaatactataaaaacattagcactgtaaaaacagcaacatattatacagcctcaaaacagttttaaactgaagtctagtatgttcagaaacgcagggtgctgacccaccatccaactgaagctgagctcaggaatgcctaagacaactcataaaaatacacagcatcaagatcagtctttgtacattatttcaatgaaaaacacatagctgtgtacaaatatacagatctcaaactgtaacactgaaacacaaaatgcaacaaagtggctttataagttttcttcactgagacagaccttctggtgacttctggtgaatctagacatttatgattattaatacataataagcaagagaaatacagattttccaacctcatgatcagtaaattcctttgaaaaatgaatgaaggtatcagagtcatcaaaaggggaaacagttggtaagtttgatggccctgcctacactgtataatgtaagacacacaataagagctataagaaactatagttaaatgttagaagtaaagccaatatcgttttctcagacttctcccagtgattatatacctgatatataaacatcttcaaatgtgaaatagttcaataacacaatgacactttgccagtgtattaatctgatatatattttgaactggaatgatttgtaaagaaataaataagaaaccctaaaaagaaaccattagttccaagtcaaattatgttaatggtctatagaaaaaagtgagtgtgggcaggaaacattggctacatgccaatttttatttcaaagagtaatgttgcacaaataatagttatcattgtcttacacaacaaaaaatcctaaagttaatctcacaaacctaaattagctgaacatggagtaacaaagtcaaagccagtattatcatcagcacattaatttgataaatcaaactacatctttaaaaaaaaaccctgcatctgctgctgtgcagaactgataattacttttcagcatgtaaacgaaaaatcattatacagctctctctcttttttttttttttcctagaaagatgtataccagggaaacacaacagaatttgttacttgttaaatcccacaaaagctacaagggagctgagagttgatggcacttaaggacagtaaaagtctgcacttttaatatttttaatgcccactgatgggctttgtgtcaatactttttaaaatgctttttatttacaatagataaaacagtaaggaaatacaatattatatcatatccccgcacagagatactatatctgtataaatgaatcactagtaaaagagttatttcttatttcaaatgaagtcttatctaggtattaattaggctgtaatctaaatgttgatggtgcctattttcaactcccaaaataaacagaaagagctcatgtatcaagattaattttctttggccgcaatggataccattttctctgggggcagtctttagtttgctttcttttcagtaccatgtcagaggttttcctggaagcagtctctgttggtgtggtttctatctgtgttataaagttctcaggtttagcatctggtttcctatgacaactggaaaagacttcttggtgaatcctctggaggtggataacaggctgcatcctgagaacttgggaaaatccctctccttgttcaattaatgcaggcaaggacttcatggcttcactgatctcctttgctactgtttcccctctgcatttcaaattttccatatgaggggctggatcagggtcatattttaggtccagtggatgtacaacagggtggtactgcttcagaatttcttgttttgcttttatggttttgatgacacattccaggatctttctgggatactgcttacgttttgtggctatatctactatgatttcatcaaactgatcttcaagtactttgatgtcagaatccataaaacaattatctgaagcttcctgccatgcttgcccattaatgctgatattctcttgcacagctgattcaaaagtccactgcgcatctcgcagagcgggctcccgaatctcctccggcagagcgtccccgagcttttgcacgaagcggccgcacagttgtagcatttcggtcacagcccgcttcgaggtgcagcgcacccgaaagtcttctcggggagtggcggagaccaaggcctggctctctgtgccagccgcgagctccttgtcccatggagggtcaaggaccaccaactcaggagaccccgccatttttcgtcggaact

SEQ ID NO: 12050 - RNA, 3522 nt, Homo sapiens
  source 1..3522: mol_type = other RNA
ctgaatagctgggactacaggtgtgtgccatgatgcccagctaatttttgtatatatgtatttttttatgtagagatgatgtttcatgatgttgcacaggctggtctcaaactcctgtgctcaagtgatcctcccacctcggcctcccaaagtgttgggattataggtgtgagcctccacgcctggcctcaaatctcttttaaccataaatttgattaagatggagctacagatacatgcaaaaatatttacataacatcctaaaatatattaactttatcaatattaaaggagggaaaacgtttagatataggcatatatatgattatatgtaacagttcttggaattctcgactttcagagaaaatgaaattttgtatatgtacatacaatgttgtagaacttctaaccaaattaaacatttttaacatttattttcagcccctaatgaatgcagttacctcaaaactaactcctttcttttattaatggttctgttgcacaatgtgcaatttaccacattagaagctagacaaagtaaaattgcatgatcctaatgtctttttactgatttcaaacttctttaagaagtccatgcaatttactttggagaagacccaaaagcaagatatttgattctttcttatactgctgaaatccctaacaatccactaatctacacattactccaatacagaaatagatataacaaggatttttcacagcaaacttggtcagctatacctgtagcctagttttatttgttttatttagttcttttaaaaaacccttcattagttttattcttatttctctgctgtagtttactcatttttatgttagcaaaagaagatcactatttgatactaaaaaaatactcactggagagcttctaaattatactcacgactcaacctcatcctctttaaatatcttaagtatagccaaatctttaaaaaatcaccccttttcttgcctctagtgctacatttggtaactttccattttaagtttgtgtgtgttctaatacttctgcatctttaaagtcccaaagcgatacagtagaggcaaaggctggctgggtatgaatctgcattccatggaaatggtcctgtgatcacagaagagcacaaaagggcagaggacaaggacaaggaagggaggtctcacaggaatggaaacatgggagagaaagggaggctcagggccgagagagctttcaggccatcatcacaagagaaggctaagtggcaaagggtctccaaattaccaatttgttctagtctttcttttggaattttctgctacaatgttaagaagtgcttaacttacccatactaccacttcgactgctctcaaatatctgaaaagtaagaatgaaagaatttttaaaattttcaaagtctgatcttagtatttcaaaatcagtgtaggaacttttatacacattgctgaattgaagcaaaacataacccaccagacatcaatgggtcagtttttacaatttaataatttcaaaggaaagattaaaagtgaacctcttttcaatatggtcagaacaacaataacaaacaaaattctttaatttttgagacagaattttcttctttgtggtcagtcacctatctcatatccctcataatatcattgctatcatctttcaataaatgttgatctataaattaattaacttttttgagacaaatccctggtatactattcttctgattcccatgaaagactcacttttaagatacaattgcagctgccccacactgccagttactgtgtcatacacacgccttaaaattctgtaatcagcaaccaccaggtgccgtatcgcattcagcacaccacagtcagtcaatacagacatccccaaacacaccaaggctggttttgtcaaatgttttattgagtgtagacatctggagtactgtaaaacatgcattatctgtagattcaaaaaggagcaagccacattgtcctcactgtcaaatgtgtcaggcttggcatacatgatggagattaatgaagtatcatgagagtaatatggttcctgaaaagcttctacaatttggagtagggtcttaatcacgtgaaaagcaaagctgttcacatttagtgaacctgcatttcatgggggggggggggtacacagtattttaattttaaaacaaataaaaataatttgtttgtcaaagattcccatctccccaactttatttgtcgcattggttttcagaaattttaattttttaaaaatcagatgccttttggaagttgtatgtttatctgagcaataactaaattttatttcttcttcggttgttgaggtgtgttaaatttgaagaagataatatctccatcttcaacaatataatttctgccttgttgtctgtactttccagcagccttgactgcattttcagaaccttcctctttaaaatcttcgtatttcattacttcagccataatgaatcccttttcaaaatctgtgtgaatctttcctgcagcctgaggagccttagtccctttcctgatggtccatgcacgcacttcatctgggcctgcagtgaaaaagtattctagttggagtgctgcaaacccagccttaatgatctttggcaaagcactttgtgtcatgttcgcttccagatacttctgtctctcctcagcactcaattcttgcaacttgagttccaaggccccacatttgtttttctttctaatgtagtctttttcagaaagattaaccaagtagaccattggttttgaagtcaaaaataagtgtttattcaacacttcaatctctttgtcattccaatcatgatagaagcgaacaggtttcttttgatctataacccaggattttactttgcacattatatcatattcaggttttagttttttatctcctcctctcacagccaccttttctagtttatctataatgggcccaatcatttcctcatctttaagctgaagctcttcatgtattatttctatatctcgaataggatctacacttccttcaacgtgcgtgatatcatcatcttcaaaagcacgtgttagatgaaagatgccatcacaggcactaatatgagataaaaaagcattccccaggccctgcccattgtgagctcctttcacaaggccagcaatatccaccacatttagaaaggcaggaattttgcttgctggtttgtggtattgacaaagaaagtcaaacctttcatctggcacaggtactctgctctcattaggatcaatagtgcagaacgggaagttttctgctgaagcctgactattggttaacacattgaagaaagtagatttcccaacatttggcaatccaacaataccaattttcagtgaggttccaaatcttccaatgattgggggtggtttaattccatcacctccctttttagggggcatcgtgctcggcctgggcgatgacacggggtcccagcggcagcgagagaaaggtcctgccggcagctggaggcggggaggaag

SEQ ID NO: 12051 - RNA, 3585 nt, Homo sapiens
  source 1..3585: mol_type = other RNA
ctgaatagctgggactacaggtgtgtgccatgatgcccagctaatttttgtatatatgtatttttttatgtagagatgatgtttcatgatgttgcacaggctggtctcaaactcctgtgctcaagtgatcctcccacctcggcctcccaaagtgttgggattataggtgtgagcctccacgcctggcctcaaatctcttttaaccataaatttgattaagatggagctacagatacatgcaaaaatatttacataacatcctaaaatatattaactttatcaatattaaaggagggaaaacgtttagatataggcatatatatgattatatgtaacagttcttggaattctcgactttcagagaaaatgaaattttgtatatgtacatacaatgttgtagaacttctaaccaaattaaacatttttaacatttattttcagcccctaatgaatgcagttacctcaaaactaactcctttcttttattaatggttctgttgcacaatgtgcaatttaccacattagaagctagacaaagtaaaattgcatgatcctaatgtctttttactgatttcaaacttctttaagaagtccatgcaatttactttggagaagacccaaaagcaagatatttgattctttcttatactgctgaaatccctaacaatccactaatctacacattactccaatacagaaatagatataacaaggatttttcacagcaaacttggtcagctatacctgtagcctagttttatttgttttatttagttcttttaaaaaacccttcattagttttattcttatttctctgctgtagtttactcatttttatgttagcaaaagaagatcactatttgatactaaaaaaatactcactggagagcttctaaattatactcacgactcaacctcatcctctttaaatatcttaagtatagccaaatctttaaaaaatcaccccttttcttgcctctagtgctacatttggtaactttccattttaagtttgtgtgtgttctaatacttctgcatctttaaagtcccaaagcgatacagtagaggcaaaggctggctgggtatgaatctgcattccatggaaatggtcctgtgatcacagaagagcacaaaagggcagaggacaaggacaaggaagggaggtctcacaggaatggaaacatgggagagaaagggaggctcagggccgagagagctttcaggccatcatcacaagagaaggctaagtggcaaagggtctccaaattaccaatttgttctagtctttcttttggaattttctgctacaatgttaagaagtgcttaacttacccatactaccacttcgactgctctcaaatatctgaaaagtaagaatgaaagaatttttaaaattttcaaagtctgatcttagtatttcaaaatcagtgtaggaacttttatacacattgctgaattgaagcaaaacataacccaccagacatcaatgggtcagtttttacaatttaataatttcaaaggaaagattaaaagtgaacctcttttcaatatggtcagaacaacaataacaaacaaaattctttaatttttgagacagaattttcttctttgtggtcagtcacctatctcatatccctcataatatcattgctatcatctttcaataaatgttgatctataaattaattaacttttttgagacaaatccctggtatactattcttctgattcccatgaaagactcacttttaagatacaattgcagctgccccacactgccagttactgtgtcatacacacgccttaaaattctgtaatcagcaaccaccaggtgccgtatcgcattcagcacaccacagtcagtcaatacagacatccccaaacacaccaaggctggttttgtcaaatgttttattgagtgtagacatctggagtactgtaaaacatgcattatctgtagattcaaaaaggagcaagccacattgtcctcactgtcaaatgtgtcaggcttggcatacatgatggagattaatgaagtatcatgagagtaatatggttcctgaaaagcttctacaatttggagtagggtcttaatcacgtgaaaagcaaagctgttcacatttagtgaacctgcatttcatgggggggggggggtacacagtattttaattttaaaacaaataaaaataatttgtttgtcaaagattcccatctccccaactttatttgtcgcattggttttcagaaattttaattttttaaaaatcagatgccttttggaagttgtatgtttatctgagcaataactaaattttatttcttcttcggttgttgaggtgtgttaaatttgaagaagataatatctccatcttcaacaatataatttctgccttgttgtctgtactttccagcagccttgactgcattttcagaaccttcctctttaaaatcttcgtatttcattacttcagccataatgaatcccttttcaaaatctgtgtgaatctttcctgcagcctgaggagccttagtccctttcctgatggtccatgcacgcacttcatctgggcctgcagtgaaaaagtattctagttggagtgctgcaaacccagccttaatgatctttggcaaagcactttgtgtcatgttcgcttccagatacttctgtctctcctcagcactcaattcttgcaacttgagttccaaggccccactaaaaggaatgaccaaagcacctgggtcatacttgtccacccactctttaatttttatcaaccatttgtttttctttctaatgtagtctttttcagaaagattaaccaagtagaccattggttttgaagtcaaaaataagtgtttattcaacacttcaatctctttgtcattccaatcatgatagaagcgaacaggtttcttttgatctataacccaggattttactttgcacattatatcatattcaggttttagttttttatctcctcctctcacagccaccttttctagtttatctataatgggcccaatcatttcctcatctttaagctgaagctcttcatgtattatttctatatctcgaataggatctacacttccttcaacgtgcgtgatatcatcatcttcaaaagcacgtgttagatgaaagatgccatcacaggcactaatatgagataaaaaagcattccccaggccctgcccattgtgagctcctttcacaaggccagcaatatccaccacatttagaaaggcaggaattttgcttgctggtttgtggtattgacaaagaaagtcaaacctttcatctggcacaggtactctgctctcattaggatcaatagtgcagaacgggaagttttctgctgaagcctgactattggttaacacattgaagaaagtagatttcccaacatttggcaatccaacaataccaattttcagtgaggttccaaatcttccaatgattgggggtggtttaattccatcacctccctttttagggggcatcgtgctcggcctgggcgatgacacggggtcccagcggcagcgagagaaaggtcctgccggcagctggaggcggggaggaag

SEQ ID NO: 12052 - RNA, 3484 nt, Homo sapiens
  source 1..3484: mol_type = other RNA
ctgaatagctgggactacaggtgtgtgccatgatgcccagctaatttttgtatatatgtatttttttatgtagagatgatgtttcatgatgttgcacaggctggtctcaaactcctgtgctcaagtgatcctcccacctcggcctcccaaagtgttgggattataggtgtgagcctccacgcctggcctcaaatctcttttaaccataaatttgattaagatggagctacagatacatgcaaaaatatttacataacatcctaaaatatattaactttatcaatattaaaggagggaaaacgtttagatataggcatatatatgattatatgtaacagttcttggaattctcgactttcagagaaaatgaaattttgtatatgtacatacaatgttgtagaacttctaaccaaattaaacatttttaacatttattttcagcccctaatgaatgcagttacctcaaaactaactcctttcttttattaatggttctgttgcacaatgtgcaatttaccacattagaagctagacaaagtaaaattgcatgatcctaatgtctttttactgatttcaaacttctttaagaagtccatgcaatttactttggagaagacccaaaagcaagatatttgattctttcttatactgctgaaatccctaacaatccactaatctacacattactccaatacagaaatagatataacaaggatttttcacagcaaacttggtcagctatacctgtagcctagttttatttgttttatttagttcttttaaaaaacccttcattagttttattcttatttctctgctgtagtttactcatttttatgttagcaaaagaagatcactatttgatactaaaaaaatactcactggagagcttctaaattatactcacgactcaacctcatcctctttaaatatcttaagtatagccaaatctttaaaaaatcaccccttttcttgcctctagtgctacatttggtaactttccattttaagtttgtgtgtgttctaatacttctgcatctttaaagtcccaaagcgatacagtagaggcaaaggctggctgggtatgaatctgcattccatggaaatggtcctgtgatcacagaagagcacaaaagggcagaggacaaggacaaggaagggaggtctcacaggaatggaaacatgggagagaaagggaggctcagggccgagagagctttcaggccatcatcacaagagaaggctaagtggcaaagggtctccaaattaccaatttgttctagtctttcttttggaattttctgctacaatgttaagaagtgcttaacttacccatactaccacttcgactgctctcaaatatctgaaaagtaagaatgaaagaatttttaaaattttcaaagtctgatcttagtatttcaaaatcagtgtaggaacttttatacacattgctgaattgaagcaaaacataacccaccagacatcaatgggtcagtttttacaatttaataatttcaaaggaaagattaaaagtgaacctcttttcaatatggtcagaacaacaataacaaacaaaattctttaatttttgagacagaattttcttctttgtggtcagtcacctatctcatatccctcataatatcattgctatcatctttcaataaatgttgatctataaattaattaacttttttgagacaaatccctggtatactattcttctgattcccatgaaagactcacttttaagatacaattgcagctgccccacactgccagttactgtgtcatacacacgccttaaaattctgtaatcagcaaccaccaggtgccgtatcgcattcagcacaccacagtcagtcaatacagacatccccaaacacaccaaggctggttttgtcaaatgttttattgagtgtagacatctggagtactgtaaaacatgcattatctgtagattcaaaaaggagcaagccacattgtcctcactgtcaaatgtgtcaggcttggcatacatgatggagattaatgaagtatcatgagagtaatatggttcctgaaaagcttctacaatttggagtagggtcttaatcacgtgaaaagcaaagctgttcacatttagtgaacctgcatttcatgggggggggggggtacacagtattttaattttaaaacaaataaaaataatttgtttgtcaaagattcccatctccccaactttatttgtcgcattggttttcagaaattttaattttttaaaaatcagatgccttttggaagttgtatgtttatctgagcaataactaaattttatttcttcttcggttgttgaggtgtgttaaatttgaagaagataatatctccatcttcaacaatataatttctgccttgttgtctgtactttccagcagccttgactgcattttcagaaccttcctctttaaaatcttcgtatttcattacttcagccataatgaatcccttttcaaaatctgtgtgaatctttcctgcagcctgaggagccttagtccctttcctgatggtccatgcacgcacttcatctgggcctgcagtgaaaaagtattctagttggagtgctgcaaacccagccttaatgatctttggcaaagcactttgtgtcatgttcgcttccagatacttctgtctctcctcagcactcaattcttgcaacttgagttccaaggccccactaaaaggaatgaccaaagcacctgggtcatacttgtccacccactctttaatttttatcaaccatttgtttttctttctaatgtagtctttttcagaaagattaaccaagtagaccattggttttgaagtcaaaaataagtgtttattcaacacttcaatctctttgtcattccaatcatgatagaagcgaacaggtttcttttgatctataacccaggattttactttgcacattatatcatattcaggttttagttttttatctcctcctctcacagccaccttttctagtttatctataatgggcccaatcatttcctcatctttaagctgaagctcttcatgtattatttctatatctcgaataggatctacacttccttcaacgtgcgtgatatcatcatcttcaaaagcacgtgttagatgaaagatgccatcacaggcactaatatgagataaaaaagcattccccaggccctgcccattgtgagctcctttcacaaggccagcaatatccaccacatttagaaaggcaggaattttgcttgctggtttgtggtattgacaaagaaagtcaaacctttcatctggcacaggtactctgctctcattaggatcaatagtgcagaacgggaagttttctgctgaagcctgactattggttaacacattgaagaaagtagatttccgtgctcggcctgggcgatgacacggggtcccagcggcagcgagagaaaggtcctgccggcagctggaggcggggaggaag

SEQ ID NO: 12053 - RNA, 1713 nt, Homo sapiens
  source 1..1713: mol_type = other RNA
ctgaatagctgggactacaggtgtgtgccatggggccccagtaattttgtttttatgtttagtggagacagggtctcgctttgtttcccagactggtctggaactcctgtcttcaatcagtcctactgccttggcctctcaaagtgctgagattacaggtgtcagccactcttttttttttttaatggccgaataatagtctgttgtataaatataccatattttgtttatccatttattcattcttggacatttgggttgtttttacttattggctattatgagcaatgataatgtgaaatctcatacccaagtttttttgtggggagatatgttttcatttctcttggctacatacccacaagtggaactgctgaatcctatggtaattttatgtttaatcctttgagaaactgccaaactgttttccaaactggttgtaccattttacatccccaccatcagtgtgtgaatttcctcccctgtctgtctcttgctccctctctcaccatgtgacacgctggctccgtttccccttctgccatgattctaagcttcctgaggccctcaccaagagcagatgccggcaccacaccctcttgtacagactgcagaactgtgagccaaagaaacctcttttctttatacatgacccagtctcaggtattcttttatagcaacgcaaacagactaacacacagcaccctgggagattttattcttccttaggtggtgactctactgttaggtttttttccaaatacttccatccctaagaatttagtgaggcagttctaaattagacaaagcgggagagagcaaaagagttgacagaaaagccttgggcagcctgagccacaatgagcttagatgaagtagttgggacattcgtgggcaaacaaatgccaggcttgattaaaggcgtccacgacagccggctccaggggcccttcctctgccgctgccaagttctgctccagctgctccaggctggacatgcccaggatgaccgcgtccccgtgggcaccctgcagctgtgagtggtggtacatccaccggagggcggccgaggtcatgctgggagcgctggcgccatacgcggcctgcagggccttctccaccagggcaatgccctcgaagtggtgctccttccagaagctggtacacagtgggcaggatccagccgttgctcttgcagagggtacagatctcggccacttcccaggcggcatagttggagaggccaagctccacgaacttgccctcctggtgcagctggtggcaggcacgcagtgtctcttccaccggggcgctgtggtcaggtgcatgtagatagaagaggtccactcagggacactgcagccgcttcagtgacgtctccagctgggatcggacactgtcaggcttcagggagttcccaatccatggattggccttggtagcaattttcactctgcagtcgctgctgcccattcggagccccaggccgccaaggatggtctcggactggccgtcgctgtacaggaaggccgtgtctatctcggtgtggccgcgctccaggaaggcgcgcgtgactgcggcgctggtgggcgcgtccatgcggcgccccatctccatggcgcccagcaccgtggctggccgggcccgcgacagctgccgggacatgacggcggcaacgggagactgtgacagcccaggagccgcgcgcagcgg

SEQ ID NO: 12054 - RNA, 1910 nt, Homo sapiens
  source 1..1910: mol_type = other RNA
ctgaatagctgggactacaggtgtgtgccatggggccccagtaattttgtttttatgtttagtggagacagggtctcgctttgtttcccagactggtctggaactcctgtcttcaatcagtcctactgccttggcctctcaaagtgctgagattacaggtgtcagccactcttttttttttttaatggccgaataatagtctgttgtataaatataccatattttgtttatccatttattcattcttggacatttgggttgtttttacttattggctattatgagcaatgataatgtgaaatctcatacccaagtttttttgtggggagatatgttttcatttctcttggctacatacccacaagtggaactgctgaatcctatggtaattttatgtttaatcctttgagaaactgccaaactgttttccaaactggttgtaccattttacatccccaccatcagtgtgtgaatttcctcccctgtctgtctcttgctccctctctcaccatgtgacacgctggctccgtttccccttctgccatgattctaagcttcctgaggccctcaccaagagcagatgccggcaccacaccctcttgtacagactgcagaactgtgagccaaagaaacctcttttctttatacatgacccagtctcaggtattcttttatagcaacgcaaacagactaacacacagcaccctgggagattttattcttccttaggtggtgactctactgttaggtttttttccaaatacttccatccctaagaatttagtgaggcagttctaaattagacaaagcgggagagagcaaaagagttgacagaaaagccttgggcagcctgagccacaatgagcttagatgaagtagttgggacattcgtgggcaaacaaatgccaggcttgattaaaggcgtccacgacagccggctccaggggcccttcctctgccgctgccaagttctgctccagctgctccaggctggacatgcccaggatgaccgcgtccccgtgggcaccctgcagctgtgagtggtggtacatccaccggagggcggccgaggtcatgctgggagcgctggcgccatacgcggcctgcagggccttctccaccagggcaatgccctcgaagtggtgctccttccagaagtgattcctgtagatctctgcccactgagtcccaaagaagcggcccacgggctgtttcccgtccttgtcctcatacttgtacttgccggtcagcaggcccccagccagagggttgtaggcatagaacctcagtccaaagtgcctgaggcaggggaagagctccgtttccacctgccgggtggtggcgctgtacatgccctggtacacagtgggcaggatccagccgttgctcttgcagagggtacagatctcggccacttcccaggcggcatagttggagaggccaagctccacgaacttgccctcctggtgcagctggtggcaggcacgcagtgtctcttccaccggggcgctgtggtcaggtgcatgtagatagaagaggtccactcagggacactgcagccgcttcagtgacgtctccagctgggatcggacactgtcaggcttcagggagttcccaatccatggattggccttggtagcaattttcactctgcagtcgctgctgcccattcggagccccaggccgccaaggatggtctcggactggccgtcgctgtacaggaaggccgtgtctatctcggtgtggccgcgctccaggaaggcgcgcgtgactgcggcgctggtgggcgcgtccatgcggcgccccatctccatggcgcccagcaccgtggctggccgggcccgcgacagctgccgggacatgacggcggcaacgggagactgtgacagcccaggagccgcgcgcagcgg

SEQ ID NO: 12055 - RNA, 1910 nt, Homo sapiens
  source 1..1910: mol_type = other RNA
ctgaatagctgggactacaggtgtgtgccatggggccccagtaattttgtttttatgtttagtggagacagggtctcgctttgtttcccagactggtctggaactcctgtcttcaatcagtcctactgccttggcctctcaaagtgctgagattacaggtgtcagccactcttttttttttttaatggccgaataatagtctgttgtataaatataccatattttgtttatccatttattcattcttggacatttgggttgtttttacttattggctattatgagcaatgataatgtgaaatctcatacccaagtttttttgtggggagatatgttttcatttctcttggctacatacccacaagtggaactgctgaatcctatggtaattttatgtttaatcctttgagaaactgccaaactgttttccaaactggttgtaccattttacatccccaccatcagtgtgtgaatttcctcccctgtctgtctcttgctccctctctcaccatgtgacacgctggctccgtttccccttctgccatgattctaagcttcctgaggccctcaccaagagcagatgccggcaccacaccctcttgtacagactgcagaactgtgagccaaagaaacctcttttctttatacatgacccagtctcaggtattcttttatagcaacgcaaacagactaacacacagcaccctgggagattttattcttccttaggtggtgactctactgttaggtttttttccaaatacttccatccctaagaatttagtgaggcagttctaaattagacaaagcgggagagagcaaaagagttgacagaaaagccttgggcagcctgagccacaatgagcttagatgaagtagttgggacattcgtgggcaaacaaatgccaggcttgattaaaggcgtccacgacagccggctccaggggcccttcctctgccgctgccaagttctgctccagctgctccaggctggacatgcccaggatgaccgcgtccccgtgggcaccctgcagctgtgagtggtggtacatccaccggagggcggccgaggtcatgctgggagcgctggcgccatacgcggcctgcagggccttctccaccagggcaatgccctcgaagtggtgctccttccagaagtgattcctgtagatctctgcccactgagtcccaaagaagcggcccacgggctgtttcccgtccttgtcctcatacttgtacttgccggtcagcaggcccccagccagagggttgtaggcatagaacctcagtccaaagtgcctgaggcaggggaagagctccgtttccacctgccgggtggtggcgctgtacatgccctggtacacagtgggcaggatccagccgttgctcttgcagagggtacagatctcggccacttcccaggcggcatagttggagaggccaagctccacgaacttgccctcctggtgcagctggtggcaggcacgcagtgtctcttccaccggggcgctgtggtcaggtgcatgtagatagaagaggtccactcggggacactgcagccgcttcagtgacgtctccagctgggatcggacactgtcaggcttcagggagttcccaatccatggattggccttggtagcaattttcactctgcagtcgctgctgcccattcggagccccaggccgccaaggatggtctcggactggccgtcgctgtacaggaaggccgtgtctatctcggtgtggccgcgctccaggaaggcgcgcgtgactgcggcgctggtgggcgcgtccatgcggcgccccatctccatggcgcccagcaccgtggctggccgggcccgcgacagctgccgggacatgacggcggcaacgggagactgtgacagcccaggagccgcgcgcagcgg

SEQ ID NO: 12056 - RNA, 3212 nt, Homo sapiens
  source 1..3212: mol_type = other RNA
ctgaatagctgggactacaggtgtgtgccattatgcctggctaatttttttttgttgggggagagggggatagagacagggttttcccatgttgtccaggctggtctcaaattcctgggctcaagtgatccttctgccttggcctcccaatgtgctgggattacaggtgtcagtatagatttttattatctgttttctcagtcttcaaagggtcccacgttaaatgctacaccatttcctaaactcatgctcacatccctggctggttctacaggccttccaccaggacctctggaaccacttcttatcatgtgctgggagtggcatctgatgtatggggagatgcaaattcccacatacccccttactggccctttgttggtcccgaatggccagaatacatagatgttcagtaccaaaattacacacttgtgaaaaaccaatttggcactgttctttccacctttactgttgctggaaacttgaaacccagaatacaattttacggttagaccctgcaaattgcagtttgtcatgtaatcttttacattttggtccatggacttatgaataggatgccaaactctagttgactatgtatatgattactttttctttctacttaagcacaaaattcattattaagtggggaaatacaaagataatctcagattagtttacaaaagcaggcaaacaatgcatagctataattgcatatatacatataaaatgtatatataatatataatacacgggggtggagatagagaaggagagaggatatgacatcaagctattaactatactgatatgtagaaagcaaacaacttgatagtcaactcttactttatcacatctcatcagccccaaatatctcagagacttgctgctctgtgcaatcagggtggctccttggtctgtgatttctttacaccatccgacatccacagtctctattgtcatgctgtatcgcccaatggctatcagtgcataatctgtgattttacaggacaccaaatatagctctttcaggttttgtccttcctttgcaatgacctccacacacctgtcatttatgatccagttcagacagagattgagagagctaagatttttgcacctcttgacaatttccatcacggtttcattatccagttcagtgatatgacgtaggtccaagctggaaaggtttcttagcttggttaggtgaatgactcctttagaagtgactgaacaacccatgaagcctacatattgaagctcaggacagtgttcagcaaatgctttcactgactgatctgtcactaatttgttttcctgcatgtatatcctttgtaatttcagacagcccttagctatgacgatcatgccttcatctgagatcttgtaacactggccgaaatgaatatctttgagttctctgcattttgagcccagctgcttgagtccttcatcagtgagtttgtcctggttgcctacatgcactttctgaagtaaaggacagtgagaggcaaccgcaataatagaggtgtcagaaagctgtttacacctgtaggctgtatacctaagaagtccaggacatttaaatgctaaaacacatacgccattatcagacatactgcgacaatcagaaatgttgatttcaattatattctgacttcttgatgcaattttttccaacaattcatcagtgacctgctgacgactactaagatccagctgcttccaaaactggaagtctaaacaaaggtcacgccagtacttgcaaaccaatgatgcggaaaggcaacgctcatccagtgacaaattggaaaatatcttgagcaggatggacggcggcagctggttgatgtctggggtttcggggggcggctccctgtgacagtcgcaggggttttcgggggactcccgacagtccgcgtcgccacattcatgctgctgctgggcggacaagggggcggtgcccccggctcggacagcgtccccgccagcttcggtgggggcaccttcggaggtgggagaagagggcggagggcagagcggctgcgggggctgctccggggcctggcagcagccggcgtcggggggccggggcggcgaagcgcctccccccgcaggccctcccccgccaccgccgccgccgccgccgccgcagcccccgccgccgcagcggggctgcttgcagggggtgcaggcggggaccccggcccccttccgcttgcacaccatttcggggggcgtagggagctcggccggtgacggtgtcggcccccggaagagctgcacggcggcgggcggccccaggaagcgcaccggccccaagctggccaggaagagacttcggccctgctgctcccaggcggcggccgcagccagccccaactctttgcagcaggaggcgggcgacgaagccgaggcggcagcggcggcggcggcggcggccgaggatagcaggaagcggcgggcagcagcggcgcagtcctcggcggccagggccgcgtagcgccgcgccaggtgctgagaggaggaggcggcagcgtaggccccgtcccgcggcggcggcgagagcggcggctcctcctctgggccggcgggggcgggcgcgccgggactgtgcacgatgaagcagagcatgcagggcccgcggaagaagcagtcccggctccggggcgccgccggctgagggggcaccttggctggggtccggcggggcagcctgaggagagggcgccggcggcggcaccaactgcaacagcgaggcctcttctggctcgggcggttacgcggctccttcgagagaaggtggcccatatagaaggccccgaggagggggaccgggacgggagggagggagacccagagaggcgggctcccggcagcggggcaggccgctcgctggctcggcccccggaggggtcgcccttcctgcgcacacacacgcacacacgggcacacacgcgacggtggggggtgggcgtcagctgcgggccgccggagtgcccgacgggggctacatgctttgcccagggaagccgggagaacgatgggcgcgagctttggggacgcgagggagggagcgagcgagcctgccggctaggcgaccagtccgggcccggccagccggctcagtcagtcagcggagcggccggggaaaggccgggtcccgctcggaccattttaactgcggatccgccgccggcgcgcgcacccgc

SEQ ID NO: 12057 - RNA, 755 nt, Homo sapiens
  source 1..755: mol_type = other RNA
ctgaatagctgggactacaggtgtgtgctatcacaaccagctaaatttttgtatattttgtaaagatagggtctcccagtgttgcccaggctgttctcaaactcttgggctcaagcaaagccccagccccagcctcccaaagtgctgggactacaagtatgagccatcacaccccaggaattaatccacaataagcttttctatttctgactccatcttagccactgctttccagagaacctgttagtgccatggccctatagctcagtttcttcacttgcaaattgaagatggagataatcattccaggcagacaggaatcaggcaatggtggtgctaagcatgaggaagtaatttcactccaaagcaaacagcacatatagaatcagagacttgtgaaacatcatggcttcgaaacagtctcacctaatgcaaaacaatcactcagtggacccagcagccctttgtgatacttgtgatacgtacaccgtttcttcagggcagttgaacagttgcccagtggcatggaatccatgttacacctgtcttctggagagaagaatatatctgtctcattagatgagaagcaaggttatctaagttttctaggtttactggagagtgagtcttgcattccccattagatgataagttcacatgcttagcaagcagagaggtagagtcgttgggttttgtaaagaaagcccactaaaagaggctgctgttcaatcccacctactggtatccaacaaaat

SEQ ID NO: 12058 - RNA, 2687 nt, Homo sapiens
  source 1..2687: mol_type = other RNA
ctgaatagctgggactacaggtgtgtgtcaccatgcccagtaatttttttgtatatttgtagaggcagggtctcccaatgttgcctgggctggtctcaaactcctgggctcaagcaatccaccagctttggccttccaaagttctaggattatacgcatgagccactgtgccctgccccaatattttgttacttactagtgagactaaacacttttctaaaagtttgttagccatactatcctataaaagctgtttgttcatgtcttttgtccatttatctttttttttgtttttcttgagacagagtcttgctctgtggcccaggctggagtgcaggggtgcaatctcggctcactgcaagctccgcctcccaggttcaaatgattctcctgcctcagcctcctgagtagctgggattacaggcatgtgccaccatgcccagctaatttttttgtgtgtgtttttcagtagagatggggtttcaccatgttggccaggctgatctcgaattcctgacctcaggtgctccacccgcctcagcctcccaaagtactgggattacaggggtgagccaccgcacccggccaattttctgtatttttaatagagacagggtttcatcctgttggccaggctggcctcgaacttcggacctcaggtgatccacccgcctcgacctcccaaagtgctgggattacaggtgtgggccaccacacccagccaatttttttgtatttttagtagagacagggtttcatcatgttggccaggctggtcgcaaactcctgacctcaggtgatccacccgcctcagcatcccaaagtgctgggattacaggcatgagccaccactcccggccaatgttttgtatttttagtagagatggggtttcatcatgttggccagactggtctcaaactctggacctcaggtgatccacctgcctcagcctcccaaagtgtagggattacaggtgtgagccaccgcgcccagcctatgtttctattttatacatattcaacaaacatgattccccaacttctgcaaaataatttctttttcaagaacattgattttagagctcacactaagaaaaagaatacaaaaataatggcatagaaagtgaaaaaacaaaaataaaaagtagaaagctaaagtttcccattaaaatgatcaatatactgtgcagtaagtcaaatgtgtacaatgaattaagaaaatatgatatataaaaatccaaatttacaaaattaagtacaaataggtgtttatattacaaagtgatactggtttataaaaggattcaacatagattttttttaaatggttgttttcctcaatcaatttaacaatgattttaaatgtataaaattttaatatctctttgagacagtgatccaagcttcttcccttgatgatgttaccagttcatactttgtttcaataacctgtccctccacagaaagtaggtgcagtctcttcaccaatacactaagaagtactgtggtcaccatatatgcaaacctcaactctggacactcctgtgtgcctgagaatccaagtgaggaaaaagttttcattactaattcatcatcaaaccgatctggatcaaacttgtgtggagatggccaagtattaggatcctgaagtaccacaccaagggcataaaggacgagggtctctctaggaataataaatcggtcaatttttccttcaatatcttgaagctgggcagaaactggagtcagtttggcagttcgaacagtttcacaaagcacatgctgacaatatattttgcagttattatgcaactggccagagaaaatatcatactgtcttctaggatctgttggtcattaaggttcccttgtactaaggagtcaatgaaaatatgttgactgaagttccttccttttcgttcttttatgatgttccttaaaacagactccagttgcatgagggcatcttcatattgttttttccgagtcatgtttttatcaagtgacccatctagaaagccttttccaatctcagaccaaactgtgccatgattcttctggaagcgaatgacttcctgatcatcttcaaatgtactacccattaccatctgtgtaacagacttcatagcaaaaccaagcatatgctggctgaggggcacgtgctgggtctctgggtaggagagccatttatctaataattcttctgaaagctttaggaggagggcaaagttactcttcagagaatcagtcacaccattttcatacaattttttcctcatgtggttttcactcacactgccaccaccagattgataccttaataatgacttcagcatggtttcaaaagggtccgatgtcttattgggattgatatgctgcttcagtacatcaacagtgcccaaactaaccacgaggcgcctgccaaaccagaaggagaccacaggcccatatctctcatgcaaattaaccaggaactcatgcaaacttccactattcacaatatctggaagattaccatctttttcttcagttggagtaatccctggaattcctgcagcttgtctggaagccggatagaggtagagcacggctcccaccaacgccagcaagaaggtaacggcgaagatcgcgaagtccaacatggttctgccgcccagggagccacgtctcggatcggccgctccagc

SEQ ID NO: 12059 - RNA, 2608 nt, Homo sapiens
  source 1..2608: mol_type = other RNA
ctgaatagctgggactacaggtgtgtgtcaccatgcccagtaatttttttgtatatttgtagaggcagggtctcccaatgttgcctgggctggtctcaaactcctgggctcaagcaatccaccagctttggccttccaaagttctaggattatacgcatgagccactgtgccctgccccaatattttgttacttactagtgagactaaacacttttctaaaagtttgttagccatactatcctataaaagctgtttgttcatgtcttttgtccatttatctttttttttgtttttcttgagacagagtcttgctctgtggcccaggctggagtgcaggggtgcaatctcggctcactgcaagctccgcctcccaggttcaaatgattctcctgcctcagcctcctgagtagctgggattacaggcatgtgccaccatgcccagctaatttttttgtgtgtgtttttcagtagagatggggtttcaccatgttggccaggctgatctcgaattcctgacctcaggtgctccacccgcctcagcctcccaaagtactgggattacaggggtgagccaccgcacccggccaattttctgtatttttaatagagacagggtttcatcctgttggccaggctggcctcgaacttcggacctcaggtgatccacccgcctcgacctcccaaagtgctgggattacaggtgtgggccaccacacccagccaatttttttgtatttttagtagagacagggtttcatcatgttggccaggctggtcgcaaactcctgacctcaggtgatccacccgcctcagcatcccaaagtgctgggattacaggcatgagccaccactcccggccaatgttttgtatttttagtagagatggggtttcatcatgttggccagactggtctcaaactctggacctcaggtgatccacctgcctcagcctcccaaagtgtagggattacaggtgtgagccaccgcgcccagcctatgtttctattttatacatattcaacaaacatgattccccaacttctgcaaaataatttctttttcaagaacattgattttagagctcacactaagaaaaagaatacaaaaataatggcatagaaagtgaaaaaacaaaaataaaaagtagaaagctaaagtttcccattaaaatgatcaatatactgtgcagtaagtcaaatgtgtacaatgaattaagaaaatatgatatataaaaatccaaatttacaaaattaagtacaaataggtgtttatattacaaagtgatactggtttataaaaggattcaacatagattttttttaaatggttgttttcctcaatcaatttaacaatgattttaaatgtataaaattttaatatctctttgagacagtgatccaagcttcttcccttgatgatgttaccagttcatactttgtttcaataacctgtccctccacagaaagtaggtgcagtctcttcaccaatacactaagaagtactgtggtcaccatatatgcaaacctcaactctggacactcctgtgtgcctgagaatccaagtgaggaaaaagttttcattactaattcatcatcaaaccgatctggatcaaacttgtgtggagatggccaagtattaggatcctgaagtaccacaccaagggcataaaggacgagggtctctctaggaataataaatcggtcaatttttccttcaatatcttgaagctgggcagaaactggagtcagtttggcagttcgaacagtttcacaaagcacatgctgacaatatattttgcagttattatgcaactggccagagaaaatatcatactgtcttctaggatctgttggtcattaaggttcccttgtactaaggagtcaatgaaaatatgttgactgaagttccttccttttcgttcttttatgatgttccttaaaacagactccagttgcatgagggtgtgccatgattcttctggaagcgaatgacttcctgatcatcttcaaatgtactacccattaccatctgtgtaacagacttcatagcaaaaccaagcatatgctggctgaggggcacgtgctgggtctctgggtaggagagccatttatctaataattcttctgaaagctttaggaggagggcaaagttactcttcagagaatcagtcacaccattttcatacaattttttcctcatgtggttttcactcacactgccaccaccagattgataccttaataatgacttcagcatggtttcaaaagggtccgatgtcttattgggattgatatgctgcttcagtacatcaacagtgcccaaactaaccacgaggcgcctgccaaaccagaaggagaccacaggcccatatctctcatgcaaattaaccaggaactcatgcaaacttccactattcacaatatctggaagattaccatctttttcttcagttggagtaatccctggaattcctgcagcttgtctggaagccggatagaggtagagcacggctcccaccaacgccagcaagaaggtaacggcgaagatcgcgaagtccaacatggttctgccgcccagggagccacgtctcggatcggccgctccagc

SEQ ID NO: 12060 - RNA, 2391 nt, Homo sapiens
  source 1..2391: mol_type = other RNA
ctgaatagctgggactacaggtgtgtgtcaccatgcccagtaatttttttgtatatttgtagaggcagggtctcccaatgttgcctgggctggtctcaaactcctgggctcaagcaatccaccagctttggccttccaaagttctaggattatacgcatgagccactgtgccctgccccaatattttgttacttactagtgagactaaacacttttctaaaagtttgttagccatactatcctataaaagctgtttgttcatgtcttttgtccatttatctttttttttgtttttcttgagacagagtcttgctctgtggcccaggctggagtgcaggggtgcaatctcggctcactgcaagctccgcctcccaggttcaaatgattctcctgcctcagcctcctgagtagctgggattacaggcatgtgccaccatgcccagctaatttttttgtgtgtgtttttcagtagagatggggtttcaccatgttggccaggctgatctcgaattcctgacctcaggtgctccacccgcctcagcctcccaaagtactgggattacaggggtgagccaccgcacccggccaattttctgtatttttaatagagacagggtttcatcctgttggccaggctggcctcgaacttcggacctcaggtgatccacccgcctcgacctcccaaagtgctgggattacaggtgtgggccaccacacccagccaatttttttgtatttttagtagagacagggtttcatcatgttggccaggctggtcgcaaactcctgacctcaggtgatccacccgcctcagcatcccaaagtgctgggattacaggcatgagccaccactcccggccaatgttttgtatttttagtagagatggggtttcatcatgttggccagactggtctcaaactctggacctcaggtgatccacctgcctcagcctcccaaagtgtagggattacaggtgtgagccaccgcgcccagcctatgtttctattttatacatattcaacaaacatgattccccaacttctgcaaaataatttctttttcaagaacattgattttagagctcacactaagaaaaagaatacaaaaataatggcatagaaagtgaaaaaacaaaaataaaaagtagaaagctaaagtttcccattaaaatgatcaatatactgtgcagtaagtcaaatgtgtacaatgaattaagaaaatatgatatataaaaatccaaatttacaaaattaagtacaaataggtgtttatattacaaagtgatactggtttataaaaggattcaacatagattttttttaaatggttgttttcctcaatcaatttaacaatgattttaaatgtataaaattttaatatctctttgagacagtgatccaagcttcttcccttgatgatgttaccagttcatactttgtttcaataacctgtccctccacagaaagtaggtgcagtctcttcaccaatacactaagaagtactgtggtcaccatatatgcaaacctcaactctggacactcctgtgtgcctgagaatccaagtgaggaaaaagttttcattactaattcatcatcaaaccgatctggatcaaacttgtgtggagatggccaagtattaggatcctgaagtaccacaccaagggcataaaggacgagggtctctctaggaataataaatcggtcaatttttccttcaatatcttgaagctgggcagaaactggagtcagtttggcagttcgaacagtttcacaaagcacatgctgacaatatattttgcagttattatgcaactggccagagaaaatatcatactgtcttctaggatctgttggtcattaaggttcccttgtactaaggagtcaatgaaaatatgttgactgaagttccttccttttcgttcttttatgatgttccttaaaacagactccagttgcatgagggtgtgccatgattcttctggaagcgaatgacttcctgatcatcttcaaatgtactacccattaccatctgtgtaacagacttcatagcaaaaccaagcatatgctggctgaggggcacgtgctgggtctctgggtaggagagccatttatctaataattcttctgaaagctttaggaggagggcaaagttactcttcagagaatcagtcacaccattttcatacaattttttcctcatgtggttttcactcacactgccaccaccagattgataccttaataatgacttcagcatggtttcaaaagggtccgcggatagaggtagagcacggctcccaccaacgccagcaagaaggtaacggcgaagatcgcgaagtccaacatggttctgccgcccagggagccacgtctcggatcggccgctccagc

SEQ ID NO: 12061 - RNA, 2832 nt, Homo sapiens
  source 1..2832: mol_type = other RNA
ctgaatagctgggactacaggtgtgtgtcaccatgcccagtaatttttttgtatatttgtagaggcagggtctcccaatgttgcctgggctggtctcaaactcctgggctcaagcaatccaccagctttggccttccaaagttctaggattatacgcatgagccactgtgccctgccccaatattttgttacttactagtgagactaaacacttttctaaaagtttgttagccatactatcctataaaagctgtttgttcatgtcttttgtccatttatctttttttttgtttttcttgagacagagtcttgctctgtggcccaggctggagtgcaggggtgcaatctcggctcactgcaagctccgcctcccaggttcaaatgattctcctgcctcagcctcctgagtagctgggattacaggcatgtgccaccatgcccagctaatttttttgtgtgtgtttttcagtagagatggggtttcaccatgttggccaggctgatctcgaattcctgacctcaggtgctccacccgcctcagcctcccaaagtactgggattacaggggtgagccaccgcacccggccaattttctgtatttttaatagagacagggtttcatcctgttggccaggctggcctcgaacttcggacctcaggtgatccacccgcctcgacctcccaaagtgctgggattacaggtgtgggccaccacacccagccaatttttttgtatttttagtagagacagggtttcatcatgttggccaggctggtcgcaaactcctgacctcaggtgatccacccgcctcagcatcccaaagtgctgggattacaggcatgagccaccactcccggccaatgttttgtatttttagtagagatggggtttcatcatgttggccagactggtctcaaactctggacctcaggtgatccacctgcctcagcctcccaaagtgtagggattacaggtgtgagccaccgcgcccagcctatgtttctattttatacatattcaacaaacatgattccccaacttctgcaaaataatttctttttcaagaacattgattttagagctcacactaagaaaaagaatacaaaaataatggcatagaaagtgaaaaaacaaaaataaaaagtagaaagctaaagtttcccattaaaatgatcaatatactgtgcagtaagtcaaatgtgtacaatgaattaagaaaatatgatatataaaaatccaaatttacaaaattaagtacaaataggtgtttatattacaaagtgatactggtttataaaaggattcaacatagattttttttaaatggttgttttcctcaatcaatttaacaatgattttaaatgtataaaattttaatatctctttgagacagtgatccaagcttcttcccttgatgatgttaccagttcatactttgtttcaataacctgtccctccacagaaagtaggtgcagtctcttcaccaatacactaagaagtactgtggtcaccatatatgcaaacctcaactctggacactcctgtgtgcctgagaatccaagtgaggaaaaagttttcattactaattcatcatcaaaccgatctggatcaaacttgtgtggagatggccaagtattaggatcctgaagtaccacaccaagggcataaaggacgagggtctctctaggaataataaatcggtcaatttttccttcaatatcttgaagctgggcagaaactggagtcagtttggcagttcgaacagtttcacaaagcacatgctgacaatatctgagctgctcaattttctctggagtaacaggaccatttccaaaaacttggtttatctcttcatataattttttttgaacttcttcagaggtggttaaaaaacagattgcccaggtacacaattttgcagttattatgcaactggccagagaaaatatcatactgtcttctaggatctgttggtcattaaggttcccttgtactaaggagtcaatgaaaatatgttgactgaagttccttccttttcgttcttttatgatgttccttaaaacagactccagttgcatgagggcatcttcatattgttttttccgagtcatgtttttatcaagtgacccatctagaaagccttttccaatctcagaccaaacctgaaaataggtaaatatacataatgtgccatgattcttctggaagcgaatgacttcctgatcatcttcaaatgtactacccattaccatctgtgtaacagacttcatagcaaaaccaagcatatgctggctgaggggcacgtgctgggtctctgggtaggagagccatttatctaataattcttctgaaagctttaggaggagggcaaagttactcttcagagaatcagtcacaccattttcatacaattttttcctcatgtggttttcactcacactgccaccaccagattgataccttaataatgacttcagcatggtttcaaaagggtccgatgtcttattgggattgatatgctgcttcagtacatcaacagtgcccaaactaaccacgaggcgcctgccaaaccagaaggagaccacaggcccatatctctcatgcaaattaaccaggaactcatgcaaacttccactattcacaatatctggaagattaccatctttttcttcagttggagtaatccctggaattcctgcagcttgtctggaagccggatagaggtagagcacggctcccaccaacgccagcaagaaggtaacggcgaagatcgcgaagtccaacatggttctgccgcccagggagccacgtctcggatcggccgctccagc

SEQ ID NO: 12062 - RNA, 2535 nt, Homo sapiens
  source 1..2535: mol_type = other RNA
ctgaatagctgggactacaggtgtgtgtcaccatgcccagtaatttttttgtatatttgtagaggcagggtctcccaatgttgcctgggctggtctcaaactcctgggctcaagcaatccaccagctttggccttccaaagttctaggattatacgcatgagccactgtgccctgccccaatattttgttacttactagtgagactaaacacttttctaaaagtttgttagccatactatcctataaaagctgtttgttcatgtcttttgtccatttatctttttttttgtttttcttgagacagagtcttgctctgtggcccaggctggagtgcaggggtgcaatctcggctcactgcaagctccgcctcccaggttcaaatgattctcctgcctcagcctcctgagtagctgggattacaggcatgtgccaccatgcccagctaatttttttgtgtgtgtttttcagtagagatggggtttcaccatgttggccaggctgatctcgaattcctgacctcaggtgctccacccgcctcagcctcccaaagtactgggattacaggggtgagccaccgcacccggccaattttctgtatttttaatagagacagggtttcatcctgttggccaggctggcctcgaacttcggacctcaggtgatccacccgcctcgacctcccaaagtgctgggattacaggtgtgggccaccacacccagccaatttttttgtatttttagtagagacagggtttcatcatgttggccaggctggtcgcaaactcctgacctcaggtgatccacccgcctcagcatcccaaagtgctgggattacaggcatgagccaccactcccggccaatgttttgtatttttagtagagatggggtttcatcatgttggccagactggtctcaaactctggacctcaggtgatccacctgcctcagcctcccaaagtgtagggattacaggtgtgagccaccgcgcccagcctatgtttctattttatacatattcaacaaacatgattccccaacttctgcaaaataatttctttttcaagaacattgattttagagctcacactaagaaaaagaatacaaaaataatggcatagaaagtgaaaaaacaaaaataaaaagtagaaagctaaagtttcccattaaaatgatcaatatactgtgcagtaagtcaaatgtgtacaatgaattaagaaaatatgatatataaaaatccaaatttacaaaattaagtacaaataggtgtttatattacaaagtgatactggtttataaaaggattcaacatagattttttttaaatggttgttttcctcaatcaatttaacaatgattttaaatgtataaaattttaatatctctttgagacagtgatccaagcttcttcccttgatgatgttaccagttcatactttgtttcaataacctgtccctccacagaaagtaggtgcagtctcttcaccaatacactaagaagtactgtggtcaccatatatgcaaacctcaactctggacactcctgtgtgcctgagaatccaagtgaggaaaaagttttcattactaattcatcatcaaaccgatctggatcaaacttgtgtggagatggccaagtattaggatcctgaagtaccacaccaagggcataaaggacgagggtctctctaggaataataaatcggtcaatttttccttcaatatcttgaagctgggcagaaactggagtcagtttggcagttcgaacagtttcacaaagcacatgctgacaatatctgagctgctcaattttctctggagtaacaggaccatttccaaaaacttggtttatctcttcatataattttttttgaacttcttcagaggtggttaaaaaacagattgcccaggtacacaattttgcagttattatgcaactggccagagaaaatatcatactgtcttctaggatctgttggtcattaaggttcccttgtactaaggagtcaatgaaaatatgttgactgaagttccttccttttcgttcttttatgatgttccttaaaacagactccagttgcatgagggcatcttcatattgttttttccgagtcatgtttttatcaagtgacccatctagaaagccttttccaatctcagaccaaactgtgccatgattcttctggaagcgaatgacttcctgatcatcttcaaatgtactacccattaccatctgtgtaacagacttcatagcaaaaccaagcatatgctggctgaggggcacgtgctgggtctctgggtaggagagccatttatctaataattcttctgaaagcttaataatgacttcagcatggtttcaaaagggtccgttttcttcagttggagtaatccctggaattcctgcagcttgtctggaagccggatagaggtagagcacggctcccaccaacgccagcaagaaggtaacggcgaagatcgcgaagtccaacatggttctgccgcccagggagccacgtctcggatcggccgctccagc

SEQ ID NO: 12063 - RNA, 2808 nt, Homo sapiens
  source 1..2808: mol_type = other RNA
ctgaatagctgggactacaggtgtgtgtcaccatgcccagtaatttttttgtatatttgtagaggcagggtctcccaatgttgcctgggctggtctcaaactcctgggctcaagcaatccaccagctttggccttccaaagttctaggattatacgcatgagccactgtgccctgccccaatattttgttacttactagtgagactaaacacttttctaaaagtttgttagccatactatcctataaaagctgtttgttcatgtcttttgtccatttatctttttttttgtttttcttgagacagagtcttgctctgtggcccaggctggagtgcaggggtgcaatctcggctcactgcaagctccgcctcccaggttcaaatgattctcctgcctcagcctcctgagtagctgggattacaggcatgtgccaccatgcccagctaatttttttgtgtgtgtttttcagtagagatggggtttcaccatgttggccaggctgatctcgaattcctgacctcaggtgctccacccgcctcagcctcccaaagtactgggattacaggggtgagccaccgcacccggccaattttctgtatttttaatagagacagggtttcatcctgttggccaggctggcctcgaacttcggacctcaggtgatccacccgcctcgacctcccaaagtgctgggattacaggtgtgggccaccacacccagccaatttttttgtatttttagtagagacagggtttcatcatgttggccaggctggtcgcaaactcctgacctcaggtgatccacccgcctcagcatcccaaagtgctgggattacaggcatgagccaccactcccggccaatgttttgtatttttagtagagatggggtttcatcatgttggccagactggtctcaaactctggacctcaggtgatccacctgcctcagcctcccaaagtgtagggattacaggtgtgagccaccgcgcccagcctatgtttctattttatacatattcaacaaacatgattccccaacttctgcaaaataatttctttttcaagaacattgattttagagctcacactaagaaaaagaatacaaaaataatggcatagaaagtgaaaaaacaaaaataaaaagtagaaagctaaagtttcccattaaaatgatcaatatactgtgcagtaagtcaaatgtgtacaatgaattaagaaaatatgatatataaaaatccaaatttacaaaattaagtacaaataggtgtttatattacaaagtgatactggtttataaaaggattcaacatagattttttttaaatggttgttttcctcaatcaatttaacaatgattttaaatgtataaaattttaatatctctttgagacagtgatccaagcttcttcccttgatgatgttaccagttcatactttgtttcaataacctgtccctccacagaaagtaggtgcagtctcttcaccaatacactaagaagtactgtggtcaccatatatgcaaacctcaactctggacactcctgtgtgcctgagaatccaagtgaggaaaaagttttcattactaattcatcatcaaaccgatctggatcaaacttgtgtggagatggccaagtattaggatcctgaagtaccacaccaagggcataaaggacgagggtctctctaggaataataaatcggtcaatttttccttcaatatcttgaagctgggcagaaactggagtcagtttggcagttcgaacagtttcacaaagcacatgctgacaatatctgagctgctcaattttctctggagtaacaggaccatttccaaaaacttggtttatctcttcatataattttttttgaacttcttcagaggtggttaaaaaacagattgcccaggtacacaattttgcagttattatgcaactggccagagaaaatatcatactgtcttctaggatctgttggtcattaaggttcccttgtactaaggagtcaatgaaaatatgttgactgaagttccttccttttcgttcttttatgatgttccttaaaacagactccagttgcatgagggcatcttcatattgttttttccgagtcatgtttttatcaagtgacccatctagaaagccttttccaatctcagaccaaactgtgccatgattcttctggaagcgaatgacttcctgatcatcttcaaatgtactacccattaccatctgtgtaacagacttcatagcaaaaccaagcatatgctggctgaggggcacgtgctgggtctctgggtaggagagccatttatctaataattcttctgaaagctttaggaggagggcaaagttactcttcagagaatcagtcacaccattttcatacaattttttcctcatgtggttttcactcacactgccaccaccagattgataccttaataatgacttcagcatggtttcaaaagggtccgatgtcttattgggattgatatgctgcttcagtacatcaacagtgcccaaactaaccacgaggcgcctgccaaaccagaaggagaccacaggcccatatctctcatgcaaattaaccaggaactcatgcaaacttccactattcacaatatctggaagattaccatctttttcttcagttggagtaatccctggaattcctgcagcttgtctggaagccggatagaggtagagcacggctcccaccaacgccagcaagaaggtaacggcgaagatcgcgaagtccaacatggttctgccgcccagggagccacgtctcggatcggccgctccagc

SEQ ID NO: 12064 - RNA, 2591 nt, Homo sapiens
  source 1..2591: mol_type = other RNA
ctgaatagctgggactacaggtgtgtgtcaccatgcccagtaatttttttgtatatttgtagaggcagggtctcccaatgttgcctgggctggtctcaaactcctgggctcaagcaatccaccagctttggccttccaaagttctaggattatacgcatgagccactgtgccctgccccaatattttgttacttactagtgagactaaacacttttctaaaagtttgttagccatactatcctataaaagctgtttgttcatgtcttttgtccatttatctttttttttgtttttcttgagacagagtcttgctctgtggcccaggctggagtgcaggggtgcaatctcggctcactgcaagctccgcctcccaggttcaaatgattctcctgcctcagcctcctgagtagctgggattacaggcatgtgccaccatgcccagctaatttttttgtgtgtgtttttcagtagagatggggtttcaccatgttggccaggctgatctcgaattcctgacctcaggtgctccacccgcctcagcctcccaaagtactgggattacaggggtgagccaccgcacccggccaattttctgtatttttaatagagacagggtttcatcctgttggccaggctggcctcgaacttcggacctcaggtgatccacccgcctcgacctcccaaagtgctgggattacaggtgtgggccaccacacccagccaatttttttgtatttttagtagagacagggtttcatcatgttggccaggctggtcgcaaactcctgacctcaggtgatccacccgcctcagcatcccaaagtgctgggattacaggcatgagccaccactcccggccaatgttttgtatttttagtagagatggggtttcatcatgttggccagactggtctcaaactctggacctcaggtgatccacctgcctcagcctcccaaagtgtagggattacaggtgtgagccaccgcgcccagcctatgtttctattttatacatattcaacaaacatgattccccaacttctgcaaaataatttctttttcaagaacattgattttagagctcacactaagaaaaagaatacaaaaataatggcatagaaagtgaaaaaacaaaaataaaaagtagaaagctaaagtttcccattaaaatgatcaatatactgtgcagtaagtcaaatgtgtacaatgaattaagaaaatatgatatataaaaatccaaatttacaaaattaagtacaaataggtgtttatattacaaagtgatactggtttataaaaggattcaacatagattttttttaaatggttgttttcctcaatcaatttaacaatgattttaaatgtataaaattttaatatctctttgagacagtgatccaagcttcttcccttgatgatgttaccagttcatactttgtttcaataacctgtccctccacagaaagtaggtgcagtctcttcaccaatacactaagaagtactgtggtcaccatatatgcaaacctcaactctggacactcctgtgtgcctgagaatccaagtgaggaaaaagttttcattactaattcatcatcaaaccgatctggatcaaacttgtgtggagatggccaagtattaggatcctgaagtaccacaccaagggcataaaggacgagggtctctctaggaataataaatcggtcaatttttccttcaatatcttgaagctgggcagaaactggagtcagtttggcagttcgaacagtttcacaaagcacatgctgacaatatctgagctgctcaattttctctggagtaacaggaccatttccaaaaacttggtttatctcttcatataattttttttgaacttcttcagaggtggttaaaaaacagattgcccaggtacacaattttgcagttattatgcaactggccagagaaaatatcatactgtcttctaggatctgttggtcattaaggttcccttgtactaaggagtcaatgaaaatatgttgactgaagttccttccttttcgttcttttatgatgttccttaaaacagactccagttgcatgagggcatcttcatattgttttttccgagtcatgtttttatcaagtgacccatctagaaagccttttccaatctcagaccaaactgtgccatgattcttctggaagcgaatgacttcctgatcatcttcaaatgtactacccattaccatctgtgtaacagacttcatagcaaaaccaagcatatgctggctgaggggcacgtgctgggtctctgggtaggagagccatttatctaataattcttctgaaagctttaggaggagggcaaagttactcttcagagaatcagtcacaccattttcatacaattttttcctcatgtggttttcactcacactgccaccaccagattgataccttaataatgacttcagcatggtttcaaaagggtccgcggatagaggtagagcacggctcccaccaacgccagcaagaaggtaacggcgaagatcgcgaagtccaacatggttctgccgcccagggagccacgtctcggatcggccgctccagc

SEQ ID NO: 12065 - RNA, 3360 nt, Homo sapiens
  source 1..3360: mol_type = other RNA
ctgaatagctgggactacaggtgtgtgtcaccatgcccagtaatttttttgtatatttgtagaggcagggtctcccaatgttgcctgggctggtctcaaactcctgggctcaagcaatccaccagctttggccttccaaagttctaggattatacgcatgagccactgtgccctgccccaatattttgttacttactagtgagactaaacacttttctaaaagtttgttagccatactatcctataaaagctgtttgttcatgtcttttgtccatttatctttttttttgtttttcttgagacagagtcttgctctgtggcccaggctggagtgcaggggtgcaatctcggctcactgcaagctccgcctcccaggttcaaatgattctcctgcctcagcctcctgagtagctgggattacaggcatgtgccaccatgcccagctaatttttttgtgtgtgtttttcagtagagatggggtttcaccatgttggccaggctgatctcgaattcctgacctcaggtgctccacccgcctcagcctcccaaagtactgggattacaggggtgagccaccgcacccggccaattttctgtatttttaatagagacagggtttcatcctgttggccaggctggcctcgaacttcggacctcaggtgatccacccgcctcgacctcccaaagtgctgggattacaggtgtgggccaccacacccagccaatttttttgtatttttagtagagacagggtttcatcatgttggccaggctggtcgcaaactcctgacctcaggtgatccacccgcctcagcatcccaaagtgctgggattacaggcatgagccaccactcccggccaatgttttgtatttttagtagagatggggtttcatcatgttggccagactggtctcaaactctggacctcaggtgatccacctgcctcagcctcccaaagtgtagggattacaggtgtgagccaccgcgcccagcctatgtttctattttatacatattcaacaaacatgattccccaacttctgcaaaataatttctttttcaagaacattgattttagagctcacactaagaaaaagaatacaaaaataatggcatagaaagtgaaaaaacaaaaataaaaagtagaaagctaaagtttcccattaaaatgatcaatatactgtgcagtaagtcaaatgtgtacaatgaattaagaaaatatgatatataaaaatccaaatttacaaaattaagtacaaataggtgtttatattacaaagtgatactggtttataaaaggattcaacatagattttttttaaatggttgttttcctcaatcaatttaacaatgattttaaatgtataaaattttaatatctctttgagacagtgatccaagcttcttcccttgatgatgttaccagttcatactttgtttcaataacctgtccctccacagaaagtaggtgcagtctcttcaccaatacactaagaagtactgtggtcaccatatatgcaaacctcaactctggacactcctgtgtgcctgagaatccaagtgaggaaaaagttttcattactaattcatcatcaaaccgatctggatcaaacttgtgtggagatggccaagtattaggatcctgaagtaccacaccaagggcataaaggacgagggtctctctaggaataataaatcggtcaatttttccttcaatatcttgaagctgggcagaaactggagtcagtttggcagttcgaacagtttcacaaagcacatgctgacaatatctgagctgctcaattttctctggagtaacaggaccatttccaaaaacttggtttatctcttcatataattttttttgaacttcttcagaggtggttaaaaaacagattgcccaggtacacaattttgcagttattatgcaactggccagagaaaatatcatactgtcttctaggatctgttggtcattaaggttcccttgtactaaggagtcaatgaaaatatgttgactgaagttccttccttttcgttcttttatgatgttccttaaaacagactccagttgcatgagggcatcttcatattgttttttccgagtcatgtttttatcaagtgacccatctagaaagccttttccaatctcagaccaaactgtgccatgattcttctggaagcgaatgacttcctgatcatcttcaaatgtactacccattaccatctgtgtaacagacttcatagcaaaaccaagcatatgctggctgaggggcacgtgctgggtctctgggtaggagagccatttatctaataattcttctgaaagctttaggaggagggcaaagttactcttcagagaatcagtcacaccattttcatacaattttttcctcatgtggttttcactcacactgccaccaccagattgataccttaataatgacttcagcatggtttcaaaagggtccgctgctcggaaaagaacatttaagaaggtgtatggtcaattccagcagttcagctacttttcaactttcactgtaaaaccaccaccttgctttgtagaacaggtgttttttgtttgtttgtttgtttgttttgagataagagtctggctctgtcgccaggctgcagtgcagtggtgcgatcttggctcactgcaagctccgcctcccaggttcaagcgattctcctgcctcagcctcctgagtagctgggattacaggcgcccgccaccacagccagctaatgtttgtatttttagtagagacggtgtgtcaccatgttggccaggatggtctcgatatcctgacctcgtgatccgcccgcctcagcctcccaaagtgtgtagaacaggttttaaagacggtcctcagtcatcaacacttttgttttcagaccctccctctctcgctgacggaggcaagtggagagaggaggaccggaggctcgcagaggcgtcagcggcagaggaaacctcgcacccgaacccgcagcgcggcgctctccccaaagaagcatttgcctggagcccctaagaggagcaagacctggacctcgagcactttggattccagtcaggatagatcgatggacagatggaaaagaggaatacacaagtgctgggagaatcctcaagaaaggagaaaggagtggcgcgcccaggagtctcgtcctgacacactgggaaatgaaatttgggtttggcgagttatggccaaaaagctgcccaaagtacttgagagccgccttggagagtggcgcggggtgcctggcaaggtgagaccggcctgcgggggcgcgggcttttcctcagcagctctacgcccgcctggcccggcgcctgaggggtagc

SEQ ID NO: 12066 - RNA, 2641 nt, Homo sapiens
  source 1..2641: mol_type = other RNA
ctgaatagctgggactacaggtgtgtgtcaccatgcccagtaatttttttgtatatttgtagaggcagggtctcccaatgttgcctgggctggtctcaaactcctgggctcaagcaatccaccagctttggccttccaaagttctaggattatacgcatgagccactgtgccctgccccaatattttgttacttactagtgagactaaacacttttctaaaagtttgttagccatactatcctataaaagctgtttgttcatgtcttttgtccatttatctttttttttgtttttcttgagacagagtcttgctctgtggcccaggctggagtgcaggggtgcaatctcggctcactgcaagctccgcctcccaggttcaaatgattctcctgcctcagcctcctgagtagctgggattacaggcatgtgccaccatgcccagctaatttttttgtgtgtgtttttcagtagagatggggtttcaccatgttggccaggctgatctcgaattcctgacctcaggtgctccacccgcctcagcctcccaaagtactgggattacaggggtgagccaccgcacccggccaattttctgtatttttaatagagacagggtttcatcctgttggccaggctggcctcgaacttcggacctcaggtgatccacccgcctcgacctcccaaagtgctgggattacaggtgtgggccaccacacccagccaatttttttgtatttttagtagagacagggtttcatcatgttggccaggctggtcgcaaactcctgacctcaggtgatccacccgcctcagcatcccaaagtgctgggattacaggcatgagccaccactcccggccaatgttttgtatttttagtagagatggggtttcatcatgttggccagactggtctcaaactctggacctcaggtgatccacctgcctcagcctcccaaagtgtagggattacaggtgtgagccaccgcgcccagcctatgtttctattttatacatattcaacaaacatgattccccaacttctgcaaaataatttctttttcaagaacattgattttagagctcacactaagaaaaagaatacaaaaataatggcatagaaagtgaaaaaacaaaaataaaaagtagaaagctaaagtttcccattaaaatgatcaatatactgtgcagtaagtcaaatgtgtacaatgaattaagaaaatatgatatataaaaatccaaatttacaaaattaagtacaaataggtgtttatattacaaagtgatactggtttataaaaggattcaacatagattttttttaaatggttgttttcctcaatcaatttaacaatgattttaaatgtataaaattttaatatctctttgagacagtgatccaagcttcttcccttgatgatgttaccagttcatactttgtttcaataacctgtccctccacagaaagtaggtgcagtctcttcaccaatacactaagaagtactgtggtcaccatatatgcaaacctcaactctggacactcctgtgtgcctgagaatccaagtgaggaaaaagttttcattactaattcatcatcaaaccgatctggatcaaacttgtgtggagatggccaagtattaggatcctgaagtaccacaccaagggcataaaggacgagggtctctctaggaataataaatcggtcaatttttccttcaatatcttgaagctgggcagaaactggagtcagtttggcagttcgaacagtttcacaaagcacatgctgacaatatctgagctgctcaattttctctggagtaacaggaccatttccaaaaacttggtttatctcttcatataattttttttgaacttcttcagaggtggttaaaaaacagattgcccaggtacacaattttgcagttattatgcaactggccagagaaaatatcatactgtcttctaggatctgttggtcattaaggttcccttgtactaaggagtcaatgaaaatatgttgactgaagttccttccttttcgttcttttatgatgttccttaaaacagactccagttgcatgagggcatcttcatattgttttttccgagtcatgtttttatcaagtgacccatctagaaagccttttccaatctcagaccaaactgtgccatgattcttctggaagcgaatgacttcctgatcatcttcaaatgtactacccattaccatctgtgtaacagacttcatagcaaaaccaagcatatgctggctgaggggcacgtgctgggtctctgggtaggagagccatttatctaataattcttctgaaagctttaggaggagggcaaagttactcttcagagaatcagtcacaccattttcatacaattttttcctcatgtggttttcactcacactgccaccaccagattgataccttaataatgacttcagcatggtttcaaaagggtccgttttcttcagttggagtaatccctggaattcctgcagcttgtctggaagccggatagaggtagagcacggctcccaccaacgccagcaagaaggtaacggcgaagatcgcgaagtccaacatggttctgccgcccagggagccacgtctcggatcggccgctccagc

SEQ ID NO: 12067 - RNA, 2456 nt, Homo sapiens
  source 1..2456: mol_type = other RNA
ctgaatagctgggactacaggtgtgtgtcaccatgcccagtaatttttttgtatatttgtagaggcagggtctcccaatgttgcctgggctggtctcaaactcctgggctcaagcaatccaccagctttggccttccaaagttctaggattatacgcatgagccactgtgccctgccccaatattttgttacttactagtgagactaaacacttttctaaaagtttgttagccatactatcctataaaagctgtttgttcatgtcttttgtccatttatctttttttttgtttttcttgagacagagtcttgctctgtggcccaggctggagtgcaggggtgcaatctcggctcactgcaagctccgcctcccaggttcaaatgattctcctgcctcagcctcctgagtagctgggattacaggcatgtgccaccatgcccagctaatttttttgtgtgtgtttttcagtagagatggggtttcaccatgttggccaggctgatctcgaattcctgacctcaggtgctccacccgcctcagcctcccaaagtactgggattacaggggtgagccaccgcacccggccaattttctgtatttttaatagagacagggtttcatcctgttggccaggctggcctcgaacttcggacctcaggtgatccacccgcctcgacctcccaaagtgctgggattacaggtgtgggccaccacacccagccaatttttttgtatttttagtagagacagggtttcatcatgttggccaggctggtcgcaaactcctgacctcaggtgatccacccgcctcagcatcccaaagtgctgggattacaggcatgagccaccactcccggccaatgttttgtatttttagtagagatggggtttcatcatgttggccagactggtctcaaactctggacctcaggtgatccacctgcctcagcctcccaaagtgtagggattacaggtgtgagccaccgcgcccagcctatgtttctattttatacatattcaacaaacatgattccccaacttctgcaaaataatttctttttcaagaacattgattttagagctcacactaagaaaaagaatacaaaaataatggcatagaaagtgaaaaaacaaaaataaaaagtagaaagctaaagtttcccattaaaatgatcaatatactgtgcagtaagtcaaatgtgtacaatgaattaagaaaatatgatatataaaaatccaaatttacaaaattaagtacaaataggtgtttatattacaaagtgatactggtttataaaaggattcaacatagattttttttaaatggttgttttcctcaatcaatttaacaatgattttaaatgtataaaattttaatatctctttgagacagtgatccaagcttcttcccttgatgatgttaccagttcatactttgtttcaataacctgtccctccacagaaagtaggtgcagtctcttcaccaatacactaagaagtactgtggtcaccatatatgcaaacctcaactctggacactcctgtgtgcctgagaatccaagtgaggaaaaagttttcattactaattcatcatcaaaccgatctggatcaaacttgtgtggagatggccaagtattaggatcctgaagtaccacaccaagggcataaaggacgagggtctctctaggaataataaatcggtcaatttttccttcaatatcttgaagctgggcagaaactggagtcagtttggcagttcgaacagtttcacaaagcacatgctgacaatatctgagctgctcaattttctctggagtaacaggaccatttccaaaaacttggtttatctcttcatataattttttttgaacttcttcagaggtggttaaaaaacagattgcccaggtacacaattttgcagttattatgcaactggccagagaaaatatcatactgtcttctaggatctgttggtcattaaggttcccttgtactaaggagtcaatgaaaatatgttgactgaagttccttccttttcgttcttttatgatgttccttaaaacagactccagttgcatgagggtgtgccatgattcttctggaagcgaatgacttcctgatcatcttcaaatgtactacccattaccatctgtgtaacagacttcatagcaaaaccaagcatatgctggctgaggggcacgtgctgggtctctgggtaggagagccatttatctaataattcttctgaaagcttaataatgacttcagcatggtttcaaaagggtccgttttcttcagttggagtaatccctggaattcctgcagcttgtctggaagccggatagaggtagagcacggctcccaccaacgccagcaagaaggtaacggcgaagatcgcgaagtccaacatggttctgccgcccagggagccacgtctcggatcggccgctccagc

SEQ ID NO: 12068 - RNA, 2729 nt, Homo sapiens
  source 1..2729: mol_type = other RNA
ctgaatagctgggactacaggtgtgtgtcaccatgcccagtaatttttttgtatatttgtagaggcagggtctcccaatgttgcctgggctggtctcaaactcctgggctcaagcaatccaccagctttggccttccaaagttctaggattatacgcatgagccactgtgccctgccccaatattttgttacttactagtgagactaaacacttttctaaaagtttgttagccatactatcctataaaagctgtttgttcatgtcttttgtccatttatctttttttttgtttttcttgagacagagtcttgctctgtggcccaggctggagtgcaggggtgcaatctcggctcactgcaagctccgcctcccaggttcaaatgattctcctgcctcagcctcctgagtagctgggattacaggcatgtgccaccatgcccagctaatttttttgtgtgtgtttttcagtagagatggggtttcaccatgttggccaggctgatctcgaattcctgacctcaggtgctccacccgcctcagcctcccaaagtactgggattacaggggtgagccaccgcacccggccaattttctgtatttttaatagagacagggtttcatcctgttggccaggctggcctcgaacttcggacctcaggtgatccacccgcctcgacctcccaaagtgctgggattacaggtgtgggccaccacacccagccaatttttttgtatttttagtagagacagggtttcatcatgttggccaggctggtcgcaaactcctgacctcaggtgatccacccgcctcagcatcccaaagtgctgggattacaggcatgagccaccactcccggccaatgttttgtatttttagtagagatggggtttcatcatgttggccagactggtctcaaactctggacctcaggtgatccacctgcctcagcctcccaaagtgtagggattacaggtgtgagccaccgcgcccagcctatgtttctattttatacatattcaacaaacatgattccccaacttctgcaaaataatttctttttcaagaacattgattttagagctcacactaagaaaaagaatacaaaaataatggcatagaaagtgaaaaaacaaaaataaaaagtagaaagctaaagtttcccattaaaatgatcaatatactgtgcagtaagtcaaatgtgtacaatgaattaagaaaatatgatatataaaaatccaaatttacaaaattaagtacaaataggtgtttatattacaaagtgatactggtttataaaaggattcaacatagattttttttaaatggttgttttcctcaatcaatttaacaatgattttaaatgtataaaattttaatatctctttgagacagtgatccaagcttcttcccttgatgatgttaccagttcatactttgtttcaataacctgtccctccacagaaagtaggtgcagtctcttcaccaatacactaagaagtactgtggtcaccatatatgcaaacctcaactctggacactcctgtgtgcctgagaatccaagtgaggaaaaagttttcattactaattcatcatcaaaccgatctggatcaaacttgtgtggagatggccaagtattaggatcctgaagtaccacaccaagggcataaaggacgagggtctctctaggaataataaatcggtcaatttttccttcaatatcttgaagctgggcagaaactggagtcagtttggcagttcgaacagtttcacaaagcacatgctgacaatatctgagctgctcaattttctctggagtaacaggaccatttccaaaaacttggtttatctcttcatataattttttttgaacttcttcagaggtggttaaaaaacagattgcccaggtacacaattttgcagttattatgcaactggccagagaaaatatcatactgtcttctaggatctgttggtcattaaggttcccttgtactaaggagtcaatgaaaatatgttgactgaagttccttccttttcgttcttttatgatgttccttaaaacagactccagttgcatgagggtgtgccatgattcttctggaagcgaatgacttcctgatcatcttcaaatgtactacccattaccatctgtgtaacagacttcatagcaaaaccaagcatatgctggctgaggggcacgtgctgggtctctgggtaggagagccatttatctaataattcttctgaaagctttaggaggagggcaaagttactcttcagagaatcagtcacaccattttcatacaattttttcctcatgtggttttcactcacactgccaccaccagattgataccttaataatgacttcagcatggtttcaaaagggtccgatgtcttattgggattgatatgctgcttcagtacatcaacagtgcccaaactaaccacgaggcgcctgccaaaccagaaggagaccacaggcccatatctctcatgcaaattaaccaggaactcatgcaaacttccactattcacaatatctggaagattaccatctttttcttcagttggagtaatccctggaattcctgcagcttgtctggaagccggatagaggtagagcacggctcccaccaacgccagcaagaaggtaacggcgaagatcgcgaagtccaacatggttctgccgcccagggagccacgtctcggatcggccgctccagc

SEQ ID NO: 12069 - RNA, 2512 nt, Homo sapiens
  source 1..2512: mol_type = other RNA
ctgaatagctgggactacaggtgtgtgtcaccatgcccagtaatttttttgtatatttgtagaggcagggtctcccaatgttgcctgggctggtctcaaactcctgggctcaagcaatccaccagctttggccttccaaagttctaggattatacgcatgagccactgtgccctgccccaatattttgttacttactagtgagactaaacacttttctaaaagtttgttagccatactatcctataaaagctgtttgttcatgtcttttgtccatttatctttttttttgtttttcttgagacagagtcttgctctgtggcccaggctggagtgcaggggtgcaatctcggctcactgcaagctccgcctcccaggttcaaatgattctcctgcctcagcctcctgagtagctgggattacaggcatgtgccaccatgcccagctaatttttttgtgtgtgtttttcagtagagatggggtttcaccatgttggccaggctgatctcgaattcctgacctcaggtgctccacccgcctcagcctcccaaagtactgggattacaggggtgagccaccgcacccggccaattttctgtatttttaatagagacagggtttcatcctgttggccaggctggcctcgaacttcggacctcaggtgatccacccgcctcgacctcccaaagtgctgggattacaggtgtgggccaccacacccagccaatttttttgtatttttagtagagacagggtttcatcatgttggccaggctggtcgcaaactcctgacctcaggtgatccacccgcctcagcatcccaaagtgctgggattacaggcatgagccaccactcccggccaatgttttgtatttttagtagagatggggtttcatcatgttggccagactggtctcaaactctggacctcaggtgatccacctgcctcagcctcccaaagtgtagggattacaggtgtgagccaccgcgcccagcctatgtttctattttatacatattcaacaaacatgattccccaacttctgcaaaataatttctttttcaagaacattgattttagagctcacactaagaaaaagaatacaaaaataatggcatagaaagtgaaaaaacaaaaataaaaagtagaaagctaaagtttcccattaaaatgatcaatatactgtgcagtaagtcaaatgtgtacaatgaattaagaaaatatgatatataaaaatccaaatttacaaaattaagtacaaataggtgtttatattacaaagtgatactggtttataaaaggattcaacatagattttttttaaatggttgttttcctcaatcaatttaacaatgattttaaatgtataaaattttaatatctctttgagacagtgatccaagcttcttcccttgatgatgttaccagttcatactttgtttcaataacctgtccctccacagaaagtaggtgcagtctcttcaccaatacactaagaagtactgtggtcaccatatatgcaaacctcaactctggacactcctgtgtgcctgagaatccaagtgaggaaaaagttttcattactaattcatcatcaaaccgatctggatcaaacttgtgtggagatggccaagtattaggatcctgaagtaccacaccaagggcataaaggacgagggtctctctaggaataataaatcggtcaatttttccttcaatatcttgaagctgggcagaaactggagtcagtttggcagttcgaacagtttcacaaagcacatgctgacaatatctgagctgctcaattttctctggagtaacaggaccatttccaaaaacttggtttatctcttcatataattttttttgaacttcttcagaggtggttaaaaaacagattgcccaggtacacaattttgcagttattatgcaactggccagagaaaatatcatactgtcttctaggatctgttggtcattaaggttcccttgtactaaggagtcaatgaaaatatgttgactgaagttccttccttttcgttcttttatgatgttccttaaaacagactccagttgcatgagggtgtgccatgattcttctggaagcgaatgacttcctgatcatcttcaaatgtactacccattaccatctgtgtaacagacttcatagcaaaaccaagcatatgctggctgaggggcacgtgctgggtctctgggtaggagagccatttatctaataattcttctgaaagctttaggaggagggcaaagttactcttcagagaatcagtcacaccattttcatacaattttttcctcatgtggttttcactcacactgccaccaccagattgataccttaataatgacttcagcatggtttcaaaagggtccgcggatagaggtagagcacggctcccaccaacgccagcaagaaggtaacggcgaagatcgcgaagtccaacatggttctgccgcccagggagccacgtctcggatcggccgctccagc

SEQ ID NO: 12070 - RNA, 3281 nt, Homo sapiens
  source 1..3281: mol_type = other RNA
ctgaatagctgggactacaggtgtgtgtcaccatgcccagtaatttttttgtatatttgtagaggcagggtctcccaatgttgcctgggctggtctcaaactcctgggctcaagcaatccaccagctttggccttccaaagttctaggattatacgcatgagccactgtgccctgccccaatattttgttacttactagtgagactaaacacttttctaaaagtttgttagccatactatcctataaaagctgtttgttcatgtcttttgtccatttatctttttttttgtttttcttgagacagagtcttgctctgtggcccaggctggagtgcaggggtgcaatctcggctcactgcaagctccgcctcccaggttcaaatgattctcctgcctcagcctcctgagtagctgggattacaggcatgtgccaccatgcccagctaatttttttgtgtgtgtttttcagtagagatggggtttcaccatgttggccaggctgatctcgaattcctgacctcaggtgctccacccgcctcagcctcccaaagtactgggattacaggggtgagccaccgcacccggccaattttctgtatttttaatagagacagggtttcatcctgttggccaggctggcctcgaacttcggacctcaggtgatccacccgcctcgacctcccaaagtgctgggattacaggtgtgggccaccacacccagccaatttttttgtatttttagtagagacagggtttcatcatgttggccaggctggtcgcaaactcctgacctcaggtgatccacccgcctcagcatcccaaagtgctgggattacaggcatgagccaccactcccggccaatgttttgtatttttagtagagatggggtttcatcatgttggccagactggtctcaaactctggacctcaggtgatccacctgcctcagcctcccaaagtgtagggattacaggtgtgagccaccgcgcccagcctatgtttctattttatacatattcaacaaacatgattccccaacttctgcaaaataatttctttttcaagaacattgattttagagctcacactaagaaaaagaatacaaaaataatggcatagaaagtgaaaaaacaaaaataaaaagtagaaagctaaagtttcccattaaaatgatcaatatactgtgcagtaagtcaaatgtgtacaatgaattaagaaaatatgatatataaaaatccaaatttacaaaattaagtacaaataggtgtttatattacaaagtgatactggtttataaaaggattcaacatagattttttttaaatggttgttttcctcaatcaatttaacaatgattttaaatgtataaaattttaatatctctttgagacagtgatccaagcttcttcccttgatgatgttaccagttcatactttgtttcaataacctgtccctccacagaaagtaggtgcagtctcttcaccaatacactaagaagtactgtggtcaccatatatgcaaacctcaactctggacactcctgtgtgcctgagaatccaagtgaggaaaaagttttcattactaattcatcatcaaaccgatctggatcaaacttgtgtggagatggccaagtattaggatcctgaagtaccacaccaagggcataaaggacgagggtctctctaggaataataaatcggtcaatttttccttcaatatcttgaagctgggcagaaactggagtcagtttggcagttcgaacagtttcacaaagcacatgctgacaatatctgagctgctcaattttctctggagtaacaggaccatttccaaaaacttggtttatctcttcatataattttttttgaacttcttcagaggtggttaaaaaacagattgcccaggtacacaattttgcagttattatgcaactggccagagaaaatatcatactgtcttctaggatctgttggtcattaaggttcccttgtactaaggagtcaatgaaaatatgttgactgaagttccttccttttcgttcttttatgatgttccttaaaacagactccagttgcatgagggtgtgccatgattcttctggaagcgaatgacttcctgatcatcttcaaatgtactacccattaccatctgtgtaacagacttcatagcaaaaccaagcatatgctggctgaggggcacgtgctgggtctctgggtaggagagccatttatctaataattcttctgaaagctttaggaggagggcaaagttactcttcagagaatcagtcacaccattttcatacaattttttcctcatgtggttttcactcacactgccaccaccagattgataccttaataatgacttcagcatggtttcaaaagggtccgctgctcggaaaagaacatttaagaaggtgtatggtcaattccagcagttcagctacttttcaactttcactgtaaaaccaccaccttgctttgtagaacaggtgttttttgtttgtttgtttgtttgttttgagataagagtctggctctgtcgccaggctgcagtgcagtggtgcgatcttggctcactgcaagctccgcctcccaggttcaagcgattctcctgcctcagcctcctgagtagctgggattacaggcgcccgccaccacagccagctaatgtttgtatttttagtagagacggtgtgtcaccatgttggccaggatggtctcgatatcctgacctcgtgatccgcccgcctcagcctcccaaagtgtgtagaacaggttttaaagacggtcctcagtcatcaacacttttgttttcagaccctccctctctcgctgacggaggcaagtggagagaggaggaccggaggctcgcagaggcgtcagcggcagaggaaacctcgcacccgaacccgcagcgcggcgctctccccaaagaagcatttgcctggagcccctaagaggagcaagacctggacctcgagcactttggattccagtcaggatagatcgatggacagatggaaaagaggaatacacaagtgctgggagaatcctcaagaaaggagaaaggagtggcgcgcccaggagtctcgtcctgacacactgggaaatgaaatttgggtttggcgagttatggccaaaaagctgcccaaagtacttgagagccgccttggagagtggcgcggggtgcctggcaaggtgagaccggcctgcgggggcgcgggcttttcctcagcagctctacgcccgcctggcccggcgcctgaggggtagc

SEQ ID NO: 12071 - RNA, 2562 nt, Homo sapiens
  source 1..2562: mol_type = other RNA
ctgaatagctgggactacaggtgtgtgtcaccatgcccagtaatttttttgtatatttgtagaggcagggtctcccaatgttgcctgggctggtctcaaactcctgggctcaagcaatccaccagctttggccttccaaagttctaggattatacgcatgagccactgtgccctgccccaatattttgttacttactagtgagactaaacacttttctaaaagtttgttagccatactatcctataaaagctgtttgttcatgtcttttgtccatttatctttttttttgtttttcttgagacagagtcttgctctgtggcccaggctggagtgcaggggtgcaatctcggctcactgcaagctccgcctcccaggttcaaatgattctcctgcctcagcctcctgagtagctgggattacaggcatgtgccaccatgcccagctaatttttttgtgtgtgtttttcagtagagatggggtttcaccatgttggccaggctgatctcgaattcctgacctcaggtgctccacccgcctcagcctcccaaagtactgggattacaggggtgagccaccgcacccggccaattttctgtatttttaatagagacagggtttcatcctgttggccaggctggcctcgaacttcggacctcaggtgatccacccgcctcgacctcccaaagtgctgggattacaggtgtgggccaccacacccagccaatttttttgtatttttagtagagacagggtttcatcatgttggccaggctggtcgcaaactcctgacctcaggtgatccacccgcctcagcatcccaaagtgctgggattacaggcatgagccaccactcccggccaatgttttgtatttttagtagagatggggtttcatcatgttggccagactggtctcaaactctggacctcaggtgatccacctgcctcagcctcccaaagtgtagggattacaggtgtgagccaccgcgcccagcctatgtttctattttatacatattcaacaaacatgattccccaacttctgcaaaataatttctttttcaagaacattgattttagagctcacactaagaaaaagaatacaaaaataatggcatagaaagtgaaaaaacaaaaataaaaagtagaaagctaaagtttcccattaaaatgatcaatatactgtgcagtaagtcaaatgtgtacaatgaattaagaaaatatgatatataaaaatccaaatttacaaaattaagtacaaataggtgtttatattacaaagtgatactggtttataaaaggattcaacatagattttttttaaatggttgttttcctcaatcaatttaacaatgattttaaatgtataaaattttaatatctctttgagacagtgatccaagcttcttcccttgatgatgttaccagttcatactttgtttcaataacctgtccctccacagaaagtaggtgcagtctcttcaccaatacactaagaagtactgtggtcaccatatatgcaaacctcaactctggacactcctgtgtgcctgagaatccaagtgaggaaaaagttttcattactaattcatcatcaaaccgatctggatcaaacttgtgtggagatggccaagtattaggatcctgaagtaccacaccaagggcataaaggacgagggtctctctaggaataataaatcggtcaatttttccttcaatatcttgaagctgggcagaaactggagtcagtttggcagttcgaacagtttcacaaagcacatgctgacaatatctgagctgctcaattttctctggagtaacaggaccatttccaaaaacttggtttatctcttcatataattttttttgaacttcttcagaggtggttaaaaaacagattgcccaggtacacaattttgcagttattatgcaactggccagagaaaatatcatactgtcttctaggatctgttggtcattaaggttcccttgtactaaggagtcaatgaaaatatgttgactgaagttccttccttttcgttcttttatgatgttccttaaaacagactccagttgcatgagggtgtgccatgattcttctggaagcgaatgacttcctgatcatcttcaaatgtactacccattaccatctgtgtaacagacttcatagcaaaaccaagcatatgctggctgaggggcacgtgctgggtctctgggtaggagagccatttatctaataattcttctgaaagctttaggaggagggcaaagttactcttcagagaatcagtcacaccattttcatacaattttttcctcatgtggttttcactcacactgccaccaccagattgataccttaataatgacttcagcatggtttcaaaagggtccgttttcttcagttggagtaatccctggaattcctgcagcttgtctggaagccggatagaggtagagcacggctcccaccaacgccagcaagaaggtaacggcgaagatcgcgaagtccaacatggttctgccgcccagggagccacgtctcggatcggccgctccagc

SEQ ID NO: 12072 - RNA, 2396 nt, Homo sapiens
  source 1..2396: mol_type = other RNA
ctgaatagctgggactacaggtgtgtgtcaccatgcccagtaatttttttgtatatttgtagaggcagggtctcccaatgttgcctgggctggtctcaaactcctgggctcaagcaatccaccagctttggccttccaaagttctaggattatacgcatgagccactgtgccctgccccaatattttgttacttactagtgagactaaacacttttctaaaagtttgttagccatactatcctataaaagctgtttgttcatgtcttttgtccatttatctttttttttgtttttcttgagacagagtcttgctctgtggcccaggctggagtgcaggggtgcaatctcggctcactgcaagctccgcctcccaggttcaaatgattctcctgcctcagcctcctgagtagctgggattacaggcatgtgccaccatgcccagctaatttttttgtgtgtgtttttcagtagagatggggtttcaccatgttggccaggctgatctcgaattcctgacctcaggtgctccacccgcctcagcctcccaaagtactgggattacaggggtgagccaccgcacccggccaattttctgtatttttaatagagacagggtttcatcctgttggccaggctggcctcgaacttcggacctcaggtgatccacccgcctcgacctcccaaagtgctgggattacaggtgtgggccaccacacccagccaatttttttgtatttttagtagagacagggtttcatcatgttggccaggctggtcgcaaactcctgacctcaggtgatccacccgcctcagcatcccaaagtgctgggattacaggcatgagccaccactcccggccaatgttttgtatttttagtagagatggggtttcatcatgttggccagactggtctcaaactctggacctcaggtgatccacctgcctcagcctcccaaagtgtagggattacaggtgtgagccaccgcgcccagcctatgtttctattttatacatattcaacaaacatgattccccaacttctgcaaaataatttctttttcaagaacattgattttagagctcacactaagaaaaagaatacaaaaataatggcatagaaagtgaaaaaacaaaaataaaaagtagaaagctaaagtttcccattaaaatgatcaatatactgtgcagtaagtcaaatgtgtacaatgaattaagaaaatatgatatataaaaatccaaatttacaaaattaagtacaaataggtgtttatattacaaagtgatactggtttataaaaggattcaacatagattttttttaaatggttgttttcctcaatcaatttaacaatgattttaaatgtataaaattttaatatctctttgagacagtgatccaagcttcttcccttgatgatgttaccagttcatactttgtttcaataacctgtccctccacagaaagtaggtgcagtctcttcaccaatacactaagaagtactgtggtcaccatatatgcaaacctcaactctggacactcctgtgtgcctgagaatccaagtgaggaaaaagttttcattactaattcatcatcaaaccgatctggatcaaacttgtgtggagatggccaagtattaggatcctgaagtaccacaccaagggcataaaggacgagggtctctctaggaataataaatcggtcaatttttccttcaatatcttgaagctgggcagaaactggagtcagtttggcagttcgaacagtttcacaaagcacatgctgacaatatctgagctgctcaattttctctggagtaacaggaccatttccaaaaacttggtttatctcttcatataattttttttgaacttcttcagaggtggttaaaaaacagattgcccaggtacacaattttgcagttattatgcaactggccagagaaaatatcatactgtcttctaggattgtgccatgattcttctggaagcgaatgacttcctgatcatcttcaaatgtactacccattaccatctgtgtaacagacttcatagcaaaaccaagcatatgctggctgaggggcacgtgctgggtctctgggtaggagagccatttatctaataattcttctgaaagctttaggaggagggcaaagttactcttcagagaatcagtcacaccattttcatacaattttttcctcatgtggttttcactcacactgccaccaccagattgataccttaataatgacttcagcatggtttcaaaagggtccgcggatagaggtagagcacggctcccaccaacgccagcaagaaggtaacggcgaagatcgcgaagtccaacatggttctgccgcccagggagccacgtctcggatcggccgctccagc

SEQ ID NO: 12073 - RNA, 2446 nt, Homo sapiens
  source 1..2446: mol_type = other RNA
ctgaatagctgggactacaggtgtgtgtcaccatgcccagtaatttttttgtatatttgtagaggcagggtctcccaatgttgcctgggctggtctcaaactcctgggctcaagcaatccaccagctttggccttccaaagttctaggattatacgcatgagccactgtgccctgccccaatattttgttacttactagtgagactaaacacttttctaaaagtttgttagccatactatcctataaaagctgtttgttcatgtcttttgtccatttatctttttttttgtttttcttgagacagagtcttgctctgtggcccaggctggagtgcaggggtgcaatctcggctcactgcaagctccgcctcccaggttcaaatgattctcctgcctcagcctcctgagtagctgggattacaggcatgtgccaccatgcccagctaatttttttgtgtgtgtttttcagtagagatggggtttcaccatgttggccaggctgatctcgaattcctgacctcaggtgctccacccgcctcagcctcccaaagtactgggattacaggggtgagccaccgcacccggccaattttctgtatttttaatagagacagggtttcatcctgttggccaggctggcctcgaacttcggacctcaggtgatccacccgcctcgacctcccaaagtgctgggattacaggtgtgggccaccacacccagccaatttttttgtatttttagtagagacagggtttcatcatgttggccaggctggtcgcaaactcctgacctcaggtgatccacccgcctcagcatcccaaagtgctgggattacaggcatgagccaccactcccggccaatgttttgtatttttagtagagatggggtttcatcatgttggccagactggtctcaaactctggacctcaggtgatccacctgcctcagcctcccaaagtgtagggattacaggtgtgagccaccgcgcccagcctatgtttctattttatacatattcaacaaacatgattccccaacttctgcaaaataatttctttttcaagaacattgattttagagctcacactaagaaaaagaatacaaaaataatggcatagaaagtgaaaaaacaaaaataaaaagtagaaagctaaagtttcccattaaaatgatcaatatactgtgcagtaagtcaaatgtgtacaatgaattaagaaaatatgatatataaaaatccaaatttacaaaattaagtacaaataggtgtttatattacaaagtgatactggtttataaaaggattcaacatagattttttttaaatggttgttttcctcaatcaatttaacaatgattttaaatgtataaaattttaatatctctttgagacagtgatccaagcttcttcccttgatgatgttaccagttcatactttgtttcaataacctgtccctccacagaaagtaggtgcagtctcttcaccaatacactaagaagtactgtggtcaccatatatgcaaacctcaactctggacactcctgtgtgcctgagaatccaagtgaggaaaaagttttcattactaattcatcatcaaaccgatctggatcaaacttgtgtggagatggccaagtattaggatcctgaagtaccacaccaagggcataaaggacgagggtctctctaggaataataaatcggtcaatttttccttcaatatcttgaagctgggcagaaactggagtcagtttggcagttcgaacagtttcacaaagcacatgctgacaatatctgagctgctcaattttctctggagtaacaggaccatttccaaaaacttggtttatctcttcatataattttttttgaacttcttcagaggtggttaaaaaacagattgcccaggtacacaattttgcagttattatgcaactggccagagaaaatatcatactgtcttctaggattgtgccatgattcttctggaagcgaatgacttcctgatcatcttcaaatgtactacccattaccatctgtgtaacagacttcatagcaaaaccaagcatatgctggctgaggggcacgtgctgggtctctgggtaggagagccatttatctaataattcttctgaaagctttaggaggagggcaaagttactcttcagagaatcagtcacaccattttcatacaattttttcctcatgtggttttcactcacactgccaccaccagattgataccttaataatgacttcagcatggtttcaaaagggtccgttttcttcagttggagtaatccctggaattcctgcagcttgtctggaagccggatagaggtagagcacggctcccaccaacgccagcaagaaggtaacggcgaagatcgcgaagtccaacatggttctgccgcccagggagccacgtctcggatcggccgctccagc

SEQ ID NO: 12074 - RNA, 2696 nt, Homo sapiens
  source 1..2696: mol_type = other RNA
ctgaatagctgggactacaggtgtgtgtcaccatgcccagtaatttttttgtatatttgtagaggcagggtctcccaatgttgcctgggctggtctcaaactcctgggctcaagcaatccaccagctttggccttccaaagttctaggattatacgcatgagccactgtgccctgccccaatattttgttacttactagtgagactaaacacttttctaaaagtttgttagccatactatcctataaaagctgtttgttcatgtcttttgtccatttatctttttttttgtttttcttgagacagagtcttgctctgtggcccaggctggagtgcaggggtgcaatctcggctcactgcaagctccgcctcccaggttcaaatgattctcctgcctcagcctcctgagtagctgggattacaggcatgtgccaccatgcccagctaatttttttgtgtgtgtttttcagtagagatggggtttcaccatgttggccaggctgatctcgaattcctgacctcaggtgctccacccgcctcagcctcccaaagtactgggattacaggggtgagccaccgcacccggccaattttctgtatttttaatagagacagggtttcatcctgttggccaggctggcctcgaacttcggacctcaggtgatccacccgcctcgacctcccaaagtgctgggattacaggtgtgggccaccacacccagccaatttttttgtatttttagtagagacagggtttcatcatgttggccaggctggtcgcaaactcctgacctcaggtgatccacccgcctcagcatcccaaagtgctgggattacaggcatgagccaccactcccggccaatgttttgtatttttagtagagatggggtttcatcatgttggccagactggtctcaaactctggacctcaggtgatccacctgcctcagcctcccaaagtgtagggattacaggtgtgagccaccgcgcccagcctatgtttctattttatacatattcaacaaacatgattccccaacttctgcaaaataatttctttttcaagaacattgattttagagctcacactaagaaaaagaatacaaaaataatggcatagaaagtgaaaaaacaaaaataaaaagtagaaagctaaagtttcccattaaaatgatcaatatactgtgcagtaagtcaaatgtgtacaatgaattaagaaaatatgatatataaaaatccaaatttacaaaattaagtacaaataggtgtttatattacaaagtgatactggtttataaaaggattcaacatagattttttttaaatggttgttttcctcaatcaatttaacaatgattttaaatgtataaaattttaatatctctttgagacagtgatccaagcttcttcccttgatgatgttaccagttcatactttgtttcaataacctgtccctccacagaaagtaggtgcagtctcttcaccaatacactaagaagtactgtggtcaccatatatgcaaacctcaactctggacactcctgtgtgcctgagaatccaagtgaggaaaaagttttcattactaattcatcatcaaaccgatctggatcaaacttgtgtggagatggccaagtattaggatcctgaagtaccacaccaagggcataaaggacgagggtctgagctgctcaattttctctggagtaacaggaccatttccaaaaacttggtttatctcttcatataattttttttgaacttcttcagaggtggttaaaaaacagattgcccaggtacacaattttgcagttattatgcaactggccagagaaaatatcatactgtcttctaggatctgttggtcattaaggttcccttgtactaaggagtcaatgaaaatatgttgactgaagttccttccttttcgttcttttatgatgttccttaaaacagactccagttgcatgagggcatcttcatattgttttttccgagtcatgtttttatcaagtgacccatctagaaagccttttccaatctcagaccaaactgtgccatgattcttctggaagcgaatgacttcctgatcatcttcaaatgtactacccattaccatctgtgtaacagacttcatagcaaaaccaagcatatgctggctgaggggcacgtgctgggtctctgggtaggagagccatttatctaataattcttctgaaagctttaggaggagggcaaagttactcttcagagaatcagtcacaccattttcatacaattttttcctcatgtggttttcactcacactgccaccaccagattgataccttaataatgacttcagcatggtttcaaaagggtccgatgtcttattgggattgatatgctgcttcagtacatcaacagtgcccaaactaaccacgaggcgcctgccaaaccagaaggagaccacaggcccatatctctcatgcaaattaaccaggaactcatgcaaacttccactattcacaatatctggaagattaccatctttttcttcagttggagtaatccctggaattcctgcagcttgtctggaagccggatagaggtagagcacggctcccaccaacgccagcaagaaggtaacggcgaagatcgcgaagtccaacatggttctgccgcccagggagccacgtctcggatcggccgctccagc

SEQ ID NO: 12075 - RNA, 2450 nt, Homo sapiens
  source 1..2450: mol_type = other RNA
ctgaatagctgggactacaggtgtgtgtcaccatgcccagtaatttttttgtatatttgtagaggcagggtctcccaatgttgcctgggctggtctcaaactcctgggctcaagcaatccaccagctttggccttccaaagttctaggattatacgcatgagccactgtgccctgccccaatattttgttacttactagtgagactaaacacttttctaaaagtttgttagccatactatcctataaaagctgtttgttcatgtcttttgtccatttatctttttttttgtttttcttgagacagagtcttgctctgtggcccaggctggagtgcaggggtgcaatctcggctcactgcaagctccgcctcccaggttcaaatgattctcctgcctcagcctcctgagtagctgggattacaggcatgtgccaccatgcccagctaatttttttgtgtgtgtttttcagtagagatggggtttcaccatgttggccaggctgatctcgaattcctgacctcaggtgctccacccgcctcagcctcccaaagtactgggattacaggggtgagccaccgcacccggccaattttctgtatttttaatagagacagggtttcatcctgttggccaggctggcctcgaacttcggacctcaggtgatccacccgcctcgacctcccaaagtgctgggattacaggtgtgggccaccacacccagccaatttttttgtatttttagtagagacagggtttcatcatgttggccaggctggtcgcaaactcctgacctcaggtgatccacccgcctcagcatcccaaagtgctgggattacaggcatgagccaccactcccggccaatgttttgtatttttagtagagatggggtttcatcatgttggccagactggtctcaaactctggacctcaggtgatccacctgcctcagcctcccaaagtgtagggattacaggtgtgagccaccgcgcccagcctatgtttctattttatacatattcaacaaacatgattccccaacttctgcaaaataatttctttttcaagaacattgattttagagctcacactaagaaaaagaatacaaaaataatggcatagaaagtgaaaaaacaaaaataaaaagtagaaagctaaagtttcccattaaaatgatcaatatactgtgcagtaagtcaaatgtgtacaatgaattaagaaaatatgatatataaaaatccaaatttacaaaattaagtacaaataggtgtttatattacaaagtgatactggtttataaaaggattcaacatagattttttttaaatggttgttttcctcaatcaatttaacaatgattttaaatgtataaaattttaatatctctttgagacagtgatccaagcttcttcccttgatgatgttaccagttcatactttgtttcaataacctgtccctccacagaaagtaggtgcagtctcttcaccaatacactaagaagtactgtggtcaccatatatgcaaacctcaactctggacactcctgtgtgcctgagaatccaagtgaggaaaaagttttcattactaattcatcatcaaaccgatctggatcaaacttgtgtggagatggccaagtattaggatcctgaagtaccacaccaagggcataaaggacgagggtctgagctgctcaattttctctggagtaacaggaccatttccaaaaacttggtttatctcttcatataattttttttgaacttcttcagaggtggttaaaaaacagattgcccaggtacacaattttgcagttattatgcaactggccagagaaaatatcatactgtcttctaggatctgttggtcattaaggttcccttgtactaaggagtcaatgaaaatatgttgactgaagttccttccttttcgttcttttatgatgttccttaaaacagactccagttgcatgagggtgtgccatgattcttctggaagcgaatgacttcctgatcatcttcaaatgtactacccattaccatctgtgtaacagacttcatagcaaaaccaagcatatgctggctgaggggcacgtgctgggtctctgggtaggagagccatttatctaataattcttctgaaagctttaggaggagggcaaagttactcttcagagaatcagtcacaccattttcatacaattttttcctcatgtggttttcactcacactgccaccaccagattgataccttaataatgacttcagcatggtttcaaaagggtccgttttcttcagttggagtaatccctggaattcctgcagcttgtctggaagccggatagaggtagagcacggctcccaccaacgccagcaagaaggtaacggcgaagatcgcgaagtccaacatggttctgccgcccagggagccacgtctcggatcggccgctccagc

SEQ ID NO: 12076 - RNA, 3965 nt, Homo sapiens
  source 1..3965: mol_type = other RNA
ctgaatagctgggactacaggtgtgtgtcgctacacctggctattttttattttttgtagagataggggtattgctttgtcgcccaggctgggctcagattcctggcttcaagcaattctcccaccttggcttcccaaagtgttgggattacaagcatgagccattgtgtctggcctgggtgattctttatctgacatagaggttgggaaacagaacaacaaaaaaaaattgataaattacataacttacaaattagtaagaaagatatgaccatactaatggaaaaaagttaattcaaaaacttttgaccttaaactaactttttggatattaggcttcctgaagttcaagagtgacatattaggcttatattaggcttatttgtaatgtttgaattatacaggaaacattgtcaagtgtgaggtggtgtttagcttcctttgggttatactgatagagatttgttgttaatatgtgttccaggattgtatgagagttctaaaattctgatatgtcttaatatatgttgtaatgattatgttaaattgttgtaagccacagaaatagccacatttgtcaactgtgtctttatggctgtcttaagacttttgtcatccataattgatgttttgctctgatccttctcaaaaaaaaaaagtgacttataatcagctacagtccaaggcttacttctttggagttcatgaaaagaactcttgaatgcaggtttctggtaactttggagagtgtgccattggattagacagaaaacttccaaggcactaattgaaaggctgatgtgttcataaagatgaatatgaagtagagcaggagttgattacatggactgaaatgaactaatggaagactgaaataatttgtatggcttttgttgtttgaaatattgctacttctttttgttttttcagagtctgaataatctttttattttgagctatttatagccttgaaatacactttaagtgtattgagtattctaatttctccagaatttgtaaactatttatgaatattcttaattcatggcatttgtctgtataaagttaataaccacgttttcttttgtaatagggcacaattgaaaccggttactttctcaggactttgactgaaatggccttgtgaaatgttctagcaaagccaatctaggagagtctatatggacaatgattcttgttgcactttgtgtgggtaatcaggcccagtatatgggactgcagtttattttgaagttaggtcggttctgctgtgatttgtctttggtggaagtggtagactggagacagaaatattgtatgtccctaaattaatatagctcccaacaaccaatccctcattatacctttaactgcaaccaccagacacaacggctaggaataacagcagaggtaggaatgggagttagcgggattgcaacttccctatcctattaccaacgcttgtccaaggattttatggaaagcctggataacattgctcaaagtattgtcaccttacaaattcggataggctccttggcagtggtcgctttgcaaaatcgaaggggactagatctcctaactgctgaaacaggtggcttatgtattttcctagaagaagaatgctgttttgatgtcaaccaatcaggattagtaagggacaccacctgaaaactagctgactgggcctctaaaatatgacaacagctggggcacctaaagggcactaagttgggtttcatggctccctcccttggccagcccattattaatgattatatttgccttggtttttggaccatatctgttaaatcttttaaccaaatccatttccttttgcctagagaccaccaagttagatgatcatgtgacaagatttctagccagtttcaggagaagacaccaccggccatcaagaagctaccctgtctcccctagacaaagcagggtgagagttacgtgatctccaataggtagggactgtgtcccaagttagcatgaagcagttacagaagaaagaccctcagtctctcagcctcccataaagatttacgaggatcacgtctctcagggggaaaatgaggcaggagaatagggtctggagacagggaacctaaggctgattcacattgacttcctagaactgaatcaaaaggaaaaccccacctctccatacctaagtaacaaaaggatcagaggctactccctttgcaatccccttgccttttctgcattgcagatgaaaaatgaaagtgcctctgattggtcccctcctgcaaccaatcagactggtcataggccaagtcctcatttacacaggagtataactttgtaacttcacttcagcctctgattggtcactttctgcaccaatcagacaggtcacgggccactacttcatttacacagggtgtacgccaagtaaccaatggcaaacctctagaggatattcattgctttgtgcgttttgttcaattatttgtccaaaatgccaagaacctggacaccctccaccagtaacagtttgaccagttatttattgtattacttaggactgcatttggctgcatataaaagaaacctgaccaaggcctaattaagcacagtgtttattcttctcactaccaagaagtcagaggtcagcaatccaagctggtgtagcagctcctccaggcatgtcagcaaggagccaagctctgagtctttttactaacatgacccaaagcacatggctgccttccttatgcctaaaagtggctctggtactcaggttttatctctgcactccaagtaggatgaaaagataagagcaaaggctcatgtttgccaagtctgtccttttgtaacaaaaaacccagcagctttatcaagcagaattccacctgtatttcttaacttgccagagctgagtctcatggccacccttagcaggagttggggaggtatttttaacaaggcacattatcatctcccccacccaaagtggagctattgctaatgaaaaagatacaatgagatgtttatgaaattatctgtagctattaatgtcaggtttttgaaatttactgacctggaagaatactcgtaatgcaatgtcaagtgagaagcaggacaaagaacatttgcaatacagttgtatttataaaattttgtttacacacaaaaaatgtattttgcttaaaaatataatttacatatatatacaaccacacaagggaaataacaaaatgttaatactagctaatttctatagagttggcattttaagtcagaggggtattgatgaatagatgtagtttattaaatttttttctctatttcctaaactttctataaagaacttgtagtatctttataataggaaaaaatgtgattttaatgaacactccatatactttcaaagtagactaaattcaaaatatttacacttactcattttcatcttcgttgtcaaaagaaaggaggctactatttttaatttgtttttgtgagttctttttgaccgagtcctgatttacttcatcttcatttggcttcttcttttttgagcttgctgttaaacctgaatatttttcatctgagggatgcttgactggttttcgatatatgattcttccatcggctggagttggttcttcatctgagcaaaaacagaatttttaagaactttcttctcctcattattttgcctttacctgctttggcagcctttatttctgctttaattttcatgacttcttcaactgacaggtctcccttttttaaaaccaccacttgaggctgttcatcttctttgtcactgtgatccccatcttcatctgggggctgaggctgaattctcttagtctctacggtgggtccctccctgtagccgacccgttccttgaagcgggccagaaacgccggctcggctggccgcacgtacgatacctggttccgcttgctcatggtagctctgggtaaag

SEQ ID NO: 12077 - RNA, 3910 nt, Homo sapiens
  source 1..3910: mol_type = other RNA
ctgaatagctgggactacaggtgtgtgtcgctacacctggctattttttattttttgtagagataggggtattgctttgtcgcccaggctgggctcagattcctggcttcaagcaattctcccaccttggcttcccaaagtgttgggattacaagcatgagccattgtgtctggcctgggtgattctttatctgacatagaggttgggaaacagaacaacaaaaaaaaattgataaattacataacttacaaattagtaagaaagatatgaccatactaatggaaaaaagttaattcaaaaacttttgaccttaaactaactttttggatattaggcttcctgaagttcaagagtgacatattaggcttatattaggcttatttgtaatgtttgaattatacaggaaacattgtcaagtgtgaggtggtgtttagcttcctttgggttatactgatagagatttgttgttaatatgtgttccaggattgtatgagagttctaaaattctgatatgtcttaatatatgttgtaatgattatgttaaattgttgtaagccacagaaatagccacatttgtcaactgtgtctttatggctgtcttaagacttttgtcatccataattgatgttttgctctgatccttctcaaaaaaaaaaagtgacttataatcagctacagtccaaggcttacttctttggagttcatgaaaagaactcttgaatgcaggtttctggtaactttggagagtgtgccattggattagacagaaaacttccaaggcactaattgaaaggctgatgtgttcataaagatgaatatgaagtagagcaggagttgattacatggactgaaatgaactaatggaagactgaaataatttgtatggcttttgttgtttgaaatattgctacttctttttgttttttcagagtctgaataatctttttattttgagctatttatagccttgaaatacactttaagtgtattgagtattctaatttctccagaatttgtaaactatttatgaatattcttaattcatggcatttgtctgtataaagttaataaccacgttttcttttgtaatagggcacaattgaaaccggttactttctcaggactttgactgaaatggccttgtgaaatgttctagcaaagccaatctaggagagtctatatggacaatgattcttgttgcactttgtgtgggtaatcaggcccagtatatgggactgcagtttattttgaagttaggtcggttctgctgtgatttgtctttggtggaagtggtagactggagacagaaatattgtatgtccctaaattaatatagctcccaacaaccaatccctcattatacctttaactgcaaccaccagacacaacggctaggaataacagcagaggtaggaatgggagttagcgggattgcaacttccctatcctattaccaacgcttgtccaaggattttatggaaagcctggataacattgctcaaagtattgtcaccttacaaattcggataggctccttggcagtggtcgctttgcaaaatcgaaggggactagatctcctaactgctgaaacaggtggcttatgtattttcctagaagaagaatgctgttttgatgtcaaccaatcaggattagtaagggacaccacctgaaaactagctgactgggcctctaaaatatgacaacagctggggcacctaaagggcactaagttgggtttcatggctccctcccttggccagcccattattaatgattatatttgccttggtttttggaccatatctgttaaatcttttaaccaaatccatttccttttgcctagagaccaccaagttagatgatcatgtgacaagatttctagccagtttcaggagaagacaccaccggccatcaagaagctaccctgtctcccctagacaaagcagggtgagagttacgtgatctccaataggtagggactgtgtcccaagttagcatgaagcagttacagaagaaagaccctcagtctctcagcctcccataaagatttacgaggatcacgtctctcagggggaaaatgaggcaggagaatagggtctggagacagggaacctaaggctgattcacattgacttcctagaactgaatcaaaaggaaaaccccacctctccatacctaagtaacaaaaggatcagaggctactccctttgcaatccccttgccttttctgcattgcagatgaaaaatgaaagtgcctctgattggtcccctcctgcaaccaatcagactggtcataggccaagtcctcatttacacaggagtataactttgtaacttcacttcagcctctgattggtcactttctgcaccaatcagacaggtcacgggccactacttcatttacacagggtgtacgccaagtaaccaatggcaaacctctagaggatattcattgctttgtgcgttttgttcaattatttgtccaaaatgccaagaacctggacaccctccaccagtaacagtttgaccagttatttattgtattacttaggactgcatttggctgcatataaaagaaacctgaccaaggcctaattaagcacagtgtttattcttctcactaccaagaagtcagaggtcagcaatccaagctggtgtagcagctcctccaggcatgtcagcaaggagccaagctctgagtctttttactaacatgacccaaagcacatggctgccttccttatgcctaaaagtggctctggtactcaggttttatctctgcactccaagtaggatgaaaagataagagcaaaggctcatgtttgccaagtctgtccttttgtaacaaaaaacccagcagctttatcaagcagaattccacctgtatttcttaacttgccagagctgagtctcatggccacccttagcaggagttggggaggtatttttaacaaggcacattatcatctcccccacccaaagtggagctattgctaatgaaaaagatacaatgagatgtttatgaaattatctgtagctattaatgtcaggtttttgaaatttactgacctggaagaatactcgtaatgcaatgtcaagtgagaagcaggacaaagaacatttgcaatacagttgtatttataaaattttgtttacacacaaaaaatgtattttgcttaaaaatataatttacatatatatacaaccacacaagggaaataacaaaatgttaatactagctaatttctatagagttggcattttaagtcagaggggtattgatgaatagatgtagtttattaaatttttttctctatttcctaaactttctataaagaacttgtagtatctttataataggaaaaaatgtgattttaatgaacactccatatactttcaaagtagactaaattcaaaatatttacacttactcattttcatcttcgttgtcaaaagaaaggaggctactatttttaatttgtttttgtgagttctttttgaccgagtcctgatttacttcatcttcatttggcttcttcttttttgagcttgctgttaaacctgaatatttttcatctgagggatgcttgactggttttcgatatatgattcttccatcggctggagttggttcttcatctgctttggcagcctttatttctgctttaattttcatgacttcttcaactgacaggtctcccttttttaaaaccaccacttgaggctgttcatcttctttgtcactgtgatccccatcttcatctgggggctgaggctgaattctcttagtctctacggtgggtccctccctgtagccgacccgttccttgaagcgggccagaaacgccggctcggctggccgcacgtacgatacctggttccgcttgctcatggtagctctgggtaaag

SEQ ID NO: 12078 - RNA, 6035 nt, Homo sapiens
  source 1..6035: mol_type = other RNA
ctgaatagctgggactacaggtgttcagtaagataatctctccaattctataccattcccttcaccatccataatatttatttatttatttatttatttatttatttattttcagtcggagtctcactctgtcaccccggctggagtgcagtggtgcaatcttggttcactgcaacctccgcctcccaggttccagcaattcttgtacctcagccttctgagtagctgggattacaggagtgcaccaccacacccagctaatttttttatttttagtagagatgtggttttgccatgttggccaggctggtctcgaactcctgacctcaagtgatctgcccaccatccataatatttaaataagcatattgacttcttcttaaactaagggttaaatataatattttattttaatagttcaggttcatgtatctcatatcttatgctcaagttaataattcctatttgctatacatttatgaaaaagccttataaatggttttaataataaatagatattttaatatttaataataaatagatatttattggaatctaaccttggaaaattttcccaaatacagcaataggattcatgcacaaagatgctcatcccaatgatcaactggagatagccttcaatgagcaaaattatggtaatcgctagaggttgcctattatgcaattattgatataatgtttaagaaggctatgaatataataaaaacatatttgataaaatactaagtgaaaaagcttacataaaaagtatatatgtagtatgataacattctgtaaaattttgaaagagaattgagacatacatagaaaaaaaatagacttgaaaaaccatccagaaattgttagcagtgattaccttaaggtaatggggacaatttatgttctttctacatctctgtatggtctaaattttctataatagccagctattatttttaatggaaaaataataagaggagtatccaataagaacaaagtcagtagtgcctttcaaggttgcattttgggcgacttttcacatatttaggaatgggggtggttccttcaataggagcctggtgagtccaagagagcaagagactgccttgtcacctcctctgacaggtaagaagcatcctgagaaatgaaaacacttttcctgaagagagcggggtcctcttgctgcagcatgttttagaatctggcctaatttgagagacttttaacaatatgccaactaattagtcacataatacaaaaaagggaaaagtagagaatcaattggaaatgaacaaaataacaatacaggagtaaagcatgaccaggttcttattcataggatagatgttctcctatatatgtgttcatcaaaaataagattaaaggaaaaaggaggcggtaagaacacacttaaactatcaacctccagtcccaggcattgagacacagagagaaacaggcaccattctggagaaacacataaaggaaatattcttcctttatatccgtcttcaagtatgaaaccaatcacacactttattctcaaggtctcagcacactagggtgatttaaaatcatccaccatgtacccaggggtctgaaaatctctcatttagtagtcgatagcaaaattgttcatcagcattccttaatatgatcttgctataattagatttttctccattagagttcatacagttttatttgattttattagcaatctctttcagaagacccttgagatcattaagctttgtatccagttgtctaaatcgatgcctcatttcctctgaggtgtcgttggcttttgtgttgatcttgacaaggtagttttccttcatgacaccctcccatgccagagtctcattgtcttcatttttgaaacagcagacagaagactccatgtttttctccttgcagcaacacttgaagcacttcttcaccaccatgtagaagtaagcgaagacgatgaaggggaaggggatattgaggcggctgcagtactcctgcaccaggaagtacctctggaacttccagacctggtcattgttctcctggacggtgcccaccgtgtagccaaacatggcgaccagcaggttgaccagcaggatgttggtggataacatgtagatgcacaccagggggatggtgatccactcggggaaccggggcaggttgtgctcatccagctccacacacagtggcttggactcattcccagtgaaggtgcagtgggcaaagtcatacgtggtaccatccacgtcactgggcacctggccgaacatggccaggtagggctcgtagatgaccgaacggaatatccacctccagcgctgctcattctgcctaaggatcccttgcctggccacgccaaaggccaccatccacaccgcaaagaggaacaggaagaagaacacatcgatcagcatcctctgcagcattataatcttgggtcctaagtttctgcttacagtaaaaatgtggatcaatcttagagtgaaaataatgtagtccagacagaaaatgactcgtccagaatacaaagagcttttattagaagagtggagccgaaatacaattcctgctatgaagtaaaaaagccccagcgtgtccatcacattccacaggtcagtaaaataattcaccccatttacgtaccactgtctcacttcatcacagaagaggacaaagaccagcgagtacaggaccagctcgggggggtgtggcaccgaatggaaatccatgagcagcacgtaggcaaacagcaggaggaaggcgatgtagaagaccacattccaggagaagaccacgaagggggaggtgaagaacgccacatagtaccaaagcagcttcttgtgcttgtcgacaggtttcttcctaaatgatacaaagccacagcccaccaagggtataataaacagacacaggataatcttccagttcttggtgtctcgggaaatctctccataccattgcttagaaagaaaattctggaccccaggctgggcgatgaaatgctggtctgtggcctccaccgccagctccagacagttgcttccaccccaagcttcacaggaatagaccagcagctgttctgccaagtcttcatcgctgctgtaacactcagtgaacagctcaacagcccgggtctcgtactcattagccagctcctcggactccccagcagcattgatgtcgttcttcactttggccagagtcttcagaagcttgctggctcccagggctgccagagtgcagcccctggtctgctcccaaatgactttggagagttccttcttattctgaagaatggcccagatgaagagagcttgcagggggtgccgagtaataggagacacgtcgtggagttctatgtccatctcgtcccggccatttctgtcttccttccggaagcctcttcggaagttcgcaaccagtttccagacaaacgtgaggagggcatcattataggaattcttggcgatctgcagattccggtacacaagcgtgctgaagtggttggagaagagttcagtgaggacatcatgggtgagaaacttccgtaggttcaagccattctccagaaagaggcggacaaacttgggtctgtcctttatgagagccgtaaacatgacttcttgaaggtcagcagactcccatcggcggtcattggtgaaaatctcatcattggctaagtccagctggttccactccagcagaagcttcagctgcccattccagttatccttgtcttgctcactggtgctgaaggctttgtatagagcgtaggagatggcattgctcacaatttcatccccagcttcttccattttaataactgttaataggtgagaacattcgagaatttctttgagccatttgatccaactctcagtctcctcctcaggcagccgggacaccgtgcggggtaaaaagcgcaccagcttctccttgacggcagaagatgtcagggcatcctccacctccaccaggctagcgatcacatcagcgatctggcccgagccttccaccaccacacaaggaattttatttttgatggaggtattgatggctttcaaagtctcttttccacctccttgggcaaaacacacaatggggatcttgccaccatagttggaatcttgaatagtgcgctcagagatatacttctctagctgattccggagctttgcttcgacagtgggatgtccatgacagccattgtccacgagcagcaaatgtgtgtggttgttgtccaggatatacagtggatctcttgtgaagtcatccataaggtactgggctaaaaaatagccctcagcatcgcaattcctgatgagggtgtcccggttggagaccatgccccaagctgctatgccaatggccacaatattctcctctgaactcctgctgatggtgttatctctcaccacctccccgatgtacttcatcaggccataatgggtgcctcccgtgagaatccaagcacctttggactgcgcgatgtagatgagccggctgaagatcttgcgcatgcgcggcttcagggcgaagttcttggcgcccccggtcacagaaatgaccaggttgggtgttttcaggtgccagtgctgggtcagcagctcgtaaaggatttccgcgtccgtgtcgcaggacagacgtatatacttccctttcttccccagtgtctcaaactgaatatccccaaaggcgtcggtaggaaattccttggtgtgtttcttgtagttccatttctcactttggttgatctgggtgccttccatgtgctggctctgggcatagccacacttgcacacattctccctctgttttggaacagttcccagggcatcactcagtgtggccaagatatgtcaaccagaattcagcacaatgttcttagccctctctcttcctaagtgttagggcacttcctgagcccaggctacttcctgatgttcctcttctctctccatagcttccactgtcccaccatcctttgggatctgtccacccacccaagcttattggaggatgggggagagaattccccgccccatctgttcttgctataactgaaaacaaactgttgggcccttttccctgctaagggtaggggtgtgtcacaggtgaccttgaccaagagagctgcctggcagctctggtctatgggctggtagccctctaagcaccaatttgtatgaactggtttataaatggagaaaagaaattgccaggaagacattaggagtgcagatacctgaaggaggaataaggatgacagacaggagaaatgaagaggacaggaaaacatcaggaccctagttctacccccttggaccaaatctgaatcctgtagaactacaccgtccaatatggtagccactgacctcacgtggttatttaattttatatttaagttaagtgaaattaaataaattaaaaacattccttcgttgtcctagccacatttcaaatgatcaatagccagatgtggctagtggctaccgtattggatggtgcggacatagaatatttccaccagggaagaaagttctgttgcacagtgctgctgttgtgaaggtagcattctttctgtttctacctggaacccagcatggccaaggaagtgagaagtgactagagcaaaaccagacctaggagcttactacccatagtgtgccagaaggtggctcctaagctggcagcacatttcagaggacacagcagcaggggcaaaagtgcggcaccatcttgcagtagcgtccacaagaagttagagtagagaggcaagggtgggttgggcttagcactagggtggcaaccctgagaactctcaggggagactttggcagcttaggtcatctagtgtggcaagtaacagcaaaaccagggtatcaataaaattaatcatcacttcatttgatgcccttgtctgatgggtaacttagattacatggagtgatcccactacctgtggagagagagaaataataaacatgggggattcaaagattatagaatcctgcatcctt

SEQ ID NO: 12079 - RNA, 5080 nt, Homo sapiens
  source 1..5080: mol_type = other RNA
ctgaatagctgggactacaggtgttcagtaagataatctctccaattctataccattcccttcaccatccataatatttatttatttatttatttatttatttatttattttcagtcggagtctcactctgtcaccccggctggagtgcagtggtgcaatcttggttcactgcaacctccgcctcccaggttccagcaattcttgtacctcagccttctgagtagctgggattacaggagtgcaccaccacacccagctaatttttttatttttagtagagatgtggttttgccatgttggccaggctggtctcgaactcctgacctcaagtgatctgcccaccatccataatatttaaataagcatattgacttcttcttaaactaagggttaaatataatattttattttaatagttcaggttcatgtatctcatatcttatgctcaagttaataattcctatttgctatacatttatgaaaaagccttataaatggttttaataataaatagatattttaatatttaataataaatagatatttattggaatctaaccttggaaaattttcccaaatacagcaataggattcatgcacaaagatgctcatcccaatgatcaactggagatagccttcaatgagcaaaattatggtaatcgctagaggttgcctattatgcaattattgatataatgtttaagaaggctatgaatataataaaaacatatttgataaaatactaagtgaaaaagcttacataaaaagtatatatgtagtatgataacattctgtaaaattttgaaagagaattgagacatacatagaaaaaaaatagacttgaaaaaccatccagaaattgttagcagtgattaccttaaggtaatggggacaatttatgttctttctacatctctgtatggtctaaattttctataatagccagctattatttttaatggaaaaataataagaggagtatccaataagaacaaagtcagtagtgcctttcaaggttgcattttgggcgacttttcacatatttaggaatgggggtggttccttcaataggagcctggtgagtccaagagagcaagagactgccttgtcacctcctctgacaggtaagaagcatcctgagaaatgaaaacacttttcctgaagagagcggggtcctcttgctgcagcatgttttagaatctggcctaatttgagagacttttaacaatatgccaactaattagtcacataatacaaaaaagggaaaagtagagaatcaattggaaatgaacaaaataacaatacaggagtaaagcatgaccaggttcttattcataggatagatgttctcctatatatgtgttcatcaaaaataagattaaaggaaaaaggaggcggtaagaacacacttaaactatcaacctccagtcccaggcattgagacacagagagaaacaggcaccattctggagaaacacataaaggaaatattcttcctttatatccgtcttcaagtatgaaaccaatcacacactttattctcaaggtctcagcacactagggtgatttaaaatcatccaccatgtacccaggggtctgaaaatctctcatttagtagtcgatagcaaaattgttcatcagcattccttaatatgatcttgctataattagatttttctccattagagttcatacagttttatttgattttattagcaatctctttcagaagacccttgagatcattaagctttgtatccagttgtctaaatcgatgcctcatttcctctgaggtgtcgttggcttttgtgttgatcttgacaaggtagttttccttcatgacaccctcccatgccagagtctcattgtcttcatttttgaaacagcagacagaagactccatgtttttctccttgcagcaacacttgaagcacttcttcaccaccatgtagaagtaagcgaagacgatgaaggggaaggggatattgaggcggctgcagtactcctgcaccaggaagtacctctggaacttccagacctggtcattgttctcctggacggtgcccaccgtgtagccaaacatggcgaccagcaggttgaccagcaggatgttggtggataacatgtagatgcacaccagggggatggtgatccactcggggaaccggggcaggttgtgctcatccagctccacacacagtggcttggactcattcccagtgaaggtgcagtgggcaaagtcatacgtggtaccatccacgtcactgggcacctggccgaacatggccaggtagggctcgtagatgaccgaacggaatatccacctccagcgctgctcattctgcctaaggatcccttgcctggccacgccaaaggccaccatccacaccgcaaagaggaacaggaagaagaacacatcgatcagcatcctctgcagcattataatcttgggtcctaagtttctgcttacagtaaaaatgtggatcaatcttagagtgaaaataatgtagtccagacagaaaatgactcgtccagaatacaaagagcttttattagaagagtggagccgaaatacaattcctgctatgaagtaaaaaagccccagcgtgtccatcacattccacaggtcagtaaaataattcaccccatttacgtaccactgtctcacttcatcacagaagaggacaaagaccagcgagtacaggaccagctcgggggggtgtggcaccgaatggaaatccatgagcagcacgtaggcaaacagcaggaggaaggcgatgtagaagaccacattccaggagaagaccacgaagggggaggtgaagaacgccacatagtaccaaagcagcttcttgtgcttgtcgacaggtttcttcctaaatgatacaaagccacagcccaccaagggtataataaacagacacaggataatcttccagttcttggtgtctcgggaaatctctccataccattgcttagaaagaaaattctggaccccaggctgggcgatgaaatgctggtctgtggcctccaccgccagctccagacagttgcttccaccccaagcttcacaggaatagaccagcagctgttctgccaagtcttcatcgctgctgtaacactcagtgaacagctcaacagcccgggtctcgtactcattagccagctcctcggactccccagcagcattgatgtcgttcttcactttggccagagtcttcagaagcttgctggctcccagggctgccagagtgcagcccctggtctgctcccaaatgactttggagagttccttcttattctgaagaatggcccagatgaagagagcttgcagggggtgccgagtaataggagacacgtcgtggagttctatgtccatctcgtcccggccatttctgtcttccttccggaagcctcttcggaagttcgcaaccagtttccagacaaacgtgaggagggcatcattataggaattcttggcgatctgcagattccggtacacaagcgtgctgaagtggttggagaagagttcagtgaggacatcatgggtgagaaacttccgtaggttcaagccattctccagaaagaggcggacaaacttgggtctgtcctttatgagagccgtaaacatgacttcttgaaggtcagcagactcccatcggcggtcattggtgaaaatctcatcattggctaagtccagctggttccactccagcagaagcttcagctgcccattccagttatccttgtcttgctcactggtgctgaaggctttgtatagagcgtaggagatggcattgctcacaatttcatccccagcttcttccattttaataactgttaataggtgagaacattcgagaatttctttgagccatttgatccaactctcagtctcctcctcaggcagccgggacaccgtgcggggtaaaaagcgcaccagcttctccttgacggcagaagatgtcagggcatcctccacctccaccaggctagcgatcacatcagcgatctggcccgagccttccaccaccacacaaggaattttatttttgatggaggtattgatggctttcaaagtctcttttccacctccttgggcaaaacacacaatggggatcttgccaccatagttggaatcttgaatagtgcgctcagagatatacttctctagctgattccggagctttgcttcgacagtgggatgtccatgacagccattgtccacgagcagcaaatgtgtgtggttgttgtccaggatatacagtggatctcttgtgaagtcatccataaggtactgggctaaaaaatagccctcagcatcgcaattcctgatgagggtgtcccggttggagaccatgccccaagctgctatgccaatggccacaatattctcctctgaactcctgctgatggtgttatctctcaccacctccccgatgtacttcatcaggccataatgggtgcctcccgtgagaatccaagcacctttggactgcgcgatgtagatgagccggctgaagatcttgcgcatgcgcggcttcagggcgaagttcttggcgcccccggtcacagaaatgaccaggttgggtgttttcaggtgccagtgctgggtcagcagctcgtaaaggatttccgcgtccgtgtcgcaggacagacgtatatacttccctttcttccccagtgtctcaaactgaatatccccaaaggcgtcggtaggaaattccttggtgtgtttcttgtagttccatttctcactttggttgatctgggtgccttccatgtgctggctctgggcatagccacacttgcacacattctccgtggccttggaatctttggtaaagaagacacattctcgtttcttaaaatttgcttgaataaaattcaccaagtcgctttcactgtaagacaagtctgtgctccgagacgcgctggagtacagggtccgggtgctgtccagagtgtcattccttctgttcctcatgctgagcctggctgcccgaaaggacatcttttcctaagtgacggtttttgtcaagcaggattttctttcacccaaggatcctgctggtctct

SEQ ID NO: 12080 - RNA, 4058 nt, Homo sapiens
  source 1..4058: mol_type = other RNA
ctgaatagctgggactacaggtgttcagtaagataatctctccaattctataccattcccttcaccatccataatatttatttatttatttatttatttatttatttattttcagtcggagtctcactctgtcaccccggctggagtgcagtggtgcaatcttggttcactgcaacctccgcctcccaggttccagcaattcttgtacctcagccttctgagtagctgggattacaggagtgcaccaccacacccagctaatttttttatttttagtagagatgtggttttgccatgttggccaggctggtctcgaactcctgacctcaagtgatctgcccaccatccataatatttaaataagcatattgacttcttcttaaactaagggttaaatataatattttattttaatagttcaggttcatgtatctcatatcttatgctcaagttaataattcctatttgctatacatttatgaaaaagccttataaatggttttaataataaatagatattttaatatttaataataaatagatatttattggaatctaaccttggaaaattttcccaaatacagcaataggattcatgcacaaagatgctcatcccaatgatcaactggagatagccttcaatgagcaaaattatggtaatcgctagaggttgcctattatgcaattattgatataatgtttaagaaggctatgaatataataaaaacatatttgataaaatactaagtgaaaaagcttacataaaaagtatatatgtagtatgataacattctgtaaaattttgaaagagaattgagacatacatagaaaaaaaatagacttgaaaaaccatccagaaattgttagcagtgattaccttaaggtaatggggacaatttatgttctttctacatctctgtatggtctaaattttctataatagccagctattatttttaatggaaaaataataagaggagtatccaataagaacaaagtcagtagtgcctttcaaggttgcattttgggcgacttttcacatatttaggaatgggggtggttccttcaataggagcctggtgagtccaagagagcaagagactgccttgtcacctcctctgacaggtaagaagcatcctgagaaatgaaaacacttttcctgaagagagcggggtcctcttgctgcagcatgttttagaatctggcctaatttgagagacttttaacaatatgccaactaattagtcacataatacaaaaaagggaaaagtagagaatcaattggaaatgaacaaaataacaatacaggagtaaagcatgaccaggttcttattcataggatagatgttctcctatatatgtgttcatcaaaaataagattaaaggaaaaaggaggcggtaagaacacacttaaactatcaacctccagtcccaggcattgagacacagagagaaacaggcaccattctggagaaacacataaaggaaatattcttcctttatatccgtcttcaagtatgaaaccaatcacacactttattctcaaggtctcagcacactagggtgatttaaaatcatccaccatgtacccaggggtctgaaaatctctcatttagtagtcgatagcaaaattgttcatcagcattccttaatatgatcttgctataattagatttttctccattagagttcatacagttttatttgattttattagcaatctctttcagaagacccttgagatcattaagctttgtatccagttgtctaaatcgatgcctcatttcctctgaggtgtcgttggcttttgtgttgatcttgacaaggtagttttccttcatgacaccctcccatgccagagtctcattgtcttcatttttgaaacagcagacagaagactccatgtttttctccttgcagcaacacttgaagcacttcttcaccaccatgtagaagtaagcgaagacgatgaaggggaaggggatattgaggcggctgcagtactcctgcaccaggaagtacctctggaacttccagacctggtcattgttctcctggacggtgcccaccgtgtagccaaacatggcgaccagcaggttgaccagcaggatgttggtggataacatgtagatgcacaccagggggatggtgatccactcggggaaccggggcaggttgtgctcatccagctccacacacagtggcttggactcattcccagtgaaggtgcagtgggcaaagtcatacgtggtaccatccacgtcactgggcacctggccgaacatggccaggtagggctcgtagatgaccgaacggaatatccacctccagcgctgctcattctgcctaaggatcccttgcctggccacgccaaaggccaccatccacaccgcaaagaggaacaggaagaagaacacatcgatcagcatcctctgcagcattataatcttgggtcctaagtttctgcttacagtaaaaatgtggatcaatcttagagtgaaaataatgtagtccagacagaaaatgactcgtccagaatacaaagagcttttattagaagagtggagccgaaatacaattcctgctatgaagtaaaaaagccccagcgtgtccatcacattccacaggtcagtaaaataattcaccccatttacgtaccactgtctcacttcatcacagaagaggacaaagaccagcgagtacaggaccagctcgggggggtgtggcaccgaatggaaatccatgagcagcacgtaggcaaacagcaggaggaaggcgatgtagaagaccacattccaggagaagaccacgaagggggaggtgaagaacgccacatagtaccaaagcagcttcttgtgcttgtcgacaggtttcttcctaaatgatacaaagccacagcccaccaagggtataataaacagacacaggataatcttccagttcttggtgtctcgggaaatctctccataccattgcttagaaagaaaattctggaccccaggctgggcgatgaaatgctggtctgtggcctccaccgccagctccagacagttgcttccaccccaagcttcacaggaatagaccagcagctgttctgccaagtcttcatcgctgctgtaacactcagtgaacagctcaacagcccgggtctcgtactcattagccagctcctcggactccccagcagcattgatgtcgttcttcactttggccagagtcttcagaagcttgctggctcccagggctgccagagtgcagcccctggtctgctcccaaatgactttggagagttccttcttattctgaagaatggcccagatgaagagagcttgcagggggtgccgagtaataggagacacgtcgtggagttctatgtccatctcgtcccggccatttctgtcttccttccggaagcctcttcggaagttcgcaaccagtttccagacaaacgtgaggagggcatcattataggaattcttggcgatctgcagattccggtacacaagcgtgctgaagtggttggagaagagttcagtgaggacatcatgggtgagaaacttccgtaggttcaagccattctccagaaagaggcggacaaacttgggtctgtcctttatgagagccgtaaacatgacttcttgaaggtcagcagactcccatcggcggtcattggtgaaaatctcatcattggctaagtccagctggttccactccagcagaagcttcagctgcccattccagttatccttgtcttgctcactggtgctgaaggctttgtatagagcgtaggagatggcattgctcacaatttcatccccagcttcttccattttaataactgttaataggtgagaacattcgagaatttctttgagctgtagtggagttccggatcagcttctcatttctgaattgcaatgagtccttgactacagtgagaataaagtattggttatacacgtatcaaaaagcccctatcaaaaagctgagagcctcatttgactagagatgtgtgcatctgcgtgcaggtgctgtgtgtgtgtgtgtgtgtcacaaag

SEQ ID NO: 12081 - RNA, 6829 nt, Homo sapiens
  source 1..6829: mol_type = other RNA
ctgaatagctgggactacaggtgttcagtaagataatctctccaattctataccattcccttcaccatccataatatttatttatttatttatttatttatttatttattttcagtcggagtctcactctgtcaccccggctggagtgcagtggtgcaatcttggttcactgcaacctccgcctcccaggttccagcaattcttgtacctcagccttctgagtagctgggattacaggagtgcaccaccacacccagctaatttttttatttttagtagagatgtggttttgccatgttggccaggctggtctcgaactcctgacctcaagtgatctgcccaccatccataatatttaaataagcatattgacttcttcttaaactaagggttaaatataatattttattttaatagttcaggttcatgtatctcatatcttatgctcaagttaataattcctatttgctatacatttatgaaaaagccttataaatggttttaataataaatagatattttaatatttaataataaatagatatttattggaatctaaccttggaaaattttcccaaatacagcaataggattcatgcacaaagatgctcatcccaatgatcaactggagatagccttcaatgagcaaaattatggtaatcgctagaggttgcctattatgcaattattgatataatgtttaagaaggctatgaatataataaaaacatatttgataaaatactaagtgaaaaagcttacataaaaagtatatatgtagtatgataacattctgtaaaattttgaaagagaattgagacatacatagaaaaaaaatagacttgaaaaaccatccagaaattgttagcagtgattaccttaaggtaatggggacaatttatgttctttctacatctctgtatggtctaaattttctataatagccagctattatttttaatggaaaaataataagaggagtatccaataagaacaaagtcagtagtgcctttcaaggttgcattttgggcgacttttcacatatttaggaatgggggtggttccttcaataggagcctggtgagtccaagagagcaagagactgccttgtcacctcctctgacaggtaagaagcatcctgagaaatgaaaacacttttcctgaagagagcggggtcctcttgctgcagcatgttttagaatctggcctaatttgagagacttttaacaatatgccaactaattagtcacataatacaaaaaagggaaaagtagagaatcaattggaaatgaacaaaataacaatacaggagtaaagcatgaccaggttcttattcataggatagatgttctcctatatatgtgttcatcaaaaataagattaaaggaaaaaggaggcggtaagaacacacttaaactatcaacctccagtcccaggcattgagacacagagagaaacaggcaccattctggagaaacacataaaggaaatattcttcctttatatccgtcttcaagtatgaaaccaatcacacactttattctcaaggtctcagcacactagggtgatttaaaatcatccaccatgtacccaggggtctgaaaatctctcatttagtagtcgatagcaaaattgttcatcagcattccttaatatgatctttgtatccagttgtctaaatcgatgcctcatttcctctgaggtgtcgttggcttttgtgttgatcttgacaaggtagttttccttcatgacaccctcccatgccagagtctcattgtcttcatttttgaaacagcagacagaagactccatgtttttctccttgcagcaacacttgaagcacttcttcaccaccatgtagaagtaagcgaagacgatgaaggggaaggggatattgaggcggctgcagtactcctgcaccaggaagtacctctggaacttccagacctggtcattgttctcctggacggtgcccaccgtgtagccaaacatggcgaccagcaggttgaccagcaggatgttggtggataacatgtagatgcacaccagggggatggtgatccactcggggaaccggggcaggttgtgctcatccagctccacacacagtggcttggactcattcccagtgaaggtgcagtgggcaaagtcatacgtggtaccatccacgtcactgggcacctggccgaacatggccaggtagggctcgtagatgaccgaacggaatatccacctccagcgctgctcattctgcctaaggatcccttgcctggccacgccaaaggccaccatccacaccgcaaagaggaacaggaagaagaacacatcgatcagcatcctctgcagcattataatcttgggtcctaagtttctgcttacagtaaaaatgtggatcaatcttagagtgaaaataatgtagtccagacagaaaatgactcgtccagaatacaaagagcttttattagaagagtggagccgaaatacaattcctgctatgaagtaaaaaagccccagcgtgtccatcacattccacaggtcagtaaaataattcaccccatttacgtaccactgtctcacttcatcacagaagaggacaaagaccagcgagtacaggaccagctcgggggggtgtggcaccgaatggaaatccatgagcagcacgtaggcaaacagcaggaggaaggcgatgtagaagaccacattccaggagaagaccacgaagggggaggtgaagaacgccacatagtaccaaagcagcttcttgtgcttgtcgacaggtttcttcctaaatgatacaaagccacagcccaccaagggtataataaacagacacaggataatcttccagttcttggtgtctcgggaaatctctccataccattgcttagaaagaaaattctggaccccaggctgggcgatgaaatgctggtctgtggcctccaccgccagctccagacagttgcttccaccccaagcttcacaggaatagaccagcagctgttctgccaagtcttcatcgctgctgtaacactcagtgaacagctcaacagcccgggtctcgtactcattagccagctcctcggactccccagcagcattgatgtcgttcttcactttggccagagtcttcagaagcttgctggctcccagggctgccagagtgcagcccctggtctgctcccaaatgactttggagagttccttcttattctgaagaatggcccagatgaagagagcttgcagggggtgccgagtaataggagacacgtcgtggagttctatgtccatctcgtcccggccatttctgtcttccttccggaagcctcttcggaagttcgcaaccagtttccagacaaacgtgaggagggcatcattataggaattcttggcgatctgcagattccggtacacaagcgtgctgaagtggttggagaagagttcagtgaggacatcatgggtgagaaacttccgtaggttcaagccattctccagaaagaggcggacaaacttgggtctgtcctttatgagagccgtaaacatgacttcttgaaggtcagcagactcccatcggcggtcattggtgaaaatctcatcattggctaagtccagctggttccactccagcagaagcttcagctgcccattccagttatccttgtcttgctcactggtgctgaaggctttgtatagagcgtaggagatggcattgctcacaatttcatccccagcttcttccattttaataactgttaataggtgagaacattcgagaatttctttgagccatttgatccaactctcagtctcctcctcaggcagccgggacaccgtgcggggtaaaaagcgcaccagcttctccttgacggcagaagatgtcagggcatcctccacctccaccaggctagcgatcacatcagcgatctggcccgagccttccaccaccacacaaggaattttatttttgatggaggtattgatggctttcaaagtctcttttccacctccttgggcaaaacacacaatggggatcttgccaccatagttggaatcttgaatagtgcgctcagagatatacttctctagctgattccggagctttgcttcgacagtgggatgtccatgacagccattgtccacgagcagcaaatgtgtgtggttgttgtccaggatatacagtggatctcttgtgaagtcatccataaggtactgggctaaaaaatagccctcagcatcgcaattcctgatgagggtgtcccggttggagaccatgccccaagctgctatgccaatggccacaatattctcctctgaactcctgctgatggtgttatctctcaccacctccccgatgtacttcatcaggccataatgggtgcctcccgtgagaatccaagcacctttggactgcgcgatgtagatgagccggctgaagatcttgcgcatgcgcggcttcagggcgaagttcttggcgcccccggtcacagaaatgaccaggttgggtgttttcaggtgccagtgctgggtcagcagctcgtaaaggatttccgcgtccgtgtcgcaggacagacgtatatacttccctttcttccccagtgtctcaaactgaatatccccaaaggcgtcggtaggaaattccttggtgtgtttcttgtagttccatttctcactttggttgatctgggtgccttccatgtgctggctctgggcatagccacacttgcacacattctcccttctgagatgggaactggaagaccctgaggtgttcctgtgctccgcttgtgttgctgagggctgcggctgcccaccacatctcccttcattttgacccagacttgagctgtaatcaagcactgtaaggtgaacagccacaggtttccctaacctgcatctacttccccttccactagtaagtgcgccctgattttccttgaggaatcatgcctttctgcattgagttcacctggacacatctcccaagccttgccaatcaacatattccactgtccctcaacttccatcctccagccccagggattagtttagagataggcacatgctccaagcaagaccattaagagccataaacatcagcccaggacttttgatggaattgctaggagcaaggccctctttgctctaactggcaaatggaaagctgataacgcacaaccaacaatgaccattttgcctccaatagtgaagagcccatccatcagagaagggcaggaacaacaggtggaaagagacagagtctcggcgacgttgttgaagccctggatctggctgtgcttttcagccacaagatcccattatcacaccccacagaatccctgctccagcttccacttatgccagttagattgaacatatgtaactgagaacgtgttgaggaatttgttctgcccaaagcaacgccattcttagaaagggaggcaactgacggtatagagaaggcacagccttggaatcagaaagcccgggctcaagtctctcatccatcttccactgcacatgtgaccatgggtaaaatactgaacttctctgggcctcacttgccttaaaggtagcaacagcttccttgcaaggaggttgataatattagcaatccagtatgtaagtcccattcatgaaacatacaggggataaatagtggtcttacaaagcttacactttgtcagaatgactcatgatgcgtatgtttttaccagtgacaaggcagagatctcttagtttttctggtgttcattttctaattcacatgaagtaagaattatgctctgaagcattatggtaggtattttatatgctgcgtcttgaataccacaacccatgaggtatacttttgctagatttttaggataagagaattagctttagaaaagagaataattggctcaaggccacacagtgaggagtcagccaagtcaaggttgaaaccaaagctggttctaaagcttttttccttatttctatatccttcctctgttcattgaccctgttcaacagagagtcttttcattataaactacagcagcaacttgcaattaatagctagactctttcttgcattgccagccaacagaaaggaaggggcagagaggaataaggagagtgggaggtaggacgaaaattgtttaattagattcaaatgcatcttctacacaaagggtgagcactagtcgacccattcactcactcacttgctcatcaacagttattgaagaactcctgtaggctgagctggtgaagcctgcttttgtaacccagccttaatgttccaaaacacatgagacttagagcagatgaacactcaattagaaggaaagacctaaagtcaacagcagggaagaaaagcctgacggaggagccagtaagatggacatatgtacacatgcatggtattgccagccaacagctgtaaaacaactttcattaccaaggtcactcaggtgggttcccaatctcatgggaatactgaagagagtgacagcctccctcaacgacttttccaactatggccaaagctgaaaataccaaacaaaattgtatagctctgagtaacaactataagctccttgccagatccttcctgcgcaaacagtgtttctgagaattataagacgaagacatctttaataatgaactagggagcatttgtttgttgtaagggtggctgataatttttttgaacttggaaagcaaaactggagggaaaatagtagcttacgtggccttggaatctttggtaaagaagacacattctcgtttcttaaaatttgcttgaataaaattcaccaagtcgctttcactgtaagacaagtctgtgc

SEQ ID NO: 12082 - RNA, 5018 nt, Homo sapiens
  source 1..5018: mol_type = other RNA
ctgaatagctgggactacaggtgttcagtaagataatctctccaattctataccattcccttcaccatccataatatttatttatttatttatttatttatttatttattttcagtcggagtctcactctgtcaccccggctggagtgcagtggtgcaatcttggttcactgcaacctccgcctcccaggttccagcaattcttgtacctcagccttctgagtagctgggattacaggagtgcaccaccacacccagctaatttttttatttttagtagagatgtggttttgccatgttggccaggctggtctcgaactcctgacctcaagtgatctgcccaccatccataatatttaaataagcatattgacttcttcttaaactaagggttaaatataatattttattttaatagttcaggttcatgtatctcatatcttatgctcaagttaataattcctatttgctatacatttatgaaaaagccttataaatggttttaataataaatagatattttaatatttaataataaatagatatttattggaatctaaccttggaaaattttcccaaatacagcaataggattcatgcacaaagatgctcatcccaatgatcaactggagatagccttcaatgagcaaaattatggtaatcgctagaggttgcctattatgcaattattgatataatgtttaagaaggctatgaatataataaaaacatatttgataaaatactaagtgaaaaagcttacataaaaagtatatatgtagtatgataacattctgtaaaattttgaaagagaattgagacatacatagaaaaaaaatagacttgaaaaaccatccagaaattgttagcagtgattaccttaaggtaatggggacaatttatgttctttctacatctctgtatggtctaaattttctataatagccagctattatttttaatggaaaaataataagaggagtatccaataagaacaaagtcagtagtgcctttcaaggttgcattttgggcgacttttcacatatttaggaatgggggtggttccttcaataggagcctggtgagtccaagagagcaagagactgccttgtcacctcctctgacaggtaagaagcatcctgagaaatgaaaacacttttcctgaagagagcggggtcctcttgctgcagcatgttttagaatctggcctaatttgagagacttttaacaatatgccaactaattagtcacataatacaaaaaagggaaaagtagagaatcaattggaaatgaacaaaataacaatacaggagtaaagcatgaccaggttcttattcataggatagatgttctcctatatatgtgttcatcaaaaataagattaaaggaaaaaggaggcggtaagaacacacttaaactatcaacctccagtcccaggcattgagacacagagagaaacaggcaccattctggagaaacacataaaggaaatattcttcctttatatccgtcttcaagtatgaaaccaatcacacactttattctcaaggtctcagcacactagggtgatttaaaatcatccaccatgtacccaggggtctgaaaatctctcatttagtagtcgatagcaaaattgttcatcagcattccttaatatgatctttgtatccagttgtctaaatcgatgcctcatttcctctgaggtgtcgttggcttttgtgttgatcttgacaaggtagttttccttcatgacaccctcccatgccagagtctcattgtcttcatttttgaaacagcagacagaagactccatgtttttctccttgcagcaacacttgaagcacttcttcaccaccatgtagaagtaagcgaagacgatgaaggggaaggggatattgaggcggctgcagtactcctgcaccaggaagtacctctggaacttccagacctggtcattgttctcctggacggtgcccaccgtgtagccaaacatggcgaccagcaggttgaccagcaggatgttggtggataacatgtagatgcacaccagggggatggtgatccactcggggaaccggggcaggttgtgctcatccagctccacacacagtggcttggactcattcccagtgaaggtgcagtgggcaaagtcatacgtggtaccatccacgtcactgggcacctggccgaacatggccaggtagggctcgtagatgaccgaacggaatatccacctccagcgctgctcattctgcctaaggatcccttgcctggccacgccaaaggccaccatccacaccgcaaagaggaacaggaagaagaacacatcgatcagcatcctctgcagcattataatcttgggtcctaagtttctgcttacagtaaaaatgtggatcaatcttagagtgaaaataatgtagtccagacagaaaatgactcgtccagaatacaaagagcttttattagaagagtggagccgaaatacaattcctgctatgaagtaaaaaagccccagcgtgtccatcacattccacaggtcagtaaaataattcaccccatttacgtaccactgtctcacttcatcacagaagaggacaaagaccagcgagtacaggaccagctcgggggggtgtggcaccgaatggaaatccatgagcagcacgtaggcaaacagcaggaggaaggcgatgtagaagaccacattccaggagaagaccacgaagggggaggtgaagaacgccacatagtaccaaagcagcttcttgtgcttgtcgacaggtttcttcctaaatgatacaaagccacagcccaccaagggtataataaacagacacaggataatcttccagttcttggtgtctcgggaaatctctccataccattgcttagaaagaaaattctggaccccaggctgggcgatgaaatgctggtctgtggcctccaccgccagctccagacagttgcttccaccccaagcttcacaggaatagaccagcagctgttctgccaagtcttcatcgctgctgtaacactcagtgaacagctcaacagcccgggtctcgtactcattagccagctcctcggactccccagcagcattgatgtcgttcttcactttggccagagtcttcagaagcttgctggctcccagggctgccagagtgcagcccctggtctgctcccaaatgactttggagagttccttcttattctgaagaatggcccagatgaagagagcttgcagggggtgccgagtaataggagacacgtcgtggagttctatgtccatctcgtcccggccatttctgtcttccttccggaagcctcttcggaagttcgcaaccagtttccagacaaacgtgaggagggcatcattataggaattcttggcgatctgcagattccggtacacaagcgtgctgaagtggttggagaagagttcagtgaggacatcatgggtgagaaacttccgtaggttcaagccattctccagaaagaggcggacaaacttgggtctgtcctttatgagagccgtaaacatgacttcttgaaggtcagcagactcccatcggcggtcattggtgaaaatctcatcattggctaagtccagctggttccactccagcagaagcttcagctgcccattccagttatccttgtcttgctcactggtgctgaaggctttgtatagagcgtaggagatggcattgctcacaatttcatccccagcttcttccattttaataactgttaataggtgagaacattcgagaatttctttgagccatttgatccaactctcagtctcctcctcaggcagccgggacaccgtgcggggtaaaaagcgcaccagcttctccttgacggcagaagatgtcagggcatcctccacctccaccaggctagcgatcacatcagcgatctggcccgagccttccaccaccacacaaggaattttatttttgatggaggtattgatggctttcaaagtctcttttccacctccttgggcaaaacacacaatggggatcttgccaccatagttggaatcttgaatagtgcgctcagagatatacttctctagctgattccggagctttgcttcgacagtgggatgtccatgacagccattgtccacgagcagcaaatgtgtgtggttgttgtccaggatatacagtggatctcttgtgaagtcatccataaggtactgggctaaaaaatagccctcagcatcgcaattcctgatgagggtgtcccggttggagaccatgccccaagctgctatgccaatggccacaatattctcctctgaactcctgctgatggtgttatctctcaccacctccccgatgtacttcatcaggccataatgggtgcctcccgtgagaatccaagcacctttggactgcgcgatgtagatgagccggctgaagatcttgcgcatgcgcggcttcagggcgaagttcttggcgcccccggtcacagaaatgaccaggttgggtgttttcaggtgccagtgctgggtcagcagctcgtaaaggatttccgcgtccgtgtcgcaggacagacgtatatacttccctttcttccccagtgtctcaaactgaatatccccaaaggcgtcggtaggaaattccttggtgtgtttcttgtagttccatttctcactttggttgatctgggtgccttccatgtgctggctctgggcatagccacacttgcacacattctccgtggccttggaatctttggtaaagaagacacattctcgtttcttaaaatttgcttgaataaaattcaccaagtcgctttcactgtaagacaagtctgtgctccgagacgcgctggagtacagggtccgggtgctgtccagagtgtcattccttctgttcctcatgctgagcctggctgcccgaaaggacatcttttcctaagtgacggtttttgtcaagcaggattttctttcacccaaggatcctgctggtctctccccacaggaggaggaaagcttttataactg

SEQ ID NO: 12083 - RNA, 3966 nt, Homo sapiens
  source 1..3966: mol_type = other RNA
ctgaatagctgggactacaggtgttcagtaagataatctctccaattctataccattcccttcaccatccataatatttatttatttatttatttatttatttatttattttcagtcggagtctcactctgtcaccccggctggagtgcagtggtgcaatcttggttcactgcaacctccgcctcccaggttccagcaattcttgtacctcagccttctgagtagctgggattacaggagtgcaccaccacacccagctaatttttttatttttagtagagatgtggttttgccatgttggccaggctggtctcgaactcctgacctcaagtgatctgcccaccatccataatatttaaataagcatattgacttcttcttaaactaagggttaaatataatattttattttaatagttcaggttcatgtatctcatatcttatgctcaagttaataattcctatttgctatacatttatgaaaaagccttataaatggttttaataataaatagatattttaatatttaataataaatagatatttattggaatctaaccttggaaaattttcccaaatacagcaataggattcatgcacaaagatgctcatcccaatgatcaactggagatagccttcaatgagcaaaattatggtaatcgctagaggttgcctattatgcaattattgatataatgtttaagaaggctatgaatataataaaaacatatttgataaaatactaagtgaaaaagcttacataaaaagtatatatgtagtatgataacattctgtaaaattttgaaagagaattgagacatacatagaaaaaaaatagacttgaaaaaccatccagaaattgttagcagtgattaccttaaggtaatggggacaatttatgttctttctacatctctgtatggtctaaattttctataatagccagctattatttttaatggaaaaataataagaggagtatccaataagaacaaagtcagtagtgcctttcaaggttgcattttgggcgacttttcacatatttaggaatgggggtggttccttcaataggagcctggtgagtccaagagagcaagagactgccttgtcacctcctctgacaggtaagaagcatcctgagaaatgaaaacacttttcctgaagagagcggggtcctcttgctgcagcatgttttagaatctggcctaatttgagagacttttaacaatatgccaactaattagtcacataatacaaaaaagggaaaagtagagaatcaattggaaatgaacaaaataacaatacaggagtaaagcatgaccaggttcttattcataggatagatgttctcctatatatgtgttcatcaaaaataagattaaaggaaaaaggaggcggtaagaacacacttaaactatcaacctccagtcccaggcattgagacacagagagaaacaggcaccattctggagaaacacataaaggaaatattcttcctttatatccgtcttcaagtatgaaaccaatcacacactttattctcaaggtctcagcacactagggtgatttaaaatcatccaccatgtacccaggggtctgaaaatctctcatttagtagtcgatagcaaaattgttcatcagcattccttaatatgatctttgtatccagttgtctaaatcgatgcctcatttcctctgaggtgtcgttggcttttgtgttgatcttgacaaggtagttttccttcatgacaccctcccatgccagagtctcattgtcttcatttttgaaacagcagacagaagactccatgtttttctccttgcagcaacacttgaagcacttcttcaccaccatgtagaagtaagcgaagacgatgaaggggaaggggatattgaggcggctgcagtactcctgcaccaggaagtacctctggaacttccagacctggtcattgttctcctggacggtgcccaccgtgtagccaaacatggcgaccagcaggttgaccagcaggatgttggtggataacatgtagatgcacaccagggggatggtgatccactcggggaaccggggcaggttgtgctcatccagctccacacacagtggcttggactcattcccagtgaaggtgcagtgggcaaagtcatacgtggtaccatccacgtcactgggcacctggccgaacatggccaggtagggctcgtagatgaccgaacggaatatccacctccagcgctgctcattctgcctaaggatcccttgcctggccacgccaaaggccaccatccacaccgcaaagaggaacaggaagaagaacacatcgatcagcatcctctgcagcattataatcttgggtcctaagtttctgcttacagtaaaaatgtggatcaatcttagagtgaaaataatgtagtccagacagaaaatgactcgtccagaatacaaagagcttttattagaagagtggagccgaaatacaattcctgctatgaagtaaaaaagccccagcgtgtccatcacattccacaggtcagtaaaataattcaccccatttacgtaccactgtctcacttcatcacagaagaggacaaagaccagcgagtacaggaccagctcgggggggtgtggcaccgaatggaaatccatgagcagcacgtaggcaaacagcaggaggaaggcgatgtagaagaccacattccaggagaagaccacgaagggggaggtgaagaacgccacatagtaccaaagcagcttcttgtgcttgtcgacaggtttcttcctaaatgatacaaagccacagcccaccaagggtataataaacagacacaggataatcttccagttcttggtgtctcgggaaatctctccataccattgcttagaaagaaaattctggaccccaggctgggcgatgaaatgctggtctgtggcctccaccgccagctccagacagttgcttccaccccaagcttcacaggaatagaccagcagctgttctgccaagtcttcatcgctgctgtaacactcagtgaacagctcaacagcccgggtctcgtactcattagccagctcctcggactccccagcagcattgatgtcgttcttcactttggccagagtcttcagaagcttgctggctcccagggctgccagagtgcagcccctggtctgctcccaaatgactttggagagttccttcttattctgaagaatggcccagatgaagagagcttgcagggggtgccgagtaataggagacacgtcgtggagttctatgtccatctcgtcccggccatttctgtcttccttccggaagcctcttcggaagttcgcaaccagtttccagacaaacgtgaggagggcatcattataggaattcttggcgatctgcagattccggtacacaagcgtgctgaagtggttggagaagagttcagtgaggacatcatgggtgagaaacttccgtaggttcaagccattctccagaaagaggcggacaaacttgggtctgtcctttatgagagccgtaaacatgacttcttgaaggtcagcagactcccatcggcggtcattggtgaaaatctcatcattggctaagtccagctggttccactccagcagaagcttcagctgcccattccagttatccttgtcttgctcactggtgctgaaggctttgtatagagcgtaggagatggcattgctcacaatttcatccccagcttcttccattttaataactgttaataggtgagaacattcgagaatttctttgagctgtagtggagttccggatcagcttctcatttctgaattgcaatgagtccttgactacagtgagaataaagtattggttatacacgtatcaaaaagcccctatcaaaaagctgagagcctcatttgactagagatgtgtgcatctgcgtgcaggtgctgtgtgtgtgtgtgtgtgtcacaaagc

SEQ ID NO: 12084 - RNA, 1099 nt, Homo sapiens
  source 1..1099: mol_type = other RNA
ctgaatagctgggactacaggtgtttgccaccacgcccagctaattatattttttgtagagacggggtctcactatgctgcctaggctggtcttgaatttctgggctcaagagttctgcctgccttggcctcccaaactgctaagattacaggcgtgagctaccgcacccggcccgtattggattttatttatttccttttcttggtgctcatcctccttcacaacttcaagatgggcataagatgtttgacaacatggttcttcattaagtccaactccttatcataatagggcttgggaaatattaaacacgagggcaatcgtgctaacacaaaaatgggcgccccctaaaccttgttacttgtttgctcacttataagaagagccaactcaaaggctcaactgaattctagcactaagattccttccttgctgtagaagatctgtacctggtcacttccattaaagttacataggcgttccaagaagcctcctgcaatacagttgtgactcagccggtatgggagtaatgacggtcctgtggtatttcctgcacccccagagtcccagagtttgttaaggaccgtgtaagaggacaccacgctggcttttcagtgggcgcgtctctcctgggggcatcaccagacaaccccaggcggaagtggcggtggcccatcctcatgcaaactgcagtgtaagaactggggcccgggactcctcgcaaatgtgggacactgacattctgtgatgctgtcccaatgccctttcaaagcgctcagcccccaaattcccaaccaacagccatttcagggaggggctacccaggaccaggcttttgatgaaccacgactgttcggggtgccgtcttgggagagccacgtcagtccctctgagattccaaacggccgacagcggacacctcgggaccacatccaagcctcggggacctgtcaagacgccatcgacggtcctggaccaaatcccgcccgggaagggaagggtcgcgaccggaccctggagacccacggctgcctggcgatctgagcccaccccggcgctgccgtcccgcccccacttccgatcggtcgaaggtcacgt

SEQ ID NO: 12085 - RNA, 1529 nt, Homo sapiens
  source 1..1529: mol_type = other RNA
ctgaatagctgggactacaggtgtttgggactaccagctaattttgcttgtattttgtgtagagacagggtctcaccaagttgcccaggctagtctcaaactcctgagctcaaatgatctgtcagccttggcctcccaaagtgcttggattacaggcatgagccactgtgcctggctcgctcttcctctcttgaagcaaccaatgttattcgttttatgtggaccatcccagggctatcattattaattcaggtgtttatacaaggctctctgagaactcagttttaaagattacccaaagagtccctgcaacaatccagcctaaaacgatataaaatcagttttaatataactgaagtttttagattctgcctccaaatatcagattgtgacattttacctttctctgactttatgccaaatttacttcaacttctagcatctatcgttctcatttaggaacaaatatgtatttcacaaatgtggaaatacaaccatgagccaaacaaaaccaaatcctggacttacggagctgatggtagattccccaacataaccacttgattacagttttatgcaatgtgatgggagtaagggaccaccgtagggaggtcagaagttgcctctcagaggtggagactacagctgtcgtcagaaggatgagggttggaagaatcttcaggcacagagcaaagcatgagcaaaagctctgtggagtccaggaagctgagtaaatagggaataaaagaggccagtttggctgaagcagagagagcaggatggaattggtctgacctgtaagaagacatggagaggtgggcaaagcgcctggccattcagggcttggttagttaggaggttttgtctaagagaacgggaaggtgtttaagtggtttgggctgggaagtgacagggtcacattacattttgaaaaagccactctgcctgttgtgttgagattagagaggcgataaaggggatatgggtaaaccacaaggagactaggtcagtagtccctccacccccactccccaggtgaaggtagcctagactagggtggtgatggaggaggtagaagaggacagattcaaggaaaatttggaaggtaaaaaccagtaggatttgctgatggacggaatataggaggggaaaggtagattatcagggatgtatcttagttttcttatagaagatgtatttagttgcaatgcaattgttaattgaaattgactttaaataatggcacgacttaaaattatgcaaacatttgccttagataaaatttcaagttttcaaagtttttagctgggtagatggcatggctttacttcatatttcttggtatttcctaatcttgttaaaaaaaaagtttttctttttctcaaaggcttatttcagtggaagcccatctgcgaaatctgttataaatttaaattagaaaataaatacaagtgccattgacacgttggttattgtttttgcgagtgacctaaggccacctctcgcgggagctgggggctgccttccga

SEQ ID NO: 12086 - RNA, 1852 nt, Homo sapiens
  source 1..1852: mol_type = other RNA
ctgaatagctgggactacaggttcctgccaccatgtccagctaatttttgtatttttttttatagagatggggttttgcatgttgcccaggctagtctcaaatttctgggctcaagtgatttgcccaccttggcctcccaaagtgctgggattacgggcatgaaccactgtgcctggctcctctctctttctttttaatgtctcctagttattatcaataagaattggaaaaaatccaattttccttgtatagcctttcacagtgtagatatactttttctcatcagagttgcagagtgaaaagttcaaagcaaatatgtcagccaaagctcactttctgttctagctctgcctagagcaggctgcctgaccctggacaagttacttctcctgagccttggttttctcatcttttatttttatttttatttattttttagagatagggtctcactttttcacccaggctaaagtgcagcagtgggatcatagctcactgcagcgtcgaactcttgggctcaagcgatcctcctacttcagcatcctgagtccctgggattacaggtgcgagccaccactcctagttcaggttttctcatctttaggaagggagtggtcattcccacctgcaggggtggctgtgagggcaaaaatccagactgccctgcataaccaggacctcctgggaacgtctgggaaaatcagacagtgaggctccatcttgcttttgtcttctcttcctcattcctcgggcttgtatataactccctctgtgggcagaggaaggcccctgatagagggatgcaggcagacattgcactcagtgagcctgagaagatggggatagagagggctgcgtggggttggtgggaggaggaaccaggaccctccacccagtggttattttggagctagaagtgctgtgaccacttccgtccaggtctggcttgtgtcctgactgggagaccaggctgctggagtctgcatctcattttctttctgatttgcctctggtgttgttctgctgtgtgttggttttcgagggctgccataacaaagggccacatcctggatggcggtttgtttttctcactgctctggaggctagaactccaagatcaaggtgttgtgaggattgtttcttctgatgcctctctccttggcttgtagatgaccacaccctccctgagtcttcacatggtcttttctccatgcattcttctctgtgtcctaatctcctccttttataaatgcccatcataatggattagggcccactctaatgacctcgtgtcacctttattacctctgtaaagaccctgtctccaaatacagtcaaatactgaggtacgaggtgttaggccttcaacatatgaattttgcggggatgcaatttcgttcataacagacagctgggcaagttgcatctttggtcgtcttccctcaagagaggaaaagtggcttggttggcctactgagcctctttccttggagaggagttgaatcaggaggctgaaacagcgcaaatccctctctaaaccctcttggctttacccagagccaatgggtaatccactgcctgctctggggttcctggatgcttcctcttgcctcctcaagcctgcttttcagatctgggatctgctttgtttctggtggagaaataggtgtctactctgaaattacctctcctcgggactgttcaaatgtatttgtcttgtcttttgcagacattcctttaacagaaaagagctctcagccccgaaagatcccatgcagagggctcacctactgcaggataggagagccaaggaagttgccactctttttccattcaccccttccttcctct

SEQ ID NO: 12087 - RNA, 741 nt, Homo sapiens
  source 1..741: mol_type = other RNA
ctgaatagctgggactacaggttgcgtcaccacaccctggcagccacttccacagcccctggaactctggcccaaggctctctgattgactccttcccagatcttcttggcttagcggctgaagactgatgttgccggatcgcctcggaagccttttgtttcgttgttctgtcatccctttagtgtatggtacttgtttacttcttcaaagatggcctcttgtctaggcactggccaagtggtgctgtggaaaatctccaggacatctcagctgcatgagctaatttgtctcccatggacttgtctctcaatggcttggctgtgggccattccacatggctgaggggggctcacaattatggcagaaggcaaagaggagcaagtcacatcttacgtggatggcagcaggcaaagagagctggagcatagaaactccatcactttccacttctttcttcttcgaaagcagccatctgtgtccaagagaactatagaggcactagatgttgcactgttaagagctgagccaaagctgcacctcccttcctccagctacggaaggaaaataaatccttacttgtttaagccacagaggtcagtttttctgttattttcaacatagcacattcctaactaaaactatggtatttttatttcaagaagagaacatttaaatgttcggctttcagggatctcctgattagaagagatgactacgaactcccctttcaacctatcttg

SEQ ID NO: 12088 - RNA, 2650 nt, Homo sapiens
  source 1..2650: mol_type = other RNA
ctgaatagctgggactacaggtttgcaccaccacacccagctaattttttatttttaatagagatggggttttatcatgttgtccaggctagccttgaactcctgatctcaagtgatccacccgcctcccaaagagctgggattgacagcatgagccaccatgccaggccctgttccacaaattttaatacgtagcattttcattatcctttagtcccaaatatttctaatagccattcggaattctttaactcataggtaatttataagtgtgttttaaaaattccaaatatgaaatgccactgcactccagcctgagtgacagagcaagactctatctaaaaaacaaaaaaaaatagctcaaattttttttaatgacattgggatacggtcagataacgacactgattccttgaaatatcttaagacttcttttctggacaaagtaggtggtcagtttccatccatgttccatatatgcatggaaagagtatgtattcttttcagatactgttgtgtctgtctctcagctcaagctcatgctcacctcacatcctatctttcacagggctttttcatcagttgcctctgtctggtaacagtcacaccagctcctgttcagttacagtctttgtctcataaccggagagtttcatcaaaagaattttatttacagctttatcatccatatgccactaaaattcacctgttttctttcaacctgcactcattttgattgcctggaactctggatttaattcttccatcccactttgtatcttgcattcacttcactctctctccagcttttattctttctttctctttccctaggtccaatgcacttgacccaactcacatgcgtggactccgggaaggtactgctccctccctccaaattctgagcagtaaaatgccgccccggggcactggggaacagaaaggaatgagaccccaacaggcagaagccaagagagcggggaggagccatggcgttctgccccaggatgcaccacgcctggacgtgctcccccgactcccagtgccaggtgcccatatgccacacctcagggttgtcctctgttcgggtgagctgcggactaacgtggcccggcagcagaggccaccgtcttctgtcccgtggctcctgcgaacacaggcagtggggaacaggcagtgactgcccacccccaccgttcctcctccctgaccctgcaaacctcggggaagctttcaggcccgggaaagcagaccaggccccagtctccctcaccctttccctgggtctgaaggtcccggatcctgcgttcaaggatgacgctgaaactctctctttctcacatgggatctgtgatctgggccctcacaactcagcagagcaccactgtgtccccctcacatggagaggccgaggtctgtggagatcctgggacagagccagcgtcaaggactcagagggtgtcctggagtctcctaggacggaagacggcggccccaggtgggaaagactcagaccaggcctgcgcgctccaggtcctgcggcaggatgcggcccttcttgcgggctctgagcaggcggcgctcggcgcgggccgccttcttcctgcgcaggttctgccgccgccggtcctggcgctgctgcatcttctccaccacgccggccgtgcgcttctcccaccggcgctgccgctgcgccctgcgcttctccttgcgcttcagggcctcctgcagcaggcgttcgtcgtcacggatcttcacgccctccgccttgtagaggaggttggtccacttcatcttcgcctccagctcctgcgccttcccctcatcctggccgcgcagctcgtccagccggctctgccgtgcctgcaggcgctccagcagctgccggtagttcctcccggtcagcggcgtgaggttccccttcaccctctgcctcttctcttttctgcgctgcgccttgctggccggctcgtcttcgctcacctccaccttattgaagatcagcccgggcggctcccgcggctccgtgcaggccccctctggggttgcctccaccacctcctgggcctccgtggcctcctcagccttcctggccttctctttcgcccgcagctcctttcgcttcctcttcttccggtcccgttcctgctttctccgccgccttttctccaaggcggcaggggacagctccttggcactacctggccccgggcctcctggatcttctcatgcagtcgctgtcgcagaacatccagagcaaagacagactcaggctcagtggccaggccatctgcagggttccctgctgagctggaagcccaagctgcttcctctttggctgcctcaggcctcctggccccagaggctgctggagatttctcccccaaggacttggccttgtgctcagcagccttctcttctcgcttccggaatttcttttgtgttttcttccttttcttttttgggggccctgcagtttctgagccttgagttttgccagcccgcgtgcgcgcctgctgttccggggccgaatgggagcagatcttcttggccaggctctgcaggtaggcgtccttggcgagtagagaggccatggcggagacccgggccgttcacgactcacaccttccccgctgcgcgtgcgactctc

SEQ ID NO: 12089 - RNA, 2598 nt, Homo sapiens
  source 1..2598: mol_type = other RNA
ctgaatagctgggactacaggtttgcaccaccacacccagctaattttttatttttaatagagatggggttttatcatgttgtccaggctagccttgaactcctgatctcaagtgatccacccgcctcccaaagagctgggattgacagcatgagccaccatgccaggccctgttccacaaattttaatacgtagcattttcattatcctttagtcccaaatatttctaatagccattcggaattctttaactcataggtaatttataagtgtgttttaaaaattccaaatatgaaatgccactgcactccagcctgagtgacagagcaagactctatctaaaaaacaaaaaaaaatagctcaaattttttttaatgacattgggatacggtcagataacgacactgattccttgaaatatcttaagacttcttttctggacaaagtaggtggtcagtttccatccatgttccatatatgcatggaaagagtatgtattcttttcagatactgttgtgtctgtctctcagctcaagctcatgctcacctcacatcctatctttcacagggctttttcatcagttgcctctgtctggtaacagtcacaccagctcctgttcagttacagtctttgtctcataaccggagagtttcatcaaaagaattttatttacagctttatcatccatatgccactaaaattcacctgttttctttcaacctgcactcattttgattgcctggaactctggatttaattcttccatcccactttgtatcttgcattcacttcactctctctccagcttttattctttctttctctttccctaggtccaatgcacttgacccaactcacatgcgtggactccgggaaggtactgctccctccctccaaattctgagcagtaaaatgccgccccggggcactggggaacagaaaggaatgagaccccaacaggcagaagccaagagagcggggaggagccatggcgttctgccccaggatgcaccacgcctggacgtgctcccccgactcccagtgccaggtgcccatatgccacacctcagggttgtcctctgttcgggtgagctgcggactaacgtggcccggcagcagaggccaccgtcttctgtcccgtggctcctgcgaacacaggcagtggggaacaggcagtgactgcccacccccaccgttcctcctccctgaccctgcaaacctcggggaagctttcaggcccgggaaagcagaccaggccccagtctccctcaccctttccctgggtctgaaggtcccggatcctgcgttcaaggatgacgctgaaactctctctttctcacatgggatctgtgatctgggccctcacaactcagcagagcaccactgtgtccccctcacatggagaggccgaggtctgtggagatcctgggacagagccagcgtcaaggactcagagggtgtcctggagtctcctaggacggaagacggcggccccaggtgggaaagactcagaccaggcctgcgcgctccaggtcctgcggcaggatgcggcccttcttgcgggctctgagcaggcggcgctcggcgcgggccgccttcttcctgcgcaggttctgccgccgccggtcctggcgctgctgcatcttctccaccacgccggccgtgcgcttctcccaccggcgctgccgctgcgccctgcgcttctccttgcgcttcagggcctcctgcagcaggcgttcgtcgtcacggatcttcacgccctccgccttgtagaggaggttggtccacttcatcttcgcctccagctcctgcgccttcccctcatcctggccgcgcagctcgtccagccggctctgccgtgcctgcaggcgctccagcagctgccggtagttcctcccggtcagcggcgtgaggttccccttcaccctctgcctcttctcttttctgcgctgcgccttgctggccggctcgtcttcgctcacctccaccttattgaagatcagcccgggcggctcccgcggctccgtgcaggccccctctggggttgcctccaccacctcctgggcctccgtggcctcctcagccttcctggccttctctttcgcccgcagctcctttcgcttcctcttcttccggtcccgttcctgctttctccgccgccttttctccaaggcggcaggggacagctccttggcactgccctggccccgggcctcctggatcttctcatgcagtcgctgcagggttccctgctgagctggaagcccaagctgcttcctctttggctgcctcaggcctcctggccccagaggctgctggagatttctcccccaaggacttggccttgtgctcagcagccttctcttctcgcttccggaatttcttttgtgttttcttccttttcttttttgggggccctgcagtttctgagccttgagttttgccagcccgcgtgcgcgcctgctgttccggggccgaatgggagcagatcttcttggccaggctctgcaggtaggcgtccttggcgagtagagaggccatggcggagacccgggccgttcacgactcacaccttccccgctgcgcgtgcgactctc

SEQ ID NO: 12090 - RNA, 2651 nt, Homo sapiens
  source 1..2651: mol_type = other RNA
ctgaatagctgggactacaggtttgcaccaccacacccagctaattttttatttttaatagagatggggttttatcatgttgtccaggctagccttgaactcctgatctcaagtgatccacccgcctcccaaagagctgggattgacagcatgagccaccatgccaggccctgttccacaaattttaatacgtagcattttcattatcctttagtcccaaatatttctaatagccattcggaattctttaactcataggtaatttataagtgtgttttaaaaattccaaatatgaaatgccactgcactccagcctgagtgacagagcaagactctatctaaaaaacaaaaaaaaatagctcaaattttttttaatgacattgggatacggtcagataacgacactgattccttgaaatatcttaagacttcttttctggacaaagtaggtggtcagtttccatccatgttccatatatgcatggaaagagtatgtattcttttcagatactgttgtgtctgtctctcagctcaagctcatgctcacctcacatcctatctttcacagggctttttcatcagttgcctctgtctggtaacagtcacaccagctcctgttcagttacagtctttgtctcataaccggagagtttcatcaaaagaattttatttacagctttatcatccatatgccactaaaattcacctgttttctttcaacctgcactcattttgattgcctggaactctggatttaattcttccatcccactttgtatcttgcattcacttcactctctctccagcttttattctttctttctctttccctaggtccaatgcacttgacccaactcacatgcgtggactccgggaaggtactgctccctccctccaaattctgagcagtaaaatgccgccccggggcactggggaacagaaaggaatgagaccccaacaggcagaagccaagagagcggggaggagccatggcgttctgccccaggatgcaccacgcctggacgtgctcccccgactcccagtgccaggtgcccatatgccacacctcagggttgtcctctgttcgggtgagctgcggactaacgtggcccggcagcagaggccaccgtcttctgtcccgtggctcctgcgaacacaggcagtggggaacaggcagtgactgcccacccccaccgttcctcctccctgaccctgcaaacctcggggaagctttcaggcccgggaaagcagaccaggccccagtctccctcaccctttccctgggtctgaaggtcccggatcctgcgttcaaggatgacgctgaaactctctctttctcacatgggatctgtgatctgggccctcacaactcagcagagcaccactgtgtccccctcacatggagaggccgaggtctgtggagatcctgggacagagccagcgtcaaggactcagagggtgtcctggagtctcctaggacggaagacggcggccccaggtgggaaagactcagaccaggcctgcgcgctccaggtcctgcggcaggatgcggcccttcttgcgggctctgagcaggcggcgctcggcgcgggccgccttcttcctgcgcaggttctgccgccgccggtcctggcgctgctgcatcttctccaccacgccggccgtgcgcttctcccaccggcgctgccgctgcgccctgcgcttctccttgcgcttcagggcctcctgcagcaggcgttcgtcgtcacggatcttcacgccctccgccttgtagaggaggttggtccacttcatcttcgcctccagctcctgcgccttcccctcatcctggccgcgcagctcgtccagccggctctgccgtgcctgcaggcgctccagcagctgccggtagttcctcccggtcagcggcgtgaggttccccttcaccctctgcctcttctcttttctgcgctgcgccttgctggccggctcgtcttcgctcacctccaccttattgaagatcagcccgggcggctcccgcggctccgtgcaggccccctctggggttgcctccaccacctcctgggcctccgtggcctcctcagccttcctggccttctctttcgcccgcagctcctttcgcttcctcttcttccggtcccgttcctgctttctccgccgccttttctccaaggcggcaggggacagctccttggcactgccctggccccgggcctcctggatcttctcatgcagtcgctgtcgcagaacatccagagcaaagacagactcaggctcagtggccaggccatctgcagggttccctgctgagctggaagcccaagctgcttcctctttggctgcctcaggcctcctggccccagaggctgctggagatttctcccccaaggacttggccttgtgctcagcagccttctcttctcgcttccggaatttcttttgtgttttcttccttttcttttttgggggccctgcagtttctgagccttgagttttgccagcccgcgtgcgcgcctgctgttccggggccgaatgggagcagatcttcttggccaggctctgcaggtaggcgtccttggcgagtagagaggccatggcggagacccgggccgttcacgactcacaccttccccgctgcgcgtgcgactctc

SEQ ID NO: 12091 - RNA, 2186 nt, Homo sapiens
  source 1..2186: mol_type = other RNA
ctgcagactcgacctcccaggctcaaacaatcctcccacctcagcctcccaagtcgctgggactcccaggcacgtgccaccacacctggttaattttttattttttgtagagatggggtctcactatgtcacctaggctggtctcaaattcctgggctcaagcaatcctccaacctcagcctccaaaagtgttgggaatacaggtgtgagccactgcacccagcccccacccctttgccttttgctctctggtcacttcacctgtccaggcctcagtattctcatctgtaaaatgggagtgagaactcctgccctgatgacctaagtagggttttgtgagactcaaaggaatcagtggccagcatagagttttcagaggctaaaaatcactcgacaaatttaagagtgggtaattatcagcaattatggtgagtctgaagtcttctgttccagattctaagggcagtgtctggaaggctgaagtcctacctgctatgagaatgtggctggaggccagttagcttgaacctccagtgcgaccattctgcagactgacaggccgctgcctcctgcctcccagctcgcccctcctgctgcctgcctgtccctccttctttctgtcctgctttctggggaccagctttagggactgctgggtttccactttctccataactgcaaagccatgcaaaacaacacgaagggaggttgggagacacagctggggatgaggaaggggagtggggctgagtaggggtgacttggacatagacaccctggcttttggaaccaagggaaggtgggagacctagcaggacagaggtataaatagagatgcaaacgtacacggaacatgaagtcccctccgaaggtgggggtctgggtaccagcagggtctctgaggactgggagcttcttagattttcaaagggaagggaggctcccagcttctgcctttcctccctgaccccaccaagtttcacatttctcggaatttgcagggctccgatgggggccccaggggtcctcagagcccggcctcctgccggctggtgcaagcaggcacagtcggagatgggggtgctgggggagagtggtgagggatgttgtgcggggtcccactgggcagaaggcagcaggggcagtctcctggcctcccagcaggggtcccccgcccgcgcccccaggtgctccaggcccctcggggcagtcacacggagctcctgcgcttcatgaggccgcggaaggtggacaggctgtgcagacccgtggacaccgagctgatggcggagcgtggcgccccgctgcacaggcagcgtcgcgagggcgtgtcgctgtagcggccgccccctcccggcgacgagtggctctgctccacgcacgtgtcggacgtggagaggtcccgcgggatgatcatggggatggagtactgcagcttctcgcggctcttgtaccacaggcacgagcacatggactggaagtgcagcacctccgcgtagacgttgcggaagccgccgccgcccgctgccgccgtggatgaggcggtgtccgtagtgtgcgcgctgccaccccctccgccgccgcccgcctgcccgttgcgcgtgagcagcgcgcggtgctcggcgtcgcgcttctcgtcctcggcgttcatggtcatgaagcgcagcaccacgaggttgaggaaggcgccgatgaccgtgaggcccgtaaggatgtagacgaagctgaaggccacgtactgcggctgcgtctgcagggcctggtccttctgcagcgccacgtagtcgccgaagccgatggtggtgagggtgatgaagcagtagtagtaggcctggaagaaggtccagtgctcgtagtgggagaaggcggcggcgccgatgcacagcgtgctgatgcacgagaagaagccgatgagcaccatgttggccatggacacgtcggcgcgccgcatgcccagccccttcttggcgcggtgcagcaggtacctcaccaaggtgttgatgcgctcgcccaggctctggaacatgacgagcgtgagcgggatgcccagcagcgcgtagaacatgcagaacaccttgccgccatccgtgctgggtgccgcgtgcccgtagcccttcagatgtatttttaacttaatcctcaaaaacttcttacaaggtcactattatgattatcttcatattaca

SEQ ID NO: 12092 - RNA, 2549 nt, Homo sapiens
  source 1..2549: mol_type = other RNA
ctgcagactcgacctcccaggctcaaacaatcctcccacctcagcctcccaagtcgctgggactcccaggcacgtgccaccacacctggttaattttttattttttgtagagatggggtctcactatgtcacctaggctggtctcaaattcctgggctcaagcaatcctccaacctcagcctccaaaagtgttgggaatacaggtgtgagccactgcacccagcccccacccctttgccttttgctctctggtcacttcacctgtccaggcctcagtattctcatctgtaaaatgggagtgagaactcctgccctgatgacctaagtagggttttgtgagactcaaaggaatcagtggccagcatagagttttcagaggctaaaaatcactcgacaaatttaagagtgggtaattatcagcaattatggtgagtctgaagtcttctgttccagattctaagggcagtgtctggaaggctgaagtcctacctgctatgagaatgtggctggaggccagttagcttgaacctccagtgcgaccattctgcagactgacaggccgctgcctcctgcctcccagctcgcccctcctgctgcctgcctgtccctccttctttctgtcctgctttctggggaccagctttagggactgctgggtttccactttctccataactgcaaagccatgcaaaacaacacgaagggaggttgggagacacagctggggatgaggaaggggagtggggctgagtaggggtgacttggacatagacaccctggcttttggaaccaagggaaggtgggagacctagcaggacagaggtataaatagagatgcaaacgtacacggaacatgaagtcccctccgaaggtgggggtctgggtaccagcagggtctctgaggactgggagcttcttagattttcaaagggaagggaggctcccagcttctgcctttcctccctgaccccaccaagtttcacatttctcggaatttgcagggctccgatgggggccccaggggtcctcagagcccggcctcctgccggctggtgcaagcaggcacagtcggagatgggggtgctgggggagagtggtgagggatgttgtgcggggtcccactgggcagaaggcagcaggggcagtctcctggcctcccagcaggggtcccccgcccgcgcccccaggtgctccaggcccctcggggcagtcacacggagctcctgcgcttcatgaggccgcggaaggtggacaggctgtgcagacccgtggacaccgagctgatggcggagcgtggcgccccgctgcacaggcagcgtcgcgagggcgtgtcgctgtagcggccgccccctcccggcgacgagtggctctgctccacgcacgtgtcggacgtggagaggtcccgcgggatgatcatggggatggagtactgcagcttctcgcggctcttgtaccacaggcacgagcacatggactggaagtgcagcacctccgcgtagacgttgcggaagccgccgccgcccgctgccgccgtggatgaggcggtgtccgtagtgtgcgcgctgccaccccctccgccgccgcccgcctgcccgttgcgcgtgagcagcgcgcggtgctcggcgtcgcgcttctcgtcctcggcgttcatggtcatgaagcgcagcaccacgaggttgaggaaggcgccgatgaccgtgaggcccgtaaggatgtagacgaagctgaaggccacgtactgcggctgcgtctgcagggcctggtccttctgcagcgccacgtagtcgccgaagccgatggtggtgagggtgatgaagcagtagtagtaggcctggaagaaggtccagtgctcgtagtgggagaaggcggcggcgccgatgcacagcgtgctgatgcacgagaagaagccgatgagcaccatgttggccatggacacgtcggcgcgccgcatgcccagccccttcttggcgcggtgcagcaggtacctcaccaaggtgttgatgcgctcgcccaggctctggaacatgacgagcgtgagcgggatgcccagcagcgcgtagaacatgcagaacaccttgccgccatccgtgctgggtgccgcgtgcccgtagccgatggtggtgatgacggtgatggcgaagtagaaggagccggcgaagcgccactgcacgccggccttgtgcggcttgaggcgcagcacgacgcgctccagctcctcgtagccgccctggctgaggttgtagcgcgcccgcagctcctgctgccgcagctccagccgctgccgctcgatcagctcgggctccgactccagcgcgtcgaagaccgcggcgcccaccagcaggtaggtgaaggtgcacacgatgagcgccagcgtgcgcacgttctgccgcttcatcgtcccgcccgggccgccgccggccccccggcgcccccggcccgcgcctcggccccggccgccgctgctgctgccccggaggcggcctggggcatggctgcgctcgccgctctccgcgccgggcacccgctcagcgcccggggccgccgccgcc

SEQ ID NO: 12093 - RNA, 2222 nt, Homo sapiens
  source 1..2222: mol_type = other RNA
ctgcagactcgacctcccaggctcaagcaatcctcccacctcagcctccccagtagctgggaccacagatgtgcaccatcacacccagctaatttttgtattttttgtagagatggggtttcaccatgttgcccaggctggtcttgaactcctcggctcaagctatctgcccacctcagcttccgaaagtgcagtgattacaagtgtgagctgccatggctggccaaggctgtcttttaaaaagctaaagatgtgttggttcaagaccagtctgagcaatatggcgagacctcatttctactaaaaagaaaaaaaaaatcagctggctgtggtggcccatgcctgtagtcatcccagctacttgaaaggctgaagtgggaggatcgcttgaacccagaaggttgaggttgcagtgagccttgattgtgccactgcactccggcctgggtgacagtgagacctcgtctcaaaaagcctcggaaggagtggcctagggagatgagcaagcattttgtttctagtttctgaatggccctgtgcattgagagaggtcttcggcctcccagcctctctggctgaaggtggcgattctgcatggagtctctccaccacttggtggcattgctcacagtgacttcctacttctaaacaccattgaattggagcaagtagatgatttgccacatttttcccagctagtttggaggctgaatatagaattttactggggcacaccagaatgtgtacgttggggagcagcgatccccgttttccttgataatctgccgacagcttccttagtattgaaatcacaaagtcagaaatgcacacacctctatgatgagagatccatacagaagagagcaacaaaaagaggccttttaagtttgccagacttcctgaccagtgggaagcaagagagtagataagtgtgcaacaggcacaaacccaggcctataagaacctagttgggaacagaatgtaagagaatggggagcgatggggactctagtgtgttctgggcacgtgcccatctaaagtctccatgtgactgttgccctgcaggaatgtgggccccagtgttcaccaaacctttttgtttgtttgtttttttcccgtgaagagaagccagaaacccagatattgatacaaagtatccagtttagaagtgttggtagtttttttaattttgaacattgtgctgcccaaagaaggtatctgcaagccaggtacaaaccagcagttcatgccctctggtgagcagaaatgtcggaggtcgaattctagttctgctgttgcaacagctgtaaacgaaagtcttcagatttctaatgcccaatggaaatgccactttatttccaaaggttattaaaaggaatagttcatgtatgtaagtaggcacagagcttgccacctattaggtactcaaaagcattcttccttcacttaaggaaacaatacaggcataatacaacaataaagttacgatcaagttcattatcaggaggcatacacccaaacaataggggagtgagcacctaccacgtacagagctctctgctaggttctctgggggcagcagttcccaacctggcaattcatcggcatcgtcggaatcagccagcagcttgttggatatgctgagtccagagtcccgcccatattacacctaacgttctgtgcctattacacccagatttatgagatcctcctctcccatgcagtcaaagaatctgcattctaataagttcctcagaggaagctcttttgcagccagtttgcactggtctgtgggttggtcacttatggaaaccactgctccagggaatgaatcatgatttccagtctcattagggaaagatgatatgcatatgcacacatgtaaagaggagtgacagtaattagccaaaagctctgtggacataattgcctctgatgaagtgctgactgatgacatcagacagtaggctattgacagtgtaccccggggaaagctaaatgcaaaagagaagcgaactgcctcatgaagtgagatcaggattacacggtcagaaatgtggagagggtgattcagatggacaaaggagcagaggtaggattcaagtgatgtgtttcggaggcagtgcagcctgtttgtgctgagtggaaggtgcacgaggaacatagtagacggtaacatgaaggcaggagctgtgaaggcctttgaaggtcaggccagttgt

SEQ ID NO: 12094 - RNA, 2750 nt, Homo sapiens
  source 1..2750: mol_type = other RNA
ctgcagactcgacctcccaggctcaagcaatcctcccacttcagcctctgaagtctcttatatggtgtccaagaaatggggacaaatctcacaaagggactaggctcaggagggctggaatattcagggaagtttctttttttttttttttttgaggcagagtctcgctctgtcccccaggctggagtgcagcggcccgatcttggctggctgcatgctccacctcccaggttcatgccattttcctgcttcagcctcacaagtagctgggacgacacacgcccgccaccacacccagctaattttttgcatttttagtagagaatggtctgtgttagccaggatggtctcgatctcctgaccttgtgatccgcctgccttggcctcccaaagtgctgggattacaggcgtgagccaccgcacctggcctattcagggaaggtttcaagcagaaagatgaactgagttggctttggagagattcacaggactcccacaggcagagtgaaataagggcattgtagatggacaaaggcacagatgagcagcaatggggacagtgtgactgggggacgctgaggggctgctgtggctggaatggagggctgccaccataatggaaatggccaatgaggcaaataaggttggattaggagcatagcatcaagggtgccagcttattaaatccctcttccagtatgctagcactggcctgctgggaaaagtaatacatcacataatcaaacaaaaggcaaaaagaggcgagctccaggaataggcactgtaaacaggactcgccccagggtagccagatgcaggctttagatttgttgatgcaggttgagcatctctaatccgagggggaatgtctcatatggtgtccaagaaatggtgacacatctcacagagggcctaggctcaggagggctggagtatgagacattccccctcccctgtgaatttgaaaacgtggccaaaatttttttttaaaaatggctaccctgtagttctttaactggacctatttagacaacaccttacacactggagaaggatgatactatgtgaatctagtaagtctacaagacaatacttctctcttttggctgtcttcttcctctccagggtgatgacaactccgtgagggtggagattatatgtctctcatcatttaagcaacaaggaaataaattagtggcagagtaaggggtgactcagtgagtacatccaattgttgacatagttttgggtgggagaaattttgctattatatcaacttaacttcttaaaatagtctagtgggattaacttggttttatttcacagagacctcctggaagcgaggatcctttaacaatcctggaatatacattgcagtaaaagaacaaagcacacctcagccttaaatgacagaagaagaatgtcaagtgggaaagtgacgttggttttcagtttgtggattctgaatccacacaaacacaggattgtattttgaaaacctgaattaattattgtctttacctctataaaacaaaaaattataatcaaaattattagtatgacagtcacagatattgcgaagatgagtttgttcttatagtcatatcctggaacttctttcatgagctcacttgacttctgctctttctgttcattctgttccatgttctcattaatataatttgttttttgttggtccgtatcccattctacattcaatgcctttgcttcctgctgctcgctgagaagcttcatcaggaggcctgttcgcgacatgagcttggcacagctcccttgcacatgtgtttctgaacattccattttcaaggtccagataacatgagacatgaactttctcacatcctcgttggggatgagggaccgtagctgctcggttagctgaatttcaagctgatcacatcactctcgtcattggtgtctagctgctcactcccaaagcctgacaagttgatgccactgctgtctgagggcgcctccgactcaatagtcagctcagtgctcatgtgctgcttccgggcttgtaacatcttcatgaatgctccttctggattccctacagatgcttcttcagttgtctggtaaatcattatcaaataaatgactgcagtccacaacttgtcctcctgtgccgatttggtccctggactgaagacttactactgtcttctaactgtcctttggcccaagtttgcataaatccaacctctgataaccagtgtctttgaggtggttgatggcactggaaaaagacgaacacaacggagaaatccagcaccttgtttcttatggatcttcttgtgattccatacactgattgtaactgaatcagacttttcaatatacctattatattttaaaatgctgtagaacaaaagctgtttctaacgcttttcccctgcttctttcctgtatgcaggccttgaacgagcaggactcttgcagatttcacttcacctcctgggggaggcgatcgggttacctgccggctcctgctcttttcaggtgcagccaaggatagggagatgataacatcaggcccgagacgttgggagaatggagaagcgcttgcgagccaaaagtcctccaggagcacctgaaggaagcttcgcctgcacctgggacacccttccctgatgctggcctcaaggcaggcgcgccgcacacgcttccggtccatgacgaccacagctcagaagagcacgcgaacccagcctccacaaagagaaaat

SEQ ID NO: 12095 - RNA, 4582 nt, Homo sapiens
  source 1..4582: mol_type = other RNA
ctgcagactcgacctcccaggctcaagcaatcctcccatctcagcctcctgagtagctgggaccgccggcacgcaccaccacgcccagctaatttttgtattttttttttgtagagatggggtttcaccatgttgcccaggctggtctcagactcctgggctcaagcaatccactcgccttggcctccccaagtgctggaattacaggtgtgagccactgcacccgatcataatcccaactcgcagcatctgtgtggcctggggccagttccctccttcccagccttgcttcctgtgagttgggtgtggaggtgagtgtgcaacagctggcacatagcgcagtgagtgttgaatctgtgctggggccacagcagcccgagcttgtcactagcaatggcagggatggcactttccccagctaagtcagacctccctgcagcccaccctgcggctctgggcccagcctgctcctcctgggggagccgacgggtgtgagttgggggcacagagccccagccctgtgtggggctcctggaggctgcggacagacggggaagctgtgaaaggagacaccgccccgcccggccatgcagcctgcacccgggccaggccagggcccccagggcttccaccgtttcttgtggatgctggggattttcagctggaccatctcccagagaaggatactgaggccaggagaggctagagagcttggcgggtgcgctgggcccagatacgcggctcctgcctgcctcatggcctgctcctctgtcggggcctgtcaccgggaaaccccttttttagcagcgatgacgacactggaaccacgctagtctccgtccctcccgctcacatgcgcccacgctccccctcgaggcaggttgagccccggcctggaccgccccacgctgccttccgtccacgcagagcgggctcggccctcagggctttccttcgagtcgtgttggaaagaagcagaagcagcctcacccgtggggcggaggcgtctgagggtcaggaggcagggaggagagagggcctctgtggagccggctgcctggtgtccaagtccctgctctgtgacctcaggcaacttgctccgtctctctgggctcggtcgctgtcccagctggcttgagcgttgagcatgtcagtttcctggcacagtcctcggctggtctgagggggcatttggcggaaactgacttctcccctgtcctaaagtgcaggcctgaggtgttgctgacataggggctcagcccctgacacctcagcctctgccgcccggagcccaggcggtgtctgggtctccagaaagggagccctcggccacacaccctccaaacgcagatttgagcaacttgacccctatcggggtggccttccccacggcaagggcagagcaggcctagagcccagccagtgcccccagcctccagaaactgcccctcggcagcaggtccctggggacctgctgacagagtgagacacgggggccgcctggtgggtctattcctgtggggatccaataagacaggtgggcgtctttgcagccgtgcagggaggagctcagcctatcttatcaggcagccgggctgggccctgcagacccactggccttggatccccatgtcctcagcccaggaagcaagaggctgggagctggccctctctagcccggactccactggtctgtgcccgccctgctgagtccctcggagaccccaggtcccgctgttcctggtgaccgtggccatgggtggggggcagcacgggtgggagccgcggtcccggggtggtgcccactggagcttcctgtctgctctccacgcccagtgcctgagccccccaggccttgcccacttctgctgcccctgccccagcccccacccaacctgtgctgcgggccccagacacacagaactgactgccacctgcaggccgggtcaccgtactgtcccctgacgggccctgggcctggggggcgccctgcagtgacacccctcgccctgggccagccgtgtgtcctcccagaagcccccttagtccctgggcggctactgttcttgcggccgcgatttccgaggccacttgcacgcctccagcttcctgcgggcagggcacgcgtccgaggctcctcaaacccagggccccacctggcacgtggaggaagaagagaagggcaggaggcaggtgcccaggtgggagccccctctgtgccccctgggagtgtcccccccgcccaggtactcagggccctgccttcgtggccttgtccgctcgccgcgggtggggctggcacaaggcccgttttggaggaagtggaggctcccaggagaaaggcagtggctgtgatcgcacagcccaggctctgccctgcactgccctggaccacgaggctgcccaccccagacaggtgggacccctttcccgcatgcagactctgagcagcagcctcctgtgacccccaccgcgtcctgctcctcaggctcatgccctgcgggaacagaagccaagacccggtagaaaatccaaggtgtttaaatataaataagagcgattcccacagccccacggtgctggccagcctcacaggtgcccgctggttctgtgacccatcccaggcacacgctcccctggctgggcgcctggccagggctcccctgtggctggcgtgtggagacacgtgggcccttctccacgtgcccacgagggccgtagcaggctccaaggaggcccagccccggccagcctgtgtggaccccgccggcctgcggcgcccggagctgctgactgtgtcagagcccggctgcccagcgccccggcgcccctccctccagctgcccagcctgggatccgtccgctgtctgtctcctgaaccagggagtctgacccactcacagctcccatggggtccgtgcagccaaggccccgcagccacactcactctccgccccacagtggctcctggggctgatggctgggtgatcccagggggtccccaggctcttccgattggctcaggtgccctctcctgcggtggcgggcccacctgggtgcctgccagggccatcaggtgccctgaccccctggctggagggaggatgggaagtgggctccgagggcctcacaggtgggctctcaggagaggccccacctttggcaggagttggtgggtggggggaccctgttcttccccagaggcctgggcagcctgggtccctacagcactggcagcccaggcccccctacaggtcctccgaggggatcagcatccgcttctccaggctccggctcttcctgctcccgccggagccgccgctggggtgggtgccgggcctgggcgcctcgtgcgtggcctgctgcgtgtagtgctggtaggcgggggagaagttgtggatggcgtcctgcacgatgtcctgggggctcactgtctccctgatgccgctggagatgctctgcatgggtgccgggggggctggtgaattctccttcttctctgcgtacacctggcaggggaaggcataacgcagggccacggaggcgaacagcatctccacgcagatgatgaagttctggtagccggcggccagcgtgccagcccccagcttgttcccgccgctggtctccacctccgggatgaccccgcaccgctccaggatggccagcagcagcccttgccagaacgacaggaagatgacggctttgatggtgaggaacttgaggacgggctggaagggccgcaggagctccctggtggtgaagtagaagaggaacagggcgtagagggcgaggctgacggaggcgttgtagatgagggtcacatagaggtagccgctgcggacattgaagtccccgtcgtggtatttgccaaatgcctggaggatgatggtggtgacggccatgacgggcttcaccaggcagaactgcagagtggcctgcttacagaagcgcaggaacccgatggagtaggtcatgccccggaggcagcaggtgccgtacaagcagctggacttgatgggctttccacgaatctcagccatgatggcgccctcgcctcccaggtactggaaacacaggctcaggaagctgtaaatgacaaaggcttcgtagcagtcccgcacagagtcgaagtagacgtagtactggtggtctccgaggaggaggaggctgagccaggagtcgaaggcgtagatgggcacgatgaggagcaggcggatgatgtaacgttgctcctgtggcacggtgtaggagcgcaggtgcagatagatctggtggcaggtgagcaccagggcagtccacacgaagatccccgagacgcctcgggccagtgcggaggtgaggaagagccagggggccccctgggagctgttccccatgtggtccatctgcggcccagctggcacagccggtggggggctgggctgcggccagttcgctgacaccagggggacgccggctgtctccaggatccctgagacattactcatctttgctggcaggaagcacctggcccagtccagggaggcctggcctccagggaagcctagctggtcattctcatggccacgtggccccaact

SEQ ID NO: 12096 - RNA, 8017 nt, Homo sapiens
  source 1..8017: mol_type = other RNA
ctgcagactcgacctcccaggctcaagcaatccttccccctcagcctaccaagcagctgggactacaggtgcatgccatcttgcccagctcatttatttttttgtatagacggcataaccctgtgttaccccgttggtattacaggcatgagccactgcacctagccaggcatattggttttaaaagggttacaagaaacaagatgcacttttaggcctcctataatcctgcatttccaaagcatccatttagtcatctcatcaaaattttcattgatttaaataagttaatatgaacagactgacataattttactttaatgatgttgtttattgtcctaagccatccatacacaaaacgtttaatgtgttatggaaggctaacagtttttcagcttttctcaatactttcagccatccatacataaaatgtttaatgtgttatggaaggctaacagtttttcaacttttctcaatactatcagatgaatgtattcttaccaatcatgatttacgtttttcaaatgtggatttcttaggcctttgactgatagctttaggcttttgcactacacaaagaaaaagacacctttctattcatttcttaataatttgtttccataaagctaaaatgtccactgatgacataatctacctttggttaatcacagcaaatagttcacattttaaaggaatgcagatatttggatagaagcctctaacaatgtaaatattgtgcatttcaagttccatagtgtgtctaaccagggatagcaactgattatatgtggattaacaatagtgaataactgagcacatattaacatgaataacatacacagcagtcaaaacttactgtttttcatatgtgtaaagtaaaaattcaatctatctttaaccggctcatactgttttcatgttgttcaactatttgacacaaaaggagctttttcctttctttaaaaggattttgattcagtcataacagatttttgaaagtgacagtaaaattatgcatttggtccaggattaagagggaagttttgcttgctagtgtctatctggttagacatcagaataaaatgaatggactgtaaaggatcttataaccagtctctctctttaatatgaaggcccaacattacataattctttttaagagttgaccaggaatgaaatgtaacctcttttaaagatgaagaaaaactgaaaaaatgagattaagaaaatatgtgggtagtttacagctgctgatagaattgtgtgcacgcgtgcatgcatgcataaacacaaagtgaatctagaagggaaaaaattgagtttgatgaagtctaagatgaaaggttccatttcatgtaagattatgtgaccttggaaaaatttactggcttgctagtggaatacgtccttatatagggacttgaagagtttatctaaatagactgacttaaggatgcttttcctcttgttagacttgtatgacattactgagaagatttagagttctagaagtagagaagactgattagcttgtgcctgtgtatgaagaatgacaaattaagacaaaaggttatgtaaaccatttactaaaaaagtctaaatttttatattcctaggcccctacttatcttttacaaactttgaaggacctgaaattctttggacaccatcagatttagtttataagagttctgattttgaatcaagaaattattcatgtagttttaaaacacaattaaaattttcagtcaggctgaacttttgtgcacttcctcatttattcgagaaaccccaccactaatgtatttagaccttaatatgatggctttgagtcttaaatcattgtccacctaaaataatataccaaataaagatttttaaagtgctgcatatggtttctgtaagaggtacataattagattaccagcattatcctttagcttcaaaagtaaaactcatagtcaggattttactgatagtacaggaagaaaaaaaataaccactgttgaaaaataaatgaaaaaaattttattgagtattactttatacatgcaaattgaaagtgaatctatattaagttgactattccacaataaaaacctatgaaatgggaatgatcaaagctgtctaacacaatactaatgtgttcaataaattatccagatgtttttccacaaatatttggattacctgaattagctgattcttcagcaaaagttaaattttagctttaatatggtagcagcaggatgctacttaaatttagaagaaaaacataagaataaaaaccctgaatagcatagccaaatcttccaagaaataagttcaccaaaaaagtagcatacacctatttggtatccagaggaggaaacaaaacacaggcacttaatcaacatccaccaagtgatcatcactaacattctattattaccagagtaactgtcgatatgtgaactgtagattagaacagacttacatatctaaaaacaaaccagtaatcaataatatatacagaaatactaacttgaagtcacatttaaataccatcaacagtttggtgtatctgatataactgaattcatttcatcactgctataaattccttaaaagtgttcttttcctaattaacattatctttaaaaaatggtagatatttcccagtatgcatcagttttttcactccaccattcagtaaatgttgtagcaaattaaatagaacctattaactagatctaaaaacagtggctgaatacttaacacaaagaagtacttttgagtaaactattcagattagacaggctaatgctaagactgcattttgtgctactgacatgcactatatagatcgtacactactagatggaaagttggtccatgtccatttatttaaagattctgtaacacctgtaatagtatttaatacagctcccacatactatattcctctcacatagacatagttatttttagtggggataaggatatgactttaacatgctatgagattctagctaagtaaaataaaaacaatatggactcagattttcttaggagatattagttcaagtttttaaactgggaaacaatcaacttccatatatccaggagaaacttagcatggggggaggtgccttagttgatgtgcctgataagcaaactgttagttgtctattagtattatgttttcggcttaatgtaacaacaaaagaaagttgtcacactacctctcagataatatcaattacaatcttagagactgtaattgggaatacaatcctataacaagttattaacaatatcatgaatagttattaagtaagtgccagcactacatgcaacttactggtcaccaactcagaacccataaaactatacacatatgcacaaaaaaaaaactccaaagaaagatacctatcactgtacatatgaatactgtccaggatatcagatcaattatcaaatccaaggtctctgctgttttgtcttacagtgttgaatatatgaatgcttctctattacactgacttgtactattttcaagaaattaagtggattcaaaatcttacatttttatttctaattataaaatccagattaatccaaaaaacacaaaccacatgtaaccgaggtaggtttttcaccttaagaatacattgcttctaccacaattaaaaattttttaaactgaagaaaaaaaaaaactacattgctccacatacctgatacttaattttctatgtttgaaactacttgaacaagtgtgacagtgctaatctactatatttagtaaatcccttagtacctataaatacacacccaaaagcccttccctccttctctaatggtaactgttgtataataaaattgtcaacaactctagaaagatgaaataaagattactatagcaatcttcaattaattcatttcagaaatcaaggaggcaagtcatgttcattttaaagatgacaaacttactattttgaaaatgagctcataaatacattagaactttgaatgtgctttattatgccacaaattcccaggagatttaagaaatagtatttctgaacaggaataataatttcacaaatactaacactttattgacaatagacaagtcttttagggtagtgcacatgtacttaaaaactaccttctaccaatctcaacactttttataaattttcaggtgaaactgtagcagatcctactttatttttcaatggttagtgtaaaattctgtatgtaaaataagtacatattttgagatggaagaaggactgcatgtgaaatgctttgcctaagttgtaaggctcctgtctttacgctatcattaaaggccaaaaaaatcactgctagaaatgttccccaaaaaattcttaaacagctcagtctttaaaagtattaataatttttttttttttttttttggagacagagtttcgctcttcttgcccaggctggagtacaatggcgcaatctcagctcaccgcaacctctgtctcctgggttttcaagcgattctcctgcctcagcctcctgagtagccaggattacaggcatgcgccaccacacctggctaattttgtatttttagtagagacggggtttctccatgttggtcaagctggtctcaaactcccgaactctggtaatccacccgccttggcctcccaaagtgctgggattacaggcatgagccactgcacccagcctaataactgatataatttttttaagtgaaatgaaatgttcctttatttacatatgaattaaatagaaaattcaaagtaattcttttaataaaaacccatatactaatatattttaaggttggatactaacagcattttcacaagatccaaagtgtggatgacgaactaggcaataaggacatgtgtgccacataactaagggtaactaaaggaagatgagtacctcacaaccaaaagcagttaactatgcctggcataccaccctgtcatgtgggcagatcactgttcccatgctgggtaagagtctccaagaagggaagcccttatgcagtaattctgtaactatattaaatttggtaatctaacattaaactttttcgtgagcagtgaatatacacatggtcatatgaaaactgccctggagaccgggttaattattaaataaactaaaaggggagaaatgctgatagataaaattatgtcaattccagggtgttcaatggaataaagaaacagcagcagctgcttcaaaagtagactatgatcagaaacctcagatggtaacctttaaaaattgtggaatccagagtctcaacctaaacctacataggagctacagccagggagttctttctaagttcctcaagtgattctgatgattggccaagctggaaacttctgaactgggggagaaagccaacctaggtaaatgtagagacttttagaattcaacatttgattatcatttactccacattttcccccagctgtctcaccttctctatttttctaacagtgaacaataaaagggcttggcaagtgaaggaaaaagtcagtagagtacctaaaatggatttgactatattcaagccactttcatatattaactagataaaaggataccatactgctatttgaaattcaatcacaaagcaaaaatgtcataattttaatgtattttaagggaagacggggttcttaacatgaatatgtaatacaaaaacaattctaaataataatatttaatagaagaaaaaatctgtataattatttagaagtaactctgtttttaaaatttcaatgttaggaagaaaatcccttaaatttgaaatagcggaatattctctcatatgaaaaaactgtgtcccagtgttattcttcaacttagaaattaggcaaagtattttagtactatttctgcttacatattgttttgtatgaatgttttaagtatgaataatattttggtttttagtgtgcatgctaatataaaaatatggatttttttctcctacactgactttgtacactttccaggcccgaagaataaaaaacttttaaaatatcctgtgttcactagcaaaccttggaacgataaaaaaaggtagtacctacataagaaattttacattgaaattacaattgtatgtttttcaggagttaaagtgattcaatttttcaatattcaaacacaaaatagtaaatttttatttactatagcacaattcaagtattctcttaaatttatatttagtcaactaaaacatgacagtgactttataagagctttccttttaaaaggttgctgttataaaaaagtatgactctattactctaaatgcttagaataagtggaaagaacaaatgacagtagacaaaaacctttatgagtgagtcatcaacacataaaaggttgcacacatcagtaataggacatgtgaaggtaacatcccaaaagtatttgaactcatgtaaacaaagactatgtatattcctaagggagaaaatgtactaccaagataaaatatattcaaacggctgtgactttaaaccatgtattagttgaataccacacaaaaccaaaaaggcattatctatcatttaataactgaaagatattacttatttgtgagataaaaggataatgcttttttaaaaccaataatgaaaaagaagtattttgaaaacaaacatctgtttgctagaaataaatatacttgcttagttattttaatgtattgcagcataggaatattgtgctagcattgaccattaacattcaatcagtagtttaaaatattttttccacattgagtcttgaatcctctacctggtcagctgacccacaactttcaaaagagttttattttcctgctttagctgttcattttcatcttctatgtcatctaggtctctatttaataaatcaatttcttctttgagttttccaatcatttcctctttatcttgcatcagtctcacaagtcttaggttttcttgtctttctcttactacttccttttcaagatcttcaattttcttttccagtgtgctacttgaaaccagagtacctgaaacatttgcatccctgttatatctagggaacccacttctatctgttcgagaatatctacttgagacatcttcttcagagacactggttgtgcttttatatctgcctgaaactgttctaggtggctcctgtagcagataggaactgcctggatctagtaagtttacagcttcattctgaatagtgttctgttgtgtaattgcatcttctcgtttccgctctttctgccctgcttcatcatcttcgtactcatctaagcactctgcggcagggatgttgaccacgccggtggagcgccgcttctcccgcagcttcctcttctcgatctgccccttgcctttcctggcactggggcccgagctcttgcccttctctgggacgccgtccggctcctcctcgtcacgctggggcggcggtgcagccgaggcagaggcggctgggggctcgtcctccgaccgccgcgggccgggggccgcccgcgtcagcatggcggagccgaccgcgcagttcacgcccccgggaccggggacggcaggtgcggccggcgcgccgcccgggaggttgttgttgagctcgttggcagcggcggccgccggggtgcccagagcccccgcggggggcttcccagcggcgtcgctgctgccccctcccgggggggccgggcccggggggttctgcttggcgcgcatcttctcgcgtttcgccttccactcctccaggaagtctgtggtgctgccgccgaggccgctgctggtccggtagccaccggtcgccatattcccaaaggggccggtcgggctctcacctcaggccgcccaccagggctccggccgctgcctcctcttccttcctgcggccccgaggatgccaggagacgacctccaggagagggacggccgccgctcccacagcagccggcggggctacagtacggaccccgacgatcgcc

SEQ ID NO: 12097 - RNA, 8084 nt, Homo sapiens
  source 1..8084: mol_type = other RNA
ctgcagactcgacctcccaggctcaagcaatccttccccctcagcctaccaagcagctgggactacaggtgcatgccatcttgcccagctcatttatttttttgtatagacggcataaccctgtgttaccccgttggtattacaggcatgagccactgcacctagccaggcatattggttttaaaagggttacaagaaacaagatgcacttttaggcctcctataatcctgcatttccaaagcatccatttagtcatctcatcaaaattttcattgatttaaataagttaatatgaacagactgacataattttactttaatgatgttgtttattgtcctaagccatccatacacaaaacgtttaatgtgttatggaaggctaacagtttttcagcttttctcaatactttcagccatccatacataaaatgtttaatgtgttatggaaggctaacagtttttcaacttttctcaatactatcagatgaatgtattcttaccaatcatgatttacgtttttcaaatgtggatttcttaggcctttgactgatagctttaggcttttgcactacacaaagaaaaagacacctttctattcatttcttaataatttgtttccataaagctaaaatgtccactgatgacataatctacctttggttaatcacagcaaatagttcacattttaaaggaatgcagatatttggatagaagcctctaacaatgtaaatattgtgcatttcaagttccatagtgtgtctaaccagggatagcaactgattatatgtggattaacaatagtgaataactgagcacatattaacatgaataacatacacagcagtcaaaacttactgtttttcatatgtgtaaagtaaaaattcaatctatctttaaccggctcatactgttttcatgttgttcaactatttgacacaaaaggagctttttcctttctttaaaaggattttgattcagtcataacagatttttgaaagtgacagtaaaattatgcatttggtccaggattaagagggaagttttgcttgctagtgtctatctggttagacatcagaataaaatgaatggactgtaaaggatcttataaccagtctctctctttaatatgaaggcccaacattacataattctttttaagagttgaccaggaatgaaatgtaacctcttttaaagatgaagaaaaactgaaaaaatgagattaagaaaatatgtgggtagtttacagctgctgatagaattgtgtgcacgcgtgcatgcatgcataaacacaaagtgaatctagaagggaaaaaattgagtttgatgaagtctaagatgaaaggttccatttcatgtaagattatgtgaccttggaaaaatttactggcttgctagtggaatacgtccttatatagggacttgaagagtttatctaaatagactgacttaaggatgcttttcctcttgttagacttgtatgacattactgagaagatttagagttctagaagtagagaagactgattagcttgtgcctgtgtatgaagaatgacaaattaagacaaaaggttatgtaaaccatttactaaaaaagtctaaatttttatattcctaggcccctacttatcttttacaaactttgaaggacctgaaattctttggacaccatcagatttagtttataagagttctgattttgaatcaagaaattattcatgtagttttaaaacacaattaaaattttcagtcaggctgaacttttgtgcacttcctcatttattcgagaaaccccaccactaatgtatttagaccttaatatgatggctttgagtcttaaatcattgtccacctaaaataatataccaaataaagatttttaaagtgctgcatatggtttctgtaagaggtacataattagattaccagcattatcctttagcttcaaaagtaaaactcatagtcaggattttactgatagtacaggaagaaaaaaaataaccactgttgaaaaataaatgaaaaaaattttattgagtattactttatacatgcaaattgaaagtgaatctatattaagttgactattccacaataaaaacctatgaaatgggaatgatcaaagctgtctaacacaatactaatgtgttcaataaattatccagatgtttttccacaaatatttggattacctgaattagctgattcttcagcaaaagttaaattttagctttaatatggtagcagcaggatgctacttaaatttagaagaaaaacataagaataaaaaccctgaatagcatagccaaatcttccaagaaataagttcaccaaaaaagtagcatacacctatttggtatccagaggaggaaacaaaacacaggcacttaatcaacatccaccaagtgatcatcactaacattctattattaccagagtaactgtcgatatgtgaactgtagattagaacagacttacatatctaaaaacaaaccagtaatcaataatatatacagaaatactaacttgaagtcacatttaaataccatcaacagtttggtgtatctgatataactgaattcatttcatcactgctataaattccttaaaagtgttcttttcctaattaacattatctttaaaaaatggtagatatttcccagtatgcatcagttttttcactccaccattcagtaaatgttgtagcaaattaaatagaacctattaactagatctaaaaacagtggctgaatacttaacacaaagaagtacttttgagtaaactattcagattagacaggctaatgctaagactgcattttgtgctactgacatgcactatatagatcgtacactactagatggaaagttggtccatgtccatttatttaaagattctgtaacacctgtaatagtatttaatacagctcccacatactatattcctctcacatagacatagttatttttagtggggataaggatatgactttaacatgctatgagattctagctaagtaaaataaaaacaatatggactcagattttcttaggagatattagttcaagtttttaaactgggaaacaatcaacttccatatatccaggagaaacttagcatggggggaggtgccttagttgatgtgcctgataagcaaactgttagttgtctattagtattatgttttcggcttaatgtaacaacaaaagaaagttgtcacactacctctcagataatatcaattacaatcttagagactgtaattgggaatacaatcctataacaagttattaacaatatcatgaatagttattaagtaagtgccagcactacatgcaacttactggtcaccaactcagaacccataaaactatacacatatgcacaaaaaaaaaactccaaagaaagatacctatcactgtacatatgaatactgtccaggatatcagatcaattatcaaatccaaggtctctgctgttttgtcttacagtgttgaatatatgaatgcttctctattacactgacttgtactattttcaagaaattaagtggattcaaaatcttacatttttatttctaattataaaatccagattaatccaaaaaacacaaaccacatgtaaccgaggtaggtttttcaccttaagaatacattgcttctaccacaattaaaaattttttaaactgaagaaaaaaaaaaactacattgctccacatacctgatacttaattttctatgtttgaaactacttgaacaagtgtgacagtgctaatctactatatttagtaaatcccttagtacctataaatacacacccaaaagcccttccctccttctctaatggtaactgttgtataataaaattgtcaacaactctagaaagatgaaataaagattactatagcaatcttcaattaattcatttcagaaatcaaggaggcaagtcatgttcattttaaagatgacaaacttactattttgaaaatgagctcataaatacattagaactttgaatgtgctttattatgccacaaattcccaggagatttaagaaatagtatttctgaacaggaataataatttcacaaatactaacactttattgacaatagacaagtcttttagggtagtgcacatgtacttaaaaactaccttctaccaatctcaacactttttataaattttcaggtgaaactgtagcagatcctactttatttttcaatggttagtgtaaaattctgtatgtaaaataagtacatattttgagatggaagaaggactgcatgtgaaatgctttgcctaagttgtaaggctcctgtctttacgctatcattaaaggccaaaaaaatcactgctagaaatgttccccaaaaaattcttaaacagctcagtctttaaaagtattaataatttttttttttttttttttggagacagagtttcgctcttcttgcccaggctggagtacaatggcgcaatctcagctcaccgcaacctctgtctcctgggttttcaagcgattctcctgcctcagcctcctgagtagccaggattacaggcatgcgccaccacacctggctaattttgtatttttagtagagacggggtttctccatgttggtcaagctggtctcaaactcccgaactctggtaatccacccgccttggcctcccaaagtgctgggattacaggcatgagccactgcacccagcctaataactgatataatttttttaagtgaaatgaaatgttcctttatttacatatgaattaaatagaaaattcaaagtaattcttttaataaaaacccatatactaatatattttaaggttggatactaacagcattttcacaagatccaaagtgtggatgacgaactaggcaataaggacatgtgtgccacataactaagggtaactaaaggaagatgagtacctcacaaccaaaagcagttaactatgcctggcataccaccctgtcatgtgggcagatcactgttcccatgctgggtaagagtctccaagaagggaagcccttatgcagtaattctgtaactatattaaatttggtaatctaacattaaactttttcgtgagcagtgaatatacacatggtcatatgaaaactgccctggagaccgggttaattattaaataaactaaaaggggagaaatgctgatagataaaattatgtcaattccagggtgttcaatggaataaagaaacagcagcagctgcttcaaaagtagactatgatcagaaacctcagatggtaacctttaaaaattgtggaatccagagtctcaacctaaacctacataggagctacagccagggagttctttctaagttcctcaagtgattctgatgattggccaagctggaaacttctgaactgggggagaaagccaacctaggtaaatgtagagacttttagaattcaacatttgattatcatttactccacattttcccccagctgtctcaccttctctatttttctaacagtgaacaataaaagggcttggcaagtgaaggaaaaagtcagtagagtacctaaaatggatttgactatattcaagccactttcatatattaactagataaaaggataccatactgctatttgaaattcaatcacaaagcaaaaatgtcataattttaatgtattttaagggaagacggggttcttaacatgaatatgtaatacaaaaacaattctaaataataatatttaatagaagaaaaaatctgtataattatttagaagtaactctgtttttaaaatttcaatgttaggaagaaaatcccttaaatttgaaatagcggaatattctctcatatgaaaaaactgtgtcccagtgttattcttcaacttagaaattaggcaaagtattttagtactatttctgcttacatattgttttgtatgaatgttttaagtatgaataatattttggtttttagtgtgcatgctaatataaaaatatggatttttttctcctacactgactttgtacactttccaggcccgaagaataaaaaacttttaaaatatcctgtgttcactagcaaaccttggaacgataaaaaaaggtagtacctacataagaaattttacattgaaattacaattgtatgtttttcaggagttaaagtgattcaatttttcaatattcaaacacaaaatagtaaatttttatttactatagcacaattcaagtattctcttaaatttatatttagtcaactaaaacatgacagtgactttataagagctttccttttaaaaggttgctgttataaaaaagtatgactctattactctaaatgcttagaataagtggaaagaacaaatgacagtagacaaaaacctttatgagtgagtcatcaacacataaaaggttgcacacatcagtaataggacatgtgaaggtaacatcccaaaagtatttgaactcatgtaaacaaagactatgtatattcctaagggagaaaatgtactaccaagataaaatatattcaaacggctgtgactttaaaccatgtattagttgaataccacacaaaaccaaaaaggcattatctatcatttaataactgaaagatattacttatttgtgagataaaaggataatgcttttttaaaaccaataatgaaaaagaagtattttgaaaacaaacatctgtttgctagaaataaatatacttgcttagttattttaatgtattgcagcataggaatattgtgctagcattgaccattaacattcaatcagtagtttaaaatattttttccacattgagtcttgaatcctctacctggtcagctgacccacaactttcaaaagagttttattttcctgctttagctgttcattttcatcttctatgtcatctaggtctctatttaataaatcaatttcttctttgagttttccaatcatttcctctttatcttgcatcagtctcacaagtcttaggttttcttgtctttctcttactacttccttttcaagatcttcaattttcttttccagtgtgctacttgaaaccagagtacctgaaacatttgcatccctgttatatctagggaacccacttctatctgttcgagaatatctacttgagacatcttcttcagagacactggttgtgcttttatatctgcctgaaactgttctaggtggctcctgtagcagataggaactgcctggatctagtaagtttacagcttcattctgaatagtgttctgttgtgtaattgcatcttctcgtttccgctctttctgccctgcttcatcatcttcgtactcatctaagcactctgcggcagggatgttgaccacgccggtggagcgccgcttctcccgcagcttcctcttctcgatctgccccttgcctttcctggcactggggcccgagctcttgcccttctctgggacgccgtccggctcctcctcgtcacgctggggcggcggtgcagccgaggcagaggcggctgggggctcgtcctccgaccgccgcgggccgggggccgcccgcgtcagcatggcggagccgaccgcgcagttcacgcccccgggaccggggacggcaggtgcggccggcgcgccgcccgggaggttgttgttgagctcgttggcagcggcggccgccggggtgcccagagcccccgcggggggcttcccagcggcgtcgctgctgccccctcccgggggggccgggcccggggggttctgcttggcgcgcatcttctcgcgtttcgccttccactcctccaggaagtctgtggtgctgccgccgaggccgctgctggtccggtagccaccggtcgccatattcccaaaggggccggtcgggctctcacctcaggccgcccaccagggctccggccgctgcctcctcttccttcctgcggccccgaggatgccaggagacgacctccaggagagggacggccgccgctcccacagcagccggcggggcttggaggagcttgtaggggacgaggcgtagggctgggatccggctcccaggtgtgccgaagctggcgcgcgctcttccgccgcgcggaaagt

SEQ ID NO: 12098 - RNA, 2181 nt, Homo sapiens
  source 1..2181: mol_type = other RNA
ctgcagactcgacctcccaggctcaagcaatctccccatctcagcctcccaagtagcagggaccacaggcacgtgccaccacaccaggctgagggctacatagttttaaagatgactacttataacatttccaaaattttttcaagaaaagacaataaaatttaaagaaagtatactgtggatagcatgacttcaattaattatgaaaagtatgtaggcaaagctaaagactactgataaaccttaactaatctgatacgatttctaaaaactgaaataccatcagtaaacatgaagagaaagactttcccaagtacttaaacatatgttccaaaacactcagcaataacaaaggctaatgaaatattagatttaagagaaagctccaatacgagaaattctctttacctataggtaatcgattctttttatttgctggagtggttgctggagatagctgaggtgtattgtagggagtcatttctaaactgctactttttcctggcttggccgggggtaggtttgccaataaattgtcaagagccattctatcttctctcagttgatctccagacatcacactcttcataaaattcaccagagtaataagctgactgtaggttatataaaccacagttctgctcaatccttccagaagattgacggaagacaatggaggggtctccactgcacggcccccaatcacaacatcaaggaaagcggcaacacagcttttgtcaaactttccaaggctgctctttgttcggggatctccctcttcagagccagtcattgctaactgctgcaaaaggcggcctacctgcatcagattaaatcgtgctacttcattaataggagcatcggaaattattccatattgttctggattgacaactgcaggacaaatgaagcaggccaacaggagatcagtacacattgccctgacctccccaacttccagcctatctacacaggagagggttttgtacatctgagacacgatccaccttaaactatgtggaaaacaatatgtgttctgtttgagataaccaataaatttgttcaccaaagccactagctttgcttcattggactccaccatttcttgaactttttgcctgaatctatctgagcccttctctccaaagagtttttcctgctgagatggagagaacctctcaattagcttgtttggatctgtttccaggtgatcttcatcttcaacaagcagttgcataattggctcatgtaaagtggctgtgaggaaaagtttggcagaaaacagtccttcagaaaaaagtttaaataagatgctgaaggcacaagttcctctcctcaaaagtcgcctagggttgtcactttctttaagttcaaattcaatcaagtatcgcaaaacctgaaggaggtagctttcatcttcttgcatgatgcaattgccatacagggaggtaaaaactgtgtaaataacactttgtgtgttctcctgattaagtttctctccagcaaccaaagaggaggcaataagacgaggattttccctcaatcgactcaagaattctccataagcagtctcctgaaatcccaattgcttatacccatcaacaaattgtgtatcttccaaaattttggcatgttggcaacattcagcaggggaagcttcagcactggttatgataagccgatccaaattgattctctgttgcttcgcaatccatgctgtacgatacaacttttcagctgtcttaagtacatctgcattgagcctctgaatgagctgtttctcagagtttacatataagcgttcctgcttgaggtgatgagccagagtatgaatatctagtttcaccatcttcaatgtgggaaaggctcaaaggctgatcactgaatgccagctacttgggagggtcagatgggaggatcgcttgaacccgggaggcggaggttacagtgagctgagatcgtgtcactgcactccagcctgggtgacagagccagaccctttgagattcctagaatgtataaccaactctctccagtacacttaccccaagggggtcatgcgggggaggacacggaggactctgtcggaccgccactcggcctcggagccgtcgccctagccggtgactgcccccgccgccgctgccgccaccttcgccactcgcctgttggcttccctgc

SEQ ID NO: 12099 - RNA, 1982 nt, Homo sapiens
  source 1..1982: mol_type = other RNA
ctgcagactcgacctcccaggctcaagccatcctcccaactcagttcttttgccagttggcatccttttacttattcattgatgaatcccacatattcatttattcactctacagtggtgaaatctcttagaattattttcactaagtaataaaagttaacatcaccaagaatggaacacattgacactgtgtgtctctcgatgggataaaccacatgagttatgtggtattcctcccaaagatacataaaagatgaggtacatccaaattaaagaacactctacaaaataactgtcccggcgcggtggctcatgcctgtaatcctagcactttgggcagcagaagtgggaggatctcttgagcccaagagtttgagaccacactgggcaacatagaacaccccatctctacaaaaaataaaaaattacccgggcgtggtggcgcaggcctgtagtcccagctactcgggaggctgaagcaggagggtcccttgagcccaggagttcgaggctgcagtgagctatcatcgcgccactgtattccagcctgggcgatacagcaaagccctgtctccaaaaataaaaccaaaaaccaaaaaacaaaaccccaaaaaaactcaccaccaccaaaaaacaaaataagtaacctgtattctttgaaaatgtcaaggtcgggaacaggtaggatacacagaaaacaaataggtggaagatttaaatcgaaatattttagtagtttcattaaatgtacagaggagagtatgtgcctatcattgggagtctgagacaagataaaagcacggatctcataacaataaattactttgaaatcttctttcttgctcagtacaggtcccgccgccgcgccgcctggctctcgtattcctggttctcggcgggctgtggggcttccgcgccgcagccgttagtctcgtcgggtaggtgactccttcagcgagcaggcgcagcgacgagaaaggcctggcggggttgcgctgtcttcccgcccaccggaaggccctgaggagaagcctcgggccctgagggagggcttggggtcgggggcggccgctgccgccgccatgttgggctggaggtacgcacgctcccaacgctctctggctgcgctcccaacggtatctggctgcaaatcacggcgggagcgcctcgggcctcttgtcttttgaccctgtccttggaacccgaggagacttgccgttcccgggggagggtgtgtgtgagtcgggcggcggaggccgtctacgccattgtaggggcggggggagccgagattagagcatcagcctgagagaagtggtgcttctggttctccgctctgcctcgcatctttcagcgaggcctcgtacctcagttttcccatccgtgaagtggagctgggcctgcctgactcattcattcatcaggtggaggccttgacgctctaggagccctttcaaaggactttgccttacacgaaatagtacctatcgttattcactctgcagtaaccacccggatttgagtggcgggtgtttgcacagtaattcagtttcctcttcaccctcctgccattcgtcttcccctccagtttatctcattgacactcacacagcttccactcacacctgcgatcacaaggcagcatcttcgggccctcgtcggccacgatccgctcccagagagcattcgcgcacaatcttatcccatccacgattttgattccttttctcccacttcttcaaccctatccgggacgagaccatcaggtcccacctccaccttcaccttcattttccgcgcaatgcagactgagccctggactcacccatatacagattgaattgtccggtcagtgtttcatcccctctgcattctgagggcgagttagcatctgggtgcatgagttccaaactaacagccaggaccaggcttggagccaagaatcctttggctcgcatcgtggctgggttgaccgcttttct

SEQ ID NO: 12100 - RNA, 1753 nt, Homo sapiens
  source 1..1753: mol_type = other RNA
ctgcagactcgacctcccaggctcaagccatcctcccaactcagttcttttgccagttggcatccttttacttattcattgatgaatcccacatattcatttattcactctacagtggtgaaatctcttagaattattttcactaagtaataaaagttaacatcaccaagaatggaacacattgacactgtgtgtctctcgatgggataaaccacatgagttatgtggtattcctcccaaagatacataaaagatgaggtacatccaaattaaagaacactctacaaaataactgtcccggcgcggtggctcatgcctgtaatcctagcactttgggcagcagaagtgggaggatctcttgagcccaagagtttgagaccacactgggcaacatagaacaccccatctctacaaaaaataaaaaattacccgggcgtggtggcgcaggcctgtagtcccagctactcgggaggctgaagcaggagggtcccttgagcccaggagttcgaggctgcagtgagctatcatcgcgccactgtattccagcctgggcgatacagcaaagccctgtctccaaaaataaaaccaaaaaccaaaaaacaaaaccccaaaaaaactcaccaccaccaaaaaacaaaataagtaacctgtattctttgaaaatgtcaaggtcgggaacaggtaggatacacagaaaacaaataggtggaagatttaaatcgaaatattttagtagtttcattaaatgtacagaggagagtatgtgcctatcattgggagtctgagacaagataaaagcacggatctcataacaataaattactttgaaatcttctttcttgctcagtacaggtcccgccgccgcgccgcctggctctcgtattcctggttctcggcgggctgtggggcttccgcgccgcagccgttagtctcgtcgggtaggtgactccttcagcgagcaggcgcagcgacgagaaaggcctggcggggttgcgctgtcttcccgcccaccggaaggccctgaggagaagcctcgggccctgagggagggcttggggtcgggggcggccgctgccgccgccatgttgggctggaggtacgcacgctcccaacgctctctggctgcgctcccaacggtatctggctgcaaatcacggcgggagcgcctcgggcctcttgtcttttgaccctgtccttggaacccgaggagacttgccgttcccgggggagggtgtgtgtgagtcgggcggcggaggccgtctacgccattgtaggggcggggggagccgagattagagcatcagcctgagagaagtggtgcttctggttctccgctctgcctcgcatctttcagcgaggcctcgtacctcagttttcccatccgtgaagtggagctgggcctgcctgactcattcattcatcaggtggaggccttgacgctctaggagccctttcaaaggactttgccttacacgaaatagtacctatcgttattcactctgcagtaaccacccggatttgagtggcgggtgtttgcacagtaattcagtttcctcttcaccctcctgccattcgtcttcccctccagtttatctcccatatacagattgaattgtccggtcagtgtttcatcccctctgcattctgagggcgagttagcatctgggtgcatgagttccaaactaacagccaggaccaggcttggagccaagaatcctttggctcgcatcgtggctgggttgaccgcttttct

SEQ ID NO: 12101 - RNA, 1953 nt, Homo sapiens
  source 1..1953: mol_type = other RNA
ctgcagactcgacctcccaggctcaagccatcctcccaactcagttcttttgccagttggcatccttttacttattcattgatgaatcccacatattcatttattcactctacagtggtgaaatctcttagaattattttcactaagtaataaaagttaacatcaccaagaatggaacacattgacactgtgtgtctctcgatgggataaaccacatgagttatgtggtattcctcccaaagatacataaaagatgaggtacatccaaattaaagaacactctacaaaataactgtcccggcgcggtggctcatgcctgtaatcctagcactttgggcagcagaagtgggaggatctcttgagcccaagagtttgagaccacactgggcaacatagaacaccccatctctacaaaaaataaaaaattacccgggcgtggtggcgcaggcctgtagtcccagctactcgggaggctgaagcaggagggtcccttgagcccaggagttcgaggctgcagtgagctatcatcgcgccactgtattccagcctgggcgatacagcaaagccctgtctccaaaaataaaaccaaaaaccaaaaaacaaaaccccaaaaaaactcaccaccaccaaaaaacaaaataagtaacctgtattctttgaaaatgtcaaggtcgggaacaggtaggatacacagaaaacaaataggtggaagatttaaatcgaaatattttagtagtttcattaaatgtacagaggagagtatgtgcctatcattgggagtctgagacaagataaaagcacggatctcataacaataaattactttgaaatcttctttcttgctcagtacaggtcccgccgccgcgccgcctggctctcgtattcctggttctcggcgggctgtggggcttccgcgccgcagccgttagtctcgtcgggtaggtgactccttcagcgagcaggcgcagcgacgagaaaggcctggcggggttgcgctgtcttcccgcccaccggaaggccctgaggagaagcctcgggccctgagggagggcttggggtcgggggcggccgctgccgccgccatgttgggctggaggtacgcacgctcccaacgctctctggctgcgctcccaacggtatctggctgcaaatcacggcgggagcgcctcgggcctcttgtcttttgaccctgtccttggaacccgaggagacttgccgttcccgggggagggtgtgtgtgagtcgggcggcggaggccgtctacgccattgtaggggcggggggagccgagattagagcatcagcctgagagaagtggtgcttctggttctccgctctgcctcgcatctttcagcgaggcctcgtacctcagttttcccatccgtgaagtggagctgggcctgcctgactcattcattcatcaggtggaggccttgacgctctaggagccctttcaaaggactttgccttacacgaaatagtacctatcgttattcactctgcagtaaccacccggatttgagtggcgggtgtttgcacagtaattcagtttcctcttcaccctcctgccattcgtcttcccctccagtttatctcctgcgatcacaaggcagcatcttcgggccctcgtcggccacgatccgctcccagagagcattcgcgcacaatcttatcccatccacgattttgattccttttctcccacttcttcaaccctatccgggacgagaccatcaggtcccacctccaccttcaccttcattttccgcgcaatgcagactgagccctggactcacccatatacagattgaattgtccggtcagtgtttcatcccctctgcattctgagggcgagttagcatctgggtgcatgagttccaaactaacagccaggaccaggcttggagccaagaatcctttggctcgcatcgtggctgggttgaccgcttttct

SEQ ID NO: 12102 - RNA, 1202 nt, Homo sapiens
  source 1..1202: mol_type = other RNA
ctgcagactcgacctcccaggctcaagcgatctccccgcctaggcctccagggtagctgggaccacaggcacgtgccaccacacctggctatttttctgtttgttttgttttgtattgttttgttttgttttgtagagacagggttttgccatgttgcccagaatggtctctaactcctgagctcaagggatcctcctgtctgggcctcccaaagtgctgggattacaggcgtgagccaccacacctggcctttttttttttttttctctcaaaatcgcatcacacgcagcacaggggtcccttagtctctgcatttcaccgaaggtcggagattttccttgattgtcttttcccgtggccaacatcagggctggtggctttaagagtcctgggggacacttttctcttaaggatctggtagctttcactccattgtctcaggcattgacggttgcatgagaagttcacggttgtcctgattattaagatcttcggaaatcatctaagtttgaattttttctatttttagatggtggttgaccgcaggtaactgaaaccacagaaagcaaaactgcaatgtgggggggctgcttgcatgctcctttcagacccatgtcaccccaagtcatggggcatttccagtgagcacatacagacttaggaacccgggagaaagcctggaggctagaaaagctgagaccacagtcagctgggctgcagatctttgctccgccttcctccagacagcacaagtgactcagccctccccagggtgctgcttctcgctctgacaccacgatttggcctcctctcactcacaactctatctcctctctgtgtcattcctcctactcagggccgatagtcaaaatatcaaaccactaataaagcatgggcacctgccagtcagactacacaccagctgggaacaatggctagaggtagcaaattgccccaaaacttagtggcatgaaacaacaaacatttgttacataacacactaatgggtcaggagtttgggtggttctggctcagggcctctcatgaagttgtcagcatgtcagagttggaaccatttgaaagcttggctggggctggaggatcctctttcaaggtgtctcattcacaaggctgtcggcagaaagccgcagtgcctccccagtgtgtgggcctctccatagggctgcttgagtatcttcac

SEQ ID NO: 12103 - RNA, 7575 nt, Homo sapiens
  source 1..7575: mol_type = other RNA
ctgcagactcgacctcccaggctcaagggatcctcccacatcaggctcccgagtagctgggactacaggtgcaagccaccacctctggctaatttttgaatttttctgtagagacgggtttcaccatattacccaggctggttccgaactcctgaggtcaagccatctgcccacctcgacttcccagtgttgagattacaggcgtaagccaccatgtccagccaattcttacttgtttttatcctttttaaatgtatataaagctcatattaatctcaatgtttaattttagaagtgttttgggtctttattagaaatttggtagtgtttttgtaaccagaaatatatgccatagggacttaactcttatttatatcagttcacctatggtaaaattgatttcattatatgttgtttttcttaaactcgcagtttcccagaacctatcaacaacattgaggacttattgtattataaattatctttatatgaatataaagactttccctatttcaattgcgaatatacagatctgtgcactcaaaaataacaagcctattaggactcaaacagttatttgtatacccacgttcacagaagcattattcacaatagccaaaaagcagaagcaacccagtgtccattaatggatgaactgataaacaaaatacggtatttacatactacggcatatttggcctttaagaggaaagaaattctaatacatgctacaacatgaatgaactttgaagacattatggtaaatgaaataagaatgaatccatttagatatccagagtagtcaattcatagagactgaatgctggttaccagaggctgaggagagaggaggtaatgggtggttattgtttaatgaatacataatttcagtttgggaagatgaagagttctgtagacggatggtggtggtggttgcacaatagtatgaatatacttaatgccacagaattgaacacttaaaactggttaaagtggtgaattttacgatatgcatatttaatcacaataaaaaatgcttattaaaagatgtactagttatgaaatagcatacctcatctgtttcaaactgggtgtggctaacaatgaggtagaaaagcagcaagcaggtacagagatttataatggctgctctaggtcctatcgggtaaagggatcagcagatgtgaagtcaagagtctcctgtaagatttgactttcttggaaacatattttaatcctgggcctcctctttccaaatcacctatttcttttagtctttttgcagtgatactgtgtgttgcttctaacagaggttcagtttcacagcctttccctcaagtgtcttatcctaaaagtaaaacctagatgatctaaggtggtggttttcaacagggtgcaattttgcctcctatactcgcaacacccagggacagttggctatgtctggagacatttttgggttgtcacaactggaagtagggtggggagtggtgctaatgacatcaagtgggcataagccaattatgctgctagaaatcctacaatgcacaggataggctcccacaaacaaagacttaaccaaccccaaatactaacaatgcttggtttgagaaaccctgttctaaggtttttctaagttgcttgatttatggtagaaactgatcataagttaaaagtttcctccttttggattgcttgagcccaggagtttgaggctatggtgcattatgattatgcctgtgaatagtcactgtaatctagccactgcaatctatattaagaaacataggccgggcgcagtggctcacgcctgtaatcccagcactttgggaggccaaggcgggtggatcacgaggtcaggagatcgagaccatcctggctaacacggtgaaaccctgtctctactaaaaaaaaacaaaaaaaattagctgggcgtgctagcgggcacctgtagtcccagctactcaggaggctgaggcaggagaatggcgtgaacccgggaggcggagcttgcagtgagccgagatcgcgccactgcattccagcctgggtgacagagcaagactctgtctcaaaaaaaaaaaaaaaaaaaagaaagaaaagaaaagaaaaaagaaaaaggaaacatagtgagaccctgtttctttaaaaaaaaaaaaaaagtttcttcctcttattccttactttctcttctcatttattttgaggaaataggataagaaccagtggtaatactttaggtgaaaggaggctacttatgttatcattctcttcaccctggccgatcctaaccatgacactttatatcctgggggatggtgaaaaacagaggaggtggggtaggacttgtggtcaaattgttggggacagaggcaaaaaagaaaacagcaacaaaaaaatacaaatgaagaaattggaaggcagtgcctatgccatctgaattggataattcttcctaatggccatttggatatagatgagttggacagacataatttagaaacctatataaggaaatatcatgcattttaatgaggttataacccaaaatttaaaattcaattaaaaaattaaatcacagattttcccacaacatactaattcaacatactacttacgattacttaaaatttgcattttttctaaggagcaataacctaatgagtatgtaatactaatgtgtcagttaataagggcaattacttttgctcttattttcctgttatatgaaattaacaacatacctgctgcaatataactcatttggtacaatttaggtgtttcgagaaattcaacccactaagatcattagcgtaattcatttttatgctacacattaaaatggtgccttcttacagtcactttggaaaactgtttgacagtaaatactaaaactgaaaatatacacaccctacaacctggcaattccattcttaggtttatactcaatggaaatgtatacactcaccaaaagacatgtataagaatgttctacacagtactattcataatagctcagaattgaaaaattctcaaaagactattaatgggagaatgaataacttttggatgtaatgaaaaatggataaacaaacggaagactatacagcaatgagaatgaatgaactacaaatacatgcaacaataagaatggatctcactttggcaggttgaataacggcctccaaagatagccagcgtatgaatccctggaacctgtgaatgtcacttatatggcaaaagagattctgcagatgtgattaaattaaggatcttgagatagggggattatccctgctttatgcaggtgagccctaaacttagaggcagggaaagatctgactacagaagagaagatgatataatgacaaaagcaagctttgatcatagagaggaaggggtcacaagcccataaatacaggccgtcactggaagccaaaaaagggaagaaaacattctccctcacaacctcaataaagagccaaccctgctgatactttgatttaggcctaatgaaactgatttttggacttctgatctccaggactataaaagaataaatctgtgttgttttaagtcactaagtttgtggtagtttgttacagtggcaacaagaaactaaaatattcacaaaaatgatgaatgaaaaaaagtgtattatgtatgattacatttacataaaataaaaaacaggcaaaactaatctatgattttagaagtcaggatagtaactttcagcaagaaagaagacagtgttaagatggggaaagaggagggcttctggggtacacataatgctctgtgttttgatctgaagactagtatgtgagtttgtttaatttgtgaaaacctttatttgtgtactgttttgtgtgtgtgtggtatatgcagttttaaaaactgatgccttttaaacacttactaatctgataatctgccgaaaaagaatatataacatatattcaaggggatggaaaaatacttactgaacaataattttatttctcaagaacgctgaagattttgtttctctcttcaaaagatttaaaaaattttaactggcaaaacataatagtgactcttaaatgctaaaaaaaaaaaaaaaaaaaaaaaaaaaagaaaaaacctaaaaataaaatattgcataagtaagctttgttatgcctcgatcttaggactgtaaattataaaaatacaagtaaaaccacattttttgaaataacagtaaacaaaaacaaaaggcaggtactacataccaaatgaccaaaatgtcttttgggcctaagattcttgaaaatagtaaaaatggtaataatagaaatctctctatagaacattaaatataaaaaccatttataaaacacatcacaattttattgcttgaagaatacagcatatgaaatcacaagaatgtcaaaatgaaaagtcactaggcttcaaacgtataatacattatcagatgcagtaaaatattaacctgaactctgcatcagaaaaaaaaaaaaaggtgtggaaaatatctaagttgtttacttaagaaacagatatacttaaaatagaaagtataaggatgttacagtacaaattagaaaagccaacacgtattaacttatcgttctagactagactacctttggtacttaaactttttaaaaaacaatttcttctatctcatccaaatgcacttcatgggtatgacatccatgaagtaacttcaacttaaaacattcagcaaaattaaccttttcacttcatgggggaagtatatttaataaatgtataacaatatttcccttttactaaaactgcaaaatatgatcattaagaaacctaacagttataaaactttacttacttagctctccaattaaaattggaatcctgggagccacaatctatttttgggcttggtgaatacataagtttaaaagatttggcaactgacataggaatttaattacttaatactatcttaagtgacttttcctttctgtttccaaaatatagacattatgccatttcttcaacatcctggattcctataaacactaccatactgtatttattagaaccaaattaaagcttctctaacaagcaggtagaaactatttatgttccatatacggctgataagttataacacaacttatgtttcatatagggctgatcagttaattcatatagggctgatcagttgtaacataacttcttaagcaaaactaatcttttttttaaagctatcactcaattatggagacaataatgtcatctcaaaaggtaatgttggactctaggccatctagttgggaaaatgtaaaagtaattctaaaaacaataagtaaactataactacaagttaaattaaaaatccctctctcatagcaagcatgctcattaactttcatttctttcccccagcaaaggtttgaatattcataaacctcagttaaaccaagagaaccaatgtaattgtttcaaaagtaccacctatatatttgaataatatgagtatggatggactaggtaagtaatactatcaacaattactgaattggagtgaaagagtaaaaatcatgacagacttccaaactgggcagtctttgaaatgtcatagtggagctcaaaatgaattatgctgtaataaaactatagtttttacctctacacaaaacagaaacaaaataaaaaaacataaccaccaaatttatacaaatactattaaacatactccttcctagtttttgaatgtcttgaagtttttctaaacaagtatattgatctgagcatatatatttattgcctatatatgtactcattttaaaagacaaattcagatactacagaactgaactctttcaccaacccaatccaatgtctactgattcacacagcaccccccccttaataatttaaaattcacaagttttagtttagttaaaagggcagaggaaatgcaaatgcagatttagagctttgtagaaatttcactgtatttttataaacttgaagttatctgtaacactgtttattgatcaaacgaaggactcgctgctatctaaaatttcataaacaccattaaaaattcaaaattgatattatactgaaccttaaattttcaatagttcaaagagacagtttttacatgtatagcacacaatagatgaaacttaatagcagacatccctagaataccaatgacaagtccaccaagatgcatacaaaattacagataagcatttctttcactgtttttgttgtgcagggaaaaacatttatagaagaaatagaaactcagctggtgaatttcagatatcatcatcatcttcttcatcctgagaagatcccgcctgattagatgcactggctgaggcagcagcaagctgggcttgttgggcagcttgctgcatttgaagccattcctgttgggccaattctgcttgttgctgtctagcttttgcaaataattcttgttgctgtctcaataactcttcttcaggaatgccaaggttttccaaacgagaactggcctttcttctttttaatgctactgttttacactcttgcaagacttcttttacttcactgatgtaagagccaaatcccaaactttctagtgcttgtatgacatgctctggtgagatggtcttcttttccgatttgttacaaatctcattggcttcagaagatataaggtgaatgaattcagtgcagcagttcaccaccagctctcgagcatcgttggccacccggacattaggaagagtctctttgatcattttattgatagcagctctggggatagtgagatcatcatcgttgccagacgaggaagccatagtaccttcctgtttctcgcgccccggcttttaaaaactccccagctctggtccactactccaccgagatttctcaaaaagtcgccctcggagagtgatcccggggggtgctttgcgaagagggtgcagaaaatgaacggaggagcagctggcttgagggctgggaacactcgcgtgtgtgagagatttaggatgagtttgggaagaaagtgggggcccgaggattctagagagagcacagcccaggctgaggaggggaaagcgcggtggtccggaaatttgagcggctggggaaccaccttcgtgtctcctcagaggggcgggcgctgtcgcctaactggtccccaacggcgtcggagcagaggcaagatccaggggcactggcctcgccgcggtaccgggcgggtacccagcgggctcggctctatagagcccgaggccccgctgccgctgccgccgccgccagcagccgttgccgccgcctcggccaaaccatccttcagacacccgcgccgccgcctcacaacatgtccgccgctgccgctgccgctgccgctgctggaacggcgacggccgcctgggaactaatatggacagagccaggcacagtgggagtcgcagtggctgccgccgtggccgcgtagcccgaacgcagatcgtggaagccgaagacgcggcaacggtggtccctccagatgccagggaaggtttgcaggaagccgctcccgacaccctttgc

SEQ ID NO: 12104 - RNA, 2174 nt, Homo sapiens
  source 1..2174: mol_type = other RNA
ctgcagactcgacctcccaggctcaagtgatcctcccatttcagcctcctgagtagctgggaccacaggcatgtaccaccacacccagctaattttttttttttttttttttggtagaaacaggatcttactatgtggcccaggctggtctcaaacttctggtctcaaagcaatcttcccatcttggcctcccaaagtgctgggattacaggcatcagccacctcacctggccaacctgtatttttctttcactgcatttcctgagtctgtaattattattattatgttttaaagagatgaagtctccctctgtcacccagtctggcatgcagtggtgtgattgtagcttactgctaccttgaactcttggactcaagtgatcctgctgcctcagcctcctgagtagctagagctgttagcacataccaccatgcccagctaatgtttaaaattttttgtagagatagggggtctcactatgttacctaggctggtttcaaactctggcctcaattgatcctcccaccttggcctcccaaagtgctgggattacagtcatgagctgccacaaccagcctgtaattatgttgttactgattttctgtcagttaattacctttagcctggaataccacgctcaccattgattgctaagcacctggagccatgtctgcacacaaagggtgctcaataaacactccttaaatgaggaatgcaggagggagtgaggaccagggccctggcaggaagcagaggacaggacagtagctggctttggctctggccacccctttgggactagagttctgttgactggataacctccaggctcctccacgtggggccctgggcccgcctggggaagttgagtctgtgtaattccttggagatctcttggaaggtcttgcctttggtctcaggaaggaacaggccagtgtagatggccccacagacacagacaccaaggaaagggacatagaggaagtgggacaaggcctccatgataaagggaaatcccaggccgaccaggatgagcatgatccacatgagcgccccgcagaccatgcaggcagcaggcctggccatctggtcaaacagctctgtggccaggatccccgtcactccggcagggccaatgccaaagctgaggatgaaggcaaagatgcaggccatggccaggtagagtgtccaggggaaggagctctgcaggcacagggccacagtgaagatgctcccccagcaggtcatcaggctgtacccaccgatgagcagcacgcgccgacccaccctctcgattaccacacaactaacaaccgccgtgagcagctcgcagctcccagtcccgatgatcgcgtactggatcttcgcttccggcactcctgccttccggaacacggaggaggcgtaggcgtacaccgagtcattcccgcagagctccatggcactgcccagaaccacgaggcttgtcacctgtctcctcagggcccgatgctggaacagctcccatgggcgccgggcacggcagccctggcaggcagcgcgctcctcctccagctcctccagctcccctgccaagtccccggagccccggagccgccgtagtgctgagtccgaccacctgtcccatcacgatccccagagccgtaaagatggctgagctcatggccacagctcctcggagctccttaggggcgctctcccccaggtacatgggctggatgttcatgctcacacctgcattgactcccacgagcagtcttcccagcatgatcatctcaaaggagcctgctttgcggctgaatccaaacaggattgctgctgacaccacaaagatgttattcaccaggagggacttcttcccagcgtgatggccaagggacctgcaagcagtgctccaaagaggcctcccaggggatacagagacacgatgagggaccacataagcaggactaggtgatcgggcagtggctctccagtacgcgcctgccatgtctcattggtgaattcctgaatgtgcaaggtcggggcattgatgatagagaggttatagccaaactgaaaagtcccaccaatgccggcagcgcagatggtcaggagcaggatcctgccctgaatcagtcttcggagcgctctcatctgtgcgtcctgggcagagcgagagacttggcggaat

SEQ ID NO: 12105 - RNA, 2327 nt, Homo sapiens
  source 1..2327: mol_type = other RNA
ctgcagactcgacctcccaggctcaagtgatcctcccatttcagcctcctgagtagctgggaccacaggcatgtaccaccacacccagctaattttttttttttttttttttggtagaaacaggatcttactatgtggcccaggctggtctcaaacttctggtctcaaagcaatcttcccatcttggcctcccaaagtgctgggattacaggcatcagccacctcacctggccaacctgtatttttctttcactgcatttcctgagtctgtaattattattattatgttttaaagagatgaagtctccctctgtcacccagtctggcatgcagtggtgtgattgtagcttactgctaccttgaactcttggactcaagtgatcctgctgcctcagcctcctgagtagctagagctgttagcacataccaccatgcccagctaatgtttaaaattttttgtagagatagggggtctcactatgttacctaggctggtttcaaactctggcctcaattgatcctcccaccttggcctcccaaagtgctgggattacagtcatgagctgccacaaccagcctgtaattatgttgttactgattttctgtcagttaattacctttagcctggaataccacgctcaccattgattgctaagcacctggagccatgtctgcacacaaagggtgctcaataaacactccttaaatgaggaatgcaggagggagtgaggaccagggccctggcaggaagcagaggacaggacagtagctggctttggctctggccacccctttgggactagagttctgttgactggataacctccaggctcctccacgtggggccctgggcccgcctggggaagttgagtctgtgtaattccttggagatctcttggaaggtcttgcctttggtctcaggaaggaacaggccagtgtagatggccccacagacacagacaccaaggaaagggacatagaggaagtgggacaaggcctccatgataaagggaaatcccaggccgaccaggatgagcatgatccacatgagcgccccgcagaccatgcaggcagcaggcctggccatctggtcaaacagctctgtggccaggatccccgtcactccggcagggccaatgccaaagctgaggatgaaggcaaagatgcaggccatggccaggtagagtgtccaggggaaggagctctgcaggcacagggccacagtgaagatgctcccccagcaggtcatcaggctgtacccaccgatgagcagcacgcgccgacccaccctctcgattaccacacaactaacaaccgccgtgagcagctcgcagctcccagtcccgatgatcgcgtactggatcttcgcttccggcactcctgccttccggaacacggaggaggcgtaggcgtacaccgagtcattcccgcagagctccatggcactgcccagaaccacgaggcttgtcacctgtctcctcagggcccgatgctggaacagctcccatgggcgccgggcacggcagccctggcaggcagcgcgctcctcctccagctcctccagctcccctgccaagtccccggagccccggagccgccgtagtgctgccaggcaggcctcggtgtctccacagtcaatgaggaggtagcgcgggctttcagggagcagaggcagggaggcgagctggagcgccccgggcaccaggcagctggccagcagcaggggccaggcctgagggccacctaggagctccctgagtccgaccacctgtcccatcacgatccccagagccgtaaagatggctgagctcatggccacagctcctcggagctccttaggggcgctctcccccaggtacatgggctggatgttcatgctcacacctgcattgactcccacgagcagtcttcccagcatgatcatctcaaaggagcctgctttgcggctgaatccaaacaggattgctgctgacaccacaaagatgttattcaccaggagggacttcttccttcccagcgtgatggccaagggacctgcaagcagtgctccaaagaggcctcccaggggatacagagacacgatgagggaccacataagcaggactaggtgatcgggcagtggctctccagtacgcgcctgccatgtctcattggtgaattcctgaatgtgcaaggtcggggcattgatgatagagaggttatagccaaactgaaaagtcccaccaatgccggcagcgcagatggtcaggagcaggatcctgccctgaatcagtcttcggagcgctctcatctgtgcgtcctgggcagagcgagagacttggcggaat

SEQ ID NO: 12106 - RNA, 2424 nt, Homo sapiens
  source 1..2424: mol_type = other RNA
ctgcagactcgacctcccaggctcaagtgatcctcccatttcagcctcctgagtagctgggaccacaggcatgtaccaccacacccagctaattttttttttttttttttttggtagaaacaggatcttactatgtggcccaggctggtctcaaacttctggtctcaaagcaatcttcccatcttggcctcccaaagtgctgggattacaggcatcagccacctcacctggccaacctgtatttttctttcactgcatttcctgagtctgtaattattattattatgttttaaagagatgaagtctccctctgtcacccagtctggcatgcagtggtgtgattgtagcttactgctaccttgaactcttggactcaagtgatcctgctgcctcagcctcctgagtagctagagctgttagcacataccaccatgcccagctaatgtttaaaattttttgtagagatagggggtctcactatgttacctaggctggtttcaaactctggcctcaattgatcctcccaccttggcctcccaaagtgctgggattacagtcatgagctgccacaaccagcctgtaattatgttgttactgattttctgtcagttaattacctttagcctggaataccacgctcaccattgattgctaagcacctggagccatgtctgcacacaaagggtgctcaataaacactccttaaatgaggaatgcaggagggagtgaggaccagggccctggcaggaagcagaggacaggacagtagctggctttggctctggccacccctttgggactagagttctgttgactggataacctccaggctcctccacgtggggccctgggcccgcctggggaagttgagtctgtgtaattccttggagatctcttggaaggtcttgcctttggtctcaggaaggaacaggccagtgtagatggccccacagacacagacaccaaggaaagggacatagaggaagtgggacaaggcctccatgataaagggaaatcccaggccgaccaggatgagcatgatccacatgagcgccccgcagaccatgcaggcagcaggcctggccatctggtcaaacagctctgtggccaggatccccgtcactccggcagggccaatgccaaagctgaggatgaaggcaaagatgcaggccatggccaggtagagtgtccaggggaaggagctctgcaggcacagggccacagtgaagatgctcccccagcaggtcatcaggctgtacccaccgatgagcagcacgcgccgacccaccctctcgattaccacacaactaacaaccgccgtgagcagctcgcagctcccagtcccgatgatcgcgtactggatcttcgcttccggcactcctgccttccggaacacggaggaggcgtaggcgtacaccgagtcattcccgcagagctccatggcactgcccagaaccacgaggcttgtcacctgtctcctcagggcccgatgctggaacagctcccatgggcgccgggcacggcagccctggcaggcagcgcgctcctcctccagctcctccagctcccctgccaagtccccggagccccggagccgccgtagtgctgccaggcaggcctcggtgtctccacagtcaatgaggaggtagcgcgggctttcagggagcagaggcagggaggcgagctggagcgccccgggcaccaggcagctggccagcagcaggggccaggcctgagggccacctaggagctccctgagtccgaccacctgtcccatcacgatccccagagccgtaaagatggctgagctcatggccacagctcctcggagctccttaggggcgctctcccccaggtacatgggctggatgttcatgctcacacctgcattgactcccacgagcagtcttcccagcatgatcatctcaaaggagcctgctttgcggctgaatccaaacaggattgctgctgacaccacaaagatgttattcaccaggagggacttcttccttcccagcgtgatggccaagggacctgcaagcagtgctccaaagaggcctcccaggggatacagagacacgatgagggaccacataagcaggactaggtgatcgggcagtggctctccagtacgcgcctgccatgtctcattggtgaattcctgaatgtgcaaggtcggggcattgatgatagagaggttatagccaaactgaaaagtcccaccaatgccggcagcgcagatggtcaggagcaggatcctgccctgaatcattctagatcgcaggagggcgtggagcattcgaaagaggggcctgagcggaggtcttgctgtcccagggagaccccggctgccattagcaagcggtgagccggcagcctgtgcgcggagggaagggcagcgcgcagcgcccagtggtgaaagag

SEQ ID NO: 12107 - RNA, 2438 nt, Homo sapiens
  source 1..2438: mol_type = other RNA
ctgcagactcgacctcccaggctcaagtgatcctcccatttcagcctcctgagtagctgggaccacaggcatgtaccaccacacccagctaattttttttttttttttttttggtagaaacaggatcttactatgtggcccaggctggtctcaaacttctggtctcaaagcaatcttcccatcttggcctcccaaagtgctgggattacaggcatcagccacctcacctggccaacctgtatttttctttcactgcatttcctgagtctgtaattattattattatgttttaaagagatgaagtctccctctgtcacccagtctggcatgcagtggtgtgattgtagcttactgctaccttgaactcttggactcaagtgatcctgctgcctcagcctcctgagtagctagagctgttagcacataccaccatgcccagctaatgtttaaaattttttgtagagatagggggtctcactatgttacctaggctggtttcaaactctggcctcaattgatcctcccaccttggcctcccaaagtgctgggattacagtcatgagctgccacaaccagcctgtaattatgttgttactgattttctgtcagttaattacctttagcctggaataccacgctcaccattgattgctaagcacctggagccatgtctgcacacaaagggtgctcaataaacactccttaaatgaggaatgcaggagggagtgaggaccagggccctggcaggaagcagaggacaggacagtagctggctttggctctggccacccctttgggactagagttctgttgactggataacctccaggctcctccacgtggggccctgggcccgcctggggaagttgagtctgtgtaattccttggagatctcttggaaggtcttgcctttggtctcaggaaggaacaggccagtgtagatggccccacagacacagacaccaaggaaagggacatagaggaagtgggacaaggcctccatgataaagggaaatcccaggccgaccaggatgagcatgatccacatgagcgccccgcagaccatgcaggcagcaggcctggccatctggtcaaacagctctgtggccaggatccccgtcactccggcagggccaatgccaaagctgaggatgaaggcaaagatgcaggccatggccaggtagagtgtccaggggaaggagctctgcaggcacagggccacagtgaagatgctcccccagcaggtcatcaggctgtacccaccgatgagcagcacgcgccgacccaccctctcgattaccacacaactaacaaccgccgtgagcagctcgcagctcccagtcccgatgatcgcgtactggatcttcgcttccggcactcctgccttccggaacacggaggaggcgtaggcgtacaccgagtcattcccgcagagctccatggcactgcccagaaccacgaggcttgtcacctgtctcctcagggcccgatgctggaacagctcccatgggcgccgggcacggcagccctggcaggcagcgcgctcctcctccagctcctccagctcccctgccaagtccccggagccccggagccgccgtagtgctgccaggcaggcctcggtgtctccacagtcaatgaggaggtagcgcgggctttcagggagcagaggcagggaggcgagctggagcgccccgggcaccaggcagctggccagcagcaggggccaggcctgagggccacctaggagctccctgagtccgaccacctgtcccatcacgatccccagagccgtaaagatggctgagctcatggccacagctcctcggagctccttaggggcgctctcccccaggtacatgggctggatgttcatgctcacacctgcattgactcccacgagcagtcttcccagcatgatcatctcaaaggagcctgctttgcggctgaatccaaacaggattgctgctgacaccacaaagatgttattcaccaggagggacttcttccttcccagcgtgatggccaagggacctgcaagcagtgctccaaagaggcctcccaggggatacagagacacgatgagggaccacataagcaggactaggtgatcgggcagtggctctccagtacgcgcctgccatgtctcattggtgaattcctgaatgtgcaaggtcggggcattgatgatagagaggttatagccaaactgaaaagtcccaccaatgccggcagcgcagatggtcaggagcaggatcctgccctgaatctgcgtccgaggccgtaaggacggctccagttcatcctccatccgcctctgccgcagcactgaggctgaaaagccgctcactccttactcggctaagccccaagctcatctcagtcttcggagcgctctcatctgtgcgtcctgggcagagcgagagacttggcggaat

SEQ ID NO: 12108 - RNA, 2648 nt, Homo sapiens
  source 1..2648: mol_type = other RNA
ctgcagactcgacctcccaggctcaagtgatcctcccatttcagcctcctgagtagctgggaccacaggcatgtaccaccacacccagctaattttttttttttttttttttggtagaaacaggatcttactatgtggcccaggctggtctcaaacttctggtctcaaagcaatcttcccatcttggcctcccaaagtgctgggattacaggcatcagccacctcacctggccaacctgtatttttctttcactgcatttcctgagtctgtaattattattattatgttttaaagagatgaagtctccctctgtcacccagtctggcatgcagtggtgtgattgtagcttactgctaccttgaactcttggactcaagtgatcctgctgcctcagcctcctgagtagctagagctgttagcacataccaccatgcccagctaatgtttaaaattttttgtagagatagggggtctcactatgttacctaggctggtttcaaactctggcctcaattgatcctcccaccttggcctcccaaagtgctgggattacagtcatgagctgccacaaccagcctgtaattatgttgttactgattttctgtcagttaattacctttagcctggaataccacgctcaccattgattgctaagcacctggagccatgtctgcacacaaagggtgctcaataaacactccttaaatgaggaatgcaggagggagtgaggaccagggccctggcaggaagcagaggacaggacagtagctggctttggctctggccacccctttgggactagagttctgttgactggataacctccaggctcctccacgtggggccctgggcccgcctggggaagttgagtctgtgtaattccttggagatctcttggaaggtcttgcctttggtctcaggaaggaacaggccagtgtagatggccccacagacacagacaccaaggaaagggacatagaggaagtgggacaaggcctcctgcggattaaaaaagaccccaagaccatgataaagggaaatcccaggccgaccaggatgagcatgatccacatgagcgccccgcagaccatgcaggcagcaggcctggccatctggtcaaacagctctgtggccaggatccccgtcactccggcagggccaatgccaaagctgaggatgaaggcaaagatgcaggccatggccaggtagagtgtccaggggaaggagctctgccgtggacggggcgggggtgaggtggaagtcagcccggcctggaccccccagccctcatccaccccagctacactaacaaccgccgtgagcagctcgcagctcccagtcccgatgatcgcgtactggatcttcgcttccggcactcctgccttccggaacacggaggaggcgtaggcgtacaccgagtcattcccgcagagctccatggcactgcccagaaccacgaggcttgtcacctgtctcctcagggcccgatgctggaacagctcccatgggcgccgggcacggcagccctggcaggcagcgcgctcctcctccagctcctccagctcccctgccaagtccccggagccccggagccgccgtagtgctgccaggcaggcctcggtgtctccacagtcaatgaggaggtagcgcgggctttcagggagcagaggcagggaggcgagctggagcgccccgggcaccaggcagctggccagcagcaggggccaggcctgagggccacctaggagctccctgagtccgaccacctgtcccatcacgatccccagagccgtaaagatggctgagctcatggccacagctcctcggagctccttaggggcgctctcccccaggtacatgggctggatgttcatgctcacacctgcattgactcccacgagcagtcttcccagcatgatcatctcaaaggagcctgctttgcggctgaatccaaacaggattgctgctgacaccacaaagatgttattcaccaggagggacttcttccttcccagcgtgatggccaagggacctgcaagcagtgctccaaagaggcctcccaggggatacagagacacgatgagggaccacataagcaggactaggtgatcgggcagtggctctccagtacgcgcctgccatgtctcattggtgaattcctgaatgtgcaaggtcggggcattgatgatagagaggttatagccaaactgaaaagtcccaccaatgccggcagcgcagatggtcaggagcaggatcctgccctgaatctgcgtccgaggccgtaaggacggctccagttcatcctccatccgcctctgccgcagcactgaggctgaaaagccgctcactccttactcggctaagccccaagctcatctctgcaggccggaagggagctctggtccaaggtcatctcggccaagcccctgcattcgccctcgcaagtgccagcaagcgactctggtcgccgcgctcccaagtcctcccccgaaattccggctctggcccctcgtccccctcctttgctacagtctctggactaaatgtctgcgggtctctgtctctcgctggtctgacctcagccgcaaccctgcgcgattccctgcgccggtcgccactgccggccgccagaacctcggaggccact

SEQ ID NO: 12109 - RNA, 5531 nt, Homo sapiens
  source 1..5531: mol_type = other RNA
ctgcagactcgacctcccaggctcaagtgatcctcctacctcagcctcctgagtagctaggaccacaggcacatgccaccaggcccggctaatttttttttattttttgtagatagagtcttgctatgttgcccaggctggtctggaactcctgggctcaagagatcctccactatggcctcccaaagtgctgggattataggcatgagccatcacgcccagccaaatctttttacgtgaaacaccatggggccccaaaattaacctaattaatgaagacaggagaagaggtaagtcaaggaatacacacaaaaaacaaggaatgacaagaaagcaaatagatcagagaattgagagaggaaacatagtctcagcagccattagtggagactgagtgtagctgctcagaaccgaatgctgctttaagattaaggaaagttgagaactaagaaaagatttaaattggactgtggcattagcattaactattttaagcacttggccaagctcggtggctcacacctgtaatcccagcactttgggaggccaaggccagcagatcacttgaggccaggagttcgagaccagcctggccaacacaatgaaaccccgtctctactaaaaatacaaaaaattagctgagcgtggtggcacatgcctatagtcccagctgcttgtgaggtggaggttgccgtgagccaagatcgtgccactgcactccagcctgggcaacagagtgagattctgtctcaaaaaaaaaaaaagcacctgctttgaggtaactttgattacagctgaaatacagggaattttactaaaggacaaataccttccctcccagtagcttgtttcagattctggcacactggtaaataaaaactagaatcttgcaggctaaccttgcacatatgtatgtaagacagtcagaattccagccaggctttctcaaaactagggcagaattttttttaacttgtacttaactctcttctcccaggttatgttaaaatatgccttgggtcaggatgatagatgcctgtttttttctggagattcttagacattcagtcactcaatatcaaactgacaattaataaaatggttgtcatttcctcttccttctctgccataatctaccatcagcatatgaccatagaaagatgacaaatttttagataacctaaccaacccatatatgattaaactgacctttccttactaaaataaaatacacttactccatgtcttcactgcttttatcccctctaatgtgaaaatagcctcaaaatgatcttctaagacacaaaagaggacttaaacagtgtcatttgtcacttgctttatgcaaacattcgagtgtacctctttcaccacagggctagagatggtctactctgtacatacatttcacaacaaagaaaaattctgtcattccccaactctatgaccaaggaaaacttttaggatttctttaatttgtagcagagacacagtggcctagccaatcggcagtgctatacacacagtatgccagtttcccacccctaccctctttctccttttttaaagcttcaaaggttagatcaataaaatttaaaatttcctcatttaaggagaaatataatgacccacatgttaatttatattaaaaactaaaaataaataatggggttcttaaacaaggacatctttaactaggttatgattagaccagcctgtgggtgaaatgagagattatctcttctccctggaaatgtcttcaaggctcagacaattcagtagtttttaaaaggccccaactcacacatctcaggtgaaaagtataggcaatgggcaacaaacaagacgctagtatgcacttggcttctgataaattgaaacaaagatttggtggcccagcctaataaatgacagcacgaaactagaggtttaaagtaagttttgacatcacatatagatccctcaaccctaagttactttggagggaagccatgagaggctggatcagtcctcaagcctcagctaaggatggatcctatttcttcccagtgcaaaacaccaaatgtacctataaggtggagtcggcaaggagagttcccctcttactttgaagcaagagatggaaaaagtcagaaagatttctagataaaattgagaaacacaaaaggcaaagtaaagtcaatttaaacaggcctcacaaaaatcagccggaattcttattaaaaaaaacaaaacagaacattcatggatgggcaaagaaaggaaacaatgcagacgcctttggacttcaagagaaagcccatcaggaatctctgagagtgtcagctgagagagttctgtctctctccatgtaggatcctttctgcatcatgtatatcccaaaaggagttctgcgtgaaggtcatccatcttccctacagttcttagctgagcactgacacacacacatactccaccaatccaccaaactgcagctgtagctgcttatctgacccacactcccctggctctccacttttaggcacagtctttgttctttatcgccaggcccgattcaggagcttcacctgtgccagtctcttagtgatcatggtggcaaaaaccaggccaaagaggacgctgctgattaacacgtagtcatagtcatccttcagaacgtcaaactgcttggatgggtagactcgagtttggtaaatgtccaaaccataggccacaaccaaacaagtggactccagacccgagggagctgtgtagatacctcgcattcgagaaactgtctggttatagttgatgaatcgctctgcgtgtatctgtacatctggagaatacgggattaagttctcctctctgctttgttctgttgggatctcggggcggcggggatccagcaaagccttaggaagggaaagaattgctccagaaggtagtccaatcagcaggtgtcggctggtgatgccccgttcggtgatggtggcctccatggcactgatggaggacgggaagatataggactgctggaggacctggggcagctgggggcggtccagggagctgaaggcggtggcgttgtattgctcagtgccctcatagagctccagtacggtaaactcgttgcgccgagccttggtgttccagtactggtacaccacccagttctctgaatgcacgatatggacagggcctttggctttcttctgcacagaggagtgaatgatacgcccagtgacgccatcaatgaggaagatgccaataaaggtgcgctcatggtgcgcgtctgtgctctctgtcaccacggccagcaggttggggttcaggctcttgtagagcacactgcggtcccccatcacacggccctgggaatgaacgtgctcactgctgcgtttccccttcaccttgacgatccgctgtacttctgggggaatggtcagctcccaactcagctcagtggtgagatcctttcgaagccgatatccacacagccgtccctgctctgcatccaccaaatagaagaagatggaaggggcaagctcatgtagctgtcgcaagacattccgagtggctggaaaagctgtgaccttgtattcatcatctatcaacagcaacaccttggcgtagtcttgatccatgactgggagaagcaaggactgcaagatggggcgcttcagcactgggggagctacctgactccacttcccaaaaatgggattgaagacatacagagaactcattcccgactccttgtccttcaccagcagggtgcactgtgggggatgggggaaatgagcagtagttctctggaccatcagtttaaaggaggagtctggcttgacattgggtagatactgtttccacaggatggtgccagagctgctctcaatgccaaaaagcttgcctgaggctgttaccatcaccatcatcttctggaggttgaattcatctctggccagggtgtcaatgttgatctcattcttaatctgactccggggcttccgagcatcataaaacattttccagaggtgggaagtccatgcttgcagcaggataagctgagacgagaggcgtttcaggaacatccccagcaagccatctgcctttttgccaaattctccttccagctcggcctgtgccccagtcagggggaggtccaccatctctaggcacaccacttctgccagggactcctcacggctccacagcaccaccttccccaactgctgcaggaaaagtagcagatgatcctctgtctgcaccaaagcccggtagcccactgagtcatccttcttcaagaacacctggatatacagccgctcaggccgagtgccgctctgttccaggctaaatgttatcgtggtgtccagcagccgccgacctgtctccacgaggtataggttaatggtgtaggtctgattgaagcaagccagagagtcctttgaactagacttctccgaaaagctccccattgacccatcttcagaactgctacttttctgcacttcattccgacaggccatgactgcagccaccgtcttctccccagtggtggcaaagctcactagggcagtctgtgggaagtttttaagcaaactcagcgttccataatggtactgcagcagagcatagtggcttggggacaagtgcaggaagaactgggcccgggaagcgtccactgggttgggctgggtaggcaggacccggggttggaatccacttccaaattctaagtcgagagactgcagtgggatctgtctcaactcccattccgtctccagagccaaagtttggagggaacgtgagctcgggtcaggacacaccaggacagcctcatccaccacaccacaggctccagacaggtgctgcagccacggagttgaaaccctaacctgctgaacaatctctccatcttccacattaaacttgacaatgttcacatggctgaagggaacaactccgagggcccacaccaccccagagccgtaagaatacaccatctggtagtggatgctgtcactttctgggagatgttccacccacttgaggtgcccactggagaggtgatggagggcaagtgtagtcttcttcaggactgcgatgtaccttacagactcctgcaggccaaccagcccaagtgcctggaaactgccactgtccagggttatctcccagttcaggcccccgatgttagtctcccaggaacgcatgattcggcctccattggacacagtgatcacatcctgtccgtgcagcagcatggcatccacagccccttctgccgtgcccttgtcaacatggcgccacaagatctccccagttcgggaatttaatgctgcaatcacattcttctctgtggctacaaccaacttcttggatccaggggaaaattccaaggaggcaaacttgaccttcccaacatattgctgtctccaatcaaacttgcccacttggtcttcgtagaccgcggccgcaggaatcagcagcgtagcccaaagccagaaacgagaagcccactcagccgccatgatgcgagcgcatgc

SEQ ID NO: 12110 - RNA, 5531 nt, Homo sapiens
  source 1..5531: mol_type = other RNA
ctgcagactcgacctcccaggctcaagtgatcctcctacctcagcctcctgagtagctaggaccacaggcacatgccaccaggcccggctaatttttttttattttttgtagatagagtcttgctatgttgcccaggctggtctggaactcctgggctcaagagatcctccactatggcctcccaaagtgctgggattataggcatgagccatcacgcccagccaaatctttttacgtgaaacaccatggggccccaaaattaacctaattaatgaagacaggagaagaggtaagtcaaggaatacacacaaaaaacaaggaatgacaagaaagcaaatagatcagagaattgagagaggaaacatagtctcagcagccattagtggagactgagtgtagctgctcagaaccgaatgctgctttaagattaaggaaagttgagaactaagaaaagatttaaattggactgtggcattagcattaactattttaagcacttggccaagctcggtggctcacacctgtaatcccagcactttgggaggccaaggccagcagatcacttgaggccaggagttcgagaccagcctggccaacacaatgaaaccccgtctctactaaaaatacaaaaaattagctgagcgtggtggcacatgcctatagtcccagctgcttgtgaggtggaggttgccgtgagccaagatcgtgccactgcactccagcctgggcaacagagtgagattctgtctcaaaaaaaaaaaaagcacctgctttgaggtaactttgattacagctgaaatacagggaattttactaaaggacaaataccttccctcccagtagcttgtttcagattctggcacactggtaaataaaaactagaatcttgcaggctaaccttgcacatatgtatgtaagacagtcagaattccagccaggctttctcaaaactagggcagaattttttttaacttgtacttaactctcttctcccaggttatgttaaaatatgccttgggtcaggatgatagatgcctgtttttttctggagattcttagacattcagtcactcaatatcaaactgacaattaataaaatggttgtcatttcctcttccttctctgccataatctaccatcagcatatgaccatagaaagatgacaaatttttagataacctaaccaacccatatatgattaaactgacctttccttactaaaataaaatacacttactccatgtcttcactgcttttatcccctctaatgtgaaaatagcctcaaaatgatcttctaagacacaaaagaggacttaaacagtgtcatttgtcacttgctttatgcaaacattcgagtgtacctctttcaccacagggctagagatggtctactctgtacatacatttcacaacaaagaaaaattctgtcattccccaactctatgaccaaggaaaacttttaggatttctttaatttgtagcagagacacagtggcctagccaatcggcagtgctatacacacagtatgccagtttcccacccctaccctctttctccttttttaaagcttcaaaggttagatcaataaaatttaaaatttcctcatttaaggagaaatataatgacccacatgttaatttatattaaaaactaaaaataaataatggggttcttaaacaaggacatctttaactaggttatgattagaccagcctgtgggtgaaatgagagattatctcttctccctggaaatgtcttcaaggctcagacaattcagtagtttttaaaaggccccaactcacacatctcaggtgaaaagtataggcaatgggcaacaaacaagacgctagtatgcacttggcttctgataaattgaaacaaagatttggtggcccagcctaataaatgacagcacgaaactagaggtttaaagtaagttttgacatcacatatagatccctcaaccctaagttactttggagggaagccatgagaggctggatcagtcctcaagcctcagctaaggatggatcctatttcttcccagtgcaaaacaccaaatgtacctataaggtggagtcggcaaggagagttcccctcttactttgaagcaagagatggaaaaagtcagaaagatttctagataaaattgagaaacacaaaaggcaaagtaaagtcaatttaaacaggcctcacaaaaatcagccggaattcttattaaaaaaaacaaaacagaacattcatggatgggcaaagaaaggaaacaatgcagacgcctttggacttcaagagaaagcccatcaggaatctctgagagtgtcagctgagagagttctgtctctctccatgtaggatcctttctgcatcatgtatatcccaaaaggagttctgcgtgaaggtcatccatcttccctacagttcttagctgagcactgacacacacacatactccaccaatccaccaaactgcagctgtagctgcttatctgacccacactcccctggctctccacttttaggcacagtctttgttctttatcgccaggcccgattcaggagcttcacctgtgccagtctcttagtgatcatggtggcaaaaaccaggccaaagaggacgctgctgattaacacgtagtcatagtcatccttcagaacgtcaaactgcttggatgggtagactcgagtttggtaaatgtccaaaccataggccacaaccaaacaagtggactccagacccgagggagctgtgtagatacctcgcattcgagaaactgtctggttatagttgatgaatcgctctgcgtgtatctgtacatctggagaatacgggattaagttctcctctctgctttgttctgttgggatctcggggcggcggggatccagcaaagccttaggaagggaaagaattgctccagaaggtagtccaatcagcaggtgtcggctggtgatgccccgttcggtgatggtggcctccatggcactgatggaggacgggaagatataggactgctggaggacctggggcagctgggggcggtccagggagctgaaggcggtggcgttgtattgctcagtgccctcatagagctccagtacggtaaactcgttgcgccgagccttggtgttccagtactggtacaccacccagttctctgaatgcacgatatggacagggcctttggctttcttctgcacagaggagtgaatgatacgcccagtgacgccatcaatgaggaagatgccaataaaggtgcgctcatggtgcgcgtctgtgctctctgtcaccacggccagcaggttggggttcaggctcttgtagagcacactgcggtcccccatcacacggccctgggaatgaacgtgctcactgctgcgtttccccttcaccttgacgatccgctgtacttctgggggaatggtcagctcccaactcagctcagtggtgagatcctttcgaagccgatatccacacagccgtccctgctctgcatccaccaaatagaagaagatggaaggggcaagctcatgtagctgtcgcaagacattccgagtggctggaaaagctgtgaccttgtattcatcatctatcaacagcaacaccttggcgtagtcttgatccatgactgggagaagcaaggactgcaagatggggcgcttcagcactgggggagctacctgactccacttcccaaaaatgggattgaagacatacagagaactcattcccgactccttgtccttcaccagcagggtgcactgtgggggatgggggaaatgagcagtagttctctggaccatcagtttaaaggaggagtctggcttgacattgggtagatactgtttccacaggatggtgccagagctgctctcaatgccaaaaagcttgcctgaggctgttaccatcaccatcatcttctggaggttgaattcatctctggccagggtgtcaatgttgatctcattcttaatctgactccggggcttccgagcatcataaaacattttccagaggtgggaagtccatgcttgcagcaggataagctgagacgagaggcgtttcaggaacatccccagcaagccatctgcctttttgccaaattctccttccagctcggcctgtgccccagtcagggggaggtccaccatctctaggcacaccacttctgccagggactcctcacggctccacagcaccaccttccctgccaactgctgcaggaaaagtagcagatgatcctctgtctgcaccaaagcccggtagcccactgagtcatccttcttcaagaacacctggatatacagccgctcaggccgagtgccgctctgttccaggctaaatgttatcgtggtgtccagcagccgccgacctgtctccacgaggtataggttaatggtgtaggtctgattgaagcaagccagagagtcctttgaactagacttctccgaaaagctccccattgacccatcttcagaactgctacttttcacttcattccgacaggccatgactgcagccaccgtcttctccccagtggtggcaaagctcactagggcagtctgtgggaagtttttaagcaaactcagcgttccataatggtactgcagcagagcatagtggcttggggacaagtgcaggaagaactgggcccgggaagcgtccactgggttgggctgggtaggcaggacccggggttggaatccacttccaaattctaagtcgagagactgcagtgggatctgtctcaactcccattccgtctccagagccaaagtttggagggaacgtgagctcgggtcaggacacaccaggacagcctcatccaccacaccacaggctccagacaggtgctgcagccacggagttgaaaccctaacctgctgaacaatctctccatcttccacattaaacttgacaatgttcacatggctgaagggaacaactccgagggcccacaccaccccagagccgtaagaatacaccatctggtagtggatgctgtcactttctgggagatgttccacccacttgaggtgcccactggagaggtgatggagggcaagtgtagtcttcttcaggactgcgatgtaccttacagactcctgcaggccaaccagcccaagtgcctggaaactgccactgtccagggttatctcccagttcaggcccccgatgttagtctcccaggaacgcatgattcggcctccattggacacagtgatcacatcctgtccgtgcagcagcatggcatccacagccccttctgccgtgcccttgtcaacatggcgccacaagatctccccagttcgggaatttaatgctgcaatcacattcttctctgtggctacaaccaacttcttggatccaggggaaaattccaaggaggcaaacttgaccttcccaacatattgctgtctccaatcaaacttgcccacttggtcttcgtagaccgcggccgcaggaatcagcagcgtagcccaaagccagaaacgagaagcccactcagccgccatgatgcgagcgcatgc

SEQ ID NO: 12111 - RNA, 5468 nt, Homo sapiens
  source 1..5468: mol_type = other RNA
ctgcagactcgacctcccaggctcaagtgatcctcctacctcagcctcctgagtagctaggaccacaggcacatgccaccaggcccggctaatttttttttattttttgtagatagagtcttgctatgttgcccaggctggtctggaactcctgggctcaagagatcctccactatggcctcccaaagtgctgggattataggcatgagccatcacgcccagccaaatctttttacgtgaaacaccatggggccccaaaattaacctaattaatgaagacaggagaagaggtaagtcaaggaatacacacaaaaaacaaggaatgacaagaaagcaaatagatcagagaattgagagaggaaacatagtctcagcagccattagtggagactgagtgtagctgctcagaaccgaatgctgctttaagattaaggaaagttgagaactaagaaaagatttaaattggactgtggcattagcattaactattttaagcacttggccaagctcggtggctcacacctgtaatcccagcactttgggaggccaaggccagcagatcacttgaggccaggagttcgagaccagcctggccaacacaatgaaaccccgtctctactaaaaatacaaaaaattagctgagcgtggtggcacatgcctatagtcccagctgcttgtgaggtggaggttgccgtgagccaagatcgtgccactgcactccagcctgggcaacagagtgagattctgtctcaaaaaaaaaaaaagcacctgctttgaggtaactttgattacagctgaaatacagggaattttactaaaggacaaataccttccctcccagtagcttgtttcagattctggcacactggtaaataaaaactagaatcttgcaggctaaccttgcacatatgtatgtaagacagtcagaattccagccaggctttctcaaaactagggcagaattttttttaacttgtacttaactctcttctcccaggttatgttaaaatatgccttgggtcaggatgatagatgcctgtttttttctggagattcttagacattcagtcactcaatatcaaactgacaattaataaaatggttgtcatttcctcttccttctctgccataatctaccatcagcatatgaccatagaaagatgacaaatttttagataacctaaccaacccatatatgattaaactgacctttccttactaaaataaaatacacttactccatgtcttcactgcttttatcccctctaatgtgaaaatagcctcaaaatgatcttctaagacacaaaagaggacttaaacagtgtcatttgtcacttgctttatgcaaacattcgagtgtacctctttcaccacagggctagagatggtctactctgtacatacatttcacaacaaagaaaaattctgtcattccccaactctatgaccaaggaaaacttttaggatttctttaatttgtagcagagacacagtggcctagccaatcggcagtgctatacacacagtatgccagtttcccacccctaccctctttctccttttttaaagcttcaaaggttagatcaataaaatttaaaatttcctcatttaaggagaaatataatgacccacatgttaatttatattaaaaactaaaaataaataatggggttcttaaacaaggacatctttaactaggttatgattagaccagcctgtgggtgaaatgagagattatctcttctccctggaaatgtcttcaaggctcagacaattcagtagtttttaaaaggccccaactcacacatctcaggtgaaaagtataggcaatgggcaacaaacaagacgctagtatgcacttggcttctgataaattgaaacaaagatttggtggcccagcctaataaatgacagcacgaaactagaggtttaaagtaagttttgacatcacatatagatccctcaaccctaagttactttggagggaagccatgagaggctggatcagtcctcaagcctcagctaaggatggatcctatttcttcccagtgcaaaacaccaaatgtacctataaggtggagtcggcaaggagagttcccctcttactttgaagcaagagatggaaaaagtcagaaagatttctagataaaattgagaaacacaaaaggcaaagtaaagtcaatttaaacaggcctcacaaaaatcagccggaattcttattaaaaaaaacaaaacagaacattcatggatgggcaaagaaaggaaacaatgcagacgcctttggacttcaagagaaagcccatcaggaatctctgagagtgtcagctgagagagttctgtctctctccatgtaggatcctttctgcatcatgtatatcccaaaaggagttctgcgtgaaggtcatccatcttccctacagttcttagctgagcactgacacacacacatactccaccaatccaccaaactgcagctgtagctgcttatctgacccacactcccctggctctccacttttaggcacagtctttgttctttatcgccaggcccgattcaggagcttcacctgtgccagtctcttagtgatcatggtggcaaaaaccaggccaaagaggacgctgctgattaacacgtagtcatagtcatccttcagaacgtcaaactgcttggatgggtagactcgagtttggtaaatgtccaaaccataggccacaaccaaacaagtggactccagacccgagggagctgtgtagatacctcgcattcgagaaactgtctggttatagttgatgaatcgctctgcgtgtatctgtacatctggagaatacgggattaagttctcctctctgctttgttctgttgggatctcggggcggcggggatccagcaaagccttaggaagggaaagaattgctccagaaggtagtccaatcagcaggtgtcggctggtgatgccccgttcggtgatggtggcctccatggcactgatggaggacgggaagatataggactgctggaggacctggggcagctgggggcggtccagggagctgaaggcggtggcgttgtattgctcagtgccctcatagagctccagtacggtaaactcgttgcgccgagccttggtgttccagtactggtacaccacccagttctctgaatgcacgatatggacagggcctttggctttcttctgcacagaggagtgaatgatacgcccagtgacgccatcaatgaggaagatgccaataaaggtgcgctcatggtgcgcgtctgtgctctctgtcaccacggccagcaggttggggttcaggctcttgtagagcacactgcggtcccccatcacacggccctgggaatgaacgtgctcactgctgcgtttccccttcaccttgacgatccgctgtacttctgggggaatggtcagctcccaactcagctcagtggtgagatcctttcgaagccgatatccacacagccgtccctgctctgcatccaccaaatagaagaagatggaaggggcaagctcatgtagctgtcgcaagacattccgagtggctggaaaagctgtgaccttgtattcatcatctatcaacagcaacaccttggcgtagtcttgatccatgactgggagaagcaaggactgcaagatggggcgcttcagcactgggggagctacctgactccacttcccaaaaatgggattgaagacatacagagaactcattcccgactccttgtccttcaccagcagggtgcactgtgggggatgggggaaatgagcagtagttctctggaccatcagtttaaaggaggagtctggcttgacattgggtagatactgtttccacaggatggtgccagagctgctctcaatgccaaaaagcttgcctgaggctgttaccatcaccatcatcttctggaggttgaattcatctctggccagggtgtcaatgttgatctcattcttaatctgactccggggcttccgagcatcataaaacattttccagaggtgggaagtccatgcttgcagcaggataagctgagacgagaggcgtttcaggaacatccccagcaagccatctgcctttttgccaaattctccttccagctcggcctgtgccccagtcagggggaggtccaccatctctaggcacaccacttctgccagggactcctcacggctccacagcaccaccttccctgccaactgctgcaggaaaagtagcagatgatcctctgtctgcaccaaagcccggtagcccactgagtcatccttcttcaagaacacctggatatacagccgctcaggccgagtgccgctctgttccaggctaaatgttatcgtggtgtccagcagccgccgacctgtctccacgaggtataggttaatggtgtaggtctgattgaagcaagccagagagtcctttgaactagacttctccgaaaagctccccattgacccatcttcagaactgctacttttctgcacttcattccgacaggccatgactgcagccaccgtcttctccccagtggtggcaaagctcactagggcagtctgtgggaagtttttaagcaaactcagcgttccataatggtactgcagcagagcatagtggcttggggacaagtgcaggaagaactgggcccgggaagcgtccactgggttgggctgggtaggcaggacccggggttggaatccacttccaaattctaagtcgagagactgcagtgggatctgtctcaactcccattccgtctccagagccaaagtttggagggaacgtgagctcgggtcaggacacaccaggacagcctcatccaccacaccacaggctccagacaggtgctgcagccacggagttgaaaccctaacctgctgaacaatctctccatcttccacattaaacttgacaatgttcacatggctgaagggaacaactccgagggcccacaccaccccagagccgtaagaatacaccatctggtagtggatgctgtcactttctgggagatgttccacccacttgaggtgcccactggagaggtgatggagggcaagtgtagtcttcttcaggactgcgatgtaccttacagactcctgcaggccaaccagcccaagtgcctggaaactgccactgtccagggttatctcccagttcaggcccccgatgttagtctcccaggaacgcatgattcggcctccattggacacagtgatcacatagatctccccagttcgggaatttaatgctgcaatcacattcttctctgtggctacaaccaacttcttggatccaggggaaaattccaaggaggcaaacttgaccttcccaacatattgctgtctccaatcaaacttgcccacttggtcttcgtagaccgcggccgcaggaatcagcagcgtagcccaaagccagaaacgagaagcccactcagccgccatgatgcgagcgcatgc

SEQ ID NO: 12112 - RNA, 5534 nt, Homo sapiens
  source 1..5534: mol_type = other RNA
ctgcagactcgacctcccaggctcaagtgatcctcctacctcagcctcctgagtagctaggaccacaggcacatgccaccaggcccggctaatttttttttattttttgtagatagagtcttgctatgttgcccaggctggtctggaactcctgggctcaagagatcctccactatggcctcccaaagtgctgggattataggcatgagccatcacgcccagccaaatctttttacgtgaaacaccatggggccccaaaattaacctaattaatgaagacaggagaagaggtaagtcaaggaatacacacaaaaaacaaggaatgacaagaaagcaaatagatcagagaattgagagaggaaacatagtctcagcagccattagtggagactgagtgtagctgctcagaaccgaatgctgctttaagattaaggaaagttgagaactaagaaaagatttaaattggactgtggcattagcattaactattttaagcacttggccaagctcggtggctcacacctgtaatcccagcactttgggaggccaaggccagcagatcacttgaggccaggagttcgagaccagcctggccaacacaatgaaaccccgtctctactaaaaatacaaaaaattagctgagcgtggtggcacatgcctatagtcccagctgcttgtgaggtggaggttgccgtgagccaagatcgtgccactgcactccagcctgggcaacagagtgagattctgtctcaaaaaaaaaaaaagcacctgctttgaggtaactttgattacagctgaaatacagggaattttactaaaggacaaataccttccctcccagtagcttgtttcagattctggcacactggtaaataaaaactagaatcttgcaggctaaccttgcacatatgtatgtaagacagtcagaattccagccaggctttctcaaaactagggcagaattttttttaacttgtacttaactctcttctcccaggttatgttaaaatatgccttgggtcaggatgatagatgcctgtttttttctggagattcttagacattcagtcactcaatatcaaactgacaattaataaaatggttgtcatttcctcttccttctctgccataatctaccatcagcatatgaccatagaaagatgacaaatttttagataacctaaccaacccatatatgattaaactgacctttccttactaaaataaaatacacttactccatgtcttcactgcttttatcccctctaatgtgaaaatagcctcaaaatgatcttctaagacacaaaagaggacttaaacagtgtcatttgtcacttgctttatgcaaacattcgagtgtacctctttcaccacagggctagagatggtctactctgtacatacatttcacaacaaagaaaaattctgtcattccccaactctatgaccaaggaaaacttttaggatttctttaatttgtagcagagacacagtggcctagccaatcggcagtgctatacacacagtatgccagtttcccacccctaccctctttctccttttttaaagcttcaaaggttagatcaataaaatttaaaatttcctcatttaaggagaaatataatgacccacatgttaatttatattaaaaactaaaaataaataatggggttcttaaacaaggacatctttaactaggttatgattagaccagcctgtgggtgaaatgagagattatctcttctccctggaaatgtcttcaaggctcagacaattcagtagtttttaaaaggccccaactcacacatctcaggtgaaaagtataggcaatgggcaacaaacaagacgctagtatgcacttggcttctgataaattgaaacaaagatttggtggcccagcctaataaatgacagcacgaaactagaggtttaaagtaagttttgacatcacatatagatccctcaaccctaagttactttggagggaagccatgagaggctggatcagtcctcaagcctcagctaaggatggatcctatttcttcccagtgcaaaacaccaaatgtacctataaggtggagtcggcaaggagagttcccctcttactttgaagcaagagatggaaaaagtcagaaagatttctagataaaattgagaaacacaaaaggcaaagtaaagtcaatttaaacaggcctcacaaaaatcagccggaattcttattaaaaaaaacaaaacagaacattcatggatgggcaaagaaaggaaacaatgcagacgcctttggacttcaagagaaagcccatcaggaatctctgagagtgtcagctgagagagttctgtctctctccatgtaggatcctttctgcatcatgtatatcccaaaaggagttctgcgtgaaggtcatccatcttccctacagttcttagctgagcactgacacacacacatactccaccaatccaccaaactgcagctgtagctgcttatctgacccacactcccctggctctccacttttaggcacagtctttgttctttatcgccaggcccgattcaggagcttcacctgtgccagtctcttagtgatcatggtggcaaaaaccaggccaaagaggacgctgctgattaacacgtagtcatagtcatccttcagaacgtcaaactgcttggatgggtagactcgagtttggtaaatgtccaaaccataggccacaaccaaacaagtggactccagacccgagggagctgtgtagatacctcgcattcgagaaactgtctggttatagttgatgaatcgctctgcgtgtatctgtacatctggagaatacgggattaagttctcctctctgctttgttctgttgggatctcggggcggcggggatccagcaaagccttaggaagggaaagaattgctccagaaggtagtccaatcagcaggtgtcggctggtgatgccccgttcggtgatggtggcctccatggcactgatggaggacgggaagatataggactgctggaggacctggggcagctgggggcggtccagggagctgaaggcggtggcgttgtattgctcagtgccctcatagagctccagtacggtaaactcgttgcgccgagccttggtgttccagtactggtacaccacccagttctctgaatgcacgatatggacagggcctttggctttcttctgcacagaggagtgaatgatacgcccagtgacgccatcaatgaggaagatgccaataaaggtgcgctcatggtgcgcgtctgtgctctctgtcaccacggccagcaggttggggttcaggctcttgtagagcacactgcggtcccccatcacacggccctgggaatgaacgtgctcactgctgcgtttccccttcaccttgacgatccgctgtacttctgggggaatggtcagctcccaactcagctcagtggtgagatcctttcgaagccgatatccacacagccgtccctgctctgcatccaccaaatagaagaagatggaaggggcaagctcatgtagctgtcgcaagacattccgagtggctggaaaagctgtgaccttgtattcatcatctatcaacagcaacaccttggcgtagtcttgatccatgactgggagaagcaaggactgcaagatggggcgcttcagcactgggggagctacctgactccacttcccaaaaatgggattgaagacatacagagaactcattcccgactccttgtccttcaccagcagggtgcactgtgggggatgggggaaatgagcagtagttctctggaccatcagtttaaaggaggagtctggcttgacattgggtagatactgtttccacaggatggtgccagagctgctctcaatgccaaaaagcttgcctgaggctgttaccatcaccatcatcttctggaggttgaattcatctctggccagggtgtcaatgttgatctcattcttaatctgactccggggcttccgagcatcataaaacattttccagaggtgggaagtccatgcttgcagcaggataagctgagacgagaggcgtttcaggaacatccccagcaagccatctgcctttttgccaaattctccttccagctcggcctgtgccccagtcagggggaggtccaccatctctaggcacaccacttctgccagggactcctcacggctccacagcaccaccttccctgccaactgctgcaggaaaagtagcagatgatcctctgtctgcaccaaagcccggtagcccactgagtcatccttcttcaagaacacctggatatacagccgctcaggccgagtgccgctctgttccaggctaaatgttatcgtggtgtccagcagccgccgacctgtctccacgaggtataggttaatggtgtaggtctgattgaagcaagccagagagtcctttgaactagacttctccgaaaagctccccattgacccatcttcagaactgctacttttctgcacttcattccgacaggccatgactgcagccaccgtcttctccccagtggtggcaaagctcactagggcagtctgtgggaagtttttaagcaaactcagcgttccataatggtactgcagcagagcatagtggcttggggacaagtgcaggaagaactgggcccgggaagcgtccactgggttgggctgggtaggcaggacccggggttggaatccacttccaaattctaagtcgagagactgcagtgggatctgtctcaactcccattccgtctccagagccaaagtttggagggaacgtgagctcgggtcaggacacaccaggacagcctcatccaccacaccacaggctccagacaggtgctgcagccacggagttgaaaccctaacctgctgaacaatctctccatcttccacattaaacttgacaatgttcacatggctgaagggaacaactccgagggcccacaccaccccagagccgtaagaatacaccatctggtagtggatgctgtcactttctgggagatgttccacccacttgaggtgcccactggagaggtgatggagggcaagtgtagtcttcttcaggactgcgatgtaccttacagactcctgcaggccaaccagcccaagtgcctggaaactgccactgtccagggttatctcccagttcaggcccccgatgttagtctcccaggaacgcatgattcggcctccattggacacagtgatcacatcctgtccgtgcagcagcatggcatccacagccccttctgccgtgcccttgtcaacatggcgccacaagatctccccagttcgggaatttaatgctgcaatcacattcttctctgtggctacaaccaacttcttggatccaggggaaaattccaaggaggcaaacttgaccttcccaacatattgctgtctccaatcaaacttgcccacttggtcttcgtagaccgcggccgcaggaatcagcagcgtagcccaaagccagaaacgagaagcccactcagccgccatgatgcgagcgcatgc

SEQ ID NO: 12113 - RNA, 5540 nt, Homo sapiens
  source 1..5540: mol_type = other RNA
ctgcagactcgacctcccaggctcaagtgatcctcctacctcagcctcctgagtagctaggaccacaggcacatgccaccaggcccggctaatttttttttattttttgtagatagagtcttgctatgttgcccaggctggtctggaactcctgggctcaagagatcctccactatggcctcccaaagtgctgggattataggcatgagccatcacgcccagccaaatctttttacgtgaaacaccatggggccccaaaattaacctaattaatgaagacaggagaagaggtaagtcaaggaatacacacaaaaaacaaggaatgacaagaaagcaaatagatcagagaattgagagaggaaacatagtctcagcagccattagtggagactgagtgtagctgctcagaaccgaatgctgctttaagattaaggaaagttgagaactaagaaaagatttaaattggactgtggcattagcattaactattttaagcacttggccaagctcggtggctcacacctgtaatcccagcactttgggaggccaaggccagcagatcacttgaggccaggagttcgagaccagcctggccaacacaatgaaaccccgtctctactaaaaatacaaaaaattagctgagcgtggtggcacatgcctatagtcccagctgcttgtgaggtggaggttgccgtgagccaagatcgtgccactgcactccagcctgggcaacagagtgagattctgtctcaaaaaaaaaaaaagcacctgctttgaggtaactttgattacagctgaaatacagggaattttactaaaggacaaataccttccctcccagtagcttgtttcagattctggcacactggtaaataaaaactagaatcttgcaggctaaccttgcacatatgtatgtaagacagtcagaattccagccaggctttctcaaaactagggcagaattttttttaacttgtacttaactctcttctcccaggttatgttaaaatatgccttgggtcaggatgatagatgcctgtttttttctggagattcttagacattcagtcactcaatatcaaactgacaattaataaaatggttgtcatttcctcttccttctctgccataatctaccatcagcatatgaccatagaaagatgacaaatttttagataacctaaccaacccatatatgattaaactgacctttccttactaaaataaaatacacttactccatgtcttcactgcttttatcccctctaatgtgaaaatagcctcaaaatgatcttctaagacacaaaagaggacttaaacagtgtcatttgtcacttgctttatgcaaacattcgagtgtacctctttcaccacagggctagagatggtctactctgtacatacatttcacaacaaagaaaaattctgtcattccccaactctatgaccaaggaaaacttttaggatttctttaatttgtagcagagacacagtggcctagccaatcggcagtgctatacacacagtatgccagtttcccacccctaccctctttctccttttttaaagcttcaaaggttagatcaataaaatttaaaatttcctcatttaaggagaaatataatgacccacatgttaatttatattaaaaactaaaaataaataatggggttcttaaacaaggacatctttaactaggttatgattagaccagcctgtgggtgaaatgagagattatctcttctccctggaaatgtcttcaaggctcagacaattcagtagtttttaaaaggccccaactcacacatctcaggtgaaaagtataggcaatgggcaacaaacaagacgctagtatgcacttggcttctgataaattgaaacaaagatttggtggcccagcctaataaatgacagcacgaaactagaggtttaaagtaagttttgacatcacatatagatccctcaaccctaagttactttggagggaagccatgagaggctggatcagtcctcaagcctcagctaaggatggatcctatttcttcccagtgcaaaacaccaaatgtacctataaggtggagtcggcaaggagagttcccctcttactttgaagcaagagatggaaaaagtcagaaagatttctagataaaattgagaaacacaaaaggcaaagtaaagtcaatttaaacaggcctcacaaaaatcagccggaattcttattaaaaaaaacaaaacagaacattcatggatgggcaaagaaaggaaacaatgcagacgcctttggacttcaagagaaagcccatcaggaatctctgagagtgtcagctgagagagttctgtctctctccatgtaggatcctttctgcatcatgtatatcccaaaaggagttctgcgtgaaggtcatccatcttccctacagttcttagctgagcactgacacacacacatactccaccaatccaccaaactgcagctgtagctgcttatctgacccacactcccctggctctccacttttaggcacagtctttgttctttatcgccaggcccgattcaggagcttcacctgtgccagtctcttagtgatcatggtggcaaaaaccaggccaaagaggacgctgctgattaacacgtagtcatagtcatccttcagaacgtcaaactgcttggatgggtagactcgagtttggtaaatgtccaaaccataggccacaaccaaacaagtggactccagacccgagggagctgtgtagatacctcgcattcgagaaactgtctggttatagttgatgaatcgctctgcgtgtatctgtacatctggagaatacgggattaagttctcctctctgctttgttctgttgggatctcggggcggcggggatccagcaaagccttaggaagggaaagaattgctccagaaggtagtccaatcagcaggtgtcggctggtgatgccccgttcggtgatggtggcctccatggcactgatggaggacgggaagatataggactgctggaggacctggggcagctgggggcggtccagggagctgaaggcggtggcgttgtattgctcagtgccctcatagagctccagtacggtaaactcgttgcgccgagccttggtgttccagtactggtacaccacccagttctctgaatgcacgatatggacagggcctttggctttcttctgcacagaggagtgaatgatacgcccagtgacgccatcaatgaggaagatgccaataaaggtgcgctcatggtgcgcgtctgtgctctctgtcaccacggccagcaggttggggttcaggctcttgtagagcacactgcggtcccccatcacacggccctgggaatgaacgtgctcactgctgcgtttccccttcaccttgacgatccgctgtacttctgggggaatggtcagctcccaactcagctcagtggtgagatcctttcgaagccgatatccacacagccgtccctgctctgcatccaccaaatagaagaagatggaaggggcaagctcatgtagctgtcgcaagacattccgagtggctggaaaagctgtgaccttgtattcatcatctatcaacagcaacaccttggcgtagtcttgatccatgactgggagaagcaaggactgcaagatggggcgcttcagcactgggggagctacctgactccacttcccaaaaatgggattgaagacatacagagaactcattcccgactccttgtccttcaccagcagggtgcactgtgggggatgggggaaatgagcagtagttctctggaccatcagtttaaaggaggagtctggcttgacattgggtagatactgtttccacaggatggtgccagagctgctctcaatgccaaaaagcttgcctgaggctgttaccatcaccatcatcttctggaggttgaattcatctctggccagggtgtcaatgttgatctcattcttaatctgactccggggcttccgagcatcataaaacattttccagaggtgggaagtccatgcttgcagcaggataagctgagacgagaggcgtttcaggaacatccccagcaagccatcttgaattgctgcctttttgccaaattctccttccagctcggcctgtgccccagtcagggggaggtccaccatctctaggcacaccacttctgccagggactcctcacggctccacagcaccaccttccctgccaactgctgcaggaaaagtagcagatgatcctctgtctgcaccaaagcccggtagcccactgagtcatccttcttcaagaacacctggatatacagccgctcaggccgagtgccgctctgttccaggctaaatgttatcgtggtgtccagcagccgccgacctgtctccacgaggtataggttaatggtgtaggtctgattgaagcaagccagagagtcctttgaactagacttctccgaaaagctccccattgacccatcttcagaactgctacttttcacttcattccgacaggccatgactgcagccaccgtcttctccccagtggtggcaaagctcactagggcagtctgtgggaagtttttaagcaaactcagcgttccataatggtactgcagcagagcatagtggcttggggacaagtgcaggaagaactgggcccgggaagcgtccactgggttgggctgggtaggcaggacccggggttggaatccacttccaaattctaagtcgagagactgcagtgggatctgtctcaactcccattccgtctccagagccaaagtttggagggaacgtgagctcgggtcaggacacaccaggacagcctcatccaccacaccacaggctccagacaggtgctgcagccacggagttgaaaccctaacctgctgaacaatctctccatcttccacattaaacttgacaatgttcacatggctgaagggaacaactccgagggcccacaccaccccagagccgtaagaatacaccatctggtagtggatgctgtcactttctgggagatgttccacccacttgaggtgcccactggagaggtgatggagggcaagtgtagtcttcttcaggactgcgatgtaccttacagactcctgcaggccaaccagcccaagtgcctggaaactgccactgtccagggttatctcccagttcaggcccccgatgttagtctcccaggaacgcatgattcggcctccattggacacagtgatcacatcctgtccgtgcagcagcatggcatccacagccccttctgccgtgcccttgtcaacatggcgccacaagatctccccagttcgggaatttaatgctgcaatcacattcttctctgtggctacaaccaacttcttggatccaggggaaaattccaaggaggcaaacttgaccttcccaacatattgctgtctccaatcaaacttgcccacttggtcttcgtagaccgcggccgcaggaatcagcagcgtagcccaaagccagaaacgagaagcccactcagccgccatgatgcgagcgcatgc

SEQ ID NO: 12114 - RNA, 5543 nt, Homo sapiens
  source 1..5543: mol_type = other RNA
ctgcagactcgacctcccaggctcaagtgatcctcctacctcagcctcctgagtagctaggaccacaggcacatgccaccaggcccggctaatttttttttattttttgtagatagagtcttgctatgttgcccaggctggtctggaactcctgggctcaagagatcctccactatggcctcccaaagtgctgggattataggcatgagccatcacgcccagccaaatctttttacgtgaaacaccatggggccccaaaattaacctaattaatgaagacaggagaagaggtaagtcaaggaatacacacaaaaaacaaggaatgacaagaaagcaaatagatcagagaattgagagaggaaacatagtctcagcagccattagtggagactgagtgtagctgctcagaaccgaatgctgctttaagattaaggaaagttgagaactaagaaaagatttaaattggactgtggcattagcattaactattttaagcacttggccaagctcggtggctcacacctgtaatcccagcactttgggaggccaaggccagcagatcacttgaggccaggagttcgagaccagcctggccaacacaatgaaaccccgtctctactaaaaatacaaaaaattagctgagcgtggtggcacatgcctatagtcccagctgcttgtgaggtggaggttgccgtgagccaagatcgtgccactgcactccagcctgggcaacagagtgagattctgtctcaaaaaaaaaaaaagcacctgctttgaggtaactttgattacagctgaaatacagggaattttactaaaggacaaataccttccctcccagtagcttgtttcagattctggcacactggtaaataaaaactagaatcttgcaggctaaccttgcacatatgtatgtaagacagtcagaattccagccaggctttctcaaaactagggcagaattttttttaacttgtacttaactctcttctcccaggttatgttaaaatatgccttgggtcaggatgatagatgcctgtttttttctggagattcttagacattcagtcactcaatatcaaactgacaattaataaaatggttgtcatttcctcttccttctctgccataatctaccatcagcatatgaccatagaaagatgacaaatttttagataacctaaccaacccatatatgattaaactgacctttccttactaaaataaaatacacttactccatgtcttcactgcttttatcccctctaatgtgaaaatagcctcaaaatgatcttctaagacacaaaagaggacttaaacagtgtcatttgtcacttgctttatgcaaacattcgagtgtacctctttcaccacagggctagagatggtctactctgtacatacatttcacaacaaagaaaaattctgtcattccccaactctatgaccaaggaaaacttttaggatttctttaatttgtagcagagacacagtggcctagccaatcggcagtgctatacacacagtatgccagtttcccacccctaccctctttctccttttttaaagcttcaaaggttagatcaataaaatttaaaatttcctcatttaaggagaaatataatgacccacatgttaatttatattaaaaactaaaaataaataatggggttcttaaacaaggacatctttaactaggttatgattagaccagcctgtgggtgaaatgagagattatctcttctccctggaaatgtcttcaaggctcagacaattcagtagtttttaaaaggccccaactcacacatctcaggtgaaaagtataggcaatgggcaacaaacaagacgctagtatgcacttggcttctgataaattgaaacaaagatttggtggcccagcctaataaatgacagcacgaaactagaggtttaaagtaagttttgacatcacatatagatccctcaaccctaagttactttggagggaagccatgagaggctggatcagtcctcaagcctcagctaaggatggatcctatttcttcccagtgcaaaacaccaaatgtacctataaggtggagtcggcaaggagagttcccctcttactttgaagcaagagatggaaaaagtcagaaagatttctagataaaattgagaaacacaaaaggcaaagtaaagtcaatttaaacaggcctcacaaaaatcagccggaattcttattaaaaaaaacaaaacagaacattcatggatgggcaaagaaaggaaacaatgcagacgcctttggacttcaagagaaagcccatcaggaatctctgagagtgtcagctgagagagttctgtctctctccatgtaggatcctttctgcatcatgtatatcccaaaaggagttctgcgtgaaggtcatccatcttccctacagttcttagctgagcactgacacacacacatactccaccaatccaccaaactgcagctgtagctgcttatctgacccacactcccctggctctccacttttaggcacagtctttgttctttatcgccaggcccgattcaggagcttcacctgtgccagtctcttagtgatcatggtggcaaaaaccaggccaaagaggacgctgctgattaacacgtagtcatagtcatccttcagaacgtcaaactgcttggatgggtagactcgagtttggtaaatgtccaaaccataggccacaaccaaacaagtggactccagacccgagggagctgtgtagatacctcgcattcgagaaactgtctggttatagttgatgaatcgctctgcgtgtatctgtacatctggagaatacgggattaagttctcctctctgctttgttctgttgggatctcggggcggcggggatccagcaaagccttaggaagggaaagaattgctccagaaggtagtccaatcagcaggtgtcggctggtgatgccccgttcggtgatggtggcctccatggcactgatggaggacgggaagatataggactgctggaggacctggggcagctgggggcggtccagggagctgaaggcggtggcgttgtattgctcagtgccctcatagagctccagtacggtaaactcgttgcgccgagccttggtgttccagtactggtacaccacccagttctctgaatgcacgatatggacagggcctttggctttcttctgcacagaggagtgaatgatacgcccagtgacgccatcaatgaggaagatgccaataaaggtgcgctcatggtgcgcgtctgtgctctctgtcaccacggccagcaggttggggttcaggctcttgtagagcacactgcggtcccccatcacacggccctgggaatgaacgtgctcactgctgcgtttccccttcaccttgacgatccgctgtacttctgggggaatggtcagctcccaactcagctcagtggtgagatcctttcgaagccgatatccacacagccgtccctgctctgcatccaccaaatagaagaagatggaaggggcaagctcatgtagctgtcgcaagacattccgagtggctggaaaagctgtgaccttgtattcatcatctatcaacagcaacaccttggcgtagtcttgatccatgactgggagaagcaaggactgcaagatggggcgcttcagcactgggggagctacctgactccacttcccaaaaatgggattgaagacatacagagaactcattcccgactccttgtccttcaccagcagggtgcactgtgggggatgggggaaatgagcagtagttctctggaccatcagtttaaaggaggagtctggcttgacattgggtagatactgtttccacaggatggtgccagagctgctctcaatgccaaaaagcttgcctgaggctgttaccatcaccatcatcttctggaggttgaattcatctctggccagggtgtcaatgttgatctcattcttaatctgactccggggcttccgagcatcataaaacattttccagaggtgggaagtccatgcttgcagcaggataagctgagacgagaggcgtttcaggaacatccccagcaagccatcttgaattgctgcctttttgccaaattctccttccagctcggcctgtgccccagtcagggggaggtccaccatctctaggcacaccacttctgccagggactcctcacggctccacagcaccaccttccctgccaactgctgcaggaaaagtagcagatgatcctctgtctgcaccaaagcccggtagcccactgagtcatccttcttcaagaacacctggatatacagccgctcaggccgagtgccgctctgttccaggctaaatgttatcgtggtgtccagcagccgccgacctgtctccacgaggtataggttaatggtgtaggtctgattgaagcaagccagagagtcctttgaactagacttctccgaaaagctccccattgacccatcttcagaactgctacttttctgcacttcattccgacaggccatgactgcagccaccgtcttctccccagtggtggcaaagctcactagggcagtctgtgggaagtttttaagcaaactcagcgttccataatggtactgcagcagagcatagtggcttggggacaagtgcaggaagaactgggcccgggaagcgtccactgggttgggctgggtaggcaggacccggggttggaatccacttccaaattctaagtcgagagactgcagtgggatctgtctcaactcccattccgtctccagagccaaagtttggagggaacgtgagctcgggtcaggacacaccaggacagcctcatccaccacaccacaggctccagacaggtgctgcagccacggagttgaaaccctaacctgctgaacaatctctccatcttccacattaaacttgacaatgttcacatggctgaagggaacaactccgagggcccacaccaccccagagccgtaagaatacaccatctggtagtggatgctgtcactttctgggagatgttccacccacttgaggtgcccactggagaggtgatggagggcaagtgtagtcttcttcaggactgcgatgtaccttacagactcctgcaggccaaccagcccaagtgcctggaaactgccactgtccagggttatctcccagttcaggcccccgatgttagtctcccaggaacgcatgattcggcctccattggacacagtgatcacatcctgtccgtgcagcagcatggcatccacagccccttctgccgtgcccttgtcaacatggcgccacaagatctccccagttcgggaatttaatgctgcaatcacattcttctctgtggctacaaccaacttcttggatccaggggaaaattccaaggaggcaaacttgaccttcccaacatattgctgtctccaatcaaacttgcccacttggtcttcgtagaccgcggccgcaggaatcagcagcgtagcccaaagccagaaacgagaagcccactcagccgccatgatgcgagcgcatgc

SEQ ID NO: 12115 - RNA, 5592 nt, Homo sapiens
  source 1..5592: mol_type = other RNA
ctgcagactcgacctcccaggctcaagtgatcctcctgctgtggccttccaaagtgctaggattacaagtgtgacccactgaacacggcctgcacactattaatggcatctcaatagtgtctttaacacattcgtaaatggtattatatactgagactgaaagctacaagtcattctcattttctaatgttcggagtgatcagtggtttcactgggctgatccattcaaatttcctgtaagtttttcacctcaaagatagagcatttatcaatgaatattatttgcttacaagttataaaatgttagtattctagttctataattccttttattagctgaattaaagaaaaattttccgtcagtcatttgattgtcctgctcaagccagaattagctatatttccagaaaactctggctcattttgacgggaatggtatttgaacatggtttccaggcctttctagtgtcttttatatagagaaaacataacttcgtgttatttcccattcaaatttaggattacagattgtttttactctttgattttgtatgtatcttttctcatacactaaaaatcctcatttctaattatattaacatagttatgattaacaatttaattactgaagagtttaagatttcttcacatttctttttgcccttggatatatcccattaagaatggacatacaaattactatgctttaaagataactgaaacatacctgtgtattcaagccatcaacttgatatgcaatgcaggtcgtctgtttcattttgctttggacttgtagggcttttcttaactttgcttaaatctcgttttagaataacatatgtaccaaagtcaaatgttgaaaattcaagatatattctgagaaatctagcttccatcctggtcctttccatctggttcctctcctcctgcctccaccataagtaaccattttttaaagttttggttatgggtccattgtttcttttttttaactacacacacacacgcacttttatattccctttcttaaatatgatacatacacacacacacacacacacatatatatatataccttctccattttgtttttacttaataagaccactctgtagcgttaaacagaaatatacctcatggatttttacaggtacatactactcaatcatgtggctatacaaggatttagaataacctatttttaagtatagtatttaaatttaaataaccagtatttcattgaatgcttctgacttgtgagttaagaattagaccaaaaggtatcagaagccaaggcaatcaggctgattaaaaaatccagttttaaataggatatgtataacatatttagatgactagtacatctcaatacagtgggttttatatatattttgagggagggctgaaaatgttttgaaaattaattggatgttttcttccagtcatatccacaaaaaacatttgagatgcctatccaagtcctgatttcttctctgaagtctgcttcccacctagaaagaccggcatgacttgaactaaggaaaaggcagtgctttcctggccaacaagtttgtcattcaattgtctggctaatgagtcagcatgctaaatgaggtatgcctatatacagaactagacattaagggaaacagtctagaaatagctaattctcttgtgctcttatatactacacactgaactaaagcactctgaatattaacttatttatcttcaatatccttgaggtaggtactattactgccttaaaaataagataaggcagcacaggaagattaaataacttaaagagagtcacacagttagtattataaatggcagggctatgattaaactcaggccttctggctccagagctcagaatcctaaccactatattaccccatctttaaaagttattaggaccagaagaaataacattcagaagttaaaatagtaaactgagatgataaaagttttaattctgatgcaacagccaaatataaaacaagcaacaagtaggggtgtatggttttatttttttaaaaatgtatatgctcaataacagtttacttggaaattttcactagaagaaataacatgaaagaacaccagcataaatacataatacatactttaattgtggctatattaaatgtatcttaatgtaataccgctgtaacatggtatcatctcattgttaaaaattaaaaaaaaaaaaagaacatagggaagtgaaactaaaaaactatagaatcctggattctgtggcagatggagtacccttatttaagctagaaaaggagccctgtaaggtagaaagagaaaagaggcaagcaatctgaaaccatcatgttaaccaactgtgagtttttaaaaatgtggttaaaatgaatctaagaatgccttttaacacagctcacactttaatgaacaccagagaattcacagcaagactgtaaagctaggaatgtaaagttattgtggggttttagccacgaccctcacctcactctactatatgcaaaagaagaaagaaaagtctttagtcatgatttgcaccttaatcagcatcaattattctcagcagcccaaaaccctataaatgcagcagagcacacaggtctttaactaagtctaaaagcctagttaacatcaaaaaaattcatattgggaaagagccatacacatttaacgactgtgaaaagtcctttaacagagttttggtaaccatgagagaattcaaaccgaagagaaaccccaagtgtaaaaaatgcaacaaggcctttaggtatcactcaaccattagcaaaatccataggggagagaaaccttttatgtgtagctgaaatgataaagtcttaagtagtgacccattccttaattcaatatcagaacttctgtaagaaagaaactttatcaatgtgcggaatacgcaaggtatataaccaaaggagagaaatttgaagacacaaatgctaaagcagtagacagttcccaaccacccctaaatatgatggcatcccacccctctccctatcacactagccccttaccctcatttattcttcttcatggtactcatcacttgacactctctatacatttattacttaaaatgcttgtctaacttcctccactagaatataagctctgaaacaggagggggttttaaaaagctatatcctcagggtctaggataaaatctggcatatggtaggcatacaatagttgagtgaatttagtgtagtactttccttatgtggggtatttggtaccttgaggttacttcattctaagtgaatgatttagcaggctttaacatatataaaaatgtgttcattattctataatacaccagagtaaaaagcattttaactgccatggtctacaaattattctccaactgtgtgggggatggaaagttgtataaaaagcacccagtactaccctcataattgtaccaaccagtgagaccaagtggtctaccagggtcacgaaggtaaaatgaagtttccaacttcttaagagaaagttctcttttctcaggttcagaatctaaacactttactcctctcaggatggcatatatccctatatgccttgtcagccactggtatagagggcatagcagtttggaatccaatagcaacaactttttgtgcaaagtttggcatttagaatcatgcctcattaattcaaaaacattactaagggcctaccatgcattaagcactatgtatacaggtaaatttttaaaatatggagtttaccaacaataaagaaaataattacaaagcagtgtgatcagtgcgacaacatgggaggggaagagtaaaggaccagaacaaaggagcatctaatttgactgaaaagggctttaaaaagcctatgaaaacagaatcactgaagctgagtcctaagaggtaggtaggtattcacttggtcacaaagaaggatgcagaagtaatgatgtgtgcaaggctactgaggtggaaaacacacaaagcgcatttagggaagaagtggaagtacttgcaattgatcaggatgctctaaaaagagggatagtctgtggttctaaaaaccgtattaaaaataatttaaatctttatacttagaaagcacaaaggtattttcataagaaaacttgctaaaatgctaagttaaataaaaatcttagctgtgtaatgataaacaagggggctggggcaggaactgagaaattccctttgccacagaggctctatatcagaatttgtatgtttaccaaaagcagcctggattttaactgtttgagcaacactggactagaacatgattacacaggatgactgcagagacatggctgggaaggtagtcattctgtgttgccctgatctgcggaaaatcccaaaaagagaaaacttacaaagcagaaaggattttatataacagatgaggacttgacgtttggaaacactgagcttaaaattactgtgggatgtctaatgaagatatttgatagacagttagaaacaaggtttagaaagcaagagataagtcaggatacaagttacaggtttgagactcagtctgttattacaggtggtaaaagaagccatagttatgaatgacattgtataaaatatgtaaagtaaaaaaaaaaaagagagagagagaaaaaaatatagtgaagatcaatacctaaaaggtaggcagaaagtgagacaacactttgtggggaaatgagagagacagcgaagatgaaaccaacatgtagcacagagtcgcctttgataggaagcaggcaacctcttttcctctaaaatgggaaaatgagtaaagttggtaaatacaagttgacctcttcatagtctcaattttctgttcaataggagaaagagccatatgctaggggaggggcagagggcctaaggaaagtaatgaagtttggctcagccacagcgggaaatgggagagaggccaccctagtaacaaacataaggtttacattgagggcttttctaaggctgaagtgagacacttgtagtgattctactttgaaggactacccatcacaaagaactcagcatccccgaaaaggtagataataaataggattaatctgaggttgagggcttgccaaaggactagactaaaagaccagggaaagaagaataactggtgagattagttcatatagtatcccataaagctgagggtggatagggaagaaagcctgaaaggggctgacagtttaggaggaaggggagcagtcaagaaaagggggtaagaaggaactgaagaatgtggaatgagcataaaggagagaaaagtcaataaaataaggaagtgaaaaaactgaaaagagggcagttatcagttactgaaattttaccagaaagagaaactcaaggtggtgacattcaaagtgcggccacgggagtaagctgctggaatgtaataaagtcactgggcagaagtccaaggtatcagcaaggtatcagaaagatcatccaaagatgacaacaggagttgaggtagacagaaagaccatgagcaagatatcaagttaggctctctggcctttaacactcacccctattattaaag

SEQ ID NO: 12116 - RNA, 6311 nt, Homo sapiens
  source 1..6311: mol_type = other RNA
ctgcagactcgacctcccaggctcaatccatcctcctgagtagctgggactacaggtgggcaccagcactcctcgctaattttttttgtgtgtgtgtgttttgtttgcttgtttgtttgttgttgttttggttttttggggttttttttgtttttttttttttttttgcagagatggggttttgtcatgttgcctaggctggtctcaaactcctggactcaagcaatctgcccacctctgcctcccaaagtcctgggattacaggagtgagccactgcgcctagccctcctatctgctgctttgtatcctctgacctacatctctccaccctcctccacctcaggttttgttatctctgtatacctgtatttgagtgttttctttagattccccatgtgagtgaaatcgtgtaatatttttctttctgtatctgccttatttcacttaatatcctccagtttcatccatgttgtggcaaatggcaagatattctttttagggctgaataatattccattgtgtgtgtgtgtgtgtgtatacagtttctttatccattcattcttcaacaggcatttaggttgcttccctatattggctgcaatgctgcaatgaacgtgggatcacatttatctctacaaggtggctatctcattttatttgtgtatatcccctaaagagggattgttgggtcatatgtagccctattttcagtttatttagaaacctccatactgttttccacaatggctgtacattctcaccaacaatgcacaaaggttttctgttctcttcacccttatccacgtttatgattaatatcttttgactttttgataatagtcatcctattattatctagtgtctcataatggtttcaattcacatttcccttatgattagtgatgttgaacaccttttcatatccatcttggccatttttcttcttggagaaatgtcttttcaggtttttgcccatttttaactgggatcatttgttttcctgctattgagttgtatgagttctttatcaatttgttgtatcttattagatatatagtttgcaaatattttttccaatccataggttgccatttcattttgttgcttgttgtctttgctatgcagaagcttttcagcttgatgtagtcccatttatttatttttgcttttgtggcctgggcttttgatgtgatagccaaaaaatcattgctaaggccaaggttcaggagcttatcattacattttaacagctggaagagctcttccactctcatcagaatttttcttatctgtctcacttttgttttttagttgaggattagtatcattttgtcaagttaaaaaattgtatattgattaatttagggagaattgacatctttacaatactgagtcttcctatccaaagcaatatgtcttctttacattattttttactttgataagtgtggtttaaatgtagcttttattaatttactaaatgatacattttatttattcttgttaattattattgtcctaactcactattatttgtataaaagaaagttattttttattttaatatttcctttcactttactgaattttatcttaccacttttaccactttatttattattattattatttttattattttgagacagagttttgctcttgttgtctagactggagtgcaatggtgcgatctcggctcaccacaacttctgcctcccaggttcaagcaattctcccgcctcagcctcccgagtagctgggattacaggcatgcaccactacgcccggctaatttttattttaagtagagatggagtttctccatgttgtcaagctggtctcgaactcctgacctcaggtgatccgcccgacttggcctcccaaagtgctgagattacaggtgtgagccaccacgccctgcctattattattatttttattattttccagacagagtcttgctctgtcactaggctggagtgctctggtgcgaccttggctcactgcaacctctgcctcccaggatcaagcacttctcatgcttcagcctcctgagtagctgggactacaggtgtgtgccaccaaaccaggctaatttttgtatttttagaagagatggggtttcgccatgttggccaggctggtcttgaactcctgacctcaggtgatccacccacctcagcctcccaaaatgctgggattataggcatgaaccactgcgcctggccataatactttattattatttggttctcatggatttcctaggtgtataatcacttacaaataaaagtaattttggcatttctttaaatattataacttatttttcttgtataattggattggccacctgttctaaaacactgtaaaataagatagatagtaatcaatttttttcatgttcctaactttagtaggaatgcttctgtttcttcatcattaggtatgtattagcttttgtttacatgtatataaaattatggccaaataacatctgtctatcctattttagtaactaatttaataattaagaatggatgttgaatatttttgttttagcccagttgtctaagacttccaggaatatacctgtagtgtaataaaattaggtttattgatccattgcaatgagacagactgcgtcccaggggagccatggggtatctcaccaaacaaaggaaaaggcagagttataggatttggggtaagtttaggttaatattaaataaggcagatcgttgataggctcagaggaaagcagggctgtgtgtaaaacggtccatatcaggtctggactgcaaagtggacccagagtcctattttcttgaatactagacagttgagagaggtgtggaatgttgtgtccagataccccttatctgcacttctgtatttgagtataagatgaggctgtgttaggagtcaggaaaagaaaggagccaactgaagttatttagaaagcaaaatcaacagaacttggtgacgctggatgtagtgtgagggaaaatggcgaactgaaatttcacccctctatttatggcttatgtgattgggtagatgaccaggtcttcagctgatatggaatatactataacaacagttggtttagggaagcaagagagagaagaacaggatgatcacttcaatttttgatttgttgggtttctgactgctgcaagactcgagtatagacccacaggtaggtagtaggatgtataagtgcagggatactgctggaggctggggtcacagctatagatacagatgcctaggagtcatgagcatcactgaaggagggcctgcaaagtgagaggagcactgaccagatcaagagaaaaccccaggaagatttccctaaggtttccaggccagtaggatgagcccacagtgaagactacaaatgaacagagagaggtaggaatcaaagcagagacctgccatgtcagagaaactgaggaaaagagttccaaggaggagggagtggtcaactttatcaactgcaggaaatgggctcaggaatggaagacctgaattggtttaacagttggcaggtagacggtgacttttgccagggtacattcaggtaagttggtgaagcagaagaccaaattctgtatgttcagccaataataagtgagacagaaaagtcagcctccaccttacaggaagctgggctgagaagggcaggagacagggcagtaactgctgtggcatcaagctcagggaatgcttttcagcaaaaaagatgtcagtgtttcacttttttcagctagttagaatcaggacctcagcctgatggaattcatttaaaataccaaataaaggtaagtcttctgtagtctttctgtactcacttgagtacttgatctctgtaactcactctgcatcctccttcttgccccttccttagcatgacacacgcacgcgcacgtgcacacacacaccagtatacatttgattatattttaatgatcacgcagacccttttagaaaagatgtctccttgaactgtacccaggagatgtggccatggcacacacaaagctgtagggaaagaccagacgaatcttgagctgagaaggaagggctcagttgcataggtatttaggcagaatgcataaagaaatcctttgttgaaaatatttaggaaagaatggagtttttgaaatataaaatcaataataatttttattttttgttcagcacacatggcaacacagagctgtgaagacagacgtggttagcacaaaccacttgggccagtgaaaccagggcaaactcatggatcatctgcgttcccatcttcaccttggtggcagccctacctctgagattttaaggtctacggaaagtgcaggcttccaggagtgatgaggtggagcattttctcaggttaccaacagccttgacatattcttctcctaagtatttttcatatgtgtttctgtcatgaagtttggccaaacatactgtgtcatctctgaacagaaggtccttggtttccgaccggaacaaacaaaagttgcccgagcagtcagttacgttgcttccaaataggtgctgctgttgacgtaatatcttgtggacgcaagcttccttatctttccgtgtgaccacagcgtgattcggggctctggccaggtggcagttcgcatactcctccacaggtttcctggtaccatcaaggcacagcaactcatagtctttttcattcagattcttagcccatggatcagggttttttcccccagtgttctgtgggacagtctggtgtttcacaaaggccacatctcccttctcaaccagacacctgaaagcgcctgtgtagccgtagtatccctctttgttgttgggttcacacaggtttaggcctgagcccatacacagcttacagagactggagtctttcttagacccaggggcacaaccttcactgaaaaattcatcaaatctgcagtggttgatcttattgtagagcaggcccatggggatgttccagccagcggttctgccaactgccgtatggcaggacttcttgcctttcagattgtcccaggtgaggtcagaagctgatttcttcaccactgctatagcaaaataccctgcctctggtgtatcctcacaattatcgctcttattgtagttttctgccaagacaggcaccagaccacacttgcccgctatgtagacaaaccctccatccaagctcatggcatcagcttctccattcatgatcttggcgatgcagtcttcggtggtctctgctgatacacactctattttccctacactgttaacactccactcatcacacttgagcctctcgtggtggctcagcgcacaccacttcacaggcttgcattcatctgttggggcttctgggcatgtgccttcccgtagattccggatggcagtgacatactcatagcccaggtacatcttggcatccatcctgggggggacttttaaaaacccgtgggcagagtccttaaacagcaggtccttcccatgaggagagctgaatagttggaattcttttgatttgtctttgccaaaatgttcctgggcctggttgagaagctcccagatcaagtcctccttgccgcccatacttcgggccacgacggtatgagaagggacctgggccaagtggcagtccttgtattcatctaccggcttccgggtgttgtccaggcaaagcagctcatactggtccctgtcagccttgtttgccaagttctcaaatatagtcgagtgcttgacaaaggccacatccccagcaccatccttcagacacttgaaggctcccgagtagccgaagtattggttaagggtggagcagccacaccctggacacagttgacacagctgggggaagtccgtcccatccgcacaaggggcacagctgcccgagaagaaattggccactgctttctcaagaggtttacgtggctcaggtaagtcacagtaaagtaagcctatggggatgttccacccagcggacctgcctagacccgtgtggcaggacttcttgcctcgaagctggttcatctggaagccactatccttcttcaccacagcaacagcataatagaaagtctgtggatcctcttttgacccatagaactctgccaccacaggcttcaggttattgggagccaggtaagcatcatacaccaaacctgcatccagtgtcacagcatccgcttcgtttgcccaggacggcgcagaccagcagggctcccacggcgagcctcatcttccgggtgcggcgctgagcagcgagcacagtcggactcgcttctgt

SEQ ID NO: 12117 - RNA, 7452 nt, Homo sapiens
  source 1..7452: mol_type = other RNA
ctgcagactcgacctcccaggctcaatccatcctcctgagtagctgggactacaggtgggcaccagcactcctcgctaattttttttgtgtgtgtgtgttttgtttgcttgtttgtttgttgttgttttggttttttggggttttttttgtttttttttttttttttgcagagatggggttttgtcatgttgcctaggctggtctcaaactcctggactcaagcaatctgcccacctctgcctcccaaagtcctgggattacaggagtgagccactgcgcctagccctcctatctgctgctttgtatcctctgacctacatctctccaccctcctccacctcaggttttgttatctctgtatacctgtatttgagtgttttctttagattccccatgtgagtgaaatcgtgtaatatttttctttctgtatctgccttatttcacttaatatcctccagtttcatccatgttgtggcaaatggcaagatattctttttagggctgaataatattccattgtgtgtgtgtgtgtgtgtatacagtttctttatccattcattcttcaacaggcatttaggttgcttccctatattggctgcaatgctgcaatgaacgtgggatcacatttatctctacaaggtggctatctcattttatttgtgtatatcccctaaagagggattgttgggtcatatgtagccctattttcagtttatttagaaacctccatactgttttccacaatggctgtacattctcaccaacaatgcacaaaggttttctgttctcttcacccttatccacgtttatgattaatatcttttgactttttgataatagtcatcctattattatctagtgtctcataatggtttcaattcacatttcccttatgattagtgatgttgaacaccttttcatatccatcttggccatttttcttcttggagaaatgtcttttcaggtttttgcccatttttaactgggatcatttgttttcctgctattgagttgtatgagttctttatcaatttgttgtatcttattagatatatagtttgcaaatattttttccaatccataggttgccatttcattttgttgcttgttgtctttgctatgcagaagcttttcagcttgatgtagtcccatttatttatttttgcttttgtggcctgggcttttgatgtgatagccaaaaaatcattgctaaggccaaggttcaggagcttatcattacattttaacagctggaagagctcttccactctcatcagaatttttcttatctgtctcacttttgttttttagttgaggattagtatcattttgtcaagttaaaaaattgtatattgattaatttagggagaattgacatctttacaatactgagtcttcctatccaaagcaatatgtcttctttacattattttttactttgataagtgtggtttaaatgtagcttttattaatttactaaatgatacattttatttattcttgttaattattattgtcctaactcactattatttgtataaaagaaagttattttttattttaatatttcctttcactttactgaattttatcttaccacttttaccactttatttattattattattatttttattattttgagacagagttttgctcttgttgtctagactggagtgcaatggtgcgatctcggctcaccacaacttctgcctcccaggttcaagcaattctcccgcctcagcctcccgagtagctgggattacaggcatgcaccactacgcccggctaatttttattttaagtagagatggagtttctccatgttgtcaagctggtctcgaactcctgacctcaggtgatccgcccgacttggcctcccaaagtgctgagattacaggtgtgagccaccacgccctgcctattattattatttttattattttccagacagagtcttgctctgtcactaggctggagtgctctggtgcgaccttggctcactgcaacctctgcctcccaggatcaagcacttctcatgcttcagcctcctgagtagctgggactacaggtgtgtgccaccaaaccaggctaatttttgtatttttagaagagatggggtttcgccatgttggccaggctggtcttgaactcctgacctcaggtgatccacccacctcagcctcccaaaatgctgggattataggcatgaaccactgcgcctggccataatactttattattatttggttctcatggatttcctaggtgtataatcacttacaaataaaagtaattttggcatttctttaaatattataacttatttttcttgtataattggattggccacctgttctaaaacactgtaaaataagatagatagtaatcaatttttttcatgttcctaactttagtaggaatgcttctgtttcttcatcattaggtatgtattagcttttgtttacatgtatataaaattatggccaaataacatctgtctatcctattttagtaactaatttaataattaagaatggatgttgaatatttttgttttagcccagttgtctaagacttccaggaatatacctgtagtgtaataaaattaggtttattgatccattgcaatgagacagactgcgtcccaggggagccatggggtatctcaccaaacaaaggaaaaggcagagttataggatttggggtaagtttaggttaatattaaataaggcagatcgttgataggctcagaggaaagcagggctgtgtgtaaaacggtccatatcaggtctggactgcaaagtggacccagagtcctattttcttgaatactagacagttgagagaggtgtggaatgttgtgtccagataccccttatctgcacttctgtatttgagtataagatgaggctgtgttaggagtcaggaaaagaaaggagccaactgaagttatttagaaagcaaaatcaacagaacttggtgacgctggatgtagtgtgagggaaaatggcgaactgaaatttcacccctctatttatggcttatgtgattgggtagatgaccaggtcttcagctgatatggaatatactataacaacagttggtttagggaagcaagagagagaagaacaggatgatcacttcaatttttgatttgttgggtttctgactgctgcaagactcgagtatagacccacaggtaggtagtaggatgtataagtgcagggatactgctggaggctggggtcacagctatagatacagatgcctaggagtcatgagcatcactgaaggagggcctgcaaagtgagaggagcactgaccagatcaagagaaaaccccaggaagatttccctaaggtttccaggccagtaggatgagcccacagtgaagactacaaatgaacagagagaggtaggaatcaaagcagagacctgccatgtcagagaaactgaggaaaagagttccaaggaggagggagtggtcaactttatcaactgcaggaaatgggctcaggaatggaagacctgaattggtttaacagttggcaggtagacggtgacttttgccagggtacattcaggtaagttggtgaagcagaagaccaaattctgtatgttcagccaataataagtgagacagaaaagtcagcctccaccttacaggaagctgggctgagaagggcaggagacagggcagtaactgctgtggcatcaagctcagggaatgcttttcagcaaaaaagatgtcagtgtttcacttttttcagctagttagaatcaggacctcagcctgatggaattcatttaaaataccaaataaaggtaagtcttctgtagtctttctgtactcacttgagtacttgatctctgtaactcactctgcatcctccttcttgccccttccttagcatgacacacgcacgcgcacgtgcacacacacaccagtatacatttgattatattttaatgatcacgcagacccttttagaaaagatgtctccttgaactgtacccaggagatgtggccatggcacacacaaagctgtagggaaagaccagacgaatcttgagctgagaaggaagggctcagttgcataggtatttaggcagaatgcataaagaaatcctttgttgaaaatatttaggaaagaatggagtttttgaaatataaaatcaataataatttttattttttgttcagcacacatggcaacacagagctgtgaagacagacgtggttagcacaaaccacttgggccagtgaaaccagggcaaactcatggatcatctgcgttcccatcttcaccttggtggcagccctacctctgagattttaaggtctacggaaagtgcaggcttccaggagtgatgaggtggagcattttctcaggttaccaacagccttgacatattcttctcctaagtatttttcatatgtgtttctgtcatgaagtttggccaaacatactgtgtcatctctgaacagaaggtccttggtttccgaccggaacaaacaaaagttgcccgagcagtcagttacgttgcttccaaataggtgctgctgttgacgtaatatcttgtggacgcaagcttccttatctttccgtgtgaccacagcgtgattcggggctctggccaggtggcagttcgcatactcctccacaggtttcctggtaccatcaaggcacagcaactcatagtctttttcattcagattcttagcccatggatcagggttttttcccccagtgttctgtgggacagtctggtgtttcacaaaggccacatctcccttctcaaccagacacctgaaagcgcctgtgtagccgtagtatccctctttgttgttgggttcacacaggtttaggcctgagcccatacacagcttacagagactggagtctttcttagacccaggggcacaaccttcactgaaaaattcatcaaatctgcagtggttgatcttattgtagagcaggcccatggggatgttccagccagcggttctgccaactgccgtatggcaggacttcttgcctttcagattgtcccaggtgaggtcagaagctgatttcttcaccactgctatagcaaaataccctgcctctggtgtatcctcacaattatcgctcttattgtagttttctgccaagacaggcaccagaccacacttgcccgctatgtagacaaaccctccatccaagctcatggcatcagcttctccattcatgatcttggcgatgcagtcttcggtggtctctgctgatacacactctattttccctacactgttaacactccactcatcacacttgagcctctcgtggtggctcagcgcacaccacttcacaggcttgcattcatctgttggggcttctgggcatgtgccttcccgtagattccggatggcagtgacatactcatagcccaggtacatcttggcatccatcctgggggggacttttaaaaacccgtgggcagagtccttaaacagcaggtccttcccatgaggagagctgaatagttggaattcttttgatttgtctttgccaaaatgttcctgggcctggttgagaagctcccagatcaagtcctccttgccgcccatacttcgggccacgacggtatgagaagggacctgggccaagtggcagtccttgtattcatctaccggcttccgggtgttgtccaggcaaagcagctcatactggtccctgtcagccttgtttgccaagttctcaaatatagtcgagtgcttgacaaaggccacatccccagcaccatccttcagacacttgaaggctcccgagtagccgaagtattggttaagggtggagcagccacaccctggacacagttgacacagctgggggaagtccgtcccatccgcacaaggggcacagctgcccgagaagaaattggccactgctttctcaagaggtttacgtggctcaggtaagtcacagtaaagtaagcctatggggatgttccacccagcggacctgcctagacccgtgtggcaggacttcttgcctcgaagctggttcatctggaagccactatccttcttcaccacagcaacagcataatagaaagtctgtggatcctcttttgacccatagaactctgccaccacaggcttcaggttattgggagccaggtaagcatcatacaccaaacctgcatccagtgtcacagcatccgcttcgtttgccgcaatggccctgatgcaatcaaggtaggaggctttcttcacacaagcaacactgggaccatcggatggaatgacgcttttcatatggtcgcggaaactctggcacttagtggcctcatgctccgacactgcacaccatctcacagttttatcagggacagccagacacagcccagccaagtgtaagaagtgaggtgtctggtgtcccccctgtgattttaaaccaaggctctgatggattcttgacttgtccacagtcacacagaagaaagtggcaaaagtagaactagagttgtgactctgccgccatcattcttgcttctccctaggtgccctaaggtgccctaaatcatctgggtctgcaggagagtgccctgaaagccccactggagccgtagtatctctcctggctgttgtaagcccatatgtgggcaggattgcacctgccaccacacagagcacagagaggggaatccggattagacccaggggcacaactgcgactgaagaaatcatcacatttacaggacccggtttgattgtatattaagcccatggggatgttccagcttgcagaagtgccaactgcagtgtggcaggacttcttgcctcaaagagagttccaggtgacatcagcatctgatttcttaaccacagccatgacataatagccttttctctgtgttgtagatcaggtctctacaaattcaaacttggagaagttgggagtcaacatggcagatggaaggtccgtcttgtccttcttaggtgacctcagacacgtccttatcatctaggagcctaaatttttcttcagttaaatggtggcagtggaacccctcctggagtgactctttttggatcctgagtcgcggaaaaatactcatatcccaggtacagcttggcatctatcttaggtgggaccattaaaaacccatgggcagcatcagtaaacagcagatctgtctcatgaggagagccaaagagctgaaattctgacgacttgtcttttccaaaatgttctgtgatggctttaatgtactcaagggaagacgctctctccacgcaggtgacaaggggaccatctgctggaaacacttttttcatattgtctcggaaactggtgcacttcgtggcctcgtgatctgacatggcacaccatcttccagttttctcaggagcagccaggcacagccctccacgtttgacatttccgctcttctgctgcagct

SEQ ID NO: 12118 - RNA, 6484 nt, Homo sapiens
  source 1..6484: mol_type = other RNA
ctgcagactcgacctcccaggctcaatccatcctcctgagtagctgggactacaggtgggcaccagcactcctcgctaattttttttgtgtgtgtgtgttttgtttgcttgtttgtttgttgttgttttggttttttggggttttttttgtttttttttttttttttgcagagatggggttttgtcatgttgcctaggctggtctcaaactcctggactcaagcaatctgcccacctctgcctcccaaagtcctgggattacaggagtgagccactgcgcctagccctcctatctgctgctttgtatcctctgacctacatctctccaccctcctccacctcaggttttgttatctctgtatacctgtatttgagtgttttctttagattccccatgtgagtgaaatcgtgtaatatttttctttctgtatctgccttatttcacttaatatcctccagtttcatccatgttgtggcaaatggcaagatattctttttagggctgaataatattccattgtgtgtgtgtgtgtgtgtatacagtttctttatccattcattcttcaacaggcatttaggttgcttccctatattggctgcaatgctgcaatgaacgtgggatcacatttatctctacaaggtggctatctcattttatttgtgtatatcccctaaagagggattgttgggtcatatgtagccctattttcagtttatttagaaacctccatactgttttccacaatggctgtacattctcaccaacaatgcacaaaggttttctgttctcttcacccttatccacgtttatgattaatatcttttgactttttgataatagtcatcctattattatctagtgtctcataatggtttcaattcacatttcccttatgattagtgatgttgaacaccttttcatatccatcttggccatttttcttcttggagaaatgtcttttcaggtttttgcccatttttaactgggatcatttgttttcctgctattgagttgtatgagttctttatcaatttgttgtatcttattagatatatagtttgcaaatattttttccaatccataggttgccatttcattttgttgcttgttgtctttgctatgcagaagcttttcagcttgatgtagtcccatttatttatttttgcttttgtggcctgggcttttgatgtgatagccaaaaaatcattgctaaggccaaggttcaggagcttatcattacattttaacagctggaagagctcttccactctcatcagaatttttcttatctgtctcacttttgttttttagttgaggattagtatcattttgtcaagttaaaaaattgtatattgattaatttagggagaattgacatctttacaatactgagtcttcctatccaaagcaatatgtcttctttacattattttttactttgataagtgtggtttaaatgtagcttttattaatttactaaatgatacattttatttattcttgttaattattattgtcctaactcactattatttgtataaaagaaagttattttttattttaatatttcctttcactttactgaattttatcttaccacttttaccactttatttattattattattatttttattattttgagacagagttttgctcttgttgtctagactggagtgcaatggtgcgatctcggctcaccacaacttctgcctcccaggttcaagcaattctcccgcctcagcctcccgagtagctgggattacaggcatgcaccactacgcccggctaatttttattttaagtagagatggagtttctccatgttgtcaagctggtctcgaactcctgacctcaggtgatccgcccgacttggcctcccaaagtgctgagattacaggtgtgagccaccacgccctgcctattattattatttttattattttccagacagagtcttgctctgtcactaggctggagtgctctggtgcgaccttggctcactgcaacctctgcctcccaggatcaagcacttctcatgcttcagcctcctgagtagctgggactacaggtgtgtgccaccaaaccaggctaatttttgtatttttagaagagatggggtttcgccatgttggccaggctggtcttgaactcctgacctcaggtgatccacccacctcagcctcccaaaatgctgggattataggcatgaaccactgcgcctggccataatactttattattatttggttctcatggatttcctaggtgtataatcacttacaaataaaagtaattttggcatttctttaaatattataacttatttttcttgtataattggattggccacctgttctaaaacactgtaaaataagatagatagtaatcaatttttttcatgttcctaactttagtaggaatgcttctgtttcttcatcattaggtatgtattagcttttgtttacatgtatataaaattatggccaaataacatctgtctatcctattttagtaactaatttaataattaagaatggatgttgaatatttttgttttagcccagttgtctaagacttccaggaatatacctgtagtgtaataaaattaggtttattgatccattgcaatgagacagactgcgtcccaggggagccatggggtatctcaccaaacaaaggaaaaggcagagttataggatttggggtaagtttaggttaatattaaataaggcagatcgttgataggctcagaggaaagcagggctgtgtgtaaaacggtccatatcaggtctggactgcaaagtggacccagagtcctattttcttgaatactagacagttgagagaggtgtggaatgttgtgtccagataccccttatctgcacttctgtatttgagtataagatgaggctgtgttaggagtcaggaaaagaaaggagccaactgaagttatttagaaagcaaaatcaacagaacttggtgacgctggatgtagtgtgagggaaaatggcgaactgaaatttcacccctctatttatggcttatgtgattgggtagatgaccaggtcttcagctgatatggaatatactataacaacagttggtttagggaagcaagagagagaagaacaggatgatcacttcaatttttgatttgttgggtttctgactgctgcaagactcgagtatagacccacaggtaggtagtaggatgtataagtgcagggatactgctggaggctggggtcacagctatagatacagatgcctaggagtcatgagcatcactgaaggagggcctgcaaagtgagaggagcactgaccagatcaagagaaaaccccaggaagatttccctaaggtttccaggccagtaggatgagcccacagtgaagactacaaatgaacagagagaggtaggaatcaaagcagagacctgccatgtcagagaaactgaggaaaagagttccaaggaggagggagtggtcaactttatcaactgcaggaaatgggctcaggaatggaagacctgaattggtttaacagttggcaggtagacggtgacttttgccagggtacattcaggtaagttggtgaagcagaagaccaaattctgtatgttcagccaataataagtgagacagaaaagtcagcctccaccttacaggaagctgggctgagaagggcaggagacagggcagtaactgctgtggcatcaagctcagggaatgcttttcagcaaaaaagatgtcagtgtttcacttttttcagctagttagaatcaggacctcagcctgatggaattcatttaaaataccaaataaaggtaagtcttctgtagtctttctgtactcacttgagtacttgatctctgtaactcactctgcatcctccttcttgccccttccttagcatgacacacgcacgcgcacgtgcacacacacaccagtatacatttgattatattttaatgatcacgcagacccttttagaaaagatgtctccttgaactgtacccaggagatgtggccatggcacacacaaagctgtagggaaagaccagacgaatcttgagctgagaaggaagggctcagttgcataggtatttaggcagaatgcataaagaaatcctttgttgaaaatatttaggaaagaatggagtttttgaaatataaaatcaataataatttttattttttgttcagcacacatggcaacacagagctgtgaagacagacgtggttagcacaaaccacttgggccagtgaaaccagggcaaactcatggatcatctgcgttcccatcttcaccttggtggcagccctacctctgagattttaaggtctacggaaagtgcaggcttccaggagtgatgaggtggagcattttctcaggttaccaacagccttgacatattcttctcctaagtatttttcatatgtgtttctgtcatgaagtttggccaaacatactgtgtcatctctgaacagaaggtccttggtttccgaccggaacaaacaaaagttgcccgagcagtcagttacgttgcttccaaataggtgctgctgttgacgtaatatcttgtggacgcaagcttccttatctttccgtgtgaccacagcgtgattcggggctctggccaggtggcagttcgcatactcctccacaggtttcctggtaccatcaaggcacagcaactcatagtctttttcattcagattcttagcccatggatcagggttttttcccccagtgttctgtgggacagtctggtgtttcacaaaggccacatctcccttctcaaccagacacctgaaagcgcctgtgtagccgtagtatccctctttgttgttgggttcacacaggtttaggcctgagcccatacacagcttacagagactggagtctttcttagacccaggggcacaaccttcactgaaaaattcatcaaatctgcagtggttgatcttattgtagagcaggcccatggggatgttccagccagcggttctgccaactgccgtatggcaggacttcttgcctttcagattgtcccaggtgaggtcagaagctgatttcttcaccactgctatagcaaaataccctgcctctggtgtatcctcacaattatcgctcttattgtagttttctgccaagacaggcaccagaccacacttgcccgctatgtagacaaaccctccatccaagctcatggcatcagcttctccattcatgatcttggcgatgcagtcttcggtggtctctgctgatacacactctattttccctacactgttaacactccactcatcacacttgagcctctcgtggtggctcagcgcacaccacttcacaggcttgcattcatctgttggggcttctgggcatgtgccttcccgtagattccggatggcagtgacatactcatagcccaggtacatcttggcatccatcctgggggggacttttaaaaacccgtgggcagagtccttaaacagcaggtccttcccatgaggagagctgaatagttggaattcttttgatttgtctttgccaaaatgttcctgggcctggttgagaagctcccagatcaagtcctccttgccgcccatacttcgggccacgacggtatgagaagggacctgggccaagtggcagtccttgtattcatctaccggcttccgggtgttgtccaggcaaagcagctcatactggtccctgtcagccttgtttgccaagttctcaaatatagtcgagtgcttgacaaaggccacatccccagcaccatccttcagacacttgaaggctcccgagtagccgaagtattggttaagggtggagcagccacaccctggacacagttgacacagctgggggaagtccgtcccatccgcacaaggggcacagctgcccgagaagaaattggccactgctttctcaagaggtttacgtggctcaggtaagtcacagtaaagtaagcctatggggatgttccacccagcggacctgcctagacccgtgtggcaggacttcttgcctcgaagctggttcatctggaagccactatccttcttcaccacagcaacagcataatagaaagtctgtggatcctcttttgacccatagaactctgccaccacaggcttcaggttattgggagccaggtaagcatcatacaccaaacctgcatccagtgtcacagcatccgcttcgtttgccgcaatggccctgatgcaatcaaggtaggaggctttcttcacacaagcaacactgggaccatcggatggaatgacgcttttcatatggtcgcggaaactctggcacttagtggcctcatgctccgacactgcacaccatctcacagttttatcagggacagccagacacagccccaggacggcgcagaccagcagggctcccacggcgagcctcatcttccgggtgcggcgctgagcagcgagcacagtcggactcgcttctgt

SEQ ID NO: 12119 - RNA, 94 nt, Homo sapiens
  source 1..94: mol_type = other RNA
ctgcagactcgacctcccaggctcaggtgatcctcccacctcagcctcctgagtagctgggactacaggcatgtgccaccacgcctagctaatt

SEQ ID NO: 12120 - RNA, 2409 nt, Homo sapiens
  source 1..2409: mol_type = other RNA
ctgcagactcgacctcccaggctcaggtgatcctcctgtctcagcttcctgagtagctgggaccacaggcatacatcaccacgcctagctaatgtttttttcttttgtagtgacaaggtctgtgttgcccagcctggtcttgaattcctgggctcaagcaatccgcccaccttggcctcccaaaatgttgaaattacatgtatgagccactgcccaaaaatgtaatcagccctaaaatagtctttaattataaaattatttcttactactacagcattgtgagacagccagggagttagccaggaagttattactgttcctattttataaagagagatcacttaattctagaactccctcaaggcctcccatagctaataaataagactagaacttgagtcttaagaatcttagtctactgctgtcttacctacacttcccttttctgtgtggacaacaaagtattcttctgtgtctttttttttttttttggtcatttcctttttatctgtcaggcagccagctctgacttactctctgtttctgtcatctctcccccacataccaacttcttcaccatgatgattataccaataatacagttccttatatgaggggctctggaaaattagacagtgaagcatgttgcagattacatgttaaacaggtctaattcacaatgaatgacaacttgagacaatatgagacagttttcagacaacagttttgtggcaggtaggggactcctttctctgcatactcttcttggctgaggttgtgttgcactggctgaggttgctgaaacagtggcccatggatggagatgtagaatcagaagcaaggagacacagttctccgctggagtcttctaaagaaatcaagcctgcccatacttttgattttggccttctggtctccagaacttaacccaaaagtccaagtcaaaagtctcatccaagacaaggaaaattccttctgcctgtgagcccatactgttgcaaacaaggtacacatgtggtttccagagggaaacaaaatgagactcaaggcagtagcatttgtagtggttcctaagcatggagagaggacctgagctgtaagccgttctctcttctctctctctctcttcagctatctgctcctggacaaatcttcaacttcctggctggctctcttcttcccattgatcctcactcatttcctctgggttttccatgcgtgtggcgtgcttcgggcagggctacatgcttgggctttttggctttgctggattcctcttggcagtcacacttggactccacagctccattagccacttccttcttctgtctgtttgttttgaggacatctggtgaaacagacaatggagaacagccatccatgggtcggggggaattgagaaggatgttcagtagtaacccagggatgacttggtgacggaaaagaaggcacacattttaaatctgcagaggacatcaaattagatgtggttgagcagtaaatgcagatccttcagctggtaaagttgaccctcaagtctgagctgaagattttctcagaaactttcaaatcaagatctagatctccacagataagaataatggagtgactccaccagtagattttactcgtctcaggtaattctgctggaaagggaaggaagtaaatcttggagtcctgcacttccatccgttaatcatatacatgcacgccctcaaaagcagtaaatcactgtctttcactgtattgccatgattcacacctgaagagcactcatcagtcattctgactgtcttgtgataatgcttcagcaaacccaccagtgaaatgagcttgttgccaattcctggaaatcttccccatccagaaagtctcctaccggaacatgctgggtgttaacacatctgtagtcacctgagggtacttctttaaggtggagaattcccagcgatcaaattgtaatccatatagaaaaggtatcatcaaaaattccaatgatttaacttttaagcaactccagatgaatccaggaatgatttgaccttgtattggtacttccatattgttggctgatggaaagatccagtaagaacaacgcagaatgaaggaggtcagtgctaggaagtactccagcaaattcatgatgctttctagatgctgataatagtaattacaccttcttccccacttcgtcgcacttttaagggacatttcccccgctgcagtccacgaggcgttcggacactttttcccggcctgacagcagagaaagtcggggcggcaaagttgcgagagggagataccccggcgtccgggggagaggggaggaaagagagttcatcagagttcccccttttgttccaagtcccggagcagacaaagaggcggcgagcggcggcaggtttctcc

SEQ ID NO: 12121 - RNA, 1659 nt, Homo sapiens
  source 1..1659: mol_type = other RNA
ctgcagactcgacctcccaggctcaggtgattctcccgcctcagcctcccaggtagttgggactacaagcgtgcataactccgccaggataattttttgtatttattgtagagacggggtttcgccatgttgcccaggctgatcttgaactcctgacctcaggtgatcatcccgcctcagcctctcacagtgctgggattacaggcgtgagccaccgcacctggctaatagctatttattgaaagtactgtgataagcattttagattcattgtatcattttaaatttacagggcaactcattgaggttaaaatcattctatctcctttagaaacttcaaaactgatcttagttcaagaaagaagttactattcagtgatcaccgaggctctaacaagtggagcctagattcgaaaccaaaccctgtgacttcaacacccaaacatttacgttcttacgttttactgtacagccttcctcctggataaatcagattaaaattttgaagacatgtatatagcttgtcagggtagtacagttattaattctgtggttaccacattcttttatatctcaagactcccagccccaggatctaagtcatagctcttgattatggcccacccccagtagggagctgaacttactacttctgatatgaaagaagccagagtagttgtttcttccaagtcactcacatctgagatggccctcaaaccctccttggtggtctccggctgagagatgtttgcgtctttctgatcttggtaatactggatcaactgctgaaccccagaccttaatgcaggtttaagtgcagcactgatcgctagacccataggcccccctgacatcccagccatggtcatcagaaggtcatatcccagatctatggccccatctcggcctcgttccctggccttgcccaggcagttttgagtagcataatacaaagctgtgcccaggttgtagaaggttcccactcctggcagcagctggactacattgtgcacagcttgctccttctcattctcacagtcctctgtcgggagggagcgcccgacccttcctgtgctttgctgctccctggctaacagctgcagagcagaggccagggcttccactgacacgttcctctctgtgcttctgcctttctggagccctcgaagatgctggatgaggacctgtgtagcattcacaccaccctggcggtagagctgtagctgtagagcccaaacatcagcctgacaaccagcttcctccagggcattccttagagccaggcttaccaagaacttgggtagaggggccatgtggctgaaaccaggcagtgactttgggtgcagaaattggcaggacaaggggtctgaggagggtgtctgggattccaaggacaagggaaagtgcatcaagacatttgtctgctttccatatgaagtggcatccacagggtgcagcaggaggtagcaaagtagcagctcaactggtatcatgatgagtctgaggccacgcatgtctggagcagagtacccacacagtccagtcattgagaagtgagactgccttggtaggtttgatcgcttcctgatcctgttctgcctagttctgtgtcccatgaggaaaggagatatttgctttcccctatgatcagtgaaggat

SEQ ID NO: 12122 - RNA, 5921 nt, Homo sapiens
  source 1..5921: mol_type = other RNA
ctgcagactcgacctcccaggctcaggtgtttctgcctcctaagtagctgggactacatgggactacatgcacatgccaccatgcctggctaattgtttgtatattttttttgtagagatgggctttcatcatgttgcccaggctgggcttgaactcctgggcttaagtgatctgcctgcctcggcctcccacgtgctgggattataggcatgagccaatgtgcccggcctcaaccatttcttgataagttaagggccttcacagtaatatcaattactgtgcttggctataaagtcattacactggagagcatataactgatgctcagaatgaaggctctgaaatcatcgagaaatggtttggctgctcagaactctttctttttccttctttcttgctcatggattttcagctgtccattccctactggagggctgggtccaactgcttgttcactggcacagtgccttccatgtacaaagtgatcaaacctgtctattaattaagcaaatgagtggtgaatcactgagacggctggatggctgagctgagggatgtgatgtgtgcccaacgtcctgcagggtgctggtgaataacatgagaaagaacttaaaatggcttgatgatctcaccatttagtgaccttggttgtcacactgctttccaagagccctttaaaggtaggaatgagagctgtttccagtatgcattccaataggaatgcagctttgctaaagttagagacataaactaaaaccctgtgaagtcctatagagcccttggacttatttcctagcaagcatttatcatccccaccatcctctacttcaggacacttgagcagaaacagtcaaggtttttgccgttttcatcctgctcttcaaaacactgtaagtagtggcgcaggtaagcacagccacaggtgaagaccgttttcagctgaggctgcacatcagaaccacagatcacaggggatggtgcgtgacaatcgtctcagttctcccagtaatgcccatgctagccccaggctcgatgccaggagggaagtgcattccttactgagggagggcatcaggcgtgggtcttccacggaaccccaataggaatcagcaacccccaagcagatattactcaaaggtggtattacatacaacagtagtcagactcagacttcaagcagcccaaagagtggaaccacaggcttgcacaattataaaatgtttttatttcaattacataataacacgttttcctcaaattttattgaggttttggtctttttgcattcaattctatcttgtaacagtaatatgaatccacataatttcataaaatgtcaacaacattcataaggtacattcctttgtgattttatattttacaattttaaatctaactttacaattattttaaaaaatttttttatatagaaaacagatattttcttcaggcagatcaaaacaagaattttccagtaagaatatactgggacataacaaatgaaaatatttataccaaaataccaaaagtgattcagctctttaaaatatcctactatagtctaattagtagcttgtacaagaacaagtaaccattttttactgctcttttgaatgatgattagaaattcaaacaaagtattttaaggttcaaaaactttttttttttttttttttttttttagagacagtgtctcactctgtctcccaggctagagtacagtgtgcaatcatagctcactgcagccttgaactcctggcctcaagcaatcctcccaccttggcttcccaatgtgctaggtttacaggcgtgaaaacattgtgttgtgtgtgtgtgtgtttttttttttttttttagacagagtttcgctcttgttgtccaggctggagtacaatggcttgatcttggctcactgcaatctctgcctcgcaggttcaagcgattctcctgcctcagcctctggagtggctgggattacaggcgcccaccatcacgcccggccaattttttgtatttttagtagagacagggtttcaccatgttggccaggctggcctcgaactcttgacctcaggtgatccacctgccttggcctcccaatgtactgagattacaggcatgagccaccacgcccggccaaaaacatttaaaaaatgactgtccctgctcaaatactgcagtaggaaatgtaatttgacatatatcacttccagaaaaaaactttaaatctttctataaaatgaatttgatacatcatcagcatgaagtgaagttaaaatctcttacaaagtaaattcaggtatatcaacaatgagatccaaaagtatcggttcaagatcaaagactcatatgaggtaaaggcaaataaagcccctcatgctttcagacatttacttgttatccttaaaatgattattgttctaaggtgcaaatcttatcattcagtgacctatttgctatttggctgtttatctcctttaaataaaataccatacaggttataatgtacattttaaaatcaaatatgaaagtacacatatgtgaacaagacattaatttaaatatcaattatattcataatacagaagtctaagaatgctatttggtcatttcaattagatgctgatatatttggtcaagaaaacccacattcctatcagcctaaggcaaatagtaaatgcctctatttttattaagtggactataaacagtagacattattgtttgatactactggaatgctctcaattagaacgtacactgataacaaatatgtctttctaatctgggtgataacctcaatgattacatggaaatctacaagtaacagtctataacttaaagcagtagagcacctggtaattgtcatacagtgcctctctatgaatttagaacattctacttacattggcagtggagagaaaagaccccttcacactgagacttcctgtgcaccgcgcctgccgcctgcctcagcttaggacatggtacagtcttctttgcttttgcccttctcattccctcctctggtatcttctctgctttctggattgaagtgccctggctctcttcctggtgccgacaagtcatcgttctctaggctattgctgtctaaagctttcctgacggtctgacttggatgttctgacatctcacacctctctgtactttctgcttcacaggcatcactaatgtcctgtgagggactttcatgttcgggcagggtgcagcgatctgcgtcttcgctctttggttctgcaggactgctttgagtggcaccatctattttagcattatcttttgcaacaccttcatctaattcttcaccaccagccctcgggcctgatgattgaacggtgtcatcctcaaaatctaatgtgtctccatcagctagtacctcctcagctgctgtttgtacatcatcaccttcttggtcaagttttccatccaacttaattttaggattctccggacaatcaacattttcactgctttctgctgcaattttctgttttggattttcagtcacctcgttttgggcttccactgctgactttctgtcagtagactttacctgctcttcttccttaatttcacttaaatctgtgttctgatacgttaactcttttttaacatctttaagggtttctacgggtactggggattttttcttcttgtttttctttttcttgttctttgtcttcttctgcgatgagtccaatgcctctccctgttggtcactcttttcttcatcgggctctttcatatctaagggttcattttgagtgtctactgtacttggacctgtcgcttcctgacagttgccctcagttcctgctggagaaccaggaacttctgtcttgattggtttctcgtcccttaatcctgtttcttcaccctcttcttcgttgtgatccctacctacttctgtactgtgcgctggaacctccttgggctcagctgcttcctggttggtgaattctttctctaaactatgccctgtgcttgtctctaactcttgggggacctctaccatacatttgtcatcatgataaactgtgtcatcactatgccctaaaggacacgaggccactgtgcctgcctgctcttcaacctgagtcactgctgcctctcccacattctctgtgtggttcccaccatctaagtcactccaacagttggatggctcaaggggagttctggtcctgtcatctggtgcacccatgacctcatttgactcaacctgtactgtgttttcagggagagaactgctctcaagaatttggctttgaacctgttcctcataggtagcacctgctaaggttcctaggaatggggcagtgtcttcagaggatttctggtcctcggtattctcaccagcagggaatacctctatgtccacacagtccttcactgtgtcctctgtgtgttgttctttctcagtattgtgcaagatttctcttttccccacattcgccacgatttcatttttcacctccacttcactggctcttcctagggtcccatcccctgtcgacttgagggcatttaactcttcttttgtcatcttggtaggaccttggtatccaacattattgagggtgtcggaagtctctccattggtagctatttctgaatttaggattattccatgtttctcgagcatttcctctctttgcttcagggcctccttgacttcagcaaactgaaattgcagtatactgtgggcgtgtttttccctttcaaattctttgtttttctcttcgtactgccgcctagattcagccagctgttcttcaagctccagcaacatatcttttagggtatcaacctggtacatgaagtttgtcttttcattgtctagctgagcattggaaaccatagccttcttatatttctcttcaacttctgctagagagtccttcatctctttcaatccctgcatgtatttgccttctacatcctgaatctggtcctttaactcattgagttccttgatttccctgatggatgcctcggtgtcgatggagatggaggtgtctccgctgcctctccgagaggaagtcccacccagagaggccagcgtggctgcagacaggcccggcatgttacgagaccccttctcagtaaaatctttttctggtctctcttctaccacagggctggcccgggccgagctggccctggaggaggcgcgggagctggagttgaggtggccgctgtactccgagggagcacgggagccggaggtgctgccccgtcgggtcccaccgaagctgccttcatccaacacagacgcccggtaactccccgaaggccgggcagcgctgtacagacaggagggcaacttctcctccctggatgatgacaaagtagagaatctgctgtcaccgctgtagctggaattcctgccagatcttctattcagggactgtgatccatacaattctccatcataaccatttgtccaggcgtaaggacccccatactccaagtcaggctgcgacctcaggcttccacgactacccactgacatgcgctcgtcttcatcagaagccgatgtgtttcttctggatctacgagagtagcgctcactgtcttccatccactgctcgatgtcaccccattttgtatccagcccataatatttcttttggacctgatagatctccttctgctgccgctccagctccttcatgcggatctcgcgagcctccgcgcgggccgcccgttttgcagcgagccgggcttccgcctcccgcgcgatctggttgagcgcgtcgtcctccgccgtgagccgctcccggttggggagccgcttgcgccccgatccctgggtgcccatgtccatcgaccgcgtcgcccgcagctgccgcggggcccgttgctccagccgctcgcgccgccccggcccggcccc

SEQ ID NO: 12123 - RNA, 5499 nt, Homo sapiens
  source 1..5499: mol_type = other RNA
ctgcagactcgacctcccaggctcaggtgtttctgcctcctaagtagctgggactacatgggactacatgcacatgccaccatgcctggctaattgtttgtatattttttttgtagagatgggctttcatcatgttgcccaggctgggcttgaactcctgggcttaagtgatctgcctgcctcggcctcccacgtgctgggattataggcatgagccaatgtgcccggcctcaaccatttcttgataagttaagggccttcacagtaatatcaattactgtgcttggctataaagtcattacactggagagcatataactgatgctcagaatgaaggctctgaaatcatcgagaaatggtttggctgctcagaactctttctttttccttctttcttgctcatggattttcagctgtccattccctactggagggctgggtccaactgcttgttcactggcacagtgccttccatgtacaaagtgatcaaacctgtctattaattaagcaaatgagtggtgaatcactgagacggctggatggctgagctgagggatgtgatgtgtgcccaacgtcctgcagggtgctggtgaataacatgagaaagaacttaaaatggcttgatgatctcaccatttagtgaccttggttgtcacactgctttccaagagccctttaaaggtaggaatgagagctgtttccagtatgcattccaataggaatgcagctttgctaaagttagagacataaactaaaaccctgtgaagtcctatagagcccttggacttatttcctagcaagcatttatcatccccaccatcctctacttcaggacacttgagcagaaacagtcaaggtttttgccgttttcatcctgctcttcaaaacactgtaagtagtggcgcaggtaagcacagccacaggtgaagaccgttttcagctgaggctgcacatcagaaccacagatcacaggggatggtgcgtgacaatcgtctcagttctcccagtaatgcccatgctagccccaggctcgatgccaggagggaagtgcattccttactgagggagggcatcaggcgtgggtcttccacggaaccccaataggaatcagcaacccccaagcagatattactcaaaggtggtattacatacaacagtagtcagactcagacttcaagcagcccaaagagtggaaccacaggcttgcacaattataaaatgtttttatttcaattacataataacacgttttcctcaaattttattgaggttttggtctttttgcattcaattctatcttgtaacagtaatatgaatccacataatttcataaaatgtcaacaacattcataaggtacattcctttgtgattttatattttacaattttaaatctaactttacaattattttaaaaaatttttttatatagaaaacagatattttcttcaggcagatcaaaacaagaattttccagtaagaatatactgggacataacaaatgaaaatatttataccaaaataccaaaagtgattcagctctttaaaatatcctactatagtctaattagtagcttgtacaagaacaagtaaccattttttactgctcttttgaatgatgattagaaattcaaacaaagtattttaaggttcaaaaactttttttttttttttttttttttttagagacagtgtctcactctgtctcccaggctagagtacagtgtgcaatcatagctcactgcagccttgaactcctggcctcaagcaatcctcccaccttggcttcccaatgtgctaggtttacaggcgtgaaaacattgtgttgtgtgtgtgtgtgtttttttttttttttttagacagagtttcgctcttgttgtccaggctggagtacaatggcttgatcttggctcactgcaatctctgcctcgcaggttcaagcgattctcctgcctcagcctctggagtggctgggattacaggcgcccaccatcacgcccggccaattttttgtatttttagtagagacagggtttcaccatgttggccaggctggcctcgaactcttgacctcaggtgatccacctgccttggcctcccaatgtactgagattacaggcatgagccaccacgcccggccaaaaacatttaaaaaatgactgtccctgctcaaatactgcagtaggaaatgtaatttgacatatatcacttccagaaaaaaactttaaatctttctataaaatgaatttgatacatcatcagcatgaagtgaagttaaaatctcttacaaagtaaattcaggtatatcaacaatgagatccaaaagtatcggttcaagatcaaagactcatatgaggtaaaggcaaataaagcccctcatgctttcagacatttacttgttatccttaaaatgattattgttctaaggtgcaaatcttatcattcagtgacctatttgctatttggctgtttatctcctttaaataaaataccatacaggttataatgtacattttaaaatcaaatatgaaagtacacatatgtgaacaagacattaatttaaatatcaattatattcataatacagaagtctaagaatgctatttggtcatttcaattagatgctgatatatttggtcaagaaaacccacattcctatcagcctaaggcaaatagtaaatgcctctatttttattaagtggactataaacagtagacattattgtttgatactactggaatgctctcaattagaacgtacactgataacaaatatgtctttctaatctgggtgataacctcaatgattacatggaaatctacaagtaacagtctataacttaaagcagtagagcacctggtaattgtcatacagtgcctctctatgaatttagaacattctacttacattggcagtggagagaaaagaccccttcacactgagacttcctgtgcaccgcgcctgccgcctgcctcagcttaggacatggtacagtcttctttgcttttgcccttctcattccctcctctggtatcttctctgctttctggattgaagtgccctggctctcttcctggtgccgacaagtcatcgttctctaggctattgctgtctaaagctttcctgacggtctgacttggatgttctgacatctcacacctctctgtactttctgcttcacaggcatcactaatgtcctgtgagggactttcatgttcgggcagggtgcagcgatctgcgtcttcgctctttggttctgcaggactgctttgagtggcaccatctattttagcattatcttttgcaacaccttcatctaattcttcaccaccagccctcgggcctgatgattgaacggtgtcatcctcaaaatctaatgtgtctccatcagctagtacctcctcagctgctgtttgtacatcatcaccttcttggtcaagttttccatccaacttaattttaggattctccggacaatcaacattttcactgctttctgctgcaattttctgttttggattttcagtcacctcgttttgggcttccactgctgactttctgtcagtagactttacctgctcttcttccttaatttcacttaaatctgtgttctgatacgttaactcttttttaacatctttaagggtttctacgggtactggggattttttcttcttgtttttctttttcttgttctttgtcttcttctgcgatgagtccaatgcctctccctgttggtcactcttttcttcatcgggctctttcatatctaagggttcattttgagtgtctactgtacttggacctgtcgcttcctgacagttgccctcagttcctgctggagaaccaggaacttctgtcttgattggtttctcgtcccttaatcctgtttcttcaccctcttcttcgttgtgatccctacctacttctgtactgtgcgctggaacctccttgggctcagctgcttcctggttggtgaattctttctctaaactatgccctgtgcttgtctctaactcttgggggacctctaccatacatttgtcatcatgataaactgtgtcatcactatgccctaaaggacacgaggccactgtgcctgcctgctcttcaacctgagtcactgctgcctctcccacattctctgtgtggttcccaccatctaagtcactccaacagttggatggctcaaggggagttctggtcctgtcatctggtgcacccatgacctcatttgactcaacctgtactgtgttttcagggagagaactgctctcaagaatttggctttgaacctgttcctcataggtagcacctgctaaggttcctaggaatggggcagtgtcttcagaggatttctggtcctcggtattctcaccagcagggaatacctctatgtccacacagtccttcactgtgtcctctgtgtgttgttctttctcagtattgtgcaagatttctcttttccccacattcgccacgatttcatttttcacctccacttcactggctcttcctagggtcccatcccctgtcgacttgagggcatttaactcttcttttgtcatcttggtaggaccttggtatccaacattattgagggtgtcggaagtctctccattggtagctatttctgaatttaggattattccatgtttctcgagcatttcctctctttgcttcagggcctccttgacttcagcaaactgaaattgcagtatactgtgggcgtgtttttccctttcaaattctttgtttttctcttcgtactgccgcctagattcagccagctgttcttcaagctccagcaacatatcttttagggtatcaacctggtacatgaagtttgtcttttcattgtctagctgagcattggaaaccatagccttcttatatttctcttcaacttctgctagagagtccttcatctctttcaatccctgcatgtatttgccttctacatcctgaatctggtcctttaactcattgagttccttgatttccctgatggatgcctcggtgtcgatggagatggaggtgtctccgctgcctctccgagaggaagtcccacccagagaggccagcgtggctgcagacaggcccggcatgttacgagaccccttctcagtaaaatctttttctggtctctcttctaccctcaggcttccacgactacccactgacatgcgctcgtcttcatcagaagccgatgtgtttcttctggatctacgagagtagcgctcactgtcttcctccttctgctgccgctccagctccttcatgcggatctcgcgagcctccgcgcgggccgcccgttttgcagcgagccgggcttccgccagcttctgcgcttccgggctcaaacagtcgatctcccggctttgagcggccgcggggctggtcatcctgccgggctcggcccgctccacccggcgggaaatgctcggggaccgcgccgggagcccctcgcgggccgggccagggggcgcgcgctctgtc

SEQ ID NO: 12124 - RNA, 5669 nt, Homo sapiens
  source 1..5669: mol_type = other RNA
ctgcagactcgacctcccaggctcaggtgtttctgcctcctaagtagctgggactacatgggactacatgcacatgccaccatgcctggctaattgtttgtatattttttttgtagagatgggctttcatcatgttgcccaggctgggcttgaactcctgggcttaagtgatctgcctgcctcggcctcccacgtgctgggattataggcatgagccaatgtgcccggcctcaaccatttcttgataagttaagggccttcacagtaatatcaattactgtgcttggctataaagtcattacactggagagcatataactgatgctcagaatgaaggctctgaaatcatcgagaaatggtttggctgctcagaactctttctttttccttctttcttgctcatggattttcagctgtccattccctactggagggctgggtccaactgcttgttcactggcacagtgccttccatgtacaaagtgatcaaacctgtctattaattaagcaaatgagtggtgaatcactgagacggctggatggctgagctgagggatgtgatgtgtgcccaacgtcctgcagggtgctggtgaataacatgagaaagaacttaaaatggcttgatgatctcaccatttagtgaccttggttgtcacactgctttccaagagccctttaaaggtaggaatgagagctgtttccagtatgcattccaataggaatgcagctttgctaaagttagagacataaactaaaaccctgtgaagtcctatagagcccttggacttatttcctagcaagcatttatcatccccaccatcctctacttcaggacacttgagcagaaacagtcaaggtttttgccgttttcatcctgctcttcaaaacactgtaagtagtggcgcaggtaagcacagccacaggtgaagaccgttttcagctgaggctgcacatcagaaccacagatcacaggggatggtgcgtgacaatcgtctcagttctcccagtaatgcccatgctagccccaggctcgatgccaggagggaagtgcattccttactgagggagggcatcaggcgtgggtcttccacggaaccccaataggaatcagcaacccccaagcagatattactcaaaggtggtattacatacaacagtagtcagactcagacttcaagcagcccaaagagtggaaccacaggcttgcacaattataaaatgtttttatttcaattacataataacacgttttcctcaaattttattgaggttttggtctttttgcattcaattctatcttgtaacagtaatatgaatccacataatttcataaaatgtcaacaacattcataaggtacattcctttgtgattttatattttacaattttaaatctaactttacaattattttaaaaaatttttttatatagaaaacagatattttcttcaggcagatcaaaacaagaattttccagtaagaatatactgggacataacaaatgaaaatatttataccaaaataccaaaagtgattcagctctttaaaatatcctactatagtctaattagtagcttgtacaagaacaagtaaccattttttactgctcttttgaatgatgattagaaattcaaacaaagtattttaaggttcaaaaactttttttttttttttttttttttttagagacagtgtctcactctgtctcccaggctagagtacagtgtgcaatcatagctcactgcagccttgaactcctggcctcaagcaatcctcccaccttggcttcccaatgtgctaggtttacaggcgtgaaaacattgtgttgtgtgtgtgtgtgtttttttttttttttttagacagagtttcgctcttgttgtccaggctggagtacaatggcttgatcttggctcactgcaatctctgcctcgcaggttcaagcgattctcctgcctcagcctctggagtggctgggattacaggcgcccaccatcacgcccggccaattttttgtatttttagtagagacagggtttcaccatgttggccaggctggcctcgaactcttgacctcaggtgatccacctgccttggcctcccaatgtactgagattacaggcatgagccaccacgcccggccaaaaacatttaaaaaatgactgtccctgctcaaatactgcagtaggaaatgtaatttgacatatatcacttccagaaaaaaactttaaatctttctataaaatgaatttgatacatcatcagcatgaagtgaagttaaaatctcttacaaagtaaattcaggtatatcaacaatgagatccaaaagtatcggttcaagatcaaagactcatatgaggtaaaggcaaataaagcccctcatgctttcagacatttacttgttatccttaaaatgattattgttctaaggtgcaaatcttatcattcagtgacctatttgctatttggctgtttatctcctttaaataaaataccatacaggttataatgtacattttaaaatcaaatatgaaagtacacatatgtgaacaagacattaatttaaatatcaattatattcataatacagaagtctaagaatgctatttggtcatttcaattagatgctgatatatttggtcaagaaaacccacattcctatcagcctaaggcaaatagtaaatgcctctatttttattaagtggactataaacagtagacattattgtttgatactactggaatgctctcaattagaacgtacactgataacaaatatgtctttctaatctgggtgataacctcaatgattacatggaaatctacaagtaacagtctataacttaaagcagtagagcacctggtaattgtcatacagtgcctctctatgaatttagaacattctacttacattggcagtggagagaaaagaccccttcacactgagacttcctgtgcaccgcgcctgccgcctgcctcagcttaggacatggtacagtcttctttgcttttgcccttctcattccctcctctggtatcttctctgctttctggattgaagtgccctggctctcttcctggtgccgacaagtcatcgttctctaggctattgctgtctaaagctttcctgacggtctgacttggatgttctgacatctcacacctctctgtactttctgcttcacaggcatcactaatgtcctgtgagggactttcatgttcgggcagggtgcagcgatctgcgtcttcgctctttggttctgcaggactgctttgagtggcaccatctattttagcattatcttttgcaacaccttcatctaattcttcaccaccagccctcgggcctgatgattgaacggtgtcatcctcaaaatctaatgtgtctccatcagctagtacctcctcagctgctgtttgtacatcatcaccttcttggtcaagttttccatccaacttaattttaggattctccggacaatcaacattttcactgctttctgctgcaattttctgttttggattttcagtcacctcgttttgggcttccactgctgactttctgtcagtagactttacctgctcttcttccttaatttcacttaaatctgtgttctgatacgttaactcttttttaacatctttaagggtttctacgggtactggggattttttcttcttgtttttctttttcttgttctttgtcttcttctgcgatgagtccaatgcctctccctgttggtcactcttttcttcatcgggctctttcatatctaagggttcattttgagtgtctactgtacttggacctgtcgcttcctgacagttgccctcagttcctgctggagaaccaggaacttctgtcttgattggtttctcgtcccttaatcctgtttcttcaccctcttcttcgttgtgatccctacctacttctgtactgtgcgctggaacctccttgggctcagctgcttcctggttggtgaattctttctctaaactatgccctgtgcttgtctctaactcttgggggacctctaccatacatttgtcatcatgataaactgtgtcatcactatgccctaaaggacacgaggccactgtgcctgcctgctcttcaacctgagtcactgctgcctctcccacattctctgtgtggttcccaccatctaagtcactccaacagttggatggctcaaggggagttctggtcctgtcatctggtgcacccatgacctcatttgactcaacctgtactgtgttttcagggagagaactgctctcaagaatttggctttgaacctgttcctcataggtagcacctgctaaggttcctaggaatggggcagtgtcttcagaggatttctggtcctcggtattctcaccagcagggaatacctctatgtccacacagtccttcactgtgtcctctgtgtgttgttctttctcagtattgtgcaagatttctcttttccccacattcgccacgatttcatttttcacctccacttcactggctcttcctagggtcccatcccctgtcgacttgagggcatttaactcttcttttgtcatcttggtaggaccttggtatccaacattattgagggtgtcggaagtctctccattggtagctatttctgaatttaggattattccatgtttctcgagcatttcctctctttgcttcagggcctccttgacttcagcaaactgaaattgcagtatactgtgggcgtgtttttccctttcaaattctttgtttttctcttcgtactgccgcctagattcagccagctgttcttcaagctccagcaacatatcttttagggtatcaacctggtacatgaagtttgtcttttcattgtctagctgagcattggaaaccatagccttcttatatttctcttcaacttctgctagagagtccttcatctctttcaatccctgcatgtatttgccttctacatcctgaatctggtcctttaactcattgagttccttgatttccctgatggatgcctcggtgtcgatggagatggaggtgtctccgctgcctctccgagaggaagtcccacccagagaggccagcgtggctgcagacaggcccggcatgttacgagaccccttctcagtaaaatctttttctggtctctcttctaccctgccagatcttctattcagggactgtgatccatacaattctccatcataaccatttgtccaggcgtaaggacccccatactccaagtcaggctgcgacctcaggcttccacgactacccactgacatgcgctcgtcttcatcagaagccgatgtgtttcttctggatctacgagagtagcgctcactgtcttccatccactgctcgatgtcaccccattttgtatccagcccataatatttcttttggacctgatagatctccttctgctgccgctccagctccttcatgcggatctcgcgagcctccgcgcgggccgcccgttttgcagcgagccgggcttccgcctcccgcgcgatctggttgagcgcgtcgtcctccgccgtgagccgctcccggttggggagccgcttgcgccccgatccctgggtgcccatgtccatcgaccgcgtcgcccgcagctgccgcggggcccgttgctccagccgctcgcgccgccccggcccggcccc

SEQ ID NO: 12125 - RNA, 5604 nt, Homo sapiens
  source 1..5604: mol_type = other RNA
ctgcagactcgacctcccaggctcaggtgtttctgcctcctaagtagctgggactacatgggactacatgcacatgccaccatgcctggctaattgtttgtatattttttttgtagagatgggctttcatcatgttgcccaggctgggcttgaactcctgggcttaagtgatctgcctgcctcggcctcccacgtgctgggattataggcatgagccaatgtgcccggcctcaaccatttcttgataagttaagggccttcacagtaatatcaattactgtgcttggctataaagtcattacactggagagcatataactgatgctcagaatgaaggctctgaaatcatcgagaaatggtttggctgctcagaactctttctttttccttctttcttgctcatggattttcagctgtccattccctactggagggctgggtccaactgcttgttcactggcacagtgccttccatgtacaaagtgatcaaacctgtctattaattaagcaaatgagtggtgaatcactgagacggctggatggctgagctgagggatgtgatgtgtgcccaacgtcctgcagggtgctggtgaataacatgagaaagaacttaaaatggcttgatgatctcaccatttagtgaccttggttgtcacactgctttccaagagccctttaaaggtaggaatgagagctgtttccagtatgcattccaataggaatgcagctttgctaaagttagagacataaactaaaaccctgtgaagtcctatagagcccttggacttatttcctagcaagcatttatcatccccaccatcctctacttcaggacacttgagcagaaacagtcaaggtttttgccgttttcatcctgctcttcaaaacactgtaagtagtggcgcaggtaagcacagccacaggtgaagaccgttttcagctgaggctgcacatcagaaccacagatcacaggggatggtgcgtgacaatcgtctcagttctcccagtaatgcccatgctagccccaggctcgatgccaggagggaagtgcattccttactgagggagggcatcaggcgtgggtcttccacggaaccccaataggaatcagcaacccccaagcagatattactcaaaggtggtattacatacaacagtagtcagactcagacttcaagcagcccaaagagtggaaccacaggcttgcacaattataaaatgtttttatttcaattacataataacacgttttcctcaaattttattgaggttttggtctttttgcattcaattctatcttgtaacagtaatatgaatccacataatttcataaaatgtcaacaacattcataaggtacattcctttgtgattttatattttacaattttaaatctaactttacaattattttaaaaaatttttttatatagaaaacagatattttcttcaggcagatcaaaacaagaattttccagtaagaatatactgggacataacaaatgaaaatatttataccaaaataccaaaagtgattcagctctttaaaatatcctactatagtctaattagtagcttgtacaagaacaagtaaccattttttactgctcttttgaatgatgattagaaattcaaacaaagtattttaaggttcaaaaactttttttttttttttttttttttttagagacagtgtctcactctgtctcccaggctagagtacagtgtgcaatcatagctcactgcagccttgaactcctggcctcaagcaatcctcccaccttggcttcccaatgtgctaggtttacaggcgtgaaaacattgtgttgtgtgtgtgtgtgtttttttttttttttttagacagagtttcgctcttgttgtccaggctggagtacaatggcttgatcttggctcactgcaatctctgcctcgcaggttcaagcgattctcctgcctcagcctctggagtggctgggattacaggcgcccaccatcacgcccggccaattttttgtatttttagtagagacagggtttcaccatgttggccaggctggcctcgaactcttgacctcaggtgatccacctgccttggcctcccaatgtactgagattacaggcatgagccaccacgcccggccaaaaacatttaaaaaatgactgtccctgctcaaatactgcagtaggaaatgtaatttgacatatatcacttccagaaaaaaactttaaatctttctataaaatgaatttgatacatcatcagcatgaagtgaagttaaaatctcttacaaagtaaattcaggtatatcaacaatgagatccaaaagtatcggttcaagatcaaagactcatatgaggtaaaggcaaataaagcccctcatgctttcagacatttacttgttatccttaaaatgattattgttctaaggtgcaaatcttatcattcagtgacctatttgctatttggctgtttatctcctttaaataaaataccatacaggttataatgtacattttaaaatcaaatatgaaagtacacatatgtgaacaagacattaatttaaatatcaattatattcataatacagaagtctaagaatgctatttggtcatttcaattagatgctgatatatttggtcaagaaaacccacattcctatcagcctaaggcaaatagtaaatgcctctatttttattaagtggactataaacagtagacattattgtttgatactactggaatgctctcaattagaacgtacactgataacaaatatgtctttctaatctgggtgataacctcaatgattacatggaaatctacaagtaacagtctataacttaaagcagtagagcacctggtaattgtcatacagtgcctctctatgaatttagaacattctacttacattggcagtggagagaaaagaccccttcacactgagacttcctgtgcaccgcgcctgccgcctgcctcagcttaggacatggtacagtcttctttgcttttgcccttctcattccctcctctggtatcttctctgctttctggattgaagtgccctggctctcttcctggtgccgacaagtcatcgttctctaggctattgctgtctaaagctttcctgacggtctgacttggatgttctgacatctcacacctctctgtactttctgcttcacaggcatcactaatgtcctgtgagggactttcatgttcgggcagggtgcagcgatctgcgtcttcgctctttggttctgcaggactgctttgagtggcaccatctattttagcattatcttttgcaacaccttcatctaattcttcaccaccagccctcgggcctgatgattgaacggtgtcatcctcaaaatctaatgtgtctccatcagctagtacctcctcagctgctgtttgtacatcatcaccttcttggtcaagttttccatccaacttaattttaggattctccggacaatcaacattttcactgctttctgctgcaattttctgttttggattttcagtcacctcgttttgggcttccactgctgactttctgtcagtagactttacctgctcttcttccttaatttcacttaaatctgtgttctgatacgttaactcttttttaacatctttaagggtttctacgggtactggggattttttcttcttgtttttctttttcttgttctttgtcttcttctgcgatgagtccaatgcctctccctgttggtcactcttttcttcatcgggctctttcatatctaagggttcattttgagtgtctactgtacttggacctgtcgcttcctgacagttgccctcagttcctgctggagaaccaggaacttctgtcttgattggtttctcgtcccttaatcctgtttcttcaccctcttcttcgttgtgatccctacctacttctgtactgtgcgctggaacctccttgggctcagctgcttcctggttggtgaattctttctctaaactatgccctgtgcttgtctctaactcttgggggacctctaccatacatttgtcatcatgataaactgtgtcatcactatgccctaaaggacacgaggccactgtgcctgcctgctcttcaacctgagtcactgctgcctctcccacattctctgtgtggttcccaccatctaagtcactccaacagttggatggctcaaggggagttctggtcctgtcatctggtgcacccatgacctcatttgactcaacctgtactgtgttttcagggagagaactgctctcaagaatttggctttgaacctgttcctcataggtagcacctgctaaggttcctaggaatggggcagtgtcttcagaggatttctggtcctcggtattctcaccagcagggaatacctctatgtccacacagtccttcactgtgtcctctgtgtgttgttctttctcagtattgtgcaagatttctcttttccccacattcgccacgatttcatttttcacctccacttcactggctcttcctagggtcccatcccctgtcgacttgagggcatttaactcttcttttgtcatcttggtaggaccttggtatccaacattattgagggtgtcggaagtctctccattggtagctatttctgaatttaggattattccatgtttctcgagcatttcctctctttgcttcagggcctccttgacttcagcaaactgaaattgcagtatactgtgggcgtgtttttccctttcaaattctttgtttttctcttcgtactgccgcctagattcagccagctgttcttcaagctccagcaacatatcttttagggtatcaacctggtacatgaagtttgtcttttcattgtctagctgagcattggaaaccatagccttcttatatttctcttcaacttctgctagagagtccttcatctctttcaatccctgcatgtatttgccttctacatcctgaatctggtcctttaactcattgagttccttgatttccctgatggatgcctcggtgtcgatggagatggaggtgtctccgctgcctctccgagaggaagtcccacccagagaggccagcgtggctgcagacaggcccggcatgttacgagaccccttctcagtaaaatctttttctggtctctcttctacctccttctgctgccgctccagctccttcatgcggatctcgcgagcctccgcgcgggccgcccgttttgcagcgagccgggcttccgccagcttctgcgcttccgggctcaaacagtcgatctcccggctttgagcggccgcggggctggtcatcctgccgggctcggcccgctccacccggcgggaaatgctcggggaccgcgccgggagcccctcgcgggccgggccagggggcgcgcgctctgtccgcggagacggagccactcgccgctaagtgaacgctcgcgcttccggggccaggagccagcccgccggggagcggctcgcggcgctgggctcgggcgcggccgacaggggcggggcgcaggtggccgcgggctgagtcgggctcggggtggaagggcgccggggaagcgggactcgggcgcctccgcccgtcccacggccc

SEQ ID NO: 12126 - RNA, 5498 nt, Homo sapiens
  source 1..5498: mol_type = other RNA
ctgcagactcgacctcccaggctcaggtgtttctgcctcctaagtagctgggactacatgggactacatgcacatgccaccatgcctggctaattgtttgtatattttttttgtagagatgggctttcatcatgttgcccaggctgggcttgaactcctgggcttaagtgatctgcctgcctcggcctcccacgtgctgggattataggcatgagccaatgtgcccggcctcaaccatttcttgataagttaagggccttcacagtaatatcaattactgtgcttggctataaagtcattacactggagagcatataactgatgctcagaatgaaggctctgaaatcatcgagaaatggtttggctgctcagaactctttctttttccttctttcttgctcatggattttcagctgtccattccctactggagggctgggtccaactgcttgttcactggcacagtgccttccatgtacaaagtgatcaaacctgtctattaattaagcaaatgagtggtgaatcactgagacggctggatggctgagctgagggatgtgatgtgtgcccaacgtcctgcagggtgctggtgaataacatgagaaagaacttaaaatggcttgatgatctcaccatttagtgaccttggttgtcacactgctttccaagagccctttaaaggtaggaatgagagctgtttccagtatgcattccaataggaatgcagctttgctaaagttagagacataaactaaaaccctgtgaagtcctatagagcccttggacttatttcctagcaagcatttatcatccccaccatcctctacttcaggacacttgagcagaaacagtcaaggtttttgccgttttcatcctgctcttcaaaacactgtaagtagtggcgcaggtaagcacagccacaggtgaagaccgttttcagctgaggctgcacatcagaaccacagatcacaggggatggtgcgtgacaatcgtctcagttctcccagtaatgcccatgctagccccaggctcgatgccaggagggaagtgcattccttactgagggagggcatcaggcgtgggtcttccacggaaccccaataggaatcagcaacccccaagcagatattactcaaaggtggtattacatacaacagtagtcagactcagacttcaagcagcccaaagagtggaaccacaggcttgcacaattataaaatgtttttatttcaattacataataacacgttttcctcaaattttattgaggttttggtctttttgcattcaattctatcttgtaacagtaatatgaatccacataatttcataaaatgtcaacaacattcataaggtacattcctttgtgattttatattttacaattttaaatctaactttacaattattttaaaaaatttttttatatagaaaacagatattttcttcaggcagatcaaaacaagaattttccagtaagaatatactgggacataacaaatgaaaatatttataccaaaataccaaaagtgattcagctctttaaaatatcctactatagtctaattagtagcttgtacaagaacaagtaaccattttttactgctcttttgaatgatgattagaaattcaaacaaagtattttaaggttcaaaaactttttttttttttttttttttttttagagacagtgtctcactctgtctcccaggctagagtacagtgtgcaatcatagctcactgcagccttgaactcctggcctcaagcaatcctcccaccttggcttcccaatgtgctaggtttacaggcgtgaaaacattgtgttgtgtgtgtgtgtgtttttttttttttttttagacagagtttcgctcttgttgtccaggctggagtacaatggcttgatcttggctcactgcaatctctgcctcgcaggttcaagcgattctcctgcctcagcctctggagtggctgggattacaggcgcccaccatcacgcccggccaattttttgtatttttagtagagacagggtttcaccatgttggccaggctggcctcgaactcttgacctcaggtgatccacctgccttggcctcccaatgtactgagattacaggcatgagccaccacgcccggccaaaaacatttaaaaaatgactgtccctgctcaaatactgcagtaggaaatgtaatttgacatatatcacttccagaaaaaaactttaaatctttctataaaatgaatttgatacatcatcagcatgaagtgaagttaaaatctcttacaaagtaaattcaggtatatcaacaatgagatccaaaagtatcggttcaagatcaaagactcatatgaggtaaaggcaaataaagcccctcatgctttcagacatttacttgttatccttaaaatgattattgttctaaggtgcaaatcttatcattcagtgacctatttgctatttggctgtttatctcctttaaataaaataccatacaggttataatgtacattttaaaatcaaatatgaaagtacacatatgtgaacaagacattaatttaaatatcaattatattcataatacagaagtctaagaatgctatttggtcatttcaattagatgctgatatatttggtcaagaaaacccacattcctatcagcctaaggcaaatagtaaatgcctctatttttattaagtggactataaacagtagacattattgtttgatactactggaatgctctcaattagaacgtacactgataacaaatatgtctttctaatctgggtgataacctcaatgattacatggaaatctacaagtaacagtctataacttaaagcagtagagcacctggtaattgtcatacagtgcctctctatgaatttagaacattctacttacattggcagtggagagaaaagaccccttcacactgagacttcctgtgcaccgcgcctgccgcctgcctcagcttaggacatggtacagtcttctttgcttttgcccttctcattccctcctctggtatcttctctgctttctggattgaagtgccctggctctcttcctggtgccgacaagtcatcgttctctaggctattgctgtctaaagctttcctgacggtctgacttggatgttctgacatctcacacctctctgtactttctgcttcacaggcatcactaatgtcctgtgagggactttcatgttcgggcagggtgcagcgatctgcgtcttcgctctttggttctgcaggactgctttgagtggcaccatctattttagcattatcttttgcaacaccttcatctaattcttcaccaccagccctcgggcctgatgattgaacggtgtcatcctcaaaatctaatgtgtctccatcagctagtacctcctcagctgctgtttgtacatcatcaccttcttggtcaagttttccatccaacttaattttaggattctccggacaatcaacattttcactgctttctgctgcaattttctgttttggattttcagtcacctcgttttgggcttccactgctgactttctgtcagtagactttacctgctcttcttccttaatttcacttaaatctgtgttctgatacgttaactcttttttaacatctttaagggtttctacgggtactggggattttttcttcttgtttttctttttcttgttctttgtcttcttctgcgatgagtccaatgcctctccctgttggtcactcttttcttcatcgggctctttcatatctaagggttcattttgagtgtctactgtacttggacctgtcgcttcctgacagttgccctcagttcctgctggagaaccaggaacttctgtcttgattggtttctcgtcccttaatcctgtttcttcaccctcttcttcgttgtgatccctacctacttctgtactgtgcgctggaacctccttgggctcagctgcttcctggttggtgaattctttctctaaactatgccctgtgcttgtctctaactcttgggggacctctaccatacatttgtcatcatgataaactgtgtcatcactatgccctaaaggacacgaggccactgtgcctgcctgctcttcaacctgagtcactgctgcctctcccacattctctgtgtggttcccaccatctaagtcactccaacagttggatggctcaaggggagttctggtcctgtcatctggtgcacccatgacctcatttgactcaacctgtactgtgttttcagggagagaactgctctcaagaatttggctttgaacctgttcctcataggtagcacctgctaaggttcctaggaatggggcagtgtcttcagaggatttctggtcctcggtattctcaccagcagggaatacctctatgtccacacagtccttcactgtgtcctctgtgtgttgttctttctcagtattgtgcaagatttctcttttccccacattcgccacgatttcatttttcacctccacttcactggctcttcctagggtcccatcccctgtcgacttgagggcatttaactcttcttttgtcatcttggtaggaccttggtatccaacattattgagggtgtcggaagtctctccattggtagctatttctgaatttaggattattccatgtttctcgagcatttcctctctttgcttcagggcctccttgacttcagcaaactgaaattgcagtatactgtgggcgtgtttttccctttcaaattctttgtttttctcttcgtactgccgcctagattcagccagctgttcttcaagctccagcaacatatcttttagggtatcaacctggtacatgaagtttgtcttttcattgtctagctgagcattggaaaccatagccttcttatatttctcttcaacttctgctagagagtccttgatttccctgatggatgcctcggtgtcgatggagatggaggtgtctccgctgcctctccgagaggaagtcccacccagagaggccagcgtggctgcagacaggcccggcatgttacgagaccccttctcagtaaaatctttttctggtctctcttctaccctcaggcttccacgactacccactgacatgcgctcgtcttcatcagaagccgatgtgtttcttctggatctacgagagtagcgctcactgtcttccatccactgctcgatgtcaccccattttgtatccagcccataatatttcttttggacctgatagatctccttctgctgccgctccagctccttcatgcggatctcgcgagcctccgcgcgggccgcccgttttgcagcgagccgggcttccgcctcccgcgcgatctggttgagcgcgtcgtcctccgccgtgagccgctcccggttggggagccgcttgcgccccgatccctgggtgcccatgtccatcgaccgcgtcgcccgcagctgccgcggggcccgttgctccagccgctcgcgccgccccggcccggcccc

SEQ ID NO: 12127 - RNA, 5427 nt, Homo sapiens
  source 1..5427: mol_type = other RNA
ctgcagactcgacctcccaggctcaggtgtttctgcctcctaagtagctgggactacatgggactacatgcacatgccaccatgcctggctaattgtttgtatattttttttgtagagatgggctttcatcatgttgcccaggctgggcttgaactcctgggcttaagtgatctgcctgcctcggcctcccacgtgctgggattataggcatgagccaatgtgcccggcctcaaccatttcttgataagttaagggccttcacagtaatatcaattactgtgcttggctataaagtcattacactggagagcatataactgatgctcagaatgaaggctctgaaatcatcgagaaatggtttggctgctcagaactctttctttttccttctttcttgctcatggattttcagctgtccattccctactggagggctgggtccaactgcttgttcactggcacagtgccttccatgtacaaagtgatcaaacctgtctattaattaagcaaatgagtggtgaatcactgagacggctggatggctgagctgagggatgtgatgtgtgcccaacgtcctgcagggtgctggtgaataacatgagaaagaacttaaaatggcttgatgatctcaccatttagtgaccttggttgtcacactgctttccaagagccctttaaaggtaggaatgagagctgtttccagtatgcattccaataggaatgcagctttgctaaagttagagacataaactaaaaccctgtgaagtcctatagagcccttggacttatttcctagcaagcatttatcatccccaccatcctctacttcaggacacttgagcagaaacagtcaaggtttttgccgttttcatcctgctcttcaaaacactgtaagtagtggcgcaggtaagcacagccacaggtgaagaccgttttcagctgaggctgcacatcagaaccacagatcacaggggatggtgcgtgacaatcgtctcagttctcccagtaatgcccatgctagccccaggctcgatgccaggagggaagtgcattccttactgagggagggcatcaggcgtgggtcttccacggaaccccaataggaatcagcaacccccaagcagatattactcaaaggtggtattacatacaacagtagtcagactcagacttcaagcagcccaaagagtggaaccacaggcttgcacaattataaaatgtttttatttcaattacataataacacgttttcctcaaattttattgaggttttggtctttttgcattcaattctatcttgtaacagtaatatgaatccacataatttcataaaatgtcaacaacattcataaggtacattcctttgtgattttatattttacaattttaaatctaactttacaattattttaaaaaatttttttatatagaaaacagatattttcttcaggcagatcaaaacaagaattttccagtaagaatatactgggacataacaaatgaaaatatttataccaaaataccaaaagtgattcagctctttaaaatatcctactatagtctaattagtagcttgtacaagaacaagtaaccattttttactgctcttttgaatgatgattagaaattcaaacaaagtattttaaggttcaaaaactttttttttttttttttttttttttagagacagtgtctcactctgtctcccaggctagagtacagtgtgcaatcatagctcactgcagccttgaactcctggcctcaagcaatcctcccaccttggcttcccaatgtgctaggtttacaggcgtgaaaacattgtgttgtgtgtgtgtgtgtttttttttttttttttagacagagtttcgctcttgttgtccaggctggagtacaatggcttgatcttggctcactgcaatctctgcctcgcaggttcaagcgattctcctgcctcagcctctggagtggctgggattacaggcgcccaccatcacgcccggccaattttttgtatttttagtagagacagggtttcaccatgttggccaggctggcctcgaactcttgacctcaggtgatccacctgccttggcctcccaatgtactgagattacaggcatgagccaccacgcccggccaaaaacatttaaaaaatgactgtccctgctcaaatactgcagtaggaaatgtaatttgacatatatcacttccagaaaaaaactttaaatctttctataaaatgaatttgatacatcatcagcatgaagtgaagttaaaatctcttacaaagtaaattcaggtatatcaacaatgagatccaaaagtatcggttcaagatcaaagactcatatgaggtaaaggcaaataaagcccctcatgctttcagacatttacttgttatccttaaaatgattattgttctaaggtgcaaatcttatcattcagtgacctatttgctatttggctgtttatctcctttaaataaaataccatacaggttataatgtacattttaaaatcaaatatgaaagtacacatatgtgaacaagacattaatttaaatatcaattatattcataatacagaagtctaagaatgctatttggtcatttcaattagatgctgatatatttggtcaagaaaacccacattcctatcagcctaaggcaaatagtaaatgcctctatttttattaagtggactataaacagtagacattattgtttgatactactggaatgctctcaattagaacgtacactgataacaaatatgtctttctaatctgggtgataacctcaatgattacatggaaatctacaagtaacagtctataacttaaagcagtagagcacctggtaattgtcatacagtgcctctctatgaatttagaacattctacttacattggcagtggagagaaaagaccccttcacactgagacttcctgtgcaccgcgcctgccgcctgcctcagcttaggacatggtacagtcttctttgcttttgcccttctcattccctcctctggtatcttctctgctttctggattgaagtgccctggctctcttcctggtgccgacaagtcatcgttctctaggctattgctgtctaaagctttcctgacggtctgacttggatgttctgacatctcacacctctctgtactttctgcttcacaggcatcactaatgtcctgtgagggactttcatgttcgggcagggtgcagcgatctgcgtcttcgctctttggttctgcaggactgctttgagtggcaccatctattttagcattatcttttgcaacaccttcatctaattcttcaccaccagccctcgggcctgatgattgaacggtgtcatcctcaaaatctaatgtgtctccatcagctagtacctcctcagctgctgtttgtacatcatcaccttcttggtcaagttttccatccaacttaattttaggattctccggacaatcaacattttcactgctttctgctgcaattttctgttttggattttcagtcacctcgttttgggcttccactgctgactttctgtcagtagactttacctgctcttcttccttaatttcacttaaatctgtgttctgatacgttaactcttttttaacatctttaagggtttctacgggtactggggattttttcttcttgtttttctttttcttgttctttgtcttcttctgcgatgagtccaatgcctctccctgttggtcactcttttcttcatcgggctctttcatatctaagggttcattttgagtgtctactgtacttggacctgtcgcttcctgacagttgccctcagttcctgctggagaaccaggaacttctgtcttgattggtttctcgtcccttaatcctgtttcttcaccctcttcttcgttgtgatccctacctacttctgtactgtgcgctggaacctccttgggctcagctgcttcctggttggtgaattctttctctaaactatgccctgtgcttgtctctaactcttgggggacctctaccatacatttgtcatcatgataaactgtgtcatcactatgccctaaaggacacgaggccactgtgcctgcctgctcttcaacctgagtcactgctgcctctcccacattctctgtgtggttcccaccatctaagtcactccaacagttggatggctcaaggggagttctggtcctgtcatctggtgcacccatgacctcatttgactcaacctgtactgtgttttcagggagagaactgctctcaagaatttggctttgaacctgttcctcataggtagcacctgctaaggttcctaggaatggggcagtgtcttcagaggatttctggtcctcggtattctcaccagcagggaatacctctatgtccacacagtccttcactgtgtcctctgtgtgttgttctttctcagtattgtgcaagatttctcttttccccacattcgccacgatttcatttttcacctccacttcactggctcttcctagggtcccatcccctgtcgacttgagggcatttaactcttcttttgtcatcttggtaggaccttggtatccaacattattgagggtgtcggaagtctctccattggtagctatttctgaatttaggattattccatgtttctcgagcatttcctctctttgcttcagggcctccttgacttcagcaaactgaaattgcagtatactgtgggcgtgtttttccctttcaaattctttgtttttctcttcgtactgccgcctagattcagccagctgttcttcaagctccagcaacatatcttttagggtatcaacctggtacatgaagtttgtcttttcattgtctagctgagcattggaaaccatagccttcttatatttctcttcaacttctgctagagagtccttgatttccctgatggatgcctcggtgtcgatggagatggaggtgtctccgctgcctctccgagaggaagtcccacccagagaggccagcgtggctgcagacaggcccggcatgttacgagaccccttctcagtaaaatctttttctggtctctcttctaccctcaggcttccacgactacccactgacatgcgctcgtcttcatcagaagccgatgtgtttcttctggatctacgagagtagcgctcactgtcttcctccttctgctgccgctccagctccttcatgcggatctcgcgagcctccgcgcgggccgcccgttttgcagcgagccgggcttccgccagcttctgcgcttccgggctcaaacagtcgatctcccggctttgagcggccgcggggctggtcatcctgccgggctcggcccgctccacccggcgggaaatgctcggggaccgcgccgggagcccctcgcgggccgggccagggggcgcgcgctctgtc

SEQ ID NO: 12128 - RNA, 5406 nt, Homo sapiens
  source 1..5406: mol_type = other RNA
ctgcagactcgacctcccaggctcaggtgtttctgcctcctaagtagctgggactacatgggactacatgcacatgccaccatgcctggctaattgtttgtatattttttttgtagagatgggctttcatcatgttgcccaggctgggcttgaactcctgggcttaagtgatctgcctgcctcggcctcccacgtgctgggattataggcatgagccaatgtgcccggcctcaaccatttcttgataagttaagggccttcacagtaatatcaattactgtgcttggctataaagtcattacactggagagcatataactgatgctcagaatgaaggctctgaaatcatcgagaaatggtttggctgctcagaactctttctttttccttctttcttgctcatggattttcagctgtccattccctactggagggctgggtccaactgcttgttcactggcacagtgccttccatgtacaaagtgatcaaacctgtctattaattaagcaaatgagtggtgaatcactgagacggctggatggctgagctgagggatgtgatgtgtgcccaacgtcctgcagggtgctggtgaataacatgagaaagaacttaaaatggcttgatgatctcaccatttagtgaccttggttgtcacactgctttccaagagccctttaaaggtaggaatgagagctgtttccagtatgcattccaataggaatgcagctttgctaaagttagagacataaactaaaaccctgtgaagtcctatagagcccttggacttatttcctagcaagcatttatcatccccaccatcctctacttcaggacacttgagcagaaacagtcaaggtttttgccgttttcatcctgctcttcaaaacactgtaagtagtggcgcaggtaagcacagccacaggtgaagaccgttttcagctgaggctgcacatcagaaccacagatcacaggggatggtgcgtgacaatcgtctcagttctcccagtaatgcccatgctagccccaggctcgatgccaggagggaagtgcattccttactgagggagggcatcaggcgtgggtcttccacggaaccccaataggaatcagcaacccccaagcagatattactcaaaggtggtattacatacaacagtagtcagactcagacttcaagcagcccaaagagtggaaccacaggcttgcacaattataaaatgtttttatttcaattacataataacacgttttcctcaaattttattgaggttttggtctttttgcattcaattctatcttgtaacagtaatatgaatccacataatttcataaaatgtcaacaacattcataaggtacattcctttgtgattttatattttacaattttaaatctaactttacaattattttaaaaaatttttttatatagaaaacagatattttcttcaggcagatcaaaacaagaattttccagtaagaatatactgggacataacaaatgaaaatatttataccaaaataccaaaagtgattcagctctttaaaatatcctactatagtctaattagtagcttgtacaagaacaagtaaccattttttactgctcttttgaatgatgattagaaattcaaacaaagtattttaaggttcaaaaactttttttttttttttttttttttttagagacagtgtctcactctgtctcccaggctagagtacagtgtgcaatcatagctcactgcagccttgaactcctggcctcaagcaatcctcccaccttggcttcccaatgtgctaggtttacaggcgtgaaaacattgtgttgtgtgtgtgtgtgtttttttttttttttttagacagagtttcgctcttgttgtccaggctggagtacaatggcttgatcttggctcactgcaatctctgcctcgcaggttcaagcgattctcctgcctcagcctctggagtggctgggattacaggcgcccaccatcacgcccggccaattttttgtatttttagtagagacagggtttcaccatgttggccaggctggcctcgaactcttgacctcaggtgatccacctgccttggcctcccaatgtactgagattacaggcatgagccaccacgcccggccaaaaacatttaaaaaatgactgtccctgctcaaatactgcagtaggaaatgtaatttgacatatatcacttccagaaaaaaactttaaatctttctataaaatgaatttgatacatcatcagcatgaagtgaagttaaaatctcttacaaagtaaattcaggtatatcaacaatgagatccaaaagtatcggttcaagatcaaagactcatatgaggtaaaggcaaataaagcccctcatgctttcagacatttacttgttatccttaaaatgattattgttctaaggtgcaaatcttatcattcagtgacctatttgctatttggctgtttatctcctttaaataaaataccatacaggttataatgtacattttaaaatcaaatatgaaagtacacatatgtgaacaagacattaatttaaatatcaattatattcataatacagaagtctaagaatgctatttggtcatttcaattagatgctgatatatttggtcaagaaaacccacattcctatcagcctaaggcaaatagtaaatgcctctatttttattaagtggactataaacagtagacattattgtttgatactactggaatgctctcaattagaacgtacactgataacaaatatgtctttctaatctgggtgataacctcaatgattacatggaaatctacaagtaacagtctataacttaaagcagtagagcacctggtaattgtcatacagtgcctctctatgaatttagaacattctacttacattggcagtggagagaaaagaccccttcacactgagacttcctgtgcaccgcgcctgccgcctgcctcagcttaggacatggtacagtcttctttgcttttgcccttctcattccctcctctggtatcttctctgctttctggattgaagtgccctggctctcttcctggtgccgacaagtcatcgttctctaggctattgctgtctaaagctttcctgacggtctgacttggatgttctgacatctcacacctctctgtactttctgcttcacaggcatcactaatgtcctgtgagggactttcatgttcgggcagggtgcagcgatctgcgtcttcgctctttggttctgcaggactgctttgagtggcaccatctattttagcattatcttttgcaacaccttcatctaattcttcaccaccagccctcgggcctgatgattgaacggtgtcatcctcaaaatctaatgtgtctccatcagctagtacctcctcagctgctgtttgtacatcatcaccttcttggtcaagttttccatccaacttaattttaggattctccggacaatcaacattttcactgctttctgctgcaattttctgttttggattttcagtcacctcgttttgggcttccactgctgactttctgtcagtagactttacctgctcttcttccttaatttcacttaaatctgtgttctgatacgttaactcttttttaacatctttaagggtttctacgggtactggggattttttcttcttgtttttctttttcttgttctttgtcttcttctgcgatgagtccaatgcctctccctgttggtcactcttttcttcatcgggctctttcatatctaagggttcattttgagtgtctactgtacttggacctgtcgcttcctgacagttgccctcagttcctgctggagaaccaggaacttctgtcttgattggtttctcgtcccttaatcctgtttcttcaccctcttcttcgttgtgatccctacctacttctgtactgtgcgctggaacctccttgggctcagctgcttcctggttggtgaattctttctctaaactatgccctgtgcttgtctctaactcttgggggacctctaccatacatttgtcatcatgataaactgtgtcatcactatgccctaaaggacacgaggccactgtgcctgcctgctcttcaacctgagtcactgctgcctctcccacattctctgtgtggttcccaccatctaagtcactccaacagttggatggctcaaggggagttctggtcctgtcatctggtgcacccatgacctcatttgactcaacctgtactgtgttttcagggagagaactgctctcaagaatttggctttgaacctgttcctcataggtagcacctgctaaggttcctaggaatggggcagtgtcttcagaggatttctggtcctcggtattctcaccagcagggaatacctctatgtccacacagtccttcactgtgtcctctgtgtgttgttctttctcagtattgtgcaagatttctcttttccccacattcgccacgatttcatttttcacctccacttcactggctcttcctagggtcccatcccctgtcgacttgagggcatttaactcttcttttgtcatcttggtaggaccttggtatccaacattattgagggtgtcggaagtctctccattggtagctatttctgaatttaggattattccatgtttctcgagcatttcctctctttgcttcagggcctccttgacttcagcaaactgaaattgcagtatactgtgggcgtgtttttccctttcaaattctttgtttttctcttcgtactgccgcctagattcagccagctgttcttcaagctccagcaacatatcttttagggtatcaacctggtacatgaagtttgtcttttcattgtctagctgagcattggaaaccatagccttcttatatttctcttcaacttctgctagagagtccttgatttccctgatggatgcctcggtgtcgatggagatggaggtgtctccgctgcctctccgagaggaagtcccacccagagaggccagcgtggctgcagacaggcccggcatgttacgagaccccttctcagtaaaatctttttctggtctctcttctaccctcaggcttccacgactacccactgacatgcgctcgtcttcatcagaagccgatgtgtttcttctggatctacgagagtagcgctcactgtcttcctccttctgctgccgctccagctccttcatgcggatctcgcgagcctccgcgcgggccgcccgttttgcagcgagccgggcttccgcctcccgcgcgatctggttgagcgcgtcgtcctccgccgtgagccgctcccggttggggagccgcttgcgccccgatccctgggtgcccatgtccatcgaccgcgtcgcccgcagctgccgcggggcccgttgctccagc

SEQ ID NO: 12129 - RNA, 5597 nt, Homo sapiens
  source 1..5597: mol_type = other RNA
ctgcagactcgacctcccaggctcaggtgtttctgcctcctaagtagctgggactacatgggactacatgcacatgccaccatgcctggctaattgtttgtatattttttttgtagagatgggctttcatcatgttgcccaggctgggcttgaactcctgggcttaagtgatctgcctgcctcggcctcccacgtgctgggattataggcatgagccaatgtgcccggcctcaaccatttcttgataagttaagggccttcacagtaatatcaattactgtgcttggctataaagtcattacactggagagcatataactgatgctcagaatgaaggctctgaaatcatcgagaaatggtttggctgctcagaactctttctttttccttctttcttgctcatggattttcagctgtccattccctactggagggctgggtccaactgcttgttcactggcacagtgccttccatgtacaaagtgatcaaacctgtctattaattaagcaaatgagtggtgaatcactgagacggctggatggctgagctgagggatgtgatgtgtgcccaacgtcctgcagggtgctggtgaataacatgagaaagaacttaaaatggcttgatgatctcaccatttagtgaccttggttgtcacactgctttccaagagccctttaaaggtaggaatgagagctgtttccagtatgcattccaataggaatgcagctttgctaaagttagagacataaactaaaaccctgtgaagtcctatagagcccttggacttatttcctagcaagcatttatcatccccaccatcctctacttcaggacacttgagcagaaacagtcaaggtttttgccgttttcatcctgctcttcaaaacactgtaagtagtggcgcaggtaagcacagccacaggtgaagaccgttttcagctgaggctgcacatcagaaccacagatcacaggggatggtgcgtgacaatcgtctcagttctcccagtaatgcccatgctagccccaggctcgatgccaggagggaagtgcattccttactgagggagggcatcaggcgtgggtcttccacggaaccccaataggaatcagcaacccccaagcagatattactcaaaggtggtattacatacaacagtagtcagactcagacttcaagcagcccaaagagtggaaccacaggcttgcacaattataaaatgtttttatttcaattacataataacacgttttcctcaaattttattgaggttttggtctttttgcattcaattctatcttgtaacagtaatatgaatccacataatttcataaaatgtcaacaacattcataaggtacattcctttgtgattttatattttacaattttaaatctaactttacaattattttaaaaaatttttttatatagaaaacagatattttcttcaggcagatcaaaacaagaattttccagtaagaatatactgggacataacaaatgaaaatatttataccaaaataccaaaagtgattcagctctttaaaatatcctactatagtctaattagtagcttgtacaagaacaagtaaccattttttactgctcttttgaatgatgattagaaattcaaacaaagtattttaaggttcaaaaactttttttttttttttttttttttttagagacagtgtctcactctgtctcccaggctagagtacagtgtgcaatcatagctcactgcagccttgaactcctggcctcaagcaatcctcccaccttggcttcccaatgtgctaggtttacaggcgtgaaaacattgtgttgtgtgtgtgtgtgtttttttttttttttttagacagagtttcgctcttgttgtccaggctggagtacaatggcttgatcttggctcactgcaatctctgcctcgcaggttcaagcgattctcctgcctcagcctctggagtggctgggattacaggcgcccaccatcacgcccggccaattttttgtatttttagtagagacagggtttcaccatgttggccaggctggcctcgaactcttgacctcaggtgatccacctgccttggcctcccaatgtactgagattacaggcatgagccaccacgcccggccaaaaacatttaaaaaatgactgtccctgctcaaatactgcagtaggaaatgtaatttgacatatatcacttccagaaaaaaactttaaatctttctataaaatgaatttgatacatcatcagcatgaagtgaagttaaaatctcttacaaagtaaattcaggtatatcaacaatgagatccaaaagtatcggttcaagatcaaagactcatatgaggtaaaggcaaataaagcccctcatgctttcagacatttacttgttatccttaaaatgattattgttctaaggtgcaaatcttatcattcagtgacctatttgctatttggctgtttatctcctttaaataaaataccatacaggttataatgtacattttaaaatcaaatatgaaagtacacatatgtgaacaagacattaatttaaatatcaattatattcataatacagaagtctaagaatgctatttggtcatttcaattagatgctgatatatttggtcaagaaaacccacattcctatcagcctaaggcaaatagtaaatgcctctatttttattaagtggactataaacagtagacattattgtttgatactactggaatgctctcaattagaacgtacactgataacaaatatgtctttctaatctgggtgataacctcaatgattacatggaaatctacaagtaacagtctataacttaaagcagtagagcacctggtaattgtcatacagtgcctctctatgaatttagaacattctacttacattggcagtggagagaaaagaccccttcacactgagacttcctgtgcaccgcgcctgccgcctgcctcagcttaggacatggtacagtcttctttgcttttgcccttctcattccctcctctggtatcttctctgctttctggattgaagtgccctggctctcttcctggtgccgacaagtcatcgttctctaggctattgctgtctaaagctttcctgacggtctgacttggatgttctgacatctcacacctctctgtactttctgcttcacaggcatcactaatgtcctgtgagggactttcatgttcgggcagggtgcagcgatctgcgtcttcgctctttggttctgcaggactgctttgagtggcaccatctattttagcattatcttttgcaacaccttcatctaattcttcaccaccagccctcgggcctgatgattgaacggtgtcatcctcaaaatctaatgtgtctccatcagctagtacctcctcagctgctgtttgtacatcatcaccttcttggtcaagttttccatccaacttaattttaggattctccggacaatcaacattttcactgctttctgctgcaattttctgttttggattttcagtcacctcgttttgggcttccactgctgactttctgtcagtagactttacctgctcttcttccttaatttcacttaaatctgtgttctgatacgttaactcttttttaacatctttaagggtttctacgggtactggggattttttcttcttgtttttctttttcttgttctttgtcttcttctgcgatgagtccaatgcctctccctgttggtcactcttttcttcatcgggctctttcatatctaagggttcattttgagtgtctactgtacttggacctgtcgcttcctgacagttgccctcagttcctgctggagaaccaggaacttctgtcttgattggtttctcgtcccttaatcctgtttcttcaccctcttcttcgttgtgatccctacctacttctgtactgtgcgctggaacctccttgggctcagctgcttcctggttggtgaattctttctctaaactatgccctgtgcttgtctctaactcttgggggacctctaccatacatttgtcatcatgataaactgtgtcatcactatgccctaaaggacacgaggccactgtgcctgcctgctcttcaacctgagtcactgctgcctctcccacattctctgtgtggttcccaccatctaagtcactccaacagttggatggctcaaggggagttctggtcctgtcatctggtgcacccatgacctcatttgactcaacctgtactgtgttttcagggagagaactgctctcaagaatttggctttgaacctgttcctcataggtagcacctgctaaggttcctaggaatggggcagtgtcttcagaggatttctggtcctcggtattctcaccagcagggaatacctctatgtccacacagtccttcactgtgtcctctgtgtgttgttctttctcagtattgtgcaagatttctcttttccccacattcgccacgatttcatttttcacctccacttcactggctcttcctagggtcccatcccctgtcgacttgagggcatttaactcttcttttgtcatcttggtaggaccttggtatccaacattattgagggtgtcggaagtctctccattggtagctatttctgaatttaggattattccatgtttctcgagcatttcctctctttgcttcagggcctccttgacttcagcaaactgaaattgcagtatactgtgggcgtgtttttccctttcaaattctttgtttttctcttcgtactgccgcctagattcagccagctgttcttcaagctccagcaacatatcttttagggtatcaacctggtacatgaagtttgtcttttcattgtctagctgagcattggaaaccatagccttcttatatttctcttcaacttctgctagagagtccttgatttccctgatggatgcctcggtgtcgatggagatggaggtgtctccgctgcctctccgagaggaagtcccacccagagaggccagcgtggctgcagacaggcccggcatgttacgagaccccttctcagtaaaatctttttctggtctctcttctaccctgccagatcttctattcagggactgtgatccatacaattctccatcataaccatttgtccaggcgtaaggacccccatactccaagtcaggctgcgacctcaggcttccacgactacccactgacatgcgctcgtcttcatcagaagccgatgtgtttcttctggatctacgagagtagcgctcactgtcttccatccactgctcgatgtcaccccattttgtatccagcccataatatttcttttggacctgatagatctccttctgctgccgctccagctccttcatgcggatctcgcgagcctccgcgcgggccgcccgttttgcagcgagccgggcttccgcctcccgcgcgatctggttgagcgcgtcgtcctccgccgtgagccgctcccggttggggagccgcttgcgccccgatccctgggtgcccatgtccatcgaccgcgtcgcccgcagctgccgcggggcccgttgctccagccgctcgcgccgccccggcccggcccc

SEQ ID NO: 12130 - RNA, 5572 nt, Homo sapiens
  source 1..5572: mol_type = other RNA
ctgcagactcgacctcccaggctcaggtgtttctgcctcctaagtagctgggactacatgggactacatgcacatgccaccatgcctggctaattgtttgtatattttttttgtagagatgggctttcatcatgttgcccaggctgggcttgaactcctgggcttaagtgatctgcctgcctcggcctcccacgtgctgggattataggcatgagccaatgtgcccggcctcaaccatttcttgataagttaagggccttcacagtaatatcaattactgtgcttggctataaagtcattacactggagagcatataactgatgctcagaatgaaggctctgaaatcatcgagaaatggtttggctgctcagaactctttctttttccttctttcttgctcatggattttcagctgtccattccctactggagggctgggtccaactgcttgttcactggcacagtgccttccatgtacaaagtgatcaaacctgtctattaattaagcaaatgagtggtgaatcactgagacggctggatggctgagctgagggatgtgatgtgtgcccaacgtcctgcagggtgctggtgaataacatgagaaagaacttaaaatggcttgatgatctcaccatttagtgaccttggttgtcacactgctttccaagagccctttaaaggtaggaatgagagctgtttccagtatgcattccaataggaatgcagctttgctaaagttagagacataaactaaaaccctgtgaagtcctatagagcccttggacttatttcctagcaagcatttatcatccccaccatcctctacttcaggacacttgagcagaaacagtcaaggtttttgccgttttcatcctgctcttcaaaacactgtaagtagtggcgcaggtaagcacagccacaggtgaagaccgttttcagctgaggctgcacatcagaaccacagatcacaggggatggtgcgtgacaatcgtctcagttctcccagtaatgcccatgctagccccaggctcgatgccaggagggaagtgcattccttactgagggagggcatcaggcgtgggtcttccacggaaccccaataggaatcagcaacccccaagcagatattactcaaaggtggtattacatacaacagtagtcagactcagacttcaagcagcccaaagagtggaaccacaggcttgcacaattataaaatgtttttatttcaattacataataacacgttttcctcaaattttattgaggttttggtctttttgcattcaattctatcttgtaacagtaatatgaatccacataatttcataaaatgtcaacaacattcataaggtacattcctttgtgattttatattttacaattttaaatctaactttacaattattttaaaaaatttttttatatagaaaacagatattttcttcaggcagatcaaaacaagaattttccagtaagaatatactgggacataacaaatgaaaatatttataccaaaataccaaaagtgattcagctctttaaaatatcctactatagtctaattagtagcttgtacaagaacaagtaaccattttttactgctcttttgaatgatgattagaaattcaaacaaagtattttaaggttcaaaaactttttttttttttttttttttttttagagacagtgtctcactctgtctcccaggctagagtacagtgtgcaatcatagctcactgcagccttgaactcctggcctcaagcaatcctcccaccttggcttcccaatgtgctaggtttacaggcgtgaaaacattgtgttgtgtgtgtgtgtgtttttttttttttttttagacagagtttcgctcttgttgtccaggctggagtacaatggcttgatcttggctcactgcaatctctgcctcgcaggttcaagcgattctcctgcctcagcctctggagtggctgggattacaggcgcccaccatcacgcccggccaattttttgtatttttagtagagacagggtttcaccatgttggccaggctggcctcgaactcttgacctcaggtgatccacctgccttggcctcccaatgtactgagattacaggcatgagccaccacgcccggccaaaaacatttaaaaaatgactgtccctgctcaaatactgcagtaggaaatgtaatttgacatatatcacttccagaaaaaaactttaaatctttctataaaatgaatttgatacatcatcagcatgaagtgaagttaaaatctcttacaaagtaaattcaggtatatcaacaatgagatccaaaagtatcggttcaagatcaaagactcatatgaggtaaaggcaaataaagcccctcatgctttcagacatttacttgttatccttaaaatgattattgttctaaggtgcaaatcttatcattcagtgacctatttgctatttggctgtttatctcctttaaataaaataccatacaggttataatgtacattttaaaatcaaatatgaaagtacacatatgtgaacaagacattaatttaaatatcaattatattcataatacagaagtctaagaatgctatttggtcatttcaattagatgctgatatatttggtcaagaaaacccacattcctatcagcctaaggcaaatagtaaatgcctctatttttattaagtggactataaacagtagacattattgtttgatactactggaatgctctcaattagaacgtacactgataacaaatatgtctttctaatctgggtgataacctcaatgattacatggaaatctacaagtaacagtctataacttaaagcagtagagcacctggtaattgtcatacagtgcctctctatgaatttagaacattctacttacattggcagtggagagaaaagaccccttcacactgagacttcctgtgcaccgcgcctgccgcctgcctcagcttaggacatggtacagtcttctttgcttttgcccttctcattccctcctctggtatcttctctgctttctggattgaagtgccctggctctcttcctggtgccgacaagtcatcgttctctaggctattgctgtctaaagctttcctgacggtctgacttggatgttctgacatctcacacctctctgtactttctgcttcacaggcatcactaatgtcctgtgagggactttcatgttcgggcagggtgcagcgatctgcgtcttcgctctttggttctgcaggactgctttgagtggcaccatctattttagcattatcttttgcaacaccttcatctaattcttcaccaccagccctcgggcctgatgattgaacggtgtcatcctcaaaatctaatgtgtctccatcagctagtacctcctcagctgctgtttgtacatcatcaccttcttggtcaagttttccatccaacttaattttaggattctccggacaatcaacattttcactgctttctgctgcaattttctgttttggattttcagtcacctcgttttgggcttccactgctgactttctgtcagtagactttacctgctcttcttccttaatttcacttaaatctgtgttctgatacgttaactcttttttaacatctttaagggtttctacgggtactggggattttttcttcttgtttttctttttcttgttctttgtcttcttctgcgatgagtccaatgcctctccctgttggtcactcttttcttcatcgggctctttcatatctaagggttcattttgagtgtctactgtacttggacctgtcgcttcctgacagttgccctcagttcctgctggagaaccaggaacttctgtcttgattggtttctcgtcccttaatcctgtttcttcaccctcttcttcgttgtgatccctacctacttctgtactgtgcgctggaacctccttgggctcagctgcttcctggttggtgaattctttctctaaactatgccctgtgcttgtctctaactcttgggggacctctaccatacatttgtcatcatgataaactgtgtcatcactatgccctaaaggacacgaggccactgtgcctgcctgctcttcaacctgagtcactgctgcctctcccacattctctgtgtggttcccaccatctaagtcactccaacagttggatggctcaaggggagttctggtcctgtcatctggtgcacccatgacctcatttgactcaacctgtactgtgttttcagggagagaactgctctcaagaatttggctttgaacctgttcctcataggtagcacctgctaaggttcctaggaatggggcagtgtcttcagaggatttctggtcctcggtattctcaccagcagggaatacctctatgtccacacagtccttcactgtgtcctctgtgtgttgttctttctcagtattgtgcaagatttctcttttccccacattcgccacgatttcatttttcacctccacttcactggctcttcctagggtcccatcccctgtcgacttgagggcatttaactcttcttttgtcatcttggtaggaccttggtatccaacattattgagggtgtcggaagtctctccattggtagctatttctgaatttaggattattccatgtttctcgagcatttcctctctttgcttcagggcctccttgacttcagcaaactgaaattgcagtatactgtgggcgtgtttttccctttcaaattctttgtttttctcttcgtactgccgcctagattcagccagctgttcttcaagctccagcaacatatcttttagggtatcaacctggtacatgaagtttgtcttttcattgtctagctgagcattggaaaccatagccttcttatatttctcttcaacttctgctagagagtccttgatttccctgatggatgcctcggtgtcgatggagatggaggtgtctccgctgcctctccgagaggaagtcccacccagagaggccagcgtggctgcagacaggcccggcatgttacgagaccccttctcagtaaaatctttttctggtctctcttctacctccttctgctgccgctccagctccttcatgcggatctcgcgagcctccgcgcgggccgcccgttttgcagcgagccgggcttccgccagcttctgcgcttccgggctcaaacagtcgatctcccggctttgagcggccgcggggctggtcatcctgccgggctcggcccgctccacccggcgggaaatgctcggggaccgcgccgggagcccctcgcgggccgggccagggggcgcgcgctctgtccgcggagacggagccactcgccgctaagtgaacgctcgcgcttccggggccaggagccagcccgccggggagcggctcgcggcgctgggctcgggcgcggccgacaggggcggggcgcaggtggccgcgggctgagtcgggctcggggtggaagggcgccggggaagcgggactcgggcgcctccgcccgtcccacggcccgccccgccccccacgcagttccgcctcggaggggccctcc

SEQ ID NO: 12131 - RNA, 5326 nt, Homo sapiens
  source 1..5326: mol_type = other RNA
ctgcagactcgacctcccaggctcaggtgtttctgcctcctaagtagctgggactacatgggactacatgcacatgccaccatgcctggctaattgtttgtatattttttttgtagagatgggctttcatcatgttgcccaggctgggcttgaactcctgggcttaagtgatctgcctgcctcggcctcccacgtgctgggattataggcatgagccaatgtgcccggcctcaaccatttcttgataagttaagggccttcacagtaatatcaattactgtgcttggctataaagtcattacactggagagcatataactgatgctcagaatgaaggctctgaaatcatcgagaaatggtttggctgctcagaactctttctttttccttctttcttgctcatggattttcagctgtccattccctactggagggctgggtccaactgcttgttcactggcacagtgccttccatgtacaaagtgatcaaacctgtctattaattaagcaaatgagtggtgaatcactgagacggctggatggctgagctgagggatgtgatgtgtgcccaacgtcctgcagggtgctggtgaataacatgagaaagaacttaaaatggcttgatgatctcaccatttagtgaccttggttgtcacactgctttccaagagccctttaaaggtaggaatgagagctgtttccagtatgcattccaataggaatgcagctttgctaaagttagagacataaactaaaaccctgtgaagtcctatagagcccttggacttatttcctagcaagcatttatcatccccaccatcctctacttcaggacacttgagcagaaacagtcaaggtttttgccgttttcatcctgctcttcaaaacactgtaagtagtggcgcaggtaagcacagccacaggtgaagaccgttttcagctgaggctgcacatcagaaccacagatcacaggggatggtgcgtgacaatcgtctcagttctcccagtaatgcccatgctagccccaggctcgatgccaggagggaagtgcattccttactgagggagggcatcaggcgtgggtcttccacggaaccccaataggaatcagcaacccccaagcagatattactcaaaggtggtattacatacaacagtagtcagactcagacttcaagcagcccaaagagtggaaccacaggcttgcacaattataaaatgtttttatttcaattacataataacacgttttcctcaaattttattgaggttttggtctttttgcattcaattctatcttgtaacagtaatatgaatccacataatttcataaaatgtcaacaacattcataaggtacattcctttgtgattttatattttacaattttaaatctaactttacaattattttaaaaaatttttttatatagaaaacagatattttcttcaggcagatcaaaacaagaattttccagtaagaatatactgggacataacaaatgaaaatatttataccaaaataccaaaagtgattcagctctttaaaatatcctactatagtctaattagtagcttgtacaagaacaagtaaccattttttactgctcttttgaatgatgattagaaattcaaacaaagtattttaaggttcaaaaactttttttttttttttttttttttttagagacagtgtctcactctgtctcccaggctagagtacagtgtgcaatcatagctcactgcagccttgaactcctggcctcaagcaatcctcccaccttggcttcccaatgtgctaggtttacaggcgtgaaaacattgtgttgtgtgtgtgtgtgtttttttttttttttttagacagagtttcgctcttgttgtccaggctggagtacaatggcttgatcttggctcactgcaatctctgcctcgcaggttcaagcgattctcctgcctcagcctctggagtggctgggattacaggcgcccaccatcacgcccggccaattttttgtatttttagtagagacagggtttcaccatgttggccaggctggcctcgaactcttgacctcaggtgatccacctgccttggcctcccaatgtactgagattacaggcatgagccaccacgcccggccaaaaacatttaaaaaatgactgtccctgctcaaatactgcagtaggaaatgtaatttgacatatatcacttccagaaaaaaactttaaatctttctataaaatgaatttgatacatcatcagcatgaagtgaagttaaaatctcttacaaagtaaattcaggtatatcaacaatgagatccaaaagtatcggttcaagatcaaagactcatatgaggtaaaggcaaataaagcccctcatgctttcagacatttacttgttatccttaaaatgattattgttctaaggtgcaaatcttatcattcagtgacctatttgctatttggctgtttatctcctttaaataaaataccatacaggttataatgtacattttaaaatcaaatatgaaagtacacatatgtgaacaagacattaatttaaatatcaattatattcataatacagaagtctaagaatgctatttggtcatttcaattagatgctgatatatttggtcaagaaaacccacattcctatcagcctaaggcaaatagtaaatgcctctatttttattaagtggactataaacagtagacattattgtttgatactactggaatgctctcaattagaacgtacactgataacaaatatgtctttctaatctgggtgataacctcaatgattacatggaaatctacaagtaacagtctataacttaaagcagtagagcacctggtaattgtcatacagtgcctctctatgaatttagaacattctacttacattggcagtggagagaaaagaccccttcacactgagacttcctgtgcaccgcgcctgccgcctgcctcagcttaggacatggtacagtcttctttgcttttgcccttctcattccctcctctggtatcttctctgctttctggattgaagtgccctggctctcttcctggtgccgacaagtcatcgttctctaggctattgctgtctaaagctttcctgacggtctgacttggatgttctgacatctcacacctctctgtactttctgcttcacaggcatcactaatgtcctgtgagggactttcatgttcgggcagggtgcagcgatctgcgtcttcgctctttggttctgcaggactgctttgagtggcaccatctattttagcattatcttttgcaacaccttcatctaattcttcaccaccagccctcgggcctgatgattgaacggtgtcatcctcaaaatctaatgtgtctccatcagctagtacctcctcagctgctgtttgtacatcatcaccttcttggtcaagttttccatccaacttaattttaggattctccggacaatcaacattttcactgctttctgctgcaattttctgttttggattttcagtcacctcgttttgggcttccactgctgactttctgtcagtagactttacctgctcttcttccttaatttcacttaaatctgtgttctgatacgttaactcttttttaacatctttaagggtttctacgggtactggggattttttcttcttgtttttctttttcttgttctttgtcttcttctgcgatgagtccaatgcctctccctgttggtcactcttttcttcatcgggctctttcatatctaagggttcattttgagtgtctactgtacttggacctgtcgcttcctgacagttgccctcagttcctgctggagaaccaggaacttctgtcttgattggtttctcgtcccttaatcctgtttcttcaccctcttcttcgttgtgatccctacctacttctgtactgtgcgctggaacctccttgggctcagctgcttcctggttggtgaattctttctctaaactatgccctgtgcttgtctctaactcttgggggacctctaccatacatttgtcatcatgataaactgtgtcatcactatgccctaaaggacacgaggccactgtgcctgcctgctcttcaacctgagtcactgctgcctctcccacattctctgtgtggttcccaccatctaagtcactccaacagttggatggctcaaggggagttctggtcctgtcatctggtgcacccatgacctcatttgactcaacctgtactgtgttttcagggagagaactgctctcaagaatttggctttgaacctgttcctcataggtagcacctgctaaggttcctaggaatggggcagtgtcttcagaggatttctggtcctcggtattctcaccagcagggaatacctctatgtccacacagtccttcactgtgtcctctgtgtgttgttctttctcagtattgtgcaagatttctcttttccccacattcgccacgatttcatttttcacctccacttcactggctcttcctagggtcccatcccctgtcgacttgagggcatttaactcttcttttgtcatcttggtaggaccttggtatccaacattattgagggtgtcggaagtctctccattggtagctatttctgaatttaggattattccatgtttctcgagcatttcctctctttgcttcagggcctccttgacttcagcaaactgaaattgcagtatactgtgggcgtgtttttccctttcaaattctttgtttttctcttcgtactgccgcctagattcagccagctgttcttcaagctccagcaacatatcttttagggtatcaacctggtacatgaagtttgtcttttcattgtctagctgagcattggaaaccatagccttcttatatttctcttcaacttctgctagagagtccttgatttccctgatggatgcctcggtgtcgatggagatggaggtgtctccgctgcctctccgagaggaagtcccacccagagaggccagcgtggctgcagacaggcccggcatgttacgagaccccttctcagtaaaatctttttctggtctctcttctacctccttctgctgccgctccagctccttcatgcggatctcgcgagcctccgcgcgggccgcccgttttgcagcgagccgggcttccgcctcccgcgcgatctggttgagcgcgtcgtcctccgccgtgagccgctcccggttggggagccgcttgcgccccgatccctgggtgcccatgtccatcgaccgcgtcgcccgcagctgccgcggggcccgttgctccagccgctcgcgccgccccg

SEQ ID NO: 12132 - RNA, 6272 nt, Homo sapiens
  source 1..6272: mol_type = other RNA
ctgcagactcgacctcccaggctcaggtgtttctgcctcctaagtagctgggactacatgggactacatgcacatgccaccatgcctggctaattgtttgtatattttttttgtagagatgggctttcatcatgttgcccaggctgggcttgaactcctgggcttaagtgatctgcctgcctcggcctcccacgtgctgggattataggcatgagccaatgtgcccggcctcaaccatttcttgataagttaagggccttcacagtaatatcaattactgtgcttggctataaagtcattacactggagagcatataactgatgctcagaatgaaggctctgaaatcatcgagaaatggtttggctgctcagaactctttctttttccttctttcttgctcatggattttcagctgtccattccctactggagggctgggtccaactgcttgttcactggcacagtgccttccatgtacaaagtgatcaaacctgtctattaattaagcaaatgagtggtgaatcactgagacggctggatggctgagctgagggatgtgatgtgtgcccaacgtcctgcagggtgctggtgaataacatgagaaagaacttaaaatggcttgatgatctcaccatttagtgaccttggttgtcacactgctttccaagagccctttaaaggtaggaatgagagctgtttccagtatgcattccaataggaatgcagctttgctaaagttagagacataaactaaaaccctgtgaagtcctatagagcccttggacttatttcctagcaagcatttatcatccccaccatcctctacttcaggacacttgagcagaaacagtcaaggtttttgccgttttcatcctgctcttcaaaacactgtaagtagtggcgcaggtaagcacagccacaggtgaagaccgttttcagctgaggctgcacatcagaaccacagatcacaggggatggtgcgtgacaatcgtctcagttctcccagtaatgcccatgctagccccaggctcgatgccaggagggaagtgcattccttactgagggagggcatcaggcgtgggtcttccacggaaccccaataggaatcagcaacccccaagcagatattactcaaaggtggtattacatacaacagtagtcagactcagacttcaagcagcccaaagagtggaaccacaggcttgcacaattataaaatgtttttatttcaattacataataacacgttttcctcaaattttattgaggttttggtctttttgcattcaattctatcttgtaacagtaatatgaatccacataatttcataaaatgtcaacaacattcataaggtacattcctttgtgattttatattttacaattttaaatctaactttacaattattttaaaaaatttttttatatagaaaacagatattttcttcaggcagatcaaaacaagaattttccagtaagaatatactgggacataacaaatgaaaatatttataccaaaataccaaaagtgattcagctctttaaaatatcctactatagtctaattagtagcttgtacaagaacaagtaaccattttttactgctcttttgaatgatgattagaaattcaaacaaagtattttaaggttcaaaaactttttttttttttttttttttttttagagacagtgtctcactctgtctcccaggctagagtacagtgtgcaatcatagctcactgcagccttgaactcctggcctcaagcaatcctcccaccttggcttcccaatgtgctaggtttacaggcgtgaaaacattgtgttgtgtgtgtgtgtgtttttttttttttttttagacagagtttcgctcttgttgtccaggctggagtacaatggcttgatcttggctcactgcaatctctgcctcgcaggttcaagcgattctcctgcctcagcctctggagtggctgggattacaggcgcccaccatcacgcccggccaattttttgtatttttagtagagacagggtttcaccatgttggccaggctggcctcgaactcttgacctcaggtgatccacctgccttggcctcccaatgtactgagattacaggcatgagccaccacgcccggccaaaaacatttaaaaaatgactgtccctgctcaaatactgcagtaggaaatgtaatttgacatatatcacttccagaaaaaaactttaaatctttctataaaatgaatttgatacatcatcagcatgaagtgaagttaaaatctcttacaaagtaaattcaggtatatcaacaatgagatccaaaagtatcggttcaagatcaaagactcatatgaggtaaaggcaaataaagcccctcatgctttcagacatttacttgttatccttaaaatgattattgttctaaggtgcaaatcttatcattcagtgacctatttgctatttggctgtttatctcctttaaataaaataccatacaggttataatgtacattttaaaatcaaatatgaaagtacacatatgtgaacaagacattaatttaaatatcaattatattcataatacagaagtctaagaatgctatttggtcatttcaattagatgctgatatatttggtcaagaaaacccacattcctatcagcctaaggcaaatagtaaatgcctctatttttattaagtggactataaacagtagacattattgtttgatactactggaatgctctcaattagaacgtacactgataacaaatatgtctttctaatctgggtgataacctcaatgattacatggaaatctacaagtaacagtctataacttaaagcagtagagcacctggtaattgtcatacagtgcctctctatgaatttagaacattctacttacattggcagtggagagaaaagaccccttcacactgagacttcctgtgcaccgcgcctgccgcctgcctcagcttaggacatggtacagtcttctttgcttttgcccttctcattccctcctctggtatcttctctgctttctggattgaagtgccctggctctcttcctggtgccgacaagtcatcgttctctaggctattgctgtctaaagctttcctgacggtctgacttggatgttctgacatctcacacctctctgtactttctgcttcacaggcatcactaatgtcctgtgagggactttcatgttcgggcagggtgcagcgatctgcgtcttcgctctttggttctgcaggactgctttgagtggcaccatctattttagcattatcttttgcaacaccttcatctaattcttcaccaccagccctcgggcctgatgattgaacggtgtcatcctcaaaatctaatgtgtctccatcagctagtacctcctcagctgctgtttgtacatcatcaccttcttggtcaagttttccatccaacttaattttaggattctccggacaatcaacattttcactgctttctgctgcaattttctgttttggattttcagtcacctcgttttgggcttccactgctgactttctgtcagtagactttacctgctcttcttccttaatttcacttaaatctgtgttctgatacgttaactcttttttaacatctttaagggtttctacgggtactggggattttttcttcttgtttttctttttcttgttctttgtcttcttctgcgatgagtccaatgcctctccctgttggtcactcttttcttcatcgggctctttcatatctaagggttcattttgagtgtctactgtacttggacctgtcgcttcctgacagttgccctcagttcctgctggagaaccaggaacttctgtcttgattggtttctcgtcccttaatcctgtttcttcaccctcttcttcgttgtgatccctacctacttctgtactgtgcgctggaacctccttgggctcagctgcttcctggttggtgaattctttctctaaactatgccctgtgcttgtctctaactcttgggggacctctaccatacatttgtcatcatgataaactgtgtcatcactatgccctaaaggacacgaggccactgtgcctgcctgctcttcaacctgagtcactgctgcctctcccacattctctgtgtggttcccaccatctaagtcactccaacagttggatggctcaaggggagttctggtcctgtcatctggtgcacccatgacctcatttgactcaacctgtactgtgttttcagggagagaactgctctcaagaatttggctttgaacctgttcctcataggtagcacctgctaaggttcctaggaatggggcagtgtcttcagaggatttctggtcctcggtattctcaccagcagggaatacctctatgtccacacagtccttcactgtgtcctctgtgtgttgttctttctcagtattgtgcaagatttctcttttccccacattcgccacgatttcatttttcacctccacttcactggctcttcctagggtcccatcccctgtcgacttgagggcatttaactcttcttttgtcatcttggtaggaccttggtatccaacattattgagggtgtcggaagtctctccattggtagctatttctgaatttaggattattccatgtttctttaattcctctttcagcatgactacttcttctctaagatcatcccgttcactccttacggaatcaaagaactctttctgcctctctaatgcccctatctttttgtctttccactctattgtttcctgaagatcagaaatctccctgatagaactcgcctgtttctgctgtagctgtcggatttcctcgagcatttcctctctttgcttcagggcctccttgacttcagcaaactgaaattgcagtatactgtgggcgtgtttttccctttcaaattctttgtttttctcttcgtactgccgcctagattcagccagctgttcttcaagctccagcaacatatcttttagggtatcaacctggtacatgaagtttgtcttttcattgtctagctgagcattggaaaccatagccttcttatatttctcttcaacttctgctagagagtccttcatctctttcaatccctgcatgtatttgccttctacatcctgaatctggtcctttaactcattgagttccttgatttccctgatggatgcctcggtgtcgatggagatggaggtgtctccgctgcctctccgagaggaagtcccacccagagaggccagcgtggctgcagacaggcccggcatgttacgagaccccttctcagtaaaatctttttctggtctctcttctaccacagggctggcccgggccgagctggccctggaggaggcgcgggagctggagttgaggtggccgctgtactccgagggagcacgggagccggaggtgctgccccgtcgggtcccaccgaagctgccttcatccaacacagacgcccggtaactccccgaaggccgggcagcgctgtacagacaggagggcaacttctcctccctggatgatgacaaagtagagaatctgctgtcaccgctgtagctggaattcctgccagatcttctattcagggactgtgatccatacaattctccatcataaccatttgtccaggcgtaaggacccccatactccaagtcaggctgcgacctcaggcttccacgactacccactgacatgcgctcgtcttcatcagaagccgatgtgtttcttctggatctacgagagtagcgctcactgtcttccatccactgctcgatgtcaccccattttgtatccagcccataatatttcttttggacctgatagatctccttctgctgccgctccagctccttcatgcggatctcgcgagcctccgcgcgggccgcccgttttgcagcgagccgggcttccgccagcttctgcgcttccgggctcaaacagtcgatctcccggctttgagcggccgcggggctggtcatcctgccgggctcggcccgctccacccggcgggaaatgctcggggaccgcgccgggagcccctcgcgggccgggccagggggcgcgcgctctgtccgcggagacggagccactcgccgctaagtgaacgctcgcgcttccggggccaggagccagcccgccggggagcggctcgcggcgctgggctcgggcgcggccgacaggggcggggcgcaggtggccgcgggctgagtcgggctcggggtggaagggcgccggggaagcgg

SEQ ID NO: 12133 - RNA, 6107 nt, Homo sapiens
  source 1..6107: mol_type = other RNA
ctgcagactcgacctcccaggctcaggtgtttctgcctcctaagtagctgggactacatgggactacatgcacatgccaccatgcctggctaattgtttgtatattttttttgtagagatgggctttcatcatgttgcccaggctgggcttgaactcctgggcttaagtgatctgcctgcctcggcctcccacgtgctgggattataggcatgagccaatgtgcccggcctcaaccatttcttgataagttaagggccttcacagtaatatcaattactgtgcttggctataaagtcattacactggagagcatataactgatgctcagaatgaaggctctgaaatcatcgagaaatggtttggctgctcagaactctttctttttccttctttcttgctcatggattttcagctgtccattccctactggagggctgggtccaactgcttgttcactggcacagtgccttccatgtacaaagtgatcaaacctgtctattaattaagcaaatgagtggtgaatcactgagacggctggatggctgagctgagggatgtgatgtgtgcccaacgtcctgcagggtgctggtgaataacatgagaaagaacttaaaatggcttgatgatctcaccatttagtgaccttggttgtcacactgctttccaagagccctttaaaggtaggaatgagagctgtttccagtatgcattccaataggaatgcagctttgctaaagttagagacataaactaaaaccctgtgaagtcctatagagcccttggacttatttcctagcaagcatttatcatccccaccatcctctacttcaggacacttgagcagaaacagtcaaggtttttgccgttttcatcctgctcttcaaaacactgtaagtagtggcgcaggtaagcacagccacaggtgaagaccgttttcagctgaggctgcacatcagaaccacagatcacaggggatggtgcgtgacaatcgtctcagttctcccagtaatgcccatgctagccccaggctcgatgccaggagggaagtgcattccttactgagggagggcatcaggcgtgggtcttccacggaaccccaataggaatcagcaacccccaagcagatattactcaaaggtggtattacatacaacagtagtcagactcagacttcaagcagcccaaagagtggaaccacaggcttgcacaattataaaatgtttttatttcaattacataataacacgttttcctcaaattttattgaggttttggtctttttgcattcaattctatcttgtaacagtaatatgaatccacataatttcataaaatgtcaacaacattcataaggtacattcctttgtgattttatattttacaattttaaatctaactttacaattattttaaaaaatttttttatatagaaaacagatattttcttcaggcagatcaaaacaagaattttccagtaagaatatactgggacataacaaatgaaaatatttataccaaaataccaaaagtgattcagctctttaaaatatcctactatagtctaattagtagcttgtacaagaacaagtaaccattttttactgctcttttgaatgatgattagaaattcaaacaaagtattttaaggttcaaaaactttttttttttttttttttttttttagagacagtgtctcactctgtctcccaggctagagtacagtgtgcaatcatagctcactgcagccttgaactcctggcctcaagcaatcctcccaccttggcttcccaatgtgctaggtttacaggcgtgaaaacattgtgttgtgtgtgtgtgtgtttttttttttttttttagacagagtttcgctcttgttgtccaggctggagtacaatggcttgatcttggctcactgcaatctctgcctcgcaggttcaagcgattctcctgcctcagcctctggagtggctgggattacaggcgcccaccatcacgcccggccaattttttgtatttttagtagagacagggtttcaccatgttggccaggctggcctcgaactcttgacctcaggtgatccacctgccttggcctcccaatgtactgagattacaggcatgagccaccacgcccggccaaaaacatttaaaaaatgactgtccctgctcaaatactgcagtaggaaatgtaatttgacatatatcacttccagaaaaaaactttaaatctttctataaaatgaatttgatacatcatcagcatgaagtgaagttaaaatctcttacaaagtaaattcaggtatatcaacaatgagatccaaaagtatcggttcaagatcaaagactcatatgaggtaaaggcaaataaagcccctcatgctttcagacatttacttgttatccttaaaatgattattgttctaaggtgcaaatcttatcattcagtgacctatttgctatttggctgtttatctcctttaaataaaataccatacaggttataatgtacattttaaaatcaaatatgaaagtacacatatgtgaacaagacattaatttaaatatcaattatattcataatacagaagtctaagaatgctatttggtcatttcaattagatgctgatatatttggtcaagaaaacccacattcctatcagcctaaggcaaatagtaaatgcctctatttttattaagtggactataaacagtagacattattgtttgatactactggaatgctctcaattagaacgtacactgataacaaatatgtctttctaatctgggtgataacctcaatgattacatggaaatctacaagtaacagtctataacttaaagcagtagagcacctggtaattgtcatacagtgcctctctatgaatttagaacattctacttacattggcagtggagagaaaagaccccttcacactgagacttcctgtgcaccgcgcctgccgcctgcctcagcttaggacatggtacagtcttctttgcttttgcccttctcattccctcctctggtatcttctctgctttctggattgaagtgccctggctctcttcctggtgccgacaagtcatcgttctctaggctattgctgtctaaagctttcctgacggtctgacttggatgttctgacatctcacacctctctgtactttctgcttcacaggcatcactaatgtcctgtgagggactttcatgttcgggcagggtgcagcgatctgcgtcttcgctctttggttctgcaggactgctttgagtggcaccatctattttagcattatcttttgcaacaccttcatctaattcttcaccaccagccctcgggcctgatgattgaacggtgtcatcctcaaaatctaatgtgtctccatcagctagtacctcctcagctgctgtttgtacatcatcaccttcttggtcaagttttccatccaacttaattttaggattctccggacaatcaacattttcactgctttctgctgcaattttctgttttggattttcagtcacctcgttttgggcttccactgctgactttctgtcagtagactttacctgctcttcttccttaatttcacttaaatctgtgttctgatacgttaactcttttttaacatctttaagggtttctacgggtactggggattttttcttcttgtttttctttttcttgttctttgtcttcttctgcgatgagtccaatgcctctccctgttggtcactcttttcttcatcgggctctttcatatctaagggttcattttgagtgtctactgtacttggacctgtcgcttcctgacagttgccctcagttcctgctggagaaccaggaacttctgtcttgattggtttctcgtcccttaatcctgtttcttcaccctcttcttcgttgtgatccctacctacttctgtactgtgcgctggaacctccttgggctcagctgcttcctggttggtgaattctttctctaaactatgccctgtgcttgtctctaactcttgggggacctctaccatacatttgtcatcatgataaactgtgtcatcactatgccctaaaggacacgaggccactgtgcctgcctgctcttcaacctgagtcactgctgcctctcccacattctctgtgtggttcccaccatctaagtcactccaacagttggatggctcaaggggagttctggtcctgtcatctggtgcacccatgacctcatttgactcaacctgtactgtgttttcagggagagaactgctctcaagaatttggctttgaacctgttcctcataggtagcacctgctaaggttcctaggaatggggcagtgtcttcagaggatttctggtcctcggtattctcaccagcagggaatacctctatgtccacacagtccttcactgtgtcctctgtgtgttgttctttctcagtattgtgcaagatttctcttttccccacattcgccacgatttcatttttcacctccacttcactggctcttcctagggtcccatcccctgtcgacttgagggcatttaactcttcttttgtcatcttggtaggaccttggtatccaacattattgagggtgtcggaagtctctccattggtagctatttctgaatttaggattattccatgtttctttaattcctctttcagcatgactacttcttctctaagatcatcccgttcactccttacggaatcaaagaactctttctgcctctctaatgcccctatctttttgtctttccactctattgtttcctgaagatcagaaatctccctgatagaactcgcctgtttctgctgtagctgtcggatttcctcgagcatttcctctctttgcttcagggcctccttgacttcagcaaactgaaattgcagtatactgtgggcgtgtttttccctttcaaattctttgtttttctcttcgtactgccgcctagattcagccagctgttcttcaagctccagcaacatatcttttagggtatcaacctggtacatgaagtttgtcttttcattgtctagctgagcattggaaaccatagccttcttatatttctcttcaacttctgctagagagtccttcatctctttcaatccctgcatgtatttgccttctacatcctgaatctggtcctttaactcattgagttccttgatttccctgatggatgcctcggtgtcgatggagatggaggtgtctccgctgcctctccgagaggaagtcccacccagagaggccagcgtggctgcagacaggcccggcatgttacgagaccccttctcagtaaaatctttttctggtctctcttctaccacagggctggcccgggccgagctggccctggaggaggcgcgggagctggagttgaggtggccgctgtactccgagggagcacgggagccggaggtgctgccccgtcgggtcccaccgaagctgccttcatccaacacagacgcccggtaactccccgaaggccgggcagcgctgtacagacaggagggcaacttctcctccctggatgatgacaaagtagagaatctgctgtcaccgctgtagctggaattcctgccagatcttctattcagggactgtgatccatacaattctccatcataaccatttgtccaggcgtaaggacccccatactccaagtcaggctgcgacctcaggcttccacgactacccactgacatgcgctcgtcttcatcagaagccgatgtgtttcttctggatctacgagagtagcgctcactgtcttccatccactgctcgatgtcaccccattttgtatccagcccataatatttcttttggacctgatagatctccttctgctgccgctccagctccttcatgcggatctcgcgagcctccgcgcgggccgcccgttttgcagcgagccgggcttccgcctcccgcgcgatctggttgagcgcgtcgtcctccgccgtgagccgctcccggttggggagccgcttgcgccccgatccctgggtgcccatgtccatcgaccgcgtcgcccgcagctgccgcggggcccgttgctccagccgctcgcgccgccccggcccggcccc

SEQ ID NO: 12134 - RNA, 6352 nt, Homo sapiens
  source 1..6352: mol_type = other RNA
ctgcagactcgacctcccaggctcaggtgtttctgcctcctaagtagctgggactacatgggactacatgcacatgccaccatgcctggctaattgtttgtatattttttttgtagagatgggctttcatcatgttgcccaggctgggcttgaactcctgggcttaagtgatctgcctgcctcggcctcccacgtgctgggattataggcatgagccaatgtgcccggcctcaaccatttcttgataagttaagggccttcacagtaatatcaattactgtgcttggctataaagtcattacactggagagcatataactgatgctcagaatgaaggctctgaaatcatcgagaaatggtttggctgctcagaactctttctttttccttctttcttgctcatggattttcagctgtccattccctactggagggctgggtccaactgcttgttcactggcacagtgccttccatgtacaaagtgatcaaacctgtctattaattaagcaaatgagtggtgaatcactgagacggctggatggctgagctgagggatgtgatgtgtgcccaacgtcctgcagggtgctggtgaataacatgagaaagaacttaaaatggcttgatgatctcaccatttagtgaccttggttgtcacactgctttccaagagccctttaaaggtaggaatgagagctgtttccagtatgcattccaataggaatgcagctttgctaaagttagagacataaactaaaaccctgtgaagtcctatagagcccttggacttatttcctagcaagcatttatcatccccaccatcctctacttcaggacacttgagcagaaacagtcaaggtttttgccgttttcatcctgctcttcaaaacactgtaagtagtggcgcaggtaagcacagccacaggtgaagaccgttttcagctgaggctgcacatcagaaccacagatcacaggggatggtgcgtgacaatcgtctcagttctcccagtaatgcccatgctagccccaggctcgatgccaggagggaagtgcattccttactgagggagggcatcaggcgtgggtcttccacggaaccccaataggaatcagcaacccccaagcagatattactcaaaggtggtattacatacaacagtagtcagactcagacttcaagcagcccaaagagtggaaccacaggcttgcacaattataaaatgtttttatttcaattacataataacacgttttcctcaaattttattgaggttttggtctttttgcattcaattctatcttgtaacagtaatatgaatccacataatttcataaaatgtcaacaacattcataaggtacattcctttgtgattttatattttacaattttaaatctaactttacaattattttaaaaaatttttttatatagaaaacagatattttcttcaggcagatcaaaacaagaattttccagtaagaatatactgggacataacaaatgaaaatatttataccaaaataccaaaagtgattcagctctttaaaatatcctactatagtctaattagtagcttgtacaagaacaagtaaccattttttactgctcttttgaatgatgattagaaattcaaacaaagtattttaaggttcaaaaactttttttttttttttttttttttttagagacagtgtctcactctgtctcccaggctagagtacagtgtgcaatcatagctcactgcagccttgaactcctggcctcaagcaatcctcccaccttggcttcccaatgtgctaggtttacaggcgtgaaaacattgtgttgtgtgtgtgtgtgtttttttttttttttttagacagagtttcgctcttgttgtccaggctggagtacaatggcttgatcttggctcactgcaatctctgcctcgcaggttcaagcgattctcctgcctcagcctctggagtggctgggattacaggcgcccaccatcacgcccggccaattttttgtatttttagtagagacagggtttcaccatgttggccaggctggcctcgaactcttgacctcaggtgatccacctgccttggcctcccaatgtactgagattacaggcatgagccaccacgcccggccaaaaacatttaaaaaatgactgtccctgctcaaatactgcagtaggaaatgtaatttgacatatatcacttccagaaaaaaactttaaatctttctataaaatgaatttgatacatcatcagcatgaagtgaagttaaaatctcttacaaagtaaattcaggtatatcaacaatgagatccaaaagtatcggttcaagatcaaagactcatatgaggtaaaggcaaataaagcccctcatgctttcagacatttacttgttatccttaaaatgattattgttctaaggtgcaaatcttatcattcagtgacctatttgctatttggctgtttatctcctttaaataaaataccatacaggttataatgtacattttaaaatcaaatatgaaagtacacatatgtgaacaagacattaatttaaatatcaattatattcataatacagaagtctaagaatgctatttggtcatttcaattagatgctgatatatttggtcaagaaaacccacattcctatcagcctaaggcaaatagtaaatgcctctatttttattaagtggactataaacagtagacattattgtttgatactactggaatgctctcaattagaacgtacactgataacaaatatgtctttctaatctgggtgataacctcaatgattacatggaaatctacaagtaacagtctataacttaaagcagtagagcacctggtaattgtcatacagtgcctctctatgaatttagaacattctacttacattggcagtggagagaaaagaccccttcacactgagacttcctgtgcaccgcgcctgccgcctgcctcagcttaggacatggtacagtcttctttgcttttgcccttctcattccctcctctggtatcttctctgctttctggattgaagtgccctggctctcttcctggtgccgacaagtcatcgttctctaggctattgctgtctaaagctttcctgacggtctgacttggatgttctgacatctcacacctctctgtactttctgcttcacaggcatcactaatgtcctgtgagggactttcatgttcgggcagggtgcagcgatctgcgtcttcgctctttggttctgcaggactgctttgagtggcaccatctattttagcattatcttttgcaacaccttcatctaattcttcaccaccagccctcgggcctgatgattgaacggtgtcatcctcaaaatctaatgtgtctccatcagctagtacctcctcagctgctgtttgtacatcatcaccttcttggtcaagttttccatccaacttaattttaggattctccggacaatcaacattttcactgctttctgctgcaattttctgttttggattttcagtcacctcgttttgggcttccactgctgactttctgtcagtagactttacctgctcttcttccttaatttcacttaaatctgtgttctgatacgttaactcttttttaacatctttaagggtttctacgggtactggggattttttcttcttgtttttctttttcttgttctttgtcttcttctgcgatgagtccaatgcctctccctgttggtcactcttttcttcatcgggctctttcatatctaagggttcattttgagtgtctactgtacttggacctgtcgcttcctgacagttgccctcagttcctgctggagaaccaggaacttctgtcttgattggtttctcgtcccttaatcctgtttcttcaccctcttcttcgttgtgatccctacctacttctgtactgtgcgctggaacctccttgggctcagctgcttcctggttggtgaattctttctctaaactatgccctgtgcttgtctctaactcttgggggacctctaccatacatttgtcatcatgataaactgtgtcatcactatgccctaaaggacacgaggccactgtgcctgcctgctcttcaacctgagtcactgctgcctctcccacattctctgtgtggttcccaccatctaagtcactccaacagttggatggctcaaggggagttctggtcctgtcatctggtgcacccatgacctcatttgactcaacctgtactgtgttttcagggagagaactgctctcaagaatttggctttgaacctgttcctcataggtagcacctgctaaggttcctaggaatggggcagtgtcttcagaggatttctggtcctcggtattctcaccagcagggaatacctctatgtccacacagtccttcactgtgtcctctgtgtgttgttctttctcagtattgtgcaagatttctcttttccccacattcgccacgatttcatttttcacctccacttcactggctcttcctagggtcccatcccctgtcgacttgagggcatttaactcttcttttgtcatcttggtaggaccttggtatccaacattattgagggtgtcggaagtctctccattggtagctatttctgaatttaggattattccatgtttctttaattcctctttcagcatgactacttcttctctaagatcatcccgttcactccttacggaatcaaagaactctttctgcctctctaatgcccctatctttttgtctttccactctattgtttcctgaagatcagaaatctccctgatagaactcgcctgtttctgctgtagctgtcggatttcctcgagcatttcctctctttgcttcagggcctccttgacttcagcaaactgaaattgcagtatactgtgggcgtgtttttccctttcaaattctttgtttttctcttcgtactgccgcctagattcagccagctgttcttcaagctccagcaacatatcttttagggtatcaacctggtacatgaagtttgtcttttcattgtctagctgagcattggaaaccatagccttcttatatttctcttcaacttctgctagagagtccttcatctctttcaatccctgcatgtatttgccttctacatcctgaatctggtcctttaactcattgagttccttgatttccctgatggatgcctcggtgtcgatggagatggaggtgtctccgctgcctctccgagaggaagtcccacccagagaggccagcgtggctgcagacaggcccggcatgttacgagaccccttctcagtaaaatctttttctggtctctcttctaccacagggctggcccgggccgagctggccctggaggaggcgcgggagctggagttgaggtggccgctgtactccgagggagcacgggagccggaggtgctgccccgtcgggtcccaccgaagctgccttcatccaacacagacgcccggtaactccccgaaggccgggcagcgctgtacagacaggagggcaacttctcctccctggatgatgacaaagtagagaatctgctgtcaccgctgtagctggaattcctgccagatcttctattcagggactgtgatccatacaattctccatcataaccatttgtccaggcgtaaggacccccatactccaagtcaggctgcgacctcaggcttccacgactacccactgacatgcgctcgtcttcatcagaagccgatgtgtttcttctggatctacgagagtagcgctcactgtcttccatccactgctcgatgtcaccccattttgtatccagcccataatatttcttttggacctgatagatctccttctgctgccgctccagctccttcatgcggatctcgcgagcctccgcgcgggccgcccgttttgcagcgagccgggcttccgcctttgaagaatgaagatcttagatgaacttcagggggagtgtgaggaacgccagagagcagccatttggagagacatgcttggcacgagagtggaaattctggaataactggagatcaaatagccactcctgaccacgtcacctttataccctgtacctcactgggcagctgccttggcatgatgagagggcgtggtcccctaaacgcactggaggctttccaaatgcttctctgacctgaccgtcggcttgattttagttgctgagattccactgaagccctcgccccttgtctccaccccgttggtggcatctgtatcaaatgtgctgtcgggctttttgggaaaccctaggattgataaagagcagggtcccctgacgtttggggttgcacagttccttgtcgtggg

SEQ ID NO: 12135 - RNA, 6020 nt, Homo sapiens
  source 1..6020: mol_type = other RNA
ctgcagactcgacctcccaggctcaggtgtttctgcctcctaagtagctgggactacatgggactacatgcacatgccaccatgcctggctaattgtttgtatattttttttgtagagatgggctttcatcatgttgcccaggctgggcttgaactcctgggcttaagtgatctgcctgcctcggcctcccacgtgctgggattataggcatgagccaatgtgcccggcctcaaccatttcttgataagttaagggccttcacagtaatatcaattactgtgcttggctataaagtcattacactggagagcatataactgatgctcagaatgaaggctctgaaatcatcgagaaatggtttggctgctcagaactctttctttttccttctttcttgctcatggattttcagctgtccattccctactggagggctgggtccaactgcttgttcactggcacagtgccttccatgtacaaagtgatcaaacctgtctattaattaagcaaatgagtggtgaatcactgagacggctggatggctgagctgagggatgtgatgtgtgcccaacgtcctgcagggtgctggtgaataacatgagaaagaacttaaaatggcttgatgatctcaccatttagtgaccttggttgtcacactgctttccaagagccctttaaaggtaggaatgagagctgtttccagtatgcattccaataggaatgcagctttgctaaagttagagacataaactaaaaccctgtgaagtcctatagagcccttggacttatttcctagcaagcatttatcatccccaccatcctctacttcaggacacttgagcagaaacagtcaaggtttttgccgttttcatcctgctcttcaaaacactgtaagtagtggcgcaggtaagcacagccacaggtgaagaccgttttcagctgaggctgcacatcagaaccacagatcacaggggatggtgcgtgacaatcgtctcagttctcccagtaatgcccatgctagccccaggctcgatgccaggagggaagtgcattccttactgagggagggcatcaggcgtgggtcttccacggaaccccaataggaatcagcaacccccaagcagatattactcaaaggtggtattacatacaacagtagtcagactcagacttcaagcagcccaaagagtggaaccacaggcttgcacaattataaaatgtttttatttcaattacataataacacgttttcctcaaattttattgaggttttggtctttttgcattcaattctatcttgtaacagtaatatgaatccacataatttcataaaatgtcaacaacattcataaggtacattcctttgtgattttatattttacaattttaaatctaactttacaattattttaaaaaatttttttatatagaaaacagatattttcttcaggcagatcaaaacaagaattttccagtaagaatatactgggacataacaaatgaaaatatttataccaaaataccaaaagtgattcagctctttaaaatatcctactatagtctaattagtagcttgtacaagaacaagtaaccattttttactgctcttttgaatgatgattagaaattcaaacaaagtattttaaggttcaaaaactttttttttttttttttttttttttagagacagtgtctcactctgtctcccaggctagagtacagtgtgcaatcatagctcactgcagccttgaactcctggcctcaagcaatcctcccaccttggcttcccaatgtgctaggtttacaggcgtgaaaacattgtgttgtgtgtgtgtgtgtttttttttttttttttagacagagtttcgctcttgttgtccaggctggagtacaatggcttgatcttggctcactgcaatctctgcctcgcaggttcaagcgattctcctgcctcagcctctggagtggctgggattacaggcgcccaccatcacgcccggccaattttttgtatttttagtagagacagggtttcaccatgttggccaggctggcctcgaactcttgacctcaggtgatccacctgccttggcctcccaatgtactgagattacaggcatgagccaccacgcccggccaaaaacatttaaaaaatgactgtccctgctcaaatactgcagtaggaaatgtaatttgacatatatcacttccagaaaaaaactttaaatctttctataaaatgaatttgatacatcatcagcatgaagtgaagttaaaatctcttacaaagtaaattcaggtatatcaacaatgagatccaaaagtatcggttcaagatcaaagactcatatgaggtaaaggcaaataaagcccctcatgctttcagacatttacttgttatccttaaaatgattattgttctaaggtgcaaatcttatcattcagtgacctatttgctatttggctgtttatctcctttaaataaaataccatacaggttataatgtacattttaaaatcaaatatgaaagtacacatatgtgaacaagacattaatttaaatatcaattatattcataatacagaagtctaagaatgctatttggtcatttcaattagatgctgatatatttggtcaagaaaacccacattcctatcagcctaaggcaaatagtaaatgcctctatttttattaagtggactataaacagtagacattattgtttgatactactggaatgctctcaattagaacgtacactgataacaaatatgtctttctaatctgggtgataacctcaatgattacatggaaatctacaagtaacagtctataacttaaagcagtagagcacctggtaattgtcatacagtgcctctctatgaatttagaacattctacttacattggcagtggagagaaaagaccccttcacactgagacttcctgtgcaccgcgcctgccgcctgcctcagcttaggacatggtacagtcttctttgcttttgcccttctcattccctcctctggtatcttctctgctttctggattgaagtgccctggctctcttcctggtgccgacaagtcatcgttctctaggctattgctgtctaaagctttcctgacggtctgacttggatgttctgacatctcacacctctctgtactttctgcttcacaggcatcactaatgtcctgtgagggactttcatgttcgggcagggtgcagcgatctgcgtcttcgctctttggttctgcaggactgctttgagtggcaccatctattttagcattatcttttgcaacaccttcatctaattcttcaccaccagccctcgggcctgatgattgaacggtgtcatcctcaaaatctaatgtgtctccatcagctagtacctcctcagctgctgtttgtacatcatcaccttcttggtcaagttttccatccaacttaattttaggattctccggacaatcaacattttcactgctttctgctgcaattttctgttttggattttcagtcacctcgttttgggcttccactgctgactttctgtcagtagactttacctgctcttcttccttaatttcacttaaatctgtgttctgatacgttaactcttttttaacatctttaagggtttctacgggtactggggattttttcttcttgtttttctttttcttgttctttgtcttcttctgcgatgagtccaatgcctctccctgttggtcactcttttcttcatcgggctctttcatatctaagggttcattttgagtgtctactgtacttggacctgtcgcttcctgacagttgccctcagttcctgctggagaaccaggaacttctgtcttgattggtttctcgtcccttaatcctgtttcttcaccctcttcttcgttgtgatccctacctacttctgtactgtgcgctggaacctccttgggctcagctgcttcctggttggtgaattctttctctaaactatgccctgtgcttgtctctaactcttgggggacctctaccatacatttgtcatcatgataaactgtgtcatcactatgccctaaaggacacgaggccactgtgcctgcctgctcttcaacctgagtcactgctgcctctcccacattctctgtgtggttcccaccatctaagtcactccaacagttggatggctcaaggggagttctggtcctgtcatctggtgcacccatgacctcatttgactcaacctgtactgtgttttcagggagagaactgctctcaagaatttggctttgaacctgttcctcataggtagcacctgctaaggttcctaggaatggggcagtgtcttcagaggatttctggtcctcggtattctcaccagcagggaatacctctatgtccacacagtccttcactgtgtcctctgtgtgttgttctttctcagtattgtgcaagatttctcttttccccacattcgccacgatttcatttttcacctccacttcactggctcttcctagggtcccatcccctgtcgacttgagggcatttaactcttcttttgtcatcttggtaggaccttggtatccaacattattgagggtgtcggaagtctctccattggtagctatttctgaatttaggattattccatgtttctttaattcctctttcagcatgactacttcttctctaagatcatcccgttcactccttacggaatcaaagaactctttctgcctctctaatgcccctatctttttgtctttccactctattgtttcctgaagatcagaaatctccctgatagaactcgcctgtttctgctgtagctgtcggatttcctcgagcatttcctctctttgcttcagggcctccttgacttcagcaaactgaaattgcagtatactgtgggcgtgtttttccctttcaaattctttgtttttctcttcgtactgccgcctagattcagccagctgttcttcaagctccagcaacatatcttttagggtatcaacctggtacatgaagtttgtcttttcattgtctagctgagcattggaaaccatagccttcttatatttctcttcaacttctgctagagagtccttcatctctttcaatccctgcatgtatttgccttctacatcctgaatctggtcctttaactcattgagttccttgatttccctgatggatgcctcggtgtcgatggagatggaggtgtctccgctgcctctccgagaggaagtcccacccagagaggccagcgtggctgcagacaggcccggcatgttacgagaccccttctcagtaaaatctttttctggtctctcttctaccacagggctggcccgggccgagctggccctggaggaggcgcgggagctggagttgaggtggccgctgtactccgagggagcacgggagccggaggtgctgccccgtcgggtcccaccgaagctgccttcatccaacacagacgcccggtaactccccgaaggccgggcagcgctgtacagacaggagggcaacttctcctccctggatgatgacaaagtagagaatctgctgtcaccgctgtagctggaattcctgccagatcttctattcagggactgtgatccatacaattctccatcataaccatttgtccaggcgtaaggacccccatactccaagtcaggctgcgacctcaggcttccacgactacccactgacatgcgctcgtcttcatcagaagccgatgtgtttcttctggatctacgagagtagcgctcactgtcttcctccttctgctgccgctccagctccttcatgcggatctcgcgagcctccgcgcgggccgcccgttttgcagcgagccgggcttccgcctcccgcgcgatctggttgagcgcgtcgtcctccgccgtgagccgctcccggttggggagccgcttgcgccccgatccctgggtgcccatgtccatcgaccgcgtcgcccgcagctgccgcggggcccgttgctccagccgctc

SEQ ID NO: 12136 - RNA, 6068 nt, Homo sapiens
  source 1..6068: mol_type = other RNA
ctgcagactcgacctcccaggctcaggtgtttctgcctcctaagtagctgggactacatgggactacatgcacatgccaccatgcctggctaattgtttgtatattttttttgtagagatgggctttcatcatgttgcccaggctgggcttgaactcctgggcttaagtgatctgcctgcctcggcctcccacgtgctgggattataggcatgagccaatgtgcccggcctcaaccatttcttgataagttaagggccttcacagtaatatcaattactgtgcttggctataaagtcattacactggagagcatataactgatgctcagaatgaaggctctgaaatcatcgagaaatggtttggctgctcagaactctttctttttccttctttcttgctcatggattttcagctgtccattccctactggagggctgggtccaactgcttgttcactggcacagtgccttccatgtacaaagtgatcaaacctgtctattaattaagcaaatgagtggtgaatcactgagacggctggatggctgagctgagggatgtgatgtgtgcccaacgtcctgcagggtgctggtgaataacatgagaaagaacttaaaatggcttgatgatctcaccatttagtgaccttggttgtcacactgctttccaagagccctttaaaggtaggaatgagagctgtttccagtatgcattccaataggaatgcagctttgctaaagttagagacataaactaaaaccctgtgaagtcctatagagcccttggacttatttcctagcaagcatttatcatccccaccatcctctacttcaggacacttgagcagaaacagtcaaggtttttgccgttttcatcctgctcttcaaaacactgtaagtagtggcgcaggtaagcacagccacaggtgaagaccgttttcagctgaggctgcacatcagaaccacagatcacaggggatggtgcgtgacaatcgtctcagttctcccagtaatgcccatgctagccccaggctcgatgccaggagggaagtgcattccttactgagggagggcatcaggcgtgggtcttccacggaaccccaataggaatcagcaacccccaagcagatattactcaaaggtggtattacatacaacagtagtcagactcagacttcaagcagcccaaagagtggaaccacaggcttgcacaattataaaatgtttttatttcaattacataataacacgttttcctcaaattttattgaggttttggtctttttgcattcaattctatcttgtaacagtaatatgaatccacataatttcataaaatgtcaacaacattcataaggtacattcctttgtgattttatattttacaattttaaatctaactttacaattattttaaaaaatttttttatatagaaaacagatattttcttcaggcagatcaaaacaagaattttccagtaagaatatactgggacataacaaatgaaaatatttataccaaaataccaaaagtgattcagctctttaaaatatcctactatagtctaattagtagcttgtacaagaacaagtaaccattttttactgctcttttgaatgatgattagaaattcaaacaaagtattttaaggttcaaaaactttttttttttttttttttttttttagagacagtgtctcactctgtctcccaggctagagtacagtgtgcaatcatagctcactgcagccttgaactcctggcctcaagcaatcctcccaccttggcttcccaatgtgctaggtttacaggcgtgaaaacattgtgttgtgtgtgtgtgtgtttttttttttttttttagacagagtttcgctcttgttgtccaggctggagtacaatggcttgatcttggctcactgcaatctctgcctcgcaggttcaagcgattctcctgcctcagcctctggagtggctgggattacaggcgcccaccatcacgcccggccaattttttgtatttttagtagagacagggtttcaccatgttggccaggctggcctcgaactcttgacctcaggtgatccacctgccttggcctcccaatgtactgagattacaggcatgagccaccacgcccggccaaaaacatttaaaaaatgactgtccctgctcaaatactgcagtaggaaatgtaatttgacatatatcacttccagaaaaaaactttaaatctttctataaaatgaatttgatacatcatcagcatgaagtgaagttaaaatctcttacaaagtaaattcaggtatatcaacaatgagatccaaaagtatcggttcaagatcaaagactcatatgaggtaaaggcaaataaagcccctcatgctttcagacatttacttgttatccttaaaatgattattgttctaaggtgcaaatcttatcattcagtgacctatttgctatttggctgtttatctcctttaaataaaataccatacaggttataatgtacattttaaaatcaaatatgaaagtacacatatgtgaacaagacattaatttaaatatcaattatattcataatacagaagtctaagaatgctatttggtcatttcaattagatgctgatatatttggtcaagaaaacccacattcctatcagcctaaggcaaatagtaaatgcctctatttttattaagtggactataaacagtagacattattgtttgatactactggaatgctctcaattagaacgtacactgataacaaatatgtctttctaatctgggtgataacctcaatgattacatggaaatctacaagtaacagtctataacttaaagcagtagagcacctggtaattgtcatacagtgcctctctatgaatttagaacattctacttacattggcagtggagagaaaagaccccttcacactgagacttcctgtgcaccgcgcctgccgcctgcctcagcttaggacatggtacagtcttctttgcttttgcccttctcattccctcctctggtatcttctctgctttctggattgaagtgccctggctctcttcctggtgccgacaagtcatcgttctctaggctattgctgtctaaagctttcctgacggtctgacttggatgttctgacatctcacacctctctgtactttctgcttcacaggcatcactaatgtcctgtgagggactttcatgttcgggcagggtgcagcgatctgcgtcttcgctctttggttctgcaggactgctttgagtggcaccatctattttagcattatcttttgcaacaccttcatctaattcttcaccaccagccctcgggcctgatgattgaacggtgtcatcctcaaaatctaatgtgtctccatcagctagtacctcctcagctgctgtttgtacatcatcaccttcttggtcaagttttccatccaacttaattttaggattctccggacaatcaacattttcactgctttctgctgcaattttctgttttggattttcagtcacctcgttttgggcttccactgctgactttctgtcagtagactttacctgctcttcttccttaatttcacttaaatctgtgttctgatacgttaactcttttttaacatctttaagggtttctacgggtactggggattttttcttcttgtttttctttttcttgttctttgtcttcttctgcgatgagtccaatgcctctccctgttggtcactcttttcttcatcgggctctttcatatctaagggttcattttgagtgtctactgtacttggacctgtcgcttcctgacagttgccctcagttcctgctggagaaccaggaacttctgtcttgattggtttctcgtcccttaatcctgtttcttcaccctcttcttcgttgtgatccctacctacttctgtactgtgcgctggaacctccttgggctcagctgcttcctggttggtgaattctttctctaaactatgccctgtgcttgtctctaactcttgggggacctctaccatacatttgtcatcatgataaactgtgtcatcactatgccctaaaggacacgaggccactgtgcctgcctgctcttcaacctgagtcactgctgcctctcccacattctctgtgtggttcccaccatctaagtcactccaacagttggatggctcaaggggagttctggtcctgtcatctggtgcacccatgacctcatttgactcaacctgtactgtgttttcagggagagaactgctctcaagaatttggctttgaacctgttcctcataggtagcacctgctaaggttcctaggaatggggcagtgtcttcagaggatttctggtcctcggtattctcaccagcagggaatacctctatgtccacacagtccttcactgtgtcctctgtgtgttgttctttctcagtattgtgcaagatttctcttttccccacattcgccacgatttcatttttcacctccacttcactggctcttcctagggtcccatcccctgtcgacttgagggcatttaactcttcttttgtcatcttggtaggaccttggtatccaacattattgagggtgtcggaagtctctccattggtagctatttctgaatttaggattattccatgtttctttaattcctctttcagcatgactacttcttctctaagatcatcccgttcactccttacggaatcaaagaactctttctgcctctctaatgcccctatctttttgtctttccactctattgtttcctgaagatcagaaatctccctgatagaactcgcctgtttctgctgtagctgtcggatttcctcgagcatttcctctctttgcttcagggcctccttgacttcagcaaactgaaattgcagtatactgtgggcgtgtttttccctttcaaattctttgtttttctcttcgtactgccgcctagattcagccagctgttcttcaagctccagcaacatatcttttagggtatcaacctggtacatgaagtttgtcttttcattgtctagctgagcattggaaaccatagccttcttatatttctcttcaacttctgctagagagtccttcatctctttcaatccctgcatgtatttgccttctacatcctgaatctggtcctttaactcattgagttccttgatttccctgatggatgcctcggtgtcgatggagatggaggtgtctccgctgcctctccgagaggaagtcccacccagagaggccagcgtggctgcagacaggcccggcatgttacgagaccccttctcagtaaaatctttttctggtctctcttctaccacagggctggcccgggccgagctggccctggaggaggcgcgggagctggagttgaggtggccgctgtactccgagggagcacgggagccggaggtgctgccccgtcgggtcccaccgaagctgccttcatccaacacagacgcccggtaactccccgaaggccgggcagcgctgtacagacaggagggcaacttctcctccctggatgatgacaaagtagagaatctgctgtcaccgctgtagctggaattcctgccagatcttctattcagggactgtgatccatacaattctccatcataaccatttgtcctcaggcttccacgactacccactgacatgcgctcgtcttcatcagaagccgatgtgtttcttctggatctacgagagtagcgctcactgtcttccatccactgctcgatgtcaccccattttgtatccagcccataatatttcttttggacctgatagatctccttctgctgccgctccagctccttcatgcggatctcgcgagcctccgcgcgggccgcccgttttgcagcgagccgggcttccgcctcccgcgcgatctggttgagcgcgtcgtcctccgccgtgagccgctcccggttggggagccgcttgcgccccgatccctgggtgcccatgtccatcgaccgcgtcgcccgcagctgccgcggggcccgttgctccagccgctcgcgccgccccggcccggcccc

SEQ ID NO: 12137 - RNA, 6110 nt, Homo sapiens
  source 1..6110: mol_type = other RNA
ctgcagactcgacctcccaggctcaggtgtttctgcctcctaagtagctgggactacatgggactacatgcacatgccaccatgcctggctaattgtttgtatattttttttgtagagatgggctttcatcatgttgcccaggctgggcttgaactcctgggcttaagtgatctgcctgcctcggcctcccacgtgctgggattataggcatgagccaatgtgcccggcctcaaccatttcttgataagttaagggccttcacagtaatatcaattactgtgcttggctataaagtcattacactggagagcatataactgatgctcagaatgaaggctctgaaatcatcgagaaatggtttggctgctcagaactctttctttttccttctttcttgctcatggattttcagctgtccattccctactggagggctgggtccaactgcttgttcactggcacagtgccttccatgtacaaagtgatcaaacctgtctattaattaagcaaatgagtggtgaatcactgagacggctggatggctgagctgagggatgtgatgtgtgcccaacgtcctgcagggtgctggtgaataacatgagaaagaacttaaaatggcttgatgatctcaccatttagtgaccttggttgtcacactgctttccaagagccctttaaaggtaggaatgagagctgtttccagtatgcattccaataggaatgcagctttgctaaagttagagacataaactaaaaccctgtgaagtcctatagagcccttggacttatttcctagcaagcatttatcatccccaccatcctctacttcaggacacttgagcagaaacagtcaaggtttttgccgttttcatcctgctcttcaaaacactgtaagtagtggcgcaggtaagcacagccacaggtgaagaccgttttcagctgaggctgcacatcagaaccacagatcacaggggatggtgcgtgacaatcgtctcagttctcccagtaatgcccatgctagccccaggctcgatgccaggagggaagtgcattccttactgagggagggcatcaggcgtgggtcttccacggaaccccaataggaatcagcaacccccaagcagatattactcaaaggtggtattacatacaacagtagtcagactcagacttcaagcagcccaaagagtggaaccacaggcttgcacaattataaaatgtttttatttcaattacataataacacgttttcctcaaattttattgaggttttggtctttttgcattcaattctatcttgtaacagtaatatgaatccacataatttcataaaatgtcaacaacattcataaggtacattcctttgtgattttatattttacaattttaaatctaactttacaattattttaaaaaatttttttatatagaaaacagatattttcttcaggcagatcaaaacaagaattttccagtaagaatatactgggacataacaaatgaaaatatttataccaaaataccaaaagtgattcagctctttaaaatatcctactatagtctaattagtagcttgtacaagaacaagtaaccattttttactgctcttttgaatgatgattagaaattcaaacaaagtattttaaggttcaaaaactttttttttttttttttttttttttagagacagtgtctcactctgtctcccaggctagagtacagtgtgcaatcatagctcactgcagccttgaactcctggcctcaagcaatcctcccaccttggcttcccaatgtgctaggtttacaggcgtgaaaacattgtgttgtgtgtgtgtgtgtttttttttttttttttagacagagtttcgctcttgttgtccaggctggagtacaatggcttgatcttggctcactgcaatctctgcctcgcaggttcaagcgattctcctgcctcagcctctggagtggctgggattacaggcgcccaccatcacgcccggccaattttttgtatttttagtagagacagggtttcaccatgttggccaggctggcctcgaactcttgacctcaggtgatccacctgccttggcctcccaatgtactgagattacaggcatgagccaccacgcccggccaaaaacatttaaaaaatgactgtccctgctcaaatactgcagtaggaaatgtaatttgacatatatcacttccagaaaaaaactttaaatctttctataaaatgaatttgatacatcatcagcatgaagtgaagttaaaatctcttacaaagtaaattcaggtatatcaacaatgagatccaaaagtatcggttcaagatcaaagactcatatgaggtaaaggcaaataaagcccctcatgctttcagacatttacttgttatccttaaaatgattattgttctaaggtgcaaatcttatcattcagtgacctatttgctatttggctgtttatctcctttaaataaaataccatacaggttataatgtacattttaaaatcaaatatgaaagtacacatatgtgaacaagacattaatttaaatatcaattatattcataatacagaagtctaagaatgctatttggtcatttcaattagatgctgatatatttggtcaagaaaacccacattcctatcagcctaaggcaaatagtaaatgcctctatttttattaagtggactataaacagtagacattattgtttgatactactggaatgctctcaattagaacgtacactgataacaaatatgtctttctaatctgggtgataacctcaatgattacatggaaatctacaagtaacagtctataacttaaagcagtagagcacctggtaattgtcatacagtgcctctctatgaatttagaacattctacttacattggcagtggagagaaaagaccccttcacactgagacttcctgtgcaccgcgcctgccgcctgcctcagcttaggacatggtacagtcttctttgcttttgcccttctcattccctcctctggtatcttctctgctttctggattgaagtgccctggctctcttcctggtgccgacaagtcatcgttctctaggctattgctgtctaaagctttcctgacggtctgacttggatgttctgacatctcacacctctctgtactttctgcttcacaggcatcactaatgtcctgtgagggactttcatgttcgggcagggtgcagcgatctgcgtcttcgctctttggttctgcaggactgctttgagtggcaccatctattttagcattatcttttgcaacaccttcatctaattcttcaccaccagccctcgggcctgatgattgaacggtgtcatcctcaaaatctaatgtgtctccatcagctagtacctcctcagctgctgtttgtacatcatcaccttcttggtcaagttttccatccaacttaattttaggattctccggacaatcaacattttcactgctttctgctgcaattttctgttttggattttcagtcacctcgttttgggcttccactgctgactttctgtcagtagactttacctgctcttcttccttaatttcacttaaatctgtgttctgatacgttaactcttttttaacatctttaagggtttctacgggtactggggattttttcttcttgtttttctttttcttgttctttgtcttcttctgcgatgagtccaatgcctctccctgttggtcactcttttcttcatcgggctctttcatatctaagggttcattttgagtgtctactgtacttggacctgtcgcttcctgacagttgccctcagttcctgctggagaaccaggaacttctgtcttgattggtttctcgtcccttaatcctgtttcttcaccctcttcttcgttgtgatccctacctacttctgtactgtgcgctggaacctccttgggctcagctgcttcctggttggtgaattctttctctaaactatgccctgtgcttgtctctaactcttgggggacctctaccatacatttgtcatcatgataaactgtgtcatcactatgccctaaaggacacgaggccactgtgcctgcctgctcttcaacctgagtcactgctgcctctcccacattctctgtgtggttcccaccatctaagtcactccaacagttggatggctcaaggggagttctggtcctgtcatctggtgcacccatgacctcatttgactcaacctgtactgtgttttcagggagagaactgctctcaagaatttggctttgaacctgttcctcataggtagcacctgctaaggttcctaggaatggggcagtgtcttcagaggatttctggtcctcggtattctcaccagcagggaatacctctatgtccacacagtccttcactgtgtcctctgtgtgttgttctttctcagtattgtgcaagatttctcttttccccacattcgccacgatttcatttttcacctccacttcactggctcttcctagggtcccatcccctgtcgacttgagggcatttaactcttcttttgtcatcttggtaggaccttggtatccaacattattgagggtgtcggaagtctctccattggtagctatttctgaatttaggattattccatgtttctttaattcctctttcagcatgactacttcttctctaagatcatcccgttcactccttacggaatcaaagaactctttctgcctctctaatgcccctatctttttgtctttccactctattgtttcctgaagatcagaaatctccctgatagaactcgcctgtttctgctgtagctgtcggatttcctcgagcatttcctctctttgcttcagggcctccttgacttcagcaaactgaaattgcagtatactgtgggcgtgtttttccctttcaaattctttgtttttctcttcgtactgccgcctagattcagccagctgttcttcaagctccagcaacatatcttttagggtatcaacctggtacatgaagtttgtcttttcattgtctagctgagcattggaaaccatagccttcttatatttctcttcaacttctgctagagagtccttcatctctttcaatccctgcatgtatttgccttctacatcctgaatctggtcctttaactcattgagttccttgatttccctgatggatgcctcggtgtcgatggagatggaggtgtctccgctgcctctccgagaggaagtcccacccagagaggccagcgtggctgcagacaggcccggcatgttacgagaccccttctcagtaaaatctttttctggtctctcttctaccacagggctggcccgggccgagctggccctggaggaggcgcgggagctggagttgaggtggccgctgtactccgagggagcacgggagccggaggtgctgccccgtcgggtcccaccgaagctgccttcatccaacacagacgcccggtaactccccgaaggccgggcagcgctgtacagacaggagggcctcaggcttccacgactacccactgacatgcgctcgtcttcatcagaagccgatgtgtttcttctggatctacgagagtagcgctcactgtcttccatccactgctcgatgtcaccccattttgtatccagcccataatatttcttttggacctgatagatctccttctgctgccgctccagctccttcatgcggatctcgcgagcctccgcgcgggccgcccgttttgcagcgagccgggcttccgccagcttctgcgcttccgggctcaaacagtcgatctcccggctttgagcggccgcggggctggtcatcctgccgggctcggcccgctccacccggcgggaaatgctcggggaccgcgccgggagcccctcgcgggccgggccagggggcgcgcgctctgtccgcggagacggagccactcgccgctaagtgaacgctcgcgcttccggggccaggagccagcccgccggggagcggctcgcggcgctgggctcgggcgcggccgacaggggcggggcgcaggtggccgcgggctgagtcgggctcggggtggaagggcgccggggaagcgg

SEQ ID NO: 12138 - RNA, 6044 nt, Homo sapiens
  source 1..6044: mol_type = other RNA
ctgcagactcgacctcccaggctcaggtgtttctgcctcctaagtagctgggactacatgggactacatgcacatgccaccatgcctggctaattgtttgtatattttttttgtagagatgggctttcatcatgttgcccaggctgggcttgaactcctgggcttaagtgatctgcctgcctcggcctcccacgtgctgggattataggcatgagccaatgtgcccggcctcaaccatttcttgataagttaagggccttcacagtaatatcaattactgtgcttggctataaagtcattacactggagagcatataactgatgctcagaatgaaggctctgaaatcatcgagaaatggtttggctgctcagaactctttctttttccttctttcttgctcatggattttcagctgtccattccctactggagggctgggtccaactgcttgttcactggcacagtgccttccatgtacaaagtgatcaaacctgtctattaattaagcaaatgagtggtgaatcactgagacggctggatggctgagctgagggatgtgatgtgtgcccaacgtcctgcagggtgctggtgaataacatgagaaagaacttaaaatggcttgatgatctcaccatttagtgaccttggttgtcacactgctttccaagagccctttaaaggtaggaatgagagctgtttccagtatgcattccaataggaatgcagctttgctaaagttagagacataaactaaaaccctgtgaagtcctatagagcccttggacttatttcctagcaagcatttatcatccccaccatcctctacttcaggacacttgagcagaaacagtcaaggtttttgccgttttcatcctgctcttcaaaacactgtaagtagtggcgcaggtaagcacagccacaggtgaagaccgttttcagctgaggctgcacatcagaaccacagatcacaggggatggtgcgtgacaatcgtctcagttctcccagtaatgcccatgctagccccaggctcgatgccaggagggaagtgcattccttactgagggagggcatcaggcgtgggtcttccacggaaccccaataggaatcagcaacccccaagcagatattactcaaaggtggtattacatacaacagtagtcagactcagacttcaagcagcccaaagagtggaaccacaggcttgcacaattataaaatgtttttatttcaattacataataacacgttttcctcaaattttattgaggttttggtctttttgcattcaattctatcttgtaacagtaatatgaatccacataatttcataaaatgtcaacaacattcataaggtacattcctttgtgattttatattttacaattttaaatctaactttacaattattttaaaaaatttttttatatagaaaacagatattttcttcaggcagatcaaaacaagaattttccagtaagaatatactgggacataacaaatgaaaatatttataccaaaataccaaaagtgattcagctctttaaaatatcctactatagtctaattagtagcttgtacaagaacaagtaaccattttttactgctcttttgaatgatgattagaaattcaaacaaagtattttaaggttcaaaaactttttttttttttttttttttttttagagacagtgtctcactctgtctcccaggctagagtacagtgtgcaatcatagctcactgcagccttgaactcctggcctcaagcaatcctcccaccttggcttcccaatgtgctaggtttacaggcgtgaaaacattgtgttgtgtgtgtgtgtgtttttttttttttttttagacagagtttcgctcttgttgtccaggctggagtacaatggcttgatcttggctcactgcaatctctgcctcgcaggttcaagcgattctcctgcctcagcctctggagtggctgggattacaggcgcccaccatcacgcccggccaattttttgtatttttagtagagacagggtttcaccatgttggccaggctggcctcgaactcttgacctcaggtgatccacctgccttggcctcccaatgtactgagattacaggcatgagccaccacgcccggccaaaaacatttaaaaaatgactgtccctgctcaaatactgcagtaggaaatgtaatttgacatatatcacttccagaaaaaaactttaaatctttctataaaatgaatttgatacatcatcagcatgaagtgaagttaaaatctcttacaaagtaaattcaggtatatcaacaatgagatccaaaagtatcggttcaagatcaaagactcatatgaggtaaaggcaaataaagcccctcatgctttcagacatttacttgttatccttaaaatgattattgttctaaggtgcaaatcttatcattcagtgacctatttgctatttggctgtttatctcctttaaataaaataccatacaggttataatgtacattttaaaatcaaatatgaaagtacacatatgtgaacaagacattaatttaaatatcaattatattcataatacagaagtctaagaatgctatttggtcatttcaattagatgctgatatatttggtcaagaaaacccacattcctatcagcctaaggcaaatagtaaatgcctctatttttattaagtggactataaacagtagacattattgtttgatactactggaatgctctcaattagaacgtacactgataacaaatatgtctttctaatctgggtgataacctcaatgattacatggaaatctacaagtaacagtctataacttaaagcagtagagcacctggtaattgtcatacagtgcctctctatgaatttagaacattctacttacattggcagtggagagaaaagaccccttcacactgagacttcctgtgcaccgcgcctgccgcctgcctcagcttaggacatggtacagtcttctttgcttttgcccttctcattccctcctctggtatcttctctgctttctggattgaagtgccctggctctcttcctggtgccgacaagtcatcgttctctaggctattgctgtctaaagctttcctgacggtctgacttggatgttctgacatctcacacctctctgtactttctgcttcacaggcatcactaatgtcctgtgagggactttcatgttcgggcagggtgcagcgatctgcgtcttcgctctttggttctgcaggactgctttgagtggcaccatctattttagcattatcttttgcaacaccttcatctaattcttcaccaccagccctcgggcctgatgattgaacggtgtcatcctcaaaatctaatgtgtctccatcagctagtacctcctcagctgctgtttgtacatcatcaccttcttggtcaagttttccatccaacttaattttaggattctccggacaatcaacattttcactgctttctgctgcaattttctgttttggattttcagtcacctcgttttgggcttccactgctgactttctgtcagtagactttacctgctcttcttccttaatttcacttaaatctgtgttctgatacgttaactcttttttaacatctttaagggtttctacgggtactggggattttttcttcttgtttttctttttcttgttctttgtcttcttctgcgatgagtccaatgcctctccctgttggtcactcttttcttcatcgggctctttcatatctaagggttcattttgagtgtctactgtacttggacctgtcgcttcctgacagttgccctcagttcctgctggagaaccaggaacttctgtcttgattggtttctcgtcccttaatcctgtttcttcaccctcttcttcgttgtgatccctacctacttctgtactgtgcgctggaacctccttgggctcagctgcttcctggttggtgaattctttctctaaactatgccctgtgcttgtctctaactcttgggggacctctaccatacatttgtcatcatgataaactgtgtcatcactatgccctaaaggacacgaggccactgtgcctgcctgctcttcaacctgagtcactgctgcctctcccacattctctgtgtggttcccaccatctaagtcactccaacagttggatggctcaaggggagttctggtcctgtcatctggtgcacccatgacctcatttgactcaacctgtactgtgttttcagggagagaactgctctcaagaatttggctttgaacctgttcctcataggtagcacctgctaaggttcctaggaatggggcagtgtcttcagaggatttctggtcctcggtattctcaccagcagggaatacctctatgtccacacagtccttcactgtgtcctctgtgtgttgttctttctcagtattgtgcaagatttctcttttccccacattcgccacgatttcatttttcacctccacttcactggctcttcctagggtcccatcccctgtcgacttgagggcatttaactcttcttttgtcatcttggtaggaccttggtatccaacattattgagggtgtcggaagtctctccattggtagctatttctgaatttaggattattccatgtttctttaattcctctttcagcatgactacttcttctctaagatcatcccgttcactccttacggaatcaaagaactctttctgcctctctaatgcccctatctttttgtctttccactctattgtttcctgaagatcagaaatctccctgatagaactcgcctgtttctgctgtagctgtcggatttcctcgagcatttcctctctttgcttcagggcctccttgacttcagcaaactgaaattgcagtatactgtgggcgtgtttttccctttcaaattctttgtttttctcttcgtactgccgcctagattcagccagctgttcttcaagctccagcaacatatcttttagggtatcaacctggtacatgaagtttgtcttttcattgtctagctgagcattggaaaccatagccttcttatatttctcttcaacttctgctagagagtccttcatctctttcaatccctgcatgtatttgccttctacatcctgaatctggtcctttaactcattgagttccttgatttccctgatggatgcctcggtgtcgatggagatggaggtgtctccgctgcctctccgagaggaagtcccacccagagaggccagcgtggctgcagacaggcccggcatgttacgagaccccttctcagtaaaatctttttctggtctctcttctaccacagggctggcccgggccgagctggccctggaggaggcgcgggagctggagttgaggtggccgctgtactccgagggagcacgggagccggaggtgctgccccgtcgggtcccaccgaagctgccttcatccaacacagacgcccggtaactccccgaaggccgggcagcgctgtacagacaggagggcctgccagatcttctattcagggactgtgatccatacaattctccatcataaccatttgtccaggcgtaaggacccccatactccaagtcaggctgcgacctcaggcttccacgactacccactgacatgcgctcgtcttcatcagaagccgatgtgtttcttctggatctacgagagtagcgctcactgtcttccatccactgctcgatgtcaccccattttgtatccagcccataatatttcttttggacctgatagatctccttctgctgccgctccagctccttcatgcggatctcgcgagcctccgcgcgggccgcccgttttgcagcgagccgggcttccgcctcccgcgcgatctggttgagcgcgtcgtcctccgccgtgagccgctcccggttggggagccgcttgcgccccgatccctgggtgcccatgtccatcgaccgcgtcgcccgcagctgccgcggggcccgttgctccagccgctcgcgccgccccggcccggcccc

SEQ ID NO: 12139 - RNA, 6005 nt, Homo sapiens
  source 1..6005: mol_type = other RNA
ctgcagactcgacctcccaggctcaggtgtttctgcctcctaagtagctgggactacatgggactacatgcacatgccaccatgcctggctaattgtttgtatattttttttgtagagatgggctttcatcatgttgcccaggctgggcttgaactcctgggcttaagtgatctgcctgcctcggcctcccacgtgctgggattataggcatgagccaatgtgcccggcctcaaccatttcttgataagttaagggccttcacagtaatatcaattactgtgcttggctataaagtcattacactggagagcatataactgatgctcagaatgaaggctctgaaatcatcgagaaatggtttggctgctcagaactctttctttttccttctttcttgctcatggattttcagctgtccattccctactggagggctgggtccaactgcttgttcactggcacagtgccttccatgtacaaagtgatcaaacctgtctattaattaagcaaatgagtggtgaatcactgagacggctggatggctgagctgagggatgtgatgtgtgcccaacgtcctgcagggtgctggtgaataacatgagaaagaacttaaaatggcttgatgatctcaccatttagtgaccttggttgtcacactgctttccaagagccctttaaaggtaggaatgagagctgtttccagtatgcattccaataggaatgcagctttgctaaagttagagacataaactaaaaccctgtgaagtcctatagagcccttggacttatttcctagcaagcatttatcatccccaccatcctctacttcaggacacttgagcagaaacagtcaaggtttttgccgttttcatcctgctcttcaaaacactgtaagtagtggcgcaggtaagcacagccacaggtgaagaccgttttcagctgaggctgcacatcagaaccacagatcacaggggatggtgcgtgacaatcgtctcagttctcccagtaatgcccatgctagccccaggctcgatgccaggagggaagtgcattccttactgagggagggcatcaggcgtgggtcttccacggaaccccaataggaatcagcaacccccaagcagatattactcaaaggtggtattacatacaacagtagtcagactcagacttcaagcagcccaaagagtggaaccacaggcttgcacaattataaaatgtttttatttcaattacataataacacgttttcctcaaattttattgaggttttggtctttttgcattcaattctatcttgtaacagtaatatgaatccacataatttcataaaatgtcaacaacattcataaggtacattcctttgtgattttatattttacaattttaaatctaactttacaattattttaaaaaatttttttatatagaaaacagatattttcttcaggcagatcaaaacaagaattttccagtaagaatatactgggacataacaaatgaaaatatttataccaaaataccaaaagtgattcagctctttaaaatatcctactatagtctaattagtagcttgtacaagaacaagtaaccattttttactgctcttttgaatgatgattagaaattcaaacaaagtattttaaggttcaaaaactttttttttttttttttttttttttagagacagtgtctcactctgtctcccaggctagagtacagtgtgcaatcatagctcactgcagccttgaactcctggcctcaagcaatcctcccaccttggcttcccaatgtgctaggtttacaggcgtgaaaacattgtgttgtgtgtgtgtgtgtttttttttttttttttagacagagtttcgctcttgttgtccaggctggagtacaatggcttgatcttggctcactgcaatctctgcctcgcaggttcaagcgattctcctgcctcagcctctggagtggctgggattacaggcgcccaccatcacgcccggccaattttttgtatttttagtagagacagggtttcaccatgttggccaggctggcctcgaactcttgacctcaggtgatccacctgccttggcctcccaatgtactgagattacaggcatgagccaccacgcccggccaaaaacatttaaaaaatgactgtccctgctcaaatactgcagtaggaaatgtaatttgacatatatcacttccagaaaaaaactttaaatctttctataaaatgaatttgatacatcatcagcatgaagtgaagttaaaatctcttacaaagtaaattcaggtatatcaacaatgagatccaaaagtatcggttcaagatcaaagactcatatgaggtaaaggcaaataaagcccctcatgctttcagacatttacttgttatccttaaaatgattattgttctaaggtgcaaatcttatcattcagtgacctatttgctatttggctgtttatctcctttaaataaaataccatacaggttataatgtacattttaaaatcaaatatgaaagtacacatatgtgaacaagacattaatttaaatatcaattatattcataatacagaagtctaagaatgctatttggtcatttcaattagatgctgatatatttggtcaagaaaacccacattcctatcagcctaaggcaaatagtaaatgcctctatttttattaagtggactataaacagtagacattattgtttgatactactggaatgctctcaattagaacgtacactgataacaaatatgtctttctaatctgggtgataacctcaatgattacatggaaatctacaagtaacagtctataacttaaagcagtagagcacctggtaattgtcatacagtgcctctctatgaatttagaacattctacttacattggcagtggagagaaaagaccccttcacactgagacttcctgtgcaccgcgcctgccgcctgcctcagcttaggacatggtacagtcttctttgcttttgcccttctcattccctcctctggtatcttctctgctttctggattgaagtgccctggctctcttcctggtgccgacaagtcatcgttctctaggctattgctgtctaaagctttcctgacggtctgacttggatgttctgacatctcacacctctctgtactttctgcttcacaggcatcactaatgtcctgtgagggactttcatgttcgggcagggtgcagcgatctgcgtcttcgctctttggttctgcaggactgctttgagtggcaccatctattttagcattatcttttgcaacaccttcatctaattcttcaccaccagccctcgggcctgatgattgaacggtgtcatcctcaaaatctaatgtgtctccatcagctagtacctcctcagctgctgtttgtacatcatcaccttcttggtcaagttttccatccaacttaattttaggattctccggacaatcaacattttcactgctttctgctgcaattttctgttttggattttcagtcacctcgttttgggcttccactgctgactttctgtcagtagactttacctgctcttcttccttaatttcacttaaatctgtgttctgatacgttaactcttttttaacatctttaagggtttctacgggtactggggattttttcttcttgtttttctttttcttgttctttgtcttcttctgcgatgagtccaatgcctctccctgttggtcactcttttcttcatcgggctctttcatatctaagggttcattttgagtgtctactgtacttggacctgtcgcttcctgacagttgccctcagttcctgctggagaaccaggaacttctgtcttgattggtttctcgtcccttaatcctgtttcttcaccctcttcttcgttgtgatccctacctacttctgtactgtgcgctggaacctccttgggctcagctgcttcctggttggtgaattctttctctaaactatgccctgtgcttgtctctaactcttgggggacctctaccatacatttgtcatcatgataaactgtgtcatcactatgccctaaaggacacgaggccactgtgcctgcctgctcttcaacctgagtcactgctgcctctcccacattctctgtgtggttcccaccatctaagtcactccaacagttggatggctcaaggggagttctggtcctgtcatctggtgcacccatgacctcatttgactcaacctgtactgtgttttcagggagagaactgctctcaagaatttggctttgaacctgttcctcataggtagcacctgctaaggttcctaggaatggggcagtgtcttcagaggatttctggtcctcggtattctcaccagcagggaatacctctatgtccacacagtccttcactgtgtcctctgtgtgttgttctttctcagtattgtgcaagatttctcttttccccacattcgccacgatttcatttttcacctccacttcactggctcttcctagggtcccatcccctgtcgacttgagggcatttaactcttcttttgtcatcttggtaggaccttggtatccaacattattgagggtgtcggaagtctctccattggtagctatttctgaatttaggattattccatgtttctttaattcctctttcagcatgactacttcttctctaagatcatcccgttcactccttacggaatcaaagaactctttctgcctctctaatgcccctatctttttgtctttccactctattgtttcctgaagatcagaaatctccctgatagaactcgcctgtttctgctgtagctgtcggatttcctcgagcatttcctctctttgcttcagggcctccttgacttcagcaaactgaaattgcagtatactgtgggcgtgtttttccctttcaaattctttgtttttctcttcgtactgccgcctagattcagccagctgttcttcaagctccagcaacatatcttttagggtatcaacctggtacatgaagtttgtcttttcattgtctagctgagcattggaaaccatagccttcttatatttctcttcaacttctgctagagagtccttcatctctttcaatccctgcatgtatttgccttctacatcctgaatctggtcctttaactcattgagttccttgatttccctgatggatgcctcggtgtcgatggagatggaggtgtctccgctgcctctccgagaggaagtcccacccagagaggccagcgtggctgcagacaggcccggcatgttacgagaccccttctcagtaaaatctttttctggtctctcttctaccacagggctggcccgggccgagctggccctggaggaggcgcgggagctggagttgaggtggccgctgtactccgagggagcacgggagccggaggtgctgccccgtcgggtcccaccgaagctgccttcatccaacacagacgcccggtaactccccgaaggccgggcagcgctgtacagacaggagggcctgccagatcttctattcagggactgtgatccatacaattctccatcataaccatttgtcctcaggcttccacgactacccactgacatgcgctcgtcttcatcagaagccgatgtgtttcttctggatctacgagagtagcgctcactgtcttccatccactgctcgatgtcaccccattttgtatccagcccataatatttcttttggacctgatagatctccttctgctgccgctccagctccttcatgcggatctcgcgagcctccgcgcgggccgcccgttttgcagcgagccgggcttccgcctcccgcgcgatctggttgagcgcgtcgtcctccgccgtgagccgctcccggttggggagccgcttgcgccccgatccctgggtgcccatgtccatcgaccgcgtcgcccgcagctgccgcggggcccgttgctccagccgctcgcgccgccccggcccggcccc

SEQ ID NO: 12140 - RNA, 5702 nt, Homo sapiens
  source 1..5702: mol_type = other RNA
ctgcagactcgacctcccaggctcaggtgtttctgcctcctaagtagctgggactacatgggactacatgcacatgccaccatgcctggctaattgtttgtatattttttttgtagagatgggctttcatcatgttgcccaggctgggcttgaactcctgggcttaagtgatctgcctgcctcggcctcccacgtgctgggattataggcatgagccaatgtgcccggcctcaaccatttcttgataagttaagggccttcacagtaatatcaattactgtgcttggctataaagtcattacactggagagcatataactgatgctcagaatgaaggctctgaaatcatcgagaaatggtttggctgctcagaactctttctttttccttctttcttgctcatggattttcagctgtccattccctactggagggctgggtccaactgcttgttcactggcacagtgccttccatgtacaaagtgatcaaacctgtctattaattaagcaaatgagtggtgaatcactgagacggctggatggctgagctgagggatgtgatgtgtgcccaacgtcctgcagggtgctggtgaataacatgagaaagaacttaaaatggcttgatgatctcaccatttagtgaccttggttgtcacactgctttccaagagccctttaaaggtaggaatgagagctgtttccagtatgcattccaataggaatgcagctttgctaaagttagagacataaactaaaaccctgtgaagtcctatagagcccttggacttatttcctagcaagcatttatcatccccaccatcctctacttcaggacacttgagcagaaacagtcaaggtttttgccgttttcatcctgctcttcaaaacactgtaagtagtggcgcaggtaagcacagccacaggtgaagaccgttttcagctgaggctgcacatcagaaccacagatcacaggggatggtgcgtgacaatcgtctcagttctcccagtaatgcccatgctagccccaggctcgatgccaggagggaagtgcattccttactgagggagggcatcaggcgtgggtcttccacggaaccccaataggaatcagcaacccccaagcagatattactcaaaggtggtattacatacaacagtagtcagactcagacttcaagcagcccaaagagtggaaccacaggcttgcacaattataaaatgtttttatttcaattacataataacacgttttcctcaaattttattgaggttttggtctttttgcattcaattctatcttgtaacagtaatatgaatccacataatttcataaaatgtcaacaacattcataaggtacattcctttgtgattttatattttacaattttaaatctaactttacaattattttaaaaaatttttttatatagaaaacagatattttcttcaggcagatcaaaacaagaattttccagtaagaatatactgggacataacaaatgaaaatatttataccaaaataccaaaagtgattcagctctttaaaatatcctactatagtctaattagtagcttgtacaagaacaagtaaccattttttactgctcttttgaatgatgattagaaattcaaacaaagtattttaaggttcaaaaactttttttttttttttttttttttttagagacagtgtctcactctgtctcccaggctagagtacagtgtgcaatcatagctcactgcagccttgaactcctggcctcaagcaatcctcccaccttggcttcccaatgtgctaggtttacaggcgtgaaaacattgtgttgtgtgtgtgtgtgtttttttttttttttttagacagagtttcgctcttgttgtccaggctggagtacaatggcttgatcttggctcactgcaatctctgcctcgcaggttcaagcgattctcctgcctcagcctctggagtggctgggattacaggcgcccaccatcacgcccggccaattttttgtatttttagtagagacagggtttcaccatgttggccaggctggcctcgaactcttgacctcaggtgatccacctgccttggcctcccaatgtactgagattacaggcatgagccaccacgcccggccaaaaacatttaaaaaatgactgtccctgctcaaatactgcagtaggaaatgtaatttgacatatatcacttccagaaaaaaactttaaatctttctataaaatgaatttgatacatcatcagcatgaagtgaagttaaaatctcttacaaagtaaattcaggtatatcaacaatgagatccaaaagtatcggttcaagatcaaagactcatatgaggtaaaggcaaataaagcccctcatgctttcagacatttacttgttatccttaaaatgattattgttctaaggtgcaaatcttatcattcagtgacctatttgctatttggctgtttatctcctttaaataaaataccatacaggttataatgtacattttaaaatcaaatatgaaagtacacatatgtgaacaagacattaatttaaatatcaattatattcataatacagaagtctaagaatgctatttggtcatttcaattagatgctgatatatttggtcaagaaaacccacattcctatcagcctaaggcaaatagtaaatgcctctatttttattaagtggactataaacagtagacattattgtttgatactactggaatgctctcaattagaacgtacactgataacaaatatgtctttctaatctgggtgataacctcaatgattacatggaaatctacaagtaacagtctataacttaaagcagtagagcacctggtaattgtcatacagtgcctctctatgaatttagaacattctacttacattggcagtggagagaaaagaccccttcacactgagacttcctgtgcaccgcgcctgccgcctgcctcagcttaggacatggtacagtcttctttgcttttgcccttctcattccctcctctggtatcttctctgctttctggattgaagtgccctggctctcttcctggtgccgacaagtcatcgttctctaggctattgctgtctaaagctttcctgacggtctgacttggatgttctgacatctcacacctctctgtactttctgcttcacaggcatcactaatgtcctgtgagggactttcatgttcgggcagggtgcagcgatctgcgtcttcgctctttggttctgcaggactgctttgagtggcaccatctattttagcattatcttttgcaacaccttcatctaattcttcaccaccagccctcgggcctgatgattgaacggtgtcatcctcaaaatctaatgtgtctccatcagctagtacctcctcagctgctgtttgtacatcatcaccttcttggtcaagttttccatccaacttaattttaggattctccggacaatcaacattttcactgctttctgctgcaattttctgttttggattttcagtcacctcgttttgggcttccactgctgactttctgtcagtagactttacctgctcttcttccttaatttcacttaaatctgtgttctgatacgttaactcttttttaacatctttaagggtttctacgggtactggggattttttcttcttgtttttctttttcttgttctttgtcttcttctgcgatgagtccaatgcctctccctgttggtcactcttttcttcatcgggctctttcatatctaagggttcattttgagtgtctactgtacttggacctgtcgcttcctgacagttgccctcagttcctgctggagaaccaggaacttctgtcttgattggtttctcgtcccttaatcctgtttcttcaccctcttcttcgttgtgatccctacctacttctgtactgtgcgctggaacctccttgggctcagctgcttcctggttggtgaattctttctctaaactatgccctgtgcttgtctctaactcttgggggacctctaccatacatttgtcatcatgataaactgtgtcatcactatgccctaaaggacacgaggccactgtgcctgcctgctcttcaacctgagtcactgctgcctctcccacattctctgtgtggttcccaccatctaagtcactccaacagttggatggctcaaggggagttctggtcctgtcatctggtgcacccatgacctcatttgactcaacctgtactgtgttttcagggagagaactgctctcaagaatttggctttgaacctgttcctcataggtagcacctgctaaggttcctaggaatggggcagtgtcttcagaggatttctggtcctcggtattctcaccagcagggaatacctctatgtccacacagtccttcactgtgtcctctgtgtgttgttctttctcagtattgtgcaagatttctcttttccccacattcgccacgatttcatttttcacctccacttcactggctcttcctagggtcccatcccctgtcgacttgagggcatttaactcttcttttgtcatcttggtaggaccttggtatccaacattattgagggtgtcggaagtctctccattggtagctatttctgaatttaggattattccatgtttctttaattcctctttcagcatgactacttcttctctaagatcatcccgttcactccttacggaatcaaagaactctttctgcctctctaatgcccctatctttttgtctttccactctattgtttcctgaagatcagaaatctccctgatagaactcgcctgtttctgctgtagctgtcggatttcctcgagcatttcctctctttgcttcagggcctccttgacttcagcaaactgaaattgcagtatactgtgggcgtgtttttccctttcaaattctttgtttttctcttcgtactgccgcctagattcagccagctgttcttcaagctccagcaacatatcttttagggtatcaacctggtacatgaagtttgtcttttcattgtctagctgagcattggaaaccatagccttcttatatttctcttcaacttctgctagagagtccttcatctctttcaatccctgcatgtatttgccttctacatcctgaatctggtcctttaactcattgagttccttgatttccctgatggatgcctcggtgtcgatggagatggaggtgtctccgctgcctctccgagaggaagtcccacccagagaggccagcgtggctgcagacaggcccggcatgttacgagaccccttctcagtaaaatctttttctggtctctcttctaccagcttctgcgcttccgggctcaaacagtcgatctcccggctttgagcggccgcggggctggtcatcctgccgggctcggcccgctccacccggcgggaaatgctcggggaccgcgccgggagcccctcgcgggccgggccagggggcgcgcgctctgtccgcggagacggagccactcgccgctaagtgaacgctcgcgcttccggggccaggagccagcccgccggggagcggctcgcggcgctgggctcgggcgcggccgacaggggcggggcgcaggtggccgcgggctgagtcgggctcggggtggaagggcgccggggaagcgggactcgggcgcctccgcccgtcccacggcc

SEQ ID NO: 12141 - RNA, 5756 nt, Homo sapiens
  source 1..5756: mol_type = other RNA
ctgcagactcgacctcccaggctcaggtgtttctgcctcctaagtagctgggactacatgggactacatgcacatgccaccatgcctggctaattgtttgtatattttttttgtagagatgggctttcatcatgttgcccaggctgggcttgaactcctgggcttaagtgatctgcctgcctcggcctcccacgtgctgggattataggcatgagccaatgtgcccggcctcaaccatttcttgataagttaagggccttcacagtaatatcaattactgtgcttggctataaagtcattacactggagagcatataactgatgctcagaatgaaggctctgaaatcatcgagaaatggtttggctgctcagaactctttctttttccttctttcttgctcatggattttcagctgtccattccctactggagggctgggtccaactgcttgttcactggcacagtgccttccatgtacaaagtgatcaaacctgtctattaattaagcaaatgagtggtgaatcactgagacggctggatggctgagctgagggatgtgatgtgtgcccaacgtcctgcagggtgctggtgaataacatgagaaagaacttaaaatggcttgatgatctcaccatttagtgaccttggttgtcacactgctttccaagagccctttaaaggtaggaatgagagctgtttccagtatgcattccaataggaatgcagctttgctaaagttagagacataaactaaaaccctgtgaagtcctatagagcccttggacttatttcctagcaagcatttatcatccccaccatcctctacttcaggacacttgagcagaaacagtcaaggtttttgccgttttcatcctgctcttcaaaacactgtaagtagtggcgcaggtaagcacagccacaggtgaagaccgttttcagctgaggctgcacatcagaaccacagatcacaggggatggtgcgtgacaatcgtctcagttctcccagtaatgcccatgctagccccaggctcgatgccaggagggaagtgcattccttactgagggagggcatcaggcgtgggtcttccacggaaccccaataggaatcagcaacccccaagcagatattactcaaaggtggtattacatacaacagtagtcagactcagacttcaagcagcccaaagagtggaaccacaggcttgcacaattataaaatgtttttatttcaattacataataacacgttttcctcaaattttattgaggttttggtctttttgcattcaattctatcttgtaacagtaatatgaatccacataatttcataaaatgtcaacaacattcataaggtacattcctttgtgattttatattttacaattttaaatctaactttacaattattttaaaaaatttttttatatagaaaacagatattttcttcaggcagatcaaaacaagaattttccagtaagaatatactgggacataacaaatgaaaatatttataccaaaataccaaaagtgattcagctctttaaaatatcctactatagtctaattagtagcttgtacaagaacaagtaaccattttttactgctcttttgaatgatgattagaaattcaaacaaagtattttaaggttcaaaaactttttttttttttttttttttttttagagacagtgtctcactctgtctcccaggctagagtacagtgtgcaatcatagctcactgcagccttgaactcctggcctcaagcaatcctcccaccttggcttcccaatgtgctaggtttacaggcgtgaaaacattgtgttgtgtgtgtgtgtgtttttttttttttttttagacagagtttcgctcttgttgtccaggctggagtacaatggcttgatcttggctcactgcaatctctgcctcgcaggttcaagcgattctcctgcctcagcctctggagtggctgggattacaggcgcccaccatcacgcccggccaattttttgtatttttagtagagacagggtttcaccatgttggccaggctggcctcgaactcttgacctcaggtgatccacctgccttggcctcccaatgtactgagattacaggcatgagccaccacgcccggccaaaaacatttaaaaaatgactgtccctgctcaaatactgcagtaggaaatgtaatttgacatatatcacttccagaaaaaaactttaaatctttctataaaatgaatttgatacatcatcagcatgaagtgaagttaaaatctcttacaaagtaaattcaggtatatcaacaatgagatccaaaagtatcggttcaagatcaaagactcatatgaggtaaaggcaaataaagcccctcatgctttcagacatttacttgttatccttaaaatgattattgttctaaggtgcaaatcttatcattcagtgacctatttgctatttggctgtttatctcctttaaataaaataccatacaggttataatgtacattttaaaatcaaatatgaaagtacacatatgtgaacaagacattaatttaaatatcaattatattcataatacagaagtctaagaatgctatttggtcatttcaattagatgctgatatatttggtcaagaaaacccacattcctatcagcctaaggcaaatagtaaatgcctctatttttattaagtggactataaacagtagacattattgtttgatactactggaatgctctcaattagaacgtacactgataacaaatatgtctttctaatctgggtgataacctcaatgattacatggaaatctacaagtaacagtctataacttaaagcagtagagcacctggtaattgtcatacagtgcctctctatgaatttagaacattctacttacattggcagtggagagaaaagaccccttcacactgagacttcctgtgcaccgcgcctgccgcctgcctcagcttaggacatggtacagtcttctttgcttttgcccttctcattccctcctctggtatcttctctgctttctggattgaagtgccctggctctcttcctggtgccgacaagtcatcgttctctaggctattgctgtctaaagctttcctgacggtctgacttggatgttctgacatctcacacctctctgtactttctgcttcacaggcatcactaatgtcctgtgagggactttcatgttcgggcagggtgcagcgatctgcgtcttcgctctttggttctgcaggactgctttgagtggcaccatctattttagcattatcttttgcaacaccttcatctaattcttcaccaccagccctcgggcctgatgattgaacggtgtcatcctcaaaatctaatgtgtctccatcagctagtacctcctcagctgctgtttgtacatcatcaccttcttggtcaagttttccatccaacttaattttaggattctccggacaatcaacattttcactgctttctgctgcaattttctgttttggattttcagtcacctcgttttgggcttccactgctgactttctgtcagtagactttacctgctcttcttccttaatttcacttaaatctgtgttctgatacgttaactcttttttaacatctttaagggtttctacgggtactggggattttttcttcttgtttttctttttcttgttctttgtcttcttctgcgatgagtccaatgcctctccctgttggtcactcttttcttcatcgggctctttcatatctaagggttcattttgagtgtctactgtacttggacctgtcgcttcctgacagttgccctcagttcctgctggagaaccaggaacttctgtcttgattggtttctcgtcccttaatcctgtttcttcaccctcttcttcgttgtgatccctacctacttctgtactgtgcgctggaacctccttgggctcagctgcttcctggttggtgaattctttctctaaactatgccctgtgcttgtctctaactcttgggggacctctaccatacatttgtcatcatgataaactgtgtcatcactatgccctaaaggacacgaggccactgtgcctgcctgctcttcaacctgagtcactgctgcctctcccacattctctgtgtggttcccaccatctaagtcactccaacagttggatggctcaaggggagttctggtcctgtcatctggtgcacccatgacctcatttgactcaacctgtactgtgttttcagggagagaactgctctcaagaatttggctttgaacctgttcctcataggtagcacctgctaaggttcctaggaatggggcagtgtcttcagaggatttctggtcctcggtattctcaccagcagggaatacctctatgtccacacagtccttcactgtgtcctctgtgtgttgttctttctcagtattgtgcaagatttctcttttccccacattcgccacgatttcatttttcacctccacttcactggctcttcctagggtcccatcccctgtcgacttgagggcatttaactcttcttttgtcatcttggtaggaccttggtatccaacattattgagggtgtcggaagtctctccattggtagctatttctgaatttaggattattccatgtttctttaattcctctttcagcatgactacttcttctctaagatcatcccgttcactccttacggaatcaaagaactctttctgcctctctaatgcccctatctttttgtctttccactctattgtttcctgaagatcagaaatctccctgatagaactcgcctgtttctgctgtagctgtcggatttcctcgagcatttcctctctttgcttcagggcctccttgacttcagcaaactgaaattgcagtatactgtgggcgtgtttttccctttcaaattctttgtttttctcttcgtactgccgcctagattcagccagctgttcttcaagctccagcaacatatcttttagggtatcaacctggtacatgaagtttgtcttttcattgtctagctgagcattggaaaccatagccttcttatatttctcttcaacttctgctagagagtccttcatctctttcaatccctgcatgtatttgccttctacatcctgaatctggtcctttaactcattgagttccttgatttccctgatggatgcctcggtgtcgatggagatggaggtgtctccgctgcctctccgagaggaagtcccacccagagaggccagcgtggctgcagacaggcccggcatgttacgagaccccttctcagtaaaatctttttctggtctctcttctaccctcaggcttccacgactacccactgacatgcgctcgtcttcatcagaagccgatgtgtttcttctggatctacgagagtagcgctcactgtcttccatccactgctcgatgtcaccccattttgtatccagcccataatatttcttttggacctgatagatctccttctgctgccgctccagctccttcatgcggatctcgcgagcctccgcgcgggccgcccgttttgcagcgagccgggcttccgcctcccgcgcgatctggttgagcgcgtcgtcctccgccgtgagccgctcccggttggggagccgcttgcgccccgatccctgggtgcccatgtccatcgaccgcgtcgcccgcagctgccgcggggcccgttgctccagccgctcgcgccgccccggcccggcccc

SEQ ID NO: 12142 - RNA, 5685 nt, Homo sapiens
  source 1..5685: mol_type = other RNA
ctgcagactcgacctcccaggctcaggtgtttctgcctcctaagtagctgggactacatgggactacatgcacatgccaccatgcctggctaattgtttgtatattttttttgtagagatgggctttcatcatgttgcccaggctgggcttgaactcctgggcttaagtgatctgcctgcctcggcctcccacgtgctgggattataggcatgagccaatgtgcccggcctcaaccatttcttgataagttaagggccttcacagtaatatcaattactgtgcttggctataaagtcattacactggagagcatataactgatgctcagaatgaaggctctgaaatcatcgagaaatggtttggctgctcagaactctttctttttccttctttcttgctcatggattttcagctgtccattccctactggagggctgggtccaactgcttgttcactggcacagtgccttccatgtacaaagtgatcaaacctgtctattaattaagcaaatgagtggtgaatcactgagacggctggatggctgagctgagggatgtgatgtgtgcccaacgtcctgcagggtgctggtgaataacatgagaaagaacttaaaatggcttgatgatctcaccatttagtgaccttggttgtcacactgctttccaagagccctttaaaggtaggaatgagagctgtttccagtatgcattccaataggaatgcagctttgctaaagttagagacataaactaaaaccctgtgaagtcctatagagcccttggacttatttcctagcaagcatttatcatccccaccatcctctacttcaggacacttgagcagaaacagtcaaggtttttgccgttttcatcctgctcttcaaaacactgtaagtagtggcgcaggtaagcacagccacaggtgaagaccgttttcagctgaggctgcacatcagaaccacagatcacaggggatggtgcgtgacaatcgtctcagttctcccagtaatgcccatgctagccccaggctcgatgccaggagggaagtgcattccttactgagggagggcatcaggcgtgggtcttccacggaaccccaataggaatcagcaacccccaagcagatattactcaaaggtggtattacatacaacagtagtcagactcagacttcaagcagcccaaagagtggaaccacaggcttgcacaattataaaatgtttttatttcaattacataataacacgttttcctcaaattttattgaggttttggtctttttgcattcaattctatcttgtaacagtaatatgaatccacataatttcataaaatgtcaacaacattcataaggtacattcctttgtgattttatattttacaattttaaatctaactttacaattattttaaaaaatttttttatatagaaaacagatattttcttcaggcagatcaaaacaagaattttccagtaagaatatactgggacataacaaatgaaaatatttataccaaaataccaaaagtgattcagctctttaaaatatcctactatagtctaattagtagcttgtacaagaacaagtaaccattttttactgctcttttgaatgatgattagaaattcaaacaaagtattttaaggttcaaaaactttttttttttttttttttttttttagagacagtgtctcactctgtctcccaggctagagtacagtgtgcaatcatagctcactgcagccttgaactcctggcctcaagcaatcctcccaccttggcttcccaatgtgctaggtttacaggcgtgaaaacattgtgttgtgtgtgtgtgtgtttttttttttttttttagacagagtttcgctcttgttgtccaggctggagtacaatggcttgatcttggctcactgcaatctctgcctcgcaggttcaagcgattctcctgcctcagcctctggagtggctgggattacaggcgcccaccatcacgcccggccaattttttgtatttttagtagagacagggtttcaccatgttggccaggctggcctcgaactcttgacctcaggtgatccacctgccttggcctcccaatgtactgagattacaggcatgagccaccacgcccggccaaaaacatttaaaaaatgactgtccctgctcaaatactgcagtaggaaatgtaatttgacatatatcacttccagaaaaaaactttaaatctttctataaaatgaatttgatacatcatcagcatgaagtgaagttaaaatctcttacaaagtaaattcaggtatatcaacaatgagatccaaaagtatcggttcaagatcaaagactcatatgaggtaaaggcaaataaagcccctcatgctttcagacatttacttgttatccttaaaatgattattgttctaaggtgcaaatcttatcattcagtgacctatttgctatttggctgtttatctcctttaaataaaataccatacaggttataatgtacattttaaaatcaaatatgaaagtacacatatgtgaacaagacattaatttaaatatcaattatattcataatacagaagtctaagaatgctatttggtcatttcaattagatgctgatatatttggtcaagaaaacccacattcctatcagcctaaggcaaatagtaaatgcctctatttttattaagtggactataaacagtagacattattgtttgatactactggaatgctctcaattagaacgtacactgataacaaatatgtctttctaatctgggtgataacctcaatgattacatggaaatctacaagtaacagtctataacttaaagcagtagagcacctggtaattgtcatacagtgcctctctatgaatttagaacattctacttacattggcagtggagagaaaagaccccttcacactgagacttcctgtgcaccgcgcctgccgcctgcctcagcttaggacatggtacagtcttctttgcttttgcccttctcattccctcctctggtatcttctctgctttctggattgaagtgccctggctctcttcctggtgccgacaagtcatcgttctctaggctattgctgtctaaagctttcctgacggtctgacttggatgttctgacatctcacacctctctgtactttctgcttcacaggcatcactaatgtcctgtgagggactttcatgttcgggcagggtgcagcgatctgcgtcttcgctctttggttctgcaggactgctttgagtggcaccatctattttagcattatcttttgcaacaccttcatctaattcttcaccaccagccctcgggcctgatgattgaacggtgtcatcctcaaaatctaatgtgtctccatcagctagtacctcctcagctgctgtttgtacatcatcaccttcttggtcaagttttccatccaacttaattttaggattctccggacaatcaacattttcactgctttctgctgcaattttctgttttggattttcagtcacctcgttttgggcttccactgctgactttctgtcagtagactttacctgctcttcttccttaatttcacttaaatctgtgttctgatacgttaactcttttttaacatctttaagggtttctacgggtactggggattttttcttcttgtttttctttttcttgttctttgtcttcttctgcgatgagtccaatgcctctccctgttggtcactcttttcttcatcgggctctttcatatctaagggttcattttgagtgtctactgtacttggacctgtcgcttcctgacagttgccctcagttcctgctggagaaccaggaacttctgtcttgattggtttctcgtcccttaatcctgtttcttcaccctcttcttcgttgtgatccctacctacttctgtactgtgcgctggaacctccttgggctcagctgcttcctggttggtgaattctttctctaaactatgccctgtgcttgtctctaactcttgggggacctctaccatacatttgtcatcatgataaactgtgtcatcactatgccctaaaggacacgaggccactgtgcctgcctgctcttcaacctgagtcactgctgcctctcccacattctctgtgtggttcccaccatctaagtcactccaacagttggatggctcaaggggagttctggtcctgtcatctggtgcacccatgacctcatttgactcaacctgtactgtgttttcagggagagaactgctctcaagaatttggctttgaacctgttcctcataggtagcacctgctaaggttcctaggaatggggcagtgtcttcagaggatttctggtcctcggtattctcaccagcagggaatacctctatgtccacacagtccttcactgtgtcctctgtgtgttgttctttctcagtattgtgcaagatttctcttttccccacattcgccacgatttcatttttcacctccacttcactggctcttcctagggtcccatcccctgtcgacttgagggcatttaactcttcttttgtcatcttggtaggaccttggtatccaacattattgagggtgtcggaagtctctccattggtagctatttctgaatttaggattattccatgtttctttaattcctctttcagcatgactacttcttctctaagatcatcccgttcactccttacggaatcaaagaactctttctgcctctctaatgcccctatctttttgtctttccactctattgtttcctgaagatcagaaatctccctgatagaactcgcctgtttctgctgtagctgtcggatttcctcgagcatttcctctctttgcttcagggcctccttgacttcagcaaactgaaattgcagtatactgtgggcgtgtttttccctttcaaattctttgtttttctcttcgtactgccgcctagattcagccagctgttcttcaagctccagcaacatatcttttagggtatcaacctggtacatgaagtttgtcttttcattgtctagctgagcattggaaaccatagccttcttatatttctcttcaacttctgctagagagtccttcatctctttcaatccctgcatgtatttgccttctacatcctgaatctggtcctttaactcattgagttccttgatttccctgatggatgcctcggtgtcgatggagatggaggtgtctccgctgcctctccgagaggaagtcccacccagagaggccagcgtggctgcagacaggcccggcatgttacgagaccccttctcagtaaaatctttttctggtctctcttctaccctcaggcttccacgactacccactgacatgcgctcgtcttcatcagaagccgatgtgtttcttctggatctacgagagtagcgctcactgtcttcctccttctgctgccgctccagctccttcatgcggatctcgcgagcctccgcgcgggccgcccgttttgcagcgagccgggcttccgccagcttctgcgcttccgggctcaaacagtcgatctcccggctttgagcggccgcggggctggtcatcctgccgggctcggcccgctccacccggcgggaaatgctcggggaccgcgccgggagcccctcgcgggccgggccagggggcgcgcgctctgtc

SEQ ID NO: 12143 - RNA, 5667 nt, Homo sapiens
  source 1..5667: mol_type = other RNA
ctgcagactcgacctcccaggctcaggtgtttctgcctcctaagtagctgggactacatgggactacatgcacatgccaccatgcctggctaattgtttgtatattttttttgtagagatgggctttcatcatgttgcccaggctgggcttgaactcctgggcttaagtgatctgcctgcctcggcctcccacgtgctgggattataggcatgagccaatgtgcccggcctcaaccatttcttgataagttaagggccttcacagtaatatcaattactgtgcttggctataaagtcattacactggagagcatataactgatgctcagaatgaaggctctgaaatcatcgagaaatggtttggctgctcagaactctttctttttccttctttcttgctcatggattttcagctgtccattccctactggagggctgggtccaactgcttgttcactggcacagtgccttccatgtacaaagtgatcaaacctgtctattaattaagcaaatgagtggtgaatcactgagacggctggatggctgagctgagggatgtgatgtgtgcccaacgtcctgcagggtgctggtgaataacatgagaaagaacttaaaatggcttgatgatctcaccatttagtgaccttggttgtcacactgctttccaagagccctttaaaggtaggaatgagagctgtttccagtatgcattccaataggaatgcagctttgctaaagttagagacataaactaaaaccctgtgaagtcctatagagcccttggacttatttcctagcaagcatttatcatccccaccatcctctacttcaggacacttgagcagaaacagtcaaggtttttgccgttttcatcctgctcttcaaaacactgtaagtagtggcgcaggtaagcacagccacaggtgaagaccgttttcagctgaggctgcacatcagaaccacagatcacaggggatggtgcgtgacaatcgtctcagttctcccagtaatgcccatgctagccccaggctcgatgccaggagggaagtgcattccttactgagggagggcatcaggcgtgggtcttccacggaaccccaataggaatcagcaacccccaagcagatattactcaaaggtggtattacatacaacagtagtcagactcagacttcaagcagcccaaagagtggaaccacaggcttgcacaattataaaatgtttttatttcaattacataataacacgttttcctcaaattttattgaggttttggtctttttgcattcaattctatcttgtaacagtaatatgaatccacataatttcataaaatgtcaacaacattcataaggtacattcctttgtgattttatattttacaattttaaatctaactttacaattattttaaaaaatttttttatatagaaaacagatattttcttcaggcagatcaaaacaagaattttccagtaagaatatactgggacataacaaatgaaaatatttataccaaaataccaaaagtgattcagctctttaaaatatcctactatagtctaattagtagcttgtacaagaacaagtaaccattttttactgctcttttgaatgatgattagaaattcaaacaaagtattttaaggttcaaaaactttttttttttttttttttttttttagagacagtgtctcactctgtctcccaggctagagtacagtgtgcaatcatagctcactgcagccttgaactcctggcctcaagcaatcctcccaccttggcttcccaatgtgctaggtttacaggcgtgaaaacattgtgttgtgtgtgtgtgtgtttttttttttttttttagacagagtttcgctcttgttgtccaggctggagtacaatggcttgatcttggctcactgcaatctctgcctcgcaggttcaagcgattctcctgcctcagcctctggagtggctgggattacaggcgcccaccatcacgcccggccaattttttgtatttttagtagagacagggtttcaccatgttggccaggctggcctcgaactcttgacctcaggtgatccacctgccttggcctcccaatgtactgagattacaggcatgagccaccacgcccggccaaaaacatttaaaaaatgactgtccctgctcaaatactgcagtaggaaatgtaatttgacatatatcacttccagaaaaaaactttaaatctttctataaaatgaatttgatacatcatcagcatgaagtgaagttaaaatctcttacaaagtaaattcaggtatatcaacaatgagatccaaaagtatcggttcaagatcaaagactcatatgaggtaaaggcaaataaagcccctcatgctttcagacatttacttgttatccttaaaatgattattgttctaaggtgcaaatcttatcattcagtgacctatttgctatttggctgtttatctcctttaaataaaataccatacaggttataatgtacattttaaaatcaaatatgaaagtacacatatgtgaacaagacattaatttaaatatcaattatattcataatacagaagtctaagaatgctatttggtcatttcaattagatgctgatatatttggtcaagaaaacccacattcctatcagcctaaggcaaatagtaaatgcctctatttttattaagtggactataaacagtagacattattgtttgatactactggaatgctctcaattagaacgtacactgataacaaatatgtctttctaatctgggtgataacctcaatgattacatggaaatctacaagtaacagtctataacttaaagcagtagagcacctggtaattgtcatacagtgcctctctatgaatttagaacattctacttacattggcagtggagagaaaagaccccttcacactgagacttcctgtgcaccgcgcctgccgcctgcctcagcttaggacatggtacagtcttctttgcttttgcccttctcattccctcctctggtatcttctctgctttctggattgaagtgccctggctctcttcctggtgccgacaagtcatcgttctctaggctattgctgtctaaagctttcctgacggtctgacttggatgttctgacatctcacacctctctgtactttctgcttcacaggcatcactaatgtcctgtgagggactttcatgttcgggcagggtgcagcgatctgcgtcttcgctctttggttctgcaggactgctttgagtggcaccatctattttagcattatcttttgcaacaccttcatctaattcttcaccaccagccctcgggcctgatgattgaacggtgtcatcctcaaaatctaatgtgtctccatcagctagtacctcctcagctgctgtttgtacatcatcaccttcttggtcaagttttccatccaacttaattttaggattctccggacaatcaacattttcactgctttctgctgcaattttctgttttggattttcagtcacctcgttttgggcttccactgctgactttctgtcagtagactttacctgctcttcttccttaatttcacttaaatctgtgttctgatacgttaactcttttttaacatctttaagggtttctacgggtactggggattttttcttcttgtttttctttttcttgttctttgtcttcttctgcgatgagtccaatgcctctccctgttggtcactcttttcttcatcgggctctttcatatctaagggttcattttgagtgtctactgtacttggacctgtcgcttcctgacagttgccctcagttcctgctggagaaccaggaacttctgtcttgattggtttctcgtcccttaatcctgtttcttcaccctcttcttcgttgtgatccctacctacttctgtactgtgcgctggaacctccttgggctcagctgcttcctggttggtgaattctttctctaaactatgccctgtgcttgtctctaactcttgggggacctctaccatacatttgtcatcatgataaactgtgtcatcactatgccctaaaggacacgaggccactgtgcctgcctgctcttcaacctgagtcactgctgcctctcccacattctctgtgtggttcccaccatctaagtcactccaacagttggatggctcaaggggagttctggtcctgtcatctggtgcacccatgacctcatttgactcaacctgtactgtgttttcagggagagaactgctctcaagaatttggctttgaacctgttcctcataggtagcacctgctaaggttcctaggaatggggcagtgtcttcagaggatttctggtcctcggtattctcaccagcagggaatacctctatgtccacacagtccttcactgtgtcctctgtgtgttgttctttctcagtattgtgcaagatttctcttttccccacattcgccacgatttcatttttcacctccacttcactggctcttcctagggtcccatcccctgtcgacttgagggcatttaactcttcttttgtcatcttggtaggaccttggtatccaacattattgagggtgtcggaagtctctccattggtagctatttctgaatttaggattattccatgtttctttaattcctctttcagcatgactacttcttctctaagatcatcccgttcactccttacggaatcaaagaactctttctgcctctctaatgcccctatctttttgtctttccactctattgtttcctgaagatcagaaatctccctgatagaactcgcctgtttctgctgtagctgtcggatttcctcgagcatttcctctctttgcttcagggcctccttgacttcagcaaactgaaattgcagtatactgtgggcgtgtttttccctttcaaattctttgtttttctcttcgtactgccgcctagattcagccagctgttcttcaagctccagcaacatatcttttagggtatcaacctggtacatgaagtttgtcttttcattgtctagctgagcattggaaaccatagccttcttatatttctcttcaacttctgctagagagtccttcatctctttcaatccctgcatgtatttgccttctacatcctgaatctggtcctttaactcattgagttccttgatttccctgatggatgcctcggtgtcgatggagatggaggtgtctccgctgcctctccgagaggaagtcccacccagagaggccagcgtggctgcagacaggcccggcatgttacgagaccccttctcagtaaaatctttttctggtctctcttctaccctcaggcttccacgactacccactgacatgcgctcgtcttcatcagaagccgatgtgtttcttctggatctacgagagtagcgctcactgtcttcctccttctgctgccgctccagctccttcatgcggatctcgcgagcctccgcgcgggccgcccgttttgcagcgagccgggcttccgcctcccgcgcgatctggttgagcgcgtcgtcctccgccgtgagccgctcccggttggggagccgcttgcgccccgatccctgggtgcccatgtccatcgaccgcgtcgcccgcagctgccgcggggcccgttgctccagccgc

SEQ ID NO: 12144 - RNA, 5855 nt, Homo sapiens
  source 1..5855: mol_type = other RNA
ctgcagactcgacctcccaggctcaggtgtttctgcctcctaagtagctgggactacatgggactacatgcacatgccaccatgcctggctaattgtttgtatattttttttgtagagatgggctttcatcatgttgcccaggctgggcttgaactcctgggcttaagtgatctgcctgcctcggcctcccacgtgctgggattataggcatgagccaatgtgcccggcctcaaccatttcttgataagttaagggccttcacagtaatatcaattactgtgcttggctataaagtcattacactggagagcatataactgatgctcagaatgaaggctctgaaatcatcgagaaatggtttggctgctcagaactctttctttttccttctttcttgctcatggattttcagctgtccattccctactggagggctgggtccaactgcttgttcactggcacagtgccttccatgtacaaagtgatcaaacctgtctattaattaagcaaatgagtggtgaatcactgagacggctggatggctgagctgagggatgtgatgtgtgcccaacgtcctgcagggtgctggtgaataacatgagaaagaacttaaaatggcttgatgatctcaccatttagtgaccttggttgtcacactgctttccaagagccctttaaaggtaggaatgagagctgtttccagtatgcattccaataggaatgcagctttgctaaagttagagacataaactaaaaccctgtgaagtcctatagagcccttggacttatttcctagcaagcatttatcatccccaccatcctctacttcaggacacttgagcagaaacagtcaaggtttttgccgttttcatcctgctcttcaaaacactgtaagtagtggcgcaggtaagcacagccacaggtgaagaccgttttcagctgaggctgcacatcagaaccacagatcacaggggatggtgcgtgacaatcgtctcagttctcccagtaatgcccatgctagccccaggctcgatgccaggagggaagtgcattccttactgagggagggcatcaggcgtgggtcttccacggaaccccaataggaatcagcaacccccaagcagatattactcaaaggtggtattacatacaacagtagtcagactcagacttcaagcagcccaaagagtggaaccacaggcttgcacaattataaaatgtttttatttcaattacataataacacgttttcctcaaattttattgaggttttggtctttttgcattcaattctatcttgtaacagtaatatgaatccacataatttcataaaatgtcaacaacattcataaggtacattcctttgtgattttatattttacaattttaaatctaactttacaattattttaaaaaatttttttatatagaaaacagatattttcttcaggcagatcaaaacaagaattttccagtaagaatatactgggacataacaaatgaaaatatttataccaaaataccaaaagtgattcagctctttaaaatatcctactatagtctaattagtagcttgtacaagaacaagtaaccattttttactgctcttttgaatgatgattagaaattcaaacaaagtattttaaggttcaaaaactttttttttttttttttttttttttagagacagtgtctcactctgtctcccaggctagagtacagtgtgcaatcatagctcactgcagccttgaactcctggcctcaagcaatcctcccaccttggcttcccaatgtgctaggtttacaggcgtgaaaacattgtgttgtgtgtgtgtgtgtttttttttttttttttagacagagtttcgctcttgttgtccaggctggagtacaatggcttgatcttggctcactgcaatctctgcctcgcaggttcaagcgattctcctgcctcagcctctggagtggctgggattacaggcgcccaccatcacgcccggccaattttttgtatttttagtagagacagggtttcaccatgttggccaggctggcctcgaactcttgacctcaggtgatccacctgccttggcctcccaatgtactgagattacaggcatgagccaccacgcccggccaaaaacatttaaaaaatgactgtccctgctcaaatactgcagtaggaaatgtaatttgacatatatcacttccagaaaaaaactttaaatctttctataaaatgaatttgatacatcatcagcatgaagtgaagttaaaatctcttacaaagtaaattcaggtatatcaacaatgagatccaaaagtatcggttcaagatcaaagactcatatgaggtaaaggcaaataaagcccctcatgctttcagacatttacttgttatccttaaaatgattattgttctaaggtgcaaatcttatcattcagtgacctatttgctatttggctgtttatctcctttaaataaaataccatacaggttataatgtacattttaaaatcaaatatgaaagtacacatatgtgaacaagacattaatttaaatatcaattatattcataatacagaagtctaagaatgctatttggtcatttcaattagatgctgatatatttggtcaagaaaacccacattcctatcagcctaaggcaaatagtaaatgcctctatttttattaagtggactataaacagtagacattattgtttgatactactggaatgctctcaattagaacgtacactgataacaaatatgtctttctaatctgggtgataacctcaatgattacatggaaatctacaagtaacagtctataacttaaagcagtagagcacctggtaattgtcatacagtgcctctctatgaatttagaacattctacttacattggcagtggagagaaaagaccccttcacactgagacttcctgtgcaccgcgcctgccgcctgcctcagcttaggacatggtacagtcttctttgcttttgcccttctcattccctcctctggtatcttctctgctttctggattgaagtgccctggctctcttcctggtgccgacaagtcatcgttctctaggctattgctgtctaaagctttcctgacggtctgacttggatgttctgacatctcacacctctctgtactttctgcttcacaggcatcactaatgtcctgtgagggactttcatgttcgggcagggtgcagcgatctgcgtcttcgctctttggttctgcaggactgctttgagtggcaccatctattttagcattatcttttgcaacaccttcatctaattcttcaccaccagccctcgggcctgatgattgaacggtgtcatcctcaaaatctaatgtgtctccatcagctagtacctcctcagctgctgtttgtacatcatcaccttcttggtcaagttttccatccaacttaattttaggattctccggacaatcaacattttcactgctttctgctgcaattttctgttttggattttcagtcacctcgttttgggcttccactgctgactttctgtcagtagactttacctgctcttcttccttaatttcacttaaatctgtgttctgatacgttaactcttttttaacatctttaagggtttctacgggtactggggattttttcttcttgtttttctttttcttgttctttgtcttcttctgcgatgagtccaatgcctctccctgttggtcactcttttcttcatcgggctctttcatatctaagggttcattttgagtgtctactgtacttggacctgtcgcttcctgacagttgccctcagttcctgctggagaaccaggaacttctgtcttgattggtttctcgtcccttaatcctgtttcttcaccctcttcttcgttgtgatccctacctacttctgtactgtgcgctggaacctccttgggctcagctgcttcctggttggtgaattctttctctaaactatgccctgtgcttgtctctaactcttgggggacctctaccatacatttgtcatcatgataaactgtgtcatcactatgccctaaaggacacgaggccactgtgcctgcctgctcttcaacctgagtcactgctgcctctcccacattctctgtgtggttcccaccatctaagtcactccaacagttggatggctcaaggggagttctggtcctgtcatctggtgcacccatgacctcatttgactcaacctgtactgtgttttcagggagagaactgctctcaagaatttggctttgaacctgttcctcataggtagcacctgctaaggttcctaggaatggggcagtgtcttcagaggatttctggtcctcggtattctcaccagcagggaatacctctatgtccacacagtccttcactgtgtcctctgtgtgttgttctttctcagtattgtgcaagatttctcttttccccacattcgccacgatttcatttttcacctccacttcactggctcttcctagggtcccatcccctgtcgacttgagggcatttaactcttcttttgtcatcttggtaggaccttggtatccaacattattgagggtgtcggaagtctctccattggtagctatttctgaatttaggattattccatgtttctttaattcctctttcagcatgactacttcttctctaagatcatcccgttcactccttacggaatcaaagaactctttctgcctctctaatgcccctatctttttgtctttccactctattgtttcctgaagatcagaaatctccctgatagaactcgcctgtttctgctgtagctgtcggatttcctcgagcatttcctctctttgcttcagggcctccttgacttcagcaaactgaaattgcagtatactgtgggcgtgtttttccctttcaaattctttgtttttctcttcgtactgccgcctagattcagccagctgttcttcaagctccagcaacatatcttttagggtatcaacctggtacatgaagtttgtcttttcattgtctagctgagcattggaaaccatagccttcttatatttctcttcaacttctgctagagagtccttcatctctttcaatccctgcatgtatttgccttctacatcctgaatctggtcctttaactcattgagttccttgatttccctgatggatgcctcggtgtcgatggagatggaggtgtctccgctgcctctccgagaggaagtcccacccagagaggccagcgtggctgcagacaggcccggcatgttacgagaccccttctcagtaaaatctttttctggtctctcttctaccctgccagatcttctattcagggactgtgatccatacaattctccatcataaccatttgtccaggcgtaaggacccccatactccaagtcaggctgcgacctcaggcttccacgactacccactgacatgcgctcgtcttcatcagaagccgatgtgtttcttctggatctacgagagtagcgctcactgtcttccatccactgctcgatgtcaccccattttgtatccagcccataatatttcttttggacctgatagatctccttctgctgccgctccagctccttcatgcggatctcgcgagcctccgcgcgggccgcccgttttgcagcgagccgggcttccgcctcccgcgcgatctggttgagcgcgtcgtcctccgccgtgagccgctcccggttggggagccgcttgcgccccgatccctgggtgcccatgtccatcgaccgcgtcgcccgcagctgccgcggggcccgttgctccagccgctcgcgccgccccggcccggcccc

SEQ ID NO: 12145 - RNA, 5816 nt, Homo sapiens
  source 1..5816: mol_type = other RNA
ctgcagactcgacctcccaggctcaggtgtttctgcctcctaagtagctgggactacatgggactacatgcacatgccaccatgcctggctaattgtttgtatattttttttgtagagatgggctttcatcatgttgcccaggctgggcttgaactcctgggcttaagtgatctgcctgcctcggcctcccacgtgctgggattataggcatgagccaatgtgcccggcctcaaccatttcttgataagttaagggccttcacagtaatatcaattactgtgcttggctataaagtcattacactggagagcatataactgatgctcagaatgaaggctctgaaatcatcgagaaatggtttggctgctcagaactctttctttttccttctttcttgctcatggattttcagctgtccattccctactggagggctgggtccaactgcttgttcactggcacagtgccttccatgtacaaagtgatcaaacctgtctattaattaagcaaatgagtggtgaatcactgagacggctggatggctgagctgagggatgtgatgtgtgcccaacgtcctgcagggtgctggtgaataacatgagaaagaacttaaaatggcttgatgatctcaccatttagtgaccttggttgtcacactgctttccaagagccctttaaaggtaggaatgagagctgtttccagtatgcattccaataggaatgcagctttgctaaagttagagacataaactaaaaccctgtgaagtcctatagagcccttggacttatttcctagcaagcatttatcatccccaccatcctctacttcaggacacttgagcagaaacagtcaaggtttttgccgttttcatcctgctcttcaaaacactgtaagtagtggcgcaggtaagcacagccacaggtgaagaccgttttcagctgaggctgcacatcagaaccacagatcacaggggatggtgcgtgacaatcgtctcagttctcccagtaatgcccatgctagccccaggctcgatgccaggagggaagtgcattccttactgagggagggcatcaggcgtgggtcttccacggaaccccaataggaatcagcaacccccaagcagatattactcaaaggtggtattacatacaacagtagtcagactcagacttcaagcagcccaaagagtggaaccacaggcttgcacaattataaaatgtttttatttcaattacataataacacgttttcctcaaattttattgaggttttggtctttttgcattcaattctatcttgtaacagtaatatgaatccacataatttcataaaatgtcaacaacattcataaggtacattcctttgtgattttatattttacaattttaaatctaactttacaattattttaaaaaatttttttatatagaaaacagatattttcttcaggcagatcaaaacaagaattttccagtaagaatatactgggacataacaaatgaaaatatttataccaaaataccaaaagtgattcagctctttaaaatatcctactatagtctaattagtagcttgtacaagaacaagtaaccattttttactgctcttttgaatgatgattagaaattcaaacaaagtattttaaggttcaaaaactttttttttttttttttttttttttagagacagtgtctcactctgtctcccaggctagagtacagtgtgcaatcatagctcactgcagccttgaactcctggcctcaagcaatcctcccaccttggcttcccaatgtgctaggtttacaggcgtgaaaacattgtgttgtgtgtgtgtgtgtttttttttttttttttagacagagtttcgctcttgttgtccaggctggagtacaatggcttgatcttggctcactgcaatctctgcctcgcaggttcaagcgattctcctgcctcagcctctggagtggctgggattacaggcgcccaccatcacgcccggccaattttttgtatttttagtagagacagggtttcaccatgttggccaggctggcctcgaactcttgacctcaggtgatccacctgccttggcctcccaatgtactgagattacaggcatgagccaccacgcccggccaaaaacatttaaaaaatgactgtccctgctcaaatactgcagtaggaaatgtaatttgacatatatcacttccagaaaaaaactttaaatctttctataaaatgaatttgatacatcatcagcatgaagtgaagttaaaatctcttacaaagtaaattcaggtatatcaacaatgagatccaaaagtatcggttcaagatcaaagactcatatgaggtaaaggcaaataaagcccctcatgctttcagacatttacttgttatccttaaaatgattattgttctaaggtgcaaatcttatcattcagtgacctatttgctatttggctgtttatctcctttaaataaaataccatacaggttataatgtacattttaaaatcaaatatgaaagtacacatatgtgaacaagacattaatttaaatatcaattatattcataatacagaagtctaagaatgctatttggtcatttcaattagatgctgatatatttggtcaagaaaacccacattcctatcagcctaaggcaaatagtaaatgcctctatttttattaagtggactataaacagtagacattattgtttgatactactggaatgctctcaattagaacgtacactgataacaaatatgtctttctaatctgggtgataacctcaatgattacatggaaatctacaagtaacagtctataacttaaagcagtagagcacctggtaattgtcatacagtgcctctctatgaatttagaacattctacttacattggcagtggagagaaaagaccccttcacactgagacttcctgtgcaccgcgcctgccgcctgcctcagcttaggacatggtacagtcttctttgcttttgcccttctcattccctcctctggtatcttctctgctttctggattgaagtgccctggctctcttcctggtgccgacaagtcatcgttctctaggctattgctgtctaaagctttcctgacggtctgacttggatgttctgacatctcacacctctctgtactttctgcttcacaggcatcactaatgtcctgtgagggactttcatgttcgggcagggtgcagcgatctgcgtcttcgctctttggttctgcaggactgctttgagtggcaccatctattttagcattatcttttgcaacaccttcatctaattcttcaccaccagccctcgggcctgatgattgaacggtgtcatcctcaaaatctaatgtgtctccatcagctagtacctcctcagctgctgtttgtacatcatcaccttcttggtcaagttttccatccaacttaattttaggattctccggacaatcaacattttcactgctttctgctgcaattttctgttttggattttcagtcacctcgttttgggcttccactgctgactttctgtcagtagactttacctgctcttcttccttaatttcacttaaatctgtgttctgatacgttaactcttttttaacatctttaagggtttctacgggtactggggattttttcttcttgtttttctttttcttgttctttgtcttcttctgcgatgagtccaatgcctctccctgttggtcactcttttcttcatcgggctctttcatatctaagggttcattttgagtgtctactgtacttggacctgtcgcttcctgacagttgccctcagttcctgctggagaaccaggaacttctgtcttgattggtttctcgtcccttaatcctgtttcttcaccctcttcttcgttgtgatccctacctacttctgtactgtgcgctggaacctccttgggctcagctgcttcctggttggtgaattctttctctaaactatgccctgtgcttgtctctaactcttgggggacctctaccatacatttgtcatcatgataaactgtgtcatcactatgccctaaaggacacgaggccactgtgcctgcctgctcttcaacctgagtcactgctgcctctcccacattctctgtgtggttcccaccatctaagtcactccaacagttggatggctcaaggggagttctggtcctgtcatctggtgcacccatgacctcatttgactcaacctgtactgtgttttcagggagagaactgctctcaagaatttggctttgaacctgttcctcataggtagcacctgctaaggttcctaggaatggggcagtgtcttcagaggatttctggtcctcggtattctcaccagcagggaatacctctatgtccacacagtccttcactgtgtcctctgtgtgttgttctttctcagtattgtgcaagatttctcttttccccacattcgccacgatttcatttttcacctccacttcactggctcttcctagggtcccatcccctgtcgacttgagggcatttaactcttcttttgtcatcttggtaggaccttggtatccaacattattgagggtgtcggaagtctctccattggtagctatttctgaatttaggattattccatgtttctttaattcctctttcagcatgactacttcttctctaagatcatcccgttcactccttacggaatcaaagaactctttctgcctctctaatgcccctatctttttgtctttccactctattgtttcctgaagatcagaaatctccctgatagaactcgcctgtttctgctgtagctgtcggatttcctcgagcatttcctctctttgcttcagggcctccttgacttcagcaaactgaaattgcagtatactgtgggcgtgtttttccctttcaaattctttgtttttctcttcgtactgccgcctagattcagccagctgttcttcaagctccagcaacatatcttttagggtatcaacctggtacatgaagtttgtcttttcattgtctagctgagcattggaaaccatagccttcttatatttctcttcaacttctgctagagagtccttcatctctttcaatccctgcatgtatttgccttctacatcctgaatctggtcctttaactcattgagttccttgatttccctgatggatgcctcggtgtcgatggagatggaggtgtctccgctgcctctccgagaggaagtcccacccagagaggccagcgtggctgcagacaggcccggcatgttacgagaccccttctcagtaaaatctttttctggtctctcttctaccctgccagatcttctattcagggactgtgatccatacaattctccatcataaccatttgtcctcaggcttccacgactacccactgacatgcgctcgtcttcatcagaagccgatgtgtttcttctggatctacgagagtagcgctcactgtcttccatccactgctcgatgtcaccccattttgtatccagcccataatatttcttttggacctgatagatctccttctgctgccgctccagctccttcatgcggatctcgcgagcctccgcgcgggccgcccgttttgcagcgagccgggcttccgcctcccgcgcgatctggttgagcgcgtcgtcctccgccgtgagccgctcccggttggggagccgcttgcgccccgatccctgggtgcccatgtccatcgaccgcgtcgcccgcagctgccgcggggcccgttgctccagccgctcgcgccgccccggcccggcccc

SEQ ID NO: 12146 - RNA, 5745 nt, Homo sapiens
  source 1..5745: mol_type = other RNA
ctgcagactcgacctcccaggctcaggtgtttctgcctcctaagtagctgggactacatgggactacatgcacatgccaccatgcctggctaattgtttgtatattttttttgtagagatgggctttcatcatgttgcccaggctgggcttgaactcctgggcttaagtgatctgcctgcctcggcctcccacgtgctgggattataggcatgagccaatgtgcccggcctcaaccatttcttgataagttaagggccttcacagtaatatcaattactgtgcttggctataaagtcattacactggagagcatataactgatgctcagaatgaaggctctgaaatcatcgagaaatggtttggctgctcagaactctttctttttccttctttcttgctcatggattttcagctgtccattccctactggagggctgggtccaactgcttgttcactggcacagtgccttccatgtacaaagtgatcaaacctgtctattaattaagcaaatgagtggtgaatcactgagacggctggatggctgagctgagggatgtgatgtgtgcccaacgtcctgcagggtgctggtgaataacatgagaaagaacttaaaatggcttgatgatctcaccatttagtgaccttggttgtcacactgctttccaagagccctttaaaggtaggaatgagagctgtttccagtatgcattccaataggaatgcagctttgctaaagttagagacataaactaaaaccctgtgaagtcctatagagcccttggacttatttcctagcaagcatttatcatccccaccatcctctacttcaggacacttgagcagaaacagtcaaggtttttgccgttttcatcctgctcttcaaaacactgtaagtagtggcgcaggtaagcacagccacaggtgaagaccgttttcagctgaggctgcacatcagaaccacagatcacaggggatggtgcgtgacaatcgtctcagttctcccagtaatgcccatgctagccccaggctcgatgccaggagggaagtgcattccttactgagggagggcatcaggcgtgggtcttccacggaaccccaataggaatcagcaacccccaagcagatattactcaaaggtggtattacatacaacagtagtcagactcagacttcaagcagcccaaagagtggaaccacaggcttgcacaattataaaatgtttttatttcaattacataataacacgttttcctcaaattttattgaggttttggtctttttgcattcaattctatcttgtaacagtaatatgaatccacataatttcataaaatgtcaacaacattcataaggtacattcctttgtgattttatattttacaattttaaatctaactttacaattattttaaaaaatttttttatatagaaaacagatattttcttcaggcagatcaaaacaagaattttccagtaagaatatactgggacataacaaatgaaaatatttataccaaaataccaaaagtgattcagctctttaaaatatcctactatagtctaattagtagcttgtacaagaacaagtaaccattttttactgctcttttgaatgatgattagaaattcaaacaaagtattttaaggttcaaaaactttttttttttttttttttttttttagagacagtgtctcactctgtctcccaggctagagtacagtgtgcaatcatagctcactgcagccttgaactcctggcctcaagcaatcctcccaccttggcttcccaatgtgctaggtttacaggcgtgaaaacattgtgttgtgtgtgtgtgtgtttttttttttttttttagacagagtttcgctcttgttgtccaggctggagtacaatggcttgatcttggctcactgcaatctctgcctcgcaggttcaagcgattctcctgcctcagcctctggagtggctgggattacaggcgcccaccatcacgcccggccaattttttgtatttttagtagagacagggtttcaccatgttggccaggctggcctcgaactcttgacctcaggtgatccacctgccttggcctcccaatgtactgagattacaggcatgagccaccacgcccggccaaaaacatttaaaaaatgactgtccctgctcaaatactgcagtaggaaatgtaatttgacatatatcacttccagaaaaaaactttaaatctttctataaaatgaatttgatacatcatcagcatgaagtgaagttaaaatctcttacaaagtaaattcaggtatatcaacaatgagatccaaaagtatcggttcaagatcaaagactcatatgaggtaaaggcaaataaagcccctcatgctttcagacatttacttgttatccttaaaatgattattgttctaaggtgcaaatcttatcattcagtgacctatttgctatttggctgtttatctcctttaaataaaataccatacaggttataatgtacattttaaaatcaaatatgaaagtacacatatgtgaacaagacattaatttaaatatcaattatattcataatacagaagtctaagaatgctatttggtcatttcaattagatgctgatatatttggtcaagaaaacccacattcctatcagcctaaggcaaatagtaaatgcctctatttttattaagtggactataaacagtagacattattgtttgatactactggaatgctctcaattagaacgtacactgataacaaatatgtctttctaatctgggtgataacctcaatgattacatggaaatctacaagtaacagtctataacttaaagcagtagagcacctggtaattgtcatacagtgcctctctatgaatttagaacattctacttacattggcagtggagagaaaagaccccttcacactgagacttcctgtgcaccgcgcctgccgcctgcctcagcttaggacatggtacagtcttctttgcttttgcccttctcattccctcctctggtatcttctctgctttctggattgaagtgccctggctctcttcctggtgccgacaagtcatcgttctctaggctattgctgtctaaagctttcctgacggtctgacttggatgttctgacatctcacacctctctgtactttctgcttcacaggcatcactaatgtcctgtgagggactttcatgttcgggcagggtgcagcgatctgcgtcttcgctctttggttctgcaggactgctttgagtggcaccatctattttagcattatcttttgcaacaccttcatctaattcttcaccaccagccctcgggcctgatgattgaacggtgtcatcctcaaaatctaatgtgtctccatcagctagtacctcctcagctgctgtttgtacatcatcaccttcttggtcaagttttccatccaacttaattttaggattctccggacaatcaacattttcactgctttctgctgcaattttctgttttggattttcagtcacctcgttttgggcttccactgctgactttctgtcagtagactttacctgctcttcttccttaatttcacttaaatctgtgttctgatacgttaactcttttttaacatctttaagggtttctacgggtactggggattttttcttcttgtttttctttttcttgttctttgtcttcttctgcgatgagtccaatgcctctccctgttggtcactcttttcttcatcgggctctttcatatctaagggttcattttgagtgtctactgtacttggacctgtcgcttcctgacagttgccctcagttcctgctggagaaccaggaacttctgtcttgattggtttctcgtcccttaatcctgtttcttcaccctcttcttcgttgtgatccctacctacttctgtactgtgcgctggaacctccttgggctcagctgcttcctggttggtgaattctttctctaaactatgccctgtgcttgtctctaactcttgggggacctctaccatacatttgtcatcatgataaactgtgtcatcactatgccctaaaggacacgaggccactgtgcctgcctgctcttcaacctgagtcactgctgcctctcccacattctctgtgtggttcccaccatctaagtcactccaacagttggatggctcaaggggagttctggtcctgtcatctggtgcacccatgacctcatttgactcaacctgtactgtgttttcagggagagaactgctctcaagaatttggctttgaacctgttcctcataggtagcacctgctaaggttcctaggaatggggcagtgtcttcagaggatttctggtcctcggtattctcaccagcagggaatacctctatgtccacacagtccttcactgtgtcctctgtgtgttgttctttctcagtattgtgcaagatttctcttttccccacattcgccacgatttcatttttcacctccacttcactggctcttcctagggtcccatcccctgtcgacttgagggcatttaactcttcttttgtcatcttggtaggaccttggtatccaacattattgagggtgtcggaagtctctccattggtagctatttctgaatttaggattattccatgtttctttaattcctctttcagcatgactacttcttctctaagatcatcccgttcactccttacggaatcaaagaactctttctgcctctctaatgcccctatctttttgtctttccactctattgtttcctgaagatcagaaatctccctgatagaactcgcctgtttctgctgtagctgtcggatttcctcgagcatttcctctctttgcttcagggcctccttgacttcagcaaactgaaattgcagtatactgtgggcgtgtttttccctttcaaattctttgtttttctcttcgtactgccgcctagattcagccagctgttcttcaagctccagcaacatatcttttagggtatcaacctggtacatgaagtttgtcttttcattgtctagctgagcattggaaaccatagccttcttatatttctcttcaacttctgctagagagtccttcatctctttcaatccctgcatgtatttgccttctacatcctgaatctggtcctttaactcattgagttccttgatttccctgatggatgcctcggtgtcgatggagatggaggtgtctccgctgcctctccgagaggaagtcccacccagagaggccagcgtggctgcagacaggcccggcatgttacgagaccccttctcagtaaaatctttttctggtctctcttctaccctgccagatcttctattcagggactgtgatccatacaattctccatcataaccatttgtcctcaggcttccacgactacccactgacatgcgctcgtcttcatcagaagccgatgtgtttcttctggatctacgagagtagcgctcactgtcttcctccttctgctgccgctccagctccttcatgcggatctcgcgagcctccgcgcgggccgcccgttttgcagcgagccgggcttccgccagcttctgcgcttccgggctcaaacagtcgatctcccggctttgagcggccgcggggctggtcatcctgccgggctcggcccgctccacccggcgggaaatgctcggggaccgcgccgggagcccctcgcgggccgggccagggggcgcgcgctctgtc

SEQ ID NO: 12147 - RNA, 5790 nt, Homo sapiens
  source 1..5790: mol_type = other RNA
ctgcagactcgacctcccaggctcaggtgtttctgcctcctaagtagctgggactacatgggactacatgcacatgccaccatgcctggctaattgtttgtatattttttttgtagagatgggctttcatcatgttgcccaggctgggcttgaactcctgggcttaagtgatctgcctgcctcggcctcccacgtgctgggattataggcatgagccaatgtgcccggcctcaaccatttcttgataagttaagggccttcacagtaatatcaattactgtgcttggctataaagtcattacactggagagcatataactgatgctcagaatgaaggctctgaaatcatcgagaaatggtttggctgctcagaactctttctttttccttctttcttgctcatggattttcagctgtccattccctactggagggctgggtccaactgcttgttcactggcacagtgccttccatgtacaaagtgatcaaacctgtctattaattaagcaaatgagtggtgaatcactgagacggctggatggctgagctgagggatgtgatgtgtgcccaacgtcctgcagggtgctggtgaataacatgagaaagaacttaaaatggcttgatgatctcaccatttagtgaccttggttgtcacactgctttccaagagccctttaaaggtaggaatgagagctgtttccagtatgcattccaataggaatgcagctttgctaaagttagagacataaactaaaaccctgtgaagtcctatagagcccttggacttatttcctagcaagcatttatcatccccaccatcctctacttcaggacacttgagcagaaacagtcaaggtttttgccgttttcatcctgctcttcaaaacactgtaagtagtggcgcaggtaagcacagccacaggtgaagaccgttttcagctgaggctgcacatcagaaccacagatcacaggggatggtgcgtgacaatcgtctcagttctcccagtaatgcccatgctagccccaggctcgatgccaggagggaagtgcattccttactgagggagggcatcaggcgtgggtcttccacggaaccccaataggaatcagcaacccccaagcagatattactcaaaggtggtattacatacaacagtagtcagactcagacttcaagcagcccaaagagtggaaccacaggcttgcacaattataaaatgtttttatttcaattacataataacacgttttcctcaaattttattgaggttttggtctttttgcattcaattctatcttgtaacagtaatatgaatccacataatttcataaaatgtcaacaacattcataaggtacattcctttgtgattttatattttacaattttaaatctaactttacaattattttaaaaaatttttttatatagaaaacagatattttcttcaggcagatcaaaacaagaattttccagtaagaatatactgggacataacaaatgaaaatatttataccaaaataccaaaagtgattcagctctttaaaatatcctactatagtctaattagtagcttgtacaagaacaagtaaccattttttactgctcttttgaatgatgattagaaattcaaacaaagtattttaaggttcaaaaactttttttttttttttttttttttttagagacagtgtctcactctgtctcccaggctagagtacagtgtgcaatcatagctcactgcagccttgaactcctggcctcaagcaatcctcccaccttggcttcccaatgtgctaggtttacaggcgtgaaaacattgtgttgtgtgtgtgtgtgtttttttttttttttttagacagagtttcgctcttgttgtccaggctggagtacaatggcttgatcttggctcactgcaatctctgcctcgcaggttcaagcgattctcctgcctcagcctctggagtggctgggattacaggcgcccaccatcacgcccggccaattttttgtatttttagtagagacagggtttcaccatgttggccaggctggcctcgaactcttgacctcaggtgatccacctgccttggcctcccaatgtactgagattacaggcatgagccaccacgcccggccaaaaacatttaaaaaatgactgtccctgctcaaatactgcagtaggaaatgtaatttgacatatatcacttccagaaaaaaactttaaatctttctataaaatgaatttgatacatcatcagcatgaagtgaagttaaaatctcttacaaagtaaattcaggtatatcaacaatgagatccaaaagtatcggttcaagatcaaagactcatatgaggtaaaggcaaataaagcccctcatgctttcagacatttacttgttatccttaaaatgattattgttctaaggtgcaaatcttatcattcagtgacctatttgctatttggctgtttatctcctttaaataaaataccatacaggttataatgtacattttaaaatcaaatatgaaagtacacatatgtgaacaagacattaatttaaatatcaattatattcataatacagaagtctaagaatgctatttggtcatttcaattagatgctgatatatttggtcaagaaaacccacattcctatcagcctaaggcaaatagtaaatgcctctatttttattaagtggactataaacagtagacattattgtttgatactactggaatgctctcaattagaacgtacactgataacaaatatgtctttctaatctgggtgataacctcaatgattacatggaaatctacaagtaacagtctataacttaaagcagtagagcacctggtaattgtcatacagtgcctctctatgaatttagaacattctacttacattggcagtggagagaaaagaccccttcacactgagacttcctgtgcaccgcgcctgccgcctgcctcagcttaggacatggtacagtcttctttgcttttgcccttctcattccctcctctggtatcttctctgctttctggattgaagtgccctggctctcttcctggtgccgacaagtcatcgttctctaggctattgctgtctaaagctttcctgacggtctgacttggatgttctgacatctcacacctctctgtactttctgcttcacaggcatcactaatgtcctgtgagggactttcatgttcgggcagggtgcagcgatctgcgtcttcgctctttggttctgcaggactgctttgagtggcaccatctattttagcattatcttttgcaacaccttcatctaattcttcaccaccagccctcgggcctgatgattgaacggtgtcatcctcaaaatctaatgtgtctccatcagctagtacctcctcagctgctgtttgtacatcatcaccttcttggtcaagttttccatccaacttaattttaggattctccggacaatcaacattttcactgctttctgctgcaattttctgttttggattttcagtcacctcgttttgggcttccactgctgactttctgtcagtagactttacctgctcttcttccttaatttcacttaaatctgtgttctgatacgttaactcttttttaacatctttaagggtttctacgggtactggggattttttcttcttgtttttctttttcttgttctttgtcttcttctgcgatgagtccaatgcctctccctgttggtcactcttttcttcatcgggctctttcatatctaagggttcattttgagtgtctactgtacttggacctgtcgcttcctgacagttgccctcagttcctgctggagaaccaggaacttctgtcttgattggtttctcgtcccttaatcctgtttcttcaccctcttcttcgttgtgatccctacctacttctgtactgtgcgctggaacctccttgggctcagctgcttcctggttggtgaattctttctctaaactatgccctgtgcttgtctctaactcttgggggacctctaccatacatttgtcatcatgataaactgtgtcatcactatgccctaaaggacacgaggccactgtgcctgcctgctcttcaacctgagtcactgctgcctctcccacattctctgtgtggttcccaccatctaagtcactccaacagttggatggctcaaggggagttctggtcctgtcatctggtgcacccatgacctcatttgactcaacctgtactgtgttttcagggagagaactgctctcaagaatttggctttgaacctgttcctcataggtagcacctgctaaggttcctaggaatggggcagtgtcttcagaggatttctggtcctcggtattctcaccagcagggaatacctctatgtccacacagtccttcactgtgtcctctgtgtgttgttctttctcagtattgtgcaagatttctcttttccccacattcgccacgatttcatttttcacctccacttcactggctcttcctagggtcccatcccctgtcgacttgagggcatttaactcttcttttgtcatcttggtaggaccttggtatccaacattattgagggtgtcggaagtctctccattggtagctatttctgaatttaggattattccatgtttctttaattcctctttcagcatgactacttcttctctaagatcatcccgttcactccttacggaatcaaagaactctttctgcctctctaatgcccctatctttttgtctttccactctattgtttcctgaagatcagaaatctccctgatagaactcgcctgtttctgctgtagctgtcggatttcctcgagcatttcctctctttgcttcagggcctccttgacttcagcaaactgaaattgcagtatactgtgggcgtgtttttccctttcaaattctttgtttttctcttcgtactgccgcctagattcagccagctgttcttcaagctccagcaacatatcttttagggtatcaacctggtacatgaagtttgtcttttcattgtctagctgagcattggaaaccatagccttcttatatttctcttcaacttctgctagagagtccttcatctctttcaatccctgcatgtatttgccttctacatcctgaatctggtcctttaactcattgagttccttgatttccctgatggatgcctcggtgtcgatggagatggaggtgtctccgctgcctctccgagaggaagtcccacccagagaggccagcgtggctgcagacaggcccggcatgttacgagaccccttctcagtaaaatctttttctggtctctcttctacctccttctgctgccgctccagctccttcatgcggatctcgcgagcctccgcgcgggccgcccgttttgcagcgagccgggcttccgccagcttctgcgcttccgggctcaaacagtcgatctcccggctttgagcggccgcggggctggtcatcctgccgggctcggcccgctccacccggcgggaaatgctcggggaccgcgccgggagcccctcgcgggccgggccagggggcgcgcgctctgtccgcggagacggagccactcgccgctaagtgaacgctcgcgcttccggggccaggagccagcccgccggggagcggctcgcggcgctgggctcgggcgcggccgacaggggcggggcgcaggtggccgcgggctgagtcgggctcggggtggaagggcgccggggaagcgggactcgggcgcctccgcccgtcccacggccc

SEQ ID NO: 12148 - RNA, 5571 nt, Homo sapiens
  source 1..5571: mol_type = other RNA
ctgcagactcgacctcccaggctcaggtgtttctgcctcctaagtagctgggactacatgggactacatgcacatgccaccatgcctggctaattgtttgtatattttttttgtagagatgggctttcatcatgttgcccaggctgggcttgaactcctgggcttaagtgatctgcctgcctcggcctcccacgtgctgggattataggcatgagccaatgtgcccggcctcaaccatttcttgataagttaagggccttcacagtaatatcaattactgtgcttggctataaagtcattacactggagagcatataactgatgctcagaatgaaggctctgaaatcatcgagaaatggtttggctgctcagaactctttctttttccttctttcttgctcatggattttcagctgtccattccctactggagggctgggtccaactgcttgttcactggcacagtgccttccatgtacaaagtgatcaaacctgtctattaattaagcaaatgagtggtgaatcactgagacggctggatggctgagctgagggatgtgatgtgtgcccaacgtcctgcagggtgctggtgaataacatgagaaagaacttaaaatggcttgatgatctcaccatttagtgaccttggttgtcacactgctttccaagagccctttaaaggtaggaatgagagctgtttccagtatgcattccaataggaatgcagctttgctaaagttagagacataaactaaaaccctgtgaagtcctatagagcccttggacttatttcctagcaagcatttatcatccccaccatcctctacttcaggacacttgagcagaaacagtcaaggtttttgccgttttcatcctgctcttcaaaacactgtaagtagtggcgcaggtaagcacagccacaggtgaagaccgttttcagctgaggctgcacatcagaaccacagatcacaggggatggtgcgtgacaatcgtctcagttctcccagtaatgcccatgctagccccaggctcgatgccaggagggaagtgcattccttactgagggagggcatcaggcgtgggtcttccacggaaccccaataggaatcagcaacccccaagcagatattactcaaaggtggtattacatacaacagtagtcagactcagacttcaagcagcccaaagagtggaaccacaggcttgcacaattataaaatgtttttatttcaattacataataacacgttttcctcaaattttattgaggttttggtctttttgcattcaattctatcttgtaacagtaatatgaatccacataatttcataaaatgtcaacaacattcataaggtacattcctttgtgattttatattttacaattttaaatctaactttacaattattttaaaaaatttttttatatagaaaacagatattttcttcaggcagatcaaaacaagaattttccagtaagaatatactgggacataacaaatgaaaatatttataccaaaataccaaaagtgattcagctctttaaaatatcctactatagtctaattagtagcttgtacaagaacaagtaaccattttttactgctcttttgaatgatgattagaaattcaaacaaagtattttaaggttcaaaaactttttttttttttttttttttttttagagacagtgtctcactctgtctcccaggctagagtacagtgtgcaatcatagctcactgcagccttgaactcctggcctcaagcaatcctcccaccttggcttcccaatgtgctaggtttacaggcgtgaaaacattgtgttgtgtgtgtgtgtgtttttttttttttttttagacagagtttcgctcttgttgtccaggctggagtacaatggcttgatcttggctcactgcaatctctgcctcgcaggttcaagcgattctcctgcctcagcctctggagtggctgggattacaggcgcccaccatcacgcccggccaattttttgtatttttagtagagacagggtttcaccatgttggccaggctggcctcgaactcttgacctcaggtgatccacctgccttggcctcccaatgtactgagattacaggcatgagccaccacgcccggccaaaaacatttaaaaaatgactgtccctgctcaaatactgcagtaggaaatgtaatttgacatatatcacttccagaaaaaaactttaaatctttctataaaatgaatttgatacatcatcagcatgaagtgaagttaaaatctcttacaaagtaaattcaggtatatcaacaatgagatccaaaagtatcggttcaagatcaaagactcatatgaggtaaaggcaaataaagcccctcatgctttcagacatttacttgttatccttaaaatgattattgttctaaggtgcaaatcttatcattcagtgacctatttgctatttggctgtttatctcctttaaataaaataccatacaggttataatgtacattttaaaatcaaatatgaaagtacacatatgtgaacaagacattaatttaaatatcaattatattcataatacagaagtctaagaatgctatttggtcatttcaattagatgctgatatatttggtcaagaaaacccacattcctatcagcctaaggcaaatagtaaatgcctctatttttattaagtggactataaacagtagacattattgtttgatactactggaatgctctcaattagaacgtacactgataacaaatatgtctttctaatctgggtgataacctcaatgattacatggaaatctacaagtaacagtctataacttaaagcagtagagcacctggtaattgtcatacagtgcctctctatgaatttagaacattctacttacattggcagtggagagaaaagaccccttcacactgagacttcctgtgcaccgcgcctgccgcctgcctcagcttaggacatggtacagtcttctttgcttttgcccttctcattccctcctctggtatcttctctgctttctggattgaagtgccctggctctcttcctggtgccgacaagtcatcgttctctaggctattgctgtctaaagctttcctgacggtctgacttggatgttctgacatctcacacctctctgtactttctgcttcacaggcatcactaatgtcctgtgagggactttcatgttcgggcagggtgcagcgatctgcgtcttcgctctttggttctgcaggactgctttgagtggcaccatctattttagcattatcttttgcaacaccttcatctaattcttcaccaccagccctcgggcctgatgattgaacggtgtcatcctcaaaatctaatgtgtctccatcagctagtacctcctcagctgctgtttgtacatcatcaccttcttggtcaagttttccatccaacttaattttaggattctccggacaatcaacattttcactgctttctgctgcaattttctgttttggattttcagtcacctcgttttgggcttccactgctgactttctgtcagtagactttacctgctcttcttccttaatttcacttaaatctgtgttctgatacgttaactcttttttaacatctttaagggtttctacgggtactggggattttttcttcttgtttttctttttcttgttctttgtcttcttctgcgatgagtccaatgcctctccctgttggtcactcttttcttcatcgggctctttcatatctaagggttcattttgagtgtctactgtacttggacctgtcgcttcctgacagttgccctcagttcctgctggagaaccaggaacttctgtcttgattggtttctcgtcccttaatcctgtttcttcaccctcttcttcgttgtgatccctacctacttctgtactgtgcgctggaacctccttgggctcagctgcttcctggttggtgaattctttctctaaactatgccctgtgcttgtctctaactcttgggggacctctaccatacatttgtcatcatgataaactgtgtcatcactatgccctaaaggacacgaggccactgtgcctgcctgctcttcaacctgagtcactgctgcctctcccacattctctgtgtggttcccaccatctaagtcactccaacagttggatggctcaaggggagttctggtcctgtcatctggtgcacccatgacctcatttgactcaacctgtactgtgttttcagggagagaactgctctcaagaatttggctttgaacctgttcctcataggtagcacctgctaaggttcctaggaatggggcagtgtcttcagaggatttctggtcctcggtattctcaccagcagggaatacctctatgtccacacagtccttcactgtgtcctctgtgtgttgttctttctcagtattgtgcaagatttctcttttccccacattcgccacgatttcatttttcacctccacttcactggctcttcctagggtcccatcccctgtcgacttgagggcatttaactcttcttttgtcatcttggtaggaccttggtatccaacattattgagggtgtcggaagtctctccattggtagctatttctgaatttaggattattccatgtttctttaattcctctttcagcatgactacttcttctctaagatcatcccgttcactccttacggaatcaaagaactctttctgcctctctaatgcccctatctttttgtctttccactctattgtttcctgaagatcagaaatctccctgatagaactcgcctgtttctgctgtagctgtcggatttcctcgagcatttcctctctttgcttcagggcctccttgacttcagcaaactgaaattgcagtatactgtgggcgtgtttttccctttcaaattctttgtttttctcttcgtactgccgcctagattcagccagctgttcttcaagctccagcaacatatcttttagggtatcaacctggtacatgaagtttgtcttttcattgtctagctgagcattggaaaccatagccttcttatatttctcttcaacttctgctagagagtccttcatctctttcaatccctgcatgtatttgccttctacatcctgaatctggtcctttaactcattgagttccttgatttccctgatggatgcctcggtgtcgatggagatggaggtgtctccgctgcctctccgagaggaagtcccacccagagaggccagcgtggctgcagacaggcccggcatgttacgagaccccttctcagtaaaatctttttctggtctctcttctacctccttctgctgccgctccagctccttcatgcggatctcgcgagcctccgcgcgggccgcccgttttgcagcgagccgggcttccgcctcccgcgcgatctggttgagcgcgtcgtcctccgccgtgagccgctcccggttggggagccgcttgcgccccgatccctgggtgcccatgtccatcgaccgcgtcgcccgcagctgccgcggggcccgttgctccagccgc

SEQ ID NO: 12149 - RNA, 6035 nt, Homo sapiens
  source 1..6035: mol_type = other RNA
ctgcagactcgacctcccaggctcaggtgtttctgcctcctaagtagctgggactacatgggactacatgcacatgccaccatgcctggctaattgtttgtatattttttttgtagagatgggctttcatcatgttgcccaggctgggcttgaactcctgggcttaagtgatctgcctgcctcggcctcccacgtgctgggattataggcatgagccaatgtgcccggcctcaaccatttcttgataagttaagggccttcacagtaatatcaattactgtgcttggctataaagtcattacactggagagcatataactgatgctcagaatgaaggctctgaaatcatcgagaaatggtttggctgctcagaactctttctttttccttctttcttgctcatggattttcagctgtccattccctactggagggctgggtccaactgcttgttcactggcacagtgccttccatgtacaaagtgatcaaacctgtctattaattaagcaaatgagtggtgaatcactgagacggctggatggctgagctgagggatgtgatgtgtgcccaacgtcctgcagggtgctggtgaataacatgagaaagaacttaaaatggcttgatgatctcaccatttagtgaccttggttgtcacactgctttccaagagccctttaaaggtaggaatgagagctgtttccagtatgcattccaataggaatgcagctttgctaaagttagagacataaactaaaaccctgtgaagtcctatagagcccttggacttatttcctagcaagcatttatcatccccaccatcctctacttcaggacacttgagcagaaacagtcaaggtttttgccgttttcatcctgctcttcaaaacactgtaagtagtggcgcaggtaagcacagccacaggtgaagaccgttttcagctgaggctgcacatcagaaccacagatcacaggggatggtgcgtgacaatcgtctcagttctcccagtaatgcccatgctagccccaggctcgatgccaggagggaagtgcattccttactgagggagggcatcaggcgtgggtcttccacggaaccccaataggaatcagcaacccccaagcagatattactcaaaggtggtattacatacaacagtagtcagactcagacttcaagcagcccaaagagtggaaccacaggcttgcacaattataaaatgtttttatttcaattacataataacacgttttcctcaaattttattgaggttttggtctttttgcattcaattctatcttgtaacagtaatatgaatccacataatttcataaaatgtcaacaacattcataaggtacattcctttgtgattttatattttacaattttaaatctaactttacaattattttaaaaaatttttttatatagaaaacagatattttcttcaggcagatcaaaacaagaattttccagtaagaatatactgggacataacaaatgaaaatatttataccaaaataccaaaagtgattcagctctttaaaatatcctactatagtctaattagtagcttgtacaagaacaagtaaccattttttactgctcttttgaatgatgattagaaattcaaacaaagtattttaaggttcaaaaactttttttttttttttttttttttttagagacagtgtctcactctgtctcccaggctagagtacagtgtgcaatcatagctcactgcagccttgaactcctggcctcaagcaatcctcccaccttggcttcccaatgtgctaggtttacaggcgtgaaaacattgtgttgtgtgtgtgtgtgtttttttttttttttttagacagagtttcgctcttgttgtccaggctggagtacaatggcttgatcttggctcactgcaatctctgcctcgcaggttcaagcgattctcctgcctcagcctctggagtggctgggattacaggcgcccaccatcacgcccggccaattttttgtatttttagtagagacagggtttcaccatgttggccaggctggcctcgaactcttgacctcaggtgatccacctgccttggcctcccaatgtactgagattacaggcatgagccaccacgcccggccaaaaacatttaaaaaatgactgtccctgctcaaatactgcagtaggaaatgtaatttgacatatatcacttccagaaaaaaactttaaatctttctataaaatgaatttgatacatcatcagcatgaagtgaagttaaaatctcttacaaagtaaattcaggtatatcaacaatgagatccaaaagtatcggttcaagatcaaagactcatatgaggtaaaggcaaataaagcccctcatgctttcagacatttacttgttatccttaaaatgattattgttctaaggtgcaaatcttatcattcagtgacctatttgctatttggctgtttatctcctttaaataaaataccatacaggttataatgtacattttaaaatcaaatatgaaagtacacatatgtgaacaagacattaatttaaatatcaattatattcataatacagaagtctaagaatgctatttggtcatttcaattagatgctgatatatttggtcaagaaaacccacattcctatcagcctaaggcaaatagtaaatgcctctatttttattaagtggactataaacagtagacattattgtttgatactactggaatgctctcaattagaacgtacactgataacaaatatgtctttctaatctgggtgataacctcaatgattacatggaaatctacaagtaacagtctataacttaaagcagtagagcacctggtaattgtcatacagtgcctctctatgaatttagaacattctacttacattggcagtggagagaaaagaccccttcacactgagacttcctgtgcaccgcgcctgccgcctgcctcagcttaggacatggtacagtcttctttgcttttgcccttctcattccctcctctggtatcttctctgctttctggattgaagtgccctggctctcttcctggtgccgacaagtcatcgttctctaggctattgctgtctaaagctttcctgacggtctgacttggatgttctgacatctcacacctctctgtactttctgcttcacaggcatcactaatgtcctgtgagggactttcatgttcgggcagggtgcagcgatctgcgtcttcgctctttggttctgcaggactgctttgagtggcaccatctattttagcattatcttttgcaacaccttcatctaattcttcaccaccagccctcgggcctgatgattgaacggtgtcatcctcaaaatctaatgtgtctccatcagctagtacctcctcagctgctgtttgtacatcatcaccttcttggtcaagttttccatccaacttaattttaggattctccggacaatcaacattttcactgctttctgctgcaattttctgttttggattttcagtcacctcgttttgggcttccactgctgactttctgtcagtagactttacctgctcttcttccttaatttcacttaaatctgtgttctgatacgttaactcttttttaacatctttaagggtttctacgggtactggggattttttcttcttgtttttctttttcttgttctttgtcttcttctgcgatgagtccaatgcctctccctgttggtcactcttttcttcatcgggctctttcatatctaagggttcattttgagtgtctactgtacttggacctgtcgcttcctgacagttgccctcagttcctgctggagaaccaggaacttctgtcttgattggtttctcgtcccttaatcctgtttcttcaccctcttcttcgttgtgatccctacctacttctgtactgtgcgctggaacctccttgggctcagctgcttcctggttggtgaattctttctctaaactatgccctgtgcttgtctctaactcttgggggacctctaccatacatttgtcatcatgataaactgtgtcatcactatgccctaaaggacacgaggccactgtgcctgcctgctcttcaacctgagtcactgctgcctctcccacattctctgtgtggttcccaccatctaagtcactccaacagttggatggctcaaggggagttctggtcctgtcatctggtgcacccatgacctcatttgactcaacctgtactgtgttttcagggagagaactgctctcaagaatttggctttgaacctgttcctcataggtagcacctgctaaggttcctaggaatggggcagtgtcttcagaggatttctggtcctcggtattctcaccagcagggaatacctctatgtccacacagtccttcactgtgtcctctgtgtgttgttctttctcagtattgtgcaagatttctcttttccccacattcgccacgatttcatttttcacctccacttcactggctcttcctagggtcccatcccctgtcgacttgagggcatttaactcttcttttgtcatcttggtaggaccttggtatccaacattattgagggtgtcggaagtctctccattggtagctatttctgaatttaggattattccatgtttctttaattcctctttcagcatgactacttcttctctaagatcatcccgttcactccttacggaatcaaagaactctttctgcctctctaatgcccctatctttttgtctttccactctattgtttcctgaagatcagaaatctccctgatagaactcgcctgtttctgctgtagctgtcggatttcctcgagcatttcctctctttgcttcagggcctccttgacttcagcaaactgaaattgcagtatactgtgggcgtgtttttccctttcaaattctttgtttttctcttcgtactgccgcctagattcagccagctgttcttcaagctccagcaacatatcttttagggtatcaacctggtacatgaagtttgtcttttcattgtctagctgagcattggaaaccatagccttcttatatttctcttcaacttctgctagagagtccttgatttccctgatggatgcctcggtgtcgatggagatggaggtgtctccgctgcctctccgagaggaagtcccacccagagaggccagcgtggctgcagacaggcccggcatgttacgagaccccttctcagtaaaatctttttctggtctctcttctaccacagggctggcccgggccgagctggccctggaggaggcgcgggagctggagttgaggtggccgctgtactccgagggagcacgggagccggaggtgctgccccgtcgggtcccaccgaagctgccttcatccaacacagacgcccggtaactccccgaaggccgggcagcgctgtacagacaggagggcaacttctcctccctggatgatgacaaagtagagaatctgctgtcaccgctgtagctggaattcctgccagatcttctattcagggactgtgatccatacaattctccatcataaccatttgtccaggcgtaaggacccccatactccaagtcaggctgcgacctcaggcttccacgactacccactgacatgcgctcgtcttcatcagaagccgatgtgtttcttctggatctacgagagtagcgctcactgtcttccatccactgctcgatgtcaccccattttgtatccagcccataatatttcttttggacctgatagatctccttctgctgccgctccagctccttcatgcggatctcgcgagcctccgcgcgggccgcccgttttgcagcgagccgggcttccgcctcccgcgcgatctggttgagcgcgtcgtcctccgccgtgagccgctcccggttggggagccgcttgcgccccgatccctgggtgcccatgtccatcgaccgcgtcgcccgcagctgccgcggggcccgttgctccagccgctcgcgccgccccggcccggcccc

SEQ ID NO: 12150 - RNA, 5864 nt, Homo sapiens
  source 1..5864: mol_type = other RNA
ctgcagactcgacctcccaggctcaggtgtttctgcctcctaagtagctgggactacatgggactacatgcacatgccaccatgcctggctaattgtttgtatattttttttgtagagatgggctttcatcatgttgcccaggctgggcttgaactcctgggcttaagtgatctgcctgcctcggcctcccacgtgctgggattataggcatgagccaatgtgcccggcctcaaccatttcttgataagttaagggccttcacagtaatatcaattactgtgcttggctataaagtcattacactggagagcatataactgatgctcagaatgaaggctctgaaatcatcgagaaatggtttggctgctcagaactctttctttttccttctttcttgctcatggattttcagctgtccattccctactggagggctgggtccaactgcttgttcactggcacagtgccttccatgtacaaagtgatcaaacctgtctattaattaagcaaatgagtggtgaatcactgagacggctggatggctgagctgagggatgtgatgtgtgcccaacgtcctgcagggtgctggtgaataacatgagaaagaacttaaaatggcttgatgatctcaccatttagtgaccttggttgtcacactgctttccaagagccctttaaaggtaggaatgagagctgtttccagtatgcattccaataggaatgcagctttgctaaagttagagacataaactaaaaccctgtgaagtcctatagagcccttggacttatttcctagcaagcatttatcatccccaccatcctctacttcaggacacttgagcagaaacagtcaaggtttttgccgttttcatcctgctcttcaaaacactgtaagtagtggcgcaggtaagcacagccacaggtgaagaccgttttcagctgaggctgcacatcagaaccacagatcacaggggatggtgcgtgacaatcgtctcagttctcccagtaatgcccatgctagccccaggctcgatgccaggagggaagtgcattccttactgagggagggcatcaggcgtgggtcttccacggaaccccaataggaatcagcaacccccaagcagatattactcaaaggtggtattacatacaacagtagtcagactcagacttcaagcagcccaaagagtggaaccacaggcttgcacaattataaaatgtttttatttcaattacataataacacgttttcctcaaattttattgaggttttggtctttttgcattcaattctatcttgtaacagtaatatgaatccacataatttcataaaatgtcaacaacattcataaggtacattcctttgtgattttatattttacaattttaaatctaactttacaattattttaaaaaatttttttatatagaaaacagatattttcttcaggcagatcaaaacaagaattttccagtaagaatatactgggacataacaaatgaaaatatttataccaaaataccaaaagtgattcagctctttaaaatatcctactatagtctaattagtagcttgtacaagaacaagtaaccattttttactgctcttttgaatgatgattagaaattcaaacaaagtattttaaggttcaaaaactttttttttttttttttttttttttagagacagtgtctcactctgtctcccaggctagagtacagtgtgcaatcatagctcactgcagccttgaactcctggcctcaagcaatcctcccaccttggcttcccaatgtgctaggtttacaggcgtgaaaacattgtgttgtgtgtgtgtgtgtttttttttttttttttagacagagtttcgctcttgttgtccaggctggagtacaatggcttgatcttggctcactgcaatctctgcctcgcaggttcaagcgattctcctgcctcagcctctggagtggctgggattacaggcgcccaccatcacgcccggccaattttttgtatttttagtagagacagggtttcaccatgttggccaggctggcctcgaactcttgacctcaggtgatccacctgccttggcctcccaatgtactgagattacaggcatgagccaccacgcccggccaaaaacatttaaaaaatgactgtccctgctcaaatactgcagtaggaaatgtaatttgacatatatcacttccagaaaaaaactttaaatctttctataaaatgaatttgatacatcatcagcatgaagtgaagttaaaatctcttacaaagtaaattcaggtatatcaacaatgagatccaaaagtatcggttcaagatcaaagactcatatgaggtaaaggcaaataaagcccctcatgctttcagacatttacttgttatccttaaaatgattattgttctaaggtgcaaatcttatcattcagtgacctatttgctatttggctgtttatctcctttaaataaaataccatacaggttataatgtacattttaaaatcaaatatgaaagtacacatatgtgaacaagacattaatttaaatatcaattatattcataatacagaagtctaagaatgctatttggtcatttcaattagatgctgatatatttggtcaagaaaacccacattcctatcagcctaaggcaaatagtaaatgcctctatttttattaagtggactataaacagtagacattattgtttgatactactggaatgctctcaattagaacgtacactgataacaaatatgtctttctaatctgggtgataacctcaatgattacatggaaatctacaagtaacagtctataacttaaagcagtagagcacctggtaattgtcatacagtgcctctctatgaatttagaacattctacttacattggcagtggagagaaaagaccccttcacactgagacttcctgtgcaccgcgcctgccgcctgcctcagcttaggacatggtacagtcttctttgcttttgcccttctcattccctcctctggtatcttctctgctttctggattgaagtgccctggctctcttcctggtgccgacaagtcatcgttctctaggctattgctgtctaaagctttcctgacggtctgacttggatgttctgacatctcacacctctctgtactttctgcttcacaggcatcactaatgtcctgtgagggactttcatgttcgggcagggtgcagcgatctgcgtcttcgctctttggttctgcaggactgctttgagtggcaccatctattttagcattatcttttgcaacaccttcatctaattcttcaccaccagccctcgggcctgatgattgaacggtgtcatcctcaaaatctaatgtgtctccatcagctagtacctcctcagctgctgtttgtacatcatcaccttcttggtcaagttttccatccaacttaattttaggattctccggacaatcaacattttcactgctttctgctgcaattttctgttttggattttcagtcacctcgttttgggcttccactgctgactttctgtcagtagactttacctgctcttcttccttaatttcacttaaatctgtgttctgatacgttaactcttttttaacatctttaagggtttctacgggtactggggattttttcttcttgtttttctttttcttgttctttgtcttcttctgcgatgagtccaatgcctctccctgttggtcactcttttcttcatcgggctctttcatatctaagggttcattttgagtgtctactgtacttggacctgtcgcttcctgacagttgccctcagttcctgctggagaaccaggaacttctgtcttgattggtttctcgtcccttaatcctgtttcttcaccctcttcttcgttgtgatccctacctacttctgtactgtgcgctggaacctccttgggctcagctgcttcctggttggtgaattctttctctaaactatgccctgtgcttgtctctaactcttgggggacctctaccatacatttgtcatcatgataaactgtgtcatcactatgccctaaaggacacgaggccactgtgcctgcctgctcttcaacctgagtcactgctgcctctcccacattctctgtgtggttcccaccatctaagtcactccaacagttggatggctcaaggggagttctggtcctgtcatctggtgcacccatgacctcatttgactcaacctgtactgtgttttcagggagagaactgctctcaagaatttggctttgaacctgttcctcataggtagcacctgctaaggttcctaggaatggggcagtgtcttcagaggatttctggtcctcggtattctcaccagcagggaatacctctatgtccacacagtccttcactgtgtcctctgtgtgttgttctttctcagtattgtgcaagatttctcttttccccacattcgccacgatttcatttttcacctccacttcactggctcttcctagggtcccatcccctgtcgacttgagggcatttaactcttcttttgtcatcttggtaggaccttggtatccaacattattgagggtgtcggaagtctctccattggtagctatttctgaatttaggattattccatgtttctttaattcctctttcagcatgactacttcttctctaagatcatcccgttcactccttacggaatcaaagaactctttctgcctctctaatgcccctatctttttgtctttccactctattgtttcctgaagatcagaaatctccctgatagaactcgcctgtttctgctgtagctgtcggatttcctcgagcatttcctctctttgcttcagggcctccttgacttcagcaaactgaaattgcagtatactgtgggcgtgtttttccctttcaaattctttgtttttctcttcgtactgccgcctagattcagccagctgttcttcaagctccagcaacatatcttttagggtatcaacctggtacatgaagtttgtcttttcattgtctagctgagcattggaaaccatagccttcttatatttctcttcaacttctgctagagagtccttgatttccctgatggatgcctcggtgtcgatggagatggaggtgtctccgctgcctctccgagaggaagtcccacccagagaggccagcgtggctgcagacaggcccggcatgttacgagaccccttctcagtaaaatctttttctggtctctcttctaccctcaggcttccacgactacccactgacatgcgctcgtcttcatcagaagccgatgtgtttcttctggatctacgagagtagcgctcactgtcttccatccactgctcgatgtcaccccattttgtatccagcccataatatttcttttggacctgatagatctccttctgctgccgctccagctccttcatgcggatctcgcgagcctccgcgcgggccgcccgttttgcagcgagccgggcttccgccagcttctgcgcttccgggctcaaacagtcgatctcccggctttgagcggccgcggggctggtcatcctgccgggctcggcccgctccacccggcgggaaatgctcggggaccgcgccgggagcccctcgcgggccgggccagggggcgcgcgctctgtccgcggagacggagccactcgccgctaagtgaacgctcgcgcttccggggccaggagccagcccgccggggagcggctcgcggcgctgggctcgggcgcggccgacaggggcggggcgcaggtggccgcgggctgagtcgggctcggggtggaagggcgccggggaagcgggactcgggcgcctcc

SEQ ID NO: 12151 - RNA, 5684 nt, Homo sapiens
  source 1..5684: mol_type = other RNA
ctgcagactcgacctcccaggctcaggtgtttctgcctcctaagtagctgggactacatgggactacatgcacatgccaccatgcctggctaattgtttgtatattttttttgtagagatgggctttcatcatgttgcccaggctgggcttgaactcctgggcttaagtgatctgcctgcctcggcctcccacgtgctgggattataggcatgagccaatgtgcccggcctcaaccatttcttgataagttaagggccttcacagtaatatcaattactgtgcttggctataaagtcattacactggagagcatataactgatgctcagaatgaaggctctgaaatcatcgagaaatggtttggctgctcagaactctttctttttccttctttcttgctcatggattttcagctgtccattccctactggagggctgggtccaactgcttgttcactggcacagtgccttccatgtacaaagtgatcaaacctgtctattaattaagcaaatgagtggtgaatcactgagacggctggatggctgagctgagggatgtgatgtgtgcccaacgtcctgcagggtgctggtgaataacatgagaaagaacttaaaatggcttgatgatctcaccatttagtgaccttggttgtcacactgctttccaagagccctttaaaggtaggaatgagagctgtttccagtatgcattccaataggaatgcagctttgctaaagttagagacataaactaaaaccctgtgaagtcctatagagcccttggacttatttcctagcaagcatttatcatccccaccatcctctacttcaggacacttgagcagaaacagtcaaggtttttgccgttttcatcctgctcttcaaaacactgtaagtagtggcgcaggtaagcacagccacaggtgaagaccgttttcagctgaggctgcacatcagaaccacagatcacaggggatggtgcgtgacaatcgtctcagttctcccagtaatgcccatgctagccccaggctcgatgccaggagggaagtgcattccttactgagggagggcatcaggcgtgggtcttccacggaaccccaataggaatcagcaacccccaagcagatattactcaaaggtggtattacatacaacagtagtcagactcagacttcaagcagcccaaagagtggaaccacaggcttgcacaattataaaatgtttttatttcaattacataataacacgttttcctcaaattttattgaggttttggtctttttgcattcaattctatcttgtaacagtaatatgaatccacataatttcataaaatgtcaacaacattcataaggtacattcctttgtgattttatattttacaattttaaatctaactttacaattattttaaaaaatttttttatatagaaaacagatattttcttcaggcagatcaaaacaagaattttccagtaagaatatactgggacataacaaatgaaaatatttataccaaaataccaaaagtgattcagctctttaaaatatcctactatagtctaattagtagcttgtacaagaacaagtaaccattttttactgctcttttgaatgatgattagaaattcaaacaaagtattttaaggttcaaaaactttttttttttttttttttttttttagagacagtgtctcactctgtctcccaggctagagtacagtgtgcaatcatagctcactgcagccttgaactcctggcctcaagcaatcctcccaccttggcttcccaatgtgctaggtttacaggcgtgaaaacattgtgttgtgtgtgtgtgtgtttttttttttttttttagacagagtttcgctcttgttgtccaggctggagtacaatggcttgatcttggctcactgcaatctctgcctcgcaggttcaagcgattctcctgcctcagcctctggagtggctgggattacaggcgcccaccatcacgcccggccaattttttgtatttttagtagagacagggtttcaccatgttggccaggctggcctcgaactcttgacctcaggtgatccacctgccttggcctcccaatgtactgagattacaggcatgagccaccacgcccggccaaaaacatttaaaaaatgactgtccctgctcaaatactgcagtaggaaatgtaatttgacatatatcacttccagaaaaaaactttaaatctttctataaaatgaatttgatacatcatcagcatgaagtgaagttaaaatctcttacaaagtaaattcaggtatatcaacaatgagatccaaaagtatcggttcaagatcaaagactcatatgaggtaaaggcaaataaagcccctcatgctttcagacatttacttgttatccttaaaatgattattgttctaaggtgcaaatcttatcattcagtgacctatttgctatttggctgtttatctcctttaaataaaataccatacaggttataatgtacattttaaaatcaaatatgaaagtacacatatgtgaacaagacattaatttaaatatcaattatattcataatacagaagtctaagaatgctatttggtcatttcaattagatgctgatatatttggtcaagaaaacccacattcctatcagcctaaggcaaatagtaaatgcctctatttttattaagtggactataaacagtagacattattgtttgatactactggaatgctctcaattagaacgtacactgataacaaatatgtctttctaatctgggtgataacctcaatgattacatggaaatctacaagtaacagtctataacttaaagcagtagagcacctggtaattgtcatacagtgcctctctatgaatttagaacattctacttacattggcagtggagagaaaagaccccttcacactgagacttcctgtgcaccgcgcctgccgcctgcctcagcttaggacatggtacagtcttctttgcttttgcccttctcattccctcctctggtatcttctctgctttctggattgaagtgccctggctctcttcctggtgccgacaagtcatcgttctctaggctattgctgtctaaagctttcctgacggtctgacttggatgttctgacatctcacacctctctgtactttctgcttcacaggcatcactaatgtcctgtgagggactttcatgttcgggcagggtgcagcgatctgcgtcttcgctctttggttctgcaggactgctttgagtggcaccatctattttagcattatcttttgcaacaccttcatctaattcttcaccaccagccctcgggcctgatgattgaacggtgtcatcctcaaaatctaatgtgtctccatcagctagtacctcctcagctgctgtttgtacatcatcaccttcttggtcaagttttccatccaacttaattttaggattctccggacaatcaacattttcactgctttctgctgcaattttctgttttggattttcagtcacctcgttttgggcttccactgctgactttctgtcagtagactttacctgctcttcttccttaatttcacttaaatctgtgttctgatacgttaactcttttttaacatctttaagggtttctacgggtactggggattttttcttcttgtttttctttttcttgttctttgtcttcttctgcgatgagtccaatgcctctccctgttggtcactcttttcttcatcgggctctttcatatctaagggttcattttgagtgtctactgtacttggacctgtcgcttcctgacagttgccctcagttcctgctggagaaccaggaacttctgtcttgattggtttctcgtcccttaatcctgtttcttcaccctcttcttcgttgtgatccctacctacttctgtactgtgcgctggaacctccttgggctcagctgcttcctggttggtgaattctttctctaaactatgccctgtgcttgtctctaactcttgggggacctctaccatacatttgtcatcatgataaactgtgtcatcactatgccctaaaggacacgaggccactgtgcctgcctgctcttcaacctgagtcactgctgcctctcccacattctctgtgtggttcccaccatctaagtcactccaacagttggatggctcaaggggagttctggtcctgtcatctggtgcacccatgacctcatttgactcaacctgtactgtgttttcagggagagaactgctctcaagaatttggctttgaacctgttcctcataggtagcacctgctaaggttcctaggaatggggcagtgtcttcagaggatttctggtcctcggtattctcaccagcagggaatacctctatgtccacacagtccttcactgtgtcctctgtgtgttgttctttctcagtattgtgcaagatttctcttttccccacattcgccacgatttcatttttcacctccacttcactggctcttcctagggtcccatcccctgtcgacttgagggcatttaactcttcttttgtcatcttggtaggaccttggtatccaacattattgagggtgtcggaagtctctccattggtagctatttctgaatttaggattattccatgtttctttaattcctctttcagcatgactacttcttctctaagatcatcccgttcactccttacggaatcaaagaactctttctgcctctctaatgcccctatctttttgtctttccactctattgtttcctgaagatcagaaatctccctgatagaactcgcctgtttctgctgtagctgtcggatttcctcgagcatttcctctctttgcttcagggcctccttgacttcagcaaactgaaattgcagtatactgtgggcgtgtttttccctttcaaattctttgtttttctcttcgtactgccgcctagattcagccagctgttcttcaagctccagcaacatatcttttagggtatcaacctggtacatgaagtttgtcttttcattgtctagctgagcattggaaaccatagccttcttatatttctcttcaacttctgctagagagtccttgatttccctgatggatgcctcggtgtcgatggagatggaggtgtctccgctgcctctccgagaggaagtcccacccagagaggccagcgtggctgcagacaggcccggcatgttacgagaccccttctcagtaaaatctttttctggtctctcttctaccctcaggcttccacgactacccactgacatgcgctcgtcttcatcagaagccgatgtgtttcttctggatctacgagagtagcgctcactgtcttccatccactgctcgatgtcaccccattttgtatccagcccataatatttcttttggacctgatagatctccttctgctgccgctccagctccttcatgcggatctcgcgagcctccgcgcgggccgcccgttttgcagcgagccgggcttccgcctcccgcgcgatctggttgagcgcgtcgtcctccgccgtgagccgctcccggttggggagccgcttgcgccccgatccctgggtgcccatgtccatcgaccgcgtcgcccgcagctgccgcggggcccgttgctccagccgctcgcgccgccccggcccggcccc

SEQ ID NO: 12152 - RNA, 5613 nt, Homo sapiens
  source 1..5613: mol_type = other RNA
ctgcagactcgacctcccaggctcaggtgtttctgcctcctaagtagctgggactacatgggactacatgcacatgccaccatgcctggctaattgtttgtatattttttttgtagagatgggctttcatcatgttgcccaggctgggcttgaactcctgggcttaagtgatctgcctgcctcggcctcccacgtgctgggattataggcatgagccaatgtgcccggcctcaaccatttcttgataagttaagggccttcacagtaatatcaattactgtgcttggctataaagtcattacactggagagcatataactgatgctcagaatgaaggctctgaaatcatcgagaaatggtttggctgctcagaactctttctttttccttctttcttgctcatggattttcagctgtccattccctactggagggctgggtccaactgcttgttcactggcacagtgccttccatgtacaaagtgatcaaacctgtctattaattaagcaaatgagtggtgaatcactgagacggctggatggctgagctgagggatgtgatgtgtgcccaacgtcctgcagggtgctggtgaataacatgagaaagaacttaaaatggcttgatgatctcaccatttagtgaccttggttgtcacactgctttccaagagccctttaaaggtaggaatgagagctgtttccagtatgcattccaataggaatgcagctttgctaaagttagagacataaactaaaaccctgtgaagtcctatagagcccttggacttatttcctagcaagcatttatcatccccaccatcctctacttcaggacacttgagcagaaacagtcaaggtttttgccgttttcatcctgctcttcaaaacactgtaagtagtggcgcaggtaagcacagccacaggtgaagaccgttttcagctgaggctgcacatcagaaccacagatcacaggggatggtgcgtgacaatcgtctcagttctcccagtaatgcccatgctagccccaggctcgatgccaggagggaagtgcattccttactgagggagggcatcaggcgtgggtcttccacggaaccccaataggaatcagcaacccccaagcagatattactcaaaggtggtattacatacaacagtagtcagactcagacttcaagcagcccaaagagtggaaccacaggcttgcacaattataaaatgtttttatttcaattacataataacacgttttcctcaaattttattgaggttttggtctttttgcattcaattctatcttgtaacagtaatatgaatccacataatttcataaaatgtcaacaacattcataaggtacattcctttgtgattttatattttacaattttaaatctaactttacaattattttaaaaaatttttttatatagaaaacagatattttcttcaggcagatcaaaacaagaattttccagtaagaatatactgggacataacaaatgaaaatatttataccaaaataccaaaagtgattcagctctttaaaatatcctactatagtctaattagtagcttgtacaagaacaagtaaccattttttactgctcttttgaatgatgattagaaattcaaacaaagtattttaaggttcaaaaactttttttttttttttttttttttttagagacagtgtctcactctgtctcccaggctagagtacagtgtgcaatcatagctcactgcagccttgaactcctggcctcaagcaatcctcccaccttggcttcccaatgtgctaggtttacaggcgtgaaaacattgtgttgtgtgtgtgtgtgtttttttttttttttttagacagagtttcgctcttgttgtccaggctggagtacaatggcttgatcttggctcactgcaatctctgcctcgcaggttcaagcgattctcctgcctcagcctctggagtggctgggattacaggcgcccaccatcacgcccggccaattttttgtatttttagtagagacagggtttcaccatgttggccaggctggcctcgaactcttgacctcaggtgatccacctgccttggcctcccaatgtactgagattacaggcatgagccaccacgcccggccaaaaacatttaaaaaatgactgtccctgctcaaatactgcagtaggaaatgtaatttgacatatatcacttccagaaaaaaactttaaatctttctataaaatgaatttgatacatcatcagcatgaagtgaagttaaaatctcttacaaagtaaattcaggtatatcaacaatgagatccaaaagtatcggttcaagatcaaagactcatatgaggtaaaggcaaataaagcccctcatgctttcagacatttacttgttatccttaaaatgattattgttctaaggtgcaaatcttatcattcagtgacctatttgctatttggctgtttatctcctttaaataaaataccatacaggttataatgtacattttaaaatcaaatatgaaagtacacatatgtgaacaagacattaatttaaatatcaattatattcataatacagaagtctaagaatgctatttggtcatttcaattagatgctgatatatttggtcaagaaaacccacattcctatcagcctaaggcaaatagtaaatgcctctatttttattaagtggactataaacagtagacattattgtttgatactactggaatgctctcaattagaacgtacactgataacaaatatgtctttctaatctgggtgataacctcaatgattacatggaaatctacaagtaacagtctataacttaaagcagtagagcacctggtaattgtcatacagtgcctctctatgaatttagaacattctacttacattggcagtggagagaaaagaccccttcacactgagacttcctgtgcaccgcgcctgccgcctgcctcagcttaggacatggtacagtcttctttgcttttgcccttctcattccctcctctggtatcttctctgctttctggattgaagtgccctggctctcttcctggtgccgacaagtcatcgttctctaggctattgctgtctaaagctttcctgacggtctgacttggatgttctgacatctcacacctctctgtactttctgcttcacaggcatcactaatgtcctgtgagggactttcatgttcgggcagggtgcagcgatctgcgtcttcgctctttggttctgcaggactgctttgagtggcaccatctattttagcattatcttttgcaacaccttcatctaattcttcaccaccagccctcgggcctgatgattgaacggtgtcatcctcaaaatctaatgtgtctccatcagctagtacctcctcagctgctgtttgtacatcatcaccttcttggtcaagttttccatccaacttaattttaggattctccggacaatcaacattttcactgctttctgctgcaattttctgttttggattttcagtcacctcgttttgggcttccactgctgactttctgtcagtagactttacctgctcttcttccttaatttcacttaaatctgtgttctgatacgttaactcttttttaacatctttaagggtttctacgggtactggggattttttcttcttgtttttctttttcttgttctttgtcttcttctgcgatgagtccaatgcctctccctgttggtcactcttttcttcatcgggctctttcatatctaagggttcattttgagtgtctactgtacttggacctgtcgcttcctgacagttgccctcagttcctgctggagaaccaggaacttctgtcttgattggtttctcgtcccttaatcctgtttcttcaccctcttcttcgttgtgatccctacctacttctgtactgtgcgctggaacctccttgggctcagctgcttcctggttggtgaattctttctctaaactatgccctgtgcttgtctctaactcttgggggacctctaccatacatttgtcatcatgataaactgtgtcatcactatgccctaaaggacacgaggccactgtgcctgcctgctcttcaacctgagtcactgctgcctctcccacattctctgtgtggttcccaccatctaagtcactccaacagttggatggctcaaggggagttctggtcctgtcatctggtgcacccatgacctcatttgactcaacctgtactgtgttttcagggagagaactgctctcaagaatttggctttgaacctgttcctcataggtagcacctgctaaggttcctaggaatggggcagtgtcttcagaggatttctggtcctcggtattctcaccagcagggaatacctctatgtccacacagtccttcactgtgtcctctgtgtgttgttctttctcagtattgtgcaagatttctcttttccccacattcgccacgatttcatttttcacctccacttcactggctcttcctagggtcccatcccctgtcgacttgagggcatttaactcttcttttgtcatcttggtaggaccttggtatccaacattattgagggtgtcggaagtctctccattggtagctatttctgaatttaggattattccatgtttctttaattcctctttcagcatgactacttcttctctaagatcatcccgttcactccttacggaatcaaagaactctttctgcctctctaatgcccctatctttttgtctttccactctattgtttcctgaagatcagaaatctccctgatagaactcgcctgtttctgctgtagctgtcggatttcctcgagcatttcctctctttgcttcagggcctccttgacttcagcaaactgaaattgcagtatactgtgggcgtgtttttccctttcaaattctttgtttttctcttcgtactgccgcctagattcagccagctgttcttcaagctccagcaacatatcttttagggtatcaacctggtacatgaagtttgtcttttcattgtctagctgagcattggaaaccatagccttcttatatttctcttcaacttctgctagagagtccttgatttccctgatggatgcctcggtgtcgatggagatggaggtgtctccgctgcctctccgagaggaagtcccacccagagaggccagcgtggctgcagacaggcccggcatgttacgagaccccttctcagtaaaatctttttctggtctctcttctaccctcaggcttccacgactacccactgacatgcgctcgtcttcatcagaagccgatgtgtttcttctggatctacgagagtagcgctcactgtcttcctccttctgctgccgctccagctccttcatgcggatctcgcgagcctccgcgcgggccgcccgttttgcagcgagccgggcttccgccagcttctgcgcttccgggctcaaacagtcgatctcccggctttgagcggccgcggggctggtcatcctgccgggctcggcccgctccacccggcgggaaatgctcggggaccgcgccgggagcccctcgcgggccgggccagggggcgcgcgctctgtc

SEQ ID NO: 12153 - RNA, 5783 nt, Homo sapiens
  source 1..5783: mol_type = other RNA
ctgcagactcgacctcccaggctcaggtgtttctgcctcctaagtagctgggactacatgggactacatgcacatgccaccatgcctggctaattgtttgtatattttttttgtagagatgggctttcatcatgttgcccaggctgggcttgaactcctgggcttaagtgatctgcctgcctcggcctcccacgtgctgggattataggcatgagccaatgtgcccggcctcaaccatttcttgataagttaagggccttcacagtaatatcaattactgtgcttggctataaagtcattacactggagagcatataactgatgctcagaatgaaggctctgaaatcatcgagaaatggtttggctgctcagaactctttctttttccttctttcttgctcatggattttcagctgtccattccctactggagggctgggtccaactgcttgttcactggcacagtgccttccatgtacaaagtgatcaaacctgtctattaattaagcaaatgagtggtgaatcactgagacggctggatggctgagctgagggatgtgatgtgtgcccaacgtcctgcagggtgctggtgaataacatgagaaagaacttaaaatggcttgatgatctcaccatttagtgaccttggttgtcacactgctttccaagagccctttaaaggtaggaatgagagctgtttccagtatgcattccaataggaatgcagctttgctaaagttagagacataaactaaaaccctgtgaagtcctatagagcccttggacttatttcctagcaagcatttatcatccccaccatcctctacttcaggacacttgagcagaaacagtcaaggtttttgccgttttcatcctgctcttcaaaacactgtaagtagtggcgcaggtaagcacagccacaggtgaagaccgttttcagctgaggctgcacatcagaaccacagatcacaggggatggtgcgtgacaatcgtctcagttctcccagtaatgcccatgctagccccaggctcgatgccaggagggaagtgcattccttactgagggagggcatcaggcgtgggtcttccacggaaccccaataggaatcagcaacccccaagcagatattactcaaaggtggtattacatacaacagtagtcagactcagacttcaagcagcccaaagagtggaaccacaggcttgcacaattataaaatgtttttatttcaattacataataacacgttttcctcaaattttattgaggttttggtctttttgcattcaattctatcttgtaacagtaatatgaatccacataatttcataaaatgtcaacaacattcataaggtacattcctttgtgattttatattttacaattttaaatctaactttacaattattttaaaaaatttttttatatagaaaacagatattttcttcaggcagatcaaaacaagaattttccagtaagaatatactgggacataacaaatgaaaatatttataccaaaataccaaaagtgattcagctctttaaaatatcctactatagtctaattagtagcttgtacaagaacaagtaaccattttttactgctcttttgaatgatgattagaaattcaaacaaagtattttaaggttcaaaaactttttttttttttttttttttttttagagacagtgtctcactctgtctcccaggctagagtacagtgtgcaatcatagctcactgcagccttgaactcctggcctcaagcaatcctcccaccttggcttcccaatgtgctaggtttacaggcgtgaaaacattgtgttgtgtgtgtgtgtgtttttttttttttttttagacagagtttcgctcttgttgtccaggctggagtacaatggcttgatcttggctcactgcaatctctgcctcgcaggttcaagcgattctcctgcctcagcctctggagtggctgggattacaggcgcccaccatcacgcccggccaattttttgtatttttagtagagacagggtttcaccatgttggccaggctggcctcgaactcttgacctcaggtgatccacctgccttggcctcccaatgtactgagattacaggcatgagccaccacgcccggccaaaaacatttaaaaaatgactgtccctgctcaaatactgcagtaggaaatgtaatttgacatatatcacttccagaaaaaaactttaaatctttctataaaatgaatttgatacatcatcagcatgaagtgaagttaaaatctcttacaaagtaaattcaggtatatcaacaatgagatccaaaagtatcggttcaagatcaaagactcatatgaggtaaaggcaaataaagcccctcatgctttcagacatttacttgttatccttaaaatgattattgttctaaggtgcaaatcttatcattcagtgacctatttgctatttggctgtttatctcctttaaataaaataccatacaggttataatgtacattttaaaatcaaatatgaaagtacacatatgtgaacaagacattaatttaaatatcaattatattcataatacagaagtctaagaatgctatttggtcatttcaattagatgctgatatatttggtcaagaaaacccacattcctatcagcctaaggcaaatagtaaatgcctctatttttattaagtggactataaacagtagacattattgtttgatactactggaatgctctcaattagaacgtacactgataacaaatatgtctttctaatctgggtgataacctcaatgattacatggaaatctacaagtaacagtctataacttaaagcagtagagcacctggtaattgtcatacagtgcctctctatgaatttagaacattctacttacattggcagtggagagaaaagaccccttcacactgagacttcctgtgcaccgcgcctgccgcctgcctcagcttaggacatggtacagtcttctttgcttttgcccttctcattccctcctctggtatcttctctgctttctggattgaagtgccctggctctcttcctggtgccgacaagtcatcgttctctaggctattgctgtctaaagctttcctgacggtctgacttggatgttctgacatctcacacctctctgtactttctgcttcacaggcatcactaatgtcctgtgagggactttcatgttcgggcagggtgcagcgatctgcgtcttcgctctttggttctgcaggactgctttgagtggcaccatctattttagcattatcttttgcaacaccttcatctaattcttcaccaccagccctcgggcctgatgattgaacggtgtcatcctcaaaatctaatgtgtctccatcagctagtacctcctcagctgctgtttgtacatcatcaccttcttggtcaagttttccatccaacttaattttaggattctccggacaatcaacattttcactgctttctgctgcaattttctgttttggattttcagtcacctcgttttgggcttccactgctgactttctgtcagtagactttacctgctcttcttccttaatttcacttaaatctgtgttctgatacgttaactcttttttaacatctttaagggtttctacgggtactggggattttttcttcttgtttttctttttcttgttctttgtcttcttctgcgatgagtccaatgcctctccctgttggtcactcttttcttcatcgggctctttcatatctaagggttcattttgagtgtctactgtacttggacctgtcgcttcctgacagttgccctcagttcctgctggagaaccaggaacttctgtcttgattggtttctcgtcccttaatcctgtttcttcaccctcttcttcgttgtgatccctacctacttctgtactgtgcgctggaacctccttgggctcagctgcttcctggttggtgaattctttctctaaactatgccctgtgcttgtctctaactcttgggggacctctaccatacatttgtcatcatgataaactgtgtcatcactatgccctaaaggacacgaggccactgtgcctgcctgctcttcaacctgagtcactgctgcctctcccacattctctgtgtggttcccaccatctaagtcactccaacagttggatggctcaaggggagttctggtcctgtcatctggtgcacccatgacctcatttgactcaacctgtactgtgttttcagggagagaactgctctcaagaatttggctttgaacctgttcctcataggtagcacctgctaaggttcctaggaatggggcagtgtcttcagaggatttctggtcctcggtattctcaccagcagggaatacctctatgtccacacagtccttcactgtgtcctctgtgtgttgttctttctcagtattgtgcaagatttctcttttccccacattcgccacgatttcatttttcacctccacttcactggctcttcctagggtcccatcccctgtcgacttgagggcatttaactcttcttttgtcatcttggtaggaccttggtatccaacattattgagggtgtcggaagtctctccattggtagctatttctgaatttaggattattccatgtttctttaattcctctttcagcatgactacttcttctctaagatcatcccgttcactccttacggaatcaaagaactctttctgcctctctaatgcccctatctttttgtctttccactctattgtttcctgaagatcagaaatctccctgatagaactcgcctgtttctgctgtagctgtcggatttcctcgagcatttcctctctttgcttcagggcctccttgacttcagcaaactgaaattgcagtatactgtgggcgtgtttttccctttcaaattctttgtttttctcttcgtactgccgcctagattcagccagctgttcttcaagctccagcaacatatcttttagggtatcaacctggtacatgaagtttgtcttttcattgtctagctgagcattggaaaccatagccttcttatatttctcttcaacttctgctagagagtccttgatttccctgatggatgcctcggtgtcgatggagatggaggtgtctccgctgcctctccgagaggaagtcccacccagagaggccagcgtggctgcagacaggcccggcatgttacgagaccccttctcagtaaaatctttttctggtctctcttctaccctgccagatcttctattcagggactgtgatccatacaattctccatcataaccatttgtccaggcgtaaggacccccatactccaagtcaggctgcgacctcaggcttccacgactacccactgacatgcgctcgtcttcatcagaagccgatgtgtttcttctggatctacgagagtagcgctcactgtcttccatccactgctcgatgtcaccccattttgtatccagcccataatatttcttttggacctgatagatctccttctgctgccgctccagctccttcatgcggatctcgcgagcctccgcgcgggccgcccgttttgcagcgagccgggcttccgcctcccgcgcgatctggttgagcgcgtcgtcctccgccgtgagccgctcccggttggggagccgcttgcgccccgatccctgggtgcccatgtccatcgaccgcgtcgcccgcagctgccgcggggcccgttgctccagccgctcgcgccgccccggcccggcccc

SEQ ID NO: 12154 - RNA, 5758 nt, Homo sapiens
  source 1..5758: mol_type = other RNA
ctgcagactcgacctcccaggctcaggtgtttctgcctcctaagtagctgggactacatgggactacatgcacatgccaccatgcctggctaattgtttgtatattttttttgtagagatgggctttcatcatgttgcccaggctgggcttgaactcctgggcttaagtgatctgcctgcctcggcctcccacgtgctgggattataggcatgagccaatgtgcccggcctcaaccatttcttgataagttaagggccttcacagtaatatcaattactgtgcttggctataaagtcattacactggagagcatataactgatgctcagaatgaaggctctgaaatcatcgagaaatggtttggctgctcagaactctttctttttccttctttcttgctcatggattttcagctgtccattccctactggagggctgggtccaactgcttgttcactggcacagtgccttccatgtacaaagtgatcaaacctgtctattaattaagcaaatgagtggtgaatcactgagacggctggatggctgagctgagggatgtgatgtgtgcccaacgtcctgcagggtgctggtgaataacatgagaaagaacttaaaatggcttgatgatctcaccatttagtgaccttggttgtcacactgctttccaagagccctttaaaggtaggaatgagagctgtttccagtatgcattccaataggaatgcagctttgctaaagttagagacataaactaaaaccctgtgaagtcctatagagcccttggacttatttcctagcaagcatttatcatccccaccatcctctacttcaggacacttgagcagaaacagtcaaggtttttgccgttttcatcctgctcttcaaaacactgtaagtagtggcgcaggtaagcacagccacaggtgaagaccgttttcagctgaggctgcacatcagaaccacagatcacaggggatggtgcgtgacaatcgtctcagttctcccagtaatgcccatgctagccccaggctcgatgccaggagggaagtgcattccttactgagggagggcatcaggcgtgggtcttccacggaaccccaataggaatcagcaacccccaagcagatattactcaaaggtggtattacatacaacagtagtcagactcagacttcaagcagcccaaagagtggaaccacaggcttgcacaattataaaatgtttttatttcaattacataataacacgttttcctcaaattttattgaggttttggtctttttgcattcaattctatcttgtaacagtaatatgaatccacataatttcataaaatgtcaacaacattcataaggtacattcctttgtgattttatattttacaattttaaatctaactttacaattattttaaaaaatttttttatatagaaaacagatattttcttcaggcagatcaaaacaagaattttccagtaagaatatactgggacataacaaatgaaaatatttataccaaaataccaaaagtgattcagctctttaaaatatcctactatagtctaattagtagcttgtacaagaacaagtaaccattttttactgctcttttgaatgatgattagaaattcaaacaaagtattttaaggttcaaaaactttttttttttttttttttttttttagagacagtgtctcactctgtctcccaggctagagtacagtgtgcaatcatagctcactgcagccttgaactcctggcctcaagcaatcctcccaccttggcttcccaatgtgctaggtttacaggcgtgaaaacattgtgttgtgtgtgtgtgtgtttttttttttttttttagacagagtttcgctcttgttgtccaggctggagtacaatggcttgatcttggctcactgcaatctctgcctcgcaggttcaagcgattctcctgcctcagcctctggagtggctgggattacaggcgcccaccatcacgcccggccaattttttgtatttttagtagagacagggtttcaccatgttggccaggctggcctcgaactcttgacctcaggtgatccacctgccttggcctcccaatgtactgagattacaggcatgagccaccacgcccggccaaaaacatttaaaaaatgactgtccctgctcaaatactgcagtaggaaatgtaatttgacatatatcacttccagaaaaaaactttaaatctttctataaaatgaatttgatacatcatcagcatgaagtgaagttaaaatctcttacaaagtaaattcaggtatatcaacaatgagatccaaaagtatcggttcaagatcaaagactcatatgaggtaaaggcaaataaagcccctcatgctttcagacatttacttgttatccttaaaatgattattgttctaaggtgcaaatcttatcattcagtgacctatttgctatttggctgtttatctcctttaaataaaataccatacaggttataatgtacattttaaaatcaaatatgaaagtacacatatgtgaacaagacattaatttaaatatcaattatattcataatacagaagtctaagaatgctatttggtcatttcaattagatgctgatatatttggtcaagaaaacccacattcctatcagcctaaggcaaatagtaaatgcctctatttttattaagtggactataaacagtagacattattgtttgatactactggaatgctctcaattagaacgtacactgataacaaatatgtctttctaatctgggtgataacctcaatgattacatggaaatctacaagtaacagtctataacttaaagcagtagagcacctggtaattgtcatacagtgcctctctatgaatttagaacattctacttacattggcagtggagagaaaagaccccttcacactgagacttcctgtgcaccgcgcctgccgcctgcctcagcttaggacatggtacagtcttctttgcttttgcccttctcattccctcctctggtatcttctctgctttctggattgaagtgccctggctctcttcctggtgccgacaagtcatcgttctctaggctattgctgtctaaagctttcctgacggtctgacttggatgttctgacatctcacacctctctgtactttctgcttcacaggcatcactaatgtcctgtgagggactttcatgttcgggcagggtgcagcgatctgcgtcttcgctctttggttctgcaggactgctttgagtggcaccatctattttagcattatcttttgcaacaccttcatctaattcttcaccaccagccctcgggcctgatgattgaacggtgtcatcctcaaaatctaatgtgtctccatcagctagtacctcctcagctgctgtttgtacatcatcaccttcttggtcaagttttccatccaacttaattttaggattctccggacaatcaacattttcactgctttctgctgcaattttctgttttggattttcagtcacctcgttttgggcttccactgctgactttctgtcagtagactttacctgctcttcttccttaatttcacttaaatctgtgttctgatacgttaactcttttttaacatctttaagggtttctacgggtactggggattttttcttcttgtttttctttttcttgttctttgtcttcttctgcgatgagtccaatgcctctccctgttggtcactcttttcttcatcgggctctttcatatctaagggttcattttgagtgtctactgtacttggacctgtcgcttcctgacagttgccctcagttcctgctggagaaccaggaacttctgtcttgattggtttctcgtcccttaatcctgtttcttcaccctcttcttcgttgtgatccctacctacttctgtactgtgcgctggaacctccttgggctcagctgcttcctggttggtgaattctttctctaaactatgccctgtgcttgtctctaactcttgggggacctctaccatacatttgtcatcatgataaactgtgtcatcactatgccctaaaggacacgaggccactgtgcctgcctgctcttcaacctgagtcactgctgcctctcccacattctctgtgtggttcccaccatctaagtcactccaacagttggatggctcaaggggagttctggtcctgtcatctggtgcacccatgacctcatttgactcaacctgtactgtgttttcagggagagaactgctctcaagaatttggctttgaacctgttcctcataggtagcacctgctaaggttcctaggaatggggcagtgtcttcagaggatttctggtcctcggtattctcaccagcagggaatacctctatgtccacacagtccttcactgtgtcctctgtgtgttgttctttctcagtattgtgcaagatttctcttttccccacattcgccacgatttcatttttcacctccacttcactggctcttcctagggtcccatcccctgtcgacttgagggcatttaactcttcttttgtcatcttggtaggaccttggtatccaacattattgagggtgtcggaagtctctccattggtagctatttctgaatttaggattattccatgtttctttaattcctctttcagcatgactacttcttctctaagatcatcccgttcactccttacggaatcaaagaactctttctgcctctctaatgcccctatctttttgtctttccactctattgtttcctgaagatcagaaatctccctgatagaactcgcctgtttctgctgtagctgtcggatttcctcgagcatttcctctctttgcttcagggcctccttgacttcagcaaactgaaattgcagtatactgtgggcgtgtttttccctttcaaattctttgtttttctcttcgtactgccgcctagattcagccagctgttcttcaagctccagcaacatatcttttagggtatcaacctggtacatgaagtttgtcttttcattgtctagctgagcattggaaaccatagccttcttatatttctcttcaacttctgctagagagtccttgatttccctgatggatgcctcggtgtcgatggagatggaggtgtctccgctgcctctccgagaggaagtcccacccagagaggccagcgtggctgcagacaggcccggcatgttacgagaccccttctcagtaaaatctttttctggtctctcttctacctccttctgctgccgctccagctccttcatgcggatctcgcgagcctccgcgcgggccgcccgttttgcagcgagccgggcttccgccagcttctgcgcttccgggctcaaacagtcgatctcccggctttgagcggccgcggggctggtcatcctgccgggctcggcccgctccacccggcgggaaatgctcggggaccgcgccgggagcccctcgcgggccgggccagggggcgcgcgctctgtccgcggagacggagccactcgccgctaagtgaacgctcgcgcttccggggccaggagccagcccgccggggagcggctcgcggcgctgggctcgggcgcggccgacaggggcggggcgcaggtggccgcgggctgagtcgggctcggggtggaagggcgccggggaagcgggactcgggcgcctccgcccgtcccacggcccgccccgccccccacgcagttccgcctcggaggggccctcc

SEQ ID NO: 12155 - RNA, 5497 nt, Homo sapiens
  source 1..5497: mol_type = other RNA
ctgcagactcgacctcccaggctcaggtgtttctgcctcctaagtagctgggactacatgggactacatgcacatgccaccatgcctggctaattgtttgtatattttttttgtagagatgggctttcatcatgttgcccaggctgggcttgaactcctgggcttaagtgatctgcctgcctcggcctcccacgtgctgggattataggcatgagccaatgtgcccggcctcaaccatttcttgataagttaagggccttcacagtaatatcaattactgtgcttggctataaagtcattacactggagagcatataactgatgctcagaatgaaggctctgaaatcatcgagaaatggtttggctgctcagaactctttctttttccttctttcttgctcatggattttcagctgtccattccctactggagggctgggtccaactgcttgttcactggcacagtgccttccatgtacaaagtgatcaaacctgtctattaattaagcaaatgagtggtgaatcactgagacggctggatggctgagctgagggatgtgatgtgtgcccaacgtcctgcagggtgctggtgaataacatgagaaagaacttaaaatggcttgatgatctcaccatttagtgaccttggttgtcacactgctttccaagagccctttaaaggtaggaatgagagctgtttccagtatgcattccaataggaatgcagctttgctaaagttagagacataaactaaaaccctgtgaagtcctatagagcccttggacttatttcctagcaagcatttatcatccccaccatcctctacttcaggacacttgagcagaaacagtcaaggtttttgccgttttcatcctgctcttcaaaacactgtaagtagtggcgcaggtaagcacagccacaggtgaagaccgttttcagctgaggctgcacatcagaaccacagatcacaggggatggtgcgtgacaatcgtctcagttctcccagtaatgcccatgctagccccaggctcgatgccaggagggaagtgcattccttactgagggagggcatcaggcgtgggtcttccacggaaccccaataggaatcagcaacccccaagcagatattactcaaaggtggtattacatacaacagtagtcagactcagacttcaagcagcccaaagagtggaaccacaggcttgcacaattataaaatgtttttatttcaattacataataacacgttttcctcaaattttattgaggttttggtctttttgcattcaattctatcttgtaacagtaatatgaatccacataatttcataaaatgtcaacaacattcataaggtacattcctttgtgattttatattttacaattttaaatctaactttacaattattttaaaaaatttttttatatagaaaacagatattttcttcaggcagatcaaaacaagaattttccagtaagaatatactgggacataacaaatgaaaatatttataccaaaataccaaaagtgattcagctctttaaaatatcctactatagtctaattagtagcttgtacaagaacaagtaaccattttttactgctcttttgaatgatgattagaaattcaaacaaagtattttaaggttcaaaaactttttttttttttttttttttttttagagacagtgtctcactctgtctcccaggctagagtacagtgtgcaatcatagctcactgcagccttgaactcctggcctcaagcaatcctcccaccttggcttcccaatgtgctaggtttacaggcgtgaaaacattgtgttgtgtgtgtgtgtgtttttttttttttttttagacagagtttcgctcttgttgtccaggctggagtacaatggcttgatcttggctcactgcaatctctgcctcgcaggttcaagcgattctcctgcctcagcctctggagtggctgggattacaggcgcccaccatcacgcccggccaattttttgtatttttagtagagacagggtttcaccatgttggccaggctggcctcgaactcttgacctcaggtgatccacctgccttggcctcccaatgtactgagattacaggcatgagccaccacgcccggccaaaaacatttaaaaaatgactgtccctgctcaaatactgcagtaggaaatgtaatttgacatatatcacttccagaaaaaaactttaaatctttctataaaatgaatttgatacatcatcagcatgaagtgaagttaaaatctcttacaaagtaaattcaggtatatcaacaatgagatccaaaagtatcggttcaagatcaaagactcatatgaggtaaaggcaaataaagcccctcatgctttcagacatttacttgttatccttaaaatgattattgttctaaggtgcaaatcttatcattcagtgacctatttgctatttggctgtttatctcctttaaataaaataccatacaggttataatgtacattttaaaatcaaatatgaaagtacacatatgtgaacaagacattaatttaaatatcaattatattcataatacagaagtctaagaatgctatttggtcatttcaattagatgctgatatatttggtcaagaaaacccacattcctatcagcctaaggcaaatagtaaatgcctctatttttattaagtggactataaacagtagacattattgtttgatactactggaatgctctcaattagaacgtacactgataacaaatatgtctttctaatctgggtgataacctcaatgattacatggaaatctacaagtaacagtctataacttaaagcagtagagcacctggtaattgtcatacagtgcctctctatgaatttagaacattctacttacattggcagtggagagaaaagaccccttcacactgagacttcctgtgcaccgcgcctgccgcctgcctcagcttaggacatggtacagtcttctttgcttttgcccttctcattccctcctctggtatcttctctgctttctggattgaagtgccctggctctcttcctggtgccgacaagtcatcgttctctaggctattgctgtctaaagctttcctgacggtctgacttggatgttctgacatctcacacctctctgtactttctgcttcacaggcatcactaatgtcctgtgagggactttcatgttcgggcagggtgcagcgatctgcgtcttcgctctttggttctgcaggactgctttgagtggcaccatctattttagcattatcttttgcaacaccttcatctaattcttcaccaccagccctcgggcctgatgattgaacggtgtcatcctcaaaatctaatgtgtctccatcagctagtacctcctcagctgctgtttgtacatcatcaccttcttggtcaagttttccatccaacttaattttaggattctccggacaatcaacattttcactgctttctgctgcaattttctgttttggattttcagtcacctcgttttgggcttccactgctgactttctgtcagtagactttacctgctcttcttccttaatttcacttaaatctgtgttctgatacgttaactcttttttaacatctttaagggtttctacgggtactggggattttttcttcttgtttttctttttcttgttctttgtcttcttctgcgatgagtccaatgcctctccctgttggtcactcttttcttcatcgggctctttcatatctaagggttcattttgagtgtctactgtacttggacctgtcgcttcctgacagttgccctcagttcctgctggagaaccaggaacttctgtcttgattggtttctcgtcccttaatcctgtttcttcaccctcttcttcgttgtgatccctacctacttctgtactgtgcgctggaacctccttgggctcagctgcttcctggttggtgaattctttctctaaactatgccctgtgcttgtctctaactcttgggggacctctaccatacatttgtcatcatgataaactgtgtcatcactatgccctaaaggacacgaggccactgtgcctgcctgctcttcaacctgagtcactgctgcctctcccacattctctgtgtggttcccaccatctaagtcactccaacagttggatggctcaaggggagttctggtcctgtcatctggtgcacccatgacctcatttgactcaacctgtactgtgttttcagggagagaactgctctcaagaatttggctttgaacctgttcctcataggtagcacctgctaaggttcctaggaatggggcagtgtcttcagaggatttctggtcctcggtattctcaccagcagggaatacctctatgtccacacagtccttcactgtgtcctctgtgtgttgttctttctcagtattgtgcaagatttctcttttccccacattcgccacgatttcatttttcacctccacttcactggctcttcctagggtcccatcccctgtcgacttgagggcatttaactcttcttttgtcatcttggtaggaccttggtatccaacattattgagggtgtcggaagtctctccattggtagctatttctgaatttaggattattccatgtttctttaattcctctttcagcatgactacttcttctctaagatcatcccgttcactccttacggaatcaaagaactctttctgcctctctaatgcccctatctttttgtctttccactctattgtttcctgaagatcagaaatctccctgatagaactcgcctgtttctgctgtagctgtcggatttcctcgagcatttcctctctttgcttcagggcctccttgacttcagcaaactgaaattgcagtatactgtgggcgtgtttttccctttcaaattctttgtttttctcttcgtactgccgcctagattcagccagctgttcttcaagctccagcaacatatcttttagggtatcaacctggtacatgaagtttgtcttttcattgtctagctgagcattggaaaccatagccttcttatatttctcttcaacttctgctagagagtccttgatttccctgatggatgcctcggtgtcgatggagatggaggtgtctccgctgcctctccgagaggaagtcccacccagagaggccagcgtggctgcagacaggcccggcatgttacgagaccccttctcagtaaaatctttttctggtctctcttctacctccttctgctgccgctccagctccttcatgcggatctcgcgagcctccgcgcgggccgcccgttttgcagcgagccgggcttccgcctcccgcgcgatctggttgagcgcgtcgtcctccgccgtgagccgctcccggttggggagccgcttgcgccccgatccctgggtgcccatgtccatcgaccgcgtcgcccgcagctgccgcggggcccgttgctccagcc

SEQ ID NO: 12156 - RNA, 5468 nt, Homo sapiens
  source 1..5468: mol_type = other RNA
ctgcagactcgacctcccaggctcaggtgtttctgcctcctaagtagctgggactacatgggactacatgcacatgccaccatgcctggctaattgtttgtatattttttttgtagagatgggctttcatcatgttgcccaggctgggcttgaactcctgggcttaagtgatctgcctgcctcggcctcccacgtgctgggattataggcatgagccaatgtgcccggcctcaaccatttcttgataagttaagggccttcacagtaatatcaattactgtgcttggctataaagtcattacactggagagcatataactgatgctcagaatgaaggctctgaaatcatcgagaaatggtttggctgctcagaactctttctttttccttctttcttgctcatggattttcagctgtccattccctactggagggctgggtccaactgcttgttcactggcacagtgccttccatgtacaaagtgatcaaacctgtctattaattaagcaaatgagtggtgaatcactgagacggctggatggctgagctgagggatgtgatgtgtgcccaacgtcctgcagggtgctggtgaataacatgagaaagaacttaaaatggcttgatgatctcaccatttagtgaccttggttgtcacactgctttccaagagccctttaaaggtaggaatgagagctgtttccagtatgcattccaataggaatgcagctttgctaaagttagagacataaactaaaaccctgtgaagtcctatagagcccttggacttatttcctagcaagcatttatcatccccaccatcctctacttcaggacacttgagcagaaacagtcaaggtttttgccgttttcatcctgctcttcaaaacactgtaagtagtggcgcaggtaagcacagccacaggtgaagaccgttttcagctgaggctgcacatcagaaccacagatcacaggggatggtgcgtgacaatcgtctcagttctcccagtaatgcccatgctagccccaggctcgatgccaggagggaagtgcattccttactgagggagggcatcaggcgtgggtcttccacggaaccccaataggaatcagcaacccccaagcagatattactcaaaggtggtattacatacaacagtagtcagactcagacttcaagcagcccaaagagtggaaccacaggcttgcacaattataaaatgtttttatttcaattacataataacacgttttcctcaaattttattgaggttttggtctttttgcattcaattctatcttgtaacagtaatatgaatccacataatttcataaaatgtcaacaacattcataaggtacattcctttgtgattttatattttacaattttaaatctaactttacaattattttaaaaaatttttttatatagaaaacagatattttcttcaggcagatcaaaacaagaattttccagtaagaatatactgggacataacaaatgaaaatatttataccaaaataccaaaagtgattcagctctttaaaatatcctactatagtctaattagtagcttgtacaagaacaagtaaccattttttactgctcttttgaatgatgattagaaattcaaacaaagtattttaaggttcaaaaactttttttttttttttttttttttttagagacagtgtctcactctgtctcccaggctagagtacagtgtgcaatcatagctcactgcagccttgaactcctggcctcaagcaatcctcccaccttggcttcccaatgtgctaggtttacaggcgtgaaaacattgtgttgtgtgtgtgtgtgtttttttttttttttttagacagagtttcgctcttgttgtccaggctggagtacaatggcttgatcttggctcactgcaatctctgcctcgcaggttcaagcgattctcctgcctcagcctctggagtggctgggattacaggcgcccaccatcacgcccggccaattttttgtatttttagtagagacagggtttcaccatgttggccaggctggcctcgaactcttgacctcaggtgatccacctgccttggcctcccaatgtactgagattacaggcatgagccaccacgcccggccaaaaacatttaaaaaatgactgtccctgctcaaatactgcagtaggaaatgtaatttgacatatatcacttccagaaaaaaactttaaatctttctataaaatgaatttgatacatcatcagcatgaagtgaagttaaaatctcttacaaagtaaattcaggtatatcaacaatgagatccaaaagtatcggttcaagatcaaagactcatatgaggtaaaggcaaataaagcccctcatgctttcagacatttacttgttatccttaaaatgattattgttctaaggtgcaaatcttatcattcagtgacctatttgctatttggctgtttatctcctttaaataaaataccatacaggttataatgtacattttaaaatcaaatatgaaagtacacatatgtgaacaagacattaatttaaatatcaattatattcataatacagaagtctaagaatgctatttggtcatttcaattagatgctgatatatttggtcaagaaaacccacattcctatcagcctaaggcaaatagtaaatgcctctatttttattaagtggactataaacagtagacattattgtttgatactactggaatgctctcaattagaacgtacactgataacaaatatgtctttctaatctgggtgataacctcaatgattacatggaaatctacaagtaacagtctataacttaaagcagtagagcacctggtaattgtcatacagtgcctctctatgaatttagaacattctacttacattggcagtggagagaaaagaccccttcacactgagacttcctgtgcaccgcgcctgccgcctgcctcagcttaggacatggtacagtcttctttgcttttgcccttctcattccctcctctggtatcttctctgctttctggattgaagtgccctggctctcttcctggtgccgacaagtcatcgttctctaggctattgctgtctaaagctttcctgacggtctgacttggatgttctgacatctcacacctctctgtactttctgcttcacaggcatcactaatgtcctgtgagggactttcatgttcgggcagggtgcagcgatctgcgtcttcgctctttggttctgcaggactgctttgagtggcaccatctattttagcattatcttttgcaacaccttcatctaattcttcaccaccagccctcgggcctgatgattgaacggtgtcatcctcaaaatctaatgtgtctccatcagctagtacctcctcagctgctgtttgtacatcatcaccttcttggtcaagttttccatccaacttaattttaggattctccggacaatcaacattttcactgctttctgctgcaattttctgttttggattttcagtcacctcgttttgggcttccactgctgactttctgtcagtagactttacctgctcttcttccttaatttcacttaaatctgtgttctgatacgttaactcttttttaacatctttaagggtttctacgggtactggggattttttcttcttgtttttctttttcttgttctttgtcttcttctgcgatgagtccaatgcctctccctgttggtcactcttttcttcatcgggctctttcatatctaagggttcattttgagtgtctactgtacttggacctgtcgcttcctgacagttgccctcagttcctgctggagaaccaggaacttctgtcttgattggtttctcgtcccttaatcctgtttcttcaccctcttcttcgttgtgatccctacctacttctgtactgtgcgctggaacctccttgggctcagctgcttcctggttggtgaattctttctctaaactatgccctgtgcttgtctctaactcttgggggacctctaccatacatttgtcatcatgataaactgtgtcatcactatgccctaaaggacacgaggccactgtgcctgcctgctcttcaacctgagtcactgctgcctctcccacattctctgtgtggttcccaccatctaagtcactccaacagttggatggctcaaggggagttctggtcctgtcatctggtgcacccatgacctcatttgactcaacctgtactgtgttttcagggagagaactgctctcaagaatttggctttgaacctgttcctcataggtagcacctgctaaggttcctaggaatggggcagtgtcttcagaggatttctggtcctcggtattctcaccagcagggaatacctctatgtccacacagtccttcactgtgtcctctgtgtgttgttctttctcagtattgtgcaagatttctcttttccccacattcgccacgatttcatttttcacctccacttcactggctcttcctagggtcccatcccctgtcgacttgagggcatttaactcttcttttgtcatcttggtaggaccttggtatccaacattattgagggtgtcggaagtctctccattggtagctatttctgaatttaggattattccatgtttctttaattcctctttcagcatgactacttcttctctaagatcatcccgttcactccttacggaatcaaagaactctttctgcctctctaatgcccctatctttttgtctttccactctattgtttcctgaagatcagaaatctccctgatagaactcgcctgtttctgctgtagctgtcggatttcctcgagcatttcctctctttgcttcagggcctccttgacttcagcaaactgaaattgcagtatactgtgggcgtgtttttccctttcaaattctttgtttttctcttcgtactgccgcctagattcagccagctgttcttcaagctccagcaacatatcttttagggtatcaacctggtacatgaagtttgtcttttcattgtctagctgagcattggaaaccatagccttcttatatttctcttcaacttctgctagagagtccttgatttccctgatggatgcctcggtgtcgatggagatggaggtgtctccgctgcctctccgagaggaagtcccacccagagaggccagcgtggctgcagacaggcccggcatgttacgagaccccttctcagtaaaatctttttctggtctctcttctacctccttctgctgccgctccagctccttcatgcggatctcgcgagcctccgcgcgggccgcccgttttgcagcgagccgggcttccgcctttgaagaatgaagatcttagatgaacttcagggggagtgtgaggaacgccagagagcagccatttggagagacatgcttggcacgagagtggaaattctggaataactg

SEQ ID NO: 12157 - RNA, 182 nt, Homo sapiens
  source 1..182: mol_type = other RNA
ctgcagactcgacctcccaggctcgcacgggcggccgcccgggctctcagcccgacacagcgctccaggggctgacaaggaggccgcggggtcacgctccctggggcaacggcccgagggtctcgcggaatcccggtgcagaagtctggaccctccgagcagcctccgcgccccctccggct

SEQ ID NO: 12158 - RNA, 1972 nt, Homo sapiens
  source 1..1972: mol_type = other RNA
ctgcagactcgacctcccaggctctaagaatcctcccaccttagcctcctgagtagctgagattacaggcatgagccactgtgcccaggaacttactcttgcctgtaaaaatacagctctgaagtgaagaaatcccaggcgccacatcaaggaggcgaaactagagtccgcaggaggccagccccgcacgaggagtttcaaacactaaggatcctgacagggaaaagttatatgaagcaagaaaggcaatttaaagcgatagtttatcatatgaatgtttcgttcttaaaaatgaacaagctctatttataatgcccatttagaaatgaatccattaaaaaaaatcagtagatcagcacttattttaattactgagatagagtcacacttgacagaagcaagccctgcggtatatggcatcatcacaccaccggtgggtattttaatcctaaaactgagacagagtttacttaaacatttaaggcttgagtttcctctgtacagtgtggaggtgattaagaaaattaatcctaacatgaagatttttcatccagttaaaaaaagaaatactttaaaaacgacctgcccttccaaaacatgaagttaacttggagtttttctgtgatatgacaaactaggcataatcctatctcggaattgttgagtagaaaatttatgtactaatactcctgttaaaattcaacagctttattgtgaaagaatccagagatctcacactgaaaaaatactaacacagctcatatataaattacttatctataagaacaattatagaaggaatctaaatggggcaattttaacaaaccaggcaaaatatcacatatacctgaatataaggtaactccaagccatgagtataagattaaggcagttactttattttgaacaaggaagtggcataagcaactcagtgtgtgccccttagggtgggagctcttccccctaccactccccaccccaaggcatcattttggagaaaaaagtgtcttctatctggctagctgtgttatctaggattgcaccttcttacacggcaggcgcggcatcacgtccagatgggcatctaaggaactgcatttcgggagatgaaactttcatttgggactcaactgaatgcatgaactaacacagggccatggacccaccagtcttgattgagttacagaaaatgaaggtgactctttacacttccaagttgctttctagatcctttcattacaaaatattctgatcaaataatcttacaaaggaaagataatctagcctcaaggctatcctctaaaagcaaagagaaagtgattgattttctgctcagtcattacattggggacctttacgaggcacgtgttagttcccaggcagcactgctaggcggtctgtgccagaaatttcacgtactgcccgcgggcttcaaaatggtcagcgggccggttgtacgctgtccacaccggttctcccacaaacagccgcatggccttcgtgtagttcttctcgtccaccgtgaagcggtgatagatccccgcggggagcgtcaccatgtctcccttctccatgaagatccggatccactggtcctccttgtccctcacatcgaagtacccactgccatccaggatgtagcggatctcatcgtccaagtgcaaatgctcctcgtagaacatcttaatcttttcttcataatttggtagtttatctttgcatatggttatgatgtccatccaggagtagttcctctctcttcggatcttttctaattctggatcattctcatatttgtcagcatccagcttccagtagagcaccccgagccgccgcagctgctccaggcccactgggcggccggggtcggggcggtggggttgccgcgggtcgcccggggcgtcgtccatataccaggcctgcaccatgacgcgcagtgcgggtgccgtgttcgaacccaggggccgcgctc

SEQ ID NO: 12159 - RNA, 4748 nt, Homo sapiens
  source 1..4748: mol_type = other RNA
ctgcagactcgacctcccaggctctaagaatcctcccaccttagcctcctgagtagctgagattacaggcatgagccactgtgcccaggaacttactcttgcctgtaaaaatacagctctgaagtgaagaaatcccaggcgccacatcaaggaggcgaaactagagtccgcaggaggccagccccgcacgaggagtttcaaacactaaggatcctgacagggaaaagttatatgaagcaagaaaggcaatttaaagcgatagtttatcatatgaatgtttcgttcttaaaaatgaacaagctctatttataatgcccatttagaaatgaatccattaaaaaaaatcagtagatcagcacttattttaattactgagatagagtcacacttgacagaagcaagccctgcggtatatggcatcatcacaccaccggtgggtattttaatcctaaaactgagacagagtttacttaaacatttaaggcttgagtttcctctgtacagtgtggaggtgattaagaaaattaatcctaacatgaagatttttcatccagttaaaaaaagaaatactttaaaaacgacctgcccttccaaaacatgaagttaacttggagtttttctgtgatatgacaaactaggcataatcctatctcggaattgttgagtagaaaatttatgtactaatactcctgttaaaattcaacagctttattgtgaaagaatccagagatctcacactgaaaaaatactaacacagctcatatataaattacttatctataagaacaattatagaaggaatctaaatggggcaattttaacaaaccaggcaaaatatcacatatacctgaatataaggtaactccaagccatgagtataagattaaggcagttactttattttgaacaaggaagtggcataagcaactcagtgtgtgccccttagggtgggagctcttccccctaccactccccaccccaaggcatcattttggagaaaaaagtgtcttctatctggctagctgtgttatctaggattgcaccttcttacacggcaggcgcggcatcacgtccagatgggcatctaaggaactgcatttcgggagatgaaactttcatttgggactcaactgaatgcatgaactaacacagggccatggacccaccagtcttgattgagttacagaaaatgaaggtgactctttacacttccaagttgctttctagatcctttcattacaaaatattctgatcaaataatcttacaaaggaaagataatctagcctcaaggctatcctctaaaagcaaagagaaagtgattgattttctgctcagtcattacattggggacctttacgaggcacgtgttagttcccaggcagcactgctaggcggtctgtgccagaaatttcacgtactgcccgcgggcttcaaaatggtcagcgggccggttgtacgctgtccacaccggttctcccacaaacagccgcatggccttcgtgtagttcttctcgtccaccgtgaagcggtgatagatccccgcggggagcgtcaccatgtctcccttctccatgaagatccggatccactggtcctccttgtccctcacatcgaagtacccactgccatccaggatgtagcggatctcatcgtccaagtgcaaatgctcctcgtagaacatcttaatcttttcttcataatttggtagtttatctttgcatatggttatgatgtccatccaggagtagttcctctctcttcggatcttttctaattctggatcattctcatatttgtcagcatccagtgaacaacaaactccagtgttgcaggaagtcagggaccccgaatggagggaccggctggagccatggcagaggaacataagttttgaagatttcacggacatctatcagttctcaaataatacttttataatttattatgcctgtctttaatctcttaatcctgttatcttcgtaagctgaggatgtatgtcacctcaggaccactgtgataattgtgttaactgtacaaattgattgtaaaacatgtgtgtttgaacaatatgaaatcagtacaccttaaaaaataaaataacagcgatttttagggaacaagggaagacaaccataaggtttgactgcctgcagggtcaggcaaaaacacccatatttttcttcttgcagagagcctataaatgggcgtgcaagtagagaaggtatcactaaattcttttcctaggaaggaatattaatattaatactctggggaaggaatgcatttctggggggaggtctataaacagctgctctgggaatgtctgtcttatgcggttgagataaggactgagatacgccctggtcttctgcagtaccctcaggcttactaaggtggggaaaaactccaccctggtaaatttgtggtcagaccagttctctgctctcgaaccctgttttctgttatttaagatgtttatcaagacaatatgtgcagcactgaacatagatctttatcagtggttctgcttttgccctttgccctgtgatctttgttggacccttatcagtggttctgcttttgccctttgtcctgttccctcagaagcatgtgatctttgttagacccttattagtagttctgctttttgccctttgaagcctgtgatatttgtacctactccctgttcttacaccccctccccttttgaaacccttaataaaaacttgctggtctgagactcaggcgggcatcacggtcctaccgatatgtgatgtcacccctggcggcccagctgtaaaattcctctctttatactgtctctctttatttctcagctggccgacacttatggaaaatggaacctatgttgaaatattgggggtgggttcccccgatactccagaacatattaaagtactagtcatcaatacgttattttctacaaagttgactctaaaacttagcctatccactgcatgatatgcacagtactatttgctatggtctgaatgtgtccatattatgacacataatatgtaatatgacacattatatgacacgtgtcataagtttaaatatacgaatgttgaaacttaacacaaatgtgatagtattaaggggtgggacctttaggatgtgattaagtcatgagggcaagccctcatttataggattagtggccttgtaagagagatggagctgggcactgtggctcacacctataatcccagaactttgggaggccaaggtgggcagatcacctgaggtcaggggttcaagaccagcctgtccaacatggtgaaaccccatctctactaaaaatacaaaaattagccaggcatggtggtccacgcctgtgatcccagctactcgggaggctgaggcaggagaatcacttgaatccaggaggcagaggttgcagtgagccaagactgcgctaccagcctgggtgacagagcgaggctccatctcaaaaaaaaaaaaaaaaaaaaaaaagagcaagagagatgtaagagagcagtttgccccttccaccacatgaggacagagcaaggaaatggccgtctatgaggacaggatcctcatcagacactaaatctgctggcaccttaatcttggacttcttagcctctagaactataagaattctataaattgctgttgtttataaattgcccagtttaagctatttttgtcattttgttatagcagcaggtatttagtttattccaagctaaaataatcttccaattgtttgtatgtatgacaaaaggttttttagaactctatgtcactaataacagattgattaaacagatacacaaacatgtccacatgtgttacctctgttaaaaattatgggagatgttacatatatataatgttaatatggggtgtgtgtgtggcttttttgttttttgggtttttttagagatgaggtctcaaacttctggcttcaggcaatctgccgcctcagcctcccaaagtgctgggatgacagaagccaccatgcctggcccaggagaggtcactgttttggactgagcccctgcactaggccccaggatgagaccaaaccaaaatgcagccactcatgccatatgccacttgatcaaactaaaactttaaagaaggaggtgcatctcaaacagaccagcttttcctgcgatcagaagattccagtcttcctgagtcagaataataaggaagtcgcttctgctttaacccttaggaaaaaagtaacctaatgtaacttgacgttaaccaatcagcttttctacctattgttctgtttctttgttgccgccctacaaaacccactgttgtgctattaccctatcgagctcttattctattttgtagaacggaggttgccctattcacaaatcaagaataaaagctaattagatctttaactaaatttgttgtaattttgtcttccaacagcactgatccagaatggatattaagaaagcatataggccgggtgcggtggttcgtgtctataatgccagcactttgggaggccgaagtgggtggatcacctgaggtcagcagttcaagatcagcctgaccaacatggagaaaccctgtctctactaaaaatacaaaattagcccggcatggtgctgtgcaccttgtaatcccagctactcgggaggctgacacatgagaatggcttgaactcgggaagatgaggttgcggtgagccgagatcatgccactgcactccagcctgggcaaa

SEQ ID NO: 12160 - RNA, 3341 nt, Homo sapiens
  source 1..3341: mol_type = other RNA
ctgcagactcgacctcccaggctgaagccatcctcccacctccgcctcccgagtagctgaggctacaggtgcacgtcatcatgcctggctaatttttgtatttgttgtagagacggggttttgccatgttgcccaggctggccttgaactcctgggctcaagtgatctgcccaacttcggcccccacaaagtgctgggactacaggcgtgagccactgcacccagcaggggttgaactttttaagccaattgcggaaacatgccctatcggccccagccccacctaactcttgctgaattctcctctcttcagacttgaaactccacatgtccttgagtgtcctggagagaccctgggacgtgccgttattcatggttagctctgttcagtgtcaccggttggttctttgatactcctcaccgatgcagagcaaaaaccccgctttggttataaaataacatcccatcaacagctgtgcaccgcggtccttggggttggagacccgtttggaggaggcggacggaagcatgtgccacaggcctcctgtttgtagctttcttcctgtctcaacatctgcctagtacacagctgctgctttgcttgggaatcgacttttcactgttgtgtgtcgggtacctaggaggcgcatcctgacgtgggtttatgcattttggaagtaattcacctttctgcacctcctcagctgatcataggcggcctggataaaatagacttgaacgactggaagtcgaacacgcggctgaagcactgtgtggccgacagcaacatcgtgcggtggttctggcaagcggtggagacgttcgatgaagaaaggagggccaggctcctgcagtttgtgactgggtccacgcgagtcccgctccaaggcttcaaggctttgcaaggtgactgacgtggaggcagggctattcgatgacgcgtctatgtgcgctgtgggcaggaagagctggaaggtggctgggatgtttttctgagatgtgtgctggtaagcaccgcggccaggaagtcacggcgtcctgggagccccagaggatgctgacgttcacgttttttttttgttgtttttttttgagatggagtctctgccaaaatatttttgtcatcatcagaactcaaaagccacagcaccctagaaagccagaagtcactgtacatcctctgggtcacaattttgtattttttggtttgctacgatagcttcttaaaggatgtctttttctttgcacaaatactggaaatgagcttcccctttactgtgtgttgattgggcacagtggctcccagcacgttgagagggcaaggcaggaggttcacttgaggccaggagtttgagagcagcctgggcaacctagcgagaccctgtcttgcctgtccttggccttgaggttggtcctagggctggactgcccacacggtgactctcttttgtcctttttcagctttaaccggatcgacattccaccatatgagtcctatgagaagctctacgagaagctgctgacagccgtggaggagacctgcgggtttgcttgaaatggtgtttggagaaaaagggcatattgtctgcatggtctggaccctcctcactctggagccggcagcctcccgggtccagctcccagcaatgctgtgccgggtggacagagctgaggttcatggtcactgagttgctgcctgaagggctccagactccagatccttgatctttccacgtggagctcatgagagctcctggatcttcaccggggaggtgctatctcctgccttggccattccaaggttggttttcccaacaaccagggggaaggtgtgggcgaacctggcagcaggccgggcctcttcctcaccagtagcaccagctccagactcccattctccagtgtgaaagacaaatgtcccccaaccctaacgccacccacacatctgcacagacaccaggcttcatggagcgcaagacgactcacacagtggcccaggccttgtcacacgcagtgaggacaatcagaggagcacggtcaccgctcaggcctgatgccagcaggacacccaccagctgccagatgagcacgcaatcactcctcatttgcaaagcacggctcccatcattccagaacccaagacactgtctcacaaagacagctctctgcaaggaactgggaagtaacttgagtccagtcagaccggcaaaaatcagtccctcggccttgacctgtgagcagcatgtgggcttggaatcaggctggacgggcttccctcccagtttctccacagctgctccaggcctgggacaagcttctcaccttctgtgagctggaaaccccctctctataaagtggggaaccacccctctgggctgagggctggagcccagcacagagaccttgatggtagctgccagtaccgcccactgcaaaccagcctgcacccaggccataacccagcaacacaactgcgatctcaagctgccaagggacatcttgtcaaggccctttcatttgaccctgtggtgggatttgggtaaactcagctgtaatcatcattccgtggtagcctggaacaatggagggtaaatgaaaggcaaggagagtcaagggctggagaaggttctgtggcctgcggcagaggtccagagagggctccgtgctgcccccgtcccctggggcctgtaaagggccatcttcctcgaagaagatgtttctgacatcatggcgtgtgctccttggggactgcccctcccacacgagggcaggcctggctgaaggtacacactggatgaaggacaatgaggaggtagagctgggtacagagtgcttcatgctgagcctccgggcatgcttcgtgtacactccgcacactctccacacacacacgttacatggcagcagtcctgaaacacatgaagatagctgagggctccgagagtctggcatgccgacccgctgctgagatcaggccgccattctgagagtcccgcacgccgacctgctgctgaggtcgggccgccattcctcatcaacttgactgaatatgctctgagctggcttcccaggtgccaagtcatggcctcccctgtgatcacagcagcactgtgcctgcccaggcagcgcacgctgtcaccaagaggctacgctgaggagcccacactgtctctggggcctctggttcccaaggggctagggacattgagagggaagaaacccctcatggaaacaagcattttaacataaacaagggacaataaacccttttataaaatatttattctaaaaaaaaaaatcacactgtacaaatttagatagaacattatcaatgctcagat

SEQ ID NO: 12161 - RNA, 26 nt, Homo sapiens
  source 1..26: mol_type = other RNA
ctgcagagtttgtacggaccggattc

SEQ ID NO: 12162 - RNA, 4302 nt, Homo sapiens
  source 1..4302: mol_type = other RNA
ctgcagccacttggggaactggtgtctgaccctggcatgctgtactgctctggctggcagatatttacagagaccagaggtgggactttctgctgggttgggtgatggtggaatccggatgtgatcttatgagtgggtagatggggagtcattttgtatgtgtgccaggggaggaggtggaacagactgtctctcgtgtttcttacaaggtgttaacaacttatcaggatctgccatttgagggtgcagaaagaggctgtgagtacatccttacaaccttatctcgccctcacctccatatttcccatttccttctgcaggaaaaccacctaggccattggcctggcagggcctgggacagcctctggctgtggtgccttccccatagctctttcttgctgcaggctccagctcccactgtttcctaaagcttaaagctgcccacctcctccccatgcctgggcttctgttctttttcatcctgtctgcagagcagggcatgatctctgagtttcttcttccttccttgttgtccccaaagagcagcacacaggcccttttccttctgaggccatggttctcagctttgtctccactttagaatctcctgaggagctgcagaaaaaatactccaactccatccccatccctagagtcagattccaatagtctgggatgaggcctgggcagcgccatttcaaaagctccccaggtgatattaatgtgcagccacagatgggaacattggatttaaaggttcctgctgtctatacatcagggaatcgggcaggggagaccctgataacagacggggaagggacaaagggttaatagacgtcaaaggtcttccaggagccctgagtctccttcatgcattactctcttaggagaaaataatggcactggttcacaccacagctcaaggcacagtgccaagtgctttatgtgtattacttcactgaatcctcaggaccaccttaggagatattatcagtaacttcattttacattgaggaaactgaggcatcaagaggttaagcaatgggtccaagagtacacaaacagcaagtggcatagctgggatttgaactcaggcatgcagctggccatcaaccactatgccctggctgccaagcatcaaaccgagtactgctctaagacgttcccttcatacctggaagagccctcattccacaccccaggtctggaaatgtgcactggggctgaaaaaaatggtgtcacttagtttccactcaggtgtcctttgccctaaatgggtcatttgtttttgagggaactccatttaagggctggcagtcaccttccagaggagacagagagctgcagtggttacaaaatggactctggtcggacagacctggatgtgtgtcccagctccgcacttacatgctggtgactgtagacaaggcttccctcctgtctagcgctggtctcctgtgtgtcaagtgggataatcacaccgagttcctggagttgggagggtgaggtgagagtgcataggtgaggtgcctggtacagagcctggccaagcctccagcccaccctctatcaggagtgccttctaggccatggcgtggacccctttgtcatgcctttggcagtctggcacggcttagggaccctttctaggaaaaaaataggtgggagatctttgggggtagaaaatagtagctattattttgtgtttttaaagttttattttatttttcattgacaaataattgtatatatttatagggtacattgtgaggttttgatacatgtatacattgtggaatggtcaaatcagggaaattagtatatccatgacctcaaataggtatcattatgatcatttatcacacatttattatgtgtgagaatatttaaaatctaagacattggtcaataggcactaagttacagttagagaggaggaaaaagttttggtgtcctattgcacaacataggcaactatagttaataacaatgtattgcatatttcaaaaaatgcttctaaatgtattagataaattacctaggattataaaggaaactgattactgtatcttgagatgcaatttacaatatagtcatatgtgcttcttgattaacaccttcaatataacacgatcaagcagtgggtctaatgactattatcattttgaagtggtgatgagcatagatgattttctgagatccctgccacaaccgtaatgtgatatgaaaatagctgtgattctagtagtgacagtcacagatgctgctaatagcactgtggcttactgccccagaaacagctttgtgtgctcttttgttctttagctatgtgatctagaccacccactcagcctctctgtgcccgtcctcatctgtgaaatgaaggtacctgtgaggatgaaatgagttaatgaaccagcaaaaatggctcaaacaccatgcagagtactgtgccatttgtattcttttgggatctgggatcttcaaatgtctcctttaaaatactgccaaggccacatcttcctaggtcaagaagtaagcccgtgtttcaaggactgccaactcttgggcttcacctgaggagaagtccccagggcctctcctggtagccccatttgtagcctcagtcgctgtccttacctcaccaccaaaccattatagttacaagccctaccatagatctcagcttcctgtgtaagagttcagaattttcctacaaacttctaacaaattaaagactgatttggaaacccacagcgctccctaatttgttatagttgttaggggtcagggaggggtttagggagcatcagagccatctctttactgtgcagatgtggcaactgaaacagaaagagaccctaaggtcacatggaagcttgttggcagtgttaggcctgggacccaagattcctctccctcaggcctcctagggcacagtcaaatctccatcctctttggttcctcctccttcatcctcaccatctcatcagttgacagttcccgtcggttccatttcctcctaaatatgtcaccaatctgtcagctcctgccttggctcaggccctctcccactctactcctactggcactgctgcctcggcctccccaccagcctccctgcctccagtctcaacctccaatagaaccttcctaatccatgcttctcttcctgttgcatgccaagaatgtcaagagctcagaggaagcttgcagtccctgagtccaagctcctcactcaccaccccactccacatcctgccatgtcatagaggaggaaactgaggctgagccaggggaatggagctagccaagtctgatagtgaacaagaggtagagctgaaaccaaaactcaggtcaaagggtcatggaatttgagggctagaaagcttagtttagtgctattcccattacatcacccacctctgagaatcacacccccagatcctattgtttcaggtaacaactggaaatattgttttcatcaggaccataattgccacttccctttctaggcactcattttggaaaaagcagacaatactccatctccttctcccatttctccccaaggttcttgaagcaggcctccagcatccgccagcctgattttcttccttatctgttctaggcataggcaggccctgcctgttccccaaccattttcacacgtatttctactggcctgggcccaaagtcaatttgccaatcttatgtcattggacttccctgttgccttgaatttactagaatatattagaccatatttgtctcccctctgctgccccaacacctagtatcaagcctggcagagaatgaacattcagtctttaagaaataaatgaatgaataaaagaaaatgctggtattgcaaaggataaagaaaagaataagacacagacagtcctgccttccaggagcttagagtttacttatgaagacaagatctagaaagtagtagaaatagtgaatggataaccaggcagccatgtttgactttcctttcaggccaagcagggacctggggtactgtatccaggctggaatgcaaagagctgttgggtgcaaggtataataggtaagtcatggaggtggggtgatctgaagcagcatctaggatcaaaaagtggggattaagttaagcctcagactctaacagggctgggaaagttgtgaaaaccagatacggtctctaggacctagacacactaagtgtcatggattgaatgtctgtgcacccttcttcatatgttgaaaccctactccccagtgagatggtacggggagatggggcctttggga

SEQ ID NO: 12163 - RNA, 4304 nt, Homo sapiens
  source 1..4304: mol_type = other RNA
ctgcagccacttggggaactggtgtctgaccctggcatgctgtactgctctggctggcagatatttacagagaccagaggtgggactttctgctgggttgggtgatggtggaatccggatgtgatcttatgagtgggtagatggggagtcattttgtatgtgtgccaggggaggaggtggaacagactgtctctcgtgtttcttacaaggtgttaacaacttatcaggatctgccatttgagggtgcagaaagaggctgtgagtacatccttacaaccttatctcgccctcacctccatatttcccatttccttctgcaggaaaaccacctaggccattggcctggcagggcctgggacagcctctggctgtggtgccttccccatagctctttcttgctgcaggctccagctcccactgtttcctaaagcttaaagctgcccacctcctccccatgcctgggcttctgttctttttcatcctgtctgcagagcagggcatgatctctgagtttcttcttccttccttgttgtccccaaagagcagcacacaggcccttttccttctgaggccatggttctcagctttgtctccactttagaatctcctgaggagctgcagaaaaaatactccaactccatccccatccctagagtcagattccaatagtctgggatgaggcctgggcagcgccatttcaaaagctccccaggtgatattaatgtgcagccacagatgggaacattggatttaaaggttcctgctgtctatacatcagggaatcgggcaggggagaccctgataacagacggggaagggacaaagggttaatagacgtcaaaggtcttccaggagccctgagtctccttcatgcattactctcttaggagaaaataatggcactggttcacaccacagctcaaggcacagtgccaagtgctttatgtgtattacttcactgaatcctcaggaccaccttaggagatattatcagtaacttcattttacattgaggaaactgaggcatcaagaggttaagcaatgggtccaagagtacacaaacagcaagtggcatagctgggatttgaactcaggcatgcagctggccatcaaccactatgccctggctgccaagcatcaaaccgagtactgctctaagacgttcccttcatacctggaagagccctcattccacaccccaggtctggaaatgtgcactggggctgaaaaaaatggtgtcacttagtttccactcaggtgtcctttgccctaaatgggtcatttgtttttgagggaactccatttaagggctggcagtcaccttccagaggagacagagagctgcagtggttacaaaatggactctggtcggacagacctggatgtgtgtcccagctccgcacttacatgctggtgactgtagacaaggcttccctcctgtctagcgctggtctcctgtgtgtcaagtgggataatcacaccgagttcctggagttgggagggtgaggtgagagtgcataggtgaggtgcctggtacagagcctggccaagcctccagcccaccctctatcaggagtgccttctaggccatggcgtggacccctttgtcatgcctttggcagtctggcacggcttagggaccctttctaggaaaaaaataggtgggagatctttgggggtagaaaatagtagctattattttgtgtttttaaagttttattttatttttcattgacaaataattgtatatatttatagggtacattgtgaggttttgatacatgtatacattgtggaatggtcaaatcagggaaattagtatatccatgacctcaaataggtatcattatgatcatttatcacacatttattatgtgtgagaatatttaaaatctaagacattggtcaataggcactaagttacagttagagaggaggaaaaagttttggtgtcctattgcacaacataggcaactatagttaataacaatgtattgcatatttcaaaaaatgcttctaaatgtattagataaattacctaggattataaaggaaactgattactgtatcttgagatgcaatttacaatatagtcatatgtgcttcttgattaacaccttcaatataacacgatcaagcagtgggtctaatgactattatcattttgaagtggtgatgagcatagatgattttctgagatccctgccacaaccgtaatgtgatatgaaaatagctgtgattctagtagtgacagtcacagatgctgctaatagcactgtggcttactgccccagaaacagctttgtgtgctcttttgttctttagctatgtgatctagaccacccactcagcctctctgtgcccgtcctcatctgtgaaatgaaggtacctgtgaggatgaaatgagttaatgaaccagcaaaaatggctcaaacaccatgcagagtactgtgccatttgtattcttttgggatctgggatcttcaaatgtctcctttaaaatactgccaaggccacatcttcctaggtcaagaagtaagcccgtgtttcaaggactgccaactcttgggcttcacctgaggagaagtccccagggcctctcctggtagccccatttgtagcctcagtcgctgtccttacctcaccaccaaaccattatagttacaagccctaccatagatctcagcttcctgtgtaagagttcagaattttcctacaaacttctaacaaattaaagactgatttggaaacccacagcgctccctaatttgttatagttgttaggggtcagggaggggtttagggagcatcagagccatctctttactgtgcagatgtggcaactgaaacagaaagagaccctaaggtcacatggaagcttgttggcagtgttaggcctgggacccaagattcctctccctcaggcctcctagggcacagtcaaatctccatcctctttggttcctcctccttcatcctcaccatctcatcagttgacagttcccgtcggttccatttcctcctaaatatgtcaccaatctgtcagctcctgccttggctcaggccctctcccactctactcctactggcactgctgcctcggcctccccaccagcctccctgcctccagtctcaacctccaatagaaccttcctaatccatgcttctcttcctgttgcatgccaagaatgtcaagagctcagaggaagcttgcagtccctgagtccaagctcctcactcaccaccccactccacatcctgccatgtcatagaggaggaaactgaggctgagccaggggaatggagctagccaagtctgatagtgaacaagaggtagagctgaaaccaaaactcaggtcaaagggtcatggaatttgagggctagaaagcttagtttagtgctattcccattacatcacccacctctgagaatcacacccccagatcctattgtttcaggtaacaactggaaatattgttttcatcaggaccataattgccacttccctttctaggcactcattttggaaaaagcagacaatactccatctccttctcccatttctccccaaggttcttgaagcaggcctccagcatccgccagcctgattttcttccttatctgttctaggcataggcaggccctgcctgttccccaaccattttcacacgtatttctactggcctgggcccaaagtcaatttgccaatcttatgtcattggacttccctgttgccttgaatttactagaatatattagaccatatttgtctcccctctgctgccccaacacctagtatcaagcctggcagagaatgaacattcagtctttaagaaataaatgaatgaataaaagaaaatgctggtattgcaaaggataaagaaaagaataagacacagacagtcctgccttccaggagcttagagtttacttatgaagacaagatctagaaagtagtagaaatagtgaatggataaccaggcagccatgtttgactttcctttcaggccaagcagggacctggggtactgtatccaggctggaatgcaaagagctgttgggtgcaaggtataataggtaagtcatggaggtggggtgatctgaagcagcatctaggatcaaaaagtggggattaagttaagcctcagactctaacagggctgggaaagttgtgaaaaccagatacggtctctaggacctagacacactaagtgtcatggattgaatgtctgtgcacccttcttcatatgttgaaaccctactccccagtgagatggtacggggagatggggcctttgggagg

SEQ ID NO: 12164 - RNA, 64 nt, Homo sapiens
  source 1..64: mol_type = other RNA
ctgccatgtctaagaagaaaactttggagaaaaattttcttcttagacatggcaacgtcaacag

SEQ ID NO: 12165 - RNA, 4039 nt, Homo sapiens
  source 1..4039: mol_type = other RNA
ctgcgcaagctactgccttgcttggggctttatttggagactgaaaatggtttaaggggatgcggatggatgccaagttgacaaggggtggacctgtggacttcattttgggtgtgaactcgactgggttaagggatacctagagacctgggagatcattattctgggcatgtctgtgaggtgtttccagagattagtgtgtgaatctgaggggcctaggtgtggaagatccaccctcaatgttggtgggcagcattcaatctgctgaggcccagggagaacaaataaagaaggcaaactggtctctctctcagagctgggacaggcttttcttccactgccttgacatcagagcttcaggctcgctggcctttggactctggaacttacacccatggccctcctgggtcctgaggctttcgtcctgagccaccctgccggcatcccaggttgactgtgtgtgtaagcattgtgcgtgtgtataaaaacgtcaaaacttcctcaataaatgaagagatgtaatttttgtacatctgcaattgtgagagatgaaagttcttgccatctccgctctttgggcaactgtgtgtgtggtggtgacgcatcatagattgacttcgtcaaaagacttaggttgttggtcatgatatgactgcaagtataaagcgaggtgcacacaattaccaagcatagtgacatgcatgtatacatttcccattttgacctatttcttcatgaatatagtttgtctgctaataactcacaccggtgtaactgtctgtatacctgtttatgcttccaaaaatatgtattattgcctattttattgtgtgaagtggctgatgtgttctgttgtgtttttatgtttctcaaataaatccttttaaaatgtaagtatcttttaaaaaattaaaaaaaaattttcccagaattatatttccaggatttagatcttttgggattgtgattttcggattttagagtatagtaattttaatattttggattctcaacacttgggactatggcatttgggattgcgtcttttgggattcacacacatcccaggcagactcattggctctctgcttcccatttacaatgtgcagctctttctccccctcagtttcaagccctagcccctctctccagcccctgcatgaggagcagctaggtggttgcagcttcgcgctgtctttggcggtgggctgcctgagctggtgggttcaggcaaggatgcctccacatgaacatgctaccctctgcatgcctgagtcctgccaccccccacccccaacacagtccccacatcagggacaaaagatagagatttgagtcctaggctctcctgaaagtggtcatgaagacacatgcagttcctggtgcatgtgagcctgtcctacagatggggctcagccatggctggcccagaggcccccacttctggctggccacagaggaggccctcacgggccaggaggctgcagcggcattctggggcacttgcagagacccccccttcctgctggctgttcaaagtgaggcccaggctttctggatggtggccctgggaactccaccgggcagcaggggctgagcggggctcagagtccagctggctgccgtgtgccacctgctccacagcctctgtgctgagctgcaagggctggtcctccacagaggcccaggcctggacacctagcccggtgggctccaccctgagccagctcaggtcctggacacgatctcgacacctctggtcctgtgtgctggctgagtagggtaggccatggatggtggtcatgctgggggagctgctggactgtttctgctccagcatgtcagggcccctggcccagcgctgcccaaagagcccactgcccatgtcttgccttggaggccatgcggccgggggctgttcgtttgagctgatcttcagggctgccacacgggccacacagcctgccagcatgggctctgcatccagagtgtcacctccgtgacctggcctccaggggcctcggaaacaccccaggacccctggtggcccaggctccttctgggagcagggccaggtagaaggaactggggccttatttttaccggaagtatctgttgtcgaagtggctgcagactccatagaggagaacaagccttcagagtgacctcgtgtctcttcctctcgagaggcatccctggacagtgtgccagtcccttgtgtggcccctccgagggccttgctctctccggcgagcaggcctgtggtgcccgggtgtgcccacagctcctgcctgctgggtgctgagcaaactgtcgccccccctgcatctgaggccaggccctccctgccccccagcttctctgtgggtgccctaggggctccctgggaaccaggtggagctgcaggctgcccaggggtgggtggggcacggggcgtggggcctcggcgcagccagctgacgatgcccatggtgatggcgagctcagtgtcacacagcttcagcaggcactccttgcccttccaggagctctgtaggaagccctggctgagcaggtcagggcctggtgctggggccaagttctcctcggcccccactcggaagctgcatatggacagtggcgtccccagggccggccctgacagactctcagacacgcacaggtcatcatctgggctggggccaagaggaccctcgctggggtcgtggaagagctcgtagagggcgtccccactgtagctgtcccgtgggaaggtggcggcaggagtgcctgggctctcagcttccttcttgtcctcctcaagtcctggcgagaaggaatcatagtagccctcgtcacttgtggacacggattcgggctgctcgctcttgggggtgcctgtgtcgatggagctggctttggagccgctgcgagggtccctgcaggggcagaggggcagctcagcgagcccagctgtgtccagccgggattggtccctgtctgtcccctgggggcctgaaagccacgggcctaggagggcacgctgctgctgacgcactgagcgattcacactgtcccagaacctggtgaagtcagaggcttcattctgggcgggcgaggccagctgctccacactgccctggagagggcccctgggaaccttgctctccaggccctgagcagcctgggttgggctctccgggccctcgttcagctccagagatggcaccgagctctcatctgcgaacacctccccacaacccgtgagcgagtcgaagctctggagtgaggccacgtcctcacacagggccctgcagagaccaaaggatgcatcggccaggagctcgctgtccaacaggtcctggcacaggccgtccagccccggcccctcacccggggggaggaaggctttgcttcgccgccccccagggtctgacgggtcccctggggagggcaggcttttcccctcggccgccagcgaggccaagtcctcagtcttgtttctccgaatgtggaataggttccgaaagcacttcttgggcctcttcagggaaatcctcttcctcgggatgctcttggccacagctggcacaaagggcatctggggcacaaagtggcggtagtcgatcatgcgccggctgcccggggagcccgggaagcttgcactgcccaccagctgccctgtggcagccgtggccctgcctgccccagacatgctgtcgtgagtcttgcactttcgcaccggtttgaaggtggctccacagagggctgcgggtccccctttggggtccagctgcgcccctttgttggggcatctgtcgtattcttgggcactggggctggcttgggggcccttctcactgtggggcctctgttgccctcctggaaggactgaccaggggcctgtcccctccctggctgcagccacggctgctgggtctgggggtttctcgtgggaaacctgcaggctggacttgatgaaggtctttcctctcttcagctccatgctgccagtgccccagcgctgggggcccgcagtgcagcagggcgcggccgcgac

SEQ ID NO: 12166 - RNA, 4270 nt, Homo sapiens
  source 1..4270: mol_type = other RNA
ctgcgcaagctactgccttgcttggggctttatttggagactgaaaatggtttaaggggatgcggatggatgccaagttgacaaggggtggacctgtggacttcattttgggtgtgaactcgactgggttaagggatacctagagacctgggagatcattattctgggcatgtctgtgaggtgtttccagagattagtgtgtgaatctgaggggcctaggtgtggaagatccaccctcaatgttggtgggcagcattcaatctgctgaggcccagggagaacaaataaagaaggcaaactggtctctctctcagagctgggacaggcttttcttccactgccttgacatcagagcttcaggctcgctggcctttggactctggaacttacacccatggccctcctgggtcctgaggctttcgtcctgagccaccctgccggcatcccaggttgactgtgtgtgtaagcattgtgcgtgtgtataaaaacgtcaaaacttcctcaataaatgaagagatgtaatttttgtacatctgcaattgtgagagatgaaagttcttgccatctccgctctttgggcaactgtgtgtgtggtggtgacgcatcatagattgacttcgtcaaaagacttaggttgttggtcatgatatgactgcaagtataaagcgaggtgcacacaattaccaagcatagtgacatgcatgtatacatttcccattttgacctatttcttcatgaatatagtttgtctgctaataactcacaccggtgtaactgtctgtatacctgtttatgcttccaaaaatatgtattattgcctattttattgtgtgaagtggctgatgtgttctgttgtgtttttatgtttctcaaataaatccttttaaaatgtaagtatcttttaaaaaattaaaaaaaaattttcccagaattatatttccaggatttagatcttttgggattgtgattttcggattttagagtatagtaattttaatattttggattctcaacacttgggactatggcatttgggattgcgtcttttgggattcacacacatcccaggcagactcattggctctctgcttcccatttacaatgtgcagctctttctccccctcagtttcaagccctagcccctctctccagcccctgcatgaggagcagctaggtggttgcagcttcgcgctgtctttggcggtgggctgcctgagctggtgggttcaggcaaggatgcctccacatgaacatgctaccctctgcatgcctgagtcctgccaccccccacccccaacacagtccccacatcagggacaaaagatagagatttgagtcctaggctctcctgaaagtggtcatgaagacacatgcagttcctggtgcatgtgagcctgtcctacagatggggctcagccatggctggcccagaggcccccacttctggctggccacagaggaggccctcacgggccaggaggctgcagcggcattctggggcacttgcagagacccccccttcctgctggctgttcaaagtgaggcccaggctttctggatggtggccctgggaactccaccgggcagcaggggctgagcggggctcagagtccagctggctgccgtgtgccacctgctccacagcctctgtgctgagctgcaagggctggtcctccacagaggcccaggcctggacacctagcccggtgggctccaccctgagccagctcaggtcctggacacgatctcgacacctctggtcctgtgtgctggctgagtagggtaggccatggatggtggtcatgctgggggagctgctggactgtttctgctccagcatgtcagggcccctggcccagcgctgcccaaagagcccactgcccatgtcttgccttggaggccatgcggccgggggctgttcgtttgagctgatcttcagggctgccacacgggccacacagcctgccagcatgggctctgcatccagagtgtcacctccgtgacctggcctccaggggcctcggaaacaccccaggacccctggtggcccaggctccttctgggagcagggccaggtagaaggaactggggccttatttttaccggaagtatctgttgtcgaagtggctgcagactccatagaggagaacaagccttcagagtgacctcgtgtctcttcctctcgagaggcatccctggacagtgtgccagtcccttgtgtggcccctccgagggccttgctctctccggcgagcaggcctgtggtgcccgggtgtgcccacagctcctgcctgctgggtgctgagcaaactgtcgccccccctgcatctgaggccaggccctccctgccccccagcttctctgtgggtgccctaggggctccctgggaaccaggtggagctgcaggctgcccaggggtgggtggggcacggggcgtggggcctcggcgcagccagctgacgatgcccatggtgatggcgagctcagtgtcacacagcttcagcaggcactccttgcccttccaggagctctgtaggaagccctggctgagcaggtcagggcctggtgctggggccaagttctcctcggcccccactcggaagctgcatatggacagtggcgtccccagggccggccctgacagactctcagacacgcacaggtcatcatctgggctggggccaagaggaccctcgctggggtcgtggaagagctcgtagagggcgtccccactgtagctgtcccgtgggaaggtggcggcaggagtgcctgggctctcagcttccttcttgtcctcctcaagtcctggcgagaaggaatcatagtagccctcgtcacttgtggacacggattcgggctgctcgctcttgggggtgcctgtgtcgatggagctggctttggagccgctgcgagggtccctgcaggggcagaggggcagctcagcgagcccagctgtgtccagccgggattggtccctgtctgtcccctgggggcctgaaagccacgggcctaggagggcacgctgctgctgacgcactgagcgattcacactgtcccagaacctggtgaagtcagaggcttcattctgggcgggcgaggccagctgctccacactgccctggagagggcccctgggaaccttgctctccaggccctgagcagcctgggttgggctctccgggccctcgttcagctccagagatggcaccgagctctcatctgcgaacacctccccacaacccgtgagcgagtcgaagctctggagtgaggccacgtcctcacacagggccctgcagagaccaaaggatgcatcggccaggagctcgctgtccaacaggtcctggcacaggccgtccagccccggcccctcacccggggggaggaaggctttgcttcgccgccccccagggtctgacgggtcccctggggagggcaggcttttcccctcggccgccagcgaggccaagtcctcagtcttgtttctccgaatgtggaataggttccgaaagcacttcttgggcctcttcagggaaatcctcttcctcgggatgctcttggccacagctggcacaaagggcatctggggcacaaagtggcggtagtcgatcatgcgccggctgcccggggagcccgggaagcttgcactgcccaccagctgccctgtggcagccgtggccctgcctgccccagacatgctgtcgtgagtcttgcactttcgcaccggtttgaaggtggctccacagagggctgcgggtccccctttggggtccagctgcgcccctttgttggggcatctgtcgtattcttgggcactggggctggcttgggggcccttctcactgtggggcctctgttgccctcctggaaggactgaccaggggcctgtcccctccctggctgcagccacggctgctgggtctgggggtttctcgtgggaaacctgcaggctggacttgatgaaggtctttcctctcttcagctccatgctgccagtgccccagctgccagggttcggagcgggcctgcaagaaggggcaggccaggctggggctgcaaggcagggtcttcccttggagaagggacctgactctattattaagagaacgaaagaggcacttgccctacaggtactcactgtgtggggtctactggtgctgtgctctgccgcagtcttgagggaggagcagaaatgctgtggggactctgtctccgcagaactgaggacgaggggtctgcacgcgtggttcagtgcctggggctggggtggatt

SEQ ID NO: 12167 - RNA, 4042 nt, Homo sapiens
  source 1..4042: mol_type = other RNA
ctgcgcaagctactgccttgcttggggctttatttggagactgaaaatggtttaaggggatgcggatggatgccaagttgacaaggggtggacctgtggacttcattttgggtgtgaactcgactgggttaagggatacctagagacctgggagatcattattctgggcatgtctgtgaggtgtttccagagattagtgtgtgaatctgaggggcctaggtgtggaagatccaccctcaatgttggtgggcagcattcaatctgctgaggcccagggagaacaaataaagaaggcaaactggtctctctctcagagctgggacaggcttttcttccactgccttgacatcagagcttcaggctcgctggcctttggactctggaacttacacccatggccctcctgggtcctgaggctttcgtcctgagccaccctgccggcatcccaggttgactgtgtgtgtaagcattgtgcgtgtgtataaaaacgtcaaaacttcctcaataaatgaagagatgtaatttttgtacatctgcaattgtgagagatgaaagttcttgccatctccgctctttgggcaactgtgtgtgtggtggtgacgcatcatagattgacttcgtcaaaagacttaggttgttggtcatgatatgactgcaagtataaagcgaggtgcacacaattaccaagcatagtgacatgcatgtatacatttcccattttgacctatttcttcatgaatatagtttgtctgctaataactcacaccggtgtaactgtctgtatacctgtttatgcttccaaaaatatgtattattgcctattttattgtgtgaagtggctgatgtgttctgttgtgtttttatgtttctcaaataaatccttttaaaatgtaagtatcttttaaaaaattaaaaaaaaattttcccagaattatatttccaggatttagatcttttgggattgtgattttcggattttagagtatagtaattttaatattttggattctcaacacttgggactatggcatttgggattgcgtcttttgggattcacacacatcccaggcagactcattggctctctgcttcccatttacaatgtgcagctctttctccccctcagtttcaagccctagcccctctctccagcccctgcatgaggagcagctaggtggttgcagcttcgcgctgtctttggcggtgggctgcctgagctggtgggttcaggcaaggatgcctccacatgaacatgctaccctctgcatgcctgagtcctgccaccccccacccccaacacagtccccacatcagggacaaaagatagagatttgagtcctaggctctcctgaaagtggtcatgaagacacatgcagttcctggtgcatgtgagcctgtcctacagatggggctcagccatggctggcccagaggcccccacttctggctggccacagaggaggccctcacgggccaggaggctgcagcggcattctggggcacttgcagagacccccccttcctgctggctgttcaaagtgaggcccaggctttctggatggtggccctgggaactccaccgggcagcaggggctgagcggggctcagagtccagctggctgccgtgtgccacctgctccacagcctctgtgctgagctgcaagggctggtcctccacagaggcccaggcctggacacctagcccggtgggctccaccctgagccagctcaggtcctggacacgatctcgacacctctggtcctgtgtgctggctgagtagggtaggccatggatggtggtcatgctgggggagctgctggactgtttctgctccagcatgtcagggcccctggcccagcgctgcccaaagagcccactgcccatgtcttgccttggaggccatgcggccgggggctgttcgtttgagctgatcttcagggctgccacacgggccacacagcctgccagcatgggctctgcatccagagtgtcacctccgtgacctggcctccaggggcctcggaaacaccccaggacccctggtggcccaggctccttctgggagcagggccaggtagaaggaactggggccttatttttaccggaagtatctgttgtcgaagtggctgcagactccatagaggagaacaagccttcagagtgacctcgtgtctcttcctctcgagaggcatccctggacagtgtgccagtcccttgtgtggcccctccgagggccttgctctctccggcgagcaggcctgtggtgcccgggtgtgcccacagctcctgcctgctgggtgctgagcaaactgtcgccccccctgcatctgaggccaggccctccctgccccccagcttctctgtgggtgccctaggggctccctgggaaccaggtggagctgcaggctgcccaggggtgggtggggcacggggcgtggggcctcggcgcagccagctgacgatgcccatggtgatggcgagctcagtgtcacacagcttcagcaggcactccttgcccttccaggagctctgtaggaagccctggctgagcaggtcagggcctggtgctggggccaagttctcctcggcccccactcggaagctgcatatggacagtggcgtccccagggccggccctgacagactctcagacacgcacaggtcatcatctgggctggggccaagaggaccctcgctggggtcgtggaagagctcgtagagggcgtccccactgtagctgtcccgtgggaaggtggcggcaggagtgcctgggctctcagcttccttcttgtcctcctcaagtcctggcgagaaggaatcatagtagccctcgtcacttgtggacacggattcgggctgctcgctcttgggggtgcctgtgtcgatggagctggctttggagccgctgcgagggtccctgcaggggcagaggggcagctcagcgagcccagctgtgtccagccgggattggtccctgtctgtcccctgggggcctgaaagccacgggcctaggagggcacgctgctgctgacgcactgagcgattcacactgtcccagaacctggtgaagtcagaggcttcattctgggcgggcgaggccagctgctccacactgccctggagagggcccctgggaaccttgctctccaggccctgagcagcctgggttgggctctccgggccctcgttcagctccagagatggcaccgagctctcatctgcgaacacctccccacaacccgtgagcgagtcgaagctctggagtgaggccacgtcctcacacagggccctgcagagaccaaaggatgcatcggccaggagctcgctgtccaacaggtcctggcacaggccgtccagccccggcccctcacccggggggaggaaggctttgcttcgccgccccccagggtctgacgggtcccctggggagggcaggcttttcccctcggccgccagcgaggccaagtcctcagtcttgtttctccgaatgtggaataggttccgaaagcacttcttgggcctcttcagggaaatcctcttcctcgggatgctcttggccacagctggcacaaagggcatctggggcacaaagtggcggtagtcgatcatgcgccggctgcccggggagcccgggaagcttgcactgcccaccagctgccctgtggcagccgtggccctgcctgccccagacatgctgtcgtgagtcttgcactttcgcaccggtttgaaggtggctccacagagggctgcgggtccccctttggggtccagctgcgcccctttgttggggcatctgtcgtattcttgggcactggggctggcttgggggcccttctcactgtggggcctctgttgccctcctggaaggactgaccaggggcctgtcccctccctggctgcagccacggctgctgggtctgggggtttctcgtgggaaacctgcaggctggacttgatgaaggtctttcctctcttcagctccatgctgccagtgccccagctgcgctgggggcccgcagtgcagcagggcgcggccgcgac

SEQ ID NO: 12168 - RNA, 4139 nt, Homo sapiens
  source 1..4139: mol_type = other RNA
ctgcgcaagctactgccttgcttggggctttatttggagactgaaaatggtttaaggggatgcggatggatgccaagttgacaaggggtggacctgtggacttcattttgggtgtgaactcgactgggttaagggatacctagagacctgggagatcattattctgggcatgtctgtgaggtgtttccagagattagtgtgtgaatctgaggggcctaggtgtggaagatccaccctcaatgttggtgggcagcattcaatctgctgaggcccagggagaacaaataaagaaggcaaactggtctctctctcagagctgggacaggcttttcttccactgccttgacatcagagcttcaggctcgctggcctttggactctggaacttacacccatggccctcctgggtcctgaggctttcgtcctgagccaccctgccggcatcccaggttgactgtgtgtgtaagcattgtgcgtgtgtataaaaacgtcaaaacttcctcaataaatgaagagatgtaatttttgtacatctgcaattgtgagagatgaaagttcttgccatctccgctctttgggcaactgtgtgtgtggtggtgacgcatcatagattgacttcgtcaaaagacttaggttgttggtcatgatatgactgcaagtataaagcgaggtgcacacaattaccaagcatagtgacatgcatgtatacatttcccattttgacctatttcttcatgaatatagtttgtctgctaataactcacaccggtgtaactgtctgtatacctgtttatgcttccaaaaatatgtattattgcctattttattgtgtgaagtggctgatgtgttctgttgtgtttttatgtttctcaaataaatccttttaaaatgtaagtatcttttaaaaaattaaaaaaaaattttcccagaattatatttccaggatttagatcttttgggattgtgattttcggattttagagtatagtaattttaatattttggattctcaacacttgggactatggcatttgggattgcgtcttttgggattcacacacatcccaggcagactcattggctctctgcttcccatttacaatgtgcagctctttctccccctcagtttcaagccctagcccctctctccagcccctgcatgaggagcagctaggtggttgcagcttcgcgctgtctttggcggtgggctgcctgagctggtgggttcaggcaaggatgcctccacatgaacatgctaccctctgcatgcctgagtcctgccaccccccacccccaacacagtccccacatcagggacaaaagatagagatttgagtcctaggctctcctgaaagtggtcatgaagacacatgcagttcctggtgcatgtgagcctgtcctacagatggggctcagccatggctggcccagaggcccccacttctggctggccacagaggaggccctcacgggccaggaggctgcagcggcattctggggcacttgcagagacccccccttcctgctggctgttcaaagtgaggcccaggctttctggatggtggccctgggaactccaccgggcagcaggggctgagcggggctcagagtccagctggctgccgtgtgccacctgctccacagcctctgtgctgagctgcaagggctggtcctccacagaggcccaggcctggacacctagcccggtgggctccaccctgagccagctcaggtcctggacacgatctcgacacctctggtcctgtgtgctggctgagtagggtaggccatggatggtggtcatgctgggggagctgctggactgtttctgctccagcatgtcagggcccctggcccagcgctgcccaaagagcccactgcccatgtcttgccttggaggccatgcggccgggggctgttcgtttgagctgatcttcagggctgccacacgggccacacagcctgccagcatgggctctgcatccagagtgtcacctccgtgacctggcctccaggggcctcggaaacaccccaggacccctggtggcccaggctccttctgggagcagggccaggtagaaggaactggggccttatttttaccggaagtatctgttgtcgaagtggctgcagactccatagaggagaacaagccttcagagtgacctcgtgtctcttcctctcgagaggcatccctggacagtgtgccagtcccttgtgtggcccctccgagggccttgctctctccggcgagcaggcctgtggtgcccgggtgtgcccacagctcctgcctgctgggtgctgagcaaactgtcgccccccctgcatctgaggccaggccctccctgccccccagcttctctgtgggtgccctaggggctccctgggaaccaggtggagctgcaggctgcccaggggtgggtggggcacggggcgtggggcctcggcgcagccagctgacgatgcccatggtgatggcgagctcagtgtcacacagcttcagcaggcactccttgcccttccaggagctctgtaggaagccctggctgagcaggtcagggcctggtgctggggccaagttctcctcggcccccactcggaagctgcatatggacagtggcgtccccagggccggccctgacagactctcagacacgcacaggtcatcatctgggctggggccaagaggaccctcgctggggtcgtggaagagctcgtagagggcgtccccactgtagctgtcccgtgggaaggtggcggcaggagtgcctgggctctcagcttccttcttgtcctcctcaagtcctggcgagaaggaatcatagtagccctcgtcacttgtggacacggattcgggctgctcgctcttgggggtgcctgtgtcgatggagctggctttggagccgctgcgagggtccctgcaggggcagaggggcagctcagcgagcccagctgtgtccagccgggattggtccctgtctgtcccctgggggcctgaaagccacgggcctaggagggcacgctgctgctgacgcactgagcgattcacactgtcccagaacctggtgaagtcagaggcttcattctgggcgggcgaggccagctgctccacactgccctggagagggcccctgggaaccttgctctccaggccctgagcagcctgggttgggctctccgggccctcgttcagctccagagatggcaccgagctctcatctgcgaacacctccccacaacccgtgagcgagtcgaagctctggagtgaggccacgtcctcacacagggccctgcagagaccaaaggatgcatcggccaggagctcgctgtccaacaggtcctggcacaggccgtccagccccggcccctcacccggggggaggaaggctttgcttcgccgccccccagggtctgacgggtcccctggggagggcaggcttttcccctcggccgccagcgaggccaagtcctcagtcttgtttctccgaatgtggaataggttccgaaagcacttcttgggcctcttcagggaaatcctcttcctcgggatgctcttggccacagctggcacaaagggcatctggggcacaaagtggcggtagtcgatcatgcgccggctgcccggggagcccgggaagcttgcactgcccaccagctgccctgtggcagccgtggccctgcctgccccagacatgctgtcgtgagtcttgcactttcgcaccggtttgaaggtggctccacagagggctgcgggtccccctttggggtccagctgcgcccctttgttggggcatctgtcgtattcttgggcactggggctggcttgggggcccttctcactgtggggcctctgttgccctcctggaaggactgaccaggggcctgtcccctccctggctgcagccacggctgctgggtctgggggtttctcgtgggaaacctgcaggctggacttgatgaaggtctttcctctcttcagctccatgctgccagtgccccagctgtgtgtggggtctactggtgctgtgctctgccgcagtcttgagggaggagcagaaatgctgtggggactctgtctccgcagaactgaggacgaggggtctgcacgcgtggttcagtgcctggggctggggtggatt

SEQ ID NO: 12169 - RNA, 5201 nt, Homo sapiens
  source 1..5201: mol_type = other RNA
ctgcgcaagctactgccttgcttggggctttatttggagactgaaaatggtttaaggggatgcggatggatgccaagttgacaaggggtggacctgtggacttcattttgggtgtgaactcgactgggttaagggatacctagagacctgggagatcattattctgggcatgtctgtgaggtgtttccagagattagtgtgtgaatctgaggggcctaggtgtggaagatccaccctcaatgttggtgggcagcattcaatctgctgaggcccagggagaacaaataaagaaggcaaactggtctctctctcagagctgggacaggcttttcttccactgccttgacatcagagcttcaggctcgctggcctttggactctggaacttacacccatggccctcctgggtcctgaggctttcgtcctgagccaccctgccggcatcccaggttgactgtgtgtgtaagcattgtgcgtgtgtataaaaacgtcaaaacttcctcaataaatgaagagatgtaatttttgtacatctgcaattgtgagagatgaaagttcttgccatctccgctctttgggcaactgtgtgtgtggtggtgacgcatcatagattgacttcgtcaaaagacttaggttgttggtcatgatatgactgcaagtataaagcgaggtgcacacaattaccaagcatagtgacatgcatgtatacatttcccattttgacctatttcttcatgaatatagtttgtctgctaataactcacaccggtgtaactgtctgtatacctgtttatgcttccaaaaatatgtattattgcctattttattgtgtgaagtggctgatgtgttctgttgtgtttttatgtttctcaaataaatccttttaaaatgtaagtatcttttaaaaaattaaaaaaaaattttcccagaattatatttccaggatttagatcttttgggattgtgattttcggattttagagtatagtaattttaatattttggattctcaacacttgggactatggcatttgggattgcgtcttttgggattcacacacatcccaggcagactcattggctctctgcttcccatttacaatgtgcagctctttctccccctcagtttcaagccctagcccctctctccagcccctgcatgaggagcagctaggtggttgcagcttcgcgctgtctttggcggtgggctgcctgagctggtgggttcaggcaaggatgcctccacatgaacatgctaccctctgcatgcctgagtcctgccaccccccacccccaacacagtccccacatcagggacaaaagatagagatttgagtcctaggctctcctgaaagtggtcatgaagacacatgcagttcctggtgcatgtgagcctgtcctacagatggggctcagccatggctggcccagaggcccccacttctggctggccacagaggaggccctcacgggccaggaggctgcagcggcattctggggcacttgcagagacccccccttcctgctggctgttcaaagtgaggcccaggctttctggatggtggccctgggaactccaccgggcagcaggggctgagcggggctcagagtccagctggctgccgtgtgccacctgctccacagcctctgtgctgagctgcaagggctggtcctccacagaggcccaggcctggacacctagcccggtgggctccaccctgagccagctcaggtcctggacacgatctcgacacctctggtcctgtgtgctggctgagtagggtaggccatggatggtggtcatgctgggggagctgctggactgtttctgctccagcatgtcagggcccctggcccagcgctgcccaaagagcccactgcccatgtcttgccttggaggccatgcggccgggggctgttcgtttgagctgatcttcagggctgccacacgggccacacagcctgccagcatgggctctgcatccagagtgtcacctccgtgacctggcctccaggggcctcggaaacaccccaggacccctggtggcccaggctccttctgggagcagggccaggtagaaggaactggggccttatttttaccggaagtatctgttgtcgaagtggctgcagactccatagaggagaacaagccttcagagtgacctcgtgtctcttcctctcgagaggcatccctggacagtgtgccagtcccttgtgtggcccctccgagggccttgctctctccggcgagcaggcctgtggtgcccgggtgtgcccacagctcctgcctgctgggtgctgagcaaactgtcgccccccctgcatctgaggccaggccctccctgccccccagcttctctgtgggtgccctaggggctccctgggaaccaggtggagctgcaggctgcccaggggtgggtggggcacggggcgtggggcctcggcgcagccagctgacgatgcccatggtgatggcgagctcagtgtcacacagcttcagcaggcactccttgcccttccaggagctctgtaggaagccctggctgagcaggtcagggcctggtgctggggccaagttctcctcggcccccactcggaagctgcatatggacagtggcgtccccagggccggccctgacagactctcagacacgcacaggtcatcatctgggctggggccaagaggaccctcgctggggtcgtggaagagctcgtagagggcgtccccactgtagctgtcccgtgggaaggtggcggcaggagtgcctgggctctcagcttccttcttgtcctcctcaagtcctggcgagaaggaatcatagtagccctcgtcacttgtggacacggattcgggctgctcgctcttgggggtgcctgtgtcgatggagctggctttggagccgctgcgagggtccctgcaggggcagaggggcagctcagcgagcccagctgtgtccagccgggattggtccctgtctgtcccctgggggcctgaaagccacgggcctaggagggcacgctgctgctgacgcactgagcgattcacactgtcccagaacctggtgaagtcagaggcttcattctgggcgggcgaggccagctgctccacactgccctggagagggcccctgggaaccttgctctccaggccctgagcagcctgggttgggctctccgggccctcgttcagctccagagatggcaccgagctctcatctgcgaacacctccccacaacccgtgagcgagtcgaagctctggagtgaggccacgtcctcacacagggccctgcagagaccaaaggatgcatcggccaggagctcgctgtccaacaggtcctggcacaggccgtccagccccggcccctcacccggggggaggaaggctttgcttcgccgccccccagggtctgacgggtcccctggggagggcaggcttttcccctcggccgccagcgaggccaagtcctcagtcttgtttctccgaatgtggaataggttccgaaagcacttcttgggcctcttcagggaaatcctcttcctcgggatgctcttggccacagctggcacaaagggcatctggggcacaaagtggcggtagtcgatcatgcgccggctgcccggggagcccgggaagcttgcactgcccaccagctgccctgtggcagccgtggccctgcctgccccagacatgctgtcgtgagtcttgcactttcgcaccggtttgaaggtggctccacagagggctgcgggtccccctttggggtccagctgcgcccctttgttggggcatctgtcgtattcttgggcactggggctggcttgggggcccttctcactgtggggcctctgttgccctcctggaaggactgaccaggggcctgtcccctccctggctgcagccacggctgctgggtctgggggtttctcgtgggaaacctgcaggctggacttgatgaaggtctttcctctcttcagctccatgctgccagtgccccagtgtgtggggtctactggtgctgtgctctgccgcagtcttgagggaggagcagaaatgctgtggggactctgtctccgcagaactgaggacgaggggtctgcacgcgtggttcagtgcctggggctggggtggattaagtaactccaggaaggctcaggcagcagtgccagtagtgtggggcggggttgtggggaggaggggggagcgggagcgcacagtcggtgctggggagaggctgatgccaacaggaggctctcggccgtggtgtgcccaggcggggcaggacgggaggatgcaggagtcccgggtccacgctgaggctaaggctgaagggaaggcagagctcaggtggatgacggaggccaggcctttccctgagcttggtgggctccctcccggtcaccttgtctgagaacccaggacacagagtccccttgctttggactggtttggtttgtcattccccttgacatcgcctcgccccagagacaagaggccccttcatcctccagccaagaccttccccacccttgggtgacctaccctcttgcattttttagatttgagccctctttctatgcagcgactaactcaacgtgaccccagaggccccctcgcccatgttgctggtagtcttgaccttttttggcagatcctggctgtgggagttccctgtctttctcttaggtaggacagaaggcagtttctgcctcgttgccacatacaccccaagtcaggggtaggactcccgcagaccccacagtcctcctcttgttaaaattagtaagcattagccttccttattaggctctccccgcttttgcatttaaggattttttaatgtgtcttataaaatcatgtaattgtgaggataattacagattcagcttcttccagtgagtgacaattgctcattttcgatgctcacatggtcatcgttcggccactgcaaactgttccaacccttctactttgtcatttcagacagttttcaaacacccctaacttttgggtaacatgaaaatatatatttcaaattttttatttccccaagatgtgggatcaggtcttccccagggactcctggaaaaatcttttacactaggctacccagttcagataccactgaatgatttttcttaaatattattctaatgtgaacttacattttatttttacaatacactgacttacacgcct

SEQ ID NO: 12170 - RNA, 47 nt, Homo sapiens
  source 1..47: mol_type = other RNA
ctggactgagccgtgctactggcgcctcacgcgggtgcggcccgact

SEQ ID NO: 12171 - RNA, 1104 nt, Homo sapiens
  source 1..1104: mol_type = other RNA
ctggagatatggaagagctgtgtgcagaggtccagggatcggcaggcggacagccagaaagccaccatggaagccatgccaaagatgatgctgggcaagaagcagatggtgtagacggccaccaccatggccagcacacgcatggccctctgcgggcctgcctgcccgcccagaccacggttccggatggtgagcccaatgctcacaatagcaaagaggatgagcgccagtggcaggaagaactccagcaggtacagtgcctggtgccagcggagcgaggccgagggcttcgtgcccaccctgtagctgaggcaggaggggccggagaaggtgctcaggagcaggtgcccgttgaggagcaggatgcccacccagagtcccccggccacccgggcagctgcccccacggaagcacggctcagcacgtggtggggctgcaccaccttcaggtagcggttgagtgcgatggctgtgaggaagacaacgctggccgtgcggttggtggacagcatgaagaggttgactttgcaggcagcagccccaaagcgccaggtctcatggaggaggtagtagtccacgcggaggggcaggttgctgatcaggaggaagtcagcggccaccaggctgaccaggaacaccgtgttggaggtccagggccgcgtgtggatgcagaagatgaagagggccaaactgttccccaccaggcccaggacaaactccagggccaggattggtgccaggaaggcagacaccagcgaggaagaggtggggtggcagggccctccagaggacccccccacagtggtaaaggcagagggagcagaggagggtgagggagagaaggagggagggagaacagaggaggagagagagggagatggagagctcaggttatgaagttccatgggctgcttgggccatgggcctgagagaaggttctggagtcttctacccctgcaggagtgctcagggcaaagtgggatgattggcactatcagctggccaccacggtgacacaacatcctggggttttcatcagcattctcgcagccactgagaaacaccctgtgttcctgtttgcaggccaaggggaaccctgcagcc

SEQ ID NO: 12172 - RNA, 607 nt, Homo sapiens
  source 1..607: mol_type = other RNA
ctggatggctcctccatgtcttggagtagatcagtgggcagctcttccatttcctggagtgggccactggggggctccttcttttcctgggctgggccgctggctggccctgcctctccccgcactccactgcccgacgtcgcctcggtggtgttggatgagccctcggaggactccatttgttttgatgatggattcttatgctccatcatcgtctcaaatgagtcttcagagggttctatcatttcgtcggatggaaaggagtgtattctgaagattggtaaggttgtgatggcgtccagtcagtagctgggaccgtggagatcagaaccttggctgcaagcgttcaagtggatctcctcccgtcctgtgccactcgatcctcgctgcttgcttccccgggcccagtcccaagcgtgaggctggggatgaagtgatgccggtggcttagtgatgccggtggcttcctgtcctcgaagctcagtcggtcgtctctcagctggtgtgaggctgggccaggatggaaccccagactctccgaggctccccaccacaccctgctgctgaaggctgctcagcgaggctgtgccgagtgctgggggggtgt

SEQ ID NO: 12173 - RNA, 1434 nt, Homo sapiens
  source 1..1434: mol_type = other RNA
ctggcctcttctttctcctaggagtaagtcccctatttttagcaatttgataggtaatagctctctttgcattttgatcttcaagagcctgttcttcagtgctattttcttctttctttctctttagcttttgcctgtcttctatttctttatagtacttcagttttgctttttcatcaaaatcagaatcatcagaaagatctgtaacagcacaggcagcagcagaagtctttgaaacagactttggtttgggcttggtggattttgcttttggaatcagttctttctttacagcatcatccttaagtgtcaacagatgacgaatttctgaggacagcttctgatccacaacggacagcttgttgatcaaatttcggtaggtaacaagcctttctatgacaggatgtccatgtgctgggactctcctagctttcaggatcaaataaaaactgatgttcgagcaataattcaagtagaggttgtacttggtcctcaagtattggcttccttttccgggtggaatgatcccttgttccaccaactctaacaatggctccagctcatccttaacctctgtcaacttgactttcaggtcttctatcagctccaagagttctggtgattcctttcgcaacattttcagcttctctttcactgaaactttagccaaatccttcacgacccgtgtctcagcctcatctacctgaggcactggttttgcaaaggcctcaacccaggcgacaccaaaatcatcctcttgcagcgcttgggctaggcgccgctgaatgatctgtgcctcctcctcctcctctctttcctcctcctctgcctcctgttgactctgccggcctcgggacttggaaccatagtccgtgtcatagtaaagttttttcctctgaccccacgacaaactgggatccacagaggcctcagcttcactttgcacggagctcccaccatcatcatcggcattctcctcctcctcctcctcccccgcattccctccatcttcgtcgtcctcatcgtccatatctagggctagcacctcctcctcctcctcctcgccatcctcctcgtctccactctgtacttcattccagcccttagctaaggcggcccgggatcgtgcctcatgaaagtcatctacctgatcttggtagtagctggtgtcccctggtgagggtggcaatcctaaatcatctccattttcgtcggtgagcgtgggacctgccttggctcgcacagctgcccacttagctgctccgcgccgccgggatctccccaccatggctcacaatctcaggttttacagcgactccggactttcggccaccactgacttcggcgcaggaatcaggcgctccggtaactcgtggctctaaacagcagcgcgctcccctaccaccggagtttgcagactcctgatcggctact

SEQ ID NO: 12174 - RNA, 1425 nt, Homo sapiens
  source 1..1425: mol_type = other RNA
ctggcctcttctttctcctagtagctccgtgatgaacacaaatgcccttctcctgtcggaccctccagacactccagtccagtctaccttgggattgcggtcattactctcctcttgactttccttgtgcttcttgttctgtcctggtctctgtcagtcctttccctgtctgacgcgagtcccagctccttataccactcctgggaattctccagttcctgactcactgtctgcagcctgcaggctctgacagcaccgcaggtgtcagaaggcgcctcttatgttcaagggtcctgggcttccagcatgggagtagacggcaagttaccagtggccccaaatgttagatactgtggcttgattacagagaaataggagacagctccatgagatccaacagatggtctgattagggaagaaggaagccagtgcagaacacttacaaaataaccatgcttgatagtgagctgttttggacagggacggtttggcaggcccttctgaaatcttcacagccggcgtcaggcctggcactcagcagcacgcaacaaataattgttaaatgaataaataaaacataagggctggacacagtggctcacacctgtaatcccagcactttgggaggctgaggcgggtggattgcttgaggccaggtgtttgagaccagcctagccaacatgacaaaaccccgtctctgctaaaaatattatacaaaaattagccaggcgcggcgaagagtgcctgtaatctcagctacttagaaggctgaggcaggagaattacttgaacccaggaggcagaggttacagttagccaagatcgtgccactacactccagcctgggtgactctgtggtccgagctactcgagaggcagacgtgggaggatgtcttgagcccaggaggttaaggctgcagtgagctgtgattgtaccactgcactccagcctggacaacagaacaagatcccgattcttggtggtattcagagaggtttggtctgactgagctgcagcagctgtccgactcccaggggaaaaagcgaaaggctgagagaatcccagacactggcctgacacgttggaactgccgaaattccatgaaggatccagataatggccatcacatcatcatttaaggcaggacgtaaggactaaccatgtctcttctccagctctacatatttcatcctgagcagcaagggaggctgagaaagtgggcgctggagccttggcagcctctgttaagagggtcatccagggcttccttgccgcctcggtgcacagctcaatcatgcttccttcttgttcattttgacaaagcaggtgagtgatgagcaggaaaaaattatgaggaggtgttggagcaactcgctaatcagcactgctacaagatcgccagcatttacaggaccgcattcact

SEQ ID NO: 12175 - RNA, 576 nt, Homo sapiens
  source 1..576: mol_type = other RNA
ctgggacaggaggaggaggcagacgggcagtgggacccggccctctgcggcggcggggaggggccgcacctgcccgcctgtggcgccctgcccacccccatgccacgcaccgtccacgggggccacgcggtctgagggccccttccttgccggccccatgtgcatgagcgctcctcacgggctccagggcggccccgggacagcggctgatgctggctgtaggacccgacgcctgtttctctctctctctctgcccccatctgtctgctgtgtccctcaggtggccatcgcgggtgccccggtcaccgtctggatggccgaaattgccccgcagacgggctttatttgaaactgagaaattgcgtagaagaaaccgctgagtgctgaaggccctagcaggctccttcctaaggcgctggggccaagcattccctgaggaggcagcagtgaagggtgctagagtgagtggagccagccaggcttgggggaccgagcgggaggagagtgggggagtgggtggagccttggcagcaacgtggggctcagtctaggtgggcggggcttctgcgctaaggg

SEQ ID NO: 12176 - RNA, 1708 nt, Homo sapiens
  source 1..1708: mol_type = other RNA
ctgggacaggaggaggaggcagaggagaagagcacggaggtgggcgtggcgttctcctggcccgcccacagcggggggctagtctcggccacgccgtagtacacatcctgcttgcccacgccatagcccggaaagaggtacccgccgtagccaaagtccccgccctgctcacccaggcgtggggcctcaaagccagagtccactccgcactcgccgatgcagcccaggctgttctgccggaaggtggagaggggcttgcagccgggctggtgcacccgccaggcgtcggagtagcggctatcgattgctgcgtcggggctccccgccaggaagtcgttttcattgttgtactcgaggatcttgccagtgcgcaccgcgatgtgcgtctcgatctcctcgcgcgcacgctccacgttgcctggggcacccgtgatctcgaacacggggtcgcggtcacggcttggtgtgataatgtatgtgttggtttgctgctggatgcgcttgatggttgcccctttggggcccaccaccagccccaccacgcggtagggcacccgcacacggatggtcacctggccgggcagagcaggagccacaccaaaggcggcgcctgacttgttgcgggaggcacggatcatggagaagtgctccgctgctgagatgatttcccgccgggctgtggccacgtcctcccgtcgccctgtcaccatgaacactggttcctcgcccctcaccggtgtcttgatgtaggtgttggtcttggccctcaaggccttaatcttgcagccttgcctgcccacgatctcggccacgtgctcggaggtgggcacgggaacacactccgtggtgttgctgctgcccttcaggcgcagctcggcctctttgtagagagcgcagagcttggcgtcgctcgcccctttgggggcggtggggggctggggcgtctgcgctgcgggggccgccgtcggggcggccgggggcgccgcgggcggcggcggcggggccggctgcgggggggcggccggctgcgcgggggcgccgccccccccacctcccccgtcctcgcccgccgtgggggcggggggctcccccaaacccaggaggcagagttgatcgagagccagctgaagggcgcgctcgtcttccagcagccctcggtccttagcgcttcccccgaaacatcctagttctccaaagcccccatttctttccattattccagataccactagactaggcatggcgaaacaaaagctgggggagagagagagggagagagagagagagaggtggtggaagggaaaagaggagagaggaggggaggggagaggagaggagggggtgtgtggggaggggggaacaaagaactggggaggggggaagaaagcgagatagaaagatagaccctccccctaagcccccctccccaaacaccctgtaacccgactcccctcgccccagcccccggggtgggggtggggggaaagagaagcaaaaccaagaaagcagatctcctctcctctccgggggtgacggggggcggggggctgcaggatctctgcccccacccctcccgcctcggacctgggagtctctagcccccgctgtccaggcgcccccgttaggctcccgcaccgagccccagtccgggagcggcgctcagtggcccccaatagagcccagccccttccagcgctcaaactctttt

SEQ ID NO: 12177 - RNA, 661 nt, Homo sapiens
  source 1..661: mol_type = other RNA
ctgggacaggaggaggaggcagaggcggcaaagcagagaaagagggggcgcgcgcgcgcgcacgcaacccgaactgggggagttgtgcaaagccccaggaggccggggcacggcgggagcaaagctcggtaggcgcagcgcggccgaggccacccgcgtccggatcggcgactcctttcagaaagaagatgacgcgggcgcgagccggcggcgttggccacgcggctcccgagctcgccgcgcggggctgttgccggttccactgattccagcgcgcccgagaggagcctccatccccgaggctcgggatcggaggggggaccaaggcgagggcgaaatggcccgatgacaaaggaaatgtgatcccccttctctgccaaggtttcagagaggacggacgtgaggaggaggaggggcgcagggcgcgcgcggagctcggatagcattgcacgacggcccgcgcggagcgggtacatctaatatcttcctgccgatgaataattcagggcggcccgcggggacctgcggccccgcgcgctaagccgaaggggaaggagcgtgcgtgaggcgcccaggccaggcgaggcgggggcacgagggctccgggccgcgtggggcgcgcgtgcgtgttaagcgcgggcagccgcggcccggctgggca

SEQ ID NO: 12178 - RNA, 238 nt, Homo sapiens
  source 1..238: mol_type = other RNA
ctgggacaggaggaggaggcagcaaacgaggaggaggagacccgagaggaggaggcggcgagcggcggggcggaggacggcggagaggaggagaccggccttctgagagccgccgccatcttgtctcctaacacccggagccgcggcccggcccccgccacccgcggcccgccagcgcccccactgccgccgccgcgacccccgccggccgccagccctgggccaggcagagaaagag

SEQ ID NO: 12179 - RNA, 254 nt, Homo sapiens
  source 1..254: mol_type = other RNA
ctgggacaggaggaggaggcagcaaacgaggaggaggagacccgagaggaggaggcggcgagcggcggggcggaggacggcggagaggaggagaccggccttctgagagccgccgccatcttgtctcctaacacccggagccgcggcccggcccccgccacccgcggcccgccagcgcccccactgccgccgccgcgacccccgccggccgccagccctgggccaggcagagaaagaggcccggcgccagggag

SEQ ID NO: 12180 - RNA, 496 nt, Homo sapiens
  source 1..496: mol_type = other RNA
ctgggacaggaggaggaggcagcaagaaggagggagcactagaagaacattttcttagccaacttctgccttccaattttctgacaacggccataggcgatgctaagccatttctcattctttgaatatatacaagtcaggttccgcaggcagggacacgctctatattggccaaagaacacctgcgtttgacacagactgccctcggaccccttctccgcgcagtgcgactcgcaattgtctggagcacgttggcagcagccagtctcgcagtcctggttccggatgcaagactccttgagctccaaaaggttgtattttgttggagaaagtgagcccctggtgaggaggaagagaaagaagaagagaaggaacagcagcagcagccattggggtagcatcatggcccacaggtcgtggtggcttttctagggtccagcgaaatatcctgcacgccgaccatgtgggtgtcctcccagctgtgggaacaccatgt

SEQ ID NO: 12181 - RNA, 540 nt, Homo sapiens
  source 1..540: mol_type = other RNA
ctgggacaggaggaggaggcagcaagaaggagggagcactagaagaacattttcttagccaacttctgccttccaattttctgacaacggccataggcgatgctaagccatttctcattctttgaatatatacaagtcaggttccgcaggcagggacacgctctatattggccaaagaacacctgcgtttgacacagactgccctcggaccccttctccgcgcagtgcgactcgcaattgtctggagcacgttggcagcagccagtctcgcagtcctggttccggatgcaagactccttgagctcctgcagggagggacacggcaccgccaggctccaccgcccgccttccgccctcgccgccccgcctggggctttctccctacggggctcctccccagactctgctcccaccatcacctctggctcctgccaggcagggtggtctctacgtgggggccggggtaagtctgtgcagacggtggatgcctggaggggactgaacagtttttaaaaggtttactcttggtgtcctcaacat

SEQ ID NO: 12182 - RNA, 54 nt, Homo sapiens
  source 1..54: mol_type = other RNA
ctgggacaggaggaggaggcagcggcagcaccaacagcggcgcggagaaacggc

SEQ ID NO: 12183 - RNA, 7998 nt, Homo sapiens
  source 1..7998: mol_type = other RNA
ctgggacaggaggaggaggcaggaagaaagattcgcagcagggaccctccccacttgtagcctcttccactgggcctagggaggctcctgctgctgggctcgccctgacagtggacttgagaaacagaaggaaagaccgaggcatttctggctcatcttccctcaacaagaaactccgtgaaccaagacctgggtggtttattgttggtttgcaggttcgtgtgtgtgtgtgtgtgtgtgtgtgtgtgtgtgtgtgtgtgtgtgtctgaagtcattttgaaacattcttgttttagaagttttactgtattatgcttaattgtatttcctatattttaatttctcctactcattatgataaaataaaactccaataggctgtattttgtaggattttttttgtaaatgccgtagtgcaaactttataaaccatttgcagatgtgaaaatgtaaatggtagcactgggtccctggaggagcaagttgaaaatgcattcagctgattgtgaggagtgggcgtgtcagctttccaccagggatgtggcacagtgctggggaggtggccaccactgggcgggtctcagctcagctccctgtgcgggtcacagggaaactgcacaaggccaagtgtggaaataaaaataaattctctgtgtgtgtgtgcatgtgtatggctgtagtcatcgctaaatgtaaacctttaattctcaatcacaaagcagcacactgaaggtggtgttattaatgattgaggagcaggcatgaagcgtggggaagattctgagctcgggctttgccctgattttgaggagcaggcatgaagcgtgggaaagcttctgagacaggctttgtccttgcagtcgattgtctctacatctcaactgggcagtccaaccacctgttcctcagttctcacatccgtaaaatgggtctaagcaccccttccccgctttcctcacgaaggtgacagtctgtgcagaagcattttgtccattgtcaggcaccctacaagcctgcagtatttcagcacaagcgggtaccaccacagatctggggaaggctctggggcaggagctcaatccccgtgccctgggccgtgcttgctggagccccagtggacgctatgcacgggagtgacccacacccgagaaaccccaggccatcacctcttctcccccgagacattcccattcacgcgcatggctgatcacgtgcacccgggtgctctcgggtgagccaagtcagctgccgaatggttcaattctttataacagaaacaagggtgctacaggagcaagcttcgaagtgggagatcacacattagctctcctcccaatgtggaggctgaaatcacacagctttctgtcctaaaagagctgaatttacacagaggtcaactcattcccctgataaggaaatacggcctcctggtaaagaaaccagaccccagccgagggcagttgtaattcacagagttctgtggattgactattgtaaactgtgaaagcaaaagattaccgaaatgaggattattcctaagaacttggtgagcagtcaaagcggatgaccttcctgcacccgaacaatggaagctgtggggtgagcaaagctcacatctccctccaggagagcctggtaaataatctccctgtgcctgcattaagtttacagtggagaatctaagcctcgggatggtctagaaataagtagccttagcaaaaagcaacatcttgacctacattcaaaatgttaattctttgatttatgatgtattttaaaatgcatgtaaccaggttaaaaagatgtgttagatgtggctaaaattcctgtatgctcaagctgaaaatgcctaggatacaagcctagggactactgcgcgtacgggaccatcgcaaggccaagggaccaaaagtacaatctgctcactgccgtgatgactcagtccaggctgagacatcaggaaaactaacaagtgtcccaaggttctttttcctacaaggagttacactaatgtcgggactcgtggtattataagataaaggcatggataataaggaggaatcttaatttggccaaccgaagcatcaatggaagcctatttgttggctcctcttaagagccaattctctgtgatcgaaatgagtttgtatttggctcacattggtcatacctacaccatgcccatgtcaacaacggcacacatatctggaagcagaaaaacataattcctggctgggagaatatggttccttaagaaaatgaaaaagaaaaagaaaaggctgaccagctctgataggttttgcaagctctttcctgctgtttctttcagggaatcctagcaaatgaaatgtcacgagaagaaacttttctgagaatcagagctcatggtgggcagagttctcaccccccaaaactctaatttgcacaaatgtattctttttcgctttttggcctgtggtctcagtgaacgtcacagccaggcagggctcacggtgaccctgtgaggtcgactcctagaaagggcatacaaggtgacggtgaactccacctcaaagcatcgacgcgcaaaagtctgccaggcacagaggctttcggaactgggtgtccctcctccgtctgcctcctcgaagtgtcccttttaccctgggggcttcctccctgacttctgagcctctgaactatgtcttcgacacaccagatgggctagggagcaaagaaagcaacagtcccagagttggagtaagattcaggtgcacgttaaattttaatccagtttcagtttacatattatacataattagacaatgaagtgatggattttcttttcaaaacgtcccatgtttgctgctttgggtaagaccaggcaaagtgttatctcaggaagtttaagagcttagaggatccaagagcgagagtttatctggaaaatttgttttgtccatgatcaagaatgtcctgttaaaggccaaatatcacaattcagtgttggaagtgacaagaagaaaatttccagaaagttccatttgttagctgacatgtattgtagagaataattttgggggtaattggggcccactttctactatgtgtttatgaacgattagagactgttacaggacacagtgaatggcttaatatcacgatgttaatcagggacgatgctgctgcaggacaaattaaccaaacccttgaaaatatacacaaagaatataaaaaaggactcatgcgggaattattctaaagaaagttgttgcgagtcatgaggggctcagtccatgctcctgggcttgagagacccactcaacagatcttgctgacccagatccaacaagtaacagataaaaggggtcaccaattacaaggttaaagcaaagaaattataacatgtggttataccatgaagcaacatttggtcattgaaacattagtgtttttatagaagatgcttgattgaaattcttagttttgaagatccattcatagaaagggacaatttaagaaattcagtcaagttcagatttcccagaaaggctctatcagaataggattgactttttgcaaagataggtttagacacatgtgtggcttttcgatcaaccaaaattagcaaaaggccatccacctcctgtaagatacagtctcccctccaggacaagacaggaaggaggggctgcccatgcgcaccctgccctggaaggcatgaagagctaaccggctccctcggaaaatgctaaaggtggggaccgtcacaccatcttgcaagatgaagtaagagaagaagaaagtgccgatgctggagaaacagcaagttggctcggaatttcaaatcaacataagccgccaagcccaacgtgaagggatgcaagccaaagaaaacgaatccctgcagtctctgaccagttagaggcaacactagaagcaacttttacagaggctgttttcctgtctacagctggcctgttggaactggagatgtgccaatctttggcaaagtgtccctcatcaagaaattcaaaggaatgctgccatgttctgatgtattggccaagttccaagtggagttagtcatgttttgaccatgagggaaatgtggtttcgagccatacaaaagacgcctgaacaaagtgggttgaactgctcttgctaatgctgtccgttttgagatcctaaatctacttttccatgaggcactgttttggatgaggctacagactttacagccgttaggtaagaggaagccctccaggcgtttacattccatgaagaaagttccaagggtcttgtggcgaaagagctagttcaggaagtcactgaacataagcaggtgatctagggccctagggccttggacagggatcttgagttcttgggagctggtggccagcatacttcgaatgcttttgtccgccagggggcagccagacagagttattaagtcctttttgctctccttgcactgagggtacttgggtttgggacttgggatggtcacctccccgggataccgtctttcttctagagcctcctggaatgggtccaagtcttctggagtaatgtctttggactcgtcctcgtctatcctccggggtttcattttggtgtagtctacgggcaagtcccagcagtcgccctcgcccagctggaaacaccggttgttcatcactgcctgctgctggggggacatgggctccagaggggtcaggatggggcagcagctgtcccgcggcctctgcttgttcatgctgaggtccagggtcccgttctcatccacctccatgtcagggttccgcgtggcgcacaggtcctgcggcttggtgctcaggttctgcggcatctcgcggcagcgcgtggacaggttgaggatggcggtggccgccatgtgggccgcctccatgtcgtgcgtgtagtcgaagctgctcttgctgcacgtgctgctggcgctgctgcccccgccgcagctcaggttgctgctgctgctgggcgcgtagctgctggtgctgctgctgctggggctggggtccttgcagtaccgcttcgcatcatcatatcctttgggggatatatccctggtttgcaccttgggagctatggctcgcttgccataagtatggttgtcgtaactgttgtattcaaacgaggtcttggaatatttctcgagctccttggccaggttggaacgcggcgtagttgtggggacattgtttctgtagccatactgaggaatctccagctgcttcacaaagcacattggcctgagcacgcggtccgaggcctggctggacttggacacgtcgcagctctggtgcttttcctgtgccttggccagtttctctgctgcagcgatcgggcatccggagaggcttcggtgggagttcctgttgctgttgacatgcccgcgccccgtgcagcccggagtggggcacttgaggacactttcatgcatggcaaggatttctggagggaccctatctttgtgcgggcatccggacaggctgcggtgatgtgggtacagcccagttacgtggccggttccatcacacccgggggttggacacttgctctctttcttttctgttcttgagggatctttaccatagtatggctttttgacatggctgtcactggatttaggctttctgtcctccccgggaagttgtctcggagactggtcctcatatgacctcatattgtccctcctcccagcttccatggccatcttctccctcatggcctttgctctttccgtttccaaagcgatggctttctccagcagggtcaggttccccttggtcatgtcgaacacctcttcagacctgtccgagttcacagaggtggtatcgtcgtcccgctcatgacacccatcctccttcgcacagctggcaaacactctcgaccgggggctcaactgctcctccagccgcatgaggttcagcatgtccgagtagtttctgtccggcgtccttccggggaagtcctcttctggccggacatgctgacggatgttcatgttctgctgcggattcctctcctgcgggttggtctcactgagcttcctggccaggtcgaagcactgattcctcaaacactccagactgctcagacacacctcctcatcgctctcctccaccatcttttccatgagtccgttgttcatgggcttccccaacatgacgtaattcatatttctactgtcttgctgcgacatgctgtctgcataatttctgtcattcatgttttctgagagcacaacaccgtgtccttgggctaatagtttaagggagtccactgtttctctaacaacatcactgtctaagtctaaactcaactcacttttccgacccaggttttcgtttttgtcactatcgtcttccagactattggaggtattgctgttcatttctgactcagtcctggcccggtaggctgcatcctcagcgattttgccgaggtttaacaatgacttggccaccagttcatcgtaattgtcatattcgtcattattgttatcatccttttctgtgtcttgcattattcgagtattgtgacaattcatttgatggtcttcgttttcttcttcctcttcctcctcctcctcctcctcctcttcctcttcttcatcctccacatcttctccatcctcgtcatcgtcctcatcctcctcctcgatctcctcctcctcctcccggtccccctcctcgtcctcctcgtcctcatcccctggctcatcattgtcctcggagtactcctccccctcatcctcctccttctcatccatgtcctcagtcccatcactgtcgtcacactcatccactgaggagctgtctgctttcacggcaaatggctttcgtttaggagcaggttcctggggctgtttatcttgtgtttttctttttttcgccaagggacaaccatatacacttctgtgtcttgcatatttgccactgacatgaccactgccgtcacagccaggggtgggacagctgaacagctcttgtatggctggttccacgggaactcgaacccctttggaccgcgtgcgatgccgcttctcctcggtgtccacctccatcttacaggaagtcttctctcctaggaacggaggcagcgtgactcctggcaggacgcaggcccagagtcaggggctcgctctaagctctactcctggtcctctccagcttgtgactgtggcaaagtcacttaatctctctatgccttgatttctccatctttaggtggctcctcggatatccatacgtctgtgagaccaactggaacctttcttgatggaattttgttgatagcttgaaagatgcaaacacttgattgaattcaataactacatttttttcttcttccaccagatgtggccactctgcactgttgccgcgccgggtgggtgatctcaggacctgatattcttccgccgtcgaccagggtttgaagatgcccactggataggaattcaccaattctcctctgagttcattttcacacgctgtgatccctcaaatgtcaacgtggattggacaaacgtccaggcaacagccgcacacacctcgtccttggctacagcctcctcatgacccgccctcacaatgaccacaaccgctcacaagcgaaagacaagttcaattttggtaactgtgctggctcaaaatacacagacagggaagaaaaccctgttccaccacaagtttgaaaggatgatgagacacatgcatgccaccaagacgcagaaaaggtggctttttgtcttcagtgagtatggatatcataacccatagtccagggaatgaaaaaattaaaatgcacccaccaacaatgagcaaaaaacccggggtgcttcaacaagactgcagggaaaagctctctcactgtttagtgtgcagtagcttagggaaaaaaaaaatgtcgcccgggcaggaatgacaaatgcagcgcgataggctcgcaggcctcagggatctgtttgacttccacacacccccatgcacacgc

SEQ ID NO: 12184 - RNA, 6658 nt, Homo sapiens
  source 1..6658: mol_type = other RNA
ctgggacaggaggaggaggcaggaagaaagattcgcagcagggaccctccccacttgtagcctcttccactgggcctagggaggctcctgctgctgggctcgccctgacagtggacttgagaaacagaaggaaagaccgaggcatttctggctcatcttccctcaacaagaaactccgtgaaccaagacctgggtggtttattgttggtttgcaggttcgtgtgtgtgtgtgtgtgtgtgtgtgtgtgtgtgtgtgtgtgtgtgtctgaagtcattttgaaacattcttgttttagaagttttactgtattatgcttaattgtatttcctatattttaatttctcctactcattatgataaaataaaactccaataggctgtattttgtaggattttttttgtaaatgccgtagtgcaaactttataaaccatttgcagatgtgaaaatgtaaatggtagcactgggtccctggaggagcaagttgaaaatgcattcagctgattgtgaggagtgggcgtgtcagctttccaccagggatgtggcacagtgctggggaggtggccaccactgggcgggtctcagctcagctccctgtgcgggtcacagggaaactgcacaaggccaagtgtggaaataaaaataaattctctgtgtgtgtgtgcatgtgtatggctgtagtcatcgctaaatgtaaacctttaattctcaatcacaaagcagcacactgaaggtggtgttattaatgattgaggagcaggcatgaagcgtggggaagattctgagctcgggctttgccctgattttgaggagcaggcatgaagcgtgggaaagcttctgagacaggctttgtccttgcagtcgattgtctctacatctcaactgggcagtccaaccacctgttcctcagttctcacatccgtaaaatgggtctaagcaccccttccccgctttcctcacgaaggtgacagtctgtgcagaagcattttgtccattgtcaggcaccctacaagcctgcagtatttcagcacaagcgggtaccaccacagatctggggaaggctctggggcaggagctcaatccccgtgccctgggccgtgcttgctggagccccagtggacgctatgcacgggagtgacccacacccgagaaaccccaggccatcacctcttctcccccgagacattcccattcacgcgcatggctgatcacgtgcacccgggtgctctcgggtgagccaagtcagctgccgaatggttcaattctttataacagaaacaagggtgctacaggagcaagcttcgaagtgggagatcacacattagctctcctcccaatgtggaggctgaaatcacacagctttctgtcctaaaagagctgaatttacacagaggtcaactcattcccctgataaggaaatacggcctcctggtaaagaaaccagaccccagccgagggcagttgtaattcacagagttctgtggattgactattgtaaactgtgaaagcaaaagattaccgaaatgaggattattcctaagaacttggtgagcagtcaaagcggatgaccttcctgcacccgaacaatggaagctgtggggtgagcaaagctcacatctccctccaggagagcctggtaaataatctccctgtgcctgcattaagtttacagtggagaatctaagcctcgggatggtctagaaataagtagccttagcaaaaagcaacatcttgacctacattcaaaatgttaattctttgatttatgatgtattttaaaatgcatgtaaccaggttaaaaagatgtgttagatgtggctaaaattcctgtatgctcaagctgaaaatgcctaggatacaagcctagggactactgcgcgtacgggaccatcgcaaggccaagggaccaaaagtacaatctgctcactgccgtgatgactcagtccaggctgagacatcaggaaaactaacaagtgtcccaaggttctttttcctacaaggagttacactaatgtcgggactcgtggtattataagataaaggcatggataataaggaggaatcttaatttggccaaccgaagcatcaatggaagcctatttgttggctcctcttaagagccaattctctgtgatcgaaatgagtttgtatttggctcacattggtcatacctacaccatgcccatgtcaacaacggcacacatatctggaagcagaaaaacataattcctggctgggagaatatggttccttaagaaaatgaaaaagaaaaagaaaaggctgaccagctctgataggttttgcaagctctttcctgctgtttctttcagggaatcctagcaaatgaaatgtcacgagaagaaacttttctgagaatcagagctcatggtgggcagagttctcaccccccaaaactctaatttgcacaaatgtattctttttcgctttttggcctgtggtctcagtgaacgtcacagccaggcagggctcacggtgaccctgtgaggtcgactcctagaaagggcatacaaggtgacggtgaactccacctcaaagcatcgacgcgcaaaagtctgccaggcacagaggctttcggaactgggtgtccctcctccgtctgcctcctcgaagtgtcccttttaccctgggggcttcctccctgacttctgagcctctgaactatgtcttcgacacaccagatgggctagggagcaaagaaagcaacagtcccagagttggagtaagattcaggtgcacgttaaattttaatccagtttcagtttacatattatacataattagacaatgaagtgatggattttcttttcaaaacgtcccatgtttgctgctttgggtaagaccaggcaaagtgttatctcaggaagtttaagagcttagaggatccaagagcgagagtttatctggaaaatttgttttgtccatgatcaagaatgtcttgagttcttgggagctggtggccagcatacttcgaatgcttttgtccgccagggggcagccagacagacttctgtgtgaggcgtaattaccagtcacatgaccactcccatcacaccctggagttggacatgttattaagtcctttttgctctccttgcactgagggtacttgggtttgggacttgggatggtcacctccccgggataccgtctttcttctagagcctcctggaatgggtccaagtcttctggagtaatgtctttggactcgtcctcgtctatcctccggggtttcattttggtgtagtctacgggcaagtcccagcagtcgccctcgcccagctggaaacaccggttgttcatcactgcctgctgctggggggacatgggctccagaggggtcaggatggggcagcagctgtcccgcggcctctgcttgttcatgctgaggtccagggtcccgttctcatccacctccatgtcagggttccgcgtggcgcacaggtcctgcggcttggtgctcaggttctgcggcatctcgcggcagcgcgtggacaggttgaggatggcggtggccgccatgtgggccgcctccatgtcgtgcgtgtagtcgaagctgctcttgctgcacgtgctgctggcgctgctgcccccgccgcagctcaggttgctgctgctgctgggcgcgtagctgctggtgctgctgctgctggggctggggtccttgcagtaccgcttcgcatcatcatatcctttgggggatatatccctggtttgcaccttgggagctatggctcgcttgccataagtatggttgtcgtaactgttgtattcaaacgaggtcttggaatatttctcgagctccttggccaggttggaacgcggcgtagttgtggggacattgtttctgtagccatactgaggaatctccagctgcttcacaaagcacattggcctgagcacgcggtccgaggcctggctggacttggacacgtcgcagctctggtgcttttcctgtgccttggccagtttctctgctgcagcgatcgggcatccggagaggcttcggtgggagttcctgttgctgttgacatgcccgcgccccgtgcagcccggagtggggcacttgaggacactttcatgcatggcaaggatttctggagggaccctatctttgtgcgggcatccggacaggctgcggtgatgtgggtacagcccagttacgtggccggttccatcacacccgggggttggacacttgctctctttcttttctgttcttgagggatctttaccatagtatggctttttgacatggctgtcactggatttaggctttctgtcctccccgggaagttgtctcggagactggtcctcatatgacctcatattgtccctcctcccagcttccatggccatcttctccctcatggcctttgctctttccgtttccaaagcgatggctttctccagcagggtcaggttccccttggtcatgtcgaacacctcttcagacctgtccgagttcacagaggtggtatcgtcgtcccgctcatgacacccatcctccttcgcacagctggcaaacactctcgaccgggggctcaactgctcctccagccgcatgaggttcagcatgtccgagtagtttctgtccggcgtccttccggggaagtcctcttctggccggacatgctgacggatgttcatgttctgctgcggattcctctcctgcgggttggtctcactgagcttcctggccaggtcgaagcactgattcctcaaacactccagactgctcagacacacctcctcatcgctctcctccaccatcttttccatgagtccgttgttcatgggcttccccaacatgacgtaattcatatttctactgtcttgctgcgacatgctgtctgcataatttctgtcattcatgttttctgagagcacaacaccgtgtccttgggctaatagtttaagggagtccactgtttctctaacaacatcactgtctaagtctaaactcaactcacttttccgacccaggttttcgtttttgtcactatcgtcttccagactattggaggtattgctgttcatttctgactcagtcctggcccggtaggctgcatcctcagcgattttgccgaggtttaacaatgacttggccaccagttcatcgtaattgtcatattcgtcattattgttatcatccttttctgtgtcttgcattattcgagtattgtgacaattcatttgatggtcttcgttttcttcttcctcttcctcctcctcctcctcctcctcttcctcttcttcatcctccacatcttctccatcctcgtcatcgtcctcatcctcctcctcgatctcctcctcctcctcccggtccccctcctcgtcctcctcgtcctcatcccctggctcatcattgtcctcggagtactcctccccctcatcctcctccttctcatccatgtcctcagtcccatcactgtcgtcacactcatccactgaggagctgtctgctttcacggcaaatggctttcgtttaggagcaggttcctggggctgtttatcttgtgtttttctttttttcgccaagggacaaccatatacacttctgtgtcttgcatatttgccactgacatgaccactgccgtcacagccaggggtgggacagctgaacagctcttgtatggctggttccacgggaactcgaacccctttggaccgcgtgcgatgccgcttctcctcggtgtccacctccatcttacaggaagtcttctctcctaggaacggaggcagcgtgactcctggcaggacgcaggcccagagtcaggggctcgctctaagctctactcctggtcctctccagcttgtgactgtggcaaagtcacttaatctctctatgccttgatttctccatctttaggtggctcctcggatatccatacgtctgtgagaccaactggaacctttcttgatggaattttgttgatagcttgaaagatgcaaacacttgattgaattcaataactacatttttttcttcttccaccagatgtggccactctgcactgttgccgcgccgggtgggtgatctcaggacctgatattcttccgccgtcgaccagggtttgaagatgcccactggataggaattcaccaattctcctctgagttcattttcacacgctgtgatccctcaaatgtcaacgtggattggacaaacgtccaggcaacagccgcacacacctcgtccttggctacagcctcctcatgacccgccctcacaatgaccacaaccgctcacaagcgaaagacaagttcaattttggtaactgtgctggctcaaaatacacagacagggaagaaaaccctgttccaccacaagtttgaaaggatgatgagacacatgcatgccaccaagacgcagaaaaggtggctttttgtcttcagtgagtatggatatcataacccatagtccagggaatgaaaaaattaaaatgcacccaccaacaatgagcaaaaaacccggggtgcttcaacaagactgcagggaaaagctctctcactgtttagtgtgcagtagcttagggaaaaaaaaaatgtcgcccgggcaggaatgacaaatgcagcgcgataggctcgcaggcctcagggatctgtttgacttccacacacccccatgcacacgc

SEQ ID NO: 12185 - RNA, 6595 nt, Homo sapiens
  source 1..6595: mol_type = other RNA
ctgggacaggaggaggaggcaggaagaaagattcgcagcagggaccctccccacttgtagcctcttccactgggcctagggaggctcctgctgctgggctcgccctgacagtggacttgagaaacagaaggaaagaccgaggcatttctggctcatcttccctcaacaagaaactccgtgaaccaagacctgggtggtttattgttggtttgcaggttcgtgtgtgtgtgtgtgtgtgtgtgtgtgtgtgtgtgtgtgtgtgtgtctgaagtcattttgaaacattcttgttttagaagttttactgtattatgcttaattgtatttcctatattttaatttctcctactcattatgataaaataaaactccaataggctgtattttgtaggattttttttgtaaatgccgtagtgcaaactttataaaccatttgcagatgtgaaaatgtaaatggtagcactgggtccctggaggagcaagttgaaaatgcattcagctgattgtgaggagtgggcgtgtcagctttccaccagggatgtggcacagtgctggggaggtggccaccactgggcgggtctcagctcagctccctgtgcgggtcacagggaaactgcacaaggccaagtgtggaaataaaaataaattctctgtgtgtgtgtgcatgtgtatggctgtagtcatcgctaaatgtaaacctttaattctcaatcacaaagcagcacactgaaggtggtgttattaatgattgaggagcaggcatgaagcgtggggaagattctgagctcgggctttgccctgattttgaggagcaggcatgaagcgtgggaaagcttctgagacaggctttgtccttgcagtcgattgtctctacatctcaactgggcagtccaaccacctgttcctcagttctcacatccgtaaaatgggtctaagcaccccttccccgctttcctcacgaaggtgacagtctgtgcagaagcattttgtccattgtcaggcaccctacaagcctgcagtatttcagcacaagcgggtaccaccacagatctggggaaggctctggggcaggagctcaatccccgtgccctgggccgtgcttgctggagccccagtggacgctatgcacgggagtgacccacacccgagaaaccccaggccatcacctcttctcccccgagacattcccattcacgcgcatggctgatcacgtgcacccgggtgctctcgggtgagccaagtcagctgccgaatggttcaattctttataacagaaacaagggtgctacaggagcaagcttcgaagtgggagatcacacattagctctcctcccaatgtggaggctgaaatcacacagctttctgtcctaaaagagctgaatttacacagaggtcaactcattcccctgataaggaaatacggcctcctggtaaagaaaccagaccccagccgagggcagttgtaattcacagagttctgtggattgactattgtaaactgtgaaagcaaaagattaccgaaatgaggattattcctaagaacttggtgagcagtcaaagcggatgaccttcctgcacccgaacaatggaagctgtggggtgagcaaagctcacatctccctccaggagagcctggtaaataatctccctgtgcctgcattaagtttacagtggagaatctaagcctcgggatggtctagaaataagtagccttagcaaaaagcaacatcttgacctacattcaaaatgttaattctttgatttatgatgtattttaaaatgcatgtaaccaggttaaaaagatgtgttagatgtggctaaaattcctgtatgctcaagctgaaaatgcctaggatacaagcctagggactactgcgcgtacgggaccatcgcaaggccaagggaccaaaagtacaatctgctcactgccgtgatgactcagtccaggctgagacatcaggaaaactaacaagtgtcccaaggttctttttcctacaaggagttacactaatgtcgggactcgtggtattataagataaaggcatggataataaggaggaatcttaatttggccaaccgaagcatcaatggaagcctatttgttggctcctcttaagagccaattctctgtgatcgaaatgagtttgtatttggctcacattggtcatacctacaccatgcccatgtcaacaacggcacacatatctggaagcagaaaaacataattcctggctgggagaatatggttccttaagaaaatgaaaaagaaaaagaaaaggctgaccagctctgataggttttgcaagctctttcctgctgtttctttcagggaatcctagcaaatgaaatgtcacgagaagaaacttttctgagaatcagagctcatggtgggcagagttctcaccccccaaaactctaatttgcacaaatgtattctttttcgctttttggcctgtggtctcagtgaacgtcacagccaggcagggctcacggtgaccctgtgaggtcgactcctagaaagggcatacaaggtgacggtgaactccacctcaaagcatcgacgcgcaaaagtctgccaggcacagaggctttcggaactgggtgtccctcctccgtctgcctcctcgaagtgtcccttttaccctgggggcttcctccctgacttctgagcctctgaactatgtcttcgacacaccagatgggctagggagcaaagaaagcaacagtcccagagttggagtaagattcaggtgcacgttaaattttaatccagtttcagtttacatattatacataattagacaatgaagtgatggattttcttttcaaaacgtcccatgtttgctgctttgggtaagaccaggcaaagtgttatctcaggaagtttaagagcttagaggatccaagagcgagagtttatctggaaaatttgttttgtccatgatcaagaatgtcttgagttcttgggagctggtggccagcatacttcgaatgcttttgtccgccagggggcagccagacagagttattaagtcctttttgctctccttgcactgagggtacttgggtttgggacttgggatggtcacctccccgggataccgtctttcttctagagcctcctggaatgggtccaagtcttctggagtaatgtctttggactcgtcctcgtctatcctccggggtttcattttggtgtagtctacgggcaagtcccagcagtcgccctcgcccagctggaaacaccggttgttcatcactgcctgctgctggggggacatgggctccagaggggtcaggatggggcagcagctgtcccgcggcctctgcttgttcatgctgaggtccagggtcccgttctcatccacctccatgtcagggttccgcgtggcgcacaggtcctgcggcttggtgctcaggttctgcggcatctcgcggcagcgcgtggacaggttgaggatggcggtggccgccatgtgggccgcctccatgtcgtgcgtgtagtcgaagctgctcttgctgcacgtgctgctggcgctgctgcccccgccgcagctcaggttgctgctgctgctgggcgcgtagctgctggtgctgctgctgctggggctggggtccttgcagtaccgcttcgcatcatcatatcctttgggggatatatccctggtttgcaccttgggagctatggctcgcttgccataagtatggttgtcgtaactgttgtattcaaacgaggtcttggaatatttctcgagctccttggccaggttggaacgcggcgtagttgtggggacattgtttctgtagccatactgaggaatctccagctgcttcacaaagcacattggcctgagcacgcggtccgaggcctggctggacttggacacgtcgcagctctggtgcttttcctgtgccttggccagtttctctgctgcagcgatcgggcatccggagaggcttcggtgggagttcctgttgctgttgacatgcccgcgccccgtgcagcccggagtggggcacttgaggacactttcatgcatggcaaggatttctggagggaccctatctttgtgcgggcatccggacaggctgcggtgatgtgggtacagcccagttacgtggccggttccatcacacccgggggttggacacttgctctctttcttttctgttcttgagggatctttaccatagtatggctttttgacatggctgtcactggatttaggctttctgtcctccccgggaagttgtctcggagactggtcctcatatgacctcatattgtccctcctcccagcttccatggccatcttctccctcatggcctttgctctttccgtttccaaagcgatggctttctccagcagggtcaggttccccttggtcatgtcgaacacctcttcagacctgtccgagttcacagaggtggtatcgtcgtcccgctcatgacacccatcctccttcgcacagctggcaaacactctcgaccgggggctcaactgctcctccagccgcatgaggttcagcatgtccgagtagtttctgtccggcgtccttccggggaagtcctcttctggccggacatgctgacggatgttcatgttctgctgcggattcctctcctgcgggttggtctcactgagcttcctggccaggtcgaagcactgattcctcaaacactccagactgctcagacacacctcctcatcgctctcctccaccatcttttccatgagtccgttgttcatgggcttccccaacatgacgtaattcatatttctactgtcttgctgcgacatgctgtctgcataatttctgtcattcatgttttctgagagcacaacaccgtgtccttgggctaatagtttaagggagtccactgtttctctaacaacatcactgtctaagtctaaactcaactcacttttccgacccaggttttcgtttttgtcactatcgtcttccagactattggaggtattgctgttcatttctgactcagtcctggcccggtaggctgcatcctcagcgattttgccgaggtttaacaatgacttggccaccagttcatcgtaattgtcatattcgtcattattgttatcatccttttctgtgtcttgcattattcgagtattgtgacaattcatttgatggtcttcgttttcttcttcctcttcctcctcctcctcctcctcctcttcctcttcttcatcctccacatcttctccatcctcgtcatcgtcctcatcctcctcctcgatctcctcctcctcctcccggtccccctcctcgtcctcctcgtcctcatcccctggctcatcattgtcctcggagtactcctccccctcatcctcctccttctcatccatgtcctcagtcccatcactgtcgtcacactcatccactgaggagctgtctgctttcacggcaaatggctttcgtttaggagcaggttcctggggctgtttatcttgtgtttttctttttttcgccaagggacaaccatatacacttctgtgtcttgcatatttgccactgacatgaccactgccgtcacagccaggggtgggacagctgaacagctcttgtatggctggttccacgggaactcgaacccctttggaccgcgtgcgatgccgcttctcctcggtgtccacctccatcttacaggaagtcttctctcctaggaacggaggcagcgtgactcctggcaggacgcaggcccagagtcaggggctcgctctaagctctactcctggtcctctccagcttgtgactgtggcaaagtcacttaatctctctatgccttgatttctccatctttaggtggctcctcggatatccatacgtctgtgagaccaactggaacctttcttgatggaattttgttgatagcttgaaagatgcaaacacttgattgaattcaataactacatttttttcttcttccaccagatgtggccactctgcactgttgccgcgccgggtgggtgatctcaggacctgatattcttccgccgtcgaccagggtttgaagatgcccactggataggaattcaccaattctcctctgagttcattttcacacgctgtgatccctcaaatgtcaacgtggattggacaaacgtccaggcaacagccgcacacacctcgtccttggctacagcctcctcatgacccgccctcacaatgaccacaaccgctcacaagcgaaagacaagttcaattttggtaactgtgctggctcaaaatacacagacagggaagaaaaccctgttccaccacaagtttgaaaggatgatgagacacatgcatgccaccaagacgcagaaaaggtggctttttgtcttcagtgagtatggatatcataacccatagtccagggaatgaaaaaattaaaatgcacccaccaacaatgagcaaaaaacccggggtgcttcaacaagactgcagggaaaagctctctcactgtttagtgtgcagtagcttagggaaaaaaaaaatgtcgcccgggcaggaatgacaaatgcagcgcgataggctcgcaggcctcagggatctgtttgacttccacacacccccatgcacacgc

SEQ ID NO: 12186 - RNA, 223 nt, Homo sapiens
  source 1..223: mol_type = other RNA
ctgggacaggaggaggaggcaggaggaagaaaggggggttgggaggtagcgtccggtaggtctgcgcagacagcgctgccagacctctgactcccccagtcctgccgccgccgatagccccacaaggcgacatgggaagtccgccggagcagaggggagaaaattcaaaacgagtctactcaacctcgtcttggctccgaggccccgccatgcagacccctct

SEQ ID NO: 12187 - RNA, 114 nt, Homo sapiens
  source 1..114: mol_type = other RNA
ctgggacaggaggaggaggcaggaggaagacggggggttgggaggtagcgtccggtaggtctgcgcagacagcgctgccagacctctgactcccccagtcctgccgccgccgat

SEQ ID NO: 12188 - RNA, 233 nt, Homo sapiens
  source 1..233: mol_type = other RNA
ctgggacaggaggaggaggcaggaggaagacggggggttgggaggtagcgtccggtaggtctgcgcagacagcgctgccagacctctgactcccccagtcctgccgccgccgatagccccacaaggcgacatgggaagtccgccggagcagaggggagaaaattcaaaacgagtctactcaacctcgtcttggctccgaggccccgccatggagaccagcataatgcgcaggc

SEQ ID NO: 12189 - RNA, 2831 nt, Homo sapiens
  source 1..2831: mol_type = other RNA
ctgggacaggaggaggaggcaggcacaggctgcaggtacggccacctccagcagtgggaatggcagcggcaggggcaggcccttcgccacttcacagaactggccggagaatctggcattgcagatacattcagacacccctccagctgcccggcaggtgcccccattcaagcaggggttggcttcacaggggagagtggggacctgacacctctggccagcaagaccctccaggcagctgcagttggcagcgggagagccaccctcacatgggctgccatcgaggcaggtgacattcaggctgcactccttggatgggacaggcaacctgcagcgcgggcccccgaagccaggcgggcagcggcactcgaagcggccgtcggggtgcgtgtgacagcggccacgggcgcagggggcggagtgacaggggtcgacgtgggcttcgcagcgcgggccttcccaccccgggccgcaggcgcaggcaaaggcgtcgaagaggtcacggcaggcaccgtcgtgcagacagggcgagggcgcacacacgggcgcgccgcggcagccgaggatcggggccggcgtcccaggccaagacgcgaagtgctctcgggcgccaggggccgcgccgggccggggccgcgccaagggcaggggcaggccgcccagcgccacgcggcccaagcagccggtgaagttctcagccagcaggatgcgcacagcacccgggccctgcaggaagcccaggtcactggccaggccgcgcagcgccaccggggtggcggcaccatccagccacagcagccagcgcgaggtggtggccgccgggcgctccatggccagacgcacgcggtgccaggcaccatcggccacgcgcggccccggtatgggcagcacagcgccgggcaggccatggcctccgcgcacgccccccgccagcgagccattgcgcaccgccagccacacgccttccagggcgcccgccgcggcacgcagcagccaggcctcggagtcgcgcgtgcgaaaggccagcgacaggccgccgagcaagcgccctgacgacgcgttgtgcccgctgaacgcggcggggggaccctcgcggaacgtggcctccgccacacacacaaagccatcagggacctcctcacacgtggcaggtgggagacagggctggccgggacaccacagctgctgggcacacgtaggccccgtgaaattggcagggcaggtacagtggaagtcattccaggtgacgaggcaagtcccaccattgaaacaggggtcaggactgcacatgtcctcggagacgcagcccgcagtgaggttccaggactgcctgccgccgagctcgctgggctggcttgagttatccagtggcagaggaaagaaggggaggtggcagccatcgagtcgcaggtcctggaggcagcctcggaagggcccaccccagggctggctgtcggcagcaaggagcctcccacccacgtgcacgtgctgccccaggtcctgcagctggtcaggcccgaagctgagcatcaccaggtgacggagcccatcatcccagcgcccagggagcactacagcaggactgcccggcacctcagcccggatccgaccctcactcaggaatactgttaggccagctgcggagtcattggcaaactggagcaacaggccagcggactcccgagtgcggagaaggaaagacactgtgaggttgggacctggcagctcttggagcagaaaggaggcagagcttggggcgcctcccaagccaaaggtggcagcaggaatctcatcagcgcacgtgggacctctatggggccgggcacagtcgcaacggaaatgagtccacagatccacacaggaccctccgtggacacaaggcagaggccggcactgctctcggcgctcacagcccaggaggacgttctcaccgagatcctcaggcagcaggaggtggccatccacacgcacgtcctggaggcagcctgcaaaggtcgcgtcccccagctgggcagaggagatcccggcaggcagcggagttgccgaagccgtggaagccagggccacaggaccagaggccacacagagccgggcagggcagccctcatgccagagccgtagctccagggtcgctagatggagcacaacctccacctggtgccaatggccatcgtttagggccaggtccggcagtctcaggacaagcacagtggtgctgtagctccagagtgtggcctgaagtgtggctgccaccaatgccagctccaagctttccttggtgtcattgcgagtggccaaggtcccagcgggcagtgtggtgcgaaacctcagtgccagacccagggggccaccagctggcactgatgcctgaatggggctcccagccatcacagagaaggtggtattctggccacagaacggtccatgggtaccaggtgggcagtggcagacgtaactgtggaccccagactcgaagatagggatgcaggtggcagccagcgggcaggtgtggccctggcagccagtgagctgcacagaacagtcgcgcccaccccaggtctctgggcacctgcagatatagcctgccacagtgtcactgcaggttccgccgtgcaggcagggatccgacaggcattcatccacatcttcctcacatgtcggccctgccaggagccacaggtggcccaggaaggtccacagagcccccggctccattgccatgccctccagacaggttgagagtggtgggcgggcactgaggctggggaagtggggaggaggcagagctccctgcctggcccagctgcctccttcggagcctgctcaggaat

SEQ ID NO: 12190 - RNA, 3781 nt, Homo sapiens
  source 1..3781: mol_type = other RNA
ctgggacaggaggaggaggcaggcacaggctgcaggtacggccacctccagcagtgggaatggcagcggcaggggcaggcccttcgccacttcacagaactggccggagaatctggcattgcagatacattcagacacccctccagctgcccggcaggtgcccccattcaagcaggggttggcttcacaggggagagtggggacctgacacctctggccagcaagaccctccaggcagctgcagttggcagcgggagagccaccctcacatgggctgccatcgaggcaggtgacattcaggctgcactccttggatgggacaggcaacctgcagcgcgggcccccgaagccaggcgggcagcggcactcgaagcggccgtcggggtgcgtgtgacagcggccacgggcgcagggggcggagtgacaggggtcgacgtgggcttcgcagcgcgggccttcccaccccgggccgcaggcgcaggcaaaggcgtcgaagaggtcacggcaggcaccgtcgtgcagacagggcgagggcgcacacacgggcgcgccgcggcagccgaggatcggggccggcgtcccaggccaagacgcgaagtgctctcgggcgccaggggccgcgccgggccggggccgcgccaagggcaggggcaggccgcccagcgccacgcggcccaagcagccggtgaagttctcagccagcaggatgcgcacagcacccgggccctgcaggaagcccaggtcactggccaggccgcgcagcgccaccggggtggcggcaccatccagccacagcagccagcgcgaggtggtggccgccgggcgctccatggccagacgcacgcggtgccaggcaccatcggccacgcgcggccccggtatgggcagcacagcgccgggcaggccatggcctccgcgcacgccccccgccagcgagccattgcgcaccgccagccacacgccttccagggcgcccgccgcggcacgcagcagccaggcctcggagtcgcgcgtgcgaaaggccagcgacaggccgccgagcaagcgccctgacgacgcgttgtgcccgctgaacgcggcggggggaccctcgcggaacgtggcctccgccacacacacaaagccatcagggacctcctcacacgtggcaggtgggagacagggctggccgggacaccacagctgctgggcacacgtaggccccgtgaaattggcagggcaggtacagtggaagtcattccaggtgacgaggcaagtcccaccattgaaacaggggtcaggactgcacatgtcctcggagacgcagcccgcagtgaggttccaggactgcctgccgccgagctcgctgggctggcttgagttatccagtggcagaggaaagaaggggaggtggcagccatcgagtcgcaggtcctggaggcagcctcggaagggcccaccccagggctggctgtcggcagcaaggagcctcccacccacgtgcacgtgctgccccaggtcctgcagctggtcaggcccgaagctgagcatcaccaggtgacggagcccatcatcccagcgcccagggagcactacagcaggactgcccggcacctcagcccggatccgaccctcactcaggaatactgttaggccagctgcggagtcattggcaaactggagcaacaggccagcggactcccgagtgcggagaaggaaagacactgtgaggttgggacctggcagctcttggagcagaaaggaggcagagcttggggcgcctcccaagccaaaggtggcagcaggaatctcatcagcgcacgtgggacctctatggggccgggcacagtcgcaacggaaatgagtccacagatccacacaggaccctccgtggacacaaggcagaggccggcactgctctcggcgctcacagcccaggaggacgttctcaccgagatcctcaggcagcaggaggtggccatccacacgcacgtcctggaggcagcctgcaaaggtcgcgtcccccagctgggcagaggagatcccggcaggcagcggagttgccgaagccgtggaagccagggccacaggaccagaggccacacagagccgggcagggcagccctcatgccagagccgtagctccagggtcgctagatggagcacaacctccacctggtgccaatggccatcgtttagggccaggtccggcagtctcaggacaagcacagtggtgctgtagctccagagtgtggcctgaagtgtggctgccaccaatgccagctccaagctttccttggtgtcattgcgagtggccaaggtcccagcgggcagtgtggtgcgaaacctcagtgccagacccagggggccaccagctggcactgatgcctgaatggggctcccagccatcacagagaaggtggtattctggccacagaacggtccatgggtaccaggtgggcagtggcagacgtaactgtggaccccagactcgaagatagggatgcaggtggcagccagcgggcaggtgtggccctggcagccagtgagctgcacagaacagtcgcgcccaccccaggtctctgggcacctgcagatatagcctgccacagtgtcactgcaggttccgccgtgcaggcagggatccgacaggcattcatccacatcttcctcacatgtcggccctgcgtagccatctgggcagtgacactggaagccattgggcaggtcctggcagtggcctccgttgaggcatggccgtgaggcacactcgtccacctccacaccgcagtcggctccctcaaagccaggagggcagtggcacaggaaacccgcagcatggcggaagctgaaggcgccagggaaggcggcctggacacccccgtagagggccgggtcagagcgctgcaggcatcggcccccatgctggcaggggctcgatgcacactcgtcctcgtccacctcgcacagctcgccgctgtagcctggccaacagaggcagcggaagctcccgaggccctcgaggcaggacgcgttgtgctcgcagggcgccgatgcgcactccagcacctcccgctcgcagtgcgtgccctcgtagccggtgcccgcgcagtcgcaccggaacccgttgaccaggtcgtggcacgtgcccccatgtgcgcacggctggctctggcactcgtcgaggtccagctggcaacgggtgcccccgtagcctggcgcgcacacacagcggaaggagcccacgccgtccaggcacgagcccccgtgcaggcagggcgctgaggcgcactcgtccacctccatctcgcaggtcacgcctgcatagccaagggggcaatggcactcgtagcgatcggccaggttgcggcaggtggccccatggtggcacggccgggatgcacactcatcgatgtccagctcgcagcgtgggccctggaaacccggcacgcagtagcagcggaagccggtgggatctggaccctggggcacacacagagcgccgtggtggcatggctgggtggcacagccccggggctccatgggcccacaggtatagccaccactctcggtagcctggcactcggtccctggagcgcacgggtctgaggcacaggcactggggggctctgaaggcaccgtcccagccaggagggaaagggcaggggcccagagcagcagtagcaggacagaggccagggcctgggggtccggggtcccaggcctggccagcgccatggcagcccgctctgcgctctgctcggctgctgtgagaacgggagggcggcctggctggctccgc

SEQ ID NO: 12191 - RNA, 3813 nt, Homo sapiens
  source 1..3813: mol_type = other RNA
ctgggacaggaggaggaggcaggcacaggctgcaggtacggccacctccagcagtgggaatggcagcggcaggggcaggcccttcgccacttcacagaactggccggagaatctggcattgcagatacattcagacacccctccagctgcccggcaggtgcccccattcaagcaggggttggcttcacaggggagagtggggacctgacacctctggccagcaagaccctccaggcagctgcagttggcagcgggagagccaccctcacatgggctgccatcgaggcaggtgacattcaggctgcactccttggatgggacaggcaacctgcagcgcgggcccccgaagccaggcgggcagcggcactcgaagcggccgtcggggtgcgtgtgacagcggccacgggcgcagggggcggagtgacaggggtcgacgtgggcttcgcagcgcgggccttcccaccccgggccgcaggcgcaggcaaaggcgtcgaagaggtcacggcaggcaccgtcgtgcagacagggcgagggcgcacacacgggcgcgccgcggcagccgaggatcggggccggcgtcccaggccaagacgcgaagtgctctcgggcgccaggggccgcgccgggccggggccgcgccaagggcaggggcaggccgcccagcgccacgcggcccaagcagccggtgaagttctcagccagcaggatgcgcacagcacccgggccctgcaggaagcccaggtcactggccaggccgcgcagcgccaccggggtggcggcaccatccagccacagcagccagcgcgaggtggtggccgccgggcgctccatggccagacgcacgcggtgccaggcaccatcggccacgcgcggccccggtatgggcagcacagcgccgggcaggccatggcctccgcgcacgccccccgccagcgagccattgcgcaccgccagccacacgccttccagggcgcccgccgcggcacgcagcagccaggcctcggagtcgcgcgtgcgaaaggccagcgacaggccgccgagcaagcgccctgacgacgcgttgtgcccgctgaacgcggcggggggaccctcgcggaacgtggcctccgccacacacacaaagccatcagggacctcctcacacgtggcaggtgggagacagggctggccgggacaccacagctgctgggcacacgtaggccccgtgaaattggcagggcaggtacagtggaagtcattccaggtgacgaggcaagtcccaccattgaaacaggggtcaggactgcacatgtcctcggagacgcagcccgcagtgaggttccaggactgcctgccgccgagctcgctgggctggcttgagttatccagtggcagaggaaagaaggggaggtggcagccatcgagtcgcaggtcctggaggcagcctcggaagggcccaccccagggctggctgtcggcagcaaggagcctcccacccacgtgcacgtgctgccccaggtcctgcagctggtcaggcccgaagctgagcatcaccaggtgacggagcccatcatcccagcgcccagggagcactacagcaggactgcccggcacctcagcccggatccgaccctcactcaggaatactgttaggccagctgcggagtcattggcaaactggagcaacaggccagcggactcccgagtgcggagaaggaaagacactgtgaggttgggacctggcagctcttggagcagaaaggaggcagagcttggggcgcctcccaagccaaaggtggcagcaggaatctcatcagcgcacgtgggacctctatggggccgggcacagtcgcaacggaaatgagtccacagatccacacaggaccctccgtggacacaaggcagaggccggcactgctctcggcgctcacagcccaggaggacgttctcaccgagatcctcaggcagcaggaggtggccatccacacgcacgtcctggaggcagcctgcaaaggtcgcgtcccccagctgggcagaggagatcccggcaggcagcggagttgccgaagccgtggaagccagggccacaggaccagaggccacacagagccgggcagggcagccctcatgccagagccgtagctccagggtcgctagatggagcacaacctccacctggtgccaatggccatcgtttagggccaggtccggcagtctcaggacaagcacagtggtgctgtagctccagagtgtggcctgaagtgtggctgccaccaatgccagctccaagctttccttggtgtcattgcgagtggccaaggtcccagcgggcagtgtggtgcgaaacctcagtgccagacccagggggccaccagctggcactgatgcctgaatggggctcccagccatcacagagaaggtggtattctggccacagaacggtccatgggtaccaggtgggcagtggcagacgtaactgtggaccccagactcgaagatagggatgcaggtggcagccagcgggcaggtgtggccctggcagccagtgagctgcacagaacagtcgcgcccaccccaggtctctgggcacctgcagatatagcctgccacagtgtcactgcaggttccgccgtgcaggcagggatccgacaggcattcatccacatcttcctcacatgtcggccctgcgtagccatctgggcagtgacactggaagccattgggcaggtcctggcagtggcctccgttgaggcatggccgtgaggcacactcgtccacctccacaccgcagtcggctccctcaaagccaggagggcagtggcacaggaaacccgcagcatggcggaagctgaaggcgccagggaaggcggcctggacacccccgtagagggccgggtcagagcgctgcaggcatcggcccccatgctggcaggggctcgatgcacactcgtcctcgtccacctcgcacagctcgccgctgtagcctggccaacagaggcagcggaagctcccgaggccctcgaggcaggacgcgttgtgctcgcagggcgccgatgcgcactccagcacctcccgctcgcagtgcgtgccctcgtagccggtgcccgcgcagtcgcaccggaacccgttgaccaggtcgtggcacgtgcccccatgtgcgcacggctggctctggcactcgtcgaggtccagctggcaacgggtgcccccgtagcctggcgcgcacacacagcggaaggagcccacgccgtccaggcacgagcccccgtgcaggcagggcgctgaggcgcactcgtccacctccatctcgcaggtcacgcctgcatagccaagggggcaatggcactcgtagcgatcggccaggttgcggcaggtggccccatggtggcacggccgggatgcacactcatcgatgtccagctcgcagcgtgggccctggaaacccggcacgcagtagcagcggaagccggtgggatctggaccctggggcacacacagagcgccgtggtggcatggctgggtggcacagccccggggctccatgggcccacaggtatagccaccactctcggtagcctggcactcggtccctggagcgcacgggtctgaggcacaggcactggggggctctgaaggcaccgtcccttatagtctcctgctgcactcgatgtttgcttgctctccagctggcctcttgttggggtggacaggaggagctcttcagggggacctggttcaggaagccaggtcatctcagagacactacaacatagaacaacattcctttcttctaccaccctcagccccagtggggagagaatcctcttgctgaag

SEQ ID NO: 12192 - RNA, 4173 nt, Homo sapiens
  source 1..4173: mol_type = other RNA
ctgggacaggaggaggaggcaggcacaggctgcaggtacggccacctccagcagtgggaatggcagcggcaggggcaggcccttcgccacttcacagaactggccggagaatctggcattgcagatacattcagacacccctccagctgcccggcaggtgcccccattcaagcaggggttggcttcacaggggagagtggggacctgacacctctggccagcaagaccctccaggcagctgcagttggcagcgggagagccaccctcacatgggctgccatcgaggcaggtgacattcaggctgcactccttggatgggacaggcaacctgcagcgcgggcccccgaagccaggcgggcagcggcactcgaagcggccgtcggggtgcgtgtgacagcggccacgggcgcagggggcggagtgacaggggtcgacgtgggcttcgcagcgcgggccttcccaccccgggccgcaggcgcaggcaaaggcgtcgaagaggtcacggcaggcaccgtcgtgcagacagggcgagggcgcacacacgggcgcgccgcggcagccgaggatcggggccggcgtcccaggccaagacgcgaagtgctctcgggcgccaggggccgcgccgggccggggccgcgccaagggcaggggcaggccgcccagcgccacgcggcccaagcagccggtgaagttctcagccagcaggatgcgcacagcacccgggccctgcaggaagcccaggtcactggccaggccgcgcagcgccaccggggtggcggcaccatccagccacagcagccagcgcgaggtggtggccgccgggcgctccatggccagacgcacgcggtgccaggcaccatcggccacgcgcggccccggtatgggcagcacagcgccgggcaggccatggcctccgcgcacgccccccgccagcgagccattgcgcaccgccagccacacgccttccagggcgcccgccgcggcacgcagcagccaggcctcggagtcgcgcgtgcgaaaggccagcgacaggccgccgagcaagcgccctgacgacgcgttgtgcccgctgaacgcggcggggggaccctcgcggaacgtggcctccgccacacacacaaagccatcagggacctcctcacacgtggcaggtgggagacagggctggccgggacaccacagctgctgggcacacgtaggccccgtgaaattggcagggcaggtacagtggaagtcattccaggtgacgaggcaagtcccaccattgaaacaggggtcaggactgcacatgtcctcggagacgcagcccgcagtgaggttccaggactgcctgccgccgagctcgctgggctggcttgagttatccagtggcagaggaaagaaggggaggtggcagccatcgagtcgcaggtcctggaggcagcctcggaagggcccaccccagggctggctgtcggcagcaaggagcctcccacccacgtgcacgtgctgccccaggtcctgcagctggtcaggcccgaagctgagcatcaccaggtgacggagcccatcatcccagcgcccagggagcactacagcaggactgcccggcacctcagcccggatccgaccctcactcaggaatactgttaggccagctgcggagtcattggcaaactggagcaacaggccagcggactcccgagtgcggagaaggaaagacactgtgaggttgggacctggcagctcttggagcagaaaggaggcagagcttggggcgcctcccaagccaaaggtggcagcaggaatctcatcagcgcacgtgggacctctatggggccgggcacagtcgcaacggaaatgagtccacagatccacacaggaccctccgtggacacaaggcagaggccggcactgctctcggcgctcacagcccaggaggacgttctcaccgagatcctcaggcagcaggaggtggccatccacacgcacgtcctggaggcagcctgcaaaggtcgcgtcccccagctgggcagaggagatcccggcaggcagcggagttgccgaagccgtggaagccagggccacaggaccagaggccacacagagccgggcagggcagccctcatgccagagccgtagctccagggtcgctagatggagcacaacctccacctggtgccaatggccatcgtttagggccaggtccggcagtctcaggacaagcacagtggtgctgtagctccagagtgtggcctgaagtgtggctgccaccaatgccagctccaagctttccttggtgtcattgcgagtggccaaggtcccagcgggcagtgtggtgcgaaacctcagtgccagacccagggggccaccagctggcactgatgcctgaatggggctcccagccatcacagagaaggtggtattctggccacagaacggtccatgggtaccaggtgggcagtggcagacgtaactgtggaccccagactcgaagatagggatgcaggtggcagccagcgggcaggtgtggccctggcagccagtgagctgcacagaacagtcgcgcccaccccaggtctctgggcacctgcagatatagcctgccacagtgtcactgcaggttccgccgtgcaggcagggatccgacaggcattcatccacatcttcctcacatgtcggccctgcgtagccatctgggcagtgacactggaagccattgggcaggtcctggcagtggcctccgttgaggcatggccgtgaggcacactcgtccacctccacaccgcagtcggctccctcaaagccaggagggcagtggcacaggaaacccgcagcatggcggaagctgaaggcgccagggaaggcggcctggacacccccgtagagggccgggtcagagcgctgcaggcatcggcccccatgctggcaggggctcgatgcacactcgtcctcgtccacctcgcacagctcgccgctgtagcctggccaacagaggcagcggaagctcccgaggccctcgaggcaggacgcgttgtgctcgcagggcgccgatgcgcactccagcacctcccgctcgcagtgcgtgccctcgtagccggtgcccgcgcagtcgcaccggaacccgttgaccaggtcgtggcacgtgcccccatgtgcgcacggctggctctggcactcgtcgaggtccagctggcaacgggtgcccccgtagcctggcgcgcacacacagcggaaggagcccacgccgtccaggcacgagcccccgtgcaggcagggcgctgaggcgcactcgtccacctccatctcgcaggtcacgcctgcatagccaagggggcaatggcactcgtagcgatcggccaggttgcggcaggtggccccatggtggcacggccgggatgcacactcatcgatgtccagctcgcagcgtgggccctggaaacccggcacgcagtagcagcggaagccggtgggatctggaccctggggcacacacagagcgccgtggtggcatggctgggtggcacagccccggggctccatgggcccacaggtatagccaccactctcggtagcctggcactcggtccctggagcgcacgggtctgaggcacaggcactggggggctctgaaggcaccgtcccttatagtctcctgctgcactcgatgtttgcttgctctccagctggcctcttgttggggtggacaggaggagctcttcagggggacctggttcaggaagccaggtcatctcagagacactgtaaaatggtggcgttagtgagccaaggcgacagtgccagctctctttatccagcttctcagtgatcccccagagacccaggcaatcccaatggggggctggggggagcacggcaagtcaaccaccaccctctggttctctggatgcacagacacaaactcccacactttcacagagcggggaggtcacccggcgcaggtccagtctcctctgcagcccggcccccagcactgtcctgcagccgccacactccaccttgtggccagacctggaagtgtcttgtgaggtctggagggtatggaggggggctcccccgacagcaccgggtacaggagtcccacgtgacggggaggaagccagggagtcgctggacagcaggcaggacggaggtcagacaagggcacaccatcttgaccgctccctggtccgg

SEQ ID NO: 12193 - RNA, 3784 nt, Homo sapiens
  source 1..3784: mol_type = other RNA
ctgggacaggaggaggaggcaggcacaggctgcaggtacggccacctccagcagtgggaatggcagcggcaggggcaggcccttcgccacttcacagaactggccggagaatctggcattgcagatacattcagacacccctccagctgcccggcaggtgcccccattcaagcaggggttggcttcacaggggagagtggggacctgacacctctggccagcaagaccctccaggcagctgcagttggcagcgggagagccaccctcacatgggctgccatcgaggcaggtgacattcaggctgcactccttggatgggacaggcaacctgcagcgcgggcccccgaagccaggcgggcagcggcactcgaagcggccgtcggggtgcgtgtgacagcggccacgggcgcagggggcggagtgacaggggtcgacgtgggcttcgcagcgcgggccttcccaccccgggccgcaggcgcaggcaaaggcgtcgaagaggtcacggcaggcaccgtcgtgcagacagggcgagggcgcacacacgggcgcgccgcggcagccgaggatcggggccggcgtcccaggccaagacgcgaagtgctctcgggcgccaggggccgcgccgggccggggccgcgccaagggcaggggcaggccgcccagcgccacgcggcccaagcagccggtgaagttctcagccagcaggatgcgcacagcacccgggccctgcaggaagcccaggtcactggccaggccgcgcagcgccaccggggtggcggcaccatccagccacagcagccagcgcgaggtggtggccgccgggcgctccatggccagacgcacgcggtgccaggcaccatcggccacgcgcggccccggtatgggcagcacagcgccgggcaggccatggcctccgcgcacgccccccgccagcgagccattgcgcaccgccagccacacgccttccagggcgcccgccgcggcacgcagcagccaggcctcggagtcgcgcgtgcgaaaggccagcgacaggccgccgagcaagcgccctgacgacgcgttgtgcccgctgaacgcggcggggggaccctcgcggaacgtggcctccgccacacacgtggcaggtgggagacagggctggccgggacaccacagctgctgggcacacgtaggccccgtgaaattggcagggcaggtacagtggaagtcattccaggtgacgaggcaagtcccaccattgaaacaggggtcaggactgcacatgtcctcggagacgcagcccgcagtgaggttccaggactgcctgccgccgagctcgctgggctggcttgagttatccagtggcagaggaaagaaggggaggtggcagccatcgagtcgcaggtcctggaggcagcctcggaagggcccaccccagggctggctgtcggcagcaaggagcctcccacccacgtgcacgtgctgccccaggtcctgcagctggtcaggcccgaagctgagcatcaccaggtgacggagcccatcatcccagcgcccagggagcactacagcaggactgcccggcacctcagcccggatccgaccctcactcaggaatactgttaggccagctgcggagtcattggcaaactggagcaacaggccagcggactcccgagtgcggagaaggaaagacactgtgaggttgggacctggcagctcttggagcagaaaggaggcagagcttggggcgcctcccaagccaaaggtggcagcaggaatctcatcagcgcacgtgggacctctatggggccgggcacagtcgcaacggaaatgagtccacagatccacacaggaccctccgtggacacaaggcagaggccggcactgctctcggcgctcacagcccaggaggacgttctcaccgagatcctcaggcagcaggaggtggccatccacacgcacgtcctggaggcagcctgcaaaggtcgcgtcccccagctgggcagaggagatcccggcaggcagcggagttgccgaagccgtggaagccagggccacaggaccagaggccacacagagccgggcagggcagccctcatgccagagccgtagctccagggtcgctagatggagcacaacctccacctggtgccaatggccatcgtttagggccaggtccggcagtctcaggacaagcacagtggtgctgtagctccagagtgtggcctgaagtgtggctgccaccaatgccagctccaagctttccttggtgtcattgcgagtggccaaggtcccagcgggcagtgtggtgcgaaacctcagtgccagacccagggggccaccagctggcactgatgcctgaatggggctcccagccatcacagagaaggtggtattctggccacagaacggtccatgggtaccaggtgggcagtggcagacgtaactgtggaccccagactcgaagatagggatgcaggtggcagccagcgggcaggtgtggccctggcagccagtgagctgcacagaacagtcgcgcccaccccaggtctctgggcacctgcagatatagcctgccacagtgtcactgcaggttccgccgtgcaggcagggatccgacaggcattcatccacatcttcctcacatgtcggccctgcgtagccatctgggcagtgacactggaagccattgggcaggtcctggcagtggcctccgttgaggcatggccgtgaggcacactcgtccacctccacaccgcagtcggctccctcaaagccaggagggcagtggcacaggaaacccgcagcatggcggaagctgaaggcgccagggaaggcggcctggacacccccgtagagggccgggtcagagcgctgcaggcatcggcccccatgctggcaggggctcgatgcacactcgtcctcgtccacctcgcacagctcgccgctgtagcctggccaacagaggcagcggaagctcccgaggccctcgaggcaggacgcgttgtgctcgcagggcgccgatgcgcactccagcacctcccgctcgcagtgcgtgccctcgtagccggtgcccgcgcagtcgcaccggaacccgttgaccaggtcgtggcacgtgcccccatgtgcgcacggctggctctggcactcgtcgaggtccagctggcaacgggtgcccccgtagcctggcgcgcacacacagcggaaggagcccacgccgtccaggcacgagcccccgtgcaggcagggcgctgaggcgcactcgtccacctccatctcgcaggtcacgcctgcatagccaagggggcaatggcactcgtagcgatcggccaggttgcggcaggtggccccatggtggcacggccgggatgcacactcatcgatgtccagctcgcagcgtgggccctggaaacccggcacgcagtagcagcggaagccggtgggatctggaccctggggcacacacagagcgccgtggtggcatggctgggtggcacagccccggggctccatgggcccacaggtatagccaccactctcggtagcctggcactcggtccctggagcgcacgggtctgaggcacaggcactggggggctctgaaggcaccgtcccagccaggagggaaagggcaggggcccagagcagcagtagcaggacagaggccagggcctgggggtccggggtcccaggcctggccagcgccatggcagcccgctctgcgctctgctcggctgctgtgagaacgggagggcggcctggctggctccgcacccccctcgtccctccaaccagcactaat

SEQ ID NO: 12194 - RNA, 1271 nt, Homo sapiens
  source 1..1271: mol_type = other RNA
ctgggacaggaggaggaggcaggccccagcagggctgaatgtgtagaagcgagagccctcaatggaagccaggatcctgcgatgagtctcagagatggttccaaccgctgggtacacgaataccttaaggccatcgcccctgcactttgaggtatcaaagcaagattcccagttgcagctgccaccatgaggggcttgaggaggtgaaacggcatcttctgggagctctccaggctgggagaagctctgcaggagctctgcatccagccagcggggccagccttgggaagccccgggccgaggtctgggaggcaatgccaggcggagaagggagaagcctcccagcaggacaagcaggagccaggaggctgacagtgccagccacagggactttcttctcctccacgactgcatgtggccacccacagtcagggctagggaagctgggaggcctctgccagcaagcaggaagagcagggcctggggcgggagaccagagctgggaccgacctgctagtcctgtgctgtcattgtacagatgggaagactgaggcccatcgagaccaggccgcctgtctaaggtcagatagtgagtcaccagccaggcaggaggaggccaggtgggacccagcttgctggcctggcccccctgctctcaggactctgccttctcggcctttggacaaccaagccagccttttccctcccagcagggacccctgcccctgggcactgctctggctgacgcaacccctgtccagaatgcagggccgtgtccccctgccctcctggctgcaccccttgaccttgccctcaactgagaggagggctgtctgccaggccatggggaccagtcagagctcccacaggaggcggcttggccagggacaggctggagggagctgggctggtcttcccactcctccccttgcctgagcagccctggctgcccctgtgcccgctggcagacgcttctgggctgtggcccctgtggctggagctaaaattagaccctgcatcccatgtggatcatcggcgtcagctgaggtcacagcctgggtgcagccggtgtccccctgccttggagggccaggagggctcggggtcctgatccttatccactctgccgctgcaccagctcaggaagtgcagcccctcttccccgcagcccagcagctgccttgcaccatctggcttggagctatcacagtgcagaggccagggccgctgtgccaagccccccaaaccctatggtatctcctcccatccct

SEQ ID NO: 12195 - RNA, 1286 nt, Homo sapiens
  source 1..1286: mol_type = other RNA
ctgggacaggaggaggaggcaggccccagcagggctgaatgtgtagaagcgagagccctcaatggaagccaggatcctgcgatgagtctcagagatggttccaaccgctgggtacacgaataccttaaggccatcgcccctgcactttgaggtatcaaagcaagattcccagttgcagctgccaccatgaggggcttgaggaggtgaaacggcatcttctgggagctctccaggctgggagaagctctgcaggagctctgcatccagccagcggggccagccttgggaagccccgggccgaggtctgggaggcaatgccaggcggagaagggagaagcctcccagcaggacaagcaggagccaggaggctgacagtgccagccacagggactttcttctcctccacgactgcatgtggccacccacagtcagggctagggaagctgggaggcctctgccagcaagcaggaagagcagggcctggggcgggagaccagagctgggaccgacctgctagtcctgtgctgtcattgtacagatgggaagactgaggcccatcgagaccaggccgcctgtctaaggtcagatagtgagtcaccagccaggcaggaggaggccaggtgggacccagcttgctggcctggcccccctgctctcaggactctgccttctcggcctttggacaaccaagccagccttttccctcccagcagggacccctgcccctgggcactgctctggctgacgcaacccctgtccagaatgcagggccgtgtccccctgccctcctggctgcaccccttgaccttgccctcaactgagaggagggctgtctgccaggccatggggaccagtcagagctcccacaggaggcggcttggccagggacaggctggagggagctgggctggtcttcccactcctccccttgcctgagcagccctggctgcccctgtgcccgctggcagacgcttctgggctgtggcccctgtggctggagctaaaattagaccctgcatcccatgtggatcatcggcgtcagctgaggtcacagcctgggtgcagccggtgtccccctgccttggagggccaggagggctcggggtcctgatccttatccactctgccgctgcaccagctcaggaagtgcagcccctcttccccgcagcccagcagctgccttgcaccatctggcttggagctatcacagtgcagaggccagggccgctgtgccaagccccccaaaccctatggtatctcctcccatccctctccagtcggcaact

SEQ ID NO: 12196 - RNA, 1289 nt, Homo sapiens
  source 1..1289: mol_type = other RNA
ctgggacaggaggaggaggcagggaagagggaatgtcatcagtgactcaggtttggtagaaagatgctgcaggcgctgggctttgctcccacaacggggtgctggccgcagtgcaaactgagggtgagcaagtagagggcctgggttctgcagctctgcagggagagcgtggctaaaggccttggatcaagtcctggccttttctttgcggataacagcagaggtcagaagtcagggaggagctgctgggagcccagccttgttggagactggccgcccacctggtgccctgtggctcagtgggaagtgtctatgggcctggggcctgggctgagctgggtgcagcagagacctcccttgatgctgcatgtgccgattccttaaaacccaccagacgagcagggctgacagcaccaggctcttggctacgaggagtccacagaacacaggcaccagggcaatgggggctgcagggccagggcggagcgtggagttctgtggctgtgaagggacagggatggtagatggagactcaggggcttgtctggctcctgcagtgggaggcacacagctctgggtctgggtctgtgaagagaccaggtcgcggggagtccaggaggtctgtgtggaggcagaggctggagataccaccagatagaatctgacggacttagagacagagttgtcagaagggcggtagattctacaccagtaatgtcctgagtcttcctctctcagatcagtcatggtgacagtgaagaagccagcatcagggtcgtcccagattgtgaatcgagaggtccaagccatcgtcctgggcttggagctggtgactaacctgatgcacacaagtgctgaagcctccttacaccagcctttcttctcgtagagactgcccgtgggcgggtactggcatctcacggttagcgtctgccctgccacactttgaagtacctgagccttggattgtgcctgagagcctgggaacagcagcagcagcagtagcagtgggtgtagggctcgccaggccatgtggtccttttcctgtgcgctcatgggaggggacacctggagaagactggggagagggaattgggagctgggcctgattctgctgctcttccagcacgtctgatagaaaaatgagacaggctgaggcctgggttggggagatgggagactgcaaagggcagattctgtgggcacagggaagtggggatctccagctgtaggtgagtctgggtctggtgggctcggcgctgtctggcacacagcttcccaggcctctg

SEQ ID NO: 12197 - RNA, 784 nt, Homo sapiens
  source 1..784: mol_type = other RNA
ctgggacaggaggaggaggcagggcccccaaacagctgcgtcaggctgccctggctcccagacagcccggtggcccgaggacccatgaagctaggcagggacggagcccctcgaggtttgggcagcactggcttgaaggctgttgggcggatcaggatcttctccatgttcttctccagctttccagagacagggatgagctttggtggtgggccgcggaggtgggcattgtgtgcccgctgctctcgggcatcctcaacatcactgcttgggctggggggtgactctgtccggaagtcctcattgatgtaggtgaagctggtgacagggacagccttcctagggggcacagctgggcacagcggctcctgtgcctcatagccaccccgtagcaggccatcctgctggcggaagaaggtgggcccaggagggccgtggtggcggggaggagctggccccccgggacagggccggcctgagataaggctgctcacactacccatgactggagcttgtggggcagtggcagcttcaggagcaggctccagtggcactggcagagtctgcacaatggccatggtggcagaggctcaggcctggccagcggcctcgcaggcgacccagcgccacctgcgcctcggctccagttccggccccgctcctgctccagcgcgcccacctcctcgccgcgacaacgccggctccctagccggctccgaactctaggttccgaactctgggctcccggctcccagctcccggcgcccgcctggcccgacctggt

SEQ ID NO: 12198 - RNA, 752 nt, Homo sapiens
  source 1..752: mol_type = other RNA
ctgggacaggaggaggaggcagggcccccaaacagctgcgtcaggctgccctggctcccagacagcccggtggcccgaggacccatgaagctaggcagggacggagcccctcgaggtttgggcagcactggcttgaaggctgttgggcggatcaggatcttctccatgttcttctccagctttccagagacagggatgagctttggtggtgggccgcggaggtgggcattgtgtgcccgctgctctcgggcatcctcaacatcactgcttgggctggggggtgactctgtccggaagtcctcattgatgtaggtgaagctggtgacagggacagccttcctagggggcacagctgggcacagcggctcctgtgcctcatagccaccccgtagcaggccatcctgctggcggaagaaggtgggcccaggagggccgtggtggcggggaggagctggccccccgggacagggccggcctgagataaggctgctcacactacccatgactggagcttgtggggcagtggcagcttcaggagcaggctccagtggcactggcagagtctgcacaatggccatggtggcagaggctcaggcctggccagcggcctcgcaggcgaccccagaccctcagcctcacaagaacagactgagcccctctccccagcagagccccctcctctggccttgccctgatccctgcctcctggggcaccgagagcctcctcctctttctggcagcctgcccagctc

SEQ ID NO: 12199 - RNA, 765 nt, Homo sapiens
  source 1..765: mol_type = other RNA
ctgggacaggaggaggaggcagggcccccaaacagctgcgtcaggctgccctggctcccagacagcccggtggcccgaggacccatgaagctaggcagggacggagcccctcgaggtttgggcagcactggcttgaaggctgttgggcggatcaggatcttctccatgttcttctccagctttccagagacagggatgagctttggtggtgggccgcggaggtgggcattgtgtgcccgctgctctcgggcatcctcaacatcactgcttgggctggggggtgactctgtccggaagtcctcattgatgtaggtgaagctggtgacagggacagccttcctagggggcacagctgggcacagcggctcctgtgcctcatagccaccccgtagcaggccatcctgctggcggaagaaggtgggcccaggagggccgtggtggcggggaggagctggccccccgggacagggccggcctgagataaggctgctcacactacccatgactggagcttgtggggcagtggcagcttcaggagcaggctccagtggcactggcagagtctgcacaatggccatggtggcagaggctcaggcctggccagcggcctcgcaggcgacctccgccgcgctgctccatgctcagccccaggccgcccccagcgctccacaggcgcgccgcccggccccggctccggctccggccccggccccggccccggccctggcccgcgcgccgccactcggagctgcccggcccagcccc

SEQ ID NO: 12200 - RNA, 1021 nt, Homo sapiens
  source 1..1021: mol_type = other RNA
ctgggacaggaggaggaggcagggcccccaaacagctgcgtcaggctgccctggctcccagacagcccggtggcccgaggacccatgaagctaggcagggacggagcccctcgaggtttgggcagcactggcttgaaggctgttgggcggatcaggatcttctccatgttcttctccagctttccagagacagggatgagctttggtggtgggccgcggaggtgggcattgtgtgcccgctgctctcgggcatcctcaacatcactgcttgggctggggggtgactctgtccggaagtcctcattgatgtaggtgaagctggtgacagggacagccttcctagggggcacagctgggcacagcggctcctgtgcctcatagccaccccgtagcaggccatcctgctggcggaagaaggtgggcccaggagggccgtggtggcggggaggagctggccccccgggacagggccggcctgagataaggctgctcacactacccatgactggagcttgtggggcagtggcagcttcaggagcaggctccagtggcactggcagagtctgcacaatggccatggtggcagaggctcaggcctggccagcggcctcgcaggcgaccttctcgcacacaatacagtctccctaacacccacaagacctttcccacatgcagccgcagtctcagccgtcacgtgggtccgcgttccttctttccataatcttccagtccacctcacacacagacacggtgtcacaggcctgttgggcacaggcttccacaacaatccgcagtccttcgcacccagtcacagtctcaagtgcacttagtctcctaaccatctttcacgcattgacagcctctattcacagtcactcacacagacaacttcttacacgccgtgcttcacaaatattctaccgcacagcctttcccctaggggtctcggtgacccggtcaggtcagctgatgcctgcatccctgggcaaaggcagcctttctcccctaaccaccccctccc

SEQ ID NO: 12201 - RNA, 995 nt, Homo sapiens
  source 1..995: mol_type = other RNA
ctgggacaggaggaggaggcagggggagctccgaggggcgggcctcagcagggcgaggtggagatgtgcaggtggtccgggtacttgatggcgggagggtagttctgcgtcatttggatggacacgtcgctggagatgtcggaggggctccggccgcggcgccacgcctcgggctgcaggaactggcccgagtagtcggagcagtcgctgagacgcgggcggtagaaggccgggtgtggacggtacatctcctcctccgcgtagcgcttggtgaacaggtacacggacatcacgccggccccccgatagtatgaagaagatgccagagacaaaagccagaatggtcctctgcgggcggatgtggccgatgttgctgatgacgaaggccgtgaacacgaggaagaggctgaccatggggaagggggtggccgtgcgcactgtcttcagaatattctccgtgttttccgtcaccaaattgatctccggttcaagaaaatattctgaggccacacagcgacctttctcccgacctgcaaagaagcagactcgccagaggccggcgtgcagggccatcttgacctcggtggtctggttctgcggtagcactgtgccttcttccatgtacagccagtagtcagtgctgaccgcgatgcctaccaggagcaggccacacgcaccaaacacgctgctcagcagggtcagggcgcggctgctgcagtgactcatcctcagaggcagggggcgccctgcggggcctcgctcagggctgggcggacgctccgggccgcgggccccgcagccgcatgaccggccccgaggcttcccccggccgccgccgccgccaccggggtcgccggtgcccgcgccccccgcccccgccccggagcccggcgtcccggccccctcccggcctcccaccccccaccccccgcggccgcggcctcactcggcggacggagccgggagcaggaaccggcggccgctcattggctact

SEQ ID NO: 12202 - RNA, 1141 nt, Homo sapiens
  source 1..1141: mol_type = other RNA
ctgggacaggaggaggaggcagggggagctccgaggggcgggcctcagcagggcgaggtggagatgtgcaggtggtccgggtacttgatggcgggagggtagttctgcgtcatttggatggacacgtcgctggagatgtcggaggggctccggccgcggcgccacgcctcgggctgcaggaactggcccgagtagtcggagcagtcgctgagacgcgggcggtagaaggccgggtgtggacggtacatctcctcctccgcgtagcgcttggtgaacaggtacacggacatcacgccggccccctctttgagtaggaaggaggaagcggcgaaggcaaaagaccacccgtagcgataatgaaaatactgctcagagctgctgggcctgttcatgacctcgtcgttgatgctggagatgtaaagaaccaagcccaccaccaaggagaggcccgatagtatgaagaagatgccagagacaaaagccagaatggtcctctgcgggcggatgtggccgatgttgctgatgacgaaggccgtgaacacgaggaagaggctgaccatggggaagggggtggccgtgcgcactgtcttcagaatattctccgtgttttccgtcaccaaattgatctccggttcaagaaaatattctgaggccacacagcgacctttctcccgacctgcaaagaagcagactcgccagaggccggcgtgcagggccatcttgacctcggtggtctggttctgcggtagcactgtgccttcttccatgtacagccagtagtcagtgctgaccgcgatgcctaccaggagcaggccacacgcaccaaacacgctgctcagcagggtcagggcgcggctgctgcagtgactcatcctcagaggcagggggcgccctgcggggcctcgctcagggctgggcggacgctccgggccgcgggccccgcagccgcatgaccggccccgaggcttcccccggccgccgccgccgccaccggggtcgccggtgcccgcgccccccgcccccgccccggagcccggcgtcccggccccctcccggcctcccaccccccaccccccgcggccgcggcctcactcggcggacggagccgggagcaggaaccggcggccgctcattggctact

SEQ ID NO: 12203 - RNA, 5129 nt, Homo sapiens
  source 1..5129: mol_type = other RNA
ctgggacaggaggaggaggcagggggagggagcgtggtcttcaggaaggtggtgaacactgggagtcacagatcagcacgctacacacacccacactcacgtatgtgcacaccatacacacagcacgcacacacacaccccgagctctaggccctacgtctaacacacagcgaagacacagcaaaaggctacaacgagcactagcgcgcccacacctagcaagcacacagccccagctcagcccctcccgctggggcctggcccagccacacgctacaaaattaaaaatatatcaaatatacaatgaaaatagatctgtacagcactgaggatgaaaatagtccaccagccacagtataatattgggtttgtcatttaacagcatttacacccacatgtacagagtgaatatacaatagaaacagaatatatagaagagtatatatagtagagtgtctctcctggggctctgcttttcctgttgctaattctgcttgggatttggcaaggggccaggtaggaggtgttgtcgggtgagggggactgcggtgggatgttgtgccccaaaagctcatctctttggggagatgtgggtctctctctcccctcaaacactcaggaaagacaggtagggcagagggggctagaaaggggaagctgtggaagagggatgagtaagggagatggcagggttgggggatagactgctcccaggcttgggggaacagtaaggaactcaggggtaaaggaggggaccctgattctggtctgtccctccaggtcctaagagcaatctgagccacaagagtgacttgcgacccttcgtgagggtgtccgggttgagcactgtggcctgtttctgccctgcccaccagagctctcaaagatggagccagtattccctcctttctccctcctttccttccttcccccaccccatccgtccatccatccatccatctatccatccacccccaccccccaacccatccatccatccatccatccatctatccatccatccacccccactccccaacccatccatccatctatccatccatccatccatctctctgcagacatttactcttgggtcaggttcctccctggctgcactctgagaatgggttctcttccagaggaggccctgaaggtaatggcaggtggggtcgctgttgtcagctgcagccttctgcacaggctggcctccatcctgaagaccagcccttgcctttggcagcctctactgtccacagcactgcctatggcactggccactgtgggccaggaaggcttgggaaaggtttccaaggtgtctgcacatgatgtgcacactgggcggctgtgcttgtgtaataaggagagtgagtggtggctcaaaggggcagtgaaattatctgtctttccccaggagtgaggcttcctggggataagcctgtgaactccagggacccctgttccaggggaaaagctgccactagacagaacattggaccccaggtgaggagggaggggagtgtgcttcaccattgtgctccaaaccatctaatttgtgctaggaaccaacaatttgtgctctggaaacctctccgtgcactgtccttctctctccaggaaagaggcagaggccaccactgtgggctggggaggggtgctggggacagggagatggctaagccctaattgaggtggggaaggttctggtcccggtcactgcactcccagacaagatgcaggagcacacaccacacaccccaggcagggccaaggacatgggaagattccacccagggaccagggcagaggaggttcctcaccttctgctaccaaggctcatgctgaagccaagggcagcacatacctcagaaaacagaacttggggcttctgcctaggccctcccaagtctgagccctgagccctggcacacctgctcccaccctccgccttggagcaggtagcctcttggaccaggagcaaccccgtctgggctgggcaggatggtgtcctgttctcatggcagagtgagccaaagtccactctccttccccagccccaaggcctctcaccaccaccatctgaccccacagccctaagaactgcaggtggcaagttacagggagagagggaggtgagtgactcctgcagtggccacttggaatctcccatggactgggaagcaggccttatgggttgttccaattacatggctacaatttggcggaggctcttggagggctagatgagtggggtcctgaattaggaaacagagctgctcccagcctcctgctcagggctagggagcagagtctactgggactgaagaggggagtgaggcagggcagaccctctcttcttgggcaaagggcctggcctgggcctggtggccacctcaagaaagaggccaggcctggacaagtgggcaggttgagcgtggggggagaggcgggcagggcttgggcagtggtcacagctccgactcaggggtgctggccagcaggtagccgctcccatagcgtccattggggttaccgctggtctccaggggtgatgtgctgccgggccccagataggaacggtgagtgggcatgggggaaggtgcctcactgggcaccttgctgaggatgaagcgggtctcatcgttctcctccaggttggagatgtccttcatcatgcggcccttcttgtaggacacggagagggtgttggagccatcagagagcaggtggaagtgccgcaggacgaacaccacagggatgggcagcgtcgccacgacgatgagggtgatcaggagtgccatggcccagttggggaaatacaggtagcgctcggcagcctcctccttgatccaggcgctgtagcccgggggcgtgacccccagctggatgatgctggctgtggtgagcacagccatgcatagtggagacacgaacttccacatgtagaaatagaagcggtaggggcggaagcccagcatctccgtcagctcctgcatgaacttcttggttccataaatccaggccacagcgatgttctcaaggatgacgatgagagtgagtggcagggtggccgagtagtcatcgaacatggtgacaaagtagtttccggagcgctggacgaacaacagccccacgaggaatgcaaagacacagcagcccactgtgaacatctccttgggcaccttgaaggtgtcgatgatgggcgtggtgatgcctgccatggtcccgatcatgctgcccaggcccaggttgataagcatcaagaagaacatgacggaccagaacggggaggcggggaagtgcgtcatggcctcagtgaaggcgatgaaggccaggcctgtgccctgcacggacttgtccagctcgtcctccagaaggcaggggtcaaggcccagggctgagaactggtcctccttcacggtcatgatgacattgtacatctccatgtagtcctttgtggtcaggtgggagaagttgacgtggggtgggatgaggtcccggctcaggacgttggtgttaaggtaccctaggattttctcagcattctcgaccacacacttctcattcatgatgttggccttgaagcccagcacagcaaacaccacgagggtggccaacactgacgtgaagaagttgatgaaggacaccagggcggcatcgaagtggcagttgttgtcctgcttattgtagctggagaaggcaatgacaccaccaaagcccaggcccaaggcaaagaagacctgggtagctgcctcccgccacacctgggggtccagcatcttgtccagcttgggagtgaacatgtgtaggatgccatcaactgcccctcgcagcaacagcccccggaccaggaagcaggccagcaccacgtaggggaagagggagctgaaatacatcaccttccccgaggactggatgcccttaacgacagccatccccacgatgctccaggccacgaggaggcacagggtcatcttccagttgaggcccccactctccgagatggagtcagagatgtccaaggcctctcggtaccagaagtaggtagtggctgagctcttttcacactctgcctccaccactgccacgctcccattcctgacgacaggacattcactccagggcagcgggtactggaaggacttgaagaaatagaagatgctccacccgatgatcacattataatacagccccacaaagagacagactatgcagctggagaagccgatgccccccaggcggggacatatatagtgccacacaccgatgctgccgcggcggatcctctgacccacagccagctccaggaagaagagggggatcccgatgatgatcagcagcaccaggtagggcaccaggtaagcacctcctccatttttctggcacaggtaggggaacctccagatgttgccgaggcccacagagaagccaatctgggccaggatgtactgcagcttactgttccaggccggccggtcctctgcatccagctcctcctccaccgccttctgcttgccgcctgcctcaccagccacattcagtacactctgcttatagtccacaggctcctcgagggccagcaggtcggccacggactcagtgacatgctcactgctgtgctcacgctgggtcactttgctgttcttcggcattgatgccacctgggccgtgtagccctgctccccagcacacagagaagatggaattcagctgctgtcagctccttctcattcagggacctgtcacgcgtgggtagtcgcgcagactcggcccgtgcactccggccgagcagctgcgatccccgacgggtcgcggacgcacagctcctcccccgggccacaggcccccggctggggctggggcgacccggagctgcgcgccggcgcacgcgactccgctcgctcctcactccctgcctcaccaccagtcccaacctggctcccgcccgccgcgcgctcggggctcaggggagcggcgcggggacccaggtcccacggcggagagagcgcgcgggattgcgaagactggggccgagtgccgccctccctgcgccctggcagcgccggctctgcggagcagaacggagctgggcggagcgctgcgcgcactgttccctcgctttccgaaag

SEQ ID NO: 12204 - RNA, 1311 nt, Homo sapiens
  source 1..1311: mol_type = other RNA
ctgggacaggaggaggaggcagtaaggtagatgatggttcttcctcccctccttttttaggctcttctgtgtagagcagggccaaagcagccctaactaaagcccataacattaaagatgttactgggacctgttgcccttgtacataatgttgtttaagatttcttcccaattgctcccagagccctaggtctagtgtgccttcttctgggaaccatgggttatggaatacaacagtttgcattacatcccttaattgagcctccgaaaccaagtctccactagctttaagcagctgtttcaatacttttatctactgttgctgttgagcttataactgttgtcccatgatgaaaccctagcttgaaaatcccctcgaacttagaaatccccagtggggaccaattacttactgagcagtcactttatttttgagggttcagtccagatccgttgcagcattcctcatacagggcaccacttgccggatctgtcctgcagaccctggctgactgatggatgaaaagagtactcacacacagctatgcagtgtgtaagagcagctaggagactgcctggctcaagtggccaaagtgcagccccgagaagctggagctgcttgcttttattcagtgcaggcagaatgccgaaagcctggggcaaacacaatctgtgggtaattaatatttattgttcccctttcagggaatgtcacgcacacacgcacacacggatgttcaaaggtcaattccaggataacttcaaacaagcctgatcaagataatttccccttgctcccttgcacttgctccttaccctctgcctcaaggttagagaacagttgccttcagctattctcccctgaagttgtgcagagccttgctaaaagctcctctaactttataaacgaaatctgaacttccctatttcagaatgctatctctatcactttggaattggtatttccaggtgttcaatccttatgctttgtgcttgaataaattctttatattcttcagtgtgcaagaagaagggcttaaacaaaaacaagaaaaatatattctgacctttttggttatttttgtttgataagttgttttctccatgggacaatattttctccatgggacattattttctccatgggacaatgtttcatatcctagataataaggaccatgtgtggttcacctttgtggtttgattcaagtaatgtgggcatttcagatgtgaaaggctttgaggaacaacgcagagtaccttgaaatgagaaagctgaactgtttaaagcaaaaggtggctgggtgtggt

SEQ ID NO: 12205 - RNA, 313 nt, Homo sapiens
  source 1..313: mol_type = other RNA
ctgggacaggaggaggaggcagtaaggtaggtgatggttcctcctgccttcctttttgaggttcttctgtgtagagcagggccaaagcagccctgactaatgcacacaactttaaaaatgttactgggacctgaagcccttgcatacgatgttaagatttctccgcatttgttcccagagctctaggtctattgtcccttcttcaaggaaccatggcttaagggaaacaacagtttgcattaggtcctttaattgagcctgtgaaaccaaagctccagtagctttaagtagctgttccaatacttttatatac

SEQ ID NO: 12206 - RNA, 488 nt, Homo sapiens
  source 1..488: mol_type = other RNA
ctgggacaggaggaggaggcagtctcctgctcctcagtagcaggagcctgcgcacccaccaagcccagggcctctccttgggcctcaaggccttcctcaggcttgcagtgctgactcctctgctcaagtggcatgatgactctggtcagggcagcaggtaggagtgtgggcaggagctagtgctgctccggggcctgtctcctcagaacctggatgcttggtagatcttaggaccactgtgtctgtcgactacatgggggcccctgtgttgacctgagtcaccctctgaagaaaaggtcctcaactccctgagataccagagttccctgcggttaaagcggcggggggtggcggggtgaggtggtggcgactcagcctgagaagtcttcccctgcagggtggtccaggcccggcagcagaggcagcgctggattattgggggccctctgtctggggtgaggcccgcctcagtcctccctcggcatctt

SEQ ID NO: 12207 - RNA, 418 nt, Homo sapiens
  source 1..418: mol_type = other RNA
ctgggacaggaggaggaggcagtctcctgctcctcagtagcaggagcctgcgcacccaccaagcccagggcctctccttgggcctcaaggccttcctcaggcttgcagtgctgactcctctgctcaagtggcatgatgactctggtcagggcagcaggtaggagtgtgggcaggagctagtgctgctccggggcctgtctcctcagaacctggatgcttggtagatcttaggaccactgtgtctgtcgactacatgggggcccctgtgttgacctgagtcaccctctgaagaaaaggtcctcaactccctgagatcttgcctcctcacggagcctgcgcctgcttccctccaccgacgtcaggccgttgctcagggcgagaatctcgctgttctctgacctccaacgcgcaagtcagt

SEQ ID NO: 12208 - RNA, 312 nt, Homo sapiens
  source 1..312: mol_type = other RNA
ctgggacaggaggaggaggcagtctcctgctcctcagtagcaggagcctgcgcacccaccaagcccagggcctctccttgggcctcaaggccttcctcaggcttgcagtgctgactcctctgctcaagtggcatgatgactctggtcagggcagcaggtaggagtgtgggcaggagctagtgctgctccggggcctgtctcctcagaaccttgcctcctcacggagcctgcgcctgcttccctccaccgacgtcaggccgttgctcagggcgagaatctcgctgttctctgacctccaacgcgcaagtcagt

SEQ ID NO: 12209 - RNA, 584 nt, Homo sapiens
  source 1..584: mol_type = other RNA
ctgggacaggaggaggaggcagtggacatggtggctctgcgggccctggacgccgccggccgacacggaggcgcggggcgggaggcgcgcgagcgtgtgggagccggcgcgatagtgcgtgcgagtgtgtaagggggaggggcgggggtatcgctgtgggggaggagtctcggggctccccctccccaacgcacacccccgccgcctcggcgaggggggaggggaaggctgcgaaaacaaacgtccaacggccgcaaccgcccggctgggctcggtgtggcggtcacggccggggccgcaaggagcccggagccgccgccgccaccgctccaggcatcgtgctgacagggcaacggcccggatcacgcagccccgagggccgctcgcagccttctcctcagccctcgcagggctgcacgcacgggagaacccggcagctgcaaggagggccgggacccctgcttctggggaccagggtagagagaaagggcctcgaggtgctggcgctcctcggagtccgcgccaccgcaaacgccgccgccgccgccgccgcttctacccactcctcactccgaatggcaact

SEQ ID NO: 12210 - RNA, 315 nt, Homo sapiens
  source 1..315: mol_type = other RNA
ctgggacaggaggaggaggcagtggcactttctttggtgtgggctggtcctctcttaggcaggccatagacctgtgtttcccaggagtctacaactctcccagcgagagtcaggagggaaatgaaggagaaagtacacttccagggctcaatcagccagtccaccaggagttagaagtccctgagccttcattgtatatggacacaggaggcttccctggtatgagtcaggaggactgggaaattgctttcttccatgcaaaaaagtatgattatactactcgcatcctcaaatgacactctgccttttcagtca

SEQ ID NO: 12211 - RNA, 2803 nt, Homo sapiens
  source 1..2803: mol_type = other RNA
ctgggacaggaggaggaggcagttcctgcttagatttttttgtaattgcttgttctcttacacgaacagtctccaaaaggtccttctgaggaatctgagacatccccagctttgctacagcctgagtcacctggttggaggaatcttctagtctctgaaccaaagaatcccatctttgagtcagttcctctgagtcactgttgatcttcttagatgccttggaattatcaagtaattgtcccacatcctggccaatctcactcagctgatccaatgtttgacgcttcatttccatgtcttccttcaaaatagccagacgtcgaacactgacacttagttccttttggtctttgaagttgcttgtctggactttatttaaagcctcttctttttcggttaaccaagctttcaacaagcactgttcttccaataattcctgccacaatatattgatttcttgtaacctattccagcgttcttcagtccaacggcatactgctgtccagcgctcaccaagtttctgtaactggtcttctaggatagctgtagcactctcaccactgttttcatcaacaatgaccaccatgtgagttagtgaatttactttcacctgttcagcctcaagatcactttgcaaacttttatgttcttctagcagcttttgtagagattttacatcatcatccagggggcaagtttccatcttctgaatgcgctcctctgtgagtgttaaccaggcggagagctgctgcagttgcttcttctgcagttccatcagcacatcgtgcagccgggactgtctgtccatactctccaccctaagagcctcccatctagcattcagcagggtcatctgttcctgaatctcaaattcttcttcgtctgacagagttccttgtgttatcagttggttgcctgcctgcaggacgctgcccacactgctctggtgtgcagtcagttccatcataaaagcttcatgggttgcaaactggtctttgacttcttcaacatcatcagaaatatcatcctgctcctggaaagtgtcctcagcagaaagcaaccaggtcagcacttcctccaacgcaatctgatagctgtccagatccatgtcaacctcagtgacagtgctgggagtttcagctcggggactctcatgctcctcctcaggcgctgtactctgtatattaattgcctcttcttcacattcttttttatatttccttgggagtgtctctacctcacggatggcgtctatggtgacttgctgaggtagcacctcaaacaaagatgttaaatacataattatggatttcttgtcaggaagctgaacggcaacatcttcaggatctaacagcttttcaattcccaaataagtttgagccttgctgaaggcatgttcaagtctctcaattggtgacattttgacaactttatcccagctgaagagatcaggtttatgtcggtggaggacagcattaaaggcgagtccatctgtccagctggtggtgaagttgaggacgttgacttggctgtagggcctggtggtctgacgcacccagctgagcaggatcttctcactgttcgtctgctgcaggtccgacatgacatccttcatgacatctttcacctgccagtgcaaaatgatgctccaaagtaaccccaaagtcagtttgtgatttccatccacaatgtcagttccccctatattcactaattccacattgttctgatgtaaaacctgcagcactctgttgacgttatttaaggcatgtacccttgtggaaccacgttcctttggcagtgatgttcctgtgaggccttctagaagatccaatagcttccttccatctttgaggtctgtgaacatatcattgatgggtggtttcccactctttgaaaatcgagcatttatccatttggtaaaggttttcttctgtacgtcattgtgttcatcaattaggttgagttggtgatgcaatccgatggcaggagattgcagctggggaatctggtctgaatgcggaatgaggagcaaagggccattatctctctctcctgtagtaggagagggcagatctggacttaatgatatcactgaattcgttctgcccattgtcaggactggcttcatgttctccatacttggccatcttgccagagtttcaagataatccaaaaactttaccaagtcctctttctaaggctttcaacttcctacgatggttcagcttgacatcaatacctgctgcccgcgggcctcctcgcctgccggtcgccaccgccgcaccccgagctggccaagggctcctctaggagtttgacacggagtaaccgcgggggtgtgtgcgagtgttagtttggtggtgcgatgtatttaaaaaaaaaaataaagcttggagaagcagacacgaaccgaaattttaaaaaaagaaagaaagaaagagaaattgacacccgactgaaaacgccccttacttgtgcaatcttcctgcctggtagttccgccaaaaacaaaacagtcaaagcgcaaacctggaaggggcgcgcaggcaccaactttgccaaacgctacagagttttccgtttgcagaaatgacccaaaagaaggggggcgccgctccccgtgattccccaatcggcttctggagccagaggctcctcctcgcccctcggcgggagaaagcccgcggccggctgctgctgcccgcttccctgctccgaggaaaaacgactccacaactttgtgcgcgagagaggctcgctccttcggcggctcctcctcctcctccccgctgcgggcctg

SEQ ID NO: 12212 - RNA, 2344 nt, Homo sapiens
  source 1..2344: mol_type = other RNA
ctgggacaggaggaggaggcagttcctgcttagatttttttgtaattgcttgttctcttacacgaacagtctccaaaaggtccttctgaggaatctgagacatccccagctttgctacagcctgagtcacctggttggaggaatcttctagtctctgaaccaaagaatcccatctttgagtcagttcctctgagtcactgttgatcttcttagatgccttggaattatcaagtaattgtcccacatcctggccaatctcactcagctgatccaatgtttgacgcttcatttccatgtcttccttcaaaatagccagacgtcgaacactgacacttagttccttttggtctttgaagttgcttgtctggactttatttaaagcctcttctttttcggttaaccaagctttcaacaagcactgttcttccaataattcctgccacaatatattgatttcttgtaacctattccagcgttcttcagtccaacggcatactgctgtccagcgctcaccaagtttctgtaactggtcttctaggatagctgtagcactctcaccactgttttcatcaacaatgaccaccatgtgagttagtgaatttactttcacctgttcagcctcaagatcactttgcaaacttttatgttcttctagcagcttttgtagagattttacatcatcatccagggggcaagtttccatcttctgaatgcgctcctctgtgagtgttaaccaggcggagagctgctgcagttgcttcttctgcagttccatcagcacatcgtgcagccgggactgtctgtccatactctccaccctaagagcctcccatctagcattcagcagggtcatctgttcctgaatctcaaattcttcttcgtctgacagagttccttgtgttatcagttggttgcctgcctgcaggacgctgcccacactgctctggtgtgcagtcagttccatcataaaagcttcatgggttgcaaactggtctttgacttcttcaacatcatcagaaatatcatcctgctcctggaaagtgtcctcagcagaaagcaaccaggtcagcacttcctccaacgcaatctgatagctgtccagatccatgtcaacctcagtgacagtgctgggagtttcagctcggggactctcatgctcctcctcaggcgctgtactctgtatattaattgcctcttcttcacattcttttttatatttccttgggagtgtctctacctcacggatggcgtctatggtgacttgctgaggtagcacctcaaacaaagatgttaaatacataattatggatttcttgtcaggaagctgaacggcaacatcttcaggatctaacagcttttcaattcccaaataagtttgagccttgctgaaggcatgttcaagtctctcaattggtgacattttgacaactttatcccagctgaagagatcaggtttatgtcggtggaggacagcattaaaggcgagtccatctgtccagctggtggtgaagttgaggacgttgacttggctgtagggcctggtggtctgacgcacccagctgagcaggatcttctcactgttcgtctgctgcaggtccgacatgacatccttcatgacatctttcacctgccagtgcaaaatgatgctccaaagtaaccccaaagtcagtttgtgatttccatccacaatgtcagttccccctatattcactaattccacattgttctgatgtaaaacctgcagcactctgttgacgttatttaaggcatgtacccttgtggaaccacgttcctttggcagtgatgttcctgtgaggccttctagaagatccaatagcttccttccatctttgaggtctgtgaacatatcattgatgggtggtttcccactctttgaaaatcgagcatttatccatttggtaaaggttttcttctgtacgtcattgtgttcatcaattaggttgagttggtgatgcaatccgatggcaggagattgcagctggggaatctggtctgaatgcggaatgaggagcaaagggccattatctctctctcctgtagtaggagagggcagatctggacttaatgatatcactgaattcgttctgcccattgtcaggactggcttcatgttctccatacttggccatcttgccagagtttcaagataatccaaaaactttaccaagtcctctttctaaggctttcaacttcctacgatggttcagcttgacatcaataccttgtcagttgcagcaagagatccccagagtccggaaaaggagagccggcgactgcgcgggactacacaccaatggggcgcccccctcctcctgtcccctca

SEQ ID NO: 12213 - RNA, 2124 nt, Homo sapiens
  source 1..2124: mol_type = other RNA
ctgggacaggaggaggaggcagttcctgcttagatttttttgtaattgcttgttctcttacacgaacagtctccaaaaggtccttctgaggaatctgagacatccccagctttgctacagcctgagtcacctggttggaggaatcttctagtctctgaaccaaagaatcccatctttgagtcagttcctctgagtcactgttgatcttcttagatgccttggaattatcaagtaattgtcccacatcctggccaatctcactcagctgatccaatgtttgacgcttcatttccatgtcttccttcaaaatagccagacgtcgaacactgacacttagttccttttggtctttgaagttgcttgtctggactttatttaaagcctcttctttttcggttaaccaagctttcaacaagcactgttcttccaataattcctgccacaatatattgatttcttgtaacctattccagcgttcttcagtccaacggcatactgctgtccagcgctcaccaagtttctgtaactggtcttctaggatagctgtagcactctcaccactgttttcatcaacaatgaccaccatgtgagttagtgaatttactttcacctgttcagcctcaagatcactttgcaaacttttatgttcttctagcagcttttgtagagattttacatcatcatccagggggcaagtttccatcttctgaatgcgctcctctgtgagtgttaaccaggcggagagctgctgcagttgcttcttctgcagttccatcagcacatcgtgcagccgggactgtctgtccatactctccaccctaagagcctcccatctagcattcagcagggtcatctgttcctgaatctcaaattcttcttcgtctgacagagttccttgtgttatcagttggttgcctgcctgcaggacgctgcccacactgctctggtgtgcagtcagttccatcataaaagcttcatgggttgcaaactggtctttgacttcttcaacatcatcagaaatatcatcctgctcctggaaagtgtcctcagcagaaagcaaccaggtcagcacttcctccaacgcaatctgatagctgtccagatccatgtcaacctcagtgacagtgctgggagtttcagctcggggactctcatgctcctcctcaggcgctgtactctgtatattaattgcctcttcttcacattcttttttatatttccttgggagtgtctctacctcacggatggcgtctatggtgacttgctgaggtagcacctcaaacaaagatgttaaatacataattatggatttcttgtcaggaagctgaacggcaacatcttcaggatctaacagcttttcaattcccaaataagtttgagccttgctgaaggcatgttcaagtctctcaattggtgacattttgacaactttatcccagctgaagagatcaggtttatgtcggtggaggacagcattaaaggcgagtccatctgtccagctggtggtgaagttgaggacgttgacttggctgtagggcctggtggtctgacgcacccagctgagcaggatcttctcactgttcgtctgctgcaggtccgacatgacatccttcatgacatctttcacctgccagtgcaaaatgatgctccaaagtaaccccaaagtcagtttgtgatttccatccacaatgtcagttccccctatattcactaattccacattgttctgatgtaaaacctgcagcactctgttgacgttatttaaggcatgtacccttgtggaaccacgttcctttggcagtgatgttcctgtgaggccttctagaagatccaatagcttccttccatctttgaggtctgtgaacatatcattgatgggtggtttcccactctttgaaaatcgagcatttatccatttggtaaaggttttcttctgtacgtcattgtgttcatcagatctggacttaatgatatcactgaattcgttctgcccattgtcaggactggcttcatgttctccatacttggccatcttgccagagtttcaagataatccaaaaactttaccaagtcctctttctaaggctttcaacttcctacgatggttcagcttgacatcaatac

SEQ ID NO: 12214 - RNA, 2991 nt, Homo sapiens
  source 1..2991: mol_type = other RNA
ctgggacaggaggaggaggcagttcctgcttagatttttttgtaattgcttgttctcttacacgaacagtctccaaaaggtccttctgaggaatctgagacatccccagctttgctacagcctgagtcacctggttggaggaatcttctagtctctgaaccaaagaatcccatctttgagtcagttcctctgagtcactgttgatcttcttagatgccttggaattatcaagtaattgtcccacatcctggccaatctcactcagctgatccaatgtttgacgcttcatttccatgtcttccttcaaaatagccagacgtcgaacactgacacttagttccttttggtctttgaagttgcttgtctggactttatttaaagcctcttctttttcggttaaccaagctttcaacaagcactgttcttccaataattcctgccacaatatattgatttcttgtaacctattccagcgttcttcagtccaacggcatactgctgtccagcgctcaccaagtttctgtaactggtcttctaggatagctgtagcactctcaccactgttttcatcaacaatgaccaccatgtgagttagtgaatttactttcacctgttcagcctcaagatcactttgcaaacttttatgttcttctagcagcttttgtagagattttacatcatcatccagggggcaagtttccatcttctgaatgcgctcctctgtgagtgttaaccaggcggagagctgctgcagttgcttcttctgcagttccatcagcacatcgtgcagccgggactgtctgtccatactctccaccctaagagcctcccatctagcattcagcagggtcatctgttcctgaatctcaaattcttcttcgtctgacagagttccttgtgttatcagttggttgcctgcctgcaggacgctgcccacactgctctggtgtgcagtcagttccatcataaaagcttcatgggttgcaaactggtctttgacttcttcaacatcatcagaaatatcatcctgctcctggaaagtgtcctcagcagaaagcaaccaggtcagcacttcctccaacgcaatctgatagctgtccagatccatgtcaacctcagtgacagtgctgggagtttcagctcggggactctcatgctcctcctcaggcgctgtactctgtatattaattgcctcttcttcacattcttttttatatttccttgggagtgtctctacctcacggatggcgtctatggtgacttgctgaggtagcacctcaaacaaagatgttaaatacataattatggatttcttgtcaggaagctgaacggcaacatcttcaggatctaacagcttttcaattcccaaataagtttgagccttgctgaaggcatgttcaagtctctcaattggtgacattttgacaactttatcccagctgaagagatcaggtttatgtcggtggaggacagcattaaaggcgagtccatctgtccagctggtggtgaagttgaggacgttgacttggctgtagggcctggtggtctgacgcacccagctgagcaggatcttctcactgttcgtctgctgcaggtccgacatgacatccttcatgacatctttcacctgccagtgcaaaatgatgctccaaagtaaccccaaagtcagtttgtgatttccatccacaatgtcagttccccctatattcactaattccacattgttctgatgtaaaacctgcagcactctgttgacgttatttaaggcatgtacccttgtggaaccacgttcctttggcagtgatgttcctgtgaggccttctagaagatccaatagcttccttccatctttgaggtctgtgaacatatcattgatgggtggtttcccactctttgaaaatcgagcatttatccatttggtaaaggttttcttctgtacgtcattgtgttcatcagatctggacttaatgatatcactgaattcgttctgcccattgtcaggactggcttcatgttctccatacttggccatcttgccagagtttcaagataatccaaaaactttaccaagtcctctttctaaggctttcaacttcctacgatggttcagcttgacatcaatacctgctgcccgcgggcctcctcgcctgccggtcgccaccgccgcaccccgagctggccaagggctcctctaggagtttgacacggagtaaccgcgggggtgtgtgcgagtgttagtttggtggtgcgatgtatttaaaaaaaaaaataaagcttggagaagcagacacgaaccgaaattttaaaaaaagaaagaaagaaagagaaattgacacccgactgaaaacgccccttacttgtgcaatcttcctgcctggtagttccgccaaaaacaaaacagtcaaagcgcaaacctggaaggggcgcgcaggcaccaactttgccaaacgctacagagttttccgtttgcagaaatgacccaaaagaaggggggcgccgctccccgtgattccccaatcggcttctggagccagaggctcctcctcgcccctcggcgggagaaagcccgcggccggctgctgctgcccgcttccctgctccgaggaaaaacgactccacaactttgtgcgcgagagaggctcgctccttcggcggctcctcctcctcctccccgctgcgggcctgcccctttgttggagccgagcgctggaggcggaggagggagggtggggcgcaggaccgctgggtcgcgcgttgccgcccccaccccccgggaaggggctcgcctccgggcagccaggggtccgctctccagatgagaagggtgcagatcagcgccagccctccggcccgcgcctctgcagcgctccggctccccctcggcgctctcgccccgccgccgccggcccagcaactttgttccggaagatcagccccactacgttcccgggtcagcgtctgccgggcctcggcggtcaccgcggccaccgc

SEQ ID NO: 12215 - RNA, 2342 nt, Homo sapiens
  source 1..2342: mol_type = other RNA
ctgggacaggaggaggaggcagttcctgcttagatttttttgtaattgcttgttctcttacacgaacagtctccaaaaggtccttctgaggaatctgagacatccccagctttgctacagcctgagtcacctggttggaggaatcttctagtctctgaaccaaagaatcccatctttgagtcagttcctctgagtcactgttgatcttcttagatgccttggaattatcaagtaattgtcccacatcctggccaatctcactcagctgatccaatgtttgacgcttcatttccatgtcttccttcaaaatagccagacgtcgaacactgacacttagttccttttggtctttgaagttgcttgtctggactttatttaaagcctcttctttttcggttaaccaagctttcaacaagcactgttcttccaataattcctgccacaatatattgatttcttgtaacctattccagcgttcttcagtccaacggcatactgctgtccagcgctcaccaagtttctgtaactggtcttctaggatagctgtagcactctcaccactgttttcatcaacaatgaccaccatgtgagttagtgaatttactttcacctgttcagcctcaagatcactttgcaaacttttatgttcttctagcagcttttgtagagattttacatcatcatccagggggcaagtttccatcttctgaatgcgctcctctgtgagtgttaaccaggcggagagctgctgcagttgcttcttctgcagttccatcagcacatcgtgcagccgggactgtctgtccatactctccaccctaagagcctcccatctagcattcagcagggtcatctgttcctgaatctcaaattcttcttcgtctgacagagttccttgtgttatcagttggttgcctgcctgcaggacgctgcccacactgctctggtgtgcagtcagttccatcataaaagcttcatgggttgcaaactggtctttgacttcttcaacatcatcagaaatatcatcctgctcctggaaagtgtcctcagcagaaagcaaccaggtcagcacttcctccaacgcaatctgatagctgtccagatccatgtcaacctcagtgacagtgctgggagtttcagctcggggactctcatgctcctcctcaggcgctgtactctgtatattaattgcctcttcttcacattcttttttatatttccttgggagtgtctctacctcacggatggcgtctatggtgacttgctgaggtagcacctcaaacaaagatgttaaatacataattatggatttcttgtcaggaagctgaacggcaacatcttcaggatctaacagcttttcaattcccaaataagtttgagccttgctgaaggcatgttcaagtctctcaattggtgacattttgacaactttatcccagctgaagagatcaggtttatgtcggtggaggacagcattaaaggcgagtccatctgtccagctggtggtgaagttgaggacgttgacttggctgtagggcctggtggtctgacgcacccagctgagcaggatcttctcactgttcgtctgctgcaggtccgacatgacatccttcatgacatctttcacctgccagtgcaaaatgatgctccaaagtaaccccaaagtcagtttgtgatttccatccacaatgtcagttccccctatattcactaattccacattgttctgatgtaaaacctgcagcactctgttgacgttatttaaggcatgtacccttgtggaaccacgttcctttggcagtgatgttcctgtgaggccttctagaagatccaatagcttccttccatctttgaggtctgtgaacatatcattgatgggtggtttcccactctttgaaaatcgagcatttatccatttggtaaaggttttcttctgtacgtcattgtgttcatcagatctggacttaatgatatcactgaattcgttctgcccattgtcaggactggcttcatgttctccatacttggccatcttgccagagtttcaagataatccaaaaactttaccaagtcctctttctaaggctttcaacttcctacgatggttcagcttgacatcaataccttgtcagttgcagcaagagatccccagagtccggaaaaggagagccggcgactgcgcgggactacacaccaatggggcgcccccctcctcctgtcccctcagtctctccagggccgctgccagggagcttggcgatcgcgccacactctccggagccccacccttgggagcagcaaccacccagaggtcaagcacgttccccgccgggcggctggct

SEQ ID NO: 12216 - RNA, 2181 nt, Homo sapiens
  source 1..2181: mol_type = other RNA
ctgggacaggaggaggaggcagttcctgcttagatttttttgtaattgcttgttctcttacacgaacagtctccaaaaggtccttctgaggaatctgagacatccccagctttgctacagcctgagtcacctggttggaggaatcttctagtctctgaaccaaagaatcccatctttgagtcagttcctctgagtcactgttgatcttcttagatgccttggaattatcaagtaattgtcccacatcctggccaatctcactcagctgatccaatgtttgacgcttcatttccatgtcttccttcaaaatagccagacgtcgaacactgacacttagttccttttggtctttgaagttgcttgtctggactttatttaaagcctcttctttttcggttaaccaagctttcaacaagcactgttcttccaataattcctgccacaatatattgatttcttgtaacctattccagcgttcttcagtccaacggcatactgctgtccagcgctcaccaagtttctgtaactggtcttctaggatagctgtagcactctcaccactgttttcatcaacaatgaccaccatgtgagttagtgaatttactttcacctgttcagcctcaagatcactttgcaaacttttatgttcttctagcagcttttgtagagattttacatcatcatccagggggcaagtttccatcttctgaatgcgctcctctgtgagtgttaaccaggcggagagctgctgcagttgcttcttctgcagttccatcagcacatcgtgcagccgggactgtctgtccatactctccaccctaagagcctcccatctagcattcagcagggtcatctgttcctgaatctcaaattcttcttcgtctgacagagttccttgtgttatcagttggttgcctgcctgcaggacgctgcccacactgctctggtgtgcagtcagttccatcataaaagcttcatgggttgcaaactggtctttgacttcttcaacatcatcagaaatatcatcctgctcctggaaagtgtcctcagcagaaagcaaccaggtcagcacttcctccaacgcaatctgatagctgtccagatccatgtcaacctcagtgacagtgctgggagtttcagctcggggactctcatgctcctcctcaggcgctgtactctgtatattaattgcctcttcttcacattcttttttatatttccttgggagtgtctctacctcacggatggcgtctatggtgacttgctgaggtagcacctcaaacaaagatgttaaatacataattatggatttcttgtcaggaagctgaacggcaacatcttcaggatctaacagcttttcaattcccaaataagtttgagccttgctgaaggcatgttcaagtctctcaattggtgacattttgacaactttatcccagctgaagagatcaggtttatgtcggtggaggacagcattaaaggcgagtccatctgtccagctggtggtgaagttgaggacgttgacttggctgtagggcctggtggtctgacgcacccagctgagcaggatcttctcactgttcgtctgctgcaggtccgacatgacatccttcatgacatctttcacctgccagtgcaaaatgatgctccaaagtaaccccaaagtcagtttgtgatttccatccacaatgtcagttccccctatattcactaattccacattgttctgatgtaaaacctgcagcactctgttgacgttatttaaggcatgtacccttgtggaaccacgttcctttggcagtgatgttcctgtgaggccttctagaagatccaatagcttccttccatctttgaggtctgtgaacatatcattgatgggtggtttcccactctttgaaaatcgagcatttatccatttggtaaaggttttcttctgtacgtcattgtgttcatcctgacgatggcaggggtaatggaaacccagatcttgagggccaagtctcatcccttaaagaactgctcagggccaggcgccgtggctcatgcctgtaatcccagcactttgggaggctgaggcgggcggatcacgaggtcaggagatccagaccatcctggctaacacggggaaaccccgtctctactaaaaatacaaaaaattagccgggcgtgatggcgggcgcc

SEQ ID NO: 12217 - RNA, 3144 nt, Homo sapiens
  source 1..3144: mol_type = other RNA
ctgggacaggaggaggaggcagttcctgcttagatttttttgtaattgcttgttctcttacacgaacagtctccaaaaggtccttctgaggaatctgagacatccccagctttgctacagcctgagtcacctggttggaggaatcttctagtctctgaaccaaagaatcccatctttgagtcagttcctctgagtcactgttgatcttcttagatgccttggaattatcaagtaattgtcccacatcctggccaatctcactcagctgatccaatgtttgacgcttcatttccatgtcttccttcaaaatagccagacgtcgaacactgacacttagttccttttggtctttgaagttgcttgtctggactttatttaaagcctcttctttttcggttaaccaagctttcaacaagcactgttcttccaataattcctgccacaatatattgatttcttgtaacctattccagcgttcttcagtccaacggcatactgctgtccagcgctcaccaagtttctgtaactggtcttctaggatagctgtagcactctcaccactgttttcatcaacaatgaccaccatgtgagttagtgaatttactttcacctgttcagcctcaagatcactttgcaaacttttatgttcttctagcagcttttgtagagattttacatcatcatccagggggcaagtttccatcttctgaatgcgctcctctgtgagtgttaaccaggcggagagctgctgcagttgcttcttctgcagttccatcagcacatcgtgcagccgggactgtctgtccatactctccaccctaagagcctcccatctagcattcagcagggtcatctgttcctgaatctcaaattcttcttcgtctgacagagttccttgtgttatcagttggttgcctgcctgcaggacgctgcccacactgctctggtgtgcagtcagttccatcataaaagcttcatgggttgcaaactggtctttgacttcttcaacatcatcagaaatatcatcctgctcctggaaagtgtcctcagcagaaagcaaccaggtcagcacttcctccaacgcaatctgatagctgtccagatccatgtcaacctcagtgacagtgctgggagtttcagctcggggactctcatgctcctcctcaggcgctgtactctgtatattaattgcctcttcttcacattcttttttatatttccttgggagtgtctctacctcacggatggcgtctatggtgacttgctgaggtagcacctcaaacaaagatgttaaatacataattatggatttcttgtcaggaagctgaacggcaacatcttcaggatctaacagcttttcaattcccaaataagtttgagccttgctgaaggcatgttcaagtctctcaattggtgacattttgacaactttatcccagctgaagagatcaggtttatgtcggtggaggacagcattaaaggcgagtccatctgtccagctggtggtgaagttgaggacgttgacttggctgtagggcctggtggtctgacgcacccagctgagcaggatcttctcactgttcgtctgctgcaggtccgacatgacatccttcatgacatctttcacctgccagtgcaaaatgatgctccaaagtaaccccaaagtcagtttgtgatttccatccacaatgtcagttccccctatattcactaattccacattgttctgatgtaaaacctgcagcactctgttgacgttatttaaggcatgtacccttgtggaaccacgttcctttggcagtgatgttcctgtgaggccttctagaagatccaatagcttccttccatctttgaggtctgtgaacatatcattgatgggtggtttcccactctttgaaaatcgagcatttatccatttggtaaaggttttcttctgtacgtcattgtgttcatctgcctgtgactgtctgccgtctccgtttgtggattcagatctcacttccatttctcgtcggctcagcgtgtcctccaaatgtagttaagactcccaaaccaacagtgcatgatttctgaagtcacaaagggatgtgtacccctcggctggagaatgtgctttgatggagtcaaattgaaaaacagggccaaacagtatgggaaccgtggatagatgagttcctccccaactgcccggaccagaatggtcacattcctgcctctgtgaatagcccaatcctggtctgctctgtctgagcctctgccaggtgtggagcctgtcgccttaaaatctgaagacgtgtgacaacacttatctgcctaggaacagcaaggtatgcatttctacaaacaccactgttgaaactgcttggtatacagagaagccaagcacttcctctcttctcaggttttccttagattcaagccaaatagaaatctgagtgaggaaaaatgttaaggaatttagctttagaaaaatttgtttttatgtttctaactcttgcaagagagcttgttctcatcaattttataacctatttttcaacctacatactccagactaattcctaatgcttttagggatccatccattaatgcactaaataatacatgccctcaaactaagaggtaaaccatgccccttcaatcaggataagaaatactactgagtgaaatgcagactgcatctttctgccaattttaatccacagccctctgctcacttcactcccaatcaccggcctcaatcaggctttctgtgggccaagttctgccagcttagagcctgcacacagctctgccttcagccagtgccctccaccaccttgaactatggacttgaatagattcctcaagaaggccttccctgaccactcaaactatcactcattccaggtccctatgaagtccccgagtgatttgccatgacagcactgcagaatgtctaccctctaagcagttaaacaactatttgtatgctctgcaatttgatgtctggttctcgtactagtctacacactcaagaggccagatgccatcatagagctcatcagttttgtcaactacacccagtgcagtgcctgccatatggggcattcacccaagactactttccatttaaaattgttgtctcttttgaaacactctgtg

SEQ ID NO: 12218 - RNA, 2062 nt, Homo sapiens
  source 1..2062: mol_type = other RNA
ctgggacaggaggaggaggcagttcctgcttagatttttttgtaattgcttgttctcttacacgaacagtctccaaaaggtccttctgaggaatctgagacatccccagctttgctacagcctgagtcacctggttggaggaatcttctagtctctgaaccaaagaatcccatctttgagtcagttcctctgagtcactgttgatcttcttagatgccttggaattatcaagtaattgtcccacatcctggccaatctcactcagctgatccaatgtttgacgcttcatttccatgtcttccttcaaaatagccagacgtcgaacactgacacttagttccttttggtctttgaagttgcttgtctggactttatttaaagcctcttctttttcggttaaccaagctttcaacaagcactgttcttccaataattcctgccacaatatattgatttcttgtaacctattccagcgttcttcagtccaacggcatactgctgtccagcgctcaccaagtttctgtaactggtcttctaggatagctgtagcactctcaccactgttttcatcaacaatgaccaccatgtgagttagtgaatttactttcacctgttcagcctcaagatcactttgcaaacttttatgttcttctagcagcttttgtagagattttacatcatcatccagggggcaagtttccatcttctgaatgcgctcctctgtgagtgttaaccaggcggagagctgctgcagttgcttcttctgcagttccatcagcacatcgtgcagccgggactgtctgtccatactctccaccctaagagcctcccatctagcattcagcagggtcatctgttcctgaatctcaaattcttcttcgtctgacagagttccttgtgttatcagttggttgcctgcctgcaggacgctgcccacactgctctggtgtgcagtcagttccatcataaaagcttcatgggttgcaaactggtctttgacttcttcaacatcatcagaaatatcatcctgctcctggaaagtgtcctcagcagaaagcaaccaggtcagcacttcctccaacgcaatctgatagctgtccagatccatgtcaacctcagtgacagtgctgggagtttcagctcggggactctcatgctcctcctcaggcgctgtactctgtatattaattgcctcttcttcacattcttttttatatttccttgggagtgtctctacctcacggatggcgtctatggtgacttgctgaggtagcacctcaaacaaagatgttaaatacataattatggatttcttgtcaggaagctgaacggcaacatcttcaggatctaacagcttttcaattcccaaataagtttgagccttgctgaaggcatgttcaagtctctcaattggtgacattttgacaactttatcccagctgaagagatcaggtttatgtcggtggaggacagcattaaaggcgagtccatctgtccagctggtggtgaagttgaggacgttgacttggctgtagggcctggtggtctgacgcacccagctgagcaggatcttctcactgttcgtctgctgcaggtccgacatgacatccttcatgacatctttcacctgccagtgcaaaatgatgctccaaagtaaccccaaagtcagtttgtgatttccatccacaatgtcagttccccctatattcactaattccacattgttctgatgtaaaacctgcagcactctgttgacgttatttaaggcatgtacccttgtggaaccacgttcctttggcagtgatgttcctgtgaggccttctagaagatccaatagcttccttccatctttgaggtctgtgaacatatcattgatgggtggtttcccactctttgaaaatcgagcatttatccatttggtaaaggttttcttctgtacgtcattgtgttcatctggtaatcgcttgcaagcctggagagctacatgccctggcaaatccaatctgcactttttccaatgaaacgtggtggctgccaggccgctcatcacctacatctgctt

SEQ ID NO: 12219 - RNA, 489 nt, Homo sapiens
  source 1..489: mol_type = other RNA
ctgggagaagagtggtgaagatattccaggaccatctcgcagagccaagcacttcactcacacctgctgcatccaaattgggagggaaccaactgtgcttgcacctaccggcagcagcccgctcgcctgcagctgtggtgtgcttcagcagctagcctcaccacggaaggtaaattgcggctcctgtcatgtgtcttggcaccgggtctagggaatgctgccatctggcttgtcatcaaacatggtcattgaatctctcagagataaaatggctttttaaaaatcttgctgtttttttaaaaattgacacacataaaatgtattatctttctctttacaggcatggtatattctaaaataagtgtttgagcttatttgagcaatagcttccagagtgttgtttttcctcactgattcccacgctcaaagggatttatagtctaaacctattatatgttaatggaaaatttaaattcatcggatctggcc

SEQ ID NO: 12220 - RNA, 3415 nt, Homo sapiens
  source 1..3415: mol_type = other RNA
ctgggaggggctgggtttggcaccggtgggagccggggccccacgggactcagaggctgggccgcccccgctgctggcacggtagtcacattggccacggagatggctacgaatagggaatccaataaattaggctgtagaaagaggtggtgaggggccgagggggcggggcctgcattctcgcttggcaggcagtgctgtgcgtccctctcccctctcccgtgggatctttggggctcttgtgggggagaggatgcaggtgaggcgctctgtgtgactgtgggtcccactgggcggcttttatggcatcccacggaacgggagccttggctgaccaccctcaggggatggaccatggggtctttgagagactgacgaggagggaatcatggggactcgagtctctggagggaggccacctgcagtgccaggggctgtggcctgacgggctcctggggctcggctgcgctgctgtgtggccagcactgggccccttgtaccccagcttcctccacggagcaaagtagaggactcactgccctggacagggcccagtcactgtggaacagcgcccccagggagtgggagggacagggcgagggttacgcagggcgccaccctccacatctactttcccgagggcgggaagggttttctaggaggaggggccaggcatgcaggggcggggtgcgtgcatgggtgggtgctgctgtctccttcatgtgatccgagcttgggggcggggcaggggccggggacggttgtgtcaggtggaggcaccctggaggccaccagggccttgcgggctaggtgccggcacatgcgctggggccacggcctcgcccaggatctggcagagctcctggaggcgccgctgcatcttgggaatgcccgccagctgctgctccagccgctgcttctcctccgtcaggctcaggcgggcagctgagtccagcttctcgaacttccagccgccctccccatcgaactgtagcaagtgtgtgtggtatttccacagggagggccggtgggtgatggagagcagggcaatgcccgcgtccttggccgcctggaagatcttgccttccacgtcgatgctcacggcgctggtgcattcatccaggagggcgtacttgggcctgtggtagaacatgcgggccatgccgattctctgcttctcgccacccgacaggacgtccttccagtcacacatagcctcccaacctccctcccgctgcaggatgtggtgcaggtgcacgacgtccaggatggcttccaggtcctgctccgagtagcccttcctttgcatgtcctccactgagtccgggtagatcacctggtcacgcagggagcccacagacatgtagggcctctgcgggatgtagaacatgcgctggggtgggggcttgtagagcacaccaccgtacgtgggccagagcccacccaggatccggaacagggagctcttgccgcagccattggggcctgtgatgagcagatgcatgccttcctccaccctgatgttgaggctggccaccaccacctctcctgagggcgtgacgatggggatgttctcgcagatgatcccctgttccacatccaccacctggcctcggatcttcagggggccctccacacggacaccagaccggcctatggtcccagaccccgcctgagcgtcctctagctccctgggcctcttgaagtgacagcgctgaacatcttcaaatacctggaacatctcgtgcacccgggctgtgtagccagccagctccgtcacctccttgtacgacgacatgatccgctcaatggcatctgcagccgctgtcaggaggttgcgggcaatagtgaaggcttctgtgcgctcgctcaccagctcctcctccttcttttccaaggctgccttcttcacggcctctgcatctgactctgagtagccagtggcagtgatgatggggacagccaccatgagcaggcccgaggcgctccacacatacttcatgaggaactgctccagcataacataccacaggcgttccagaaggatgaggttgatctgcgaggccaggtcctggtaggagcgctgtagcagggccagctccacctcatggcccccatagaaggcgatctcctccgagttggccaccacacgcgagtgcatgtagcgcagctcccccttccgccgcgcctcctctgccaccagctccccgaacttgggcgagaaggcccgcagcacgttggccgtgaggaacaccacgaggccggcgatggccgagggccaggctgtgccggctccacgggagcgggccgcccgaagcagggtgtaggaagtcacagccacgtccaggagtggcttggtcaggttggagtagaggtgggccacagaggccgcaaaggccaccacgtcctccgtcagagactggtcagggttgcgaagccgcccgtccatgttgctgacccggtagtaggtctgctgggagaagtagaggcggtaggcgtgggccaccagacggctgcggaacgacagggccagttggccctccaggtaacggatggcactgttgacgaaggtagcagggagggcgatgaggagccactgcagcagctgccagccaaaagcccgcgggtccttgcggacgatgcagcgggccagccttccgtccaggcgggccacatacaccgacaggaaggtgcggctcaccaaggcggccgagtgcagggccagcagccccgtctcccggcacaggacccgggggaacagcagccgcaggagccacaggagccgctgcaggaatacccggttcatgccagctttggccgccgcgaccccggaggcctcctgcgtgggctccccggcgggcgcctgaagacccctggccggggccaggcactggcgcaccaaggggtagactttgtgggctccataggccgcgagggccaggagcacggccgtgcgcttcagcgtgttcccccgccagggccggggcctggagagcaccggcatgtcacctgggctggctgccgcgtagggactggggctggtgcctggggcagcagttgaggcaggtggctggaaggattgttgctctgaccctgggcctgttgtctaggcaactggaaaccttgcgatggcccctgagactgtcgctttaggcccccggggtggtgctggggcccctggtgcggtgggctcagggccctccagggtcgcggcctcttcgggcagcccaagtggaggaacttggctctcctgtcctgtcagtgccctggcccctgaggtcagggccttgagaggtctcgggcagagggggcgtctcttcctctccaccttctcctcctcctcctcccccggtggcgcccctccccggggcaccaggcgcgtccgtccgctccgcagcctggctgaagcgacagt

SEQ ID NO: 12221 - RNA, 3476 nt, Homo sapiens
  source 1..3476: mol_type = other RNA
ctgggaggggctgggtttggcaccggtgggagccggggccccacgggactcagaggctgggccgcccccgctgctggcacggtagtcacattggccacggagatggctacgaatagggaatccaataaattaggctgtagaaagaggtggtgaggggccgagggggcggggcctgcattctcgcttggcaggcagtgctgtgcgtccctctcccctctcccgtgggatctttggggctcttgtgggggagaggatgcaggtgaggcgctctgtgtgactgtgggtcccactgggcggcttttatggcatcccacggaacgggagccttggctgaccaccctcaggggatggaccatggggtctttgagagactgacgaggagggaatcatggggactcgagtctctggagggaggccacctgcagtgccaggggctgtggcctgacgggctcctggggctcggctgcgctgctgtgtggccagcactgggccccttgtaccccagcttcctccacggagcaaagtagaggactcactgccctggacagggcccagtcactgtggaacagcgcccccagggagtgggagggacagggcgagggttacgcagggcgccaccctccacatctactttcccgagggcgggaagggttttctaggaggaggggccaggcatgcaggggcggggtgcgtgcatgggtgggtgctgctgtctccttcatgtgatccgagcttgggggcggggcaggggccggggacggttgtgtcaggtggaggcaccctggaggccaccagggccttgcgggctaggtgccggcacatgcgctggggccacggcctcgcccaggatctggcagagctcctggaggcgccgctgcatcttgggaatgcccgccagctgctgctccagccgctgcttctcctccgtcaggctcaggcgggcagctgagtccagcttctcgaacttccagccgccctccccatcgaactgtagcaagtgtgtgtggtatttccacagggagggccggtgggtgatggagagcagggcaatgcccgcgtccttggccgcctggaagatcttgccttccacgtcgatgctcacggcgctggtgcattcatccaggagggcgtacttgggcctgtggtagaacatgcgggccatgccgattctctgcttctcgccacccgacaggacgtccttccagtcacacatagcctcccaacctccctcccgctgcaggatgtggtgcaggtgcacgacgtccaggatggcttccaggtcctgctccgagtagcccttcctttgcatgtcctccactgagtccgggtagatcacctggtcacgcagggagcccacagacatgtagggcctctgcgggatgtagaacatgcgctggggtgggggcttgtagagcacaccaccgtacgtgggccagagcccacccaggatccggaacagggagctcttgccgcagccattggggcctgtgatgagcagatgcatgccttcctccaccctgatgttgaggctggccaccaccacctctcctgagggcgtgacgatggggatgttctcgcagatgatcccctgttccacatccaccacctggcctgcctcccgtggcagccagcagctggcacactgactggaactttctcttgctgtcctcggatcttcagggggccctccacacggacaccagaccggcctatggtcccagaccccgcctgagcgtcctctagctccctgggcctcttgaagtgacagcgctgaacatcttcaaatacctggaacatctcgtgcacccgggctgtgtagccagccagctccgtcacctccttgtacgacgacatgatccgctcaatggcatctgcagccgctgtcaggaggttgcgggcaatagtgaaggcttctgtgcgctcgctcaccagctcctcctccttcttttccaaggctgccttcttcacggcctctgcatctgactctgagtagccagtggcagtgatgatggggacagccaccatgagcaggcccgaggcgctccacacatacttcatgaggaactgctccagcataacataccacaggcgttccagaaggatgaggttgatctgcgaggccaggtcctggtaggagcgctgtagcagggccagctccacctcatggcccccatagaaggcgatctcctccgagttggccaccacacgcgagtgcatgtagcgcagctcccccttccgccgcgcctcctctgccaccagctccccgaacttgggcgagaaggcccgcagcacgttggccgtgaggaacaccacgaggccggcgatggccgagggccaggctgtgccggctccacgggagcgggccgcccgaagcagggtgtaggaagtcacagccacgtccaggagtggcttggtcaggttggagtagaggtgggccacagaggccgcaaaggccaccacgtcctccgtcagagactggtcagggttgcgaagccgcccgtccatgttgctgacccggtagtaggtctgctgggagaagtagaggcggtaggcgtgggccaccagacggctgcggaacgacagggccagttggccctccaggtaacggatggcactgttgacgaaggtagcagggagggcgatgaggagccactgcagcagctgccagccaaaagcccgcgggtccttgcggacgatgcagcgggccagccttccgtccaggcgggccacatacaccgacaggaaggtgcggctcaccaaggcggccgagtgcagggccagcagccccgtctcccggcacaggacccgggggaacagcagccgcaggagccacaggagccgctgcaggaatacccggttcatgccagctttggccgccgcgaccccggaggcctcctgcgtgggctccccggcgggcgcctgaagacccctggccggggccaggcactggcgcaccaaggggtagactttgtgggctccataggccgcgagggccaggagcacggccgtgcgcttcagcgtgttcccccgccagggccggggcctggagagcaccggcatgtcacctgggctggctgccgcgtagggactggggctggtgcctggggcagcagttgaggcaggtggctggaaggattgttgctctgaccctgggcctgttgtctaggcaactggaaaccttgcgatggcccctgagactgtcgctttaggcccccggggtggtgctggggcccctggtgcggtgggctcagggccctccagggtcgcggcctcttcgggcagcccaagtggaggaacttggctctcctgtcctgtcagtgccctggcccctgaggtcagggccttgagaggtctcgggcagagggggcgtctcttcctctccaccttctcctcctcctcctcccccggtggcgcccctccccggggcaccaggcgcgtccgtccgctccgcagcctggctgaagcgacagtgactc

SEQ ID NO: 12222 - RNA, 4845 nt, Homo sapiens
  source 1..4845: mol_type = other RNA
ctgggaggggctgggtttggcccactggccatagtttgcctaccttgatctagaatagaataagcttttaggggccctgggtttagggctcatgccacaaaagggagaggacagtgccatctgactcaccctagccaggctcctcccagaggaagagaaaaggagtctcagagaaggctagatcctctacttctctagttcccaatttggtaaaatccagtgtccactgtattacttagaaatcactgggccagccgggtgcggtggctcatgcctgtaatcccagcactttgggaggccgaggcgggcggatcacgaggtcaggagatcaagaccatcctggctaacatggtgaaaccccgtctctactaaaaatacaaaaaaaaaaaaaaattagccgggcgtgttggcgggtgcctgtagtcccagctgctcgggaggctgaggcaggagaatcgcgtgaacccaggaggcggagcttgcagtgagccgagatcacgccactgcgctccagcctcggtgacagagtgagactctgtctcaaaaaacaaaaaaaaagaaatcactgggccagctctgcttctcccacagccgcattttttttttttttttagacggagttttactcttgttgcccaggctggagtgcaatggcacaatctcagctcactgcaaactccacctcctgggatcaagcaattctcctgcctcagcctcccaagtagctggggttataggcatgtgccaccacacccagctaatttcgtatttttagtagagacagggtttcaccatgttggtcaggctggtcttgaactcctgacctcagatgatccacccccgaccccggcctcccaaagtgctgggattacaggcatcagccaccacacccagccccacagccccatctaagcctccaccctgccatcctgttcctcagaaagcacatgctctgtggagggagccagcagggaagtcttgttccccacctccacctccatcccaatcccaagtcctggggatggggcaggtggtgcaggaagaccaggtaggccaggccaatcccctatggagcagctgagcctccaactcctgagccaggccaccctagtgtcatttgtcatccatgctcaaatgttttcatccatattttcttttatttcttttcttttctttttttttctttcatttttttttcccgagatggggtcttgctctgtcgcccaggctggagtgcagtggcgtgatcttggctcactgcaacctccgcctcctaggttcaagcaattctcctgcctcagcctcccaagtagctaggattacaggtgcccactacgacatctggctaatttttgtatttttagtaaagaaggggtttcatcatgttggcgaggctggtctcgaactcctgacctcatgatccgcccgcctcgactccccaaagtgctgggattacaggcatgagccactgagcctggctgtgtttttctttctcattgcagagacaaagcgggttacttctggttcattcacgcatccaagtcctgacatgtctcaagggcattactgtgcttgtcagggagggagggcccagtccatcctctggttattcccatccatcccctaggccttcccttggctcaccctgccccctgccaggcccctttgcttgctggcctgacggggctgggtctctgtggctggaggagatggcctctgccccacccccctcgactgtcctgggcacaaaggagaacagctttgcctggaaagggcccaagacaccctgagaaacttgtagcgatgggacctgcctcctgcagccctccacctgcgtcatccttcctgtgccctccttgtctacaccagggccatgcggtcacccctgagggctctaatgttactaggcaaaggcctgagtctgagcaggacagggtggggcaagctccaacccaaagtctactctattatcaggagaagctccatgctatccagaggaccccgacacacaccccaagccaatttcccttcatccccaggaaagtgtgccaccaactgaggaggaaatgtatctgcttctcttcctagcactcccgtgaactcaaccaggaagatactgctgtttggctttaaaaatagtacattctagctggacttttatggtcttgtgaagaacactgtgctcatgccctcccacacctggcctctgcccctgcctggccctgtccagctgcccacatcagctctgcacaagctcttcagggtccctctgcagagacgtggttcaaggcagatttacgagttcagccttggccgaggccttctccccatggctcccatccacattccagctgttctcccacatcccaggcagctcggggctgggatgttctgtgtctctttttctacctctaccacaactggctcagtcgcacccccagccctatttcagctctgccctggccagccctgtggaggtacagggtcctgtcatgccagaacccagaccccaaccattcccagcctgcccagagctcacttacattcatgataacaacaatggtgtgtgtctaaggataaccttgttgggactctagttggtcatgcccgtcccctcccactctgaagggctgaaatttaaccgaaaggtaatttgttccatctggacttcaggtgccaggtttgaggctacatccgatctggaaagttattttcagtgtgtgtagattctatgattagtcctcaagttatttctttagggccagagatgagtttcaccgaagctatatcacatttctggcaccccatggtaggacttagagaaagcccccaaggacgatctccatgaggcggagccggccctagggagctaatagactatagaaataactccagagccagggaagcctcgaacacaaattttacaaggagccaattgagtggttgagcagttgaaggcaggcctatcttgtttttgcttgagggcaggtttctaacataatggaaagagaagactgtaatgatcaccccctatatacctgatcttctcttaaggtccttcaaggatgtaattgattctgtcaatatccttcatatttaaggccataagttgctgcttggttcaattaaggtagaattgcttctggttaagatctcaaactaggcatctgggactatctaaaagtttctctggaaactggaatgtaagcaatgcaagatgtatggcttaacctgtagatataactcatgtcaagaaaacagtggggttgggcatggtggctcatgcctgtaatcccagcactttaggaggctgaggtgggaggatcacttgaggccaggggttcgaggccagcctgggcaacatatcaagacccccatctctacataaaaagaagaagaaacgaaaagaaaagaaaagaaaagaaaagagtggaagagtgcaggagccgagagggagagaaaatgtagtggtgaggggcagcttctggaaaggcccatactacagagggaggaatcctgaattcctcactatctctctaacatcaggtaagcatctcatgatgcagttagaaagcacatttccttcttcagtttcccctctggctgtgtgacccagcccagatctgtttacacttggagctaccaggagcctatccggccacctggctttcccatcagcacctggggctggtgccatcccaggcccctccctctgcacctgcctttttgctatctgcagagggtttgtagaaaccttaggggaagaaagctagggtggttccctacctcaactttgagcccaattatacctctttctctcccacttcccagtagctgtcacagaagagccatggggaagtcccctcctggggaccaaggaggaggctctccaacctgtgcccctctaggtactgtccatcacagaagtgctactgcttctcttggtctgcatgctggaacttgggagctgagtctgagtcaagtctgatggctgagaatctgggggctggtagaaaatccaggcccataagcatgagtcacagtctaggagaaaagggcgagtgtgataattatttgtcaccaagagctggtgagagtggtgtggtggaaaggagagcatctgcctctccagggacttgggaccccacctctgcatctcttgttctttggctgggggtgctggctgtggtggagtcaagatcggagtaccccaggcctccagcatagagacgagatcgcatcggccacttcttgagagggtgcaagtagcggagtccacgcaggaagggcggccaggcagggccaggcaactcgtggccgagtgtgcgggtgaggtgggctatgtagctggcggcgagcaccagcacgtccaacttggagagcttggtgtcgggcggcacggcaggcagagcagcctgcaaggccaagaaggcctggcgcagcgtcctgacccggctccgctcccgcgcggcattctcaggactggcctcgctcctgccaagagccaggcccccagccctggtccctcgagggccaggggtagctctgctccatctctggttgctccagcttctttcttcccacgggtcctgccttgtcctgctgaggcggctcctcttcctgtcagcgcctggcagcaaccgtgctttggcctgagtctggctatgccccacccctggcatggctggtggccctctggccttcctctgtgacatgccaccccactggggctgcagcccacagagcagaaacacagtgcctgaggaggccttggactcaagctagctggctgtggctggtcatccagccagcaatatctacatccgaggaagctggcgccaactc

SEQ ID NO: 12223 - RNA, 1336 nt, Homo sapiens
  source 1..1336: mol_type = other RNA
ctgggaggggctgggtttggccccagaagtgtggcacaggacagggagggagggcaggggctcctgcctgctgccacagtcttggggagggggaagggctaggaaactccagcagagggagggggttgggacccactatggacagtcctcacacagcccacggagttcaccccgtttccaccacctcctgccctgcctggggcccccacactctctctcacatatacacatctcatctccccatgcttgcccgctccccccagactctctctctctctctctctctctcctcaccaaccctctcctctaccacggtcttatccctctgcatacccccaccacacaccctcaccagttccaagcctgagccccgcggggtgcggctggtctggcccaagctgacatccctccaaacgaggttcttaggttctttccttgggttggcttcgacctgcctaaagttgcagggccggtgccattgagtggaggcaggggagctggggacttcacgaagaaatgagggctccggagcctcaggacaggcagccatagacatgcctgagtccagtggagggcagagtgctgcgcagcgcaaaggcactggggcccagcggaggatgcccctgagcttgggagggtgggctctgggtgagtcggcttgacacggagagcaagccctgggccagccaggcacctaagtgccccacctccactgccagcgcacctggggcctctgtcgggagggcccaggctgcagagggatagcgtggagggccaacaggccggcctccctctgccttgggggtctccgggctgggcgggcggggcgggctgggggagggcgcccggtgccgcccgcctatcccctttgcaagtcggctcagacctccgggccgccgaaggccaggttgtcgcgcaccattagcgtcttgcggaggtcgcggtccaccagggggcgctgcatgcgccacttgtgcgcctcctgcaggcccggctcgaagtagtagatgcaggcgccgaagcccaccagaatgaggaccgagatgaccaagtagaccggcacgaaccagtccaggaagtgcggcatcgcggcggccttggctcacgccctgcagatgccagttccgggggctctgtgctgagcacaccgcctcagcctgagcagctcagcattggcccgtggactcattcgcagctgctgtccccagagacactgccatctgcggccgccctgggtgctggaggcagagatagggcagagccaatgcaacccacgggagacgagcttctcacacccaggggctctgagtgggccaggagggggcagtcctggact

SEQ ID NO: 12224 - RNA, 231 nt, Homo sapiens
  source 1..231: mol_type = other RNA
ctgggaggtcaaggctgcagtaaaccatgatcatggcactgaactccagcctgggcaacaaagtgagaccctgccaggcttgtttggtccccgagggcactgtcagctgagatcagagctcccgaggaggcgggcggggacgctgcagctgggagcctctcagccagcctgagccggaggccgccccgccaaggccgggccacagcacccagagctcgccactgagactgc

SEQ ID NO: 12225 - RNA, 2774 nt, Homo sapiens
  source 1..2774: mol_type = other RNA
ctgggaggtcaaggctgcagtaagatccagcctaggcaacagagaccctatcttaaaaaaacaaaacaaaacaaaactttggtctaggtgctggcatttatatccaaaaaaaaagtctacatctcactaaagaaaaagcttccatatttaaaataaatcctgaatcaagactgcccattttagttaagatttagggccttaaagtgtcctcatgtactggccagaaacaagtatcagcttccttttgtacaatcaccatttgtagcacagaatataataatactctttcttctctacctcaaatattaaaaggaaattctgaaattatacacagagatagtaatgtccttgtcaaaactgctgagttaaaatgtgtatgaaagtatacatagttccagaaaacaggaagccccaagcaataaaagtttttgagttggcatgttgttcatctgaactgcttaagtttttgcagagtcctaaggtcaaccacataaggcattcatttatttaaattagaatctaataccatctaccctaccgttcatataccgattacaccccactacatgacacgtctataagatttacaaggagggcaattaaaaaaacaaaaaactaaaagtgatcagggcaataactcatgtcataaaactatgcagcaacagttagggccttgtcatgctaaagattacagcaatagacactgggttaataaataaccttttaattaatctgtagtacccacaaaagcagccaagcaaaatgaacaaaaatcaacagagcaaaatgatttaatgaccaaaaaaaaaacaaaaaaacaaaaaaacaaaagaccagtggcaaaaaaagaaaacacacctactatgtgctgacaacttgaaggaaaaaggtggtaagaaatattacacaaaccaaaacttttgttcaacgtaaaaattaagaagtttttaagaattccattgaattgaggtttatataacccctttcttctgaagtttaatttttaaaaatcctagaagagaacagtgtatttctatgtattccctccaatgactatccgataactttcatgtgtaaaggcagtatgaggtaaggaaaaatgcagcatgtgtgcttgaacccacgcactaccaattaggctcctgctaagttttgttcacacagtttgctcatcaggcttaattttggtgtttttataccccaaaagttcttgggaggattaagggagacaagaaggccactctataaactgtgaattttatacaaacattattattactaagtgcaatctccagctcatcaaagctactagtctctaaactagaatgacctgtactttttaggcccacagtcatgatggggatttctcaaccaacgacaatgtgatacatggctctagagaaccattaatttgcctataaatcactccgtctcattcctgtaaaatgatctaaggattcggaaggctagatctaggccacattaactttcacatcatgcttgttttaaaaaatgtaatggctttaatacatgaagtttatctcacaatttcaaaattctatgctaaaaaatccaaactgcataaccttagttccagctcttcccacagctgcaattaacaccactagaaagtttagataaacatttcccatcctatttgagaaacaccctagaagaggttaggaattacttcccatcaaaatcaggacactggtactcaatgagataaattacagacaggtttttccccttaactggactatatataatttggagaactaaagacagtttgaaaataagagctctgatatctttaagactttattagagtcttttataacagcaataataaaagggcagggggagacagcctgaaacattacacagcactgaacacaaaaaaattatcataggtttttcatgtatcccacccaacctcagtatcggaatacaatttcttctaattcttagaatagtttattttttagtatcttggaataatgttatatatattcaagacataccatggattaaaataattcataacacttaaaacagaaaataaaatgtgtctggactagaaaccaaccaatagacaaacatgatacatgcagggtggcagtctgctcctctaaataaatctcatcatgcaatctatccttcagggaacaggggaaaatcagctggggagaaatcacctgaaatacctttgggaaggtaaataactattattaaggcttgaaacaaagtaatattaaataaaaaaacctttcccaaaatcatataaagaataggacatggatctgcaaatggcacctgaagcagtttttcattagcaccttgctgtgtgtgatgttagaaagtttgggggttcaacaaatgaaaacacctaaaggattaacattacagggttagacaagatggaaagcatttcccatgcaagaatgagcaggatagtcaaacctgtactggtcccttctacagtgggaggctgtccataagaagttgcataggcggtctgcccataggttgcagtggtctgagcctgggtatagctgacatcagtgggctgtccataggttccatagctttgttgcccatatgcctgggtggtctgtgcatatccttgagtgggctgggcggtgtaagcactgtagccctgctgcgctgcagcttggctataggtactgtaatccgtggacgccattttctctccttcctcctcgttctctcaacgtccgtctccctctcgctttccctctaggcgccgcact

SEQ ID NO: 12226 - RNA, 3755 nt, Homo sapiens
  source 1..3755: mol_type = other RNA
ctgggaggtcaaggctgcagtaagccatgatcacaccactgtaccccagcctgcgcaatgaagcaagaccccgcctcaaaaaataaaaataaagtttatattttaaagcacataattactattctcattcatctttaatttaaatacttggtattaattcccatttacagttgtgtttttctcagtctcaacctcagcttcaagtaacttggtatcttagattgcatttgcagtgacttagagctctgcttcctttctttatgtatgataaagcagaaagagacagacacaggatgtagtgataggagggcacaggaaacataaaacccctcaggtatttttcggtcacctgggctctcttctctttctcattcaagagtgtttttgctgcaactgtacagcaaaaacacaaaactactcatctctgaatagctgatacctttataacttcccacccactccttgttatggtgatttcagttacaaatggacttaattaaatggaatgtaccacttacaaagatcaaaaggctttcaaaaatttttcttaagatttttgaacaaagatttaactgtttctattaaaatgcaataagatggaaactctgtttcctctgatgtgattattatgcattgtatacctatatcaaaatatctcaagcaccccataaatatataaacctactatgtacccacaaaaattaaaaattaaaaacttttttttaatgcaataagaattaaacctgttttgcagagaaataagacagtggaaaaaatcaagttatacatatacatatatattacatacatatacatatataacatgcatatacatatataaaatatacatgtattattatatataataatatacatatatattaaacctattaaggtattaatgacatataagatcttgtaaagacagtgaatgtaaataaaactaaagatgttattccagtcagaaagttaccacctttatgccctctgagctcatcaagcttcataggatttgaatgaaataataaagtatatctgtatttgataaagacattatgagaaggcagaactgacattgtgtctgctgcataaacctgtctattttggtctctgttccaaagttattgtttccccaaatttttgtttattaccctgtcatgtaaagatagaagaatgatgaaacttgcaaatcaaagtatataataattatgagagaatggttttcttagcctgggcaacatggcaaaccccatctctacaaaaaatacaaaaattagctgagcagggtagcaaatgcctgtagtcccagctgcttgggaggctgaggtgggaggatcacttgagctgggggtcgaggccacagtgagccgtgatcacaccattgcactccagcctgggtgacagcgagaccgtgtctcaaaaacaaaaaaaaaaaggagttttcttgaggcttcatcactagaccattattctgtaacatcttcagagagttacctttactccctgtctccactcttcacctccctctcactcatcacctcattgttacggctttcagccccatctctccaaataaactgctctaggtaagctgttataggtaagtttagcaatggcctccatattattgaatctagccattgttttttaatctttattttttccctttagcagtattcagcattgttaaccaccctatccttaactctatcgtttccctgtggtttctatgacatgacactctcctgattgtgtccctctgtctttactgcttcctctctgttccctttggaggtcattcttccttacctggctgttaaattgctgaagctccctagggcttgtttgatctcaggtccttcatcatataaagctacacactgtccttagattatttcagccatactctagctttaattatgtaagatgactcacaaactcatcttcctagttctggctacactctgaactccagactcttctttgactttttcaccttgatatttcaaagcacttcaacaacatgctcaaaacaaactcatcatctcccttcccagtcgtggctctcttttagtgttcccgatcctagtgcaccacctatccaattgtgcaaaccagaaatctagtcatcagtcatgacatctccctctttctcactccccatttccagtctatccccatttcctgttggttttcatttccatgtatttctagaattcattcattgctgtctcttcccctgccttcccaccaaaactaccatcctcacttgcctgcactgcagcaatagtccactcattaatctcctagcacttacccttgttcctttgtaaatcattctctatcctgtaatcttttcaaaacacaaatctgacctcttacgataaagacaagaagacttaccctgtcctgcaagcccagcatagtctggcccctgtgtcccactccaccctccttgcatggcacattcgttcttgccctctctactttagctatgctggtctctgtttgggccctcatactggccatgtgtatcagtcaagatcaagtcaggagataagaaccatactggttatttgaataggagaaatgtaatgtaaagcattgttaattaaaacagtaggaggttactaactactagaaggggtaaaagaggaccataaggtgtccacatttagcatgagagcagttactatatctgtactgaagaaaatgagacaataaaggaactaaggcctaggggaggcccccaagccaagactgagattctgacctgatcgaagaaggtgtgtggctaccagaggaacgtgcagccttgtggtggtgaagaaacttgtcaaagggcacagactgagctcttctgttaagaggctgccattgccagagggtgtagatggattggagctgctcaaagccactgacagtggcgggaggtggggaatggcacgaggatgtaggttggagctcctctgaatggctgctgggttctcaagatcagatgatgtgctttgctgcaattacctccatacgttatgtcagtcacacacttggcactggcagtcagctccgctggcactgcagccttctttgcagaataaaggcccacaataagagcttgaggagttcagaaatctttcccttgtaaaggagcttaatccattgcgtccttactgctcatccatttacgttcctggtcagtgatgtgttgaaggaatgattttttaatagaggcttcaaattttctttgcttataactgtggcttagagatttggttttcctgatgtctactggtgtcatcagtggcttgctggcatctgatacttatctcttttcttttttggtagaatggatcttctaaccaaagacggagatttaatccacagtatcataacaacaggctaaatgggcctgccaagtcgcagggcagtgggaatgaagccgagccactgggaaagggcaacagccgccacgaacacagaagacagccgcacaacggcttccggcccaaaaacaaaggcggtgccaaaaatcaagaggcttccttggggatgaagacccccgaggccccggcccattctgaaaagccccggcgaaggcagcacgctgcagacacctcggaggccaggcccttccggggtagtgtcggtagggtttcacagtgcaatctctgccccacgagaatagaagtttccacagatgcagcagttctctcagtcccggctgtgacgttggtggcctgagctaggaggaaaaa

SEQ ID NO: 12227 - RNA, 55 nt, Homo sapiens
  source 1..55: mol_type = other RNA
ctgggaggtcaaggctgcagtaagccatgatcatgccaatgtactccagcctggg

SEQ ID NO: 12228 - RNA, 366 nt, Homo sapiens
  source 1..366: mol_type = other RNA
ctgggaggtcaaggctgcagtaagccatgattgtgccactgcactccaccctggaccacagagtgagaccctgtcaaaaaataataaaaaaataaaaataaatcactgttgttttaagtttcctggtttgtggtcatttttatggcagccctaggaaatgaacacagctggcgacgccagtctctggaggtgggggaactggccctggcgggggttggtactgttccccactccaagcctgagggtgcaggacaagtttgggtggccgagaacccctttgtgcctgggagtgcatgaagccccattcggggagtctggactttccaggaaggacgccttgcttgaacctgcctttcttgccgagaa

SEQ ID NO: 12229 - RNA, 385 nt, Homo sapiens
  source 1..385: mol_type = other RNA
ctgggaggtcaaggctgcagtaagcccacattgcaccactgcacaccagcctggatgacagagtgagaactgggtgttgggcaccgggctaaacatttcatcttcttcacaacgcaatgaggcaggtgctgttatctccattttgcagatttgtttggaaaagttaaatgacttgccaaccacacgacccttacggctcgcaggcgcggctgggcgttcgcgggggcctggtgctctacaacctgcccttccccttgctgcttacggcgctggcagccctgactctgctcggcctgggcgcggggctgccgccaccgctgcaaaacccactcctgctgggagcagtggcgctggtgcatggtgtagggttgctcgcgacagacct

SEQ ID NO: 12230 - RNA, 199 nt, Homo sapiens
  source 1..199: mol_type = other RNA
ctgggaggtcaaggctgcagtaagccgtgattgcagcactgcactccaacctgacctagggagagattccccgaactgccgcgaggtggaaagggcgaaggcgaagggagcagctgtgcgcgggctgcagcagccgggcagccaaagcagacattagagaagtcgcagccatagaccgcgccggtgactgcgccgggag

SEQ ID NO: 12231 - RNA, 70 nt, Homo sapiens
  source 1..70: mol_type = other RNA
ctgggaggtcaaggctgcagtaagctataatcactccactgcactccagcctgggtaacagagtgagacc

SEQ ID NO: 12232 - RNA, 543 nt, Homo sapiens
  source 1..543: mol_type = other RNA
ctgggaggtcaaggctgcagtaagctataatcactccactgcactccagcctgggtaacagagtgagaccctgctctctgcatagggttgcggcagagcacctcacacgcgcagatacacgcctggctttaggggaagtcgcggcactgggtctgcagagtccgctgagcacgcaccttcgttgtgaaactaaggaaaccctggagtgtccttgggcttgggtgggatggaacatgcccgtgacagacaggcccacctgtggttgatccaaggggtaaccggaggtgtgtggccctgtgccaccaccccaaattgtgcctgttgtccaaacacagcttcctttagttcgggctttcagcaagatggccgtgccgcatccctcctctttgtaaatgctggggctgccaccattatggttttatcatcagcgacattccagggggtgaagactggtcccaacctctcttctcctctcctcttctgatgagagtgagggatgggggaggggtcccagctcctagcactttctcccctcaccccaaa

SEQ ID NO: 12233 - RNA, 5951 nt, Homo sapiens
  source 1..5951: mol_type = other RNA
ctgggaggtcaaggctgcagtaagctgtgatcctgccactgcactccaccctgggcaaccctgtctcaaaaaataaaaaagacagtaaaaatatccctatactggggcaggaactttacaaggtatcctgtggcaaagggagcagagatggggggaaaggggtgctaaaagtttgattggaaagggacttttccatggttacaacaccaactgacatggaagctgcacctctgagagggccctggtcctagaggtcaaccacctgatggagagccttggtaaaccaagccctctttcaccaatctcaggaatcaggtagcacagccaagcactctaacttcacacataaggaaattgatgcagaggttcattgacttgctcaagatcaatcctgccaagaaaaggcacaccatgcctggaacccagatctgatgactccaagacccttcctatgactctggcccccctgcccagccacttctagtgccagttttgggacagtgaagggacatcttcagtgccatgaacagctgctgccgtaggaaggcaagaggatggcagaaccaagatgaccaaaccttcctgaggacaaagctgaacaggcatcagaacaccaacaggagacttctgccccgcccccaccatcctgtgacaccaccacacaatatcagagccttcattttcacctgctcatggcaatccagagcaggtaagattattccatactctactgaaaaagacatcttccaggttggtttcttctcatttcaagaaatgaccagctccatgaacgggcccctatagtcaggacactgctctactattaaaacattttatcctttcattcataatctgacctcttcaataatcagaagcaatgattactcacatgctttagcaatatcactcctttgcctttaagtaattgattcttgctttttgcttcaacacaagtgggtgggccagtgagggagctcctcccagaacaggctgccttttctcctgagagcagcaggcacatgcacttgttccttcgggttgaatctgattgctagcaccagatctcatacatggagaggggtatgtgaagctgagaggggcctgcagtgtgcaggggctagagacatgaacacaacaatggtaagcgtttatatctgctgaggccgaggatcctatagaaaattcagaaacggagtggggaggagtctgatttatgggaactggcagcaaggctaactgcatgagaagcctttcacccttttactgagtccttggatctgtggttaacccttataaaatataattcagattcaaaccacatcactcctcaactcaaaattgtccaaaagctccctgcctccctctgagccagctcaagcccccgtaatgacccatgatgctcatatggccgggcctgtggcctccctggcccctctccttcccttccagctggctccctgcactccatcccaggggcttccttcctgaggacaccagtcaagacccaatctcctctgcctgcaactctccctagagagctacctgctacctccctggcttccttcacgtctttgctcacatttcaccttctcagttgaggccctccctgaccagactatctaaaatcacgactgatctcccaatccagcactccctctgctcttctctgattcactttgtccactacacacatcaccatccagaatactgcgtatcccatttgtttgtcatctgtaaagatccaagatggcaggattttcatctgttctggtccctgctgggtctctggcaaacacaccagcgcctggtgtatgggagtgctcagcacatttctgttaaacagatggaccgctgctgcctatgcaggcctgtgggatggggatggcaacagggtactggtagagatccacacgccaagcgcttgagcccagcatcctgctctcctccacctgccgctgagaccactctaaccccctagcagatatccaaaagccagccaggaaggctgaagccccagccagaactccccagggggcatttgggaaggctaggagttcttgatgctgctgcttttaaagtcaacagaataggcatggccacaggccaaacttgaagacaaatctaggatcccactggcccctttccagcagccatagcccatgatgccacagatattctgtccaaccacaaagggcagtggtctctctcttcagagttgtggaaggagacctgaataggggagccgcaggctatggtgcagaggccactcctaggggccggagtctccagaagggctccaaaggacatggtgctgcacttccccagcgtcacatcctagcaggcaggctggggactccccgagctttcaaatccttgggattctgtcactagcttccaaaacagaaagggctgggccctttatcaaagttactccacaatgcctataattaagggttctctagcaggggactgagaacccacccccactgtcactgtcaggtcccaggctaatctctaatatggtttttcatatgccgagccaggttcgaagaccacctgaaggtctttccacacttgctgcatttgaagggcctctctcgagtatgaaatctcttgtggctaatgagttgtgaactcttgttaaaagttttcccacatatgctgcatttgtggcactttttcccaatgcttatgtcctggagtccagtgagcctggagctctggctgcaagcttctttgcagtcttcgaggggcatctcttcacttggttttagcttctgtaatctcaactttgtgtcctgagaggaagaccgtgcaggcgggctacgttcagcctgtgctgctctggtgtgtttcctctggtgactggaaagggtatgtctcccaatgaactctttcccacaccactgacatttgaaaggtctctctgtagagtggatcctctgatggttaacaaggcgatagtttctatcataagatttcccacatagattacatttatagcgcttctctccactgtgtattcccttatgatctaaaagggttcttttacgtgtaaaggttttcccacattcttgacaccaaaaacgtttctcaccagtgaggatttttggctccacatttggagtcttttcactttcatggcaatcatactgtttttgaagagagtgaatcctctgatgtcggtagagattggaactccatctgaaggctttcccacactccctgcacttatatggcttctctccagtgtgaactctctgatggatgaggaggaatgagtgattgcggaaggccttgccacactggctgcatttgtagggctcctctttggagtgactgctctgaggaacctggaacactgtgtcctgactaaaagatggcccgccctcaggttttcttttcatggcatgcttcttcttatgaacaataaaggctgacctataggcaaagtccttcccacaatcgctacactggtaaggtttctcacctgtgtgaattctctggtggtcaacgagagttttctttctagtaaaagttttcccacactgctgacacagaaatgttttctccacagcgggagcaccctggggctgactgcagtcaggagattgcctgaagccttcacgacattcatcttgtttgtagaatttttcctcctcatgcaacctcatatgacgagtaaagtttgatctccatctaaaggttttcctacatttggtacatttatagggcttctcctgggtgtgaatcctttgatgttcaagaacatatgacttacagtggaaggatttcctgcactggctgcagtcaaagagtttctccccactttggtctcccaaatgatgatcaaaccctgagctgtaggtgagagctgccctatactgattcaattcaagaaatttcttcttagcatgggtttctcggtgcagacggtaggctgacaggcgtcggaaagctttctcacataaatcgcatttataaggcttcactccagtgtgaattttctcatgccgcgcacagttggaactccaccggaaggctttcccacacaccctacatttaaatgctttctcttgagtgtgaagtctctgatgatacgcaagatgggagctatgactgaaagtccttccacagtcactgcacttaaatgacactcccactgtgtgaagactctgcccacgttggtgatgagagctaaggctgaagtcttttccacacacgtcctttttgttccctttcagtccactatgaattctctgatgtaggctgaagcccccaatcatgtgtctgagccccttcccatatttcttgtagtcatagtggtgtgaactcattctgaagtgtttgccacagccatgtttaagggattcctttcttccagaaactctcaaatatgtaacatgttttaagtcaagactattacttcctgatacttcagagtcttttcctgtcctgtgactgaaattggtctcttctttcttaactcttacttgtatgggattttcacattgatccttctgcctgctcttctgttgaaaagattctctgagcccaattccctcagaaacacttgtcgcaggacatcctgatgacacagctaaggtttctgcttcttccaaaggttcctgatttaagatgaatttgtttgttttactctggaggtcatctcctgtaggagcagcaactggattccccttaggctgagctgcctgcatgttcaggccccatggctcccttgcttccaaccaggagatcagagcaggtttggtgaatggtcccaccagggaagccatgttcctataattctccagcatcacatccctgtacaggttcctctgagcagagtccagccacccccactcgtcctgggagaaggtcacctccacatccttgaaagtcatggtctcctggagctgggctgtcagggacctggttggtgttacctggtctcccgggcacccctctctcgggaaaagggcaggcatctgggcagcaggagtatcggattgcccagccaggaagtcacgtgcttctatttcatagggaggctccaggtggtcccccagagcagagctgctcctgagaggtgaagcaagggaccatatctgtgcagatcgcagggctcctgtacccatccaatgcacatctgggctctgggcagggcccgggtccctccaggatgtcccatcaaggtccctctgcagctcctccagcaaggccacagcctcctcgccactctcagggttatgaagctgcacccaaacccggagctccccaggcaggatgctcaggaactgttccagcaccagcagctctaggatctgtgccttggagagaacgtcaggcctcagccaccagcgacagagttcccggagccggctcagagtttctaggggccctgaagactcatggtagcgaagctgtctgaagagctggcggaacagctcctggccagggcggttgagagtctgtggcctggcagcctgcactggagtatagctttcatcctcttcttccttctttactgtctgaagccgccctcgctccctcgaagactgggcctgagctggataggcagcatgccacctgcctggaggcatcactcctgttcagggactaaccagaagagtgcgaaccaagtccaccttagacgtgggtcctcagaagtatcttctcagcagtcaacaatgccaacatttgctgggacatcagaagtcatcagcaagtgactgaaattaccagcatttctgtagtcccagctactcgggaggctgaggcagaagaatcacttgaacccaggaggcggaggctgcagtgagccgagatcatgccattgcactccagccttgcgaaagagcgagactccaccgactcccgccgccgagcgacaatcggtccacccgccgccaccgcagccgcccgtcccgcgcctacctcccggcggctcc

SEQ ID NO: 12234 - RNA, 5794 nt, Homo sapiens
  source 1..5794: mol_type = other RNA
ctgggaggtcaaggctgcagtaagctgtgatcctgccactgcactccaccctgggcaaccctgtctcaaaaaataaaaaagacagtaaaaatatccctatactggggcaggaactttacaaggtatcctgtggcaaagggagcagagatggggggaaaggggtgctaaaagtttgattggaaagggacttttccatggttacaacaccaactgacatggaagctgcacctctgagagggccctggtcctagaggtcaaccacctgatggagagccttggtaaaccaagccctctttcaccaatctcaggaatcaggtagcacagccaagcactctaacttcacacataaggaaattgatgcagaggttcattgacttgctcaagatcaatcctgccaagaaaaggcacaccatgcctggaacccagatctgatgactccaagacccttcctatgactctggcccccctgcccagccacttctagtgccagttttgggacagtgaagggacatcttcagtgccatgaacagctgctgccgtaggaaggcaagaggatggcagaaccaagatgaccaaaccttcctgaggacaaagctgaacaggcatcagaacaccaacaggagacttctgccccgcccccaccatcctgtgacaccaccacacaatatcagagccttcattttcacctgctcatggcaatccagagcaggtaagattattccatactctactgaaaaagacatcttccaggttggtttcttctcatttcaagaaatgaccagctccatgaacgggcccctatagtcaggacactgctctactattaaaacattttatcctttcattcataatctgacctcttcaataatcagaagcaatgattactcacatgctttagcaatatcactcctttgcctttaagtaattgattcttgctttttgcttcaacacaagtgggtgggccagtgagggagctcctcccagaacaggctgccttttctcctgagagcagcaggcacatgcacttgttccttcgggttgaatctgattgctagcaccagatctcatacatggagaggggtatgtgaagctgagaggggcctgcagtgtgcaggggctagagacatgaacacaacaatggtaagcgtttatatctgctgaggccgaggatcctatagaaaattcagaaacggagtggggaggagtctgatttatgggaactggcagcaaggctaactgcatgagaagcctttcacccttttactgagtccttggatctgtggttaacccttataaaatataattcagattcaaaccacatcactcctcaactcaaaattgtccaaaagctccctgcctccctctgagccagctcaagcccccgtaatgacccatgatgctcatatggccgggcctgtggcctccctggcccctctccttcccttccagctggctccctgcactccatcccaggggcttccttcctgaggacaccagtcaagacccaatctcctctgcctgcaactctccctagagagctacctgctacctccctggcttccttcacgtctttgctcacatttcaccttctcagttgaggccctccctgaccagactatctaaaatcacgactgatctcccaatccagcactccctctgctcttctctgattcactttgtccactacacacatcaccatccagaatactgcgtatcccatttgtttgtcatctgtaaagatccaagatggcaggattttcatctgttctggtccctgctgggtctctggcaaacacaccagcgcctggtgtatgggagtgctcagcacatttctgttaaacagatggaccgctgctgcctatgcaggcctgtgggatggggatggcaacagggtactggtagagatccacacgccaagcgcttgagcccagcatcctgctctcctccacctgccgctgagaccactctaaccccctagcagatatccaaaagccagccaggaaggctgaagccccagccagaactccccagggggcatttgggaaggctaggagttcttgatgctgctgcttttaaagtcaacagaataggcatggccacaggccaaacttgaagacaaatctaggatcccactggcccctttccagcagccatagcccatgatgccacagatattctgtccaaccacaaagggcagtggtctctctcttcagagttgtggaaggagacctgaataggggagccgcaggctatggtgcagaggccactcctaggggccggagtctccagaagggctccaaaggacatggtgctgcacttccccagcgtcacatcctagcaggcaggctggggactccccgagctttcaaatccttgggattctgtcactagcttccaaaacagaaagggctgggccctttatcaaagttactccacaatgcctataattaagggttctctagcaggggactgagaacccacccccactgtcactgtcaggtcccaggctaatctctaatatggtttttcatatgccgagccaggttcgaagaccacctgaaggtctttccacacttgctgcatttgaagggcctctctcgagtatgaaatctcttgtggctaatgagttgtgaactcttgttaaaagttttcccacatatgctgcatttgtggcactttttcccaatgcttatgtcctggagtccagtgagcctggagctctggctgcaagcttctttgcagtcttcgaggggcatctcttcacttggttttagcttctgtaatctcaactttgtgtcctgagaggaagaccgtgcaggcgggctacgttcagcctgtgctgctctggtgtgtttcctctggtgactggaaagggtatgtctcccaatgaactctttcccacaccactgacatttgaaaggtctctctgtagagtggatcctctgatggttaacaaggcgatagtttctatcataagatttcccacatagattacatttatagcgcttctctccactgtgtattcccttatgatctaaaagggttcttttacgtgtaaaggttttcccacattcttgacaccaaaaacgtttctcaccagtgaggatttttggctccacatttggagtcttttcactttcatggcaatcatactgtttttgaagagagtgaatcctctgatgtcggtagagattggaactccatctgaaggctttcccacactccctgcacttatatggcttctctccagtgtgaactctctgatggatgaggaggaatgagtgattgcggaaggccttgccacactggctgcatttgtagggctcctctttggagtgactgctctgaggaacctggaacactgtgtcctgactaaaagatggcccgccctcaggttttcttttcatggcatgcttcttcttatgaacaataaaggctgacctataggcaaagtccttcccacaatcgctacactggtaaggtttctcacctgtgtgaattctctggtggtcaacgagagttttctttctagtaaaagttttcccacactgctgacacagaaatgttttctccacagcgggagcaccctggggctgactgcagtcaggagattgcctgaagccttcacgacattcatcttgtttgtagaatttttcctcctcatgcaacctcatatgacgagtaaagtttgatctccatctaaaggttttcctacatttggtacatttatagggcttctcctgggtgtgaatcctttgatgttcaagaacatatgacttacagtggaaggatttcctgcactggctgcagtcaaagagtttctccccactttggtctcccaaatgatgatcaaaccctgagctgtaggtgagagctgccctatactgattcaattcaagaaatttcttcttagcatgggtttctcggtgcagacggtaggctgacaggcgtcggaaagctttctcacataaatcgcatttataaggcttcactccagtgtgaattttctcatgccgcgcacagttggaactccaccggaaggctttcccacacaccctacatttaaatgctttctcttgagtgtgaagtctctgatgatacgcaagatgggagctatgactgaaagtccttccacagtcactgcacttaaatgacactcccactgtgtgaagactctgcccacgttggtgatgagagctaaggctgaagtcttttccacacacgtcctttttgttccctttcagtccactatgaattctctgatgtaggctgaagcccccaatcatgtgtctgagccccttcccatatttcttgtagtcatagtggtgtgaactcattctgaagtgtttgccacagccatgtttaagggattcctttcttccagaaactctcaaatatgtaacatgttttaagtcaagactattacttcctgatacttcagagtcttttcctgtcctgtgactgaaattggtctcttctttcttaactcttacttgtatgggattttcacattgatccttctgcctgctcttctgttgaaaagattctctgagcccaattccctcagaaacacttgtcgcaggacatcctgatgacacagctaaggtttctgcttcttccaaaggttcctgatttaagatgaatttgtttgttttactctggaggtcatctcctgtaggagcagcaactggattccccttaggctgagctgcctgcatgttcaggccccatggctcccttgcttccaaccaggagatcagagcaggtttggtgaatggtcccaccagggaagccatgttcctataattctccagcatcacatccctgtacaggttcctctgagcagagtccagccacccccactcgtcctgggagaaggtcacctccacatccttgaaagtcatggtctcctggtctcccgggcacccctctctcgggaaaagggcaggcatctgggcagcaggagtatcggattgcccagccaggaagtcacgtgcttctatttcatagggaggctccaggtggtcccccagagcagagctgctcctgagaggtgaagcaagggaccatatctgtgcagatcgcagggctcctgtacccatccaatgcacatctgggctctgggcagggcccgggtccctccaggatgtcccatcaaggtccctctgcagctcctccagcaaggccacagcctcctcgccactctcagggttatgaagctgcacccaaacccggagctccccaggcaggatgctcaggaactgttccagcaccagcagctctaggatctgtgccttggagagaacgtcaggcctcagccaccagcgacagagttcccggagccggctcagagtttctaggggccctgaagactcatggtagcgaagctgtctgaagagctggcggaacagctcctggccagggcggttgagagtctgtggcctggcagcctgcactggagtatagctttcatcctcttcttccttctttactgtctgaagccgccctcgctccctcgaagactgggcctgagctggataggcagcatgccacctgcctggaggcatcactcctgttcagggactaaccagaagagtgcgaaccaagtccaccttagacgtgggtcctcagaagtatcttctcagcagtcaacaatgccaacatttgctgggacatcagaagtcatcagcaagtgactgaaattaccagcatttcgactcccgccgccgagcgacaatcggtccacccgccgccaccgcagccgcccgtcccgcgcctacctcccggcggctcc

SEQ ID NO: 12235 - RNA, 1689 nt, Homo sapiens
  source 1..1689: mol_type = other RNA
ctgggaggtcaaggctgcagtaagctgtggttgtgccgccgcactccagcctgggcaacagagccagaccttgtctcaaaaaaaaaaaagaaaaaaaagaaaaaaaaaagtcacccctgtgtgaagttgtgaagttttccagtaacccacaactcaataccactcccaccaggtaagattaattacctcctcttttatgctccacatttgtaccttgtacaaacttattctagctcctggtgcactttattgtctcccagattcaagcatcctgaactttgaatccagctcttccacctgagagctgagtgatcttaggcaagataatgtgtgtgcctggcatactatagcatctagcccatatcataaacactataaatggtagtgctactattattactattatgatttgtctttggagaagtagtataaaataacattttgatttaaaaagcaggttttcgtgccagactgccccagttcaaatcctagctgtgctacttaccagctgtgtggccttgggcaagttagttcacttctctatgcctttgcctccttattcctggggtcgataataatggctatttcatagggttgctgtgaggtttaaatgggttaatatatataaagtgcttaggataatgctgacaacagtagaagcacaatacatattatctattcatagggtaacatctggaactctctgctctcagtgattgttgcttgaaaaaaacgattgaccaattcctctaagaggtcataacctctccttccctctgcagctcccctgtgctcatgtctcaggagcttagcctcaggagacgctttttgtgcatatttcgtcccccatggtatctccctagtaatgtgtggagtaggtactggagcatttttacattggattacctgacatgataagtcaatttcaaatctagttttgtgaattgtatttctcccacctagttgttgcctacgttctttcattaagaaattgtgttcttttgacttgaggccaaatgataagacctctcacctgaaatgttctttttcatgccttctgaactgtatctcttccctgtctagactagctaaccactcagttccatagtttttctacagtcagtccctaaaggaggcccttcaccacacatagctttctctgtgcagttgtgatgaattcttgcctcgcttgtctgtgcttgctaggtcgggctcagttcttcgtgggtggctgtgtgtaattcactggagatcaaaaccggagctctttggtgccatgcttgcctctcttcccgccacactgaccaccagtccttcagactttgttttgtcatggcatactctacgactcttgccactttgccataagtgctctcagctcaaactcaggatgtcccaaactgcattcattttcttcatcctgtcccacctgagttatccatctggacatctgctgtcagttctgggtcctctttctgttgtatccccttttcttccttctcactgccattcttctaggtcaggcctttgttatgtcacacccagacctctgagctggctcccagctgatatccctgccttcttctgctttcctcttgataatataccttgctgttgccaagtttgtctttttttctttctttcttctgagacagtcttgctctgtcgcccaggctggagtgcagtggt

SEQ ID NO: 12236 - RNA, 1878 nt, Homo sapiens
  source 1..1878: mol_type = other RNA
ctgggaggtcaaggctgcagtaagcttagatcatgccactgtacgccagcctaggcaacagaatgagaccctgtctcaaaaaaaaaaaaaaaagttatgtttacactacactatagtctattgtacaatagcataatgtctaaaaatgtacattctttaatttaaaaatactttattgctgaaaatgctaacagtcatctgagtcttcagcgagttgtaatccttttgctggtggagggtcttgcctcaatattgatggctgctgactgctcagggtggtggttggttgctgaaggctagggtaactgtgacaatttctatgtgatttactttggctaagtggtgtgtgtatcttctgggaagaagctttaggagccagctcagggttaaccatgttctctgttttctgtacgtatgagaatcttgaagcatgtgctgagacagatcctctatcagtctgggtccatgagcgacttcaaagggcagggcttccatgcagatcaaaatgtttggagttactctttcttcttgatgggtggagagggggtattttcttccatttgtttatgtttgtagcccatatttctgccatctcagtatcctcaaatcttccagattaacgggatcatgctttctgccaccaagaggacacaacaaaatcctcaggttctttgttttcatatgcagagtatgaggccctccctcacaaaatccacttcttccagcaataagatcttgtcttttatgttggaaatttcatcaagaaaccttttgagagtcatctcctccaacttgaaaaagcagcaggagtcggttctggttgtcttcccactccgtgcataatgattgcgcattttctatcatgactgtgcattgtttttgtaattcaactattttcagcaagagaagtatcaaaagaaatcaggagtggttgttgaagcagcatccacctgtgagcaggtgtaaacatcaagtcccaagggtccagcaactacccaaaacctcctgctttgtgccaggctgagggaatgttcactaaggcagtgtggcaggtggaggccagggcaggcccagagttccctggggctgctgagcccagtgtgggcaggttggcaacaggactccaaagagacatgtagccagtacaaaccatgccccagctaagcgtgatgccttcccctttcttccatattgatatcacctgctccaggcctggcacaggtgcagcaccttccccagaagccttccctgacggcctccttcttcaccagctctagtatttatcagctgtgtggcaagttagttcacctcccccatgccttggtttccccacctataaaatgaggataagaatgtttgtaagaatcaaatgagtaatatttgtaaagtacttgtaacggtgcttggcttagagttagtactctatcatgttactcatcatcaccatcaccattatgatttccaccatgcccatggaatctgcccttgatcaagacatccacttggtcttgtgtgggaggctgcctaggggaagcagggcctgatattatttatttctgttcacatcccagccagcaaaggtgccagcactgaatttatgctcagtacctacctggctgattaaactttggaaagaagcagcaggccagttaagaaaccacatgcaagcataactgtcctgaaaccctacttagttctgtgacgtcccttcttagaaattctgagttttctttccctagacatggtcactatttctacctagattctttcataacccactcatcagagaaatgtaagaaccaaagtaagacctttatcaggaaaactataaaacactgatgaaagaaatagaagaggatacaaacaaatggaaagcta

SEQ ID NO: 12237 - RNA, 419 nt, Homo sapiens
  source 1..419: mol_type = other RNA
ctgggaggtcaaggctgcagtatgccatgatcataccactgtactccagcctgggcaacagagtgagatcctgtctcaaaaattgaaaaaaaaaaaaaaaaaaggtttaatgtgtagaagggaaaaggctaaatggaaatgtgttaaagtcttaacggtgatcttccttggagcaatgatatagtgggtggttgctattcttttctttatacttttatgtacttttatgttatgcaaggttgaaaaaatgggcacatattgctttcatagtcatttctgttaagataatcatatgattatgaaagagggagtgtgtgtgtgaaagtggaatggaccaatcaaatagaacagtaggaagacctcagaagatatgacacatgagctcaaccccaaagatgagaagaaccagccatttagtg

SEQ ID NO: 12238 - RNA, 249 nt, Homo sapiens
  source 1..249: mol_type = other RNA
ctgggaggtcaaggctgcagtcagccatgattatgccactgcattccagcctgagcaagagtgagaccctgctcacttccgacccagcgcggtcgcacgaggactggacgtttgagtccgagcaactccccccggctgaggcggctcttcgggggctgggccgggacctatgagtctgggactccagctcccggcccagggccgacaactcgccccgcagccccggccccggcttccggcgccactgtc

SEQ ID NO: 12239 - RNA, 1938 nt, Homo sapiens
  source 1..1938: mol_type = other RNA
ctgggaggtcaaggctgcagtcagctgtgattgcactactgtactcctgcctgggcaagagcaagaccctgtctcaaaagaaaaaaaaaaaaaaagtggcctgggggaaacaggacagtcatataccccaagaatggaaattttcatgccaccccccttccttccttacaaattctaatgctgattgcatgaacgaggtgttgagagagacttttcttcatttagacatttgccctagtgaatgagggagcaagagaatgctaagagggatgagagaatatatttctggctctaggactttgacatccaggtaattgaatctgggacattctcattaggttagaaaaggaaagatgagaaaatcactagcaggatatgcaattccagagaccatctgctccaaaaattagttttgtttctcattgctccttattcagcgacagttatttcaataagctacattatttagcagagtctgagagacaaaggctgtgaaaacatgtatttatgatagaaaacaaactcagaaaaatataatagatagttcactttttatctcattcacattctatagctggagaactcaaaatcccatttagatatttctgcttatccaaaagcacactgggtgaaactaaaccaccaaatgggagaaaatgttcattgggtgtgtgtggcttcacccagtttatttacctatggagtggaagtgtagggagaaataaggtctgcttataatggtcaaggtctatggagaagccctgaagttgctctccccaaatcacaagtctgattcaagaaaaggaaacaaaaatgatgaaaacatctcatcacacaaaactcagtgatggggtctctgacagtcaccagccagcaggggaaaaggagaaatccacctgccggctttaagatttattgaaggctgccagcacagcccagatcatttctgtggcactaggctttgtcccttccacttcagggtccagttctactaagtccttggctcgattcattgccacatcatacttgtcatctgtcagagaggagaagacattctctagcacatcagaggagtgggctagcaccaggagtgctagtgttcgcttgtccatacgctgagggtcatttacccaccgctctagtacactatcttgaagttttttcactagtcgctgtttctctgttgtattggtcactggatgagtagtcatgtcaaatagcaggaaattctgcttctcagtggttagaatacctttctctactaggttctttgcgatgcgctctcgtacatttctcagctggtactgtaatttgaaggggttccaggtctcaccagtgagtagctctatccatgtttggacagtttctgtgggttcagttgctttgatgtgtttcagagtttcatccagtaaaacatcacctgttgggctgtctgactttagcagtacctttctgtctagtagtcgcttcttacgcatggtcgggggttccagatagattcgaccccgcatggccagctctatcaggatgccccctcgcaggcctgatgatatgcagtcattccagaaagatgtgtacccctctttatcttttagtcccagaagcaatacttcttccataagagtaaggcggatatccttagagtctccagaatcttcattgtctggacttttctcccaattactgtcttcctcactttccatcttcttttcagagttcttgcttatttcagtgcgacgggcccggtgagttaaagtggtcattctcacctgtttctgatgttactcctgggttatggctggacgcaggctgtagcttgtgctgtattttagaaggacacctgttctccccaccccacccccgtcctagtaggtgaaaaacttagccacgcagagagcacaaacttcctgatccttcgatgcagagaaggaataacac

SEQ ID NO: 12240 - RNA, 2814 nt, Homo sapiens
  source 1..2814: mol_type = other RNA
ctgggaggtcaaggctgcagtcagctgtgattgcactactgtactcctgcctgggcaagagcaagaccctgtctcaaaagaaaaaaaaaaaaaaagtggcctgggggaaacaggacagtcatataccccaagaatggaaattttcatgccaccccccttccttccttacaaattctaatgctgattgcatgaacgaggtgttgagagagacttttcttcatttagacatttgccctagtgaatgagggagcaagagaatgctaagagggatgagagaatatatttctggctctaggactttgacatccaggtaattgaatctgggacattctcattaggttagaaaaggaaagatgagaaaatcactagcaggatatgcaattccagagaccatctgctccaaaaattagttttgtttctcattgctccttattcagcgacagttatttcaataagctacattatttagcagagtctgagagacaaaggctgtgaaaacatgtatttatgatagaaaacaaactcagaaaaatataatagatagttcactttttatctcattcacattctatagctggagaactcaaaatcccatttagatatttctgcttatccaaaagcacactgggtgaaactaaaccaccaaatgggagaaaatgttcattgggtgtgtgtggcttcacccagtttatttacctatggagtggaagtgtagggagaaataaggtctgcttataatggtcaaggtctatggagaagccctgaagttgctctccccaaatcacaagtctgattcaagaaaaggaaacaaaaatgatgaaaacatctcatcacacaaaactcagtgatggggtctctgacagtcaccagccagcaggggaaaaggagaaatccacctgccggctttaagatttattgaaggctgccagcacagcccagatcatttctgtggcactaggctttgtcccttccacttcagggtccagttctactaagtccttggctcgattcattgccacatcatacttgtcatctgtcagagaggagaagacattctctagcacatcagaggagtgggctagcaccaggagtgctagtgttcgcttgtccatacgctgagggtcatttacccaccgctctagtacactatcttgaagttttttcactagtcgctgtttctctgttgtattggtcactggatgagtagtcatgtcaaatagcaggaaattctgcttctcagtggttagaatacctttctctactaggttctttgcgatgcgctctcgtacatttctcagctggtactgtaatttgaaggggttccaggtctcaccagtgagtagctctatccatgtttggacagtttctgtgggttcagttgctttgatgtgtttcagagtttcatccagtaaaacatcacctgttgggctgtctgactttagcagtacctttctgtctagtagtcgcttcttacgcatggtcgggggttccagatagattcgaccccgcatggccagctctatcaggatgccccctcgcaggcctgatgatatgcagtcattccagaaagatgtgtacccctctttatcttttagtcccagaagcaatacttcttccataagagtaaggcggatatccttagagtctccagaatcttcattgtctggacttttctcccaattactgtcttcctcactttccatcttcttttcagagttcttgcttatttcagtgcgacgggcccggtgagttaaagtggtcattctcacctgttttttggagatcacaagtctagacgataacattcagaaaatcatgtgtagtaattccacagtcagtaaacttagcagctctagtcctagctagccatatcttgcaaatacacaaggagctgcaaacaaaaattactggcaagagagtgttgaaagattaacaaattttctcaatttaaaaaaaaaagtcaaagaacatgtcttttattctatgtactacggtcaaaagaaactgcactaaatcatttgtgataaagtttatagttagcatactttattttatataaatctagatatcagtttttaagataatatataacaaatattttaaatcagcaattatataaaggagtatctttttcaagatcaaaataatggtatttaagagttgctatgactggactcgtttctactcctctagcaatatttcccattgctcctaataagtagtgttgccagactttttctcaaaaatgtctcatgctttctttctgcttctgctcctctgtacttgctggggtcttcacccttttctcttcctctttacattctacccattctttaaaggccttgtgaaggcctttaagtgacctcctcttttctattacctatgtgtctcatggccactccctcagctgtttcacagagctttatttatactcacttcctttaaagtatttattatagtctttctcttggtatagctgtctctcaactgtaaacttcttaagaacagggatattgtcttcttgggtttatatattctccatagcaactagcactgtctttaacattgttattgctcgataaatttatattgattaaaatgaatactcagaagtgcatgtgaacatttaaaatagaaatacaaatgaagtgagctacaaaagtttttttgtacaagggtatatttcaaatataatttgttatgggaggtgggaagaaaagtgaaggaggaagagaaccatgaaataaattcttaagcgcactaagcctatctggcactgtgaatagggactatttcctaaaccaatccaagaaa

SEQ ID NO: 12241 - RNA, 1684 nt, Homo sapiens
  source 1..1684: mol_type = other RNA
ctgggaggtcaaggctgcagtgaaatgtgattgtaccactgtacttcagattgggcgacacagtgagcctctatctcaaaaacaaactaacaacaacaaaaaacagtacttggtacacacaaggtgcttaatatatattgttaaataaatggttacctatagatacacacttgcatgcttatgcacagctatacataattactgtttatagttactatggtttaataggggcaattcttccaggtgagaaaagcagacgtttccagttgcagttttgacataatgtcctagaaagatttcatttaaatagattttttcaataaaagaggcattgcacaaagtcccttattggtgcagcctcaacattttctttggcggtttggatgctctgctgtctaggctgtggccctgtgcatgtggtcttgatggaatgtcccgattagttatgagatgttcccgaggagcctgggggaatagcttgtcagttcaagtctcaccacggaaggtttctcattagcagttctcttgaaattcttcttgggccgtctctatcctccggcgactcaaaacagcatgcttgcttatagtttcttttgtcaatctttttccttatcgactgagttctggaggctgaaagtcaaggtgttggttgatctacagagttggttctgtctgagggctgggagggaaggatgtgttccaggtccatgtccttagcttatagatggctgtcttctccctttgtcttcacatcatattcctcctgtatgtggctgtgttcaaatttcctgcaagtaggtctgtctgatgataaaacctttgctcttaaagggaattcctagctattcatggccttagttgtgaacgtcttgagccgttcctattctcaatcattcttgattattctgtttcatgcttataggctcctaatgttagctgacgagatgttgtcaataattgttgcatcattgctgttgggtcttgaaatatcatttcatcatagaactctgaaaccactgtctttttccccagcattgcattggtgtctgattgaaacagctttagcaaatgatacagggttacaggtctttcattagggtcaatgaaaaatattttgatgattatttcgaattcaccccatcctgtttcagtaatttcatatggaggtttagtaacaactcttaaaggattgccatagctttcatgtaatttaaactggattttcttcacatatgctgacatatcctcatttctatatggtttcacatatactgtccactgatgagtgtgcccatcttcttctcttttctttccaaaataccgagcaacattaccgtaaactattggtttaacgatagtaacaccctttactctcccgccggagtcaggcccaaattcggccattctcttgaacatattgtcccacggaagaagccgccgccgccagggaaagagaccggggctggcggggtcgccgctcccctcagagaccgcgctcctgtcgcgcgggcccaggcggagggtttctagccgaaggagggcgagttacttgggctcacggcggtgagtaaccgtcaactcctcaggccgactgtgctcctgaaggccattcaggcccgcgcaggtggagaacgccgcgaaaagaggggcgacggccgcaccgcgcgcaggcgcaacgggctcg

SEQ ID NO: 12242 - RNA, 2561 nt, Homo sapiens
  source 1..2561: mol_type = other RNA
ctgggaggtcaaggctgcagtgaacagtgatcccaccactgcactccagcccaggtgacggagtgactctgtctcaaagaaaaagtacctgcacaaaccaaagccaattactctgtcttcagaatagacatccaaaaccaaggctacaatccaagtcttcaataatgaaagttttctggccaggtgtggtggctcgtgcctataatcccagtattttggggacagaggtgggaggatcacttgggcctaggagtttgaaaccagcctgtgcaacaaagtgagatccctccatctctacaaaaaataaagaataaaaaaaatccgggcacggtggtacacacctgtggtcccagctacttgggaagctgaggcgggaggacagcttgagcctgggaggtcgagactacagtgagccgtgattgcccccctgcactccagtctgggtgacagaatgagactatctccaaaaaaaagaaagttttctaacatttagacttgcaaaagaaaaagaaaatcagaattgactgtgtcagaaaacacggtgtttcctgtttctagaatgacaggtggagaccaccgattcctgtgctgggcaggaggctggaggttatagccaatgattcgtttgaggtctaagaaccaacaaaaactctctgctataatgaaagtgcatccaggggcacagggaatactagttttttccttagtgtgaaagcaggctggggcatctgtttctttgttccctgtttgtccactcttcgactcacatcatcgttgacagcagtgaggatggataagatgtcttcatgtcttgggaccaatttcttcagatgattacacagagactgaatataccagctgccttcctccacatgccgaaaggatacatagcctgggacagtggccagaccaagtaggaagtcagcctcggcaggaatactgtcctgcagggaagtgggtgcctgctcagggttcagagcatctgcttcgatggatacggaaggctgtatctcttcaccttggcaggcctggatgaaaaagagtttaggtttttcagccagtctagggcactgcagggctgtgaagtgagacatgatctcccgaatgggaatgagggcctcatccgaagagtagacagctccaaatctcccatgggtcagaatacagaacacgaagcagtccccgtcggcatgggctggattgcacttctgcttctgcaggaccatctccatttccactttcgtcacattattgtgtatatgcactgtgaacccaagccactggaacacatgactcaggatctcagcatctttatgggttccttgtctgtccttcagggaggtaaagctgtggttgttgacaatgacacagaggcctctgtggttccgattcatcctgtacacagctgccctcattactacctgcatgcttattttgccaggactccggtaaggcttccaagaatgtcttaacatctgtttgggaaactagttcttcctctccttgatacgactcggcttccttgtctacaggaggtgtcactatctggatagctttctctcttttgtatttctctatgtttctcaaaagtttaggtacaactgttttgcagaggtcctccaggcatgtcagattatcttcatctattttaccttgtttctctagaaatgccaggaaacttagggaggtcatttcagttttgggaagcgagtctttcagaaggaagatcatgtcctttaagttctctgagtcaatgccttctgacagttcgtagagcaggtttctaaacagagaaaccctttgtcgggtgggcagcagtcgctccacttcctctttggtacagttgaggtgctgcagcagcttcttctgccgtatgatatagaggagttctgccaggaagaaagggtcttcctcactcagcagatcctctgccaagagatgttcaaaaacatctgaggctgagctggacttctccagcttcttgttggggaccaatcctatgcagagaaacttgaggttctccacatcttggacccccaggtttgaatcaataatcagaagcttctcacgaaagctcactttacagtttttatctgaactggaataccaatgttgaccttgagatttcatggccagccttcagatcaagctccaccaatcttctggaagtaaacggttctcagggaaattgcctgaaaacaaagttttaaagaaagtagaatcctctgtgtgctccaaggtccaaagaagctcccatttgcttgggaagagacttcaagacttgctggttgtttaagtgaaaactgaatcttcaggactgggtagcctgatactagtttcctgctgatgtcatcactgcttatctgcctttttccctccccttttccagggttaagataactttgacaaacagcgtctcctaaaggctaatttacaactttctcactgtagagcttggggtttccccaggtaaagcaaaagcttcctagaaacgaacccgtggaagccacaaagtgcttcaggctttcctttggatctccatttccttggtaagtcaaaaa

SEQ ID NO: 12243 - RNA, 2308 nt, Homo sapiens
  source 1..2308: mol_type = other RNA
ctgggaggtcaaggctgcagtgaacagtgatcccaccactgcactccagcccaggtgacggagtgactctgtctcaaagaaaaagtacctgcacaaaccaaagccaattactctgtcttcagaatagacatccaaaaccaaggctacaatccaagtcttcaataatgaaagttttctggccaggtgtggtggctcgtgcctataatcccagtattttggggacagaggtgggaggatcacttgggcctaggagtttgaaaccagcctgtgcaacaaagtgagatccctccatctctacaaaaaataaagaataaaaaaaatccgggcacggtggtacacacctgtggtcccagctacttgggaagctgaggcgggaggacagcttgagcctgggaggtcgagactacagtgagccgtgattgcccccctgcactccagtctgggtgacagaatgagactatctccaaaaaaaagaaagttttctaacatttagacttgcaaaagaaaaagaaaatcagaattgactgtgtcagaaaacacggtgtttcctgtttctagaatgacaggtggagaccaccgattcctgtgctgggcaggaggctggaggttatagccaatgattcgtttgaggtctaagaaccaacaaaaactctctgctataatgaaagtgcatccaggggcacagggaatactagttttttccttagtgtgaaagcaggctggggcatctgtttctttgttccctgtttgtccactcttcgactcacatcatcgttgacagcagtgaggatggataagatgtcttcatgtcttgggaccaatttcttcagatgattacacagagactgaatataccagctgccttcctccacatgccgaaaggatacatagcctgggacagtggccagaccaagtaggaagtcagcctcggcaggaatactgtcctgcagggaagtgggtgcctgctcagggttcagagcatctgcttcgatggatacggaaggctgtatctcttcaccttggcaggcctggatgaaaaagagtttaggtttttcagccagtctagggcactgcagggctgtgaagtgagacatgatctcccgaatgggaatgagggcctcatccgaagagtagacagctccaaatctcccatgggtcagaatacagaacacgaagcagtccccgtcggcatgggctggattgcacttctgcttctgcaggaccatctccatttccactttcgtcacattattgtgtatatgcactgtgaacccaagccactggaacacatgactcaggatctcagcatctttatgggttccttgtctgtccttcagggaggtaaagctgtggttgttgacaatgacacagaggcctctgtggttccgattcatcctgtacacagctgccctcattactacctgcatgcttattttgccaggactcctgcggtaaggcttccaagaatgtcttaacatctgtttgggaaactagttcttcctctccttgatacgactcggcttccttgtctacaggaggtgtcactatctggatagctttctctcttttgtatttctctatgtttctcaaaagtttaggtacaactgttttgcagaggtcctccaggcatgtcagattatcttcatctattttaccttgtttctctagaaatgccaggaaacttagggaggtcatttcagttttgggaagcgagtctttcagaaggaagatcatgtcctttaagttctctgagtcaatgccttctgacagttcgtagagcaggtttctaaacagagaaaccctttgtcgggtgggcagcagtcgctccacttcctctttggtacagttgaggtgctgcagcagcttcttctgccgtatgatatagaggagttctgccaggaagaaagggtcttcctcactcagcagatcctctgccaagagatgttcaaaaacatctgaggctgagctggacttctccagcttcttgttggggaccaatcctatgcagagaaacttgaggttctccacatcttggacccccaggtttgaatcaataatcagaagcttctcacgaaagctcactttacagtttttatctgaactggaataccaatgttgaccttgagatttcatggccagccttcagatcaagctccaccaatcttctggaagtaaacggttctcagggaaattgcctgaaaacaaagttttaaagaaagtagaatcctctgtgtgctccaaggtccaaagaagctcccatttgcttgggaagagacttcaagacttgctggttgtttaagtgaaaact

SEQ ID NO: 12244 - RNA, 2271 nt, Homo sapiens
  source 1..2271: mol_type = other RNA
ctgggaggtcaaggctgcagtgaacagtgatcccaccactgcactccagcccaggtgacggagtgactctgtctcaaagaaaaagtacctgcacaaaccaaagccaattactctgtcttcagaatagacatccaaaaccaaggctacaatccaagtcttcaataatgaaagttttctggccaggtgtggtggctcgtgcctataatcccagtattttggggacagaggtgggaggatcacttgggcctaggagtttgaaaccagcctgtgcaacaaagtgagatccctccatctctacaaaaaataaagaataaaaaaaatccgggcacggtggtacacacctgtggtcccagctacttgggaagctgaggcgggaggacagcttgagcctgggaggtcgagactacagtgagccgtgattgcccccctgcactccagtctgggtgacagaatgagactatctccaaaaaaaagaaagttttctaacatttagacttgcaaaagaaaaagaaaatcagaattgactgtgtcagaaaacacggtgtttcctgtttctagaatgacaggtggagaccaccgattcctgtgctgggcaggaggctggaggttatagccaatgattcgtttgaggtctaagaaccaacaaaaactctctgctataatgaaagtgcatccaggggcacagggaatactagttttttccttagtgtgaaagcaggctggggcatctgtttctttgttccctgtttgtccactcttcgactcacatcatcgttgacagcagtgaggatggataagatgtcttcatgtcttgggaccaatttcttcagatgattacacagagactgaatataccagctgccttcctccacatgccgaaaggatacatagcctgggacagtggccagaccaagtaggaagtcagcctcggcaggaatactgtcctgcagggaagtgggtgcctgctcagggttcagagcatctgcttcgatggatacggaaggctgtatctcttcaccttggcaggcctggatgaaaaagagtttaggtttttcagccagtctagggcactgcagggctgtgaagtgagacatgatctcccgaatgggaatgagggcctcatccgaagagtagacagctccaaatctcccatgggtcagaatacagaacacgaagcagtccccgtcggcatgggctggattgcacttctgcttctgcaggaccatctccatttccactttcgtcacattattgtgtatatgcactgtgaacccaagccactggaacacatgactcaggatctcagcatctttatgggttccttgtctgtccttcagggaggtaaagctgtggttgttgacaatgacacagaggcctctgtggttccgattcatcctgtacacagctgccctcggtaaggcttccaagaatgtcttaacatctgtttgggaaactagttcttcctctccttgatacgactcggcttccttgtctacaggaggtgtcactatctggatagctttctctcttttgtatttctctatgtttctcaaaagtttaggtacaactgttttgcagaggtcctccaggcatgtcagattatcttcatctattttaccttgtttctctagaaatgccaggaaacttagggaggtcatttcagttttgggaagcgagtctttcagaaggaagatcatgtcctttaagttctctgagtcaatgccttctgacagttcgtagagcaggtttctaaacagagaaaccctttgtcgggtgggcagcagtcgctccacttcctctttggtacagttgaggtgctgcagcagcttcttctgccgtatgatatagaggagttctgccaggaagaaagggtcttcctcactcagcagatcctctgccaagagatgttcaaaaacatctgaggctgagctggacttctccagcttcttgttggggaccaatcctatgcagagaaacttgaggttctccacatcttggacccccaggtttgaatcaataatcagaagcttctcacgaaagctcactttacagtttttatctgaactggaataccaatgttgaccttgagatttcatggccagccttcagatcaagctccaccaatcttctggaagtaaacggttctcagggaaattgcctgaaaacaaagttttaaagaaagtagaatcctctgtgtgctccaaggtccaaagaagctcccatttgcttgggaagagacttcaagacttgctggttgtttaagtgaaaact

SEQ ID NO: 12245 - RNA, 2426 nt, Homo sapiens
  source 1..2426: mol_type = other RNA
ctgggaggtcaaggctgcagtgaacagtgatcccaccactgcactccagcccaggtgacggagtgactctgtctcaaagaaaaagtacctgcacaaaccaaagccaattactctgtcttcagaatagacatccaaaaccaaggctacaatccaagtcttcaataatgaaagttttctggccaggtgtggtggctcgtgcctataatcccagtattttggggacagaggtgggaggatcacttgggcctaggagtttgaaaccagcctgtgcaacaaagtgagatccctccatctctacaaaaaataaagaataaaaaaaatccgggcacggtggtacacacctgtggtcccagctacttgggaagctgaggcgggaggacagcttgagcctgggaggtcgagactacagtgagccgtgattgcccccctgcactccagtctgggtgacagaatgagactatctccaaaaaaaagaaagttttctaacatttagacttgcaaaagaaaaagaaaatcagaattgactgtgtcagaaaacacggtgtttcctgtttctagaatgacaggtggagaccaccgattcctgtgctgggcaggaggctggaggttatagccaatgattcgtttgaggtctaagaaccaacaaaaactctctgctataatgaaagtgcatccaggggcacagggaatactagttttttccttagtgtgaaagcaggctggggcatctgtttctttgttccctgtttgtccactcttcgactcacatcatcgttgacagcagtgaggatggataagatgtcttcatgtcttgggaccaatttcttcagatgattacacagagactgaatataccagctgccttcctccacatgccgaaaggatacatagcctgggacagtggccagaccaagtaggaagtcagcctcggcaggaatactgtcctgcagggaagtgggtgcctgctcagggttcagagcatctgcttcgatggatacggaaggctgtatctcttcaccttggcaggcctggatgaaaaagagtttaggtttttcagccagtctagggcactgcagggctgtgaagtgagacatgatctcccgaatgggaatgagggcctcatccgaagagtagacagctccaaatctcccatgggtcagaatacagaacacgaagcagtccccgtcggcatgggctggattgcacttctgcttctgcaggaccatctccatttccactttcgtcacattattgtgtatatgcactgtgaacccaagccactggaacacatgactcaggatctcagcatctttatgggttccttgtctgtccttcagggaggtaaagctgtggttgttgacaatgacacagaggcctctgtggttccgattcatcctgtacacagctgccctctttgtgctggtttcagagtttagagtgttagcagatgctccttgcatccccctggagaccaggcttggtgcaccatttgtggctctgttaccattactacctgcatgcttattttgccaggactccggtaaggcttccaagaatgtcttaacatctgtttgggaaactagttcttcctctccttgatacgactcggcttccttgtctacaggaggtgtcactatctggatagctttctctcttttgtatttctctatgtttctcaaaagtttaggtacaactgttttgcagaggtcctccaggcatgtcagattatcttcatctattttaccttgtttctctagaaatgccaggaaacttagggaggtcatttcagttttgggaagcgagtctttcagaaggaagatcatgtcctttaagttctctgagtcaatgccttctgacagttcgtagagcaggtttctaaacagagaaaccctttgtcgggtgggcagcagtcgctccacttcctctttggtacagttgaggtgctgcagcagcttcttctgccgtatgatatagaggagttctgccaggaagaaagggtcttcctcactcagcagatcctctgccaagagatgttcaaaaacatctgaggctgagctggacttctccagcttcttgttggggaccaatcctatgcagagaaacttgaggttctccacatcttggacccccaggtttgaatcaataatcagaagcttctcacgaaagctcactttacagtttttatctgaactggaataccaatgttgaccttgagatttcatggccagccttcagatcaagctccaccaatcttctggaagtaaacggttctcagggaaattgcctgaaaacaaagttttaaagaaagtagaatcctctgtgtgctccaaggtccaaagaagctcccatttgcttgggaagagacttcaagacttgctggttgtttaagtgaaaactgaatcttcaggactgggtagcctgatact

SEQ ID NO: 12246 - RNA, 2400 nt, Homo sapiens
  source 1..2400: mol_type = other RNA
ctgggaggtcaaggctgcagtgaacagtgatcccaccactgcactccagcccaggtgacggagtgactctgtctcaaagaaaaagtacctgcacaaaccaaagccaattactctgtcttcagaatagacatccaaaaccaaggctacaatccaagtcttcaataatgaaagttttctggccaggtgtggtggctcgtgcctataatcccagtattttggggacagaggtgggaggatcacttgggcctaggagtttgaaaccagcctgtgcaacaaagtgagatccctccatctctacaaaaaataaagaataaaaaaaatccgggcacggtggtacacacctgtggtcccagctacttgggaagctgaggcgggaggacagcttgagcctgggaggtcgagactacagtgagccgtgattgcccccctgcactccagtctgggtgacagaatgagactatctccaaaaaaaagaaagttttctaacatttagacttgcaaaagaaaaagaaaatcagaattgactgtgtcagaaaacacggtgtttcctgtttctagaatgacaggtggagaccaccgattcctgtgctgggcaggaggctggaggttatagccaatgattcgtttgaggtctaagaaccaacaaaaactctctgctataatgaaagtgcatccaggggcacagggaatactagttttttccttagtgtgaaagcaggctggggcatctgtttctttgttccctgtttgtccactcttcgactcacatcatcgttgacagcagtgaggatggataagatgtcttcatgtcttgggaccaatttcttcagatgattacacagagactgaatataccagctgccttcctccacatgccgaaaggatacatagcctgggacagtggccagaccaagtaggaagtcagcctcggcaggaatactgtcctgcagggaagtgggtgcctgctcagggttcagagcatctgcttcgatggatacggaaggctgtatctcttcaccttggcaggcctggatgaaaaagagtttaggtttttcagccagtctagggcactgcagggctgtgaagtgagacatgatctcccgaatgggaatgagggcctcatccgaagagtagacagctccaaatctcccatgggtcagaatacagaacacgaagcagtccccgtcggcatgggctggattgcacttctgcttctgcaggaccatctccatttccactttcgtcacattattgtgtatatgcactgtgaacccaagccactggaacacatgactcaggatctcagcatctttatgggttccttgtctgtccttcagggaggtaaagctgtggttgttgacaatgacacagaggcctctgtggttccgattcatcctgtacacagctgccctctttgtgctggtttcagagtttagagtgttagcagatgctccttgcatccccctggagaccaggcttggtgcaccatttgtggctctgttaccattactacctgcatgcttattttgccaggactcctgcggtaaggcttccaagaatgtcttaacatctgtttgggaaactagttcttcctctccttgatacgactcggcttccttgtctacaggaggtgtcactatctggatagctttctctcttttgtatttctctatgtttctcaaaagtttaggtacaactgttttgcagaggtcctccaggcatgtcagattatcttcatctattttaccttgtttctctagaaatgccaggaaacttagggaggtcatttcagttttgggaagcgagtctttcagaaggaagatcatgtcctttaagttctctgagtcaatgccttctgacagttcgtagagcaggtttctaaacagagaaaccctttgtcgggtgggcagcagtcgctccacttcctctttggtacagttgaggtgctgcagcagcttcttctgccgtatgatatagaggagttctgccaggaagaaagggtcttcctcactcagcagatcctctgccaagagatgttcaaaaacatctgaggctgagctggacttctccagcttcttgttggggaccaatcctatgcagagaaacttgaggttctccacatcttggacccccaggtttgaatcaataatcagaagcttctcacgaaagctcactttacagtttttatctgaactggaataccaatgttgaccttgagatttcatggccagccttcagatcaagctccaccaatcttctggaagtaaacggttctcagggaaattgcctgaaaacaaagttttaaagaaagtagaatcctctgtgtgctccaaggtccaaagaagctcccatttgcttgggaagagacttcaagacttgctggttgtttaagtgaaaact

SEQ ID NO: 12247 - RNA, 2199 nt, Homo sapiens
  source 1..2199: mol_type = other RNA
ctgggaggtcaaggctgcagtgaacagtgatcccaccactgcactccagcccaggtgacggagtgactctgtctcaaagaaaaagtacctgcacaaaccaaagccaattactctgtcttcagaatagacatccaaaaccaaggctacaatccaagtcttcaataatgaaagttttctggccaggtgtggtggctcgtgcctataatcccagtattttggggacagaggtgggaggatcacttgggcctaggagtttgaaaccagcctgtgcaacaaagtgagatccctccatctctacaaaaaataaagaataaaaaaaatccgggcacggtggtacacacctgtggtcccagctacttgggaagctgaggcgggaggacagcttgagcctgggaggtcgagactacagtgagccgtgattgcccccctgcactccagtctgggtgacagaatgagactatctccaaaaaaaagaaagttttctaacatttagacttgcaaaagaaaaagaaaatcagaattgactgtgtcagaaaacacggtgtttcctgtttctagaatgacaggtggagaccaccgattcctgtgctgggcaggaggctggaggttatagccaatgattcgtttgaggtctaagaaccaacaaaaactctctgctataatgaaagtgcatccaggggcacagggaatactagttttttccttagtgtgaaagcaggctggggcatctgtttctttgttccctgtttgtccactcttcgactcacatcatcgttgacagcagtgaggatggataagatgtcttcatgtcttgggaccaatttcttcagatgattacacagagactgaatataccagctgccttcctccacatgccgaaaggatacatagcctgggacagtggccagaccaagtaggaagtcagcctcggcaggaatactgtcctgcagggaagtgggtgcctgctcagggttcagagcatctgcttcgatggatacggaaggctgtatctcttcaccttggcaggcctggatgaaaaagagtttaggtttttcagccagtctagggcactgcagggctgtgaagtgagacatgatctcccgaatgggaatgagggcctcatccgaagagtagacagctccaaatctcccatgggtcagaatacagaacacgaagcagtccccgtcggcatgggctggattgcacttctgcttctgcaggaccatctccatttccactttcgtcacattattgtgtatatgcactgtgaacccaagccactggaacacatgactcaggatctcattactacctgcatgcttattttgccaggactcctgcggtaaggcttccaagaatgtcttaacatctgtttgggaaactagttcttcctctccttgatacgactcggcttccttgtctacaggaggtgtcactatctggatagctttctctcttttgtatttctctatgtttctcaaaagtttaggtacaactgttttgcagaggtcctccaggcatgtcagattatcttcatctattttaccttgtttctctagaaatgccaggaaacttagggaggtcatttcagttttgggaagcgagtctttcagaaggaagatcatgtcctttaagttctctgagtcaatgccttctgacagttcgtagagcaggtttctaaacagagaaaccctttgtcgggtgggcagcagtcgctccacttcctctttggtacagttgaggtgctgcagcagcttcttctgccgtatgatatagaggagttctgccaggaagaaagggtcttcctcactcagcagatcctctgccaagagatgttcaaaaacatctgaggctgagctggacttctccagcttcttgttggggaccaatcctatgcagagaaacttgaggttctccacatcttggacccccaggtttgaatcaataatcagaagcttctcacgaaagctcactttacagtttttatctgaactggaataccaatgttgaccttgagatttcatggccagccttcagatcaagctccaccaatcttctggaagtaaacggttctcagggaaattgcctgaaaacaaagttttaaagaaagtagaatcctctgtgtgctccaaggtccaaagaagctcccatttgcttgggaagagacttcaagacttgctggttgtttaagtgaaaact

SEQ ID NO: 12248 - RNA, 1931 nt, Homo sapiens
  source 1..1931: mol_type = other RNA
ctgggaggtcaaggctgcagtgaaccactgcacttggcctgggagacagaacaagaccaaaaaagtaaaaataataataataataataataatacaagatcctgcattataggcactaatggaatgcaataaatgcacagagaaaacagccataaatctcatgttcgagaagacacccaagaaagcatcactgagaggtagatctgaactaagaacaatcagtaggattttacaggatagaaggtaggatagaaggtaggtgggaaggggtgacatgaaggcaaagatttcaggaagaagaaaaattcataattaaaaacataaaagggccgagtgcagtggctcacacctgtatctcagcactttgcggggttacggcaggaggactgctcaagcccaggaattcgagatcagcctgggcaatgaagtgagacccttgtctccacaaaaaatttgtttttaattagccagtcatggtggtgcacgcccatggccacagctacttgggagagtgggatgggagaactgcttgagcctgggaggttaagactgtagtgagccatcatcacgtcactgcactcaggcctagactatagagcaagactctgcctcataaaaaatacaaaaagatgtttaggacaacattctagaacttaccagtatgtaggaacatggccagatgtagaggtagacaaactaaggtaggtggagaaatataacagaaggccttgaatatatcatactaagaagtttaaaccttactttgtaagttttaagcaagtgtaaattgggtgggagagtttctggctcctgagcctagcctacaccataacgtataaatcttagcagaagtcctcaccttgtgcattccacccacacaagtcattagatctctgaactcacaaggtaactggcataaacaatgacacataactaaaaacaaatccctcagagcaactgcaattcaaaaatatagtcaaactctttttttctggacctgctatcagttccagcattcacaaatcccttttctcacaaatgcttctattaaatgtaattccaaataaacataaaggaagcagaagttgtcactgcttctggaattttcccttgcttacaccaagaatatatttaaaattatatacttttaaaaaaacaaaaacattacaacatgctacattcttcaagacaccagaagtcttattcaatgtaacaatttagcacactataatctctgaggaacagtgagttccaagataattcaatataatcttcaagtgacaatctgaaataagattaggcataaataatatgcaaaagaatattaacctccaacacagtaaacttgaagtgttagtaactttgactcaagtgctaaaattcaaaacagcaattaagttactgaaacattttacaaccctaacacaaatagattatcaatgcctccaccctacccataaatatctcacttcataatttcttcttccaaataactaatgaataattacgtacatctaaaagtacaaattcaagaccaataccaaaattcagattttttacagccaattattaagctttaaagtatcaagtatacagtttataacccaagctacaaaatttatgtaattaaaacatttaactcaagtgaataacccaagttttaaattatattgtatcaataaaaaaaatgttatgtagtaattctcaacagaaggcaatccttctatccatattcaaatgcaacctgttccaatttttaatacaacagaggtaactgggttactatcactactactagttttagctgtcataaattgagcaagtgtctgttctcacttctttagccagcattgtgtaataaagaatttggggcccaggcacagtggcacatgcctgtataccagcactctgggaggccaaggcaggaggat

SEQ ID NO: 12249 - RNA, 71 nt, Homo sapiens
  source 1..71: mol_type = other RNA
ctgggaggtcaaggctgcagtgaaccatgattgtggcactatactccaggctgggcgccagagagaaactc

SEQ ID NO: 12250 - RNA, 1243 nt, Homo sapiens
  source 1..1243: mol_type = other RNA
ctgggaggtcaaggctgcagtgaaccgtgtttgcaccacggtattccagctgggccacaaagtgagaccccaagatcatatagcgtggactccctgtgacctgattttcaaactactgatctttggaactcctgtgctacccctctgtgttgctgaaggccatctattcttagttggttctattgatgttggttgaaaccatcccgaacatacctgtggctaggcacagtggctcacgtctgtaatcccagcactttgggaggttgaggggggcggatcacttcaggtcaggagttggagtccagcctggccaacatgatgaaaccccatctctgctaaaaatacaaaaattagcaaggcatggtggtgcacacctgtgactctagctactcgggaggcggaggcaggagaattgcttgaaccctggaggcagaggttgcagtgaattgagaccacaccactgcactccagcctgggtgacagagtgagaccctgcctcaaaacaaaacaaaacaaccatcctgcacaattatgagtgagagtaaatccaacacatctcacagcatcttgggaaaatgataaggctcactttcttctttcccttcagtgtgaactcatgtaataacttcagagaaaggcatttccctgctgtctggaagttgaactccttctacaaactggtggagcttgctgcccagtcctgtgccctccgagctgaggggaaggcgtggggattttctgttctactgaaatggcaggattatgtcatagcagtggttttgagtgtttagaggtagtgttattttaattatttttctaactctggtttaaataaaaacttacaaatcaggaaagaactggctatctgtatgttaaaaaaattaagagagggctgggtgcagtgtctcacgcctgtaatcccaacactttgggaggccgaggtgggtggatcacgaagtcaggagatcgagaccatcctggccaaccaacatggtgaaaccccgtctctactaaaaatacaaaaattagctgggcgtggtggcgtgcgcctgtaatcccagctacgcaggaggctgaggcaggagaatcgcttgaacctgggaggcggaggttgcagtgaaccgagattgtgccagtgcactccagcctggccaacagaacaagactccgtcttaaaaaaaaaaaaaggagagagagagagggaacattgactcttaccttgtaccatcccaaaaattcattt

SEQ ID NO: 12251 - RNA, 6794 nt, Homo sapiens
  source 1..6794: mol_type = other RNA
ctgggaggtcaaggctgcagtgaactgagatcacgctactgtacttcagtctgggtgacagagcaagaccctttctcaaaaaaacaaaaacacaaattgagtcttctcattcacaagagccagagatgggtgcaggctcctcccagctgtaagtttctgctggcaaccatggacctccagggtttcggcatctagggcaacctctcttctaaggacaccattccttacccacgtttcaacatctcccaccaaccaaacaaaccatccatttgatcattctaagaccctgttcagttctttaggtgccgaggataagacacaataattttatgaggatttttctgagctctaagcataaatccatctttcatattagatgctaccacctatgtgcaggatgttttaattattttaatttcataccgtttcaaagacatcatcagatagatagtgctcctcaagggaaattttggcttggggtggaggcacatgttcaaatttctgcacttaggccagtatggtggctcatgcctgcaatcccagcactttgggaggccgaggtgggaggattgcttgagcccaggagttccagagcagcctgggctacatagtagaacctcatctctagtaaaaaaatacaaaaaaattagccgggcatggtgatgtgcacctgtagtcccagctactcaggagactgaggtgggaggatggcttgaaccagggaggttgaggttgcaatcaaccatgattgcaccactgcactccagcctgggtgacagagccgaggtcttgtcccaaaaaaaaaaaaaaaaaaaaaaaaagtctgtactttggcccagcgcttctcaacatacatgaagacgtattggttttctccaaactgtgctccccgggatacttacccttaagggcaccccaacatgcttcctgaggacagtcaagcctcctgggatgcagtgagtgagcaccaatgggcaggtctataatgggcaagaatagactcgaggacaatgtggaccacagagcccctttagtcttgctgctgtgtcacactagctactcagccagggaaacaattaaacaggattcaagcagacataattgaaataggtccttttttgacttcctgtgaatatcaactactactaagaatcacttgatctgatacatattattaaaatgttatttgtgtgttttgtgtaacttttttttttcttttgccaacattccatagtttgttcatggtaacagcagtaaggttctcatgccaagcattcctccttttacaagggggatagcatgatgctataagcctaggaaaaataaaattcaaagtttaaaatgaaaaaaatagagtaagacctactatttgatagcaaacagggtgactataagcaataataactgtacatttttaaataactgagtgtagctggattgtttgcaactcaatggataaatgcttgaggaggtagacaccccattctccatgatgtgcttatttatttcacattgcatgcctgtttcaagacatctcatgtaccccataaatatatacaccttctatatacccgtaagaattaaaaatagaaaaaaaatgaaaacaaactttaaagcgaccacaccaaccatattggtaatccagtttaaagtgaccacaccaactgtattgatgataaaccaaagtgaccacaccaaccgtactgataatcccgcttaaagtgaccacggcaaccatactgatagtccagtttaaagtgaccacaccaaccgttttgataatccagttttgtattttgacttctgaaatatgatcataaatgtttaattctgggccataactgggaaattagttactgaacatctaactttcaacaaaaaagcccatgaagtttacatagataattcttgtgtttaaccaagtaataaaatatttaataaaatgaaagtatacagaagaaaattatgaattcatcaaatcaggccgttttgcatccagattgtattcagaaaacttgtttaacacctaggaaattactgtccaaagttgatagtgcttggtcttttttatcagtttttattctgaaagctgtgcattactaatctacttttatgtaaatctgaaatacagtatttatcccatatgtccacatggtaaagtaatcaagaaagatattttcagtgcttagcacccccaccccaatttaaaggaaactctgactgtagtaaattcatgctaattgagaactctggggaaggggttaaaacattacccaggtacaagtcgggtggccattataaacgttacccaaataaaagccagaaacaggaagccaaaaaccaggtccctaaggcaggcatgtgtcttaaatgatatcatttgtcaagcttccagcatcttgtggtggtgaacacaaaaagaaggtctgcgttgtactgaggacattacatcctcattagctggaatgttcctcaagtacataatgcaggattttcattttaataagaagcagctacttgtcactgcactttcattagataaacacagaatgtaatactaatgaccatttacagaggctctatcctactcctgaggaacttcatccagatgaaatcatataatgacaagttatagaatatatcatgcaaaacttccttcatttctttgcaaactattccctgaatttttttttttttaatgctgaggtcagttaacagcagtagtcatcatcaaaggaacccctaaatgacactgctggtattttctgcctgcaaaacaggcttgaaggaatagcatttggctctttagaagtcataaccaaatggtaacagatcactgggactccttggtttctcaaagaggcaagctccttccaccctgcccggctggtgaccttaagcccgacatgcagagaagtccacgctgagaaataatttactcactgggattgttccaccctggccccttctctaaaaagactgacaattgccctgaattatggatgtactttttgtgatatgtattacagttcagaagaaaggtgttgagaccatcgtaccgtttcacctcccattagaggctggtcttgaacaataatcccagaagatgaaactgatgctgaactatgaccctcaatttacaaatcatttttcaaaagaataaaaaaaagtttaaacatatttttggcattatctgaatgggcggaatctttcatgcttgttttctaagaataagtgaaaacagcatgcagtgcactttcttagtttggggaaagagagaacatgaggttttcagattatattttattttaatcctgggcgtttgaattttatttttacatagctgcatttagtatattccctcaaaacacaataaatttctattctgtagcttaagggatccatcagttaaaatgttggtctttcatctttattaccctcccattaaaatgaaacaaaccgggactcacttcagtttcgaagaagcaatttagttggtaatgtccttactccccaagtctttacaaagggagaaagtacattactgcttagatttcacacatctatctgcataagaagcaactaagccttttggacatagactatgttaaatttaataatattctttgattagattattttattacaacattttttccattaccagtcatttcctgtgcacagttacattcataaaacctgctcccccctcctttgtttgtttgtgaatgtaaaagtgaggcaaagtctctttccgtgtggctgtggctgttaggtctgaaagggatggatgaataactaagcaccacactggacgggtttttcctagtcccctgcaccagtaaccctttgctataatgaggacacaaagagcctcgcatcaggccgctacccttcttcataactcaaaagcgtcacagtggcaatagcctctagtgctatttgtctttagtgcagttgtgacacttcggcatgatccataatttggcagctatttaccgtgacatttcccttcagtgcagccataacattcagtgaagccattatttggttccatttaccatataaattgtattgttgtgcatgcatgctagcagctacattaggtacctgaaaatgagtaaatcttgtaaaatagatactaacagctattcagcagtaggatttccttgctcctcagatggaaggaaagaaaaattaaatacagtccccaaatttcctagagcatctttaattgcgtccatatttactgagcaggttagatacaccgaaacctaagactttgaaaaataatctggtgggcttcaccttcaatcagaacgggcccatggggtttcagcgcaacggtgacagcggcagcagtcttcagggcactaaaggttaagagggaagccgatgagccacaggcgtgactcagaagagagggtgcaggtttcgctgcttttcctgtgtggtcagtgggtcaatgtgggacatcaggctatagtgccaaggagcatctcattccaccagaacacgtggagagaaaaatgggaatgcagaatgagtggctgctattctgtttccagaatcagaggtaacgcatagcttctagttcgaacgcctctaaggagaagcaaatgtattcttccttgagatgactgaggtctctacggtgcacagggcgatgggacataccgtacctcgagcagtgtagcatgctgttactaaggccttgccgtgtgcctagacagcgcttccctcctggggcccgtgttttgtggtgaacccccactgagaatggagcgcacacttttctctttcctgtgcctatattaattttaagtccccctaatctctgtggtttccctttccaaaacctactttctgtctatgtaagttttcaacattaatttgctgcttcagaggaaagagaacatttccatttcacatgtgccttatcaggttgatggtagataaaagccattacgtgctacttcttcaaaacacatctgtgttcacggaatcatttttctaataacaaaatcaaatttgggagggaattcccccaaatgtccatttagatagttggttggtgatttatagaaaaaaaaaggaccatttcctgaggatatagattctgaaaatatatggctggcttttgctacacttgtcactcatgaactgcttatgagcataagaccaaattctcccaaagcaaagaagtcgggaaccactttcaaaactgattttaaaatctgatcaagctgaagacatactgactcgatcagatctggcatcaggaatgaatttagttccctggaacaataacatctggaacgagaccatccatgactaaagaattgaatgtaagcgttttccctcttagccatggagggaagttttattagcacatttttttttttcccccaagggaagaggaggaggaggaggagaaggagagacctattcattaacaccttacttttgttttaagaaatattatatccattaccaactaaaaataaattgatttgagtaattctgagacataaagtgcccattttctttctcccttgatttatgtcattgttctgtttttacagcttactgttgacagagtgaggtaattcaactacaatttttccagtgttttttcccatgtacatataattgacagcacggaatatggactccaggccagtaaacctgccctctggagacagatctccaaggtccacctcacaaaccaggtctccgctcacacacatctcgagcaagtggctcatggctgcttgatacttagaaaggtaatggttcaggaagaagccctgtacgctggcagatttcttgagcagtttggctggcaatgttcctgctttcacaggcgaaaggccagtaggagtttggtagccagagataaaccctattactatcaagcgccctttcgtagccagggcgtctacagccaagtcaaacatggctcccccaacagattcatagaccacatcgacaccttcagggtactcctgcttaaggacggtacctacgggttcagttttatagttgataggacgatcacagccaagagatttcagaaaagcagacttttcatcagaagagcaggttccaattacatggcactttgccttctttgaaagctgcatggcaaactggcccgttcccccagctgctgctgtcaccaaaacttttttcccttccgacagtcctccgagctctttcaggctgatgtatgcggtggtgccacttaccagcagggtaagatactcgggtttcactgagggcactggagttgcaatgctggcaggcacaactgtgtactcagcaaaagaaccaggtgccatgtaagccacagcttggccaactgtgtatctggcactagcagagaggcctagggccaccacctccccaatgccttcgaaacctatgtcaaagggaggcttaactgaggggtcatagcggcctgctgaatagttgatgtcagatgcgttaacaccaacaaatcggttccggacgaggaggtctccgtccccggggagcggcaccgggcagtcccggctcagggtgacggcctcgcggaagttggggctcagccgggtcaccaccagcttctgcatggcttggggaatggcggagccctggaagtccaggaagtggcgggcgtacgacatgtccacgatggcccgggccccggtgggcaccagccgcagcatggcctgcgcctccgcccgctctctgcgccgacgctggccggggtcggcccccgcccgggccgctcggctcggctgtgctct

SEQ ID NO: 12252 - RNA, 6825 nt, Homo sapiens
  source 1..6825: mol_type = other RNA
ctgggaggtcaaggctgcagtgaactgagatcacgctactgtacttcagtctgggtgacagagcaagaccctttctcaaaaaaacaaaaacacaaattgagtcttctcattcacaagagccagagatgggtgcaggctcctcccagctgtaagtttctgctggcaaccatggacctccagggtttcggcatctagggcaacctctcttctaaggacaccattccttacccacgtttcaacatctcccaccaaccaaacaaaccatccatttgatcattctaagaccctgttcagttctttaggtgccgaggataagacacaataattttatgaggatttttctgagctctaagcataaatccatctttcatattagatgctaccacctatgtgcaggatgttttaattattttaatttcataccgtttcaaagacatcatcagatagatagtgctcctcaagggaaattttggcttggggtggaggcacatgttcaaatttctgcacttaggccagtatggtggctcatgcctgcaatcccagcactttgggaggccgaggtgggaggattgcttgagcccaggagttccagagcagcctgggctacatagtagaacctcatctctagtaaaaaaatacaaaaaaattagccgggcatggtgatgtgcacctgtagtcccagctactcaggagactgaggtgggaggatggcttgaaccagggaggttgaggttgcaatcaaccatgattgcaccactgcactccagcctgggtgacagagccgaggtcttgtcccaaaaaaaaaaaaaaaaaaaaaaaaagtctgtactttggcccagcgcttctcaacatacatgaagacgtattggttttctccaaactgtgctccccgggatacttacccttaagggcaccccaacatgcttcctgaggacagtcaagcctcctgggatgcagtgagtgagcaccaatgggcaggtctataatgggcaagaatagactcgaggacaatgtggaccacagagcccctttagtcttgctgctgtgtcacactagctactcagccagggaaacaattaaacaggattcaagcagacataattgaaataggtccttttttgacttcctgtgaatatcaactactactaagaatcacttgatctgatacatattattaaaatgttatttgtgtgttttgtgtaacttttttttttcttttgccaacattccatagtttgttcatggtaacagcagtaaggttctcatgccaagcattcctccttttacaagggggatagcatgatgctataagcctaggaaaaataaaattcaaagtttaaaatgaaaaaaatagagtaagacctactatttgatagcaaacagggtgactataagcaataataactgtacatttttaaataactgagtgtagctggattgtttgcaactcaatggataaatgcttgaggaggtagacaccccattctccatgatgtgcttatttatttcacattgcatgcctgtttcaagacatctcatgtaccccataaatatatacaccttctatatacccgtaagaattaaaaatagaaaaaaaatgaaaacaaactttaaagcgaccacaccaaccatattggtaatccagtttaaagtgaccacaccaactgtattgatgataaaccaaagtgaccacaccaaccgtactgataatcccgcttaaagtgaccacggcaaccatactgatagtccagtttaaagtgaccacaccaaccgttttgataatccagttttgtattttgacttctgaaatatgatcataaatgtttaattctgggccataactgggaaattagttactgaacatctaactttcaacaaaaaagcccatgaagtttacatagataattcttgtgtttaaccaagtaataaaatatttaataaaatgaaagtatacagaagaaaattatgaattcatcaaatcaggccgttttgcatccagattgtattcagaaaacttgtttaacacctaggaaattactgtccaaagttgatagtgcttggtcttttttatcagtttttattctgaaagctgtgcattactaatctacttttatgtaaatctgaaatacagtatttatcccatatgtccacatggtaaagtaatcaagaaagatattttcagtgcttagcacccccaccccaatttaaaggaaactctgactgtagtaaattcatgctaattgagaactctggggaaggggttaaaacattacccaggtacaagtcgggtggccattataaacgttacccaaataaaagccagaaacaggaagccaaaaaccaggtccctaaggcaggcatgtgtcttaaatgatatcatttgtcaagcttccagcatcttgtggtggtgaacacaaaaagaaggtctgcgttgtactgaggacattacatcctcattagctggaatgttcctcaagtacataatgcaggattttcattttaataagaagcagctacttgtcactgcactttcattagataaacacagaatgtaatactaatgaccatttacagaggctctatcctactcctgaggaacttcatccagatgaaatcatataatgacaagttatagaatatatcatgcaaaacttccttcatttctttgcaaactattccctgaatttttttttttttaatgctgaggtcagttaacagcagtagtcatcatcaaaggaacccctaaatgacactgctggtattttctgcctgcaaaacaggcttgaaggaatagcatttggctctttagaagtcataaccaaatggtaacagatcactgggactccttggtttctcaaagaggcaagctccttccaccctgcccggctggtgaccttaagcccgacatgcagagaagtccacgctgagaaataatttactcactgggattgttccaccctggccccttctctaaaaagactgacaattgccctgaattatggatgtactttttgtgatatgtattacagttcagaagaaaggtgttgagaccatcgtaccgtttcacctcccattagaggctggtcttgaacaataatcccagaagatgaaactgatgctgaactatgaccctcaatttacaaatcatttttcaaaagaataaaaaaaagtttaaacatatttttggcattatctgaatgggcggaatctttcatgcttgttttctaagaataagtgaaaacagcatgcagtgcactttcttagtttggggaaagagagaacatgaggttttcagattatattttattttaatcctgggcgtttgaattttatttttacatagctgcatttagtatattccctcaaaacacaataaatttctattctgtagcttaagggatccatcagttaaaatgttggtctttcatctttattaccctcccattaaaatgaaacaaaccgggactcacttcagtttcgaagaagcaatttagttggtaatgtccttactccccaagtctttacaaagggagaaagtacattactgcttagatttcacacatctatctgcataagaagcaactaagccttttggacatagactatgttaaatttaataatattctttgattagattattttattacaacattttttccattaccagtcatttcctgtgcacagttacattcataaaacctgctcccccctcctttgtttgtttgtgaatgtaaaagtgaggcaaagtctctttccgtgtggctgtggctgttaggtctgaaagggatggatgaataactaagcaccacactggacgggtttttcctagtcccctgcaccagtaaccctttgctataatgaggacacaaagagcctcgcatcaggccgctacccttcttcataactcaaaagcgtcacagtggcaatagcctctagtgctatttgtctttagtgcagttgtgacacttcggcatgatccataatttggcagctatttaccgtgacatttcccttcagtgcagccataacattcagtgaagccattatttggttccatttaccatataaattgtattgttgtgcatgcatgctagcagctacattaggtacctgaaaatgagtaaatcttgtaaaatagatactaacagctattcagcagtaggatttccttgctcctcagatggaaggaaagaaaaattaaatacagtccccaaatttcctagagcatctttaattgcgtccatatttactgagcaggttagatacaccgaaacctaagactttgaaaaataatctggtgggcttcaccttcaatcagaacgggcccatggggtttcagcgcaacggtgacagcggcagcagtcttcagggcactaaaggttaagagggaagccgatgagccacaggcgtgactcagaagagagggtgcaggtttcgctgcttttcctgtgtggtcagtgggtcaatgtgggacatcaggctatagtgccaaggagcatctcattccaccagaacacgtggagagaaaaatgggaatgcagaatgagtggctgctattctgtttccagaatcagaggtaacgcatagcttctagttcgaacgcctctaaggagaagcaaatgtattcttccttgagatgactgaggtctctacggtgcacagggcgatgggacataccgtacctcgagcagtgtagcatgctgttactaaggccttgccgtgtgcctagacagcgcttccctcctggggcccgtgttttgtggtgaacccccactgagaatggagcgcacacttttctctttcctgtgcctatattaattttaagtccccctaatctctgtggtttccctttccaaaacctactttctgtctatgtaagttttcaacattaatttgctgcttcagaggaaagagaacatttccatttcacatgtgccttatcaggttgatggtagataaaagccattacgtgctacttcttcaaaacacatctgtgttcacggaatcatttttctaataacaaaatcaaatttgggagggaattcccccaaatgtccatttagatagttggttggtgatttatagaaaaaaaaaggaccatttcctgaggatatagattctgaaaatatatggctggcttttgctacacttgtcactcatgaactgcttatgagcataagaccaaattctcccaaagcaaagaagtcgggaaccactttcaaaactgattttaaaatctgatcaagctgaagacatactgactcgatcagatctggcatcaggaatgaatttagttccctggaacaataacatctggaacgagaccatccatgactaaagaattgaatgtaagcgttttccctcttagccatggagggaagttttattagcacatttttttttttcccccaagggaagaggaggaggaggaggagaaggagagacctattcattaacaccttacttttgttttaagaaatattatatccattaccaactaaaaataaattgatttgagtaattctgagacataaagtgcccattttctttctcccttgatttatgtcattgttctgtttttacagcttactgttgacagagtgaggtaattcaactacaatttttccagtgttttttcccatgtacatataattgacagcacggaatatggactccaggccagtaaacctgccctctggagacagatctccaaggtccacctcacaaaccaggtctccgctcacacacatctcgagcaagtggctcatggctgcttgatacttagaaaggtaatggttcaggaagaagccctgtacgctggcagatttcttgagcagtttggctggcaatgttcctgctttcacaggcgaaaggccagtaggagtttggtagccagagataaaccctattactatcaagcgccctttcgtagccagggcgtctacagccaagtcaaacatggctcccccaacagattcatagaccacatcgacaccttcagggtactcctgcttaaggacggtacctacgggttcagttttatagttgataggacgatcacagccaagagatttcagaaaagcagacttttcatcagaagagcaggttccaattacatggcactttgccttctttgaaagctgcatggcaaactggcccgttcccccagctgctgctgtcaccaaaacttttttcccttccgacagtcctccgagctctttcaggctgatgtatgcggtggtgccacttaccagcagggtaagatactcgggtttcactgagggcactggagttgcaatgctggcaggcacaactgtgtactcagcaaaagaaccaggtgccatgtaagccacagcttggccaactgtgtatctggcactagcagagaggcctagggccaccacctccccaatgccttcgaaacctatgtcaaagggaggcttaactgaggggtcatagcggcctgctgaatagttgatgtcagatgcgttaacaccaacaaatctctgcgtgagggtccgcagctcgcgccttccgctccaccagaaacaagttcaagcgcagcaggcgcaaagcgaatgcggggctcgggatggggagcaggggcggaagggccagggagccacagaaagacaagaaagacacactgggaaggattcgcgcatttggagaccctccttgtacccccaccccccctttaattgaaactgtgtgcatgcagtgagcgcaggattctagtaatccgacgggaggatccacttaaaagactaaaatccagaaaccccaggaaaaaagaataggaccggcgcaggcattctccaaatc

SEQ ID NO: 12253 - RNA, 67 nt, Homo sapiens
  source 1..67: mol_type = other RNA
ctgggaggtcaaggctgcagtgaactgagattgcaccactgcagtctcagcctaggcaccaaagtga

SEQ ID NO: 12254 - RNA, 4548 nt, Homo sapiens
  source 1..4548: mol_type = other RNA
ctgggaggtcaaggctgcagtgacctatgttcataccactgcactccagcctgggcgacagagtgagaccaactcaaaaaacaaacaaacaaacaaacaaacaaactttctctctcgagtccagtgattctccctcaacgctcaagactccagcatgaactgttaggcattgggtttttctgtgtttacagcagaccatggtaaaaagaagtcccaagtcacagccagaacgccaaagtaagatctgttgagtgctaggctcatggactgagcctaatcttattttccactctgcctcaaacaaaacaactcatttgcccatacaacccatggcatcctttcacagtaacaaggacaacaggacacctccagtactttttattttttttgagatgggagtcacccaggctggagtgcagtggcgcgatctcggctcactgcaacctccgcttccccgattcaagcgattctcctgcttcagcctcctgagtagctgggattaaaggtgcgtcccaccgtgcctggctaatttttgtatttttagtagagacggagctctgccatgttggtcaggctggccttgaactcctgacctcatgacccgcccgccttggcctcccaaagcgctaggattacagacgtgagccaccgcgcccggcaatatctccaatactttaatacttggttgaaaagaacccattgcactgtttcccactgtttgtcccagtactttagttttatgatctcatttgggtttttgtaaaagcagtcttcctacaagcctagtaaaggaaattctttctttctcattttgccaaatgtagcatttaattgattttttttttttttttttttttgagctagagagagtcttgctctgtcacccaggcaggagtacagtggcatgatctcggctcacttcaatctccacctcctagttcaagcgattctccgcctcagcctccagagtagctgggagctactccatgtaccacaatgcccagctaatttttttgtattttagtagtgatggggtttcaccctgttccccaggctggtctcaaactcctgagctcagacaatccacccacctcagcctcccaaagtgctaggattacagcgtgagccaccacacctggccaattctaattctgtgtaaaatgagtgaaacacagctaaactagaactagtccttgctagcatgttaatatagattttgctcaaacatctgccatccccatcctgttgcagagatgaccaacaaccctgggtccacagcatgttccaaatctctcaagtagtactaaatctattacttctagtaccccagcctttttccccctcctggtggcaaaattcaagtatctcacacgcaccctaaatgtctcttcctctatgcagggaacttttggttgcctccccaaataaacggcattgttcaaactcagagctcagaacaaaccaatgaaaaaaaaaaaaggaaatagcgtatttgttttaactttttattaaaatgcttaggatacagattgactttctttcgtaaatgactgttttacttttcctgaagtaggacatatatgcactctgataaaacagaatgagaagtcataattcatgggaattcctatacaaggtgctgatcctgtgtttggagctgagctcctcacagcagcttctttcagctatcttataggaatagtgttccgtggggcaagaaatacattggttctaactgattttcaatcccctttctccagtggaataaaccactttcacaaagagctgccctatgtataacccacagatttctagcttgcaacaaagtgacaagggacaaataggggaaaaaaaaaattaagaaaactaacactgaagtaatcatacttctcatgtctccgaacagagaagtatgggggacctttaaccaaaggaaattaaaaatatgcaagttatattacctagttcattcactgttagctagatttgttcacttaaggctttaacccctttccaaaccaacaactttgtcttaatccagctatgtttgctaataaacgaaatgcatgcacttcccacatatatacttcactgagcctctgcattcagtacctggcagtgaaaaagtatgctttccccacaagtcagtactggagaataagaatgagaactccaactaaagaacaatgcctccctcaccccagtaatgttatccacattttccctaccctcacattagaataaagacatcctcccaacttttcatctcctatctccaatctgttcataggagatatatcttttgatcttttattataagggtagaatatagattaagatcatcaaaatccaatttcacatgtggcactaggaaaatggaatgctataaaattaatccccatcacccaagtagggatgccggtgcttttatactgagtctttactgccaataagtgatgctgcctccaaaggaacagctctacagaaagtttttgggttagtgtttccctagcttatttctgcaatggagaaagacaatttcataccaaaaaaaaaaaaaaaaaaaaaaaaacctggaaaagctacagatgttaacctttactttaaacaccaataaaataggtgtcaaaggagaaaaaatgtaaaaaaaagagctcccaaacagcctgagagaccaaattctgcaaatggaaattttaaagcccactgaatacatttttcatggatccaaacaaatgctacaatacttttaagtcctcaactcacagaattaagagcccttaagctgttaactttgtcctgtcttcctattcagaaaaatgtccccctagaatctgtgcaaaagtaactgatgcacctgcagtatgtgacacgagagatgttctcaactcttttatgaggtcaaagtcacttttgataactgaaaacgaaaaaggaaggtgctatagagagaaattaaatttcacaaaagtataaaagcaaagactggctaaaatctgtaacttcatgagtaagaataacaacaataacccattctataattaactcctccacagtgaacaatctgctacacattccttgatgaggaatgaacctagcttaccacagtggaaacctgccacaactgcaaggccggggttctgccccttttctagttctctgtgcacaaggttatgccacctactccaaggcagtcagagagacaggtgagctcaggggagcttctctcaccaacctgctaactcagcaggagtaagtttacccaaatgagctctggcctccatatctgttcataattttatgaagtatctaaatgtcattcattagtttaaaaaaaaaaaagaatagaaaactctggaccaagtaaattgtgaactcaaaaagttaggagggataccaattacattaacaacgctttctttaaaaaatagaatcactttcttttgaatcaaccacagtggtgagacgtgtttttcttttcaggtgccccatgatggcatacagctttacccggcaaatcctgccagcttccaagtcccaggatactgacctgcaccagcacgtggggcagcattacctcccaacagtgtggagaagagcacatgtcaccactgggcaatgagagagttgacagagactcttggcttctcaacgccagacatggttggagagctttccttgttctattagaaaagttcatgaggaagctgtgaataggatcagtccagagaagtaaaactcttttattttcaccgtccaaacatcagtcaatatactgggagagccagcggaaaccctcgccgtaaccttgcctcttgagcacactgcacatgaacacttccatggggcgagcattcagctccttcagggtcacattcccctttcctgtggtctgtccataaagcccaaatatctcacggagtttttcttcactgattgcatctgttctgtcaattttgttacccaagataaggattggcacattggatattgtttcatcagtcattaaagcattaagctcaactttggattccacgaggcgagaatgatctgcacagtccaccagaaagacaatcccattaattgctgggagataatttttccaaacgcgacgtgcttgctcgtgcccaccaagatcaaaagttgtaaaggtcattccagcaattgttagctcttctgatgtcggatgtagtgttggaacatgttggcccaatctgtcatctttgagcatgtgaagaagagtggttttgcctgcattatccaaacctaagaatacaagttttccagatttcttgtacagtcctaggaactggagcacactgctgaagccattgtagatccactcaaagatgaaagacattattaatgcttactacctcatttgatgatactttgtggatcctgaggttttctggtttttttacaaattgaaggttggaagcagccggcctgaggggctcctccggcaaaacagcggctggctcggaccctccctcagagcacactaaccagcagcacccgggaccgccagctactcgccggatgtac

SEQ ID NO: 12255 - RNA, 4478 nt, Homo sapiens
  source 1..4478: mol_type = other RNA
ctgggaggtcaaggctgcagtgacctatgttcataccactgcactccagcctgggcgacagagtgagaccaactcaaaaaacaaacaaacaaacaaacaaacaaactttctctctcgagtccagtgattctccctcaacgctcaagactccagcatgaactgttaggcattgggtttttctgtgtttacagcagaccatggtaaaaagaagtcccaagtcacagccagaacgccaaagtaagatctgttgagtgctaggctcatggactgagcctaatcttattttccactctgcctcaaacaaaacaactcatttgcccatacaacccatggcatcctttcacagtaacaaggacaacaggacacctccagtactttttattttttttgagatgggagtcacccaggctggagtgcagtggcgcgatctcggctcactgcaacctccgcttccccgattcaagcgattctcctgcttcagcctcctgagtagctgggattaaaggtgcgtcccaccgtgcctggctaatttttgtatttttagtagagacggagctctgccatgttggtcaggctggccttgaactcctgacctcatgacccgcccgccttggcctcccaaagcgctaggattacagacgtgagccaccgcgcccggcaatatctccaatactttaatacttggttgaaaagaacccattgcactgtttcccactgtttgtcccagtactttagttttatgatctcatttgggtttttgtaaaagcagtcttcctacaagcctagtaaaggaaattctttctttctcattttgccaaatgtagcatttaattgattttttttttttttttttttttgagctagagagagtcttgctctgtcacccaggcaggagtacagtggcatgatctcggctcacttcaatctccacctcctagttcaagcgattctccgcctcagcctccagagtagctgggagctactccatgtaccacaatgcccagctaatttttttgtattttagtagtgatggggtttcaccctgttccccaggctggtctcaaactcctgagctcagacaatccacccacctcagcctcccaaagtgctaggattacagcgtgagccaccacacctggccaattctaattctgtgtaaaatgagtgaaacacagctaaactagaactagtccttgctagcatgttaatatagattttgctcaaacatctgccatccccatcctgttgcagagatgaccaacaaccctgggtccacagcatgttccaaatctctcaagtagtactaaatctattacttctagtaccccagcctttttccccctcctggtggcaaaattcaagtatctcacacgcaccctaaatgtctcttcctctatgcagggaacttttggttgcctccccaaataaacggcattgttcaaactcagagctcagaacaaaccaatgaaaaaaaaaaaaggaaatagcgtatttgttttaactttttattaaaatgcttaggatacagattgactttctttcgtaaatgactgttttacttttcctgaagtaggacatatatgcactctgataaaacagaatgagaagtcataattcatgggaattcctatacaaggtgctgatcctgtgtttggagctgagctcctcacagcagcttctttcagctatcttataggaatagtgttccgtggggcaagaaatacattggttctaactgattttcaatcccctttctccagtggaataaaccactttcacaaagagctgccctatgtataacccacagatttctagcttgcaacaaagtgacaagggacaaataggggaaaaaaaaaattaagaaaactaacactgaagtaatcatacttctcatgtctccgaacagagaagtatgggggacctttaaccaaaggaaattaaaaatatgcaagttatattacctagttcattcactgttagctagatttgttcacttaaggctttaacccctttccaaaccaacaactttgtcttaatccagctatgtttgctaataaacgaaatgcatgcacttcccacatatatacttcactgagcctctgcattcagtacctggcagtgaaaaagtatgctttccccacaagtcagtactggagaataagaatgagaactccaactaaagaacaatgcctccctcaccccagtaatgttatccacattttccctaccctcacattagaataaagacatcctcccaacttttcatctcctatctccaatctgttcataggagatatatcttttgatcttttattataagggtagaatatagattaagatcatcaaaatccaatttcacatgtggcactaggaaaatggaatgctataaaattaatccccatcacccaagtagggatgccggtgcttttatactgagtctttactgccaataagtgatgctgcctccaaaggaacagctctacagaaagtttttgggttagtgtttccctagcttatttctgcaatggagaaagacaatttcataccaaaaaaaaaaaaaaaaaaaaaaaaacctggaaaagctacagatgttaacctttactttaaacaccaataaaataggtgtcaaaggagaaaaaatgtaaaaaaaagagctcccaaacagcctgagagaccaaattctgcaaatggaaattttaaagcccactgaatacatttttcatggatccaaacaaatgctacaatacttttaagtcctcaactcacagaattaagagcccttaagctgttaactttgtcctgtcttcctattcagaaaaatgtccccctagaatctgtgcaaaagtaactgatgcacctgcagtatgtgacacgagagatgttctcaactcttttatgaggtcaaagtcacttttgataactgaaaacgaaaaaggaaggtgctatagagagaaattaaatttcacaaaagtataaaagcaaagactggctaaaatctgtaacttcatgagtaagaataacaacaataacccattctataattaactcctccacagtgaacaatctgctacacattccttgatgaggaatgaacctagcttaccacagtggaaacctgccacaactgcaaggccggggttctgccccttttctagttctctgtgcacaaggttatgccacctactccaaggcagtcagagagacaggtgagctcaggggagcttctctcaccaacctgctaactcagcaggagtaagtttacccaaatgagctctggcctccatatctgttcataattttatgaagtatctaaatgtcattcattagtttaaaaaaaaaaaagaatagaaaactctggaccaagtaaattgtgaactcaaaaagttaggagggataccaattacattaacaacgctttctttaaaaaatagaatcactttcttttgaatcaaccacagtggtgagacgtgtttttcttttcaggtgccccatgatggcatacagctttacccggcaaatcctgccagcttccaagtcccaggatactgacctgcaccagcacgtggggcagcattacctcccaacagtgtggagaagagcacatgtcaccactgggcaatgagagagttgacagagactcttggcttctcaacgccagacatggttggagagctttccttgttctattagaaaagttcatgaggaagctgtgaataggatcagtccagagaagtaaaactcttttattttcaccgtccaaacatcagtcaatatactgggagagccagcggaaaccctcgccgtaaccttgcctcttgagcacactgcacatgaacacttccatggggcgagcattcagctccttcagggtcacattcccctttcctgtggtctgtccataaagcccaaatatctcacggagtttttcttcactgattgcatctgttctgtcaattttgttacccaagataaggattggcacattggatattgtttcatcagtcattaaagcattaagctcaactttggattccacgaggcgagaatgatctgcacagtccaccagaaagacaatcccattaattgctgggagataatttttccaaacgcgacgtgcttgctcgtgcccaccaagatcaaaagttgtaaaggtcattccagcaattgttagctcttctgatgtcggatgtagtgttggaacatgttggcccaatctgtcatctttgagcatgtgaagaagagtggttttgcctgcattatccaaacctaagaatacaagttttccagatttcttgtacagtcctaggaactggagcacactgctgaagccattgtagatccactcaaagatgaaagacattattaatgcttactacggcctgaggggctcctccggcaaaacagcggctggctcggaccctccctcagagcacactaaccagcagcacccgggaccgccagctactcgccggatgtac

SEQ ID NO: 12256 - RNA, 159 nt, Homo sapiens
  source 1..159: mol_type = other RNA
ctgggaggtcaaggctgcagtgagacttaatcacaccactgtattccagcctgggagacagagcaagacctattgggttgtgtccgcaccagccaggagcattccctgacacagaagagggagatgatctgaaagtctacaggcagcggcagcagcagt

SEQ ID NO: 12257 - RNA, 910 nt, Homo sapiens
  source 1..910: mol_type = other RNA
ctgggaggtcaaggctgcagtgagatgtgatcatgccaccgaattccagcctgggtgacacagcaagacccaataaaatgccgtgatgacgctgtcacccattccggattcacgaatcattcttcaaaagtccggctccaaaactatgtggagactgaaatcccccaggaagacctccgctccctcagacgcggggcgggccctgcgacttcactctgggagggacatttccgctcacccagctctgcgaccctcgctcctgcggagtcagcttctgctcgcggagggggaagggcaaaaggacagtgcgtcccaacccgtccctctccagctgagcctgtcagagaccagcccagctctgaaatcaagccgttgagaaaagggaattcggccctccgccgcctcttcagtttaaaatcgtttcccgactcgctctgcggccccacgcaggaagcctccttggcgcctcgccgattccgtatcagtgaagcaactaaaattgccattttaactgagggcaaggccgagccacttaaccactatcgtcaacctttccaatcgtgctcggttgctcctcagttttcctaccggtgcgaagctttctctcaaatttccgcccgtagtaggcatggcggcggcacctcaccactgattcgttgaattccttcccggtaatcttgggcactagcgggcggagttgaagggcgcttggaccccagcggcgatctgtgtttgggttcgcgctctgggagaattttggctttgctcgccttcctctttcagaagactcgaaatcggccagcaggtctgcgagatttgaaacgcgactgttactccttgttttccggttctggccgcgggagcctctcgagaagcgtggaaagaggagaagggcgtataccttgtgacc

SEQ ID NO: 12258 - RNA, 838 nt, Homo sapiens
  source 1..838: mol_type = other RNA
ctgggaggtcaaggctgcagtgagatgtgatcatgccaccgaattccagcctgggtgacacagcaagaccctcaataaaatgccgtgatgacgctgtcacccattccggattcacgaatcattcttcaaaagtccggctccaaaactatgtggagactgaaatcccccagctctgcgaccctcgctcctgcggagtcagcttctgctcgcggagggggaagggcaaaaggacagtgcgtcccaacccgtccctctccagctgagcctgtcagagaccagcccagctctgaaatcaagccgttgagaaaagggaattcggccctccgccgcctcttcagtttaaaatcgtttcccgactcgctctgcggccccacgcaggaagcctccttggcgcctcgccgattccgtatcagtgaagcaactaaaattgccattttaactgagggcaaggccgagccacttaaccactatcgtcaacctttccaatcgtgctcggttgctcctcagttttcctaccggtgcgaagctttctctcaaatttccgcccgtagtaggcatggcggcggcacctcaccactgattcgttgaattccttcccggtaatcttgggcactagcgggcggagttgaagggcgcttggaccccagcggcgatctgtgtttgggttcgcgctctgggagaattttggctttgctcgccttcctctttcagaagactcgaaatcggccagcaggtctgcgagatttgaaacgcgactgttactccttgttttccggttctggccgcgggagcctctcgagaagcgtggaaagaggagaagggcgtataccttgtgacc

SEQ ID NO: 12259 - RNA, 912 nt, Homo sapiens
  source 1..912: mol_type = other RNA
ctgggaggtcaaggctgcagtgagatgtgatcatgccaccgaattccagcctgggtgacacagcaagaccctcaataaaatgccgtgatgacgctgtcacccattccggattcacgaatcattcttcaaaagtccggctccaaaactatgtggagactgaaatcccccaggaagacctccgctccctcagacgcggggcgggccctgcgacttcactctgggagggacatttccgctcacccagctctgcgaccctcgctcctgcggagtcagcttctgctcgcggagggggaagggcaaaaggacagtgcgtcccaacccgtccctctccagctgagcctgtcagagaccagcccagctctgaaatcaagccgttgagaaaagggaattcggccctccgccgcctcttcagtttaaaatcgtttcccgactcgctctgcggccccacgcaggaagcctccttggcgcctcgccgattccgtatcagtgaagcaactaaaattgccattttaactgagggcaaggccgagccacttaaccactatcgtcaacctttccaatcgtgctcggttgctcctcagttttcctaccggtgcgaagctttctctcaaatttccgcccgtagtaggcatggcggcggcacctcaccactgattcgttgaattccttcccggtaatcttgggcactagcgggcggagttgaagggcgcttggaccccagcggcgatctgtgtttgggttcgcgctctgggagaattttggctttgctcgccttcctctttcagaagactcgaaatcggccagcaggtctgcgagatttgaaacgcgactgttactccttgttttccggttctggccgcgggagcctctcgagaagcgtggaaagaggagaagggcgtataccttgtgacc

SEQ ID NO: 12260 - RNA, 1149 nt, Homo sapiens
  source 1..1149: mol_type = other RNA
ctgggaggtcaaggctgcagtgagccaaaaaaaagaccaatgaattcaagtgtctaccccctaacccaaacagaagcagaccctaaatctttcagggtgtcatcctaagctaagtagaaatctaaaagtttcctagagcacagataagagtgacctagcactccagccaaccagaaagggaaaagcagaacataagcttactttctacaaaggaagcagctatacaaattatgccagagaactagaaaaacactaatttgagtatccaaaaggggggaagtagttccaaatatttctaataaagagcattctgtaagccttccaacaagctattaaaggttgagaaaacctatctggcaacccagttaatttcaggacacataattacaggaacttagtccctcaagtcagagatgcctgtgaggaattgcacggtttgaatcacagcagatttgcagcctatttaagtttttggaccactagaaaactggaaaaacaattcatttaatatagttgagagaatacttaaaaatcctacatcaattcaattatatactgacttagaattatatgattacttcctatggagggttaattccctggcatttaggttgagcccctacatataccttcaattatcaaaaaaaaaatcaaaactttatttgaactcaaagttttacttatgagaataatgaaatcttacttagattaacactcaaaacatttcttggggataggctttttaaaatgaaacccataatttatttttgttacaaaaggaaatgtttacgtccctgttaaagtataaaaagggtctcattagtgtatctgaagagtactacattgtacattgtcttccagaggtggaaaaaaaaagaagttaacttttacatatacttgaaagggaaagtctgcattctgcactaagttttcttgaatggaataagtttaaattgtcctcagttctagcaaagaatgttcttaaatatctgtctttaaaaatccaatagtagggccgggtgaggtggctcacgtctgtaatcccagcattttgggaggcagatggatcatctgaggtcaggagttcgaaaacagcccggccaacatggtgaaaacagcatggccaacatggtgaaaccctgtctccgt

SEQ ID NO: 12261 - RNA, 2906 nt, Homo sapiens
  source 1..2906: mol_type = other RNA
ctgggaggtcaaggctgcagtgagccaagatagtgccattgcactccagccagggtgacagagtgagaccttgactcaaaaaaaaaaaaaaacaaaaacaaaaaaaaaaccccaatggatcaaaaatgtgagaaaatgggcacaattagttttcgacaaatccagttttccagtttcatatttcacagaatgttgccaggagtcctttagctggcagactctccccgtgcattccaaaagcattcaggttcccagaacaggtttctatacacttttcaggaacacatctgctgtgaaaaatacaatgtttgtagcactgggactccaaacaaagcctgaaggggaagatgcacttaaaaatatttattaaagaggccgggcgcagtggctcacgcctgtaatcctagcactttgggaggccgaggcgggcggatcacttgaggtcaggagttcgagactagcctggccaacatggtgaaactccgtctctactgaaaacacaaaaaaattgtctgggcttggtggcgcatgcctgtaatcccagctacttgggaggctgaggcaggagaatcgtttgaacccaggaggcagaggttgcagtgacctgagatcgtgccactgcaccactccagcctgggggacaagagcgaaactccatctggaaaaaaaaaacaaagaaaaagtttattaaagatagaaaattcttccacatgaggaaaagatggccagagccactgtacaattaggttctgacttaaagattagagattgaaacaaacagaaaaaaatgcaaccgcttgcatttcttgctaaaagtaaaccaaaagcagtttaatttgaaggatgtgctatggtagcggtgattaggttttaggtcaaataaccaatgggcccaactcaatgtgagacagggggagcctcattaagaagagtggctgagaaggaggcagcatgaccagtacaaattattgcccttggagaatggagatgtcgctttcctgttcattgaagattttaattagaaatgtattcttctttatagatgtttccattagttgtattctaattatagaccttgacaaaaaaagcaaaaagaagacccagcagagccaagcccacggacatcctcagcgcacagtcttgatgtagccttggcatgggcagcaccattctggaactcgctgagtcacactgagatgcagcagaggtgtgggatcctgaactcagctggttcccaagcccatttctgaagtcctttgtcaaacccgagacttctccctttgctagcggtttgctgatggagggcgtgtacactttggcatcagatactggctgccctttcataaaatgtttgcctgattcatagatgtccacttcaaccatcttccccatgaacgcagggttctttggcactaaaacctgctcatagaattgattgtgtgcaacataaaacttggaatcaaaagattcttctgttactaacacttgttgtctttcaccaatcacttgtgctggaacttgttccatttttgcagcaggagttcctggtcttgggtaaaattggttaataaacaggcttgggaatttgtactcttcaacaagtttcactgtttcttgaaaatcctgatctgtttctccaggaaaaccacagataatatctgtagcaatagttattccaggaactttctctttcagaaaatccactactcttttgaagtcagccacacagtattctcttttcatttccatgagtacgctgtcggaggcagactggactggtatgtgcagaaaagcgtagactctggggtgattaaggatttttgccatttcctccagatgctctaaaatatagggcggatttgtcatgccaagcctcagcattgctccctcaggaatcacttcaaccagtttccacaggagtgtggggagattggtgccaatatctctgccataagcccccgtgtcttcactggtcaaccatatctcacaaacaccctcttgaaaagattgtttggctctatctactagttcatcaattggataactggccaaatttcctctggcgtgtttagttttgcagtaggtacaagcattgagacacccggtattgatggaaatgatttctatcagtggattcttcctaatcttcggcaaatccaatcgtgctcccccaagccgccttccattatcctttttctgacccagcagtctcacagagtgacctttaattgtctcctccacaacttctaccacacgatctatctgctgaaccccaatgatactcagtcccttaaggtagtcctggcgaggctgggcttgaggaacgcatccagccagtacgattttcttgttctcctcttgagcttttttaattgagtttctaaagtggtcttcagctgggttttttacagtgcaactgttcaggagccataaatctgcatcggatgcattttctgtaattttatagccataagcagctagctgtccagccatatattctccatctgaattattatgagaacaaccccatgttcgtatccaaattttctgtatgcctggaatagtgctgtcacttggtggactgttttcttcctcttgcaaatatttttgggtatttcgccttcgtaccttcgggacaacatcctttcttacaaaatgcctatcttgtggttttgaatcttcctgagacacgatatcttcgatgtcatccagtagtgtatcacaggatgcagaaggcatattctcttaattatctgcaattagtctaaagtcctcttgaaagatgagtccagaagtcgggaagtaaaaaccagtccaaagtgagaaaatcaacccgccactctccggaagctgcacagactttagatggagagcgccatgacacatacgtcccgccacgtttattt

SEQ ID NO: 12262 - RNA, 2739 nt, Homo sapiens
  source 1..2739: mol_type = other RNA
ctgggaggtcaaggctgcagtgagccaagatagtgccattgcactccagccagggtgacagagtgagaccttgactcaaaaaaaaaaaaaaacaaaaacaaaaaaaaaaccccaatggatcaaaaatgtgagaaaatgggcacaattagttttcgacaaatccagttttccagtttcatatttcacagaatgttgccaggagtcctttagctggcagactctccccgtgcattccaaaagcattcaggttcccagaacaggtttctatacacttttcaggaacacatctgctgtgaaaaatacaatgtttgtagcactgggactccaaacaaagcctgaaggggaagatgcacttaaaaatatttattaaagaggccgggcgcagtggctcacgcctgtaatcctagcactttgggaggccgaggcgggcggatcacttgaggtcaggagttcgagactagcctggccaacatggtgaaactccgtctctactgaaaacacaaaaaaattgtctgggcttggtggcgcatgcctgtaatcccagctacttgggaggctgaggcaggagaatcgtttgaacccaggaggcagaggttgcagtgacctgagatcgtgccactgcaccactccagcctgggggacaagagcgaaactccatctggaaaaaaaaaacaaagaaaaagtttattaaagatagaaaattcttccacatgaggaaaagatggccagagccactgtacaattaggttctgacttaaagattagagattgaaacaaacagaaaaaaatgcaaccgcttgcatttcttgctaaaagtaaaccaaaagcagtttaatttgaaggatgtgctatggtagcggtgattaggttttaggtcaaataaccaatgggcccaactcaatgtgagacagggggagcctcattaagaagagtggctgagaaggaggcagcatgaccagtacaaattattgcccttggagaatggagatgtcgctttcctgttcattgaagattttaattagaaatgtattcttctttatagatgtttccattagttgtattctaattatagaccttgacaaaaaaagcaaaaagaagacccagcagagccaagcccacggacatcctcagcgcacagtcttgatgtagccttggcatgggcagcaccattctggaactcgctgagtcacactgagatgcagcagaggtgtgggatcctgaactcagctggttcccaagcccatttctgaagtcctttgtcaaacccgagacttctccctttgctagcggtttgctgatggagggcgtgtacactttggcatcagatactggctgccctttcataaaatgtttgcctgattcatagatgtccacttcaaccatcttccccatgaacgcagggttctttggcactaaaacctgctcatagaattgattgtgtgcaacataaaacttggaatcaaaagattcttctgttactaacacttgttgtctttcaccaatcacttgtgctggaacttgttccatttttgcagcaggagttcctggtcttgggtaaaattggttaataaacaggcttgggaatttgtactcttcaacaagtttcactgtttcttgaaaatcctgatctgtttctccaggaaaaccacagataatatctgtagcaatagttattccaggaactttctctttcagaaaatccactactcttttgaagtcagccacacagtattctcttttcatttccatgagtacgctgtcggaggcagactggactggtatgtgcagaaaagcgtagactctggggtgattaaggatttttgccatttccttgaaaagattgtttggctctatctactagttcatcaattggataactggccaaatttcctctggcgtgtttagttttgcagtaggtacaagcattgagacacccggtattgatggaaatgatttctatcagtggattcttcctaatcttcggcaaatccaatcgtgctcccccaagccgccttccattatcctttttctgacccagcagtctcacagagtgacctttaattgtctcctccacaacttctaccacacgatctatctgctgaaccccaatgatactcagtcccttaaggtagtcctggcgaggctgggcttgaggaacgcatccagccagtacgattttcttgttctcctcttgagcttttttaattgagtttctaaagtggtcttcagctgggttttttacagtgcaactgttcaggagccataaatctgcatcggatgcattttctgtaattttatagccataagcagctagctgtccagccatatattctccatctgaattattatgagaacaaccccatgttcgtatccaaattttctgtatgcctggaatagtgctgtcacttggtggactgttttcttcctcttgcaaatatttttgggtatttcgccttcgtaccttcgggacaacatcctttcttacaaaatgcctatcttgtggttttgaatcttcctgagacacgatatcttcgatgtcatccagtagtgtatcacaggatgcagaaggcatattctcttaattatctgcaattagtctaaagtcctcttgaaagatgagtccagaagtcgggaagtaaaaaccagtccaaagtgagaaaatcaacccgccactctccggaagctgcacagactttagatggagagcgccatgacacatacgtcccgccacgtttattt

SEQ ID NO: 12263 - RNA, 2862 nt, Homo sapiens
  source 1..2862: mol_type = other RNA
ctgggaggtcaaggctgcagtgagccaagatagtgccattgcactccagccagggtgacagagtgagaccttgactcaaaaaaaaaaaaaaacaaaaacaaaaaaaaaaccccaatggatcaaaaatgtgagaaaatgggcacaattagttttcgacaaatccagttttccagtttcatatttcacagaatgttgccaggagtcctttagctggcagactctccccgtgcattccaaaagcattcaggttcccagaacaggtttctatacacttttcaggaacacatctgctgtgaaaaatacaatgtttgtagcactgggactccaaacaaagcctgaaggggaagatgcacttaaaaatatttattaaagaggccgggcgcagtggctcacgcctgtaatcctagcactttgggaggccgaggcgggcggatcacttgaggtcaggagttcgagactagcctggccaacatggtgaaactccgtctctactgaaaacacaaaaaaattgtctgggcttggtggcgcatgcctgtaatcccagctacttgggaggctgaggcaggagaatcgtttgaacccaggaggcagaggttgcagtgacctgagatcgtgccactgcaccactccagcctgggggacaagagcgaaactccatctggaaaaaaaaaacaaagaaaaagtttattaaagatagaaaattcttccacatgaggaaaagatggccagagccactgtacaattaggttctgacttaaagattagagattgaaacaaacagaaaaaaatgcaaccgcttgcatttcttgctaaaagtaaaccaaaagcagtttaatttgaaggatgtgctatggtagcggtgattaggttttaggtcaaataaccaatgggcccaactcaatgtgagacagggggagcctcattaagaagagtggctgagaaggaggcagcatgaccagtacaaattattgcccttggagaatggagatgtcgctttcctgttcattgaagattttaattagaaatgtattcttctttatagatgtttccattagttgtattctaattatagaccttgacaaaaaaagcaaaaagaagacccagcagagccaagcccacggacatcctcagcgcacagtcttgatgtagccttggcatgggcagcaccattctggaactcgctgagtcacactgagatgcagcagaggtgtgggatcctgaactcagctggttcccaagcccatttctgaagtcctttgtcaaacccgagacttctccctttgctagcggtttgctgatggagggcgtgtacactttggcatcagatactggctgccctttcataaaatgtttgcctgattcatagatgtccacttcaaccatcttccccatgaacgcagggttctttggcactaaaacctgctcatagaattgattgtgtgcaacataaaacttggaatcaaaagattcttctgttactaacacttgttgtctttcaccaatcttgtgatcatatggactgtaagaatgaaacacccgagaaagatcttttgtcctttgctttttcacttgtgctggaacttgttccatttttgcagcaggagttcctggtcttgggtaaaattggttaataaacaggcttgggaatttgtactcttcaacaagtttcactgtttcttgaaaatcctgatctgtttctccaggaaaaccacagataatatctgtagcaatagttattccaggaactttctctttcagaaaatccactactcttttgaagtcagccacacagtattctcttttcatttccatgagtacgctgtcggaggcagactggactggtatgtgcagaaaagcgtagactctggggtgattaaggatttttgccatttcctccagatgctctaaaatatagggcggatttgtcatgccaagcctcagcattgctccctcaggaatcacttcaaccagtttccacaggagtgtggggagattggtgccaatatctctgccataagcccccgtgtcttcactggtcaaccatatctcacaaacaccctccggtattgatggaaatgatttctatcagtggattcttcctaatcttcggcaaatccaatcgtgctcccccaagccgccttccattatcctttttctgacccagcagtctcacagagtgacctttaattgtctcctccacaacttctaccacacgatctatctgctgaaccccaatgatactcagtcccttaaggtagtcctggcgaggctgggcttgaggaacgcatccagccagtacgattttcttgttctcctcttgagcttttttaattgagtttctaaagtggtcttcagctgggttttttacagtgcaactgttcaggagccataaatctgcatcggatgcattttctgtaattttatagccataagcagctagctgtccagccatatattctccatctgaattattatgagaacaaccccatgttcgtatccaaattttctgtatgcctggaatagtgctgtcacttggtggactgttttcttcctcttgcaaatatttttgggtatttcgccttcgtaccttcgggacaacatcctttcttacaaaatgcctatcttgtggttttgaatcttcctgagacacgatatcttcgatgtcatccagtagtgtatcacaggatgcagaaggcatattctcttaattatctgcaattagtctaaagtcctcttgaaagatgagtccagaagtcgggaagtaaaaaccagtccaaagtgagaaaatcaacccgccactctccggaagctgcacagactttagatggagagcgccatgacacatacgtcccgccacgttta

SEQ ID NO: 12264 - RNA, 2969 nt, Homo sapiens
  source 1..2969: mol_type = other RNA
ctgggaggtcaaggctgcagtgagccaagatagtgccattgcactccagccagggtgacagagtgagaccttgactcaaaaaaaaaaaaaaacaaaaacaaaaaaaaaaccccaatggatcaaaaatgtgagaaaatgggcacaattagttttcgacaaatccagttttccagtttcatatttcacagaatgttgccaggagtcctttagctggcagactctccccgtgcattccaaaagcattcaggttcccagaacaggtttctatacacttttcaggaacacatctgctgtgaaaaatacaatgtttgtagcactgggactccaaacaaagcctgaaggggaagatgcacttaaaaatatttattaaagaggccgggcgcagtggctcacgcctgtaatcctagcactttgggaggccgaggcgggcggatcacttgaggtcaggagttcgagactagcctggccaacatggtgaaactccgtctctactgaaaacacaaaaaaattgtctgggcttggtggcgcatgcctgtaatcccagctacttgggaggctgaggcaggagaatcgtttgaacccaggaggcagaggttgcagtgacctgagatcgtgccactgcaccactccagcctgggggacaagagcgaaactccatctggaaaaaaaaaacaaagaaaaagtttattaaagatagaaaattcttccacatgaggaaaagatggccagagccactgtacaattaggttctgacttaaagattagagattgaaacaaacagaaaaaaatgcaaccgcttgcatttcttgctaaaagtaaaccaaaagcagtttaatttgaaggatgtgctatggtagcggtgattaggttttaggtcaaataaccaatgggcccaactcaatgtgagacagggggagcctcattaagaagagtggctgagaaggaggcagcatgaccagtacaaattattgcccttggagaatggagatgtcgctttcctgttcattgaagattttaattagaaatgtattcttctttatagatgtttccattagttgtattctaattatagaccttgacaaaaaaagcaaaaagaagacccagcagagccaagcccacggacatcctcagcgcacagtcttgatgtagccttggcatgggcagcaccattctggaactcgctgagtcacactgagatgcagcagaggtgtgggatcctgaactcagctggttcccaagcccatttctgaagtcctttgtcaaacccgagacttctccctttgctagcggtttgctgatggagggcgtgtacactttggcatcagatactggctgccctttcataaaatgtttgcctgattcatagatgtccacttcaaccatcttccccatgaacgcagggttctttggcactaaaacctgctcatagaattgattgtgtgcaacataaaacttggaatcaaaagattcttctgttactaacacttgttgtctttcaccaatcttgtgatcatatggactgtaagaatgaaacacccgagaaagatcttttgtcctttgctttttcacttgtgctggaacttgttccatttttgcagcaggagttcctggtcttgggtaaaattggttaataaacaggcttgggaatttgtactcttcaacaagtttcactgtttcttgaaaatcctgatctgtttctccaggaaaaccacagataatatctgtagcaatagttattccaggaactttctctttcagaaaatccactactcttttgaagtcagccacacagtattctcttttcatttccatgagtacgctgtcggaggcagactggactggtatgtgcagaaaagcgtagactctggggtgattaaggatttttgccatttcctccagatgctctaaaatatagggcggatttgtcatgccaagcctcagcattgctccctcaggaatcacttcaaccagtttccacaggagtgtggggagattggtgccaatatctctgccataagcccccgtgtcttcactggtcaaccatatctcacaaacaccctcttgaaaagattgtttggctctatctactagttcatcaattggataactggccaaatttcctctggcgtgtttagttttgcagtaggtacaagcattgagacacccggtattgatggaaatgatttctatcagtggattcttcctaatcttcggcaaatccaatcgtgctcccccaagccgccttccattatcctttttctgacccagcagtctcacagagtgacctttaattgtctcctccacaacttctaccacacgatctatctgctgaaccccaatgatactcagtcccttaaggtagtcctggcgaggctgggcttgaggaacgcatccagccagtacgattttcttgttctcctcttgagcttttttaattgagtttctaaagtggtcttcagctgggttttttacagtgcaactgttcaggagccataaatctgcatcggatgcattttctgtaattttatagccataagcagctagctgtccagccatatattctccatctgaattattatgagaacaaccccatgttcgtatccaaattttctgtatgcctggaatagtgctgtcacttggtggactgttttcttcctcttgcaaatatttttgggtatttcgccttcgtaccttcgggacaacatcctttcttacaaaatgcctatcttgtggttttgaatcttcctgagacacgatatcttcgatgtcatccagtagtgtatcacaggatgcagaaggcatattctcttaattatctgcaattagtctaaagtcctcttgaaagatgagtccagaagtcgggaagtaaaaaccagtccaaagtgagaaaatcaacccgccactctccggaagctgcacagactttagatggagagcgccatgacacatacgtcccgccacgtttattt

SEQ ID NO: 12265 - RNA, 2802 nt, Homo sapiens
  source 1..2802: mol_type = other RNA
ctgggaggtcaaggctgcagtgagccaagatagtgccattgcactccagccagggtgacagagtgagaccttgactcaaaaaaaaaaaaaaacaaaaacaaaaaaaaaaccccaatggatcaaaaatgtgagaaaatgggcacaattagttttcgacaaatccagttttccagtttcatatttcacagaatgttgccaggagtcctttagctggcagactctccccgtgcattccaaaagcattcaggttcccagaacaggtttctatacacttttcaggaacacatctgctgtgaaaaatacaatgtttgtagcactgggactccaaacaaagcctgaaggggaagatgcacttaaaaatatttattaaagaggccgggcgcagtggctcacgcctgtaatcctagcactttgggaggccgaggcgggcggatcacttgaggtcaggagttcgagactagcctggccaacatggtgaaactccgtctctactgaaaacacaaaaaaattgtctgggcttggtggcgcatgcctgtaatcccagctacttgggaggctgaggcaggagaatcgtttgaacccaggaggcagaggttgcagtgacctgagatcgtgccactgcaccactccagcctgggggacaagagcgaaactccatctggaaaaaaaaaacaaagaaaaagtttattaaagatagaaaattcttccacatgaggaaaagatggccagagccactgtacaattaggttctgacttaaagattagagattgaaacaaacagaaaaaaatgcaaccgcttgcatttcttgctaaaagtaaaccaaaagcagtttaatttgaaggatgtgctatggtagcggtgattaggttttaggtcaaataaccaatgggcccaactcaatgtgagacagggggagcctcattaagaagagtggctgagaaggaggcagcatgaccagtacaaattattgcccttggagaatggagatgtcgctttcctgttcattgaagattttaattagaaatgtattcttctttatagatgtttccattagttgtattctaattatagaccttgacaaaaaaagcaaaaagaagacccagcagagccaagcccacggacatcctcagcgcacagtcttgatgtagccttggcatgggcagcaccattctggaactcgctgagtcacactgagatgcagcagaggtgtgggatcctgaactcagctggttcccaagcccatttctgaagtcctttgtcaaacccgagacttctccctttgctagcggtttgctgatggagggcgtgtacactttggcatcagatactggctgccctttcataaaatgtttgcctgattcatagatgtccacttcaaccatcttccccatgaacgcagggttctttggcactaaaacctgctcatagaattgattgtgtgcaacataaaacttggaatcaaaagattcttctgttactaacacttgttgtctttcaccaatcttgtgatcatatggactgtaagaatgaaacacccgagaaagatcttttgtcctttgctttttcacttgtgctggaacttgttccatttttgcagcaggagttcctggtcttgggtaaaattggttaataaacaggcttgggaatttgtactcttcaacaagtttcactgtttcttgaaaatcctgatctgtttctccaggaaaaccacagataatatctgtagcaatagttattccaggaactttctctttcagaaaatccactactcttttgaagtcagccacacagtattctcttttcatttccatgagtacgctgtcggaggcagactggactggtatgtgcagaaaagcgtagactctggggtgattaaggatttttgccatttccttgaaaagattgtttggctctatctactagttcatcaattggataactggccaaatttcctctggcgtgtttagttttgcagtaggtacaagcattgagacacccggtattgatggaaatgatttctatcagtggattcttcctaatcttcggcaaatccaatcgtgctcccccaagccgccttccattatcctttttctgacccagcagtctcacagagtgacctttaattgtctcctccacaacttctaccacacgatctatctgctgaaccccaatgatactcagtcccttaaggtagtcctggcgaggctgggcttgaggaacgcatccagccagtacgattttcttgttctcctcttgagcttttttaattgagtttctaaagtggtcttcagctgggttttttacagtgcaactgttcaggagccataaatctgcatcggatgcattttctgtaattttatagccataagcagctagctgtccagccatatattctccatctgaattattatgagaacaaccccatgttcgtatccaaattttctgtatgcctggaatagtgctgtcacttggtggactgttttcttcctcttgcaaatatttttgggtatttcgccttcgtaccttcgggacaacatcctttcttacaaaatgcctatcttgtggttttgaatcttcctgagacacgatatcttcgatgtcatccagtagtgtatcacaggatgcagaaggcatattctcttaattatctgcaattagtctaaagtcctcttgaaagatgagtccagaagtcgggaagtaaaaaccagtccaaagtgagaaaatcaacccgccactctccggaagctgcacagactttagatggagagcgccatgacacatacgtcccgccacgtttattt

SEQ ID NO: 12266 - RNA, 3730 nt, Homo sapiens
  source 1..3730: mol_type = other RNA
ctgggaggtcaaggctgcagtgagccaagatcacaccatgccctccagcctgagcaatataatgagactctaacacacacacgtgcacacacacacacacacacacacaaataagactttatatgagtggtcattggttatgatgttcttattctttataagagaaaatctgtgtatactgttacagctgaatggcatttggtatatggcatgccagtcttccacatgtactgatgtttaagaaaggcttggatccagtgtgtattctggatgtcgggggaaaaaaaggcttggaaaccaggttatcctattatttaaaatattaaaaattacattattttagaaacagagaaccaaatacaagctgatactaccataaaattaccataaaatagttttgctcttttttcactgtttacacctttcctccctatattaagttgttaagtacttgagaaacgtacttaacactgaacttcccaatatatttgggaaggtatgatatgaatgttaagtataaaataatacgggtagttaatgttaaaagaactcagaggaaatttccccgcagggtaactacaaagatgttttctatgctgcatttgtcccgagatgtttatgtaactcattcctctatctcaatcattacatacccctcattacaaacactcctatgtgctctctgagctcatctgaagagaacagaattgagtcgatgatttgagttatgattttctccattctcctagggactgtacataattagtaccattctagatgacacagggacttagggctttttctcctgcaaacctaattgagaaagcctgtgatagacactagcacacctccttctctttccccctactcccagactgctctggcctcaaacccatcctatctatttcaccaatggccaacactgtcctgtctgcacccagagtgagaagctcccacagggaaaagttattttaaaatatccaactttatatatttaaagcctcatatttcctcataagctactatttttctctcccattcctacctttgtcaagctcagcatataacaagtcatctttttgtgacatcaaagtcttcaaagtctttctggagatctagaatctacaatttctaaatattttgcataacgcataaagtgcatataaattgagttatcctatatctgtgaactgatgagaattattctgctcaaacaggtggtgaaaacctttgcttgactctcctaaaaggataaacaaatactaaagaaagatggctttcaactacagtgaggttcttgtgatatgtgctactggaaaaagtacatttttaccaagccatagcaaataattttaaaagaatatcattccacagtatatggatctttttcattatactgcaatgtaatttgaaactagattattttccttgctaacactgagaagcaacaatttgtttagattatctagtgatgacctttttcctcttaaaggtgacaatgattctaaaacaagaacatctgaaaacatttgaaaaaactatcccaacacttcaatacattggaacagtagtcatatcacactatactatagaccatgggttgataaattttttccataaacagacagacagtaaatatcaggctttgtgggctatagtttctgtggcagctactctgccacagaaaagcagccatagacaagtaaaagaatgatcttggttgtgtttcaacaaactttatttatgaacactaaatattcatgttaattttcaagtatcataaaagtctttaaaaaaaaacatttaaaattataaacacaattcctagctcacaggccataaaaagcaggcagcaggctggatttgatccacaggccatagttggctgtctcttaaacaggcttttatacgttatgcaaagtgtttcaaattccagagactttggagacttttcgttttttagatttctcattttaaaacacacataatacaagttttctttctggatcaatatactcacgagagaaaataattcagaaaaaaataaaattccttacttaaaaaaagggaaaagctatagaacaaatgtttcgtcttaaaatatatttaggaaatgtaaaattaaagattaaaaattttattctatgcaacataaaataatatgcataaatctggcacataatttctttgtttttactttagaaaaaagacagtaagaaaaaagtttataaatttctcagtcccttttatacaaagttgcaactaaaaccagcaatcacttatatgtacaaccatcaactctgaatacaatgtgaattatacctaggaactgtaatttacctagatgagttctgcctgctttatgaaaaacacacacttatatcacagaacaccgtggcttctacaatttgtaacaattttgaaaacgaaactcctgcctccataatataaggaaacaagagtactctttccatagtcatcatcctgtataaaaaaaacttcatagtctgatttacctttgtcaaaggtaaaatgattcacatttgcttggattactctgatcctcagtagttcctaaacacaaaataaagtttgcatgaacctttatctgggttttccaaagcaagtattatgctggcagaagtccatgagctgaataaaaagatactaaatataaaaggtttaccaactttatcctttcttaattttacgatagcttcaggtattgagacctaactggtttcctgtgcctatccattgtgaacacatctcaatcttctacttttaacactcctcagcaccatattttcgttgtttctttattgtgcgacgtagaagatcctttcgtccaacttcaatcatttgttcttcccaagacttcatttcattatgataacgagtttcgtcctctttagcatgctgaatatataattccttttcagagtcagacagatttttccagttttcctttacagtcttcagcttttcctgcggtgaatcacccttagcttcttggaatctttcagctacataaacgttataagctgaacgaggtctttttggttttccaagcagtgttaactcttttttttttgtcatagctttcctttttaaatgtttgtccatgatttctttttccaaagacataatctgacttggagttagctgttctttaaatctgcttatctcttctttatatacctgccactccgccctataagcatcttgatatatttttttctttgaatcaggaagttccctccaacgctgggcaattcttctaattagttctgtagtttttgcatagtttatggatgcttccacagaagttgcaactttattaacaattccctgagccagaaaaaggaggagctgggttctgagctttaaatatgggtagttgttctttagaaaatcgaaggtaagaacttacaggtttctttggacaacttgccaagacagatgaaaaccacctcggtaaatacacaaaactgaagggggagcgcagtcgacttccacagccggtgcacagctctgctccagaccttcccagggcactcagcacgccccacatgcttcggagaaacgccatcgctccggtggatgaggcagtgacccgaccccaatctcggagagcctcctggcaatacacaactccagcaatcacaactggaacccgcgtgcgaccctccggcgtgtgttatcatgcccgccactagcgaggcactat

SEQ ID NO: 12267 - RNA, 3663 nt, Homo sapiens
  source 1..3663: mol_type = other RNA
ctgggaggtcaaggctgcagtgagccaagatcacaccatgccctccagcctgagcaatataatgagactctaacacacacacgtgcacacacacacacacacacacacaaataagactttatatgagtggtcattggttatgatgttcttattctttataagagaaaatctgtgtatactgttacagctgaatggcatttggtatatggcatgccagtcttccacatgtactgatgtttaagaaaggcttggatccagtgtgtattctggatgtcgggggaaaaaaaggcttggaaaccaggttatcctattatttaaaatattaaaaattacattattttagaaacagagaaccaaatacaagctgatactaccataaaattaccataaaatagttttgctcttttttcactgtttacacctttcctccctatattaagttgttaagtacttgagaaacgtacttaacactgaacttcccaatatatttgggaaggtatgatatgaatgttaagtataaaataatacgggtagttaatgttaaaagaactcagaggaaatttccccgcagggtaactacaaagatgttttctatgctgcatttgtcccgagatgtttatgtaactcattcctctatctcaatcattacatacccctcattacaaacactcctatgtgctctctgagctcatctgaagagaacagaattgagtcgatgatttgagttatgattttctccattctcctagggactgtacataattagtaccattctagatgacacagggacttagggctttttctcctgcaaacctaattgagaaagcctgtgatagacactagcacacctccttctctttccccctactcccagactgctctggcctcaaacccatcctatctatttcaccaatggccaacactgtcctgtctgcacccagagtgagaagctcccacagggaaaagttattttaaaatatccaactttatatatttaaagcctcatatttcctcataagctactatttttctctcccattcctacctttgtcaagctcagcatataacaagtcatctttttgtgacatcaaagtcttcaaagtctttctggagatctagaatctacaatttctaaatattttgcataacgcataaagtgcatataaattgagttatcctatatctgtgaactgatgagaattattctgctcaaacaggtggtgaaaacctttgcttgactctcctaaaaggataaacaaatactaaagaaagatggctttcaactacagtgaggttcttgtgatatgtgctactggaaaaagtacatttttaccaagccatagcaaataattttaaaagaatatcattccacagtatatggatctttttcattatactgcaatgtaatttgaaactagattattttccttgctaacactgagaagcaacaatttgtttagattatctagtgatgacctttttcctcttaaaggtgacaatgattctaaaacaagaacatctgaaaacatttgaaaaaactatcccaacacttcaatacattggaacagtagtcatatcacactatactatagaccatgggttgataaattttttccataaacagacagacagtaaatatcaggctttgtgggctatagtttctgtggcagctactctgccacagaaaagcagccatagacaagtaaaagaatgatcttggttgtgtttcaacaaactttatttatgaacactaaatattcatgttaattttcaagtatcataaaagtctttaaaaaaaaacatttaaaattataaacacaattcctagctcacaggccataaaaagcaggcagcaggctggatttgatccacaggccatagttggctgtctcttaaacaggcttttatacgttatgcaaagtgtttcaaattccagagactttggagacttttcgttttttagatttctcattttaaaacacacataatacaagttttctttctggatcaatatactcacgagagaaaataattcagaaaaaaataaaattccttacttaaaaaaagggaaaagctatagaacaaatgtttcgtcttaaaatatatttaggaaatgtaaaattaaagattaaaaattttattctatgcaacataaaataatatgcataaatctggcacataatttctttgtttttactttagaaaaaagacagtaagaaaaaagtttataaatttctcagtcccttttatacaaagttgcaactaaaaccagcaatcacttatatgtacaaccatcaactctgaatacaatgtgaattatacctaggaactgtaatttacctagatgagttctgcctgctttatgaaaaacacacacttatatcacagaacaccgtggcttctacaatttgtaacaattttgaaaacgaaactcctgcctccataatataaggaaacaagagtactctttccatagtcatcatcctgtataaaaaaaacttcatagtctgatttacctttgtcaaaggtaaaatgattcacatttgcttggattactctgatcctcagtagttcctaaacacaaaataaagtttgcatgaacctttatctgggttttccaaagcaagtattatgctggcagaagtccatgagctgaataaaaagatactaaatataaaaggtttaccaactttatcctttcttaattttacgatagcttcaggtattgagacctaactggtttcctgtgcctatccattgtgaacacatctcaatcttctacttttaacactcctcagcaccatattttcgttgtttctttattgtgcgacgtagaagatcctttcgtccaacttcaatcatttgttcttcccaagacttcatttcattatgataacgagtttcgtcctctttagcatgctgaatatataattccttttcagagtcagacagatttttccagttttcctttacagtcttcagcttttcctgcggtgaatcacccttagcttcttggaatctttcagctacataaacgttataagctgaacgaggtctttttggttttccaagcagtgttaactcttttttttttgtcatagctttcctttttaaatgtttgtccatgatttctttttccaaagacataatctgacttggagttagctgttctttaaatctgcttatctcttctttatatacctgccactccgccctataagcatcttgatatatttttttctttgaatcaggaagttccctccaacgctgggcaattcttctaattagttctgtagtttttgcatctgggttctgagctttaaatatgggtagttgttctttagaaaatcgaaggtaagaacttacaggtttctttggacaacttgccaagacagatgaaaaccacctcggtaaatacacaaaactgaagggggagcgcagtcgacttccacagccggtgcacagctctgctccagaccttcccagggcactcagcacgccccacatgcttcggagaaacgccatcgctccggtggatgaggcagtgacccgaccccaatctcggagagcctcctggcaatacacaactccagcaatcacaactggaacccgcgtgcgaccctccggcgtgtgttatcatgcccgccactagcgaggcactat

SEQ ID NO: 12268 - RNA, 3567 nt, Homo sapiens
  source 1..3567: mol_type = other RNA
ctgggaggtcaaggctgcagtgagccaagatcacaccatgccctccagcctgagcaatataatgagactctaacacacacacgtgcacacacacacacacacacacacaaataagactttatatgagtggtcattggttatgatgttcttattctttataagagaaaatctgtgtatactgttacagctgaatggcatttggtatatggcatgccagtcttccacatgtactgatgtttaagaaaggcttggatccagtgtgtattctggatgtcgggggaaaaaaaggcttggaaaccaggttatcctattatttaaaatattaaaaattacattattttagaaacagagaaccaaatacaagctgatactaccataaaattaccataaaatagttttgctcttttttcactgtttacacctttcctccctatattaagttgttaagtacttgagaaacgtacttaacactgaacttcccaatatatttgggaaggtatgatatgaatgttaagtataaaataatacgggtagttaatgttaaaagaactcagaggaaatttccccgcagggtaactacaaagatgttttctatgctgcatttgtcccgagatgtttatgtaactcattcctctatctcaatcattacatacccctcattacaaacactcctatgtgctctctgagctcatctgaagagaacagaattgagtcgatgatttgagttatgattttctccattctcctagggactgtacataattagtaccattctagatgacacagggacttagggctttttctcctgcaaacctaattgagaaagcctgtgatagacactagcacacctccttctctttccccctactcccagactgctctggcctcaaacccatcctatctatttcaccaatggccaacactgtcctgtctgcacccagagtgagaagctcccacagggaaaagttattttaaaatatccaactttatatatttaaagcctcatatttcctcataagctactatttttctctcccattcctacctttgtcaagctcagcatataacaagtcatctttttgtgacatcaaagtcttcaaagtctttctggagatctagaatctacaatttctaaatattttgcataacgcataaagtgcatataaattgagttatcctatatctgtgaactgatgagaattattctgctcaaacaggtggtgaaaacctttgcttgactctcctaaaaggataaacaaatactaaagaaagatggctttcaactacagtgaggttcttgtgatatgtgctactggaaaaagtacatttttaccaagccatagcaaataattttaaaagaatatcattccacagtatatggatctttttcattatactgcaatgtaatttgaaactagattattttccttgctaacactgagaagcaacaatttgtttagattatctagtgatgacctttttcctcttaaaggtgacaatgattctaaaacaagaacatctgaaaacatttgaaaaaactatcccaacacttcaatacattggaacagtagtcatatcacactatactatagaccatgggttgataaattttttccataaacagacagacagtaaatatcaggctttgtgggctatagtttctgtggcagctactctgccacagaaaagcagccatagacaagtaaaagaatgatcttggttgtgtttcaacaaactttatttatgaacactaaatattcatgttaattttcaagtatcataaaagtctttaaaaaaaaacatttaaaattataaacacaattcctagctcacaggccataaaaagcaggcagcaggctggatttgatccacaggccatagttggctgtctcttaaacaggcttttatacgttatgcaaagtgtttcaaattccagagactttggagacttttcgttttttagatttctcattttaaaacacacataatacaagttttctttctggatcaatatactcacgagagaaaataattcagaaaaaaataaaattccttacttaaaaaaagggaaaagctatagaacaaatgtttcgtcttaaaatatatttaggaaatgtaaaattaaagattaaaaattttattctatgcaacataaaataatatgcataaatctggcacataatttctttgtttttactttagaaaaaagacagtaagaaaaaagtttataaatttctcagtcccttttatacaaagttgcaactaaaaccagcaatcacttatatgtacaaccatcaactctgaatacaatgtgaattatacctaggaactgtaatttacctagatgagttctgcctgctttatgaaaaacacacacttatatcacagaacaccgtggcttctacaatttgtaacaattttgaaaacgaaactcctgcctccataatataaggaaacaagagtactctttccatagtcatcatcctgtataaaaaaaacttcatagtctgatttacctttgtcaaaggtaaaatgattcacatttgcttggattactctgatcctcagtagttcctaaacacaaaataaagtttgcatgaacctttatctgggttttccaaagcaagtattatgctggcagaagtccatgagctgaataaaaagatactaaatataaaaggtttaccaactttatcctttcttaattttacgatagcttcaggtattgagacctaactggtttcctgtgcctatccattgtgaacacatctcaatcttctacttttaacactcctcagcaccatattttcgttgtttctttattgtgcgacgtagaagatcctttcgtccaacttcaatcatttgttcttcccaagacttcatttcattatgataacgagtttcgtcctctttagcatgctgaatatataattccttttcagagtcagacagatttttccagttttcctttacagtcttcagcttttcttttttttttgtcatagctttcctttttaaatgtttgtccatgatttctttttccaaagacataatctgacttggagttagctgttctttaaatctgcttatctcttctttatatacctgccactccgccctataagcatcttgatatatttttttctttgaatcaggaagttccctccaacgctgggcaattcttctaattagttctgtagtttttgcatctgggttctgagctttaaatatgggtagttgttctttagaaaatcgaaggtaagaacttacaggtttctttggacaacttgccaagacagatgaaaaccacctcggtaaatacacaaaactgaagggggagcgcagtcgacttccacagccggtgcacagctctgctccagaccttcccagggcactcagcacgccccacatgcttcggagaaacgccatcgctccggtggatgaggcagtgacccgaccccaatctcggagagcctcctggcaatacacaactccagcaatcacaactggaacccgcgtgcgaccctccggcgtgtgttatcatgcccgccactagcgaggcactat

SEQ ID NO: 12269 - RNA, 1145 nt, Homo sapiens
  source 1..1145: mol_type = other RNA
ctgggaggtcaaggctgcagtgagccaagatcataccactgcactccagcccccacaacaaagcaaaaccctgtctcaaaagacaaaaataaaaccttctaaaacagtgagcttgctaagcacagtggctcacgcctgtaatcccagcactctgagaggccaaggcaggcagatcacgaggtcaggagatcaagaccatcctggctaacacggtgaaaccccgtctctactaaaaataccaaaaaaaaaaaaaaaaaaattagctgggcatggtggcaggcgcctgtagtcccagctactcgggaggctgaggcaggagaacggcgtgaacccgggaggcggagcttgcagtgagccaagattgcaccactgcactccagcctgggtgacagagtgagattccatctcaaaacaaaaaactgtgagcttacaaaatgcaacagactgctaggcacacttaatgtaacgtggaagtatgttcactgaaatgatgaaaatttgaaacacgaccataaacctttgtgaaaaaccatagtatgccctttacttcatttgcttttagctatttcataaacaccacagagaaactggacacagtttgtgatgaaacttagaaaaatttctttttccataacataaacatgtcagtttttccctttagatccttcttccactcccgcttcactgtgctgaagagatattgagttcttccagatttttgcttagctgggtggtttccgaactcaacggactctccaggtaggtagttccagcacagggctttcctgtcactggatctatgacttttccaactttgaaaacgatctcagccagttcatgtttcacatgctttgctcgtggaacaggtaaagctctgagaagcacaatatccccaactgtgcactgctgaagggcatcgtgagcaaagtaggttttccgcttattaaaatactttaataaatagggatccagaacaagcctggtcactctcactttagcagtcttttgcatttttgtcccaatcaccttccccacaatccatctggcatggacggatgagcgaactacggacattacgtggctttggtcacctccgccaagactatgcagccacctgccccggggagcgccggtcgcagcgggat

SEQ ID NO: 12270 - RNA, 4589 nt, Homo sapiens
  source 1..4589: mol_type = other RNA
ctgggaggtcaaggctgcagtgagccacaatcacaccattgcactccagcctgtgcgacagagcaagaccttgtctcaaaaaaaaaaattgttttttaactaaaaacagatgaagctggaaggccagcctgtaatcccagcactttgggaggccaaaatgggtggatcacctgaggtcaggagttcgagaccagcctggcgggcacctgtaatcccagctactcgggaggctgaggcaggagaatcccttgaacctaggaggcggaggttacggtgatcacaccactgcactccagcctgggcgacagagcgagactctgtctcaaacaaaacaaacaaaccaaccaacaaaaaaaatggcagaacagctcaaatgctaagccaaagactgggggctttatcctgtaggcaagagggagttgttgaaagttttgagcaactgagtcccgtgaccacatttgcatttttggaaacattaccaagtcaggattaaaggctggagggcaattaggaggccttgcagtaggtcacatgtcttttcatgtggatttaatgaggaaggagtcagaatataacagttttattaatggtgttggattttacaaccaaataatcccttagctatattgttttattttctaacatgaaagagcttctaccgttaatcctctcttctgtctcctgaagccagggctccacaggccttcctctgggagacacacccaggtgtgccgccttcccctgccagatcctcaggcctttcttacccaactcacaacttccctttcacccttagtcccatacccaccatctcccgagaaaacctccgcaatgggctgccggggccccaggcccttccacccatcccgccagcacaccctccccgtgaaaatgagtgaccccaggccagcgtcttccctcaggagagaagcctgtctggatccccaaaggcctctccctccagggaagagggactctcactctggcctcagtggttactccagagcccaagaaatgccctgtgcgctaaaaccaaagaaggtgtgaaccagcaagtaagtggggagcggccagttctgggacatctagttgggggccttctcttccccatgagcagcagggaccagtgtgaccttggcatcaggctctttctcttggctggcttcctcaacgttcaagacgctcgataaacatatcccagaggcaaagcaagttaagtcgagggttgtttattcacctagaatcagctccagccattttccaatgtcttctttttgttgtttttctggtttttgttgcaacagggtctcactatgttccccaggctggtctcaaactcctggcctcaaatgagcctcctgcctcaaactcccaaagtgttgggtttacaggcatgagtacccagcccttaagtgtctttgctttggtttatgtttgtttgtttccttccactcctggtgcaaaccttacatgtttttgactggggaaacatattttggacctatgcctctacactgacagtgaagagcccaatgggttgtgcactaggtcagggcttcccgcagcgtcagcccctgtggccagcagcgtcacctgggaacctgctagaaatgcacatttttggcagggcgtggtggctcacacctgtaatcccagcacttggaaggccaaggcaggaggatcacctgaggccaagagttcaagatcagcctgggcaatgtaacgagacaccatttctacaaaaactaaattaaaaaaaaaaaaatgagcattttcagccaggtgcagtggctcatgtctgtaatcccagcactatgggaggccaaggcgggtgaatcacttgaggtcaggagttcgagaccagcttggccaacatagtgaaacccctactaaaaataaaaataaatagccaggtgtggtggcgggcgtctgtagtcccagctacttgggaggctgaggcatgagaattgcttgaaccctggaggcagaggttgcagtgagccgagatggcaccactgcactctagccttgagtgacagagcaagactctgtctcaaaaaaaaaaaaaaaaaaaaaaaaaagaaataaaaaaaagaaatgagcatttttgacctgtccaacctactaaatcagaaacttagcaccctatgctttaacaagtcatggctaagggctttaaaaaggtgattttaatgcatgcctaaggtggagaactaaggagaaggcttttgggtaaggtgaatctggagcgggggacccaaggcctaaggaggaggggagtgtgaggcaaaaggagccccttatctacaggttctcaagctcctcccatcaatcccccaacctggccctgtccctccctcgctcaaccttagtttcttcctggaattctcaggcctcctggttcccaaattctgatttccccactgacctgactccagatctccctaccccactgggtcttgtccccagcgtcactccaacccctcaccagcagtccccaggccatgccaacccccacacttttttttttttttgagacagagtctcactcttgtcacccaggctagagtgcagtgccgcaatgtctgctcactgcaacctccacctcctgggttcaagcaattatcctgcctcagcctcccaactagctgggattacaggcgtatgccaccgcgcccagctcatttttgtattttcagtagagaggagtttcaccatgttggccaggctggtcttgaactcctgacctcaggtgatccacccgcctccgtctcccaaagtgctgggattacaggcatgagccaccaagccagtcctaccccacgcttgtcagtattctgggagatcccccagttcccagccccctgggccctggcaacccgctccccacccttctcccgtcagacccgaccaaggagacctaagcttcaacccaggcccccgcgcccctccactacccgtccggcggctcaggcctcggcgccttcgggacccacgagcagcagcggctgggcattcttgcccttgtcgtgccagcacacgtcgaagaaggggtacacgggcctgggcaggcgctcgtggaaggcaaaaagcggcacgagcgcgtcggcgtcgctggcatcgtagaaggagaggacgccgtcgccgaagctcaggtaaaggccaatgcgcgtgggccgcctctcggggctgcgcagagcgcgcggctccttggcctccacgtgtgcctccaggatcttgccctcgcgcagccccagcagccacaggccctgcgagggcaccgcgtgcaggcgcccgcggcggggggcctcggccgcgatcacgcccagcgcccagcgcggcttgtcgccaacatccacctcccagtagtgctcgccctcggagagctgctggtgcgccaccaccgccaccgccttgtcgaactggcgcgggtcctccccggccggcggcgccttctgctccgagcactccacgcggcggccagaggaagacaccaccaggctcgggtgcgcagagctcgggtcaaaggtcagctcctccagcgctggcatcagagcccggaacatcttcctccacacctggaatttgaagtcatctgagataattggcagctggatgtccagacgggcgggtgggggagactctgccaggatcttctgcagcctgctggtcaccaggcagtatttcatgaggaactcagtctgcggcttgtccgccacctcctccaggaccttctccatctgccgcagctgctccaggtaagagttcaggctccccagctcccggcgcaaggcgacccctgcctcaccccgtacacgctctgcctcgcggtccaaggagccctccagtgcagccaggaacacccgcatcttgcccagctgctcccccacggccccccggaactgacgcactgtctcctccacctccaccagctgatgctccagcacagccacactcttctccttgcgcatgcatgcctcctgcagctgcagtttctgctgtggcagctgtgtcttgaggcgtgcgtgggcctcggcggcaggcaggaggcgatgaccgcggtgcgagccgagtgaggcgcacactccgcacaccagcgcgcggtcctgctcgcagtagatgctcagcgggtccaggtgctcctcgcagtggccctgcggcacctgggccagcccctccaccaggcgcgccagctgcaggttggtgctgagtgcctgcggccgcgtgggggcctggcagcaggggcagagaacggtgccatccgccgccggctccccggccacgcggcctaggcaggcgcggcagaaactgtggccgcactcggctgtcacgggcgcgtcgaacagctgcaggcacagcgggcaggacagctcctggtgcaggaggccgggcgcagccgacatggcgggcaggtctggttggagatcttaggctgaaagagtctcgaaggaggaccggtcagggttgagcttagctggactggggtcagggctgggtccaaggatctgagacaagcagcaggctccaagcaaggacagggactcacaggggcagctggcagtggacaccacgcgtgatgggcacacagt

SEQ ID NO: 12271 - RNA, 955 nt, Homo sapiens
  source 1..955: mol_type = other RNA
ctgggaggtcaaggctgcagtgagccacgatcatgccactgcactctagcctgagcaacagagtgagatcctgtctcaaaagacaataaaatttactttagtgagagtttgctgatggcaaattctctcagtttttatcagtgaaaggttctcatcttttcattgttattgaacaggggtttagctggtatcgtagtcagggttcttcagagaaacaggaccaattggatgtgggtggatatatgggtagatagatagacatagattgattgatacagatagatagatctgtatcggtagacagagaaatatagctctatcatctatctatctatcatctatctatatggagattaattttaaggagttgattcatgaaattatggaggctggcaagtcccacgattttccgtatgggaatcagggaataagaatccgagtagaggaggggcagggagtgctaatagcaggacaacagcaactgcagagagaagacggtcaggccggtgagggaagggaggagaacgggtgtcccggacaggttcttcttgcagtcctactcgatcccagaggaggcaggacgaggccttgagctccctggccagtgtcccgggcctgggcaggagggtgatgctggtgacgtgtaggagtgaatccgtgagtgagtcgtggcggtggggcgccagcaccagttccccgaaagtgagagcccgggaacagccagagatcagaagaggcgtgggactgcagccttgaaaggcgctaatgagaggagcctgccactgtagagggtatagcttggtggaagagcctctgcctacacgccaagaggttcctgcttcaagtccaggtgtctcctatggtttacgtttttatccagcaagagtattttgttttcttcctctcccacccctcaaaagccagcctgtaaggctgtaatgtcttatttgtctgt

SEQ ID NO: 12272 - RNA, 386 nt, Homo sapiens
  source 1..386: mol_type = other RNA
ctgggaggtcaaggctgcagtgagccatatcacaccactgcactccagcctgggcaacagagcaaaaccctgtgggaccgcgttgtcagtctcggcgcctgcgctccgctccaggaagaaagcgccaaggcgaggcatggcggtctccgtgcgcaccggcagcttctcgtgggacatcaggatgtcgtccaaagaaagaaagttctcctcaggccccagcgcacccgactccactcggaaataagcctctgacatggcggccacttgagcttctccgcttccactcgcgtgattcggaggagcctcaggagttaggggtgtacaagacggggaagcggagactgggcaggatggttggggtcaggaaagtggattgaaactcgttt
